European Patent Application EP 4 520 821 A1 - sequence listing, part 6

SEQ ID NO: 12273 - RNA, 6104 nt, Homo sapiens
  source 1..6104: mol_type = other RNA
ctgggaggtcaaggctgcagtgagccatgaccacgccactacactccagcctgggcaacacagtgagacctcgtttgaaaaataaaagaataggcctggcatggtggctcatgcctgcaataccagcgctttgggaggccaacgcgggtggatcacctgaggtcaagagttcaagaccagcctggccaacatggtgaaaccccacctctactaaaaatacaaaaaaaattagccgggcatggtggcgggcccctgtaatcccagcttctggggaggctgagacaggagaatcgcttgaacccaggaggcggagattgcagtgagcccagattaaaaaaagaataaactatggatacacgaaacaacacaggtgaatgcaagggaatcatgctccaaagattatccgctctgattccatttacctggcattctcaaaataacaaaattacagacgggtagggggaaaatggcttagtggttgcaggtgttgaggggagagatgaagttatggaagagcagctggaaggatcctgtgcagatgggctgtttgttgactatggttgagattacacaaatctgtcctccgcctccccttcaggctcagggtctgagtcctccacctcaaggccggctccattcagcttcacgtcctgcgagggcgcagcagctgggaggcgcgggctccaggggcgcggcctggcggcaggcggcctcccgcaggcggcaggcgctggcgtagaccaccccgtcggagccgcacaccgggttcccctgggcgccgcagtcgtggtcgcagccgcatcgcgcgatcgccgccccctcctcaggggccacggcagggcccgactcgccggggaaccagcccgggccccgggcaggggcgcgctccacttcgttgcacgcgggtccggcgcacagttcccgggcgagtgggctgtgggtgctgacgttgtagaagcgagtggcctcgaaggcgggttcgtagtagtcgtacacggagactggcagcgccgacgtcctgcccaccacgcactcccggagagcacggaaccgcacgcacgtcaggcaccggctggggatctcatcaaagtagaagagcactcggcgtccagccacttcatacctcttcatccccatgtgcttgtcaaggagcagctgctccaggctctcgatgtctgcccggaagcctgacagcaggggcacctccaggacagccatattggaagaccctgcatgcagccacctggtgcacacctccagcatcaccttgtattcctggtgatgctgatcggccgctgggtcatcatcgtcagctgggggccagtctcctcgggaaccctcagctgcggaggcaggcatggggggcgggcgtccctgggcctcaggctcctggaggcttacgagcagctggaaagctggcttggccaccgggtcaggcacattgtaggtgacatcaatctgcatcaggcagcagccgtcccccttggcactcacaaacagccccgtggggaggctggggatcgctgctgtctgcagaaccttctggttggtcctgtgcagctcgaaggtttcctggtagtccaggttggtggaggccagggagacagtgaggttgatgcctccagcataggacaagatggcatattcagccaaggcctgcagagccacgcaggtgtcctgagtggaggagaagcccccaagtgcatttcgctgctgggacagccacttcaccacaggcagggcggcagccacgtcacccagcagagtgtaggtcagaagggcgtaggctgtcatttccacctcggccgagaccactgactgagagaccctgtcactgaagctcaagaatgtgcccttgtccacgtcccaggaatttgacaggctccagtgggtgaccccatctcgcatgatggccaggctacggagcttgcgcagtgcctcaggggctgccgggctgcggagcagggtcagcgcgtaggtagtcagggcacagctataagggtccatggccaggggcgcagcagactccaggaagtgcctcgctttgtcagtggagcctctctcctcctctgaggctgtgcctgtttccaggagagcaaccaccacgtaggctgtcagcgggacagtgccgtggatcccaccctggatgtccttgttcaggaccctgcccacggccaggaaggagccatcggcctgctgctgctggatgatccagctcttggcggcagccagctcccgggggtccacgaagataaagctgcgagcctgtgcgaaggacttcaggacaaaggctgtgagccacatgctccccgatgcgtcccgctccccaaacgcgctgtaggagccatcctggcgcttgtaggtcagctggcgctggtagccttgtactaggtagtcggtggtctctctctccacctcagggctgagctgctgggttttctgaagatacttcaagacaaagacgttgggtgcaaagtggatcatgttctgctctccacagccaaacggcagccgcaggaggttgttgaggtggttcagggttggccccatgacgtccccgatgatggaggcggtggctcgctcagacccagggatggcgccgtgtgggacccccagggtgaaggcctcgctgtagctctcgtccacctccatcttcctccagattcggaattcacccatggagccccagccggtggaaaagccaatgaactggacctctggtggcctcgggagggtccaggccacaatgacagactcattggatggctctggaccatggccaacctggataaggccaccacgccagctgatccagaatgttctgaattcatcccaggagaggatcttggccgtgtgtgcactggccacgggctctcccatcttgctggtggagatccatgacctggtgttctgatgcccccccaggacgatctcgatcatgcctgctgtgtcctggggcccagaagacaaggccacacgggcatcattgtgagctcgcacagccacatcaaagcgggtgaggcgcagtggccgctgcacatactggaactcatacttgttgggggtggagatgtggactctctcactgggacagaagaatgcgctgtaggtgtacgcccgggggactccttccgcctcaaccatcacactgcgcctgacgtgatccaccccgatggggaccctcctgtcggcgtgattctcctcagggtgtttgctggacctcccatcccggcagcaatttgtgtctccgtaagcaagggctttggccgtgatgttgttgagtcccaggtcgctgaaggacagaacgacccagatgggctcagcctccccgggggccacacacatcttcttggtcacatggcgtttgccaggatgcccaacaaactggatgcccttgggaaccgagagcttcatgtacacctcagcgcaggtgcccatgtagttgtagacactgagcgggatcttgacctgctccccacggatgatgagagcggggagcatgaagtccacgaagaagggcttgaaggtcttcagcagggagggctcggcgatgcctaagccctgagaggtggacagggccacggcctcacccacccagctggtgatggagtccgggaccttcacactgagtgtcccctcaccagatgggtcactgatgttgagacaatgccaaatccatgtttcggggaagaaagtcctttttctcttctctgttctgggggggtgcctggaaggagccactgccaccaggctccctgtgtggggctggaaagcggggacagcctcatcggtgtagaggccaccgtcctgccggtggttcaggctcactcggtcggtcatcaccaccagtcccgtttcggtgaaggcaaacccagagtccttggtgatgccccaaggccacgggaagacagaggagcgccggcgtcgttgtgccgtcagcccagcccaccaaaaaggaccatcctccctggacacgccaaaggaatcagaaacatcataatcttccagttcctggaaaacctgggcaggagtcagccggaacccagacctgagcaggtagacactcttatcaactgcggcgacgcacacacagctgccccttgcagccctgatccgcaggtcgacaacctccccaggttgggtctcatttgctgaatacgtcactgaaacctggttttcgaagaaggtctcgactgcaaactgaaggctgtcggcgaccccttctccattctccctgacgtagaagaccagcaggcgaccaagggggaccatgctgggggtcacggccagatgaagagaggtcacacacacgtcgacctcagcttctggggctggtgggggctctgtctcagaaaggtgtgttaaacgaatcggtttctccagggcaggggccgcccgcttgcttcgctgctgggtggtgtgggcaggctgctggcccgatagcacaatattgccccgtgcagccacctcgtagtacagggtaaagttgcagggacatgtggacttcacagaaaaataggcttcttccccaacctgcagtgggtgggagggtggctgcagctgcaggtagcactggctgggggagtaccagctgccgagggagaggtagctgggcaggtactgagcccccacaggcttcccgttcagtgccatcaccttggtctccagccacacgtgctgggctgacgtggggatggaggggatttcaaaccccactagtccacgctgggacacaacttcactggtgtagatgttatcctttggtgtcagctctgccttaatctggaccgtcaccccctcagctgggctgccatcggggtaggatagctccaccttccccacgtaggccaggcccggcttgaactgcttcctcgtgtccttggagtaccggatgtccaccagctgcctctgcacgggggtggagtcatcgaacgcgacctgctggctcccgtccacactggtcaccatggcccagatgctgaccctgccccggaagtgctcagggacgtccgctgggatcatgtccctcacgcagatgtcgaagtcccgggagccgaggatcttggttgttctgaggacagggcgtcccacctcgtggctgtagtaccctacaccattaacagtcatgttgatcattaaggcaccagccacaggtttcccaaaggtatacctggcccgcacagtgcctgtctcacaggcgtccaggtcttggatataccggggcgggtcaatcagaagctcaaacttgggcaacacatacttctgaacttcaaaagacttgttgtacgcgtggccttgcatttcaacaaaaatgaaccattctcccaacacaggctggtcggacaaggggaagctcatgttggtgatgccgcagcagaacggctttaagtgtctccactctatcatccgagagcctcgggggtccaggatgtaggcttccagcttctcgttgacaggcctcagatttggagagacggtgaagatgcttatgagcactcggtgctggggtctgtacacaggcttgtccgtctggatgaatacagaagcgccccggccgtccacggtcaccgaggtctggttgtgaaagaggggcccctcctccgcctgccagccgcggccccacactttcagaagcgcttggccccggaggcccgtgggcaccttgagtttgattgtccctttatccaggatggctccctggctctgcaccaccggctcaccctgggccaccagctgagcctggaccgtgacttcccttggagagttaaagatggtcacgctgatgacttcctccacgcccgcgcgaaaaacagagggagctgcaatcaagtaacccggggcctgaggctgcgcggcgcgcacgccgtcccgcgccgacagcagcaggagcaggagcgggagcaacggccagagcagggcgccgctcatttttcggctcctggggggcgccgcgcctggggagggggccgggccagggctgggccagggccagggtccgagcgcggccgtcctcgcgccgccgccgggggccctttgttcgcagcccccgcgcagtgcgcccggcgccatgcgccccgctccgcgcccggccaagctggggcagc

SEQ ID NO: 12274 - RNA, 6178 nt, Homo sapiens
  source 1..6178: mol_type = other RNA
ctgggaggtcaaggctgcagtgagccatgaccacgccactacactccagcctgggcaacacagtgagacctcgtttgaaaaataaaagaataggcctggcatggtggctcatgcctgcaataccagcgctttgggaggccaacgcgggtggatcacctgaggtcaagagttcaagaccagcctggccaacatggtgaaaccccacctctactaaaaatacaaaaaaaattagccgggcatggtggcgggcccctgtaatcccagcttctggggaggctgagacaggagaatcgcttgaacccaggaggcggagattgcagtgagcccagattaaaaaaagaataaactatggatacacgaaacaacacaggtgaatgcaagggaatcatgctccaaagattatccgctctgattccatttacctggcattctcaaaataacaaaattacagacgggtagggggaaaatggcttagtggttgcaggtgttgaggggagagatgaagttatggaagagcagctggaaggatcctgtgcagatgggctgtttgttgactatggttgagattacacaaatctgtcctccgcctccccttcaggctcagggtctgagtcctccacctcaaggccggctccattcagcttcacgtcctgctgtaaaggccccggggccacagaagccaggtcatccccgtaggtggaggacgacgaggccggcagccgctgctcgagggcgcagcagctgggaggcgcgggctccaggggcgcggcctggcggcaggcggcctcccgcaggcggcaggcgctggcgtagaccaccccgtcggagccgcacaccgggttcccctgggcgccgcagtcgtggtcgcagccgcatcgcgcgatcgccgccccctcctcaggggccacggcagggcccgactcgccggggaaccagcccgggccccgggcaggggcgcgctccacttcgttgcacgcgggtccggcgcacagttcccgggcgagtgggctgtgggtgctgacgttgtagaagcgagtggcctcgaaggcgggttcgtagtagtcgtacacggagactggcagcgccgacgtcctgcccaccacgcactcccggagagcacggaaccgcacgcacgtcaggcaccggctggggatctcatcaaagtagaagagcactcggcgtccagccacttcatacctcttcatccccatgtgcttgtcaaggagcagctgctccaggctctcgatgtctgcccggaagcctgacagcaggggcacctccaggacagccatattggaagaccctgcatgcagccacctggtgcacacctccagcatcaccttgtattcctggtgatgctgatcggccgctgggtcatcatcgtcagctgggggccagtctcctcgggaaccctcagctgcggaggcaggcatggggggcgggcgtccctgggcctcaggctcctggaggcttacgagcagctggaaagctggcttggccaccgggtcaggcacattgtaggtgacatcaatctgcatcaggcagcagccgtcccccttggcactcacaaacagccccgtggggaggctggggatcgctgctgtctgcagaaccttctggttggtcctgtgcagctcgaaggtttcctggtagtccaggttggtggaggccagggagacagtgaggttgatgcctccagcataggacaagatggcatattcagccaaggcctgcagagccacgcaggtgtcctgagtggaggagaagcccccaagtgcatttcgctgctgggacagccacttcaccacaggcagggcggcagccacgtcacccagcagagtgtaggtcagaagggcgtaggctgtcatttccacctcggccgagaccactgactgagagaccctgtcactgaagctcaagaatgtgcccttgtccacgtcccaggaatttgacaggctccagtgggtgaccccatctcgcatgatggccaggctacggagcttgcgcagtgcctcaggggctgccgggctgcggagcagggtcagcgcgtaggtagtcagggcacagctataagggtccatggccaggggcgcagcagactccaggaagtgcctcgctttgtcagtggagcctctctcctcctctgaggctgtgcctgtttccaggagagcaaccaccacgtaggctgtcagcgggacagtgccgtggatcccaccctggatgtccttgttcaggaccctgcccacggccaggaaggagccatcggcctgctgctgctggatgatccagctcttggcggcagccagctcccgggggtccacgaagataaagctgcgagcctgtgcgaaggacttcaggacaaaggctgtgagccacatgctccccgatgcgtcccgctccccaaacgcgctgtaggagccatcctggcgcttgtaggtcagctggcgctggtagccttgtactaggtagtcggtggtctctctctccacctcagggctgagctgctgggttttctgaagatacttcaagacaaagacgttgggtgcaaagtggatcatgttctgctctccacagccaaacggcagccgcaggaggttgttgaggtggttcagggttggccccatgacgtccccgatgatggaggcggtggctcgctcagacccagggatggcgccgtgtgggacccccagggtgaaggcctcgctgtagctctcgtccacctccatcttcctccagattcggaattcacccatggagccccagccggtggaaaagccaatgaactggacctctggtggcctcgggagggtccaggccacaatgacagactcattggatggctctggaccatggccaacctggataaggccaccacgccagctgatccagaatgttctgaattcatcccaggagaggatcttggccgtgtgtgcactggccacgggctctcccatcttgctggtggagatccatgacctggtgttctgatgcccccccaggacgatctcgatcatgcctgctgtgtcctggggcccagaagacaaggccacacgggcatcattgtgagctcgcacagccacatcaaagcgggtgaggcgcagtggccgctgcacatactggaactcatacttgttgggggtggagatgtggactctctcactgggacagaagaatgcgctgtaggtgtacgcccgggggactccttccgcctcaaccatcacactgcgcctgacgtgatccaccccgatggggaccctcctgtcggcgtgattctcctcagggtgtttgctggacctcccatcccggcagcaatttgtgtctccgtaagcaagggctttggccgtgatgttgttgagtcccaggtcgctgaaggacagaacgacccagatgggctcagcctccccgggggccacacacatcttcttggtcacatggcgtttgccaggatgcccaacaaactggatgcccttgggaaccgagagcttcatgtacacctcagcgcaggtgcccatgtagttgtagacactgagcgggatcttgacctgctccccacggatgatgagagcggggagcatgaagtccacgaagaagggcttgaaggtcttcagcagggagggctcggcgatgcctaagccctgagaggtggacagggccacggcctcacccacccagctggtgatggagtccgggaccttcacactgagtgtcccctcaccagatgggtcactgatgttgagacaatgccaaatccatgtttcggggaagaaagtcctttttctcttctctgttctgggggggtgcctggaaggagccactgccaccaggctccctgtgtggggctggaaagcggggacagcctcatcggtgtagaggccaccgtcctgccggtggttcaggctcactcggtcggtcatcaccaccagtcccgtttcggtgaaggcaaacccagagtccttggtgatgccccaaggccacgggaagacagaggagcgccggcgtcgttgtgccgtcagcccagcccaccaaaaaggaccatcctccctggacacgccaaaggaatcagaaacatcataatcttccagttcctggaaaacctgggcaggagtcagccggaacccagacctgagcaggtagacactcttatcaactgcggcgacgcacacacagctgccccttgcagccctgatccgcaggtcgacaacctccccaggttgggtctcatttgctgaatacgtcactgaaacctggttttcgaagaaggtctcgactgcaaactgaaggctgtcggcgaccccttctccattctccctgacgtagaagaccagcaggcgaccaagggggaccatgctgggggtcacggccagatgaagagaggtcacacacacgtcgacctcagcttctggggctggtgggggctctgtctcagaaaggtgtgttaaacgaatcggtttctccagggcaggggccgcccgcttgcttcgctgctgggtggtgtgggcaggctgctggcccgatagcacaatattgccccgtgcagccacctcgtagtacagggtaaagttgcagggacatgtggacttcacagaaaaataggcttcttccccaacctgcagtgggtgggagggtggctgcagctgcaggtagcactggctgggggagtaccagctgccgagggagaggtagctgggcaggtactgagcccccacaggcttcccgttcagtgccatcaccttggtctccagccacacgtgctgggctgacgtggggatggaggggatttcaaaccccactagtccacgctgggacacaacttcactggtgtagatgttatcctttggtgtcagctctgccttaatctggaccgtcaccccctcagctgggctgccatcggggtaggatagctccaccttccccacgtaggccaggcccggcttgaactgcttcctcgtgtccttggagtaccggatgtccaccagctgcctctgcacgggggtggagtcatcgaacgcgacctgctggctcccgtccacactggtcaccatggcccagatgctgaccctgccccggaagtgctcagggacgtccgctgggatcatgtccctcacgcagatgtcgaagtcccgggagccgaggatcttggttgttctgaggacagggcgtcccacctcgtggctgtagtaccctacaccattaacagtcatgttgatcattaaggcaccagccacaggtttcccaaaggtatacctggcccgcacagtgcctgtctcacaggcgtccaggtcttggatataccggggcgggtcaatcagaagctcaaacttgggcaacacatacttctgaacttcaaaagacttgttgtacgcgtggccttgcatttcaacaaaaatgaaccattctcccaacacaggctggtcggacaaggggaagctcatgttggtgatgccgcagcagaacggctttaagtgtctccactctatcatccgagagcctcgggggtccaggatgtaggcttccagcttctcgttgacaggcctcagatttggagagacggtgaagatgcttatgagcactcggtgctggggtctgtacacaggcttgtccgtctggatgaatacagaagcgccccggccgtccacggtcaccgaggtctggttgtgaaagaggggcccctcctccgcctgccagccgcggccccacactttcagaagcgcttggccccggaggcccgtgggcaccttgagtttgattgtccctttatccaggatggctccctggctctgcaccaccggctcaccctgggccaccagctgagcctggaccgtgacttcccttggagagttaaagatggtcacgctgatgacttcctccacgcccgcgcgaaaaacagagggagctgcaatcaagtaacccggggcctgaggctgcgcggcgcgcacgccgtcccgcgccgacagcagcaggagcaggagcgggagcaacggccagagcagggcgccgctcatttttcggctcctggggggcgccgcgcctggggagggggccgggccagggctgggccagggccagggtccgagcgcggccgtcctcgcgccgccgccgggggccctttgttcgcagcccccgcgcagtgcgcccggcgccatgcgccccgctccgcgcccggccaagctggggcagc

SEQ ID NO: 12275 - RNA, 1478 nt, Homo sapiens
  source 1..1478: mol_type = other RNA
ctgggaggtcaaggctgcagtgagccatgatcacactcctgcctgcgtgacagactgagaccctgtctcacaaaacaaaaactcaaaagtaaacaatgggaaataaatgcatgaaaaatgtttgcaataccagctgcagagaaacaaggtagtgccacacacctgagctccagtgagttccggcacggggagtgagttccaaggactcagcagcataaagcatcggttgaacatccaaatggccaggctgtgatttcagcgtccagttacgagtgcactataaaaagcaccgttctagtaccaaaaatgtgactggtgagaatataggacaacttcttgcagagccaggcttaaggcaggaatcaacttcatggtctaccagccagacccttgggaggcagccttggactcgatgagacaactatgaagtgccaagacaggaggtgctgtggctccacaggaacctcggagaatctgtgtatcaagcagaagtgctcgttgttttgagtccgctacgtcagccatcaacaaaacatcagtttaaaatggattgctctaacttcaggatgtttcgtgtaatccccatggtaatgacaacatatcgcgctccctcctgtttcagggcctttgctcgtgccgctccctcgtcccgtgcatcaggagtgctgtctaccagccggggtcggggtcgaggcagacaaatgaagtcgggtcggcttttgtccagctgacgccccacggcgcctgcactctcgagaggccaccacgcgccgcgccagtgacgtcattgcgccgctctccccaccaaccgctgccccaggcccactcggcgtggctcggccacgctcggcttgacttggctcggctcggccacactcggcttccctcggcttcctctcggcctctcggcagcactgcgggctccgcagcccttctggccttcacgtggttcccagttctcgtggtacgtcctgcctgccgggatctcagggctcttggaagaccccaggcccggggagggcatgtcccaagggcatgccaggtcaaggccacaatagcgagccctctcccacgccctgtagtcgtcggagaccaacgtgttctcccaccccattccggtccacagcaatccctgcctacccaacctcacatagaccttaggtcttgaacctcttttcctacctggaaatgaggttaagaactacccacctcatgggtgaagttcaatcagaggatgcctgaaaagtgcttaatacgtgatgtgtgcccagtcattggaatcagccctctctgcttgattctttcattgctgctgtttgtttgtttgttgttgttgtttgaaacaccgtctcattgactaggcgcggtggctcacgcctgtaatcccagcactttgggaggccgaggtgggcagatcacttgagaccaggagttcgtcaccagcctggccaacatggtgaaaccccgtctctactaaa

SEQ ID NO: 12276 - RNA, 1993 nt, Homo sapiens
  source 1..1993: mol_type = other RNA
ctgggaggtcaaggctgcagtgagccatgatcactccactgcactccagcctgggcaagagagtgagaccctatctcaaaaaatgaataaattacataaataaaaagtaataagaaaaaagtatatatgtaaattatacatccataaaggtgattaaaagaaaacgtgtgggtggatttttgcccatatatggcacagtccaacccatgaaactctctgaagacaacagcatgggttcttacctcaggacctgcaaatatggcaccaagtatcatactagaatgtgtgagagacactgagctccacagtcacacagatggggacacaaagggacacctgtcagtaaatacacacatttgctctctctctctctctctctggaagtgcaagagagtgttttgatcagaggcagcagatgtgaactgaaatagtgcctctctatgttagggacacattgccctaaagctgaatccaagtttttaaaaatatacctaattatgtgtcatcccatggctcatgtgtctaaccaaagttgctactgtcttggttacctattattgcatggtgccccaatcctagtggcttagtaccacaacttattattatctctcacagttctatgagttgactgggctcagctggtggattttcattcctggtttctcatgtggttgcagtcaggtgtcagctggggctggagtcatctgaaggtttaaccaagctggatgtccaagatagctcactcacaagactggtagttgatgttggctgccggctgggaacttaactgtggctgttgactacgatgccttatatgtggtgtctgcatgtagattgggcttcttacagcatggtggctgggttccaagaaggagtatcccaagagcaagtgttcttcacaggccaggtggaagttgcaaggctttctgtgacctcacctttcaggtcacacagtctgtcttccacatcattctatcagtcaaaacagtcacagaactcactcagattcaaaggaggggagaaattgtctcctctacttgatggagaagtggcagattatacagcagaaaagtgtgtgggatattgttgcagccaccttttgaaaatgcaatcagtcccagctctataatgaaacctctttttcccttagtcttcaatgtagaatttttcattgggctccaacaaccagtgccaaagacacaggccagccacagtcctctcatctactgaaattttgaggtcaatttcttcaagtccctaagaaaatcctctctgaatagcggtgtatccttctgctttctggcacattttgcaactccagacatcacggaagcagccaacaggcaccatcagaatccttaggctcaatccatcagatgcccccatcaaaggcttggagttgggaactaataatacagagatgcaaggagcacagaagtccattctggtggatggtggcagtcgccaagtcaatggcattccagttcctggggcgacagggaccatatccacgtcccaaggtggcagtgtatgccagggagtcctggatttggcagcgaggtcatccctggattgcctgactttggctgtggtcctgactgctgtgcagcctccttggtcgactcaccaactgtattcttcagccctcttggttattttgtgagttccccaagatccttttgataaagtccttttctgcttaaataagccagaattgtttcctgttgcttgggagccaagagctccggctgttacagctgagccgctagattttgcctggcttccctcagcgagaccacacaggacactgctaattcttggatccctcaggcatcccagtccacttcctgggagctcccatatcccaggaccttggcctgctgatcttacattaagagaactggcctggtctgacagagggtcccacatccatcctggacagcttcatggtgatgttcctgggtcccatctcagactctccccatcaaaggct

SEQ ID NO: 12277 - RNA, 3369 nt, Homo sapiens
  source 1..3369: mol_type = other RNA
ctgggaggtcaaggctgcagtgagccatgatcatgccactgcactccagcctaggtgacagagcaagaactcatctctaaaaaaaaatttttaaataaagcaaaatatgccacagcatagatctgattgtagaaaattattatatggagaactgaaaaatctcctaatcaagacaaaaattttaaatagaggaaaaaaatactatctatcattagttcaagtttccattaagagtagagtgtgaagtagctccaagttcagagctggagaattttgcatctctccctcttaccagccaattgactttaggtaaagaatactagagttttttagttagtaaaatatagttaataattctgtataaaggagcaaaagtaagtttctcattgtttcctatctcccttcataggtttgacatgttgaaattgtgaaattatttaatgttaatagtttttaacttctttaattatgtaaaataattaatttttaaattattttaacagttaaaacacaaagcatacttttcatggaaccaagtgttccaaacacaaaaaggtcattctctgatggctcctgataacatacaacataaaatatagttataacaaatataatttagaatttatatttcagaatccatcctggtgtaaagctatttactataaccttactaaaaataccaacggtaaggatgttggatcttttaaaggtaaaacatcagagaaaagagaaaaagacctgtttgtccaattctctgtgctttccatgctctagcaccatcccaaagttgcctcctaacttctgttccctccctgggaagggaagtccaggcaaatctgtgatcagttaataacttttaacaattgtttgccattacatctgaaagtgaacagttaatcacttattgttatatctcaaaggtaaatttcactatctaaatgcctagaggtaactggaagatgaaagatacataaaggtttgatgaatagaggggaaaaaatgggggggagggttgtttctgtttttccaatgaaaaggtttgctccttctctctgcaaaatcttggaactgagaaagccgtctggagtgcagatggaaagcatgcatcaaattgatgtaactacacaacatactcctgccctacaccaggttcattctgccacctctatcccactctacgaatgtcccatttgccacagcctaacttctatcatagttctaattcctcagtgaagatcacaagaaaggtacttccaggttgttaaaagaaacgagaatgttacaccaacacatttctggggtggaaggagactactgacactccatatttattgcttacattacaagaattaaacaaaaaaagcagactagaaaatcactttctgtaatttcacaatcaccaatttgcaacagaaactgaagcataatatttatgctaacaaatatgttggatgaattatcacctcagcacataactgcagatggatactcctggattttcacttaatccattactcaatgatgaacactataaaatgaaaggtgacatacttatgaactaaaatcacaagaagaaactctccaagatcaatcttaaatgagctcctattccaataagccataaagagcagtaaaaggcaatattcatttaacagtacaagaatctcgatgacaagaaatcaggtatttatattcctctagagacatttcttctccacctaacaaaggcacttgacatgtactgaaatggacagttaattcaggtactgccctgggcaactgttaccttgctaaaattagatgaagtggtgattaagttcaaattagttctcccaaataagcctgaaacacacatgaatagatcataagttctctatttttggcagatgatataaccaagaagaaaagctaatgttggtatccatgctgaactggctgacttaagcagtcaaggatactctctctgcacaatatattccttgatgactatggaatgtatatataattataggcaaattaacctttcctatagtttcaggtattaatgttcattcctcttcttgtcttttcttacttttttgttctttcccaaagccttagatgactcctcaggtgaatttgtgtagttcttttccactagtatgtttctggcacagttgttgatatgtttaaagcgatctggtcctagcagaatccctccataccagcgtgatactaccaccatgacattcttcacattcaaaatctccatgagatgaagaagacgcccaccagctgctgtttccccatcatcctcacaatcctgtaagaaggtctgtttatcctcacaatatattctgtaggcatagatgttgtgggtggcactagctattttcttattctcatacaatttggaaagaaccattttcacctgtttgggacaaaccactggagccaagtgtgcctgaaaagtacttcttcggtctgtaataggaatgccatgatcaatcggaggtaattcttctacttctacttctgtccgagtttcactgatatcaaaatccaatgctttaagcgaactttccggctgacatgctaaaatgagatcatcttcacattcaacatcttcctcttcagttttcttctttacatctgggcctggttctgtcatctgagatttttgtataagaacatctcttattttctccacccacaggtaaagaatactttcaccgatattctgaatatatatttcctcaaggctatttgataaatccgcacgttcttgccctttaagccaaggagcattcaactggtagataggtggagctgtacctgggtattcattcggcagcatcacctgcaagcaaagtgtccatttggggtcatctatatcgtcgctaattctaatacaaaatattttggcacagtcatcaatgacacaccactcctcgccataaatggctgccattgcttcaatttcctcattagccctgtaggaaaagacttatgatcgcccacgtgaacaaggcacagggaaagctcgatgccaaggaccagaaggagtgagattcggtgggctctcgggacctgcagggtctgggctattgccattttgcaaagggggaaacccgaattcttaagtgatttgtccaagatgactcggcggcggcagggtggggatcgaaaccccggtttttgccttcggcccagagctgcttagtcgcgtgttaatggttgacgaggacaccgtccgagacaggccgagaccgcggccgccgaggagccgccggcctaagagcgctcggccgacgggaagcgccgggaaaatggaacgcggtggagcaaatggcgtggccagtgctggcggaacccggggcggccccaggc

SEQ ID NO: 12278 - RNA, 3091 nt, Homo sapiens
  source 1..3091: mol_type = other RNA
ctgggaggtcaaggctgcagtgagccatgatcatgccactgcactccagcctaggtgacagagcaagaactcatctctaaaaaaaaatttttaaataaagcaaaatatgccacagcatagatctgattgtagaaaattattatatggagaactgaaaaatctcctaatcaagacaaaaattttaaatagaggaaaaaaatactatctatcattagttcaagtttccattaagagtagagtgtgaagtagctccaagttcagagctggagaattttgcatctctccctcttaccagccaattgactttaggtaaagaatactagagttttttagttagtaaaatatagttaataattctgtataaaggagcaaaagtaagtttctcattgtttcctatctcccttcataggtttgacatgttgaaattgtgaaattatttaatgttaatagtttttaacttctttaattatgtaaaataattaatttttaaattattttaacagttaaaacacaaagcatacttttcatggaaccaagtgttccaaacacaaaaaggtcattctctgatggctcctgataacatacaacataaaatatagttataacaaatataatttagaatttatatttcagaatccatcctggtgtaaagctatttactataaccttactaaaaataccaacggtaaggatgttggatcttttaaaggtaaaacatcagagaaaagagaaaaagacctgtttgtccaattctctgtgctttccatgctctagcaccatcccaaagttgcctcctaacttctgttccctccctgggaagggaagtccaggcaaatctgtgatcagttaataacttttaacaattgtttgccattacatctgaaagtgaacagttaatcacttattgttatatctcaaaggtaaatttcactatctaaatgcctagaggtaactggaagatgaaagatacataaaggtttgatgaatagaggggaaaaaatgggggggagggttgtttctgtttttccaatgaaaaggtttgctccttctctctgcaaaatcttggaactgagaaagccgtctggagtgcagatggaaagcatgcatcaaattgatgtaactacacaacatactcctgccctacaccaggttcattctgccacctctatcccactctacgaatgtcccatttgccacagcctaacttctatcatagttctaattcctcagtgaagatcacaagaaaggtacttccaggttgttaaaagaaacgagaatgttacaccaacacatttctggggtggaaggagactactgacactccatatttattgcttacattacaagaattaaacaaaaaaagcagactagaaaatcactttctgtaatttcacaatcaccaatttgcaacagaaactgaagcataatatttatgctaacaaatatgttggatgaattatcacctcagcacataactgcagatggatactcctggattttcacttaatccattactcaatgatgaacactataaaatgaaaggtgacatacttatgaactaaaatcacaagaagaaactctccaagatcaatcttaaatgagctcctattccaataagccataaagagcagtaaaaggcaatattcatttaacagtacaagaatctcgatgacaagaaatcaggtatttatattcctctagagacatttcttctccacctaacaaaggcacttgacatgtactgaaatggacagttaattcaggtactgccctgggcaactgttaccttgctaaaattagatgaagtggtgattaagttcaaattagttctcccaaataagcctgaaacacacatgaatagatcataagttctctatttttggcagatgatataaccaagaagaaaagctaatgttggtatccatgctgaactggctgacttaagcagtcaaggatactctctctgcacaatatattccttgatgactatggaatgtatatataattataggcaaattaacctttcctatagtttcaggtattaatgttcattcctcttcttgtcttttcttacttttttgttctttcccaaagccttagatgactcctcaggtgaatttgtgtagttcttttccactagtatgtttctggcacagttgttgatatgtttaaagcgatctggtcctagcagaatccctccataccagcgtgatactaccaccatgacattcttcacattcaaaatctccatgagatgaagaagacgcccaccagctgctgtttccccatcatcctcacaatcctgtaagaaggtctgtttatcctcacaatatattctgtaggcatagatgttgtgggtggcactagctattttcttattctcatacaatttggaaagaaccattttcacctgtttgggacaaaccactggagccaagtgtgcctgaaaagtacttcttcggtctgtaataggaatgccatgatcaatcggaggtaattcttctacttctacttctgtccgagtttcactgatatcaaaatccaatgctttaagcgaactttccggctgacatgctaaaatgagatcatcttcacattcaacatcttcctcttcagttttcttctttacatctgggcctggttctgtcatctgagatttttgtataagaacatctcttattttctccacccacaggtaaagaatactttcaccgatattctgaatatatatttcctcaaggctatttgataaatccgcacgttcttgccctttaagccaaggagcattcaactggtagataggtggagctgtacctgggtattcattcggcagcatcacctgcaagcaaagtgtccatttggggtcatctatatcgtcgctaattctaatacaaaatattttggcacagtcatcaatgacacaccactcctcgccataaatggctgccattgcttcaatttcctcattctgcctctggtcgctccctgcgtccccctcagccatgtggcccctggacctgccctgcagccgccgcctgccaggtccggagcgcgggggcggggcgctgcggctgcgagccgagagctggct

SEQ ID NO: 12279 - RNA, 776 nt, Homo sapiens
  source 1..776: mol_type = other RNA
ctgggaggtcaaggctgcagtgagccatgatcatgccactgcactccagcctggataacacagcgagaccctttttggatcttcccagcttcaatgtaaggggtgagaaataatggctgtcctgagtctcccttaggtggcatggaaacacttctgtatagggagcgaaacagcccatcacaggggccaggcatcaacaggaccagcgaaacaatcaccttccacatggcaccaaccatctctcagggtattgtagtttgaactggggctcctggcagcaacatttatatagaatatactgtgtttggtggctcctagggttgtgcagctggtgcccatgccactgacgtgttcaacttacagcaatcaagctgattacggagtgagtcccagatctgcaggatgacttggcatgtaagagacccaggagagctgatggtatagttcctgtcaagacagcaggctggaaccccaggaagagccaatgtttccgtttggatcatttccagtcaagctcttcaacaatataatctgttctctgaatctcatttctcttatcaaaccttagcagcatatcaaaatcacctgtggccatcccgcccgctctctcggaatgggggcaggcgtccggggtgatacttgtttggttcgccagcacctcggtgcccagagcacctccgcgcctgacatctgacagcgcagaggtgggagagcggtggtgcccttagtgtgcggacgcgggtgttccggggcttggagtgcagcgagcgaaaagc

SEQ ID NO: 12280 - RNA, 58 nt, Homo sapiens
  source 1..58: mol_type = other RNA
ctgggaggtcaaggctgcagtgagccatgatcatgccactgtactccagcctgggtga

SEQ ID NO: 12281 - RNA, 2903 nt, Homo sapiens
  source 1..2903: mol_type = other RNA
ctgggaggtcaaggctgcagtgagccatgatcctgtcactaagttccagcctgggtgatacagcaagaccctgtctctaaaaataacaataataatataaaaagcaagttccagaaaactacatatgataccatttttacagagctcaaaaccaggcaaatctaaacaatatttattgtttaaaggtataatacatacatgacaaagtatataaaaatccaatccaagccaaactaaataaaatattgcttcctcatgggaggaggcaaaggagtggatggggaaaagaacacaggtaaaaagcaagttactcctgatgctccatttcttgggctaagtgatgagtccatggggtttgttaaatcacactccacatccaatatttttgttacatataatcctttgtatgtagcaaatatgtcctgtccctggtatcaggattaagccatccatttgtgacacctaggacaccatttcctttgacttgttaattccctttgaaggtcattgatgtcctcaaccaccttggctagtgggatgaagacaatctgtggaagtatgtcttggcccacccaggcctcagctcagccttctaaaactaatagcccagctggtcagatgttaggaagaggtgggcgaagcccactgataaaactcatctactaaaacctccctctatgacctaaagcctcttgtcgtaggctcgctggtctccacctagccctgttccacttgctgtgactattctggcttcccaaccaccccttccagaacctagattggtcatggaggtcacagaggtccatggtaaccgaaacctcgtgtcagtcccacttctgaggccaggtgcaggcacgtgtgcttcagaccccacttgctcaagctactaacaaaggtcagctccgtggccttgaggagttaagcctgtgtcctcgcctggaggatgctgcaccaacaatctgagacttctctaagatgttgaggacctcagtcactttgatgctcccaatatgatgaaaatctgctaaaagctggttatgttcacgagcacaccccatgaggaggaaggtggtattgagaaaccctgcctgaaattttaaggtggaactgtaacacgtagaagcagccaaggggcaagaattagtggtgacaaaatttgggaggcaatccttcatgtgctcgcccacacaggtcgggcagctacaggacgcagatgtgatagacttaggagtgctggccttgagtttcacaaaaggctccaaattggtgaggttgttgcagagataagaccggcagacgcgactgtaggaggcaatggacactccgggtggggaaacaaggtaggagatttgcgcagggtaagacgaagacgagctgcagcctttaaagcccacgactccccttgcagtccctgtctcaatgaacactagcgtctcctcgcagccctcttgcagcttacacaccatgttcctcatcagaagccacttccagttatggaaagcaacagctctgaatcttgaggctgttgcttcatagcacaaaagagctccagcccctttctgggtcttatagcatccagccccacaggacatacgaggcagagtggagatggcccctagaaggcagaacagctgcacaagtctcaaatgctggggtcccatggccctgtgtctgggtcctgggtgctagaggtcagtctggaatcagtttcagtctggatcccaagctcagttcccatcagtccccgaattctttgtccacctgtctctgggtcactgtttctttccaattttatctaggacagctcccctgcccagcagtccagctagaggtcacgtcggccacccttttctgcctgcaatgcctcagacacacatgctctgtaacccagaaatctgtggccaagaaaggtgccaagacccgcagaaaagctgggacacaggaaagagaaacgaaggctgacaacagatctcacgggggtgagggagattaggccaatcagagaagacagcacacgccagcctcagatgcagaacaactggacctggacctaacaagctgagtacaagtggagacgcaaccagaaaagattgaagtgaaatcctcaagcaaaaaaaaaaaaaaaaaaaaaaaaaaaaaggatggagcagtagtcagaggggatgccacccctacaaaagacaaacaaattgatggaatggaaccttgcagggagagagaggaccagcagagagagggaggcgtaggaaaatgaggagtggggcacaaaggtggggctctcagggagaagaggagtcgattttagagggggagaagaaaaggacacagagctggctgtacagagaaaaggggccaaggcagagaagatggcgggatggtgtgagacggagttcacagaaatacccagagaaggcgacgattacacagaggagcccccagaggggcgaactcttgaggaagatgaacgcggagggtggagccagccagaaattcagaaaaactagaggcgtccccggtagcgaaggaagccgggaaggggccaggctatcagggcatgaagcacgggagaaaatgggtccgaagagggagagcgtccgagagaaaaggaaaatcagagattaggaaaatcacaaccgacacaaagacaagaagagacacaaggaaaggggtgcaatctgaggaaggagggcccggtaagcaacccggtaatcacagcgctgggagagaacgcataaaagaagggtagctcaggagttgtggggcaccggaagagacataacagaaaacgcaggcctccactcagcaaaaacaagccacgcgcgaagtcgaggtacaaggcaagggaaggccagaaacgaggcaacccgtgcacagaccgggcttggtcaacgccccaggggcgg

SEQ ID NO: 12282 - RNA, 1827 nt, Homo sapiens
  source 1..1827: mol_type = other RNA
ctgggaggtcaaggctgcagtgagccatgatcctgtcactaagttccagcctgggtgatacagcaagaccctgtctctaaaaataacaataataatataaaaagcaagttccagaaaactacatatgataccatttttacagagctcaaaaccaggcaaatctaaacaatatttattgtttaaaggtataatacatacatgacaaagtatataaaaatccaatccaagccaaactaaataaaatattgcttcctcatgggaggaggcaaaggagtggatggggaaaagaacacaggtaaaaagcaagttactcctgatgctccatttcttgggctaagtgatgagtccatggggtttgttaaatcacactccacatccaatatttttgttacatataatcctttgtatgtagcaaatatgtcctgtccctggtatcaggattaagccatccatttgtgacacctaggacaccatttcctttgacttgttaattccctttgaaggtcattgatgtcctcaaccaccttggctagtgggatgaagacaatctgtggaagtatgtcttggcccacccaggcctcagctcagccttctaaaactaatagcccagctggtcagatgttaggaagaggtgggcgaagcccactgataaaactcatctactaaaacctccctctatgacctaaagcctcttgtcgtaggctcgctggtctccacctagccctgttccacttgctgtgactattctggcttcccaaccaccccttccagaacctagattggtcatggaggtcacagaggtccatggtaaccgaaacctcgtgtcagtcccacttctgaggccaggtgcaggcacgtgtgcttcagaccccacttgctcaagctactaacaaaggtcagctccgtggccttgaggagttaagcctgtgtcctcgcctggaggatgctgcaccaacaatctgagacttctctaagatgttgaggacctcagtcactttgatgctcccaatatgatgaaaatctgctaaaagctggttatgttcacgagcacaccccatgaggaggaaggtggtattgagaaaccctgcctgaaattttaaggtggaactgtaacacgtagaagcagccaaggggcaagaattagtggtgacaaaatttgggaggcaatccttcatgtgctcgcccacacaggtcgggcagctacaggacgcagatgtgatagacttaggagtgctggccttgagtttcacaaaaggctccaaattggtgaggttgttgcagagataagaccggcagacgcgactgtaggaggcaatggacactccgggtggggaaacaaggtaggagatttgcgcagggtaagacgaagacgagctgcagcctttaaagcccacgactccccttgcagtccctgtctcaatgaacactagcgtctcctcgcagccctcttgcagcttacacaccatgttcctcatcagaagccacttccagttatggaaagcaacagctctgaatcttgaggctgttgcttcatagcacaaaagagctccagcccgaggcagagtggagatggcccctagaaggcagaacagctgcacaagtctcaaatgctggggtcccatggccctgtgtctgggtcctgggtgctagaggtcagtctggaatcagtttcagtctggatcccaagctcagttcccatcagtccccgaattctttgtccacctgtctctgggtcactgtttcgggcttggtcaacgccccaggggcggggccaggcgggccgttcctggggggcggggccagcctcggtccaataaggggtactcg

SEQ ID NO: 12283 - RNA, 1759 nt, Homo sapiens
  source 1..1759: mol_type = other RNA
ctgggaggtcaaggctgcagtgagccatgatcctgtcactaagttccagcctgggtgatacagcaagaccctgtctctaaaaataacaataataatataaaaagcaagttccagaaaactacatatgataccatttttacagagctcaaaaccaggcaaatctaaacaatatttattgtttaaaggtataatacatacatgacaaagtatataaaaatccaatccaagccaaactaaataaaatattgcttcctcatgggaggaggcaaaggagtggatggggaaaagaacacaggtaaaaagcaagttactcctgatgctccatttcttgggctaagtgatgagtccatggggtttgttaaatcacactccacatccaatatttttgttacatataatcctttgtatgtagcaaatatgtcctgtccctggtatcaggattaagccatccatttgtgacacctaggacaccatttcctttgacttgttaattccctttgaaggtcattgatgtcctcaaccaccttggctagtgggatgaagacaatctgtggaagtatgtcttggcccacccaggcctcagctcagccttctaaaactaatagcccagctggtcagatgttaggaagaggtgggcgaagcccactgataaaactcatctactaaaacctccctctatgacctaaagcctcttgtcgtaggctcgctggtctccacctagccctgttccacttgctgtgactattctggcttcccaaccaccccttccagaacctagattggtcatggaggtcacagaggtccatggtaaccgaaacctcgtgtcagtcccacttctgaggccaggtgcaggcacgtgtgcttcagaccccacttgctcaagctactaacaaaggtcagctccgtggccttgaggagttaagcctgtgtcctcgcctggaggatgctgcaccaacaatctgagacttctctaagatgttgaggacctcagtcactttgatgctcccaatatgatgaaaatctgctaaaagctggttatgttcacgagcacaccccatgaggaggaaggtggtattgagaaaccctgcctgaaattttaaggtggaactgtaacacgtagaagcagccaaggggcaagaattagtggtgacaaaatttgggaggcaatccttcatgtgctcgcccacacaggtcgggcagctacaggacgcagatgtgatagacttaggagtgctggccttgagtttcacaaaaggctccaaattggtgaggttgttgcagagataagaccggcagacgcgactgtaggaggcaatggacactccgggtggggaaacaaggtaggagatttgcgcagggtaagacgaagacgagctgcagcctttaaagcccacgactccccttgcagtccctgtctcaatgaacactagcgtctcctcgcagccctcttgcagcttacacaccatgttcctcatcagaagccacttccagttatggaaagcaacagctctgaatcttgaggctgttgcttcatagcacaaaagagctccagcccgaggcagagtggagatggcccctagaaggcagaacagctgcacaagtctcaaatgctggggtcccatggccctgtgtctgggtcctgggtgctagaggtcagtctggaatcagtttcagtctggatcccaagctcagttcccatcagtccccgaattctttgtccacctgtctctgggtcactgtttctcgaaagggggaagac

SEQ ID NO: 12284 - RNA, 1541 nt, Homo sapiens
  source 1..1541: mol_type = other RNA
ctgggaggtcaaggctgcagtgagccatgatcgggccactgtaatttagcctgagtgacagaatgagaccctggctggaaaaaaaaataaaataaaaaagaaagattttcctacccaaataatttaggttatcctcctaataactttggcagtaattttactttttcatatttgtctttactgctcatataattttttgtttatatcaaggtatagagatataatttaatcatggcatgtttagtagactatcgatgctgggaaagggcttaggagatgatgatgaatcaaaacatgggatagaggctgggtacgtggctcaggcctgtaatcccagcattctggggagccaaggtgggtgaattgtttgaacccaggagtttgagaccagcctcggcaacatagtgatacctcatctctacaaaaaaattttttaaaaaattagttgggcatggtggcatgttcctgtagtttcagctactcatgaggctgaggctggaggattgcttcagacagggaggtcgaggctgcagtgagcaatgattgtgccactgcactgcagcctgtgacgtttgtttgtttgagacagggtctcactgtgtctgaaaaaaccaaacaaacaaaaattaaataaaaaacccacaggatagaaatctctatggataataatacatgaatgaaaagaaagaatgacagagatcaaattaatgaagtcatttctgtgtggaagacttcctgatgattttgatgctttttccccaaggaatttttctttttttttccaggaaatatgtatgatatgaattatggtaaatggccctttcctttgacttttgaatctctggttttccttcatctccgctgacatcaggacattcctgagcatcacaaaggtcagttccagtgtttggtatgattccttcttctcttatgatccatttcatctcccttctgctctctggagcctccctccttcctggaccgaggccccaaggttggagctcacagactgattcctgggatgagcagcctccacctgcaggagcagtggcaggaacaagggaggggacaggaggccaaggtcccatcctggaggctgggggactgggtcgtgcattagcaagggtttggggttgagtcagctccagacctgatcctgctgttttggtctggaggcctccctctgccctgagacaaaagtccagtcaatcagttgtgggagaaaacgttcatatcaacatggattttgggaagctggatgaactcagagcctgacacgagaccgggagactctcttctgtgcagagtcccgtccaggtgcggggaacagggggagagcctgggacgtcctggctggggagaaaggggagcggggtcctctgtcttcagtcctgtggccacacgggggcgccgccacagtgctctcggattctgactgagcgctttcggggaccaggctgcgggctgagtggggcagacggggctgatcctgaggtcatccacgccaggatggaggcgtctcctgagcagccctggaatcc

SEQ ID NO: 12285 - RNA, 1511 nt, Homo sapiens
  source 1..1511: mol_type = other RNA
ctgggaggtcaaggctgcagtgagccatgatcgtgccagtgcactccagcctggacgatgaaatgaaactcttcgttagcgcgaaggccactgtcccgtcatcctcagtggaaaggtcaagcagcttctggtaaaatgcttcatcataaggcccatctatttgtaaggtttttctctcctcgggaaactcttccaggtatcgctcaacccggttgtacagagggtagaggccttcgatgtccagcaggtccaacatctgcacctggagggttttgtacagaagacagcccttcggtaaccccgagcgctctggggtgttttttccttggcagcgaaggctcctactgaaagggctggcttcgcagactcgcgggccctgaggcccgagccccggactcagggtgcctgcccggcccttgtccgagccactcagcagcacccgtgtgatcacgtgcaccagctccctgatcacagcccttgtgcagtggggcccactggccaggccgttggaagggaagaagaacggcttcaggtggtgtgcaagctcgctccagtcagccacggggctccgggcatctttgcagccgtaaatcagctcaccattcttaaatatcttcaagttgttctgtgcctcctgcagcaaactcttcaaggcaaagtgcattctctgtttgtttcctgagtagagatcaaggggacagtatttgctgatctgcttccacttcccagttgctaccttgaggtgctggtgcatgcagtatcgacagaccttatgcttcatctcatgcgtgacatcactcgagaaaggaataaacccacattttggcttaatctctacacacagaatcggccggtgctctgcaaagcggtaggtttggagtctggttaaattaggaaggcacatagcgtaaccactgagagtatccaggtccttgtcacagcgagactctggtctttcagattgtatctttaaacaaagctgtttcacaaactctaaaggtagctgaacgacctccccataatgaacatagttctcccccaaaaactccttcatgacatttttcccaaagtccactatgttctgcaggtgttgaaatatctcttccgaggtcttcttcctatttggaggaaacttcagaaaccgcagcacgacgcagcgctgcgcgtgggccaccaccaggctcttattgccctctccgtggtacccccattcattctcgtccatcttcccctcttccatgcccaggcgcagccctggcgcctcgcgggctaggactcggggacgcgagctgggggccgcccgcctcgctgggaaccagccgctgcggtcgggggaggagcgcctgtcagctgccgcccccgctcgaccccgccgcggcgactagcaagctgtggccgccggaagccacgcccccggcgcctgccatgacggagtcgggcaattccgggttcgtgacactttcctcacaccgatcgcgacggtggatgggccggcggccatcttaggtact

SEQ ID NO: 12286 - RNA, 5561 nt, Homo sapiens
  source 1..5561: mol_type = other RNA
ctgggaggtcaaggctgcagtgagccatgatggcgccactgcactccagcctaggtgacagaacgagactctgtctcaaaaaaacaaaacaaaacaagtaagactctaccttattccccagttctaacttctgcttttgctttcttgccctacatctttcctcatcctaaagatttagtatgtgccatatgtttggtatatgttattgcacttaaacctcacaacagtatgaggtaggtattattacacaacctttttcacagatgaagaaactagatacagagaggttaaaatgcctaaggtcatttaatagtatcagaattagaatagaaacccagctggctgcaaggccattattttgcctctataaaaagcaattttcaagctgtgtccccaaaattccatggagactcagggttgccagggagactggagagatgaacgggctgcggctcatctcacttttacagacagctatgacatgtggactgccacatattctttggatgccatggactcatttctgccttcctgtttgcctgggcttccttcacctgtaactcagagatgaatcttacctcactcactcatatcccccaacagccacctctttggtggatgtattttctttccggtctgcccttgcatgtttccattaaccttttcactccctggactgccataaaataacagggagtagttataatggtcattttagaaatgctaccataacatataagcaatattaccaactcttccacactataaaaatagagacgagtgtagctcacactatttaaaacactggataaccctccagatcatttgtcattacaattaattttaccaacacagcatttatattttaataaaattcattattcatatcaactatggagtattctagaataacctgcaatattttaagccatatgaagacatactagaaagacctaaggtgaaaagctttgttcaaaggcttcctcaattttctcctttgctcaattttatgagctctactacatgatgttgatttctgacagcttatcatataacaggtatgtgatgtttgaaggcaaagtaaccctcttaatattaaaattaatatttttgattcatttttcttgcccatatattcacatagtttataatgacactgaacaaaactgtttgtgaagaagactgaaacattcctgattagtttaattaatgagaaaaatgtggctgagttatgacctaaattattaacagtgatcttcagtctgacatgaaatctctttttacatagccagtattaccaaataaatggtactatcttgcagtactatgagtattctgctcccatccttttaagccagataagtaaacactatggacatattactacagcatttctcaaagtatggtctagagagcacctgcatcagaatctccaaaggtactatttatatcttttatgttgtttttttttcttgaaagagacagtggtctgactatcttgcccaggctggtcttgaactcctgggctcaagtgatcctgctgcctcaacctctgaagtagctgtggtaacaggtacatgccatggcacccggcatgaggtgttatttataatatgcagattcctgggccctacaagcaacctgaggaatcaaaatttctaaagcagaccaagaaatctccatttttaaacaagctctcacaggtactgcttaggtattgatttgagaaatcaatgatataaatccttttaatctgatcttactatttaatggagatattgactaaaacaaaaacaaaaaccttttctctattttgctgatatttaaattttcacatttgtagaatgtttcttagtatatgtccttgtaacataagcattctctaataattaaaaaatttaggggcaataatactgatcataatactattctcgaaagcactctctcaaagtaaattttcactttttaggaggagttgtaggatagtgaaattcttcattaaagagttagtgataaactaactagtcttcagtcaatttagcagttcacatagtttattcagcaatataacaggagagaacctccattgtaagagacataaggcagatacagggtgcatctctggggtacattcttcatacagactaacaaataacttcaggtttcacaacatgtagcaagtatgatttgttgcacaccaacagccattcattcctcacgttttccttgctaaaagagccctggtcaggcacggtggctatgcctgtaatcccagcactgtcggaggtcagggcaggtggatcatctgaggtcaggagttcaagaccagcctggccaacatggtgaaaccccgtctctactaaaaacacaaaaattagccagacatggtggcgggcacctgtaatccccactactcaggaggctgaggcaggagaattgcttgaacctaggaggtggaggttacagtaagccgagatcgtgccactacactccatcctgggcaagagagcgagactccgtcaaaaaaaaaaaaaaaaaagggctgggcacagtggctcatgcctgtaatcccagcactttgggaggccaaggcgggtggatcatgagatcaagagatcaagaccatcctggccaacaatggtgaaaccccatctctactaaaaatacaaaaattagccaagtgtggtggcgcacacctgtagtcccagctactcgggaggctgaggcaggagaattgcttgaacccggaaggcagaggttgcagtgaaccaagactgccactgcactccagcctgggcgacagagtgagactctgtctcaaaaaaaaaaaaaaaaaaaaaaaagccctgatttcttcaatggaggcaatgtggcctacccaggcaatgctaaccctattcccctttgccaaggtttcccaggctcccttgtaaactggtactttctaatgagatgtaagaagaaatttgctagggatttttgggaaagacttgattcccaaataaaacactgacttgaaagaaagccttttgctctctacttccagcctttcctagggattaaaatgtctgttacaacaagaagtcatattgtactcattgagaaaaaaaaacctaacgataaaaagcaaacatggatcctaggccgggtagggtggctcacgcctgtaatcccagcaccttgggagaccgaggtgggaggatggcttgagcctaggagttggagaccagcctgggtcatacagcaagactctgtcactattttttaaaaagcaaaaaaaaaaaaaaaaaaaaagaggatcgcaagggggaaggacacaaagaagctgggaccttgataatattgataatattgctaaaagcactagatacctagatacctggcatgttaagtgtaatttaaaaattgttcagtggcctttgagatgttttcaacagctttttctaagtggcttaaccccaactctgggtccatgattttcatgaaagtccagaatgtggccaatgttcagcagacctccttagttctaagaaagatgcttcctctagactgttcataatatatatgaagtcaggcttgataatttcttttgtcatacatctcctgataggtacttttccatttccaggggaggacgttgtaaattcagtcaccacaaagacaagacagtcttttgtttatgtaaagccacgtaagtatggacaggtggcatttctgcatgtttctgcataacctatataggtgtttcctaatagaatgtgatttatctgacagtgaccagttatcaataatctcacagccacactgaggatgggccaaacagggccaatgatgaataaatggctatataagagcaaattttatctatctatctatttatatatatatctcatcactgaccaatgcataagaggtgagtttacaacagtgtaatttcttattaaaattcactggactaatctaggatccagctataacgaggctgctttcccacaaaagttatcattagaaataccactatgaagcacacagtataggacttcccctctaggactactttgtcatatgacactcattaggttgcagaaatttttttaggagtggtaagttagttccaaaacagtttataggaaatacggattagcctcagtctagatgaacagattagcctcagtctagatgaacaggctggctggaatactaactaaattcatgtgaataaaatatgtataggccacggaagcagatccaacaatttaagcagttcccaaagtagtgacaatctgggtcagacttagaaatgaattatttttccatcttccttgggctacctacacaaaagcctctagacttgacaattttgactattatagaagctatttgttttggcccagttttttgtttaaggttttatctgttctggtcaagattaactgtaatgcagggttaaaaccagctactcgagagtcatgtattctttttctaaccagtggaggacccagaagaaatggatggcaagctttctcaaaggtccatctggtgagattctggggagcccactcaagtgggaaagaccaaggaagaacaaggcttctattagcaggattatcaggataacactcaggacaataatcagctctgttaatacggtctaagaatacctggtaacattcattttcaacaagttcagtttggtacaaccagtggcctagttctaaactagggaaccactgttgtccacaatcagggcaatgtgaattatctgaaaacatctggacctagaaagacaacacagacagcaatgtgacagcaagagacaacagtgacagagagagacgcccaaacaccagtcctattacaggtttcgtttaccaatttcttagttcaaccaatattatttggagagccaaataaacttggcttgcacctccgtgcaattcttcaagatttcgttgtctatttttcactcaattgcaactcagtctctgaactcagggaccgatccagtttataatgttatcagtcacttactagcagtacagatctcaggatagctccttcaaatcccagcttctcaagaagagatagggctctagtctaaattagttatatttttcttatgcgtcatcagctgctggtggtgtcacacagaggcacttggcttactctgctttgttggtaaggttattgtgtctgcttggtgaaacagaggagctgacaggtccaatgggtcttttgttggcgctggcactcttgccgttgtaacacacgtacccaagtcttaaggccttggcactttatagcaatgtagaggggtcagaaaaacctggcagagtcctcttgatcgtggatccaatgaagtctgtcttgggaggacattaatcaggacccaattgctgtgaagaagctgatgctcagttggctgaagagtctgggaatgcgtcacatacaaattctggcgaagttttaaatcgtaaaactgttagtatcaggagagcccttcgagtattctctccgctccacaccgctcggctgcacccagcggccgccgcggcccgaat

SEQ ID NO: 12287 - RNA, 5483 nt, Homo sapiens
  source 1..5483: mol_type = other RNA
ctgggaggtcaaggctgcagtgagccatgatggcgccactgcactccagcctaggtgacagaacgagactctgtctcaaaaaaacaaaacaaaacaagtaagactctaccttattccccagttctaacttctgcttttgctttcttgccctacatctttcctcatcctaaagatttagtatgtgccatatgtttggtatatgttattgcacttaaacctcacaacagtatgaggtaggtattattacacaacctttttcacagatgaagaaactagatacagagaggttaaaatgcctaaggtcatttaatagtatcagaattagaatagaaacccagctggctgcaaggccattattttgcctctataaaaagcaattttcaagctgtgtccccaaaattccatggagactcagggttgccagggagactggagagatgaacgggctgcggctcatctcacttttacagacagctatgacatgtggactgccacatattctttggatgccatggactcatttctgccttcctgtttgcctgggcttccttcacctgtaactcagagatgaatcttacctcactcactcatatcccccaacagccacctctttggtggatgtattttctttccggtctgcccttgcatgtttccattaaccttttcactccctggactgccataaaataacagggagtagttataatggtcattttagaaatgctaccataacatataagcaatattaccaactcttccacactataaaaatagagacgagtgtagctcacactatttaaaacactggataaccctccagatcatttgtcattacaattaattttaccaacacagcatttatattttaataaaattcattattcatatcaactatggagtattctagaataacctgcaatattttaagccatatgaagacatactagaaagacctaaggtgaaaagctttgttcaaaggcttcctcaattttctcctttgctcaattttatgagctctactacatgatgttgatttctgacagcttatcatataacaggtatgtgatgtttgaaggcaaagtaaccctcttaatattaaaattaatatttttgattcatttttcttgcccatatattcacatagtttataatgacactgaacaaaactgtttgtgaagaagactgaaacattcctgattagtttaattaatgagaaaaatgtggctgagttatgacctaaattattaacagtgatcttcagtctgacatgaaatctctttttacatagccagtattaccaaataaatggtactatcttgcagtactatgagtattctgctcccatccttttaagccagataagtaaacactatggacatattactacagcatttctcaaagtatggtctagagagcacctgcatcagaatctccaaaggtactatttatatcttttatgttgtttttttttcttgaaagagacagtggtctgactatcttgcccaggctggtcttgaactcctgggctcaagtgatcctgctgcctcaacctctgaagtagctgtggtaacaggtacatgccatggcacccggcatgaggtgttatttataatatgcagattcctgggccctacaagcaacctgaggaatcaaaatttctaaagcagaccaagaaatctccatttttaaacaagctctcacaggtactgcttaggtattgatttgagaaatcaatgatataaatccttttaatctgatcttactatttaatggagatattgactaaaacaaaaacaaaaaccttttctctattttgctgatatttaaattttcacatttgtagaatgtttcttagtatatgtccttgtaacataagcattctctaataattaaaaaatttaggggcaataatactgatcataatactattctcgaaagcactctctcaaagtaaattttcactttttaggaggagttgtaggatagtgaaattcttcattaaagagttagtgataaactaactagtcttcagtcaatttagcagttcacatagtttattcagcaatataacaggagagaacctccattgtaagagacataaggcagatacagggtgcatctctggggtacattcttcatacagactaacaaataacttcaggtttcacaacatgtagcaagtatgatttgttgcacaccaacagccattcattcctcacgttttccttgctaaaagagccctggtcaggcacggtggctatgcctgtaatcccagcactgtcggaggtcagggcaggtggatcatctgaggtcaggagttcaagaccagcctggccaacatggtgaaaccccgtctctactaaaaacacaaaaattagccagacatggtggcgggcacctgtaatccccactactcaggaggctgaggcaggagaattgcttgaacctaggaggtggaggttacagtaagccgagatcgtgccactacactccatcctgggcaagagagcgagactccgtcaaaaaaaaaaaaaaaaaagggctgggcacagtggctcatgcctgtaatcccagcactttgggaggccaaggcgggtggatcatgagatcaagagatcaagaccatcctggccaacaatggtgaaaccccatctctactaaaaatacaaaaattagccaagtgtggtggcgcacacctgtagtcccagctactcgggaggctgaggcaggagaattgcttgaacccggaaggcagaggttgcagtgaaccaagactgccactgcactccagcctgggcgacagagtgagactctgtctcaaaaaaaaaaaaaaaaaaaaaaaagccctgatttcttcaatggaggcaatgtggcctacccaggcaatgctaaccctattcccctttgccaaggtttcccaggctcccttgtaaactggtactttctaatgagatgtaagaagaaatttgctagggatttttgggaaagacttgattcccaaataaaacactgacttgaaagaaagccttttgctctctacttccagcctttcctagggattaaaatgtctgttacaacaagaagtcatattgtactcattgagaaaaaaaaacctaacgataaaaagcaaacatggatcctaggccgggtagggtggctcacgcctgtaatcccagcaccttgggagaccgaggtgggaggatggcttgagcctaggagttggagaccagcctgggtcatacagcaagactctgtcactattttttaaaaagcaaaaaaaaaaaaaaaaaaaaagaggatcgcaagggggaaggacacaaagaagctgggaccttgataatattgataatattgctaaaagcactagatacctagatacctggcatgttaagtgtaatttaaaaattgttcagtggcctttgagatgttttcaacagctttttctaagtggcttaaccccaactctgggtccatgattttcatgaaagtccagaatgtggccaatgttcagcagacctccttagttctaagaaagatgcttcctctagactgttcataatatatatgaagtcaggcttgataatttcttttgtcatacatctcctgataggtacttttccatttccaggggaggacgttgtaaattcagtcaccacaaagacaagacagtcttttgtttatgtaaagccacgtaagtatggacaggtggcatttctgcatgtttctgcataacctatataggtgtttcctaatagaatgtgatttatctgacagtgaccagttatcaataatctcacagccacactgaggatgggccaaacagggccaatgatgaataaatggctatataagagcaaattttatctatctatctatttatatatatatctcatcactgaccaatgcataagaggtgagtttacaacagtgtaatttcttattaaaattcactggactaatctaggatccagctataacgaggctgctttcccacaaaagttatcattagaaataccactatgaagcacacagtataggacttcccctctaggactactttgtcatatgacactcattaggttgcagaaatttttttaggagtggtaagttagttccaaaacagtttataggaaatacggattagcctcagtctagatgaacagattagcctcagtctagatgaacaggctggctggaatactaactaaattcatgtgaataaaatatgtataggccacggaagcagatccaacaatttaagcagttcccaaagtagtgacaatctgggtcagacttagaaatgaattatttttccatcttccttgggctacctacacaaaagcctctagacttgacaattttgactattatagaagctatttgttttggcccagttttttgtttaaggttttatctgttctggtcaagattaactgtaatgcagggttaaaaccagctactcgagagtcatgtattctttttctaaccagtggaggacccagaagaaatggatggcaagctttctcaaaggtccatctggtgagattctggggagcccactcaagtgggaaagaccaaggaagaacaaggcttctattagcaggattatcaggataacactcaggacaataatcagctctgttaatacggtctaagaatacctggtaacattcattttcaacaagttcagtttggtacaaccagtggcctagttctaaactagggaaccactgttgtccacaatcagggcaatgtgaattatctgaaaacatctggacctagaaagacaacacagacagcaatgtgacagcaagagacaacagtgacagagagagacgcccaaacaccagtcctattacaggtttcgtttaccaatttcttagttcaaccaatattatttggagagccaaataaacttggcttgcacctccgtgcaattcttcaagatttcgttgtctatttttcactcaattgcaactcagtctctgaactcagggaccgatccagtttataatgttatcagtcacttactagcagtacagatctcaggatagctccttcaaatcccagcttctcaagaagagatagggctctagtctaaattagttatatttttcttatgcgtcatcagctgctggtggtgtcacacagaggcacttggcttactctgctttgttggtaaggttattgtgtctgcttggtgaaacagaggagctgacaggtccaatgggtcttttgttggcgctggcactcttgccgttgtaacacacgtacccaagtcttaaggccttggcactttatagcaatgtagaggggtcagaaaaacctggcagagtcctcttgatcgtggatccaatgaagtctgtcttgggaggacattaatcaggacccaattgctgtgaagaagctgatgctcagttggctgaagagtctgggaatgcgtcacatacataaagtttcaaaaggatataaaattaatgtgt

SEQ ID NO: 12288 - RNA, 5696 nt, Homo sapiens
  source 1..5696: mol_type = other RNA
ctgggaggtcaaggctgcagtgagccatgatggcgccactgcactccagcctaggtgacagaacgagactctgtctcaaaaaaacaaaacaaaacaagtaagactctaccttattccccagttctaacttctgcttttgctttcttgccctacatctttcctcatcctaaagatttagtatgtgccatatgtttggtatatgttattgcacttaaacctcacaacagtatgaggtaggtattattacacaacctttttcacagatgaagaaactagatacagagaggttaaaatgcctaaggtcatttaatagtatcagaattagaatagaaacccagctggctgcaaggccattattttgcctctataaaaagcaattttcaagctgtgtccccaaaattccatggagactcagggttgccagggagactggagagatgaacgggctgcggctcatctcacttttacagacagctatgacatgtggactgccacatattctttggatgccatggactcatttctgccttcctgtttgcctgggcttccttcacctgtaactcagagatgaatcttacctcactcactcatatcccccaacagccacctctttggtggatgtattttctttccggtctgcccttgcatgtttccattaaccttttcactccctggactgccataaaataacagggagtagttataatggtcattttagaaatgctaccataacatataagcaatattaccaactcttccacactataaaaatagagacgagtgtagctcacactatttaaaacactggataaccctccagatcatttgtcattacaattaattttaccaacacagcatttatattttaataaaattcattattcatatcaactatggagtattctagaataacctgcaatattttaagccatatgaagacatactagaaagacctaaggtgaaaagctttgttcaaaggcttcctcaattttctcctttgctcaattttatgagctctactacatgatgttgatttctgacagcttatcatataacaggtatgtgatgtttgaaggcaaagtaaccctcttaatattaaaattaatatttttgattcatttttcttgcccatatattcacatagtttataatgacactgaacaaaactgtttgtgaagaagactgaaacattcctgattagtttaattaatgagaaaaatgtggctgagttatgacctaaattattaacagtgatcttcagtctgacatgaaatctctttttacatagccagtattaccaaataaatggtactatcttgcagtactatgagtattctgctcccatccttttaagccagataagtaaacactatggacatattactacagcatttctcaaagtatggtctagagagcacctgcatcagaatctccaaaggtactatttatatcttttatgttgtttttttttcttgaaagagacagtggtctgactatcttgcccaggctggtcttgaactcctgggctcaagtgatcctgctgcctcaacctctgaagtagctgtggtaacaggtacatgccatggcacccggcatgaggtgttatttataatatgcagattcctgggccctacaagcaacctgaggaatcaaaatttctaaagcagaccaagaaatctccatttttaaacaagctctcacaggtactgcttaggtattgatttgagaaatcaatgatataaatccttttaatctgatcttactatttaatggagatattgactaaaacaaaaacaaaaaccttttctctattttgctgatatttaaattttcacatttgtagaatgtttcttagtatatgtccttgtaacataagcattctctaataattaaaaaatttaggggcaataatactgatcataatactattctcgaaagcactctctcaaagtaaattttcactttttaggaggagttgtaggatagtgaaattcttcattaaagagttagtgataaactaactagtcttcagtcaatttagcagttcacatagtttattcagcaatataacaggagagaacctccattgtaagagacataaggcagatacagggtgcatctctggggtacattcttcatacagactaacaaataacttcaggtttcacaacatgtagcaagtatgatttgttgcacaccaacagccattcattcctcacgttttccttgctaaaagagccctggtcaggcacggtggctatgcctgtaatcccagcactgtcggaggtcagggcaggtggatcatctgaggtcaggagttcaagaccagcctggccaacatggtgaaaccccgtctctactaaaaacacaaaaattagccagacatggtggcgggcacctgtaatccccactactcaggaggctgaggcaggagaattgcttgaacctaggaggtggaggttacagtaagccgagatcgtgccactacactccatcctgggcaagagagcgagactccgtcaaaaaaaaaaaaaaaaaagggctgggcacagtggctcatgcctgtaatcccagcactttgggaggccaaggcgggtggatcatgagatcaagagatcaagaccatcctggccaacaatggtgaaaccccatctctactaaaaatacaaaaattagccaagtgtggtggcgcacacctgtagtcccagctactcgggaggctgaggcaggagaattgcttgaacccggaaggcagaggttgcagtgaaccaagactgccactgcactccagcctgggcgacagagtgagactctgtctcaaaaaaaaaaaaaaaaaaaaaaaagccctgatttcttcaatggaggcaatgtggcctacccaggcaatgctaaccctattcccctttgccaaggtttcccaggctcccttgtaaactggtactttctaatgagatgtaagaagaaatttgctagggatttttgggaaagacttgattcccaaataaaacactgacttgaaagaaagccttttgctctctacttccagcctttcctagggattaaaatgtctgttacaacaagaagtcatattgtactcattgagaaaaaaaaacctaacgataaaaagcaaacatggatcctaggccgggtagggtggctcacgcctgtaatcccagcaccttgggagaccgaggtgggaggatggcttgagcctaggagttggagaccagcctgggtcatacagcaagactctgtcactattttttaaaaagcaaaaaaaaaaaaaaaaaaaaagaggatcgcaagggggaaggacacaaagaagctgggaccttgataatattgataatattgctaaaagcactagatacctagatacctggcatgttaagtgtaatttaaaaattgttcagtggcctttgagatgttttcaacagctttttctaagtggcttaaccccaactctgggtccatgattttcatgaaagtccagaatgtggccaatgttcagcagacctccttagttctaagaaagatgcttcctctagactgttcataatatatatgaagtcaggcttgataatttcttttgtcatacatctcctgataggtacttttccatttccaggggaggacgttgtaaattcagtcaccacaaagacaagacagtcttttgtttatgtaaagccacgtaagtatggacaggtggcatttctgcatgtttctgcataacctatataggtgtttcctaatagaatgtgatttatctgacagtgaccagttatcaataatctcacagccacactgaggatgggccaaacagggccaatgatgaataaatggctatataagagcaaattttatctatctatctatttatatatatatctcatcactgaccaatgcataagaggtgagtttacaacagtgtaatttcttattaaaattcactggactaatctaggatccagctataacgaggctgctttcccacaaaagttatcattagaaataccactatgaagcacacagtataggacttcccctctaggactactttgtcatatgacactcattaggttgcagaaatttttttaggagtggtaagttagttccaaaacagtttataggaaatacggattagcctcagtctagatgaacagattagcctcagtctagatgaacaggctggctggaatactaactaaattcatgtgaataaaatatgtataggccacggaagcagatccaacaatttaagcagttcccaaagtagtgacaatctgggtcagacttagaaatgaattatttttccatcttccttgggctacctacacaaaagcctctagacttgacaattttgactattatagaagctatttgttttggcccagttttttgtttaaggttttatctgttctggtcaagattaactgtaatgcagggttaaaaccagctactcgagagtcatgtattctttttctaaccagtggaggacccagaagaaatggatggcaagctttctcaaaggtccatctggtgagattctggggagcccactcaagtgggaaagaccaaggaagaacaaggcttctattagcaggattatcaggataacactcaggacaataatcagctctgttaatacggtctaagaatacctggtaacattcattttcaacaagttcagtttggtacaaccagtggcctagttctaaactagggaaccactgttgtccacaatcagggcaatgtgaattatctgaaaacatctggacctagaaagacaacacagacagcaatgtgacagcaagagacaacagtgacagagagagacgcccaaacaccagtcctattacaggtttcgtttaccaatttcttagttcaaccaatattatttggagagccaaataaacttggcttgcacctccgtgcaattcttcaagatttcgttgtctatttttcactcaattgcaactcagtctctgaactcagggaccgatccagtttataatgttatcagtcacttactagcagtacagatctcaggatagctccttcaaatcccagcttctcaagaagagatagggctctagtctaaattagttatatttttcttatgcgtcatcagctgctggtggtgtcacacagaggcacttggcttactctgctttgttggtaaggttattgtgtctgcttggtgaaacagaggagctgacaggtccaatgggtcttttgttggcgctggcactcttgccgttgtaacacacgtacccaagtcttaaggccttggcactttatagcaatgtagaggggtcagaaaaacctggcagagtcctcttgatcgtggatccaatgaagtctgtcttgggaggacattaatcaggacccaattgctgtgaagaagctgatgctcagttggctgaagagtctgggaatgcgtcacatacctcgtttactgtttgagtgaggccaggcgtggtggctcacgcctgtaatcccagcactttgggaggctgaggtgggagaatcgcttgaagccaggagttcgagaccaacctgggcaatacagtgagaccctgtcgaaattctggcgaagttttaaatcgtaaaactgttagtatcaggagagcccttcgagtattctctccgctccacaccgctcggctgcacccagcggccgccgcggcccgaat

SEQ ID NO: 12289 - RNA, 2776 nt, Homo sapiens
  source 1..2776: mol_type = other RNA
ctgggaggtcaaggctgcagtgagccatgattgagccactgcactccagcctgggcaacagagcaagaccctgtccaaaaaagaaaagtctaaatcacttgaaaattccacttccaccccagattctgcctgcattttactcttcatttgcattgatgttttcatgcttttttcatgtgtatcataatgagaatatgaagtaaaattacaaccacagattaaatcacttttttctataattgcacagttctcttaaaatacttgaggttgacgaattgatgaagttcaatcgttttgggaaaagaaagcaagaaagaggctgagacacacaaagatacacagagagatagagacagaattaaatcagaaagtaaaagtttggtcaaatataagaatacatttattaaaatgcttctaaatatttcattttttttgctgttttggaaaccaaacatataactatgatcgttaacgtgagacagtgtgtgggattcatatttcaaatttttgaagtataaaattacataagtaactgttttccagagtttaaggccaaaaacaataacttattttatgaattttgtataaatgttaaaacacattttagtatatggcaattttactcaacttttaatcaatctccttaattcaagtttgcttatttgattcctttaataaaatattagtcattatttgcatcccacaattctgtggaaccaaagcatcacaactcttaatatttgtgtttctcgtgttgtaaataagccaatagagtgggatggttccattctccagttaaaagtgacatattctgggaaaatggtcatgtattttttcagtctgttatatacattgctttgcctagttagagatatatgtatacatatatctcaaatgtgaaatgtagaaatggtagtgtggatcaagtgctatggaaacatattatgaaacagttaattctgcacaaggatgagaaggatggtgtttcaggacagctagtgagtgcaggtgacatttcagctgagttttgaagcattagtagaagtctatcagatgggctggcacattagaaggaaataatggatacatgaaccttgatggcaggtggatgaaggacaaacatttttttccagatagaacacagggtcttggattgacaagaggaatgtctgggaggatgaaccctcatgctgctttggtgtgtttctcttctttagaattccaatgcttcctagtccctgtggctttgggattgacaagaggaatgtctggggaggatgaatcctcacgctgccttgaggtgtttcccttctttagaattccaatgcttcctagtccctgtggctttgggattgacaagaggaatgtctggggaggatgaaccctcactctgccttgaggtgtttcccttgtttagaattccaggtgtttcctagtccttgtggctttgtccagcagcactacccagtatcagggtcctcaaggcccctttcacatctttgtttctcagagtgtagataatggggtttaaaagtggggtgactatggtatagaaaagagaaacaaactttccctggtttttggatctcctattggccggttgaaggtacatgaatatgatggtcccatagaaaatgatgaccacaaccaggtgagacgaacaggtcccaaaggccttttggcggcccgcagctgattttatccttaacacagcttgagtgataaagccataggagactaagatgagtaacaccgggacaattagaaagactacactggccacaaagagttctgcctcgttgaaagtcgtatccacacaggccagtttgatgagcactggcacctcacagaaaatatgatccagtgtgcgatgaccacagaggggcagctgcacagtgagggagcactgaattagggaggtgatgaggccgctgagccatgctccaccggccagagacgcacagaacctggggtgcataatggctatgtagcgcagtggccggcagacagcagcatagcggtcataagccatgacggccaagagaatacactcagacgagcccaaccccatggccacatagagctgggccacacagccaccgtagctcatggttttgtctttcttattcatggtaaccagcaactgtggggcaacactggtggtaaagcagatgtccacacacgagaggttgctgaggaagaagtacattggagtgtggagtctggagtccagacaacatactagtatgagggcagtgttccccagaaggctcaagacgtagaagtacaaaatgatggcaaaaagaaacctctctagctgaggctgatctgaaaatcccaggagaagaaatcccttttcagagctgttgttggtttcctccatttttcctgcagcttcaggactcttcagcttcaaatactgatattgtgggtgatctcaatttcttcctgggtgatctttcctggtttaatatttgtatgattccaatgataaatctcagataatataaatagcaaaaaattaaaatactgagaaaataatatacaacttattaggggagaaagaggaagagatgctcccttagtggcacacagaaggtgggatgcctggtctgctttttctatatttttgcatatttggggttcagaaaactgaaacccatagagtcaccatatgctacatacactgaacctaaagtaataagtagttctgaaagagaacagaggagaagagggactccctacagggataaatggtccagacttaaggtatggc

SEQ ID NO: 12290 - RNA, 179 nt, Homo sapiens
  source 1..179: mol_type = other RNA
ctgggaggtcaaggctgcagtgagccatgattgcgccactgcactccagactgggtgacagagtgagaccctgtctcaaaaaaaaaaaaaaaaaaaaaagaatttggtattcaatatataaagctaaattttccaaagacaaaaaacttagaaaaaaaagtttcctacaaatgttaagt

SEQ ID NO: 12291 - RNA, 1939 nt, Homo sapiens
  source 1..1939: mol_type = other RNA
ctgggaggtcaaggctgcagtgagccgtaactgtgccactgcactctagcctgggtggcagagcaagaccctgtctcaacaaaacccccaaaaccaaaagaaaacaaaaaaagcaaagcaaacaacaaaaaagatggtttctttttcttactgtggctctttgaattttaaagatattaactctttcttacatattgcgaatgtttttcctaggctttttatttttttaaatttctttcaccatatggaagtttggaaatattatatggtcaaattagctaatctttcccaatattctttgtcactatactacagtgccaactgaagtggtgacaactatggctggaggacggtaattaaaaaacagggaagcttcctaaaaataagaggtgaggataatgggatgaataaagggagaatctttcatctgagataaatacaaatgctcaactcctacttttttgttttgttttgtttttttaaagagatgggggtctcactatattgcccaggctggagtgcagtggctattcacaggtatgatcataacatacggcagcctctaactcctgggctcaagcaatcttcctgcctcagcctcccaagtagctgagactacaggtgcatgccactgtaccaggcctcaactcttattcttaacaacatgcctcggatgagtaaagtatgttatacacaaaaaactagggcagggaaataccagatcacttctggaaagccctgccaagcccagggtggtagagacagggtttttgcttaatccctggctgcagttcctgggtaggagggtcaatatggaggaaagaatctccaaggactgtaagagtagggacaagccaggattgggcggaggtgtcagaaaggtcttactttctggattactgcctagcacacatgaagcccttgcaggacagactgccaaaagcttggtagaaggctgtgcaccacttcgccagccttcaatcaacatgcaccaactgcaaaccaaatgacaacatctccaagtataaaaataggatgctaccttgtgttctcatcatatttatacagaatcaaaaataacccagacaaaacctcagagctgcttgtcccactggcctgcttgcaactgtgtttgtacctggggtctctccaggagcacctggggtcagggttccagctactgtctccacaatgatctccatgttccctggtccctcttcagttgctgtggcctctaccagcaggcagcctggctcagtaggtataggtgcagggtcccgggaaggacaggggctctggacaggccccaggattccacggttagagagaggcggggggatcagcaatagctcagggcacagtccatccatctccccggtgctactggctggctgtgagtccaaaagggggtctgtcatcaccaccgacttgtgtgttttggcttcttaaatgtgaatattatcgctgttctggggaatcttcaagcttgaccatacatggcctccggggggagccaaggaggacgctgagccgtcaagattaagaaccttcacctgcgggagggcagggtgaggtaggagacaggtgggcaccagagaagaaatacgcttatcttccgggcaggagggcgcgtggtcttggacagacacagtcgcttcgcttctctgggcctcagctttcctatctccagacccagagccggcgggagccgcatctctatggtcggccgcggctggaacggcccccggggcccgctttgtgcgaccgcctccggctcagccgcctctaggatattggggatgtggaagccactctctcttcctcttgccggctgccggggtactctatgttttgtctctgtggtttttcccgccctccacccccactccagccctgaagccggagaagcaccatcgagagctctggggtagagtggcgt

SEQ ID NO: 12292 - RNA, 2034 nt, Homo sapiens
  source 1..2034: mol_type = other RNA
ctgggaggtcaaggctgcagtgagccgtaactgtgccactgcactctagcctgggtggcagagcaagaccctgtctcaacaaaacccccaaaaccaaaagaaaacaaaaaaagcaaagcaaacaacaaaaaagatggtttctttttcttactgtggctctttgaattttaaagatattaactctttcttacatattgcgaatgtttttcctaggctttttatttttttaaatttctttcaccatatggaagtttggaaatattatatggtcaaattagctaatctttcccaatattctttgtcactatactacagtgccaactgaagtggtgacaactatggctggaggacggtaattaaaaaacagggaagcttcctaaaaataagaggtgaggataatgggatgaataaagggagaatctttcatctgagataaatacaaatgctcaactcctacttttttgttttgttttgtttttttaaagagatgggggtctcactatattgcccaggctggagtgcagtggctattcacaggtatgatcataacatacggcagcctctaactcctgggctcaagcaatcttcctgcctcagcctcccaagtagctgagactacaggtgcatgccactgtaccaggcctcaactcttattcttaacaacatgcctcggatgagtaaagtatgttatacacaaaaaactagggcagggaaataccagatcacttctggaaagccctgccaagcccagggtggtagagacagggtttttgcttaatccctggctgcagttcctgggtaggagggtcaatatggaggaaagaatctccaaggactgtaagagtagggacaagccaggattgggcggaggtgtcagaaaggtcttactttctggattactgcctagcacacatgaagcccttgcaggacagactgccaaaagcttggtagaaggctgtgcaccacttcgccagccttcaatcaacatgcaccaactgcaaaccaaatgacaacatctccaagtataaaaataggatgctaccttgtgttctcatcatatttatacagaatcaaaaataacccagacaaaacctcagagctgcttgtcccactggcctgcttgcaactgtgtttgtacctggggtctctccaggagcacctggggtcagggttccagctactgtctccacaatgatctccatgttccctggtccctcttcagttgctgtggcctctaccagcaggcagcctggctcagtaggtataggtgcagggtcccgggaaggacaggggctctggacaggccccaggattccacggttagagagaggcggggggatcagcaatagctcagggcacagtccatccatctccccggtgctactggctggctgtgagtccaaaagggggtctgtcatcaccaccgacttgtgtgttttggcttcttaaatgtgaatattatcgctgttctggggaatcttcaagcttgaccatacatggcctccggggggagccaaggaggacgctgagccgtcaagattaagaaccttcacctgcgggagggcagggtgaggtaggagacaggtgggcaccagagaagaaatacgcttatcttccgggcaggagggcgcgtggtcttggacagacacagtcgcttcgcttctctgggcctcagctttcctatctgtaaaatggaggtgatgacagtgtccacatcgtcgggcaggagctggatcataagagccagcgaactggaaaggcggtttgtaacctggaaggctccagacccagagccggcgggagccgcatctctatggtcggccgcggctggaacggcccccggggcccgctttgtgcgaccgcctccggctcagccgcctctaggatattggggatgtggaagccactctctcttcctcttgccggctgccggggtactctatgttttgtctctgtggtttttcccgccctccacccccactccagccctgaagccggagaagcaccatcgagagctctggggtagagtggcgt

SEQ ID NO: 12293 - RNA, 2272 nt, Homo sapiens
  source 1..2272: mol_type = other RNA
ctgggaggtcaaggctgcagtgagccgtaactgtgccactgcactctagcctgggtggcagagcaagaccctgtctcaacaaaacccccaaaaccaaaagaaaacaaaaaaagcaaagcaaacaacaaaaaagatggtttctttttcttactgtggctctttgaattttaaagatattaactctttcttacatattgcgaatgtttttcctaggctttttatttttttaaatttctttcaccatatggaagtttggaaatattatatggtcaaattagctaatctttcccaatattctttgtcactatactacagtgccaactgaagtggtgacaactatggctggaggacggtaattaaaaaacagggaagcttcctaaaaataagaggtgaggataatgggatgaataaagggagaatctttcatctgagataaatacaaatgctcaactcctacttttttgttttgttttgtttttttaaagagatgggggtctcactatattgcccaggctggagtgcagtggctattcacaggtatgatcataacatacggcagcctctaactcctgggctcaagcaatcttcctgcctcagcctcccaagtagctgagactacaggtgcatgccactgtaccaggcctcaactcttattcttaacaacatgcctcggatgagtaaagtatgttatacacaaaaaactagggcagggaaataccagatcacttctggaaagccctgccaagcccagggtggtagagacagggtttttgcttaatccctggctgcagttcctgggtaggagggtcaatatggaggaaagaatctccaaggactgtaagagtagggacaagccaggattgggcggaggtgtcagaaaggtcttactttctggattactgcctagcacacatgaagcccttgcaggacagactgccaaaagcttggtagaaggctgtgcaccacttcgccagccttcaatcaacatgcaccaactgcaaaccaaatgacaacatctccaagtataaaaataggatgctaccttgtgttctcatcatatttatacagaatcaaaaataacccagacaaaacctcagagctgcttgtcccactggcctgcttgcaactgtgtttgtacctggggtctctccaggagcacctggggtcagggttccagctactgtctccacaatgatctccatgttccctggtccctcttcagttgctgtggcctctaccagcaggcagcctggctcagtaggtataggtgcagggtcccgggaaggacaggggctctggacaggccccaggattccacggttagagagaggcggggggatcagcaatagctcagggcacagtccatccatctccccggtgctactggctggctgtgagtccaaaagggggtctgtcatcaccaccgacttgtgtgttttggcttcttaaatgtgaatattatcgctgttctggggaatcttcaagcttgaccatacatggcctccggggggagccaaggaggacgctgagccgtcaagattaagaaccttcacctgcgggagggcagggtgaggtaggagacaggtgggcaccagagaagaaatacgcttatcttccgggcaggagggcgcgtggtcttggacagacacagtcgcttcgcttctctgggcctcagctttcctatctgtaaaatggaggtgatgacagtgtccacatcgtcgggcaggagctggatcataagagccagcgaactggaaaggcggtttgtaacctggaaggcttgggatggagcatcgtcatgattttgtcctgagagcagcaggtacccgggcggggtccagaaccgtgacgcgactgcagcgccggggcccagctcgtctgggtgctcccttcagtacctccttccgagagttcccagcgcccaggcccaccctgatcccggggctcgaaaaactttgcctccagctcgctccacccgcattcccttcccagttccgccccgcagccgctcactcacctccagacccagagccggcgggagccgcatctctatggtcggccgcggctggaacggcccccggggcccgctttgtgcgaccgcctccggctcagccgcctctaggatattggggatgtggaagccactctctcttcctcttgccggctgccggggtactctatgttttgtctctgtggtttttcccgccctccacccccactccagccctgaagccggagaagcaccatcgagagctctggggtagagtggcgt

SEQ ID NO: 12294 - RNA, 1960 nt, Homo sapiens
  source 1..1960: mol_type = other RNA
ctgggaggtcaaggctgcagtgagccgtaactgtgccactgcactctagcctgggtggcagagcaagaccctgtctcaacaaaacccccaaaaccaaaagaaaacaaaaaaagcaaagcaaacaacaaaaaagatggtttctttttcttactgtggctctttgaattttaaagatattaactctttcttacatattgcgaatgtttttcctaggctttttatttttttaaatttctttcaccatatggaagtttggaaatattatatggtcaaattagctaatctttcccaatattctttgtcactatactacagtgccaactgaagtggtgacaactatggctggaggacggtaattaaaaaacagggaagcttcctaaaaataagaggtgaggataatgggatgaataaagggagaatctttcatctgagataaatacaaatgctcaactcctacttttttgttttgttttgtttttttaaagagatgggggtctcactatattgcccaggctggagtgcagtggctattcacaggtatgatcataacatacggcagcctctaactcctgggctcaagcaatcttcctgcctcagcctcccaagtagctgagactacaggtgcatgccactgtaccaggcctcaactcttattcttaacaacatgcctcggatgagtaaagtatgttatacacaaaaaactagggcagggaaataccagatcacttctggaaagccctgccaagcccagggtggtagagacagggtttttgcttaatccctggctgcagttcctgggtaggagggtcaatatggaggaaagaatctccaaggactgtaagagtagggacaagccaggattgggcggaggtgtcagaaaggtcttactttctggattactgcctagcacacatgaagcccttgcaggacagactgccaaaagcttggtagaaggctgtgcaccacttcgccagccttcaatcaacatgcaccaactgcaaaccaaatgacaacatctccaagtataaaaataggatgctaccttgtgttctcatcatatttatacagaatcaaaaataacccagacaaaacctcagagctgcttgtcccactggcctgcttgcaactgtgtttgtacctggggtctctccaggagcacctggggtcagggttccagctactgtctccacaatgatctccatgttccctggtccctcttcagttgctgtggcctctaccagcaggcagcctggctcagtaggtataggtgcagggtcccgggaaggacaggggctctggacaggccccaggattccacggttagagagaggcggggggatcagcaatagctcagggcacagtccatccatctccccggtgctactggctggctgtgagtccaaaagggggtctgtcatcaccaccgacttgtgtgttttggcttcttaaatgtgaatattatcgctgttctggggaatcttcaagcttgaccatacatggcctccggggggagccaaggaggacgctgagccgtcaagattaagaaccttcacctgcgggagggcagggtgaggtaggagacaggtgggcaccagagaagaaatacgcttatcttccgggcaggagggctgaggaagagaaaggacagacgcgtggtcttggacagacacagtcgcttcgcttctctgggcctcagctttcctatctccagacccagagccggcgggagccgcatctctatggtcggccgcggctggaacggcccccggggcccgctttgtgcgaccgcctccggctcagccgcctctaggatattggggatgtggaagccactctctcttcctcttgccggctgccggggtactctatgttttgtctctgtggtttttcccgccctccacccccactccagccctgaagccggagaagcaccatcgagagctctggggtagagtggcgt

SEQ ID NO: 12295 - RNA, 29208 nt, Homo sapiens
  source 1..29208: mol_type = other RNA
ctgggaggtcaaggctgcagtgagccgtaatcatacctctccactccagcctggatgacagagcaagaccctcttaaaaaacaaacaaacaaaaaaaaaacaaacaaaaaaacaaaaacaacagaaaaatcagagccaagatttcaagtcttgtcttcccccttttttttttaaacaaatctcagattttcaaatcaaacttactgtataattttcagattattgttaaagcagttctgttgtccaaaaaaaatttggggtttaaggaagtatctccagaagtaaagagaatcactatatctgggaagaatctggctttatgttagagcttgctactttctggaatgttcagggagaaacaagaatttttgttcagtacaaaggaaagtacaagagagaccctcacagataatctctctgagacagtaacttcaaagagataacaatacattatcctgggagattcctggaactagggattagccctgctggcttctagccagggctgccatacatgagctcacccaggctccttggccatgagacagagttcttctaaatggtctctagaaggtcctttccagtactaggactataggaggagcatgtggcttttaataaagtgatgttgaaatgtgcctcatgattggcatgtgaaaagctaaatatgtctatgctattttcttaccaagatagctaagggggagatactattatttaacttggataatttagcaatcaaggtatagaaagagagatcatttagaatccatatataaagccagtaacaggactgggactgggagtggggtgggaaacaatcagcaaaacaagggctggtttgcttttctgacacctccaagcaatggaagtatgcattaaagagtaaaacaattaccaatttacattgtcttcattaatattgggaagaaccagcaaaatccaactgtgggaacctctaaaggataaagtgctctattcctttaacaagtatatgtcaagaaaaagttagaaagcaaatctttagatttaaaatacatttgagaaatagcaactaattgtatggaccttatgacttatgggaaaaaaacccaccaccaccccataaaacagtattacatttgagacaattagtgaacactggatatttcttatcaaggaattatggctaccttatgatgtcacaatggtattgttaaactaaaaaagagtccttagtaaaagagatatatactgtaatgtttacagatgaaaccatataattatgggatttgtttcagaataatacatgagggggagatgagtgtaaccaagggctccagcaccagctatagtagaaacagatcccaacccaagtagattcgccagtccaagactcctaccaacaattggaaaccaactgggcaaggggtttttcccaaacagcacttttaacaatctttttggaatcacagtaaagaaagcacaaagaccaagaaaaaaactctgattctggattttttttaaccctgataatttgtggtaggtttctttattttttgaatataaagtgacagaaataatttgccattagaaaagagaaagaatctttgactatttacagcttttatacatcacaaagtttttcttgtttttttatgttgtcttttttttaattcgttttaatttttgttcctgcatcatttgaacaagtccaaactggaaatctatacagctcacaaaaaagccctccacccaaaagaccccccacccccacccgaccccaatgagaaacaagataaatcaaaagaatgaaatcaacttatttcttttgtttaaaggtaagtcatttgcttatatatatacttgtaattatttttttcaagttcaaacaccaaaatccaagagagaaaggaaaaaataaaaagacccagtcatccgcccctccccccactccagaatctcaattgatccctgcatgtccaaaataagaaatagatatttacagaaaacagaagcaaaacaaataaacaaaaaaagaacttggaggtggatgggctggggatctgagagtcaagaggaaggagagccggccccagggaggagtgtggagtctgggcctcgcagagctgaggcaagcctgagtcgtcggtgctccctggagaggacatcacacaggaaagctatgaccatttcccctctgccatgtgactttgggaggggtgcagctgtgaatttgcaacgcaaccccatagtggatgcatatcatgtttccatcatcacccccttacacacgtgcgctcacacacacgctcacacacatgtgcacaggcacacacacgcatcagtcattgtggctaagtgtaattctgatgctgttggagcactggctcctgtcacgtggaggaaaagagatttcccctagggacaagagctcactgccccatcccttctctgatctccactgtaacattgcctctagctcccttgaaatgtttccacaagcgtcagggctactctgaagtattaatgctgggatagtcactgggtaacaaagctcccataaatctattccctctgctccaacaattttgcccctcacttcccacaaattcctttaacaaataggcgtacccaggttaccccattaaccaggggtgggagccagtctgaaggaggggagatctgaggcagggtaaatggaagtcacattgttttctgcacatcttccaaagagtggattccgggaggtcagaaagcaaagagaggtcatgacaaaaccatccctggcttcctttgcttccctcttccttcctaaatagagtttaatgcgtactcagtgcataaagtaaggtatgactgagttggctgtgataccttaagaactcaagatgtggcgttagatgagccaagatgaacataatttaatcttttgggggaaaacggctggcaggatatgaccatgctgaagggtttgcctttattagtggacagagaggctgaaccagcagcagcagtagttgtgatctcattcacaccctgttcagggttccgtgagggtttggaaaaatagttcactagaaatggcctaacagtttctcttctcaaattatgattttttcaggtggcacaggaaatagaattagtgcatcctctgtgtcagaaacaacgtgcagtgtctctgggggcagactctaggttgctcttgctaaatctccaaatgcctacacagtggaattttatttttctgctctccttgccaaactacttgtttttttcagaccctccccaagagtcctcacttacccccttttcatgcagccccactcagagtccttttctttctaagccctctcctgatccttgaaaacgctctctcaaggcttttaaagactttcattcatttccatgctcctgtcccactgtttctgtcacaaaagaaaatacaaaatcaaaatgatctgtcagagaaaactttcatttagcagaattgggcagaagcaaagttgctttccaatcctttttatttgattttttttttaaagatgaacaaggagtaaggtaagtaagaacaaataattatgacccccccacaacgagactagcttagttgggaaccttagaaaggacaagatttcctgtgaaaatgtgtactttccaggataaatagtcaaaatgtggtctcaatccaggataacatttgttgacatctataaaaacatgttgtggcctatcacagttagcagtggggtttttagtagaagttaaaaaagcaaatatcaggactgaggaagaggtaccagagttccatgtgctgccatcaagtccctgccccgggcacttgcagcatcaccacctcaatctgacatagagacaattagggccaaccccaaatgcccacagcctcgcttagggcaatcaccacgagaagcccaagacccccagtccctcttatcacttggactttcatccccagatacccatgcacatctcccatctcagctcatttcccttcctttaccaactcccaaatcctgcctaagaatcagtggttcatcaccagccacaaccctggcaattcctttcctcttgctcttacagaaacctggctcctctttgaggaccctgaatcactcccaggtggtgagcatttccacttgcaccttcctcatgccctggggcctggaggtggagatgcccttcttgcccctcattgccattccagaccatcctccctcctttttaaaaaaaaataacatgcaacaaccataaaatccagctttgatgcacatcagactaggctagctgcaccccttacttgatgcaatgattgaaatgttctcgaatcactctccctcattcctgtcataatttacattcctatcatatggaagtcaacattttgttgacttcaatatctatataattcccatatcctggcctctcagttccttgacccctgctccttctataaccttttcctctatcttatctcagcccaccaccccaacaacagaccccaaaccaccaataactgcaagccctccataacctcaagcatccacctctccaacccacctcctaatttctacgttattgcttctgactcactaactgagtgatcccagcttgaatctcaatcctctgcctctaatatgcttcattgttcctccttccctaaaaatcctcactttcctctacacccagcttagattccatgaccaaacattatagttaacacactgcagttgcccttgactccacatctcttgctttcattatattcacctggttataccccaaccctgttccaatctaacttgccaccctgtttaagcagctgaaggtgactgaagaaaacaaatttctttaaactcataatcataaaaactcaaataattcctttatgccccctagcatgtctcctatatttttggtgtctccgacatttttgttctcactcttcctgccggatggctatatgactcattcatgctttcttccttccaaaacctccaatactcttcccctatactcactcttaactgatgaactcctttcatagtttactaaaaatcaatcagaaaaagcatactcccattatcccatttaccagcccacttgcatctgtgcccaaatgcactatctccctgctattaatacaaacaaacctggttagtcccctgaagccagtccctctatgtttgtattgaatcccatgccctctcacttcatcaaagacattactccagcaattgtcctctctccctaggcatcatcaatttttcctttctcctggattagtcttgtcaacataaaatgggctgttatttttcccatcttaaaaaaagaagtccctccctgggcgtcacattctctatgatctgctatttccatgtcctctttacagccaaactcctaaagcgttgcctattcctgttgtctctacctcctctccttcccctctttcttgaatccaccccatcatgcttttgcccccaccagtccactgaaacagctctcttccaggtcatcaatgggatgacctccatgtttccagatagtcttatcctactcaataatagtacttgctttacccattaaccactcctcccattgctggtcccttctcatctcctggagctttgaacaatcctccaccctgggcctcagtctagagaatcctcttctgtcgctactcattctctagttccagtatcatggcttcaaataccaaccaaacgcatacaaattttaaatatgtatcttcaggctatacattttccctgaactccaggtccatatatctaattgcctaatcatcatttctacttgcaacatctgtagacaccttaaactataaggctttccttcccagtcagcctcacctgcaggattcctgtcttacactgatggcaactccaaactttcaatagctcaggccaaacattctaaggttattcttaagatttttctttctcttattcaatgtctaattcatcagcaaactgtgtgatatcgattctttaaaacatttctggaatccaactgcttcttatcacctcccctgctaacatcatggcccaagcaactatgatctcttaccaggattattgcaagagcttcctaaccggtctttcagccgcttccattgtctgccctctcagggtatactctcaacacagcagtcccaaagcttcctcttcaactgaagtcagatcatatcactctatgctccgaaccttctagcaacttctcatcttgctcttggtaaaagccaaatcctgacagtgtcctacaaggccctacctgacttgcgttattgccccctctctgacctcacctctcatactctcctcctccctcattggcctcccggctcttcctcaagtttgccaagcatttggtttgacagcagggcctttgcaattgctttctctttgcctttgcatagaaagccccaagtctcactccctcatttcctccaaacctttacttaaatgtcatctttgcttactcaaaaatagcaaccccacacccatcctatcatctatcccccttaatctgcctcatttttctgcatgacactttgcactatctgacatgagatctattgatttgcttttttgtccatttcctctcatcaacatacaaacttcaagagggtatggactttgtgtggttcgttcttatattccagcacctagaacagcctggcatgggtttccactcaataaatatcaacatggataagtcatttatccaaaacatgctctgaagccacagaccaaatatccccaaaataagagctccagtaaacaaaacaatgcaagcaaggaaacaactcctcccccaaaacctggatatttattctaagtgtttctaaattttaaccaatggcaagtgcagagctcacttttcatgatttttctggtttgagaattgtccttgggttaattattatttttaataggtaagaaaaaagttactccgagtttcattaatctatggcactttgtccctcctctcccctgcggcctaactcccaaatccccttcagctatagtgaaatacacagacgctgaatatttgggaggattacttaacgttttagctttcctggtttgcttagaacatatgatctactacccgccagtaatattttatagcttagaagatcatgtctgagtcagtaaattccatgttaatatgtgtaagactcaggattaaatcaatctgtaaaatgcctatttgtaatcgaatctagcaattttctttctgaagtaaacagtaatcacattaacaacctagtgatttcactggagatgggaagatataattttatttaacagattttctctctcagaggtgacctaactttgtgatccaaaatcattccaatattgaaaaaaaaaggttcagctaactccattcccctgatatattcagttctcagtgccccttggcttcccaatttaagtcaatgtaatcacaatgcacacaaggctcttccactcagaatcttcttgactggagaatggaaatcattggagaggggctgccctaaaggtttgtagacaaggttttgaagaatcgagctacaatgcttatcaatgtctgtctggaagaaagcctacgtctctttctaaagccagcctgtcaccatttctgagccatcaatggcagcacagcctctccttctgccagagctcacagggaatgacaaatctctgagggaatacaccagagcatctggatgtgggtgtcatcgtctcttcaccaccaaaccattctaccccaatttccctcttctttgtttctagattatttttttttcaactcagtgaagaacatttctcagaaccaagctttttgtctgcttgtcactgaatctatttcccattcaaccttctgtttctcattccaatagacacacaatattaatggttaaaaataacatgcaacaactcactgggcgagaaatttagaaacacttgcctcctatgaacccagggccaaggggagctgaggatagtgtcacattaccagcatgttcaagctagacatcctccatcacaaagggcttgtgccttgaaataaatttaaaaagagagaacaagaaaagccacaaaatacctccacatacacaacaggcatcttgaccagagcaccaggacacatgctcagaggtggcttaatattccagagcacatccctctccactaagagccactcactatcccagcacttgatcttgagttgaagcactcaggaacaagacctcatttgcctgcttgtcattctttctccaacttcctaagttaaaaaatgatgagaaaaccatgaaaaattactgtcaagggtttcttttaacagtctgatagtttagataagaatacagtttaagggatatatcccattttcataggaaaggaaagtcggggaggggagccaaaaacatgaaggggaaccaggagagctgccaggaggctgggaggtgaggaagggtttccaagtaaggagcttggaaggttgttctcaacgataaaacccactttgcagtggctaaaaatataagtattttggtctattttatattatagctgtctttccttttgtgaagcaccaaccactgaagttcattttggaatcatggccacccagaagaggaaaggggtgatcatgtgtctcaaagaagagataactttgagggagaggatgaaaactgcaaagacccttgggattaaatgaaatctgctgattctactcttttttcatgaatttctgtatgatatttagcaattagaatgtttgactggcaatggccaggtagatttcaccattatgtaacaaagagaataaaaaagaaaggaaaggagaaaacaataattggcctaggagatgggagttttgttcttggtcttagttgtctccctaggagaagcagctcttttccatccaaaggtgaacagaagactctgcagagcataatgttgctatggcttgttttactgaagtaaagacactgtaaatctcaaaaatactccaacttccctgattcttttggaagttattgggcatctgcattttcccaggagacttctctccacattgtcgcagtgttgaaactctgagataagaattccttgcccatcttctaacttccacccagatatctggcttctgtcaataggccttacccaaacagggttatgtatatgtatgtatgtatgtatgtgtgtgtatatatatatatatatatatattttttttttttttctgaaagctacagaagagaccacggagatgtgtgagctgccaaggtgccaatgatcaaatagagaagtctagcttggaaataaatcaaaaccatcagaggaattacattccacccctaggctcagtgggaaagagtttaagttcatgtggatcttgctgttccggagcaagctctgggctctaaaattgagcttatcttctctgtctttcataggatagctaagcacccatgccccctaagggatacttgaaataggaagatatctttatgttgtgtatactcggtttagtggcttcagtcttgtgcagatatagattttctttgtaagacttcctccattggccgctatggtacagctcagaaaagctgaacttttcatttctattttaatatttaatactaagtacaagagctctgtggtttcaatcaaataattctccattcatgccctcagagtccccaagaatcctgctattttcccacctcccccccccgatgaatataggtgtagcagaagacagggagtggtcatcttgggggaataagatgctccaaatactcatcagctgttggccctgtgacctgtttttcaggatcatcatgatccaggtatctgtaatgacactcatgaaaaagatgaagtcaccacggagtcaaggtagaaatagctactgcccctctctcttagcttactatgataacacgattttatgtgaattattgggaggcaaaaggacaagggaaaaatgagatttgtaataggcttgattttttttagattaaaaaattagtctagtgcccacctcctccccccatcttcatgcatgggaataaaagctacctcctccatttcctccgatcatctgaaactagcctcctgaaccaggctccggggatcagtacactctgaagttgatggtatagaagtctcctcactcattcatctaaggacttttccatcttcctacctcctctcctatcttccctctagggctaggaaggactgataaaaaaaaaaagttactctacattaagcaggacactagagctctttcactgtttttggtttaagcataatgctgtgagccaaaatttcttctgcagcccaaactaaagatactaaaatctttggaaagatggattatatcctgagcttgatatcattcataagtgaacaggtgggttgtaagagaaggttgttgcaagattctctgatctgcgggtgcttaataaataattcaccattgcaaccttgtgacaaaatcaaggtctcataagtattctcaggagactattaattttggagcccccatgcttccctttcttcaggattttggcaggcagtaattatttattatcggtctgggggctataggttctttcttcaagaattcattgtgtatgtgaactgccttatatttttctgttcagaactaacttatgccttaatcctagaatcaggcttgtatgtttgaacttaattagacagaggtgcccagaaaaggatgtaaggggctctcccttgaggctgccctgctcactgtgggctgaccaaaactactgacaccttcggagtatcatgacacccctgcacacgttcctgaaggctcttttgccatgtagcactctggaagaaatcctctgtcccagtttattcttgagttttttatttatgtggattacatgctacctaaaaaaaatttttaataataaaaaattattcacaatatcttaccctatagaattcaaaaacatttttatttgaccaagttttcttcaccgtggaaacctctctaacctttctgattttcaaatttttgctttcttcttgctctttttgacttgtctctgtagatgtatgtggagtgtgtgtgtgtctacaaagggaaatttcatagataagatctggctaaatcagctgcctagatttcgtgacttttctccactgctagatgctgaaaacctacagtgggggcagacaattcaggcagcattactcgctgagctagactgagagttagaaatttggacaagttttggttcagccaagttttggttctgtcaagaattttctgtataatcttacttttggctaattatccaattttgtgctttgacttctcatctgtaaaactgaaagatgatcttatttccaagtcaaaggaggttatttggagaagtggttatggtaaattcttctgtattcacataccaactactgtgatttactcagaatgtaccataggctaagtgtggtggagcctaatgggttgctggttatcctagaaactccaccattccccaaggaggggagcagaggcaggctagaactgcaggagctcagtgcctctttacatgggaataagctaaaaatgctcgagaaatgactcttcagatttctatgtgacccatttctcgtgcctgttaccaagaaataaccaaagtgaatgcgctgatcactgaaggtgtgcaagagtctcaggaggaattctgtcataaagaatatgtatgtatctaagcaacaggactgtctgttctcagtagaatgacttctgcttctccatcctcttagaaccaacccatcaacaggaccttatggattccatcaggtcaaataggacagttagcaggataactatgttgctctaccacaaagaaaatgctgccttcacataaagcctcttttctgtaatccaagatgtccagctatgtacagcaggccccatcctagtcattaaaatgcagtgggattgactgtgctagactgattgggctcgagtttggaaacattaagtaccatgcacgtgttcgagctctgtgctcactcaacttctcatcctaacattgtttgtgttttgaggatgggctgctcagagtcaactcaggataagtatacctcaagatgaataaattgagaaagagaagtaaagaatgcaagagatgaaaagttagtgaagggaaacacagctgtaagtgccctcattgacttctaaatgcatttatatcaaagaaagggtgattttactacttcatgtttttctcagtaagagttccacctccacctagatgcttcactatcctccttgcttcctgcctatgtgaaaccttgatatttttcttgctcctgaccctgggagagagagaacagataaattattgaatccgtgaaggcatttatccctattccttgagaatagggattctcaaggaattctcctacccttattcctcccattgagaacagacctctccacctctgctcatgatgtttccaagaagagatgtgggcacatgtgcgaatatgtatgtatctaagcaacaggactgtctgttctcagggggactggcttctgcttctccatcctcttagtaccagtccatcaacaggaccttagaaggccacatggattccatagggtaaaatgggaaaatggagacgataactaggttgtttcatcacaaagaacatgctgccttcacatgaagcctgaatatttctgtcaaaccttgagggatcaatgatccacaagccaggtagagcaaagagaaaacactggctgcataaattatgatatgtctctttatcccattctaaatgaacactttcatctaccataacatgattgacataggaaatttggatctatttgttaagattgtgtgtgtgcattagggaggtacataggcatcagaatgctcatggcaaagagatcaaattctgtgtagttgtgctgttcaggtgaatatctgagagcaaagtataaactactgagagtataactcagccagaggcaacctaatggccaggtctctggtttgcagagggttcttatgtcatggtcaaagggagcattaaaatagccatggatttcaaaagaaaatcaattacaattaaaatgtgacaatgacagttaactgcaagactgttctgaatagggctgaagttttaggcaggcatgttttgtttcatttcgaaaaaaaaacaatcccctctggaaacaggtaatatacttatcctagaggagcaggcagctcaacaaattcgcattcctgtggccccttcccctgatgctgttctcctgtcagatttcagagactatgaatctcttactgcaagggggacagatggagtcacagcctggtggcctaaattctgtgggtaagggtggtgtgataagtcactccctctgcccagggtgatgatcaagggctccttgggtgctgtaatctgaaggacctgggcaggaatgacatggggccaggttccttgtggatatcaggacctcacacataaggttgcattcaggttcctcactcatctccgctttggtccttgctctttcaagtttccctactttccgaagctatcattgaagccagtaaccaagggggaaccatgtgcctcacatgtcagcttctggctttattggtgacacaaaaggaagctccagtgtagacttcctgttcttttccttcctcatatcctccctttccttttatgggtatttgtaggcaaaataattgacatgaacagttcatggctaaaatgcctagaattttggtccatttattggcccaaatgagattcatgaacgtccttcatgaggatggctgtcttcctaccctcccaccagctgtttaccagataatttgtttcatcagctaaaaaaaaaagtctcatagtataatgaaatgggttttgctctaaaatattaactattctcattttcaggagcaaggctatctagaccccataggacttttgaaaagcaaaattatctctctagacttatattttaattttcactaggtatctcccaagttgtcacaagttttgccctaccttgccaataataattgtcctacccactcctgtctcaatgaagagtggactttcttcactttttttttaaaaaaagagacttgtcactgcctgtaacttatttgagttcagttctctatagtatgctttaaattagcacacagtggcagaagatgcctcccaaaggggaataattcatagccaatggcataatgagatttacagagaaggctggccgggagaaggaacgaaaacattatcggttaccagagcagctgaagtgaaaggacagtacgagctccaagagtttcttcagagggacagagactgacactggctagaaagaatgattgatagattgctaagtagagccaagagaggaggaggaagggttaacagggcttcaagaatacagggaccagaggataagggagggccataaggtcagaagtgatgttgtctccccctgaggtaatgaatccctttatatttacagagaaaggagtagtttagagactagcattctctctgagccagctcattcaaatcctaacttactttcattgtaaatatacagataagaggtaaagtgctcaattacctcaactcttatcctccctttgggagaagtgatcctgtagacaaagcctcagaaagggtgagaagccaaagaactcaggaaagaaatataaagacaaggtggtgaccagcacagacagttcccccaaggccacaaatgtggaagtagcgtgtggtgaaatacagtggtcctgttggaccaccacctggggtctacaaggctgtgtgattagtgagccagaactgtgacaaggttcttttggtgctgaaagtgttaaaaaagaagctaaatattggatcacagatcagtcccagcatggatcaggttattagagactcaatcttggtagtaaagtgtctggatacaagctctacccaaagcatctgaaaagctgatacctaaaatttgatcaatatccttcatagtttctccctctgtcacttacttgaacacatgtagtgttccaagtacactttcctaaccataaaacagtccaaaacaacttcaaaggacaaagcacttagaaaaaggacaaagcacttagaaaaatccagattccatttgaaataatgaactgtatacatgtagtatatacatgtgattgtgtgtgcagatatatatagagaaactggggggattcatccttaggtgctactgcagatacaaatgggcaaaataaagtgactccttctcaattataatttataataatatcaaatatttactaatgcctttcatatacaaggcactctgtttagtgctacaggagataaaaagatttaaaaatacatggccctgaacacagggagcttatgctgtagcaggagagatgagatgtataaccaaatacctatgaaataagatggcccatgatagctgccactagggagaaacaacgaaagtgttatgggcattcataaaatgcctaaaattattttctgaatggaagataaagaagttgttctggtctttgaagacttatatagagggaatggatattattcaagaagggagtgagatgggagataggaaggagagtattttggacaaagggaacagtttaagggaagacgcaagtgggaaaacaagctggtagggaaaggtgaaacaaatgttattcagcttgtctggattatgggacacacacatagtcaagtaacaagaaattattgctggcagactacggcaagtgaagcccactgaaggttgtttcttgatctgaagaatgacatctgatttatatgtaggaagtgagtactgacaagagtagattcaaatataaaatattggaacaatgctaaaagacgctgaaataatccagactagaaggaagggtctgaatgaaaaggaaagactggaaaccttagggggaagaattagtaggcttttcaaatttttagatatgcaggatgaagaaaatggaggaggcaaaagtgcctgaaaagcttgagttcggtgacggaagacatggtgataccattaagcaaaaggaggaagttggtgattatgttggtttgcagcaatggttttggatatttgagtcaagatgaagttgagtgttcagaaggtgactggaagtatgtgtatgaaggaaaagcaaaaggtaggggctaaaagtgaagatttgggattcatcttcattcaaagagttattgaaatcatagaagacagaaagattgctacagaagcattaagataaggagaagagggtcaagctcagatataccatggcaagtcaatgctaaggagataagaggaagagcaggaaccaatgaggttagaggaccagagaactaagattaaaaccagaatgtattgcctcccaatggtaattgtcaatgaggttgaagagcagggtaagtaaagaaaaaaggctattgacttttgtaacaagaacttcattggaacgttgcctgagagtagtttcagaagagtggtagggtgtagcccattgatgaagccatgagcataaggtgaggaagtggagaaagaaagactacccttttgagaagttgggaagtgaaaagatagcgataggacagaaattcaagagtcaaattggattgagagatttgtctttagagatagttgtaggacgggtgtttttgagatagttgcaggtagatgtgtggaaggaattaaagatgcaaaagagagaaatacaattggctggagagcacctcagaagaggtcagagcatagggaagaggagcacttggttgggagaaaggatggaaaagatgtgtgaaagacaagagaaatctaaaggcagagaggacagcatatgtgaggattcaataatcagattttcttgcaaacacagtaggaaagattgcctgttgaaagacaggacatgaacatgaaaggaaaataaaacaaatttatcaagcacagaatgtgacactgagtcaacattggagaaattaaaaagtccaagtgagtaggcttcaggtgaggttaaattgattgaatttgtgctcttcacgtaggtttaagacttgctcttcttggggatgcaatgaatgacaaggggatgggatgcagttagctaagcatggttggtgtagtgagatggcaagaggaaaaaggaattgccggtgagaatattgctaatgtgggtaaatacagggttagaccaaagagggaattcaatgaggcctgatggatttatggaccagaacaacagaggggtcttgaaggaaggaagatatagaaaaggcaaggttgtggttagagaggaaatcccagagttttagctctgggaggtgtaataatttcaaaagaataagtccaggcctggccatgacatgggaagctgaatctctgcaatgttttttcaaatagcataatggatatctttgactcctaccctgaaaccagaaaatattaaacttgcatgtataatcatacaaatgtatgcatacctatttatacatacatttacatattttatacttatgctttcatatattctacgtgagtacaatatactccattttgaaaccttttatatcattcacagaactagcctagggacatagtacgtgcacaatagacgttggtttaattaaactcacatatttaaccagagagcttttatttttttctcctgcatagtactagaatctgctccacctcctaaatcacaacattaaaataattaccgataaaagagttcaggtttaaagtgtggaaacctaatctttaaaataacagtttaaattgggcttagtgttgtgctttttaattgtaccttaattcttgcactgagttctttcaccttctccaaaacacagattctacacaccagagtgccaaggctctgaggaattctactcatctactctgcttttcaccttcagttctttcaggagcccttaaccacataatcaccccagcaattatattcaaagcatgaagcagctccagaaactcactgtacagagctcttgagagatgtagagagaaatgtggaagatttctaactttccctacttattcccagtactgctattctaacccattactctgaacaaaattcttttttcttgcttcaatattgtaaatgagaagccctaaacgtcacagttctctccaaggcatgaaagtagcagcactggctttcaatttaaggttttgggtgagggcctttgtcataggaatagataggctatctcttctaagtcatagagctcacagggccactgtgtgactgaatcaatgtggttggaatgagttgagggtgggatgttctcagatatcctatgattttatacaatactgcaaccccaccccccaaactagaatagaatcctagattcagatcaatattagacattctcagactgactaatctgccattttagtgtcatcccaaacatctgctaggcctaagaaacaattgccccccaggttaagtagcacctgaggtcataagtggctcttttaccagataacagggcaccccctatggaggtggaaagtataggatatagaccaactcagctaattggaagattaattaaactgggacagaaaccagacaatgacagtaaattttattgtatcactaattcaatttgatttttctagctgcctactcagtaacatgtaatggaggagaagcatcactcttctattttctatggaaagaatcatagttctcaacctgccctacaagatactgaatttagaaattcataaattatacactcatatgattgtgtattgaaaataattcctaaccaggagtcctatttaggtgtcaaatgaggcttaaataaaagcaggcggaggccaaaatatggtttaaatgtctttgccatctagaacctgtatccttgttccctactctattgctctcagtgctctctgctcccttcctcttctcttgtatcataacttattcccaggaaaaggagtgagattcctaatgtaaattaggtgattaaatgtatacatccctaatatggcttaatatgtcacctttcctgggattactttcattcgaatgacagacagctcagctcagtgctaaagcaacaaatctgtgtgggaaggtggtagttgcagtggggtgggaaatgaaaaagaccttttcaggaccttcaacacaccatggaccacatagcatacataaggccagacccatcccagtgtgactattcactttcagctgcttctcctccatgaagagctccttaaacaggaggaaaagtctctgacacccaagtgaagaaagcaaaagctctgctgtagtgtgtagcagcctactgagcatgtatttcctatatggctttgggctcagagagcacataaggtatggccacagtccctggaaatgctgaatgcattcatcaatatcactgcagtgacatcatttatgcacacatctgaatcattcctaacatacaaaaacagacattcacagggtgtcaagcaatgacagggcctttttagagagatgatgattgaaagaataaagtgagttctggaatagtttttccaaaagcttattgcccaaacaatctggttattctatctgtaaatcttgaactaactaactaaaaaccgaccaaaaaaaaaaaaaaaatgaaccaaagaaacctagttcttagtgacatgtgcaggtgaccagcactctgcagagaattctcccttgggcaactcctgatggccacggaagaccgggtgagtgatagtcacttaactgtatagacaactcctactgtatcatgtcatacatgcgtttttggcactactgacaccagcaacatttaatggaatcatttgggattttcccctcaatcacaacatggctgtggccagtgcagggaaatacatatgaaggatgtttcccaagttctggctgaggatacacagtgacagattttgaaataacaaagtccactgtacatgcatcactttgaagggtgtgcaaagtctcgactcaggcaaattcaagggtcagattattgtcagtggaaatgctgagatttaagcattgccactgaaaggagttcatacaggaccacactcaccaaccacttctgcaatggaagggaatgatagagggtacaaagcgagaaagcatggattctgaagaacatgggaatattaggtgctcctgagggtatctgcggaatctcacagttttggatggattgggtgttgtttcatacccatctgtgatatagattgggcttatagctgaattcttcctcatgcattttacttgcttgttattctggaattaagtaacatctagattttaacaatgcccagccttcctttctttaagttttcttaagcagaccatgagtaacttagtcccagtgcaaatatccagttgaagaaaagcaaccaactggggccaaataagtttagaaaaataaaattgtccagctaacagcttttatgatgggaggataggaaaaaatgtagtgaatatactgggtaaatggatttggaaattttatcctgtgatagaggctgccaacctccacaaagccaacagtctaggaaaagaagttctatttgtctggttaacccaaggccagattatgaacacctggctcgaggccagtagcaccttcctgatggcagtaatgaggacaaggcaaataaagagccgctattggcaccattgctcacatacccaccctcccacgtctaaacctaacttcagcaatcttgctaagggaatcatctcaccactgagtttctagtggatcccatcatcttttctagaaaagcatgcaaatttgtaagacacatatccagcactacctctctgtgaccagatatcacatgcttcaaaaagtagagttagtggagatttttccacgtgtgtttgccaggctgacttctgagggtggagatggggcagggagtgagtcagcgcccaggtcctaaagaagaaaagactcagatgactgagacgattgtttcagcatcagaggaggccgctgggagatttctcaggattgagcttcctgaaacctttcagtcacgccaagaatgggaagttaatttgaccttaattctgtttaagcccttttgggaatctttcctaccctaggtactgacagaggaaatatggtgccaccagcctgtctttgtgtggaatgtggtaacctagggtctacctagaagataggagtcagacctggggtttgcttagagccaaattgaaccctatgtaaaaccctggccaaagtgcatgaacatttctcacaaaccagtaagaagactggttttctgggggggatggacacaattactttcccctggctttttcaccatagtggcctccatgagcattcgctttttccagacaccctgaagcaaaaaagccatacaaaacaattcccccaatgggaaatgaaaacccataacaaaacactttttccctctcattcccatcaccaccccactccctccagcccaacaccctgaatactcacaagagaacactttatctatacaaaattagaaaacaaaatatttacatatgaaataaacaccatcttgatttctgttgccagcggagactgaaagagctcccttggttctagattgctgttcgctaggttagttggtttggtttttttgtttgaaaggggtgaggtaagaggaagatgaggggatgagtccctgacccctggacagagtcagggcgaagcagtgtttacgtggcccttcgccttcttcctcctggaggtgcctcatgccctctgtcctctctcagtcttttctgttatctaaggtaaagcactccgtgctcctctcaccaaatctgtgagaggttcagccccttgcccccatgttcattttagaaagaaaacaaagctttacaaggccttcagttggctttaaaatgaaagatactgaggtaaaaatcaaggaggagggttggggacagcagtcaagggcgggatgaggaagggtcacgagtgagggcaaacaggggcgaagagcagccctggagggagtgacttgaagagacatggcagcttccttccagaggaggatgagcacctttctggtttatgtgtcctgtgtgcaacatggcgatcctgcagtcaagcttccacacagacctggggctctctggatgccaccctgtgtaggggaggatggcaggacagtggaactgacccatagaataaatagccctaccgcaagtttcaggaccggcagtgatacatattcatttcccttctcaattttccaatgttaagtgaagggagcatcagttctgctggtaccctcatccctggagttttatacatgtatatctttttttattcctcaatggtacaatctgagagggaaacaaggtgttgcaggaaggtagaagggcttctaccaagagtgttcactctgggctcaagtcacattcccagggagccaggcccaaagaggtggtggagggtccctctctgcccccgtctcccatttccaagtctcttcccctcttttcgtacctccagagctgcactcatggagtgcagctcatttctcttaaaggtcaagctcatttctcttaactgtctgctctgtagcagttgtaatcagttttggggggaagaagcctgctcgtctagcttcaggttaagtaagaagggatcaaagcattggaaacatccccctctctcacttaccctaccatacacgactccttacttcttcaaaggtggcttcgttcttccccaaaccttggccagtcgagagtctaaatgctcaaaagagctttgtagaatcttttgctcccaagtgtgggcaaaagaatcatggctgtgaaaattcggtttccctttagccttcctggaaagttcttggttcaaactggttgaaacaattgccaaccactgaggacttgtttatgtaccttgttcttgcaggattgctcaccgcctttttttgtttagaccacagaatcttctttatcaagaattttcattctccttattccagaaggatgaagggagacacagccaaaattcaggtaatacatggccatctctgtctgtatataagccaaacaatcacactgcttggggatattgaaagaaacaatagaaagagtcaaggttgccttctcttgaggcacctgactacacatgggtgcaagtgtgcatgaacacacatgcacgcacaatccacctgctcttgtccccaaggcaccgtgggacactatcataacgtactttccagtttgttcaagaatccactctgccaccaatgaccttttgttctgttcaccaccactatcgagtctcatggggttgaagcaagcattttttggcttatatataaacacaaatggcctcccaacctctgcttggcacatgattcctagacagatgtcatctaagcagcatgaatttagccagagcctctttcctttcacaagcagtgtgctaaatggtctcacatagatgcttttgcttcctcacctaaatgaaaagatcagtttgggaaaagctacctttgtgctcacatagcctctttttggttctcccagcttcactcaaagaggatatcaaggagctcttccacaccaggaggaagcccgcatgcagcccttcctttctccgctctaccctcccctgctgagagggcccatggcatcatctcatgggaacaggaatggctgacagcggggggaagaaggagagaactgtgaaaaggaggagagatggtgctggtcaccagggttgcccccagtaggaaccagaactccaggatcccataaataaattaaaacaagaaaggagcaaatgggaaccaagttcacccccgtcaccctccgtgacatgcgcatcacgcgacccacagccttaccctcccgtacccaccttaacctctctgttccctcactcagacatcagactcaatactagaaagtttctcataaacatgcccattgctggagccattgaaagccctggggtttttgttgttaggcacacaggggttggactggttccctatacagatgtccttctggaaacgggctggcacggccccatgaagggccgagaccaccggcttgttggtgacaagggcccggaagtccggcctggctttcgacgcccccgccaccgtgggctgcctgaagaagtaggatttgctgccatggagcaagcactggtcgtccccaaaagtggggatgaaagggttttgcgtgacccggtcagggtagagcgacttgctgagcatgtacccgccgccggggttgttgtggtggtgatgtccggcagtgggcactgaggacttgttgttggcaaaggtgctctcgccagctgacatctcaaacatgtgggcgtaggggctcccatccatgaatcggcccttgtctttcaggcttacgctgcgcggggccagggcggcttcttccttctgcaggtccacgaaggtgtcgtaggagtgctgccggcgcagtttgttccggttcttcttctgggccttggaattagtcgggctctgagggtacttagtggtggaggcgtttgacgtcaccgccactggggcagccggctggtccagttcctgcagggagttgtcctcactgatgtcatacaggttgcctgctttcttgcaagcctcacaccggatgcacgcctgcctgcccgagttctgacccgtcaccgtcgtggagtagttgtgcagcttggagggacagctgcggcagaagttgcccccggaccggtcctcccactccacgttggtcaggttcttctcccaaggtgcaggtaccccgctgaccacgccgtgtttgtcgcccgtcccgtgcttgatgtgagacctgttggtacagggccctcctccgctgacggagtcgcgcttaaagtcatcactccgctccttgtagatgtcggtcaggtctacgtgctcccagtggggtgagttctcctttgttcggaactggtccaggtagaagtcccgtagcccttccttgtccctgaagtagcgcttgtggtcaggggagcggggcggtcggcgacggtaggccagctcgatctcgtcaaactccctgcgggacttggccgaggcaggccgcttcttcaggctgtccttatattgctgcttacgcctcttggcggcattgccctcgatgttcccataggtgacggtgtgggttgagatgtcagagacatcggagcggatcaagtcgtcgtggccactgtagcggtcgctcttgaaggagaatttgccgtacaggtcactgagctggctgtgcttggaggaggggaggccgatgtccaggggcttcttgctgatggacctggactgggtggtgaagggtgggttgtcacagtcgtagagcccatcgatggagctggcactgccaatactatggggccggtggtgatggtggtagtgatcttggtacacgttgctgtccttcagctgcaggttcccgaacgttctctctacctcactgatgtagtcactgaagaggttctcctcacagggcgggttgttgtaggatttgcagtcagaatgcgtgaagctgcggcggtgctctgagatgtcatagacggatgactcccgtcggatgaagtccagggcgctctgcggtgagccattcacaccagacaggttagccatgttcttggccgtgcgcagcaggcgcaggatgttggagtgtgtgttgttcatggttgcggtgggggagttcattacagactggcgctcctcgatcgccaccccatggatgcagctgtagatacctctgctgatggagaagaccatgccaggcttgccagaacagacacccataaagcaatgtcggaactgccaatagaaaaggtgttcgcagatgaaggtgatgaggctgagagccatggccgcccccaacatgtagaagacccctgccatgttgtcaatgtccagctggctgctcatgacctcattcttctcattgtgacaaatgccagtgagccagagagcttccagttcttccatctccccatctccaaagagctgcaggatagcaaggtccacctggcgcttccacccagaatctttttggatggcaatgccatagccagtggaagcaaagaccttcccactgccaatggtcaccagcttgcagccttcatctctgcctgccatatagttcagcactgctgcatcatagatgaaggcatccagtttccctgttttcagggagagcaatgcatcatctacacccctctggttgaactttcccatgtaggcatgcatttctgcatagttattgcgaatatttctctctgtgctgccgttgggcacggtcccaaagcggaaagggggtgagaagtcattaggtctctggaactttttgtcgctcaggccagaaacctggtccacatattcctcttggatcatgaaggcagctaagttggcagtgtagctggccaggaagatgacagcaaagaaggcccacactgacaccatgatcttggaggtggtcccctttgggttctgcacaggtacggagttgttaaacaccagaccccagagcaaccaaatagctttgccgatggtgaaagagggtccaccaggctctctgccatcagcgaggcacctgttataacccacagggctgaagtactcaaagacaaagacagccacggctgagacgatgagcagcatcacaaacatcatcacccatacgtcagcgctgaatggctctaagaaggcagaaggtgagacagtcccattgctgcgtgacaccatgacactgatgcctgtctctatgaagggcacagagaagtcgaccacctccgatcgttcctcattgatggtgagtgagcccactgccatgtaggccctcttcatgaccacctctccaatcataccattccaggttccattgattttcttcccatgcttgccattggtaaccaggtaaaggtcataggtgaacttcacagatttagaaattttcttaaggatgtcaatacagaaccccttgcagcattttttgatgtaacccggctcctcgtctgttttattctcagtgactatgcgtttttggcaggggactgtgttcctcatgcaggttccactcagagggtccacactttccacaatgacaaatggtgcctcctccagggtcacaatgctcagatggtcatcctcctgctcttcagtctctggacacattcggggccacacatagtacttcatctgcagggacttgtctttccacttccccaccctttcccacttcctctccttgttcagaagaattatcaccagtttcgggtgcatctggtagccatcttcactgaaggacaaattcctcccctcaaaagtgacattgatcagatacctatttagcatattggactggtagattctcttctcgtgggtgttgtaacaactgcttttgggctcagggatgaagctgtgctcagacagcatgtcagaagcagcagtggtgattatggcaattccatctctcactctggcggggaggccatagtcccattcatcatatgatacagagatgagcccagtggggaactccgcaggcactgtgtctgtatcccctgccaccagactgggcacgatccacgtgtagccatagccagtcagccctactgagttggccacttcaaagatgtaggtggcttcttccttggtacagtaaagaagaatgatggggctttgaagtttcttgagctgattctggatcttagaatctccatcgtccagggacatgtccagtaggaggacctcctctagctcccagcccacaaagctattctcaatggtgctgcggatcttgtttacaaagtcctggtagccagggaaataggtggtgacgatagaaaagatgtaccagtcatattcttccatgatgttgagcattacggaagcttgctgttcaattgatgggccaaactggaagaacatggaggattcatccttatctgccattatcatagaggagcccccgtggatgcccaggatgggggtgagagtctgtgctgaaatgaaatcgaggatctgggcgatggcttcctggtctgtgtcatcagcaaacaccaccccctggatcttccggtcagacatgagatcacagatgcgggtgatgatgctctttgggtcggtctcattcatggctaccagttccacccggggtaccacggagagatggtggaaatcatctttctcgtgggcatccttgatggccacctcgtcggaagtgcccacgaggatgacagcaatgccaatgctgggggggctcttctgagaacgagctctgctgcctgacacggccaggacggccaacaccaaccagaacttgggagaacagcactccgctctgggcttcatcttcaactcgtcgactcccttggtttgtagaagccaaacctctagacggacagattaagggagtgagcatgttgggaatgtccagtcccttcttctcgcttgcatatccacataagaaagacgaaggataaatgaacggaagataatttaaaatccaatttagcgtaaattttgttttaatcttgtgtcttgaagagatgcaaattcaaaaaaaaaaagatttaattcaaaggtaattcagggtatggagagcagctcacaatgcagaatccagagtaattattccgtgtgcatgtgaggttagtggctggaatagatttttaacgcttcttctggcaattacggtttttggtttttggagcgttagtggaggaggctctgtgtggagaagctgggggccggctccgtccctcggtggagcatggtcattcccaaagcgtccccttccggctccgagcgcctccgcggttgcagtctgcggagaggggtggccggtggctgggaatggagggttttcctttcctgcaaagcaggattaatgatccgtctcgggggttttgaagttcatgactcttctttgcaaggcaaaaggatatgcattcggacgccagcactactggatggtggtgatcaagaatcacccttgacgagcactctcgatagagcgaagccccgagatttcctagaggtgaagaagccggaggaagt

SEQ ID NO: 12296 - RNA, 29279 nt, Homo sapiens
  source 1..29279: mol_type = other RNA
ctgggaggtcaaggctgcagtgagccgtaatcatacctctccactccagcctggatgacagagcaagaccctcttaaaaaacaaacaaacaaaaaaaaaacaaacaaaaaaacaaaaacaacagaaaaatcagagccaagatttcaagtcttgtcttcccccttttttttttaaacaaatctcagattttcaaatcaaacttactgtataattttcagattattgttaaagcagttctgttgtccaaaaaaaatttggggtttaaggaagtatctccagaagtaaagagaatcactatatctgggaagaatctggctttatgttagagcttgctactttctggaatgttcagggagaaacaagaatttttgttcagtacaaaggaaagtacaagagagaccctcacagataatctctctgagacagtaacttcaaagagataacaatacattatcctgggagattcctggaactagggattagccctgctggcttctagccagggctgccatacatgagctcacccaggctccttggccatgagacagagttcttctaaatggtctctagaaggtcctttccagtactaggactataggaggagcatgtggcttttaataaagtgatgttgaaatgtgcctcatgattggcatgtgaaaagctaaatatgtctatgctattttcttaccaagatagctaagggggagatactattatttaacttggataatttagcaatcaaggtatagaaagagagatcatttagaatccatatataaagccagtaacaggactgggactgggagtggggtgggaaacaatcagcaaaacaagggctggtttgcttttctgacacctccaagcaatggaagtatgcattaaagagtaaaacaattaccaatttacattgtcttcattaatattgggaagaaccagcaaaatccaactgtgggaacctctaaaggataaagtgctctattcctttaacaagtatatgtcaagaaaaagttagaaagcaaatctttagatttaaaatacatttgagaaatagcaactaattgtatggaccttatgacttatgggaaaaaaacccaccaccaccccataaaacagtattacatttgagacaattagtgaacactggatatttcttatcaaggaattatggctaccttatgatgtcacaatggtattgttaaactaaaaaagagtccttagtaaaagagatatatactgtaatgtttacagatgaaaccatataattatgggatttgtttcagaataatacatgagggggagatgagtgtaaccaagggctccagcaccagctatagtagaaacagatcccaacccaagtagattcgccagtccaagactcctaccaacaattggaaaccaactgggcaaggggtttttcccaaacagcacttttaacaatctttttggaatcacagtaaagaaagcacaaagaccaagaaaaaaactctgattctggattttttttaaccctgataatttgtggtaggtttctttattttttgaatataaagtgacagaaataatttgccattagaaaagagaaagaatctttgactatttacagcttttatacatcacaaagtttttcttgtttttttatgttgtcttttttttaattcgttttaatttttgttcctgcatcatttgaacaagtccaaactggaaatctatacagctcacaaaaaagccctccacccaaaagaccccccacccccacccgaccccaatgagaaacaagataaatcaaaagaatgaaatcaacttatttcttttgtttaaaggtaagtcatttgcttatatatatacttgtaattatttttttcaagttcaaacaccaaaatccaagagagaaaggaaaaaataaaaagacccagtcatccgcccctccccccactccagaatctcaattgatccctgcatgtccaaaataagaaatagatatttacagaaaacagaagcaaaacaaataaacaaaaaaagaacttggaggtggatgggctggggatctgagagtcaagaggaaggagagccggccccagggaggagtgtggagtctgggcctcgcagagctgaggcaagcctgagtcgtcggtgctccctggagaggacatcacacaggaaagctatgaccatttcccctctgccatgtgactttgggaggggtgcagctgtgaatttgcaacgcaaccccatagtggatgcatatcatgtttccatcatcacccccttacacacgtgcgctcacacacacgctcacacacatgtgcacaggcacacacacgcatcagtcattgtggctaagtgtaattctgatgctgttggagcactggctcctgtcacgtggaggaaaagagatttcccctagggacaagagctcactgccccatcccttctctgatctccactgtaacattgcctctagctcccttgaaatgtttccacaagcgtcagggctactctgaagtattaatgctgggatagtcactgggtaacaaagctcccataaatctattccctctgctccaacaattttgcccctcacttcccacaaattcctttaacaaataggcgtacccaggttaccccattaaccaggggtgggagccagtctgaaggaggggagatctgaggcagggtaaatggaagtcacattgttttctgcacatcttccaaagagtggattccgggaggtcagaaagcaaagagaggtcatgacaaaaccatccctggcttcctttgcttccctcttccttcctaaatagagtttaatgcgtactcagtgcataaagtaaggtatgactgagttggctgtgataccttaagaactcaagatgtggcgttagatgagccaagatgaacataatttaatcttttgggggaaaacggctggcaggatatgaccatgctgaagggtttgcctttattagtggacagagaggctgaaccagcagcagcagtagttgtgatctcattcacaccctgttcagggttccgtgagggtttggaaaaatagttcactagaaatggcctaacagtttctcttctcaaattatgattttttcaggtggcacaggaaatagaattagtgcatcctctgtgtcagaaacaacgtgcagtgtctctgggggcagactctaggttgctcttgctaaatctccaaatgcctacacagtggaattttatttttctgctctccttgccaaactacttgtttttttcagaccctccccaagagtcctcacttacccccttttcatgcagccccactcagagtccttttctttctaagccctctcctgatccttgaaaacgctctctcaaggcttttaaagactttcattcatttccatgctcctgtcccactgtttctgtcacaaaagaaaatacaaaatcaaaatgatctgtcagagaaaactttcatttagcagaattgggcagaagcaaagttgctttccaatcctttttatttgattttttttttaaagatgaacaaggagtaaggtaagtaagaacaaataattatgacccccccacaacgagactagcttagttgggaaccttagaaaggacaagatttcctgtgaaaatgtgtactttccaggataaatagtcaaaatgtggtctcaatccaggataacatttgttgacatctataaaaacatgttgtggcctatcacagttagcagtggggtttttagtagaagttaaaaaagcaaatatcaggactgaggaagaggtaccagagttccatgtgctgccatcaagtccctgccccgggcacttgcagcatcaccacctcaatctgacatagagacaattagggccaaccccaaatgcccacagcctcgcttagggcaatcaccacgagaagcccaagacccccagtccctcttatcacttggactttcatccccagatacccatgcacatctcccatctcagctcatttcccttcctttaccaactcccaaatcctgcctaagaatcagtggttcatcaccagccacaaccctggcaattcctttcctcttgctcttacagaaacctggctcctctttgaggaccctgaatcactcccaggtggtgagcatttccacttgcaccttcctcatgccctggggcctggaggtggagatgcccttcttgcccctcattgccattccagaccatcctccctcctttttaaaaaaaaataacatgcaacaaccataaaatccagctttgatgcacatcagactaggctagctgcaccccttacttgatgcaatgattgaaatgttctcgaatcactctccctcattcctgtcataatttacattcctatcatatggaagtcaacattttgttgacttcaatatctatataattcccatatcctggcctctcagttccttgacccctgctccttctataaccttttcctctatcttatctcagcccaccaccccaacaacagaccccaaaccaccaataactgcaagccctccataacctcaagcatccacctctccaacccacctcctaatttctacgttattgcttctgactcactaactgagtgatcccagcttgaatctcaatcctctgcctctaatatgcttcattgttcctccttccctaaaaatcctcactttcctctacacccagcttagattccatgaccaaacattatagttaacacactgcagttgcccttgactccacatctcttgctttcattatattcacctggttataccccaaccctgttccaatctaacttgccaccctgtttaagcagctgaaggtgactgaagaaaacaaatttctttaaactcataatcataaaaactcaaataattcctttatgccccctagcatgtctcctatatttttggtgtctccgacatttttgttctcactcttcctgccggatggctatatgactcattcatgctttcttccttccaaaacctccaatactcttcccctatactcactcttaactgatgaactcctttcatagtttactaaaaatcaatcagaaaaagcatactcccattatcccatttaccagcccacttgcatctgtgcccaaatgcactatctccctgctattaatacaaacaaacctggttagtcccctgaagccagtccctctatgtttgtattgaatcccatgccctctcacttcatcaaagacattactccagcaattgtcctctctccctaggcatcatcaatttttcctttctcctggattagtcttgtcaacataaaatgggctgttatttttcccatcttaaaaaaagaagtccctccctgggcgtcacattctctatgatctgctatttccatgtcctctttacagccaaactcctaaagcgttgcctattcctgttgtctctacctcctctccttcccctctttcttgaatccaccccatcatgcttttgcccccaccagtccactgaaacagctctcttccaggtcatcaatgggatgacctccatgtttccagatagtcttatcctactcaataatagtacttgctttacccattaaccactcctcccattgctggtcccttctcatctcctggagctttgaacaatcctccaccctgggcctcagtctagagaatcctcttctgtcgctactcattctctagttccagtatcatggcttcaaataccaaccaaacgcatacaaattttaaatatgtatcttcaggctatacattttccctgaactccaggtccatatatctaattgcctaatcatcatttctacttgcaacatctgtagacaccttaaactataaggctttccttcccagtcagcctcacctgcaggattcctgtcttacactgatggcaactccaaactttcaatagctcaggccaaacattctaaggttattcttaagatttttctttctcttattcaatgtctaattcatcagcaaactgtgtgatatcgattctttaaaacatttctggaatccaactgcttcttatcacctcccctgctaacatcatggcccaagcaactatgatctcttaccaggattattgcaagagcttcctaaccggtctttcagccgcttccattgtctgccctctcagggtatactctcaacacagcagtcccaaagcttcctcttcaactgaagtcagatcatatcactctatgctccgaaccttctagcaacttctcatcttgctcttggtaaaagccaaatcctgacagtgtcctacaaggccctacctgacttgcgttattgccccctctctgacctcacctctcatactctcctcctccctcattggcctcccggctcttcctcaagtttgccaagcatttggtttgacagcagggcctttgcaattgctttctctttgcctttgcatagaaagccccaagtctcactccctcatttcctccaaacctttacttaaatgtcatctttgcttactcaaaaatagcaaccccacacccatcctatcatctatcccccttaatctgcctcatttttctgcatgacactttgcactatctgacatgagatctattgatttgcttttttgtccatttcctctcatcaacatacaaacttcaagagggtatggactttgtgtggttcgttcttatattccagcacctagaacagcctggcatgggtttccactcaataaatatcaacatggataagtcatttatccaaaacatgctctgaagccacagaccaaatatccccaaaataagagctccagtaaacaaaacaatgcaagcaaggaaacaactcctcccccaaaacctggatatttattctaagtgtttctaaattttaaccaatggcaagtgcagagctcacttttcatgatttttctggtttgagaattgtccttgggttaattattatttttaataggtaagaaaaaagttactccgagtttcattaatctatggcactttgtccctcctctcccctgcggcctaactcccaaatccccttcagctatagtgaaatacacagacgctgaatatttgggaggattacttaacgttttagctttcctggtttgcttagaacatatgatctactacccgccagtaatattttatagcttagaagatcatgtctgagtcagtaaattccatgttaatatgtgtaagactcaggattaaatcaatctgtaaaatgcctatttgtaatcgaatctagcaattttctttctgaagtaaacagtaatcacattaacaacctagtgatttcactggagatgggaagatataattttatttaacagattttctctctcagaggtgacctaactttgtgatccaaaatcattccaatattgaaaaaaaaaggttcagctaactccattcccctgatatattcagttctcagtgccccttggcttcccaatttaagtcaatgtaatcacaatgcacacaaggctcttccactcagaatcttcttgactggagaatggaaatcattggagaggggctgccctaaaggtttgtagacaaggttttgaagaatcgagctacaatgcttatcaatgtctgtctggaagaaagcctacgtctctttctaaagccagcctgtcaccatttctgagccatcaatggcagcacagcctctccttctgccagagctcacagggaatgacaaatctctgagggaatacaccagagcatctggatgtgggtgtcatcgtctcttcaccaccaaaccattctaccccaatttccctcttctttgtttctagattatttttttttcaactcagtgaagaacatttctcagaaccaagctttttgtctgcttgtcactgaatctatttcccattcaaccttctgtttctcattccaatagacacacaatattaatggttaaaaataacatgcaacaactcactgggcgagaaatttagaaacacttgcctcctatgaacccagggccaaggggagctgaggatagtgtcacattaccagcatgttcaagctagacatcctccatcacaaagggcttgtgccttgaaataaatttaaaaagagagaacaagaaaagccacaaaatacctccacatacacaacaggcatcttgaccagagcaccaggacacatgctcagaggtggcttaatattccagagcacatccctctccactaagagccactcactatcccagcacttgatcttgagttgaagcactcaggaacaagacctcatttgcctgcttgtcattctttctccaacttcctaagttaaaaaatgatgagaaaaccatgaaaaattactgtcaagggtttcttttaacagtctgatagtttagataagaatacagtttaagggatatatcccattttcataggaaaggaaagtcggggaggggagccaaaaacatgaaggggaaccaggagagctgccaggaggctgggaggtgaggaagggtttccaagtaaggagcttggaaggttgttctcaacgataaaacccactttgcagtggctaaaaatataagtattttggtctattttatattatagctgtctttccttttgtgaagcaccaaccactgaagttcattttggaatcatggccacccagaagaggaaaggggtgatcatgtgtctcaaagaagagataactttgagggagaggatgaaaactgcaaagacccttgggattaaatgaaatctgctgattctactcttttttcatgaatttctgtatgatatttagcaattagaatgtttgactggcaatggccaggtagatttcaccattatgtaacaaagagaataaaaaagaaaggaaaggagaaaacaataattggcctaggagatgggagttttgttcttggtcttagttgtctccctaggagaagcagctcttttccatccaaaggtgaacagaagactctgcagagcataatgttgctatggcttgttttactgaagtaaagacactgtaaatctcaaaaatactccaacttccctgattcttttggaagttattgggcatctgcattttcccaggagacttctctccacattgtcgcagtgttgaaactctgagataagaattccttgcccatcttctaacttccacccagatatctggcttctgtcaataggccttacccaaacagggttatgtatatgtatgtatgtatgtatgtgtgtgtatatatatatatatatatatattttttttttttttctgaaagctacagaagagaccacggagatgtgtgagctgccaaggtgccaatgatcaaatagagaagtctagcttggaaataaatcaaaaccatcagaggaattacattccacccctaggctcagtgggaaagagtttaagttcatgtggatcttgctgttccggagcaagctctgggctctaaaattgagcttatcttctctgtctttcataggatagctaagcacccatgccccctaagggatacttgaaataggaagatatctttatgttgtgtatactcggtttagtggcttcagtcttgtgcagatatagattttctttgtaagacttcctccattggccgctatggtacagctcagaaaagctgaacttttcatttctattttaatatttaatactaagtacaagagctctgtggtttcaatcaaataattctccattcatgccctcagagtccccaagaatcctgctattttcccacctcccccccccgatgaatataggtgtagcagaagacagggagtggtcatcttgggggaataagatgctccaaatactcatcagctgttggccctgtgacctgtttttcaggatcatcatgatccaggtatctgtaatgacactcatgaaaaagatgaagtcaccacggagtcaaggtagaaatagctactgcccctctctcttagcttactatgataacacgattttatgtgaattattgggaggcaaaaggacaagggaaaaatgagatttgtaataggcttgattttttttagattaaaaaattagtctagtgcccacctcctccccccatcttcatgcatgggaataaaagctacctcctccatttcctccgatcatctgaaactagcctcctgaaccaggctccggggatcagtacactctgaagttgatggtatagaagtctcctcactcattcatctaaggacttttccatcttcctacctcctctcctatcttccctctagggctaggaaggactgataaaaaaaaaaagttactctacattaagcaggacactagagctctttcactgtttttggtttaagcataatgctgtgagccaaaatttcttctgcagcccaaactaaagatactaaaatctttggaaagatggattatatcctgagcttgatatcattcataagtgaacaggtgggttgtaagagaaggttgttgcaagattctctgatctgcgggtgcttaataaataattcaccattgcaaccttgtgacaaaatcaaggtctcataagtattctcaggagactattaattttggagcccccatgcttccctttcttcaggattttggcaggcagtaattatttattatcggtctgggggctataggttctttcttcaagaattcattgtgtatgtgaactgccttatatttttctgttcagaactaacttatgccttaatcctagaatcaggcttgtatgtttgaacttaattagacagaggtgcccagaaaaggatgtaaggggctctcccttgaggctgccctgctcactgtgggctgaccaaaactactgacaccttcggagtatcatgacacccctgcacacgttcctgaaggctcttttgccatgtagcactctggaagaaatcctctgtcccagtttattcttgagttttttatttatgtggattacatgctacctaaaaaaaatttttaataataaaaaattattcacaatatcttaccctatagaattcaaaaacatttttatttgaccaagttttcttcaccgtggaaacctctctaacctttctgattttcaaatttttgctttcttcttgctctttttgacttgtctctgtagatgtatgtggagtgtgtgtgtgtctacaaagggaaatttcatagataagatctggctaaatcagctgcctagatttcgtgacttttctccactgctagatgctgaaaacctacagtgggggcagacaattcaggcagcattactcgctgagctagactgagagttagaaatttggacaagttttggttcagccaagttttggttctgtcaagaattttctgtataatcttacttttggctaattatccaattttgtgctttgacttctcatctgtaaaactgaaagatgatcttatttccaagtcaaaggaggttatttggagaagtggttatggtaaattcttctgtattcacataccaactactgtgatttactcagaatgtaccataggctaagtgtggtggagcctaatgggttgctggttatcctagaaactccaccattccccaaggaggggagcagaggcaggctagaactgcaggagctcagtgcctctttacatgggaataagctaaaaatgctcgagaaatgactcttcagatttctatgtgacccatttctcgtgcctgttaccaagaaataaccaaagtgaatgcgctgatcactgaaggtgtgcaagagtctcaggaggaattctgtcataaagaatatgtatgtatctaagcaacaggactgtctgttctcagtagaatgacttctgcttctccatcctcttagaaccaacccatcaacaggaccttatggattccatcaggtcaaataggacagttagcaggataactatgttgctctaccacaaagaaaatgctgccttcacataaagcctcttttctgtaatccaagatgtccagctatgtacagcaggccccatcctagtcattaaaatgcagtgggattgactgtgctagactgattgggctcgagtttggaaacattaagtaccatgcacgtgttcgagctctgtgctcactcaacttctcatcctaacattgtttgtgttttgaggatgggctgctcagagtcaactcaggataagtatacctcaagatgaataaattgagaaagagaagtaaagaatgcaagagatgaaaagttagtgaagggaaacacagctgtaagtgccctcattgacttctaaatgcatttatatcaaagaaagggtgattttactacttcatgtttttctcagtaagagttccacctccacctagatgcttcactatcctccttgcttcctgcctatgtgaaaccttgatatttttcttgctcctgaccctgggagagagagaacagataaattattgaatccgtgaaggcatttatccctattccttgagaatagggattctcaaggaattctcctacccttattcctcccattgagaacagacctctccacctctgctcatgatgtttccaagaagagatgtgggcacatgtgcgaatatgtatgtatctaagcaacaggactgtctgttctcagggggactggcttctgcttctccatcctcttagtaccagtccatcaacaggaccttagaaggccacatggattccatagggtaaaatgggaaaatggagacgataactaggttgtttcatcacaaagaacatgctgccttcacatgaagcctgaatatttctgtcaaaccttgagggatcaatgatccacaagccaggtagagcaaagagaaaacactggctgcataaattatgatatgtctctttatcccattctaaatgaacactttcatctaccataacatgattgacataggaaatttggatctatttgttaagattgtgtgtgtgcattagggaggtacataggcatcagaatgctcatggcaaagagatcaaattctgtgtagttgtgctgttcaggtgaatatctgagagcaaagtataaactactgagagtataactcagccagaggcaacctaatggccaggtctctggtttgcagagggttcttatgtcatggtcaaagggagcattaaaatagccatggatttcaaaagaaaatcaattacaattaaaatgtgacaatgacagttaactgcaagactgttctgaatagggctgaagttttaggcaggcatgttttgtttcatttcgaaaaaaaaacaatcccctctggaaacaggtaatatacttatcctagaggagcaggcagctcaacaaattcgcattcctgtggccccttcccctgatgctgttctcctgtcagatttcagagactatgaatctcttactgcaagggggacagatggagtcacagcctggtggcctaaattctgtgggtaagggtggtgtgataagtcactccctctgcccagggtgatgatcaagggctccttgggtgctgtaatctgaaggacctgggcaggaatgacatggggccaggttccttgtggatatcaggacctcacacataaggttgcattcaggttcctcactcatctccgctttggtccttgctctttcaagtttccctactttccgaagctatcattgaagccagtaaccaagggggaaccatgtgcctcacatgtcagcttctggctttattggtgacacaaaaggaagctccagtgtagacttcctgttcttttccttcctcatatcctccctttccttttatgggtatttgtaggcaaaataattgacatgaacagttcatggctaaaatgcctagaattttggtccatttattggcccaaatgagattcatgaacgtccttcatgaggatggctgtcttcctaccctcccaccagctgtttaccagataatttgtttcatcagctaaaaaaaaaagtctcatagtataatgaaatgggttttgctctaaaatattaactattctcattttcaggagcaaggctatctagaccccataggacttttgaaaagcaaaattatctctctagacttatattttaattttcactaggtatctcccaagttgtcacaagttttgccctaccttgccaataataattgtcctacccactcctgtctcaatgaagagtggactttcttcactttttttttaaaaaaagagacttgtcactgcctgtaacttatttgagttcagttctctatagtatgctttaaattagcacacagtggcagaagatgcctcccaaaggggaataattcatagccaatggcataatgagatttacagagaaggctggccgggagaaggaacgaaaacattatcggttaccagagcagctgaagtgaaaggacagtacgagctccaagagtttcttcagagggacagagactgacactggctagaaagaatgattgatagattgctaagtagagccaagagaggaggaggaagggttaacagggcttcaagaatacagggaccagaggataagggagggccataaggtcagaagtgatgttgtctccccctgaggtaatgaatccctttatatttacagagaaaggagtagtttagagactagcattctctctgagccagctcattcaaatcctaacttactttcattgtaaatatacagataagaggtaaagtgctcaattacctcaactcttatcctccctttgggagaagtgatcctgtagacaaagcctcagaaagggtgagaagccaaagaactcaggaaagaaatataaagacaaggtggtgaccagcacagacagttcccccaaggccacaaatgtggaagtagcgtgtggtgaaatacagtggtcctgttggaccaccacctggggtctacaaggctgtgtgattagtgagccagaactgtgacaaggttcttttggtgctgaaagtgttaaaaaagaagctaaatattggatcacagatcagtcccagcatggatcaggttattagagactcaatcttggtagtaaagtgtctggatacaagctctacccaaagcatctgaaaagctgatacctaaaatttgatcaatatccttcatagtttctccctctgtcacttacttgaacacatgtagtgttccaagtacactttcctaaccataaaacagtccaaaacaacttcaaaggacaaagcacttagaaaaaggacaaagcacttagaaaaatccagattccatttgaaataatgaactgtatacatgtagtatatacatgtgattgtgtgtgcagatatatatagagaaactggggggattcatccttaggtgctactgcagatacaaatgggcaaaataaagtgactccttctcaattataatttataataatatcaaatatttactaatgcctttcatatacaaggcactctgtttagtgctacaggagataaaaagatttaaaaatacatggccctgaacacagggagcttatgctgtagcaggagagatgagatgtataaccaaatacctatgaaataagatggcccatgatagctgccactagggagaaacaacgaaagtgttatgggcattcataaaatgcctaaaattattttctgaatggaagataaagaagttgttctggtctttgaagacttatatagagggaatggatattattcaagaagggagtgagatgggagataggaaggagagtattttggacaaagggaacagtttaagggaagacgcaagtgggaaaacaagctggtagggaaaggtgaaacaaatgttattcagcttgtctggattatgggacacacacatagtcaagtaacaagaaattattgctggcagactacggcaagtgaagcccactgaaggttgtttcttgatctgaagaatgacatctgatttatatgtaggaagtgagtactgacaagagtagattcaaatataaaatattggaacaatgctaaaagacgctgaaataatccagactagaaggaagggtctgaatgaaaaggaaagactggaaaccttagggggaagaattagtaggcttttcaaatttttagatatgcaggatgaagaaaatggaggaggcaaaagtgcctgaaaagcttgagttcggtgacggaagacatggtgataccattaagcaaaaggaggaagttggtgattatgttggtttgcagcaatggttttggatatttgagtcaagatgaagttgagtgttcagaaggtgactggaagtatgtgtatgaaggaaaagcaaaaggtaggggctaaaagtgaagatttgggattcatcttcattcaaagagttattgaaatcatagaagacagaaagattgctacagaagcattaagataaggagaagagggtcaagctcagatataccatggcaagtcaatgctaaggagataagaggaagagcaggaaccaatgaggttagaggaccagagaactaagattaaaaccagaatgtattgcctcccaatggtaattgtcaatgaggttgaagagcagggtaagtaaagaaaaaaggctattgacttttgtaacaagaacttcattggaacgttgcctgagagtagtttcagaagagtggtagggtgtagcccattgatgaagccatgagcataaggtgaggaagtggagaaagaaagactacccttttgagaagttgggaagtgaaaagatagcgataggacagaaattcaagagtcaaattggattgagagatttgtctttagagatagttgtaggacgggtgtttttgagatagttgcaggtagatgtgtggaaggaattaaagatgcaaaagagagaaatacaattggctggagagcacctcagaagaggtcagagcatagggaagaggagcacttggttgggagaaaggatggaaaagatgtgtgaaagacaagagaaatctaaaggcagagaggacagcatatgtgaggattcaataatcagattttcttgcaaacacagtaggaaagattgcctgttgaaagacaggacatgaacatgaaaggaaaataaaacaaatttatcaagcacagaatgtgacactgagtcaacattggagaaattaaaaagtccaagtgagtaggcttcaggtgaggttaaattgattgaatttgtgctcttcacgtaggtttaagacttgctcttcttggggatgcaatgaatgacaaggggatgggatgcagttagctaagcatggttggtgtagtgagatggcaagaggaaaaaggaattgccggtgagaatattgctaatgtgggtaaatacagggttagaccaaagagggaattcaatgaggcctgatggatttatggaccagaacaacagaggggtcttgaaggaaggaagatatagaaaaggcaaggttgtggttagagaggaaatcccagagttttagctctgggaggtgtaataatttcaaaagaataagtccaggcctggccatgacatgggaagctgaatctctgcaatgttttttcaaatagcataatggatatctttgactcctaccctgaaaccagaaaatattaaacttgcatgtataatcatacaaatgtatgcatacctatttatacatacatttacatattttatacttatgctttcatatattctacgtgagtacaatatactccattttgaaaccttttatatcattcacagaactagcctagggacatagtacgtgcacaatagacgttggtttaattaaactcacatatttaaccagagagcttttatttttttctcctgcatagtactagaatctgctccacctcctaaatcacaacattaaaataattaccgataaaagagttcaggtttaaagtgtggaaacctaatctttaaaataacagtttaaattgggcttagtgttgtgctttttaattgtaccttaattcttgcactgagttctttcaccttctccaaaacacagattctacacaccagagtgccaaggctctgaggaattctactcatctactctgcttttcaccttcagttctttcaggagcccttaaccacataatcaccccagcaattatattcaaagcatgaagcagctccagaaactcactgtacagagctcttgagagatgtagagagaaatgtggaagatttctaactttccctacttattcccagtactgctattctaacccattactctgaacaaaattcttttttcttgcttcaatattgtaaatgagaagccctaaacgtcacagttctctccaaggcatgaaagtagcagcactggctttcaatttaaggttttgggtgagggcctttgtcataggaatagataggctatctcttctaagtcatagagctcacagggccactgtgtgactgaatcaatgtggttggaatgagttgagggtgggatgttctcagatatcctatgattttatacaatactgcaaccccaccccccaaactagaatagaatcctagattcagatcaatattagacattctcagactgactaatctgccattttagtgtcatcccaaacatctgctaggcctaagaaacaattgccccccaggttaagtagcacctgaggtcataagtggctcttttaccagataacagggcaccccctatggaggtggaaagtataggatatagaccaactcagctaattggaagattaattaaactgggacagaaaccagacaatgacagtaaattttattgtatcactaattcaatttgatttttctagctgcctactcagtaacatgtaatggaggagaagcatcactcttctattttctatggaaagaatcatagttctcaacctgccctacaagatactgaatttagaaattcataaattatacactcatatgattgtgtattgaaaataattcctaaccaggagtcctatttaggtgtcaaatgaggcttaaataaaagcaggcggaggccaaaatatggtttaaatgtctttgccatctagaacctgtatccttgttccctactctattgctctcagtgctctctgctcccttcctcttctcttgtatcataacttattcccaggaaaaggagtgagattcctaatgtaaattaggtgattaaatgtatacatccctaatatggcttaatatgtcacctttcctgggattactttcattcgaatgacagacagctcagctcagtgctaaagcaacaaatctgtgtgggaaggtggtagttgcagtggggtgggaaatgaaaaagaccttttcaggaccttcaacacaccatggaccacatagcatacataaggccagacccatcccagtgtgactattcactttcagctgcttctcctccatgaagagctccttaaacaggaggaaaagtctctgacacccaagtgaagaaagcaaaagctctgctgtagtgtgtagcagcctactgagcatgtatttcctatatggctttgggctcagagagcacataaggtatggccacagtccctggaaatgctgaatgcattcatcaatatcactgcagtgacatcatttatgcacacatctgaatcattcctaacatacaaaaacagacattcacagggtgtcaagcaatgacagggcctttttagagagatgatgattgaaagaataaagtgagttctggaatagtttttccaaaagcttattgcccaaacaatctggttattctatctgtaaatcttgaactaactaactaaaaaccgaccaaaaaaaaaaaaaaaatgaaccaaagaaacctagttcttagtgacatgtgcaggtgaccagcactctgcagagaattctcccttgggcaactcctgatggccacggaagaccgggtgagtgatagtcacttaactgtatagacaactcctactgtatcatgtcatacatgcgtttttggcactactgacaccagcaacatttaatggaatcatttgggattttcccctcaatcacaacatggctgtggccagtgcagggaaatacatatgaaggatgtttcccaagttctggctgaggatacacagtgacagattttgaaataacaaagtccactgtacatgcatcactttgaagggtgtgcaaagtctcgactcaggcaaattcaagggtcagattattgtcagtggaaatgctgagatttaagcattgccactgaaaggagttcatacaggaccacactcaccaaccacttctgcaatggaagggaatgatagagggtacaaagcgagaaagcatggattctgaagaacatgggaatattaggtgctcctgagggtatctgcggaatctcacagttttggatggattgggtgttgtttcatacccatctgtgatatagattgggcttatagctgaattcttcctcatgcattttacttgcttgttattctggaattaagtaacatctagattttaacaatgcccagccttcctttctttaagttttcttaagcagaccatgagtaacttagtcccagtgcaaatatccagttgaagaaaagcaaccaactggggccaaataagtttagaaaaataaaattgtccagctaacagcttttatgatgggaggataggaaaaaatgtagtgaatatactgggtaaatggatttggaaattttatcctgtgatagaggctgccaacctccacaaagccaacagtctaggaaaagaagttctatttgtctggttaacccaaggccagattatgaacacctggctcgaggccagtagcaccttcctgatggcagtaatgaggacaaggcaaataaagagccgctattggcaccattgctcacatacccaccctcccacgtctaaacctaacttcagcaatcttgctaagggaatcatctcaccactgagtttctagtggatcccatcatcttttctagaaaagcatgcaaatttgtaagacacatatccagcactacctctctgtgaccagatatcacatgcttcaaaaagtagagttagtggagatttttccacgtgtgtttgccaggctgacttctgagggtggagatggggcagggagtgagtcagcgcccaggtcctaaagaagaaaagactcagatgactgagacgattgtttcagcatcagaggaggccgctgggagatttctcaggattgagcttcctgaaacctttcagtcacgccaagaatgggaagttaatttgaccttaattctgtttaagcccttttgggaatctttcctaccctaggtactgacagaggaaatatggtgccaccagcctgtctttgtgtggaatgtggtaacctagggtctacctagaagataggagtcagacctggggtttgcttagagccaaattgaaccctatgtaaaaccctggccaaagtgcatgaacatttctcacaaaccagtaagaagactggttttctgggggggatggacacaattactttcccctggctttttcaccatagtggcctccatgagcattcgctttttccagacaccctgaagcaaaaaagccatacaaaacaattcccccaatgggaaatgaaaacccataacaaaacactttttccctctcattcccatcaccaccccactccctccagcccaacaccctgaatactcacaagagaacactttatctatacaaaattagaaaacaaaatatttacatatgaaataaacaccatcttgatttctgttgccagcggagactgaaagagctcccttggttctagattgctgttcgctaggttagttggtttggtttttttgtttgaaaggggtgaggtaagaggaagatgaggggatgagtccctgacccctggacagagtcagggcgaagcagtgtttacgtggcccttcgccttcttcctcctggaggtgcctcatgccctctgtcctctctcagtcttttctgttatctaaggtaaagcactccgtgctcctctcaccaaatctgtgagaggttcagccccttgcccccatgttcattttagaaagaaaacaaagctttacaaggccttcagttggctttaaaatgaaagatactgaggtaaaaatcaaggaggagggttggggacagcagtcaagggcgggatgaggaagggtcacgagtgagggcaaacaggggcgaagagcagccctggagggagtgacttgaagagacatggcagcttccttccagaggaggatgagcacctttctggtttatgtgtcctgtgtgcaacatggcgatcctgcagtcaagcttccacacagacctggggctctctggatgccaccctgtgtaggggaggatggcaggacagtggaactgacccatagaataaatagccctaccgcaagtttcaggaccggcagtgatacatattcatttcccttctcaattttccaatgttaagtgaagggagcatcagttctgctggtaccctcatccctggagttttatacatgtatatctttttttattcctcaatggtacaatctgagagggaaacaaggtgttgcaggaaggtagaagggcttctaccaagagtgttcactctgggctcaagtcacattcccagggagccaggcccaaagaggtggtggagggtccctctctgcccccgtctcccatttccaagtctcttcccctcttttcgtacctccagagctgcactcatggagtgcagctcatttctcttaaaggtcaagctcatttctcttaactgtctgctctgtagcagttgtaatcagttttggggggaagaagcctgctcgtctagcttcaggttaagtaagaagggatcaaagcattggaaacatccccctctctcacttaccctaccatacacgactccttacttcttcaaaggtggcttcgttcttccccaaaccttggccagtcgagagtctaaatgctcaaaagagctttgtagaatcttttgctcccaagtgtgggcaaaagaatcatggctgtgaaaattcggtttccctttagccttcctggaaagttcttggttcaaactggttgaaacaattgccaaccactgaggacttgtttatgtaccttgttcttgcaggattgctcaccgcctttttttgtttagaccacagaatcttctttatcaagaattttcattctccttattccagaaggatgaagggagacacagccaaaattcaggtaatacatggccatctctgtctgtatataagccaaacaatcacactgcttggggatattgaaagaaacaatagaaagagtcaaggttgccttctcttgaggcacctgactacacatgggtgcaagtgtgcatgaacacacatgcacgcacaatccacctgctcttgtccccaaggcaccgtgggacactatcataacgtactttccagtttgttcaagaatccactctgccaccaatgaccttttgttctgttcaccaccactatcgagtctcatggggttgaagcaagcattttttggcttatatataaacacaaatggcctcccaacctctgcttggcacatgattcctagacagatgtcatctaagcagcatgaatttagccagagcctctttcctttcacaagcagtgtgctaaatggtctcacatagatgcttttgcttcctcacctaaatgaaaagatcagtttgggaaaagctacctttgtgctcacatagcctctttttggttctcccagcttcactcaaagaggatatcaaggagctcttccacaccaggaggaagcccgcatgcagcccttcctttctccgctctaccctcccctgctgagagggcccatggcatcatctcatgggaacaggaatggctgacagcggggggaagaaggagagaactgtgaaaaggaggagagatggtgctggtcaccagggttgcccccagtaggaaccagaactccaggatcccataaataaattaaaacaagaaaggagcaaatgggaaccaagttcacccccgtcaccctccgtgacatgcgcatcacgcgacccacagccttaccctcccgtacccaccttaacctctctgttccctcactcagacatcagactcaatactagaaagtttctcataaacatgcccattgctggagccattgaaagccctggggtttttgttgttaggcacacaggggttggactggttccctatacagatgtccttctggaaacgggctggcacggccccatgaagggccgagaccaccggcttgttggtgacaagggcccggaagtccggcctggctttcgacgcccccgccaccgtgggctgcctgaagaagtaggatttgctgccatggagcaagcactggtcgtccccaaaagtggggatgaaagggttttgcgtgacccggtcagggtagagcgacttgctgagcatgtacccgccgccggggttgttgtggtggtgatgtccggcagtgggcactgaggacttgttgttggcaaaggtgctctcgccagctgacatctcaaacatgtgggcgtaggggctcccatccatgaatcggcccttgtctttcaggcttacgctgcgcggggccagggcggcttcttccttctgcaggtccacgaaggtgtcgtaggagtgctgccggcgcagtttgttccggttcttcttctgggccttggaattagtcgggctctgagggtacttagtggtggaggcgtttgacgtcaccgccactggggcagccggctggtccagttcctgcagggagttgtcctcactgatgtcatacaggttgcctgctttcttgcaagcctcacaccggatgcacgcctgcctgcccgagttctgacccgtcaccgtcgtggagtagttgtgcagcttggagggacagctgcggcagaagttgcccccggaccggtcctcccactccacgttggtcaggttcttctcccaaggtgcaggtaccccgctgaccacgccgtgtttgtcgcccgtcccgtgcttgatgtgagacctgttggtacagggccctcctccgctgacggagtcgcgcttaaagtcatcactccgctccttgtagatgtcggtcaggtctacgtgctcccagtggggtgagttctcctttgttcggaactggtccaggtagaagtcccgtagcccttccttgtccctgaagtagcgcttgtggtcaggggagcggggcggtcggcgacggtaggccagctcgatctcgtcaaactccctgcgggacttggccgaggcaggccgcttcttcaggctgtccttatattgctgcttacgcctcttggcggcattgccctcgatgttcccataggtgacggtgtgggttgagatgtcagagacatcggagcggatcaagtcgtcgtggccactgtagcggtcgctcttgaaggagaatttgccgtacaggtcactgagctggctgtgcttggaggaggggaggccgatgtccaggggcttcttgctgatggacctggactgggtggtgaagggtgggttgtcacagtcgtagagcccatcgatggagctggcactgccaatactatggggccggtggtgatggtggtagtgatcttggtacacgttgctgtccttcagctgcaggttcccgaacgttctctctacctcactgatgtagtcactgaagaggttctcctcacagggcgggttgttgtaggatttgcagtcagaatgcgtgaagctgcggcggtgctctgagatgtcatagacggatgactcccgtcggatgaagtccagggcgctctgcggtgagccattcacaccagacaggttagccatgttcttggccgtgcgcagcaggcgcaggatgttggagtgtgtgttgttcatggttgcggtgggggagttcattacagactggcgctcctcgatcgccaccccatggatgcagctgtagatacctctgctgatggagaagaccatgccaggcttgccagaacagacacccataaagcaatgtcggaactgccaatagaaaaggtgttcgcagatgaaggtgatgaggctgagagccatggccgcccccaacatgtagaagacccctgccatgttgtcaatgtccagctggctgctcatgacctcattcttctcattgtgacaaatgccagtgagccagagagcttccagttcttccatctccccatctccaaagagctgcaggatagcaaggtccacctggcgcttccacccagaatctttttggatggcaatgccatagccagtggaagcaaagaccttcccactgccaatggtcaccagcttgcagccttcatctctgcctgccatatagttcagcactgctgcatcatagatgaaggcatccagtttccctgttttcagggagagcaatgcatcatctacacccctctggttgaactttcccatgtaggcatgcatttctgcatagttattgcgaatatttctctctgtgctgccgttgggcacggtcccaaagcggaaagggggtgagaagtcattaggtctctggaactttttgtcgctcaggccagaaacctggtccacatattcctcttggatcatgaaggcagctaagttggcagtgtagctggccaggaagatgacagcaaagaaggcccacactgacaccatgatcttggaggtggtcccctttgggttctgcacaggtacggagttgttaaacaccagaccccagagcaaccaaatagctttgccgatggtgaaagagggtccaccaggctctctgccatcagcgaggcacctgttataacccacagggctgaagtactcaaagacaaagacagccacggctgagacgatgagcagcatcacaaacatcatcacccatacgtcagcgctgaatggctctaagaaggcagaaggtgagacagtcccattgctgcgtgacaccatgacactgatgcctgtctctatgaagggcacagagaagtcgaccacctccgatcgttcctcattgatggtgagtgagcccactgccatgtaggccctcttcatgaccacctctccaatcataccattccaggttccattgattttcttcccatgcttgccattggtaaccaggtaaaggtcataggtgaacttcacagatttagaaattttcttaaggatgtcaatacagaaccccttgcagcattttttgatgtaacccggctcctcgtctgttttattctcagtgactatgcgtttttggcaggggactgtgttcctcatgcaggttccactcagagggtccacactttccacaatgacaaatggtgcctcctccagggtcacaatgctcagatggtcatcctcctgctcttcagtctctggacacattcggggccacacatagtacttcatctgcagggacttgtctttccacttccccaccctttcccacttcctctccttgttcagaagaattatcaccagtttcgggtgcatctggtagccatcttcactgaaggacaaattcctcccctcaaaagtgacattgatcagatacctatttagcatattggactggtagattctcttctcgtgggtgttgtaacaactgcttttgggctcagggatgaagctgtgctcagacagcatgtcagaagcagcagtggtgattatggcaattccatctctcactctggcggggaggccatagtcccattcatcatatgatacagagatgagcccagtggggaactccgcaggcactgtgtctgtatcccctgccaccagactgggcacgatccacgtgtagccatagccagtcagccctactgagttggccacttcaaagatgtaggtggcttcttccttggtacagtaaagaagaatgatggggctttgaagtttcttgagctgattctggatcttagaatctccatcgtccagggacatgtccagtaggaggacctcctctagctcccagcccacaaagctattctcaatggtgctgcggatcttgtttacaaagtcctggtagccagggaaataggtggtgacgatagaaaagatgtaccagtcatattcttccatgatgttgagcattacggaagcttgctgttcaattgatgggccaaactggaagaacatggaggattcatccttatctgccattatcatagaggagcccccgtggatgcccaggatgggggtgagagtctgtgctgaaatgaaatcgaggatctgggcgatggcttcctggtctgtgtcatcagcaaacaccaccccctggatcttccggtcagacatgagatcacagatgcgggtgatgatgctctttgggtcggtctcattcatggctaccagttccacccggggtaccacggagagatggtggaaatcatctttctcgtgggcatccttgatggccacctcgtcggaagtgcccacgaggatgacagcaatgccaatgctgggggggctcttctgagaacgagctctgctgcctgacacggccaggacggccaacaccaaccagaacttgggagaacagcactccgctctgggcttcatcttcaactcgtcgactcccttggtttgtagaagccaaacctctagacggacagattaagggagtgagcatgttgggaatgtccagtcccttcttctcgcttgcatatccacataagaaagacgaaggataaatgaacggaagataatttaaaatccaatttagcgtaaattttgttttaatcttgtgtcttgaagagatgcaaattcaaaaaaaaaaagatttaattcaaaggtaattcagggtatggagagcagctcacaatgcagaatccagagtaattattccgtgtgcatgtgaggttagtggctggaatagatttttaacgcttcttctggcaattacggtttttggtttttggagcgttagtggaggaggctctgtgtggagaagctgggggccggctccgtccctcggtggagcatggtcattcccaaagcgtccccttccggctccgagcgcctccgcggttgcagtctgcggagaggggtggccggtggctgggaatggagggttttcctttcctgcaaagcaggattaatgatccgtctcgggggttttgaagttcatgactcttctttgcaaggcaaaaggatatgcattcggacgccagcactactggatggtggtgatcaagaatcacccttgacgagcactctcgatagagcgaagccccgagatttcctcgcacaccctgactccggggggaggagaaacccacgaagctggggaagatactgcttctgctcccaggggcgggtgtgagcgcgcgtgtcctctt

SEQ ID NO: 12297 - RNA, 29028 nt, Homo sapiens
  source 1..29028: mol_type = other RNA
ctgggaggtcaaggctgcagtgagccgtaatcatacctctccactccagcctggatgacagagcaagaccctcttaaaaaacaaacaaacaaaaaaaaaacaaacaaaaaaacaaaaacaacagaaaaatcagagccaagatttcaagtcttgtcttcccccttttttttttaaacaaatctcagattttcaaatcaaacttactgtataattttcagattattgttaaagcagttctgttgtccaaaaaaaatttggggtttaaggaagtatctccagaagtaaagagaatcactatatctgggaagaatctggctttatgttagagcttgctactttctggaatgttcagggagaaacaagaatttttgttcagtacaaaggaaagtacaagagagaccctcacagataatctctctgagacagtaacttcaaagagataacaatacattatcctgggagattcctggaactagggattagccctgctggcttctagccagggctgccatacatgagctcacccaggctccttggccatgagacagagttcttctaaatggtctctagaaggtcctttccagtactaggactataggaggagcatgtggcttttaataaagtgatgttgaaatgtgcctcatgattggcatgtgaaaagctaaatatgtctatgctattttcttaccaagatagctaagggggagatactattatttaacttggataatttagcaatcaaggtatagaaagagagatcatttagaatccatatataaagccagtaacaggactgggactgggagtggggtgggaaacaatcagcaaaacaagggctggtttgcttttctgacacctccaagcaatggaagtatgcattaaagagtaaaacaattaccaatttacattgtcttcattaatattgggaagaaccagcaaaatccaactgtgggaacctctaaaggataaagtgctctattcctttaacaagtatatgtcaagaaaaagttagaaagcaaatctttagatttaaaatacatttgagaaatagcaactaattgtatggaccttatgacttatgggaaaaaaacccaccaccaccccataaaacagtattacatttgagacaattagtgaacactggatatttcttatcaaggaattatggctaccttatgatgtcacaatggtattgttaaactaaaaaagagtccttagtaaaagagatatatactgtaatgtttacagatgaaaccatataattatgggatttgtttcagaataatacatgagggggagatgagtgtaaccaagggctccagcaccagctatagtagaaacagatcccaacccaagtagattcgccagtccaagactcctaccaacaattggaaaccaactgggcaaggggtttttcccaaacagcacttttaacaatctttttggaatcacagtaaagaaagcacaaagaccaagaaaaaaactctgattctggattttttttaaccctgataatttgtggtaggtttctttattttttgaatataaagtgacagaaataatttgccattagaaaagagaaagaatctttgactatttacagcttttatacatcacaaagtttttcttgtttttttatgttgtcttttttttaattcgttttaatttttgttcctgcatcatttgaacaagtccaaactggaaatctatacagctcacaaaaaagccctccacccaaaagaccccccacccccacccgaccccaatgagaaacaagataaatcaaaagaatgaaatcaacttatttcttttgtttaaaggtaagtcatttgcttatatatatacttgtaattatttttttcaagttcaaacaccaaaatccaagagagaaaggaaaaaataaaaagacccagtcatccgcccctccccccactccagaatctcaattgatccctgcatgtccaaaataagaaatagatatttacagaaaacagaagcaaaacaaataaacaaaaaaagaacttggaggtggatgggctggggatctgagagtcaagaggaaggagagccggccccagggaggagtgtggagtctgggcctcgcagagctgaggcaagcctgagtcgtcggtgctccctggagaggacatcacacaggaaagctatgaccatttcccctctgccatgtgactttgggaggggtgcagctgtgaatttgcaacgcaaccccatagtggatgcatatcatgtttccatcatcacccccttacacacgtgcgctcacacacacgctcacacacatgtgcacaggcacacacacgcatcagtcattgtggctaagtgtaattctgatgctgttggagcactggctcctgtcacgtggaggaaaagagatttcccctagggacaagagctcactgccccatcccttctctgatctccactgtaacattgcctctagctcccttgaaatgtttccacaagcgtcagggctactctgaagtattaatgctgggatagtcactgggtaacaaagctcccataaatctattccctctgctccaacaattttgcccctcacttcccacaaattcctttaacaaataggcgtacccaggttaccccattaaccaggggtgggagccagtctgaaggaggggagatctgaggcagggtaaatggaagtcacattgttttctgcacatcttccaaagagtggattccgggaggtcagaaagcaaagagaggtcatgacaaaaccatccctggcttcctttgcttccctcttccttcctaaatagagtttaatgcgtactcagtgcataaagtaaggtatgactgagttggctgtgataccttaagaactcaagatgtggcgttagatgagccaagatgaacataatttaatcttttgggggaaaacggctggcaggatatgaccatgctgaagggtttgcctttattagtggacagagaggctgaaccagcagcagcagtagttgtgatctcattcacaccctgttcagggttccgtgagggtttggaaaaatagttcactagaaatggcctaacagtttctcttctcaaattatgattttttcaggtggcacaggaaatagaattagtgcatcctctgtgtcagaaacaacgtgcagtgtctctgggggcagactctaggttgctcttgctaaatctccaaatgcctacacagtggaattttatttttctgctctccttgccaaactacttgtttttttcagaccctccccaagagtcctcacttacccccttttcatgcagccccactcagagtccttttctttctaagccctctcctgatccttgaaaacgctctctcaaggcttttaaagactttcattcatttccatgctcctgtcccactgtttctgtcacaaaagaaaatacaaaatcaaaatgatctgtcagagaaaactttcatttagcagaattgggcagaagcaaagttgctttccaatcctttttatttgattttttttttaaagatgaacaaggagtaaggtaagtaagaacaaataattatgacccccccacaacgagactagcttagttgggaaccttagaaaggacaagatttcctgtgaaaatgtgtactttccaggataaatagtcaaaatgtggtctcaatccaggataacatttgttgacatctataaaaacatgttgtggcctatcacagttagcagtggggtttttagtagaagttaaaaaagcaaatatcaggactgaggaagaggtaccagagttccatgtgctgccatcaagtccctgccccgggcacttgcagcatcaccacctcaatctgacatagagacaattagggccaaccccaaatgcccacagcctcgcttagggcaatcaccacgagaagcccaagacccccagtccctcttatcacttggactttcatccccagatacccatgcacatctcccatctcagctcatttcccttcctttaccaactcccaaatcctgcctaagaatcagtggttcatcaccagccacaaccctggcaattcctttcctcttgctcttacagaaacctggctcctctttgaggaccctgaatcactcccaggtggtgagcatttccacttgcaccttcctcatgccctggggcctggaggtggagatgcccttcttgcccctcattgccattccagaccatcctccctcctttttaaaaaaaaataacatgcaacaaccataaaatccagctttgatgcacatcagactaggctagctgcaccccttacttgatgcaatgattgaaatgttctcgaatcactctccctcattcctgtcataatttacattcctatcatatggaagtcaacattttgttgacttcaatatctatataattcccatatcctggcctctcagttccttgacccctgctccttctataaccttttcctctatcttatctcagcccaccaccccaacaacagaccccaaaccaccaataactgcaagccctccataacctcaagcatccacctctccaacccacctcctaatttctacgttattgcttctgactcactaactgagtgatcccagcttgaatctcaatcctctgcctctaatatgcttcattgttcctccttccctaaaaatcctcactttcctctacacccagcttagattccatgaccaaacattatagttaacacactgcagttgcccttgactccacatctcttgctttcattatattcacctggttataccccaaccctgttccaatctaacttgccaccctgtttaagcagctgaaggtgactgaagaaaacaaatttctttaaactcataatcataaaaactcaaataattcctttatgccccctagcatgtctcctatatttttggtgtctccgacatttttgttctcactcttcctgccggatggctatatgactcattcatgctttcttccttccaaaacctccaatactcttcccctatactcactcttaactgatgaactcctttcatagtttactaaaaatcaatcagaaaaagcatactcccattatcccatttaccagcccacttgcatctgtgcccaaatgcactatctccctgctattaatacaaacaaacctggttagtcccctgaagccagtccctctatgtttgtattgaatcccatgccctctcacttcatcaaagacattactccagcaattgtcctctctccctaggcatcatcaatttttcctttctcctggattagtcttgtcaacataaaatgggctgttatttttcccatcttaaaaaaagaagtccctccctgggcgtcacattctctatgatctgctatttccatgtcctctttacagccaaactcctaaagcgttgcctattcctgttgtctctacctcctctccttcccctctttcttgaatccaccccatcatgcttttgcccccaccagtccactgaaacagctctcttccaggtcatcaatgggatgacctccatgtttccagatagtcttatcctactcaataatagtacttgctttacccattaaccactcctcccattgctggtcccttctcatctcctggagctttgaacaatcctccaccctgggcctcagtctagagaatcctcttctgtcgctactcattctctagttccagtatcatggcttcaaataccaaccaaacgcatacaaattttaaatatgtatcttcaggctatacattttccctgaactccaggtccatatatctaattgcctaatcatcatttctacttgcaacatctgtagacaccttaaactataaggctttccttcccagtcagcctcacctgcaggattcctgtcttacactgatggcaactccaaactttcaatagctcaggccaaacattctaaggttattcttaagatttttctttctcttattcaatgtctaattcatcagcaaactgtgtgatatcgattctttaaaacatttctggaatccaactgcttcttatcacctcccctgctaacatcatggcccaagcaactatgatctcttaccaggattattgcaagagcttcctaaccggtctttcagccgcttccattgtctgccctctcagggtatactctcaacacagcagtcccaaagcttcctcttcaactgaagtcagatcatatcactctatgctccgaaccttctagcaacttctcatcttgctcttggtaaaagccaaatcctgacagtgtcctacaaggccctacctgacttgcgttattgccccctctctgacctcacctctcatactctcctcctccctcattggcctcccggctcttcctcaagtttgccaagcatttggtttgacagcagggcctttgcaattgctttctctttgcctttgcatagaaagccccaagtctcactccctcatttcctccaaacctttacttaaatgtcatctttgcttactcaaaaatagcaaccccacacccatcctatcatctatcccccttaatctgcctcatttttctgcatgacactttgcactatctgacatgagatctattgatttgcttttttgtccatttcctctcatcaacatacaaacttcaagagggtatggactttgtgtggttcgttcttatattccagcacctagaacagcctggcatgggtttccactcaataaatatcaacatggataagtcatttatccaaaacatgctctgaagccacagaccaaatatccccaaaataagagctccagtaaacaaaacaatgcaagcaaggaaacaactcctcccccaaaacctggatatttattctaagtgtttctaaattttaaccaatggcaagtgcagagctcacttttcatgatttttctggtttgagaattgtccttgggttaattattatttttaataggtaagaaaaaagttactccgagtttcattaatctatggcactttgtccctcctctcccctgcggcctaactcccaaatccccttcagctatagtgaaatacacagacgctgaatatttgggaggattacttaacgttttagctttcctggtttgcttagaacatatgatctactacccgccagtaatattttatagcttagaagatcatgtctgagtcagtaaattccatgttaatatgtgtaagactcaggattaaatcaatctgtaaaatgcctatttgtaatcgaatctagcaattttctttctgaagtaaacagtaatcacattaacaacctagtgatttcactggagatgggaagatataattttatttaacagattttctctctcagaggtgacctaactttgtgatccaaaatcattccaatattgaaaaaaaaaggttcagctaactccattcccctgatatattcagttctcagtgccccttggcttcccaatttaagtcaatgtaatcacaatgcacacaaggctcttccactcagaatcttcttgactggagaatggaaatcattggagaggggctgccctaaaggtttgtagacaaggttttgaagaatcgagctacaatgcttatcaatgtctgtctggaagaaagcctacgtctctttctaaagccagcctgtcaccatttctgagccatcaatggcagcacagcctctccttctgccagagctcacagggaatgacaaatctctgagggaatacaccagagcatctggatgtgggtgtcatcgtctcttcaccaccaaaccattctaccccaatttccctcttctttgtttctagattatttttttttcaactcagtgaagaacatttctcagaaccaagctttttgtctgcttgtcactgaatctatttcccattcaaccttctgtttctcattccaatagacacacaatattaatggttaaaaataacatgcaacaactcactgggcgagaaatttagaaacacttgcctcctatgaacccagggccaaggggagctgaggatagtgtcacattaccagcatgttcaagctagacatcctccatcacaaagggcttgtgccttgaaataaatttaaaaagagagaacaagaaaagccacaaaatacctccacatacacaacaggcatcttgaccagagcaccaggacacatgctcagaggtggcttaatattccagagcacatccctctccactaagagccactcactatcccagcacttgatcttgagttgaagcactcaggaacaagacctcatttgcctgcttgtcattctttctccaacttcctaagttaaaaaatgatgagaaaaccatgaaaaattactgtcaagggtttcttttaacagtctgatagtttagataagaatacagtttaagggatatatcccattttcataggaaaggaaagtcggggaggggagccaaaaacatgaaggggaaccaggagagctgccaggaggctgggaggtgaggaagggtttccaagtaaggagcttggaaggttgttctcaacgataaaacccactttgcagtggctaaaaatataagtattttggtctattttatattatagctgtctttccttttgtgaagcaccaaccactgaagttcattttggaatcatggccacccagaagaggaaaggggtgatcatgtgtctcaaagaagagataactttgagggagaggatgaaaactgcaaagacccttgggattaaatgaaatctgctgattctactcttttttcatgaatttctgtatgatatttagcaattagaatgtttgactggcaatggccaggtagatttcaccattatgtaacaaagagaataaaaaagaaaggaaaggagaaaacaataattggcctaggagatgggagttttgttcttggtcttagttgtctccctaggagaagcagctcttttccatccaaaggtgaacagaagactctgcagagcataatgttgctatggcttgttttactgaagtaaagacactgtaaatctcaaaaatactccaacttccctgattcttttggaagttattgggcatctgcattttcccaggagacttctctccacattgtcgcagtgttgaaactctgagataagaattccttgcccatcttctaacttccacccagatatctggcttctgtcaataggccttacccaaacagggttatgtatatgtatgtatgtatgtatgtgtgtgtatatatatatatatatatatattttttttttttttctgaaagctacagaagagaccacggagatgtgtgagctgccaaggtgccaatgatcaaatagagaagtctagcttggaaataaatcaaaaccatcagaggaattacattccacccctaggctcagtgggaaagagtttaagttcatgtggatcttgctgttccggagcaagctctgggctctaaaattgagcttatcttctctgtctttcataggatagctaagcacccatgccccctaagggatacttgaaataggaagatatctttatgttgtgtatactcggtttagtggcttcagtcttgtgcagatatagattttctttgtaagacttcctccattggccgctatggtacagctcagaaaagctgaacttttcatttctattttaatatttaatactaagtacaagagctctgtggtttcaatcaaataattctccattcatgccctcagagtccccaagaatcctgctattttcccacctcccccccccgatgaatataggtgtagcagaagacagggagtggtcatcttgggggaataagatgctccaaatactcatcagctgttggccctgtgacctgtttttcaggatcatcatgatccaggtatctgtaatgacactcatgaaaaagatgaagtcaccacggagtcaaggtagaaatagctactgcccctctctcttagcttactatgataacacgattttatgtgaattattgggaggcaaaaggacaagggaaaaatgagatttgtaataggcttgattttttttagattaaaaaattagtctagtgcccacctcctccccccatcttcatgcatgggaataaaagctacctcctccatttcctccgatcatctgaaactagcctcctgaaccaggctccggggatcagtacactctgaagttgatggtatagaagtctcctcactcattcatctaaggacttttccatcttcctacctcctctcctatcttccctctagggctaggaaggactgataaaaaaaaaaagttactctacattaagcaggacactagagctctttcactgtttttggtttaagcataatgctgtgagccaaaatttcttctgcagcccaaactaaagatactaaaatctttggaaagatggattatatcctgagcttgatatcattcataagtgaacaggtgggttgtaagagaaggttgttgcaagattctctgatctgcgggtgcttaataaataattcaccattgcaaccttgtgacaaaatcaaggtctcataagtattctcaggagactattaattttggagcccccatgcttccctttcttcaggattttggcaggcagtaattatttattatcggtctgggggctataggttctttcttcaagaattcattgtgtatgtgaactgccttatatttttctgttcagaactaacttatgccttaatcctagaatcaggcttgtatgtttgaacttaattagacagaggtgcccagaaaaggatgtaaggggctctcccttgaggctgccctgctcactgtgggctgaccaaaactactgacaccttcggagtatcatgacacccctgcacacgttcctgaaggctcttttgccatgtagcactctggaagaaatcctctgtcccagtttattcttgagttttttatttatgtggattacatgctacctaaaaaaaatttttaataataaaaaattattcacaatatcttaccctatagaattcaaaaacatttttatttgaccaagttttcttcaccgtggaaacctctctaacctttctgattttcaaatttttgctttcttcttgctctttttgacttgtctctgtagatgtatgtggagtgtgtgtgtgtctacaaagggaaatttcatagataagatctggctaaatcagctgcctagatttcgtgacttttctccactgctagatgctgaaaacctacagtgggggcagacaattcaggcagcattactcgctgagctagactgagagttagaaatttggacaagttttggttcagccaagttttggttctgtcaagaattttctgtataatcttacttttggctaattatccaattttgtgctttgacttctcatctgtaaaactgaaagatgatcttatttccaagtcaaaggaggttatttggagaagtggttatggtaaattcttctgtattcacataccaactactgtgatttactcagaatgtaccataggctaagtgtggtggagcctaatgggttgctggttatcctagaaactccaccattccccaaggaggggagcagaggcaggctagaactgcaggagctcagtgcctctttacatgggaataagctaaaaatgctcgagaaatgactcttcagatttctatgtgacccatttctcgtgcctgttaccaagaaataaccaaagtgaatgcgctgatcactgaaggtgtgcaagagtctcaggaggaattctgtcataaagaatatgtatgtatctaagcaacaggactgtctgttctcagtagaatgacttctgcttctccatcctcttagaaccaacccatcaacaggaccttatggattccatcaggtcaaataggacagttagcaggataactatgttgctctaccacaaagaaaatgctgccttcacataaagcctcttttctgtaatccaagatgtccagctatgtacagcaggccccatcctagtcattaaaatgcagtgggattgactgtgctagactgattgggctcgagtttggaaacattaagtaccatgcacgtgttcgagctctgtgctcactcaacttctcatcctaacattgtttgtgttttgaggatgggctgctcagagtcaactcaggataagtatacctcaagatgaataaattgagaaagagaagtaaagaatgcaagagatgaaaagttagtgaagggaaacacagctgtaagtgccctcattgacttctaaatgcatttatatcaaagaaagggtgattttactacttcatgtttttctcagtaagagttccacctccacctagatgcttcactatcctccttgcttcctgcctatgtgaaaccttgatatttttcttgctcctgaccctgggagagagagaacagataaattattgaatccgtgaaggcatttatccctattccttgagaatagggattctcaaggaattctcctacccttattcctcccattgagaacagacctctccacctctgctcatgatgtttccaagaagagatgtgggcacatgtgcgaatatgtatgtatctaagcaacaggactgtctgttctcagggggactggcttctgcttctccatcctcttagtaccagtccatcaacaggaccttagaaggccacatggattccatagggtaaaatgggaaaatggagacgataactaggttgtttcatcacaaagaacatgctgccttcacatgaagcctgaatatttctgtcaaaccttgagggatcaatgatccacaagccaggtagagcaaagagaaaacactggctgcataaattatgatatgtctctttatcccattctaaatgaacactttcatctaccataacatgattgacataggaaatttggatctatttgttaagattgtgtgtgtgcattagggaggtacataggcatcagaatgctcatggcaaagagatcaaattctgtgtagttgtgctgttcaggtgaatatctgagagcaaagtataaactactgagagtataactcagccagaggcaacctaatggccaggtctctggtttgcagagggttcttatgtcatggtcaaagggagcattaaaatagccatggatttcaaaagaaaatcaattacaattaaaatgtgacaatgacagttaactgcaagactgttctgaatagggctgaagttttaggcaggcatgttttgtttcatttcgaaaaaaaaacaatcccctctggaaacaggtaatatacttatcctagaggagcaggcagctcaacaaattcgcattcctgtggccccttcccctgatgctgttctcctgtcagatttcagagactatgaatctcttactgcaagggggacagatggagtcacagcctggtggcctaaattctgtgggtaagggtggtgtgataagtcactccctctgcccagggtgatgatcaagggctccttgggtgctgtaatctgaaggacctgggcaggaatgacatggggccaggttccttgtggatatcaggacctcacacataaggttgcattcaggttcctcactcatctccgctttggtccttgctctttcaagtttccctactttccgaagctatcattgaagccagtaaccaagggggaaccatgtgcctcacatgtcagcttctggctttattggtgacacaaaaggaagctccagtgtagacttcctgttcttttccttcctcatatcctccctttccttttatgggtatttgtaggcaaaataattgacatgaacagttcatggctaaaatgcctagaattttggtccatttattggcccaaatgagattcatgaacgtccttcatgaggatggctgtcttcctaccctcccaccagctgtttaccagataatttgtttcatcagctaaaaaaaaaagtctcatagtataatgaaatgggttttgctctaaaatattaactattctcattttcaggagcaaggctatctagaccccataggacttttgaaaagcaaaattatctctctagacttatattttaattttcactaggtatctcccaagttgtcacaagttttgccctaccttgccaataataattgtcctacccactcctgtctcaatgaagagtggactttcttcactttttttttaaaaaaagagacttgtcactgcctgtaacttatttgagttcagttctctatagtatgctttaaattagcacacagtggcagaagatgcctcccaaaggggaataattcatagccaatggcataatgagatttacagagaaggctggccgggagaaggaacgaaaacattatcggttaccagagcagctgaagtgaaaggacagtacgagctccaagagtttcttcagagggacagagactgacactggctagaaagaatgattgatagattgctaagtagagccaagagaggaggaggaagggttaacagggcttcaagaatacagggaccagaggataagggagggccataaggtcagaagtgatgttgtctccccctgaggtaatgaatccctttatatttacagagaaaggagtagtttagagactagcattctctctgagccagctcattcaaatcctaacttactttcattgtaaatatacagataagaggtaaagtgctcaattacctcaactcttatcctccctttgggagaagtgatcctgtagacaaagcctcagaaagggtgagaagccaaagaactcaggaaagaaatataaagacaaggtggtgaccagcacagacagttcccccaaggccacaaatgtggaagtagcgtgtggtgaaatacagtggtcctgttggaccaccacctggggtctacaaggctgtgtgattagtgagccagaactgtgacaaggttcttttggtgctgaaagtgttaaaaaagaagctaaatattggatcacagatcagtcccagcatggatcaggttattagagactcaatcttggtagtaaagtgtctggatacaagctctacccaaagcatctgaaaagctgatacctaaaatttgatcaatatccttcatagtttctccctctgtcacttacttgaacacatgtagtgttccaagtacactttcctaaccataaaacagtccaaaacaacttcaaaggacaaagcacttagaaaaaggacaaagcacttagaaaaatccagattccatttgaaataatgaactgtatacatgtagtatatacatgtgattgtgtgtgcagatatatatagagaaactggggggattcatccttaggtgctactgcagatacaaatgggcaaaataaagtgactccttctcaattataatttataataatatcaaatatttactaatgcctttcatatacaaggcactctgtttagtgctacaggagataaaaagatttaaaaatacatggccctgaacacagggagcttatgctgtagcaggagagatgagatgtataaccaaatacctatgaaataagatggcccatgatagctgccactagggagaaacaacgaaagtgttatgggcattcataaaatgcctaaaattattttctgaatggaagataaagaagttgttctggtctttgaagacttatatagagggaatggatattattcaagaagggagtgagatgggagataggaaggagagtattttggacaaagggaacagtttaagggaagacgcaagtgggaaaacaagctggtagggaaaggtgaaacaaatgttattcagcttgtctggattatgggacacacacatagtcaagtaacaagaaattattgctggcagactacggcaagtgaagcccactgaaggttgtttcttgatctgaagaatgacatctgatttatatgtaggaagtgagtactgacaagagtagattcaaatataaaatattggaacaatgctaaaagacgctgaaataatccagactagaaggaagggtctgaatgaaaaggaaagactggaaaccttagggggaagaattagtaggcttttcaaatttttagatatgcaggatgaagaaaatggaggaggcaaaagtgcctgaaaagcttgagttcggtgacggaagacatggtgataccattaagcaaaaggaggaagttggtgattatgttggtttgcagcaatggttttggatatttgagtcaagatgaagttgagtgttcagaaggtgactggaagtatgtgtatgaaggaaaagcaaaaggtaggggctaaaagtgaagatttgggattcatcttcattcaaagagttattgaaatcatagaagacagaaagattgctacagaagcattaagataaggagaagagggtcaagctcagatataccatggcaagtcaatgctaaggagataagaggaagagcaggaaccaatgaggttagaggaccagagaactaagattaaaaccagaatgtattgcctcccaatggtaattgtcaatgaggttgaagagcagggtaagtaaagaaaaaaggctattgacttttgtaacaagaacttcattggaacgttgcctgagagtagtttcagaagagtggtagggtgtagcccattgatgaagccatgagcataaggtgaggaagtggagaaagaaagactacccttttgagaagttgggaagtgaaaagatagcgataggacagaaattcaagagtcaaattggattgagagatttgtctttagagatagttgtaggacgggtgtttttgagatagttgcaggtagatgtgtggaaggaattaaagatgcaaaagagagaaatacaattggctggagagcacctcagaagaggtcagagcatagggaagaggagcacttggttgggagaaaggatggaaaagatgtgtgaaagacaagagaaatctaaaggcagagaggacagcatatgtgaggattcaataatcagattttcttgcaaacacagtaggaaagattgcctgttgaaagacaggacatgaacatgaaaggaaaataaaacaaatttatcaagcacagaatgtgacactgagtcaacattggagaaattaaaaagtccaagtgagtaggcttcaggtgaggttaaattgattgaatttgtgctcttcacgtaggtttaagacttgctcttcttggggatgcaatgaatgacaaggggatgggatgcagttagctaagcatggttggtgtagtgagatggcaagaggaaaaaggaattgccggtgagaatattgctaatgtgggtaaatacagggttagaccaaagagggaattcaatgaggcctgatggatttatggaccagaacaacagaggggtcttgaaggaaggaagatatagaaaaggcaaggttgtggttagagaggaaatcccagagttttagctctgggaggtgtaataatttcaaaagaataagtccaggcctggccatgacatgggaagctgaatctctgcaatgttttttcaaatagcataatggatatctttgactcctaccctgaaaccagaaaatattaaacttgcatgtataatcatacaaatgtatgcatacctatttatacatacatttacatattttatacttatgctttcatatattctacgtgagtacaatatactccattttgaaaccttttatatcattcacagaactagcctagggacatagtacgtgcacaatagacgttggtttaattaaactcacatatttaaccagagagcttttatttttttctcctgcatagtactagaatctgctccacctcctaaatcacaacattaaaataattaccgataaaagagttcaggtttaaagtgtggaaacctaatctttaaaataacagtttaaattgggcttagtgttgtgctttttaattgtaccttaattcttgcactgagttctttcaccttctccaaaacacagattctacacaccagagtgccaaggctctgaggaattctactcatctactctgcttttcaccttcagttctttcaggagcccttaaccacataatcaccccagcaattatattcaaagcatgaagcagctccagaaactcactgtacagagctcttgagagatgtagagagaaatgtggaagatttctaactttccctacttattcccagtactgctattctaacccattactctgaacaaaattcttttttcttgcttcaatattgtaaatgagaagccctaaacgtcacagttctctccaaggcatgaaagtagcagcactggctttcaatttaaggttttgggtgagggcctttgtcataggaatagataggctatctcttctaagtcatagagctcacagggccactgtgtgactgaatcaatgtggttggaatgagttgagggtgggatgttctcagatatcctatgattttatacaatactgcaaccccaccccccaaactagaatagaatcctagattcagatcaatattagacattctcagactgactaatctgccattttagtgtcatcccaaacatctgctaggcctaagaaacaattgccccccaggttaagtagcacctgaggtcataagtggctcttttaccagataacagggcaccccctatggaggtggaaagtataggatatagaccaactcagctaattggaagattaattaaactgggacagaaaccagacaatgacagtaaattttattgtatcactaattcaatttgatttttctagctgcctactcagtaacatgtaatggaggagaagcatcactcttctattttctatggaaagaatcatagttctcaacctgccctacaagatactgaatttagaaattcataaattatacactcatatgattgtgtattgaaaataattcctaaccaggagtcctatttaggtgtcaaatgaggcttaaataaaagcaggcggaggccaaaatatggtttaaatgtctttgccatctagaacctgtatccttgttccctactctattgctctcagtgctctctgctcccttcctcttctcttgtatcataacttattcccaggaaaaggagtgagattcctaatgtaaattaggtgattaaatgtatacatccctaatatggcttaatatgtcacctttcctgggattactttcattcgaatgacagacagctcagctcagtgctaaagcaacaaatctgtgtgggaaggtggtagttgcagtggggtgggaaatgaaaaagaccttttcaggaccttcaacacaccatggaccacatagcatacataaggccagacccatcccagtgtgactattcactttcagctgcttctcctccatgaagagctccttaaacaggaggaaaagtctctgacacccaagtgaagaaagcaaaagctctgctgtagtgtgtagcagcctactgagcatgtatttcctatatggctttgggctcagagagcacataaggtatggccacagtccctggaaatgctgaatgcattcatcaatatcactgcagtgacatcatttatgcacacatctgaatcattcctaacatacaaaaacagacattcacagggtgtcaagcaatgacagggcctttttagagagatgatgattgaaagaataaagtgagttctggaatagtttttccaaaagcttattgcccaaacaatctggttattctatctgtaaatcttgaactaactaactaaaaaccgaccaaaaaaaaaaaaaaaatgaaccaaagaaacctagttcttagtgacatgtgcaggtgaccagcactctgcagagaattctcccttgggcaactcctgatggccacggaagaccgggtgagtgatagtcacttaactgtatagacaactcctactgtatcatgtcatacatgcgtttttggcactactgacaccagcaacatttaatggaatcatttgggattttcccctcaatcacaacatggctgtggccagtgcagggaaatacatatgaaggatgtttcccaagttctggctgaggatacacagtgacagattttgaaataacaaagtccactgtacatgcatcactttgaagggtgtgcaaagtctcgactcaggcaaattcaagggtcagattattgtcagtggaaatgctgagatttaagcattgccactgaaaggagttcatacaggaccacactcaccaaccacttctgcaatggaagggaatgatagagggtacaaagcgagaaagcatggattctgaagaacatgggaatattaggtgctcctgagggtatctgcggaatctcacagttttggatggattgggtgttgtttcatacccatctgtgatatagattgggcttatagctgaattcttcctcatgcattttacttgcttgttattctggaattaagtaacatctagattttaacaatgcccagccttcctttctttaagttttcttaagcagaccatgagtaacttagtcccagtgcaaatatccagttgaagaaaagcaaccaactggggccaaataagtttagaaaaataaaattgtccagctaacagcttttatgatgggaggataggaaaaaatgtagtgaatatactgggtaaatggatttggaaattttatcctgtgatagaggctgccaacctccacaaagccaacagtctaggaaaagaagttctatttgtctggttaacccaaggccagattatgaacacctggctcgaggccagtagcaccttcctgatggcagtaatgaggacaaggcaaataaagagccgctattggcaccattgctcacatacccaccctcccacgtctaaacctaacttcagcaatcttgctaagggaatcatctcaccactgagtttctagtggatcccatcatcttttctagaaaagcatgcaaatttgtaagacacatatccagcactacctctctgtgaccagatatcacatgcttcaaaaagtagagttagtggagatttttccacgtgtgtttgccaggctgacttctgagggtggagatggggcagggagtgagtcagcgcccaggtcctaaagaagaaaagactcagatgactgagacgattgtttcagcatcagaggaggccgctgggagatttctcaggattgagcttcctgaaacctttcagtcacgccaagaatgggaagttaatttgaccttaattctgtttaagcccttttgggaatctttcctaccctaggtactgacagaggaaatatggtgccaccagcctgtctttgtgtggaatgtggtaacctagggtctacctagaagataggagtcagacctggggtttgcttagagccaaattgaaccctatgtaaaaccctggccaaagtgcatgaacatttctcacaaaccagtaagaagactggttttctgggggggatggacacaattactttcccctggctttttcaccatagtggcctccatgagcattcgctttttccagacaccctgaagcaaaaaagccatacaaaacaattcccccaatgggaaatgaaaacccataacaaaacactttttccctctcattcccatcaccaccccactccctccagcccaacaccctgaatactcacaagagaacactttatctatacaaaattagaaaacaaaatatttacatatgaaataaacaccatcttgatttctgttgccagcggagactgaaagagctcccttggttctagattgctgttcgctaggttagttggtttggtttttttgtttgaaaggggtgaggtaagaggaagatgaggggatgagtccctgacccctggacagagtcagggcgaagcagtgtttacgtggcccttcgccttcttcctcctggaggtgcctcatgccctctgtcctctctcagtcttttctgttatctaaggtaaagcactccgtgctcctctcaccaaatctgtgagaggttcagccccttgcccccatgttcattttagaaagaaaacaaagctttacaaggccttcagttggctttaaaatgaaagatactgaggtaaaaatcaaggaggagggttggggacagcagtcaagggcgggatgaggaagggtcacgagtgagggcaaacaggggcgaagagcagccctggagggagtgacttgaagagacatggcagcttccttccagaggaggatgagcacctttctggtttatgtgtcctgtgtgcaacatggcgatcctgcagtcaagcttccacacagacctggggctctctggatgccaccctgtgtaggggaggatggcaggacagtggaactgacccatagaataaatagccctaccgcaagtttcaggaccggcagtgatacatattcatttcccttctcaattttccaatgttaagtgaagggagcatcagttctgctggtaccctcatccctggagttttatacatgtatatctttttttattcctcaatggtacaatctgagagggaaacaaggtgttgcaggaaggtagaagggcttctaccaagagtgttcactctgggctcaagtcacattcccagggagccaggcccaaagaggtggtggagggtccctctctgcccccgtctcccatttccaagtctcttcccctcttttcgtacctccagagctgcactcatggagtgcagctcatttctcttaaaggtcaagctcatttctcttaactgtctgctctgtagcagttgtaatcagttttggggggaagaagcctgctcgtctagcttcaggttaagtaagaagggatcaaagcattggaaacatccccctctctcacttaccctaccatacacgactccttacttcttcaaaggtggcttcgttcttccccaaaccttggccagtcgagagtctaaatgctcaaaagagctttgtagaatcttttgctcccaagtgtgggcaaaagaatcatggctgtgaaaattcggtttccctttagccttcctggaaagttcttggttcaaactggttgaaacaattgccaaccactgaggacttgtttatgtaccttgttcttgcaggattgctcaccgcctttttttgtttagaccacagaatcttctttatcaagaattttcattctccttattccagaaggatgaagggagacacagccaaaattcaggtaatacatggccatctctgtctgtatataagccaaacaatcacactgcttggggatattgaaagaaacaatagaaagagtcaaggttgccttctcttgaggcacctgactacacatgggtgcaagtgtgcatgaacacacatgcacgcacaatccacctgctcttgtccccaaggcaccgtgggacactatcataacgtactttccagtttgttcaagaatccactctgccaccaatgaccttttgttctgttcaccaccactatcgagtctcatggggttgaagcaagcattttttggcttatatataaacacaaatggcctcccaacctctgcttggcacatgattcctagacagatgtcatctaagcagcatgaatttagccagagcctctttcctttcacaagcagtgtgctaaatggtctcacatagatgcttttgcttcctcacctaaatgaaaagatcagtttgggaaaagctacctttgtgctcacatagcctctttttggttctcccagcttcactcaaagaggatatcaaggagctcttccacaccaggaggaagcccgcatgcagcccttcctttctccgctctaccctcccctgctgagagggcccatggcatcatctcatgggaacaggaatggctgacagcggggggaagaaggagagaactgtgaaaaggaggagagatggtgctggtcaccagggttgcccccagtaggaaccagaactccaggatcccataaataaattaaaacaagaaaggagcaaatgggaaccaagttcacccccgtcaccctccgtgacatgcgcatcacgcgacccacagccttaccctcccgtacccaccttaacctctctgttccctcactcagacatcagactcaatactagaaagtttctcataaacatgcccattgctggagccattgaaagccctggggtttttgttgttaggcacacaggggttggactggttccctatacagatgtccttctggaaacgggctggcacggccccatgaagggccgagaccaccggcttgttggtgacaagggcccggaagtccggcctggctttcgacgcccccgccaccgtgggctgcctgaagaagtaggatttgctgccatggagcaagcactggtcgtccccaaaagtggggatgaaagggttttgcgtgacccggtcagggtagagcgacttgctgagcatgtacccgccgccggggttgttgtggtggtgatgtccggcagtgggcactgaggacttgttgttggcaaaggtgctctcgccagctgacatctcaaacatgtgggcgtaggggctcccatccatgaatcggcccttgtctttcaggcttacgctgcgcggggccagggcggcttcttccttctgcaggtccacgaaggtgtcgtaggagtgctgccggcgcagtttgttccggttcttcttctgggccttggaattagtcgggctctgagggtacttagtggtggaggcgtttgacgtcaccgccactggggcagccggctggtccagttcctgcagggagttgtcctcactgatgtcatacaggttgcctgctttcttgcaagcctcacaccggatgcacgcctgcctgcccgagttctgacccgtcaccgtcgtggagtagttgtgcagcttggagggacagctgcggcagaagttgcccccggaccggtcctcccactccacgttggtcaggttcttctcccaaggtgcaggtaccccgctgaccacgccgtgtttgtcgcccgtcccgtgcttgatgtgagacctgttggtacagggccctcctccgctgacggagtcgcgcttaaagtcatcactccgctccttgtagatgtcggtcaggtctacgtgctcccagtggggtgagttctcctttgttcggaactggtccaggtagaagtcccgtagcccttccttgtccctgaagtagcgcttgtggtcaggggagcggggcggtcggcgacggtaggccagctcgatctcgtcaaactccctgcgggacttggccgaggcaggccgcttcttcaggctgtccttatattgctgcttacgcctcttggcggcattgccctcgatgttcccataggtgacggtgtgggttgagatgtcagagacatcggagcggatcaagtcgtcgtggccactgtagcggtcgctcttgaaggagaatttgccgtacaggtcactgagctggctgtgcttggaggaggggaggccgatgtccaggggcttcttgctgatggacctggactgggtggtgaagggtgggttgtcacagtcgtagagcccatcgatggagctggcactgccaatactatggggccggtggtgatggtggtagtgatcttggtacacgttgctgtccttcagctgcaggttcccgaacgttctctctacctcactgatgtagtcactgaagaggttctcctcacagggcgggttgttgtaggatttgcagtcagaatgcgtgaagctgcggcggtgctctgagatgtcatagacggatgactcccgtcggatgaagtccagggcgctctgcggtgagccattcacaccagacaggttagccatgttcttggccgtgcgcagcaggcgcaggatgttggagtgtgtgttgttcatggttgcggtgggggagttcattacagactggcgctcctcgatcgccaccccatggatgcagctgtagatacctctgctgatggagaagaccatgccaggcttgccagaacagacacccataaagcaatgtcggaactgccaatagaaaaggtgttcgcagatgaaggtgatgaggctgagagccatggccgcccccaacatgtagaagacccctgccatgttgtcaatgtccagctggctgctcatgacctcattcttctcattgtgacaaatgccagtgagccagagagcttccagttcttccatctccccatctccaaagagctgcaggatagcaaggtccacctggcgcttccacccagaatctttttggatggcaatgccatagccagtggaagcaaagaccttcccactgccaatggtcaccagcttgcagccttcatctctgcctgccatatagttcagcactgctgcatcatagatgaaggcatccagtttccctgttttcagggagagcaatgcatcatctacacccctctggttgaactttcccatgtaggcatgcatttctgcatagttattgcgaatatttctctctgtgctgccgttgggcacggtcccaaagcggaaagggggtgagaagtcattaggtctctggaactttttgtcgctcaggccagaaacctggtccacatattcctcttggatcatgaaggcagctaagttggcagtgtagctggccaggaagatgacagcaaagaaggcccacactgacaccatgatcttggaggtggtcccctttgggttctgcacaggtacggagttgttaaacaccagaccccagagcaaccaaatagctttgccgatggtgaaagagggtccaccaggctctctgccatcagcgaggcacctgttataacccacagggctgaagtactcaaagacaaagacagccacggctgagacgatgagcagcatcacaaacatcatcacccatacgtcagcgctgaatggctctaagaaggcagaaggtgagacagtcccattgctgcgtgacaccatgacactgatgcctgtctctatgaagggcacagagaagtcgaccacctccgatcgttcctcattgatggtgagtgagcccactgccatgtaggccctcttcatgaccacctctccaatcataccattccaggttccattgattttcttcccatgcttgccattggtaaccaggtaaaggtcataggtgaacttcacagatttagaaattttcttaaggatgtcaatacagaaccccttgcagcattttttgatgtaacccggctcctcgtctgttttattctcagtgactatgcgtttttggcaggggactgtgttcctcatgcaggttccactcagagggtccacactttccacaatgacaaatggtgcctcctccagggtcacaatgctcagatggtcatcctcctgctcttcagtctctggacacattcggggccacacatagtacttcatctgcagggacttgtctttccacttccccaccctttcccacttcctctccttgttcagaagaattatcaccagtttcgggtgcatctggtagccatcttcactgaaggacaaattcctcccctcaaaagtgacattgatcagatacctatttagcatattggactggtagattctcttctcgtgggtgttgtaacaactgcttttgggctcagggatgaagctgtgctcagacagcatgtcagaagcagcagtggtgattatggcaattccatctctcactctggcggggaggccatagtcccattcatcatatgatacagagatgagcccagtggggaactccgcaggcactgtgtctgtatcccctgccaccagactgggcacgatccacgtgtagccatagccagtcagccctactgagttggccacttcaaagatgtaggtggcttcttccttggtacagtaaagaagaatgatggggctttgaagtttcttgagctgattctggatcttagaatctccatcgtccagggacatgtccagtaggaggacctcctctagctcccagcccacaaagctattctcaatggtgctgcggatcttgtttacaaagtcctggtagccagggaaataggtggtgacgatagaaaagatgtaccagtcatattcttccatgatgttgagcattacggaagcttgctgttcaattgatgggccaaactggaagaacatggaggattcatccttatctgccattatcatagaggagcccccgtggatgcccaggatgggggtgagagtctgtgctgaaatgaaatcgaggatctgggcgatggcttcctggtctgtgtcatcagcaaacaccaccccctggatcttccggtcagacatgagatcacagatgcgggtgatgatgctctttgggtcggtctcattcatggctaccagttccacccggggtaccacggagagatggtggaaatcatctttctcgtgggcatccttgatggccacctcgtcggaagtgcccacgaggatgacagcaatgccaatgctgggggggctcttctgagaacgagctctgctgcctgacacggccaggacggccaacaccaaccagaacttgggagaacagcactccgctctgggcttcatcttcaactcgtcgactcccttggtttgtagaagccaaacctctagacggacagattaagggagtgagcatgttgggaatgtccagtcccttcttctcgcttgcatatccacataagaaagacgaaggataaatgaacggaagataatttaaaatccaatttagcgtaaattttgttttaatcttgtgtcttgaagagatgcaaattcaaaaaaaaaaagatttaattcaaaggtaattcagggtatggagagcagctcacaatgcagaatccagagtaattattccgtgtgcatgtgaggttagtggctggaatagatttttaacgcttcttctggcaattacggtttttggtttttggagcgttagtggaggaggctctgtgtggagaagctgggggccggctccgtccctcggtggagcatggtcattcccaaagcgtccccttcctgcaacgtgtcgattggacggatgggctcggcgcgtgggtccggcccggggcgccgctgccctgcccctctgctaggtga

SEQ ID NO: 12298 - RNA, 26406 nt, Homo sapiens
  source 1..26406: mol_type = other RNA
ctgggaggtcaaggctgcagtgagccgtaatcatacctctccactccagcctggatgacagagcaagaccctcttaaaaaacaaacaaacaaaaaaaaaacaaacaaaaaaacaaaaacaacagaaaaatcagagccaagatttcaagtcttgtcttcccccttttttttttaaacaaatctcagattttcaaatcaaacttactgtataattttcagattattgttaaagcagttctgttgtccaaaaaaaatttggggtttaaggaagtatctccagaagtaaagagaatcactatatctgggaagaatctggctttatgttagagcttgctactttctggaatgttcagggagaaacaagaatttttgttcagtacaaaggaaagtacaagagagaccctcacagataatctctctgagacagtaacttcaaagagataacaatacattatcctgggagattcctggaactagggattagccctgctggcttctagccagggctgccatacatgagctcacccaggctccttggccatgagacagagttcttctaaatggtctctagaaggtcctttccagtactaggactataggaggagcatgtggcttttaataaagtgatgttgaaatgtgcctcatgattggcatgtgaaaagctaaatatgtctatgctattttcttaccaagatagctaagggggagatactattatttaacttggataatttagcaatcaaggtatagaaagagagatcatttagaatccatatataaagccagtaacaggactgggactgggagtggggtgggaaacaatcagcaaaacaagggctggtttgcttttctgacacctccaagcaatggaagtatgcattaaagagtaaaacaattaccaatttacattgtcttcattaatattgggaagaaccagcaaaatccaactgtgggaacctctaaaggataaagtgctctattcctttaacaagtatatgtcaagaaaaagttagaaagcaaatctttagatttaaaatacatttgagaaatagcaactaattgtatggaccttatgacttatgggaaaaaaacccaccaccaccccataaaacagtattacatttgagacaattagtgaacactggatatttcttatcaaggaattatggctaccttatgatgtcacaatggtattgttaaactaaaaaagagtccttagtaaaagagatatatactgtaatgtttacagatgaaaccatataattatgggatttgtttcagaataatacatgagggggagatgagtgtaaccaagggctccagcaccagctatagtagaaacagatcccaacccaagtagattcgccagtccaagactcctaccaacaattggaaaccaactgggcaaggggtttttcccaaacagcacttttaacaatctttttggaatcacagtaaagaaagcacaaagaccaagaaaaaaactctgattctggattttttttaaccctgataatttgtggtaggtttctttattttttgaatataaagtgacagaaataatttgccattagaaaagagaaagaatctttgactatttacagcttttatacatcacaaagtttttcttgtttttttatgttgtcttttttttaattcgttttaatttttgttcctgcatcatttgaacaagtccaaactggaaatctatacagctcacaaaaaagccctccacccaaaagaccccccacccccacccgaccccaatgagaaacaagataaatcaaaagaatgaaatcaacttatttcttttgtttaaaggtaagtcatttgcttatatatatacttgtaattatttttttcaagttcaaacaccaaaatccaagagagaaaggaaaaaataaaaagacccagtcatccgcccctccccccactccagaatctcaattgatccctgcatgtccaaaataagaaatagatatttacagaaaacagaagcaaaacaaataaacaaaaaaagaacttggaggtggatgggctggggatctgagagtcaagaggaaggagagccggccccagggaggagtgtggagtctgggcctcgcagagctgaggcaagcctgagtcgtcggtgctccctggagaggacatcacacaggaaagctatgaccatttcccctctgccatgtgactttgggaggggtgcagctgtgaatttgcaacgcaaccccatagtggatgcatatcatgtttccatcatcacccccttacacacgtgcgctcacacacacgctcacacacatgtgcacaggcacacacacgcatcagtcattgtggctaagtgtaattctgatgctgttggagcactggctcctgtcacgtggaggaaaagagatttcccctagggacaagagctcactgccccatcccttctctgatctccactgtaacattgcctctagctcccttgaaatgtttccacaagcgtcagggctactctgaagtattaatgctgggatagtcactgggtaacaaagctcccataaatctattccctctgctccaacaattttgcccctcacttcccacaaattcctttaacaaataggcgtacccaggttaccccattaaccaggggtgggagccagtctgaaggaggggagatctgaggcagggtaaatggaagtcacattgttttctgcacatcttccaaagagtggattccgggaggtcagaaagcaaagagaggtcatgacaaaaccatccctggcttcctttgcttccctcttccttcctaaatagagtttaatgcgtactcagtgcataaagtaaggtatgactgagttggctgtgataccttaagaactcaagatgtggcgttagatgagccaagatgaacataatttaatcttttgggggaaaacggctggcaggatatgaccatgctgaagggtttgcctttattagtggacagagaggctgaaccagcagcagcagtagttgtgatctcattcacaccctgttcagggttccgtgagggtttggaaaaatagttcactagaaatggcctaacagtttctcttctcaaattatgattttttcaggtggcacaggaaatagaattagtgcatcctctgtgtcagaaacaacgtgcagtgtctctgggggcagactctaggttgctcttgctaaatctccaaatgcctacacagtggaattttatttttctgctctccttgccaaactacttgtttttttcagaccctccccaagagtcctcacttacccccttttcatgcagccccactcagagtccttttctttctaagccctctcctgatccttgaaaacgctctctcaaggcttttaaagactttcattcatttccatgctcctgtcccactgtttctgtcacaaaagaaaatacaaaatcaaaatgatctgtcagagaaaactttcatttagcagaattgggcagaagcaaagttgctttccaatcctttttatttgattttttttttaaagatgaacaaggagtaaggtaagtaagaacaaataattatgacccccccacaacgagactagcttagttgggaaccttagaaaggacaagatttcctgtgaaaatgtgtactttccaggataaatagtcaaaatgtggtctcaatccaggataacatttgttgacatctataaaaacatgttgtggcctatcacagttagcagtggggtttttagtagaagttaaaaaagcaaatatcaggactgaggaagaggtaccagagttccatgtgctgccatcaagtccctgccccgggcacttgcagcatcaccacctcaatctgacatagagacaattagggccaaccccaaatgcccacagcctcgcttagggcaatcaccacgagaagcccaagacccccagtccctcttatcacttggactttcatccccagatacccatgcacatctcccatctcagctcatttcccttcctttaccaactcccaaatcctgcctaagaatcagtggttcatcaccagccacaaccctggcaattcctttcctcttgctcttacagaaacctggctcctctttgaggaccctgaatcactcccaggtggtgagcatttccacttgcaccttcctcatgccctggggcctggaggtggagatgcccttcttgcccctcattgccattccagaccatcctccctcctttttaaaaaaaaataacatgcaacaaccataaaatccagctttgatgcacatcagactaggctagctgcaccccttacttgatgcaatgattgaaatgttctcgaatcactctccctcattcctgtcataatttacattcctatcatatggaagtcaacattttgttgacttcaatatctatataattcccatatcctggcctctcagttccttgacccctgctccttctataaccttttcctctatcttatctcagcccaccaccccaacaacagaccccaaaccaccaataactgcaagccctccataacctcaagcatccacctctccaacccacctcctaatttctacgttattgcttctgactcactaactgagtgatcccagcttgaatctcaatcctctgcctctaatatgcttcattgttcctccttccctaaaaatcctcactttcctctacacccagcttagattccatgaccaaacattatagttaacacactgcagttgcccttgactccacatctcttgctttcattatattcacctggttataccccaaccctgttccaatctaacttgccaccctgtttaagcagctgaaggtgactgaagaaaacaaatttctttaaactcataatcataaaaactcaaataattcctttatgccccctagcatgtctcctatatttttggtgtctccgacatttttgttctcactcttcctgccggatggctatatgactcattcatgctttcttccttccaaaacctccaatactcttcccctatactcactcttaactgatgaactcctttcatagtttactaaaaatcaatcagaaaaagcatactcccattatcccatttaccagcccacttgcatctgtgcccaaatgcactatctccctgctattaatacaaacaaacctggttagtcccctgaagccagtccctctatgtttgtattgaatcccatgccctctcacttcatcaaagacattactccagcaattgtcctctctccctaggcatcatcaatttttcctttctcctggattagtcttgtcaacataaaatgggctgttatttttcccatcttaaaaaaagaagtccctccctgggcgtcacattctctatgatctgctatttccatgtcctctttacagccaaactcctaaagcgttgcctattcctgttgtctctacctcctctccttcccctctttcttgaatccaccccatcatgcttttgcccccaccagtccactgaaacagctctcttccaggtcatcaatgggatgacctccatgtttccagatagtcttatcctactcaataatagtacttgctttacccattaaccactcctcccattgctggtcccttctcatctcctggagctttgaacaatcctccaccctgggcctcagtctagagaatcctcttctgtcgctactcattctctagttccagtatcatggcttcaaataccaaccaaacgcatacaaattttaaatatgtatcttcaggctatacattttccctgaactccaggtccatatatctaattgcctaatcatcatttctacttgcaacatctgtagacaccttaaactataaggctttccttcccagtcagcctcacctgcaggattcctgtcttacactgatggcaactccaaactttcaatagctcaggccaaacattctaaggttattcttaagatttttctttctcttattcaatgtctaattcatcagcaaactgtgtgatatcgattctttaaaacatttctggaatccaactgcttcttatcacctcccctgctaacatcatggcccaagcaactatgatctcttaccaggattattgcaagagcttcctaaccggtctttcagccgcttccattgtctgccctctcagggtatactctcaacacagcagtcccaaagcttcctcttcaactgaagtcagatcatatcactctatgctccgaaccttctagcaacttctcatcttgctcttggtaaaagccaaatcctgacagtgtcctacaaggccctacctgacttgcgttattgccccctctctgacctcacctctcatactctcctcctccctcattggcctcccggctcttcctcaagtttgccaagcatttggtttgacagcagggcctttgcaattgctttctctttgcctttgcatagaaagccccaagtctcactccctcatttcctccaaacctttacttaaatgtcatctttgcttactcaaaaatagcaaccccacacccatcctatcatctatcccccttaatctgcctcatttttctgcatgacactttgcactatctgacatgagatctattgatttgcttttttgtccatttcctctcatcaacatacaaacttcaagagggtatggactttgtgtggttcgttcttatattccagcacctagaacagcctggcatgggtttccactcaataaatatcaacatggataagtcatttatccaaaacatgctctgaagccacagaccaaatatccccaaaataagagctccagtaaacaaaacaatgcaagcaaggaaacaactcctcccccaaaacctggatatttattctaagtgtttctaaattttaaccaatggcaagtgcagagctcacttttcatgatttttctggtttgagaattgtccttgggttaattattatttttaataggtaagaaaaaagttactccgagtttcattaatctatggcactttgtccctcctctcccctgcggcctaactcccaaatccccttcagctatagtgaaatacacagacgctgaatatttgggaggattacttaacgttttagctttcctggtttgcttagaacatatgatctactacccgccagtaatattttatagcttagaagatcatgtctgagtcagtaaattccatgttaatatgtgtaagactcaggattaaatcaatctgtaaaatgcctatttgtaatcgaatctagcaattttctttctgaagtaaacagtaatcacattaacaacctagtgatttcactggagatgggaagatataattttatttaacagattttctctctcagaggtgacctaactttgtgatccaaaatcattccaatattgaaaaaaaaaggttcagctaactccattcccctgatatattcagttctcagtgccccttggcttcccaatttaagtcaatgtaatcacaatgcacacaaggctcttccactcagaatcttcttgactggagaatggaaatcattggagaggggctgccctaaaggtttgtagacaaggttttgaagaatcgagctacaatgcttatcaatgtctgtctggaagaaagcctacgtctctttctaaagccagcctgtcaccatttctgagccatcaatggcagcacagcctctccttctgccagagctcacagggaatgacaaatctctgagggaatacaccagagcatctggatgtgggtgtcatcgtctcttcaccaccaaaccattctaccccaatttccctcttctttgtttctagattatttttttttcaactcagtgaagaacatttctcagaaccaagctttttgtctgcttgtcactgaatctatttcccattcaaccttctgtttctcattccaatagacacacaatattaatggttaaaaataacatgcaacaactcactgggcgagaaatttagaaacacttgcctcctatgaacccagggccaaggggagctgaggatagtgtcacattaccagcatgttcaagctagacatcctccatcacaaagggcttgtgccttgaaataaatttaaaaagagagaacaagaaaagccacaaaatacctccacatacacaacaggcatcttgaccagagcaccaggacacatgctcagaggtggcttaatattccagagcacatccctctccactaagagccactcactatcccagcacttgatcttgagttgaagcactcaggaacaagacctcatttgcctgcttgtcattctttctccaacttcctaagttaaaaaatgatgagaaaaccatgaaaaattactgtcaagggtttcttttaacagtctgatagtttagataagaatacagtttaagggatatatcccattttcataggaaaggaaagtcggggaggggagccaaaaacatgaaggggaaccaggagagctgccaggaggctgggaggtgaggaagggtttccaagtaaggagcttggaaggttgttctcaacgataaaacccactttgcagtggctaaaaatataagtattttggtctattttatattatagctgtctttccttttgtgaagcaccaaccactgaagttcattttggaatcatggccacccagaagaggaaaggggtgatcatgtgtctcaaagaagagataactttgagggagaggatgaaaactgcaaagacccttgggattaaatgaaatctgctgattctactcttttttcatgaatttctgtatgatatttagcaattagaatgtttgactggcaatggccaggtagatttcaccattatgtaacaaagagaataaaaaagaaaggaaaggagaaaacaataattggcctaggagatgggagttttgttcttggtcttagttgtctccctaggagaagcagctcttttccatccaaaggtgaacagaagactctgcagagcataatgttgctatggcttgttttactgaagtaaagacactgtaaatctcaaaaatactccaacttccctgattcttttggaagttattgggcatctgcattttcccaggagacttctctccacattgtcgcagtgttgaaactctgagataagaattccttgcccatcttctaacttccacccagatatctggcttctgtcaataggccttacccaaacagggttatgtatatgtatgtatgtatgtatgtgtgtgtatatatatatatatatatatattttttttttttttctgaaagctacagaagagaccacggagatgtgtgagctgccaaggtgccaatgatcaaatagagaagtctagcttggaaataaatcaaaaccatcagaggaattacattccacccctaggctcagtgggaaagagtttaagttcatgtggatcttgctgttccggagcaagctctgggctctaaaattgagcttatcttctctgtctttcataggatagctaagcacccatgccccctaagggatacttgaaataggaagatatctttatgttgtgtatactcggtttagtggcttcagtcttgtgcagatatagattttctttgtaagacttcctccattggccgctatggtacagctcagaaaagctgaacttttcatttctattttaatatttaatactaagtacaagagctctgtggtttcaatcaaataattctccattcatgccctcagagtccccaagaatcctgctattttcccacctcccccccccgatgaatataggtgtagcagaagacagggagtggtcatcttgggggaataagatgctccaaatactcatcagctgttggccctgtgacctgtttttcaggatcatcatgatccaggtatctgtaatgacactcatgaaaaagatgaagtcaccacggagtcaaggtagaaatagctactgcccctctctcttagcttactatgataacacgattttatgtgaattattgggaggcaaaaggacaagggaaaaatgagatttgtaataggcttgattttttttagattaaaaaattagtctagtgcccacctcctccccccatcttcatgcatgggaataaaagctacctcctccatttcctccgatcatctgaaactagcctcctgaaccaggctccggggatcagtacactctgaagttgatggtatagaagtctcctcactcattcatctaaggacttttccatcttcctacctcctctcctatcttccctctagggctaggaaggactgataaaaaaaaaaagttactctacattaagcaggacactagagctctttcactgtttttggtttaagcataatgctgtgagccaaaatttcttctgcagcccaaactaaagatactaaaatctttggaaagatggattatatcctgagcttgatatcattcataagtgaacaggtgggttgtaagagaaggttgttgcaagattctctgatctgcgggtgcttaataaataattcaccattgcaaccttgtgacaaaatcaaggtctcataagtattctcaggagactattaattttggagcccccatgcttccctttcttcaggattttggcaggcagtaattatttattatcggtctgggggctataggttctttcttcaagaattcattgtgtatgtgaactgccttatatttttctgttcagaactaacttatgccttaatcctagaatcaggcttgtatgtttgaacttaattagacagaggtgcccagaaaaggatgtaaggggctctcccttgaggctgccctgctcactgtgggctgaccaaaactactgacaccttcggagtatcatgacacccctgcacacgttcctgaaggctcttttgccatgtagcactctggaagaaatcctctgtcccagtttattcttgagttttttatttatgtggattacatgctacctaaaaaaaatttttaataataaaaaattattcacaatatcttaccctatagaattcaaaaacatttttatttgaccaagttttcttcaccgtggaaacctctctaacctttctgattttcaaatttttgctttcttcttgctctttttgacttgtctctgtagatgtatgtggagtgtgtgtgtgtctacaaagggaaatttcatagataagatctggctaaatcagctgcctagatttcgtgacttttctccactgctagatgctgaaaacctacagtgggggcagacaattcaggcagcattactcgctgagctagactgagagttagaaatttggacaagttttggttcagccaagttttggttctgtcaagaattttctgtataatcttacttttggctaattatccaattttgtgctttgacttctcatctgtaaaactgaaagatgatcttatttccaagtcaaaggaggttatttggagaagtggttatggtaaattcttctgtattcacataccaactactgtgatttactcagaatgtaccataggctaagtgtggtggagcctaatgggttgctggttatcctagaaactccaccattccccaaggaggggagcagaggcaggctagaactgcaggagctcagtgcctctttacatgggaataagctaaaaatgctcgagaaatgactcttcagatttctatgtgacccatttctcgtgcctgttaccaagaaataaccaaagtgaatgcgctgatcactgaaggtgtgcaagagtctcaggaggaattctgtcataaagaatatgtatgtatctaagcaacaggactgtctgttctcagtagaatgacttctgcttctccatcctcttagaaccaacccatcaacaggaccttatggattccatcaggtcaaataggacagttagcaggataactatgttgctctaccacaaagaaaatgctgccttcacataaagcctcttttctgtaatccaagatgtccagctatgtacagcaggccccatcctagtcattaaaatgcagtgggattgactgtgctagactgattgggctcgagtttggaaacattaagtaccatgcacgtgttcgagctctgtgctcactcaacttctcatcctaacattgtttgtgttttgaggatgggctgctcagagtcaactcaggataagtatacctcaagatgaataaattgagaaagagaagtaaagaatgcaagagatgaaaagttagtgaagggaaacacagctgtaagtgccctcattgacttctaaatgcatttatatcaaagaaagggtgattttactacttcatgtttttctcagtaagagttccacctccacctagatgcttcactatcctccttgcttcctgcctatgtgaaaccttgatatttttcttgctcctgaccctgggagagagagaacagataaattattgaatccgtgaaggcatttatccctattccttgagaatagggattctcaaggaattctcctacccttattcctcccattgagaacagacctctccacctctgctcatgatgtttccaagaagagatgtgggcacatgtgcgaatatgtatgtatctaagcaacaggactgtctgttctcagggggactggcttctgcttctccatcctcttagtaccagtccatcaacaggaccttagaaggccacatggattccatagggtaaaatgggaaaatggagacgataactaggttgtttcatcacaaagaacatgctgccttcacatgaagcctgaatatttctgtcaaaccttgagggatcaatgatccacaagccaggtagagcaaagagaaaacactggctgcataaattatgatatgtctctttatcccattctaaatgaacactttcatctaccataacatgattgacataggaaatttggatctatttgttaagattgtgtgtgtgcattagggaggtacataggcatcagaatgctcatggcaaagagatcaaattctgtgtagttgtgctgttcaggtgaatatctgagagcaaagtataaactactgagagtataactcagccagaggcaacctaatggccaggtctctggtttgcagagggttcttatgtcatggtcaaagggagcattaaaatagccatggatttcaaaagaaaatcaattacaattaaaatgtgacaatgacagttaactgcaagactgttctgaatagggctgaagttttaggcaggcatgttttgtttcatttcgaaaaaaaaacaatcccctctggaaacaggtaatatacttatcctagaggagcaggcagctcaacaaattcgcattcctgtggccccttcccctgatgctgttctcctgtcagatttcagagactatgaatctcttactgcaagggggacagatggagtcacagcctggtggcctaaattctgtgggtaagggtggtgtgataagtcactccctctgcccagggtgatgatcaagggctccttgggtgctgtaatctgaaggacctgggcaggaatgacatggggccaggttccttgtggatatcaggacctcacacataaggttgcattcaggttcctcactcatctccgctttggtccttgctctttcaagtttccctactttccgaagctatcattgaagccagtaaccaagggggaaccatgtgcctcacatgtcagcttctggctttattggtgacacaaaaggaagctccagtgtagacttcctgttcttttccttcctcatatcctccctttccttttatgggtatttgtaggcaaaataattgacatgaacagttcatggctaaaatgcctagaattttggtccatttattggcccaaatgagattcatgaacgtccttcatgaggatggctgtcttcctaccctcccaccagctgtttaccagataatttgtttcatcagctaaaaaaaaaagtctcatagtataatgaaatgggttttgctctaaaatattaactattctcattttcaggagcaaggctatctagaccccataggacttttgaaaagcaaaattatctctctagacttatattttaattttcactaggtatctcccaagttgtcacaagttttgccctaccttgccaataataattgtcctacccactcctgtctcaatgaagagtggactttcttcactttttttttaaaaaaagagacttgtcactgcctgtaacttatttgagttcagttctctatagtatgctttaaattagcacacagtggcagaagatgcctcccaaaggggaataattcatagccaatggcataatgagatttacagagaaggctggccgggagaaggaacgaaaacattatcggttaccagagcagctgaagtgaaaggacagtacgagctccaagagtttcttcagagggacagagactgacactggctagaaagaatgattgatagattgctaagtagagccaagagaggaggaggaagggttaacagggcttcaagaatacagggaccagaggataagggagggccataaggtcagaagtgatgttgtctccccctgaggtaatgaatccctttatatttacagagaaaggagtagtttagagactagcattctctctgagccagctcattcaaatcctaacttactttcattgtaaatatacagataagaggtaaagtgctcaattacctcaactcttatcctccctttgggagaagtgatcctgtagacaaagcctcagaaagggtgagaagccaaagaactcaggaaagaaatataaagacaaggtggtgaccagcacagacagttcccccaaggccacaaatgtggaagtagcgtgtggtgaaatacagtggtcctgttggaccaccacctggggtctacaaggctgtgtgattagtgagccagaactgtgacaaggttcttttggtgctgaaagtgttaaaaaagaagctaaatattggatcacagatcagtcccagcatggatcaggttattagagactcaatcttggtagtaaagtgtctggatacaagctctacccaaagcatctgaaaagctgatacctaaaatttgatcaatatccttcatagtttctccctctgtcacttacttgaacacatgtagtgttccaagtacactttcctaaccataaaacagtccaaaacaacttcaaaggacaaagcacttagaaaaaggacaaagcacttagaaaaatccagattccatttgaaataatgaactgtatacatgtagtatatacatgtgattgtgtgtgcagatatatatagagaaactggggggattcatccttaggtgctactgcagatacaaatgggcaaaataaagtgactccttctcaattataatttataataatatcaaatatttactaatgcctttcatatacaaggcactctgtttagtgctacaggagataaaaagatttaaaaatacatggccctgaacacagggagcttatgctgtagcaggagagatgagatgtataaccaaatacctatgaaataagatggcccatgatagctgccactagggagaaacaacgaaagtgttatgggcattcataaaatgcctaaaattattttctgaatggaagataaagaagttgttctggtctttgaagacttatatagagggaatggatattattcaagaagggagtgagatgggagataggaaggagagtattttggacaaagggaacagtttaagggaagacgcaagtgggaaaacaagctggtagggaaaggtgaaacaaatgttattcagcttgtctggattatgggacacacacatagtcaagtaacaagaaattattgctggcagactacggcaagtgaagcccactgaaggttgtttcttgatctgaagaatgacatctgatttatatgtaggaagtgagtactgacaagagtagattcaaatataaaatattggaacaatgctaaaagacgctgaaataatccagactagaaggaagggtctgaatgaaaaggaaagactggaaaccttagggggaagaattagtaggcttttcaaatttttagatatgcaggatgaagaaaatggaggaggcaaaagtgcctgaaaagcttgagttcggtgacggaagacatggtgataccattaagcaaaaggaggaagttggtgattatgttggtttgcagcaatggttttggatatttgagtcaagatgaagttgagtgttcagaaggtgactggaagtatgtgtatgaaggaaaagcaaaaggtaggggctaaaagtgaagatttgggattcatcttcattcaaagagttattgaaatcatagaagacagaaagattgctacagaagcattaagataaggagaagagggtcaagctcagatataccatggcaagtcaatgctaaggagataagaggaagagcaggaaccaatgaggttagaggaccagagaactaagattaaaaccagaatgtattgcctcccaatggtaattgtcaatgaggttgaagagcagggtaagtaaagaaaaaaggctattgacttttgtaacaagaacttcattggaacgttgcctgagagtagtttcagaagagtggtagggtgtagcccattgatgaagccatgagcataaggtgaggaagtggagaaagaaagactacccttttgagaagttgggaagtgaaaagatagcgataggacagaaattcaagagtcaaattggattgagagatttgtctttagagatagttgtaggacgggtgtttttgagatagttgcaggtagatgtgtggaaggaattaaagatgcaaaagagagaaatacaattggctggagagcacctcagaagaggtcagagcatagggaagaggagcacttggttgggagaaaggatggaaaagatgtgtgaaagacaagagaaatctaaaggcagagaggacagcatatgtgaggattcaataatcagattttcttgcaaacacagtaggaaagattgcctgttgaaagacaggacatgaacatgaaaggaaaataaaacaaatttatcaagcacagaatgtgacactgagtcaacattggagaaattaaaaagtccaagtgagtaggcttcaggtgaggttaaattgattgaatttgtgctcttcacgtaggtttaagacttgctcttcttggggatgcaatgaatgacaaggggatgggatgcagttagctaagcatggttggtgtagtgagatggcaagaggaaaaaggaattgccggtgagaatattgctaatgtgggtaaatacagggttagaccaaagagggaattcaatgaggcctgatggatttatggaccagaacaacagaggggtcttgaaggaaggaagatatagaaaaggcaaggttgtggttagagaggaaatcccagagttttagctctgggaggtgtaataatttcaaaagaataagtccaggcctggccatgacatgggaagctgaatctctgcaatgttttttcaaatagcataatggatatctttgactcctaccctgaaaccagaaaatattaaacttgcatgtataatcatacaaatgtatgcatacctatttatacatacatttacatattttatacttatgctttcatatattctacgtgagtacaatatactccattttgaaaccttttatatcattcacagaactagcctagggacatagtacgtgcacaatagacgttggtttaattaaactcacatatttaaccagagagcttttatttttttctcctgcatagtactagaatctgctccacctcctaaatcacaacattaaaataattaccgataaaagagttcaggtttaaagtgtggaaacctaatctttaaaataacagtttaaattgggcttagtgttgtgctttttaattgtaccttaattcttgcactgagttctttcaccttctccaaaacacagattctacacaccagagtgccaaggctctgaggaattctactcatctactctgcttttcaccttcagttctttcaggagcccttaaccacataatcaccccagcaattatattcaaagcatgaagcagctccagaaactcactgtacagagctcttgagagatgtagagagaaatgtggaagatttctaactttccctacttattcccagtactgctattctaacccattactctgaacaaaattcttttttcttgcttcaatattgtaaatgagaagccctaaacgtcacagttctctccaaggcatgaaagtagcagcactggctttcaatttaaggttttgggtgagggcctttgtcataggaatagataggctatctcttctaagtcatagagctcacagggccactgtgtgactgaatcaatgtggttggaatgagttgagggtgggatgttctcagatatcctatgattttatacaatactgcaaccccaccccccaaactagaatagaatcctagattcagatcaatattagacattctcagactgactaatctgccattttagtgtcatcccaaacatctgctaggcctaagaaacaattgccccccaggttaagtagcacctgaggtcataagtggctcttttaccagataacagggcaccccctatggaggtggaaagtataggatatagaccaactcagctaattggaagattaattaaactgggacagaaaccagacaatgacagtaaattttattgtatcactaattcaatttgatttttctagctgcctactcagtaacatgtaatggaggagaagcatcactcttctattttctatggaaagaatcatagttctcaacctgccctacaagatactgaatttagaaattcataaattatacactcatatgattgtgtattgaaaataattcctaaccaggagtcctatttaggtgtcaaatgaggcttaaataaaagcaggcggaggccaaaatatggtttaaatgtctttgccatctagaacctgtatccttgttccctactctattgctctcagtgctctctgctcccttcctcttctcttgtatcataacttattcccaggaaaaggagtgagattcctaatgtaaattaggtgattaaatgtatacatccctaatatggcttaatatgtcacctttcctgggattactttcattcgaatgacagacagctcagctcagtgctaaagcaacaaatctgtgtgggaaggtggtagttgcagtggggtgggaaatgaaaaagaccttttcaggaccttcaacacaccatggaccacatagcatacataaggccagacccatcccagtgtgactattcactttcagctgcttctcctccatgaagagctccttaaacaggaggaaaagtctctgacacccaagtgaagaaagcaaaagctctgctgtagtgtgtagcagcctactgagcatgtatttcctatatggctttgggctcagagagcacataaggtatggccacagtccctggaaatgctgaatgcattcatcaatatcactgcagtgacatcatttatgcacacatctgaatcattcctaacatacaaaaacagacattcacagggtgtcaagcaatgacagggcctttttagagagatgatgattgaaagaataaagtgagttctggaatagtttttccaaaagcttattgcccaaacaatctggttattctatctgtaaatcttgaactaactaactaaaaaccgaccaaaaaaaaaaaaaaaatgaaccaaagaaacctagttcttagtgacatgtgcaggtgaccagcactctgcagagaattctcccttgggcaactcctgatggccacggaagaccgggtgagtgatagtcacttaactgtatagacaactcctactgtatcatgtcatacatgcgtttttggcactactgacaccagcaacatttaatggaatcatttgggattttcccctcaatcacaacatggctgtggccagtgcagggaaatacatatgaaggatgtttcccaagttctggctgaggatacacagtgacagattttgaaataacaaagtccactgtacatgcatcactttgaagggtgtgcaaagtctcgactcaggcaaattcaagggtcagattattgtcagtggaaatgctgagatttaagcattgccactgaaaggagttcatacaggaccacactcaccaaccacttctgcaatggaagggaatgatagagggtacaaagcgagaaagcatggattctgaagaacatgggaatattaggtgctcctgagggtatctgcggaatctcacagttttggatggattgggtgttgtttcatacccatctgtgatatagattgggcttatagctgaattcttcctcatgcattttacttgcttgttattctggaattaagtaacatctagattttaacaatgcccagccttcctttctttaagttttcttaagcagaccatgagtaacttagtcccagtgcaaatatccagttgaagaaaagcaaccaactggggccaaataagtttagaaaaataaaattgtccagctaacagcttttatgatgggaggataggaaaaaatgtagtgaatatactgggtaaatggatttggaaattttatcctgtgatagaggctgccaacctccacaaagccaacagtctaggaaaagaagttctatttgtctggttaacccaaggccagattatgaacacctggctcgaggccagtagcaccttcctgatggcagtaatgaggacaaggcaaataaagagccgctattggcaccattgctcacatacccaccctcccacgtctaaacctaacttcagcaatcttgctaagggaatcatctcaccactgagtttctagtggatcccatcatcttttctagaaaagcatgcaaatttgtaagacacatatccagcactacctctctgtgaccagatatcacatgcttcaaaaagtagagttagtggagatttttccacgtgtgtttgccaggctgacttctgagggtggagatggggcagggagtgagtcagcgcccaggtcctaaagaagaaaagactcagatgactgagacgattgtttcagcatcagaggaggccgctgggagatttctcaggattgagcttcctgaaacctttcagtcacgccaagaatgggaagttaatttgaccttaattctgtttaagcccttttgggaatctttcctaccctaggtactgacagaggaaatatggtgccaccagcctgtctttgtgtggaatgtggtaacctagggtctacctagaagataggagtcagacctggggtttgcttagagccaaattgaaccctatgtaaaaccctggccaaagtgcatgaacatttctcacaaaccagtaagaagactggttttctgggggggatggacacaattactttcccctggctttttcaccatagtggcctccatgagcattcgctttttccagacaccctgaagcaaaaaagccatacaaaacaattcccccaatgggaaatgaaaacccataacaaaacactttttccctctcattcccatcaccaccccactccctccagcccaacaccctgaatactcacaagagaacactttatctatacaaaattagaaaacaaaatatttacatatgaaataaacaccatcttgatttctgttgccagcggagactgaaagagctcccttggttctagattgctgttcgctaggttagttggtttggtttttttgtttgaaaggggtgaggtaagaggaagatgaggggatgagtccctgacccctggacagagtcagggcgaagcagtgtttacgtggcccttcgccttcttcctcctggaggtgcctcatgccctctgtcctctctcagtcttttctgttatctaaggtaaagcactccgtgctcctctcaccaaatctgtgagaggttcagccccttgcccccatgttcattttagaaagaaaacaaagctttacaaggccttcagttggctttaaaatgaaagatactgaggtaaaaatcaaggaggagggttggggacagcagtcaagggcgggatgaggaagggtcacgagtgagggcaaacaggggcgaagagcagccctggagggagtgacttgaagagacatggcagcttccttccagaggaggatgagcacctttctggtttatgtgtcctgtgtgcaacatggcgatcctgcagtcaagcttccacacagacctggggctctctggatgccaccctgtgtaggggaggatggcaggacagtggaactgacccatagaataaatagccctaccgcaagtttcaggaccggcagtgatacatattcatttcccttctcaattttccaatgttaagtgaagggagcatcagttctgctggtaccctcatccctggagttttatacatgtatatctttttttattcctcaatggtacaatctgagagggaaacaaggtgttgcaggaaggtagaagggcttctaccaagagtgttcactctgggctcaagtcacattcccagggagccaggcccaaagaggtggtggagggtccctctctgcccccgtctcccatttccaagtctcttcccctcttttcgtacctccagagctgcactcatggagtgcagctcatttctcttaaaggtcaagctcatttctcttaactgtctgctctgtagcagttgtaatcagttttggggggaagaagcctgctcgtctagcttcaggttaagtaagaagggatcaaagcattggaaacatccccctctctcacttaccctaccatacacgactccttacttcttcaaaggtggcttcgttcttccccaaaccttggccagtcgagagtctaaatgctcaaaagagctttgtagaatcttttgctcccaagtgtgggcaaaagaatcatggctgtgaaaattcggtttccctttagccttcctggaaagttcttggttcaaactggttgaaacaattgccaaccactgaggacttgtttatgtaccttgttcttgcaggattgctcaccgcctttttttgtttagaccacagaatcttctttatcaagaattttcattctccttattccagaaggatgaagggagacacagccaaaattcaggtaatacatggccatctctgtctgtatataagccaaacaatcacactgcttggggatattgaaagaaacaatagaaagagtcaaggttgccttctcttgaggcacctgactacacatgggtgcaagtgtgcatgaacacacatgcacgcacaatccacctgctcttgtccccaaggcaccgtgggacactatcataacgtactttccagtttgttcaagaatccactctgccaccaatgaccttttgttctgttcaccaccactatcgagtctcatggggttgaagcaagcattttttggcttatatataaacacaaatggcctcccaacctctgcttggcacatgattcctagacagatgtcatctaagcagcatgaatttagccagagcctctttcctttcacaagcagtgtgctaaatggtctcacatagatgcttttgcttcctcacctaaatgaaaagatcagtttgggaaaagctacctttgtgctcacatagcctctttttggttctcccagcttcactcaaagaggatatcaaggagctcttccacaccaggaggaagcccgcatgcagcccttcctttctccgctctaccctcccctgctgagagggcccatggcatcatctcatgggaacaggaatggctgacagcggggggaagaaggagagaactgtgaaaaggaggagagatggtgctggtcaccagggttgcccccagtaggaaccagaactccaggatcccataaataaattaaaacaagaaaggagcaaatgggaaccaagttcacccccgtcaccctccgtgacatgcgcatcacgcgacccacagccttaccctcccgtacccaccttaacctctctgttccctcactcagacatcagactcaatactagaaagtttctcataaacatgcccattgctggagccattgaaagccctggggtttttgttgttaggcacacaggggttggactggttccctatacagatgtccttctggaaacgggctggcacggccccatgaagggccgagaccaccggcttgttggtgacaagggcccggaagtccggcctggctttcgacgcccccgccaccgtgggctgcctgaagaagtaggatttgctgccatggagcaagcactggtcgtccccaaaagtggggatgaaagggttttgcgtgacccggtcagggtagagcgacttgctgagcatgtacccgccgccggggttgttgtggtggtgatgtccggcagtgggcactgaggacttgttgttggcaaaggtgctctcgccagctgacatctcaaacatgtgggcgtaggggctcccatccatgaatcggcccttgtctttcaggcttacgctgcgcggggccagggcggcttcttccttctgcaggtccacgaaggtgtcgtaggagtgctgccggcgcagtttgttccggttcttcttctgggccttggaattagtcgggctctgagggtacttagtggtggaggcgtttgacgtcaccgccactggggcagccggctggtccagttcctgcagggagttgtcctcactgatgtcatacaggttgcctgctttcttgcaagcctcacaccggatgcacgcctgcctgcccgagttctgacccgtcaccgtcgtggagtagttgtgcagcttggagggacagctgcggcagaagttgcccccggaccggtcctcccactccacgttggtcaggttcttctcccaaggtgcaggtaccccgctgaccacgccgtgtttgtcgcccgtcccgtgcttgatgtgagacctgttggtacagggccctcctccgctgacggagtcgcgcttaaagtcatcactccgctccttgtagatgtcggtcaggtctacgtgctcccagtggggtgagttctcctttgttcggaactggtccaggtagaagtcccgtagcccttccttgtccctgaagtagcgcttgtggtcaggggagcggggcggtcggcgacggtaggccagctcgatctcgtcaaactccctgcgggacttggccgaggcaggccgcttcttcaggctgtccttatattgctgcttacgcctcttggcggcattgccctcgatgttcccataggtgacggtgtgggttgagatgtcagagacatcggagcggatcaagtcgtcgtggccactgtagcggtcgctcttgaaggagaatttgccgtacaggtcactgagctggctgtgcttggaggaggggaggccgatgtccaggggcttcttgctgatggacctggactgggtggtgaagggtgggttgtcacagtcgtagagcccatcgatggagctggcactgccaatactatggggccggtggtgatggtggtagtgatcttggtacacgttgctgtccttcagctgcaggttcccgaacgttctctctacctcactgatgtagtcactgaagaggttctcctcacagggcgggttgttgtaggatttgcagtcagaatgcgtgaagctgcggcggtgctctgagatgtcatagacggatgactcccgtcggatgaagtccagggcgctctgcggtgagccattcacaccagacaggttagccatgttcttggccgtgcgcagcaggcgcaggatgttggagtgtgtgttgttcatggttgcggtgggggagttcattacagactggcgctcctcgatcgccaccccatggatgcagctgtagatacctctgctgatggagaagaccatgccaggcttgccagaacagacacccataaagcaatgtcggaactgccaatagaaaaggtgttcgcagatgaaggtgatgaggctgagagccatggccgcccccaacatgtagaagacccctgccatgttgtcaatgtccagctggctgctcatgacctcattcttctcattgtgacaaatgccagtgagccagagagcttccagttcttccatctccccatctccaaagagctgcaggatagcaaggtccacctggcgcttccacccagaatctttttggatggcaatgccatagccagtggaagcaaagaccttcccactgccaatggtcaccagcttgcagccttcatctctgcctgccatatagttcagcactgctgcatcatagatgaaggcatccagtttcctttttgtcgctcaggccagaaacctggtccacatattcctcttggatcatgaaggcagctaagttggcagtgtagc

SEQ ID NO: 12299 - RNA, 6147 nt, Homo sapiens
  source 1..6147: mol_type = other RNA
ctgggaggtcaaggctgcagtgagccgtgatcacaccagtgcgttccagcctgggtgacagagctagaccctgactcaaaaaaaacaaaaacaaaaaaattctttggtttacccagcccatttctggaggtgaccattgttaacttgctggttgtcttaccagacgcttcttctgccagtacaaacgcatactctttgttcacatatatgtgtgttaaaaaacaaacaaacagaaaaaccctgatccttgaaggtaaaaatttctgcacttgctcagggaggccaggaacctgaaggtattcagaacagctcaggtgtttgtctgtctgcagcccaggtgatctgacatgcttgtgggctttgcaggcagagctacctgcccccatggcccctgacccccaccttggcagaccctgagggcagctgcctggcctgacgggcgcagtgaggctgggaggggtgggggtccctgtggggggtgatttcccagtcggtttcctgagatctccctcggaccagagcaggagtgtggctgcgcctccctgccccacttccagctaccacaggtcatgtgccctggagcagtctctcctggcctcgcagggtcatggctgtgggacgcgggcgtgtccacaggccaggccagtgtctgacacacgcatgctgcttgtcctctgtcaccatgggccgtgtccttccggggcggctgcttgtgtgacctggtgctgctctctgctgtcacagctcccctgcgctgctgttccggctcagccaggtgtcctgggaggggtgggctcctctcctctgagtgaggactccctaagcccggtgggtccattaggccttgggggcaaattgggaaacagggtccttacccaccgggtgggggccgtcctgaggtctcctggagctccctgctccagccagggagaggcccccacctgccttcccgcccgcctccagctcctgcaggtcacatgcctgagcctcacaggctcgtggctgtgggatgcaggcgtgcctgcgggctcggcagtgttcgacacatgtgctgcttgtcctgtgtcaccaaatgggcctgcagtctgttgtgggcaggaggtaggcagtggcttcagtctttctccttctccagggaacccggccctgggcctgcagtgcaggtgctcagttctgtgcccgggctcctgactcagggggtctaccctggctctggggacccgcacttctaggcagtggggtagagttgtctgggcctgccttgtctgtggggtggggccatcccctccagaaaggacagtgtcctgccctgaagctggctttcgataggtccacgttcacctggaagctggtggcgcccatgtcatggtcccctgtggcttctcctggggatcacatcatctctctggaccagccctcaaccctcactgtcacaaggcctctgccacaggccccccgccaccacttagcactctccctgctgaccccctggtccattcagcccctgggtggcccccacacagtctgtgacagggaggaggctgggaggggcactgcctcccacaaggagctcacgttctggtgggaggaggccaagaatcaggaccaaggagaacttcagtgaagcaaaagaagaaaaatggaacaggggtgaaggggctggagaagcctcagggaggtgacagctgaaacctgcaccaggaggggcggggcctgtagtgggcactgggcagtaggaccctgtggtgagccaggtctgctcaggtaacaggaaggtcgttgggccacagtgtggtggggactgccctgaggccgggtggctgcagctgggcctggtgtgggggtggtggccttgcctgggggcccctgcagggctggcctagcagggaaggtgtccacaccatctcagctctgggcaggtggggtggacctggggcttatccaccgtctagaaaccacttggaggccaggcagccttggctactgctctgtggctgggcctccagggccctcctggtcatgcagaatggggcagagccggagcccgttgggagggagcctgggctgtgcgctcggggtactgtgaagtccctggaggcctggacccccatcctttcctgggtgggtcagggacagggtgggacagggacagagggcaagggtgagagggtagagagcgggcaacaggtagtaacagccggcccttctctcccagcacagcgactcggactccgaccccgagtactccacgctgccgccatccatccccagtgcggtgcccgtgaccggcgagtccttctgtgactgtgctgggcagagcgaggcctccttctgtagcagcctgcactcggcccaccggggcagggactgccgctgcggagaggaagacgagtgtgagcgtggggcccagcccctgctgggactgcactgcgggcgggcctgggggtgggcagggcagagccccatggagctctcagggctgccccagcctgggcctctcttgcagatttcgactgggtctgggatgacttaaataagtcatcagccaccctgctgagctgtgacaaccgtaaggtcagcttccacatggagtacagctgcggcacagcggccatccggggcaccaaggagctgggggagggccagcacttctgggagatcaagatgacctctcccgtctacggcaccgacatggtaagttgcttcggcccagggtgcttctggggaacctggctccggcagcccagccccgcgccctctgcctggcccctgttcctagatggtgggcatcgggacgtcggatgtggacctggacaaataccgccacacgttctgcagcctgctgggcagggatgaggacagctggggcctctcctacacgggtgcgtgaggcccagggtggggcggggccgagcctggagctcccgggctcactgcgaccctggctgcccccaggcctcctccaccacaagggcgacaagaccagcttctcatcgcggttcggccagggctccatcattggcgtgcacctggacacctggcacggcacactcacctttttcaagaacaggaagtgtataggtgaggccgtcacaggacttgagctcctctcagctgtcaccccgagggaggcagccaccccgccccagcccaggggacactgaggttttctgaaagggttcctcccagaagcctgaggccccagggtcccagggggtgggacagtgaggccaggctggagtggcagggccagcgcgtgcaccctgccttgcctcagctgtgccagctgcccacccgggtgactgtagcgtgaggtctgaggggctgcgcccagtagctggccccttccctgcctggggttcaggctgggcccctcccttccaggtgtggcagccaccaagctgcagaacaagagattctacccgatggtgtgctccacggcggcccggagcagcatgaaggtcacccgctcctgtgccagcgccacttccctccagtacctgtgctgccaccgcctgcgccagctgcggccagactcgggagacacgctggagggtctgccgctgccgccgggcctcaagcaggtgctacacaacaagctgggctgggtcctgagcatgagttgcagccgccgcaaggctccagtgtccgatccccaggcagcgacctccgcccaccccagcagtcgcgagcctcggccctgccagaggaagcgctgccgccggacctgactgacttcccagtggaactgccttcttgggctgggacagcccctttcctctgtcccttctttctctgtcccttccttccagccacactccagggcggagttggatgaggcccgtccggagggagccatctcttgctcccgaggctgggacagtcctttctgtgggggctctagggcccctctgctgctgtgctgggtggggaagcggctgccctgagccccaggtcttgtgggaggctgcgaggacgagagcctggctggagcccgcgttgctgttcccacagggcctcggtttttcctaacttgctctgcatgctgtcagcggctgccccgccgtcatagacttaaaggactgcaataaatgtagagttgatgtctaacacccacatggcgtgagctgaaacgtatccgtgcagaggccgggcttgcgagcagcctgggccttctcccaggcctcactgcccctccacatccttgggagtcccctactgcttctggctgagggtgccacaccccaagcctccaggtggcagtggggccctggagctgccttctggtccctgccgagtgtgtgtgtgtgttgggggggcacagccctgctgctgaggcctcccctggggcctacgtgttcaggactcagcacaggaaccgccagccatctgccagccagaagcccctcttctcccagctacctaaaacttcccctgcaaccacccacccttcccctgaggtcagacctgctcagccagagaacccacccaggctgagggtccacatgtggctgggggtcctcccccaccgcccagggtgtctggtctgtccccaaggctgcatgctgtcctggtggtcccacgtgtggtcaggagcccaggtccagcaggagatcagggttggctgtggtcaggaagaggcagatgcggcgggagaggtcaggccccaccctgcggggacgcccgccttcactgggcggcacaggaaggtcggccaggaggcccatgcgctcccgctccgtgctgcaggcctccagcgcctgctgcagaaggcggggggaggggaaggctgtgacaactgcatcagccacggctgggctgacccgactgaactgcctgatctgcctccgccaggccgcctgcagccctgcgccgtctcttgccactggctcgccggctgcccagcgccctgctgtgcagaaggagaaggcctgggattcccggtactgcttgaggggatactgggcgagagccttggtaacggcgcacacgtgccgactcagctcctgccaagaggccaccagtagcacgtccaggtttgcccagagctgcaggagtaccagggcctcttccacctccggccagctgacggccacctcggcaccggccaccttcgggctctctggctgctgtgtcccccgggaaacgtgctggcgagaccacaggtaggcatccagcccgatgacagccaggtggggccgggcggtggtctcgggggagatccagggcacccagtgggttgggccagagatctgggtcagtgtggcgacgccctgcagaaactcctcgggctccagcagcagcagcaattcctgttcacctgcagcccacacttcaggaggcaggctgcgggggcaggggtcgggactcgctcgggtccaccgcaggctgcgggccgggcgctggggctcgatgcggcactcgcagcccagggcctccagggcctccatcaggacgtcggcaccggcgtcttccaggatggctgtgtccacgcacaccgcgaggcgcttcaggacctgctccggccgcagcagccgcaacgcctcggcagccgccctgcgctcacccgctgggtcccgggctctcgcggcggcctccgagccggcggagtcctcagcgtcggagtctgagatctcccaggttggaggtcgccgctgaccgctcccgccccgtccccggccccggccctggcaagagacccccgccctcccgggtccaacccgcgccatggccggaccgacctcttcctcgcttccggccgcgaccgaacactttagcctgggacaccggcctcttccggtgacttccggccggaccgctgaggacgcggacccgccatggcgcggaagaaggtgcgtccgcggctgatcgcggagctggcccgccgcgtgcgcgccctgcgggagcaactgaacaggccgcgcgactcccagctctacgcggtggactacgagaccttgacgcggccgttctctggacgccggctgccggtccgggcctgggccgacgtgcgccgcgagagccgcctcttgcagctgctcggccgcctcccgctcttcggcctgggccgcctggtcacgcgcaagtcctggctgtggcagcacgacgagccgtgctactggcgcctcacgcgggtgcggcccgact

SEQ ID NO: 12300 - RNA, 65 nt, Homo sapiens
  source 1..65: mol_type = other RNA
ctgggaggtcaaggctgcagtgagccgtgatcacatgactgtactccagcctgggtgacagagcg

SEQ ID NO: 12301 - RNA, 668 nt, Homo sapiens
  source 1..668: mol_type = other RNA
ctgggaggtcaaggctgcagtgagccgtgatcacatgactgtactccagcctgggtgacagagcgagaccccataaagtcttcaacatgagaccctggaagttgctgtgttagttccaaaggcccagcagagaatctacgaagggcagaggcagcccaaagacctgaggaagagacagacacttttatcctcatgctcagatacaaacacaaagcaagaaaaacccaagcccttcagtagtgggtttgtaatcaactgggctctctctcctttagaggcacttgcctggaagaacagatactgttcaaggaatgacaccttttactgccttacaggtaaaacttccattcataatagatgaaaaattgaaaatgtttaataagaattaactaatttaggaagatcataatctcagcaacgtgcaaaaagatggtttaacaagttatttgttattgtttttcttgtcaggttgttcaagctcataaaaacatacattcctcggtcaagtatactacaatcagccctcctctttcttccttgagtaactaggcaagttctcaagaaatatgatgactcttcagcaccagagccaagcatataactccacagggcaccccataaaagcacgcaaactgaacttaccaccaccccctgctgatgaggaggaa

SEQ ID NO: 12302 - RNA, 861 nt, Homo sapiens
  source 1..861: mol_type = other RNA
ctgggaggtcaaggctgcagtgagccgtgatcacatgactgtactccagcctgggtgacagagcgagaccccataaagtcttcaacatgagaccctggaagttgctgtgttagttccaaaggcccagcagagaatctacgaagggcagaggcagcccaaagacctgaggaagagacagacacttttatcctcatgctcagatacaaacacaaagcaagaaaaacccaagcccttcagtagtgggtttgtaatcaactgggctctctctcctttagaggcacttgcctggaagaacagatactgttcaaggaatgacaccttttactgccttacaggtaaaacttccattcataatagatgaaaaattgaaaatgtttaataagaattaactaatttaggaagatcataatctcagcaacgtgcaaaaagatggtttaacaagttatttgttattgtttttcttgtcaggttgttcaagctcataaaaacatacattcctcggtcaagtatactacaatcagccctcctctttcttccttgagtaactaggcaagttctcaagaaatatgatgactcttcagcaccagagccaagcatataactccacagggcaccccataaaagcacgcaaactgaacttaccaccaccccctgctgatgaggaggaaggaaccatggcacagtccacagacaccaagtttaaagcacatctaaacaaatgggcatcagagtgaaagtgggcaggcttggagttaggttaatccccaaacaaatgtggctgcagcctcagcaataccatgtagaaaagggatctttgccaaatgcagtggctcacacctgtaatcctggcgcttgtggatg

SEQ ID NO: 12303 - RNA, 875 nt, Homo sapiens
  source 1..875: mol_type = other RNA
ctgggaggtcaaggctgcagtgagccgtgatcatgctactgcactccagcctgggcaacacagcaagacttggtctcaaaaataaataaataaaagttcatccaattccaagatcagaaatacatttgatgagcaataaaaggggaatgaaactacaaattctaacagagacctttcataaatctgaaagatagggtggttgtttctgcctgggacttcatggagaaagagcaacatttgaactgaatctggaagttctgagttggccaggcagatggcgatgggggtgggaagggcaaagccagccacatatacacatgtggcatgaaggaatgagacagcttgatggattctgggcacagttgtttgggatggctgtgatacaggccacaggtgggaagtactgagagatgaacctcattgacctctccatcatccggtgactcattgtagtcattcatctcgtccatgtcctgcatatcctcatcatcctctgagtcctcttcactatcctcatcatcttcatcatcctcttcttcctcgtcatcatagtgctctgaggctggcttgccaataggaaccaggttgttgtctttctccgcgatgctttggagccaggcctgatgctgctgttcctgctgctgcagctctgtctcttccacacagggtcgatccagattaaaccacagagtctcagtcacacgagggaagagtgaggggaacaaagtggacatggctcctagactggctttgagtcctggctccaccacttactagctgtttgaccttggctgagtcacttaacctctctgagcctcagtgtcttcatcgcgccgggaggctgctgccggcggcgacccggaagcgcttcaccc

SEQ ID NO: 12304 - RNA, 454 nt, Homo sapiens
  source 1..454: mol_type = other RNA
ctgggaggtcaaggctgcagtgagccgtgattgtgccgctatactccaccagcctgggtgacagaatgagaccctatctcaaaaaagagtaaagccttctctgattagtaaaggacagacaggatgagagcagtgccagaaggcagaacctcgctgtcatgaactggagcctgttgatgatgaggagaccatgcagggcttgcagccaaaagaaggaagctgaagggatgtaagcaagtcagattcagatgagaatctggtggtgagccacactctgtgctgtcattgttcacttgtctatgcttctcactagatcacaagctttgggaaggcaggaactcttttgtgtagattgctgttgaatcactggtgcctgcagagtgactaactaaataggtgctctctgacattattgaagaatcgaattaacgagtatctgctacttgtttttttc

SEQ ID NO: 12305 - RNA, 293 nt, Homo sapiens
  source 1..293: mol_type = other RNA
ctgggaggtcaaggctgcagtgagccgtgattttaccactgcactccatcctgagcaacacaacgaccctgtccaaaaaaaaaaaaaaaaaaaaagagtcagccacttttgcaggcccttcaggtttattaggacacttctaacacaaaacttgatctaattattcagaaaaccagtgcggcagaagcatcctatttcctttgcagcacactgtttaggtgcaagttttgtattgccagtttcaggtggattattccaccttcaagtactgaaggggaatctgtagagaaaga

SEQ ID NO: 12306 - RNA, 1611 nt, Homo sapiens
  source 1..1611: mol_type = other RNA
ctgggaggtcaaggctgcagtgagccttggtcatgccttggtcttgctctttcacctatgccacccagccttgggttgaagagcaagaccatgtcccaatttaaaaaagaaagaaactttaaataactatatttgaatcatttgcatagtcatgaatattttaagtctgtttttaacatttttattattgatttgtacaattagaatcagaataagcaaaaaaaaaaaaaatcaaaaggcaacaaaaaaatctacataggccaggtgtggtggctcatgcctgcaatcccagcactttgggaggccgaggcgggtggatcacgaggtcaggagtgcaagaccagcctggctaccatggtgaaaccccctctctactgaaaatacaaaaattagccaggcatggtggcacatgcctgtaatcccagctacttgggaggctgaggcaggagaatcgcttgaacccaggaggtggaggttgcagtgagccgagaccccgccactgcactccagcctggcaacagagcgagactccgtctcaaaaaaacaaaaaaaatctacatagatagcttgggttgtatacccatggcaggatgtattttccagcctcactctgcctctgcatgtagtccacttattccttttgtccagacatgaatgcctgtattgcttcacgcgagggtccgtggcttcattcttgaagtcagtgagaccaagaacccaccaattccagacacataagcagcttcagcctctctgtcaaggagaactggaaagtgtgtttcctgtctaaagggtatagctgcaatgctgagccaatatttccaaatgtgttcactttcctttttattggggttgttttactcttgttgagttttgtttgagttccttgtaaattctcgatattagtcctttgttggatacatagcttgcaagtattttctcccattctgtaggttgtctattcactctgtaaccccagttactcaggaggctgaggcaggagaatcgcttgaacccgggaagtggaggtttcagtgagccgagatggtgcccctgcactccagcctggatgacagagcaagatgaaacttcttgctcttcatttgtcctaactccagggaatgttctttactgtctctcaaaatattgaagagggatttccttctgcttctctggtggtaatttgcttagtaatcacattttattgacttcctttctggccttgtctcatgtgtccgtattctaccagtgttttctggacattctaaagttttaagcggtttatgaaattcagaggttaatatcataaagcaggcttggattttcatgcccatcagaagtcctgagtagtggcagtagagtgaattttcagcattaagtgaaatgtccgaagtcttctctcaactcgtggcacctctgaaatcctcagcaaatcctttgagatatgatgaagaaagcagtttctacagaacttcttgagttctctcctctttaaaatagacattaacacctgtatgcttgataagagtatggtggtcttaatcatgcagcatccggataaacgacacctctacaaagtcacttttgccattcaatgtaacatagctctat

SEQ ID NO: 12307 - RNA, 4873 nt, Homo sapiens
  source 1..4873: mol_type = other RNA
ctgggaggtcaaggctgcagtgagctatgatcacctcactgcactccaggctgggtgacagagcaagaccctgtctcaaaaaaaaaaaaaaaaaaaaaagatatgggtgagattcctttaattctaataaaatacctactttataccaatacattagaaaaattaagtaaaactgatgactctccagaacgatgtggatttccaaaacatgcacggaaaggtgaatagctcaaggataccaagtttgccaaagatttgttcccaactgggcattgggacttgatggttttgcaagttgagttctagcaaacccttcaaagtgaaaataagagttatcagaaaccaggctgtgagcactgtaaaagggcaggaagtattgttttattcaccactatatccccagctcctggcagagaacctggcacacagtaaactctaaataaaaatctgttaagtgtgccgggcgcggtggctcacgcctgtaatcccagcactttgggaggccgaggcgggcagatcacgaggtcaggagattgagaccatcctggctaacacggtgaaaccctgtctctactaaaaaaatacaaaaaaattagccgggcatggtggcgggcaactgtagtcccagctactcgagaggatgaggtaggagaatggagtgaacctgggaggcggagcttgcagtgatctgagattgggccactgcacttcagcctgggtgacagagcaagactgtgtcttaaaaaaaaaaaaaaattgttaagtggctgtaaagggaacatttcattagagtatttgtgtgtgtgtgtaattttcaaagatagatatatttttagttatagaaactgaaaacagggctgggcacagtggctcattcctgtaatcctggcactttgggaggctgaggtgagtggattgcttgagcccaggagttctgagatcagcctgggcaatgtggtgtaaccctgtctctacaaaaaatacaaaaactagccaggtgtggtggcacacgcctgtggtctcagctactagggaggctcaggcaggaataccacttgagccccagaagtggaggttgcagtgagttgagatcatgccactgcactccagcctgactgacagagtgaaactctgtctcaaaaaaaaaacacctgaaaacatttctggagcaatatttatttttagagtccctcgaatacagaagtgaaaatgtactattcaagacttgtatttaacttcataaaatttctttcctagatgggtattacctcttattaaacaactaataaaatatgtgctatataatcatacatttaaaacatggaaagacaactaatatcttacagtacatgaagacaaacttcaggagacaaacattaaatatatccaaaaactaaatggacctggactttgcttacaaattgcttaaatggaaatgaaatttgtgtttaagaaatgttttcactgatggaaaaataaatctaacaaaaccattatgtaaaaacatactgatttacaaagccaatgtgtctcagttttaatttgtatataccctagatgaggtttatattaaatgagaataaaatattaaaagtccatcaatgtgtagaaaagaaatacagctgctcaagtactagatagaacttcatattctttaaatctatttctagaactgaattgactttttaaaattttataatttatcaactactccttaaggttattaacaatagcaggaattatgacgacatattatgtcatttgtttctcctactgcttttatctctacattacaatataaaattttcaatccagcattttatagctctgtgtttaagttaattagtaccttaaaaaaataaaattctaaatataaacttggtggattaaggctcagtaaacagtaatcaaacaaacaacagatttgtcctcacaaagagaatatgaaagccaaagttttttttcttttgtgatcctgcttcatattattctgttctgtccaatttcttttctgtagggaaacgccaaagagatataaaaaagagatataaaacagtggtgagtggcttccaaatgactgtttgcccttgctttttaagccaaaatcctctaaaaataggtctttaattctggcagcagattaggacaaatgctcaaaaattcatgttttcttcaaaaaatttcaactggcgagctttcacactgtaagttgtatacttttcacccatgtgctcccgcaaacgtacctctctatcaaattcatcctcctcctccaaaagatcatacacctgctctaaaagctgaactcccaggccacgaattacatcagttctcaagacttcaactagtctcctgatcttttcagaacctggcataatagctgaaggtagctctttaaaatggatttcctctgcctcttctgcaaccttcccatgaagtatcagtgtgtcccgatatttccgatgaagtttgaattctgacactgggtttgctaccgggacatcttcacagctctctttagaatccagtttcagggtctgagtcatcaattgtaccaaggcattaatttcatttgtctgacctttcccttccccgtaatccccatctgacttatcagttgaacttgtagaagaacttaactcatcctcagacagacaatgaatctgtttcctttcctgagtgacgctgcagtcagaggagagccgtcgggcaggcaagggctggtcttcttcctggggttttcctggccctgctacactcagagacgctttcctcactgaagggcctgaagaggacatttcttcctgtgactgctttagtcgcctcctctctctggctgataatggtcgatcctttgatgatgacatctcactgctccttgaactgctcacagacccagtgaccactctacgttggttttcagcctctttttgtgttgatgtgacatccactttcccaacaatgggatgagaaggcaaaaatcgaggaggcgactcttggaaagcaaagagatctctgcggacctgtctcttttcccctctgtgctcagtctgttctctcctcttttgccgtcgctgtcgagacagggaaggttcagacccagagttgtgtggctgtaaatctgggtggattctgccctgtttttctataatacattcaccagcaacttgatcctgggcgtggtggcacacgcctgtaatcccagctactcgggaggctgaggctggagaatcacttgaacccaggaggcggaggttgctgtgagccaagattgtgccactgcactccagcttgggcgacagggcaagactctggtcctttggcttttgttctttgattaggggctgcagaggcttcactggttcattcttttccccagtgacaatgtcagaggaccacatgggaatcaggttttcaggctgggcactggatttagtgttgtcctgcagcatctcctcttccacttgagaaatactgcatatacctcctaactcattagaggcatccaaatatcttggctgattctcctgaacaaagccatcactcactgaatccctcccttttgcaggtaagatgtcaatatttacgctactgattgtggctagttctgtggtattgctcaagtcctgtttgcaggtatgggctttcagactggcaggtgacttcaagagaccagaggccctgggtttctcctgggacaaacatttgccttcacccattatatatgtctgggagccctcagaagagagtggttgggggtggattacttcatgatttgattctgcctctccagaaaccactgtagcaaaaggcttggattgagagtcaccatttttaatgttatttttggaggtttttatctttgtggcctccaaaaagaaggagatttgccgctttatataaggctgcctcaggatgctcctcacagacggcctttcttcaggccttttgctcagcattgttcttatcagttctgccagctctgggctgtaatctcttggcattggtggcagctttccttcaataatccgataaactaaagaattcatatcttttgcattgaaagcatgcttcaaggtggccatttcatagacacagcatcctagagcccaaacatcagacttatagttgtagggtttgtttgagaacaattcagggctcatgtagtagggtgtgccaatgagggtgctagccatgtcacagtggttctctaacactcgggcaattcctaggtcccctactttgatgatgtttgttcttgttaggaagacattttgagttttcagatctcgatgaaggatgtgtttttcatgtaaatactgcaaagccatggcgatctgtacaaaccactctaccacctgattctcaggcagaagctgccctttctgctccttgagctttcggtacaaatcacctccttcacagaagcccatgacaatgtagagcagaccatctcctccttcccatgactccttgtaggtgacaatgttgggatgcttcaactgagacaagagctgggcttcctgttcagcagctcgccgctctcggctagaggcatttcggaggttcagttttttgatgacatactgcttgccgtcccgccggtgcttcacaagcgtcacctctccatagctccccttgcccacgacccgcaggtagcagtaggcggccaggggcatgttcccagcgctggcccagagtcgggatgcggcggcagcggcgggtagggcagcgggcggcaacaagaagctcggttcatgcccgagagggggcagtgggggcggctgttgaggcagccgggcccgggcgggattgctggggcccggcccgcgacgacgccgctgccatagcgatccgggccgggagcagttct

SEQ ID NO: 12308 - RNA, 4835 nt, Homo sapiens
  source 1..4835: mol_type = other RNA
ctgggaggtcaaggctgcagtgagctatgatcacctcactgcactccaggctgggtgacagagcaagaccctgtctcaaaaaaaaaaaaaaaaaaaaaagatatgggtgagattcctttaattctaataaaatacctactttataccaatacattagaaaaattaagtaaaactgatgactctccagaacgatgtggatttccaaaacatgcacggaaaggtgaatagctcaaggataccaagtttgccaaagatttgttcccaactgggcattgggacttgatggttttgcaagttgagttctagcaaacccttcaaagtgaaaataagagttatcagaaaccaggctgtgagcactgtaaaagggcaggaagtattgttttattcaccactatatccccagctcctggcagagaacctggcacacagtaaactctaaataaaaatctgttaagtgtgccgggcgcggtggctcacgcctgtaatcccagcactttgggaggccgaggcgggcagatcacgaggtcaggagattgagaccatcctggctaacacggtgaaaccctgtctctactaaaaaaatacaaaaaaattagccgggcatggtggcgggcaactgtagtcccagctactcgagaggatgaggtaggagaatggagtgaacctgggaggcggagcttgcagtgatctgagattgggccactgcacttcagcctgggtgacagagcaagactgtgtcttaaaaaaaaaaaaaaattgttaagtggctgtaaagggaacatttcattagagtatttgtgtgtgtgtgtaattttcaaagatagatatatttttagttatagaaactgaaaacagggctgggcacagtggctcattcctgtaatcctggcactttgggaggctgaggtgagtggattgcttgagcccaggagttctgagatcagcctgggcaatgtggtgtaaccctgtctctacaaaaaatacaaaaactagccaggtgtggtggcacacgcctgtggtctcagctactagggaggctcaggcaggaataccacttgagccccagaagtggaggttgcagtgagttgagatcatgccactgcactccagcctgactgacagagtgaaactctgtctcaaaaaaaaaacacctgaaaacatttctggagcaatatttatttttagagtccctcgaatacagaagtgaaaatgtactattcaagacttgtatttaacttcataaaatttctttcctagatgggtattacctcttattaaacaactaataaaatatgtgctatataatcatacatttaaaacatggaaagacaactaatatcttacagtacatgaagacaaacttcaggagacaaacattaaatatatccaaaaactaaatggacctggactttgcttacaaattgcttaaatggaaatgaaatttgtgtttaagaaatgttttcactgatggaaaaataaatctaacaaaaccattatgtaaaaacatactgatttacaaagccaatgtgtctcagttttaatttgtatataccctagatgaggtttatattaaatgagaataaaatattaaaagtccatcaatgtgtagaaaagaaatacagctgctcaagtactagatagaacttcatattctttaaatctatttctagaactgaattgactttttaaaattttataatttatcaactactccttaaggttattaacaatagcaggaattatgacgacatattatgtcatttgtttctcctactgcttttatctctacattacaatataaaattttcaatccagcattttatagctctgtgtttaagttaattagtaccttaaaaaaataaaattctaaatataaacttggtggattaaggctcagtaaacagtaatcaaacaaacaacagatttgtcctcacaaagagaatatgaaagccaaagttttttttcttttgtgatcctgcttcatattattctgttctgtccaatttcttttctgtagggaaacgccaaagagatataaaaaagagatataaaacagtggtgagtggcttccaaatgactgtttgcccttgctttttaagccaaaatcctctaaaaataggtctttaattctggcagcagattaggacaaatgctcaaaaattcatgttttcttcaaaaaatttcaactggcgagctttcacactgtaagttgtatacttttcacccatgtgctcccgcaaacgtacctctctatcaaattcatcctcctcctccaaaagatcatacacctgctctaaaagctgaactcccaggccacgaattacatcagttctcaagacttcaactagtctcctgatcttttcagaacctggcataatagctgaaggtagctctttaaaatggatttcctctgcctcttctgcaaccttcccatgaagtatcagtgtgtcccgatatttccgatgaagtttgaattctgacactgggtttgctaccgggacatcttcacagctctctttagaatccagtttcagggtctgagtcatcaattgtaccaaggcattaatttcatttgtctgacctttcccttccccgtaatccccatctgacttatcagttgaacttgtagaagaacttaactcatcctcagacagacaatgaatctgtttcctttcctgagtgacgctgcagtcagaggagagccgtcgggcaggcaagggctggtcttcttcctggggttttcctggccctgctacactcagagacgctttcctcactgaagggcctgaagaggacatttcttcctgtgactgctttagtcgcctcctctctctggctgataatggtcgatcctttgatgatgacatctcactgctccttgaactgctcacagacccagtgaccactctacgttggttttcagcctctttttgtgttgatgtgacatccactttcccaacaatgggatgagaaggcaaaaatcgaggaggcgactcttggaaagcaaagagatctctgcggacctgtctcttttcccctctgtgctcagtctgttctctcctcttttgccgtcgctgtcgagacagggaaggttcagacccagagttgtgtggctgtaaatctgggtggattctgccctgtttttctataatacattcaccagcaacttgatcctgggcgtggtggcacacgcctgtaatcccagctactcgggaggctgaggctggagaatcacttgaacccaggaggcggaggttgctgtgagccaagattgtgccactgcactccagcttgggcgacagggcaagactctggtcctttggcttttgttctttgattaggggctgcagaggcttcactggttcattcttttccccagtgacaatgtcagaggaccacatgggaatcaggttttcaggctgggcactggatttagtgttgtcctgcagcatctcctcttccacttgagaaatactgcatatacctcctaactcattagaggcatccaaatatcttggctgattctcctgaacaaagccatcactcactgaatccctcccttttgcaggtaagatgtcaatatttacgctactgattgtggctagttctgtggtattgctcaagtcctgtttgcaggtatgggctttcagactggcaggtgacttcaagagaccagaggccctgggtttctcctgggacaaacatttgccttcacccattatatatgtctgggagccctcagaagagagtggttgggggtggattacttcatgatttgattctgcctctccagaaaccactgtagcaaaaggcttggattgagagtcaccatttttaatgttatttttggaggtttttatctttgtggcctccaaaaagaaggagatttgccgctttatataaggctgcctcaggatgctcctcacagacggcctttcttcaggccttttgctcagcattgttcttatcagttctgccagctctgggctgtaatctcttggcattggtggcagctttccttcaataatccgataaactaaagaattcatatcttttgcattgaaagcatgcttcaaggtggccatttcatagacacagcatcctagagcccaaacatcagacttatagttgtagggtttgtttgagaacaattcagggctcatgtagtagggtgtgccaatgagggtgctagccatgtcacagtggttctctaacactcgggcaattcctaggtcccctactttgatgatgtttgttcttgttaggaagacattttgagttttcagatctcgatgaaggatgtgtttttcatgtaaatactgcaaagccatggcgatctgtacaaaccactctaccacctgattctcaggcagaagctgccctttctgctccttgagctttcggtacaaatcacctccttcacagaagcccatgacaatgtagagcagaccatctcctccttcccatgactccttgtaggtgacaatgttgggatgcttcaactgagacaagagctgggcttcctgttcagcagctcgccgctctcggctgcttgccgtcccgccggtgcttcacaagcgtcacctctccatagctccccttgcccacgacccgcaggtagcagtaggcggccaggggcatgttcccagcgctggcccagagtcgggatgcggcggcagcggcgggtagggcagcgggcggcaacaagaagctcggttcatgcccgagagggggcagtgggggcggctgttgaggcagccgggcccgggcgggattgctggggcccggcccgcgacgacgccgctgccatagcgatccgggccgggagcagttct

SEQ ID NO: 12309 - RNA, 4606 nt, Homo sapiens
  source 1..4606: mol_type = other RNA
ctgggaggtcaaggctgcagtgagctatgatcacctcactgcactccaggctgggtgacagagcaagaccctgtctcaaaaaaaaaaaaaaaaaaaaaagatatgggtgagattcctttaattctaataaaatacctactttataccaatacattagaaaaattaagtaaaactgatgactctccagaacgatgtggatttccaaaacatgcacggaaaggtgaatagctcaaggataccaagtttgccaaagatttgttcccaactgggcattgggacttgatggttttgcaagttgagttctagcaaacccttcaaagtgaaaataagagttatcagaaaccaggctgtgagcactgtaaaagggcaggaagtattgttttattcaccactatatccccagctcctggcagagaacctggcacacagtaaactctaaataaaaatctgttaagtgtgccgggcgcggtggctcacgcctgtaatcccagcactttgggaggccgaggcgggcagatcacgaggtcaggagattgagaccatcctggctaacacggtgaaaccctgtctctactaaaaaaatacaaaaaaattagccgggcatggtggcgggcaactgtagtcccagctactcgagaggatgaggtaggagaatggagtgaacctgggaggcggagcttgcagtgatctgagattgggccactgcacttcagcctgggtgacagagcaagactgtgtcttaaaaaaaaaaaaaaattgttaagtggctgtaaagggaacatttcattagagtatttgtgtgtgtgtgtaattttcaaagatagatatatttttagttatagaaactgaaaacagggctgggcacagtggctcattcctgtaatcctggcactttgggaggctgaggtgagtggattgcttgagcccaggagttctgagatcagcctgggcaatgtggtgtaaccctgtctctacaaaaaatacaaaaactagccaggtgtggtggcacacgcctgtggtctcagctactagggaggctcaggcaggaataccacttgagccccagaagtggaggttgcagtgagttgagatcatgccactgcactccagcctgactgacagagtgaaactctgtctcaaaaaaaaaacacctgaaaacatttctggagcaatatttatttttagagtccctcgaatacagaagtgaaaatgtactattcaagacttgtatttaacttcataaaatttctttcctagatgggtattacctcttattaaacaactaataaaatatgtgctatataatcatacatttaaaacatggaaagacaactaatatcttacagtacatgaagacaaacttcaggagacaaacattaaatatatccaaaaactaaatggacctggactttgcttacaaattgcttaaatggaaatgaaatttgtgtttaagaaatgttttcactgatggaaaaataaatctaacaaaaccattatgtaaaaacatactgatttacaaagccaatgtgtctcagttttaatttgtatataccctagatgaggtttatattaaatgagaataaaatattaaaagtccatcaatgtgtagaaaagaaatacagctgctcaagtactagatagaacttcatattctttaaatctatttctagaactgaattgactttttaaaattttataatttatcaactactccttaaggttattaacaatagcaggaattatgacgacatattatgtcatttgtttctcctactgcttttatctctacattacaatataaaattttcaatccagcattttatagctctgtgtttaagttaattagtaccttaaaaaaataaaattctaaatataaacttggtggattaaggctcagtaaacagtaatcaaacaaacaacagatttgtcctcacaaagagaatatgaaagccaaagttttttttcttttgtgatcctgcttcatattattctgttctgtccaatttcttttctgtagggaaacgccaaagagatataaaaaagagatataaaacagtggtgagtggcttccaaatgactgtttgcccttgctttttaagccaaaatcctctaaaaataggtctttaattctggcagcagattaggacaaatgctcaaaaattcatgttttcttcaaaaaatttcaactggcgagctttcacactgtaagttgtatacttttcacccatgtgctcccgcaaacgtacctctctatcaaattcatcctcctcctccaaaagatcatacacctgctctaaaagctgaactcccaggccacgaattacatcagttctcaagacttcaactagtctcctgatcttttcagaacctggcataatagctgaaggtagctctttaaaatggatttcctctgcctcttctgcaaccttcccatgaagtatcagtgtgtcccgatatttccgatgaagtttgaattctgacactgggtttgctaccgggacatcttcacagctctctttagaatccagtttcagggtctgagtcatcaattgtaccaaggcattaatttcatttgtctgacctttcccttccccgtaatccccatctgacttatcagttgaacttgtagaagaacttaactcatcctcagacagacaatgaatctgtttcctttcctgagtgacgctgcagtcagaggagagccgtcgggcaggcaagggctggtcttcttcctggggttttcctggccctgctacactcagagacgctttcctcactgaagggcctgaagaggacatttcttcctgtgactgctttagtcgcctcctctctctggctgataatggtcgatcctttgatgatgacatctcactgctccttgaactgctcacagacccagtgaccactctacgttggttttcagcctctttttgtgttgatgtgacatccactttcccaacaatgggatgagaaggcaaaaatcgaggaggcgactcttggaaagcaaagagatctctgcggacctgtctcttttcccctctgtgctcagtctgttctctcctcttttgccgtcgctgtcgagacagggaaggttcagacccagagttgtgtggctgtaaatctgggtggattctgccctgtttttctataatacattcaccagcaacttgatcctgggcgtggtggcacacgcctgtaatcccagctactcgggaggctgaggctggagaatcacttgaacccaggaggcggaggttgctgtgagccaagattgtgccactgcactccagcttgggcgacagggcaagactctggtcctttggcttttgttctttgattaggggctgcagaggcttcactggttcattcttttccccagtgacaatgtcagaggaccacatgggaatcaggttttcaggctgggcactggatttagtgttgtcctgcagcatctcctcttccacttgagaaatactgcatatacctcctaactcattagaggcatccaaatatcttggctgattctcctgaacaaagccatcactcactgaatccctcccttttgcaggtaagatgtcaatatttacgctactgattgtggctagttctgtggtattgctcaagtcctgtttgcaggtatgggctttcagactggcaggtgacttcaagagaccagaggccctgggtttctcctgggacaaacatttgccttcacccattatatatgtctgggagccctcagaagagagtggttgggggtggattacttcatgatttgattctgcctctccagaaaccactgtagcaaaaggcttggattgagagtcaccatttttaatgttatttttggaggtttttatctttgtggcctccaaaaagaaggagatttgccgctttatataaggctgcctcaggatgctcctcacagacggcctttcttcaggccttttgctcagcattgttcttatcagttctgccagctctgggctgtaatctcttggcattggtggcagctttccttcaataatccgataaactaaagaattcatatcttttgcattgaaagcatgcttcaaggtggccatttcatagacacagcatcctagagcccaaacatcagacttatagttgtagggtttgtttgagaacaattcagggctcatgtagtagggtgtgccaatgagggtgctagccatgtcacagtggttctctaacactcgggcaattcctaggtcccctactttgatgatgtttgttcttgttaggaagacattttgagttttcagatctcgatgaaggatgtgtttttcatgtaaatactgcttgccgtcccgccggtgcttcacaagcgtcacctctccatagctccccttgcccacgacccgcaggtagcagtaggcggccaggggcatgttcccagcgctggcccagagtcgggatgcggcggcagcggcgggtagggcagcgggcggcaacaagaagctcggttcatgcccgagagggggcagtgggggcggctgttgaggcagccgggcccgggcgggattgctggggcccggcccgcgacgacgccgctgccatagcgatccgggccgggagcagttct

SEQ ID NO: 12310 - RNA, 4735 nt, Homo sapiens
  source 1..4735: mol_type = other RNA
ctgggaggtcaaggctgcagtgagctatgatcacctcactgcactccaggctgggtgacagagcaagaccctgtctcaaaaaaaaaaaaaaaaaaaaaagatatgggtgagattcctttaattctaataaaatacctactttataccaatacattagaaaaattaagtaaaactgatgactctccagaacgatgtggatttccaaaacatgcacggaaaggtgaatagctcaaggataccaagtttgccaaagatttgttcccaactgggcattgggacttgatggttttgcaagttgagttctagcaaacccttcaaagtgaaaataagagttatcagaaaccaggctgtgagcactgtaaaagggcaggaagtattgttttattcaccactatatccccagctcctggcagagaacctggcacacagtaaactctaaataaaaatctgttaagtgtgccgggcgcggtggctcacgcctgtaatcccagcactttgggaggccgaggcgggcagatcacgaggtcaggagattgagaccatcctggctaacacggtgaaaccctgtctctactaaaaaaatacaaaaaaattagccgggcatggtggcgggcaactgtagtcccagctactcgagaggatgaggtaggagaatggagtgaacctgggaggcggagcttgcagtgatctgagattgggccactgcacttcagcctgggtgacagagcaagactgtgtcttaaaaaaaaaaaaaaattgttaagtggctgtaaagggaacatttcattagagtatttgtgtgtgtgtgtaattttcaaagatagatatatttttagttatagaaactgaaaacagggctgggcacagtggctcattcctgtaatcctggcactttgggaggctgaggtgagtggattgcttgagcccaggagttctgagatcagcctgggcaatgtggtgtaaccctgtctctacaaaaaatacaaaaactagccaggtgtggtggcacacgcctgtggtctcagctactagggaggctcaggcaggaataccacttgagccccagaagtggaggttgcagtgagttgagatcatgccactgcactccagcctgactgacagagtgaaactctgtctcaaaaaaaaaacacctgaaaacatttctggagcaatatttatttttagagtccctcgaatacagaagtgaaaatgtactattcaagacttgtatttaacttcataaaatttctttcctagatgggtattacctcttattaaacaactaataaaatatgtgctatataatcatacatttaaaacatggaaagacaactaatatcttacagtacatgaagacaaacttcaggagacaaacattaaatatatccaaaaactaaatggacctggactttgcttacaaattgcttaaatggaaatgaaatttgtgtttaagaaatgttttcactgatggaaaaataaatctaacaaaaccattatgtaaaaacatactgatttacaaagccaatgtgtctcagttttaatttgtatataccctagatgaggtttatattaaatgagaataaaatattaaaagtccatcaatgtgtagaaaagaaatacagctgctcaagtactagatagaacttcatattctttaaatctatttctagaactgaattgactttttaaaattttataatttatcaactactccttaaggttattaacaatagcaggaattatgacgacatattatgtcatttgtttctcctactgcttttatctctacattacaatataaaattttcaatccagcattttatagctctgtgtttaagttaattagtaccttaaaaaaataaaattctaaatataaacttggtggattaaggctcagtaaacagtaatcaaacaaacaacagatttgtcctcacaaagagaatatgaaagccaaagttttttttcttttgtgatcctgcttcatattattctgttctgtccaatttcttttctgtagggaaacgccaaagagatataaaaaagagatataaaacagtggtgagtggcttccaaatgactgtttgcccttgctttttaagccaaaatcctctaaaaataggtctttaattctggcagcagattaggacaaatgctcaaaaattcatgttttcttcaaaaaatttcaactggcgagctttcacactgtaagttgtatacttttcacccatgtgctcccgcaaacgtacctctctatcaaattcatcctcctcctccaaaagatcatacacctgctctaaaagctgaactcccaggccacgaattacatcagttctcaagacttcaactagtctcctgatcttttcagaacctggcataatagctgaaggtagctctttaaaatggatttcctctgcctcttctgcaaccttcccatgaagtatcagtgtgtcccgatatttccgatgaagtttgaattctgacactgggtttgctaccgggacatcttcacagctctctttagaatccagtttcagggtctgagtcatcaattgtaccaaggcattaatttcatttgtctgacctttcccttccccgtaatccccatctgacttatcagttgaacttgtagaagaacttaactcatcctcagacagacaatgaatctgtttcctttcctgagtgacgctgcagtcagaggagagccgtcgggcaggcaagggctggtcttcttcctggggttttcctggccctgctacactcagagacgctttcctcactgaagggcctgaagaggacatttcttcctgtgactgctttagtcgcctcctctctctggctgataatggtcgatcctttgatgatgacatctcactgctccttgaactgctcacagacccagtgaccactctacgttggttttcagcctctttttgtgttgatgtgacatccactttcccaacaatgggatgagaaggcaaaaatcgaggaggcgactcttggaaagcaaagagatctctgcggacctgtctcttttcccctctgtgctcagtctgttctctcctcttttgccgtcgctgtcgagacagggaaggttcagacccagagttgtgtggctgtaaatctgggtggattctgccctgtttttctataatacattcaccagcaacttgatcctggtcctttggcttttgttctttgattaggggctgcagaggcttcactggttcattcttttccccagtgacaatgtcagaggaccacatgggaatcaggttttcaggctgggcactggatttagtgttgtcctgcagcatctcctcttccacttgagaaatactgcatatacctcctaactcattagaggcatccaaatatcttggctgattctcctgaacaaagccatcactcactgaatccctcccttttgcaggtaagatgtcaatatttacgctactgattgtggctagttctgtggtattgctcaagtcctgtttgcaggtatgggctttcagactggcaggtgacttcaagagaccagaggccctgggtttctcctgggacaaacatttgccttcacccattatatatgtctgggagccctcagaagagagtggttgggggtggattacttcatgatttgattctgcctctccagaaaccactgtagcaaaaggcttggattgagagtcaccatttttaatgttatttttggaggtttttatctttgtggcctccaaaaagaaggagatttgccgctttatataaggctgcctcaggatgctcctcacagacggcctttcttcaggccttttgctcagcattgttcttatcagttctgccagctctgggctgtaatctcttggcattggtggcagctttccttcaataatccgataaactaaagaattcatatcttttgcattgaaagcatgcttcaaggtggccatttcatagacacagcatcctagagcccaaacatcagacttatagttgtagggtttgtttgagaacaattcagggctcatgtagtagggtgtgccaatgagggtgctagccatgtcacagtggttctctaacactcgggcaattcctaggtcccctactttgatgatgtttgttcttgttaggaagacattttgagttttcagatctcgatgaaggatgtgtttttcatgtaaatactgcaaagccatggcgatctgtacaaaccactctaccacctgattctcaggcagaagctgccctttctgctccttgagctttcggtacaaatcacctccttcacagaagcccatgacaatgtagagcagaccatctcctccttcccatgactccttgtaggtgacaatgttgggatgcttcaactgagacaagagctgggcttcctgttcagcagctcgccgctctcggctagaggcatttcggaggttcagttttttgatgacatactgcttgccgtcccgccggtgcttcacaagcgtcacctctccatagctccccttgcccacgacccgcaggtagcagtaggcggccaggggcatgttcccagcgctggcccagagtcgggatgcggcggcagcggcgggtagggcagcgggcggcaacaagaagctcggttcatgcccgagagggggcagtgggggcggctgttgaggcagccgggcccgggcgggattgctggggcccggcccgcgacgacgccgctgccatagcgatccgggccgggagcagttct

SEQ ID NO: 12311 - RNA, 416 nt, Homo sapiens
  source 1..416: mol_type = other RNA
ctgggaggtcaaggctgcagtgagctatgatggcaccattgctctccagcctggacaacagagcaagactctgtctcttggggaggcggtgggacaggagagggcatggaagtcctgcctcccacactggctctctctggggatctcttccatctcatccagctgctcctgagttgtagtctcctgggaaaaatgctggaaataagccagactccagagtgatgtggtcatgaccagatccctccaagatgacctggaaagctgagtccacctgagctcacaggacggctggagctgggccagaatggagaggccgctggtgggccatgccccagtgaccccagcccgaggggtggcagccaagctggcgaggaagagacagaggaggaccatgtcagaaactcacaaggacaagt

SEQ ID NO: 12312 - RNA, 505 nt, Homo sapiens
  source 1..505: mol_type = other RNA
ctgggaggtcaaggctgcagtgagctatgattgcaccactgcactgcagcctgggtggcgcagcaagactctgtctgaggctggtagctctggtagacagaggccacttcgtccgcgagatcaactagctcacagcccctcagtgccgcaatgaagtactccacccagccgggccgccgctgaagggtattgaagagatgccagagggtgtcccggttccctgagagtgtgcaggtggcccgcagtcgatcctggtctcttgctgtgaggcagggcaggtaaggcagaatctctacaacatccacattgcaaaaattgctgaaattgcggcagatatacttataggtcttgtcttcagcaaacggcattgctgctcagattctggagagagggctctggccccatgaagggtggatggactgagaggaaacgagactcgggtacccccggccctgagacctggcgaccgccgcccggggcccaggacccttcccgcagcgaggag

SEQ ID NO: 12313 - RNA, 623 nt, Homo sapiens
  source 1..623: mol_type = other RNA
ctgggaggtcaaggctgcagtgagctgagatcacgctactgcattccagcctgggtgacaaaatgagaccctatctcaaaaaaataaaataaaagttacagtacgttacaaaacagtagtacaaaaggacttattcatgtatacactcaacaagtatttacagactgcctgctctctgctaggcattattctcatagtaacaataaactggggaacagacagacaaggtccatcatcacgtgtacattctggtggatcccacttttgaacagaaatgactagaaaagcctctgactagaaacttatgcaaccagataccaatatcatacatctttaagttgaaggatttatacgttttctaatgtacttttccattttgattttcctacataaatgggcactgtcaaacaataagaaataggaaataaataggaaactggccatactcaaacaacaaaaatgctattaaaaatctgagatttaggattgttgaaaggtttctcttttaaataaacccaaatcaattttcagttccatccttctactcaaaggtgtatttgaagaactgatatattatcttataataataaaagcaggaatatcagtgatctggcaattttatt

SEQ ID NO: 12314 - RNA, 1498 nt, Homo sapiens
  source 1..1498: mol_type = other RNA
ctgggaggtcaaggctgcagtgagctgagatcatgccacttcataccagcctgtgtgacagagcaagactatgtctccaaaaaacaaaacacaaattaaagaatgttgggcttgtattaacgttgtggatgctgagaggatgaataactatttcttgaaactgtcaggaatagagcagccccaagtttaccaaggaattttcaggaattgaagcaaagtggcagggccttgcactactgtgttggggaaaggtccattccctttgtataaggctctttgtgtctgtgtatcttcagtgtgtaaaatgaattttctctgagaatgatgtcatcagtataatgtcacacctgtactcctgtagaaaggtggctgcagtgagatattgtctgtgaagattgcatgcaatgacgaggctgccaaggcactccgtgtgttacctggtcccttcagagatgaaggcaggctatgactgcgactctgtccagaagcgtctcttgcaaaaatccatctttctgagcctttttaagaattttactgtcttctttacttattttaagtttgtgctcttggaagctctgaaatttctttacataattgatttcacattgttttacatttcctttgtcttcttctggaatgtcatcttttttcttggtttctctttcagcacaggatctaatcttgatcatttcttcttctcctgctgttttactttttgcttctatgtcccctgcttcattgcatctaataaagcagccatttgaggccaacaaagccattttccccttctttgtgtggagctcccagggtaaaaagaccattgtcgagtggatgtatataggttccctcatccatttcaatggctatggttcctgaaatttcatcaaagtttgttactgttcaccagattccaacatatcaaactgggtttcttcatcttcttctctttttctcttcttctctttgctctttttcttcttacaggcagaggcctgcagagatgcctcagaggactgaaactcgtgggtacggggccacgggtcacccgcccgtctatcctgtttccagggtcgtcagtgcgggaggctgcccctctctgcacaggcgccaggaactgcggtccggcctccgtccagcccggacaggggccagggcgaagcctgggaggccacaaagccggctctccgcgccacggcttccaccggattcgaggggggtggagtgcgtccgaaaagaactgaggaggctcccgccggaggtgcaggacccacctcttcgtcttggttcccttgagcacaagcttggtagacttcgcataagagtactcggccatggctccgggacacttctgcgcggagaggctgaagccggctcaggacgagtatgtgacccggagcagcaccagggcggggaggaacagaagtggaggcaaagtaaacactccctgacagcgtacgtctgtccagaacccgcctccgtcttcacccaaacgctgaat

SEQ ID NO: 12315 - RNA, 1679 nt, Homo sapiens
  source 1..1679: mol_type = other RNA
ctgggaggtcaaggctgcagtgagctgagatcgcgccactgcactctagcctgggtgacagagtaagacagagtaaaaatatatatatgtatgcgtatacagctttaaaaacagttttggaaaaaaatacaggtgcttatttcccaagtttaaaagtggatctcctgtgcctaagttaaacagcctgaaaagagaaaaccaaaaaggccaacaccaggaccctgactaagggcttcattaaaatattcgaatgctgtggaagtttattcccacgcaaggcacttactcccaacaagacacaaccgtttaaaattttacagcagtgacaccagggaggggtcccactcctatagacgtcagtattctgcatcgatatgctttgcaatggtgttcaactggatgttggaagctccttcatatatcgtaccaatctttgcatctcggaagtatttctccacagggtaatctttggtgtagcctactccccccatccactcgatacatttactcgttgtttgtcctgcaatctctgatgcatagtatttggccattgacgcttcttttatgaatggctttccagcttctaaaagcctagcagcattgtatgttagtaatcttgcagcttccagctgggtggccacgtgagccacttggtgttggaggccctgaaaatcaaatagtcttttgccaaattgtatcctttctttaatatatggaatagtgtagtcaaaacatccttgcgccagtcccagcatctgtgcagcaattcctattctaccttcattgagactccctatggcatacttatagccatgtccaatttgtcccaagatattggcttctggaaccttgacattttcgaatgttaacgggcaggtggaagaagctctgagccccaatttgttttcaggtttccctatatgaaggcccggagtatcacgatctactaagaaggaggtaattcccttatatccaatggtagggtctacatttgccatcaccagaaagagccctgcgtgctcagcactgctgatccacatctttgatccattgaggacataataatctccctctttatcagctctggtcttcaaagcaaatgagtcactacctgctccagcctctgaaaggcagaaacttcctactttttctgtagtgagctgaggcaaataggtggccttttgttcttctgttccatgttttctaatcagtgtgttaattaatgtgttctggatctcacaaaagacagccacagatgcatcaactttggctaattcctctatcacgagcacagtggataaaaatgaagctcctgtgcctccatattctgggtcaacttcaatacccatcaacccttgttgaaataatccttgtattactgatttctccattttcgaattttcatccatggttgaaaccaaaggtgcaatttgttcctgagcaaattttttaactgaactctttatcatcatttcctcatctgtaaatgtttgcaggggagcaaagtgtattccattatttgttatattgagtagagcttctgactgggaagattttgagacatgaggaggaatcttccaagaagacaaacaagtcaggaaatttcttcttagcagcctgctgccgcgcagcaaccgcactgccaggccctccatcctcgccgcaggcctctccgctct

SEQ ID NO: 12316 - RNA, 1578 nt, Homo sapiens
  source 1..1578: mol_type = other RNA
ctgggaggtcaaggctgcagtgagctgagatcgcgccactgcactctagcctgggtgacagagtaagacagagtaaaaatatatatatgtatgcgtatacagctttaaaaacagttttggaaaaaaatacaggtgcttatttcccaagtttaaaagtggatctcctgtgcctaagttaaacagcctgaaaagagaaaaccaaaaaggccaacaccaggaccctgactaagggcttcattaaaatattcgaatgctgtggaagtttattcccacgcaaggcacttactcccaacaagacacaaccgtttaaaattttacagcagtgacaccagggaggggtcccactcctatagacgtcagtattctgcatcgatatgctttgcaatggtgttcaactggatgttggaagctccttcatatatcgtaccaatctttgcatctcggaagtatttctccacagggtaatctttggtgtagcctactccccccatccactcgatacatttactcgttgtttgtcctgcaatctctgatgcatagtatttggccattgacgcttcttttatgaatggctttccagcttctaaaagcctagcagcattgtatgttagtaatcttgcagcttccagctgggtggccacgtgagccacttggtgttggaggccctgaaaatcaaatagtcttttgccaaattgtatcctttctttaatatatggaatagtgtagtcaaaacatccttgcgccagtcccagcatctgtgcagcaattcctattctaccttcattgagactccctatggcatacttatagccatgtccaatttgtcccaagatattggcttctggaaccttgacattttcgaatgttaacgggcaggtggaagaagctctgagccccaatttgttttcaggtttccctatatgaaggcccggagtatcacgatctactaagaaggaggtaattcccttatatccaatggtagggtctacatttgccatcaccagaaagagccctgcgtgctcagcactgctgatccacatctttgatccattgaggacataataatctccctctttatcagctctggtcttcaaagcaaatgagtcactacctgctccagcctctgaaaggcagaaacttcctactttttctgtagtgagctgaggcaaataggtggccttttgttcttctgttccatgttttctaatcagtgtgttaattaatgtgttctggatctcacaaaagacagccacagatgcatcaactttggctaattcctctatcacgagcacagtggataaaaatgaagctcctgtgcctccatattctgggtcaacttcaatacccatcaactgaactctttatcatcatttcctcatctgtaaatgtttgcaggggagcaaagtgtattccattatttgttatattgagtagagcttctgactgggaagattttgagacatgaggaggaatcttccaagaagacaaacaagtcaggaaatttcttcttagcagcctgctgccgcgcagcaaccgcactgccaggccctccatcctcgccgcaggcctctccgctct

SEQ ID NO: 12317 - RNA, 748 nt, Homo sapiens
  source 1..748: mol_type = other RNA
ctgggaggtcaaggctgcagtgagctgagttcacaccagtgcacgccagcctgggtcacagagtgagaccctgtctcttaaaatttttgcaaagaaaacaagcatgacaggattcttaggctgtggaggtatctcatctttttttgtttcatttctcagaggtgataagaagcagcgattttacttcctgagcagtcagctggccaatccccagctttgccaaagccttgtccagttggtgaatcacagttgtatgagtcttcaaacgatgtctcaacaagggaggaggcaggtaagatgtgagaagcatggcccggctcaaggctttctgtctcaaatgctccatctcccggtatggaagttgatgaaactttatattgtgcttccacatatttgtctttattcttctagcctttttggcatcagcccataacatctgcaatcctttcatgaagattgtgtacaggacatagaagcgggggaaatgacgacccaagaaacgatggtatttcccattaatcgcttttgtcttggttaccacataagacatcaagttcttcacatctgcctttggagaaaggtgaagctttgaagaccgaggggccccccaagccaggccagagcgaccaagttgcagcctccgggtgacaaaatgtccaggggtgactgccgagccccacacagccgaccgagcccagcacaccctggagagcgccatcttcacagcgagagaagcgggagagaagag

SEQ ID NO: 12318 - RNA, 1946 nt, Homo sapiens
  source 1..1946: mol_type = other RNA
ctgggaggtcaaggctgcagtgagctgagttcacaccagtgcacgccagcctgggtcacagagtgagaccctgtctcttaaaatttttgcaaagaaaacaagcatgacaggattcttaggctgtggaggtatctcatctttttttgtttcatttctcagaggtgataagaagcagcttaaagtgtccagcaaggagatcaacttcaaatcagtttctgcaaaacttccatcccatcagaaggttctatgccaaccaattaaatccccatttgttagattatgtcagtcttgtaaaaggagacagcaaaatgattagagtatgcataagtcatttccatcaacaggtttcaagcagtctttacttgggtttaaaaacagtgcttcatgcatttacaataagttattacagaactctaagtcactgatgcacacacaaaagctaaacccaacttactaactatgcagacctctcctgatctccccaggctgggcagtaattagtaccttacaggtgtgatccatggcccagagaaggcagccactgtcagttacagttggactgctgcatcacagtggaggcagcagagttgaagatccacagagggctgtaatacagcccagaaaagacaatggagagtgaaggctagaaacattgaggaaggggtcaagaagcacttgtacttcctgttatcttttccaatagaatattcctgcaagttacccatcagaaaaaggtgttcagagggtttgaaaaagaagtggttagcccatgccagtgaaggtgacaaaaaacaaaacaacttgatttttggtcatatcagaaaggatggagggaaacacccaagtacatgcacggacacatgtgctccagccaaaggagtgctgttttcaccagccacaaattttctaacagcaacaacaaaaacccacagatgtaagtaacatggaagtggatcagtcctaagccaaataaggattcccacctggggcaaaagctgacttcctaggacatgaactgaacacatcacagtaaaagcccagtagaggctgctgccagttccagctattagtaattatgagggggacaggatgacacctcacacggaccacccctagcaagagggtttgtttcagttctagctgtgagaggaatgtctgcagttcccacatgtgtgccatgctgtgaagcccatggcccctgctcctctctctgcctcccacacacttaacagtacacacagactttgctggcaagtgctgtttgttcctgcactgctatactatacgactgcaggacaatgccatccgctccatggttcattcagcgccttgtcccaaggtagttggtggagagcaggaccacgttgtgcagcaagagagacagctcagcttctttcaggctgcaggaaatctgcagccattctcccagccaagttcgacacctatcttcaccaatatgcgtagaattcaggccacggagataacaagccgattttacttcctgagcagtcagctggccaatccccagctttgccaaagccttgtccagttggtgaatcacagttgtatgagtcttcaaacgatgtctcaacaagggaggaggcaggtaagatgtgagaagcatggcccggctcaaggctttctttcatgaagattgtgtacaggacatagaagcgggggaaatgacgacccaagaaacgatggtatttcccattaatcgcttttgtcttggttaccacataagacatcaagttcttcacatctgcctttggagaaaggtgaagctttgaagaccgaggggccccccaagccaggccagagcgaccaagttgcagcctccgggtgacaaaatgtccaggggtgactgccgagccccacacagccgaccgagcccagcacaccctggagagcgccatcttcacagcgagagaagcgggagagaagag

SEQ ID NO: 12319 - RNA, 28 nt, Homo sapiens
  source 1..28: mol_type = other RNA
ctgggaggtcaaggctgcagtgagctgg

SEQ ID NO: 12320 - RNA, 186 nt, Homo sapiens
  source 1..186: mol_type = other RNA
ctgggaggtcaaggctgcagtgagctgtaatggcggcatcactgcactccagcctgggtgaaagagcaagaccatttgtattagtcctctttgtggattatcagtgtcattttcttctcttttttcttcttcctatgggctgccatgggagagaagatgcctgaagacaagtgacaatgcttctgt

SEQ ID NO: 12321 - RNA, 3059 nt, Homo sapiens
  source 1..3059: mol_type = other RNA
ctgggaggtcaaggctgcagtgagctgtaattgctttagcaatatgagtgagccatcttggaaatgtagtctccagctccagtcaagacttcagatgactgcaaacttggccatcatcatgtgtacaatcttgtgagaggcccggagccagaaccaagtgagggtgccattaggtaagctgttgagggtgccattaggtaaccaggtgccattaggtaagctgctcctaaattcctgatctggttcgcttgtcagggcatgggaagaaaacaattgaaagactgaggacaagattgtctgcagaggaggcactgggatgaaccaagatcaatgtgatcctttcatgaagaactgattttttcctcctccaaattgcttctcttctgtttggttgatgtgcacttcattcttctccaactcctcaatccagaccaatgttttcaaaggcctccattttgtgaaggtgttgtcatcaaagcttgcctttctctttataaatgaactcatttgtggaaaattccagactttctccagtcaatccttggcatcctacagagatggtcttcctcagtcttcagtctctgtaacgataccagcccttgtttagagacccagagtagaaatggtcactgtatacagttgtacagtttctgcaccgcacagacacctgtaaaatgggtatacatggaaggcaggtcttctgtgaagctcacacagcataaactttcgggcatcttctctaggcctccatcccaggccttggcaggagccttggcgatacattcacctggtcatatgtttatgtacaatttgcaaaagcaatatattgtcaccacaattagctgagactgaggtctctttccactaggactttccctctgccattttcccttctattgggtggtgctagggcagcctggacatgctgtgggatagggtcaggctttgtgttcctacccaaacctcatcttgaattgtaatcctcacttgttagggagagaaatgacttgattatggggacagttttcccgtgttgttctcgtgatagtaactgaattctcacgcgatctgacggttttgtgtttggcaagttcctccgctcacaattctttccgcttccttgtgaagaaggtacttgcttctccttccaccacgattgttaagtttcctgaggtctccccagccatgtggaactgtgagtcaattaaacctctttcctttataaattacccagtctcgcgcagttctttatagcagtgtgagaacggactaatacacagtatttgctttttctttaagaggaccacccaaattgcataaattgcaggccccacaaaacctgcattaccccctaagtgtgagaatagtacctatttcacaggtgtgctgtgaggattaagaggtaatggacacatggtgtgtatcaggtggatgttagccattatcactactctgaatctccatctttctattatagcaaggccacagaaatgagcattttatgtaatattcttaaaactaaattcttctcatggaatgggatttttcaaccccaggcaacagggccacatcatgtttttcttgggctctaggcctttttgccttcgttgagccccttactccattaaaatatatatacatatacacacacacatatatacatacattttaagattgtattagcacaaaaacaaatatattaatatatattaaaatactttcttaaacctaaattttttttccttctgatttgaaaagaaattaaaatattttttgtgggcctctaaaaatattgtggaccttaggcactgtgcctaatggaaaagacagtgacaggattgtgcaatatgaataatgataaatttcccaaaccatcaaggactcaagaataagggtaaacatcttaaatggggttggtttcgagtacttataatagaaaaatgttatccaaacaaggtcttaggggtaacaggaggcgtttttagtgttcaaaatacgcacatggatggagttggccattaggacgctaatagcgaccgtatctagctgtgaaatacatatttttgttttgggagtctacttttcagtaaatgtcctttcaggtgttttgttgcccatttaattacatgatcaacaaggaagagttattttacaaaacaagcttcattttgccaatttataaattgctttggagtttcatcgaaaggtctttaaaaaacacgttggccttggtgctggtgcatcacataaatcacagatgaaacaaacaagcctgtttcctactcaaggtgtgtctgtagagtcctgactgcgtgccaggggctctgtctggcacatttctgaactttgcaaaattaattgtgccgaagagaacaccatcaaacgcgtccggcatacagcgtaaacatcttcagaccgtgattctgcgccatcaaacgctctccagctaatttcatttggtgattactctgctagaaaaccgaggccaagtgaaactgcggaaatgggaacaatgtacggaggaaaaatctcaccccattaagagatccgtttcttctccgcacaaataagcccaccccgcctccgaggcaagactagatggctccaggatactctcggcgcgcccgctggccatctcgggcaggggagccccacacccggcaggaggaccaggacgcgagcggcggcgcctcggccctgggctgtttaggtaattcgcaaagtcccaacaatcatccccctctcccagaagctggttttcttgtgtgcagtggttacagaggcggcgaaaacacggttccccgctttcctctcctcaaggcactgtttgcagcggcagcagcggccgcattcggggaggcgcggtcctccccgcagagccgtcgcgcactcggcctttctcgaggatttgcctgggctcggccgcctcgctctcccctgcgcttccatgaccttctgagagcggcctcaccaccggaggctcggaggaagcaccaccctcggcgtccggggcccgtcgcgcggccgcgttcctccgactccttggagcacccgcgcgc

SEQ ID NO: 12322 - RNA, 6903 nt, Homo sapiens
  source 1..6903: mol_type = other RNA
ctgggaggtcaaggctgcagtgagctgtattcatgcctaggtgacagaatgagaccctgtctcaaaaaaaaaaaaaaaaaaaaggaaccattaattttctctcccacaacactggaagttctgagacaacacaacaactttcgaaattctgagaagataataattcctactctaaaatcccaaaccagaactatccatcaaatataagaatccaacaaaaatacagccagatatgcgagttctcaaaaaattcatttcccttgaattcttttcttgggaaaacacaagacaacataatccatcaaagtgagcgagtaaaccaaggaggaaaaaaagttagatccagccaggcgcagtggctcacacctgtagtaccaacactttgggaggccgaggagggtggatcacctgaggtcaggagttcgagaccagcgtggccaacatggtgaaaccctgtccctactaaaaatacaaaaattagctgggcatggtggtgggcgcttgtaattctagctactcaggaggctgaggcaggagaatagtttaaacctgggagacagaggttgcagtgagccgagatcaagccattgcactccagcctgggcaacaagagtgaaactctgtcttaaaggaaaaaaaaagggggggggggggagacacaagacacagtaaacagtaattccaaaacatgaaacagccaacaggaatacccaggagtatggtaaaggaaggttccagatggaatcagttctacagtccaaactagaagaatgttccagggagtagaggtgatgggatatatttggagggggaggtttattactgaatcatgagatctgttttaatatactgaggggcttatatttccagagtgattagatataaattactggtaggtaaaaaacagttaagtattaacttcagggagaaaaaaaaagctgcacaagaatgaaaataaaatcacagcatattccatggcttatctaaagctttaataatacttacacagccataataaaagtaattattgagccaatcaaaagttatataactacactaaaaagatgtaagggatcattatttcatgttgaagtggtgagaggtggtaggaatgcaggcttttcaagaaggtatttctaagaatttttaagcatttgctcttaaatatgaggaacagtaaatgatcccaaggcatctgaagaaacatcaaaataaaacactaaactaaggggaaaatcaaatgaaacagactatgtggggggtggcggggggtgggggcagagacatgacgacttttatagaaagtaggctgggcgcattggctcaggcctgtaatcccagcacttagtccgaggcagatgatcagttgaggtgaggagttcgagaccagcctggccaacatggtgaaaccacgtttctactaaaaataagaaaattagccaggtgtggtggcgcacacttctagtcccagctactcgggaggccaaggaatgagaatcacttaaacccggggggcagatgttgcagtgagccaagatcacaccactgtacttcagcccaggtgacgaagtgaaactgtttataaaaaaaaaaaaaaaaaaagccagatgtggtggctcacgcctgcaatcccagcactttgggaggccaaggcgggcagatcacaaggtcaggagttggagaccagccttaccaacatggtgaaacccagtctctactaaaaatataaaaattagccaggcatggtggcatgcacctgtaaccccagctgctcaggaggctgaggtaggagaatcgcttgaacccgggacacagagattgcagtcagctgagattgcactactgcactccagcctgggcgacagtgcgagactcaaaaaaaggggaaaaaaaggaaagaaagaaaaagtacaggcaacaagatttcctttagaatcagacatgaaatatgagggaaggaagagaagaatgactctaagatttttggtttaaataactggaagaataaagttgtcatttattgaactaaggaaaatgcaaaagaagtaaatttggattaaacaagatgaaaagtacagatatagttatcaagcacctagtaaacagtcggatatgtgaatctggaattcaggagaaaggttctggctggagatataaatttgagtcaccagcacagttcccattaaagaaatgaagaccatcaagggaatcccaaactaggcttaggatatttcaatgtttagaggatagaaaaggaaacagcaaaggaaactgagaaaagagtcagagaaataggaagaaaaagcaggaaaatatgtttcctagaagccaaataaagtaaatgttttaatggagaagagtcaacaactgtatgaaatgctgctaatagatcaagtaaaatgaggtcactgacgtcacgagaccttaaaaataccagctccaatggaaatgaatatctgattggaatgggttcagaaaaaacagaacaaactaaaaacaatgaatacaggcaaggagttttgctataatagaactctttttcaaggagctttgttataaaagaaatgagacattgcaattggctcaagctacgacaaacaatatatccgcagtatataataaagggcagatggggacagatgggcacagatgctaggtttacagatgcaacggtgacaacttttaaagattcttttctgactgcgtctattttctcagggcaatagggagcaaagtgagagggaggagatatgagacgtgcaatgacagagtaaaactatgaaaccagtcatttaggacaatgtaacaggaaagactgggtcactaaggacaagatcacgagtttcaagcaagcctaggtcagcatgcttatgtaatgggttaacattttgacttaaaaaacaaataaacctgctctatagtcttttatttaaccaaatgttctatctgaagtttttcttcaccaccaaagaacttatccatgtaaccaaaacccacctgtacctcaaaacgattaaaataaaaatttaaaagaaaagacctgtgccaataggacacagggaaaaaaaattaagtttttcttaagtgacggttccattatccttaacagatcatctgatctgcatttgaatatacatggcaacagcaatatttttccatgaaataaacactaacacagaaatgtatggcttatggagtatgtcccctctccagggtacattcaggatttctcttcctcattgtctgatatcctttcacacagggtctaaattgtgcctcttttggcctttatgctgttctattacagattgtgcattacttacatattcctaaggcctattctcttatatttggttctagttaacccactactataaattttcagggtctgtcttgttttgcatgatacactaccatttccaatttctagtcgtttctcaagaccctaaagtttcattcagaaacttctcttgtgctaacacaatgtccacttgaaatctctatatgacacactcctatagtactagtgaatgaaaccaagaaaacaaaataaccaaatcctaccgacagccaagtcttttgctattattgcacctaagctattcctgaagaaataatttaatgagatcatcttataaggaacatttatttggtaaactatctcatagaaatagactctaaaatcaaacagtttcttaaacaacagagagcataatcccaatctctccccatgaaaagcctacttcataactgaagtacctaaagcccatgaactgcattactagaagaaaggagggaaaaagacatttactaaacttccacaggaagactgtataaatctggaagtggttaagtacacatcagcctgtatccaagaatactactcagtctcaaaaattaactgaaaatctaaacttaatatggatacttctttgttcttggtaaggctcagaaaattaccatctatttaagtacgcatggtactagttacatgtcaactgatataataaaaaaggtgaagtggacaatcagtatttcaaacccaatacagggaaatcactagatgtaaataagaacttttaaaagctattcttgagctccactttaaaacaaacattcaggactggaatcttcagaattttctaatatcttgaatatccccatcttctctttaattggtcctgaagcattcatttgatcaataagatcacttcgatctaacaacaactctagatctttatcactaatgaccttctctcttgatccttttatttccctttcataatctctagattttaataattccattaattccttaggatctaagaaattcttagacagatttaatccagactgaccacctttgaaatgatttttatggatgatcaacttttccagtttccttttagcagctgctctttccacaattttctgatcgatagtatttgctgtaacaaggcgataaacaacaactggctttgtctgaccaattctatgacatctatcctgggcctgaagatccgactgggggttccaatcactatcataaatgataactgtatctgctgcagtcagattaatgcccaggccaccagctcgtgtactcactaagaagataaacacctctggatccgtgttgaagctgtgcatgtttttttctctctctgagtaagacatggacccatcaagcctgctgaagttgaaatctctgagatggcagtaatccatcaaaatgtccaacatgcttgtcatttgtgaaaaaagcagcaccttgtgacctcttttttttagttctggcagcattcgatccaaaatcaagaacttcccagaatttgttaccaattcttcatcgatcttaaattcttgtgtaacagggtctataggatattcaatcaaatatggatgattacaacatttacgaagtagcatcattatattctgcagcttcagattaacttcagattctacagggatattcacttccacaacagctctttctcggtccacctctggctgtatttgactgatcagtttttccaattcattagggaaatcatctattttgctgtaatttattgattttctagttcgtcgttttggtcgaccagtaggacttaactcaattgtttctttctcactggatccaaacatgtttgcaattgtacggttcacaatggctgtataaaagatctcctgcttctttgaaagtggagcataaacgactacttctcgtttaggaggaacttcaagagcaacatcagacttcagtcttctcaataagaaaggtgttaaaatctcaaaattggtatgaagcttgagtaaataagtattttcatatggacgtatatcatataaatcttttctggagggcaatttgccttcaaagaagccctcatctgtaaactctgacacatacattctaggaattctttcctggtgcagcatatgcaatacattctgttctctttctttagcaataatatcttcagcagtttcagaaagactagtgatgtcaaaccaagactcaaagcttttcaagtcatcaaatacatctggcaacaaaaagtttagcaatgaccaaagttctgataaattgttttgcaagggagtaccagtcaaaagaagtttgttatcagcattgaatcgttttaactccctgattagacggcacttcatattcttaatcctgtgtccttcatctactattaagtatttccaatagcaatgctgtaacgcatttcggtctctcatggctatttcaaatgacgtgattaccacaggatgaatctgcaaagtccctttccgtttgtaaatatttcttaccaatttttgacgttcctcctgggttccatgatataacattgtagggatatctggtgtaaatcttttgaattcagccatccagttaggaagtgtagacaaagggccacagacaagaaaaggtcctggtactcctctctgaatcatcaatgcaatagtagcaatgcactgaactgtcttacccaatcccatttcatctgctaaaatgccattaattccattttcccaaagcatcctaagccattccatgccttctacttggtaccatcgcatcactcctccagtgaagtgctttggttgttgaaaaggtactggctgaccattacacttccggactgggtcaaaaaagaatttagtattctgcctaaccgtttcagacaatctatctttaattatactattcgaatctttatttttctgaagatcttccacacagagattagtagaggaggagttttcatcctcattctcctttttattttttttagccacagacaaaatttcctcttttgacatgacctctgaaatattgtatgattcatcttctcttcctctttttttcctcataactggcttctcttcacttgcatcaattgaatttttaccctttttaacttttaaagactccttttttctctccaatttttctttcttcttctgttcctctaattgttgctgttccattttcgtcaataaaaatttggagtatatattgcttttttcaagcaaatgttgaagtctacggtaccgaatttctgtcgactctctatcccaagacatgcgagccttttccagcatcttccgctctctctctagtccagcagcttcaagctgttcttcctcttctagcatggccggggtaatcacagcagtgtccagttgttcaaccattgctggagcctccgagccgccgctgcccgcgggccgttccgctggcatgcctggacactcacccgggaaccgggtcccctcctctcagagcctgcaatgccgcgagctaactcctcacaaccgctgccggcccagccttctagccaaatcccccgccagggaaaaaagcgcgcttctccttcgcgggaaaat

SEQ ID NO: 12323 - RNA, 45 nt, Homo sapiens
  source 1..45: mol_type = other RNA
ctgggaggtcaaggctgcagtgagctgtgatcaaaacactgcagt

SEQ ID NO: 12324 - RNA, 2251 nt, Homo sapiens
  source 1..2251: mol_type = other RNA
ctgggaggtcaaggctgcagtgagctgtgatcacaccactacactccagcctgggcaacagagcaagaccctgtctcaaaaaaaaagtgtgggtccaccgagaagccccccagctgcaggagtggacccaggactggtcagccctcattgtcaacgtcttgtaaatcttgaactagtggacgagtagggggaaagtgcaggtgcagcaacctacttcaaaagggctaacttgaggctgattaggtcccgtgtgtctcccagtccacattagcctcgtttcttctcaatagaatcaagcactatactccggatcccaaggcactagggtcccagttcgtgctgagggcgtcgcctcaagtgctaagcgagctcacagcatctggtttctcaggaagtgagagagctacacatctgctcctgggaagcattatttgtcaaataagccttgtttctcagcaaccattgtagcccccagggccacaagtaaaggggggcttgccttcccttaccctcccccaaaagaaatttggaagagacgagctgagctgctccccgcccagctacagcaacctccagcttggacaatacaccctctgtcctcagccaggagatccgcctctggagttggctctgccccttcccccactcttcctggttcccagcacccaaaccctctactggagttctcctgacccagtggtctccagccaggacagtcccacaccttcaaatcctccccctacagtccccgcaccccaaggatctgagcacattcagttacaggcatggggtcaccccagaccatggaagagggggttccatcttcagtgccaagatggaccaccctctgcatagtcaaggtaagaaaacctgtgtggagggaggtcagaggtgctcctgaaattgtttgacctttactaacatcaacctggctttctcctcctctccttcttcctctctgaagctcctgctgctgtgagctggaaatcaggatgcctggctggcccatgaaccactcatttttgtttcactcccaccaagctacctcctgtataacttctcattctcagcttttctcagcccttcctgcagcccccttctccactatccccacattgagagtaggaatcaagcctgagctgggagtttggccacccatcttgtgacccttttccaattccttggaacctctaaagttcttcccatgggcctgccaggcagcagcaaaaccagcatgtgtgaggttctagcccttacccctcacctctctggggtccaatcaagttcctctttgagtcccagtctctccattggtaactttagagcttaagtaaaggtactcccatggcatccatcccagagcccagccaaagaccctaaggaatgctgggaagagcaagatgttaaaagagctggttgaaggctccagagacatgaacacacttaattatctcatgattctcgattacataatcaaatctggccaaaatacatgggacaaccttcagccttgccctttctccaggagcctccaatccctgccactttcctcggtattcccctaactcttgcctctcccctcctcccagtgcctccctactcattcccgcctggcttcccccacccccacctctcctgtccccagtccccagtgactcccactgctctaacctctgaaactgtctattggacaccaactcaaccaagagcagtaagatcaaggctccccagtcccaaccatatccacccctcccaaatgccaatttctgggtggggggggacacacagtcatcacgcacttcttcacagactcttcttccctgtggcaagattggaatcaggtgctccacccccttatccctaccctccaccttctgctccagggtggcacgactcaaacctgccctacggcccattagctccattccatgaagttcctatccagtaccaggcatcggtccccttccaggtgacttcagcctgtcaggccttgcctcccgtggagttggtgagtgcgctctgggatggggtggggagggcaaggaacctggccatggtgtccagaggtctggtggctccagagagggcccccaggagatgaccttgaacggagtgctgtgggtattgctcatcctacgtgacggagcgcatcttggccgccgccttccccgcgcggcccgatgaacagcggcaccggggccacctgcgcgagctggcccatgtgctgcaatccaagcaccgggacaagtac

SEQ ID NO: 12325 - RNA, 263 nt, Homo sapiens
  source 1..263: mol_type = other RNA
ctgggaggtcaaggctgcagtgagctgtgatcacgccactgcactccagcctaggtgaccggagcaagaccccatctcttctgccatttcaccatagaaactgtcaaattccaagggggaatatctaccaaaagtataagcttatgcttctgattctctcttctttcctccttctcccaaatcactctcttctgactggctactgctaaggacaacaaactgcccctcactactggcttggtttggtctactggaagcagcta

SEQ ID NO: 12326 - RNA, 4573 nt, Homo sapiens
  source 1..4573: mol_type = other RNA
ctgggaggtcaaggctgcagtgagctgtgatcatgccactccagcctgggtgacagagggatagcctgtctcaaaaaaaaaagtttgttaacagcatttcctcagagtataagcttgtttttctaggtctgtccaagaagatcttggagtatattttttctccctcttcagtagagaatagtgactttttgggtaatactttagctgtgaaaatttttcttctaaatttttctactctgaacaggaatgttttaaaacactgttaggcctattgagtgagctatttttctaaaacattttatcttttgaaatacgtatcttattaacaagaatgtttttaaccaaaaaaaaaaagaattctaacttgtattgcaagccctcttcccagtttcaatttttatacaaatattaaatcactgattcttctatgatccaagcacagatatgttactttttaaggataaaaataatcaaatcacttaggttaaactggttgtctacagtcacacagtaagttagataaagcaaaggaggtgtcaaagggtaacactaaattccattcactagcatcttgcctcactaacactctcataagatagattactaaataatataagtattaataaatggaatttccaagaactttcaactaataaagggtgggattataagattagtttttgttttactaattacaactatatcctggaactatttacatactacctaggaaataaagtttgtttattcttgcaggattgtttttaaaagcagtattttcccaaatattaatttaacagtaatcctaaaagtaactcaggaaataaaaaacttatcacttcagtacattttattcataatgaggtaaagtttttgttttttctctatatatgtagatatatatagcaacacaggttaattgtgcttgaggattcctatgaattacaagattatacatgttcccattctatttttctactcctaaagcaatcgtatatacattatttcctaataactcaataaggtaaaagtcttaaataattttattttatcctctactcttctgagaccatgtattcccatgttgtggggaaataaattctggcacaggaatgaagagaccaagatttctaggttatagtacttcaaaatcacactctgtcttggacctcagctctctaacaaaaatttaaaaaattagcttttaggtttctaaggtttcttccagctcaaatatgccatgatttgaaaagttaccttctgtggtagcttctcctacttatcctttctttcttaaatgttaccctagtccatttaattagacctacctaaatacttcagaaaggtcatatccatccaatcttgtatccttgatggatttaatattaacttatagatatatttgtctaaaagtattatggaaatagtacacaactgaaggtaatgcacttttgtactatattctatttaacatttctattaggaataaaatgatcatgttataatttttaagatcttgggtttacttaaacaattcaataactattacgtaattctattagtttctttaaactttaaattcaatctgaacgtaatattttaatgtgtcaaaagtagctaatatattcagttcaatgcttgacagggttaaaaacgtgaacaacatcagaagcaatgcatgtctggagtgggggtgagggtgctatgagctttgctgaacaaaaatatctcaggtaaatcacacttaaaaactgataccagttgccttgaaggaatgggtacatatcaaaaccagcattaatatgtcaaataaatttgaaaggaatattttcttattcccagagcccaaatttcacataaaacagaagaaaatatgtacagaaatcctcagactactaaagtccccctttcccaaaaaacataaaccctctaacccccaagcacctaaaaggctataatttacattaactacagtttgacttttcacataacagcgagaaggaccttacaaatcctcagtaaatcttcaattaatatttagagaacaacagatacgcaaacaggttttatgtgtaagctaccttagacggccataataaaattatgagcaaagataatggcatttcaacagattgctttaatgttaaacctcacaatgaaggatacttgctcaataaaataatgcactttagtgtaatgaaaagtttaatacatacaaataatactgaaaaaaattcctagtgactggctagctggtaatatgctactcaaaaattgcctttcaaacctaaaggacctagattgctttattatttgtttacactatcaaagaagaatattttgccacaaaatgaataatggacaaagaggccattgacatgtatacttttaaaaatattaactaaaaaaatagttaaaagtaaaaaattttattttaaaagtaaggaaaaagctaaactggttatagttgagattttaattgttatactttgtgaatgagggggagttaagcgcttgaaacattttatattatttacacttaagagtatgaaaaacagtgtgagactacatctggctatgttattataattcagaggaaatcattatcaagtcacaccccttgtagcaataaaatataacaaagcaaaaaaaaaaaagcaaaccaaatagaatccctcagccaacacaaacttagtctattcttaggggttgccatgatgtttctgattaatggtaacatattccacaagtgcaaataaaacatcagaaataaaatatctttttcactgaataagaaagctgttatttgtgtgatcttagtaaaactctgaaaggaatttgtaaaactcattcataatttaatcaaatgccttagtttttttttttacccccttggtataaaagtttacagatgagtttcatatttcatcacagttatatggtctagtgcatttcagagtatttggacattatcaaagctgtcctttcccaatgaaaacatttaagaaaacgttaagcacttctcaagtaacatgatgtggaattacactttttgctcttacctcttttaggtacacacgtattattcaacaaagcaaaactattttacagtgtctgttaacaaaaagttctctattagatagaggaaactacagtatcctgaagctatttccccaagagctagtttagtagatagacctttgggcccatcttatttttccttcttttttttttttcagtaaggtaactttccattatgcacatactataccatcatcattcattgggtggagattagctgggaagtagctgtatatttttagtgagatcactgatggcaatggatctctggatcgtgctgctgcttatggttaaatcatatctaatgtgaaatttcgaattacatccagagctccagtatcaaagccgcacatatccaacatgcctctatcatctgggtctgcaatggtgaaaccatttgatgtcattccacaaacaatcaatttagctggaatatccattttctttcgatactccctcagagcaatagcaggatggacacctccagcaaaggtctcattatcagtgaatacaatgaagacatcagcaggtgtgtttgtcttctgagcccagatcattggaagagagcaatcagttccacctgctgggatctgactcatagccattaaaacctgttgtaaggtcatatctgtagtcactggacatggtaccatttcatcggaaaaagcaactacataagaatctttttctgttcgtgtgacaaccatgcacattgctgcagcaactgtactagcgttgagtatactacccaaaactctttggttcatagaagcactgacatcaacagctagtaagaaacgttttccagttggttcaactgtcttaaatgttttataaaaagcagcatccaatgctttcaaaatttcttcatcagggcgccacttcagtttccctctgagaccatgacctgtcttgtaagtttctaatgcgatcaaaatatgaaatggatgtatacgagccttttttaatagtttttcattacacagtttttcacatactaaagatacttctgaatttcctggttcaagtactgaattagcagtcatctttcctagattccttagtaatgcagtaagcggcatttcttgtaacaaagccttccatacctctttagactttaagtgatttgttaaaagatgttctctaactaatctatgttcttctattagatgaatgacttctagctcatctcttgtgcgcttcactttctctacagcctccagatactttaataatttttcagtctccacagagagtgctttttctttatacaattcatgaacttctttccagccctttgtaatatatttggtcacaattgcaagtcctgtacctggcagccgaccccctggatccgcagcgccgccaggagaagtcctgcgcagcgctgggaaacgacaaaagaaggcagcctgacgggcagcgacagccacagcaacagcaacagccccactgccgccggggattccaggttcggttcccgggaacgagt

SEQ ID NO: 12327 - RNA, 5338 nt, Homo sapiens
  source 1..5338: mol_type = other RNA
ctgggaggtcaaggctgcagtgagctgtgatcatgccactccagcctgggtgacagagggatagcctgtctcaaaaaaaaaagtttgttaacagcatttcctcagagtataagcttgtttttctaggtctgtccaagaagatcttggagtatattttttctccctcttcagtagagaatagtgactttttgggtaatactttagctgtgaaaatttttcttctaaatttttctactctgaacaggaatgttttaaaacactgttaggcctattgagtgagctatttttctaaaacattttatcttttgaaatacgtatcttattaacaagaatgtttttaaccaaaaaaaaaaagaattctaacttgtattgcaagccctcttcccagtttcaatttttatacaaatattaaatcactgattcttctatgatccaagcacagatatgttactttttaaggataaaaataatcaaatcacttaggttaaactggttgtctacagtcacacagtaagttagataaagcaaaggaggtgtcaaagggtaacactaaattccattcactagcatcttgcctcactaacactctcataagatagattactaaataatataagtattaataaatggaatttccaagaactttcaactaataaagggtgggattataagattagtttttgttttactaattacaactatatcctggaactatttacatactacctaggaaataaagtttgtttattcttgcaggattgtttttaaaagcagtattttcccaaatattaatttaacagtaatcctaaaagtaactcaggaaataaaaaacttatcacttcagtacattttattcataatgaggtaaagtttttgttttttctctatatatgtagatatatatagcaacacaggttaattgtgcttgaggattcctatgaattacaagattatacatgttcccattctatttttctactcctaaagcaatcgtatatacattatttcctaataactcaataaggtaaaagtcttaaataattttattttatcctctactcttctgagaccatgtattcccatgttgtggggaaataaattctggcacaggaatgaagagaccaagatttctaggttatagtacttcaaaatcacactctgtcttggacctcagctctctaacaaaaatttaaaaaattagcttttaggtttctaaggtttcttccagctcaaatatgccatgatttgaaaagttaccttctgtggtagcttctcctacttatcctttctttcttaaatgttaccctagtccatttaattagacctacctaaatacttcagaaaggtcatatccatccaatcttgtatccttgatggatttaatattaacttatagatatatttgtctaaaagtattatggaaatagtacacaactgaaggtaatgcacttttgtactatattctatttaacatttctattaggaataaaatgatcatgttataatttttaagatcttgggtttacttaaacaattcaataactattacgtaattctattagtttctttaaactttaaattcaatctgaacgtaatattttaatgtgtcaaaagtagctaatatattcagttcaatgcttgacagggttaaaaacgtgaacaacatcagaagcaatgcatgtctggagtgggggtgagggtgctatgagctttgctgaacaaaaatatctcaggtaaatcacacttaaaaactgataccagttgccttgaaggaatgggtacatatcaaaaccagcattaatatgtcaaataaatttgaaaggaatattttcttattcccagagcccaaatttcacataaaacagaagaaaatatgtacagaaatcctcagactactaaagtccccctttcccaaaaaacataaaccctctaacccccaagcacctaaaaggctataatttacattaactacagtttgacttttcacataacagcgagaaggaccttacaaatcctcagtaaatcttcaattaatatttagagaacaacagatacgcaaacaggttttatgtgtaagctaccttagacggccataataaaattatgagcaaagataatggcatttcaacagattgctttaatgttaaacctcacaatgaaggatacttgctcaataaaataatgcactttagtgtaatgaaaagtttaatacatacaaataatactgaaaaaaattcctagtgactggctagctggtaatatgctactcaaaaattgcctttcaaacctaaaggacctagattgctttattatttgtttacactatcaaagaagaatattttgccacaaaatgaataatggacaaagaggccattgacatgtatacttttaaaaatattaactaaaaaaatagttaaaagtaaaaaattttattttaaaagtaaggaaaaagctaaactggttatagttgagattttaattgttatactttgtgaatgagggggagttaagcgcttgaaacattttatattatttacacttaagagtatgaaaaacagtgtgagactacatctggctatgttattataattcagaggaaatcattatcaagtcacaccccttgtagcaataaaatataacaaagcaaaaaaaaaaaagcaaaccaaatagaatccctcagccaacacaaacttagtctattcttaggggttgccatgatgtttctgattaatggtaacatattccacaagtgcaaataaaacatcagaaataaaatatctttttcactgaataagaaagctgttatttgtgtgatcttagtaaaactctgaaaggaatttgtaaaactcattcataatttaatcaaatgccttagtttttttttttacccccttggtataaaagtttacagatgagtttcatatttcatcacagttatatggtctagtgcatttcagagtatttggacattatcaaagctgtcctttcccaatgaaaacatttaagaaaacgttaagcacttctcaagtaacatgatgtggaattacactttttgctcttacctcttttaggtacacacgtattattcaacaaagcaaaactattttacagtgtctgttaacaaaaagttctctattagatagaggaaactacagtatcctgaagctatttccccaagagctagtttagtagatagacctttgggcccatcttatttttccttcttttttttttttcagtaaggtaactttccattatgcacatactataccatcatcattcattgggtggagattagctgggaagtagctgtatatttttagtgagatcactgatggcaatggatctctggatcgtgctgctgcttatggttaaatcatatctaatgtgaaatttcgaattacatccagagctccagtatcaaagccgcacatatccaacatgcctctatcatctgggtctgcaatggtgaaaccatttgatgtcattccacaaacaatcaatttagctggaatatccattttctttcgatactccctcagagcaatagcaggatggacacctccagcaaaggtctcattatcagtgaatacaatgaagacatcagcaggtgtgtttgtcttctgagcccagatcattggaagagagcaatcagttccacctgctgggatctgactcatagccattaaaacctgttgtaaggtcatatctgtagtcactggacatggtaccatttcatcggaaaaagcaactacataagaatctttttctgttcgtgtgacaaccatgcacattgctgcagcaactgtactagcgttgagtatactacccaaaactctttggttcatagaagcactgacatcaacagctagtaagaaacgttttccagttggttcaactgtcttaaatgttttataaaaagcagcatccaatgctttcaaaatttcttcatcagggcgccacttcagtttccctctgagaccatgacctgtcttgtaagtttctaatgcgatcaaaatatgaaatggatgtatacgagccttttttaatagtttttcattacacagtttttcacatactaaagatacttctgaatttcctggttcaagtactgaattagcagtcatctttcctagattccttagtaatgcagtaagcggcatttcttgtaacaaagccttccatacctctttagactttaagtgatttgttaaaagatgttctctaactaatctatgttcttctattagatgaatgacttctagctcatctcttgtgcgcttcactttctctacagcctccagatactttaataatttttcagtctccacagagagtgctttttctttatacaattcatgaacttctttccagccctttgtaatatatttggtcacaattgcaagtccttcactggaaggtttaagatgtgacaatcttaatagatctttgtgagaccagccatttctctgtttatattttgtaactgccagagcaagggccatgccacctttctcattgtaccagtccgctatagccttccggagggcacgaccccacatgccacatttcatgctttccttcagatctttcttaaactggataaaagtaaagagatgggtaggaatgcgacaaacttcagaaacagctttaaatgctgcttgttttgtgcttatgtcggagcactgggaacaaatggcaagtgcaaagagcataggctcttgctttgtggttctgccttcttgactaaatgactttatttcttgtatcacttcacatcctctgccatcttcaatcaatctaattaaagcttcagcattttcaaggcccaacttctgttctttgatataataagtcccaccttcagaaccgaaacataagaaccggtgtagtcgattcatgtcagtgacttgccatacatatccatcctgagaattggctatctgcttctcattcagtggctgcatttggtttacagattcctccatttttttttgtctttaggaaacaagacatatacagcaacttaatttcttctttctccaactgccatcatctcctgcctcaaagcttaagctccattatcagtggtttagaaggcaattgggcagtgagtgaggtcagaacctggtcatcagttaatccattcctggataatcaagtgttgtaaatccagattaacaacaaaaagatatagttaattctttggatgggcctgacctatctatctagtgctcttaaaacacaccatacaactaatgttgtattaaatctctataaattaagttcttgagaagttaaatattacaatactataatattaaaagcatggacactt

SEQ ID NO: 12328 - RNA, 5173 nt, Homo sapiens
  source 1..5173: mol_type = other RNA
ctgggaggtcaaggctgcagtgagctgtgatcatgccactccagcctgggtgacagagggatagcctgtctcaaaaaaaaaagtttgttaacagcatttcctcagagtataagcttgtttttctaggtctgtccaagaagatcttggagtatattttttctccctcttcagtagagaatagtgactttttgggtaatactttagctgtgaaaatttttcttctaaatttttctactctgaacaggaatgttttaaaacactgttaggcctattgagtgagctatttttctaaaacattttatcttttgaaatacgtatcttattaacaagaatgtttttaaccaaaaaaaaaaagaattctaacttgtattgcaagccctcttcccagtttcaatttttatacaaatattaaatcactgattcttctatgatccaagcacagatatgttactttttaaggataaaaataatcaaatcacttaggttaaactggttgtctacagtcacacagtaagttagataaagcaaaggaggtgtcaaagggtaacactaaattccattcactagcatcttgcctcactaacactctcataagatagattactaaataatataagtattaataaatggaatttccaagaactttcaactaataaagggtgggattataagattagtttttgttttactaattacaactatatcctggaactatttacatactacctaggaaataaagtttgtttattcttgcaggattgtttttaaaagcagtattttcccaaatattaatttaacagtaatcctaaaagtaactcaggaaataaaaaacttatcacttcagtacattttattcataatgaggtaaagtttttgttttttctctatatatgtagatatatatagcaacacaggttaattgtgcttgaggattcctatgaattacaagattatacatgttcccattctatttttctactcctaaagcaatcgtatatacattatttcctaataactcaataaggtaaaagtcttaaataattttattttatcctctactcttctgagaccatgtattcccatgttgtggggaaataaattctggcacaggaatgaagagaccaagatttctaggttatagtacttcaaaatcacactctgtcttggacctcagctctctaacaaaaatttaaaaaattagcttttaggtttctaaggtttcttccagctcaaatatgccatgatttgaaaagttaccttctgtggtagcttctcctacttatcctttctttcttaaatgttaccctagtccatttaattagacctacctaaatacttcagaaaggtcatatccatccaatcttgtatccttgatggatttaatattaacttatagatatatttgtctaaaagtattatggaaatagtacacaactgaaggtaatgcacttttgtactatattctatttaacatttctattaggaataaaatgatcatgttataatttttaagatcttgggtttacttaaacaattcaataactattacgtaattctattagtttctttaaactttaaattcaatctgaacgtaatattttaatgtgtcaaaagtagctaatatattcagttcaatgcttgacagggttaaaaacgtgaacaacatcagaagcaatgcatgtctggagtgggggtgagggtgctatgagctttgctgaacaaaaatatctcaggtaaatcacacttaaaaactgataccagttgccttgaaggaatgggtacatatcaaaaccagcattaatatgtcaaataaatttgaaaggaatattttcttattcccagagcccaaatttcacataaaacagaagaaaatatgtacagaaatcctcagactactaaagtccccctttcccaaaaaacataaaccctctaacccccaagcacctaaaaggctataatttacattaactacagtttgacttttcacataacagcgagaaggaccttacaaatcctcagtaaatcttcaattaatatttagagaacaacagatacgcaaacaggttttatgtgtaagctaccttagacggccataataaaattatgagcaaagataatggcatttcaacagattgctttaatgttaaacctcacaatgaaggatacttgctcaataaaataatgcactttagtgtaatgaaaagtttaatacatacaaataatactgaaaaaaattcctagtgactggctagctggtaatatgctactcaaaaattgcctttcaaacctaaaggacctagattgctttattatttgtttacactatcaaagaagaatattttgccacaaaatgaataatggacaaagaggccattgacatgtatacttttaaaaatattaactaaaaaaatagttaaaagtaaaaaattttattttaaaagtaaggaaaaagctaaactggttatagttgagattttaattgttatactttgtgaatgagggggagttaagcgcttgaaacattttatattatttacacttaagagtatgaaaaacagtgtgagactacatctggctatgttattataattcagaggaaatcattatcaagtcacaccccttgtagcaataaaatataacaaagcaaaaaaaaaaaagcaaaccaaatagaatccctcagccaacacaaacttagtctattcttaggggttgccatgatgtttctgattaatggtaacatattccacaagtgcaaataaaacatcagaaataaaatatctttttcactgaataagaaagctgttatttgtgtgatcttagtaaaactctgaaaggaatttgtaaaactcattcataatttaatcaaatgccttagtttttttttttacccccttggtataaaagtttacagatgagtttcatatttcatcacagttatatggtctagtgcatttcagagtatttggacattatcaaagctgtcctttcccaatgaaaacatttaagaaaacgttaagcacttctcaagtaacatgatgtggaattacactttttgctcttacctcttttaggtacacacgtattattcaacaaagcaaaactattttacagtgtctgttaacaaaaagttctctattagatagaggaaactacagtatcctgaagctatttccccaagagctagtttagtagatagacctttgggcccatcttatttttccttcttttttttttttcagtaaggtaactttccattatgcacatactataccatcatcattcattgggtggagattagctgggaagtagctgtatatttttagtgagatcactgatggcaatggatctctggatcgtgctgctgcttatggttaaatcatatctaatgtgaaatttcgaattacatccagagctccagtatcaaagccgcacatatccaacatgcctctatcatctgggtctgcaatggtgaaaccatttgatgtcattccacaaacaatcaatttagctggaatatccattttctttcgatactccctcagagcaatagcaggatggacacctccagcaaaggtctcattatcagtgaatacaatgaagacatcagcaggtgtgtttgtcttctgagcccagatcattggaagagagcaatcagttccacctgctgggatctgactcatagccattaaaacctgttgtaaggtcatatctgtagtcactggacatggtaccatttcatcggaaaaagcaactacataagaatctttttctgttcgtgtgacaaccatgcacattgctgcagcaactgtactagcgttgagtatactacccaaaactctttggttcatagaagcactgacatcaacagctagtaagaaacgttttccagttggttcaactgtcttaaatgttttataaaaagcagcatccaatgctttcaaaatttcttcatcagggcgccacttcagtttccctctgagaccatgacctgtcttgtaagtttctaatgcgatcaaaatatgaaatggatgtatacgagccttttttaatagtttttcattacacagtttttcacatactaaagatacttctgaatttcctggttcaagtactgaattagcagtcatctttcctagattccttagtaatgcagtaagcggcatttcttgtaacaaagccttccatacctctttagactttaagtgatttgttaaaagatgttctctaactaatctatgttcttctattagatgaatgacttctagctcatctcttgtgcgcttcactttctctacagcctccagatactttaataatttttcagtctccacagagagtgctttttctttatacaattcatgaacttctttccagccctttgtaatatatttggtcacaattgcaagtccttcactggaaggtttaagatgtgacaatcttaatagatctttgtgagaccagccatttctctgtttatattttgtaactgccagagcaagggccatgccacctttctcattgtaccagtccgctatagccttccggagggcacgaccccacatgccacatttcatgctttccttcagatctttcttaaactggataaaagtaaagagatgggtaggaatgcgacaaacttcagaaacagctttaaatgctgcttgttttgtgcttatgtcggagcactgggaacaaatggcaagtgcaaagagcataggctcttgctttgtggttctgccttcttgactaaatgactttatttcttgtatcacttcacatcctctgccatcttcaatcaatctaattaaagcttcagcattttcaaggcccaacttctgttctttgatataataagtcccaccttcagaaccgaaacataagaaccggtgtagtcgattcatgtcagtgacttgccatacatatccatcctgagaattggctatctgcttctcattcagtggctgcatttggtttacagattcctccatttttttttgtctttaggaaacctggcagccgaccccctggatccgcagcgccgccaggagaagtcctgcgcagcgctgggaaacgacaaaagaaggcagcctgacgggcagcgacagccacagcaacagcaacagccccactgccgccggggattccaggttcggttcccgggaacgagtcctgc

SEQ ID NO: 12329 - RNA, 5174 nt, Homo sapiens
  source 1..5174: mol_type = other RNA
ctgggaggtcaaggctgcagtgagctgtgatcatgccactccagcctgggtgacagagggatagcctgtctcaaaaaaaaaagtttgttaacagcatttcctcagagtataagcttgtttttctaggtctgtccaagaagatcttggagtatattttttctccctcttcagtagagaatagtgactttttgggtaatactttagctgtgaaaatttttcttctaaatttttctactctgaacaggaatgttttaaaacactgttaggcctattgagtgagctatttttctaaaacattttatcttttgaaatacgtatcttattaacaagaatgtttttaaccaaaaaaaaaaagaattctaacttgtattgcaagccctcttcccagtttcaatttttatacaaatattaaatcactgattcttctatgatccaagcacagatatgttactttttaaggataaaaataatcaaatcacttaggttaaactggttgtctacagtcacacagtaagttagataaagcaaaggaggtgtcaaagggtaacactaaattccattcactagcatcttgcctcactaacactctcataagatagattactaaataatataagtattaataaatggaatttccaagaactttcaactaataaagggtgggattataagattagtttttgttttactaattacaactatatcctggaactatttacatactacctaggaaataaagtttgtttattcttgcaggattgtttttaaaagcagtattttcccaaatattaatttaacagtaatcctaaaagtaactcaggaaataaaaaacttatcacttcagtacattttattcataatgaggtaaagtttttgttttttctctatatatgtagatatatatagcaacacaggttaattgtgcttgaggattcctatgaattacaagattatacatgttcccattctatttttctactcctaaagcaatcgtatatacattatttcctaataactcaataaggtaaaagtcttaaataattttattttatcctctactcttctgagaccatgtattcccatgttgtggggaaataaattctggcacaggaatgaagagaccaagatttctaggttatagtacttcaaaatcacactctgtcttggacctcagctctctaacaaaaatttaaaaaattagcttttaggtttctaaggtttcttccagctcaaatatgccatgatttgaaaagttaccttctgtggtagcttctcctacttatcctttctttcttaaatgttaccctagtccatttaattagacctacctaaatacttcagaaaggtcatatccatccaatcttgtatccttgatggatttaatattaacttatagatatatttgtctaaaagtattatggaaatagtacacaactgaaggtaatgcacttttgtactatattctatttaacatttctattaggaataaaatgatcatgttataatttttaagatcttgggtttacttaaacaattcaataactattacgtaattctattagtttctttaaactttaaattcaatctgaacgtaatattttaatgtgtcaaaagtagctaatatattcagttcaatgcttgacagggttaaaaacgtgaacaacatcagaagcaatgcatgtctggagtgggggtgagggtgctatgagctttgctgaacaaaaatatctcaggtaaatcacacttaaaaactgataccagttgccttgaaggaatgggtacatatcaaaaccagcattaatatgtcaaataaatttgaaaggaatattttcttattcccagagcccaaatttcacataaaacagaagaaaatatgtacagaaatcctcagactactaaagtccccctttcccaaaaaacataaaccctctaacccccaagcacctaaaaggctataatttacattaactacagtttgacttttcacataacagcgagaaggaccttacaaatcctcagtaaatcttcaattaatatttagagaacaacagatacgcaaacaggttttatgtgtaagctaccttagacggccataataaaattatgagcaaagataatggcatttcaacagattgctttaatgttaaacctcacaatgaaggatacttgctcaataaaataatgcactttagtgtaatgaaaagtttaatacatacaaataatactgaaaaaaattcctagtgactggctagctggtaatatgctactcaaaaattgcctttcaaacctaaaggacctagattgctttattatttgtttacactatcaaagaagaatattttgccacaaaatgaataatggacaaagaggccattgacatgtatacttttaaaaatattaactaaaaaaatagttaaaagtaaaaaattttattttaaaagtaaggaaaaagctaaactggttatagttgagattttaattgttatactttgtgaatgagggggagttaagcgcttgaaacattttatattatttacacttaagagtatgaaaaacagtgtgagactacatctggctatgttattataattcagaggaaatcattatcaagtcacaccccttgtagcaataaaatataacaaagcaaaaaaaaaaaagcaaaccaaatagaatccctcagccaacacaaacttagtctattcttaggggttgccatgatgtttctgattaatggtaacatattccacaagtgcaaataaaacatcagaaataaaatatctttttcactgaataagaaagctgttatttgtgtgatcttagtaaaactctgaaaggaatttgtaaaactcattcataatttaatcaaatgccttagtttttttttttacccccttggtataaaagtttacagatgagtttcatatttcatcacagttatatggtctagtgcatttcagagtatttggacattatcaaagctgtcctttcccaatgaaaacatttaagaaaacgttaagcacttctcaagtaacatgatgtggaattacactttttgctcttacctcttttaggtacacacgtattattcaacaaagcaaaactattttacagtgtctgttaacaaaaagttctctattagatagaggaaactacagtatcctgaagctatttccccaagagctagtttagtagatagacctttgggcccatcttatttttccttcttttttttttttcagtaaggtaactttccattatgcacatactataccatcatcattcattgggtggagattagctgggaagtagctgtatatttttagtgagatcactgatggcaatggatctctggatcgtgctgctgcttatggttaaatcatatctaatgtgaaatttcgaattacatccagagctccagtatcaaagccgcacatatccaacatgcctctatcatctgggtctgcaatggtgaaaccatttgatgtcattccacaaacaatcaatttagctggaatatccattttctttcgatactccctcagagcaatagcaggatggacacctccagcaaaggtctcattatcagtgaatacaatgaagacatcagcaggtgtgtttgtcttctgagcccagatcattggaagagagcaatcagttccacctgctgggatctgactcatagccattaaaacctgttgtaaggtcatatctgtagtcactggacatggtaccatttcatcggaaaaagcaactacataagaatctttttctgttcgtgtgacaaccatgcacattgctgcagcaactgtactagcgttgagtatactacccaaaactctttggttcatagaagcactgacatcaacagctagtaagaaacgttttccagttggttcaactgtcttaaatgttttataaaaagcagcatccaatgctttcaaaatttcttcatcagggcgccacttcagtttccctctgagaccatgacctgtcttgtaagtttctaatgcgatcaaaatatgaaatggatgtatacgagccttttttaatagtttttcattacacagtttttcacatactaaagatacttctgaatttcctggttcaagtactgaattagcagtcatctttcctagattccttagtaatgcagtaagcggcatttcttgtaacaaagccttccatacctctttagactttaagtgatttgttaaaagatgttctctaactaatctatgttcttctattagatgaatgacttctagctcatctcttgtgcgcttcactttctctacagcctccagatactttaataatttttcagtctccacagagagtgctttttctttatacaattcatgaacttctttccagccctttgtaatatatttggtcacaattgcaagtccttcactggaaggtttaagatgtgacaatcttaatagatctttgtgagaccagccatttctctgtttatattttgtaactgccagagcaagggccatgccacctttctcattgtaccagtccgctatagccttccggagggcacgaccccacatgccacatttcatgctttccttcagatctttcttaaactggataaaagtaaagagatgggtaggaatgcgacaaacttcagaaacagctttaaatgctgcttgttttgtgcttatgtcggagcactgggaacaaatggcaagtgcaaagagcataggctcttgctttgtggttctgccttcttgactaaatgactttatttcttgtatcacttcacatcctctgccatcttcaatcaatctaattaaagcttcagcattttcaaggcccaacttctgttctttgatataataagtcccaccttcagaaccgaaacataagaaccggtgtagtcgattcatgtcagtgacttgccatacatatccatcctgagaattggctatctgcttctcattcagtggctgcatttggtttacagattcctccatttttttttgtctttaggaaacctgtacctggcagccgaccccctggatccgcagcgccgccaggagaagtcctgcgcagcgctgggaaacgacaaaagaaggcagcctgacgggcagcgacagccacagcaacagcaacagccccactgccgccggggattccaggttcggttcccgggaacgagt

SEQ ID NO: 12330 - RNA, 5564 nt, Homo sapiens
  source 1..5564: mol_type = other RNA
ctgggaggtcaaggctgcagtgagctgtgatcatgccactccagcctgggtgacagagggatagcctgtctcaaaaaaaaaagtttgttaacagcatttcctcagagtataagcttgtttttctaggtctgtccaagaagatcttggagtatattttttctccctcttcagtagagaatagtgactttttgggtaatactttagctgtgaaaatttttcttctaaatttttctactctgaacaggaatgttttaaaacactgttaggcctattgagtgagctatttttctaaaacattttatcttttgaaatacgtatcttattaacaagaatgtttttaaccaaaaaaaaaaagaattctaacttgtattgcaagccctcttcccagtttcaatttttatacaaatattaaatcactgattcttctatgatccaagcacagatatgttactttttaaggataaaaataatcaaatcacttaggttaaactggttgtctacagtcacacagtaagttagataaagcaaaggaggtgtcaaagggtaacactaaattccattcactagcatcttgcctcactaacactctcataagatagattactaaataatataagtattaataaatggaatttccaagaactttcaactaataaagggtgggattataagattagtttttgttttactaattacaactatatcctggaactatttacatactacctaggaaataaagtttgtttattcttgcaggattgtttttaaaagcagtattttcccaaatattaatttaacagtaatcctaaaagtaactcaggaaataaaaaacttatcacttcagtacattttattcataatgaggtaaagtttttgttttttctctatatatgtagatatatatagcaacacaggttaattgtgcttgaggattcctatgaattacaagattatacatgttcccattctatttttctactcctaaagcaatcgtatatacattatttcctaataactcaataaggtaaaagtcttaaataattttattttatcctctactcttctgagaccatgtattcccatgttgtggggaaataaattctggcacaggaatgaagagaccaagatttctaggttatagtacttcaaaatcacactctgtcttggacctcagctctctaacaaaaatttaaaaaattagcttttaggtttctaaggtttcttccagctcaaatatgccatgatttgaaaagttaccttctgtggtagcttctcctacttatcctttctttcttaaatgttaccctagtccatttaattagacctacctaaatacttcagaaaggtcatatccatccaatcttgtatccttgatggatttaatattaacttatagatatatttgtctaaaagtattatggaaatagtacacaactgaaggtaatgcacttttgtactatattctatttaacatttctattaggaataaaatgatcatgttataatttttaagatcttgggtttacttaaacaattcaataactattacgtaattctattagtttctttaaactttaaattcaatctgaacgtaatattttaatgtgtcaaaagtagctaatatattcagttcaatgcttgacagggttaaaaacgtgaacaacatcagaagcaatgcatgtctggagtgggggtgagggtgctatgagctttgctgaacaaaaatatctcaggtaaatcacacttaaaaactgataccagttgccttgaaggaatgggtacatatcaaaaccagcattaatatgtcaaataaatttgaaaggaatattttcttattcccagagcccaaatttcacataaaacagaagaaaatatgtacagaaatcctcagactactaaagtccccctttcccaaaaaacataaaccctctaacccccaagcacctaaaaggctataatttacattaactacagtttgacttttcacataacagcgagaaggaccttacaaatcctcagtaaatcttcaattaatatttagagaacaacagatacgcaaacaggttttatgtgtaagctaccttagacggccataataaaattatgagcaaagataatggcatttcaacagattgctttaatgttaaacctcacaatgaaggatacttgctcaataaaataatgcactttagtgtaatgaaaagtttaatacatacaaataatactgaaaaaaattcctagtgactggctagctggtaatatgctactcaaaaattgcctttcaaacctaaaggacctagattgctttattatttgtttacactatcaaagaagaatattttgccacaaaatgaataatggacaaagaggccattgacatgtatacttttaaaaatattaactaaaaaaatagttaaaagtaaaaaattttattttaaaagtaaggaaaaagctaaactggttatagttgagattttaattgttatactttgtgaatgagggggagttaagcgcttgaaacattttatattatttacacttaagagtatgaaaaacagtgtgagactacatctggctatgttattataattcagaggaaatcattatcaagtcacaccccttgtagcaataaaatataacaaagcaaaaaaaaaaaagcaaaccaaatagaatccctcagccaacacaaacttagtctattcttaggggttgccatgatgtttctgattaatggtaacatattccacaagtgcaaataaaacatcagaaataaaatatctttttcactgaataagaaagctgttatttgtgtgatcttagtaaaactctgaaaggaatttgtaaaactcattcataatttaatcaaatgccttagtttttttttttacccccttggtataaaagtttacagatgagtttcatatttcatcacagttatatggtctagtgcatttcagagtatttggacattatcaaagctgtcctttcccaatgaaaacatttaagaaaacgttaagcacttctcaagtaacatgatgtggaattacactttttgctcttacctcttttaggtacacacgtattattcaacaaagcaaaactattttacagtgtctgttaacaaaaagttctctattagatagaggaaactacagtatcctgaagctatttccccaagagctagtttagtagatagacctttgggcccatcttatttttccttcttttttttttttcagtaaggtaactttccattatgcacatactataccatcatcattcattgggtggagattagctgggaagtagctgtatatttttagtgagatcactgatggcaatggatctctggatcgtgctgctgcttatggttaaatcatatctaatgtgaaatttcgaattacatccagagctccagtatcaaagccgcacatatccaacatgcctctatcatctgggtctgcaatggtgaaaccatttgatgtcattccacaaacaatcaatttagctggaatatccattttctttcgatactccctcagagcaatagcaggatggacacctccagcaaaggtctcattatcagtgaatacaatgaagacatcagcaggtgtgtttgtcttctgagcccagatcattggaagagagcaatcagttccacctgctgggatctgactcatagccattaaaacctgttgtaaggtcatatctgtagtcactggacatggtaccatttcatcggaaaaagcaactacataagaatctttttctgttcgtgtgacaaccatgcacattgctgcagcaactgtactagcgttgagtatactacccaaaactctttggttcatagaagcactgacatcaacagctagtaagaaacgttttccagttggttcaactgtcttaaatgttttataaaaagcagcatccaatgctttcaaaatttcttcatcagggcgccacttcagtttccctctgagaccatgacctgtcttgtaagtttctaatgcgatcaaaatatgaaatggatgtatacgagccttttttaatagtttttcattacacagtttttcacatactaaagatacttctgaatttcctggttcaagtactgaattagcagtcatctttcctagattccttagtaatgcagtaagcggcatttcttgtaacaaagccttccatacctctttagactttaagtgatttgttaaaagatgttctctaactaatctatgttcttctattagatgaatgacttctagctcatctcttgtgcgcttcactttctctacagcctccagatactttaataatttttcagtctccacagagagtgctttttctttatacaattcatgaacttctttccagccctttgtaatatatttggtcacaattgcaagtccttcactggaaggtttaagatgtgacaatcttaatagatctttgtgagaccagccatttctctgtttatattttgtaactgccagagcaagggccatgccacctttctcattgtaccagtccgctatagccttccggagggcacgaccccacatgccacatttcatgctttccttcagatctttcttaaactggataaaagtaaagagatgggtaggaatgcgacaaacttcagaaacagctttaaatgctgcttgttttgtgcttatgtcggagcactgggaacaaatggcaagtgcaaagagcataggctcttgctttgtggttctgccttcttgactaaatgactttatttcttgtatcacttcacatcctctgccatcttcaatcaatctaattaaagcttcagcattttcaaggcccaacttctgttctttgatataataagtcccaccttcagaaccgaaacataagaaccggtgtagtcgattcatgtcagtgacttgccatacatatccatcctgagaattggctatctgcttctcattcagtggctgcatttggtttacagattcctccatttttttttgtctttaggaaacctttctcctctccctcgttattcctctgtgataaattcaccctgtcttcccacaaagatccttcttccaaaacccagatcccgggcgacgcctctccgcgcagaagccgcgggagaaggaggagaaagaggaggagtaaagcaggccctctcgacgtcggcctgtggggagcgatgccgacaagcaggagcggtcccggcttcggaaagggcccaccctgaggaatggtccggccgggcctagcgaggatgtccctaccgcgatgctggttccgttacccagggtggacaggcgcggaagcgggacggggaagagcgatagtttcgcggcgtttgcccagcctcaacccctggcagccgaccccctggatccgcagcgccgccaggagaagtcctgcgcagcgctgggaaacgacaaaagaaggcagcctgacgggcagcgacagccacagcaacagcaacagccccactgccgccggggattccaggttcggttcccgggaacgagtcctgcccctcttcttttgccccgcctccgccccagaggggcgaggat

SEQ ID NO: 12331 - RNA, 5540 nt, Homo sapiens
  source 1..5540: mol_type = other RNA
ctgggaggtcaaggctgcagtgagctgtgatcatgccactccagcctgggtgacagagggatagcctgtctcaaaaaaaaaagtttgttaacagcatttcctcagagtataagcttgtttttctaggtctgtccaagaagatcttggagtatattttttctccctcttcagtagagaatagtgactttttgggtaatactttagctgtgaaaatttttcttctaaatttttctactctgaacaggaatgttttaaaacactgttaggcctattgagtgagctatttttctaaaacattttatcttttgaaatacgtatcttattaacaagaatgtttttaaccaaaaaaaaaaagaattctaacttgtattgcaagccctcttcccagtttcaatttttatacaaatattaaatcactgattcttctatgatccaagcacagatatgttactttttaaggataaaaataatcaaatcacttaggttaaactggttgtctacagtcacacagtaagttagataaagcaaaggaggtgtcaaagggtaacactaaattccattcactagcatcttgcctcactaacactctcataagatagattactaaataatataagtattaataaatggaatttccaagaactttcaactaataaagggtgggattataagattagtttttgttttactaattacaactatatcctggaactatttacatactacctaggaaataaagtttgtttattcttgcaggattgtttttaaaagcagtattttcccaaatattaatttaacagtaatcctaaaagtaactcaggaaataaaaaacttatcacttcagtacattttattcataatgaggtaaagtttttgttttttctctatatatgtagatatatatagcaacacaggttaattgtgcttgaggattcctatgaattacaagattatacatgttcccattctatttttctactcctaaagcaatcgtatatacattatttcctaataactcaataaggtaaaagtcttaaataattttattttatcctctactcttctgagaccatgtattcccatgttgtggggaaataaattctggcacaggaatgaagagaccaagatttctaggttatagtacttcaaaatcacactctgtcttggacctcagctctctaacaaaaatttaaaaaattagcttttaggtttctaaggtttcttccagctcaaatatgccatgatttgaaaagttaccttctgtggtagcttctcctacttatcctttctttcttaaatgttaccctagtccatttaattagacctacctaaatacttcagaaaggtcatatccatccaatcttgtatccttgatggatttaatattaacttatagatatatttgtctaaaagtattatggaaatagtacacaactgaaggtaatgcacttttgtactatattctatttaacatttctattaggaataaaatgatcatgttataatttttaagatcttgggtttacttaaacaattcaataactattacgtaattctattagtttctttaaactttaaattcaatctgaacgtaatattttaatgtgtcaaaagtagctaatatattcagttcaatgcttgacagggttaaaaacgtgaacaacatcagaagcaatgcatgtctggagtgggggtgagggtgctatgagctttgctgaacaaaaatatctcaggtaaatcacacttaaaaactgataccagttgccttgaaggaatgggtacatatcaaaaccagcattaatatgtcaaataaatttgaaaggaatattttcttattcccagagcccaaatttcacataaaacagaagaaaatatgtacagaaatcctcagactactaaagtccccctttcccaaaaaacataaaccctctaacccccaagcacctaaaaggctataatttacattaactacagtttgacttttcacataacagcgagaaggaccttacaaatcctcagtaaatcttcaattaatatttagagaacaacagatacgcaaacaggttttatgtgtaagctaccttagacggccataataaaattatgagcaaagataatggcatttcaacagattgctttaatgttaaacctcacaatgaaggatacttgctcaataaaataatgcactttagtgtaatgaaaagtttaatacatacaaataatactgaaaaaaattcctagtgactggctagctggtaatatgctactcaaaaattgcctttcaaacctaaaggacctagattgctttattatttgtttacactatcaaagaagaatattttgccacaaaatgaataatggacaaagaggccattgacatgtatacttttaaaaatattaactaaaaaaatagttaaaagtaaaaaattttattttaaaagtaaggaaaaagctaaactggttatagttgagattttaattgttatactttgtgaatgagggggagttaagcgcttgaaacattttatattatttacacttaagagtatgaaaaacagtgtgagactacatctggctatgttattataattcagaggaaatcattatcaagtcacaccccttgtagcaataaaatataacaaagcaaaaaaaaaaaagcaaaccaaatagaatccctcagccaacacaaacttagtctattcttaggggttgccatgatgtttctgattaatggtaacatattccacaagtgcaaataaaacatcagaaataaaatatctttttcactgaataagaaagctgttatttgtgtgatcttagtaaaactctgaaaggaatttgtaaaactcattcataatttaatcaaatgccttagtttttttttttacccccttggtataaaagtttacagatgagtttcatatttcatcacagttatatggtctagtgcatttcagagtatttggacattatcaaagctgtcctttcccaatgaaaacatttaagaaaacgttaagcacttctcaagtaacatgatgtggaattacactttttgctcttacctcttttaggtacacacgtattattcaacaaagcaaaactattttacagtgtctgttaacaaaaagttctctattagatagaggaaactacagtatcctgaagctatttccccaagagctagtttagtagatagacctttgggcccatcttatttttccttcttttttttttttcagtaaggtaactttccattatgcacatactataccatcatcattcattgggtggagattagctgggaagtagctgtatatttttagtgagatcactgatggcaatggatctctggatcgtgctgctgcttatggttaaatcatatctaatgtgaaatttcgaattacatccagagctccagtatcaaagccgcacatatccaacatgcctctatcatctgggtctgcaatggtgaaaccatttgatgtcattccacaaacaatcaatttagctggaatatccattttctttcgatactccctcagagcaatagcaggatggacacctccagcaaaggtctcattatcagtgaatacaatgaagacatcagcaggtgtgtttgtcttctgagcccagatcattggaagagagcaatcagttccacctgctgggatctgactcatagccattaaaacctgttgtaaggtcatatctgtagtcactggacatggtaccatttcatcggaaaaagcaactacataagaatctttttctgttcgtgtgacaaccatgcacattgctgcagcaactgtactagcgttgagtatactacccaaaactctttggttcatagaagcactgacatcaacagctagtaagaaacgttttccagttggttcaactgtcttaaatgttttataaaaagcagcatccaatgctttcaaaatttcttcatcagggcgccacttcagtttccctctgagaccatgacctgtcttgtaagtttctaatgcgatcaaaatatgaaatggatgtatacgagccttttttaatagtttttcattacacagtttttcacatactaaagatacttctgaatttcctggttcaagtactgaattagcagtcatctttcctagattccttagtaatgcagtaagcggcatttcttgtaacaaagccttccatacctctttagactttaagtgatttgttaaaagatgttctctaactaatctatgttcttctattagatgaatgacttctagctcatctcttgtgcgcttcactttctctacagcctccagatactttaataatttttcagtctccacagagagtgctttttctttatacaattcatgaacttctttccagccctttgtaatatatttggtcacaattgcaagtccttcactggaaggtttaagatgtgacaatcttaatagatctttgtgagaccagccatttctctgtttatattttgtaactgccagagcaagggccatgccacctttctcattgtaccagtccgctatagccttccggagggcacgaccccacatgccacatttcatgctttccttcagatctttcttaaactggataaaagtaaagagatgggtaggaatgcgacaaacttcagaaacagctttaaatgctgcttgttttgtgcttatgtcggagcactgggaacaaatggcaagtgcaaagagcataggctcttgctttgtggttctgccttcttgactaaatgactttatttcttgtatcacttcacatcctctgccatcttcaatcaatctaattaaagcttcagcattttcaaggcccaacttctgttctttgatataataagtcccaccttcagaaccgaaacataagaaccggtgtagtcgattcatgtcagtgacttgccatacatatccatcctgagaattggctatctgcttctcattcagtggctgcatttggtttacagattcctccatttttttttgtctttaggaaacctttctcctctccctcgttattcctctgtgataaattcaccctgtcttcccacaaagatccttcttccaaaacccagatcccgggcgacgcctctccgcgcagaagccgcgggagaaggaggagaaagaggaggagtaaagcaggccctctcgacgtcggcctgtggggagcgatgccgacaagcaggagcggtcccggcttcggaaagggcccaccctgaggaatggtccggccgggcctagcgaggatgtccctaccgcgatgctggttccgttacccagggtggacaggcgcggaagcgggacggggaagagcgatagtttcgcggcgtttgcccagcctcaacccctgtacctggcagccgaccccctggatccgcagcgccgccaggagaagtcctgcgcagcgctgggaaacgacaaaagaaggcagcctgacgggcagcgacagccacagcaacagcaacagccccactgccgccggggattccaggttcggttcccgggaacgagtcctgcccctcttctttt

SEQ ID NO: 12332 - RNA, 4939 nt, Homo sapiens
  source 1..4939: mol_type = other RNA
ctgggaggtcaaggctgcagtgagctgtgatcatgccactccagcctgggtgacagagggatagcctgtctcaaaaaaaaaagtttgttaacagcatttcctcagagtataagcttgtttttctaggtctgtccaagaagatcttggagtatattttttctccctcttcagtagagaatagtgactttttgggtaatactttagctgtgaaaatttttcttctaaatttttctactctgaacaggaatgttttaaaacactgttaggcctattgagtgagctatttttctaaaacattttatcttttgaaatacgtatcttattaacaagaatgtttttaaccaaaaaaaaaaagaattctaacttgtattgcaagccctcttcccagtttcaatttttatacaaatattaaatcactgattcttctatgatccaagcacagatatgttactttttaaggataaaaataatcaaatcacttaggttaaactggttgtctacagtcacacagtaagttagataaagcaaaggaggtgtcaaagggtaacactaaattccattcactagcatcttgcctcactaacactctcataagatagattactaaataatataagtattaataaatggaatttccaagaactttcaactaataaagggtgggattataagattagtttttgttttactaattacaactatatcctggaactatttacatactacctaggaaataaagtttgtttattcttgcaggattgtttttaaaagcagtattttcccaaatattaatttaacagtaatcctaaaagtaactcaggaaataaaaaacttatcacttcagtacattttattcataatgaggtaaagtttttgttttttctctatatatgtagatatatatagcaacacaggttaattgtgcttgaggattcctatgaattacaagattatacatgttcccattctatttttctactcctaaagcaatcgtatatacattatttcctaataactcaataaggtaaaagtcttaaataattttattttatcctctactcttctgagaccatgtattcccatgttgtggggaaataaattctggcacaggaatgaagagaccaagatttctaggttatagtacttcaaaatcacactctgtcttggacctcagctctctaacaaaaatttaaaaaattagcttttaggtttctaaggtttcttccagctcaaatatgccatgatttgaaaagttaccttctgtggtagcttctcctacttatcctttctttcttaaatgttaccctagtccatttaattagacctacctaaatacttcagaaaggtcatatccatccaatcttgtatccttgatggatttaatattaacttatagatatatttgtctaaaagtattatggaaatagtacacaactgaaggtaatgcacttttgtactatattctatttaacatttctattaggaataaaatgatcatgttataatttttaagatcttgggtttacttaaacaattcaataactattacgtaattctattagtttctttaaactttaaattcaatctgaacgtaatattttaatgtgtcaaaagtagctaatatattcagttcaatgcttgacagggttaaaaacgtgaacaacatcagaagcaatgcatgtctggagtgggggtgagggtgctatgagctttgctgaacaaaaatatctcaggtaaatcacacttaaaaactgataccagttgccttgaaggaatgggtacatatcaaaaccagcattaatatgtcaaataaatttgaaaggaatattttcttattcccagagcccaaatttcacataaaacagaagaaaatatgtacagaaatcctcagactactaaagtccccctttcccaaaaaacataaaccctctaacccccaagcacctaaaaggctataatttacattaactacagtttgacttttcacataacagcgagaaggaccttacaaatcctcagtaaatcttcaattaatatttagagaacaacagatacgcaaacaggttttatgtgtaagctaccttagacggccataataaaattatgagcaaagataatggcatttcaacagattgctttaatgttaaacctcacaatgaaggatacttgctcaataaaataatgcactttagtgtaatgaaaagtttaatacatacaaataatactgaaaaaaattcctagtgactggctagctggtaatatgctactcaaaaattgcctttcaaacctaaaggacctagattgctttattatttgtttacactatcaaagaagaatattttgccacaaaatgaataatggacaaagaggccattgacatgtatacttttaaaaatattaactaaaaaaatagttaaaagtaaaaaattttattttaaaagtaaggaaaaagctaaactggttatagttgagattttaattgttatactttgtgaatgagggggagttaagcgcttgaaacattttatattatttacacttaagagtatgaaaaacagtgtgagactacatctggctatgttattataattcagaggaaatcattatcaagtcacaccccttgtagcaataaaatataacaaagcaaaaaaaaaaaagcaaaccaaatagaatccctcagccaacacaaacttagtctattcttaggggttgccatgatgtttctgattaatggtaacatattccacaagtgcaaataaaacatcagaaataaaatatctttttcactgaataagaaagctgttatttgtgtgatcttagtaaaactctgaaaggaatttgtaaaactcattcataatttaatcaaatgccttagtttttttttttacccccttggtataaaagtttacagatgagtttcatatttcatcacagttatatggtctagtgcatttcagagtatttggacattatcaaagctgtcctttcccaatgaaaacatttaagaaaacgttaagcacttctcaagtaacatgatgtggaattacactttttgctcttacctcttttaggtacacacgtattattcaacaaagcaaaactattttacagtgtctgttaacaaaaagttctctattagatagaggaaactacagtatcctgaagctatttccccaagagctagtttagtagatagacctttgggcccatcttatttttccttcttttttttttttcagtaaggtaactttccattatgcacatactataccatcatcattcattgggtggagattagctgggaagtagctgtatatttttagtgagatcactgatggcaatggatctctggatcgtgctgctgcttatggttaaatcatatctaatgtgaaatttcgaattacatccagagctccagtatcaaagccgcacatatccaacatgcctctatcatctgggtctgcaatggtgaaaccatttgatgtcattccacaaacaatcaatttagctggaatatccattttctttcgatactccctcagagcaatagcaggatggacacctccagcaaaggtctcattatcagtgaatacaatgaagacatcagcaggtgtgtttgtcttctgagcccagatcattggaagagagcaatcagttccacctgctgggatctgactcatagccattaaaacctgttgtaaggtcatatctgtagtcactggacatggtaccatttcatcggaaaaagcaactacataagaatctttttctgttcgtgtgacaaccatgcacattgctgcagcaactgtactagcgttgagtatactacccaaaactctttggttcatagaagcactgacatcaacagctagtaagaaacgttttccagttggttcaactgtcttaaatgttttataaaaagcagcatccaatgctttcaaaatttcttcatcagggcgccacttcagtttccctctgagaccatgacctgtcttgtaagtttctaatgcgatcaaaatatgaaatggatgtatacgagccttttttaatagtttttcattacacagtttttcacatactaaagatacttctgaatttcctggttcaagtactgaattagcagtcatctttcctagattccttagtaatgcagtaagcggcatttcttgtaacaaagccttccatacctctttagactttaagtgatttgttaaaagatgttctctaactaatctatgttcttctattagatgaatgacttctagctcatctcttgtgcgcttcactttctctacagcctccagatactttaataatttttcagtctccacagagagtgctttttctttatacaattcatgaacttctttccagccctttgtaatatatttggtcacaattgcaagtcctttctcctctccctcgttattcctctgtgataaattcaccctgtcttcccacaaagatccttcttccaaaacccagatcccgggcgacgcctctccgcgcagaagccgcgggagaaggaggagaaagaggaggagtaaagcaggccctctcgacgtcggcctgtggggagcgatgccgacaagcaggagcggtcccggcttcggaaagggcccaccctgaggaatggtccggccgggcctagcgaggatgtccctaccgcgatgctggttccgttacccagggtggacaggcgcggaagcgggacggggaagagcgatagtttcgcggcgtttgcccagcctcaacccctgtacctggcagccgaccccctggatccgcagcgccgccaggagaagtcctgcgcagcgctgggaaacgacaaaagaaggcagcctgacgggcagcgacagccacagcaacagcaacagccccactgccgccggggattccaggttcggttcccgggaacgagtcctgcccctcttctttt

SEQ ID NO: 12333 - RNA, 5239 nt, Homo sapiens
  source 1..5239: mol_type = other RNA
ctgggaggtcaaggctgcagtgagctgtgatcatgccactccagcctgggtgacagagggatagcctgtctcaaaaaaaaaagtttgttaacagcatttcctcagagtataagcttgtttttctaggtctgtccaagaagatcttggagtatattttttctccctcttcagtagagaatagtgactttttgggtaatactttagctgtgaaaatttttcttctaaatttttctactctgaacaggaatgttttaaaacactgttaggcctattgagtgagctatttttctaaaacattttatcttttgaaatacgtatcttattaacaagaatgtttttaaccaaaaaaaaaaagaattctaacttgtattgcaagccctcttcccagtttcaatttttatacaaatattaaatcactgattcttctatgatccaagcacagatatgttactttttaaggataaaaataatcaaatcacttaggttaaactggttgtctacagtcacacagtaagttagataaagcaaaggaggtgtcaaagggtaacactaaattccattcactagcatcttgcctcactaacactctcataagatagattactaaataatataagtattaataaatggaatttccaagaactttcaactaataaagggtgggattataagattagtttttgttttactaattacaactatatcctggaactatttacatactacctaggaaataaagtttgtttattcttgcaggattgtttttaaaagcagtattttcccaaatattaatttaacagtaatcctaaaagtaactcaggaaataaaaaacttatcacttcagtacattttattcataatgaggtaaagtttttgttttttctctatatatgtagatatatatagcaacacaggttaattgtgcttgaggattcctatgaattacaagattatacatgttcccattctatttttctactcctaaagcaatcgtatatacattatttcctaataactcaataaggtaaaagtcttaaataattttattttatcctctactcttctgagaccatgtattcccatgttgtggggaaataaattctggcacaggaatgaagagaccaagatttctaggttatagtacttcaaaatcacactctgtcttggacctcagctctctaacaaaaatttaaaaaattagcttttaggtttctaaggtttcttccagctcaaatatgccatgatttgaaaagttaccttctgtggtagcttctcctacttatcctttctttcttaaatgttaccctagtccatttaattagacctacctaaatacttcagaaaggtcatatccatccaatcttgtatccttgatggatttaatattaacttatagatatatttgtctaaaagtattatggaaatagtacacaactgaaggtaatgcacttttgtactatattctatttaacatttctattaggaataaaatgatcatgttataatttttaagatcttgggtttacttaaacaattcaataactattacgtaattctattagtttctttaaactttaaattcaatctgaacgtaatattttaatgtgtcaaaagtagctaatatattcagttcaatgcttgacagggttaaaaacgtgaacaacatcagaagcaatgcatgtctggagtgggggtgagggtgctatgagctttgctgaacaaaaatatctcaggtaaatcacacttaaaaactgataccagttgccttgaaggaatgggtacatatcaaaaccagcattaatatgtcaaataaatttgaaaggaatattttcttattcccagagcccaaatttcacataaaacagaagaaaatatgtacagaaatcctcagactactaaagtccccctttcccaaaaaacataaaccctctaacccccaagcacctaaaaggctataatttacattaactacagtttgacttttcacataacagcgagaaggaccttacaaatcctcagtaaatcttcaattaatatttagagaacaacagatacgcaaacaggttttatgtgtaagctaccttagacggccataataaaattatgagcaaagataatggcatttcaacagattgctttaatgttaaacctcacaatgaaggatacttgctcaataaaataatgcactttagtgtaatgaaaagtttaatacatacaaataatactgaaaaaaattcctagtgactggctagctggtaatatgctactcaaaaattgcctttcaaacctaaaggacctagattgctttattatttgtttacactatcaaagaagaatattttgccacaaaatgaataatggacaaagaggccattgacatgtatacttttaaaaatattaactaaaaaaatagttaaaagtaaaaaattttattttaaaagtaaggaaaaagctaaactggttatagttgagattttaattgttatactttgtgaatgagggggagttaagcgcttgaaacattttatattatttacacttaagagtatgaaaaacagtgtgagactacatctggctatgttattataattcagaggaaatcattatcaagtcacaccccttgtagcaataaaatataacaaagcaaaaaaaaaaaagcaaaccaaatagaatccctcagccaacacaaacttagtctattcttaggggttgccatgatgtttctgattaatggtaacatattccacaagtgcaaataaaacatcagaaataaaatatctttttcactgaataagaaagctgttatttgtgtgatcttagtaaaactctgaaaggaatttgtaaaactcattcataatttaatcaaatgccttagtttttttttttacccccttggtataaaagtttacagatgagtttcatatttcatcacagttatatggtctagtgcatttcagagtatttggacattatcaaagctgtcctttcccaatgaaaacatttaagaaaacgttaagcacttctcaagtaacatgatgtggaattacactttttgctcttacctcttttaggtacacacgtattattcaacaaagcaaaactattttacagtgtctgttaacaaaaagttctctattagatagaggaaactacagtatcctgaagctatttccccaagagctagtttagtagatagacctttgggcccatcttatttttccttcttttttttttttcagtaaggtaactttccattatgcacatactataccatcatcattcattgggtggagattagctgggaagtagctgtatatttttagtgagatcactgatggcaatggatctctggatcgtgctgctgcttatggttaaatcatatctaatgtgaaatttcgaattacatccagagctccagtatcaaagccgcacatatccaacatgcctctatcatctgggtctgcaatggtgaaaccatttgatgtcattccacaaacaatcaatttagctggaatatccattttctttcgatactccctcagagcaatagcaggatggacacctccagcaaaggtctcattatcagtgaatacaatgaagacatcagcaggtgtgtttgtcttctgagcccagatcattggaagagagcaatcagttccacctgctgggatctgactcatagccattaaaacctgttgtaaggtcatatctgtagtcactggacatggtaccatttcatcggaaaaagcaactacataagaatctttttctgttcgtgtgacaaccatgcacattgctgcagcaactgtactagcgttgagtatactacccaaaactctttggttcatagaagcactgacatcaacagctagtaagaaacgttttccagttggttcaactgtcttaaatgttttataaaaagcagcatccaatgctttcaaaatttcttcatcagggcgccacttcagtttccctctgagaccatgacctgtcttgtaagtttctaatgcgatcaaaatatgaaatggatgtatacgagccttttttaatagtttttcattacacagtttttcacatactaaagatacttctgaatttcctggttcaagtactgaattagcagtcatctttcctagattccttagtaatgcagtaagcggcatttcttgtaacaaagccttccatacctctttagactttaagtgatttgttaaaagatgttctctaactaatctatgttcttctattagatgaatgacttctagctcatctcttgtgcgcttcactttctctacagcctccagatactttaataatttttcagtctccacagagagtgctttttctttatacaattcatgaacttctttccagccctttgtaatatatttggtcacaattgcaagtcttggcttaagtccacagaactgaaatgtgaacccacccttctgagtggctgtcttttcaagtttcacttcactggaaggtttaagatgtgacaatcttaatagatctttgtgagaccagccatttctctgtttatattttgtaactgccagagcaagggccatgccacctttctcattgtaccagtccgctatagccttccggagggcacgaccccacatgccacatttcatgctttccttcagatctttcttaaactggataaaagtaaagagatgggtaggaatgcgacaaacttcagaaacagctttaaatgctgcttgttttgtgcttatgtcggagcactgggaacaaatggcaagtgcaaagagcataggctcttgctttgtggttctgccttcttgactaaatgactttatttcttgtatcacttcacatcctctgccatcttcaatcaatctaattaaagcttcagcattttcaaggcccaacttctgttctttgatataataagtcccaccttcagaaccgaaacataagaaccggtgtagtcgattcatgtcagtgacttgccatacatatccatcctgagaattggctatctgcttctcattcagtggctgcatttggtttacagattcctccatttttttttgtctttaggaaacctggcagccgaccccctggatccgcagcgccgccaggagaagtcctgcgcagcgctgggaaacgacaaaagaaggcagcctgacgggcagcgacagccacagcaacagcaacagccccactgccgccggggattccaggttcggttcccgggaacgagtcctgc

SEQ ID NO: 12334 - RNA, 5368 nt, Homo sapiens
  source 1..5368: mol_type = other RNA
ctgggaggtcaaggctgcagtgagctgtgatcatgccactccagcctgggtgacagagggatagcctgtctcaaaaaaaaaagtttgttaacagcatttcctcagagtataagcttgtttttctaggtctgtccaagaagatcttggagtatattttttctccctcttcagtagagaatagtgactttttgggtaatactttagctgtgaaaatttttcttctaaatttttctactctgaacaggaatgttttaaaacactgttaggcctattgagtgagctatttttctaaaacattttatcttttgaaatacgtatcttattaacaagaatgtttttaaccaaaaaaaaaaagaattctaacttgtattgcaagccctcttcccagtttcaatttttatacaaatattaaatcactgattcttctatgatccaagcacagatatgttactttttaaggataaaaataatcaaatcacttaggttaaactggttgtctacagtcacacagtaagttagataaagcaaaggaggtgtcaaagggtaacactaaattccattcactagcatcttgcctcactaacactctcataagatagattactaaataatataagtattaataaatggaatttccaagaactttcaactaataaagggtgggattataagattagtttttgttttactaattacaactatatcctggaactatttacatactacctaggaaataaagtttgtttattcttgcaggattgtttttaaaagcagtattttcccaaatattaatttaacagtaatcctaaaagtaactcaggaaataaaaaacttatcacttcagtacattttattcataatgaggtaaagtttttgttttttctctatatatgtagatatatatagcaacacaggttaattgtgcttgaggattcctatgaattacaagattatacatgttcccattctatttttctactcctaaagcaatcgtatatacattatttcctaataactcaataaggtaaaagtcttaaataattttattttatcctctactcttctgagaccatgtattcccatgttgtggggaaataaattctggcacaggaatgaagagaccaagatttctaggttatagtacttcaaaatcacactctgtcttggacctcagctctctaacaaaaatttaaaaaattagcttttaggtttctaaggtttcttccagctcaaatatgccatgatttgaaaagttaccttctgtggtagcttctcctacttatcctttctttcttaaatgttaccctagtccatttaattagacctacctaaatacttcagaaaggtcatatccatccaatcttgtatccttgatggatttaatattaacttatagatatatttgtctaaaagtattatggaaatagtacacaactgaaggtaatgcacttttgtactatattctatttaacatttctattaggaataaaatgatcatgttataatttttaagatcttgggtttacttaaacaattcaataactattacgtaattctattagtttctttaaactttaaattcaatctgaacgtaatattttaatgtgtcaaaagtagctaatatattcagttcaatgcttgacagggttaaaaacgtgaacaacatcagaagcaatgcatgtctggagtgggggtgagggtgctatgagctttgctgaacaaaaatatctcaggtaaatcacacttaaaaactgataccagttgccttgaaggaatgggtacatatcaaaaccagcattaatatgtcaaataaatttgaaaggaatattttcttattcccagagcccaaatttcacataaaacagaagaaaatatgtacagaaatcctcagactactaaagtccccctttcccaaaaaacataaaccctctaacccccaagcacctaaaaggctataatttacattaactacagtttgacttttcacataacagcgagaaggaccttacaaatcctcagtaaatcttcaattaatatttagagaacaacagatacgcaaacaggttttatgtgtaagctaccttagacggccataataaaattatgagcaaagataatggcatttcaacagattgctttaatgttaaacctcacaatgaaggatacttgctcaataaaataatgcactttagtgtaatgaaaagtttaatacatacaaataatactgaaaaaaattcctagtgactggctagctggtaatatgctactcaaaaattgcctttcaaacctaaaggacctagattgctttattatttgtttacactatcaaagaagaatattttgccacaaaatgaataatggacaaagaggccattgacatgtatacttttaaaaatattaactaaaaaaatagttaaaagtaaaaaattttattttaaaagtaaggaaaaagctaaactggttatagttgagattttaattgttatactttgtgaatgagggggagttaagcgcttgaaacattttatattatttacacttaagagtatgaaaaacagtgtgagactacatctggctatgttattataattcagaggaaatcattatcaagtcacaccccttgtagcaataaaatataacaaagcaaaaaaaaaaaagcaaaccaaatagaatccctcagccaacacaaacttagtctattcttaggggttgccatgatgtttctgattaatggtaacatattccacaagtgcaaataaaacatcagaaataaaatatctttttcactgaataagaaagctgttatttgtgtgatcttagtaaaactctgaaaggaatttgtaaaactcattcataatttaatcaaatgccttagtttttttttttacccccttggtataaaagtttacagatgagtttcatatttcatcacagttatatggtctagtgcatttcagagtatttggacattatcaaagctgtcctttcccaatgaaaacatttaagaaaacgttaagcacttctcaagtaacatgatgtggaattacactttttgctcttacctcttttaggtacacacgtattattcaacaaagcaaaactattttacagtgtctgttaacaaaaagttctctattagatagaggaaactacagtatcctgaagctatttccccaagagctagtttagtagatagacctttgggcccatcttatttttccttcttttttttttttcagtaaggtaactttccattatgcacatactataccatcatcattcattgggtggagattagctgggaagtagctgtatatttttagtgagatcactgatggcaatggatctctggatcgtgctgctgcttatggttaaatcatatctaatgtgaaatttcgaattacatccagagctccagtatcaaagccgcacatatccaacatgcctctatcatctgggtctgcaatggtgaaaccatttgatgtcattccacaaacaatcaatttagctggaatatccattttctttcgatactccctcagagcaatagcaggatggacacctccagcaaaggtctcattatcagtgaatacaatgaagacatcagcaggtgtgtttgtcttctgagcccagatcattggaagagagcaatcagttccacctgctgggatctgactcatagccattaaaacctgttgtaaggtcatatctgtagtcactggacatggtaccatttcatcggaaaaagcaactacataagaatctttttctgttcgtgtgacaaccatgcacattgctgcagcaactgtactagcgttgagtatactacccaaaactctttggttcatagaagcactgacatcaacagctagtaagaaacgttttccagttggttcaactgtcttaaatgttttataaaaagcagcatccaatgctttcaaaatttcttcatcagggcgccacttcagtttccctctgagaccatgacctgtcttgtaagtttctaatgcgatcaaaatatgaaatggatgtatacgagccttttttaatagtttttcattacacagtttttcacatactaaagatacttctgaatttcctggttcaagtactgaattagcagtcatctttcctagattccttagtaatgcagtaagcggcatttcttgtaacaaagccttccatacctctttagactttaagtgatttgttaaaagatgttctctaactaatctatgttcttctattagatgaatgacttctagctcatctcttgtgcgcttcactttctctacagcctccagatactttaataatttttcagtctccacagagagtgctttttctttatacaattcatgaacttctttccagccctttgtaatatatttggtcacaattgcaagtcttggcttaagtccacagaactgaaatgtgaacccacccttctgagtggctgtcttttcaagtttcacttcactggaaggtttaagatgtgacaatcttaatagatctttgtgagaccagccatttctctgtttatattttgtaactgccagagcaagggccatgccacctttctcattgtaccagtccgctatagccttccggagggcacgaccccacatgccacatttcatgctttccttcagatctttcttaaactggataaaagtaaagagatgggtaggaatgcgacaaacttcagaaacagctttaaatgctgcttgttttgtgcttatgtcggagcactgggaacaaatggcaagtgcaaagagcataggctcttgctttgtggttctgccttcttgactaaatgactttatttcttgtatcacttcacatcctctgccatcttcaatcaatctaattaaagcttcagcattttcaaggcccaacttctgttctttgatataataagtcccaccttcagaaccgaaacataagaaccggtgtagtcgattcatgtcagtgacttgccatacatatccatcctgagaattggctatctgcttctcattcagtggctgcatttggtttacagattcctccatttttttttgtctttaggaaacctgtacctggcagccgaccccctggatccgcagcgccgccaggagaagtcctgcgcagcgctgggaaacgacaaaagaaggcagcctgacgggcagcgacagccacagcaacagcaacagccccactgccgccggggattccaggttcggttcccgggaacgagtcctgcccctcttcttttgccccgcctccgccccagaggggcgaggatcccggatgttgcctcctcggcgctgtgaatcaccgccctttcttctcaggccccagcccttccgaatccgctacgggtgct

SEQ ID NO: 12335 - RNA, 5606 nt, Homo sapiens
  source 1..5606: mol_type = other RNA
ctgggaggtcaaggctgcagtgagctgtgatcatgccactccagcctgggtgacagagggatagcctgtctcaaaaaaaaaagtttgttaacagcatttcctcagagtataagcttgtttttctaggtctgtccaagaagatcttggagtatattttttctccctcttcagtagagaatagtgactttttgggtaatactttagctgtgaaaatttttcttctaaatttttctactctgaacaggaatgttttaaaacactgttaggcctattgagtgagctatttttctaaaacattttatcttttgaaatacgtatcttattaacaagaatgtttttaaccaaaaaaaaaaagaattctaacttgtattgcaagccctcttcccagtttcaatttttatacaaatattaaatcactgattcttctatgatccaagcacagatatgttactttttaaggataaaaataatcaaatcacttaggttaaactggttgtctacagtcacacagtaagttagataaagcaaaggaggtgtcaaagggtaacactaaattccattcactagcatcttgcctcactaacactctcataagatagattactaaataatataagtattaataaatggaatttccaagaactttcaactaataaagggtgggattataagattagtttttgttttactaattacaactatatcctggaactatttacatactacctaggaaataaagtttgtttattcttgcaggattgtttttaaaagcagtattttcccaaatattaatttaacagtaatcctaaaagtaactcaggaaataaaaaacttatcacttcagtacattttattcataatgaggtaaagtttttgttttttctctatatatgtagatatatatagcaacacaggttaattgtgcttgaggattcctatgaattacaagattatacatgttcccattctatttttctactcctaaagcaatcgtatatacattatttcctaataactcaataaggtaaaagtcttaaataattttattttatcctctactcttctgagaccatgtattcccatgttgtggggaaataaattctggcacaggaatgaagagaccaagatttctaggttatagtacttcaaaatcacactctgtcttggacctcagctctctaacaaaaatttaaaaaattagcttttaggtttctaaggtttcttccagctcaaatatgccatgatttgaaaagttaccttctgtggtagcttctcctacttatcctttctttcttaaatgttaccctagtccatttaattagacctacctaaatacttcagaaaggtcatatccatccaatcttgtatccttgatggatttaatattaacttatagatatatttgtctaaaagtattatggaaatagtacacaactgaaggtaatgcacttttgtactatattctatttaacatttctattaggaataaaatgatcatgttataatttttaagatcttgggtttacttaaacaattcaataactattacgtaattctattagtttctttaaactttaaattcaatctgaacgtaatattttaatgtgtcaaaagtagctaatatattcagttcaatgcttgacagggttaaaaacgtgaacaacatcagaagcaatgcatgtctggagtgggggtgagggtgctatgagctttgctgaacaaaaatatctcaggtaaatcacacttaaaaactgataccagttgccttgaaggaatgggtacatatcaaaaccagcattaatatgtcaaataaatttgaaaggaatattttcttattcccagagcccaaatttcacataaaacagaagaaaatatgtacagaaatcctcagactactaaagtccccctttcccaaaaaacataaaccctctaacccccaagcacctaaaaggctataatttacattaactacagtttgacttttcacataacagcgagaaggaccttacaaatcctcagtaaatcttcaattaatatttagagaacaacagatacgcaaacaggttttatgtgtaagctaccttagacggccataataaaattatgagcaaagataatggcatttcaacagattgctttaatgttaaacctcacaatgaaggatacttgctcaataaaataatgcactttagtgtaatgaaaagtttaatacatacaaataatactgaaaaaaattcctagtgactggctagctggtaatatgctactcaaaaattgcctttcaaacctaaaggacctagattgctttattatttgtttacactatcaaagaagaatattttgccacaaaatgaataatggacaaagaggccattgacatgtatacttttaaaaatattaactaaaaaaatagttaaaagtaaaaaattttattttaaaagtaaggaaaaagctaaactggttatagttgagattttaattgttatactttgtgaatgagggggagttaagcgcttgaaacattttatattatttacacttaagagtatgaaaaacagtgtgagactacatctggctatgttattataattcagaggaaatcattatcaagtcacaccccttgtagcaataaaatataacaaagcaaaaaaaaaaaagcaaaccaaatagaatccctcagccaacacaaacttagtctattcttaggggttgccatgatgtttctgattaatggtaacatattccacaagtgcaaataaaacatcagaaataaaatatctttttcactgaataagaaagctgttatttgtgtgatcttagtaaaactctgaaaggaatttgtaaaactcattcataatttaatcaaatgccttagtttttttttttacccccttggtataaaagtttacagatgagtttcatatttcatcacagttatatggtctagtgcatttcagagtatttggacattatcaaagctgtcctttcccaatgaaaacatttaagaaaacgttaagcacttctcaagtaacatgatgtggaattacactttttgctcttacctcttttaggtacacacgtattattcaacaaagcaaaactattttacagtgtctgttaacaaaaagttctctattagatagaggaaactacagtatcctgaagctatttccccaagagctagtttagtagatagacctttgggcccatcttatttttccttcttttttttttttcagtaaggtaactttccattatgcacatactataccatcatcattcattgggtggagattagctgggaagtagctgtatatttttagtgagatcactgatggcaatggatctctggatcgtgctgctgcttatggttaaatcatatctaatgtgaaatttcgaattacatccagagctccagtatcaaagccgcacatatccaacatgcctctatcatctgggtctgcaatggtgaaaccatttgatgtcattccacaaacaatcaatttagctggaatatccattttctttcgatactccctcagagcaatagcaggatggacacctccagcaaaggtctcattatcagtgaatacaatgaagacatcagcaggtgtgtttgtcttctgagcccagatcattggaagagagcaatcagttccacctgctgggatctgactcatagccattaaaacctgttgtaaggtcatatctgtagtcactggacatggtaccatttcatcggaaaaagcaactacataagaatctttttctgttcgtgtgacaaccatgcacattgctgcagcaactgtactagcgttgagtatactacccaaaactctttggttcatagaagcactgacatcaacagctagtaagaaacgttttccagttggttcaactgtcttaaatgttttataaaaagcagcatccaatgctttcaaaatttcttcatcagggcgccacttcagtttccctctgagaccatgacctgtcttgtaagtttctaatgcgatcaaaatatgaaatggatgtatacgagccttttttaatagtttttcattacacagtttttcacatactaaagatacttctgaatttcctggttcaagtactgaattagcagtcatctttcctagattccttagtaatgcagtaagcggcatttcttgtaacaaagccttccatacctctttagactttaagtgatttgttaaaagatgttctctaactaatctatgttcttctattagatgaatgacttctagctcatctcttgtgcgcttcactttctctacagcctccagatactttaataatttttcagtctccacagagagtgctttttctttatacaattcatgaacttctttccagccctttgtaatatatttggtcacaattgcaagtcttggcttaagtccacagaactgaaatgtgaacccacccttctgagtggctgtcttttcaagtttcacttcactggaaggtttaagatgtgacaatcttaatagatctttgtgagaccagccatttctctgtttatattttgtaactgccagagcaagggccatgccacctttctcattgtaccagtccgctatagccttccggagggcacgaccccacatgccacatttcatgctttccttcagatctttcttaaactggataaaagtaaagagatgggtaggaatgcgacaaacttcagaaacagctttaaatgctgcttgttttgtgcttatgtcggagcactgggaacaaatggcaagtgcaaagagcataggctcttgctttgtggttctgccttcttgactaaatgactttatttcttgtatcacttcacatcctctgccatcttcaatcaatctaattaaagcttcagcattttcaaggcccaacttctgttctttgatataataagtcccaccttcagaaccgaaacataagaaccggtgtagtcgattcatgtcagtgacttgccatacatatccatcctgagaattggctatctgcttctcattcagtggctgcatttggtttacagattcctccatttttttttgtctttaggaaacctttctcctctccctcgttattcctctgtgataaattcaccctgtcttcccacaaagatccttcttccaaaacccagatcccgggcgacgcctctccgcgcagaagccgcgggagaaggaggagaaagaggaggagtaaagcaggccctctcgacgtcggcctgtggggagcgatgccgacaagcaggagcggtcccggcttcggaaagggcccaccctgaggaatggtccggccgggcctagcgaggatgtccctaccgcgatgctggttccgttacccagggtggacaggcgcggaagcgggacggggaagagcgatagtttcgcggcgtttgcccagcctcaacccctgtacctggcagccgaccccctggatccgcagcgccgccaggagaagtcctgcgcagcgctgggaaacgacaaaagaaggcagcctgacgggcagcgacagccacagcaacagcaacagccccactgccgccggggattccaggttcggttcccgggaacgagtcctgcccctcttctttt

SEQ ID NO: 12336 - RNA, 4510 nt, Homo sapiens
  source 1..4510: mol_type = other RNA
ctgggaggtcaaggctgcagtgagctgtgatcatgccactccagcctgggtgacagagggatagcctgtctcaaaaaaaaaagtttgttaacagcatttcctcagagtataagcttgtttttctaggtctgtccaagaagatcttggagtatattttttctccctcttcagtagagaatagtgactttttgggtaatactttagctgtgaaaatttttcttctaaatttttctactctgaacaggaatgttttaaaacactgttaggcctattgagtgagctatttttctaaaacattttatcttttgaaatacgtatcttattaacaagaatgtttttaaccaaaaaaaaaaagaattctaacttgtattgcaagccctcttcccagtttcaatttttatacaaatattaaatcactgattcttctatgatccaagcacagatatgttactttttaaggataaaaataatcaaatcacttaggttaaactggttgtctacagtcacacagtaagttagataaagcaaaggaggtgtcaaagggtaacactaaattccattcactagcatcttgcctcactaacactctcataagatagattactaaataatataagtattaataaatggaatttccaagaactttcaactaataaagggtgggattataagattagtttttgttttactaattacaactatatcctggaactatttacatactacctaggaaataaagtttgtttattcttgcaggattgtttttaaaagcagtattttcccaaatattaatttaacagtaatcctaaaagtaactcaggaaataaaaaacttatcacttcagtacattttattcataatgaggtaaagtttttgttttttctctatatatgtagatatatatagcaacacaggttaattgtgcttgaggattcctatgaattacaagattatacatgttcccattctatttttctactcctaaagcaatcgtatatacattatttcctaataactcaataaggtaaaagtcttaaataattttattttatcctctactcttctgagaccatgtattcccatgttgtggggaaataaattctggcacaggaatgaagagaccaagatttctaggttatagtacttcaaaatcacactctgtcttggacctcagctctctaacaaaaatttaaaaaattagcttttaggtttctaaggtttcttccagctcaaatatgccatgatttgaaaagttaccttctgtggtagcttctcctacttatcctttctttcttaaatgttaccctagtccatttaattagacctacctaaatacttcagaaaggtcatatccatccaatcttgtatccttgatggatttaatattaacttatagatatatttgtctaaaagtattatggaaatagtacacaactgaaggtaatgcacttttgtactatattctatttaacatttctattaggaataaaatgatcatgttataatttttaagatcttgggtttacttaaacaattcaataactattacgtaattctattagtttctttaaactttaaattcaatctgaacgtaatattttaatgtgtcaaaagtagctaatatattcagttcaatgcttgacagggttaaaaacgtgaacaacatcagaagcaatgcatgtctggagtgggggtgagggtgctatgagctttgctgaacaaaaatatctcaggtaaatcacacttaaaaactgataccagttgccttgaaggaatgggtacatatcaaaaccagcattaatatgtcaaataaatttgaaaggaatattttcttattcccagagcccaaatttcacataaaacagaagaaaatatgtacagaaatcctcagactactaaagtccccctttcccaaaaaacataaaccctctaacccccaagcacctaaaaggctataatttacattaactacagtttgacttttcacataacagcgagaaggaccttacaaatcctcagtaaatcttcaattaatatttagagaacaacagatacgcaaacaggttttatgtgtaagctaccttagacggccataataaaattatgagcaaagataatggcatttcaacagattgctttaatgttaaacctcacaatgaaggatacttgctcaataaaataatgcactttagtgtaatgaaaagtttaatacatacaaataatactgaaaaaaattcctagtgactggctagctggtaatatgctactcaaaaattgcctttcaaacctaaaggacctagattgctttattatttgtttacactatcaaagaagaatattttgccacaaaatgaataatggacaaagaggccattgacatgtatacttttaaaaatattaactaaaaaaatagttaaaagtaaaaaattttattttaaaagtaaggaaaaagctaaactggttatagttgagattttaattgttatactttgtgaatgagggggagttaagcgcttgaaacattttatattatttacacttaagagtatgaaaaacagtgtgagactacatctggctatgttattataattcagaggaaatcattatcaagtcacaccccttgtagcaataaaatataacaaagcaaaaaaaaaaaagcaaaccaaatagaatccctcagccaacacaaacttagtctattcttaggggttgccatgatgtttctgattaatggtaacatattccacaagtgcaaataaaacatcagaaataaaatatctttttcactgaataagaaagctgttatttgtgtgatcttagtaaaactctgaaaggaatttgtaaaactcattcataatttaatcaaatgccttagtttttttttttacccccttggtataaaagtttacagatgagtttcatatttcatcacagttatatggtctagtgcatttcagagtatttggacattatcaaagctgtcctttcccaatgaaaacatttaagaaaacgttaagcacttctcaagtaacatgatgtggaattacactttttgctcttacctcttttaggtacacacgtattattcaacaaagcaaaactattttacagtgtctgttaacaaaaagttctctattagatagaggaaactacagtatcctgaagctatttccccaagagctagtttagtagatagacctttgggcccatcttatttttccttcttttttttttttcagtaaggtaactttccattatgcacatactataccatcatcattcattgggtggagattagctgggaagtagctgtatatttttagtgagatcactgatggcaatggatctctggatcgtgctgctgcttatggttaaatcatatctaatgtgaaatttcgaattacatccagagctccagtatcaaagccgcacatatccaacatgcctctatcatctgggtctgcaatggtgaaaccatttgatgtcattccacaaacaatcaatttagctggaatatccattttctttcgatactccctcagagcaatagcaggatggacacctccagcaaaggtctcattatcagtgaatacaatgaagacatcagcaggtgtgtttgtcttctgagcccagatcattggaagagagcaatcagttccacctgctgggatctgactcatagccattaaaacctgttgtaaggtcatatctgtagtcactggacatggtaccatttcatcggaaaaagcaactacataagaatctttttctgttcgtgtgacaaccatgcacattgctgcagcaactgtactagcgttgagtatactacccaaaactctttggttcatagaagcactgacatcaacagctagtaagaaacgttttccagttggttcaactgtcttaaatgttttataaaaagcagcatccaatgctttcaaaatttcttcatcagggcgccacttcagtttccctctgagaccatgacctgtcttgtaagtttctaatgcgatcaaaatatgaaatggatgtatacgagccttttttaatagtttttcattacacagtttttcacatactaaagatacttctgaatttcctggttcaagtactgaattagcagtcatctttcctagattccttagtaatgcagtaagcggcatttcttgtaacaaagccttccatacctgtacctggcagccgaccccctggatccgcagcgccgccaggagaagtcctgcgcagcgctgggaaacgacaaaagaaggcagcctgacgggcagcgacagccacagcaacagcaacagccccactgccgccggggattccaggttcggttcccgggaacgagtcctgcccctcttcttttgccccgcctccgccccagaggggcgaggatcccggatgttgcctcctcggcgctgtgaatcaccgccctttcttctcaggccccagcccttccgaatccgctacgggtgctgcaaggcctgggaagagtttcgatgtctct

SEQ ID NO: 12337 - RNA, 1117 nt, Homo sapiens
  source 1..1117: mol_type = other RNA
ctgggaggtcaaggctgcagtgagctgtgatcatgccactgctctctatcttgggtaacagcataagaccctgtctcaaaaaaagaaagaaagaaagaaagagcaagctagctctagggacccaataattgagggataaaggcagagactccctagggactagagaaatgatgagccaggtttccatggtaactgatttcagtgcagcctcttcctagtctcagactgagggagaatcaattttgggggagaccacatctaatggataaaagagccacaggattacaaaagggtggaatagttgttacaagaaggtcacatcatcctggcactgctcccagaaccagtgggcctcgaagcccagcttggcactctcatcctctggtgactcaggtggtccaccttgaagcctctcccctgggggcttccacacagctctcaagctccctagcctggtggctgccacatccacctcagtcctggccctctctccaccagctataacttttgcccagtccatctcggaacgtggagccccaggtgggccctgttcatccagctcgctgggggccactgtgtccaggaagctgccaatagagacactgtccagccggtcggtggtgctggtgtctggcaggctgtcccagctgcctcgccttgagcggcctgggctcccgcctgtcaggctatattgactgctggtgaggctgctgcaatgactggtcaacgtcccccgctcctccaacagccagcgcactgcctcgatgccctcattcaaggtcaccagctgctgcaggatcttcacatcgatggctcgcaggtaagccagctccatcttcagcgccatgatcttgtcccccaagtcgtggccggtgctagacgcccctgggagcagcagggcgccagaggttcccagctcacactcgcctcgcagcccgcggagcagcccttcaggggtcttcctgcccaccttaccctccacatcccgcaggtcaggcgtctgggactccacggtcccctccatgcgggcccaagcctgaaaagggctgggcgaccggacgccggggaccggctcccgggggtcctcccttcgccgctgctaaagcggagcaaaacc

SEQ ID NO: 12338 - RNA, 202 nt, Homo sapiens
  source 1..202: mol_type = other RNA
ctgggaggtcaaggctgcagtgagctgtgatcatgcctggacaacagagtgagaccgtcacttccgctctttctcggccgccattttggctagggcaggttcggggactcggtccgaggcgcttgtattgtcgctcgacgacgccgccgccgcccgccgctctgctgcgcccgccgcgccccccggcagcacccgcggccgc

SEQ ID NO: 12339 - RNA, 297 nt, Homo sapiens
  source 1..297: mol_type = other RNA
ctgggaggtcaaggctgcagtgagctgtgatcatttcactacactccagcatgggtgacggaatgagaccatctcatcccacagtgaagagaacatccagggtgaatggtgaaaaggaatcacagttgagcaccacaggaaggctttttttcctcctcggtaatcctggtttcctcgcgctcgcggagagggccgtcgcggccgtgggaatgccccggccctcgcgcccgtcgctgccgggagagcaccgcgccaggacccggatggaggcgcgggcgggcgccgccgcggcggcct

SEQ ID NO: 12340 - RNA, 161 nt, Homo sapiens
  source 1..161: mol_type = other RNA
ctgggaggtcaaggctgcagtgagctgtgatcgtgccactgtacgccagcctgggtgacagagcaagaccctgtctcaaaaaaaaaaaaaaaaaagttaaaataatcagctaactttaacctgaagaggagagaaatcttggagaagatgtgggtatcttc

SEQ ID NO: 12341 - RNA, 3038 nt, Homo sapiens
  source 1..3038: mol_type = other RNA
ctgggaggtcaaggctgcagtgagctgtgatggtgctgctgcactccagcctgggtgtcagagtgagaccttgtctccaaaaaataaaaataaaaataagtaaaaagaaaaataggctctatttatctaaaggctctgaagacttcagttattgcttacgattaggaaggctttggagagaaaataacttgtgattttaatactgcaggtaaattctctaacacattcagattaaaaagtcaaatgttaattccctatgctacagcacagtcataatatgtaataccttaaccatattttgacaagataagagattgatgccactaaccttgaaagatctaagacattctcttaagtgaaaaataaaatatgtaaataatgtttatatttatataaagaaaatcaagctatatatttctagattttcaaatacatttgtataggaatacctcaaaaaaggcctagatagctcatacctgataacagtgatctacctttgaggaggggagtgagactgtatgagggcaaacagggacttttgctttattggcattgcctgaaattttttcatagtaggaatgtgaaaaaatagatgagagcatatactaatccactgaattccttaagccttacttgaatattgaagatggtccttgcaggaagggagcactgtggctttcagtagcacaacgtttaggcattctctctcttttttttcttttttttttgagacggagttttgctcttgttgcccaggctggagtgcaatggtgcaaacttggctcaccgcaacctccgccccaggttcaagtgattctcctgcctcagcctcccaagtagctaggattacaggcatgcgccaccatgcctggctaattttgtatttttagcagagatggggtttctccttgttggtctggctggtctcaaactcccgacctcaggggatctgccagcctcagcctcccaaagtgctgggattacaggtgtgagccaccacgcctggctaggcattcactcttacagtaggtgaaatagttttcctatagagaagaaaagctatatggctgacagcactgatattgaacattaaatatcatacttactaaaaaaaactaacccgcaaaattagaagggctaaggaaaaatatatttgctggttacatataatggtaatagaaagctagtaattaaatataattctcattagaattacaatatagcctttgaatattctattaaataaatgaattcaatttaagtttcattctcaaattaattttatcacatttgattggcccagtccattacacaaaaagacatactgactaaatacaacataatttctataacctgaggggactcgcacatcattacctgattgcttgctgacttggctgttgattggtttcatgactttgaagcttccctcctatgacaattcttcctcccctaaggacttcctcattgctgtttcttcatcttgccctaagagttctctctcttccataaacttcctttcctgggatgaccttctgtcatatgttgttctttgtaggtagcctccatctaaaagcagctcccgtgtctgtgacatgctctgctccaggaattcagaggcctccagtgactctgtcattgctccaggaccaccaggctcatcctcgggttctggagactgatgtgtgtcttccccatgctcatacatacacagcctcttttcaaccacctcacggatcaacatgtcaagcactgttcttcccaccatgctatattccatggttttttcaacttcattcattagccatggaagaaatcctatctcaatatctctttcaatgggatcataaaagtagccactatccctgaggctgccaaaaacagacgggagaaggtcagccaggtaacgctgtgcaaatgctcgggcggcgattttttgtgatgtctcgttgtgcttgtgcattatttcccactgctgtttcttacgccgttctttttcttctcggtgtcgcctctcttgctcttcaagtcgttgaacttcagcacgttcactattccgtagttcttcatactcacgctgactggcccgcaggttagccagctcttcttcttccattacttccagaagagactgctcaattgtcttccccaccaaaacttctaacactggtttaacttcaagatcaaagtcaaagagcagtggccctgtctggagtgcataagtgttacctcgaattacccttctgtcatacattatgtttccataatgcataggttcttcatctggctgcgtcaggctgtcccggtaacggctgcgctggcagggcagtgctcggggccggctggtgtaggtgtaggtgctcggggcccgagaggtgcgatcagtcagcgctgaggccatgtccgggggctgactgcctcgctttcggtggagcttggctttgaagcaggtgggcgctaaggtgttgtgggacccggagagatgtaagtagtgccaagggcaaggattccgcgacgcgaggagaggcgacaacaagggaggcgggcgggacgggaggttaccagcgcaggaggtgggagctatactgggctcgctcccagcaccacagagaccagctgcgggggccgcatcggttgcccagcaacccagggttctgtctgggggcgggaactccgggcagttccggtccccaggtttcccgggaaggactgcggcacaagggacttccggctcttgactccgcccagccgcgccacccaggtaggtgcgcctgcgctttgcgaggttcctggctagggaggcggccttggctggcttgaccgtcatccttgaggcctgcggggcaacggtggctgtccttggcccggctttggaatgtggctttgcagggctggtgttggcgccattctcgcaggcccacgtgctcctgctcttccagggtgtcctcggctgtttctcctgccgcggcgcagcagcgctcccaggctgcccccgcgataacacgcccctggcagccaggctcccagctctgttacgt

SEQ ID NO: 12342 - RNA, 2771 nt, Homo sapiens
  source 1..2771: mol_type = other RNA
ctgggaggtcaaggctgcagtgagctgtgatggtgctgctgcactccagcctgggtgtcagagtgagaccttgtctccaaaaaataaaaataaaaataagtaaaaagaaaaataggctctatttatctaaaggctctgaagacttcagttattgcttacgattaggaaggctttggagagaaaataacttgtgattttaatactgcaggtaaattctctaacacattcagattaaaaagtcaaatgttaattccctatgctacagcacagtcataatatgtaataccttaaccatattttgacaagataagagattgatgccactaaccttgaaagatctaagacattctcttaagtgaaaaataaaatatgtaaataatgtttatatttatataaagaaaatcaagctatatatttctagattttcaaatacatttgtataggaatacctcaaaaaaggcctagatagctcatacctgataacagtgatctacctttgaggaggggagtgagactgtatgagggcaaacagggacttttgctttattggcattgcctgaaattttttcatagtaggaatgtgaaaaaatagatgagagcatatactaatccactgaattccttaagccttacttgaatattgaagatggtccttgcaggaagggagcactgtggctttcagtagcacaacgtttaggcattctctctcttttttttcttttttttttgagacggagttttgctcttgttgcccaggctggagtgcaatggtgcaaacttggctcaccgcaacctccgccccaggttcaagtgattctcctgcctcagcctcccaagtagctaggattacaggcatgcgccaccatgcctggctaattttgtatttttagcagagatggggtttctccttgttggtctggctggtctcaaactcccgacctcaggggatctgccagcctcagcctcccaaagtgctgggattacaggtgtgagccaccacgcctggctaggcattcactcttacagtaggtgaaatagttttcctatagagaagaaaagctatatggctgacagcactgatattgaacattaaatatcatacttactaaaaaaaactaacccgcaaaattagaagggctaaggaaaaatatatttgctggttacatataatggtaatagaaagctagtaattaaatataattctcattagaattacaatatagcctttgaatattctattaaataaatgaattcaatttaagtttcattctcaaattaattttatcacatttgattggcccagtccattacacaaaaagacatactgactaaatacaacataatttctataacctgaggggactcgcacatcattacctgattgcttgctgacttggctgttgattggtttcatgactttgaagcttccctcctatgacaattcttcctcccctaaggacttcctcattgctgtttcttcatcttgccctaagagttctctctcttccataaacttcctttcctgggatgaccttctgtcatatgttgttctttgtaggtagcctccatctaaaagcagctcccgtgtctgtgacatgctctgctccaggaattcagaggcctccagtgactctgtcattgctccaggaccaccaggctcatcctcgggttctggagactgatgtgtgtcttccccatgctcatacatacacagcctcttttcaaccacctcacggatcaacatgtcaagcactgttcttcccaccatgctatattccatggttttttcaacttcattcattagccatggaagaaatcctatctcaatatctctttcaatgggatcataaaagtagccactatccctgaggctgccaaaaacagacgggagaaggtcagccaggtaacgctgtgcaaatgctcgggcggcgattttttgtgatgtctcgttgtgcttgtgcattatttcccactgctgtttcttacgccgttctttttcttctcggtgtcgcctctcttgctcttcaagtcgttgaacttcagcacgttcactattccgtagttcttcatactcacgctgactggcccgcaggttagccagctcttcttcttccattacttccagaagagactgctcaattgtcttccccaccaaaacttctaacactggtttaacttcaagatcaaagtcaaagagctctccttctagtatttgggtggccacatctttgccagttttggcaggaataaagagtggtgttggtggtctgtccaaaaatgcatctgtttggcattccatatcaacttctattatgcgatcagcaatttcttcaaggtataattcagtggccctgtctggagtgcataagtgttacctcgaattacccttctgtcatacattatgtttccataatgcataggttcttcatctggctgcgtcaggctgtcccggtaacggctgcgctggcagggcagtgctcggggccggctggtgtaggtgtaggtgctcggggcccgagaggtgcgatcagtcagcgctgaggccatgtccgggggctgactgcctcgctttcggtggagcttggctttgaagcaggtgggcgctaaggtgttgtgggacccggagagatgtaagtagtgccaagggcaaggattccgcgacgcgaggagaggcgacaacaagggaggcgggcgggacgggaggttaccagcgcaggaggtgggagctatactgggctcgctcccagcaccacagagaccagctgcggggg

SEQ ID NO: 12343 - RNA, 3341 nt, Homo sapiens
  source 1..3341: mol_type = other RNA
ctgggaggtcaaggctgcagtgagctgtgatggtgctgctgcactccagcctgggtgtcagagtgagaccttgtctccaaaaaataaaaataaaaataagtaaaaagaaaaataggctctatttatctaaaggctctgaagacttcagttattgcttacgattaggaaggctttggagagaaaataacttgtgattttaatactgcaggtaaattctctaacacattcagattaaaaagtcaaatgttaattccctatgctacagcacagtcataatatgtaataccttaaccatattttgacaagataagagattgatgccactaaccttgaaagatctaagacattctcttaagtgaaaaataaaatatgtaaataatgtttatatttatataaagaaaatcaagctatatatttctagattttcaaatacatttgtataggaatacctcaaaaaaggcctagatagctcatacctgataacagtgatctacctttgaggaggggagtgagactgtatgagggcaaacagggacttttgctttattggcattgcctgaaattttttcatagtaggaatgtgaaaaaatagatgagagcatatactaatccactgaattccttaagccttacttgaatattgaagatggtccttgcaggaagggagcactgtggctttcagtagcacaacgtttaggcattctctctcttttttttcttttttttttgagacggagttttgctcttgttgcccaggctggagtgcaatggtgcaaacttggctcaccgcaacctccgccccaggttcaagtgattctcctgcctcagcctcccaagtagctaggattacaggcatgcgccaccatgcctggctaattttgtatttttagcagagatggggtttctccttgttggtctggctggtctcaaactcccgacctcaggggatctgccagcctcagcctcccaaagtgctgggattacaggtgtgagccaccacgcctggctaggcattcactcttacagtaggtgaaatagttttcctatagagaagaaaagctatatggctgacagcactgatattgaacattaaatatcatacttactaaaaaaaactaacccgcaaaattagaagggctaaggaaaaatatatttgctggttacatataatggtaatagaaagctagtaattaaatataattctcattagaattacaatatagcctttgaatattctattaaataaatgaattcaatttaagtttcattctcaaattaattttatcacatttgattggcccagtccattacacaaaaagacatactgactaaatacaacataatttctataacctgaggggactcgcacatcattacctgattgcttgctgacttggctgttgattggtttcatgactttgaagcttccctcctatgacaattcttcctcccctaaggacttcctcattgctgtttcttcatcttgccctaagagttctctctcttccataaacttcctttcctgggatgaccttctgtcatatgttgttctttgtaggtagcctccatctaaaagcagctcccgtgtctgtgacatgctctgctccaggaattcagaggcctccagtgactctgtcattgctccaggaccaccaggctcatcctcgggttctggagactgatgtgtgtcttccccatgctcatacatacacagcctcttttcaaccacctcacggatcaacatgtcaagcactgttcttcccaccatgctatattccatggttttttcaacttcattcattagccatggaagaaatcctatctcaatatctctttcaatgggatcataaaagtagccactatccctgaggctgccaaaaacagacgggagaaggtcagccaggtaacgctgtgcaaatgctcgggcggcgattttttgtgatgtctcgttgtgcttgtgcattatttcccactgctgtttcttacgccgttctttttcttctcggtgtcgcctctcttgctcttcaagtcgttgaacttcagcacgttcactattccgtagttcttcatactcacgctgactggcccgcaggttagccagctcttcttcttccattacttccagaagagactgctcaattgtcttccccaccaaaacttctaacactggtttaacttcaagatcaaagtcaaagagctctccttctagtatttgggtggccacatctttgccagttttggcaggaataaagagtggtgttggtggtctgtccaaaaatgcatctgtttggcattccatatcaacttctattatgcgatcagcaatttcttcaaggtataattctgtttgcacatcgacatgctttctgccttccacaggttcaggtgtttgtggtctgagctgctcttgggcttgttttctggcaagagccctcttcctagcctcccgttgtctctggagctctagagaatcaggccgtccgagcagtggccctgtctggagtgcataagtgttacctcgaattacccttctgtcatacattatgtttccataatgcataggttcttcatctggctgcgtcaggctgtcccggtaacggctgcgctggcagggcagtgctcggggccggctggtgtaggtgtaggtgctcggggcccgagaggtgcgatcagtcagcgctgaggccatgtccgggggctgactgcctcgctttcggtggagcttggctttgaagcaggtgggcgctaaggtgttgtgggacccggagagatgtaagtagtgccaagggcaaggattccgcgacgcgaggagaggcgacaacaagggaggcgggcgggacgggaggttaccagcgcaggaggtgggagctatactgggctcgctcccagcaccacagagaccagctgcgggggccgcatcggttgcccagcaacccagggttctgtctgggggcgggaactccgggcagttccggtccccaggtttcccgggaaggactgcggcacaagggacttccggctcttgactccgcccagccgcgccacccaggtaggtgcgcctgcgctttgcgaggttcctggctagggaggcggccttggctggcttgaccgtcatccttgaggcctgcggggcaacggtggctgtccttggcccggctttggaatgtggctttgcagggctggtgttggcgccattctcgcaggcccacgtgctcctgctcttccagggtgtcctcggctgtttctcctgccgcggcgcagcagcgctcccaggctgcccccgcgataacacgcccctggcagccaggctcccagctctgttacgtgcccgggcggggaag

SEQ ID NO: 12344 - RNA, 2860 nt, Homo sapiens
  source 1..2860: mol_type = other RNA
ctgggaggtcaaggctgcagtgagctgtgatggtgctgctgcactccagcctgggtgtcagagtgagaccttgtctccaaaaaataaaaataaaaataagtaaaaagaaaaataggctctatttatctaaaggctctgaagacttcagttattgcttacgattaggaaggctttggagagaaaataacttgtgattttaatactgcaggtaaattctctaacacattcagattaaaaagtcaaatgttaattccctatgctacagcacagtcataatatgtaataccttaaccatattttgacaagataagagattgatgccactaaccttgaaagatctaagacattctcttaagtgaaaaataaaatatgtaaataatgtttatatttatataaagaaaatcaagctatatatttctagattttcaaatacatttgtataggaatacctcaaaaaaggcctagatagctcatacctgataacagtgatctacctttgaggaggggagtgagactgtatgagggcaaacagggacttttgctttattggcattgcctgaaattttttcatagtaggaatgtgaaaaaatagatgagagcatatactaatccactgaattccttaagccttacttgaatattgaagatggtccttgcaggaagggagcactgtggctttcagtagcacaacgtttaggcattctctctcttttttttcttttttttttgagacggagttttgctcttgttgcccaggctggagtgcaatggtgcaaacttggctcaccgcaacctccgccccaggttcaagtgattctcctgcctcagcctcccaagtagctaggattacaggcatgcgccaccatgcctggctaattttgtatttttagcagagatggggtttctccttgttggtctggctggtctcaaactcccgacctcaggggatctgccagcctcagcctcccaaagtgctgggattacaggtgtgagccaccacgcctggctaggcattcactcttacagtaggtgaaatagttttcctatagagaagaaaagctatatggctgacagcactgatattgaacattaaatatcatacttactaaaaaaaactaacccgcaaaattagaagggctaaggaaaaatatatttgctggttacatataatggtaatagaaagctagtaattaaatataattctcattagaattacaatatagcctttgaatattctattaaataaatgaattcaatttaagtttcattctcaaattaattttatcacatttgattggcccagtccattacacaaaaagacatactgactaaatacaacataatttctataacctgaggggactcgcacatcattacctgattgcttgctgacttggctgttgattggtttcatgactttgaagcttccctcctatgacaattcttcctcccctaaggacttcctcattgctgtttcttcatcttgccctaagagttctctctcttccataaacttcctttcctgggatgaccttctgtcatatgttgttctttgtaggtagcctccatctaaaagcagctcccgtgtctgtgacatgctctgctccaggaattcagaggcctccagtgactctgtcattgctccaggaccaccaggctcatcctcgggttctggagactgatgtgtgtcttccccatgctcatacatacacagcctcttttcaaccacctcacggatcaacatgtcaagcactgttcttcccaccatgctatattccatggttttttcaacttcattcattagccatggaagaaatcctatctcaatatctctttcaatgggatcataaaagtagccactatccctgaggctgccaaaaacagacgggagaaggtcagccaggtaacgctgtgcaaatgctcgggcggcgattttttgtgatgtctcgttgtgcttgtgcattatttcccactgctgtttcttacgccgttctttttcttctcggtgtcgcctctcttgctcttcaagtcgttgaacttcagcacgttcactattccgtagttcttcatactcacgctgactggcccgcaggttagccagctcttcttcttccattacttccagaagagactgctcaattgtcttccccaccaaaacttctaacactggtttaacttcaagatcaaagtcaaagagctctccttctagtatttgggtggccacatctttgccagttttggcaggaataaagagtggtgttggtggtctgtccaaaaatgcatctgtttggcattccatatcaacttctattatgcgatcagcaatttcttcaaggtataattctgtttgcacatcgacatgctttctgccttccacaggttcaggtgtttgtggtctgagctgctcttgggcttgttttctggcaagagccctcttcctagcctcccgttgtctctggagctctagagaatcaggccgtccgagggctgcgtcaggctgtcccggtaacggctgcgctggcagggcagtgctcggggccggctggtgtaggtgtaggtgctcggggcccgagaggtgcgatcagtcagcgctgaggccatgtccgggggctgactgcctcgctttcggtggagcttggctttgaagcaggtgggcgctaaggtgttgtgggacccggagagatgtaagtagtgccaagggcaaggattccgcgacgcgaggagaggcgacaacaagggaggcgggcgggacgggaggttaccagcgcaggaggtgggagctatactgggctcgctcccagcaccacagagaccagctgcgggggccgcatcggttgcccagcaacccagggttctgtct

SEQ ID NO: 12345 - RNA, 2943 nt, Homo sapiens
  source 1..2943: mol_type = other RNA
ctgggaggtcaaggctgcagtgagctgtgatggtgctgctgcactccagcctgggtgtcagagtgagaccttgtctccaaaaaataaaaataaaaataagtaaaaagaaaaataggctctatttatctaaaggctctgaagacttcagttattgcttacgattaggaaggctttggagagaaaataacttgtgattttaatactgcaggtaaattctctaacacattcagattaaaaagtcaaatgttaattccctatgctacagcacagtcataatatgtaataccttaaccatattttgacaagataagagattgatgccactaaccttgaaagatctaagacattctcttaagtgaaaaataaaatatgtaaataatgtttatatttatataaagaaaatcaagctatatatttctagattttcaaatacatttgtataggaatacctcaaaaaaggcctagatagctcatacctgataacagtgatctacctttgaggaggggagtgagactgtatgagggcaaacagggacttttgctttattggcattgcctgaaattttttcatagtaggaatgtgaaaaaatagatgagagcatatactaatccactgaattccttaagccttacttgaatattgaagatggtccttgcaggaagggagcactgtggctttcagtagcacaacgtttaggcattctctctcttttttttcttttttttttgagacggagttttgctcttgttgcccaggctggagtgcaatggtgcaaacttggctcaccgcaacctccgccccaggttcaagtgattctcctgcctcagcctcccaagtagctaggattacaggcatgcgccaccatgcctggctaattttgtatttttagcagagatggggtttctccttgttggtctggctggtctcaaactcccgacctcaggggatctgccagcctcagcctcccaaagtgctgggattacaggtgtgagccaccacgcctggctaggcattcactcttacagtaggtgaaatagttttcctgattgcttgctgacttggctgttgattggtttcatgactttgaagcttccctcctatgacaattcttcctcccctaaggacttcctcattgctgtttcttcatcttgccctaagagttctctctcttccataaacttcctttcctgggatgaccttctgtcatatgttgttctttgtaggtagcctccatctaaaagcagctcccgtgtctgtgacatgctctgctccaggaattcagaggcctccagtgactctgtcattgctccaggaccaccaggctcatcctcgggttctggagactgatgtgtgtcttccccatgctcatacatacacagcctcttttcaaccacctcacggatcaacatgtcaagcactgttcttcccaccatgctatattccatggttttttcaacttcattcattagccatggaagaaatcctatctcaatatctctttcaatgggatcataaaagtagccactatccctgaggctgccaaaaacagacgggagaaggtcagccaggtaacgctgtgcaaatgctcgggcggcgattttttgtgatgtctcgttgtgcttgtgcattatttcccactgctgtttcttacgccgttctttttcttctcggtgtcgcctctcttgctcttcaagtcgttgaacttcagcacgttcactattccgtagttcttcatactcacgctgactggcccgcaggttagccagctcttcttcttccattacttccagaagagactgctcaattgtcttccccaccaaaacttctaacactggtttaacttcaagatcaaagtcaaagagcagtggccctgtctggagtgcataagtgttacctcgaattacccttctgtcatacattatgtttccataatgcataggttcttcatctggctgcgtcaggctgtcccggtaacggctgcgctggcagggcagtgctcggggccggctggtgtaggtgtaggtgctcggggcccgagaggtgcgatcagtcagcgctgaggccatgtccgggggctgactgcctcgctttcggtggagcttggctttgaagcaggtgggcgctaaggtgttgtgggacccggagagatgtaagtagtgccaagggcaaggattccgcgacgcgaggagaggcgacaacaagggaggcgggcgggacgggaggttaccagcgcaggaggtgggagctatactgggctcgctcccagcaccacagagaccagctgcgggggccgcatcggttgcccagcaacccagggttctgtctgggggcgggaactccgggcagttccggtccccaggtttcccgggaaggactgcggcacaagggacttccggctcttgactccgcccagccgcgccacccaggtaggtgcgcctgcgctttgcgaggttcctggctagggaggcggccttggctggcttgaccgtcatccttgaggcctgcggggcaacggtggctgtccttggcccggctttggaatgtggctttgcagggctggtgttggcgccattctcgcaggcccacgtgctcctgctcttccagggtgtcctcggctgtttctcctgccgcggcgcagcagcgctcccaggctgcccccgcgataacacgcccctggcagccaggctcccagctctgttacgtgcccgggcggggaagagcttcctggtgtctcccggctcctgcccttctcccgccccaggggcgggctgccgccgccctctgcagctgagtcagtgcagttcctcacctaccttctctgctcaccgctgtgtgctagcaatcggaggacccttggcacacggagcgacaggggcctcccccacagacacctcattttgggaaagaagtgagcaatttattgagtcttaaaaaatacaaag

SEQ ID NO: 12346 - RNA, 2437 nt, Homo sapiens
  source 1..2437: mol_type = other RNA
ctgggaggtcaaggctgcagtgagctgtgatggtgctgctgcactccagcctgggtgtcagagtgagaccttgtctccaaaaaataaaaataaaaataagtaaaaagaaaaataggctctatttatctaaaggctctgaagacttcagttattgcttacgattaggaaggctttggagagaaaataacttgtgattttaatactgcaggtaaattctctaacacattcagattaaaaagtcaaatgttaattccctatgctacagcacagtcataatatgtaataccttaaccatattttgacaagataagagattgatgccactaaccttgaaagatctaagacattctcttaagtgaaaaataaaatatgtaaataatgtttatatttatataaagaaaatcaagctatatatttctagattttcaaatacatttgtataggaatacctcaaaaaaggcctagatagctcatacctgataacagtgatctacctttgaggaggggagtgagactgtatgagggcaaacagggacttttgctttattggcattgcctgaaattttttcatagtaggaatgtgaaaaaatagatgagagcatatactaatccactgaattccttaagccttacttgaatattgaagatggtccttgcaggaagggagcactgtggctttcagtagcacaacgtttaggcattctctctcttttttttcttttttttttgagacggagttttgctcttgttgcccaggctggagtgcaatggtgcaaacttggctcaccgcaacctccgccccaggttcaagtgattctcctgcctcagcctcccaagtagctaggattacaggcatgcgccaccatgcctggctaattttgtatttttagcagagatggggtttctccttgttggtctggctggtctcaaactcccgacctcaggggatctgccagcctcagcctcccaaagtgctgggattacaggtgtgagccaccacgcctggctaggcattcactcttacagtaggtgaaatagttttcctgattgcttgctgacttggctgttgattggtttcatgactttgaagcttccctcctatgacaattcttcctcccctaaggacttcctcattgctgtttcttcatcttgccctaagagttctctctcttccataaacttcctttcctgggatgaccttctgtcatatgttgttctttgtaggtagcctccatctaaaagcagctcccgtgtctgtgacatgctctgctccaggaattcagaggcctccagtgactctgtcattgctccaggaccaccaggctcatcctcgggttctggagactgatgtgtgtcttccccatgctcatacatacacagcctcttttcaaccacctcacggatcaacatgtcaagcactgttcttcccaccatgctatattccatggttttttcaacttcattcattagccatggaagaaatcctatctcaatatctctttcaatgggatcataaaagtagccactatccctgaggctgccaaaaacagacgggagaaggtcagccaggtaacgctgtgcaaatgctcgggcggcgattttttgtgatgtctcgttgtgcttgtgcattatttcccactgctgtttcttacgccgttctttttcttctcggtgtcgcctctcttgctcttcaagtcgttgaacttcagcacgttcactattccgtagttcttcatactcacgctgactggcccgcaggttagccagctcttcttcttccattacttccagaagagactgctcaattgtcttccccaccaaaacttctaacactggtttaacttcaagatcaaagtcaaagagctctccttctagtatttgggtggccacatctttgccagttttggcaggaataaagagtggtgttggtggtctgtccaaaaatgcatctgtttggcattccatatcaacttctattatgcgatcagcaatttcttcaaggtataattcagtggccctgtctggagtgcataagtgttacctcgaattacccttctgtcatacattatgtttccataatgcataggttcttcatctggctgcgtcaggctgtcccggtaacggctgcgctggcagggcagtgctcggggccggctggtgtaggtgtaggtgctcggggcccgagaggtgcgatcagtcagcgctgaggccatgtccgggggctgactgcctcgctttcggtggagcttggctttgaagcaggtgggcgctaaggtgttgtgggacccggagagatgtaagtagtgccaagggcaaggattccgcgacgcgaggagaggcgacaacaagggaggcgggcgggacgggaggttaccagcgcaggaggtgggagctatactgggctcgctcccagcaccacagagaccagctgcggggg

SEQ ID NO: 12347 - RNA, 2992 nt, Homo sapiens
  source 1..2992: mol_type = other RNA
ctgggaggtcaaggctgcagtgagctgtgatggtgctgctgcactccagcctgggtgtcagagtgagaccttgtctccaaaaaataaaaataaaaataagtaaaaagaaaaataggctctatttatctaaaggctctgaagacttcagttattgcttacgattaggaaggctttggagagaaaataacttgtgattttaatactgcaggtaaattctctaacacattcagattaaaaagtcaaatgttaattccctatgctacagcacagtcataatatgtaataccttaaccatattttgacaagataagagattgatgccactaaccttgaaagatctaagacattctcttaagtgaaaaataaaatatgtaaataatgtttatatttatataaagaaaatcaagctatatatttctagattttcaaatacatttgtataggaatacctcaaaaaaggcctagatagctcatacctgataacagtgatctacctttgaggaggggagtgagactgtatgagggcaaacagggacttttgctttattggcattgcctgaaattttttcatagtaggaatgtgaaaaaatagatgagagcatatactaatccactgaattccttaagccttacttgaatattgaagatggtccttgcaggaagggagcactgtggctttcagtagcacaacgtttaggcattctctctcttttttttcttttttttttgagacggagttttgctcttgttgcccaggctggagtgcaatggtgcaaacttggctcaccgcaacctccgccccaggttcaagtgattctcctgcctcagcctcccaagtagctaggattacaggcatgcgccaccatgcctggctaattttgtatttttagcagagatggggtttctccttgttggtctggctggtctcaaactcccgacctcaggggatctgccagcctcagcctcccaaagtgctgggattacaggtgtgagccaccacgcctggctaggcattcactcttacagtaggtgaaatagttttcctgattgcttgctgacttggctgttgattggtttcatgactttgaagcttccctcctatgacaattcttcctcccctaaggacttcctcattgctgtttcttcatcttgccctaagagttctctctcttccataaacttcctttcctgggatgaccttctgtcatatgttgttctttgtaggtagcctccatctaaaagcagctcccgtgtctgtgacatgctctgctccaggaattcagaggcctccagtgactctgtcattgctccaggaccaccaggctcatcctcgggttctggagactgatgtgtgtcttccccatgctcatacatacacagcctcttttcaaccacctcacggatcaacatgtcaagcactgttcttcccaccatgctatattccatggttttttcaacttcattcattagccatggaagaaatcctatctcaatatctctttcaatgggatcataaaagtagccactatccctgaggctgccaaaaacagacgggagaaggtcagccaggtaacgctgtgcaaatgctcgggcggcgattttttgtgatgtctcgttgtgcttgtgcattatttcccactgctgtttcttacgccgttctttttcttctcggtgtcgcctctcttgctcttcaagtcgttgaacttcagcacgttcactattccgtagttcttcatactcacgctgactggcccgcaggttagccagctcttcttcttccattacttccagaagagactgctcaattgtcttccccaccaaaacttctaacactggtttaacttcaagatcaaagtcaaagagctctccttctagtatttgggtggccacatctttgccagttttggcaggaataaagagtggtgttggtggtctgtccaaaaatgcatctgtttggcattccatatcaacttctattatgcgatcagcaatttcttcaaggtataattctgtttgcacatcgacatgctttctgccttccacaggttcaggtgtttgtggtctgagctgctcttgggcttgttttctggcaagagccctcttcctagcctcccgttgtctctggagctctagagaatcaggccgtccgagcagtggccctgtctggagtgcataagtgttacctcgaattacccttctgtcatacattatgtttccataatgcataggttcttcatctggctgcgtcaggctgtcccggtaacggctgcgctggcagggcagtgctcggggccggctggtgtaggtgtaggtgctcggggcccgagaggtgcgatcagtcagcgctgaggccatgtccgggggctgactgcctcgctttcggtggagcttggctttgaagcaggtgggcgctaaggtgttgtgggacccggagagatgtaagtagtgccaagggcaaggattccgcgacgcgaggagaggcgacaacaagggaggcgggcgggacgggaggttaccagcgcaggaggtgggagctatactgggctcgctcccagcaccacagagaccagctgcgggggccgcatcggttgcccagcaacccagggttctgtctgggggcgggaactccgggcagttccggtccccaggtttcccgggaaggactgcggcacaagggacttccggctcttgactccgcccagccgcgccacccaggtaggtgcgcctgcgctttgcgaggttcctggctagggaggcggccttggctggcttgaccgtcatccttgaggcctgcggggcaacggtggctgtccttggcccggctttggaatgtggctttgcagggctggtgttggcgccattctcgcaggcccacgtgctcctgctcttccagggtgtcctcggctgtttctcctgccgcggcgcagcagcgctcccaggctgcccccgcgataacacgcccctggcagccaggctcccagctctgttacgt

SEQ ID NO: 12348 - RNA, 3666 nt, Homo sapiens
  source 1..3666: mol_type = other RNA
ctgggaggtcaaggctgcagtgagctgtgattatgccactacactccagcatgggggacatctttcttctaagactacacacacatgaaatgtgatccttctgtgagctgcggctgagtggatggaactggcgatgccgaggactcaggagatggggacagacttttcactgccattgtttgatttcctctagaaacctcaggagttgattcgtaagaaataacagtttcttcctgttcgtcaacactgttctttgtattttcttcaggatgctcttctggtttatgatttgcggtctgtgtttcatcttgagggctgaatgtaacatcctcaggcattttgtctttgtttctttctttatccatcatttccacagaatttactccatttggctcaggttcaaaaagcatttcatatgaaatgttttcagttttttttaactctttgctgaagtccacattttggggttcggtttcttttagttgaacaatttctgttgcaggagtttcatggtctggctttacatcattttctctaatggcagtgtccagttccttatcatccctccttcgagtctgagtagtcctaaatggattatcccttaaatttgaagggctttgtaagggtgactggtctgaagcaccgataacatttaacccttttttcttctccctcaggcacgcttgttgatgtcttcttattctttccatttgctcttccacagtcatccttggtcgagtactttcagccaaacagagctgttccactgcacttcttggtctttccgttcttagatccatcatcttcttagttttcctcaaggttacataggaagctattgtcgaagattcgggtgttggtgattttgctcttggagggactactccaacaggaaagtgggaacctttaacaactgaagtttctatctctgaaacaggttctgatttttcttctccattagattcatcaacttctgccactgttgttaactctggttcactcttgtagagtctataatctggaccctcatttttgtacttaactgttgagaaaggctttgatcctatcatacctatttctgtagtacctctttgctgcttatgtttactcagcccttccatgacatcctgaattcgccaaagttctttctgaatctgtgcacgctgaattcctgctgattccgtctgaacttcaccaaggtgatccagctgctcttgcatctggttcctggtaacagttacatcgtattctaacttatcatattctctccatgctcgttccaattcggcagtggctcgagaaagttctcgacacgtactaagcagtccattttgtaaatcatccctttgtaacaccactgtctgaatggctgctgggttatctgcatgcatttctatctcttggctggctgatagcaaagcttgctcaagcgtgtatttctccttgtggagttgctgaagtttctcttccagagcatgcaccactttatcttgttcacataatcggcttaacttggcatcaatatctacttcttcaggtctgtatttgtataatgtgcctctaccttcatcttgtgacagctgatgatccaaatatatggtgttcctttggagatgatgtgaaagaatttcattctttgggctgtgggcctcaagctttagctgcatgagctgtgctaacgtatgctcccggatactactcagttcggcttgctgccgtctcagctttattagcagcagcgtaagctcctctggcgttttcccttggaggctctggggactaacagactgtaaagtcaggccagctggcactgaccttctgtcaggcacatagacatgcttagggtgatgggccctgtgtctgcggtctattgtcacatctcctctctgaattggtgaagacacttccgatctgtaagttcgttgaggggagtatccctgataagcagctattgacccgtgggaaggtgatgtgggaatagagtgcattgtctggtcagaaatatttaccatggttttgggactactcaaagtactgtgtcgagggagggtgctctgtttgttataaaactgacgctgctgccattcgtagagctgccacattgtgtcatctctcatggacctccgtttctcctccgctccgggtcctaatgtcttgtcatgagtggaaggggttacactgcagatactttcaggccttgtcttgctgtttcttgggagtgttctataaccttcagggtagcgggccataatctgggctctgtgacttggcatatttcttggtaatgtttggtaagaaattactcccctggtttcttcttcatgacccctccccttctggattttaatccactgttccaactgctgcattgaatttgttctctgtatgactcgatcggcctctgtgtataagggccctgtattggggcgatttccacctctaagatctgccaggctaacattgactattttgttctctgaactgctcaagttgattggtctgtagtgcacagtctgagcagggcatgctgacccactctcatattcagatggcagagaattcagctttacactattaatttttgttaagggtctatcttgaccatccttctgaaatccatatttttcagcttctaatgcctttttttcttcaattttgctcatttccttgtttttttgattgttttggatctctggtttaattagcactctatggttgggaatgttattggtttctttagttggtgcattttcagatgtaatcttgtccactcttttcacaggttctgtctgtactagggcagcatctaacatggctttcatccacaactccatttcctttcctgtatcagtgcagaaataataggtccgcatgtttggatgggctgccttaaaagcatatttgcgattaatgtgatcttcagaggtaagcaaagctatctgaaaactaggtaacagtatgcttcccaggataccctcttctttctcatctctataataaaagaggcaaaggtcagaaagcacaaaccagcgtttcttccacaatttcatgccagtactgtcctgtttataaagccaacctcgtctgacaaccggtgcattaggattccttttaattgaatttgacctctttccaaaattatgaactttttttgaagctcgtgaagttctgcctacagggctcattggatgcactgcataatctgaagtcacgttatagttagaagcttcatttatcatacttattggccgttccttcttttcttcagatgtcatggttgcaacagtctgttcattcactacaaaaatacaattgtcctgtgatggttgtcctgtgactggatgtttgcaggtcactttcctttcattatggtttatatagtatcttgcaccttcaaaagtatatgcttcttcccagccagtaggcaaatctgtgctctgccgccggtgtccggtgaccaccgcctcgccggtgacggggtgcagccaggtggtgctcttggcctcctcgttgatgaagaagactcggccgcccctggtgatcccgtaagtccaggaccggggcagggagatccactccaggttcagatccgccgccatgtctgatccctagccgccgccgccgccttctcctgctgccgccgcggctgccgagggaggagggaac

SEQ ID NO: 12349 - RNA, 1498 nt, Homo sapiens
  source 1..1498: mol_type = other RNA
ctgggaggtcaaggctgcagtgagctgtgattgagcctgggtgacagagcaagaccctgcctcaaaaaaaagaaaaaagaagccagctaattctcctcttactcatagtttgaaagagaactttaattcagaaagtttactctgtcattaatttccatggtattgtttttatacagaagcttttgaatattatcaaggccttaacatttctttatcatataagcaatcatcttctataacaactaagcaacttttgaaacaatttttttggtataagagaatttaatgcaaaagaactggaatgagtttttcttggagaaataaaaaaaaaaaagaaaaagaaaaaaatatggaatgggatcccccattagctgaaagcatattttatagaaattattttctctatattaataaaaatataaaaaataatcttaatcattcatattttcaaaatatagtacagttgagattctgtgtaattttattttaaatcctgttacataagacttttagaattcctgattactccttgggtaaaaatatgaaaagcgtaagcaacaatctacaaaaactgggcatatacatagagattttgtagtcaaaacatttttttaaaatttataatatgacacaatttcaaacacaccacaaataacaacatccatgttcccactacccagattttaagaatgttaacatattgtcacatttgcttcagaatttttttttaagaaataaaacattatagagacagttttagtcccaccaccggttagcacaataccacagaacagggccaccaaagaggctgtctcctctggcggtcaggaaggttgagaatcagaaagccaacaccgctgtgaccactgcaatggttggatcggttctgtgccagatagatctccactggtgaacaatagatgcccatgccctgccctcgacgcttgtgaagctggtaataggacactgggaggccttctggggaaaactcagcacctcatcactgtgcttaccgacagaaaccacagaagcggcagacgcatgctctccatttccttctctcctccaaatctcacacgaggtcatctgattgttcatctcagcagaatgctcgtgggaatactctagatttccttaagcacatactccaaaaacaaataaccccagtgccttttccctcttctaaatgatgctcttgagtggacttgtccctgggtaaattgattggatgtccatgtggtattgggcagggacccagcatctcaccataagttagcagcagccatcaagaatgaggtcatttccttgtgaaaaaccgtctcagcggctgcccccgcctcctctgctggatgtgaaatggcggtcggcgaggcaagtgtgagcatcgcagctcctgccaatcctgcatagccgccaaaacggccccgaacactggcgcccccctcccgcaagcccctcggagcccatccatgagatcggtgctccgccgccccttccg

SEQ ID NO: 12350 - RNA, 260 nt, Homo sapiens
  source 1..260: mol_type = other RNA
ctgggaggtcaaggctgcagtgagctgtgattgcaccactgcactccagcctgggcaaccgagtgggacccattctttttctcatcttcgtagcccagacacagcccgaggcaaagcagggagaggaattctgcggtcatagcgtcccttctgccagaaccaaggccccgccttgggttttacccttcaaaggcggagcgggactgggccggccgcagctctccggctgcccggttcgtccccaggatgtgcagatagag

SEQ ID NO: 12351 - RNA, 4466 nt, Homo sapiens
  source 1..4466: mol_type = other RNA
ctgggaggtcaaggctgcagtgagctgtgattgcaccactgcactctagcctgggcagcagagcaagaccctgtctataaaaaaattaaaaagctaccaagaaggtcctctgacacacacttggcattaaattggtggttatttgccctgtcattttcttctcttcaaggattcagtgactttcagcaagagccacccaattccataatctttattttcctgtttgtcccaaacctctacaagtcaatagatcgctttccacctgtatctcatcccagttccccacaagtgaatgacttagtgactggacaggtaccacatgccaggactattaacagtgatgcgggtcttcactccctcctggcgagtgaccaactccacaatccactctcacagcagcttcctatgaccacttgtggcaccaaatgtcttagatcaggttctctaaagcagagcctgagacagggattcagaaccatgtgattgacagtgtgatttatttgggaaacgcctttgagggagggaatgaaacaggatagagaagggagagagcttagcacggatgaaggctcagaaaaagtctagcttggcctgatccaagggtgccagagcagtcatagcaccctggagttttctccgctttaatcaaatgaaccaggtgttggggtgtagagaggaagtgactcctgggtgaggtgagatggctctcatctcctgagggcaattctccagtttctggagaacaagagctgtgagcacttgcagcccaaactcagagcagctggggatgggggtctcagcttggtagaggggactggacagggcaccacagtgtacaacacatatggtcaacaaatatttattgggcatttattgtaagccaggcaagtcagcagaaacggcctgagcagtgcccaagagcactcactcactctccctagcaaacaggctcagaactctctcacacatgtcatcctctttcccactcaaaactcccaccccaaccttcctggaaggcagggctaacaggacctcctgcctgcctgctcacgactgattactttcaatcccagctgcaatgcaaactgaaactcattctgtatatcaccactctacaggagaggtctatttctggggcacccagaagtcagcacacatactgctgggaccaggactcgtaattcgccttggtccaactccttctatgggtttagctgccctcattcctgtgggtaatacaagatcaaacagtccacaactttgcctgtcttctctgctcccctaaggtccctctcccttcgccgtaagatgtgactgaccagtacagtttctcctgaattgacaaactgaactactccttctaccggctaaaccctgacatcagtagaatcaaaccaaaaacaaggtagagtgtttcacagagaagtggtggattgaataaggcagcagaaacacataccatccagcccctgaacctgaattttgccaaaacagagatactttaagtccatttcttttcaaaggggttaatgctcaaagtgggaatagtgactagggtattctagtggttggaataataatttctagaaaaggttcattgctgaggtaccaaaacagacatcatgctaaggaattcttttactgtgcgcttccctgaatagatacgccgtcaaacaaggcagaagctacaaataaagcttacttctactgaactcatgaagctgttcctagtgtcagttttgagtttcaagtgaagactgaatgtcaactgcaggctttccgaattcctcgaccatgtccatccatggattctcttcttgtctagatttccaagcatgaagatgctaactaaagcatttctcaatggggaacacgaaaagatttctattattgtgggttctccggtgttcctaaaggctgagttataactaaaggatttcaacctatttgtgagtttgatggtaacgctggaaaaatgcttgaagttgttactttgctcattataggagtatggtttccctccaggaaggtttctctaaaattaagagctattctacaacagagacccctctacacttaaggtatttatgggatctgtcctctcatggcttctcaggtgtttaaagaggctacaactccagctgaaattcattccacattctttacattgaaaaggtttctcaccagtatggattctctgatgttgattaagatgtgacttcagagtgaagcctctgccacattcatgacattgatgggattttgtgctggagtagattttttgatgttgtttggtgtgggaacactggccaacattttctctacatatatcacattgatagggcttctctgctgtatgagttctgtaatgctgaatgaggtctgagctataaccaaaggcttttccacagatatcacactgataaggctgctcttgtaactcaatcttcttgtcttcaatcactgtcaagttccaactatatgcttcctcacagatgccatttttttcatttttctgacccatgtggagcacctgatgttcaattaggctaacgtactgaaaaaagatttccccacattcacgacactgatgggatttctctcgggagtggagtcgaagatgtccagccaggtgggaacgcctcccaaagcctttcccacattcgttacacttgaagggtctctccccactgtgcacgctctgatgctgaacaaggtgggacctcactctgaaggctttcccacataagggacaggtgtagggcttctcacctgtgtggacgcgctgatgctgagttaggtgcacgcgttggttgtagcttttcccacattcctcacacctgaatggtttctccccagtgtgtattctttgatgttgaataagatgtgcactctgaatgaagcttttcccacactcgttacatttatgtggtctctctccagtggaggattttttgtggacatatgggacttcactgtagttcatcctctttgaagatggttgtcctagtatctctttcatgggaattccctgctttctatccagcttgccttgaaactcacagccttctccaaaatcttgaacttgagaaacatttctttgggtttttccagatagttccatgtctgcttctgaatattctgaaattttcttcttaacacttaattttgtgttcttacttcttttgtcactgcatctctgggatttctccctgaagtggcgttttaggtgttcgatcagatgcgaatggcgaccgaagttcttcccacactcattgcagccatagggcctctctccgctgtggacactgtggtgctgaaccaggtgggaactcacccggaaagcctttccgcacacctgacatttgtagggtttctcccctgtgtggacgcgctggtgctgggtgaggtgcacccgctgattgtagctcttcccacattctccgcacttaaacggtttttctccagtgtggatgcgccgatgctgaataaagtttgaggcttggaggaagaatttgccacaatcgctgcatctgtgccctctctcgccatgtgtgctttgcttagggctgatgtctgtgattgcatccagatcccttttctgggaaggattctgccttgatttccccacagtggggttgacctgccacctttgtaccatgcctttaaggtcactgacttctgcaaagtctggatcctgaggaacgctcctttcggtgtgttctggcgccacccagtgtgattcagagtcatcagaaatctgcttcactatgagctccatattgtccctggactcataaccattttcctccaggagacgaggcttctgtggcgcttgctcaggctgggtgtccacggtcaggggatgggggctgcaggactcctgcactgctccaggtgttgccatcttccgaggaagcacatcagggcaggcaacaatctgctgtctgcgttcctcaagttctcgctgtatattttctatcacggccaccgcctcttctccactttcagggtgatgttccctcacccagggctggaactcttcaggcaggatggtcaggaactgctccagcaccagcagctccaggatctgctccttcgtgtgcagctcgggcctcagccactcacagcagagcacccggagttggctgagagcctcccggggtcctgaagcctcatggtactggaagtgcctgaagcgctggtaaaaagtctcaaacgttggcgggttgtactcctgcatccaggtgcagtcttcttcttccaccttcactatgaaaaggtcttcctgctcctgggaagtctcagctggggggtctaagtctataacttctcgggattcggtcattatcattccaactcagagggaagtcttcgaggctggctgtgttacactcttgaccaccgcagtcggctcagaaggccgacatcttcaacgtcacacccgcgagtcgcaggggccagct

SEQ ID NO: 12352 - RNA, 4784 nt, Homo sapiens
  source 1..4784: mol_type = other RNA
ctgggaggtcaaggctgcagtgagctgtgattgcaccactgcactctagcctgggcagcagagcaagaccctgtctataaaaaaattaaaaagctaccaagaaggtcctctgacacacacttggcattaaattggtggttatttgccctgtcattttcttctcttcaaggattcagtgactttcagcaagagccacccaattccataatctttattttcctgtttgtcccaaacctctacaagtcaatagatcgctttccacctgtatctcatcccagttccccacaagtgaatgacttagtgactggacaggtaccacatgccaggactattaacagtgatgcgggtcttcactccctcctggcgagtgaccaactccacaatccactctcacagcagcttcctatgaccacttgtggcaccaaatgtcttagatcaggttctctaaagcagagcctgagacagggattcagaaccatgtgattgacagtgtgatttatttgggaaacgcctttgagggagggaatgaaacaggatagagaagggagagagcttagcacggatgaaggctcagaaaaagtctagcttggcctgatccaagggtgccagagcagtcatagcaccctggagttttctccgctttaatcaaatgaaccaggtgttggggtgtagagaggaagtgactcctgggtgaggtgagatggctctcatctcctgagggcaattctccagtttctggagaacaagagctgtgagcacttgcagcccaaactcagagcagctggggatgggggtctcagcttggtagaggggactggacagggcaccacagtgtacaacacatatggtcaacaaatatttattgggcatttattgtaagccaggcaagtcagcagaaacggcctgagcagtgcccaagagcactcactcactctccctagcaaacaggctcagaactctctcacacatgtcatcctctttcccactcaaaactcccaccccaaccttcctggaaggcagggctaacaggacctcctgcctgcctgctcacgactgattactttcaatcccagctgcaatgcaaactgaaactcattctgtatatcaccactctacaggagaggtctatttctggggcacccagaagtcagcacacatactgctgggaccaggactcgtaattcgccttggtccaactccttctatgggtttagctgccctcattcctgtgggtaatacaagatcaaacagtccacaactttgcctgtcttctctgctcccctaaggtccctctcccttcgccgtaagatgtgactgaccagtacagtttctcctgaattgacaaactgaactactccttctaccggctaaaccctgacatcagtagaatcaaaccaaaaacaaggtagagtgtttcacagagaagtggtggattgaataaggcagcagaaacacataccatccagcccctgaacctgaattttgccaaaacagagatactttaagtccatttcttttcaaaggggttaatgctcaaagtgggaatagtgactagggtattctagtggttggaataataatttctagaaaaggttcattgctgaggtaccaaaacagacatcatgctaaggaattcttttactgtgcgcttccctgaatagatacgccgtcaaacaaggcagaagctacaaataaagcttacttctactgaactcatgaagctgttcctagtgtcagttttgagtttcaagtgaagactgaatgtcaactgcaggctttccgaattcctcgaccatgtccatccatggattctcttcttgtctagatttccaagcatgaagatgctaactaaagcatttctcaatggggaacacgaaaagatttctattattgtgggttctccggtgttcctaaaggctgagttataactaaaggatttcaacctatttgtgagtttgatggtaacgctggaaaaatgcttgaagttgttactttgctcattataggagtatggtttccctccaggaaggtttctctaaaattaagagctattctacaacagagacccctctacacttaaggtatttatgggatctgtcctctcatggcttctcaggtgtttaaagaggctacaactccagctgaaattcattccacattctttacattgaaaaggtttctcaccagtatggattctctgatgttgattaagatgtgacttcagagtgaagcctctgccacattcatgacattgatgggattttgtgctggagtagattttttgatgttgtttggtgtgggaacactggccaacattttctctacatatatcacattgatagggcttctctgctgtatgagttctgtaatgctgaatgaggtctgagctataaccaaaggcttttccacagatatcacactgataaggctgctcttgtaactcaatcttcttgtcttcaatcactgtcaagttccaactatatgcttcctcacagatgccatttttttcatttttctgacccatgtggagcacctgatgttcaattaggctaacgtactgaaaaaagatttccccacattcacgacactgatgggatttctctcgggagtggagtcgaagatgtccagccaggtgggaacgcctcccaaagcctttcccacattcgttacacttgaagggtctctccccactgtgcacgctctgatgctgaacaaggtgggacctcactctgaaggctttcccacataagggacaggtgtagggcttctcacctgtgtggacgcgctgatgctgagttaggtgcacgcgttggttgtagcttttcccacattcctcacacctgaatggtttctccccagtgtgtattctttgatgttgaataagatgtgcactctgaatgaagcttttcccacactcgttacatttatgtggtctctctccagtggaggattttttgtggacatatgggacttcactgtagttcatcctctttgaagatggttgtcctagtatctctttcatgggaattccctgctttctatccagcttgccttgaaactcacagccttctccaaaatcttgaacttgagaaacatttctttgggtttttccagatagttccatgtctgcttctgaatattctgaaattttcttcttaacacttaattttgtgttcttacttcttttgtcactgcatctctgggatttctccctgaagtggcgttttaggtgttcgatcagatgcgaatggcgaccgaagttcttcccacactcattgcagccatagggcctctctccgctgtggacactgtggtgctgaaccaggtgggaactcacccggaaagcctttccgcacacctgacatttgtagggtttctcccctgtgtggacgcgctggtgctgggtgaggtgcacccgctgattgtagctcttcccacattctccgcacttaaacggtttttctccagtgtggatgcgccgatgctgaataaagtttgaggcttggaggaagaatttgccacaatcgctgcatctgtgccctctctcgccatgtgtgctttgcttagggctgatgtctgtgattgcatccagatcccttttctgggaaggattctgccttgatttccccacagtggggttgacctgccacctttgtaccatgcctttaaggtcactgacttctgcaaagtctggatcctgaggaacgctcctttcggtgtgttctggcgccacccagtgtgattcagagtcatcagaaatctgcttcactatgagctccatattgtccctggactcataacccatggaagtaatactcccatagttctccttcctgtcatccctataaagggacttctgggactggtccaaatgcccccattcctccaggatgaaggatacagccacatcagccacctcttcaattttcaccaacttctgggacccagttgagagaagtgaagctgtcagctcctggctgtccttcaggggaagggaaggaacttggagaacaggaagggcattttcctccaggagacgaggcttctgtggcgcttgctcaggctgggtgtccacggtcaggggatgggggctgcaggactcctgcactgctccaggtgttgccatcttccgaggaagcacatcagggcaggcaacaatctgctgtctgcgttcctcaagttctcgctgtatattttctatcacggccaccgcctcttctccactttcagggtgatgttccctcacccagggctggaactcttcaggcaggatggtcaggaactgctccagcaccagcagctccaggatctgctccttcgtgtgcagctcgggcctcagccactcacagcagagcacccggagttggctgagagcctcccggggtcctgaagcctcatggtactggaagtgcctgaagcgctggtaaaaagtctcaaacgttggcgggttgtactcctgcatccaggtgcagtcttcttcttccaccttcactatgaaaaggtcttcctgctcctgggaagtctcagctggggggtctaagtctataacttctcgggattcggtcattatcattccaactcagagggaagtcttcgaggctggctgtgttacactcgcacggggggcggaccaatcggcggggagatgggacgcgggccccgagtcccagcccaccctcagtgactcggacgtctccagggcccccgaagccgctcgcacagcatcaccaaagcggggaggcaaacggagccactctctcccctgctccatcccaaagccattc

SEQ ID NO: 12353 - RNA, 4685 nt, Homo sapiens
  source 1..4685: mol_type = other RNA
ctgggaggtcaaggctgcagtgagctgtgattgcaccactgcactctagcctgggcagcagagcaagaccctgtctataaaaaaattaaaaagctaccaagaaggtcctctgacacacacttggcattaaattggtggttatttgccctgtcattttcttctcttcaaggattcagtgactttcagcaagagccacccaattccataatctttattttcctgtttgtcccaaacctctacaagtcaatagatcgctttccacctgtatctcatcccagttccccacaagtgaatgacttagtgactggacaggtaccacatgccaggactattaacagtgatgcgggtcttcactccctcctggcgagtgaccaactccacaatccactctcacagcagcttcctatgaccacttgtggcaccaaatgtcttagatcaggttctctaaagcagagcctgagacagggattcagaaccatgtgattgacagtgtgatttatttgggaaacgcctttgagggagggaatgaaacaggatagagaagggagagagcttagcacggatgaaggctcagaaaaagtctagcttggcctgatccaagggtgccagagcagtcatagcaccctggagttttctccgctttaatcaaatgaaccaggtgttggggtgtagagaggaagtgactcctgggtgaggtgagatggctctcatctcctgagggcaattctccagtttctggagaacaagagctgtgagcacttgcagcccaaactcagagcagctggggatgggggtctcagcttggtagaggggactggacagggcaccacagtgtacaacacatatggtcaacaaatatttattgggcatttattgtaagccaggcaagtcagcagaaacggcctgagcagtgcccaagagcactcactcactctccctagcaaacaggctcagaactctctcacacatgtcatcctctttcccactcaaaactcccaccccaaccttcctggaaggcagggctaacaggacctcctgcctgcctgctcacgactgattactttcaatcccagctgcaatgcaaactgaaactcattctgtatatcaccactctacaggagaggtctatttctggggcacccagaagtcagcacacatactgctgggaccaggactcgtaattcgccttggtccaactccttctatgggtttagctgccctcattcctgtgggtaatacaagatcaaacagtccacaactttgcctgtcttctctgctcccctaaggtccctctcccttcgccgtaagatgtgactgaccagtacagtttctcctgaattgacaaactgaactactccttctaccggctaaaccctgacatcagtagaatcaaaccaaaaacaaggtagagtgtttcacagagaagtggtggattgaataaggcagcagaaacacataccatccagcccctgaacctgaattttgccaaaacagagatactttaagtccatttcttttcaaaggggttaatgctcaaagtgggaatagtgactagggtattctagtggttggaataataatttctagaaaaggttcattgctgaggtaccaaaacagacatcatgctaaggaattcttttactgtgcgcttccctgaatagatacgccgtcaaacaaggcagaagctacaaataaagcttacttctactgaactcatgaagctgttcctagtgtcagttttgagtttcaagtgaagactgaatgtcaactgcaggctttccgaattcctcgaccatgtccatccatggattctcttcttgtctagatttccaagcatgaagatgctaactaaagcatttctcaatggggaacacgaaaagatttctattattgtgggttctccggtgttcctaaaggctgagttataactaaaggatttcaacctatttgtgagtttgatggtaacgctggaaaaatgcttgaagttgttactttgctcattataggagtatggtttccctccaggaaggtttctctaaaattaagagctattctacaacagagacccctctacacttaaggtatttatgggatctgtcctctcatggcttctcaggtgtttaaagaggctacaactccagctgaaattcattccacattctttacattgaaaaggtttctcaccagtatggattctctgatgttgattaagatgtgacttcagagtgaagcctctgccacattcatgacattgatgggattttgtgctggagtagattttttgatgttgtttggtgtgggaacactggccaacattttctctacatatatcacattgatagggcttctctgctgtatgagttctgtaatgctgaatgaggtctgagctataaccaaaggcttttccacagatatcacactgataaggctgctcttgtaactcaatcttcttgtcttcaatcactgtcaagttccaactatatgcttcctcacagatgccatttttttcatttttctgacccatgtggagcacctgatgttcaattaggctaacgtactgaaaaaagatttccccacattcacgacactgatgggatttctctcgggagtggagtcgaagatgtccagccaggtgggaacgcctcccaaagcctttcccacattcgttacacttgaagggtctctccccactgtgcacgctctgatgctgaacaaggtgggacctcactctgaaggctttcccacataagggacaggtgtagggcttctcacctgtgtggacgcgctgatgctgagttaggtgcacgcgttggttgtagcttttcccacattcctcacacctgaatggtttctccccagtgtgtattctttgatgttgaataagatgtgcactctgaatgaagcttttcccacactcgttacatttatgtggtctctctccagtggaggattttttgtggacatatgggacttcactgtagttcatcctctttgaagatggttgtcctagtatctctttcatgggaattccctgctttctatccagcttgccttgaaactcacagccttctccaaaatcttgaacttgagaaacatttctttgggtttttccagatagttccatgtctgcttctgaatattctgaaattttcttcttaacacttaattttgtgttcttacttcttttgtcactgcatctctgggatttctccctgaagtggcgttttaggtgttcgatcagatgcgaatggcgaccgaagttcttcccacactcattgcagccatagggcctctctccgctgtggacactgtggtgctgaaccaggtgggaactcacccggaaagcctttccgcacacctgacatttgtagggtttctcccctgtgtggacgcgctggtgctgggtgaggtgcacccgctgattgtagctcttcccacattctccgcacttaaacggtttttctccagtgtggatgcgccgatgctgaataaagtttgaggcttggaggaagaatttgccacaatcgctgcatctgtgccctctctcgccatgtgtgctttgcttagggctgatgtctgtgattgcatccagatcccttttctgggaaggattctgccttgatttccccacagtggggttgacctgccacctttgtaccatgcctttaaggtcactgacttctgcaaagtctggatcctgaggaacgctcctttcggtgtgttctggcgccacccagtgtgattcagagtcatcagaaatctgcttcactatgagctccatattgtccctggactcataacccatggaagtaatactcccatagttctccttcctgtcatccctataaagggacttctgggactggtccaaatgcccccattcctccaggatgaaggatacagccacatcagccacctcttcaattttcaccaacttctgggacccagttgagagaagtgaagctgtcagctcctggctgtccttcaggggaagggaaggaacttggagaacaggaagggcattttcctccaggagacgaggcttctgtggcgcttgctcaggctgggtgtccacggtcaggggatgggggctgcaggactcctgcactgctccaggtgttgccatcttccgaggaagcacatcagggcaggcaacaatctgctgtctgcgttcctcaagttctcgctgtatattttctatcacggccaccgcctcttctccactttcagggtgatgttccctcacccagggctggaactcttcaggcaggatggtcaggaactgctccagcaccagcagctccaggatctgctccttcgtgtgcagctcgggcctcagccactcacagcagagcacccggagttggctgagagcctcccggggtcctgaagcctcatggtactggaagtgcctgaagcgctggtaaaaagtctcaaacgttggcgggttgtactcctgcatccaggtgcagtcttcttcttccaccttcactatgaaaaggtcttcctgctcctgggaagtctcagctggggggtctaagtctataacttctcgggattcggtcattatcattccaactcagagggaagtcttcgaggctggctgtgttacactcttgaccaccgcagtcggctcagaaggccgacatcttcaacgtcacacccgcgagtcgcaggggccagct

SEQ ID NO: 12354 - RNA, 4747 nt, Homo sapiens
  source 1..4747: mol_type = other RNA
ctgggaggtcaaggctgcagtgagctgtgattgcaccactgcactctagcctgggcagcagagcaagaccctgtctataaaaaaattaaaaagctaccaagaaggtcctctgacacacacttggcattaaattggtggttatttgccctgtcattttcttctcttcaaggattcagtgactttcagcaagagccacccaattccataatctttattttcctgtttgtcccaaacctctacaagtcaatagatcgctttccacctgtatctcatcccagttccccacaagtgaatgacttagtgactggacaggtaccacatgccaggactattaacagtgatgcgggtcttcactccctcctggcgagtgaccaactccacaatccactctcacagcagcttcctatgaccacttgtggcaccaaatgtcttagatcaggttctctaaagcagagcctgagacagggattcagaaccatgtgattgacagtgtgatttatttgggaaacgcctttgagggagggaatgaaacaggatagagaagggagagagcttagcacggatgaaggctcagaaaaagtctagcttggcctgatccaagggtgccagagcagtcatagcaccctggagttttctccgctttaatcaaatgaaccaggtgttggggtgtagagaggaagtgactcctgggtgaggtgagatggctctcatctcctgagggcaattctccagtttctggagaacaagagctgtgagcacttgcagcccaaactcagagcagctggggatgggggtctcagcttggtagaggggactggacagggcaccacagtgtacaacacatatggtcaacaaatatttattgggcatttattgtaagccaggcaagtcagcagaaacggcctgagcagtgcccaagagcactcactcactctccctagcaaacaggctcagaactctctcacacatgtcatcctctttcccactcaaaactcccaccccaaccttcctggaaggcagggctaacaggacctcctgcctgcctgctcacgactgattactttcaatcccagctgcaatgcaaactgaaactcattctgtatatcaccactctacaggagaggtctatttctggggcacccagaagtcagcacacatactgctgggaccaggactcgtaattcgccttggtccaactccttctatgggtttagctgccctcattcctgtgggtaatacaagatcaaacagtccacaactttgcctgtcttctctgctcccctaaggtccctctcccttcgccgtaagatgtgactgaccagtacagtttctcctgaattgacaaactgaactactccttctaccggctaaaccctgacatcagtagaatcaaaccaaaaacaaggtagagtgtttcacagagaagtggtggattgaataaggcagcagaaacacataccatccagcccctgaacctgaattttgccaaaacagagatactttaagtccatttcttttcaaaggggttaatgctcaaagtgggaatagtgactagggtattctagtggttggaataataatttctagaaaaggttcattgctgaggtaccaaaacagacatcatgctaaggaattcttttactgtgcgcttccctgaatagatacgccgtcaaacaaggcagaagctacaaataaagcttacttctactgaactcatgaagctgttcctagtgtcagttttgagtttcaagtgaagactgaatgtcaactgcaggctttccgaattcctcgaccatgtccatccatggattctcttcttgtctagatttccaagcatgaagatgctaactaaagcatttctcaatggggaacacgaaaagatttctattattgtgggttctccggtgttcctaaaggctgagttataactaaaggatttcaacctatttgtgagtttgatggtaacgctggaaaaatgcttgaagttgttactttgctcattataggagtatggtttccctccaggaaggtttctctaaaattaagagctattctacaacagagacccctctacacttaaggtatttatgggatctgtcctctcatggcttctcaggtgtttaaagaggctacaactccagctgaaattcattccacattctttacattgaaaaggtttctcaccagtatggattctctgatgttgattaagatgtgacttcagagtgaagcctctgccacattcatgacattgatgggattttgtgctggagtagattttttgatgttgtttggtgtgggaacactggccaacattttctctacatatatcacattgatagggcttctctgctgtatgagttctgtaatgctgaatgaggtctgagctataaccaaaggcttttccacagatatcacactgataaggctgctcttgtaactcaatcttcttgtcttcaatcactgtcaagttccaactatatgcttcctcacagatgccatttttttcatttttctgacccatgtggagcacctgatgttcaattaggctaacgtactgaaaaaagatttccccacattcacgacactgatgggatttctctcgggagtggagtcgaagatgtccagccaggtgggaacgcctcccaaagcctttcccacattcgttacacttgaagggtctctccccactgtgcacgctctgatgctgaacaaggtgggacctcactctgaaggctttcccacataagggacaggtgtagggcttctcacctgtgtggacgcgctgatgctgagttaggtgcacgcgttggttgtagcttttcccacattcctcacacctgaatggtttctccccagtgtgtattctttgatgttgaataagatgtgcactctgaatgaagcttttcccacactcgttacatttatgtggtctctctccagtggaggattttttgtggacatatgggacttcactgtagttcatcctctttgaagatggttgtcctagtatctctttcatgggaattccctgctttctatccagcttgccttgaaactcacagccttctccaaaatcttgaacttgagaaacatttctttgggtttttccagatagttccatgtctgcttctgaatattctgaaattttcttcttaacacttaattttgtgttcttacttcttttgtcactgcatctctgggatttctccctgaagtggcgttttaggtgttcgatcagatgcgaatggcgaccgaagttcttcccacactcattgcagccatagggcctctctccgctgtggacactgtggtgctgaaccaggtgggaactcacccggaaagcctttccgcacacctgacatttgtagggtttctcccctgtgtggacgcgctggtgctgggtgaggtgcacccgctgattgtagctcttcccacattctccgcacttaaacggtttttctccagtgtggatgcgccgatgctgaataaagtttgaggcttggaggaagaatttgccacaatcgctgcatctgtgccctctctcgccatgtgtgctttgcttagggctgatgtctgtgattgcatccagatcccttttctgggaaggattctgccttgatttccccacagtggggttgacctgccacctttgtaccatgcctttaaggtcactgacttctgcaaagtctggatcctgaggaacgctcctttcggtgtgttctggcgccacccagtgtgattcagagtcatcagaaatctgcttcactatgagctccatattgtccctggactcataacccatggaagtaatactcccatagttctccttcctgtcatccctataaagggacttctgggactggtccaaatgcccccattcctccaggatgaaggatacagccacatcagccacctcttcaattttcaccaacttctgggacccagttgagagaagtgaagctgtcagctcctggctgtccttcaggggaagggaaggaacttggagaacaggaagggcattttcctccaggagacgaggcttctgtggcgcttgctcaggctgggtgtccacggtcaggggatgggggctgcaggactcctgcactgctccaggtgttgccatcttccgaggaagcacatcagggcaggcaacaatctgctgtctgcgttcctcaagttctcgctgtatattttctatcacggccaccgcctcttctccactttcagggtgatgttccctcacccagggctggaactcttcaggcaggatggtcaggaactgctccagcaccagcagctccaggatctgctccttcgtgtgcagctcgggcctcagccactcacagcagagcacccggagttggctgagagcctcccggggtcctgaagcctcatggtactggaagtgcctgaagcgctggtaaaaagtctcaaacgttggcgggttgtactcctgcatccaggtgcagtcttcttcttccaccttcactatgaaaaggtcttcctgctcctgggaagtctcagctggggggtctaagtctataacttctcgggattcggtcattatcattccaactcagagggaagtcttcgaggctggctgtgttacactgaaacaattgtttttctgctctttaatatcttctgaaggacactttcagtagcatgcaacctcttgaccaccgcagtcggctcagaaggccgacatcttcaacgtcacacccgcgagtcgcaggggccagct

SEQ ID NO: 12355 - RNA, 2545 nt, Homo sapiens
  source 1..2545: mol_type = other RNA
ctgggaggtcaaggctgcagtgagctgtgattgtgccactgcactccagcctgggtgacacagcgagaccctgtctagtctttcctcgtgcgtgtcctctttccaccttcaggaaggcttctggaactttagaaaaaggaaaggtttgttcaataactggccggatctttcccgcatccaccagttctgcaatgtcatctaaacatgggccactggccatgaaaaatgcccagcgataatggactcctttccagaaatgctttaatgcctttgaacctacagtgactcctgtctgcaacatgccatctgctatgcccaatcggtccatgttcaggaggaaaggagtcaccaaagtcacataggtggctcctgaccatttcttgagaaaatctggagcccatgtttcagtggatccgccaacattatcaaggataaaatcaaatggttttaaggatttcaactgctcttccacacttccagatttgtaatcaattacatcgtctgcaccaagcttccttacaagttcactggcatcttgggagcaaactgctgtcacatgagcatcccatgctttcattacctgtatagcaaaagtaccaactccgcctgaagcgcctaagattagaacacgttttcctgtgcaattcttgtcattcaggccaccaactttgtttatagcagaccaggctgtgagagccacatatggcaaagaggcagcttgagtatgagtgagtgatttgggtttgtgagagacctcattcccactgactacaacaaactctgaaagagtgccttgtttccaaggaggaactgcagcccagacctcatctccaggcttgaagtatttcacatcaagcccacattccatcaccacgccagagacatcccgacccagagtcagaggaaattcttctcctttgattttcacgtgtaaaggatcacgcttcatatttaaagctgtagctccataaccacttctcatattaacgtctataggatttacactggcagcgtgaactttgacaatgacttcatttggatagtgtatgataggcatcatcatgttctgagtgaatcgaagcacttcattcttcccatatttatctatcacccaagcaggcatgacagtgctcctaggagaggtagtactaatccttctaactgaaggcttttggacaactttgcttctccagaagcaaaccgcagtgcatgcatttcttctaagtacacaagtcttcagaaattccattgtaaacactggttgaactgcgtgctcaaattcaaatacacttggactggatcaaactctcacccctgaattcagtcaaattctgccaaaccacgggctagtttcaaaattaagcatgcaaaacggagcattcgaaaatgaagctaatctaatggagaaactgaaagaagaatacggaactgttattccgctcttcgcatatgaaatgctcgaattaacgttccagtcagtattctgtccattctcctccctcactttcaccccctccactttaaaaaaaaaagggggggcggggcattaaaaagcaggtgcgcaaaccccctagatccctgccctgtcctgggagccctcggcgggacaagcagacaccgctcgcgatccaacgccagagaatcgaacgcttgccgactgccgccgcgaccctggcccggaatctccttgcctgcccgctctccttagccgccgggatggctttgcggcgccaaccaatcgcctacaaagatcatttcctcgggctgcaattcaaccaatccaagtactcggtgttgaagggctcagtgacaattaaagatggctgcgcccatgtaacatcactagcgaccggtgacctctttttcccccttgcctggctcctgtggtggcaggctgggcacgaggaccatgctgggccggagcctccgagaagtgagtggaattggcccgctgaggcccccgggagggcggaaagtttaacggacttcgttgacaaagagtccctgggccttaccacgcatcttggcccacctcgctgcttcctctagaactgagtgggggataagtacctttcgattcttcgggtgtactcgccgtacccattcaggagttaggaccttagcagggaaatctctgcaccgcggatctgtagggtggtgaagcggcttctcaccattagacatttgctctggtgtaggtcgggatccggatggtctcggagtgggctttgccaaagggggcttgcggggccacttcagtctctcttctgtccccgacacttagctgcagttgtcgctaagaagcccggcgaaactgtagtttgcaaaattcaaatgagtaatttttggcttttttcaaagaattcgttctctaggatttacctaccactaagataccagtgatttcctaacccgtgtctccatgtcctggacgtcgtgtttgaattctagactgtatttgtgaatgctttctgggcagttcttctaaatgtcacataagcaccctcaaattcactttaatcggtgttgaagtaatcattgtaac

SEQ ID NO: 12356 - RNA, 1464 nt, Homo sapiens
  source 1..1464: mol_type = other RNA
ctgggaggtcaaggctgcagtgagctgtgattgtgccactgcactccagcctgggtgacacagcgagaccctgtctctaaaacaaaaaagacaataaagtagtttaagctagtaaaacagaaggtgccacaacaacctgcaaagccagtgtgaaggaacagcttgaaaaaacttcgaatttctactgactacagacaaatccaagtgctgatatttttatatcaattactggccaaaatggtgtgtttattttttaaagcttgtatcatggaatgtataatctaatctggaaaaatgtttgaaagggatggctagaaaaaaatttgggctcacaggcactcaccaaataagaacgtcaacaatcactaaactgcatttttatttaaacaacattaattacagtctttcctcgtgcgtgtcctctttccaccttcaggaaggcttctggaactttagaaaaaggaaaggtttgttcaataactggccggatctttcccgcatccaccagttctgcaatgtcatctaaacatgggccactggccatgaaaaatgcccagcgataatggactcctttccagaaatgctttaatgcctttgaacctacagtgactcctgtctgcaacatgccatctgctatgcccaatcggtccatgttcaggaggaaaggagtcaccaaagtcacataggtggctcctgaccatttcttgagaaaatctggagcccatgtttcagtggatccgccaacattatcaaggataaaatcaaatggttttaaggatttcaactgctcttccacacttccagatttgtaatcaattacatcgtctgcaccaagcttccttacaagttcactggcatcttgggagcaaactgctgtcacatgagcatcccatgctttcattacctgtatagcaaaagtaccaactccgcctgaagcgcctaagattagaacacgttttcctgtgcaattcttgtcattcaggccaccaactttgtttatagcagaccaggctgtgagagccacatatggcaaagaggcagcttgagtatgagtgagtgatttgggtttgtgagagacctcattcccactgactacaacaaactctgaaagagtgccttgtttccaaggaggaactgcagcccagacctcatctccaggcttgaagtatttcacatcaagcccacattccatcaccacgccagagacatcccgacccagagtcagaggaaattcttctcctttgattttcacgtgtaaaggatcacgcttcatatttaaagctgtagctccataaccacctctcaacccccgtcttaaaaaagctctggtatttctgaattcttaatagactctttttaatggcacaactattatctcatttgcctttagattcttcctcatctttcatatccaataaatcactaagccctcttcattctatcttgcagatatggctggaatct

SEQ ID NO: 12357 - RNA, 2050 nt, Homo sapiens
  source 1..2050: mol_type = other RNA
ctgggaggtcaaggctgcagtgagctgtgattgtgccactgcactccagcctgggtgacacagcgagaccctgtctctaaaacaaaaaagacaataaagtagtttaagctagtaaaacagaaggtgccacaacaacctgcaaagccagtgtgaaggaacagcttgaaaaaacttcgaatttctactgactacagacaaatccaagtgctgatatttttatatcaattactggccaaaatggtgtgtttattttttaaagcttgtatcatggaatgtataatctaatctggaaaaatgtttgaaagggatggctagaaaaaaatttgggctcacaggcactcaccaaataagaacgtcaacaatcactaaactgcatttttatttaaacaacattaattacagtctttcctcgtgcgtgtcctctttccaccttcaggaaggcttctggaactttagaaaaaggaaaggtttgttcaataactggccggatctttcccgcatccaccagttctgcaatgtcatctaaacatgggccactggccatgaaaaatgcccagcgataatggactcctttccagaaatgctttaatgcctttgaacctacagtgactcctgtctgcaacatgccatctgctatgcccaatcggtccatgttcaggaggaaaggagtcaccaaagtcacataggtggctcctgaccatttcttgagaaaatctggagcccatgtttcagtggatccgccaacattatcaaggataaaatcaaatggttttaaggatttcaactgctcttccacacttccagatttgtaatcaattacatcgtctgcaccaagcttccttacaagttcactggcatcttgggagcaaactgctgtcacatgagcatcccatgctttcattacctgtatagcaaaagtaccaactccgcctgaagcgcctaagattagaacacgttttcctgtgcaattcttgtcattcaggccaccaactttgtttatagcagaccaggctgtgagagccacatatggcaaagaggcagcttgagtatgagtgagtgatttgggtttgtgagagacctcattcccactgactacaacaaactctgaaagagtgccttgtttccaaggaggaactgcagcccagacctcatctccaggcttgaagtatttcacatcaagcccacattccatcaccacgccagagacatcccgacccagagtcagaggaaattcttctcctttgattttcacgtgtaaaggatcacgcttcatatttaaagctgtagctccataaccacttctcatattaacgtctataggatttacactggcagcgtgaactttgacaatgacttcatttggatagtgtatgataggcatcatcatgttctgagtgaatcgaagcacttcattcttcccatatttatctatcacccaagcaggcatgacagtgctcctaggagaggtagtactaatccttctaactgaaggcttttggacaactttgcttctccagaagcaaaccgcagtgcatgcatttcttctaagtacacaagtcttcagaaattccattgtaaacactggttgaactgcgtgctcaaattcaaatacacttggactggatcaaactctcacccctgaattcagtcaaattctgccaaaccacgggctagtttcaaaattaagcatgcaaaacggagcattcgaaaatgaagctaatctaatggagaaactgaaagaagaatacggaactgttattccgctcttcgcatatgaaatgctcgaattaacgttccagtcagtattctgtccattctcctccctcactttcaccccctccactttaaaaaaaaaagggggggcggggcattaaaaagcaggtgcgcaaaccccctagatccctgccctgtcctgggagccctcggcgggacaagcagacaccgctcgcgatccaacgccagagaatcgaacgcttgccgactgccgccgcgaccctggcccggaatctccttgcctgcccgctctccttagccgccgggatggctttgc

SEQ ID NO: 12358 - RNA, 2058 nt, Homo sapiens
  source 1..2058: mol_type = other RNA
ctgggaggtcaaggctgcagtgagctgtgattgtgccactgcactccagcttgggcgatacagcaagaccctgtctaaaaaaaagaaagaaaagaaaagaaaattgaattgaagccctaactttggtcagaaaggaacagagcatataatattctttggaatatttttaaaagcacacatacaactaaatatttagaaaagagcctgtggtaaaccccactagggatgtccttgattctgggccctgaggtctcctctccatcccacccgcccccaggccctgggctttgcatctgcccatcctctcaacaaggatggcctgggctggctcttgggaggctgtgggagctcggggacccgtctgtcttgtggcagattagaaagatgtcattttgccaacagtgccatttatcatggcagctgcaaaaattagtgatgcttggtgtgtaagtgttgggtgggggtgggagctggcaggtgacagcagccaatgctccccagtgttaccaggtcagggaactgcaggccaacctctgaataggggctttctgatttaacacttagcccaggtgaaggccctctgttggaaagatgaggaagctggcgctcggagcctggaaataacttcggccacgtgataatttttttttgtgacaggatcttgctccgttgcccaggctggagtgcagtggcacaatcttggttcactgcagtagctgggactacaggcacatgccaccaaacctggttaatttttaaatctttttgtagagacgtggtcttgttatgttgcctaggctggtctcgaactcatggcctcaagtgatcctcctgcttgggcctcccaaagtgggattacaggtttgagccaccatgcctagcccacatgacaaattaatggtccatctctaaataaaggtctaggttctgtgtgtgaccaggaccagggctcatctagggtgaagtgctttacttctattaggagtaagtattatttttgcctttatggctcagtctaggacagaccttcagcctggccccagctgccaccagacagaggcaggattgggagctggccctggagctaggactcactcttggggtaggtttatggtcccaagagaaggggagaaggaggatggagggttcagaaggaatattgggggggggtgaagatgttcagatgagaggtggccccgcaatcaaagggatgccgactccagggaagatgaatggggcctcccttgtgcctcggcccccaaagtaacagccgttcttggggcctggcggaggacggctgcatgggcgtgggcacgggcgctggtttgagtgtggggcctgcgggtggtgggggtggggacgcccatggtcccactgtcctttgtttgctttttctcatccggagccttcaatttttcctggaagattggaagcacgtttccctggggaccccgggaggggcgcgagggcacctgcagggggagggcctaaggggtcaggggaagcccccggtgtggagggtacgacgggcgcttcccccagggtggacgcagcaggcagaggcccaggagcagggctccgcaacccgggccgggctgggggcacggcggggagtcggcactgcgtcgtggggctggacttgggcgacctgcgtccgaccgggacgctctgcacctgcagccaggagtcatccacaggaccccgtgggtgtgctgacgatggtcgtcttgatgtcaccgatgatgctgggcgcctccctcagcacgtggtgcatgcgccgcatctcgttgcgcccctgtgcctgctctgccgactcccccatcagcgtgttctgttccccacgcgagtacaagttggccagcagctccgagaagatgaactccttggtgttgttgatcatgaggtggatgatggtcttgggcatgaggtcctgcatgttcttgttgacaatggccatgtacgagtccaccaggttctgaatggtctccacttgccactccagctgtggtccatggagagcatgaagctgtcggagccattcccctcagtcttgctggc

SEQ ID NO: 12359 - RNA, 823 nt, Homo sapiens
  source 1..823: mol_type = other RNA
ctgggaggtcaaggctgcagtgagctttgggcgacagagtgagaccctgtgttcttccatatccacggtgagagcttcccacccactgttaattgaagctaagctggcttccaaccctccttgttcatctgaaaatcagcaacaacatgtcattttaggaaatcagaagggtacttctgagccaccatgtgcccagggctccatattcctagtcctcatcctagatgcctcttgtgaaaggcccagagaccacacagaggcacacttgcattccatcctctcagggctgccatcctggaaaaaatgcctcttgtggagcgagatggccctcaggctgatgaggaagcaaaggaaagcaaagaagcagcccagctttcagaagcagccccagtgcccacagagccccaggtgagaaggctagaaactctggggtaggaagacgggctgagcttcatacccagccctgccccttctgtcccttctgccaggcctcacagctcctggatctgctagatctcctggatggggcttctggggatgtccagcatcctccccatctggacccctccccaggaggtgccctggtacacctgcttgaccttccctgtgtacctccacccccaggtaagcctaagcaaagggaagatgtcttagagaaggtaggtggaaatgtactgctcctcctcctaagccaagggctgaggctcatggaccctgcttcttcctgtgtgtcccccatcccatcgccatctcaggaggtaaaagaatgaagtcaatcatggtcatctgtcttccctttgttccagacttctttccctggcct

SEQ ID NO: 12360 - RNA, 3195 nt, Homo sapiens
  source 1..3195: mol_type = other RNA
ctgggaggtcaaggctgcagtgaggtcaagattgggccacaccacactctcagcaacctgggtgacagagtgagatcctgtctttaaaaaaaaaaaaaaaaaaaggaaagaaaagaacaaaacaaaaaacaaaactgatgtacatgttttaaagcaaaatagaaccccaagtctaaaagtaaaataagccaaggttagttacaatactgattaaaaagagtatatcctgaggcagttgttagtatatcactctctattatatgcacaataacctctgataggtaaaatatctgagcattttgcaaggtaaacctccaaagttataccacagtgtgcctttttctttgctgtttcttctttgcctattcctacagctaccagtaaacacttaggaactgctttgtatgccagggtctccaagactacctccaggttccatgatttgctaggagaattcacaagactcagcatatcatcacacagctatgatttattacagcaaaagcatatgaagcaaaacagcaaagagaaaaggtacagaggcaaagtctgggggaaaccaggtataagcttccagagtcctctaacagtggagtcacacatatctgttgtttcattccaccagcaactgaattgtgacaacatgtgagaaatgttgtttaccagggaaacttgttagagatacagtgcccagggtttttactgggggctggtcacgtaggtaccttctacctaccatgtaccaaaattctagactcccaggaagaaagcaggttttcagcacaaaccacaggttagctaccatgaacgactcttttcagtgagtggagccctcctgttaaggtttaaatatgtcccccaaagttcaagtgttggaaatttaattgacattgtaaaagtgttatgagacctttaaaaagtaattaggtaaggagggctttgccctcattaatgaattagtgctgctatcttgggagtgggctcatgataaaaggctaagtttagacccatatatctttctcatgctcacttgccatgtggtgccttctgccatggcaagaccctcactagatgctggcaccatgttcttggactgcctagcctccacacctgtcaaccaaataaacttctgttcattataaaatacttagtttgtgtaattctgttatgacagcagaacagactaagataccttctgatatctaagttcccagatgcaacagctgaggacaaaccttataatcaggcctttcaaaggataagtcaggctggctgtgttactcttttctgcatacttagtgacattcccacaggaataatcatcatagacattttcagattcaagaagacccttctaattcagaaacaccttttttttttttttttaagacagagtcttgctctgttgcccaggctagagtgcggtggcacgatctgggctcactgcaacctctgcctcctgggttcaagtgattctcctgcctcagcctcctgagtagctgggattacaggcacatgctaccatgcctggctaatttttgtattttttatttttttggagatggagtcttgctccatcacccaggttggagtgcagaggcacgatcttggcttactgcaacctctgcctcctgggttcaagcgattattctgcctcagcctcccaagtagctgggattacaggcgtccaccaccatgcccggttaattttttatatttctaccagagatggggtttcaccatgttgtcaaggctggtctcaaactcctgacctcaggtgatccacccatctgggtcggcctcccaaagtgttgggattacaggtgtgagccactgcgcccggcctaatttttgtatttttagtagagacaggtgtttcgccatgttggccaggctggtctcgaactcctgacctcatgatctgcccacctaggcctcccaaagtgctgggattacaggcgtgagccaccgtgcctggccagaaacacacttcttttttttgagacagggtcttactgtgtcgcccaggctgtagcgcagtggcgtgatcatgactcattgcaaccatgacctcacaggcttaggtgatcctcttacctcagcctcccgaatagctgggactacaggcatgcaccaccatggtcggctaattttttgtttattttgtagatatgggatttcaccatgttacccaggctggtcttgaactcctgggtttaagtgatctgcccgcctcagcctccccaagtgttaggattacaggtgtgagccaccacaccagacgataaacacacatttttaaaaaaagagaatttcccacctgagaaatggttaattcacttatattaataaattgtcatggctattttttagcttctctagttttactgaaaggtagaataaaaatatatgaaaaacaaaggaaaagtcagtttggtcttaatgaacctgagatcttgatactccaatataaagcaggttctttcagtattaccagcagcaaagactattaatacccatgttacagtcaactagaaatagacttcatatgactacacataattaagcaaaaataaagttgatgactacttggcattaatagtttggacatgaactttagaagtaaaaggtaaaggaggcattataatatcatgtttataaagataactttcttcagctaatattttggggatacaagacgaaacttcgttttgttgtttacgccacttgagtatattctctgccagttcttctgtctcagtcaccaatatatccatctttgctaaagcctggttcattttctttagatttgcagctaaatgaggaatatttctaattgtttcaaggtgggtttctaatctctcaatgaaagtcacagccaactccagcaaatgtaccatatatccaaaaagaaaggatgaacaacatctgctgtatctttttctagtttcaggagttcaatttccaggtttttctggtagatttcagcttgaatatttgtgatctgctgtagtctggtgaagttcacaaaacaagaaactgttttcttagacatgtttaacatctcctgattgaccatccccgaagctatgaagtggcctagcactagcccagcgccgttaggcgcggacgccgggtcccacgggttggcagcggccatggctcggacgcaccttccgcgaaggcgccaagagt

SEQ ID NO: 12361 - RNA, 3235 nt, Homo sapiens
  source 1..3235: mol_type = other RNA
ctgggaggtcaaggctgcagtgaggtcaagattgggccacaccacactctcagcaacctgggtgacagagtgagatcctgtctttaaaaaaaaaaaaaaaaaaaggaaagaaaagaacaaaacaaaaaacaaaactgatgtacatgttttaaagcaaaatagaaccccaagtctaaaagtaaaataagccaaggttagttacaatactgattaaaaagagtatatcctgaggcagttgttagtatatcactctctattatatgcacaataacctctgataggtaaaatatctgagcattttgcaaggtaaacctccaaagttataccacagtgtgcctttttctttgctgtttcttctttgcctattcctacagctaccagtaaacacttaggaactgctttgtatgccagggtctccaagactacctccaggttccatgatttgctaggagaattcacaagactcagcatatcatcacacagctatgatttattacagcaaaagcatatgaagcaaaacagcaaagagaaaaggtacagaggcaaagtctgggggaaaccaggtataagcttccagagtcctctaacagtggagtcacacatatctgttgtttcattccaccagcaactgaattgtgacaacatgtgagaaatgttgtttaccagggaaacttgttagagatacagtgcccagggtttttactgggggctggtcacgtaggtaccttctacctaccatgtaccaaaattctagactcccaggaagaaagcaggttttcagcacaaaccacaggttagctaccatgaacgactcttttcagtgagtggagccctcctgttaaggtttaaatatgtcccccaaagttcaagtgttggaaatttaattgacattgtaaaagtgttatgagacctttaaaaagtaattaggtaaggagggctttgccctcattaatgaattagtgctgctatcttgggagtgggctcatgataaaaggctaagtttagacccatatatctttctcatgctcacttgccatgtggtgccttctgccatggcaagaccctcactagatgctggcaccatgttcttggactgcctagcctccacacctgtcaaccaaataaacttctgttcattataaaatacttagtttgtgtaattctgttatgacagcagaacagactaagataccttctgatatctaagttcccagatgcaacagctgaggacaaaccttataatcaggcctttcaaaggataagtcaggctggctgtgttactcttttctgcatacttagtgacattcccacaggaataatcatcatagacattttcagattcaagaagacccttctaattcagaaacaccttttttttttttttttaagacagagtcttgctctgttgcccaggctagagtgcggtggcacgatctgggctcactgcaacctctgcctcctgggttcaagtgattctcctgcctcagcctcctgagtagctgggattacaggcacatgctaccatgcctggctaatttttgtattttttatttttttggagatggagtcttgctccatcacccaggttggagtgcagaggcacgatcttggcttactgcaacctctgcctcctgggttcaagcgattattctgcctcagcctcccaagtagctgggattacaggcgtccaccaccatgcccggttaattttttatatttctaccagagatggggtttcaccatgttgtcaaggctggtctcaaactcctgacctcaggtgatccacccatctgggtcggcctcccaaagtgttgggattacaggtgtgagccactgcgcccggcctaatttttgtatttttagtagagacaggtgtttcgccatgttggccaggctggtctcgaactcctgacctcatgatctgcccacctaggcctcccaaagtgctgggattacaggcgtgagccaccgtgcctggccagaaacacacttcttttttttgagacagggtcttactgtgtcgcccaggctgtagcgcagtggcgtgatcatgactcattgcaaccatgacctcacaggcttaggtgatcctcttacctcagcctcccgaatagctgggactacaggcatgcaccaccatggtcggctaattttttgtttattttgtagatatgggatttcaccatgttacccaggctggtcttgaactcctgggtttaagtgatctgcccgcctcagcctccccaagtgttaggattacaggtgtgagccaccacaccagacgataaacacacatttttaaaaaaagagaatttcccacctgagaaatggttaattcacttatattaataaattgtcatggctattttttagcttctctagttttactgaaaggtagaataaaaatatatgaaaaacaaaggaaaagtcagtttggtcttaatgaacctgagatcttgatactccaatataaagcaggttctttcagtattaccagcagcaaagactattaatacccatgttacagtcaactagaaatagacttcatatgactacacataattaagcaaaaataaagttgatgactacttggcattaatagtttggacatgaactttagaagtaaaaggtaaaggaggcattataatatcatgtttataaagataactttcttcagctaatattttggggatacaagacgaaacttcgttttgttgtttacgccacttgagtatattctctgccagttcttctgtctcagtcaccaatatatccatctttgctaaagcctggttcattttctttagatttgcagctaaatgaggaatatttctaattgtttcaaggtgggtttctaatctctcaatgaaagtcacagccaactccagcaaatgtaccatatatctgtgataaacagcttcaataggtaagttttcctggcacatgggtttcaacagtctttgcctaagggatctcttctctttcagcactgcttccaaatgattattcatgctttgcagagtatgacacttctgagccaaaaagaaaggatgaacaacatctgctgtatctttttctagtttcaggagttcaatttccaggtttttctgattgaccatccccgaagctatgaagtggcctagcactagcccagcgccgttaggcgcggacgccgggtcccacgggttggcagcggccatggctcggacgcaccttccgcgaaggcgccaagagt

SEQ ID NO: 12362 - RNA, 3328 nt, Homo sapiens
  source 1..3328: mol_type = other RNA
ctgggaggtcaaggctgcagtgaggtcaagattgggccacaccacactctcagcaacctgggtgacagagtgagatcctgtctttaaaaaaaaaaaaaaaaaaaggaaagaaaagaacaaaacaaaaaacaaaactgatgtacatgttttaaagcaaaatagaaccccaagtctaaaagtaaaataagccaaggttagttacaatactgattaaaaagagtatatcctgaggcagttgttagtatatcactctctattatatgcacaataacctctgataggtaaaatatctgagcattttgcaaggtaaacctccaaagttataccacagtgtgcctttttctttgctgtttcttctttgcctattcctacagctaccagtaaacacttaggaactgctttgtatgccagggtctccaagactacctccaggttccatgatttgctaggagaattcacaagactcagcatatcatcacacagctatgatttattacagcaaaagcatatgaagcaaaacagcaaagagaaaaggtacagaggcaaagtctgggggaaaccaggtataagcttccagagtcctctaacagtggagtcacacatatctgttgtttcattccaccagcaactgaattgtgacaacatgtgagaaatgttgtttaccagggaaacttgttagagatacagtgcccagggtttttactgggggctggtcacgtaggtaccttctacctaccatgtaccaaaattctagactcccaggaagaaagcaggttttcagcacaaaccacaggttagctaccatgaacgactcttttcagtgagtggagccctcctgttaaggtttaaatatgtcccccaaagttcaagtgttggaaatttaattgacattgtaaaagtgttatgagacctttaaaaagtaattaggtaaggagggctttgccctcattaatgaattagtgctgctatcttgggagtgggctcatgataaaaggctaagtttagacccatatatctttctcatgctcacttgccatgtggtgccttctgccatggcaagaccctcactagatgctggcaccatgttcttggactgcctagcctccacacctgtcaaccaaataaacttctgttcattataaaatacttagtttgtgtaattctgttatgacagcagaacagactaagataccttctgatatctaagttcccagatgcaacagctgaggacaaaccttataatcaggcctttcaaaggataagtcaggctggctgtgttactcttttctgcatacttagtgacattcccacaggaataatcatcatagacattttcagattcaagaagacccttctaattcagaaacaccttttttttttttttttaagacagagtcttgctctgttgcccaggctagagtgcggtggcacgatctgggctcactgcaacctctgcctcctgggttcaagtgattctcctgcctcagcctcctgagtagctgggattacaggcacatgctaccatgcctggctaatttttgtattttttatttttttggagatggagtcttgctccatcacccaggttggagtgcagaggcacgatcttggcttactgcaacctctgcctcctgggttcaagcgattattctgcctcagcctcccaagtagctgggattacaggcgtccaccaccatgcccggttaattttttatatttctaccagagatggggtttcaccatgttgtcaaggctggtctcaaactcctgacctcaggtgatccacccatctgggtcggcctcccaaagtgttgggattacaggtgtgagccactgcgcccggcctaatttttgtatttttagtagagacaggtgtttcgccatgttggccaggctggtctcgaactcctgacctcatgatctgcccacctaggcctcccaaagtgctgggattacaggcgtgagccaccgtgcctggccagaaacacacttcttttttttgagacagggtcttactgtgtcgcccaggctgtagcgcagtggcgtgatcatgactcattgcaaccatgacctcacaggcttaggtgatcctcttacctcagcctcccgaatagctgggactacaggcatgcaccaccatggtcggctaattttttgtttattttgtagatatgggatttcaccatgttacccaggctggtcttgaactcctgggtttaagtgatctgcccgcctcagcctccccaagtgttaggattacaggtgtgagccaccacaccagacgataaacacacatttttaaaaaaagagaatttcccacctgagaaatggttaattcacttatattaataaattgtcatggctattttttagcttctctagttttactgaaaggtagaataaaaatatatgaaaaacaaaggaaaagtcagtttggtcttaatgaacctgagatcttgatactccaatataaagcaggttctttcagtattaccagcagcaaagactattaatacccatgttacagtcaactagaaatagacttcatatgactacacataattaagcaaaaataaagttgatgactacttggcattaatagtttggacatgaactttagaagtaaaaggtaaaggaggcattataatatcatgtttataaagataactttcttcagctaatattttggggatacaagacgaaacttcgttttgttgtttacgccacttgagtatattctctgccagttcttctgtctcagtcaccaatatatccatctttgctaaagcctggttcattttctttagatttgcagctaaatgaggaatatttctaattgtttcaaggtgggtttctaatctctcaatgaaagtcacagccaactccagcaaatgtaccatatatctgtgataaacagcttcaataggtaagttttcctggcacatgggtttcaacagtctttgcctaagggatctcttctctttcagcactgcttccaaatgattattcatgctttgcagagtatgacacttctgagccaaaaagaaaggatgaacaacatctgctgtatctttttctagtttcaggagttcaatttccaggtttttctggtagatttcagcttgaatatttgtgatctgctgtagtctggtgaagttcacaaaacaagaaactgttttcttagacatgtttaacatctcctgattgaccatccccgaagctatgaagtggcctagcactagcccagcgccgttaggcgcggacgccgggtcccacgggttggcagcggccatggctcggacgcaccttccgcgaaggcgccaagagt

SEQ ID NO: 12363 - RNA, 3258 nt, Homo sapiens
  source 1..3258: mol_type = other RNA
ctgggaggtcaaggctgcagtgaggtcaagattgggccacaccacactctcagcaacctgggtgacagagtgagatcctgtctttaaaaaaaaaaaaaaaaaaaggaaagaaaagaacaaaacaaaaaacaaaactgatgtacatgttttaaagcaaaatagaaccccaagtctaaaagtaaaataagccaaggttagttacaatactgattaaaaagagtatatcctgaggcagttgttagtatatcactctctattatatgcacaataacctctgataggtaaaatatctgagcattttgcaaggtaaacctccaaagttataccacagtgtgcctttttctttgctgtttcttctttgcctattcctacagctaccagtaaacacttaggaactgctttgtatgccagggtctccaagactacctccaggttccatgatttgctaggagaattcacaagactcagcatatcatcacacagctatgatttattacagcaaaagcatatgaagcaaaacagcaaagagaaaaggtacagaggcaaagtctgggggaaaccaggtataagcttccagagtcctctaacagtggagtcacacatatctgttgtttcattccaccagcaactgaattgtgacaacatgtgagaaatgttgtttaccagggaaacttgttagagatacagtgcccagggtttttactgggggctggtcacgtaggtaccttctacctaccatgtaccaaaattctagactcccaggaagaaagcaggttttcagcacaaaccacaggttagctaccatgaacgactcttttcagtgagtggagccctcctgttaaggtttaaatatgtcccccaaagttcaagtgttggaaatttaattgacattgtaaaagtgttatgagacctttaaaaagtaattaggtaaggagggctttgccctcattaatgaattagtgctgctatcttgggagtgggctcatgataaaaggctaagtttagacccatatatctttctcatgctcacttgccatgtggtgccttctgccatggcaagaccctcactagatgctggcaccatgttcttggactgcctagcctccacacctgtcaaccaaataaacttctgttcattataaaatacttagtttgtgtaattctgttatgacagcagaacagactaagataccttctgatatctaagttcccagatgcaacagctgaggacaaaccttataatcaggcctttcaaaggataagtcaggctggctgtgttactcttttctgcatacttagtgacattcccacaggaataatcatcatagacattttcagattcaagaagacccttctaattcagaaacaccttttttttttttttttaagacagagtcttgctctgttgcccaggctagagtgcggtggcacgatctgggctcactgcaacctctgcctcctgggttcaagtgattctcctgcctcagcctcctgagtagctgggattacaggcacatgctaccatgcctggctaatttttgtattttttatttttttggagatggagtcttgctccatcacccaggttggagtgcagaggcacgatcttggcttactgcaacctctgcctcctgggttcaagcgattattctgcctcagcctcccaagtagctgggattacaggcgtccaccaccatgcccggttaattttttatatttctaccagagatggggtttcaccatgttgtcaaggctggtctcaaactcctgacctcaggtgatccacccatctgggtcggcctcccaaagtgttgggattacaggtgtgagccactgcgcccggcctaatttttgtatttttagtagagacaggtgtttcgccatgttggccaggctggtctcgaactcctgacctcatgatctgcccacctaggcctcccaaagtgctgggattacaggcgtgagccaccgtgcctggccagaaacacacttcttttttttgagacagggtcttactgtgtcgcccaggctgtagcgcagtggcgtgatcatgactcattgcaaccatgacctcacaggcttaggtgatcctcttacctcagcctcccgaatagctgggactacaggcatgcaccaccatggtcggctaattttttgtttattttgtagatatgggatttcaccatgttacccaggctggtcttgaactcctgggtttaagtgatctgcccgcctcagcctccccaagtgttaggattacaggtgtgagccaccacaccagacgataaacacacatttttaaaaaaagagaatttcccacctgagaaatggttaattcacttatattaataaattgtcatggctattttttagcttctctagttttactgaaaggtagaataaaaatatatgaaaaacaaaggaaaagtcagtttggtcttaatgaacctgagatcttgatactccaatataaagcaggttctttcagtattaccagcagcaaagactattaatacccatgttacagtcaactagaaatagacttcatatgactacacataattaagcaaaaataaagttgatgactacttggcattaatagtttggacatgaactttagaagtaaaaggtaaaggaggcattataatatcatgtttataaagataactttcttcagctaatattttggggatacaagacgaaacttcgttttgttgtttacgccacttgagtatattctctgccagttcttctgtctcagtcaccaatatatccatctttgctaaagcctggttcattttctttagatttgcagctaaatgaggaatatttctaattgtttcaaggtgggtttctaatctctcaatgaaagtcacagccaactccagcaaatgtaccatatatctgtgataaacagcttcaataggtaagttttcctggcacatgggtttcaacagtctttgcctaagggatctcttctctttcagcactgcttccaaatgattattcatgctttgcagagtatgacacttctgagctggtagatttcagcttgaatatttgtgatctgctgtagtctggtgaagttcacaaaacaagaaactgttttcttagacatgtttaacatctcctgattgaccatccccgaagctatgaagtggcctagcactagcccagcgccgttaggcgcggacgccgggtcccacgggttggcagcggccatggctcggacgcaccttccgcgaaggcgccaagagt

SEQ ID NO: 12364 - RNA, 3324 nt, Homo sapiens
  source 1..3324: mol_type = other RNA
ctgggaggtcaaggctgcagtgaggtcaagattgggccacaccacactctcagcaacctgggtgacagagtgagatcctgtctttaaaaaaaaaaaaaaaaaaaggaaagaaaagaacaaaacaaaaaacaaaactgatgtacatgttttaaagcaaaatagaaccccaagtctaaaagtaaaataagccaaggttagttacaatactgattaaaaagagtatatcctgaggcagttgttagtatatcactctctattatatgcacaataacctctgataggtaaaatatctgagcattttgcaaggtaaacctccaaagttataccacagtgtgcctttttctttgctgtttcttctttgcctattcctacagctaccagtaaacacttaggaactgctttgtatgccagggtctccaagactacctccaggttccatgatttgctaggagaattcacaagactcagcatatcatcacacagctatgatttattacagcaaaagcatatgaagcaaaacagcaaagagaaaaggtacagaggcaaagtctgggggaaaccaggtataagcttccagagtcctctaacagtggagtcacacatatctgttgtttcattccaccagcaactgaattgtgacaacatgtgagaaatgttgtttaccagggaaacttgttagagatacagtgcccagggtttttactgggggctggtcacgtaggtaccttctacctaccatgtaccaaaattctagactcccaggaagaaagcaggttttcagcacaaaccacaggttagctaccatgaacgactcttttcagtgagtggagccctcctgttaaggtttaaatatgtcccccaaagttcaagtgttggaaatttaattgacattgtaaaagtgttatgagacctttaaaaagtaattaggtaaggagggctttgccctcattaatgaattagtgctgctatcttgggagtgggctcatgataaaaggctaagtttagacccatatatctttctcatgctcacttgccatgtggtgccttctgccatggcaagaccctcactagatgctggcaccatgttcttggactgcctagcctccacacctgtcaaccaaataaacttctgttcattataaaatacttagtttgtgtaattctgttatgacagcagaacagactaagataccttctgatatctaagttcccagatgcaacagctgaggacaaaccttataatcaggcctttcaaaggataagtcaggctggctgtgttactcttttctgcatacttagtgacattcccacaggaataatcatcatagacattttcagattcaagaagacccttctaattcagaaacaccttttttttttttttttaagacagagtcttgctctgttgcccaggctagagtgcggtggcacgatctgggctcactgcaacctctgcctcctgggttcaagtgattctcctgcctcagcctcctgagtagctgggattacaggcacatgctaccatgcctggctaatttttgtattttttatttttttggagatggagtcttgctccatcacccaggttggagtgcagaggcacgatcttggcttactgcaacctctgcctcctgggttcaagcgattattctgcctcagcctcccaagtagctgggattacaggcgtccaccaccatgcccggttaattttttatatttctaccagagatggggtttcaccatgttgtcaaggctggtctcaaactcctgacctcaggtgatccacccatctgggtcggcctcccaaagtgttgggattacaggtgtgagccactgcgcccggcctaatttttgtatttttagtagagacaggtgtttcgccatgttggccaggctggtctcgaactcctgacctcatgatctgcccacctaggcctcccaaagtgctgggattacaggcgtgagccaccgtgcctggccagaaacacacttcttttttttgagacagggtcttactgtgtcgcccaggctgtagcgcagtggcgtgatcatgactcattgcaaccatgacctcacaggcttaggtgatcctcttacctcagcctcccgaatagctgggactacaggcatgcaccaccatggtcggctaattttttgtttattttgtagatatgggatttcaccatgttacccaggctggtcttgaactcctgggtttaagtgatctgcccgcctcagcctccccaagtgttaggattacaggtgtgagccaccacaccagacgataaacacacatttttaaaaaaagagaatttcccacctgagaaatggttaattcacttatattaataaattgtcatggctattttttagcttctctagttttactgaaaggtagaataaaaatatatgaaaaacaaaggaaaagtcagtttggtcttaatgaacctgagatcttgatactccaatataaagcaggttctttcagtattaccagcagcaaagactattaatacccatgttacagtcaactagaaatagacttcatatgactacacataattaagcaaaaataaagttgatgactacttggcattaatagtttggacatgaactttagaagtaaaaggtaaaggaggcattataatatcatgtttataaagataactttcttcagctaatattttggggatacaagacgaaacttcgttttgttgtttacgccacttgagtatattctctgccagttcttctgtctcagtcaccaatatatccatctttgctaaagcctggttcattttctttagatttgcagctaaatgaggaatatttctaattgtttcaaggtgggtttctaatctctcaatgaaagtcacagccaactccagcaaatgtaccatatatctgtgataaacagcttcaataggtaagttttcctggcacatgggtttcaacagtctttgcctaagggatctcttctctttcagcactgcttccaaatgattattcatgctttgcagagtatgacacttctgagctgtaatcgcagtgttttgggagactgaaacgggagaattgaggccatgagttcgagaccagcctgggcaacatagcaagacttcatctccaaaaagaaaggatgaacaacatctgctgtatctttttctagtttcaggagttcaatttccaggtttttctgattgaccatccccgaagctatgaagtggcctagcactagcccagcgccgttaggcgcggacgccgggtcccacgggttggcagcggccatggctcggacgcaccttccgcgaaggcgccaagagt

SEQ ID NO: 12365 - RNA, 3417 nt, Homo sapiens
  source 1..3417: mol_type = other RNA
ctgggaggtcaaggctgcagtgaggtcaagattgggccacaccacactctcagcaacctgggtgacagagtgagatcctgtctttaaaaaaaaaaaaaaaaaaaggaaagaaaagaacaaaacaaaaaacaaaactgatgtacatgttttaaagcaaaatagaaccccaagtctaaaagtaaaataagccaaggttagttacaatactgattaaaaagagtatatcctgaggcagttgttagtatatcactctctattatatgcacaataacctctgataggtaaaatatctgagcattttgcaaggtaaacctccaaagttataccacagtgtgcctttttctttgctgtttcttctttgcctattcctacagctaccagtaaacacttaggaactgctttgtatgccagggtctccaagactacctccaggttccatgatttgctaggagaattcacaagactcagcatatcatcacacagctatgatttattacagcaaaagcatatgaagcaaaacagcaaagagaaaaggtacagaggcaaagtctgggggaaaccaggtataagcttccagagtcctctaacagtggagtcacacatatctgttgtttcattccaccagcaactgaattgtgacaacatgtgagaaatgttgtttaccagggaaacttgttagagatacagtgcccagggtttttactgggggctggtcacgtaggtaccttctacctaccatgtaccaaaattctagactcccaggaagaaagcaggttttcagcacaaaccacaggttagctaccatgaacgactcttttcagtgagtggagccctcctgttaaggtttaaatatgtcccccaaagttcaagtgttggaaatttaattgacattgtaaaagtgttatgagacctttaaaaagtaattaggtaaggagggctttgccctcattaatgaattagtgctgctatcttgggagtgggctcatgataaaaggctaagtttagacccatatatctttctcatgctcacttgccatgtggtgccttctgccatggcaagaccctcactagatgctggcaccatgttcttggactgcctagcctccacacctgtcaaccaaataaacttctgttcattataaaatacttagtttgtgtaattctgttatgacagcagaacagactaagataccttctgatatctaagttcccagatgcaacagctgaggacaaaccttataatcaggcctttcaaaggataagtcaggctggctgtgttactcttttctgcatacttagtgacattcccacaggaataatcatcatagacattttcagattcaagaagacccttctaattcagaaacaccttttttttttttttttaagacagagtcttgctctgttgcccaggctagagtgcggtggcacgatctgggctcactgcaacctctgcctcctgggttcaagtgattctcctgcctcagcctcctgagtagctgggattacaggcacatgctaccatgcctggctaatttttgtattttttatttttttggagatggagtcttgctccatcacccaggttggagtgcagaggcacgatcttggcttactgcaacctctgcctcctgggttcaagcgattattctgcctcagcctcccaagtagctgggattacaggcgtccaccaccatgcccggttaattttttatatttctaccagagatggggtttcaccatgttgtcaaggctggtctcaaactcctgacctcaggtgatccacccatctgggtcggcctcccaaagtgttgggattacaggtgtgagccactgcgcccggcctaatttttgtatttttagtagagacaggtgtttcgccatgttggccaggctggtctcgaactcctgacctcatgatctgcccacctaggcctcccaaagtgctgggattacaggcgtgagccaccgtgcctggccagaaacacacttcttttttttgagacagggtcttactgtgtcgcccaggctgtagcgcagtggcgtgatcatgactcattgcaaccatgacctcacaggcttaggtgatcctcttacctcagcctcccgaatagctgggactacaggcatgcaccaccatggtcggctaattttttgtttattttgtagatatgggatttcaccatgttacccaggctggtcttgaactcctgggtttaagtgatctgcccgcctcagcctccccaagtgttaggattacaggtgtgagccaccacaccagacgataaacacacatttttaaaaaaagagaatttcccacctgagaaatggttaattcacttatattaataaattgtcatggctattttttagcttctctagttttactgaaaggtagaataaaaatatatgaaaaacaaaggaaaagtcagtttggtcttaatgaacctgagatcttgatactccaatataaagcaggttctttcagtattaccagcagcaaagactattaatacccatgttacagtcaactagaaatagacttcatatgactacacataattaagcaaaaataaagttgatgactacttggcattaatagtttggacatgaactttagaagtaaaaggtaaaggaggcattataatatcatgtttataaagataactttcttcagctaatattttggggatacaagacgaaacttcgttttgttgtttacgccacttgagtatattctctgccagttcttctgtctcagtcaccaatatatccatctttgctaaagcctggttcattttctttagatttgcagctaaatgaggaatatttctaattgtttcaaggtgggtttctaatctctcaatgaaagtcacagccaactccagcaaatgtaccatatatctgtgataaacagcttcaataggtaagttttcctggcacatgggtttcaacagtctttgcctaagggatctcttctctttcagcactgcttccaaatgattattcatgctttgcagagtatgacacttctgagctgtaatcgcagtgttttgggagactgaaacgggagaattgaggccatgagttcgagaccagcctgggcaacatagcaagacttcatctccaaaaagaaaggatgaacaacatctgctgtatctttttctagtttcaggagttcaatttccaggtttttctggtagatttcagcttgaatatttgtgatctgctgtagtctggtgaagttcacaaaacaagaaactgttttcttagacatgtttaacatctcctgattgaccatccccgaagctatgaagtggcctagcactagcccagcgccgttaggcgcggacgccgggtcccacgggttggcagcggccatggctcggacgcaccttccgcgaaggcgccaagagt

SEQ ID NO: 12366 - RNA, 3357 nt, Homo sapiens
  source 1..3357: mol_type = other RNA
ctgggaggtcaaggctgcagtgaggtcaagattgggccacaccacactctcagcaacctgggtgacagagtgagatcctgtctttaaaaaaaaaaaaaaaaaaaggaaagaaaagaacaaaacaaaaaacaaaactgatgtacatgttttaaagcaaaatagaaccccaagtctaaaagtaaaataagccaaggttagttacaatactgattaaaaagagtatatcctgaggcagttgttagtatatcactctctattatatgcacaataacctctgataggtaaaatatctgagcattttgcaaggtaaacctccaaagttataccacagtgtgcctttttctttgctgtttcttctttgcctattcctacagctaccagtaaacacttaggaactgctttgtatgccagggtctccaagactacctccaggttccatgatttgctaggagaattcacaagactcagcatatcatcacacagctatgatttattacagcaaaagcatatgaagcaaaacagcaaagagaaaaggtacagaggcaaagtctgggggaaaccaggtataagcttccagagtcctctaacagtggagtcacacatatctgttgtttcattccaccagcaactgaattgtgacaacatgtgagaaatgttgtttaccagggaaacttgttagagatacagtgcccagggtttttactgggggctggtcacgtaggtaccttctacctaccatgtaccaaaattctagactcccaggaagaaagcaggttttcagcacaaaccacaggttagctaccatgaacgactcttttcagtgagtggagccctcctgttaaggtttaaatatgtcccccaaagttcaagtgttggaaatttaattgacattgtaaaagtgttatgagacctttaaaaagtaattaggtaaggagggctttgccctcattaatgaattagtgctgctatcttgggagtgggctcatgataaaaggctaagtttagacccatatatctttctcatgctcacttgccatgtggtgccttctgccatggcaagaccctcactagatgctggcaccatgttcttggactgcctagcctccacacctgtcaaccaaataaacttctgttcattataaaatacttagtttgtgtaattctgttatgacagcagaacagactaagataccttctgatatctaagttcccagatgcaacagctgaggacaaaccttataatcaggcctttcaaaggataagtcaggctggctgtgttactcttttctgcatacttagtgacattcccacaggaataatcatcatagacattttcagattcaagaagacccttctaattcagaaacaccttttttttttttttttaagacagagtcttgctctgttgcccaggctagagtgcggtggcacgatctgggctcactgcaacctctgcctcctgggttcaagtgattctcctgcctcagcctcctgagtagctgggattacaggcacatgctaccatgcctggctaatttttgtattttttatttttttggagatggagtcttgctccatcacccaggttggagtgcagaggcacgatcttggcttactgcaacctctgcctcctgggttcaagcgattattctgcctcagcctcccaagtagctgggattacaggcgtccaccaccatgcccggttaattttttatatttctaccagagatggggtttcaccatgttgtcaaggctggtctcaaactcctgacctcaggtgatccacccatctgggtcggcctcccaaagtgttgggattacaggtgtgagccactgcgcccggcctaatttttgtatttttagtagagacaggtgtttcgccatgttggccaggctggtctcgaactcctgacctcatgatctgcccacctaggcctcccaaagtgctgggattacaggcgtgagccaccgtgcctggccagaaacacacttcttttttttgagacagggtcttactgtgtcgcccaggctgtagcgcagtggcgtgatcatgactcattgcaaccatgacctcacaggcttaggtgatcctcttacctcagcctcccgaatagctgggactacaggcatgcaccaccatggtcggctaattttttgtttattttgtagatatgggatttcaccatgttacccaggctggtcttgaactcctgggtttaagtgatctgcccgcctcagcctccccaagtgttaggattacaggtgtgagccaccacaccagacgataaacacacatttttaaaaaaagagaatttcccacctgagaaatggttaattcacttatattaataaattgtcatggctattttttagcttctctagttttactgaaaggtagaataaaaatatatgaaaaacaaaggaaaagtcagtttggtcttaatgaacctgagatcttgatactccaatataaagcaggttctttcagtattaccagcagcaaagactattaatacccatgttacagtcaactagaaatagacttcatatgactacacataattaagcaaaaataaagttgatgactacttggcattaatagtttggacatgaactttagaagtaaaaggtaaaggaggcattataatatcatgtttataaagataactttcttcagctaatattttggggatacaagacgaaacttcgttttgttgtttacgccacttgagtatattctctgccagttcttctgtctcagtcaccaatatatccatctttgctaaagcctggttcattttctttagatttgcagctaaatgaggaatatttctaattgtttcaaggtgggtttctaatctctcaatgaaagtcacagccaactccagcaaatgtaccatatatctgtgataaacagcttcaataggtaagttttcctggcacatgggtttcaacagtctttgcctaagggatctcttctctttcagcactgcttccaaatgattattcatgctttgcagagtatgacacttctgagctgtaatcgcagtgttttgggagactgaaacgggagaattgaggccatgagttcgagaccagcctgggcaacatagcaagacttcatctctggtagatttcagcttgaatatttgtgatctgctgtagtctggtgaagttcacaaaacaagaaactgttttcttagacatgtttaacatctcctgattgaccatccccgaagctatgaagtggcctagcactagcccagcgccgttaggcgcggacgccgggtcccacgggttggcagcggccatggctcggacgcaccttccgcgaaggcgccaagagtgagcgggatc

SEQ ID NO: 12367 - RNA, 1367 nt, Homo sapiens
  source 1..1367: mol_type = other RNA
ctgggaggtcaaggctgcagtgagtcatgatggcaccactgcactccagcctgggtgacagtgagacctcgtctcaaaaacaaaaacaaaacaaaaaaaccatgctcccctacagctttcttccctacagttacagaagcttccagaaatcctcgtaaggcagaataagagtgtagtattggccgggcatggtggctcacgcgtgtaatcccagcactttgggaggccaaggtgggcggatcacctgaggtcaggagttcgagacgagcctggccagcatggcaaaacgctgtctctactgaaaatacaaaattagccaggtgtgatggtgcatgcctgcaatcccagctactcgggaggctgaggcaggagagtcgcttgaatcagggaggtggaggttgcagtgagccaagatcacgccactgcactccagcctgggagacagagtgagactccatctcaaacaaacaaaaaaagatttggatcaggagagggcctcagagcccaataacagctggaacctcaccagcaagcagaaaccagaggggtcagggactttgtcttctgaataaaacaattttgattcctgcaaagtaatatacacactgcaagaactcggcaagtacctatagaatgtacgcctgcatctatgtttataagggaaaattaggcctacagaagtctggaaagaacaagggcatggggcaagggtggggacagcatcaggcatggccgctgtgcatcccgtgggcgcagtctacatgtcgtagagccggagctgctcctgcacgtcgccgtcggacatctcgccaaacgtctccttgttgtctttcatgagcttgaagatggcagccagctgttccttctgaactctctgctcctcctccagctcctctttggtcatcatcttcttgtactggtttcccctcagcttcccggggctgtatttgaaggagaagccttctccgtcctcctcctcaggcccttccgatgatggccccttctcaccatccaagtcctgctcctcttcaaatgctgagctgaggcgtgttcttgactgtgcaccccaagccctcggccttggcctttcccaggtgggtgcctgttgaggcttctgtgtgccatttggagaagtgggcccaggactcccactgcgacgctgcggccagcagacaaagggtgcaagaggaaagctggctggggtgtctgtctgggaccagggccaggcagcatggccatcgcagcctctggctttgcttccttctatgttgttttccatccccaactctctcagtgtccatgttcccaaaactggagccccacctcttcagccagttctctcccacacagagacacaataaacagat

SEQ ID NO: 12368 - RNA, 1567 nt, Homo sapiens
  source 1..1567: mol_type = other RNA
ctgggaggtcaaggctgcagtgagtcatgatggcaccactgcactccagcctgggtgacagtgagacctcgtctcaaaaacaaaaacaaaacaaaaaaaccatgctcccctacagctttcttccctacagttacagaagcttccagaaatcctcgtaaggcagaataagagtgtagtattggccgggcatggtggctcacgcgtgtaatcccagcactttgggaggccaaggtgggcggatcacctgaggtcaggagttcgagacgagcctggccagcatggcaaaacgctgtctctactgaaaatacaaaattagccaggtgtgatggtgcatgcctgcaatcccagctactcgggaggctgaggcaggagagtcgcttgaatcagggaggtggaggttgcagtgagccaagatcacgccactgcactccagcctgggagacagagtgagactccatctcaaacaaacaaaaaaagatttggatcaggagagggcctcagagcccaataacagctggaacctcaccagcaagcagaaaccagaggggtcagggactttgtcttctgaataaaacaattttgattcctgcaaagtaatatacacactgcaagaactcggcaagtacctatagaatgtacgcctgcatctatgtttataagggaaaattaggcctacagaagtctggaaagaacaagggcatggggcaagggtggggacagcatcaggcatggccgctgtgcatcccgtgggcgcagtctacatgtcgtagagccggagctgctcctgcacgtcgccgtcggacatctcgccaaacgtctccttgttgtctttcatgagcttgaagatggcagccagctgttccttctgaactctctgctcctcctccagctcctctttggtcatcatcttcttgtactggtttcccctcagcttcccggggctgtatttgaaggagaagccttctccgtcctcctcctcaggcccttccgatgatggccccttctcaccatccaagtcctgctcctcttcctgcaagacaaggacagggtcagtgcccttggcacagactgggtgatgggaagtggtgggggggcagaaggtaggggagacagaggaggccctcgaaggtccagcctgcccacgccctgtggcagcgcctgccctgtggtcatggtcaaccagcaggtgggggctgtgtacaaacgatgggccaaagtgactcggctcacaaatgctgagctgaggcgtgttcttgactgtgcaccccaagccctcggccttggcctttcccaggtgggtgcctgttgaggcttctgtgtgccatttggagaagtgggcccaggactcccactgcgacgctgcggccagcagacaaagggtgcaagaggaaagctggctggggtgtctgtctgggaccagggccaggcagcatggccatcgcagcctctggctttgcttccttctatgttgttttccatccccaactctctcagtgtccatgttcccaaaactggagccccacctcttcagccagttctctcccacacagagacacaataaacagat

SEQ ID NO: 12369 - RNA, 1391 nt, Homo sapiens
  source 1..1391: mol_type = other RNA
ctgggaggtcaaggctgcagtgagtcatgatggcaccactgcactccagcctgggtgacagtgagacctcgtctcaaaaacaaaaacaaaacaaaaaaaccatgctcccctacagctttcttccctacagttacagaagcttccagaaatcctcgtaaggcagaataagagtgtagtattggccgggcatggtggctcacgcgtgtaatcccagcactttgggaggccaaggtgggcggatcacctgaggtcaggagttcgagacgagcctggccagcatggcaaaacgctgtctctactgaaaatacaaaattagccaggtgtgatggtgcatgcctgcaatcccagctactcgggaggctgaggcaggagagtcgcttgaatcagggaggtggaggttgcagtgagccaagatcacgccactgcactccagcctgggagacagagtgagactccatctcaaacaaacaaaaaaagatttggatcaggagagggcctcagagcccaataacagctggaacctcaccagcaagcagaaaccagaggggtcagggactttgtcttctgaataaaacaattttgattcctgcaaagtaatatacacactgcaagaactcggcaagtacctatagaatgtacgcctgcatctatgtttataagggaaaattaggcctacagaagtctggaaagaacaagggcatggggcaagggtggggacagcatcaggcatggccgctgtgcatcccgtgggcgcagtctacatgtcgtagagccggagctgctcctgcacgtcgccgtcggacatctcgccaaacgtctccttgttgtctttcatgagcttgaagatggcagccagctgttccttctgaactctctgctcctcctccagctcctctttggtcatcatcttcttgtactggtttcccctcagcttcccggggctgtatttgaaggagaagccttctccgtcctcctcctcaggcccttccgatgatggccccttctcaccatccaagtcctgctcctcttcctgcctcgcctccaccgcctgctcctccgcctccgctggcgccgccgcgggatcccctggcccttcgggctcccccggtcccgcaggctccccgagctcccccagccccgcgggctctccaggctcctccggccccgcgggcgaggccgccggctcgggggcgcaggggcgggacggcgccggggccccggtggcctcggccgggggcgcgggttccgggggcgcgcgggcaggctccgggctcgcggccgccccacgccgcaccagtagccaggcgagcagaagggccagcgcggtggccagcgcaggcagcgcggccagtagctcggccggcgcctccatcgcgccgcggccgccgagt

SEQ ID NO: 12370 - RNA, 546 nt, Homo sapiens
  source 1..546: mol_type = other RNA
ctgggaggtcaaggctgcagtgagtcatgattgcatcactgcattccagcctgggccactcagcaagactttgtctctaattaaaaaaaataaaataaaacaaataaaaattttaaaaattaggactcaactaaccccctcccaagggatcctctagaccagaggttgcagcccattgtatctgtcatggatgttttattcctcccatgtaatattaaaaacaaactgaaactacttaaaatccttgcgaacatataaaaatcagatttcacatcaaaatttaggttccggtggccgggagcggtggctcacacctgtaatcccagcacttagggaggccgaggtgggtggatcacgaagtcaggagattgagaccatcctggctaacacggtgaaaccctggctctactaaaaatacaaaaaattagctgggcgtggtggtgggcacctgtagtcccagctactcaggaggctgaggcaagagaatggtgtgaaccatagaggcggagtttgcagtgagctgagattgcgccactgcactccagc

SEQ ID NO: 12371 - RNA, 3895 nt, Homo sapiens
  source 1..3895: mol_type = other RNA
ctgggaggtcaaggctgcagtgagtcatgattgtgccaacgcactgcagcctgggtgacagagtgagaaactgtctcaaaaaaaaaaaaaatttaggtctttgatccacttgaaatatttttatgaatcatgtgaagtaggaaactaatttttttctctctctctttttttttttttttttttgagacagagtttcactcttgttgcccaggctggaatgagtgcaatggcatgatctcggctcatcacaacctccatctcccaggttcaagcgttctcctgcctcagcctccagagtagctgggaatacaggcatttgccaccatgcctgcctaattgtttttttgtatttttagtagagatggggtttctccatgttggtcaggctggtcttgggctcctgacctcaggtgatccgcccaccttggcctcccaaagtgttgggattacaggtgtgagccaccacgcccggcctaattttttttcaaatggatagccaccttgccattgtgtaataatcactaacatttactgaagaacacttacttgggccaggtactattcaatttaatctcactttatcaggtttgttttgcggattaaacactttaaagaggaaacaaggaaggcaacagatggttatatggtttgtccaactcatacagatattaactggtggaattagtattctaacactaacagaatgactccagactatttggcctgttaatgaaatttccttttcccacagaaacgaaataccaccttaataatataccaaatccccacaaatacataggttttttgtttgtttgtttttgagacagagtttcactctgtcgcccaggctggagtgcagtggcgtgatctcggctcgttgcaacctctgcctcccgggttcaagcgattctcctgcctcagcctcccaagtagctgggactacaggcttgcaccaccacgcccagttaattttggaatttttagtagaggtggggtttcaccatgttggccaggctggtttcaaactcctgacctcaagtgatctgcccacctcagtctcccaaagtgctgggattatacataggttaatggattttctatggtgtactgtttcctatgcttcatcttccattcctaatttactggggaggcacctattcatttttaagattagctcaaaccacatgaccactggcctttcctccctctccatcccaaccagtagaaaaaaatcattccacctttatgtgcccatgacatgcctctgaaacttttaccctagcactgctattttacggcatttattcatttacatgtttttctttcccaccataatgagtgtcttgagggcaggaccatctcttattaagcacctagtatacatttaataaatgtttattgagtaagtcagtataaaacaatgaccgccaaattatgtgagcaatcatcagaatatctgatttctaaaaagacgcaacaaaaattttttattgtaaattgacaatttataattgtataaatgtatgggttacaaagtgatatcataaattgtggatacaatatggaatagttaaatcaagctagttaacatatgcaatacttcaaatacatttctgtgatgagaacatcaattttgaaatgtataataccccattattaagtataggcaccacactgtacaacagaactcaaaaaaagcataaaacatattcttcctgtctgagattttataccctttgaccatcattaatttttttttttttttgagacagtctcactctgtcacccaggctggaatgcagtggcgcaatctcagctcactgcaacctccacctcctgggttcaagaggttctcctgcctcagcctccccagtggctgggattacaggcacgtgacaccatacccagctaattttttttgtatttttagtagaggtggggttttgccatgttgtccaggctcatctccaactcctgacctcaggtgatccacccaccttggcctcccaaagtgctgggattacaggaatgagccaccatgcctggcctagtttttatgagacaaaatatcaatttcaaaacagcatcagtggcaaaacagcatcagtggctggacgtggtggcacgcacctatagtcccagctactccgcaggctgaggcaggagaatcgcttgaacctgggaggcggaggttgcaatgagccgagattgcgccactgcactccagcctggtgacagagcgagactccgtctcaaaacaaacaaataaacaaacaaacaacaaaaaagcagcatcagaaagtgagcaggccaggcacagtggctcatgtctgtaattccagcactttgggaggccgaggcatacttttctgtattaaaaatacaaaagtatttgtctctactaaaaatatccaccccccccgcccaaaaaagaaaaattagttgagcatggtggtgtgtacctgtaatcccagctactcgggaggctgaggcaggagaatcacttgaaggatgggaggcaggggttgcagtgagcccagatcacgccactgcactccagcctggtgacagagcaaaacttcatctcaagaaaaaaaaaaaaaagagtgagcatattgaactaccctcagctcatagtaaggcaaataggtcaacagaataataattcatgctattgcattggaaaagcaattaaaagaaatttaaaaatgtgtaagcagaaattcagttgcatgtaagaaaatccaattccccgtgagaaagagaaagagctggagtcctttaaaaattaactgcctgtttttctgtggctagtgagccttatctctcctcctttcccaggcattgtaaataccctgtttctctagctgtgcagctgcaaggtaactagacagataaactcaagtcgtaaaacatgattttccttgaaaagtaagaaatgatgtaatgcatgtctcagttaattgaataactgtctttcttgcttctgtaatatgcttccccctgcacagattccccccaacccccgcggccccacaaaatgcttaaaaggtaacttaactctgttcagggttcagtcctttggatgttaatctgactgggctggtgcacctaaataataaatatctccctgaactccatcagtctctctgattccttaaaaatcccgctacattttgtgtaatgaactggcaacaagagaaagttggtcgaagaaaggcagaggaactgtgtcttgtaagaattagaatcgaggggctccataatcatctggcatccgttcaatgttgtatctatggttagaaatgtacatgataggaactccaggaatcttacggattcttcttttcaggtcccggtcaactgtggccacaatgtaacacttatgctgagttactctctgtactaagcagtcatctgcataggttcctttgtgtgtacatggtaatcgttcaaatcttggatccttggcaatccttagagccactcgatacttctgccccaatttctcaatttcagccattacacaatcggttatacatgggatacacttggcatacagacagtccatcattgactgcactaagtccagtttggcttttatggaaaagttgataaagttggtatcaacgaggatgtggtaaggtgggcccagctgtgtattatattggaaaaataagcaggaagggtgttggggaacttctctttcctttaatgcgctgggatccttcttttctttctttttaggttttaatctatccttttctttaagcctctgatctctgagactaagcattcgcttcatggtcgcatacttccttgttttcttttgcttccccatggtcacgccaaactcctggttcttccgtaatcaccaacggcgcaatacttctac

SEQ ID NO: 12372 - RNA, 3954 nt, Homo sapiens
  source 1..3954: mol_type = other RNA
ctgggaggtcaaggctgcagtgagtcatgattgtgccaacgcactgcagcctgggtgacagagtgagaaactgtctcaaaaaaaaaaaaaatttaggtctttgatccacttgaaatatttttatgaatcatgtgaagtaggaaactaatttttttctctctctctttttttttttttttttttgagacagagtttcactcttgttgcccaggctggaatgagtgcaatggcatgatctcggctcatcacaacctccatctcccaggttcaagcgttctcctgcctcagcctccagagtagctgggaatacaggcatttgccaccatgcctgcctaattgtttttttgtatttttagtagagatggggtttctccatgttggtcaggctggtcttgggctcctgacctcaggtgatccgcccaccttggcctcccaaagtgttgggattacaggtgtgagccaccacgcccggcctaattttttttcaaatggatagccaccttgccattgtgtaataatcactaacatttactgaagaacacttacttgggccaggtactattcaatttaatctcactttatcaggtttgttttgcggattaaacactttaaagaggaaacaaggaaggcaacagatggttatatggtttgtccaactcatacagatattaactggtggaattagtattctaacactaacagaatgactccagactatttggcctgttaatgaaatttccttttcccacagaaacgaaataccaccttaataatataccaaatccccacaaatacataggttttttgtttgtttgtttttgagacagagtttcactctgtcgcccaggctggagtgcagtggcgtgatctcggctcgttgcaacctctgcctcccgggttcaagcgattctcctgcctcagcctcccaagtagctgggactacaggcttgcaccaccacgcccagttaattttggaatttttagtagaggtggggtttcaccatgttggccaggctggtttcaaactcctgacctcaagtgatctgcccacctcagtctcccaaagtgctgggattatacataggttaatggattttctatggtgtactgtttcctatgcttcatcttccattcctaatttactggggaggcacctattcatttttaagattagctcaaaccacatgaccactggcctttcctccctctccatcccaaccagtagaaaaaaatcattccacctttatgtgcccatgacatgcctctgaaacttttaccctagcactgctattttacggcatttattcatttacatgtttttctttcccaccataatgagtgtcttgagggcaggaccatctcttattaagcacctagtatacatttaataaatgtttattgagtaagtcagtataaaacaatgaccgccaaattatgtgagcaatcatcagaatatctgatttctaaaaagacgcaacaaaaattttttattgtaaattgacaatttataattgtataaatgtatgggttacaaagtgatatcataaattgtggatacaatatggaatagttaaatcaagctagttaacatatgcaatacttcaaatacatttctgtgatgagaacatcaattttgaaatgtataataccccattattaagtataggcaccacactgtacaacagaactcaaaaaaagcataaaacatattcttcctgtctgagattttataccctttgaccatcattaatttttttttttttttgagacagtctcactctgtcacccaggctggaatgcagtggcgcaatctcagctcactgcaacctccacctcctgggttcaagaggttctcctgcctcagcctccccagtggctgggattacaggcacgtgacaccatacccagctaattttttttgtatttttagtagaggtggggttttgccatgttgtccaggctcatctccaactcctgacctcaggtgatccacccaccttggcctcccaaagtgctgggattacaggaatgagccaccatgcctggcctagtttttatgagacaaaatatcaatttcaaaacagcatcagtggcaaaacagcatcagtggctggacgtggtggcacgcacctatagtcccagctactccgcaggctgaggcaggagaatcgcttgaacctgggaggcggaggttgcaatgagccgagattgcgccactgcactccagcctggtgacagagcgagactccgtctcaaaacaaacaaataaacaaacaaacaacaaaaaagcagcatcagaaagtgagcaggccaggcacagtggctcatgtctgtaattccagcactttgggaggccgaggcatacttttctgtattaaaaatacaaaagtatttgtctctactaaaaatatccaccccccccgcccaaaaaagaaaaattagttgagcatggtggtgtgtacctgtaatcccagctactcgggaggctgaggcaggagaatcacttgaaggatgggaggcaggggttgcagtgagcccagatcacgccactgcactccagcctggtgacagagcaaaacttcatctcaagaaaaaaaaaaaaaagagtgagcatattgaactaccctcagctcatagtaaggcaaataggtcaacagaataataattcatgctattgcattggaaaagcaattaaaagaaatttaaaaatgtgtaagcagaaattcagttgcatgtaagaaaatccaattccccgtgagaaagagaaagagctggagtcctttaaaaattaactgcctgtttttctgtggctagtgagccttatctctcctcctttcccaggcattgtaaataccctgtttctctagctgtgcagctgcaaggtaactagacagataaactcaagtcgtaaaacatgattttccttgaaaagtaagaaatgatgtaatgcatgtctcagttaattgaataactgtctttcttgcttctgtaatatgcttccccctgcacagattccccccaacccccgcggccccacaaaatgcttaaaaggtaacttaactctgttcagggttcagtcctttggatgttaatctgactgggctggtgcacctaaataataaatatctccctgaactccatcagtctctctgattccttaaaaatcccgctacattttgtgtaatgaactggcaacaagagaaagttggtcgaagaaaggcagaggaactgtgtcttgtaagaattagaatcgaggggctccataatcatctggcatccgttcaatgttgtatctatggttagaaatgtacatgataggaactccaggaatcttacggattcttcttttcaggtcccggtcaactgtggccacaatgtaacacttatgctgagttactctctgtactaagcagtcatctgcataggttcctttgtgtgtacatggtaatcgttcaaatcttggatccttggcaatccttagagccactcgatacttctgccccaatttctcaatttcagccattacacaatcggttatacatgggatacacttggcatacagacagtccatcattgactgcactaagtccagtttggcttttatggaaaagttgataaagttggtatcaacgaggatgtggtaaggtgggcccagctgtgtattatattggaaaaataagcaggaagggtgttggggaacttctctttcctttaatgcgctgggatccttcttttctttctttttaggttttaatctatccttttctttaagcctctgatctctgagactaagcattcgcttcatggtcgcatacttccttgttttcttttgcttcccctccttctccacccaaaaagtggcctgataacgtcccttcttggaccgtcttctctcaccatggtcacgccaaactcctggttcttccgtaatcaccaacggcgcaatacttctac

SEQ ID NO: 12373 - RNA, 2690 nt, Homo sapiens
  source 1..2690: mol_type = other RNA
ctgggaggtcaaggctgcagtgagtcgagactttgccactgcactccagcctgtgcgacggggtgagaccctgtctcaaaaaaaaaaaagaaaaaagaaaagttttatcaaaggataaaaccgaaatgctatagtatatagtgtgaccataatttcagaagaagagaattagcataatttaaaaggatagctagcatactatacgttttaataattccagtatttttgttacttgggcttaatttaacttattttcctctttttgatttttgtatttttaagagggcacttttaattttcaagttgtgtttgaaactatagagtatgctaatacaacttaatataaatataaataatatataagctctctctctgcatatatacacatataaacagacccaagcattagaccactgatgttgtactttcaggattcacacgaataagtctagatgcattcctcagatcttggagttgcttggcaggtttccccacaccttcttcaaaccttttctccaccacagggaggactgtttcatataaaaaggatgcattctgtctgataaaagctttcttctctggatcctgctcacatcgaagactataatccacatgctgaacagcaaccaaaatgatttccaccaggctctccaaaagtaccatgtgcagctctgggaaatacagcttcagggcctcttccaagaagcccatggtctgtttggtgaaagcaaccactgtgtaacttaggttcacccagcagtcatcccctgtgtactgctcaaagttacttaccccacaacttttcatctcttctttgagcttacccagggcttctggcgtcatcaagttcatcctcctccacatctcttcagagttgcgatgtttagtggcttcaatgatgatttctttgtaactgtgcaaggccccttggatgtctttcaccagaagggcatggatgatgaaggtgagatccagtccgatatcacccagttgctggcaatgctccttagccacttttacacactcagctgctgtagagaggctctccttactatcaaacacctgcttgctaaaagcatccacgaacatgcccatggctgatcttgcccagaccacaaaggcagagtagcagccgctgtcagtgcctgcaaaatcgatctcaaattctcttgcagtctcgagaaggctggtaaagaagacatggcacagcttatgaatatagagtaaagtggcaccttcgatgcgaagctgacgaattgcagtatgaacagcggctgccctgtttctcaaaaatagctcacaggccttcgtgcactggcccagccggatcagttgcgaaactgctctgcgagtagccttcggaccacctctcagggaacgatctggggagagttcgaaaactagcacctcagtgagctgtcgaactcgctcctccactttggcccttagttcttttacaggaggtgggctaggtttatcttccaggtaatggttcaatttatccagcaggtcaaccgccccttcaaagtctctctgcgcaatgcagacatccaggtcttcaggtaactcctggatccattccatggagaggtccaccttctcttcctctacctcaggaacagctggttcttcttcttcgtcatcctcaaatgggttagtggccttggaagtcacttggggtggccctcgaggggccgctgcctcctcctgctcccttcgccttttctcactgagggccctcttggtgtcctccagcacttccagccactctcgtttgattttagcattttcggcctggaaaatacggctctcggggaacataagcagcttgaacatgtccttcatgggcgggttgtccttgacattgactacggccaaaccatctagggaatagagagcgttgtagcgatacatcccacgccgctgaggcagccaggtagccaccaacaagcaatcgttcatgagaaagccgtgcacccgctgcagttgggccatgtggtccgcatcgtattccactaggtccccattgtacaccaagtactgtcccggcgtctccagcagatgcctgcagccttccaccttctcaagcagggtggtgagagtgcgctgctttccttcctcgcctggaccggagccgtcgcgggaggcacccccgggggtggagaaaaagccggcctggcctcggaggtggtctcggccccccgccccaccgactccctcctcccctccagaggcggcggcggctccggcggcagcagcggcaggcagcaacgtaagcgggatgctctccaggctgcttttctgctcggtcagcaaatggctgagctggtacatctcgctctccaggtaggagatctcgcgggccgtctctatgaactgccggtagttctggtagacgttgcgcttcaggttctgcgccgtctcctccgccagcgcctggatgcgctgccggtgctcctggaggtcccggtccccatccgactgctgcgagagctgcttcacgtacagccgcgcctcaaaaccccctgactccagctgccgacgcaggcggctcgccccactgtccgacatcgccatcgccatttctctccgggtctcacgcactcactgtcactatcggcgccgcagccgccgcggctgtctagacccacccaaggccaaccgagctcctgggctgaggaagcaggaat

SEQ ID NO: 12374 - RNA, 228 nt, Homo sapiens
  source 1..228: mol_type = other RNA
ctgggaggtcaaggctgcagtgagtcgtgatcgtgccactctactccagcctgtgcgccggggctctggatgccgagttgtggcagagccttgagaatgcaggctcatggtggtgtccccatcatcatccagcatgtccctcgtgctgctgtacttggcctgcatctggattcctacagcggtgagagtgaaatgtggtcggattgccctgggccgccgggctactgt

SEQ ID NO: 12375 - RNA, 319 nt, Homo sapiens
  source 1..319: mol_type = other RNA
ctgggaggtcaaggctgcagtgagtctagatcagaccactgcactccagcatggaattgactttgtcttctggcccctgcacttggcctgtcacggtgcctttgctggtattcttcacccagccaaccactcctattttcctagcttcatcttctgtatacattctgaagcaaacaccctgcactcttccgaacacctcgtagtccacggatttgagtgactgggcggtagacatggcggcggcgagccctctgttgaggagccggagaggggctcggggcgcagcgactgcggcggctgcgagagggaggggacacat

SEQ ID NO: 12376 - RNA, 64 nt, Homo sapiens
  source 1..64: mol_type = other RNA
ctgggaggtcaaggctgcagtgagttatgatcgtgccactgcacttcagccttggcgacagtta

SEQ ID NO: 12377 - RNA, 2352 nt, Homo sapiens
  source 1..2352: mol_type = other RNA
ctgggaggtcaaggctgcagtgagttgtgatcacactactgcactccaacctgggcaacggagcaagaccctggtccgatggccattgtcgagacacaatggtgcagtcagaagccccgatgtgacagcagcctttgacccgagctggcacgaccgtgggcacttggctgaggatgccttggtgcgtcctgtgcagggagccctggagcattggcagtgagcgtagggcaagttatatgaaaggtggtgacacaggattaaggggcgtgaggccttctcatgacctgtgtggctgggagaccatgggaacgcggcaacaacagtgcgtccagagagccacagcgcttggcctcacgtttcctagattccgtggctgtcacaatggaagacacatttttcatggagagggaacagcacagttacgccacacccttacagtgcaggggcagccaccttccagggaaggacaaggaagacagggaagacgctgaacacaaggcagcctctgttcctgagagcaagctcatcaggacgctttcctcccacacagcccggagagttcaggccagagcccaggcttcccgtgtttcacacgcagccgctccgagcgtcctcggccagcgcagcttcacctgctctcagctgagcctccagcgttgggcctgccttctctagtaaacaagctgaacgactcagatctttgacaccttttcttttcttccccccacctttttttttaagagacaggggtctcactctgtcccccaggctagagtgcaatggctcaattataggtcactgcagcctcaaactcctaggctaaggtgattctcttgcctcagcctctcagatagctggaactataggcacatgcccaccacacctggataatttatcgttattcttatttttgtagaaacagggtcttgcggcagggcacagtggctctcgcccgtaatcccagcactttgggaggccaaggtgggtggatcacctaaggtcaggagtttgagaccggcctggccaacgtggtgaaaccccatctctattaaaaatacaaaaattagctgggcgtggtggtggacacctgtaattccagctacttgggaggctgaggcagggagaattgcctgaacccggaaggcagaggttgcagtgagctgagatcgcgccactgcactccaaccttggcaacagagcaagattccatctcaaaaaaagaaggaaaagaaacagggtcttgctgtgttgcccaggctggtcttaaactcctgggctcaagtgatcctcacacctcagcctcccaaagtgttgggattataggcatgacccactgtgtctggctgatcttttctttatacgtgccgtgatagtagccatgttctttagtgttttcacaggtcctatggcccttccagaggaacggctatgtcaccctctcaaggagcagttggctgtgagagagggagggctggtcagggtgactcactatggcagctcccacatcaccccgtgctgcagctgagaggaggggagtctgcacactgatgttgtccctgccttggactctcctacagagcccgcagcttcatctcccagctcaaacaacacagcggccacaacagcagctattgtcccgggctcccagctgatgccttcaaaatcaccttccacaggaaccacagagataagcagtcatgagtcctcccacggcaccccctctcagacaacagccaagaactgggaactcacagcatccgcctcccaccagccgccaggttagcactcgctttgccccaggagaggtcagttccccattgctgcttctgagatcggggctgagatccggcacaaggcagctttataccatcaatccaaagtcaggattcactgggcagcctgctggccccggccaccagccacggcgtcctggcctgacctctttctccgtggctttctctgtggctggggcagctgcaaaagcaagcccacacccccccaagatgtgacagggccagccttatcacccgcatggcagagcctgtgcagctgggagtggcatctgtgccctcctgcagtaggaggtggtgaagctgcctacagtccggggccaggatctgtggaatggaggagctgagggtaatggggaccttctgtaaggcttatctgattcttaagtgtggccagcacctcagtgagctaccctgcttgttctttgctaaaatgagtctggttacgccagccacgagtctcccagggtgctaagatgggagccaagccatgcagattttctcctgcttcatgaggaactaggacctctaggactcgagccgtgatgctgtcctctctttt

SEQ ID NO: 12378 - RNA, 782 nt, Homo sapiens
  source 1..782: mol_type = other RNA
ctgggaggtcaaggctgcagtgagttgtgatcacatcactgcattccagtctgggtgacagagcaagatcttatctaaaaaaaaaagtcattttaaaaagataatacatgtggaagcatttagcactgtgtttgcgcgtggcaggtgctcagagaatgtgtgcgcttagttccttcttactcattacatcactttgtataagagatttgagcacctttgaatccccaaatctatgaccaatccccacttatgccccactttaccgatggacgactatatgtggtgctttggcccagggtcctcattcaatatgtttctttagcgaatgagttaaaccccataggctgttacatagctaagtacaggaaccctattaagaatatacggcagagtaggtgctctgatatttagcttcgtctaacggcagaatagaatttcctgagtcagcaggatttctggcctgatcacttttttgctattggcttcacagtggcttcatctcctgttttggagacagggaattttccccattccctgggctgcttttagagcttcaggtgtgtgactttcattaatagctctcttgcaaatggcaatcttctcggtgtggcttgtatatcagttgttggcctctcatattgctgtgtcctttgatgctttgagcttctcagttccttctggtctctttttgtttttctcctttccaaaactcattctgaaggacccatgaaaagagactgaaagcagaagaaatctgtccagtcactcagcaacacctatct

SEQ ID NO: 12379 - RNA, 6544 nt, Homo sapiens
  source 1..6544: mol_type = other RNA
ctgggaggtcaaggctgcagtgatggcttcactgcactccagcttaggtgacaaagtgagacccagtctcaaaaaaaaaacaccacacatgaaaaacctcagaacacaaaaacaggctgcttctgacaaaggcagcacagctagaccatcatccacaagagaagctagattgttacaaggcatctctccatcccctcgcagctggtggtgggcactggcatttaatccagggtgtggggcagcatgggagaacagacttgatttaatcccagacaatattccaacagcccagcccactatggtaatcagattgattctaataaataagcaaaaaaaaaaaaaaaaaaaaaggcaagtaaatgaaagatataaagtgagatccaaagagaaagagcgaacctttgctaattctggattcgaaggaaaacattttagttcctctgccccacccactcacccagggaggataaagagggaaagaggggtgcacctcgagttcctgcagatggacagaggaatgccagctttgtcccgctgagtgagcctggagaacagcaggaagctctgcagagaagggggcctgtgcaccttgctcaaatattgaaatgagacctttacgtgttttaatccgttccgctgagggagtagctgggagagggagaaaagacttgggctgcgaaatcctcgaatgtcattacttcgcggtggttctgaattattgcttcgagatacagagctcgctcttcatagaagctctggtagagtgggatgaggcacttcacagccctgctggcgttgatgcacgtggcacatacaaggcttggcagcagcttcccactcactatggctccatcaaacagaggcccaaaaaatggaacctcaggtttcttcgttatcgcgatgaagaacatgtgattcttcattgggtaaataatgattgaaacatctccaaaggcagttgggataatacccctgcggtagtctctggagtgttcagaccagacgatatggacctcgtcattccccaagtgacgaagctttttggtgagggaatcatctgagtctgacggcattcgagtggaaacatggaaaatcacttccacagttgaggtagcatagtaaggggccgtctgcccggtgctgccattgcgctgaaggccacccatgaacccacagtgggtggagagatccacctcccatccaagtccagcaacaaagtcttcatatgcttggcttcctctttcattagagaggattgaacacttgtcttcttgaccttcagcaatgtaaaacactgcgattttgtgtgtctcacggcactggcgggagtccaaatttttcagctctctcaataattttgaatttttcttcaatagatgaaaattcttccttctgtcccaagaattcattcccaagtcatcaagcaataacctgcagaaataaaagggtcctcggggctccactggggagggctgcccttggctggtgactttcattgcagaatcgaagttatgactctggatatactcatcctcttgagcattttggcgcaaaatgacctcaatgatttccttctcttggtcatagttcatgccacatggggttagggaaggttcatttagatttagctgtgacggtaaaaggcattcaggacttgtatggccaatgttttcaagtaatttgtcaagaacatcatccccctcctcaacttgagaagagtctttctgaggtccaaatgtgtcacgatgccagctcgaaatcagaaatgaaggatttcttccattgggtgctaagcagccttccaaaggtccatataaaaccttaccatcccaagagtacttccctgagatatccctcacaattactctcacatcagagagagagcccactggtgatccccctaccggtccttctgtgggtgtctgaaggtaggagatgagggtgctatcattaaatacaaacagctgcaggtttggacttctgaacacctcaaaggacagctcggagccttccacatgggcattgtcatggttctcgctgacaaggctgtgcagtatggcagggcccccactgagggggtagtgccccaggtggttcaccaggtgggccatcaccattcgagcagtcaaagggatcaactccaaacttcttctcttcttctcctcttcaacagtcagcaggttacccaattctgctgatgaatgatactggactggctcagagctcttcacatttgccagtggcaggaaggggtcataatccgtggatgacaagtcagccagggtcagtatgtagtgactctgttgggtgtacgtgcttgagccacacacacagcagtgcaaaaccctgtagatataatccagcaagggggctctggccgaatgctgctcctctaggactgctgtggacacggggtggagaaggacactcacgggcaatgccatgcaccagtccaagaggcagagtagcaaggacacaataaacttcttgtctgtttccactgaggagtactctgcacttggtaaaagaaaagcaactgtggccacgaggatttctgccattttccgaggcagagaggtttcaaacatctgaagcttctcccagtaggaaaccagcaactgaaggacatcgcaagctacctgggccacgattttgttgggaaacttcagagttactcctatcacattgatggcctctttcacctgagggtggcttgtacactgtgcaagctcttcacatatccagaccccaagggagcaaacagcaatgcatcttgcatattcatttggttcttctgtggcattcttcagtaaaatatttatgaggtaatgcttgacatcttcagttcctgtaatggcctcatttacttctggcactgactgcagtaaaggaatctcctggtaggtatttggaaagcagaccagagagccgaggacagtgacagcctctgaacgaggcgccgtcaaaatgtctgtgctaaggaccctggcagcggccgtgatgaagtcccccaccagcattgagaagccaggaaaacccagggagaaaaagcggggtggacagtgccttatgatcgtatttaagatatcctgatcctcgctggttaatcccaggtgcatcacaaggtaaaaatgcaccaggaaatctgagtttggcagaacgtcctggcgtctggtcatcatggcacagatcagcctgtaggcttgtagtttgccttccttatattcatttggcagtgtcgccgccttaaacagccatgatgcaaacattctgagtggtgggatcaaaactggaggagatggagaagactggttatccaggcttattgctagattatcccgtatctttgctagtttgtaccagagttcatagagatagcagaaaactctggcatggatcttgggtgactggatgttattcacatctccgaggatccccaagacccttcgccataacacagcagcagagtctgggtgccaaccagtgaggctccccccggcgattatactacagtcatctgtgaggcactcgctgctatctgttaaatttgaagcatcggtgggactcagttgtaaccaatgacgggcatcagcatcagccacaacatctgtgggagtattcagttctgggtcttcctcacaggtctgccatgggcccatggacagctctgcctcattggtacagcccagagttgtgtcactgttggtactttcactcttctgtctttccctacattttccttgtgtctgctgcaaatcatctttcaaatccaattcagcagggctgctgcttcttcgaactaagattgttattccttcatgttctctcttcacatgtcctttattctcttgaataggctgaggctctgaagaactcgaattctgtgtgttttctgccttttgaccctgagaagaatctgagcacagcggctcggggatgtcggaggtgctgctgctccgaaggacctgctgctgctgtcccactgtgagatggccagatccggctgcaggtgcattttctgactgttgacactcctccacttctgacagcctgtgagagcaagaagagtaagagagaccaggtaagagagcgctcacggtgtgaaggaggagcgggacgcttttagtggcaggcaaagcctcagaaaggtggacacagttgctgatagactggcttcgcttagcagttgctttttggcgaacaatatttcttgccttttccactcccggtgctccagacgtggtggcactcctaaatcgcatcggttcggtcacatctgggtggctccgccagctgagagaaaaggacctccccacggtggttcctttctgaggatctagaacacagcctttgcctcgttgcttcttttccttttgttcacttaatttatccagaggtaggtttgtcatctcaactccataaacggttcttgcaagcactgctgtcaaggagtccataatgttggcccactcgtttataagttcctcccattccgtgagggaggacagcacaccaagaaagtcatcccagagctctcgagaaatgtacacacagaggtttgctcggatccaagctaccatgagcgtcctaaatagtaaccctgccaagctctgggcaaacaagtcctttatttgtttatcctttggcttctgcatgacagcttctgttatcctgagtagtatttgcaacatctgttcccatgtctttttattcattgtaagctccattatcatgcgcctaaaaataatcaaaacagctttacaagcatcaacttgttctttcaagagcacaggaacttcagcacatggttccaacaaaaagatgtttgcagagttcgtcaaaaatacctgcaacaaagcctggacgccggctttcacatttgtattttcctcctctgtcacacaccctctgctcattgcacttgtgaaggagtatgtgcgtccccaactggaagatcgtttatgaccagaactttcagatgaggcctccttgctatcagtctcggaaaatcctaatttttcagcatcttcttgggcaacatcttttctatctggctcctccatgaacacaggtttgtcctggagaatccactttctgtacacttgaactacttttcttgttacagctatctcacaggaaggcaacaaaaatgcctggtgaaatacttcattcacgaagttgacataacctcgtgttgacaagagaatccgctgtaccatttcatacaccattcggtgctcttcttcaatgctacagaggctggagttgctgagtcttcggtccgacaaggtgctgctgttagaatggcttttgtcctgctccgtgggcccaccaccatccagctcaggcgctctctcctgcacagcaccaccaccaacagtctggatgattttaggcaatacatcaactccatttttagtgttttgtgttgcagttagatactttttttccaaaaagaaggttacaatccacttaataaaaacaacacgagctgccatatatggaatctttgtactgtaaatgttctcattgtctcgagtggtagtaatgtacacaggctttggtctcaaatgggggatgtcaagtacaggtttgtagatgtttgttaacttagtaaatgatggaaataaatgaggaagataatactttcgaaacaatgtaaaaagaaatttaaaaccagtatcttgattctccttattcttccactccaagctcgcagcctgaataaccatatacttcaacagtatttgaagaaaaaagcaggtttggtcctcagcaatcttctcccctgatatggctggtaggagtggagtgatttcttctggatatatctttacatcagctacactagggctgggattgatgagtgtctccagtgtgcaagggcccctggatgacatgactgctgggaaaccaggcaccaggcaagcaaaaatcagaacctgctcttctgcacagtttgtctgaagtgcttgaagccacagaagaaacagcctgattccttcacatcttatcttaatagaatttccagtgtgtagaagcttctttaaagttgagcctatactctggtaatgccatcgaaagaaaattcgttcaggtagaaactgcagtattttttcaaaaaggaagaggatggagtccagctcctccctttgtgacttattattcccttttaatttcaaactattttccagtgctataaaattttcatagaagatgaaatatatctgagaatagttggtctcaaaaaactgcttaagatcatttgcatccacattatccagcagcgcccgcaggtgcttcaggcgggtcagcacgtccttcttcgggtccagcaccttctgggtggacttcttcacatccccgtggctccttcgggagaacatcccgcggcaggaagcccgggccccgccggcggggcagtaggcgcctgcgccacgcgaatcaaagcatagggtcgaggccggcgcgtgtcgcgcgggccactcgccgcccccagccccgctgctgccgccgccgccgccgccgccgccgcctcagctgt

SEQ ID NO: 12380 - RNA, 272 nt, Homo sapiens
  source 1..272: mol_type = other RNA
ctgggaggtcaaggctgcagtgcagtgagctatggtcaggccactgcactccagcctggacaagagagtgagaccctgtctcaaaaaagaaagaaattataaaaagaaacaaaaaggtaagataattattatagataactcagagcaagcagaccccatctttctttgtctaggggaagcccccacaacaccctgtacaggagatggccctctgagaggagcctggtggccgctgacatccagatgtaaatttctcattgtcctggttattg

SEQ ID NO: 12381 - RNA, 701 nt, Homo sapiens
  source 1..701: mol_type = other RNA
ctgggaggtcaaggctgcagtgcgcctcgatcacaccactgcactcagcctaggcagcagagtgagactcccaactttcccaagaaaaggccctaaggtagaaagaactaggttgcataagcaaaatgtgccaaaagcctgagcgaccgaagcacttttgcagaagccccccgctcctcatctcctatcacatcttctgctcaatcaagctgggccttgtcgacttcggaaaggcgtttggattttgttctaaaagcactgggagccactcaagagttttaagcagaagcgtatctacactaggcttacgcttttacaggaccactctggttggcgtgtagtgaatacacgactctccaattactcagaacagtgagtggcaaagacaacaggtctggcaatcagagaactcgtggcccagttaggggtgcgatggttggagctactgcggtctctgtggctgaggggaggcgccaggcacgagtactgcgacagagccccgcgagtggcaggcacccggctgcactgcagagccggggccagcctagaaccccgctctcctgcaggcccgggtgtcccgagctgccccacgcggaggagtccaagtaggcccacgctaggctcctctgccgaaaccctggtgccaaggacaccatgctcgctgcacacagaaccccaaagcgaccccaccttcccagcat

SEQ ID NO: 12382 - RNA, 113 nt, Homo sapiens
  source 1..113: mol_type = other RNA
ctgggaggtcaaggctgcagtgcgcctcgatcacaccactgcactcagcctaggcagcagagtgagactccgccgcgggaaaccctccgctcgcctccgctgctaccactttt

SEQ ID NO: 12383 - RNA, 150 nt, Homo sapiens
  source 1..150: mol_type = other RNA
ctgggaggtcaaggctgcagtgcgcctcgatcacaccactgcactcagcctaggcagcagagtgagactccgccgcgggaaaccctccgctcgcctccgctgctaccacttttaccgcggccagcacgcggggcgggacctcgcagcgtc

SEQ ID NO: 12384 - RNA, 158 nt, Homo sapiens
  source 1..158: mol_type = other RNA
ctgggaggtcaaggctgcagtgcgcctcgatcacaccactgcactcagcctaggcagcagagtgagactccgccgcgggaaaccctccgctcgcctccgctgctaccacttttaccgcggccagcacgcggggcgggacctcgcagcgtcgaggagcg

SEQ ID NO: 12385 - RNA, 176 nt, Homo sapiens
  source 1..176: mol_type = other RNA
ctgggaggtcaaggctgcagtgcgcctcgatcacaccactgcactcagcctaggcagcagagtgagactccgccgcgggaaaccctccgctcgcctccgctgctaccacttttaccgcggccagcacgcggggcgggacctcgcagcgtcgaggagcgtgctggggggcgggtcct

SEQ ID NO: 12386 - RNA, 3029 nt, Homo sapiens
  source 1..3029: mol_type = other RNA
ctgggaggtcaaggctgcagtggactatgatcatgccactgcactccagcctgggtgacagagcaagactctgtcatttacaaaaaagaaagaaagaaaaataaggctgctgggattttgattggaagtgtgtaggatatgtaaaagaatataggaaaatgaacgtctttttttttttttaatttttatttgagacggagtcttgctctgtcacccaggctggagtgcagtggcgcaatctcggctcactgcaagctccgcctcctgggttcccactattcttctgcctcagcctcccaagtagctgggactacaggcgcccgccaccatgcccggctaattttttgtatttttagtagagacagggtttcaccatgttagccaggatggtctcgatctcctgacctcatgatccacctgcctcggcctcccagagtgctgagattacaggcgtgagccactgtgcccagccatgaacgtcttattaatgtgagttttcttatacatgaacatgagatatatatatagatagacagatagatagataccactatatatatatatctccatttataaagatatttaaaaatttcagcaatattctgtactttttactataaagatcatgcccatcctttactaaattcattcctatatattttatatttttatgctgttgctaaatgattacttaattttaattttcttattttttgctcctagtatatagagatgcaatgggtttttgtatattggccttctatattatgatattggtaaatcactttttaataattgccattttcttgtaaattccctaggattttctatacaaacaactatgctgtctgtgaataaatacagctttatatttttccttccaatatgtatttctttgtttgtcttatttcgttggggaggacctctagtcaaatagaataaaagtgttgggagatgagatccttgccttatttctggtttataagggaaaacatttagacttccaccattaaatttgcaattagctatccctggtgctcttgttgtcatatcaacttgacacattataaatccaatctccagtcttatcttaaaatagtcttaaaataatcttcccttacaatagtcagttgtctctcaagagaattcagagagaaaaaaatccatgcattttaatatttacgttctaatttaccacttctgctgctctccactccttcttgcagatccaagtttctgtttccattaaggatagtaaacaaattcattttcaaattatattcttggtcatcctgggctttatggctggcttcatatcatatccgattatgtgaaaacaaagtgtgacctcgtaggatggtgacattgcgaaggatttctccatgctgtgtgtccactgccttcatctcctccacgatcatggagaggttccggacgttgaggtccagccgggcactgagcaggctgaagcgctcccggagcaggtctgtggtgcccagcatgatggagacagacttgttcaggtagtagagctcctcggcatgggtgtggaagcccagcgtgcaggagagccgcacgtcatccaggtacttgagcatgctgtgcacgtggttgtcggtggcattgatgttggtgaagatggtgccaatttcaatctcgtgagaagccatgcgtccttccagagactcaaacctctccacagtgcggttctgggcgtagtgggtatggtactgaagatcatgcatgttctcttcgtggtcatccaggaaggacgagatgttatccagctgcagctgcaagcccatgacctggagtaccaggtcgtgcatgctctctgagttctggctgatgcgctgtgaggaggcccccagggtggcctggatgttcttgaccgcctctccagtcttggtggaggtggtgcgcaggccgctgaagagccgtgtgtagttctgccagtcggtgacaatcttctggagggtcagggtctcctcgtctgtcttccgctggatcccgtggatccactcggaagtctgccccacggtgaagttgatctggtgcactgcagccttgacatcgtagcactcctgggtgaggtccttcagagagaggtccaggccagctgtggtggcctgccagcctctcacctgggccaggaagagccccagagactggttaacctggtggatggagaaggagcaactgcccatctcctgggagatttgtctgctggtggtggagagcacctcctgggcctgtaaggtctggtccagctgcacctcctgggccagaagcagcttctgaattccctccagctcctcctgcagttttcggatctctggccccagctgcccagcttcatggcagaaagagcagttgttcagggctttcggatccaggccctggagatttttctgcattaacacaagcttcttgtcataaatagactgggtcaaggagatgtcttcggagagagagtccacttttctgaaaaccagagaggccaacacagccacggccaccaggagcagggccaggaagaggtaaagaatccgcaccgatgtgtgcaaagataggttcttctggcagcggctgcagcggggccctggccggcccttctgggtgcatgggaaggtcggcatgtcctcgtcgtcacccgccaggtcctcttctgtaacgcacaaggcatctccatcgccgccggccgacctcactttcatggtctcttcctctggggcctcaggagggccccgctgcaggcggctggagctgtagtggagccgggcggccggcggatcctccagggcgcggatcgccgtcctaggcgccgcccgcggccgtggggctccggccgggactcatgctccggcgcgcgggctgcggaggcggcgggaggagtggagggtcccgcggggtcgcagcctggggaagccccgccgggcgcctagcgccgcgccccgccgcccagagcgcgcatcccgccgccgcccgcgcttcccgctggggccccgcgaggtctgccgccgcccctc

SEQ ID NO: 12387 - RNA, 6051 nt, Homo sapiens
  source 1..6051: mol_type = other RNA
ctgggaggtcaaggctgcagtggctgtgattgtgccactgccctccagcctgggtgacagagcaagaccctgtctcaaaaaaaggacatatctttttttaaattgtattgatgactacatctttcatcataattagagacaggctcaagatacatctgtagtatgattgtgcttacatctaccccatatatgtaagttttattatgtctttattaagaagatgactgctttaggtttgttgctattttatttgagaagaataaaaaagaaaattatctggaaaatttctttaaagctaaacacgtcttggtcctttggtgtggggactgaataaaagtcagtgcttttatgtaatagatggagattctaagacttggagagtcctaagattacaggttcagctggtggccaagctaggagggagttccagtctgctatgcactgaatggcaccctttgcagtatgtgaagctgtccctacccaccaggattgccactacattgtagattgtgcacataatagctacatagtgactagtaagaataaatatgtctgaaaaaaatacatctcatcgaaaaagtaggatgaagttatttcaacaattaatgccaagagacctgaggaagcaaacataatctggtcagtttgagtttttacaagaaggctcatatttcaaatgtctttctccaataggaaataaacattaataataaggactgggaaacttcctttctcttttttggaaaagcagattatatggataactgcatatgcctcacattcttgcaaaattataaattgtttagaaaagggattaaaaacgcctgaaacccgcaagagttcaacctctaacctctggggttgttggcaccaggaagctgctaccttcctgtccactgcttcatagtcatggagacacagacccatggcattagtcagcagtttctaaatcttgacccacaataggaaagatacctcaagacaggagaaatagatggaggcaattacaaacagctactagattgatggttgacattgtcagggctccactgtatggcagattgcaatggtgttgaactccccttgctaccagtggatgttgctattggcaaccatgcagtgaagccaataaaacggcaagaaaatgagaggaaaactcaaccttagtggaagcttgtagggtttatgctataaattatgttccccttagcaatatgtagcatcaatgttcaggatagctacagtgctcacggcagcctgcagtctctgtcagaccctgggtccagttttgtcataaagcacatgctttaaaatgttgctgtagatggactggcatccatttgtctgggctatttatttatttattgttggggaggataacagatgtgggctcatctctgcctcacacagactgattttcaattcccgttcgtgatataaacatgatgtggcacattacccagaaacacctgcagtgcttcggagctgcagacacgtcacgatctcgcagaccagactctgtccctgactccacccaccctttgttccccacctgaaggaggagagacagccctgcagaagctattttcctttatagcagagtgatacagaaaactggcttaataaaatccataaatctgaacaacctcctcttacctgctctgcagaggcagtttcttcctgcattcatttccccctctactttctccagtcttccctgcagagacagctgtaaagggtagctaggaacattattttttagggctctcactccttccttctcccctttctcaaacccctccctgctcaagtgtctctcttttctgagcaattgatgacagggttctacaccttcattttttttggttggaagtgccatttttctttgtttggattgactttcaccttttttttttttttttcatttcccttaaccacctgtctcggtccctgtctttcctttactggtgttcttacgtttctttttcttcttgcttttattcccctcttagtctggtttatactttttttttttttttttttttttttttttttttttgagacggagtctcgctggtcgcccaggctggagggcagtgacgtgatctcgactcactgcaagctccgcctcgcgggttcccgccattctcttgcctcagcctccccagtagctgggactacagacgcctgccaccgcgcctggctaatttgttttgtgttttttagtagagacagggtttcaccgtgttagccaggacggtctcgatctcctgacctcgtgatccgcccgcctcggccttccaaattgctgggattacaggcgtgagccaccgcgcccggtctatacatttcttttactttgtttcttgccataaagagtctttttctctacaattacctgctctcccctcaattccattttggtatcttaattttacccattccttcttcagacatttcctgaattgtctactgtgtgccaggaaaacaatgtcgcatgtagaacatggcccctatttctttaatatctgtaaagttaatgattgataatgattaataacaataacaagggccgggtacggtggctcacgcctgtaatcccagcactttcggaggcagaggtgggtggctcacctgaggtcaggagtttgagatcagcctggcaaacatggtgaaaccctgtgtctactaaaagtacaaaaattagccaggcgtggtggcaggcacctgtaatcccagcttctcaggaggttgaggctggagaattgcttgaacccaggaagcagaggttgcagtaagccgagatcacgccattgcactccagcctgggcaacaagagtgaaaactcagtctcaaaaaacaaacaaacaaagaaacaaaaacaataacaagaaaaatggtttgtaaatttcagatttttttaagagctagaatggctctcaggtttaatctaggccagggattttcaaactcttcagagtccctgtggacccccatgtacgtaatcaaagagatgaaggtttgtaggtgctctggatgtccaaaccctgcttataattcacataggaattcagctttttgacgttttatatgttggggattcattgaaagatttatttgaacaaagagttgtaaggttaaaacatgttcgagaatcgtttcctagtgtaatctaatttgacaaataaggaaacaagcttgtagaagttaagtgacttgttcaagtcaatccagtcaataatgccaaagctaaggatagaaatctatcttctagcccaatgttctttggataacacataccatgtccacaatttctcaatatagggagcaaagcagctttctagtcattacatctacttaatacagtttattcttacctattgtaaacctggcttcctatagaatatgcgttctttgcccagactgttatttcttaacatttgaagcattgtttcttacacttaaggaaaaatccaaaattagggacccctatagtttgctttaagttggttactggtagtaatcttaaattttataccagaactcctcactaggagaactcaaggtagtcaatgcttagtctccatggctctgctctgtcctgtgaactatagtttctagatgtcacttgtggtaaatccagctacagatttccttccacccttactttaatcaaaatctatcaatccattccttctgggagaaaactttgtctgtaatgaaggttgaattttaaaactctggaaaagggtaccatagtcccagtctagaattacccatcaaacacatttgctatagtcctactatgtattcatttttagggggagaactgggattgatcagtatttataaggatagtatagtttaccttttaggtaggcaattctaaaggatccatcaataagaagctctaggattaaaaataaaatacctctatggaatacaaattaggattcttgggacagtctggcacaaaaaggcattcagggacaggaagcaaagacaggcagtgtttggcttgtaacaaacagaaaagccctatacaaaacgaagcagcgctaatgacgcttttactgttcagtgttccctcagctcagagtaagtaggccgactgtccacaggtccttggatccaaaacagtcccctacccagagccttcatttcagcccatgcgtgttcattagggaaaagtgagggtcctggggtgtgctccctgccccacctctttctttgtccttcccgttgctctctctgctgctgaccatgcttcaaggtgaaagcccaggcatgcttcccagtgcatccttgagatgttaggtctttctgagctaaaagaacaaaaggatgacattgctggactgaaaatggcccttcaggctgtagtcattttgcagctgcagctgacctggaggtttagttcctgtcttccttggctaccataacactggcaggggaggatgaggcagttgaggccagcagtcgtttttggtgtagctcttcccacttacttctgtttgtagctactgaatctagcatcggcttcagtttcacgttgaccttcaccagtgcctgatacaaaggcatgcagatgctatcaatccactccagttgcaaccgaggcagttcatccttccggttccgatcaaaaattgctgaaggagtgagtttgagctctaatctctcccgatctccttgttcgaagaactcactggttacaagttctgccacctgtctggagatctcccacggtttggtcacggctccaaggtcacaggctgtcattaacattgatcgaaatatatcacgatggtttttgatgttccaatcgtattctcctttactgacaagttcaaagaattcagttctcctctcaaagtacagcgtgaggtctgttgccaatattgactgcttcaaaagctgcataaggtcactatattccttggaggacaggttagcaaagatattgtgaccctcactttgaaggatcatcacggcgtggttgaaatggtgatgctccaaggtagcagaggttccatagagttgggccagggcagagccactcttagcttggaaggcattgttggttcccctgtggtcgaggtcatgacacaggcatcccacaatcaccgctaaaatttccacctcggtcagaatgtcttgaaacccagcagtggttaacatcgcgaacatcagctgacacacgttgaaggcatgtctccagttgtggtatagaaccatccgatagtttttcctcactgtcaaaagccacctacacagtgtctcatagtcaattttaaatttctgtaccatccccagctccatgaacatccggagagcagctgtgatcatggcatcaacgtcgagagaaaagtcatcaaaatgaatgtcatcgatggcaagttctgacaccagagggatgttggctgccttaaacttgtcaacttcagcttttgaacatgttgcatggtatgatagcacatcaagagccacagactgcttggcccaggacttcttcacttgatcatacataattgtgttgttgatgccaagtccacaaaagatgacaaaagcctcaaaaagtcgttgatctgcatcatcaaaaggtttcccatcaagtctgtttaacacttgagccactccaattatttggtggttgctattccaaatagggacacaaagaacagatcttatgtgaaaaccagatatctggtctgcctctgcatcaaagcgcggatcctggtaggcatcactgatgttcactggaaggcctgttgaagcaaccagctcagcaatgctgttatttattagccagtcggagtatgatgatttctccatgctttctttgaaactgttctcagcatcagcactgcactttggggacatcaattcaaaggatttggtaaatttcaccacctgttgagagaggcaatccacaaaaccaagccatgcatgtcaggactttaaggccctagttcagttctcaggattgtatttgcagtgagcaaacctgggagatgaagtaacatctttccacagacaaacatcaggctt

SEQ ID NO: 12388 - RNA, 6274 nt, Homo sapiens
  source 1..6274: mol_type = other RNA
ctgggaggtcaaggctgcagtggctgtgattgtgccactgccctccagcctgggtgacagagcaagaccctgtctcaaaaaaaggacatatctttttttaaattgtattgatgactacatctttcatcataattagagacaggctcaagatacatctgtagtatgattgtgcttacatctaccccatatatgtaagttttattatgtctttattaagaagatgactgctttaggtttgttgctattttatttgagaagaataaaaaagaaaattatctggaaaatttctttaaagctaaacacgtcttggtcctttggtgtggggactgaataaaagtcagtgcttttatgtaatagatggagattctaagacttggagagtcctaagattacaggttcagctggtggccaagctaggagggagttccagtctgctatgcactgaatggcaccctttgcagtatgtgaagctgtccctacccaccaggattgccactacattgtagattgtgcacataatagctacatagtgactagtaagaataaatatgtctgaaaaaaatacatctcatcgaaaaagtaggatgaagttatttcaacaattaatgccaagagacctgaggaagcaaacataatctggtcagtttgagtttttacaagaaggctcatatttcaaatgtctttctccaataggaaataaacattaataataaggactgggaaacttcctttctcttttttggaaaagcagattatatggataactgcatatgcctcacattcttgcaaaattataaattgtttagaaaagggattaaaaacgcctgaaacccgcaagagttcaacctctaacctctggggttgttggcaccaggaagctgctaccttcctgtccactgcttcatagtcatggagacacagacccatggcattagtcagcagtttctaaatcttgacccacaataggaaagatacctcaagacaggagaaatagatggaggcaattacaaacagctactagattgatggttgacattgtcagggctccactgtatggcagattgcaatggtgttgaactccccttgctaccagtggatgttgctattggcaaccatgcagtgaagccaataaaacggcaagaaaatgagaggaaaactcaaccttagtggaagcttgtagggtttatgctataaattatgttccccttagcaatatgtagcatcaatgttcaggatagctacagtgctcacggcagcctgcagtctctgtcagaccctgggtccagttttgtcataaagcacatgctttaaaatgttgctgtagatggactggcatccatttgtctgggctatttatttatttattgttggggaggataacagatgtgggctcatctctgcctcacacagactgattttcaattcccgttcgtgatataaacatgatgtggcacattacccagaaacacctgcagtgcttcggagctgcagacacgtcacgatctcgcagaccagactctgtccctgactccacccaccctttgttccccacctgaaggaggagagacagccctgcagaagctattttcctttatagcagagtgatacagaaaactggcttaataaaatccataaatctgaacaacctcctcttacctgctctgcagaggcagtttcttcctgcattcatttccccctctactttctccagtcttccctgcagagacagctgtaaagggtagctaggaacattattttttagggctctcactccttccttctcccctttctcaaacccctccctgctcaagtgtctctcttttctgagcaattgatgacagggttctacaccttcattttttttggttggaagtgccatttttctttgtttggattgactttcaccttttttttttttttttcatttcccttaaccacctgtctcggtccctgtctttcctttactggtgttcttacgtttctttttcttcttgcttttattcccctcttagtctggtttatactttttttttttttttttttttttttttttttttttgagacggagtctcgctggtcgcccaggctggagggcagtgacgtgatctcgactcactgcaagctccgcctcgcgggttcccgccattctcttgcctcagcctccccagtagctgggactacagacgcctgccaccgcgcctggctaatttgttttgtgttttttagtagagacagggtttcaccgtgttagccaggacggtctcgatctcctgacctcgtgatccgcccgcctcggccttccaaattgctgggattacaggcgtgagccaccgcgcccggtctatacatttcttttactttgtttcttgccataaagagtctttttctctacaattacctgctctcccctcaattccattttggtatcttaattttacccattccttcttcagacatttcctgaattgtctactgtgtgccaggaaaacaatgtcgcatgtagaacatggcccctatttctttaatatctgtaaagttaatgattgataatgattaataacaataacaagggccgggtacggtggctcacgcctgtaatcccagcactttcggaggcagaggtgggtggctcacctgaggtcaggagtttgagatcagcctggcaaacatggtgaaaccctgtgtctactaaaagtacaaaaattagccaggcgtggtggcaggcacctgtaatcccagcttctcaggaggttgaggctggagaattgcttgaacccaggaagcagaggttgcagtaagccgagatcacgccattgcactccagcctgggcaacaagagtgaaaactcagtctcaaaaaacaaacaaacaaagaaacaaaaacaataacaagaaaaatggtttgtaaatttcagatttttttaagagctagaatggctctcaggtttaatctaggccagggattttcaaactcttcagagtccctgtggacccccatgtacgtaatcaaagagatgaaggtttgtaggtgctctggatgtccaaaccctgcttataattcacataggaattcagctttttgacgttttatatgttggggattcattgaaagatttatttgaacaaagagttgtaaggttaaaacatgttcgagaatcgtttcctagtgtaatctaatttgacaaataaggaaacaagcttgtagaagttaagtgacttgttcaagtcaatccagtcaataatgccaaagctaaggatagaaatctatcttctagcccaatgttctttggataacacataccatgtccacaatttctcaatatagggagcaaagcagctttctagtcattacatctacttaatacagtttattcttacctattgtaaacctggcttcctatagaatatgcgttctttgcccagactgttatttcttaacatttgaagcattgtttcttacacttaaggaaaaatccaaaattagggacccctatagtttgctttaagttggttactggtagtaatcttaaattttataccagaactcctcactaggagaactcaaggtagtcaatgcttagtctccatggctctgctctgtcctgtgaactatagtttctagatgtcacttgtggtaaatccagctacagatttccttccacccttactttaatcaaaatctatcaatccattccttctgggagaaaactttgtctgtaatgaaggttgaattttaaaactctggaaaagggtaccatagtcccagtctagaattacccatcaaacacatttgctatagtcctactatgtattcatttttagggggagaactgggattgatcagtatttataaggatagtatagtttaccttttaggtaggcaattctaaaggatccatcaataagaagctctaggattaaaaataaaatacctctatggaatacaaattaggattcttgggacagtctggcacaaaaaggcattcagggacaggaagcaaagacaggcagtgtttggcttgtaacaaacagaaaagccctatacaaaacgaagcagcgctaatgacgcttttactgttcagtgttccctcagctcagagtaagtaggccgactgtccacaggtccttggatccaaaacagtcccctacccagagccttcatttcagcccatgcgtgttcattagggaaaagtgagggtcctggggtgtgctccctgccccacctctttctttgtccttcccgttgctctctctgctgctgaccatgcttcaaggtgaaagcccaggcatgcttcccagtgcatccttgagatgttaggtctttctgagctaaaagaacaaaaggatgacattgctggactgaaaatggcccttcaggctgtagtcattttgcagctgcagctgacctggaggtttagttcctgtcttccttggctaccataacactggcaggggaggatgaggcagttgaggccagcagtcgtttttggtgtagctcttcccacttacttctgtttgtagctactgaatctagcatcggcttcagtttcacgttgaccttcaccagtgcctgatacaaaggcatgcagatgctatcaatccactccagttgcaaccgaggcagttcatccttccggttccgatcaaaaattgctgaaggagtgagtttgagctctaatctctcccgatctccttgttcgaagaactcactggttacaagttctgccacctgtctggagatctcccacggtttggtcacggctccaaggtcacaggctgtcattaacattgatcgaaatatatcacgatggtttttgatgttccaatcgtattctcctttactgacaagttcaaagaattcagttctcctctcaaagtacagcgtgaggtctgttgccaatattgactgcttcaaaagctgcataaggtcactatattccttggaggacaggttagcaaagatattgtgaccctcactttgaaggatcatcacggcgtggttgaaatggtgatgctccaaggtagcagaggttccatagagttgggccagggcagagccactcttagcttggaaggcattgttggttcccctgtggtcgaggtcatgacacaggcatcccacaatcaccgctaaaatttccacctcggtcagaatgtcttgaaacccagcagtggttaacatcgcgaacatcagctgacacacgttgaaggcatgtctccagttgtggtatagaaccatccgatagtttttcctcactgtcaaaagccacctacacagtgtctcatagtcaattttaaatttctgtaccatccccagctccatgaacatccggagagcagctgtgatcatggcatcaacgtcgagagaaaagtcatcaaaatgaatgtcatcgatggcaagttctgacaccagagggatgttggctgccttaaacttgtcaacttcagcttttgaacatgttgcatggtatgatagcacatcaagagccacagactgcttggcccaggacttcttcacttgatcatacataattgtgttgttgatgccaagtccacaaaagatgacaaaagcctcaaaaagtcgttgatctgcatcatcaaaaggtttcccatcaagtctgtttaacacttgagccactccaattatttggtggttgctattccaaatagggacacaaagaacagatcttatgtgaaaaccagatatctggtctgcctctgcatcaaagcgcggatcctggtaggcatcactgatgttcactggaaggcctgttgaagcaaccagctcagcaatgctgttatttattagccagtcggagtatgatgatttctccatgctttctttgaaactgttctcagcatcagcactgcactttggggacatcaattcaaaggatttggtaaatttcaccactggtgattcgatgtcctctaggagtaaaacagaacagcgttcacatttcagcagagtttgggcccgatgcattattttcttgacaattttctccaggtcagtctgttcttcaaagaggtcattaaccacctctagcaaagctctgcttctttcatattctttccttgaggcagcaaagagctgagcgttagatatggcgattccacaaaatggaagatacatctgcataacctttctggctgttccatggcttcctattgcttacagggcctacactcaaagcccttcataatctattcccaacacacagtggacttttcttgactcatcttccagcactcttctccctctacatttcttg

SEQ ID NO: 12389 - RNA, 7555 nt, Homo sapiens
  source 1..7555: mol_type = other RNA
ctgggaggtcaaggctgcagtggctgtgattgtgccactgccctccagcctgggtgacagagcaagaccctgtctcaaaaaaaggacatatctttttttaaattgtattgatgactacatctttcatcataattagagacaggctcaagatacatctgtagtatgattgtgcttacatctaccccatatatgtaagttttattatgtctttattaagaagatgactgctttaggtttgttgctattttatttgagaagaataaaaaagaaaattatctggaaaatttctttaaagctaaacacgtcttggtcctttggtgtggggactgaataaaagtcagtgcttttatgtaatagatggagattctaagacttggagagtcctaagattacaggttcagctggtggccaagctaggagggagttccagtctgctatgcactgaatggcaccctttgcagtatgtgaagctgtccctacccaccaggattgccactacattgtagattgtgcacataatagctacatagtgactagtaagaataaatatgtctgaaaaaaatacatctcatcgaaaaagtaggatgaagttatttcaacaattaatgccaagagacctgaggaagcaaacataatctggtcagtttgagtttttacaagaaggctcatatttcaaatgtctttctccaataggaaataaacattaataataaggactgggaaacttcctttctcttttttggaaaagcagattatatggataactgcatatgcctcacattcttgcaaaattataaattgtttagaaaagggattaaaaacgcctgaaacccgcaagagttcaacctctaacctctggggttgttggcaccaggaagctgctaccttcctgtccactgcttcatagtcatggagacacagacccatggcattagtcagcagtttctaaatcttgacccacaataggaaagatacctcaagacaggagaaatagatggaggcaattacaaacagctactagattgatggttgacattgtcagggctccactgtatggcagattgcaatggtgttgaactccccttgctaccagtggatgttgctattggcaaccatgcagtgaagccaataaaacggcaagaaaatgagaggaaaactcaaccttagtggaagcttgtagggtttatgctataaattatgttccccttagcaatatgtagcatcaatgttcaggatagctacagtgctcacggcagcctgcagtctctgtcagaccctgggtccagttttgtcataaagcacatgctttaaaatgttgctgtagatggactggcatccatttgtctgggctatttatttatttattgttggggaggataacagatgtgggctcatctctgcctcacacagactgattttcaattcccgttcgtgatataaacatgatgtggcacattacccagaaacacctgcagtgcttcggagctgcagacacgtcacgatctcgcagaccagactctgtccctgactccacccaccctttgttccccacctgaaggaggagagacagccctgcagaagctattttcctttatagcagagtgatacagaaaactggcttaataaaatccataaatctgaacaacctcctcttacctgctctgcagaggcagtttcttcctgcattcatttccccctctactttctccagtcttccctgcagagacagctgtaaagggtagctaggaacattattttttagggctctcactccttccttctcccctttctcaaacccctccctgctcaagtgtctctcttttctgagcaattgatgacagggttctacaccttcattttttttggttggaagtgccatttttctttgtttggattgactttcaccttttttttttttttttcatttcccttaaccacctgtctcggtccctgtctttcctttactggtgttcttacgtttctttttcttcttgcttttattcccctcttagtctggtttatactttttttttttttttttttttttttttttttttttgagacggagtctcgctggtcgcccaggctggagggcagtgacgtgatctcgactcactgcaagctccgcctcgcgggttcccgccattctcttgcctcagcctccccagtagctgggactacagacgcctgccaccgcgcctggctaatttgttttgtgttttttagtagagacagggtttcaccgtgttagccaggacggtctcgatctcctgacctcgtgatccgcccgcctcggccttccaaattgctgggattacaggcgtgagccaccgcgcccggtctatacatttcttttactttgtttcttgccataaagagtctttttctctacaattacctgctctcccctcaattccattttggtatcttaattttacccattccttcttcagacatttcctgaattgtctactgtgtgccaggaaaacaatgtcgcatgtagaacatggcccctatttctttaatatctgtaaagttaatgattgataatgattaataacaataacaagggccgggtacggtggctcacgcctgtaatcccagcactttcggaggcagaggtgggtggctcacctgaggtcaggagtttgagatcagcctggcaaacatggtgaaaccctgtgtctactaaaagtacaaaaattagccaggcgtggtggcaggcacctgtaatcccagcttctcaggaggttgaggctggagaattgcttgaacccaggaagcagaggttgcagtaagccgagatcacgccattgcactccagcctgggcaacaagagtgaaaactcagtctcaaaaaacaaacaaacaaagaaacaaaaacaataacaagaaaaatggtttgtaaatttcagatttttttaagagctagaatggctctcaggtttaatctaggccagggattttcaaactcttcagagtccctgtggacccccatgtacgtaatcaaagagatgaaggtttgtaggtgctctggatgtccaaaccctgcttataattcacataggaattcagctttttgacgttttatatgttggggattcattgaaagatttatttgaacaaagagttgtaaggttaaaacatgttcgagaatcgtttcctagtgtaatctaatttgacaaataaggaaacaagcttgtagaagttaagtgacttgttcaagtcaatccagtcaataatgccaaagctaaggatagaaatctatcttctagcccaatgttctttggataacacataccatgtccacaatttctcaatatagggagcaaagcagctttctagtcattacatctacttaatacagtttattcttacctattgtaaacctggcttcctatagaatatgcgttctttgcccagactgttatttcttaacatttgaagcattgtttcttacacttaaggaaaaatccaaaattagggacccctatagtttgctttaagttggttactggtagtaatcttaaattttataccagaactcctcactaggagaactcaaggtagtcaatgcttagtctccatggctctgctctgtcctgtgaactatagtttctagatgtcacttgtggtaaatccagctacagatttccttccacccttactttaatcaaaatctatcaatccattccttctgggagaaaactttgtctgtaatgaaggttgaattttaaaactctggaaaagggtaccatagtcccagtctagaattacccatcaaacacatttgctatagtcctactatgtattcatttttagggggagaactgggattgatcagtatttataaggatagtatagtttaccttttaggtaggcaattctaaaggatccatcaataagaagctctaggattaaaaataaaatacctctatggaatacaaattaggattcttgggacagtctggcacaaaaaggcattcagggacaggaagcaaagacaggcagtgtttggcttgtaacaaacagaaaagccctatacaaaacgaagcagcgctaatgacgcttttactgttcagtgttccctcagctcagagtaagtaggccgactgtccacaggtccttggatccaaaacagtcccctacccagagccttcatttcagcccatgcgtgttcattagggaaaagtgagggtcctggggtgtgctccctgccccacctctttctttgtccttcccgttgctctctctgctgctgaccatgcttcaaggtgaaagcccaggcatgcttcccagtgcatccttgagatgttaggtctttctgagctaaaagaacaaaaggatgacattgctggactgaaaatggcccttcaggctgtagtcattttgcagctgcagctgacctggaggtttagttcctgtcttccttggctaccataacactggcaggggaggatgaggcagttgaggccagcagtcgtttttggtgtagctcttcccacttacttctgtttgtagctactgaatctagcatcggcttcagtttcacgttgaccttcaccagtgcctgatacaaaggcatgcagatgctatcaatccactccagttgcaaccgaggcagttcatccttccggttccgatcaaaaattgctgaaggagtgagtttgagctctaatctctcccgatctccttgttcgaagaactcactggttacaagttctgccacctgtctggagatctcccacggtttggtcacggctccaaggtcacaggctgtcattaacattgatcgaaatatatcacgatggtttttgatgttccaatcgtattctcctttactgacaagttcaaagaattcagttctcctctcaaagtacagcgtgaggtctgttgccaatattgactgcttcaaaagctgcataaggtcactatattccttggaggacaggttagcaaagatattgtgaccctcactttgaaggatcatcacggcgtggttgaaatggtgatgctccaaggtagcagaggttccatagagttgggccagggcagagccactcttagcttggaaggcattgttggttcccctgtggtcgaggtcatgacacaggcatcccacaatcaccgctaaaatttccacctcggtcagaatgtcttgaaacccagcagtggttaacatcgcgaacatcagctgacacacgttgaaggcatgtctccagttgtggtatagaaccatccgatagtttttcctcactgtcaaaagccacctacacagtgtctcatagtcaattttaaatttctgtaccatccccagctccatgaacatccggagagcagctgtgatcatggcatcaacgtcgagagaaaagtcatcaaaatgaatgtcatcgatggcaagttctgacaccagagggatgttggctgccttaaacttgtcaacttcagcttttgaacatgttgcatggtatgatagcacatcaagagccacagactgcttggcccaggacttcttcacttgatcatacataattgtgttgttgatgccaagtccacaaaagatgacaaaagcctcaaaaagtcgttgatctgcatcatcaaaaggtttcccatcaagtctgtttaacacttgagccactccaattatttggtggttgctattccaaatagggacacaaagaacagatcttatgtgaaaaccagatatctggtctgcctctgcatcaaagcgcggatcctggtaggcatcactgatgttcactggaaggcctgttgaagcaaccagctcagcaatgctgttatttattagccagtcggagtatgatgatttctccatgctttctttgaaactgttctcagcatcagcactgcactttggggacatcaattcaaaggatttggtaaatttcaccactggtgattcgatgtcctctaggagtaaaacagaacagcgttcacatttcagcagagtttgggcccgatgcattattttcttgacaattttctccaggtcagtctgttcttcaaagaggtcattaaccacctctagcaaagctctgcttctttcatattctttccttgaggcagcaaagagctgagcgttagatatggcgattccacaaaatggaagatacatctgcataactttttcatcatcttcagtaaatggagctccttcaggaatcttatttatcgcttgggccacaccaataatctcaccatcactgcttcggataggcatgcacaataatgattttgtcttgtatccagttagcttgtcgatttcatcattgaatcgtcgatcctggtaggcatcaggaatgttgaccgtttctccatgctccccgacatagccaatgatacctttgccccaggggacctgcacctcatttgagttctctgtgctgctgcaaggcagcagaggtgttcctgcatgcacatcaaagaatttggagaccaaggtcttcttgccagcagctgccccttccaccaggaaaagagagcagcggtcagcatccaccataaggcagacaaagatgagaatcttgtagctcaggctggtgaggtcaaggtcattggagatatctttgaccaattccagaaagaactgacgctcattatgctttttcagatggcacttgtagtcgatggctgtagggggataccgaggcagattcactctcgattccagcagcgcactgagaatatgggctgtggtggggggcagggagcttgccttccggagaagtgccctccgtcgtacactactcaggggttcctgagcccgggaggtcacctgttcatcgtaggtcctgttcacgtggatggccttggagcgggcaaaactcttccttagctctttctgagaagctctccgctgcaggttcccatcgcccctgctgccaccggcccagctgggactcaagggaaccccaccacagtccccgccaccgggaaggggctggctgtgggcagagccatttggtccagtgccaccaccaacgctgctgccacctctgcaggtgctgtgagccaagctgctggtaccagccaaagagggccttggacctaaagccccctgaccctgactgtgcctctgcagccacttttcaaccatctcctgcttccccttccgcatcaagtaatcttcaaacaactctgggtgcctgtccaggaaagtttccacctccccaaagtccaggcgggaggctgccatggtcccagacagctttccttgcctgtttacacgtgaaccaaatgttttcctgccccgaggcctctagctgttcctgcacatgttcacccccaccagtattcccagttcagcgccacctcccctggagattattcccagcagtggaatctgggagatgccccttccttctctggctcagagtggctggcgccgaccccaccccgtggtcctgctactcctgctccgcacaggtgcccagcactgagctgccgccgctgccccggctcctgttccggaaacccgagctatcgctgctcctgttctggctgccgccgctgctgctggaactgctgctgtaacc

SEQ ID NO: 12390 - RNA, 6564 nt, Homo sapiens
  source 1..6564: mol_type = other RNA
ctgggaggtcaaggctgcagtggctgtgattgtgccactgccctccagcctgggtgacagagcaagaccctgtctcaaaaaaaggacatatctttttttaaattgtattgatgactacatctttcatcataattagagacaggctcaagatacatctgtagtatgattgtgcttacatctaccccatatatgtaagttttattatgtctttattaagaagatgactgctttaggtttgttgctattttatttgagaagaataaaaaagaaaattatctggaaaatttctttaaagctaaacacgtcttggtcctttggtgtggggactgaataaaagtcagtgcttttatgtaatagatggagattctaagacttggagagtcctaagattacaggttcagctggtggccaagctaggagggagttccagtctgctatgcactgaatggcaccctttgcagtatgtgaagctgtccctacccaccaggattgccactacattgtagattgtgcacataatagctacatagtgactagtaagaataaatatgtctgaaaaaaatacatctcatcgaaaaagtaggatgaagttatttcaacaattaatgccaagagacctgaggaagcaaacataatctggtcagtttgagtttttacaagaaggctcatatttcaaatgtctttctccaataggaaataaacattaataataaggactgggaaacttcctttctcttttttggaaaagcagattatatggataactgcatatgcctcacattcttgcaaaattataaattgtttagaaaagggattaaaaacgcctgaaacccgcaagagttcaacctctaacctctggggttgttggcaccaggaagctgctaccttcctgtccactgcttcatagtcatggagacacagacccatggcattagtcagcagtttctaaatcttgacccacaataggaaagatacctcaagacaggagaaatagatggaggcaattacaaacagctactagattgatggttgacattgtcagggctccactgtatggcagattgcaatggtgttgaactccccttgctaccagtggatgttgctattggcaaccatgcagtgaagccaataaaacggcaagaaaatgagaggaaaactcaaccttagtggaagcttgtagggtttatgctataaattatgttccccttagcaatatgtagcatcaatgttcaggatagctacagtgctcacggcagcctgcagtctctgtcagaccctgggtccagttttgtcataaagcacatgctttaaaatgttgctgtagatggactggcatccatttgtctgggctatttatttatttattgttggggaggataacagatgtgggctcatctctgcctcacacagactgattttcaattcccgttcgtgatataaacatgatgtggcacattacccagaaacacctgcagtgcttcggagctgcagacacgtcacgatctcgcagaccagactctgtccctgactccacccaccctttgttccccacctgaaggaggagagacagccctgcagaagctattttcctttatagcagagtgatacagaaaactggcttaataaaatccataaatctgaacaacctcctcttacctgctctgcagaggcagtttcttcctgcattcatttccccctctactttctccagtcttccctgcagagacagctgtaaagggtagctaggaacattattttttagggctctcactccttccttctcccctttctcaaacccctccctgctcaagtgtctctcttttctgagcaattgatgacagggttctacaccttcattttttttggttggaagtgccatttttctttgtttggattgactttcaccttttttttttttttttcatttcccttaaccacctgtctcggtccctgtctttcctttactggtgttcttacgtttctttttcttcttgcttttattcccctcttagtctggtttatactttttttttttttttttttttttttttttttttttgagacggagtctcgctggtcgcccaggctggagggcagtgacgtgatctcgactcactgcaagctccgcctcgcgggttcccgccattctcttgcctcagcctccccagtagctgggactacagacgcctgccaccgcgcctggctaatttgttttgtgttttttagtagagacagggtttcaccgtgttagccaggacggtctcgatctcctgacctcgtgatccgcccgcctcggccttccaaattgctgggattacaggcgtgagccaccgcgcccggtctatacatttcttttactttgtttcttgccataaagagtctttttctctacaattacctgctctcccctcaattccattttggtatcttaattttacccattccttcttcagacatttcctgaattgtctactgtgtgccaggaaaacaatgtcgcatgtagaacatggcccctatttctttaatatctgtaaagttaatgattgataatgattaataacaataacaagggccgggtacggtggctcacgcctgtaatcccagcactttcggaggcagaggtgggtggctcacctgaggtcaggagtttgagatcagcctggcaaacatggtgaaaccctgtgtctactaaaagtacaaaaattagccaggcgtggtggcaggcacctgtaatcccagcttctcaggaggttgaggctggagaattgcttgaacccaggaagcagaggttgcagtaagccgagatcacgccattgcactccagcctgggcaacaagagtgaaaactcagtctcaaaaaacaaacaaacaaagaaacaaaaacaataacaagaaaaatggtttgtaaatttcagatttttttaagagctagaatggctctcaggtttaatctaggccagggattttcaaactcttcagagtccctgtggacccccatgtacgtaatcaaagagatgaaggtttgtaggtgctctggatgtccaaaccctgcttataattcacataggaattcagctttttgacgttttatatgttggggattcattgaaagatttatttgaacaaagagttgtaaggttaaaacatgttcgagaatcgtttcctagtgtaatctaatttgacaaataaggaaacaagcttgtagaagttaagtgacttgttcaagtcaatccagtcaataatgccaaagctaaggatagaaatctatcttctagcccaatgttctttggataacacataccatgtccacaatttctcaatatagggagcaaagcagctttctagtcattacatctacttaatacagtttattcttacctattgtaaacctggcttcctatagaatatgcgttctttgcccagactgttatttcttaacatttgaagcattgtttcttacacttaaggaaaaatccaaaattagggacccctatagtttgctttaagttggttactggtagtaatcttaaattttataccagaactcctcactaggagaactcaaggtagtcaatgcttagtctccatggctctgctctgtcctgtgaactatagtttctagatgtcacttgtggtaaatccagctacagatttccttccacccttactttaatcaaaatctatcaatccattccttctgggagaaaactttgtctgtaatgaaggttgaattttaaaactctggaaaagggtaccatagtcccagtctagaattacccatcaaacacatttgctatagtcctactatgtattcatttttagggggagaactgggattgatcagtatttataaggatagtatagtttaccttttaggtaggcaattctaaaggatccatcaataagaagctctaggattaaaaataaaatacctctatggaatacaaattaggattcttgggacagtctggcacaaaaaggcattcagggacaggaagcaaagacaggcagtgtttggcttgtaacaaacagaaaagccctatacaaaacgaagcagcgctaatgacgcttttactgttcagtgttccctcagctcagagtaagtaggccgactgtccacaggtccttggatccaaaacagtcccctacccagagccttcatttcagcccatgcgtgttcattagggaaaagtgagggtcctggggtgtgctccctgccccacctctttctttgtccttcccgttgctctctctgctgctgaccatgcttcaaggtgaaagcccaggcatgcttcccagtgcatccttgagatgttaggtctttctgagctaaaagaacaaaaggatgacattgctggactgaaaatggcccttcaggctgtagtcattttgcagctgcagctgacctggaggtttagttcctgtcttccttggctaccataacactggcaggggaggatgaggcagttgaggccagcagtcgtttttggtgtagctcttcccacttacttctgtttgtagctactgaatctagcatcggcttcagtttcacgttgaccttcaccagtgcctgatacaaaggcatgcagatgctatcaatccactccagttgcaaccgaggcagttcatccttccggttccgatcaaaaattgctgaaggagtgagtttgagctctaatctctcccgatctccttgttcgaagaactcactggttacaagttctgccacctgtctggagatctcccacggtttggtcacggctccaaggtcacaggctgtcattaacattgatcgaaatatatcacgatggtttttgatgttccaatcgtattctcctttactgacaagttcaaagaattcagttctcctctcaaagtacagcgtgaggtctgttgccaatattgactgcttcaaaagctgcataaggtcactatattccttggaggacaggttagcaaagatattgtgaccctcactttgaaggatcatcacggcgtggttgaaatggtgatgctccaaggtagcagaggttccatagagttgggccagggcagagccactcttagcttggaaggcattgttggttcccctgtggtcgaggtcatgacacaggcatcccacaatcaccgctaaaatttccacctcggtcagaatgtcttgaaacccagcagtggttaacatcgcgaacatcagctgacacacgttgaaggcatgtctccagttgtggtatagaaccatccgatagtttttcctcactgtcaaaagccacctacacagtgtctcatagtcaattttaaatttctgtaccatccccagctccatgaacatccggagagcagctgtgatcatggcatcaacgtcgagagaaaagtcatcaaaatgaatgtcatcgatggcaagttctgacaccagagggatgttggctgccttaaacttgtcaacttcagcttttgaacatgttgcatggtatgatagcacatcaagagccacagactgcttggcccaggacttcttcacttgatcatacataattgtgttgttgatgccaagtccacaaaagatgacaaaagcctcaaaaagtcgttgatctgcatcatcaaaaggtttcccatcaagtctgtttaacacttgagccactccaattatttggtggttgctattccaaatagggacacaaagaacagatcttatgtgaaaaccagatatctggtctgcctctgcatcaaagcgcggatcctggtaggcatcactgatgttcactggaaggcctgttgaagcaaccagctcagcaatgctgttatttattagccagtcggagtatgatgatttctccatgctttctttgaaactgttctcagcatcagcactgcactttggggacatcaattcaaaggatttggtaaatttcaccactggtgattcgatgtcctctaggagtaaaacagaacagcgttcacatttcagcagagtttgggcccgatgcattattttcttgacaattttctccaggtcagtctgttcttcaaagaggtcattaaccacctctagcaaagctctgcttctttcatattctttccttgaggcagcaaagagctgagcgttagatatggcgattccacaaaatggaagatacatctgcataactttttcatcatcttcagtaaatggagctccttcaggaatcttatttatcgcttgggccacaccaataatctcaccatcactgcttcggataggcatgcacaataatgattttgtcttgtatccagttagcttgtcgatttcatcattgaatcgtcgatcctttgtttttgtttgcctctgtataagaaaatcctggtgcttttcctgtttttcagccaaagaggccccagagatttggaccagtcttgtgattttcacctttttccactgtgtggcactgagcacatttctgaataaaggtcttcttgcctgcttcagcatctcccatgttgctctggaacagccacctggccagagtccacgcctcaacttcgaggctggcgatccagaaagagcacctcacgccctgggctgcaagcg

SEQ ID NO: 12391 - RNA, 20139 nt, Homo sapiens
  source 1..20139: mol_type = other RNA
ctgggaggtcaaggctgcagtgggccatgatcatgccactgcactccaacctgggtgacagagcaagaccctgtctcagaaaaaaaaaaaaaaaaaaaaaaaaggcattaaaaaagcaataaagcagaaagaaagcatttgccattttattaaactgtgagagaaggtgacaatacagtgttctttcctcatattttgtacctacacgatagcatttattagactttttgtgtgtctccccactagactgtgtttcttgaggggtaggaccatggcttatttatatcttccattgttcttataatagaattttgaacataaccccttgttcattaacatttgttgattaaattgaatgcacagtgagaaaaaggcaaattgttttaacagttaaataattttttaaaaaaggataaacatatagattggctagaggacaaaccttagaatggtccggaggcagacttacaagagaattacttaaacatctctcgattcaaacctacaggtctggatgaatactcaaaatataagtatatattttggggtataggtgaacctgcggggcatatttatggcaagaccaagcaaaagaagaaaatatagtcccttcactttgagtagtttatgatgacctagggccctaggtgacagggatagtaactatcattttttgggaaacgtggaaatgcaaaaaaaaaaaaaattgcctgataagatatatagacacacacacacacacacacacagacacacacacagacacacacagagagagagagatattaattcccaagtttgaatttctctgggaaatggccacaaagaaatgcctgaactgtttgctagcaacattcatggttttataaagaatatagcagtgatgtcctgctagaatatctgtcttgatcataatgagactgtgagaacctatcaagtgcaagatacccgttgcttagtcaaacgattctacaagtatggctgaagatttatatcccaaaactggctatcaaagatggctggtttaaaacaatcaagacagtatagacaaatattacagggcaagaatagtttggatgatgatatcctagagaaaaaatcacttttagagaatgggacttgttcactatctaacaactttctcttttacagattctagcttaatgatcatcaataaaagtgaagtcttgaatatgatggatattcacttatttgtcagggaggtgacacagttggacaagcagcacccttggagtcggggttggggaggagtgcgtgagatgtttcaaaaggatctcagtgcattttaagtgacagcttctcctgctctcttctcttcccacagctgctgggggtcctgcaccccaacccagcctagatgatatttccatttgttgtacctaaaagcagagctttttacatctttacatctttacctcatgacagaactaaaaaaatgatgtttgttctacagtatggcacggagatgggtaaaaaagtgaaaagaataagccacaagcccccgtgctttgaggagatgatcatagcctgctcctggggaactatgctagtggctggatagcaagcactgacctagaggttgctcctaggaataaaaaattaagattatccatagaagacaaagaaaaaaatacttcgctaatagtggataccaaaaatctgaggtagtgcaaaagaaaagaaaggaaaaaagaaataaaaagcgcaactggaatacatacatacaaactttcaagacgttttctcttatactcttcagtaaaattctatgtaattttcattctagtatttaaatagttctggattttacaactaaacctatcattaaaaggttatggaaaatagaaggaataaaaaagatgaaatagaacatcaggcaaatcaaaaactcaaaagctgtatccaaaacaatggtggacacctgccgtatttgctttaaaatgggtggcactgttgtgtacaatttaaatttgttaaggagatatttaacttctctgaaaagagaggaagaacacttggtaaacaaacccaaaatggtgcactaaaattggcaggcttgaggtcagaaagaacttacaaaatattaacccccaaagaaggttaaattgaatttgctaagaaagagtattctgtattagtatctggtgatcatgtggctagaaggaaattgttttttttggaggaaaacaccagaggatataaatggcttcacataaactttgggaaagaacaccttgtcttccctctacctttgctccgggttggaagaaaaaaagattaaatggttggcaggggaacacctgaaacccatataagtagggctttgatggaattagcaaagaagaagctcagaccaggaggctggctaagctgtgagggtgaggatataattagcttagaggaagtaaacaaaaacatttggcctttttagcaatgatccagccatcagaggccctggaatttcaaatgactaagaagaaccaaaatagcttgaggacacatgtcaccaaggccgccaggggttctctgccttcagcacccagatattcccactgaaaggagagaggctggggagattgcaaactaccttgggaatccaatgatcactttgtgagagacattttgaaatacatttcgaaatacatttcttattcacttcataataaaataaaatctgattgtcatattatgctgattactcatacacataaataaaatgaaaaattaggcgtttattgtagatgcctagttattgccagatggaaataaagctatacccagatgcacacatattcagattggactagttttagaattacataaagaaggctaggcaaacttaaccacagttcctgatgtttaagttttggaaagttaactttaaaaataaattttgagtaacttgagacaaatctattcccacatacttggaatgggcatacctgaaggaagtgtggctaaaataatgggagataggagcaaaatatttggaaaacacaagttagagaagaactattaaactggtgggtataataattaaactgaacaattaaggaacatcaaaactttaaacaatcaagcctcactgagaaagtggtttctgtctcattaggttttgggtgattgatacaatctgagaggtttagtaaaaaaacatataaactgcctaaaataagctcaaagctcttgtttttttcttaaattgtgtaaatttagagcattgtttcaaattttctcaaaggagaaaggaaaggggtgttgttagcaattgtatcagcacaaggggcataaaaacagactgtgtaaggccatcccagcactttgggaggccgaggcggtcggatcgatagagcccaggtgttcaagaccagcctgggcaacatggagaaaacctgtctttactaaaaatacaaaaattagccgggcgtggtggtgcatgcctgtagtcccagctactcgggaggctgaggcaggaaaatcgtttgaacccaggaggtggaggttgcagtgagccgagatcgcgccactgcactccagcctgggcgacagagcgacactgtctcaatacaaacaaacaaaaaacacccacgacaacaacaaaaatcggactgtgctcccccaagccagagaattgccaaggctgggatttaaaatgtagatatgaggtctccatctagtggtggctcttctgaactgcagacacatgtttctttaaaagagtatgcggatgtgtacaactaaatatgaggatagtatttgtcagagttgaacgcagtaatttaaactagaggattttattgagatgaaacacaatttgttgctttataagggtgggttacagagggaaatgttcaccccttcgctccaggaatttaagaatagcatgaatccttccctgaagatagacaaatgaaccagatcctctcaaggtccctttctgtcttatgataggacaataattttgctcctttctccacagagcttttacctgtagccacactgtctgacattagtctttatttaagaaaagtacggccgggcgcggtgtctcacgcctgtaatccccgtactttgggagtccgaggcaggtggatcacgaggtcaggagttcaagaccaacctggccaagaaggtgaaactccgtctctactaaaaatacaaaaaattagccgggtgcagtggcaggcgcctgtaatcccagctactcgggaggctgaggcaggagaatcgcttgaactcggagggcggaggttgcagtaagctgagatcgtgccactgcactccagcctccagcctgatgacagagtgagactccgtctcaaaaaaaaaaaaaaaaaaaaaaaaaagaaaagaaaagaaaagaaaaaagaaaagtactctggtaatttttaaaaatgagataacttttttccttgttctgagaagttgtatgactaaagcattacctatgacgttagacaaaaatagtttctagaaatgaatagcaattaaactaaatatatttctaatatgcaccttatttttcactgtaaattcttcttttgacatctggaagagcaggagggaaggcagaaaccaagaagagctgaacgattactcctctggccaagagagagcagagagagaggaagggaattcagggctgtctgaagaaggggcatggtcaccagaacgaagagactggaggatatgcctgaatctgatttcttttatccagttcctctctgattctctgtatcagtcctctattgcccttcttttgtctttctcattctttcttccttaataacttattaattcccctctttcccagccctagtctgttcttgttccttactcactcattattctcattattctaaaatgctcttacttaaaaatatttcattaaagtactcttactattctaaaatattcttactatcctaagataatgtcactctctcaattaatatttcacttttccagttcatttttcatttatttttgttcaaagagacattggcattcttttacccatgtaaatgtatagacactgggctataagataccaaagagtaggcccctggagagtttgaggcatcatgctatcaaagacagcaatggtggctgtttccttcaagatatactatgactttatctaaatctttctaaatcaaaaattttatgagaagaagacataattaacttgatagttatcaagttctctttatacaaagaaattaaaaagcagaggtagaataagagtaattaatattaatagtataagtaaaagagtcaatgacaaaacatttaatgtttcggaatatttcactcaattctggagttacttagctatgaaacccaaatagaaagacatgggaaatagttttgtgagaaagctaggacagaaatgttttacttgaaaggaaattaaggtcccatgaggtaataaagggattgtggttaggagcttaccaacctgggggtcttagatatcattagattcccagttagatatcatttttgttttaaggggctggattccattttttgtcccttcaggggaaggatctaatgaagccaaagatcatggcagtataaatagcatgctttctttctactttgagatcaacaggccagattctatctctataaaagtttgggaggggtaacatggttttgtcaaggtaaccctgattttttttctgtgctctatctaaatagttaatcatatcaattatatagcttttacagtggcttgataattttggctgaactatatgacatcttcactttagggatatagggggtgggatctattcatgaaatgatgccaaaatgcagtgtgtaaacattgtcatgctcaactgtggccaacagcctgtagacagactattcttttatctacttaaaggacgggcagcatttggcagcagtttgattaaaatttagagctaaataggtaggtggagacccctttctctcaactacacttccgtagcctcgtctctctcatgacatcttttattcttccctccacatccaaattgtaaaaattgcttaggtaacgtaatctagtgacaatgtgcatgacttcttctcaaagagaaaggaaacccaatcaaatcaaaaggatagatatggtgtgctccaattaaataaaagccacttcttaaactttttgaatggtgttactttttggatagtgttaaggtccttagaacacacaaaaggaaaattaaatgtaactgctgaaacacagcagaaaagaccaaaaatgtcttagaaaaaatgctgaagagaggaggaagactgatttaaaaaggagaaattttttttaactgggaattttgagtcaactgagaagatgaaaggttggtagtttaaggttacacaaactgaagatcaatttgctgtttagttcaatatttataaagtgcactatgtgccaggcctgtcatccacttaataattacacaaatatttattgagaacctatactatgtttctgacactatgacaggcattaaggatatatggtaaacaaaacatctggtcattttacctctcctgaggctcttctgtctagaagtcctttgttaagtattgtctgatcctctctctcaaaaagcttaaagttcataggaaaaacaaacaccaaatagctatgatctcaggcagaatgggaaagatactaaaaaacataagaaaaaattaatatggtagtgctgagtacagaaatttttttccatgaagactagggagggtttcatggttctagtgctgtttgagctgggctctgaaggctgcatatgattttaataatttagaaagggaatagggagaggaaggcattccagtagagggatagtgtgggcaaaagctgaaatataaaacacagcgaatacttggaaaagtaaggatttatatgtgtctaaaacactgagtatgcatagggtgaagaaaagaaaacaatttccagattcagaggatcagaactccttagaagaatagatgttgatgatacatggtatgtgtgatccaatctcatgcaaacagtattttcaggggatcacttgagcagcgtgtagtgaaaatgttctccacccaaaaagtgaagtaaataaacatgaaatgcagccagctgaatgattgttcaactccttgcatttcggagtgggtcattctaacattggacagcatggattcccacgctccctgacagtggtcataggagggactttttggggccgctgaacctagaagactcttttcaagcaacccccccacactttttaaagtgttgaattccatctccttctcccgtaacgtcaggggcatacagactcagtgctggaccaagttgaggaacacctttcttcatttcctttcctctttagaacaaattggcaaaattctcgctcctcttccagagattcaagagattctggttgctatttatcttgtctagcaaggcattcacacttgccacgtttagcctatcaaatgttgccctaaatcctggcaaatattcatctagctcacacttttcgtgacacttttttttttttttttaagatggagtctcactctgtcacccaggctggagagctgtggcgccatctcagctcactgcaacctccgcctgctgggttgaagcaattctcctgcctcagcctccccagtaactaggattacaggtgcgcgccacaatgcccggctaatttttcatatttttagtagagatgaggtttcagcatgttggtcaggctggtatccaattcctgacctcaagtgatccacctgcctcggcctccctaagtgctgggattacaggcataagtcaccgcacccggcttcgtgacactctttatgtgagctgtgtgaaggtcacaagaaccagcagaagacctatctgtagctccaaatggaaaaaaccatgctcaaactgaaacagatttgactagataaagactcgatttccttttgcaataggatggttgagggcaggaataaagggactcaccacattgccttgtactgtctttgatgtggaacttctctcatctttcctctggactgtgagattctgtgctgaggggaccacattacatccctcatagtacctgatatgtagttgatgcccaacaaatatttattttaatatttataatcataatatttaatgtttttgttatattcttcaatgaaatgtctccaaatgttttcagtttatgaataatatactttaggcctcagagattcagctacagtaaatgttttcctgtggaggaagtacaagagtttgctatgaaaataaagttccctgtactaagatactttactctggatgtaaagatacttggctatttgttaggctgcttattcaacctgttattttaaagaaggaaaaaaaataagcacaaacaatacacttgtgcaacagtgataaaaaaatacactttcaaaactagagaaagattgggtgattcatttaactttctttcaacaccaatttctacacccagtgaaatctatgctagcttaaagaatgaaaaaatgctgggcacagtggctcacgcctgtaatcccagcactttgggaggtcgaggcaggtggatcttttgaggccaggtgttcgagaccagcctggccaacacggtgaaaccctgtccctactaaaaatacaaaaattagcccagtgtggtggcacgcacctgtaatcccagctactcaggaggctgagacatgagaattgcctgaactcgggaggtggaagttacagtgagccaagatagcgctactgcactccagcctgggtgacacagcaagactctgtctcaagaaaaaaaaagaaagaaaagaaaaagtcacataaaagtctttttttcaaaaaaggagaagagaaaattatgccaggtttcaaaatctcacctgtggaaatttgacccagaccttgtctttgggtaggactacatagtggttccaaccgtagactaataagagtcatggaatgtttacataaatgctgcgtgaatttcacaaccttccaccttttgaggtgctgccataacaaaattaggcacaaaaggggtgttttgcagacaatttgtggaagtattgacagagctgcagaggtatccttctcatttctgcatgccttaatccaggcccatttcttacattgcttagtgctcagtgtgttgttacaaagagcatgagctcagaacccaactgggaagactctaccagctgaagaaatgcctctgaagttaaccagtaaattttctcctctctcaggtcttttctccttacttcccatagaactgttcttagggaaggttgacataatcacatggttaaaatcccaagggactcaatattcctatactttaactgtatgtttttaaataaaaacttagagtagacttgccccctcggtttttcaaaaatctctgaattctccaaagtagaagctgtgcaatttatatccttaccagggagtgtttccaaaccattctcttgcaggcagtgttgaaagtaaggaagattggaacctgtctcagtaagaagctgagaggcttagagaaagttcctcaacacagcaaaacccaacattttaaaaacagaagcagaaacagttttataaaggcattgccacccccaccattgcacacaggctttgtttgttgttgtcagtaacattataagcactccatctttgggccttagttaatgctactactccaggttcctgcgttacccaagaaagttcctcccaaattgggagctgtaaccatctgttgatactcaaggctctccgaacagctatcactctaagagggtctcttatctgtgtttcagcaggatagaagcagacatccactgcctttggaaaaacatggggagttggagggacggatctatagcagcaactgcagcaatgaagacaggtcagttttacacgctagaaacagaaatgcccccagaaggttcaggatatgactggaaaacttgattgcatctaccttagtttgtacaagtggtgcatcttggaaaatagatttcctgaacagtttagatcaaaatggagctgacactcaggatctcctgtaatagtgacccacatgctttctatacatagcgcacatctatttgtccacagcccacattctgttttcttgctataatgtattctttgggtatggtgttggtgggtgatgggaaatattctgagccaaggcaagatgcttttcttaacagaaggtggttgtattgctaaggaaaaatgttcatgcaagtgatcaccaacctggagatgccccccaagtcccagatgatcaggtagctacaagtgtgaagagaggacacattaccaacccagagtttgaacatttagttaagctcagtaagatttagcatttctgtgaaaggaactacagtggaacttcaaccccgcttttctttatactagataaaggacccatcttcttaacctattggatttcattatttgcataactttttattgacccagtgtgccaataaacttgctgtttggtcggcatatcacaaattagtcaaatatgttgtttgatcgaatttatcaaagactttgagtggtagtcctatttcagtatggcttttgacctggttatgttgtattcttgcctcttgatgagaatgtattcatcagacatatttgatcggtgtgctaatgaggggtagaaattggttagggacagcgttaagactgtccttaacagttagtaaacatactaaacggaaagacaaggtggcaagcacactacattttccaaagctttacactggaaagcttaaatattaatagatattaaatatatattaaatagattttatgattaaaaataaaatggtttttttggtttctttcatctaaccattttgacaaattcagatacttttcacttaatatttgaatatataaatctaatttcttccatgttttctcccctctgaatcttctctttttttttttttttttttttgagacggagtctcgctctgtcgcccaggctggagtgcagtggcgggatctcggctcactgcaagctccgcctcctgggttcacgccattctcctgcctcagcctcccaagtagctgggactacaggcgcccgccactacgcccggctaattttttgtatttttagtagagacggggtttcaccgttttagctgggatggtctcgatctcctgacctcgtgatccgcccgcctcggcctcccaaagtgctgggattacaggcgtgagccaccgcgcccggccctctctctttagctcaccagttgaaagatatgtcagtcctatttttaaataagtaattacattagtgatatgtgtgcaatcatctttaagattaagagcaaattaacattggcttgtcagtctctcctcaaagctgttttccatctcaaaggtcgtgatccaaggtaaggtccagaaacaactgagattgttttacatctatgtactaggttggaacaaaagtaattgtggtttttgcctgcacttttaatggtaaaaaccgcaattactttttcagcaacctaataattacaattctaagtaatggagatacatatcttttataggcttcaatgagcaatacattagcataatgttttatttcatactgactttgaatattccttgtcaaaaatgcacttatactttggagttactatgtatgtttaggttactgtgttgtcatcagaaggctggagttatcatagcagagctttaatgacaaaatattatgagccttgtaaatagttttaaaaattgtccactaatatctatttgtcttgcaaaatttgcaattttactagtaattttcatcacttgctctttctacctctaatgtttctcagtctcctccattagatcttactgacttatcacatataaacaccttcctcagaaacagtccaataaaaattaaagaccaagaggtagaatctactggagccatcatgaattccagttctttttgttgttattgatttttcttttttttttttaaaaggcacacccttgacttttttttattgttaaaataaccagattctaatttcaggcagcaaaatcagttactgcaaaaagtcaataatcaaaaatcaatgtataattggttttcatcacctatagaattagtgaggtttatacccctcaagtgtttagtgattctattcagtcaacctaaaaaaaattgcctcttttctacttaaataaataatttatttatttattttgagacagagtttcgctctgttgcccaggccggagtgcagtggcacaatctcagctcactgcaacctccgcctcccaggtcaagcgattgattctcatgcctcagcctcccaaatagctgggattataggtgcccgccaccatgctcagctaatttttgtatttttagtagagatggcgtttcaccatgttggccaggctggtcttgaactgacctcaagtgatccgcccaccttggcctcccaaagtgtggggattactagtgtgagccaccacgcctggcctgcctgttttcattattacctgcctgttctcagtatgcaacatggcagtactattgacagtgaggtgctttggcatatcagataacttttccagttggtcaaggatcccttttctcttttcctcatttctgaactgcagaacaggaagtactaaagaagtggctcaggacaatgttgtcacatcaggagtggcagaggtgtttactaggattatgatcctttcagctgtgtgtcttagaaggatctcctgaagccctgggtttgatatagaaaccataagaaaaagacttggggcagttctatatctggctcttctcccacttctcccataaaagattaagaaaaactgatgggatgatttcagatgtttcattgccaccaaactacagccatgagttttttttctttaagtgatcttatgaggccagtaaaggcctctgtcttgattaatgatgatcatcctataatatctggatatggtggcttgacatgagttttcaacaaagaaaattagtctctgaaagacatttctcatctgaaactctcaatatattaaaatgcatttaaaagttacttctgggaaacatactaaataggccaatcagttaatcattagctaattgtcaaaccctataaaatcatggtataatgtcaccctgacataaagcaacatcaaaattagtgcatcatctataaagtgaagtattattttctcccaagtgacaaattctattgccaaaaaataccactgtacttctaataagtgacactcattttaatagaccctacaaaaatacaatattttcaatgtccccataaaacagttaacttacaaatattattctcagagctctggtgacatcattcagtgatactattgtgaaaatcctcatacaatacttgaaacactagcatgtaaagtaaattcattatataacaaaagaactatgtaaaattatgaaagataatgcatgcaaccaactccgggaaattatcctggaaattcaaattaatattgtaattaaattaatgactaatatgaaagataagtattttaaaggattataaaataaattttgatcatttatgcaggaaaatagtttcaatggaaaagtaaataattctacattaaccatgcttgtctttctcttcagtgaaaaagcattcaggattttacataccttgaaactgtttttggaaaaaaagtattttatctatttctgcccagaaaaacagccattgaaattaatgatacaggtagaccacagctctgagaaattatatttgaagtttcatatttaaataccaaggatttaaaatcacctaccataactttctaacagcagtctttcgtaatgataaattttatcaatttccaaaattcgttttaaataatttaaaaagcagcaaattagattaagcaacacacaaataaattccacatttacaagtaaagaaatcacaggggctacagtttataatcaacatgaacttgaaagaaataaagcaatacctttcctgccacccatcatccactgcttaaatttgtggtgaaaaagacttaactacaatgacctttagtctgtttctaaactctgcatgtattgtaattagctaaaggcattgaacaaattagttcatcctatttttatttgggtcccagagataaatggctaatttatgaaatatttcactctgtgtcatgagaatttagcaaatgaatatggaaccaaatataaacactttataccatatgtacagttactttcataaggcattatcatgtaatttttattgaaaaagattcaatatagtaaagtcttattttaagatatattttttctctatctgagatgtttagtttatgaaaatattgtttttctctatattctttttgtatatatgccaacatataccttgtgctagaaatattttatgggaattacaattctttatatttgtattttctatataaaggcatatacaactttgaggcagtgtttctgatggagagcagaattcataaagagcttgtgtgtgcttccgtgctccgaaattatatgaaatccattttgagaagaaacttatttgattaaaaacaaaaacaaaaacagaaacaaaactgcaccaatgcacagccagaggctgacaattaaaactaatacataaccacatgaacatcatatttatagagttaacattttttaaggatggtcagtgctaacatatagtattatacatttggcactaatgtttgccattggtccagcaattggcaaaatttgtttctatgtataaatttatttttgaacattaggtctggctagacgtatcttcactatttataaaaaatatttagacagtaagctcacgttgaataactaggtctactgtgttctggaaactcttcagtagtaatacagctttttcatgttccatatgtacaaaactgtgtccatttgcctgaaggatcttatcaccaggctgcagtaggtttgatgctggcccatcaggctgaaccctagtaacaaagatacccttgtcagaaggtttgaatggatttccttgtccactaattccaccactgatactaaatccaaggccaggattcttttctattctcacacaaaactgctctggatatccatccatactcctttgccctttagtttgaattaagcaccgtccaggctgaggtccccgggtggcctgtgaagaggggatctgaataggcaatggtgactgaaattgctggatggtcactttgtttatatttccttcatacggctgctgctcccggctgcgatgctgaaggctttgggaccccatcaacgtctggatgtggctgcctgccctgtctaaccgtctagcttctatatgtctaagcagctgttgtctccagtctgcaggcattttaccacagctctcctctcccttcacaggagtaggcctcgtctttaaatcactgttatctgatggcttgtcaccatagttacccaagttatagtcagatggtattttttccaaaagagctgccatagtaggcctagctgaaactggcctggtttgggaggcaccgtaactctctgtactgtagcttctcgcagacaatggcctcctttgggtaaggtttttaaccggaaaacttcccgcctgagctttcacttcttgatatgaagggtgttcatcttcatacctgccattccttttcaggaactgggactcagtcactgtaacgctgctttggcgatccagccctcccctatatgggggtctgccgtacctatcagttgggggcagctcatgaggctcattgacccttctaaacatggccatttctgtggcgctcaccagggagtcggcccttctcaggaagcccgccctggccccttggcttgcgaactgggcattcaccacagcatcctcattcacagatggctgagaaaatgaaaacatttgctccatcggtgggtatcctctgtaagctctaggactaatcaaatccttggcgatgtttttgctggcctgttgcacgtactcgggattgtgttgaaaagggggtggtatcctcttttcggctttcacttccactgatccttgaggattgaagctttggtcaaactgatagactttttttgtcatagaagctttttgttgttgtggccccttactacttccgtaggtgagcatctcatcatccagcattgggactgactggcttcgagacatactggacataccatgctctggtcccagcatcttatccggtcgttcgtggcttcctaagtgatcactcccagaagcatagttttctaatggtatgttatacaccttatatgtaccaatgtcaatctcatcgatactctgtgactttttgaatttattagacttgatatctttcattaggggggaaagcctctctgtgcttttgctaattgaaataacacctttagaagattccgggcggcagtggatttgagaaaagacattactaagactcctgttgggattggaatcatgatactcccatggtacgcctggagaaaaaggactaggtatttcagtagattcctttatatgttctttcctttcaggcaatgggctggtagtgggggttgtctctaatttggaaggaaaagcggtcctgtcttcaaacggactaggggttctggtccaattctgccaaggattggaaggaggcacttctgtttctggtgtgtgtctgtgtgtagactgctcgagttccaggggaacaccaacaatcctgtcttgcctgatcaaaggcctgcgtccatgcgaagatgtgcttctagatttcgaacttaagagaggattactgttggcattctcggctgtggtttcctcagcaacaaaccctgtgttgtcataatgcgagccatcagtccagttgtcagtgaaagtatcactcatgggcagccggtcaggacgctgtggtatattgcctgggggaacagcctcccgctggctgagtaatggctttgaatcaagaggctgtgggaaagatggtgcaatcctgttaccccacaaagaattatgtactgcatctttagctgttgtctgcaaggaccccactttaacccgggtattagaggatcctgaggaagcctgggaaggcgagtagtctgagtaagtgccttttttgtccttccctagcagaacaagtttgggtgggtacagaggggtctcagctaatgaagggtgaagttccccaatcctcatttcattagctggatgaacaaaagaatcctccactgtaatctcctttggggctaccggccacttgtgttcatatttttctttcacagtttgctccgtgttagcagttggatttgaattctcaacacgcactccatggcttggcttacccaccaaattttgaacagattttaccatattctttaaatcctctgggtaaggagttggatatcgttttaggtttatttcaacctgtctgccacttagagagggaagagtggtggattgtgctgcaactggcaatggagtacacatgctcctttcctgctggaggccacttatacaaccccatgccagctgtgggtcattctgggggacgggcatatcttggatctgctgatcacacctggcccatggtgtgcagcaatcgccagacagtctggcaggttggagagtaatcccacgctggcccctttcccagggggcttggcaggagagatccttaactttcccagcattttcgtcatcttcttttttgtcttcaaattcaaaggcaacagtcatgcgttgttgtctctgctcttcccacagtgtagggttaaagctgtcactgtctgactggaaatcttcatcaccacgaggctgctggggaaacatgtagttagtcaatactctttgctttgtttctggatgggcttctgtttgtaaagggataagggctttggactgattgtcagaaagccacaaagctgcaagctctttaagtttggtaaatgagaatggtaaattcttcaatctgttgtcactcaaatttaggactcttagtttctgcatctgtccaatctcttcaggaagaaattctaatttgttggagcgtagagacatgactgttacattcttacaacttccaatttctctgggtaattctggaaggaaattctcatcaactgctaatgtccgaagactatgaaggtagccaatagtagaaggtagtgactccagttcattacagctacagtcaaattcttctaataaagataaatttccaattgtattgggtagcattgtaagttgattgtcatctacttttagagttgttagttttttcaaaagtcctatagaatcaggcaattgttgcaacatattggatgacaataagaggtcctcaagggcttcacatccagaaatgtccatgtcaactgtttctattctgttttttgacatatccaggtataccaacatctttaacttccctatagacccaggtaacacttgtaatgcattattatccatccataactccctcaaattttgtatttgatccagaacttcaggcagctcaccgaattcattattgcctaggtcaagtctttccaactgggccagtttgtgcattgactttggtagagttttcaagtgattttctcttaactccaagatccgcaatttgacaagtcttccaaaattggctggaagaaattcaagaaaggcgtcattcaggtagagctgggtcaggtttaggagctgtgtgaagccatcaggtagtttagaaatgggattgacactggcttcaataattgttaaacacttacagcactttatgttttctggaaattcttgtacaccatttttactgatgtcgagttctttaagattaactaaactagcaatagtggttggcagatttgaaaggtcgttatcaggaatacttagttttcgtagagcttgacagttgaacaattgcttgggtagttcttcaatttgattggcatctagataaagctcctctaatgttcgttcgaagttaaagacctcctttggcacctgctgaagactgcagtgggagtaatctaaaactgagatgatttcttcttcacctcggaaacatcggcatggcaccagacggccgatgattttccgtttggtggtcatctccaggcactgcattgctagttattcctgtctctgcagacttctaggttgtgaccactttgacttgcattttttttcatgtagcgggctcactcctcttcaggcctcttccgaagtgctgcacgaacctctttacaaggacttctctggtattgcgggggattccttccccttattaggttctccatcatcgccggcgggagaaactgcccatgaggtttcggagagcgtagtcgtgcagctgccaagggttattccttaagtgttcaggggtccgcagtggagtgggcgccagggtcttcggaggagaagaggagggaaggagtagaaggtaggaagaacaggagatagaggggaatccaggaaggtgccacgttagaccatgatgccagtgcccttcaggtggacggctggagaggttcccgcgggaagcggctgaggggaagcccgaagcgccggcgggggaggcaggagcgcgtccactccccagcctcagcctgcccagcgcgccgcgctagcgaccgcagcagcagcggcggcggcggcggcggtggcggaggcgcagctccctccccgcccccagaaggctccacagacaataaatcctgggcggagaagagacaagcaggaaaggcgaatcctgcacccaactccgtaacaacccctgcccgttgccgcgcctgtgcagggcgaggatccccaggggccagggcgcagcgggcgtctcggaggggctgagcgctccgcaactgcaggaggcggtggcggtggcccgagtgggcggctgcaggtcccgccggcgagaacccgctgcactggggctgggtgtccgtggcttcaagcccggtgttcacccggagtagggtcctcctcggtgcagtggctcggcgcacaggtgccaggattggc

SEQ ID NO: 12392 - RNA, 20242 nt, Homo sapiens
  source 1..20242: mol_type = other RNA
ctgggaggtcaaggctgcagtgggccatgatcatgccactgcactccaacctgggtgacagagcaagaccctgtctcagaaaaaaaaaaaaaaaaaaaaaaaaggcattaaaaaagcaataaagcagaaagaaagcatttgccattttattaaactgtgagagaaggtgacaatacagtgttctttcctcatattttgtacctacacgatagcatttattagactttttgtgtgtctccccactagactgtgtttcttgaggggtaggaccatggcttatttatatcttccattgttcttataatagaattttgaacataaccccttgttcattaacatttgttgattaaattgaatgcacagtgagaaaaaggcaaattgttttaacagttaaataattttttaaaaaaggataaacatatagattggctagaggacaaaccttagaatggtccggaggcagacttacaagagaattacttaaacatctctcgattcaaacctacaggtctggatgaatactcaaaatataagtatatattttggggtataggtgaacctgcggggcatatttatggcaagaccaagcaaaagaagaaaatatagtcccttcactttgagtagtttatgatgacctagggccctaggtgacagggatagtaactatcattttttgggaaacgtggaaatgcaaaaaaaaaaaaaattgcctgataagatatatagacacacacacacacacacacacagacacacacacagacacacacagagagagagagatattaattcccaagtttgaatttctctgggaaatggccacaaagaaatgcctgaactgtttgctagcaacattcatggttttataaagaatatagcagtgatgtcctgctagaatatctgtcttgatcataatgagactgtgagaacctatcaagtgcaagatacccgttgcttagtcaaacgattctacaagtatggctgaagatttatatcccaaaactggctatcaaagatggctggtttaaaacaatcaagacagtatagacaaatattacagggcaagaatagtttggatgatgatatcctagagaaaaaatcacttttagagaatgggacttgttcactatctaacaactttctcttttacagattctagcttaatgatcatcaataaaagtgaagtcttgaatatgatggatattcacttatttgtcagggaggtgacacagttggacaagcagcacccttggagtcggggttggggaggagtgcgtgagatgtttcaaaaggatctcagtgcattttaagtgacagcttctcctgctctcttctcttcccacagctgctgggggtcctgcaccccaacccagcctagatgatatttccatttgttgtacctaaaagcagagctttttacatctttacatctttacctcatgacagaactaaaaaaatgatgtttgttctacagtatggcacggagatgggtaaaaaagtgaaaagaataagccacaagcccccgtgctttgaggagatgatcatagcctgctcctggggaactatgctagtggctggatagcaagcactgacctagaggttgctcctaggaataaaaaattaagattatccatagaagacaaagaaaaaaatacttcgctaatagtggataccaaaaatctgaggtagtgcaaaagaaaagaaaggaaaaaagaaataaaaagcgcaactggaatacatacatacaaactttcaagacgttttctcttatactcttcagtaaaattctatgtaattttcattctagtatttaaatagttctggattttacaactaaacctatcattaaaaggttatggaaaatagaaggaataaaaaagatgaaatagaacatcaggcaaatcaaaaactcaaaagctgtatccaaaacaatggtggacacctgccgtatttgctttaaaatgggtggcactgttgtgtacaatttaaatttgttaaggagatatttaacttctctgaaaagagaggaagaacacttggtaaacaaacccaaaatggtgcactaaaattggcaggcttgaggtcagaaagaacttacaaaatattaacccccaaagaaggttaaattgaatttgctaagaaagagtattctgtattagtatctggtgatcatgtggctagaaggaaattgttttttttggaggaaaacaccagaggatataaatggcttcacataaactttgggaaagaacaccttgtcttccctctacctttgctccgggttggaagaaaaaaagattaaatggttggcaggggaacacctgaaacccatataagtagggctttgatggaattagcaaagaagaagctcagaccaggaggctggctaagctgtgagggtgaggatataattagcttagaggaagtaaacaaaaacatttggcctttttagcaatgatccagccatcagaggccctggaatttcaaatgactaagaagaaccaaaatagcttgaggacacatgtcaccaaggccgccaggggttctctgccttcagcacccagatattcccactgaaaggagagaggctggggagattgcaaactaccttgggaatccaatgatcactttgtgagagacattttgaaatacatttcgaaatacatttcttattcacttcataataaaataaaatctgattgtcatattatgctgattactcatacacataaataaaatgaaaaattaggcgtttattgtagatgcctagttattgccagatggaaataaagctatacccagatgcacacatattcagattggactagttttagaattacataaagaaggctaggcaaacttaaccacagttcctgatgtttaagttttggaaagttaactttaaaaataaattttgagtaacttgagacaaatctattcccacatacttggaatgggcatacctgaaggaagtgtggctaaaataatgggagataggagcaaaatatttggaaaacacaagttagagaagaactattaaactggtgggtataataattaaactgaacaattaaggaacatcaaaactttaaacaatcaagcctcactgagaaagtggtttctgtctcattaggttttgggtgattgatacaatctgagaggtttagtaaaaaaacatataaactgcctaaaataagctcaaagctcttgtttttttcttaaattgtgtaaatttagagcattgtttcaaattttctcaaaggagaaaggaaaggggtgttgttagcaattgtatcagcacaaggggcataaaaacagactgtgtaaggccatcccagcactttgggaggccgaggcggtcggatcgatagagcccaggtgttcaagaccagcctgggcaacatggagaaaacctgtctttactaaaaatacaaaaattagccgggcgtggtggtgcatgcctgtagtcccagctactcgggaggctgaggcaggaaaatcgtttgaacccaggaggtggaggttgcagtgagccgagatcgcgccactgcactccagcctgggcgacagagcgacactgtctcaatacaaacaaacaaaaaacacccacgacaacaacaaaaatcggactgtgctcccccaagccagagaattgccaaggctgggatttaaaatgtagatatgaggtctccatctagtggtggctcttctgaactgcagacacatgtttctttaaaagagtatgcggatgtgtacaactaaatatgaggatagtatttgtcagagttgaacgcagtaatttaaactagaggattttattgagatgaaacacaatttgttgctttataagggtgggttacagagggaaatgttcaccccttcgctccaggaatttaagaatagcatgaatccttccctgaagatagacaaatgaaccagatcctctcaaggtccctttctgtcttatgataggacaataattttgctcctttctccacagagcttttacctgtagccacactgtctgacattagtctttatttaagaaaagtacggccgggcgcggtgtctcacgcctgtaatccccgtactttgggagtccgaggcaggtggatcacgaggtcaggagttcaagaccaacctggccaagaaggtgaaactccgtctctactaaaaatacaaaaaattagccgggtgcagtggcaggcgcctgtaatcccagctactcgggaggctgaggcaggagaatcgcttgaactcggagggcggaggttgcagtaagctgagatcgtgccactgcactccagcctccagcctgatgacagagtgagactccgtctcaaaaaaaaaaaaaaaaaaaaaaaaaagaaaagaaaagaaaagaaaaaagaaaagtactctggtaatttttaaaaatgagataacttttttccttgttctgagaagttgtatgactaaagcattacctatgacgttagacaaaaatagtttctagaaatgaatagcaattaaactaaatatatttctaatatgcaccttatttttcactgtaaattcttcttttgacatctggaagagcaggagggaaggcagaaaccaagaagagctgaacgattactcctctggccaagagagagcagagagagaggaagggaattcagggctgtctgaagaaggggcatggtcaccagaacgaagagactggaggatatgcctgaatctgatttcttttatccagttcctctctgattctctgtatcagtcctctattgcccttcttttgtctttctcattctttcttccttaataacttattaattcccctctttcccagccctagtctgttcttgttccttactcactcattattctcattattctaaaatgctcttacttaaaaatatttcattaaagtactcttactattctaaaatattcttactatcctaagataatgtcactctctcaattaatatttcacttttccagttcatttttcatttatttttgttcaaagagacattggcattcttttacccatgtaaatgtatagacactgggctataagataccaaagagtaggcccctggagagtttgaggcatcatgctatcaaagacagcaatggtggctgtttccttcaagatatactatgactttatctaaatctttctaaatcaaaaattttatgagaagaagacataattaacttgatagttatcaagttctctttatacaaagaaattaaaaagcagaggtagaataagagtaattaatattaatagtataagtaaaagagtcaatgacaaaacatttaatgtttcggaatatttcactcaattctggagttacttagctatgaaacccaaatagaaagacatgggaaatagttttgtgagaaagctaggacagaaatgttttacttgaaaggaaattaaggtcccatgaggtaataaagggattgtggttaggagcttaccaacctgggggtcttagatatcattagattcccagttagatatcatttttgttttaaggggctggattccattttttgtcccttcaggggaaggatctaatgaagccaaagatcatggcagtataaatagcatgctttctttctactttgagatcaacaggccagattctatctctataaaagtttgggaggggtaacatggttttgtcaaggtaaccctgattttttttctgtgctctatctaaatagttaatcatatcaattatatagcttttacagtggcttgataattttggctgaactatatgacatcttcactttagggatatagggggtgggatctattcatgaaatgatgccaaaatgcagtgtgtaaacattgtcatgctcaactgtggccaacagcctgtagacagactattcttttatctacttaaaggacgggcagcatttggcagcagtttgattaaaatttagagctaaataggtaggtggagacccctttctctcaactacacttccgtagcctcgtctctctcatgacatcttttattcttccctccacatccaaattgtaaaaattgcttaggtaacgtaatctagtgacaatgtgcatgacttcttctcaaagagaaaggaaacccaatcaaatcaaaaggatagatatggtgtgctccaattaaataaaagccacttcttaaactttttgaatggtgttactttttggatagtgttaaggtccttagaacacacaaaaggaaaattaaatgtaactgctgaaacacagcagaaaagaccaaaaatgtcttagaaaaaatgctgaagagaggaggaagactgatttaaaaaggagaaattttttttaactgggaattttgagtcaactgagaagatgaaaggttggtagtttaaggttacacaaactgaagatcaatttgctgtttagttcaatatttataaagtgcactatgtgccaggcctgtcatccacttaataattacacaaatatttattgagaacctatactatgtttctgacactatgacaggcattaaggatatatggtaaacaaaacatctggtcattttacctctcctgaggctcttctgtctagaagtcctttgttaagtattgtctgatcctctctctcaaaaagcttaaagttcataggaaaaacaaacaccaaatagctatgatctcaggcagaatgggaaagatactaaaaaacataagaaaaaattaatatggtagtgctgagtacagaaatttttttccatgaagactagggagggtttcatggttctagtgctgtttgagctgggctctgaaggctgcatatgattttaataatttagaaagggaatagggagaggaaggcattccagtagagggatagtgtgggcaaaagctgaaatataaaacacagcgaatacttggaaaagtaaggatttatatgtgtctaaaacactgagtatgcatagggtgaagaaaagaaaacaatttccagattcagaggatcagaactccttagaagaatagatgttgatgatacatggtatgtgtgatccaatctcatgcaaacagtattttcaggggatcacttgagcagcgtgtagtgaaaatgttctccacccaaaaagtgaagtaaataaacatgaaatgcagccagctgaatgattgttcaactccttgcatttcggagtgggtcattctaacattggacagcatggattcccacgctccctgacagtggtcataggagggactttttggggccgctgaacctagaagactcttttcaagcaacccccccacactttttaaagtgttgaattccatctccttctcccgtaacgtcaggggcatacagactcagtgctggaccaagttgaggaacacctttcttcatttcctttcctctttagaacaaattggcaaaattctcgctcctcttccagagattcaagagattctggttgctatttatcttgtctagcaaggcattcacacttgccacgtttagcctatcaaatgttgccctaaatcctggcaaatattcatctagctcacacttttcgtgacacttttttttttttttttaagatggagtctcactctgtcacccaggctggagagctgtggcgccatctcagctcactgcaacctccgcctgctgggttgaagcaattctcctgcctcagcctccccagtaactaggattacaggtgcgcgccacaatgcccggctaatttttcatatttttagtagagatgaggtttcagcatgttggtcaggctggtatccaattcctgacctcaagtgatccacctgcctcggcctccctaagtgctgggattacaggcataagtcaccgcacccggcttcgtgacactctttatgtgagctgtgtgaaggtcacaagaaccagcagaagacctatctgtagctccaaatggaaaaaaccatgctcaaactgaaacagatttgactagataaagactcgatttccttttgcaataggatggttgagggcaggaataaagggactcaccacattgccttgtactgtctttgatgtggaacttctctcatctttcctctggactgtgagattctgtgctgaggggaccacattacatccctcatagtacctgatatgtagttgatgcccaacaaatatttattttaatatttataatcataatatttaatgtttttgttatattcttcaatgaaatgtctccaaatgttttcagtttatgaataatatactttaggcctcagagattcagctacagtaaatgttttcctgtggaggaagtacaagagtttgctatgaaaataaagttccctgtactaagatactttactctggatgtaaagatacttggctatttgttaggctgcttattcaacctgttattttaaagaaggaaaaaaaataagcacaaacaatacacttgtgcaacagtgataaaaaaatacactttcaaaactagagaaagattgggtgattcatttaactttctttcaacaccaatttctacacccagtgaaatctatgctagcttaaagaatgaaaaaatgctgggcacagtggctcacgcctgtaatcccagcactttgggaggtcgaggcaggtggatcttttgaggccaggtgttcgagaccagcctggccaacacggtgaaaccctgtccctactaaaaatacaaaaattagcccagtgtggtggcacgcacctgtaatcccagctactcaggaggctgagacatgagaattgcctgaactcgggaggtggaagttacagtgagccaagatagcgctactgcactccagcctgggtgacacagcaagactctgtctcaagaaaaaaaaagaaagaaaagaaaaagtcacataaaagtctttttttcaaaaaaggagaagagaaaattatgccaggtttcaaaatctcacctgtggaaatttgacccagaccttgtctttgggtaggactacatagtggttccaaccgtagactaataagagtcatggaatgtttacataaatgctgcgtgaatttcacaaccttccaccttttgaggtgctgccataacaaaattaggcacaaaaggggtgttttgcagacaatttgtggaagtattgacagagctgcagaggtatccttctcatttctgcatgccttaatccaggcccatttcttacattgcttagtgctcagtgtgttgttacaaagagcatgagctcagaacccaactgggaagactctaccagctgaagaaatgcctctgaagttaaccagtaaattttctcctctctcaggtcttttctccttacttcccatagaactgttcttagggaaggttgacataatcacatggttaaaatcccaagggactcaatattcctatactttaactgtatgtttttaaataaaaacttagagtagacttgccccctcggtttttcaaaaatctctgaattctccaaagtagaagctgtgcaatttatatccttaccagggagtgtttccaaaccattctcttgcaggcagtgttgaaagtaaggaagattggaacctgtctcagtaagaagctgagaggcttagagaaagttcctcaacacagcaaaacccaacattttaaaaacagaagcagaaacagttttataaaggcattgccacccccaccattgcacacaggctttgtttgttgttgtcagtaacattataagcactccatctttgggccttagttaatgctactactccaggttcctgcgttacccaagaaagttcctcccaaattgggagctgtaaccatctgttgatactcaaggctctccgaacagctatcactctaagagggtctcttatctgtgtttcagcaggatagaagcagacatccactgcctttggaaaaacatggggagttggagggacggatctatagcagcaactgcagcaatgaagacaggtcagttttacacgctagaaacagaaatgcccccagaaggttcaggatatgactggaaaacttgattgcatctaccttagtttgtacaagtggtgcatcttggaaaatagatttcctgaacagtttagatcaaaatggagctgacactcaggatctcctgtaatagtgacccacatgctttctatacatagcgcacatctatttgtccacagcccacattctgttttcttgctataatgtattctttgggtatggtgttggtgggtgatgggaaatattctgagccaaggcaagatgcttttcttaacagaaggtggttgtattgctaaggaaaaatgttcatgcaagtgatcaccaacctggagatgccccccaagtcccagatgatcaggtagctacaagtgtgaagagaggacacattaccaacccagagtttgaacatttagttaagctcagtaagatttagcatttctgtgaaaggaactacagtggaacttcaaccccgcttttctttatactagataaaggacccatcttcttaacctattggatttcattatttgcataactttttattgacccagtgtgccaataaacttgctgtttggtcggcatatcacaaattagtcaaatatgttgtttgatcgaatttatcaaagactttgagtggtagtcctatttcagtatggcttttgacctggttatgttgtattcttgcctcttgatgagaatgtattcatcagacatatttgatcggtgtgctaatgaggggtagaaattggttagggacagcgttaagactgtccttaacagttagtaaacatactaaacggaaagacaaggtggcaagcacactacattttccaaagctttacactggaaagcttaaatattaatagatattaaatatatattaaatagattttatgattaaaaataaaatggtttttttggtttctttcatctaaccattttgacaaattcagatacttttcacttaatatttgaatatataaatctaatttcttccatgttttctcccctctgaatcttctctttttttttttttttttttttgagacggagtctcgctctgtcgcccaggctggagtgcagtggcgggatctcggctcactgcaagctccgcctcctgggttcacgccattctcctgcctcagcctcccaagtagctgggactacaggcgcccgccactacgcccggctaattttttgtatttttagtagagacggggtttcaccgttttagctgggatggtctcgatctcctgacctcgtgatccgcccgcctcggcctcccaaagtgctgggattacaggcgtgagccaccgcgcccggccctctctctttagctcaccagttgaaagatatgtcagtcctatttttaaataagtaattacattagtgatatgtgtgcaatcatctttaagattaagagcaaattaacattggcttgtcagtctctcctcaaagctgttttccatctcaaaggtcgtgatccaaggtaaggtccagaaacaactgagattgttttacatctatgtactaggttggaacaaaagtaattgtggtttttgcctgcacttttaatggtaaaaaccgcaattactttttcagcaacctaataattacaattctaagtaatggagatacatatcttttataggcttcaatgagcaatacattagcataatgttttatttcatactgactttgaatattccttgtcaaaaatgcacttatactttggagttactatgtatgtttaggttactgtgttgtcatcagaaggctggagttatcatagcagagctttaatgacaaaatattatgagccttgtaaatagttttaaaaattgtccactaatatctatttgtcttgcaaaatttgcaattttactagtaattttcatcacttgctctttctacctctaatgtttctcagtctcctccattagatcttactgacttatcacatataaacaccttcctcagaaacagtccaataaaaattaaagaccaagaggtagaatctactggagccatcatgaattccagttctttttgttgttattgatttttcttttttttttttaaaaggcacacccttgacttttttttattgttaaaataaccagattctaatttcaggcagcaaaatcagttactgcaaaaagtcaataatcaaaaatcaatgtataattggttttcatcacctatagaattagtgaggtttatacccctcaagtgtttagtgattctattcagtcaacctaaaaaaaattgcctcttttctacttaaataaataatttatttatttattttgagacagagtttcgctctgttgcccaggccggagtgcagtggcacaatctcagctcactgcaacctccgcctcccaggtcaagcgattgattctcatgcctcagcctcccaaatagctgggattataggtgcccgccaccatgctcagctaatttttgtatttttagtagagatggcgtttcaccatgttggccaggctggtcttgaactgacctcaagtgatccgcccaccttggcctcccaaagtgtggggattactagtgtgagccaccacgcctggcctgcctgttttcattattacctgcctgttctcagtatgcaacatggcagtactattgacagtgaggtgctttggcatatcagataacttttccagttggtcaaggatcccttttctcttttcctcatttctgaactgcagaacaggaagtactaaagaagtggctcaggacaatgttgtcacatcaggagtggcagaggtgtttactaggattatgatcctttcagctgtgtgtcttagaaggatctcctgaagccctgggtttgatatagaaaccataagaaaaagacttggggcagttctatatctggctcttctcccacttctcccataaaagattaagaaaaactgatgggatgatttcagatgtttcattgccaccaaactacagccatgagttttttttctttaagtgatcttatgaggccagtaaaggcctctgtcttgattaatgatgatcatcctataatatctggatatggtggcttgacatgagttttcaacaaagaaaattagtctctgaaagacatttctcatctgaaactctcaatatattaaaatgcatttaaaagttacttctgggaaacatactaaataggccaatcagttaatcattagctaattgtcaaaccctataaaatcatggtataatgtcaccctgacataaagcaacatcaaaattagtgcatcatctataaagtgaagtattattttctcccaagtgacaaattctattgccaaaaaataccactgtacttctaataagtgacactcattttaatagaccctacaaaaatacaatattttcaatgtccccataaaacagttaacttacaaatattattctcagagctctggtgacatcattcagtgatactattgtgaaaatcctcatacaatacttgaaacactagcatgtaaagtaaattcattatataacaaaagaactatgtaaaattatgaaagataatgcatgcaaccaactccgggaaattatcctggaaattcaaattaatattgtaattaaattaatgactaatatgaaagataagtattttaaaggattataaaataaattttgatcatttatgcaggaaaatagtttcaatggaaaagtaaataattctacattaaccatgcttgtctttctcttcagtgaaaaagcattcaggattttacataccttgaaactgtttttggaaaaaaagtattttatctatttctgcccagaaaaacagccattgaaattaatgatacaggtagaccacagctctgagaaattatatttgaagtttcatatttaaataccaaggatttaaaatcacctaccataactttctaacagcagtctttcgtaatgataaattttatcaatttccaaaattcgttttaaataatttaaaaagcagcaaattagattaagcaacacacaaataaattccacatttacaagtaaagaaatcacaggggctacagtttataatcaacatgaacttgaaagaaataaagcaatacctttcctgccacccatcatccactgcttaaatttgtggtgaaaaagacttaactacaatgacctttagtctgtttctaaactctgcatgtattgtaattagctaaaggcattgaacaaattagttcatcctatttttatttgggtcccagagataaatggctaatttatgaaatatttcactctgtgtcatgagaatttagcaaatgaatatggaaccaaatataaacactttataccatatgtacagttactttcataaggcattatcatgtaatttttattgaaaaagattcaatatagtaaagtcttattttaagatatattttttctctatctgagatgtttagtttatgaaaatattgtttttctctatattctttttgtatatatgccaacatataccttgtgctagaaatattttatgggaattacaattctttatatttgtattttctatataaaggcatatacaactttgaggcagtgtttctgatggagagcagaattcataaagagcttgtgtgtgcttccgtgctccgaaattatatgaaatccattttgagaagaaacttatttgattaaaaacaaaaacaaaaacagaaacaaaactgcaccaatgcacagccagaggctgacaattaaaactaatacataaccacatgaacatcatatttatagagttaacattttttaaggatggtcagtgctaacatatagtattatacatttggcactaatgtttgccattggtccagcaattggcaaaatttgtttctatgtataaatttatttttgaacattaggtctggctagacgtatcttcactatttataaaaaatatttagacagtaagctcacgttgaataactaggtctactgtgttctggaaactcttcagtagtaatacagctttttcatgttccatatgtacaaaactgtgtccatttgcctgaaggatcttatcaccaggctgcagtaggtttgatgctggcccatcaggctgaaccctagtaacaaagatacccttgtcagaaggtttgaatggatttccttgtccactaattccaccactgatactaaatccaaggccaggattcttttctattctcacacaaaactgctctggatatccatccatactcctttgccctttagtttgaattaagcaccgtccaggctgaggtccccgggtggcctgtgaagaggggatctgaataggcaatggtgactgaaattgctggatggtcactttgtttatatttccttcatacggctgctgctcccggctgcgatgctgaaggctttgggaccccatcaacgtctggatgtggctgcctgccttcttagtaatggtgtccggaggtacatcccgcctcccaagtggataaggattccattggccactaggagatacatcttcttgtccattgtctaaaatgttgctttgctgggacggggtcctgtctaaccgtctagcttctatatgtctaagcagctgttgtctccagtctgcaggcattttaccacagctctcctctcccttcacaggagtaggcctcgtctttaaatcactgttatctgatggcttgtcaccatagttacccaagttatagtcagatggtattttttccaaaagagctgccatagtaggcctagctgaaactggcctggtttgggaggcaccgtaactctctgtactgtagcttctcgcagacaatggcctcctttgggtaaggtttttaaccggaaaacttcccgcctgagctttcacttcttgatatgaagggtgttcatcttcatacctgccattccttttcaggaactgggactcagtcactgtaacgctgctttggcgatccagccctcccctatatgggggtctgccgtacctatcagttgggggcagctcatgaggctcattgacccttctaaacatggccatttctgtggcgctcaccagggagtcggcccttctcaggaagcccgccctggccccttggcttgcgaactgggcattcaccacagcatcctcattcacagatggctgagaaaatgaaaacatttgctccatcggtgggtatcctctgtaagctctaggactaatcaaatccttggcgatgtttttgctggcctgttgcacgtactcgggattgtgttgaaaagggggtggtatcctcttttcggctttcacttccactgatccttgaggattgaagctttggtcaaactgatagactttttttgtcatagaagctttttgttgttgtggccccttactacttccgtaggtgagcatctcatcatccagcattgggactgactggcttcgagacatactggacataccatgctctggtcccagcatcttatccggtcgttcgtggcttcctaagtgatcactcccagaagcatagttttctaatggtatgttatacaccttatatgtaccaatgtcaatctcatcgatactctgtgactttttgaatttattagacttgatatctttcattaggggggaaagcctctctgtgcttttgctaattgaaataacacctttagaagattccgggcggcagtggatttgagaaaagacattactaagactcctgttgggattggaatcatgatactcccatggtacgcctggagaaaaaggactaggtatttcagtagattcctttatatgttctttcctttcaggcaatgggctggtagtgggggttgtctctaatttggaaggaaaagcggtcctgtcttcaaacggactaggggttctggtccaattctgccaaggattggaaggaggcacttctgtttctggtgtgtgtctgtgtgtagactgctcgagttccaggggaacaccaacaatcctgtcttgcctgatcaaaggcctgcgtccatgcgaagatgtgcttctagatttcgaacttaagagaggattactgttggcattctcggctgtggtttcctcagcaacaaaccctgtgttgtcataatgcgagccatcagtccagttgtcagtgaaagtatcactcatgggcagccggtcaggacgctgtggtatattgcctgggggaacagcctcccgctggctgagtaatggctttgaatcaagaggctgtgggaaagatggtgcaatcctgttaccccacaaagaattatgtactgcatctttagctgttgtctgcaaggaccccactttaacccgggtattagaggatcctgaggaagcctgggaaggcgagtagtctgagtaagtgcctgaggaaacactgttattcagacagtgagttttgtcaacttcagactcatcagttgattcttttttgtccttccctagcagaacaagtttgggtgggtacagaggggtctcagctaatgaagggtgaagttccccaatcctcatttcattagctggatgaacaaaagaatcctccactgtaatctcctttggggctaccggccacttgtgttcatatttttctttcacagtttgctccgtgttagcagttggatttgaattctcaacacgcactccatggcttggcttacccaccaaattttgaacagattttaccatattctttaaatcctctgggtaaggagttggatatcgttttaggtttatttcaacctgtctgccacttagagagggaagagtggtggattgtgctgcaactggcaatggagtacacatgctcctttcctgctggaggccacttatacaaccccatgccagctgtgggtcattctgggggacgggcatatcttggatctgctgatcacacctggcccatggtgtgcagcaatcgccagacagtctggcaggttggagagtaatcccacgctggcccctttcccagggggcttggcaggagagatccttaactttcccagcattttcgtcatcttcttttttgtcttcaaattcaaaggcaacagtcatgcgttgttgtctctgctcttcccacagtgtagggttaaagctgtcactgtctgactggaaatcttcatcaccacgaggctgctggggaaacatgtagttagtcaatactctttgctttgtttctggatgggcttctgtttgtaaagggataagggctttggactgattgtcagaaagccacaaagctgcaagctctttaagtttggtaaatgagaatggtaaattcttcaatctgttgtcactcaaatttaggactcttagtttctgcatctgtccaatctcttcaggaagaaattctaatttgttggagcgtagagacatgactgttacattcttacaacttccaatttctctgggtaattctggaaggaaattctcatcaactgctaatgtccgaagactatgaaggtagccaatagtagaaggtagtgactccagttcattacagctacagtcaaattcttctaataaagataaatttccaattgtattgggtagcattgtaagttgattgtcatctacttttagagttgttagttttttcaaaagtcctatagaatcaggcaattgttgcaacatattggatgacaataagaggtcctcaagggcttcacatccagaaatgtccatgtcaactgtttctattctgttttttgacatatccaggtataccaacatctttaacttccctatagacccaggtaacacttgtaatgcattattatccatccataactccctcaaattttgtatttgatccagaacttcaggcagctcaccgaattcattattgcctaggtcaagtctttccaactgggccagtttgtgcattgactttggtagagttttcaagtgattttctcttaactccaagatccgcaatttgacaagtcttccaaaattggctggaagaaattcaagaaaggcgtcattcaggtagagctgggtcaggtttaggagctgtgtgaagccatcaggtagtttagaaatgggattgacactggcttcaataattgttaaacacttacagcactttatgttttctggaaattcttgtacaccatttttactgatgtcgagttctttaagattaactaaactagcaatagtggttggcagatttgaaaggtcgttatcaggaatacttagttttcgtagagcttgacagttgaacaattgcttgggtagttcttcaatttgattggcatctagataaagctcctctaatgttcgttcgaagttaaagacctcctttggcacctgctgaagactgcagtgggagtaatctaaaactgagatgatttcttcttcacctcggaaacatcggcatggcaccagacggccgatgattttccgtttggtggtcatctccaggcactgcaactcctcttcaggcctcttccgaagtgctgcacgaacctctttacaaggacttctctggtattgcgggggattccttccccttattaggttctccatcatcgccggcgggagaaactgcccatgaggtttcggagagcgtagtcgtgcagctgccaagggttattccttaagtgttcaggggtccgcagtggagtgggcgccagggtcttcggaggagaagaggagggaaggagtagaaggtaggaagaacaggagatagaggggaatccaggaaggtgccacgttagaccatgatgccagtgcccttcaggtggacggctggagaggttcccgcgggaagcggctgaggggaagcccgaagcgccggcgggggaggcaggagcgcgtccactccccagcctcagcctgcccagcgcgccgcgctagcgaccgcagcagcagcggcggcggcggcggcggtggcggaggcgcagctccctccccgcccccagaaggctccacagacaataaatcctgggcggagaagagacaagcaggaaaggcgaatcctgcacccaactccgtaacaacccctgcccgttgccgcgcctgtgcagggcgaggatccccaggggccagggcgcagcgggcgtctcggaggggctgagcgctccgcaactgcaggaggcggtggcggtggcccgagtgggcggctgcaggtcccgccggcgagaacccgctgcactggggctgggtgtccgtggcttcaagcccggtgttcacccggagtagggtcctcctcggtgcagtggctcggcgcacaggtgccaggattggc

SEQ ID NO: 12393 - RNA, 20319 nt, Homo sapiens
  source 1..20319: mol_type = other RNA
ctgggaggtcaaggctgcagtgggccatgatcatgccactgcactccaacctgggtgacagagcaagaccctgtctcagaaaaaaaaaaaaaaaaaaaaaaaaggcattaaaaaagcaataaagcagaaagaaagcatttgccattttattaaactgtgagagaaggtgacaatacagtgttctttcctcatattttgtacctacacgatagcatttattagactttttgtgtgtctccccactagactgtgtttcttgaggggtaggaccatggcttatttatatcttccattgttcttataatagaattttgaacataaccccttgttcattaacatttgttgattaaattgaatgcacagtgagaaaaaggcaaattgttttaacagttaaataattttttaaaaaaggataaacatatagattggctagaggacaaaccttagaatggtccggaggcagacttacaagagaattacttaaacatctctcgattcaaacctacaggtctggatgaatactcaaaatataagtatatattttggggtataggtgaacctgcggggcatatttatggcaagaccaagcaaaagaagaaaatatagtcccttcactttgagtagtttatgatgacctagggccctaggtgacagggatagtaactatcattttttgggaaacgtggaaatgcaaaaaaaaaaaaaattgcctgataagatatatagacacacacacacacacacacacagacacacacacagacacacacagagagagagagatattaattcccaagtttgaatttctctgggaaatggccacaaagaaatgcctgaactgtttgctagcaacattcatggttttataaagaatatagcagtgatgtcctgctagaatatctgtcttgatcataatgagactgtgagaacctatcaagtgcaagatacccgttgcttagtcaaacgattctacaagtatggctgaagatttatatcccaaaactggctatcaaagatggctggtttaaaacaatcaagacagtatagacaaatattacagggcaagaatagtttggatgatgatatcctagagaaaaaatcacttttagagaatgggacttgttcactatctaacaactttctcttttacagattctagcttaatgatcatcaataaaagtgaagtcttgaatatgatggatattcacttatttgtcagggaggtgacacagttggacaagcagcacccttggagtcggggttggggaggagtgcgtgagatgtttcaaaaggatctcagtgcattttaagtgacagcttctcctgctctcttctcttcccacagctgctgggggtcctgcaccccaacccagcctagatgatatttccatttgttgtacctaaaagcagagctttttacatctttacatctttacctcatgacagaactaaaaaaatgatgtttgttctacagtatggcacggagatgggtaaaaaagtgaaaagaataagccacaagcccccgtgctttgaggagatgatcatagcctgctcctggggaactatgctagtggctggatagcaagcactgacctagaggttgctcctaggaataaaaaattaagattatccatagaagacaaagaaaaaaatacttcgctaatagtggataccaaaaatctgaggtagtgcaaaagaaaagaaaggaaaaaagaaataaaaagcgcaactggaatacatacatacaaactttcaagacgttttctcttatactcttcagtaaaattctatgtaattttcattctagtatttaaatagttctggattttacaactaaacctatcattaaaaggttatggaaaatagaaggaataaaaaagatgaaatagaacatcaggcaaatcaaaaactcaaaagctgtatccaaaacaatggtggacacctgccgtatttgctttaaaatgggtggcactgttgtgtacaatttaaatttgttaaggagatatttaacttctctgaaaagagaggaagaacacttggtaaacaaacccaaaatggtgcactaaaattggcaggcttgaggtcagaaagaacttacaaaatattaacccccaaagaaggttaaattgaatttgctaagaaagagtattctgtattagtatctggtgatcatgtggctagaaggaaattgttttttttggaggaaaacaccagaggatataaatggcttcacataaactttgggaaagaacaccttgtcttccctctacctttgctccgggttggaagaaaaaaagattaaatggttggcaggggaacacctgaaacccatataagtagggctttgatggaattagcaaagaagaagctcagaccaggaggctggctaagctgtgagggtgaggatataattagcttagaggaagtaaacaaaaacatttggcctttttagcaatgatccagccatcagaggccctggaatttcaaatgactaagaagaaccaaaatagcttgaggacacatgtcaccaaggccgccaggggttctctgccttcagcacccagatattcccactgaaaggagagaggctggggagattgcaaactaccttgggaatccaatgatcactttgtgagagacattttgaaatacatttcgaaatacatttcttattcacttcataataaaataaaatctgattgtcatattatgctgattactcatacacataaataaaatgaaaaattaggcgtttattgtagatgcctagttattgccagatggaaataaagctatacccagatgcacacatattcagattggactagttttagaattacataaagaaggctaggcaaacttaaccacagttcctgatgtttaagttttggaaagttaactttaaaaataaattttgagtaacttgagacaaatctattcccacatacttggaatgggcatacctgaaggaagtgtggctaaaataatgggagataggagcaaaatatttggaaaacacaagttagagaagaactattaaactggtgggtataataattaaactgaacaattaaggaacatcaaaactttaaacaatcaagcctcactgagaaagtggtttctgtctcattaggttttgggtgattgatacaatctgagaggtttagtaaaaaaacatataaactgcctaaaataagctcaaagctcttgtttttttcttaaattgtgtaaatttagagcattgtttcaaattttctcaaaggagaaaggaaaggggtgttgttagcaattgtatcagcacaaggggcataaaaacagactgtgtaaggccatcccagcactttgggaggccgaggcggtcggatcgatagagcccaggtgttcaagaccagcctgggcaacatggagaaaacctgtctttactaaaaatacaaaaattagccgggcgtggtggtgcatgcctgtagtcccagctactcgggaggctgaggcaggaaaatcgtttgaacccaggaggtggaggttgcagtgagccgagatcgcgccactgcactccagcctgggcgacagagcgacactgtctcaatacaaacaaacaaaaaacacccacgacaacaacaaaaatcggactgtgctcccccaagccagagaattgccaaggctgggatttaaaatgtagatatgaggtctccatctagtggtggctcttctgaactgcagacacatgtttctttaaaagagtatgcggatgtgtacaactaaatatgaggatagtatttgtcagagttgaacgcagtaatttaaactagaggattttattgagatgaaacacaatttgttgctttataagggtgggttacagagggaaatgttcaccccttcgctccaggaatttaagaatagcatgaatccttccctgaagatagacaaatgaaccagatcctctcaaggtccctttctgtcttatgataggacaataattttgctcctttctccacagagcttttacctgtagccacactgtctgacattagtctttatttaagaaaagtacggccgggcgcggtgtctcacgcctgtaatccccgtactttgggagtccgaggcaggtggatcacgaggtcaggagttcaagaccaacctggccaagaaggtgaaactccgtctctactaaaaatacaaaaaattagccgggtgcagtggcaggcgcctgtaatcccagctactcgggaggctgaggcaggagaatcgcttgaactcggagggcggaggttgcagtaagctgagatcgtgccactgcactccagcctccagcctgatgacagagtgagactccgtctcaaaaaaaaaaaaaaaaaaaaaaaaaagaaaagaaaagaaaagaaaaaagaaaagtactctggtaatttttaaaaatgagataacttttttccttgttctgagaagttgtatgactaaagcattacctatgacgttagacaaaaatagtttctagaaatgaatagcaattaaactaaatatatttctaatatgcaccttatttttcactgtaaattcttcttttgacatctggaagagcaggagggaaggcagaaaccaagaagagctgaacgattactcctctggccaagagagagcagagagagaggaagggaattcagggctgtctgaagaaggggcatggtcaccagaacgaagagactggaggatatgcctgaatctgatttcttttatccagttcctctctgattctctgtatcagtcctctattgcccttcttttgtctttctcattctttcttccttaataacttattaattcccctctttcccagccctagtctgttcttgttccttactcactcattattctcattattctaaaatgctcttacttaaaaatatttcattaaagtactcttactattctaaaatattcttactatcctaagataatgtcactctctcaattaatatttcacttttccagttcatttttcatttatttttgttcaaagagacattggcattcttttacccatgtaaatgtatagacactgggctataagataccaaagagtaggcccctggagagtttgaggcatcatgctatcaaagacagcaatggtggctgtttccttcaagatatactatgactttatctaaatctttctaaatcaaaaattttatgagaagaagacataattaacttgatagttatcaagttctctttatacaaagaaattaaaaagcagaggtagaataagagtaattaatattaatagtataagtaaaagagtcaatgacaaaacatttaatgtttcggaatatttcactcaattctggagttacttagctatgaaacccaaatagaaagacatgggaaatagttttgtgagaaagctaggacagaaatgttttacttgaaaggaaattaaggtcccatgaggtaataaagggattgtggttaggagcttaccaacctgggggtcttagatatcattagattcccagttagatatcatttttgttttaaggggctggattccattttttgtcccttcaggggaaggatctaatgaagccaaagatcatggcagtataaatagcatgctttctttctactttgagatcaacaggccagattctatctctataaaagtttgggaggggtaacatggttttgtcaaggtaaccctgattttttttctgtgctctatctaaatagttaatcatatcaattatatagcttttacagtggcttgataattttggctgaactatatgacatcttcactttagggatatagggggtgggatctattcatgaaatgatgccaaaatgcagtgtgtaaacattgtcatgctcaactgtggccaacagcctgtagacagactattcttttatctacttaaaggacgggcagcatttggcagcagtttgattaaaatttagagctaaataggtaggtggagacccctttctctcaactacacttccgtagcctcgtctctctcatgacatcttttattcttccctccacatccaaattgtaaaaattgcttaggtaacgtaatctagtgacaatgtgcatgacttcttctcaaagagaaaggaaacccaatcaaatcaaaaggatagatatggtgtgctccaattaaataaaagccacttcttaaactttttgaatggtgttactttttggatagtgttaaggtccttagaacacacaaaaggaaaattaaatgtaactgctgaaacacagcagaaaagaccaaaaatgtcttagaaaaaatgctgaagagaggaggaagactgatttaaaaaggagaaattttttttaactgggaattttgagtcaactgagaagatgaaaggttggtagtttaaggttacacaaactgaagatcaatttgctgtttagttcaatatttataaagtgcactatgtgccaggcctgtcatccacttaataattacacaaatatttattgagaacctatactatgtttctgacactatgacaggcattaaggatatatggtaaacaaaacatctggtcattttacctctcctgaggctcttctgtctagaagtcctttgttaagtattgtctgatcctctctctcaaaaagcttaaagttcataggaaaaacaaacaccaaatagctatgatctcaggcagaatgggaaagatactaaaaaacataagaaaaaattaatatggtagtgctgagtacagaaatttttttccatgaagactagggagggtttcatggttctagtgctgtttgagctgggctctgaaggctgcatatgattttaataatttagaaagggaatagggagaggaaggcattccagtagagggatagtgtgggcaaaagctgaaatataaaacacagcgaatacttggaaaagtaaggatttatatgtgtctaaaacactgagtatgcatagggtgaagaaaagaaaacaatttccagattcagaggatcagaactccttagaagaatagatgttgatgatacatggtatgtgtgatccaatctcatgcaaacagtattttcaggggatcacttgagcagcgtgtagtgaaaatgttctccacccaaaaagtgaagtaaataaacatgaaatgcagccagctgaatgattgttcaactccttgcatttcggagtgggtcattctaacattggacagcatggattcccacgctccctgacagtggtcataggagggactttttggggccgctgaacctagaagactcttttcaagcaacccccccacactttttaaagtgttgaattccatctccttctcccgtaacgtcaggggcatacagactcagtgctggaccaagttgaggaacacctttcttcatttcctttcctctttagaacaaattggcaaaattctcgctcctcttccagagattcaagagattctggttgctatttatcttgtctagcaaggcattcacacttgccacgtttagcctatcaaatgttgccctaaatcctggcaaatattcatctagctcacacttttcgtgacacttttttttttttttttaagatggagtctcactctgtcacccaggctggagagctgtggcgccatctcagctcactgcaacctccgcctgctgggttgaagcaattctcctgcctcagcctccccagtaactaggattacaggtgcgcgccacaatgcccggctaatttttcatatttttagtagagatgaggtttcagcatgttggtcaggctggtatccaattcctgacctcaagtgatccacctgcctcggcctccctaagtgctgggattacaggcataagtcaccgcacccggcttcgtgacactctttatgtgagctgtgtgaaggtcacaagaaccagcagaagacctatctgtagctccaaatggaaaaaaccatgctcaaactgaaacagatttgactagataaagactcgatttccttttgcaataggatggttgagggcaggaataaagggactcaccacattgccttgtactgtctttgatgtggaacttctctcatctttcctctggactgtgagattctgtgctgaggggaccacattacatccctcatagtacctgatatgtagttgatgcccaacaaatatttattttaatatttataatcataatatttaatgtttttgttatattcttcaatgaaatgtctccaaatgttttcagtttatgaataatatactttaggcctcagagattcagctacagtaaatgttttcctgtggaggaagtacaagagtttgctatgaaaataaagttccctgtactaagatactttactctggatgtaaagatacttggctatttgttaggctgcttattcaacctgttattttaaagaaggaaaaaaaataagcacaaacaatacacttgtgcaacagtgataaaaaaatacactttcaaaactagagaaagattgggtgattcatttaactttctttcaacaccaatttctacacccagtgaaatctatgctagcttaaagaatgaaaaaatgctgggcacagtggctcacgcctgtaatcccagcactttgggaggtcgaggcaggtggatcttttgaggccaggtgttcgagaccagcctggccaacacggtgaaaccctgtccctactaaaaatacaaaaattagcccagtgtggtggcacgcacctgtaatcccagctactcaggaggctgagacatgagaattgcctgaactcgggaggtggaagttacagtgagccaagatagcgctactgcactccagcctgggtgacacagcaagactctgtctcaagaaaaaaaaagaaagaaaagaaaaagtcacataaaagtctttttttcaaaaaaggagaagagaaaattatgccaggtttcaaaatctcacctgtggaaatttgacccagaccttgtctttgggtaggactacatagtggttccaaccgtagactaataagagtcatggaatgtttacataaatgctgcgtgaatttcacaaccttccaccttttgaggtgctgccataacaaaattaggcacaaaaggggtgttttgcagacaatttgtggaagtattgacagagctgcagaggtatccttctcatttctgcatgccttaatccaggcccatttcttacattgcttagtgctcagtgtgttgttacaaagagcatgagctcagaacccaactgggaagactctaccagctgaagaaatgcctctgaagttaaccagtaaattttctcctctctcaggtcttttctccttacttcccatagaactgttcttagggaaggttgacataatcacatggttaaaatcccaagggactcaatattcctatactttaactgtatgtttttaaataaaaacttagagtagacttgccccctcggtttttcaaaaatctctgaattctccaaagtagaagctgtgcaatttatatccttaccagggagtgtttccaaaccattctcttgcaggcagtgttgaaagtaaggaagattggaacctgtctcagtaagaagctgagaggcttagagaaagttcctcaacacagcaaaacccaacattttaaaaacagaagcagaaacagttttataaaggcattgccacccccaccattgcacacaggctttgtttgttgttgtcagtaacattataagcactccatctttgggccttagttaatgctactactccaggttcctgcgttacccaagaaagttcctcccaaattgggagctgtaaccatctgttgatactcaaggctctccgaacagctatcactctaagagggtctcttatctgtgtttcagcaggatagaagcagacatccactgcctttggaaaaacatggggagttggagggacggatctatagcagcaactgcagcaatgaagacaggtcagttttacacgctagaaacagaaatgcccccagaaggttcaggatatgactggaaaacttgattgcatctaccttagtttgtacaagtggtgcatcttggaaaatagatttcctgaacagtttagatcaaaatggagctgacactcaggatctcctgtaatagtgacccacatgctttctatacatagcgcacatctatttgtccacagcccacattctgttttcttgctataatgtattctttgggtatggtgttggtgggtgatgggaaatattctgagccaaggcaagatgcttttcttaacagaaggtggttgtattgctaaggaaaaatgttcatgcaagtgatcaccaacctggagatgccccccaagtcccagatgatcaggtagctacaagtgtgaagagaggacacattaccaacccagagtttgaacatttagttaagctcagtaagatttagcatttctgtgaaaggaactacagtggaacttcaaccccgcttttctttatactagataaaggacccatcttcttaacctattggatttcattatttgcataactttttattgacccagtgtgccaataaacttgctgtttggtcggcatatcacaaattagtcaaatatgttgtttgatcgaatttatcaaagactttgagtggtagtcctatttcagtatggcttttgacctggttatgttgtattcttgcctcttgatgagaatgtattcatcagacatatttgatcggtgtgctaatgaggggtagaaattggttagggacagcgttaagactgtccttaacagttagtaaacatactaaacggaaagacaaggtggcaagcacactacattttccaaagctttacactggaaagcttaaatattaatagatattaaatatatattaaatagattttatgattaaaaataaaatggtttttttggtttctttcatctaaccattttgacaaattcagatacttttcacttaatatttgaatatataaatctaatttcttccatgttttctcccctctgaatcttctctttttttttttttttttttttgagacggagtctcgctctgtcgcccaggctggagtgcagtggcgggatctcggctcactgcaagctccgcctcctgggttcacgccattctcctgcctcagcctcccaagtagctgggactacaggcgcccgccactacgcccggctaattttttgtatttttagtagagacggggtttcaccgttttagctgggatggtctcgatctcctgacctcgtgatccgcccgcctcggcctcccaaagtgctgggattacaggcgtgagccaccgcgcccggccctctctctttagctcaccagttgaaagatatgtcagtcctatttttaaataagtaattacattagtgatatgtgtgcaatcatctttaagattaagagcaaattaacattggcttgtcagtctctcctcaaagctgttttccatctcaaaggtcgtgatccaaggtaaggtccagaaacaactgagattgttttacatctatgtactaggttggaacaaaagtaattgtggtttttgcctgcacttttaatggtaaaaaccgcaattactttttcagcaacctaataattacaattctaagtaatggagatacatatcttttataggcttcaatgagcaatacattagcataatgttttatttcatactgactttgaatattccttgtcaaaaatgcacttatactttggagttactatgtatgtttaggttactgtgttgtcatcagaaggctggagttatcatagcagagctttaatgacaaaatattatgagccttgtaaatagttttaaaaattgtccactaatatctatttgtcttgcaaaatttgcaattttactagtaattttcatcacttgctctttctacctctaatgtttctcagtctcctccattagatcttactgacttatcacatataaacaccttcctcagaaacagtccaataaaaattaaagaccaagaggtagaatctactggagccatcatgaattccagttctttttgttgttattgatttttcttttttttttttaaaaggcacacccttgacttttttttattgttaaaataaccagattctaatttcaggcagcaaaatcagttactgcaaaaagtcaataatcaaaaatcaatgtataattggttttcatcacctatagaattagtgaggtttatacccctcaagtgtttagtgattctattcagtcaacctaaaaaaaattgcctcttttctacttaaataaataatttatttatttattttgagacagagtttcgctctgttgcccaggccggagtgcagtggcacaatctcagctcactgcaacctccgcctcccaggtcaagcgattgattctcatgcctcagcctcccaaatagctgggattataggtgcccgccaccatgctcagctaatttttgtatttttagtagagatggcgtttcaccatgttggccaggctggtcttgaactgacctcaagtgatccgcccaccttggcctcccaaagtgtggggattactagtgtgagccaccacgcctggcctgcctgttttcattattacctgcctgttctcagtatgcaacatggcagtactattgacagtgaggtgctttggcatatcagataacttttccagttggtcaaggatcccttttctcttttcctcatttctgaactgcagaacaggaagtactaaagaagtggctcaggacaatgttgtcacatcaggagtggcagaggtgtttactaggattatgatcctttcagctgtgtgtcttagaaggatctcctgaagccctgggtttgatatagaaaccataagaaaaagacttggggcagttctatatctggctcttctcccacttctcccataaaagattaagaaaaactgatgggatgatttcagatgtttcattgccaccaaactacagccatgagttttttttctttaagtgatcttatgaggccagtaaaggcctctgtcttgattaatgatgatcatcctataatatctggatatggtggcttgacatgagttttcaacaaagaaaattagtctctgaaagacatttctcatctgaaactctcaatatattaaaatgcatttaaaagttacttctgggaaacatactaaataggccaatcagttaatcattagctaattgtcaaaccctataaaatcatggtataatgtcaccctgacataaagcaacatcaaaattagtgcatcatctataaagtgaagtattattttctcccaagtgacaaattctattgccaaaaaataccactgtacttctaataagtgacactcattttaatagaccctacaaaaatacaatattttcaatgtccccataaaacagttaacttacaaatattattctcagagctctggtgacatcattcagtgatactattgtgaaaatcctcatacaatacttgaaacactagcatgtaaagtaaattcattatataacaaaagaactatgtaaaattatgaaagataatgcatgcaaccaactccgggaaattatcctggaaattcaaattaatattgtaattaaattaatgactaatatgaaagataagtattttaaaggattataaaataaattttgatcatttatgcaggaaaatagtttcaatggaaaagtaaataattctacattaaccatgcttgtctttctcttcagtgaaaaagcattcaggattttacataccttgaaactgtttttggaaaaaaagtattttatctatttctgcccagaaaaacagccattgaaattaatgatacaggtagaccacagctctgagaaattatatttgaagtttcatatttaaataccaaggatttaaaatcacctaccataactttctaacagcagtctttcgtaatgataaattttatcaatttccaaaattcgttttaaataatttaaaaagcagcaaattagattaagcaacacacaaataaattccacatttacaagtaaagaaatcacaggggctacagtttataatcaacatgaacttgaaagaaataaagcaatacctttcctgccacccatcatccactgcttaaatttgtggtgaaaaagacttaactacaatgacctttagtctgtttctaaactctgcatgtattgtaattagctaaaggcattgaacaaattagttcatcctatttttatttgggtcccagagataaatggctaatttatgaaatatttcactctgtgtcatgagaatttagcaaatgaatatggaaccaaatataaacactttataccatatgtacagttactttcataaggcattatcatgtaatttttattgaaaaagattcaatatagtaaagtcttattttaagatatattttttctctatctgagatgtttagtttatgaaaatattgtttttctctatattctttttgtatatatgccaacatataccttgtgctagaaatattttatgggaattacaattctttatatttgtattttctatataaaggcatatacaactttgaggcagtgtttctgatggagagcagaattcataaagagcttgtgtgtgcttccgtgctccgaaattatatgaaatccattttgagaagaaacttatttgattaaaaacaaaaacaaaaacagaaacaaaactgcaccaatgcacagccagaggctgacaattaaaactaatacataaccacatgaacatcatatttatagagttaacattttttaaggatggtcagtgctaacatatagtattatacatttggcactaatgtttgccattggtccagcaattggcaaaatttgtttctatgtataaatttatttttgaacattaggtctggctagacgtatcttcactatttataaaaaatatttagacagtaagctcacgttgaataactaggtctactgtgttctggaaactcttcagtagtaatacagctttttcatgttccatatgtacaaaactgtgtccatttgcctgaaggatcttatcaccaggctgcagtaggtttgatgctggcccatcaggctgaaccctagtaacaaagatacccttgtcagaaggtttgaatggatttccttgtccactaattccaccactgatactaaatccaaggccaggattcttttctattctcacacaaaactgctctggatatccatccatactcctttgccctttagtttgaattaagcaccgtccaggctgaggtccccgggtggcctgtgaagaggggatctgaataggcaatggtgactgaaattgctggatggtcactttgtttatatttccttcatacggctgctgctcccggctgcgatgctgaaggctttgggaccccatcaacgtctggatgtggctgcctgccttcttagtaatggtgtccggaggtacatcccgcctcccaagtggataaggattccattggccactaggagatacatcttcttgtccattgtctaaaatgttgctttgctgggacggggtcctgtctaaccgtctagcttctatatgtctaagcagctgttgtctccagtctgcaggcattttaccacagctctcctctcccttcacaggagtaggcctcgtctttaaatcactgttatctgatggcttgtcaccatagttacccaagttatagtcagatggtattttttccaaaagagctgccatagtaggcctagctgaaactggcctggtttgggaggcaccgtaactctctgtactgtagcttctcgcagacaatggcctcctttgggtaaggtttttaaccggaaaacttcccgcctgagctttcacttcttgatatgaagggtgttcatcttcatacctgccattccttttcaggaactgggactcagtcactgtaacgctgctttggcgatccagccctcccctatatgggggtctgccgtacctatcagttgggggcagctcatgaggctcattgacccttctaaacatggccatttctgtggcgctcaccagggagtcggcccttctcaggaagcccgccctggccccttggcttgcgaactgggcattcaccacagcatcctcattcacagatggctgagaaaatgaaaacatttgctccatcggtgggtatcctctgtaagctctaggactaatcaaatccttggcgatgtttttgctggcctgttgcacgtactcgggattgtgttgaaaagggggtggtatcctcttttcggctttcacttccactgatccttgaggattgaagctttggtcaaactgatagactttttttgtcatagaagctttttgttgttgtggccccttactacttccgtaggtgagcatctcatcatccagcattgggactgactggcttcgagacatactggacataccatgctctggtcccagcatcttatccggtcgttcgtggcttcctaagtgatcactcccagaagcatagttttctaatggtatgttatacaccttatatgtaccaatgtcaatctcatcgatactctgtgactttttgaatttattagacttgatatctttcattaggggggaaagcctctctgtgcttttgctaattgaaataacacctttagaagattccgggcggcagtggatttgagaaaagacattactaagactcctgttgggattggaatcatgatactcccatggtacgcctggagaaaaaggactaggtatttcagtagattcctttatatgttctttcctttcaggcaatgggctggtagtgggggttgtctctaatttggaaggaaaagcggtcctgtcttcaaacggactaggggttctggtccaattctgccaaggattggaaggaggcacttctgtttctggtgtgtgtctgtgtgtagactgctcgagttccaggggaacaccaacaatcctgtcttgcctgatcaaaggcctgcgtccatgcgaagatgtgcttctagatttcgaacttaagagaggattactgttggcattctcggctgtggtttcctcagcaacaaaccctgtgttgtcataatgcgagccatcagtccagttgtcagtgaaagtatcactcatgggcagccggtcaggacgctgtggtatattgcctgggggaacagcctcccgctggctgagtaatggctttgaatcaagaggctgtgggaaagatggtgcaatcctgttaccccacaaagaattatgtactgcatctttagctgttgtctgcaaggaccccactttaacccgggtattagaggatcctgaggaagcctgggaaggcgagtagtctgagtaagtgcctgaggaaacactgttattcagacagtgagttttgtcaacttcagactcatcagttgattcttttttgtccttccctagcagaacaagtttgggtgggtacagaggggtctcagctaatgaagggtgaagttccccaatcctcatttcattagctggatgaacaaaagaatcctccactgtaatctcctttggggctaccggccacttgtgttcatatttttctttcacagtttgctccgtgttagcagttggatttgaattctcaacacgcactccatggcttggcttacccaccaaattttgaacagattttaccatattctttaaatcctctgggtaaggagttggatatcgttttaggtttatttcaacctgtctgccacttagagagggaagagtggtggattgtgctgcaactggcaatggagtacacatgctcctttcctgctggaggccacttatacaaccccatgccagctgtgggtcattctgggggacgggcatatcttggatctgctgatcacacctggcccatggtgtgcagcaatcgccagacagtctggcaggttggagagtaatcccacgctggcccctttcccagggggcttggcaggagagatccttaactttcccagcattttcgtcatcttcttttttgtcttcaaattcaaaggcaacagtcatgcgttgttgtctctgctcttcccacagtgtagggttaaagctgtcactgtctgactggaaatcttcatcaccacgaggctgctggggaaacatgtagttagtcaatactctttgctttgtttctggatgggcttctgtttgtaaagggataagggctttggactgattgtcagaaagccacaaagctgcaagctctttaagtttggtaaatgagaatggtaaattcttcaatctgttgtcactcaaatttaggactcttagtttctgcatctgtccaatctcttcaggaagaaattctaatttgttggagcgtagagacatgactgttacattcttacaacttccaatttctctgggtaattctggaaggaaattctcatcaactgctaatgtccgaagactatgaaggtagccaatagtagaaggtagtgactccagttcattacagctacagtcaaattcttctaataaagataaatttccaattgtattgggtagcattgtaagttgattgtcatctacttttagagttgttagttttttcaaaagtcctatagaatcaggcaattgttgcaacatattggatgacaataagaggtcctcaagggcttcacatccagaaatgtccatgtcaactgtttctattctgttttttgacatatccaggtataccaacatctttaacttccctatagacccaggtaacacttgtaatgcattattatccatccataactccctcaaattttgtatttgatccagaacttcaggcagctcaccgaattcattattgcctaggtcaagtctttccaactgggccagtttgtgcattgactttggtagagttttcaagtgattttctcttaactccaagatccgcaatttgacaagtcttccaaaattggctggaagaaattcaagaaaggcgtcattcaggtagagctgggtcaggtttaggagctgtgtgaagccatcaggtagtttagaaatgggattgacactggcttcaataattgttaaacacttacagcactttatgttttctggaaattcttgtacaccatttttactgatgtcgagttctttaagattaactaaactagcaatagtggttggcagatttgaaaggtcgttatcaggaatacttagttttcgtagagcttgacagttgaacaattgcttgggtagttcttcaatttgattggcatctagataaagctcctctaatgttcgttcgaagttaaagacctcctttggcacctgctgaagactgcagtgggagtaatctaaaactgagatgatttcttcttcacctcggaaacatcggcatggcaccagacggccgatgattttccgtttggtggtcatctccaggcactgcattgctagttattcctgtctctgcagacttctaggttgtgaccactttgacttgcattttttttcatgtagcgggctcactcctcttcaggcctcttccgaagtgctgcacgaacctctttacaaggacttctctggtattgcgggggattccttccccttattaggttctccatcatcgccggcgggagaaactgcccatgaggtttcggagagcgtagtcgtgcagctgccaagggttattccttaagtgttcaggggtccgcagtggagtgggcgccagggtcttcggaggagaagaggagggaaggagtagaaggtaggaagaacaggagatagaggggaatccaggaaggtgccacgttagaccatgatgccagtgcccttcaggtggacggctggagaggttcccgcgggaagcggctgaggggaagcccgaagcgccggcgggggaggcaggagcgcgtccactccccagcctcagcctgcccagcgcgccgcgctagcgaccgcagcagcagcggcggcggcggcggcggtggcggaggcgcagctccctccccgcccccagaaggctccacagacaataaatcctgggcggagaagagacaagcaggaaaggcgaatcctgcacccaactccgtaacaacccctgcccgttgccgcgcctgtgcagggcgaggatccccaggggccagggcgcagcgggcgtctcggaggggctgagcgctccgcaactgcaggaggcggtggcggtggcccgagtgggcggctgcaggtcccgccggcgagaacccgctgcactggggctgggtgtccgtggcttcaagcccggtgttcacccggagtagggtcctcctcggtgcagtggctcggcgcacaggtgccaggattggc

SEQ ID NO: 12394 - RNA, 20383 nt, Homo sapiens
  source 1..20383: mol_type = other RNA
ctgggaggtcaaggctgcagtgggccatgatcatgccactgcactccaacctgggtgacagagcaagaccctgtctcagaaaaaaaaaaaaaaaaaaaaaaaaggcattaaaaaagcaataaagcagaaagaaagcatttgccattttattaaactgtgagagaaggtgacaatacagtgttctttcctcatattttgtacctacacgatagcatttattagactttttgtgtgtctccccactagactgtgtttcttgaggggtaggaccatggcttatttatatcttccattgttcttataatagaattttgaacataaccccttgttcattaacatttgttgattaaattgaatgcacagtgagaaaaaggcaaattgttttaacagttaaataattttttaaaaaaggataaacatatagattggctagaggacaaaccttagaatggtccggaggcagacttacaagagaattacttaaacatctctcgattcaaacctacaggtctggatgaatactcaaaatataagtatatattttggggtataggtgaacctgcggggcatatttatggcaagaccaagcaaaagaagaaaatatagtcccttcactttgagtagtttatgatgacctagggccctaggtgacagggatagtaactatcattttttgggaaacgtggaaatgcaaaaaaaaaaaaaattgcctgataagatatatagacacacacacacacacacacacagacacacacacagacacacacagagagagagagatattaattcccaagtttgaatttctctgggaaatggccacaaagaaatgcctgaactgtttgctagcaacattcatggttttataaagaatatagcagtgatgtcctgctagaatatctgtcttgatcataatgagactgtgagaacctatcaagtgcaagatacccgttgcttagtcaaacgattctacaagtatggctgaagatttatatcccaaaactggctatcaaagatggctggtttaaaacaatcaagacagtatagacaaatattacagggcaagaatagtttggatgatgatatcctagagaaaaaatcacttttagagaatgggacttgttcactatctaacaactttctcttttacagattctagcttaatgatcatcaataaaagtgaagtcttgaatatgatggatattcacttatttgtcagggaggtgacacagttggacaagcagcacccttggagtcggggttggggaggagtgcgtgagatgtttcaaaaggatctcagtgcattttaagtgacagcttctcctgctctcttctcttcccacagctgctgggggtcctgcaccccaacccagcctagatgatatttccatttgttgtacctaaaagcagagctttttacatctttacatctttacctcatgacagaactaaaaaaatgatgtttgttctacagtatggcacggagatgggtaaaaaagtgaaaagaataagccacaagcccccgtgctttgaggagatgatcatagcctgctcctggggaactatgctagtggctggatagcaagcactgacctagaggttgctcctaggaataaaaaattaagattatccatagaagacaaagaaaaaaatacttcgctaatagtggataccaaaaatctgaggtagtgcaaaagaaaagaaaggaaaaaagaaataaaaagcgcaactggaatacatacatacaaactttcaagacgttttctcttatactcttcagtaaaattctatgtaattttcattctagtatttaaatagttctggattttacaactaaacctatcattaaaaggttatggaaaatagaaggaataaaaaagatgaaatagaacatcaggcaaatcaaaaactcaaaagctgtatccaaaacaatggtggacacctgccgtatttgctttaaaatgggtggcactgttgtgtacaatttaaatttgttaaggagatatttaacttctctgaaaagagaggaagaacacttggtaaacaaacccaaaatggtgcactaaaattggcaggcttgaggtcagaaagaacttacaaaatattaacccccaaagaaggttaaattgaatttgctaagaaagagtattctgtattagtatctggtgatcatgtggctagaaggaaattgttttttttggaggaaaacaccagaggatataaatggcttcacataaactttgggaaagaacaccttgtcttccctctacctttgctccgggttggaagaaaaaaagattaaatggttggcaggggaacacctgaaacccatataagtagggctttgatggaattagcaaagaagaagctcagaccaggaggctggctaagctgtgagggtgaggatataattagcttagaggaagtaaacaaaaacatttggcctttttagcaatgatccagccatcagaggccctggaatttcaaatgactaagaagaaccaaaatagcttgaggacacatgtcaccaaggccgccaggggttctctgccttcagcacccagatattcccactgaaaggagagaggctggggagattgcaaactaccttgggaatccaatgatcactttgtgagagacattttgaaatacatttcgaaatacatttcttattcacttcataataaaataaaatctgattgtcatattatgctgattactcatacacataaataaaatgaaaaattaggcgtttattgtagatgcctagttattgccagatggaaataaagctatacccagatgcacacatattcagattggactagttttagaattacataaagaaggctaggcaaacttaaccacagttcctgatgtttaagttttggaaagttaactttaaaaataaattttgagtaacttgagacaaatctattcccacatacttggaatgggcatacctgaaggaagtgtggctaaaataatgggagataggagcaaaatatttggaaaacacaagttagagaagaactattaaactggtgggtataataattaaactgaacaattaaggaacatcaaaactttaaacaatcaagcctcactgagaaagtggtttctgtctcattaggttttgggtgattgatacaatctgagaggtttagtaaaaaaacatataaactgcctaaaataagctcaaagctcttgtttttttcttaaattgtgtaaatttagagcattgtttcaaattttctcaaaggagaaaggaaaggggtgttgttagcaattgtatcagcacaaggggcataaaaacagactgtgtaaggccatcccagcactttgggaggccgaggcggtcggatcgatagagcccaggtgttcaagaccagcctgggcaacatggagaaaacctgtctttactaaaaatacaaaaattagccgggcgtggtggtgcatgcctgtagtcccagctactcgggaggctgaggcaggaaaatcgtttgaacccaggaggtggaggttgcagtgagccgagatcgcgccactgcactccagcctgggcgacagagcgacactgtctcaatacaaacaaacaaaaaacacccacgacaacaacaaaaatcggactgtgctcccccaagccagagaattgccaaggctgggatttaaaatgtagatatgaggtctccatctagtggtggctcttctgaactgcagacacatgtttctttaaaagagtatgcggatgtgtacaactaaatatgaggatagtatttgtcagagttgaacgcagtaatttaaactagaggattttattgagatgaaacacaatttgttgctttataagggtgggttacagagggaaatgttcaccccttcgctccaggaatttaagaatagcatgaatccttccctgaagatagacaaatgaaccagatcctctcaaggtccctttctgtcttatgataggacaataattttgctcctttctccacagagcttttacctgtagccacactgtctgacattagtctttatttaagaaaagtacggccgggcgcggtgtctcacgcctgtaatccccgtactttgggagtccgaggcaggtggatcacgaggtcaggagttcaagaccaacctggccaagaaggtgaaactccgtctctactaaaaatacaaaaaattagccgggtgcagtggcaggcgcctgtaatcccagctactcgggaggctgaggcaggagaatcgcttgaactcggagggcggaggttgcagtaagctgagatcgtgccactgcactccagcctccagcctgatgacagagtgagactccgtctcaaaaaaaaaaaaaaaaaaaaaaaaaagaaaagaaaagaaaagaaaaaagaaaagtactctggtaatttttaaaaatgagataacttttttccttgttctgagaagttgtatgactaaagcattacctatgacgttagacaaaaatagtttctagaaatgaatagcaattaaactaaatatatttctaatatgcaccttatttttcactgtaaattcttcttttgacatctggaagagcaggagggaaggcagaaaccaagaagagctgaacgattactcctctggccaagagagagcagagagagaggaagggaattcagggctgtctgaagaaggggcatggtcaccagaacgaagagactggaggatatgcctgaatctgatttcttttatccagttcctctctgattctctgtatcagtcctctattgcccttcttttgtctttctcattctttcttccttaataacttattaattcccctctttcccagccctagtctgttcttgttccttactcactcattattctcattattctaaaatgctcttacttaaaaatatttcattaaagtactcttactattctaaaatattcttactatcctaagataatgtcactctctcaattaatatttcacttttccagttcatttttcatttatttttgttcaaagagacattggcattcttttacccatgtaaatgtatagacactgggctataagataccaaagagtaggcccctggagagtttgaggcatcatgctatcaaagacagcaatggtggctgtttccttcaagatatactatgactttatctaaatctttctaaatcaaaaattttatgagaagaagacataattaacttgatagttatcaagttctctttatacaaagaaattaaaaagcagaggtagaataagagtaattaatattaatagtataagtaaaagagtcaatgacaaaacatttaatgtttcggaatatttcactcaattctggagttacttagctatgaaacccaaatagaaagacatgggaaatagttttgtgagaaagctaggacagaaatgttttacttgaaaggaaattaaggtcccatgaggtaataaagggattgtggttaggagcttaccaacctgggggtcttagatatcattagattcccagttagatatcatttttgttttaaggggctggattccattttttgtcccttcaggggaaggatctaatgaagccaaagatcatggcagtataaatagcatgctttctttctactttgagatcaacaggccagattctatctctataaaagtttgggaggggtaacatggttttgtcaaggtaaccctgattttttttctgtgctctatctaaatagttaatcatatcaattatatagcttttacagtggcttgataattttggctgaactatatgacatcttcactttagggatatagggggtgggatctattcatgaaatgatgccaaaatgcagtgtgtaaacattgtcatgctcaactgtggccaacagcctgtagacagactattcttttatctacttaaaggacgggcagcatttggcagcagtttgattaaaatttagagctaaataggtaggtggagacccctttctctcaactacacttccgtagcctcgtctctctcatgacatcttttattcttccctccacatccaaattgtaaaaattgcttaggtaacgtaatctagtgacaatgtgcatgacttcttctcaaagagaaaggaaacccaatcaaatcaaaaggatagatatggtgtgctccaattaaataaaagccacttcttaaactttttgaatggtgttactttttggatagtgttaaggtccttagaacacacaaaaggaaaattaaatgtaactgctgaaacacagcagaaaagaccaaaaatgtcttagaaaaaatgctgaagagaggaggaagactgatttaaaaaggagaaattttttttaactgggaattttgagtcaactgagaagatgaaaggttggtagtttaaggttacacaaactgaagatcaatttgctgtttagttcaatatttataaagtgcactatgtgccaggcctgtcatccacttaataattacacaaatatttattgagaacctatactatgtttctgacactatgacaggcattaaggatatatggtaaacaaaacatctggtcattttacctctcctgaggctcttctgtctagaagtcctttgttaagtattgtctgatcctctctctcaaaaagcttaaagttcataggaaaaacaaacaccaaatagctatgatctcaggcagaatgggaaagatactaaaaaacataagaaaaaattaatatggtagtgctgagtacagaaatttttttccatgaagactagggagggtttcatggttctagtgctgtttgagctgggctctgaaggctgcatatgattttaataatttagaaagggaatagggagaggaaggcattccagtagagggatagtgtgggcaaaagctgaaatataaaacacagcgaatacttggaaaagtaaggatttatatgtgtctaaaacactgagtatgcatagggtgaagaaaagaaaacaatttccagattcagaggatcagaactccttagaagaatagatgttgatgatacatggtatgtgtgatccaatctcatgcaaacagtattttcaggggatcacttgagcagcgtgtagtgaaaatgttctccacccaaaaagtgaagtaaataaacatgaaatgcagccagctgaatgattgttcaactccttgcatttcggagtgggtcattctaacattggacagcatggattcccacgctccctgacagtggtcataggagggactttttggggccgctgaacctagaagactcttttcaagcaacccccccacactttttaaagtgttgaattccatctccttctcccgtaacgtcaggggcatacagactcagtgctggaccaagttgaggaacacctttcttcatttcctttcctctttagaacaaattggcaaaattctcgctcctcttccagagattcaagagattctggttgctatttatcttgtctagcaaggcattcacacttgccacgtttagcctatcaaatgttgccctaaatcctggcaaatattcatctagctcacacttttcgtgacacttttttttttttttttaagatggagtctcactctgtcacccaggctggagagctgtggcgccatctcagctcactgcaacctccgcctgctgggttgaagcaattctcctgcctcagcctccccagtaactaggattacaggtgcgcgccacaatgcccggctaatttttcatatttttagtagagatgaggtttcagcatgttggtcaggctggtatccaattcctgacctcaagtgatccacctgcctcggcctccctaagtgctgggattacaggcataagtcaccgcacccggcttcgtgacactctttatgtgagctgtgtgaaggtcacaagaaccagcagaagacctatctgtagctccaaatggaaaaaaccatgctcaaactgaaacagatttgactagataaagactcgatttccttttgcaataggatggttgagggcaggaataaagggactcaccacattgccttgtactgtctttgatgtggaacttctctcatctttcctctggactgtgagattctgtgctgaggggaccacattacatccctcatagtacctgatatgtagttgatgcccaacaaatatttattttaatatttataatcataatatttaatgtttttgttatattcttcaatgaaatgtctccaaatgttttcagtttatgaataatatactttaggcctcagagattcagctacagtaaatgttttcctgtggaggaagtacaagagtttgctatgaaaataaagttccctgtactaagatactttactctggatgtaaagatacttggctatttgttaggctgcttattcaacctgttattttaaagaaggaaaaaaaataagcacaaacaatacacttgtgcaacagtgataaaaaaatacactttcaaaactagagaaagattgggtgattcatttaactttctttcaacaccaatttctacacccagtgaaatctatgctagcttaaagaatgaaaaaatgctgggcacagtggctcacgcctgtaatcccagcactttgggaggtcgaggcaggtggatcttttgaggccaggtgttcgagaccagcctggccaacacggtgaaaccctgtccctactaaaaatacaaaaattagcccagtgtggtggcacgcacctgtaatcccagctactcaggaggctgagacatgagaattgcctgaactcgggaggtggaagttacagtgagccaagatagcgctactgcactccagcctgggtgacacagcaagactctgtctcaagaaaaaaaaagaaagaaaagaaaaagtcacataaaagtctttttttcaaaaaaggagaagagaaaattatgccaggtttcaaaatctcacctgtggaaatttgacccagaccttgtctttgggtaggactacatagtggttccaaccgtagactaataagagtcatggaatgtttacataaatgctgcgtgaatttcacaaccttccaccttttgaggtgctgccataacaaaattaggcacaaaaggggtgttttgcagacaatttgtggaagtattgacagagctgcagaggtatccttctcatttctgcatgccttaatccaggcccatttcttacattgcttagtgctcagtgtgttgttacaaagagcatgagctcagaacccaactgggaagactctaccagctgaagaaatgcctctgaagttaaccagtaaattttctcctctctcaggtcttttctccttacttcccatagaactgttcttagggaaggttgacataatcacatggttaaaatcccaagggactcaatattcctatactttaactgtatgtttttaaataaaaacttagagtagacttgccccctcggtttttcaaaaatctctgaattctccaaagtagaagctgtgcaatttatatccttaccagggagtgtttccaaaccattctcttgcaggcagtgttgaaagtaaggaagattggaacctgtctcagtaagaagctgagaggcttagagaaagttcctcaacacagcaaaacccaacattttaaaaacagaagcagaaacagttttataaaggcattgccacccccaccattgcacacaggctttgtttgttgttgtcagtaacattataagcactccatctttgggccttagttaatgctactactccaggttcctgcgttacccaagaaagttcctcccaaattgggagctgtaaccatctgttgatactcaaggctctccgaacagctatcactctaagagggtctcttatctgtgtttcagcaggatagaagcagacatccactgcctttggaaaaacatggggagttggagggacggatctatagcagcaactgcagcaatgaagacaggtcagttttacacgctagaaacagaaatgcccccagaaggttcaggatatgactggaaaacttgattgcatctaccttagtttgtacaagtggtgcatcttggaaaatagatttcctgaacagtttagatcaaaatggagctgacactcaggatctcctgtaatagtgacccacatgctttctatacatagcgcacatctatttgtccacagcccacattctgttttcttgctataatgtattctttgggtatggtgttggtgggtgatgggaaatattctgagccaaggcaagatgcttttcttaacagaaggtggttgtattgctaaggaaaaatgttcatgcaagtgatcaccaacctggagatgccccccaagtcccagatgatcaggtagctacaagtgtgaagagaggacacattaccaacccagagtttgaacatttagttaagctcagtaagatttagcatttctgtgaaaggaactacagtggaacttcaaccccgcttttctttatactagataaaggacccatcttcttaacctattggatttcattatttgcataactttttattgacccagtgtgccaataaacttgctgtttggtcggcatatcacaaattagtcaaatatgttgtttgatcgaatttatcaaagactttgagtggtagtcctatttcagtatggcttttgacctggttatgttgtattcttgcctcttgatgagaatgtattcatcagacatatttgatcggtgtgctaatgaggggtagaaattggttagggacagcgttaagactgtccttaacagttagtaaacatactaaacggaaagacaaggtggcaagcacactacattttccaaagctttacactggaaagcttaaatattaatagatattaaatatatattaaatagattttatgattaaaaataaaatggtttttttggtttctttcatctaaccattttgacaaattcagatacttttcacttaatatttgaatatataaatctaatttcttccatgttttctcccctctgaatcttctctttttttttttttttttttttgagacggagtctcgctctgtcgcccaggctggagtgcagtggcgggatctcggctcactgcaagctccgcctcctgggttcacgccattctcctgcctcagcctcccaagtagctgggactacaggcgcccgccactacgcccggctaattttttgtatttttagtagagacggggtttcaccgttttagctgggatggtctcgatctcctgacctcgtgatccgcccgcctcggcctcccaaagtgctgggattacaggcgtgagccaccgcgcccggccctctctctttagctcaccagttgaaagatatgtcagtcctatttttaaataagtaattacattagtgatatgtgtgcaatcatctttaagattaagagcaaattaacattggcttgtcagtctctcctcaaagctgttttccatctcaaaggtcgtgatccaaggtaaggtccagaaacaactgagattgttttacatctatgtactaggttggaacaaaagtaattgtggtttttgcctgcacttttaatggtaaaaaccgcaattactttttcagcaacctaataattacaattctaagtaatggagatacatatcttttataggcttcaatgagcaatacattagcataatgttttatttcatactgactttgaatattccttgtcaaaaatgcacttatactttggagttactatgtatgtttaggttactgtgttgtcatcagaaggctggagttatcatagcagagctttaatgacaaaatattatgagccttgtaaatagttttaaaaattgtccactaatatctatttgtcttgcaaaatttgcaattttactagtaattttcatcacttgctctttctacctctaatgtttctcagtctcctccattagatcttactgacttatcacatataaacaccttcctcagaaacagtccaataaaaattaaagaccaagaggtagaatctactggagccatcatgaattccagttctttttgttgttattgatttttcttttttttttttaaaaggcacacccttgacttttttttattgttaaaataaccagattctaatttcaggcagcaaaatcagttactgcaaaaagtcaataatcaaaaatcaatgtataattggttttcatcacctatagaattagtgaggtttatacccctcaagtgtttagtgattctattcagtcaacctaaaaaaaattgcctcttttctacttaaataaataatttatttatttattttgagacagagtttcgctctgttgcccaggccggagtgcagtggcacaatctcagctcactgcaacctccgcctcccaggtcaagcgattgattctcatgcctcagcctcccaaatagctgggattataggtgcccgccaccatgctcagctaatttttgtatttttagtagagatggcgtttcaccatgttggccaggctggtcttgaactgacctcaagtgatccgcccaccttggcctcccaaagtgtggggattactagtgtgagccaccacgcctggcctgcctgttttcattattacctgcctgttctcagtatgcaacatggcagtactattgacagtgaggtgctttggcatatcagataacttttccagttggtcaaggatcccttttctcttttcctcatttctgaactgcagaacaggaagtactaaagaagtggctcaggacaatgttgtcacatcaggagtggcagaggtgtttactaggattatgatcctttcagctgtgtgtcttagaaggatctcctgaagccctgggtttgatatagaaaccataagaaaaagacttggggcagttctatatctggctcttctcccacttctcccataaaagattaagaaaaactgatgggatgatttcagatgtttcattgccaccaaactacagccatgagttttttttctttaagtgatcttatgaggccagtaaaggcctctgtcttgattaatgatgatcatcctataatatctggatatggtggcttgacatgagttttcaacaaagaaaattagtctctgaaagacatttctcatctgaaactctcaatatattaaaatgcatttaaaagttacttctgggaaacatactaaataggccaatcagttaatcattagctaattgtcaaaccctataaaatcatggtataatgtcaccctgacataaagcaacatcaaaattagtgcatcatctataaagtgaagtattattttctcccaagtgacaaattctattgccaaaaaataccactgtacttctaataagtgacactcattttaatagaccctacaaaaatacaatattttcaatgtccccataaaacagttaacttacaaatattattctcagagctctggtgacatcattcagtgatactattgtgaaaatcctcatacaatacttgaaacactagcatgtaaagtaaattcattatataacaaaagaactatgtaaaattatgaaagataatgcatgcaaccaactccgggaaattatcctggaaattcaaattaatattgtaattaaattaatgactaatatgaaagataagtattttaaaggattataaaataaattttgatcatttatgcaggaaaatagtttcaatggaaaagtaaataattctacattaaccatgcttgtctttctcttcagtgaaaaagcattcaggattttacataccttgaaactgtttttggaaaaaaagtattttatctatttctgcccagaaaaacagccattgaaattaatgatacaggtagaccacagctctgagaaattatatttgaagtttcatatttaaataccaaggatttaaaatcacctaccataactttctaacagcagtctttcgtaatgataaattttatcaatttccaaaattcgttttaaataatttaaaaagcagcaaattagattaagcaacacacaaataaattccacatttacaagtaaagaaatcacaggggctacagtttataatcaacatgaacttgaaagaaataaagcaatacctttcctgccacccatcatccactgcttaaatttgtggtgaaaaagacttaactacaatgacctttagtctgtttctaaactctgcatgtattgtaattagctaaaggcattgaacaaattagttcatcctatttttatttgggtcccagagataaatggctaatttatgaaatatttcactctgtgtcatgagaatttagcaaatgaatatggaaccaaatataaacactttataccatatgtacagttactttcataaggcattatcatgtaatttttattgaaaaagattcaatatagtaaagtcttattttaagatatattttttctctatctgagatgtttagtttatgaaaatattgtttttctctatattctttttgtatatatgccaacatataccttgtgctagaaatattttatgggaattacaattctttatatttgtattttctatataaaggcatatacaactttgaggcagtgtttctgatggagagcagaattcataaagagcttgtgtgtgcttccgtgctccgaaattatatgaaatccattttgagaagaaacttatttgattaaaaacaaaaacaaaaacagaaacaaaactgcaccaatgcacagccagaggctgacaattaaaactaatacataaccacatgaacatcatatttatagagttaacattttttaaggatggtcagtgctaacatatagtattatacatttggcactaatgtttgccattggtccagcaattggcaaaatttgtttctatgtataaatttatttttgaacattaggtctggctagacgtatcttcactatttataaaaaatatttagacagtaagctcacgttgaataactaggtctactgtgttctggaaactcttcagtagtaatacagctttttcatgttccatatgtacaaaactgtgtccatttgcctgaaggatcttatcaccaggctgcagtaggtttgatgctggcccatcaggctgaaccctagtaacaaagatacccttgtcagaaggtttgaatggatttccttgtccactaattccaccactgatactaaatccaaggccaggattcttttctattctcacacaaaactgctctggatatccatccatactcctttgccctttagtttgaattaagcaccgtccaggctgaggtccccgggtggcctgtgaagaggggatctgaataggcaatggtgactgaaattgctggatggtcactttgtttatatttccttcatacggctgctgctcccggctgcgatgctgaaggctttgggaccccatcaacgtctggatgtggctgcctgccttcttagtaatggtgtccggaggtacatcccgcctcccaagtggataaggattccattggccactaggagatacatcttcttgtccattgtctaaaatgttgctttgctgggacggggttttctgaagaggtagttcttgatgatcaaatttagacttagtctgcaagtttaaagtcatgcttctgcctgcatgcattgctgaaatacctccatagggcagcatgccaaggttaactgtattgtgtttgtaagcagcattcctgtctaaccgtctagcttctatatgtctaagcagctgttgtctccagtctgcaggcattttaccacagctctcctctcccttcacaggagtaggcctcgtctttaaatcactgttatctgatggcttgtcaccatagttacccaagttatagtcagatggtattttttccaaaagagctgccatagtaggcctagctgaaactggcctggtttgggaggcaccgtaactctctgtactgtagcttctcgcagacaatggcctcctttgggtaaggtttttaaccggaaaacttcccgcctgagctttcacttcttgatatgaagggtgttcatcttcatacctgccattccttttcaggaactgggactcagtcactgtaacgctgctttggcgatccagccctcccctatatgggggtctgccgtacctatcagttgggggcagctcatgaggctcattgacccttctaaacatggccatttctgtggcgctcaccagggagtcggcccttctcaggaagcccgccctggccccttggcttgcgaactgggcattcaccacagcatcctcattcacagatggctgagaaaatgaaaacatttgctccatcggtgggtatcctctgtaagctctaggactaatcaaatccttggcgatgtttttgctggcctgttgcacgtactcgggattgtgttgaaaagggggtggtatcctcttttcggctttcacttccactgatccttgaggattgaagctttggtcaaactgatagactttttttgtcatagaagctttttgttgttgtggccccttactacttccgtaggtgagcatctcatcatccagcattgggactgactggcttcgagacatactggacataccatgctctggtcccagcatcttatccggtcgttcgtggcttcctaagtgatcactcccagaagcatagttttctaatggtatgttatacaccttatatgtaccaatgtcaatctcatcgatactctgtgactttttgaatttattagacttgatatctttcattaggggggaaagcctctctgtgcttttgctaattgaaataacacctttagaagattccgggcggcagtggatttgagaaaagacattactaagactcctgttgggattggaatcatgatactcccatggtacgcctggagaaaaaggactaggtatttcagtagattcctttatatgttctttcctttcaggcaatgggctggtagtgggggttgtctctaatttggaaggaaaagcggtcctgtcttcaaacggactaggggttctggtccaattctgccaaggattggaaggaggcacttctgtttctggtgtgtgtctgtgtgtagactgctcgagttccaggggaacaccaacaatcctgtcttgcctgatcaaaggcctgcgtccatgcgaagatgtgcttctagatttcgaacttaagagaggattactgttggcattctcggctgtggtttcctcagcaacaaaccctgtgttgtcataatgcgagccatcagtccagttgtcagtgaaagtatcactcatgggcagccggtcaggacgctgtggtatattgcctgggggaacagcctcccgctggctgagtaatggctttgaatcaagaggctgtgggaaagatggtgcaatcctgttaccccacaaagaattatgtactgcatctttagctgttgtctgcaaggaccccactttaacccgggtattagaggatcctgaggaagcctgggaaggcgagtagtctgagtaagtgcctgaggaaacactgttattcagacagtgagttttgtcaacttcagactcatcagttgattcttttttgtccttccctagcagaacaagtttgggtgggtacagaggggtctcagctaatgaagggtgaagttccccaatcctcatttcattagctggatgaacaaaagaatcctccactgtaatctcctttggggctaccggccacttgtgttcatatttttctttcacagtttgctccgtgttagcagttggatttgaattctcaacacgcactccatggcttggcttacccaccaaattttgaacagattttaccatattctttaaatcctctgggtaaggagttggatatcgttttaggtttatttcaacctgtctgccacttagagagggaagagtggtggattgtgctgcaactggcaatggagtacacatgctcctttcctgctggaggccacttatacaaccccatgccagctgtgggtcattctgggggacgggcatatcttggatctgctgatcacacctggcccatggtgtgcagcaatcgccagacagtctggcaggttggagagtaatcccacgctggcccctttcccagggggcttggcaggagagatccttaactttcccagcattttcgtcatcttcttttttgtcttcaaattcaaaggcaacagtcatgcgttgttgtctctgctcttcccacagtgtagggttaaagctgtcactgtctgactggaaatcttcatcaccacgaggctgctggggaaacatgtagttagtcaatactctttgctttgtttctggatgggcttctgtttgtaaagggataagggctttggactgattgtcagaaagccacaaagctgcaagctctttaagtttggtaaatgagaatggtaaattcttcaatctgttgtcactcaaatttaggactcttagtttctgcatctgtccaatctcttcaggaagaaattctaatttgttggagcgtagagacatgactgttacattcttacaacttccaatttctctgggtaattctggaaggaaattctcatcaactgctaatgtccgaagactatgaaggtagccaatagtagaaggtagtgactccagttcattacagctacagtcaaattcttctaataaagataaatttccaattgtattgggtagcattgtaagttgattgtcatctacttttagagttgttagttttttcaaaagtcctatagaatcaggcaattgttgcaacatattggatgacaataagaggtcctcaagggcttcacatccagaaatgtccatgtcaactgtttctattctgttttttgacatatccaggtataccaacatctttaacttccctatagacccaggtaacacttgtaatgcattattatccatccataactccctcaaattttgtatttgatccagaacttcaggcagctcaccgaattcattattgcctaggtcaagtctttccaactgggccagtttgtgcattgactttggtagagttttcaagtgattttctcttaactccaagatccgcaatttgacaagtcttccaaaattggctggaagaaattcaagaaaggcgtcattcaggtagagctgggtcaggtttaggagctgtgtgaagccatcaggtagtttagaaatgggattgacactggcttcaataattgttaaacacttacagcactttatgttttctggaaattcttgtacaccatttttactgatgtcgagttctttaagattaactaaactagcaatagtggttggcagatttgaaaggtcgttatcaggaatacttagttttcgtagagcttgacagttgaacaattgcttgggtagttcttcaatttgattggcatctagataaagctcctctaatgttcgttcgaagttaaagacctcctttggcacctgctgaagactgcagtgggagtaatctaaaactgagatgatttcttcttcacctcggaaacatcggcatggcaccagacggccgatgattttccgtttggtggtcatctccaggcactgcaactcctcttcaggcctcttccgaagtgctgcacgaacctctttacaaggacttctctggtattgcgggggattccttccccttattaggttctccatcatcgccggcgggagaaactgcccatgaggtttcggagagcgtagtcgtgcagctgccaagggttattccttaagtgttcaggggtccgcagtggagtgggcgccagggtcttcggaggagaagaggagggaaggagtagaaggtaggaagaacaggagatagaggggaatccaggaaggtgccacgttagaccatgatgccagtgcccttcaggtggacggctggagaggttcccgcgggaagcggctgaggggaagcccgaagcgccggcgggggaggcaggagcgcgtccactccccagcctcagcctgcccagcgcgccgcgctagcgaccgcagcagcagcggcggcggcggcggcggtggcggaggcgcagctccctccccgcccccagaaggctccacagacaataaatcctgggcggagaagagacaagcaggaaaggcgaatcctgcacccaactccgtaacaacccctgcccgttgccgcgcctgtgcagggcgaggatccccaggggccagggcgcagcgggcgtctcggaggggctgagcgctccgcaactgcaggaggcggtggcggtggcccgagtgggcggctgcaggtcccgccggcgagaacccgctgcactggggctgggtgtccgtggcttcaagcccggtgttcacccggagtagggtcctcctcggtgcagtggctcggcgcacaggtgccaggattggc

SEQ ID NO: 12395 - RNA, 19573 nt, Homo sapiens
  source 1..19573: mol_type = other RNA
ctgggaggtcaaggctgcagtgggccatgatcatgccactgcactccaacctgggtgacagagcaagaccctgtctcagaaaaaaaaaaaaaaaaaaaaaaaaggcattaaaaaagcaataaagcagaaagaaagcatttgccattttattaaactgtgagagaaggtgacaatacagtgttctttcctcatattttgtacctacacgatagcatttattagactttttgtgtgtctccccactagactgtgtttcttgaggggtaggaccatggcttatttatatcttccattgttcttataatagaattttgaacataaccccttgttcattaacatttgttgattaaattgaatgcacagtgagaaaaaggcaaattgttttaacagttaaataattttttaaaaaaggataaacatatagattggctagaggacaaaccttagaatggtccggaggcagacttacaagagaattacttaaacatctctcgattcaaacctacaggtctggatgaatactcaaaatataagtatatattttggggtataggtgaacctgcggggcatatttatggcaagaccaagcaaaagaagaaaatatagtcccttcactttgagtagtttatgatgacctagggccctaggtgacagggatagtaactatcattttttgggaaacgtggaaatgcaaaaaaaaaaaaaattgcctgataagatatatagacacacacacacacacacacacagacacacacacagacacacacagagagagagagatattaattcccaagtttgaatttctctgggaaatggccacaaagaaatgcctgaactgtttgctagcaacattcatggttttataaagaatatagcagtgatgtcctgctagaatatctgtcttgatcataatgagactgtgagaacctatcaagtgcaagatacccgttgcttagtcaaacgattctacaagtatggctgaagatttatatcccaaaactggctatcaaagatggctggtttaaaacaatcaagacagtatagacaaatattacagggcaagaatagtttggatgatgatatcctagagaaaaaatcacttttagagaatgggacttgttcactatctaacaactttctcttttacagattctagcttaatgatcatcaataaaagtgaagtcttgaatatgatggatattcacttatttgtcagggaggtgacacagttggacaagcagcacccttggagtcggggttggggaggagtgcgtgagatgtttcaaaaggatctcagtgcattttaagtgacagcttctcctgctctcttctcttcccacagctgctgggggtcctgcaccccaacccagcctagatgatatttccatttgttgtacctaaaagcagagctttttacatctttacatctttacctcatgacagaactaaaaaaatgatgtttgttctacagtatggcacggagatgggtaaaaaagtgaaaagaataagccacaagcccccgtgctttgaggagatgatcatagcctgctcctggggaactatgctagtggctggatagcaagcactgacctagaggttgctcctaggaataaaaaattaagattatccatagaagacaaagaaaaaaatacttcgctaatagtggataccaaaaatctgaggtagtgcaaaagaaaagaaaggaaaaaagaaataaaaagcgcaactggaatacatacatacaaactttcaagacgttttctcttatactcttcagtaaaattctatgtaattttcattctagtatttaaatagttctggattttacaactaaacctatcattaaaaggttatggaaaatagaaggaataaaaaagatgaaatagaacatcaggcaaatcaaaaactcaaaagctgtatccaaaacaatggtggacacctgccgtatttgctttaaaatgggtggcactgttgtgtacaatttaaatttgttaaggagatatttaacttctctgaaaagagaggaagaacacttggtaaacaaacccaaaatggtgcactaaaattggcaggcttgaggtcagaaagaacttacaaaatattaacccccaaagaaggttaaattgaatttgctaagaaagagtattctgtattagtatctggtgatcatgtggctagaaggaaattgttttttttggaggaaaacaccagaggatataaatggcttcacataaactttgggaaagaacaccttgtcttccctctacctttgctccgggttggaagaaaaaaagattaaatggttggcaggggaacacctgaaacccatataagtagggctttgatggaattagcaaagaagaagctcagaccaggaggctggctaagctgtgagggtgaggatataattagcttagaggaagtaaacaaaaacatttggcctttttagcaatgatccagccatcagaggccctggaatttcaaatgactaagaagaaccaaaatagcttgaggacacatgtcaccaaggccgccaggggttctctgccttcagcacccagatattcccactgaaaggagagaggctggggagattgcaaactaccttgggaatccaatgatcactttgtgagagacattttgaaatacatttcgaaatacatttcttattcacttcataataaaataaaatctgattgtcatattatgctgattactcatacacataaataaaatgaaaaattaggcgtttattgtagatgcctagttattgccagatggaaataaagctatacccagatgcacacatattcagattggactagttttagaattacataaagaaggctaggcaaacttaaccacagttcctgatgtttaagttttggaaagttaactttaaaaataaattttgagtaacttgagacaaatctattcccacatacttggaatgggcatacctgaaggaagtgtggctaaaataatgggagataggagcaaaatatttggaaaacacaagttagagaagaactattaaactggtgggtataataattaaactgaacaattaaggaacatcaaaactttaaacaatcaagcctcactgagaaagtggtttctgtctcattaggttttgggtgattgatacaatctgagaggtttagtaaaaaaacatataaactgcctaaaataagctcaaagctcttgtttttttcttaaattgtgtaaatttagagcattgtttcaaattttctcaaaggagaaaggaaaggggtgttgttagcaattgtatcagcacaaggggcataaaaacagactgtgtaaggccatcccagcactttgggaggccgaggcggtcggatcgatagagcccaggtgttcaagaccagcctgggcaacatggagaaaacctgtctttactaaaaatacaaaaattagccgggcgtggtggtgcatgcctgtagtcccagctactcgggaggctgaggcaggaaaatcgtttgaacccaggaggtggaggttgcagtgagccgagatcgcgccactgcactccagcctgggcgacagagcgacactgtctcaatacaaacaaacaaaaaacacccacgacaacaacaaaaatcggactgtgctcccccaagccagagaattgccaaggctgggatttaaaatgtagatatgaggtctccatctagtggtggctcttctgaactgcagacacatgtttctttaaaagagtatgcggatgtgtacaactaaatatgaggatagtatttgtcagagttgaacgcagtaatttaaactagaggattttattgagatgaaacacaatttgttgctttataagggtgggttacagagggaaatgttcaccccttcgctccaggaatttaagaatagcatgaatccttccctgaagatagacaaatgaaccagatcctctcaaggtccctttctgtcttatgataggacaataattttgctcctttctccacagagcttttacctgtagccacactgtctgacattagtctttatttaagaaaagtacggccgggcgcggtgtctcacgcctgtaatccccgtactttgggagtccgaggcaggtggatcacgaggtcaggagttcaagaccaacctggccaagaaggtgaaactccgtctctactaaaaatacaaaaaattagccgggtgcagtggcaggcgcctgtaatcccagctactcgggaggctgaggcaggagaatcgcttgaactcggagggcggaggttgcagtaagctgagatcgtgccactgcactccagcctccagcctgatgacagagtgagactccgtctcaaaaaaaaaaaaaaaaaaaaaaaaaagaaaagaaaagaaaagaaaaaagaaaagtactctggtaatttttaaaaatgagataacttttttccttgttctgagaagttgtatgactaaagcattacctatgacgttagacaaaaatagtttctagaaatgaatagcaattaaactaaatatatttctaatatgcaccttatttttcactgtaaattcttcttttgacatctggaagagcaggagggaaggcagaaaccaagaagagctgaacgattactcctctggccaagagagagcagagagagaggaagggaattcagggctgtctgaagaaggggcatggtcaccagaacgaagagactggaggatatgcctgaatctgatttcttttatccagttcctctctgattctctgtatcagtcctctattgcccttcttttgtctttctcattctttcttccttaataacttattaattcccctctttcccagccctagtctgttcttgttccttactcactcattattctcattattctaaaatgctcttacttaaaaatatttcattaaagtactcttactattctaaaatattcttactatcctaagataatgtcactctctcaattaatatttcacttttccagttcatttttcatttatttttgttcaaagagacattggcattcttttacccatgtaaatgtatagacactgggctataagataccaaagagtaggcccctggagagtttgaggcatcatgctatcaaagacagcaatggtggctgtttccttcaagatatactatgactttatctaaatctttctaaatcaaaaattttatgagaagaagacataattaacttgatagttatcaagttctctttatacaaagaaattaaaaagcagaggtagaataagagtaattaatattaatagtataagtaaaagagtcaatgacaaaacatttaatgtttcggaatatttcactcaattctggagttacttagctatgaaacccaaatagaaagacatgggaaatagttttgtgagaaagctaggacagaaatgttttacttgaaaggaaattaaggtcccatgaggtaataaagggattgtggttaggagcttaccaacctgggggtcttagatatcattagattcccagttagatatcatttttgttttaaggggctggattccattttttgtcccttcaggggaaggatctaatgaagccaaagatcatggcagtataaatagcatgctttctttctactttgagatcaacaggccagattctatctctataaaagtttgggaggggtaacatggttttgtcaaggtaaccctgattttttttctgtgctctatctaaatagttaatcatatcaattatatagcttttacagtggcttgataattttggctgaactatatgacatcttcactttagggatatagggggtgggatctattcatgaaatgatgccaaaatgcagtgtgtaaacattgtcatgctcaactgtggccaacagcctgtagacagactattcttttatctacttaaaggacgggcagcatttggcagcagtttgattaaaatttagagctaaataggtaggtggagacccctttctctcaactacacttccgtagcctcgtctctctcatgacatcttttattcttccctccacatccaaattgtaaaaattgcttaggtaacgtaatctagtgacaatgtgcatgacttcttctcaaagagaaaggaaacccaatcaaatcaaaaggatagatatggtgtgctccaattaaataaaagccacttcttaaactttttgaatggtgttactttttggatagtgttaaggtccttagaacacacaaaaggaaaattaaatgtaactgctgaaacacagcagaaaagaccaaaaatgtcttagaaaaaatgctgaagagaggaggaagactgatttaaaaaggagaaattttttttaactgggaattttgagtcaactgagaagatgaaaggttggtagtttaaggttacacaaactgaagatcaatttgctgtttagttcaatatttataaagtgcactatgtgccaggcctgtcatccacttaataattacacaaatatttattgagaacctatactatgtttctgacactatgacaggcattaaggatatatggtaaacaaaacatctggtcattttacctctcctgaggctcttctgtctagaagtcctttgttaagtattgtctgatcctctctctcaaaaagcttaaagttcataggaaaaacaaacaccaaatagctatgatctcaggcagaatgggaaagatactaaaaaacataagaaaaaattaatatggtagtgctgagtacagaaatttttttccatgaagactagggagggtttcatggttctagtgctgtttgagctgggctctgaaggctgcatatgattttaataatttagaaagggaatagggagaggaaggcattccagtagagggatagtgtgggcaaaagctgaaatataaaacacagcgaatacttggaaaagtaaggatttatatgtgtctaaaacactgagtatgcatagggtgaagaaaagaaaacaatttccagattcagaggatcagaactccttagaagaatagatgttgatgatacatggtatgtgtgatccaatctcatgcaaacagtattttcaggggatcacttgagcagcgtgtagtgaaaatgttctccacccaaaaagtgaagtaaataaacatgaaatgcagccagctgaatgattgttcaactccttgcatttcggagtgggtcattctaacattggacagcatggattcccacgctccctgacagtggtcataggagggactttttggggccgctgaacctagaagactcttttcaagcaacccccccacactttttaaagtgttgaattccatctccttctcccgtaacgtcaggggcatacagactcagtgctggaccaagttgaggaacacctttcttcatttcctttcctctttagaacaaattggcaaaattctcgctcctcttccagagattcaagagattctggttgctatttatcttgtctagcaaggcattcacacttgccacgtttagcctatcaaatgttgccctaaatcctggcaaatattcatctagctcacacttttcgtgacacttttttttttttttttaagatggagtctcactctgtcacccaggctggagagctgtggcgccatctcagctcactgcaacctccgcctgctgggttgaagcaattctcctgcctcagcctccccagtaactaggattacaggtgcgcgccacaatgcccggctaatttttcatatttttagtagagatgaggtttcagcatgttggtcaggctggtatccaattcctgacctcaagtgatccacctgcctcggcctccctaagtgctgggattacaggcataagtcaccgcacccggcttcgtgacactctttatgtgagctgtgtgaaggtcacaagaaccagcagaagacctatctgtagctccaaatggaaaaaaccatgctcaaactgaaacagatttgactagataaagactcgatttccttttgcaataggatggttgagggcaggaataaagggactcaccacattgccttgtactgtctttgatgtggaacttctctcatctttcctctggactgtgagattctgtgctgaggggaccacattacatccctcatagtacctgatatgtagttgatgcccaacaaatatttattttaatatttataatcataatatttaatgtttttgttatattcttcaatgaaatgtctccaaatgttttcagtttatgaataatatactttaggcctcagagattcagctacagtaaatgttttcctgtggaggaagtacaagagtttgctatgaaaataaagttccctgtactaagatactttactctggatgtaaagatacttggctatttgttaggctgcttattcaacctgttattttaaagaaggaaaaaaaataagcacaaacaatacacttgtgcaacagtgataaaaaaatacactttcaaaactagagaaagattgggtgattcatttaactttctttcaacaccaatttctacacccagtgaaatctatgctagcttaaagaatgaaaaaatgctgggcacagtggctcacgcctgtaatcccagcactttgggaggtcgaggcaggtggatcttttgaggccaggtgttcgagaccagcctggccaacacggtgaaaccctgtccctactaaaaatacaaaaattagcccagtgtggtggcacgcacctgtaatcccagctactcaggaggctgagacatgagaattgcctgaactcgggaggtggaagttacagtgagccaagatagcgctactgcactccagcctgggtgacacagcaagactctgtctcaagaaaaaaaaagaaagaaaagaaaaagtcacataaaagtctttttttcaaaaaaggagaagagaaaattatgccaggtttcaaaatctcacctgtggaaatttgacccagaccttgtctttgggtaggactacatagtggttccaaccgtagactaataagagtcatggaatgtttacataaatgctgcgtgaatttcacaaccttccaccttttgaggtgctgccataacaaaattaggcacaaaaggggtgttttgcagacaatttgtggaagtattgacagagctgcagaggtatccttctcatttctgcatgccttaatccaggcccatttcttacattgcttagtgctcagtgtgttgttacaaagagcatgagctcagaacccaactgggaagactctaccagctgaagaaatgcctctgaagttaaccagtaaattttctcctctctcaggtcttttctccttacttcccatagaactgttcttagggaaggttgacataatcacatggttaaaatcccaagggactcaatattcctatactttaactgtatgtttttaaataaaaacttagagtagacttgccccctcggtttttcaaaaatctctgaattctccaaagtagaagctgtgcaatttatatccttaccagggagtgtttccaaaccattctcttgcaggcagtgttgaaagtaaggaagattggaacctgtctcagtaagaagctgagaggcttagagaaagttcctcaacacagcaaaacccaacattttaaaaacagaagcagaaacagttttataaaggcattgccacccccaccattgcacacaggctttgtttgttgttgtcagtaacattataagcactccatctttgggccttagttaatgctactactccaggttcctgcgttacccaagaaagttcctcccaaattgggagctgtaaccatctgttgatactcaaggctctccgaacagctatcactctaagagggtctcttatctgtgtttcagcaggatagaagcagacatccactgcctttggaaaaacatggggagttggagggacggatctatagcagcaactgcagcaatgaagacaggtcagttttacacgctagaaacagaaatgcccccagaaggttcaggatatgactggaaaacttgattgcatctaccttagtttgtacaagtggtgcatcttggaaaatagatttcctgaacagtttagatcaaaatggagctgacactcaggatctcctgtaatagtgacccacatgctttctatacatagcgcacatctatttgtccacagcccacattctgttttcttgctataatgtattctttgggtatggtgttggtgggtgatgggaaatattctgagccaaggcaagatgcttttcttaacagaaggtggttgtattgctaaggaaaaatgttcatgcaagtgatcaccaacctggagatgccccccaagtcccagatgatcaggtagctacaagtgtgaagagaggacacattaccaacccagagtttgaacatttagttaagctcagtaagatttagcatttctgtgaaaggaactacagtggaacttcaaccccgcttttctttatactagataaaggacccatcttcttaacctattggatttcattatttgcataactttttattgacccagtgtgccaataaacttgctgtttggtcggcatatcacaaattagtcaaatatgttgtttgatcgaatttatcaaagactttgagtggtagtcctatttcagtatggcttttgacctggttatgttgtattcttgcctcttgatgagaatgtattcatcagacatatttgatcggtgtgctaatgaggggtagaaattggttagggacagcgttaagactgtccttaacagttagtaaacatactaaacggaaagacaaggtggcaagcacactacattttccaaagctttacactggaaagcttaaatattaatagatattaaatatatattaaatagattttatgattaaaaataaaatggtttttttggtttctttcatctaaccattttgacaaattcagatacttttcacttaatatttgaatatataaatctaatttcttccatgttttctcccctctgaatcttctctttttttttttttttttttttgagacggagtctcgctctgtcgcccaggctggagtgcagtggcgggatctcggctcactgcaagctccgcctcctgggttcacgccattctcctgcctcagcctcccaagtagctgggactacaggcgcccgccactacgcccggctaattttttgtatttttagtagagacggggtttcaccgttttagctgggatggtctcgatctcctgacctcgtgatccgcccgcctcggcctcccaaagtgctgggattacaggcgtgagccaccgcgcccggccctctctctttagctcaccagttgaaagatatgtcagtcctatttttaaataagtaattacattagtgatatgtgtgcaatcatctttaagattaagagcaaattaacattggcttgtcagtctctcctcaaagctgttttccatctcaaaggtcgtgatccaaggtaaggtccagaaacaactgagattgttttacatctatgtactaggttggaacaaaagtaattgtggtttttgcctgcacttttaatggtaaaaaccgcaattactttttcagcaacctaataattacaattctaagtaatggagatacatatcttttataggcttcaatgagcaatacattagcataatgttttatttcatactgactttgaatattccttgtcaaaaatgcacttatactttggagttactatgtatgtttaggttactgtgttgtcatcagaaggctggagttatcatagcagagctttaatgacaaaatattatgagccttgtaaatagttttaaaaattgtccactaatatctatttgtcttgcaaaatttgcaattttactagtaattttcatcacttgctctttctacctctaatgtttctcagtctcctccattagatcttactgacttatcacatataaacaccttcctcagaaacagtccaataaaaattaaagaccaagaggtagaatctactggagccatcatgaattccagttctttttgttgttattgatttttcttttttttttttaaaaggcacacccttgacttttttttattgttaaaataaccagattctaatttcaggcagcaaaatcagttactgcaaaaagtcaataatcaaaaatcaatgtataattggttttcatcacctatagaattagtgaggtttatacccctcaagtgtttagtgattctattcagtcaacctaaaaaaaattgcctcttttctacttaaataaataatttatttatttattttgagacagagtttcgctctgttgcccaggccggagtgcagtggcacaatctcagctcactgcaacctccgcctcccaggtcaagcgattgattctcatgcctcagcctcccaaatagctgggattataggtgcccgccaccatgctcagctaatttttgtatttttagtagagatggcgtttcaccatgttggccaggctggtcttgaactgacctcaagtgatccgcccaccttggcctcccaaagtgtggggattactagtgtgagccaccacgcctggcctgcctgttttcattattacctgcctgttctcagtatgcaacatggcagtactattgacagtgaggtgctttggcatatcagataacttttccagttggtcaaggatcccttttctcttttcctcatttctgaactgcagaacaggaagtactaaagaagtggctcaggacaatgttgtcacatcaggagtggcagaggtgtttactaggattatgatcctttcagctgtgtgtcttagaaggatctcctgaagccctgggtttgatatagaaaccataagaaaaagacttggggcagttctatatctggctcttctcccacttctcccataaaagattaagaaaaactgatgggatgatttcagatgtttcattgccaccaaactacagccatgagttttttttctttaagtgatcttatgaggccagtaaaggcctctgtcttgattaatgatgatcatcctataatatctggatatggtggcttgacatgagttttcaacaaagaaaattagtctctgaaagacatttctcatctgaaactctcaatatattaaaatgcatttaaaagttacttctgggaaacatactaaataggccaatcagttaatcattagctaattgtcaaaccctataaaatcatggtataatgtcaccctgacataaagcaacatcaaaattagtgcatcatctataaagtgaagtattattttctcccaagtgacaaattctattgccaaaaaataccactgtacttctaataagtgacactcattttaatagaccctacaaaaatacaatattttcaatgtccccataaaacagttaacttacaaatattattctcagagctctggtgacatcattcagtgatactattgtgaaaatcctcatacaatacttgaaacactagcatgtaaagtaaattcattatataacaaaagaactatgtaaaattatgaaagataatgcatgcaaccaactccgggaaattatcctggaaattcaaattaatattgtaattaaattaatgactaatatgaaagataagtattttaaaggattataaaataaattttgatcatttatgcaggaaaatagtttcaatggaaaagtaaataattctacattaaccatgcttgtctttctcttcagtgaaaaagcattcaggattttacataccttgaaactgtttttggaaaaaaagtattttatctatttctgcccagaaaaacagccattgaaattaatgatacaggtagaccacagctctgagaaattatatttgaagtttcatatttaaataccaaggatttaaaatcacctaccataactttctaacagcagtctttcgtaatgataaattttatcaatttccaaaattcgttttaaataatttaaaaagcagcaaattagattaagcaacacacaaataaattccacatttacaagtaaagaaatcacaggggctacagtttataatcaacatgaacttgaaagaaataaagcaatacctttcctgccacccatcatccactgcttaaatttgtggtgaaaaagacttaactacaatgacctttagtctgtttctaaactctgcatgtattgtaattagctaaaggcattgaacaaattagttcatcctatttttatttgggtcccagagataaatggctaatttatgaaatatttcactctgtgtcatgagaatttagcaaatgaatatggaaccaaatataaacactttataccatatgtacagttactttcataaggcattatcatgtaatttttattgaaaaagattcaatatagtaaagtcttattttaagatatattttttctctatctgagatgtttagtttatgaaaatattgtttttctctatattctttttgtatatatgccaacatataccttgtgctagaaatattttatgggaattacaattctttatatttgtattttctatataaaggcatatacaactttgaggcagtgtttctgatggagagcagaattcataaagagcttgtgtgtgcttccgtgctccgaaattatatgaaatccattttgagaagaaacttatttgattaaaaacaaaaacaaaaacagaaacaaaactgcaccaatgcacagccagaggctgacaattaaaactaatacataaccacatgaacatcatatttatagagttaacattttttaaggatggtcagtgctaacatatagtattatacatttggcactaatgtttgccattggtccagcaattggcaaaatttgtttctatgtataaatttatttttgaacattaggtctggctagacgtatcttcactatttataaaaaatatttagacagtaagctcacgttgaataactaggtctactgtgttctggaaactcttcagtagtaatacagctttttcatgttccatatgtacaaaactgtgtccatttgcctgaaggatcttatcaccaggctgcagtaggtttgatgctggcccatcaggctgaacccttgtcagaaggtttgaatggatttccttgtccactaattccaccactgatactaaatccaaggccaggattcttttctattctcacacaaaactgctctggatatccatccatactcctttgccctttagtttgaattaagcaccgtccaggctgaggtccccgggtggcctgtgaagaggggatctgaataggcaatggtgactgaaattgctggatggtcactttgtttatatttccttcatacggctgctgctcccggctgcgatgctgaaggctttgggaccccatcaacgtctggatgtggctgcctgccttcttagtaatggtgtccggaggtacatcccgcctcccaagtggataaggattccattggccactaggagatacatcttcttgtccattgtctaaaatgttgctttgctgggacggggtcctgtctaaccgtctagcttctatatgtctaagcagctgttgtctccagtctgcaggcattttaccacagctctcctctcccttcacaggagtaggcctcgtctttaaatcactgttatctgatggcttgtcaccatagttacccaagttatagtcagatggtattttttccaaaagagctgccatagtaggcctagctgaaactggcctggtttgggaggcaccgtaactctctgtactgtagcttctcgcagacaatggcctcctttgggtaaggtttttaaccggaaaacttcccgcctgagctttcacttcttgatatgaagggtgttcatcttcatacctgccattccttttcaggaactgggactcagtcactgtaacgctgctttggcgatccagccctcccctatatgggggtctgccgtacctatcagttgggggcagctcatgaggctcattgacccttctaaacatggccatttctgtggcgctcaccagggagtcggcccttctcaggaagcccgccctggccccttggcttgcgaactgggcattcaccacagcatcctcattcacagatggctgagaaaatgaaaacatttgctccatcggtgggtatcctctgtaagctctaggactaatcaaatccttggcgatgtttttgctggcctgttgcacgtactcgggattgtgttgaaaagggggtggtatcctcttttcggctttcacttccactgatccttgaggattgaagctttggtcaaactgatagactttttttgtcatagaagctttttgttgttgtggccccttactacttccgtaggtgagcatctcatcatccagcattgggactgactggcttcgagacatactggacataccatgctctggtcccagcatcttatccggtcgttcgtggcttcctaagtgatcactcccagaagcatagttttctaatggtatgttatacaccttatatgtaccaatgtcaatctcatcgatactctgtgactttttgaatttattagacttgatatctttcattaggggggaaagcctctctgtgcttttgctaattgaaataacacctttagaagattccgggcggcagtggatttgagaaaagacattactaagactcctgttgggattggaatcatgatactcccatggtacgcctggagaaaaaggactaggtatttcagtagattcctttatatgttctttcctttcaggcaatgggctggtagtgggggttgtctctaatttggaaggaaaagcggtcctgtcttcaaacggactaggggttctggtccaattctgccaaggattggaaggaggcacttctgtttctggtgtgtgtctgtgtgtagactgctcgagttccaggggaacaccaacaatcctgtcttgcctgatcaaaggcctgcgtccatgcgaagatgtgcttctagatttcgaacttaagagaggattactgttggcattctcggctgtggtttcctcagcaacaaaccctgtgttgtcataatgcgagccatcagtccagttgtcagtgaaagtatcactcatgggcagccggtcaggacgctgtggtatattgcctgggggaacagcctcccgctggctgagtaatggctttgaatcaagaggctgtgggaaagatggtgcaatcctgttaccccacaaagaattatgtactgcatctttagctgttgtctgcaaggaccccactttaacccgggtattagaggatcctgaggaagcctgggaaggcgagtagtctgagtaagtgcctgaggaaacactgttattcagacagtgagttttgtcaacttcagactcatcagttgattcttttttgtccttccctagcagaacaagtttgggtgggtacagaggggtctcagctaatgaagggtgaagttccccaatcctcatttcattagctggatgaacaaaagaatcctccactgtaatctcctttggggctaccggccacttgtgttcatatttttctttcacagtttgctccgtgttagcagttggatttgaattctcaacacgcactccatggcttggcttacccaccaaattttgaacagattttaccatattctttaaatcctctgggtaaggagttggatatcgttttaggtttatttcaacctgtctgccacttagagagggaagagtggtggattgtgctgcaactggcaatggagtacacatgctcctttcctgctggaggccacttatacaaccccatgccagctgtgggtcattctgggggacgggcatatcttggatctgctgatcacacctggcccatggtgtgcagcaatcgccagacagtctggcaggttggagagtaatcccacgctggcccctttcccagggggcttggcaggagagatccttaactttcccagcattttcgtcatcttcttttttgtcttcaaattcaaaggcaacagtcatgcgttgttgtctctgctcttcccacagtgtagggttaaagctgtcactgtctgactggaaatcttcatcaccacgaggctgctggggaaacatgtagttagtcaatactctttgctttgtttctggatgggcttctgtttgtaaagggataagggctttggactgattgtcagaaagccacaaagctgcaagctctttaagtttggtaaatgagaatggtaaattcttcaatctgttgtcactcaaatttaggactcttagtttctgcatctgtccaatctcttcaggaagaaattctaatttgttggagcgtagagacatgactgttacattcttacaacttccaatttctctgggtaattctggaaggaaattctcatcaactgctaatgtccgaagactatgaaggtagccaatagtagaaggtagtgactccagttcattacagctacagtcaaattcttctaataaagataaatttccaattgtattgggtagcattgtaagttgattgtcatctacttttagagttgttagttttttcaaaagtcctatagaatcaggcaattgttgcaacatattggatgacaataagaggtcctcaagggcttcacatccagaaatgtccatgtcaactgtttctattctgttttttgacatatccaggtataccaacatctttaacttccctatagacccaggtaacacttgtaatgcattattatccatccataactccctcaaattttgtatttgatccagaacttcaggcagctcaccgaattcattattgcctaggtcaagtctttccaactgggccagtttgtgcattgactttggtagagttttcaagtgattttctcttaactccaagatccgcaatttgacaagtcttccaaaattggctggaagaaattcaagaaaggcgtcattcaggtagagctgggtcaggtttaggagctgtgtgaagccatcaggtagtttagaaatgggattgacactggcttcaataattgttaaacacttacagcactttatgttttctggaaattcttgtacaccatttttactgatgtcgagttctttaagattaactaaactagcaatagtggttggcagatttgaaaggtcgttatcaggaatacttagttttcgtagagcttgacagttgaacaattgcttgggtagttcttcaatttgattggcatctagataaagctcctctaatgttcgttcgaagttaaagacctcctttggcacctgctgaagactgcagtgggagtaatctaaaactgagatgatttcttcttcacctcggaaacatcggcatggcaccagacggccgatgattttccgtttggtggtcatctccaggcactgcaactcctcttcaggcctcttccgaagtgctgcacgaacctctttacaaggacttctctggtattgcgggggattccttccccttattaggttctccatccacatcttcgccgcctccctcggccaccgcacaagcagctccccgcgagcgccgaagcctcccgccct

SEQ ID NO: 12396 - RNA, 19650 nt, Homo sapiens
  source 1..19650: mol_type = other RNA
ctgggaggtcaaggctgcagtgggccatgatcatgccactgcactccaacctgggtgacagagcaagaccctgtctcagaaaaaaaaaaaaaaaaaaaaaaaaggcattaaaaaagcaataaagcagaaagaaagcatttgccattttattaaactgtgagagaaggtgacaatacagtgttctttcctcatattttgtacctacacgatagcatttattagactttttgtgtgtctccccactagactgtgtttcttgaggggtaggaccatggcttatttatatcttccattgttcttataatagaattttgaacataaccccttgttcattaacatttgttgattaaattgaatgcacagtgagaaaaaggcaaattgttttaacagttaaataattttttaaaaaaggataaacatatagattggctagaggacaaaccttagaatggtccggaggcagacttacaagagaattacttaaacatctctcgattcaaacctacaggtctggatgaatactcaaaatataagtatatattttggggtataggtgaacctgcggggcatatttatggcaagaccaagcaaaagaagaaaatatagtcccttcactttgagtagtttatgatgacctagggccctaggtgacagggatagtaactatcattttttgggaaacgtggaaatgcaaaaaaaaaaaaaattgcctgataagatatatagacacacacacacacacacacacagacacacacacagacacacacagagagagagagatattaattcccaagtttgaatttctctgggaaatggccacaaagaaatgcctgaactgtttgctagcaacattcatggttttataaagaatatagcagtgatgtcctgctagaatatctgtcttgatcataatgagactgtgagaacctatcaagtgcaagatacccgttgcttagtcaaacgattctacaagtatggctgaagatttatatcccaaaactggctatcaaagatggctggtttaaaacaatcaagacagtatagacaaatattacagggcaagaatagtttggatgatgatatcctagagaaaaaatcacttttagagaatgggacttgttcactatctaacaactttctcttttacagattctagcttaatgatcatcaataaaagtgaagtcttgaatatgatggatattcacttatttgtcagggaggtgacacagttggacaagcagcacccttggagtcggggttggggaggagtgcgtgagatgtttcaaaaggatctcagtgcattttaagtgacagcttctcctgctctcttctcttcccacagctgctgggggtcctgcaccccaacccagcctagatgatatttccatttgttgtacctaaaagcagagctttttacatctttacatctttacctcatgacagaactaaaaaaatgatgtttgttctacagtatggcacggagatgggtaaaaaagtgaaaagaataagccacaagcccccgtgctttgaggagatgatcatagcctgctcctggggaactatgctagtggctggatagcaagcactgacctagaggttgctcctaggaataaaaaattaagattatccatagaagacaaagaaaaaaatacttcgctaatagtggataccaaaaatctgaggtagtgcaaaagaaaagaaaggaaaaaagaaataaaaagcgcaactggaatacatacatacaaactttcaagacgttttctcttatactcttcagtaaaattctatgtaattttcattctagtatttaaatagttctggattttacaactaaacctatcattaaaaggttatggaaaatagaaggaataaaaaagatgaaatagaacatcaggcaaatcaaaaactcaaaagctgtatccaaaacaatggtggacacctgccgtatttgctttaaaatgggtggcactgttgtgtacaatttaaatttgttaaggagatatttaacttctctgaaaagagaggaagaacacttggtaaacaaacccaaaatggtgcactaaaattggcaggcttgaggtcagaaagaacttacaaaatattaacccccaaagaaggttaaattgaatttgctaagaaagagtattctgtattagtatctggtgatcatgtggctagaaggaaattgttttttttggaggaaaacaccagaggatataaatggcttcacataaactttgggaaagaacaccttgtcttccctctacctttgctccgggttggaagaaaaaaagattaaatggttggcaggggaacacctgaaacccatataagtagggctttgatggaattagcaaagaagaagctcagaccaggaggctggctaagctgtgagggtgaggatataattagcttagaggaagtaaacaaaaacatttggcctttttagcaatgatccagccatcagaggccctggaatttcaaatgactaagaagaaccaaaatagcttgaggacacatgtcaccaaggccgccaggggttctctgccttcagcacccagatattcccactgaaaggagagaggctggggagattgcaaactaccttgggaatccaatgatcactttgtgagagacattttgaaatacatttcgaaatacatttcttattcacttcataataaaataaaatctgattgtcatattatgctgattactcatacacataaataaaatgaaaaattaggcgtttattgtagatgcctagttattgccagatggaaataaagctatacccagatgcacacatattcagattggactagttttagaattacataaagaaggctaggcaaacttaaccacagttcctgatgtttaagttttggaaagttaactttaaaaataaattttgagtaacttgagacaaatctattcccacatacttggaatgggcatacctgaaggaagtgtggctaaaataatgggagataggagcaaaatatttggaaaacacaagttagagaagaactattaaactggtgggtataataattaaactgaacaattaaggaacatcaaaactttaaacaatcaagcctcactgagaaagtggtttctgtctcattaggttttgggtgattgatacaatctgagaggtttagtaaaaaaacatataaactgcctaaaataagctcaaagctcttgtttttttcttaaattgtgtaaatttagagcattgtttcaaattttctcaaaggagaaaggaaaggggtgttgttagcaattgtatcagcacaaggggcataaaaacagactgtgtaaggccatcccagcactttgggaggccgaggcggtcggatcgatagagcccaggtgttcaagaccagcctgggcaacatggagaaaacctgtctttactaaaaatacaaaaattagccgggcgtggtggtgcatgcctgtagtcccagctactcgggaggctgaggcaggaaaatcgtttgaacccaggaggtggaggttgcagtgagccgagatcgcgccactgcactccagcctgggcgacagagcgacactgtctcaatacaaacaaacaaaaaacacccacgacaacaacaaaaatcggactgtgctcccccaagccagagaattgccaaggctgggatttaaaatgtagatatgaggtctccatctagtggtggctcttctgaactgcagacacatgtttctttaaaagagtatgcggatgtgtacaactaaatatgaggatagtatttgtcagagttgaacgcagtaatttaaactagaggattttattgagatgaaacacaatttgttgctttataagggtgggttacagagggaaatgttcaccccttcgctccaggaatttaagaatagcatgaatccttccctgaagatagacaaatgaaccagatcctctcaaggtccctttctgtcttatgataggacaataattttgctcctttctccacagagcttttacctgtagccacactgtctgacattagtctttatttaagaaaagtacggccgggcgcggtgtctcacgcctgtaatccccgtactttgggagtccgaggcaggtggatcacgaggtcaggagttcaagaccaacctggccaagaaggtgaaactccgtctctactaaaaatacaaaaaattagccgggtgcagtggcaggcgcctgtaatcccagctactcgggaggctgaggcaggagaatcgcttgaactcggagggcggaggttgcagtaagctgagatcgtgccactgcactccagcctccagcctgatgacagagtgagactccgtctcaaaaaaaaaaaaaaaaaaaaaaaaaagaaaagaaaagaaaagaaaaaagaaaagtactctggtaatttttaaaaatgagataacttttttccttgttctgagaagttgtatgactaaagcattacctatgacgttagacaaaaatagtttctagaaatgaatagcaattaaactaaatatatttctaatatgcaccttatttttcactgtaaattcttcttttgacatctggaagagcaggagggaaggcagaaaccaagaagagctgaacgattactcctctggccaagagagagcagagagagaggaagggaattcagggctgtctgaagaaggggcatggtcaccagaacgaagagactggaggatatgcctgaatctgatttcttttatccagttcctctctgattctctgtatcagtcctctattgcccttcttttgtctttctcattctttcttccttaataacttattaattcccctctttcccagccctagtctgttcttgttccttactcactcattattctcattattctaaaatgctcttacttaaaaatatttcattaaagtactcttactattctaaaatattcttactatcctaagataatgtcactctctcaattaatatttcacttttccagttcatttttcatttatttttgttcaaagagacattggcattcttttacccatgtaaatgtatagacactgggctataagataccaaagagtaggcccctggagagtttgaggcatcatgctatcaaagacagcaatggtggctgtttccttcaagatatactatgactttatctaaatctttctaaatcaaaaattttatgagaagaagacataattaacttgatagttatcaagttctctttatacaaagaaattaaaaagcagaggtagaataagagtaattaatattaatagtataagtaaaagagtcaatgacaaaacatttaatgtttcggaatatttcactcaattctggagttacttagctatgaaacccaaatagaaagacatgggaaatagttttgtgagaaagctaggacagaaatgttttacttgaaaggaaattaaggtcccatgaggtaataaagggattgtggttaggagcttaccaacctgggggtcttagatatcattagattcccagttagatatcatttttgttttaaggggctggattccattttttgtcccttcaggggaaggatctaatgaagccaaagatcatggcagtataaatagcatgctttctttctactttgagatcaacaggccagattctatctctataaaagtttgggaggggtaacatggttttgtcaaggtaaccctgattttttttctgtgctctatctaaatagttaatcatatcaattatatagcttttacagtggcttgataattttggctgaactatatgacatcttcactttagggatatagggggtgggatctattcatgaaatgatgccaaaatgcagtgtgtaaacattgtcatgctcaactgtggccaacagcctgtagacagactattcttttatctacttaaaggacgggcagcatttggcagcagtttgattaaaatttagagctaaataggtaggtggagacccctttctctcaactacacttccgtagcctcgtctctctcatgacatcttttattcttccctccacatccaaattgtaaaaattgcttaggtaacgtaatctagtgacaatgtgcatgacttcttctcaaagagaaaggaaacccaatcaaatcaaaaggatagatatggtgtgctccaattaaataaaagccacttcttaaactttttgaatggtgttactttttggatagtgttaaggtccttagaacacacaaaaggaaaattaaatgtaactgctgaaacacagcagaaaagaccaaaaatgtcttagaaaaaatgctgaagagaggaggaagactgatttaaaaaggagaaattttttttaactgggaattttgagtcaactgagaagatgaaaggttggtagtttaaggttacacaaactgaagatcaatttgctgtttagttcaatatttataaagtgcactatgtgccaggcctgtcatccacttaataattacacaaatatttattgagaacctatactatgtttctgacactatgacaggcattaaggatatatggtaaacaaaacatctggtcattttacctctcctgaggctcttctgtctagaagtcctttgttaagtattgtctgatcctctctctcaaaaagcttaaagttcataggaaaaacaaacaccaaatagctatgatctcaggcagaatgggaaagatactaaaaaacataagaaaaaattaatatggtagtgctgagtacagaaatttttttccatgaagactagggagggtttcatggttctagtgctgtttgagctgggctctgaaggctgcatatgattttaataatttagaaagggaatagggagaggaaggcattccagtagagggatagtgtgggcaaaagctgaaatataaaacacagcgaatacttggaaaagtaaggatttatatgtgtctaaaacactgagtatgcatagggtgaagaaaagaaaacaatttccagattcagaggatcagaactccttagaagaatagatgttgatgatacatggtatgtgtgatccaatctcatgcaaacagtattttcaggggatcacttgagcagcgtgtagtgaaaatgttctccacccaaaaagtgaagtaaataaacatgaaatgcagccagctgaatgattgttcaactccttgcatttcggagtgggtcattctaacattggacagcatggattcccacgctccctgacagtggtcataggagggactttttggggccgctgaacctagaagactcttttcaagcaacccccccacactttttaaagtgttgaattccatctccttctcccgtaacgtcaggggcatacagactcagtgctggaccaagttgaggaacacctttcttcatttcctttcctctttagaacaaattggcaaaattctcgctcctcttccagagattcaagagattctggttgctatttatcttgtctagcaaggcattcacacttgccacgtttagcctatcaaatgttgccctaaatcctggcaaatattcatctagctcacacttttcgtgacacttttttttttttttttaagatggagtctcactctgtcacccaggctggagagctgtggcgccatctcagctcactgcaacctccgcctgctgggttgaagcaattctcctgcctcagcctccccagtaactaggattacaggtgcgcgccacaatgcccggctaatttttcatatttttagtagagatgaggtttcagcatgttggtcaggctggtatccaattcctgacctcaagtgatccacctgcctcggcctccctaagtgctgggattacaggcataagtcaccgcacccggcttcgtgacactctttatgtgagctgtgtgaaggtcacaagaaccagcagaagacctatctgtagctccaaatggaaaaaaccatgctcaaactgaaacagatttgactagataaagactcgatttccttttgcaataggatggttgagggcaggaataaagggactcaccacattgccttgtactgtctttgatgtggaacttctctcatctttcctctggactgtgagattctgtgctgaggggaccacattacatccctcatagtacctgatatgtagttgatgcccaacaaatatttattttaatatttataatcataatatttaatgtttttgttatattcttcaatgaaatgtctccaaatgttttcagtttatgaataatatactttaggcctcagagattcagctacagtaaatgttttcctgtggaggaagtacaagagtttgctatgaaaataaagttccctgtactaagatactttactctggatgtaaagatacttggctatttgttaggctgcttattcaacctgttattttaaagaaggaaaaaaaataagcacaaacaatacacttgtgcaacagtgataaaaaaatacactttcaaaactagagaaagattgggtgattcatttaactttctttcaacaccaatttctacacccagtgaaatctatgctagcttaaagaatgaaaaaatgctgggcacagtggctcacgcctgtaatcccagcactttgggaggtcgaggcaggtggatcttttgaggccaggtgttcgagaccagcctggccaacacggtgaaaccctgtccctactaaaaatacaaaaattagcccagtgtggtggcacgcacctgtaatcccagctactcaggaggctgagacatgagaattgcctgaactcgggaggtggaagttacagtgagccaagatagcgctactgcactccagcctgggtgacacagcaagactctgtctcaagaaaaaaaaagaaagaaaagaaaaagtcacataaaagtctttttttcaaaaaaggagaagagaaaattatgccaggtttcaaaatctcacctgtggaaatttgacccagaccttgtctttgggtaggactacatagtggttccaaccgtagactaataagagtcatggaatgtttacataaatgctgcgtgaatttcacaaccttccaccttttgaggtgctgccataacaaaattaggcacaaaaggggtgttttgcagacaatttgtggaagtattgacagagctgcagaggtatccttctcatttctgcatgccttaatccaggcccatttcttacattgcttagtgctcagtgtgttgttacaaagagcatgagctcagaacccaactgggaagactctaccagctgaagaaatgcctctgaagttaaccagtaaattttctcctctctcaggtcttttctccttacttcccatagaactgttcttagggaaggttgacataatcacatggttaaaatcccaagggactcaatattcctatactttaactgtatgtttttaaataaaaacttagagtagacttgccccctcggtttttcaaaaatctctgaattctccaaagtagaagctgtgcaatttatatccttaccagggagtgtttccaaaccattctcttgcaggcagtgttgaaagtaaggaagattggaacctgtctcagtaagaagctgagaggcttagagaaagttcctcaacacagcaaaacccaacattttaaaaacagaagcagaaacagttttataaaggcattgccacccccaccattgcacacaggctttgtttgttgttgtcagtaacattataagcactccatctttgggccttagttaatgctactactccaggttcctgcgttacccaagaaagttcctcccaaattgggagctgtaaccatctgttgatactcaaggctctccgaacagctatcactctaagagggtctcttatctgtgtttcagcaggatagaagcagacatccactgcctttggaaaaacatggggagttggagggacggatctatagcagcaactgcagcaatgaagacaggtcagttttacacgctagaaacagaaatgcccccagaaggttcaggatatgactggaaaacttgattgcatctaccttagtttgtacaagtggtgcatcttggaaaatagatttcctgaacagtttagatcaaaatggagctgacactcaggatctcctgtaatagtgacccacatgctttctatacatagcgcacatctatttgtccacagcccacattctgttttcttgctataatgtattctttgggtatggtgttggtgggtgatgggaaatattctgagccaaggcaagatgcttttcttaacagaaggtggttgtattgctaaggaaaaatgttcatgcaagtgatcaccaacctggagatgccccccaagtcccagatgatcaggtagctacaagtgtgaagagaggacacattaccaacccagagtttgaacatttagttaagctcagtaagatttagcatttctgtgaaaggaactacagtggaacttcaaccccgcttttctttatactagataaaggacccatcttcttaacctattggatttcattatttgcataactttttattgacccagtgtgccaataaacttgctgtttggtcggcatatcacaaattagtcaaatatgttgtttgatcgaatttatcaaagactttgagtggtagtcctatttcagtatggcttttgacctggttatgttgtattcttgcctcttgatgagaatgtattcatcagacatatttgatcggtgtgctaatgaggggtagaaattggttagggacagcgttaagactgtccttaacagttagtaaacatactaaacggaaagacaaggtggcaagcacactacattttccaaagctttacactggaaagcttaaatattaatagatattaaatatatattaaatagattttatgattaaaaataaaatggtttttttggtttctttcatctaaccattttgacaaattcagatacttttcacttaatatttgaatatataaatctaatttcttccatgttttctcccctctgaatcttctctttttttttttttttttttttgagacggagtctcgctctgtcgcccaggctggagtgcagtggcgggatctcggctcactgcaagctccgcctcctgggttcacgccattctcctgcctcagcctcccaagtagctgggactacaggcgcccgccactacgcccggctaattttttgtatttttagtagagacggggtttcaccgttttagctgggatggtctcgatctcctgacctcgtgatccgcccgcctcggcctcccaaagtgctgggattacaggcgtgagccaccgcgcccggccctctctctttagctcaccagttgaaagatatgtcagtcctatttttaaataagtaattacattagtgatatgtgtgcaatcatctttaagattaagagcaaattaacattggcttgtcagtctctcctcaaagctgttttccatctcaaaggtcgtgatccaaggtaaggtccagaaacaactgagattgttttacatctatgtactaggttggaacaaaagtaattgtggtttttgcctgcacttttaatggtaaaaaccgcaattactttttcagcaacctaataattacaattctaagtaatggagatacatatcttttataggcttcaatgagcaatacattagcataatgttttatttcatactgactttgaatattccttgtcaaaaatgcacttatactttggagttactatgtatgtttaggttactgtgttgtcatcagaaggctggagttatcatagcagagctttaatgacaaaatattatgagccttgtaaatagttttaaaaattgtccactaatatctatttgtcttgcaaaatttgcaattttactagtaattttcatcacttgctctttctacctctaatgtttctcagtctcctccattagatcttactgacttatcacatataaacaccttcctcagaaacagtccaataaaaattaaagaccaagaggtagaatctactggagccatcatgaattccagttctttttgttgttattgatttttcttttttttttttaaaaggcacacccttgacttttttttattgttaaaataaccagattctaatttcaggcagcaaaatcagttactgcaaaaagtcaataatcaaaaatcaatgtataattggttttcatcacctatagaattagtgaggtttatacccctcaagtgtttagtgattctattcagtcaacctaaaaaaaattgcctcttttctacttaaataaataatttatttatttattttgagacagagtttcgctctgttgcccaggccggagtgcagtggcacaatctcagctcactgcaacctccgcctcccaggtcaagcgattgattctcatgcctcagcctcccaaatagctgggattataggtgcccgccaccatgctcagctaatttttgtatttttagtagagatggcgtttcaccatgttggccaggctggtcttgaactgacctcaagtgatccgcccaccttggcctcccaaagtgtggggattactagtgtgagccaccacgcctggcctgcctgttttcattattacctgcctgttctcagtatgcaacatggcagtactattgacagtgaggtgctttggcatatcagataacttttccagttggtcaaggatcccttttctcttttcctcatttctgaactgcagaacaggaagtactaaagaagtggctcaggacaatgttgtcacatcaggagtggcagaggtgtttactaggattatgatcctttcagctgtgtgtcttagaaggatctcctgaagccctgggtttgatatagaaaccataagaaaaagacttggggcagttctatatctggctcttctcccacttctcccataaaagattaagaaaaactgatgggatgatttcagatgtttcattgccaccaaactacagccatgagttttttttctttaagtgatcttatgaggccagtaaaggcctctgtcttgattaatgatgatcatcctataatatctggatatggtggcttgacatgagttttcaacaaagaaaattagtctctgaaagacatttctcatctgaaactctcaatatattaaaatgcatttaaaagttacttctgggaaacatactaaataggccaatcagttaatcattagctaattgtcaaaccctataaaatcatggtataatgtcaccctgacataaagcaacatcaaaattagtgcatcatctataaagtgaagtattattttctcccaagtgacaaattctattgccaaaaaataccactgtacttctaataagtgacactcattttaatagaccctacaaaaatacaatattttcaatgtccccataaaacagttaacttacaaatattattctcagagctctggtgacatcattcagtgatactattgtgaaaatcctcatacaatacttgaaacactagcatgtaaagtaaattcattatataacaaaagaactatgtaaaattatgaaagataatgcatgcaaccaactccgggaaattatcctggaaattcaaattaatattgtaattaaattaatgactaatatgaaagataagtattttaaaggattataaaataaattttgatcatttatgcaggaaaatagtttcaatggaaaagtaaataattctacattaaccatgcttgtctttctcttcagtgaaaaagcattcaggattttacataccttgaaactgtttttggaaaaaaagtattttatctatttctgcccagaaaaacagccattgaaattaatgatacaggtagaccacagctctgagaaattatatttgaagtttcatatttaaataccaaggatttaaaatcacctaccataactttctaacagcagtctttcgtaatgataaattttatcaatttccaaaattcgttttaaataatttaaaaagcagcaaattagattaagcaacacacaaataaattccacatttacaagtaaagaaatcacaggggctacagtttataatcaacatgaacttgaaagaaataaagcaatacctttcctgccacccatcatccactgcttaaatttgtggtgaaaaagacttaactacaatgacctttagtctgtttctaaactctgcatgtattgtaattagctaaaggcattgaacaaattagttcatcctatttttatttgggtcccagagataaatggctaatttatgaaatatttcactctgtgtcatgagaatttagcaaatgaatatggaaccaaatataaacactttataccatatgtacagttactttcataaggcattatcatgtaatttttattgaaaaagattcaatatagtaaagtcttattttaagatatattttttctctatctgagatgtttagtttatgaaaatattgtttttctctatattctttttgtatatatgccaacatataccttgtgctagaaatattttatgggaattacaattctttatatttgtattttctatataaaggcatatacaactttgaggcagtgtttctgatggagagcagaattcataaagagcttgtgtgtgcttccgtgctccgaaattatatgaaatccattttgagaagaaacttatttgattaaaaacaaaaacaaaaacagaaacaaaactgcaccaatgcacagccagaggctgacaattaaaactaatacataaccacatgaacatcatatttatagagttaacattttttaaggatggtcagtgctaacatatagtattatacatttggcactaatgtttgccattggtccagcaattggcaaaatttgtttctatgtataaatttatttttgaacattaggtctggctagacgtatcttcactatttataaaaaatatttagacagtaagctcacgttgaataactaggtctactgtgttctggaaactcttcagtagtaatacagctttttcatgttccatatgtacaaaactgtgtccatttgcctgaaggatcttatcaccaggctgcagtaggtttgatgctggcccatcaggctgaacccttgtcagaaggtttgaatggatttccttgtccactaattccaccactgatactaaatccaaggccaggattcttttctattctcacacaaaactgctctggatatccatccatactcctttgccctttagtttgaattaagcaccgtccaggctgaggtccccgggtggcctgtgaagaggggatctgaataggcaatggtgactgaaattgctggatggtcactttgtttatatttccttcatacggctgctgctcccggctgcgatgctgaaggctttgggaccccatcaacgtctggatgtggctgcctgccttcttagtaatggtgtccggaggtacatcccgcctcccaagtggataaggattccattggccactaggagatacatcttcttgtccattgtctaaaatgttgctttgctgggacggggtcctgtctaaccgtctagcttctatatgtctaagcagctgttgtctccagtctgcaggcattttaccacagctctcctctcccttcacaggagtaggcctcgtctttaaatcactgttatctgatggcttgtcaccatagttacccaagttatagtcagatggtattttttccaaaagagctgccatagtaggcctagctgaaactggcctggtttgggaggcaccgtaactctctgtactgtagcttctcgcagacaatggcctcctttgggtaaggtttttaaccggaaaacttcccgcctgagctttcacttcttgatatgaagggtgttcatcttcatacctgccattccttttcaggaactgggactcagtcactgtaacgctgctttggcgatccagccctcccctatatgggggtctgccgtacctatcagttgggggcagctcatgaggctcattgacccttctaaacatggccatttctgtggcgctcaccagggagtcggcccttctcaggaagcccgccctggccccttggcttgcgaactgggcattcaccacagcatcctcattcacagatggctgagaaaatgaaaacatttgctccatcggtgggtatcctctgtaagctctaggactaatcaaatccttggcgatgtttttgctggcctgttgcacgtactcgggattgtgttgaaaagggggtggtatcctcttttcggctttcacttccactgatccttgaggattgaagctttggtcaaactgatagactttttttgtcatagaagctttttgttgttgtggccccttactacttccgtaggtgagcatctcatcatccagcattgggactgactggcttcgagacatactggacataccatgctctggtcccagcatcttatccggtcgttcgtggcttcctaagtgatcactcccagaagcatagttttctaatggtatgttatacaccttatatgtaccaatgtcaatctcatcgatactctgtgactttttgaatttattagacttgatatctttcattaggggggaaagcctctctgtgcttttgctaattgaaataacacctttagaagattccgggcggcagtggatttgagaaaagacattactaagactcctgttgggattggaatcatgatactcccatggtacgcctggagaaaaaggactaggtatttcagtagattcctttatatgttctttcctttcaggcaatgggctggtagtgggggttgtctctaatttggaaggaaaagcggtcctgtcttcaaacggactaggggttctggtccaattctgccaaggattggaaggaggcacttctgtttctggtgtgtgtctgtgtgtagactgctcgagttccaggggaacaccaacaatcctgtcttgcctgatcaaaggcctgcgtccatgcgaagatgtgcttctagatttcgaacttaagagaggattactgttggcattctcggctgtggtttcctcagcaacaaaccctgtgttgtcataatgcgagccatcagtccagttgtcagtgaaagtatcactcatgggcagccggtcaggacgctgtggtatattgcctgggggaacagcctcccgctggctgagtaatggctttgaatcaagaggctgtgggaaagatggtgcaatcctgttaccccacaaagaattatgtactgcatctttagctgttgtctgcaaggaccccactttaacccgggtattagaggatcctgaggaagcctgggaaggcgagtagtctgagtaagtgcctgaggaaacactgttattcagacagtgagttttgtcaacttcagactcatcagttgattcttttttgtccttccctagcagaacaagtttgggtgggtacagaggggtctcagctaatgaagggtgaagttccccaatcctcatttcattagctggatgaacaaaagaatcctccactgtaatctcctttggggctaccggccacttgtgttcatatttttctttcacagtttgctccgtgttagcagttggatttgaattctcaacacgcactccatggcttggcttacccaccaaattttgaacagattttaccatattctttaaatcctctgggtaaggagttggatatcgttttaggtttatttcaacctgtctgccacttagagagggaagagtggtggattgtgctgcaactggcaatggagtacacatgctcctttcctgctggaggccacttatacaaccccatgccagctgtgggtcattctgggggacgggcatatcttggatctgctgatcacacctggcccatggtgtgcagcaatcgccagacagtctggcaggttggagagtaatcccacgctggcccctttcccagggggcttggcaggagagatccttaactttcccagcattttcgtcatcttcttttttgtcttcaaattcaaaggcaacagtcatgcgttgttgtctctgctcttcccacagtgtagggttaaagctgtcactgtctgactggaaatcttcatcaccacgaggctgctggggaaacatgtagttagtcaatactctttgctttgtttctggatgggcttctgtttgtaaagggataagggctttggactgattgtcagaaagccacaaagctgcaagctctttaagtttggtaaatgagaatggtaaattcttcaatctgttgtcactcaaatttaggactcttagtttctgcatctgtccaatctcttcaggaagaaattctaatttgttggagcgtagagacatgactgttacattcttacaacttccaatttctctgggtaattctggaaggaaattctcatcaactgctaatgtccgaagactatgaaggtagccaatagtagaaggtagtgactccagttcattacagctacagtcaaattcttctaataaagataaatttccaattgtattgggtagcattgtaagttgattgtcatctacttttagagttgttagttttttcaaaagtcctatagaatcaggcaattgttgcaacatattggatgacaataagaggtcctcaagggcttcacatccagaaatgtccatgtcaactgtttctattctgttttttgacatatccaggtataccaacatctttaacttccctatagacccaggtaacacttgtaatgcattattatccatccataactccctcaaattttgtatttgatccagaacttcaggcagctcaccgaattcattattgcctaggtcaagtctttccaactgggccagtttgtgcattgactttggtagagttttcaagtgattttctcttaactccaagatccgcaatttgacaagtcttccaaaattggctggaagaaattcaagaaaggcgtcattcaggtagagctgggtcaggtttaggagctgtgtgaagccatcaggtagtttagaaatgggattgacactggcttcaataattgttaaacacttacagcactttatgttttctggaaattcttgtacaccatttttactgatgtcgagttctttaagattaactaaactagcaatagtggttggcagatttgaaaggtcgttatcaggaatacttagttttcgtagagcttgacagttgaacaattgcttgggtagttcttcaatttgattggcatctagataaagctcctctaatgttcgttcgaagttaaagacctcctttggcacctgctgaagactgcagtgggagtaatctaaaactgagatgatttcttcttcacctcggaaacatcggcatggcaccagacggccgatgattttccgtttggtggtcatctccaggcactgcattgctagttattcctgtctctgcagacttctaggttgtgaccactttgacttgcattttttttcatgtagcgggctcactcctcttcaggcctcttccgaagtgctgcacgaacctctttacaaggacttctctggtattgcgggggattccttccccttattaggttctccatccacatcttcgccgcctccctcggccaccgcacaagcagctccccgcgagcgccgaagcctcccgccct

SEQ ID NO: 12397 - RNA, 7500 nt, Homo sapiens
  source 1..7500: mol_type = other RNA
ctgggaggtcaaggctgcagtgggccatgatcatgtcactgctctccaacctgggcgacatccagaccctgcctctcatcagctgaaagtgcctgtgaaaaacaaagcttctctaaaggcagtgtggtgtcctgcactggatcttatgtctcagagcgttggtggagaacactgacatcccaggcattaaaatgaggtggtgtttggtagatggtggctaatctgcattttgccaaagcagcatcagtaggtggtccaacaatagtatctcaggcttactaagcatctgtccagataacagggaagagccagctcagtcagtgttactgtctcttctgggctccctgacttgtatttagagcgcaataccaagttgcagatccaactgctggatgacaaagttttgggagttcctgccctccaaccggacgcacaaaacagcatcatctctaatcaaattggttcagtgtaaatggagggtttataaaatagaacgcaatctcaggcaaagtctctgttcttccacgtatctgccttcatcaagtgactcatgagacaatcacaggatcggcaggagtgagacctaggaaagatattcaagtaaaacatgtttcttaactagttctgtttctggtgattggaatttgcttgattttacttactaataaaatttttgctgcttatattttaagtacatctgaaaaacctgattatgaagttagaatccgtattatctcctcgaatactcttagaaagcaatgtctctctataaaaacatgaggagaaaaagacttctacagcatctttttattgtctttaccattactttaatgcattttaaaatttatctacattaattgggaacaaagaaaaatagacatttctttgtttttcataaataactaatcttcatatttgataaaaatctcaaatgattattttaccttcccacaaatataatacatacaaaatttttctgaagtaaggtcaacaaattaagtatcttgagactaacataaccacatacaactgctgtttctactgactcccaggaacgaagcagaaacaaaaactcatcaagctgctctgggtttccttttgtaagtgttacagattcagaactgtaatcatgtatcatctgccagtaataacatatggattcaaattgattgtctacaaataaagtatcgctggctctagtgtaacttctggatttaacataacagtgactacagcatgggataggcactatacatatatggaaatcataaacagtatcgaatgccctggacttcaactactgactcggtatgtgcctcatttggctcagtaataaattcacctgcaccaaacccgtatcaaaagtcaccaaatctctcatatatatatataatatatattatgtatatatacaacccacaaaacatacatactatacatagtttgtaacaacatgaagtcatactgtcttaaaatgatgcactcacagacagacactatcctggctgaaataaatcctattgtcatcaggctgctagcttttgagagtcttgactcaggttagctacttatattctgcctactcttcacccttctttaacgtcttggcagttctttcagaaccaccctccgcaatccagacagatttgtttcccaggatcacttgattggactttggaaacaagaaagagcatgcagagggagcaggcaattcttagccactgtccctcacacctgcctatacgtgtgatgtgctctgtcctgttggccacatttagtgttagaaagcagttattcaaagctctgtccctcctaccccccttgggctttctgtagagcacaaaagtgaaagaagcttctttggctggggtagcagttcattaaaatatacaactacatttcctagctctggggttcccattctgtactggagagtgcaggtcacggatgctgttattaaggtttggtgtgtgatccatgaggttttctcctggcagccggtgtcaggattagcgcagctccagcccaggaggcaacagcctaatgaataccaactttgaaacagtgctgtcggcacgttatttaagcttgtacatgcccacaattacacacaacacacacatgggccttggtcactggcaatggtcatgagaaaatatgagaaaggtttgcaaggaaaaccaataaggcaccaagaaaaattatttccagtcaattttaccatttcaaaatgtgagaaggaaaatcatagaaattaaaaagatttcctaaaatctggtcagctaattcactgagaggtcccattagttcctttagacaacctacctgaatggaatccttaccccctaagctatgaagtgaggcattgcttaaaatcaaactgaaagggacagccctgaagctgtacacataagagactccaatgggccctaagtcctccccagctccacaaagctggctgtgaagaagttgctgaactactccataaccttttattttacagttgctttcatgagcatgacttgtttccataatcacatgcaaattgggggaagtaactatatggatggaaacagggggtggctgtaagtagatccagtttctctcccctggggtggctgatctcagtaagacttagggatgcaggtgggcttttatctttgtctctcttaggggatgagggaagagagggacagcagaggtgagaacagagacaaagaagtgcttctgaaagttggtctggaattagaccccaaagatcctgactaatattgccccccacttgggcttagcgtcctttgttttaactggcttatttttaaagtaaattagttgttcagcatgttgctaaaacaaaacaaaaaaaaattctaaaaatgaattaaatcactttcatccacttcatcccacaacttttggatacactgtgcatcatttccagatttctccacaaagaaggagggacaacccaaatgaggcacaatgactgaaggcagcagagcagtctgtctactttctgggaagacatatgaaatgagggaaaaggtcaaggtgatcagaaaaggttctctcatttgaaaaacaggagaggaattggcattcagtcaagggatctatttcaagattctaggaagaggcttcttcctagaagaataaatagaggaataaaataggcacaaagttctgtagctatttgtacgaggttttgtagaatccactgaaattttaattcagaggataaattgggtaagagcagtgcattttaataaatgtgaagtttttgagagtccttacaactttaatactaggtttcttcccaccagtaaagtgtttaaattccccctgggaactatgcatttgtctatttaacatccatgaagtaaaaattgtcctaggcttaaattttacttttccaactttggtataagtgaattacaaatgcctacactcaagttgttttcctagacaggattttctcaaatgttaattgctctggccattttagcttcctaaatttagtccccaatcctggtcattggtattttgctggctgaggcactgtcaccccccttccccagtaatggccccacactcttcatgaatgaatgcttaaacagattaggaaagcaaacagaattttctaatagcaaagaaacctctgtgtgtatgttcatcaatataagcgttcataatgaatgaaggaatagttaaacagattagtaaagcaaaccaaattctctaattgcaaagtgtgtgtgtgtgtgatcatcaatatacaggctttctcagaagaggaagaaaactatagaggtagcactatactgatctatattttaaaaggttgtgcaagcatgttatgcatctcttttgttttcagagacggcagagagcaacgtcttgctgctcttggaatatctggctataaactagtccaaagtccaggaacacttattttcccttatttgggccaatgtttgttcacaggtagccagcctccctcccccagttcaagcacttcattcaagggtgggtgtggtttctaatcacagctctccaggagaggaggaataagaaaagcaaaaaggctgtttaacatgataaagggggaggggggaggggggagggggtggagcaaataagtgttggaaatttacttattagaagtatatccatttcagtccttacatttaaaaaggagccccctttagcaactgtcgctaagtattgtccagagggagtgggtttatacttttaccaaaattataacacaagttccttaaaaaaaaaaaaaaaaaaaaaaaaaggggatcactgaagcttaagaaccacccactacctctcaggcacaaagctgccatctcaccagcctaaaattcaagctccaccaatcaccatcgcttaggctctcactactgcaaatatttatgccagatcctctataatgctacctctaacttattcaagacacaacgatggtgctgttaggagtgagaattattacaagcactacagaaaagaaactgaacctccctctataaacaaagctaaggctgaacacaaaaccgctaagcactccctaaccttgtcactttggggaggccctgagctcattatgctcccctcctaggtatgacctggggctataaactgcagctcaccttaaagaatcatggacactttaagcagtggaaggagaagctggctgaaaaagcacacccaacaacttcccagtcacagcaaccgaaacgttcactgttcacatttttttttaaagacacacgtataggaaatatattttcccaattgagaccacacagttcaaagaaacctgaaccaagtggaacttcattacaacgccaaccttaggattgtaaagcccccaaagcaaaggtaaattgttgccaaaatgcaacaaagttacaaattaagaaaaatacatataaattaaaaagagggttcccataaagaaggcagtaagaaacgcaaaatagaatacacgtgagctgggccccttggagaagacctgggacaggttcttcctcgaaaacgcccctcttccctctctccaagtcgccgcgggagggggcaacagcaccatgaaggtaaacggaagtgaccttggcaaaactaccaaacaaaacgcccccctcccctcagctctccggccgagtccctcggcggcagcctcctacacgtgcgacagggacacctgcttgtggtaggtggcggcggggcccggcggcccggtcctgcctgtgagcgcggcgctcgcctcggggtagtcccctgcggccatggcgcccccgctcttgtggccgcgccgcgggcggcagcagcagcggctggtgaaacgccgccacgactccaccgtcttgcccgaccagatccagacgcccgacgtgatgcccaccaccaggcacatgaagtacttgagcatgagcacccagtactcgggcttggcgcgcggctggccggtgtcgtggcccgggcaggcgcaggtgagcgccgcctcccagctctcgcggtagtgctgctcgtacaggtagcaggccaccacaatgctggcggggaccgtgtagagcagcgtgaagatgccgatgcggatcatgagcttctccagcttgtccgtcttggtgccgccctgcttgatgacgctgcggatgcggaagagcgacacgaagcccgccagcaggaagagcgtgcccaccagcaggtagagcaccagcgggcccagcacgaagccgcgcagcgagttcaggttctggttgcccacgtagcagatgccggccactgggtccccgtccacggagctcagcgccagtgccgtgatggacttgacgctggggatgagccacgcagccaggtggaagtactgcgcgtagcccgcgatggcctcgttgccccacttcatgccggcggccaggaaccaggtgagcgacaggatgacccaccagatggagctggccatgccgaagaagtagaccaggaggaagacgatggtgcacagtgcagggcccgtggtctcgtagtggatgtggttgtgctcgcggctgcaggccacgctggcatggcccacgaccagacgcaccaggaagcccagcgacacgcacaggtagcaggctgacaggaagatgatggggcgctcaggatagcggaagcgttccatgtcgatgaggaaggtggccactgtggtggacgtggagatgaagcacagcaccgaccacaggcctatccagaaggtggcgaacgtgcgctcgtcggcactgaaggacggctggtagcagggtaccgcgcagttgggcacctggcccgtccgcaccttgttgtagagcgggtgtgactccttcagaatgggcacgaagggctcgcgacacttgcacacgaacgggcccccagcggggcattcgccccccgaggccggcgcccctggcgggcctggaagggtgggcttggctgggaaaggcctggggggcgccgtggtggcctcgctgcggttgtaatccatgcagaggacctcggcgtcgcggcccagcaccgggaggcggtcgcagctcatgcgctcgggccaggcgaagccgtactggcgcatcagcggcgagcagccggccttggcgcgctcgcacaccgagcggcagggcggcagcggcttgtggtagtcgggcagacagatgggcgtgtacatagagcataggaagaagcgcaggtccggcgagcattggatctccaccagcggccagaactggtgcacctccaggcccgcctcgtcctgcgtgtcgtggttgaactggttgggcatgtgcgtcaggttgtagccgatgccgcggcacatgggcaccgtgatttcctggcacaccggggccttggacgcggcggccgcccggcccaccagctgcgctaggagcagcagcaacagcgagggcggcgcggatgggtcaggccgagccatcgccccctccctcccctcgcctccagcagcccgcgagggacgcacacaggcagaggaatccgggccggggcttctccctccggcgtctcgtgtgtggcgccggggctggcaacctgttggttgctttttcctttaaagaaaaccgtccaaagataaactgcttcgggaaggcgctgcctccgctggcagcgctccgctcctcgccggatagggctggggagagacggttagggctcggattccagggaaaggactctccacggatcccgccgagaagagcagacagtccccagccagcctgggtcctccgtccctgggtcactccgctgagaagcgcgactcagagccgggctggcgcccggaaagtttagcgacaggctgggtacccgtggcagcggcacatggcagcaggtgggggcgactcagagtggggggcgcccccagaacaggggcggcgcaggccggtcactcgccctctcctcctcgggagccccccgcatgatccagacggagccgggcaggggcaggccgtgcgttctccccggggccgggag

SEQ ID NO: 12398 - RNA, 4251 nt, Homo sapiens
  source 1..4251: mol_type = other RNA
ctgggaggtcaaggctgcagtgggccatgattgtgccactaaactccaaattaggtaacagaccctgtttctcaaaaaaaaaaaaaaaaacaaaacaaaaaaactcataaagtaaaagttacagtaagctaaggttaatttattgaagaaaaaatatatatctaatatatataatacataatatatataatgtgtgtgtgtgtgtttattttcaagacagtcttgccctgtcgcccaggctggagtgcagtagcgcgatctcggcttactgcaacctccgcctcacaggttcaagctattctcctgcctcagactcctgagtagccgggactatgccaccacacccggctaactttttttggtattttttttagtagagatggggttttgccatgttgcccgggctggtctctaaactcctgagctcagacaacctgcccgcctaggcctcccgaagtgttaggattacaggcatgagccactacgcctggccaagaaaaatattttcaataaatttagtataggttaagtgtgcagtgtttatacaagtctacatgttccaactgtctatagcatgcaggacagtaacatgctatacgggtttgtagcctaggagcaacagactataccatatagcctaggtgtactggtaggctataccatctaggtttgtggaagtaaacaacatgatgtttacacaatgacaatatcacctaacgatgcatttctcagaacatatctctgtcattaagtgatgcgtgactctatttgctcctttatctctaacattacattgtaagggtaaggactgtgttatcaagcctgtattcctaacaaaatctatgtttaagaaatatttattgtgagtttactatgtatcaggtacagtgctaggtactcacaattggagacataattttatagatgagaacactgaaactctgagaaattaagaacttactcaaagtcacacagctggcaaatgggttgcaccagtatacctacctccagaatatatattgggtaaaggatctgtttgcatgaacaaacaaaaaaatcatattcttgtaagtatttttacaccctgtaccagtagatctttctttaaataaattccgaagatgaacaatttttgtcccatctaaaatattcaaagcaaagtccacctgttctgactctagaacaaaaagctacaaatagaggaaataaataagttgaattcaaatgctgctgagaaaaggcaatgtatattatagttctgtggtagtactgataacattcaagtcattcttaggcaccagtcttacgtatatgaagtcactttttcattccattgtacaaaactcatattttgagaaaaatctaatagctaatagtctccaacaccatatgatcataatcctttagcttaagtagagatctacttattaaatgaggcaccatcaacctaaggaaagataagctgtaagagaatgaagacagaggtatatcaagtaacaagaacattcttccttatcaggataaaatgtttatcagtattcaaataaaatatcttaaatggaaagagacaggaaagaacatggttaaatcacagaaaatgaagaaagggagaagctgatcatgatcttgtacaacattatgacagcactaaggtattacgtatccaatacaaggatacttaatagaccaaagaatttaaaatcccagggaactggaataaccagccacaaaagaggcctctctttgttgtggttcacaacacaaaaggccatcaacaaattaggaaatattaaaattaagagagcagcaggtttcttcttggtagacagctcatgctaccatccacaaagtgagcagtggaaggggtatttaatgtcaaggctttattttgaatttctgttccagatgcctctccacagcattcatcacaccttccttcacacttgaagggaaaagtccttaagagttcaccacattttggtgttatttttagcataaacatttgtttttctataagaagtatctctctggattcaaaccacagaaatgtcaatgaatgttatttccattgtataatcatttaaaagtcacctacagagctgggtgcagcagcttgtgcctgtaatctcagttactcaggaggctaaggcaggaggattgtgtgaggtcaggagttcaagaccagcctggacaacatggcaagaccctcatctctacaggaaaaaaaaaaggcacctacaaattgaaactgacttgatagtttaggatcatttatcaccagtcccatgtacttgtagttgatttcaaatgtttggtacaggtgactgtaagacttcaagtattccatgaaaataacattcatgctgggatcataaaattacatttctgggacagtatttttaaagtctgtttttaacttttgtcttcaagagctactttcttcttgctgttctgaccagtgacctttttccacatacttactgtttatccttagctttttctaagaaacattttggagttgtactaatgctctccctttccaatggtttcttaatcatctttttcttttgtttgcttagtagtttctgaaaaccttttatgtattctggtacaggacacccagcctgctgtataacattagcaacgcttcttaataatggcttatcatcctcagtgaaaaatgtaattgcttttcccttattccctgctcttccagttcgacctatcctgtggatatattccactgagctagttggaaagtcatagttgatcaccaagttcacacctttaaaatcaatccctcttgctagcaaggctgtacaaatcagaacccagatttttcctgctctgaaactgtggactgtgttatctctctgttgttgtgttctctctgcatgaataacatccacattaataccttcatatatgagctcatgaaaaagttctttagccctttcaatggactgaacaaaaacaagaacaggtggattgaaaccctttttaacaagttctctcacggccagaagttttccggtctcagatccaacaaagagaagctcttgttctacagtttctactgcagaattccttgctccaatggacacactgatgacattgtccaggttgagtttgcaccactgttcaacatcatatgcaaaagttgcactgaacatagctcttcggaccttgtgggatgtgcaggccaggaaaatggaagccagctggtctctgaacccagttttgccatcttcaaacagtttatctgattcgtctactacaagccactcaacacttgctaggtcgattccggggggatcttgctttaataaatagattagtcgatttggagtagtcacaagaatatcaaactttttagatgatttaggtccaaatttcttggctgccactgctgctttgtggatcatgtgtattctgaatcctgttccctcagaaatttttattaactctctgtgaatctggctggcaagttctcgtgttggtgatataatcagggctctgaagcctttatttgcgggttgtttcagctgcattaaaataggaatgctaaaagctaatgtttttccagatccagttggagcagaagccagaagttcccgaccatgcagcataactgggatggcttgcatttggattggcgtaggcatttggaaacctgcatctagaatgttctgaagtagtcgagaattgattttatattcctggtcaagttgctgaaatgtagcaattgggtcaggaagatcggttccttggacgtgaattttgtgtttattccgcaagaagtttatcttttcttttctgagattctccaactttccggaagttagtttactttctctctgaacttttttgtcttcaatctttgcttctacagatgacatccactgtatagtagcaccttcttcttgggaagcaatttctgaagtcatcgtcttcctttttttcttgctctgctccctcttcctttcagttaggctctcttcttttttctctccattttggggcttctgatgtgtttgtgatgctccacacacacctgggacagacttcttgtttccaaaaaagtccagtccctgaagcacctccgaagaatcaaagtcatatttcctttttcctatctggaatcgagctgcgtctgccgagaagcgtctcgtgtcgaatttggcccccgcgccgagccggcgaaagagatcgtggacgtccatctttacccagaaagcgccacagttctac

SEQ ID NO: 12399 - RNA, 4408 nt, Homo sapiens
  source 1..4408: mol_type = other RNA
ctgggaggtcaaggctgcagtgggccatgattgtgccactaaactccaaattaggtaacagaccctgtttctcaaaaaaaaaaaaaaaaacaaaacaaaaaaactcataaagtaaaagttacagtaagctaaggttaatttattgaagaaaaaatatatatctaatatatataatacataatatatataatgtgtgtgtgtgtgtttattttcaagacagtcttgccctgtcgcccaggctggagtgcagtagcgcgatctcggcttactgcaacctccgcctcacaggttcaagctattctcctgcctcagactcctgagtagccgggactatgccaccacacccggctaactttttttggtattttttttagtagagatggggttttgccatgttgcccgggctggtctctaaactcctgagctcagacaacctgcccgcctaggcctcccgaagtgttaggattacaggcatgagccactacgcctggccaagaaaaatattttcaataaatttagtataggttaagtgtgcagtgtttatacaagtctacatgttccaactgtctatagcatgcaggacagtaacatgctatacgggtttgtagcctaggagcaacagactataccatatagcctaggtgtactggtaggctataccatctaggtttgtggaagtaaacaacatgatgtttacacaatgacaatatcacctaacgatgcatttctcagaacatatctctgtcattaagtgatgcgtgactctatttgctcctttatctctaacattacattgtaagggtaaggactgtgttatcaagcctgtattcctaacaaaatctatgtttaagaaatatttattgtgagtttactatgtatcaggtacagtgctaggtactcacaattggagacataattttatagatgagaacactgaaactctgagaaattaagaacttactcaaagtcacacagctggcaaatgggttgcaccagtatacctacctccagaatatatattgggtaaaggatctgtttgcatgaacaaacaaaaaaatcatattcttgtaagtatttttacaccctgtaccagtagatctttctttaaataaattccgaagatgaacaatttttgtcccatctaaaatattcaaagcaaagtccacctgttctgactctagaacaaaaagctacaaatagaggaaataaataagttgaattcaaatgctgctgagaaaaggcaatgtatattatagttctgtggtagtactgataacattcaagtcattcttaggcaccagtcttacgtatatgaagtcactttttcattccattgtacaaaactcatattttgagaaaaatctaatagctaatagtctccaacaccatatgatcataatcctttagcttaagtagagatctacttattaaatgaggcaccatcaacctaaggaaagataagctgtaagagaatgaagacagaggtatatcaagtaacaagaacattcttccttatcaggataaaatgtttatcagtattcaaataaaatatcttaaatggaaagagacaggaaagaacatggttaaatcacagaaaatgaagaaagggagaagctgatcatgatcttgtacaacattatgacagcactaaggtattacgtatccaatacaaggatacttaatagaccaaagaatttaaaatcccagggaactggaataaccagccacaaaagaggcctctctttgttgtggttcacaacacaaaaggccatcaacaaattaggaaatattaaaattaagagagcagcaggtttcttcttggtagacagctcatgctaccatccacaaagtgagcagtggaaggggtatttaatgtcaaggctttattttgaatttctgttccagatgcctctccacagcattcatcacaccttccttcacacttgaagggaaaagtccttaagagttcaccacattttggtgttatttttagcataaacatttgtttttctataagaagtatctctctggattcaaaccacagaaatgtcaatgaatgttatttccattgtataatcatttaaaagtcacctacagagctgggtgcagcagcttgtgcctgtaatctcagttactcaggaggctaaggcaggaggattgtgtgaggtcaggagttcaagaccagcctggacaacatggcaagaccctcatctctacaggaaaaaaaaaaggcacctacaaattgaaactgacttgatagtttaggatcatttatcaccagtcccatgtacttgtagttgatttcaaatgtttggtacaggtgactgtaagacttcaagtattccatgaaaataacattcatgctgggatcataaaattacatttctgggacagtatttttaaagtctgtttttaacttttgtcttcaagagctactttcttcttgctgttctgaccagtgacctttttctgtttatccttagctttttctaagaaacattttggagttgtactaatgctctccctttccaatggtttcttaatcatctttttcttttgtttgcttagtagtttctgaaaaccttttatgtattctggtacaggacacccagcctgctgtataacattagcaacgcttcttaataatggcttatcatcctcagtgaaaaatgtaattgcttttcccttattccctgctcttccagttcgacctatcctgtggatatattccactgagctagttggaaagtcatagttgatcaccaagttcacacctttaaaatcaatccctcttgctagcaaggctgtacaaatcagaacccagatttttcctgctctgaaactgtggactgtgttatctctctgttgttgtgttctctctgcatgaataacatccacattaataccttcatatatgagctcatgaaaaagttctttagccctttcaatggactgaacaaaaacaagaacaggtggattgaaaccctttttaacaagttctctcacggccagaagttttccggtctcagatccaacaaagagaagctcttgttctacagtttctactgcagaattccttgctccaatggacacactgatgacattgtccaggttgagtttgcaccactgttcaacatcatatgcaaaagttgcactgaacatagctcttcggaccttgtgggatgtgcaggccaggaaaatggaagccagctggtctctgaacccagttttgccatcttcaaacagtttatctgattcgtctactacaagccactcaacacttgctaggtcgattccggggggatcttgctttaataaatagattagtcgatttggagtagtcacaagaatatcaaactttttagatgatttaggtccaaatttcttggctgccactgctgctttgtggatcatgtgtattctgaatcctgttccctcagaaatttttattaactctctgtgaatagaaagacttaaaagacttgcccacatggagtaagatccggagcactgtgctgtgtagaggatacttgaccatgacagaagacgtgggccttgctttttaagatctttttattaccttcaaataagaaagatcactgaagtaaaaaccaatcgcatactcttcaaaagctacaagtcatacctggctggcaagttctcgtgttggtgatataatcagggctctgaagcctttatttgcgggttgtttcagctgcattaaaataggaatgctaaaagctaatgtttttccagatccagttggagcagaagccagaagttcccgaccatgcagcataactgggatggcttgcatttggattggcgtaggcatttggaaacctgcatctagaatgttctgaagtagtcgagaattgattttatattcctggtcaagttgctgaaatgtagcaattgggtcaggaagatcggttccttggacgtgaattttgtgtttattccgcaagaagtttatcttttcttttctgagattctccaactttccggaagttagtttactttctctctgaacttttttgtcttcaatctttgcttctacagatgacatccactgtatagtagcaccttcttcttgggaagcaatttctgaagtcatcgtcttcctttttttcttgctctgctccctcttcctttcagttaggctctcttcttttttctctccattttggggcttctgatgtgtttgtgatgctccacacacacctgggacagacttcttgtttccaaaaaagtccagtccctgaagcacctccgaagaatcaaagtcatatttcctttttcctatctggaatcgagctgcgtctgccgagaagcgtctcgtgtcgaatttggcccccgcgccgagccggcgaaagagatcgtggacgtccatctttacccagaaagc

SEQ ID NO: 12400 - RNA, 4238 nt, Homo sapiens
  source 1..4238: mol_type = other RNA
ctgggaggtcaaggctgcagtgggccatgattgtgccactaaactccaaattaggtaacagaccctgtttctcaaaaaaaaaaaaaaaaacaaaacaaaaaaactcataaagtaaaagttacagtaagctaaggttaatttattgaagaaaaaatatatatctaatatatataatacataatatatataatgtgtgtgtgtgtgtttattttcaagacagtcttgccctgtcgcccaggctggagtgcagtagcgcgatctcggcttactgcaacctccgcctcacaggttcaagctattctcctgcctcagactcctgagtagccgggactatgccaccacacccggctaactttttttggtattttttttagtagagatggggttttgccatgttgcccgggctggtctctaaactcctgagctcagacaacctgcccgcctaggcctcccgaagtgttaggattacaggcatgagccactacgcctggccaagaaaaatattttcaataaatttagtataggttaagtgtgcagtgtttatacaagtctacatgttccaactgtctatagcatgcaggacagtaacatgctatacgggtttgtagcctaggagcaacagactataccatatagcctaggtgtactggtaggctataccatctaggtttgtggaagtaaacaacatgatgtttacacaatgacaatatcacctaacgatgcatttctcagaacatatctctgtcattaagtgatgcgtgactctatttgctcctttatctctaacattacattgtaagggtaaggactgtgttatcaagcctgtattcctaacaaaatctatgtttaagaaatatttattgtgagtttactatgtatcaggtacagtgctaggtactcacaattggagacataattttatagatgagaacactgaaactctgagaaattaagaacttactcaaagtcacacagctggcaaatgggttgcaccagtatacctacctccagaatatatattgggtaaaggatctgtttgcatgaacaaacaaaaaaatcatattcttgtaagtatttttacaccctgtaccagtagatctttctttaaataaattccgaagatgaacaatttttgtcccatctaaaatattcaaagcaaagtccacctgttctgactctagaacaaaaagctacaaatagaggaaataaataagttgaattcaaatgctgctgagaaaaggcaatgtatattatagttctgtggtagtactgataacattcaagtcattcttaggcaccagtcttacgtatatgaagtcactttttcattccattgtacaaaactcatattttgagaaaaatctaatagctaatagtctccaacaccatatgatcataatcctttagcttaagtagagatctacttattaaatgaggcaccatcaacctaaggaaagataagctgtaagagaatgaagacagaggtatatcaagtaacaagaacattcttccttatcaggataaaatgtttatcagtattcaaataaaatatcttaaatggaaagagacaggaaagaacatggttaaatcacagaaaatgaagaaagggagaagctgatcatgatcttgtacaacattatgacagcactaaggtattacgtatccaatacaaggatacttaatagaccaaagaatttaaaatcccagggaactggaataaccagccacaaaagaggcctctctttgttgtggttcacaacacaaaaggccatcaacaaattaggaaatattaaaattaagagagcagcaggtttcttcttggtagacagctcatgctaccatccacaaagtgagcagtggaaggggtatttaatgtcaaggctttattttgaatttctgttccagatgcctctccacagcattcatcacaccttccttcacacttgaagggaaaagtccttaagagttcaccacattttggtgttatttttagcataaacatttgtttttctataagaagtatctctctggattcaaaccacagaaatgtcaatgaatgttatttccattgtataatcatttaaaagtcacctacagagctgggtgcagcagcttgtgcctgtaatctcagttactcaggaggctaaggcaggaggattgtgtgaggtcaggagttcaagaccagcctggacaacatggcaagaccctcatctctacaggaaaaaaaaaaggcacctacaaattgaaactgacttgatagtttaggatcatttatcaccagtcccatgtacttgtagttgatttcaaatgtttggtacaggtgactgtaagacttcaagtattccatgaaaataacattcatgctgggatcataaaattacatttctgggacagtatttttaaagtctgtttttaacttttgtcttcaagagctactttcttcttgctgttctgaccagtgacctttttctgtttatccttagctttttctaagaaacattttggagttgtactaatgctctccctttccaatggtttcttaatcatctttttcttttgtttgcttagtagtttctgaaaaccttttatgtattctggtacaggacacccagcctgctgtataacattagcaacgcttcttaataatggcttatcatcctcagtgaaaaatgtaattgcttttcccttattccctgctcttccagttcgacctatcctgtggatatattccactgagctagttggaaagtcatagttgatcaccaagttcacacctttaaaatcaatccctcttgctagcaaggctgtacaaatcagaacccagatttttcctgctctgaaactgtggactgtgttatctctctgttgttgtgttctctctgcatgaataacatccacattaataccttcatatatgagctcatgaaaaagttctttagccctttcaatggactgaacaaaaacaagaacaggtggattgaaaccctttttaacaagttctctcacggccagaagttttccggtctcagatccaacaaagagaagctcttgttctacagtttctactgcagaattccttgctccaatggacacactgatgacattgtccaggttgagtttgcaccactgttcaacatcatatgcaaaagttgcactgaacatagctcttcggaccttgtgggatgtgcaggccaggaaaatggaagccagctggtctctgaacccagttttgccatcttcaaacagtttatctgattcgtctactacaagccactcaacacttgctaggtcgattccggggggatcttgctttaataaatagattagtcgatttggagtagtcacaagaatatcaaactttttagatgatttaggtccaaatttcttggctgccactgctgctttgtggatcatgtgtattctgaatcctgttccctcagaaatttttattaactctctgtgaatctggctggcaagttctcgtgttggtgatataatcagggctctgaagcctttatttgcgggttgtttcagctgcattaaaataggaatgctaaaagctaatgtttttccagatccagttggagcagaagccagaagttcccgaccatgcagcataactgggatggcttgcatttggattggcgtaggcatttggaaacctgcatctagaatgttctgaagtagtcgagaattgattttatattcctggtcaagttgctgaaatgtagcaattgggtcaggaagatcggttccttggacgtgaattttgtgtttattccgcaagaagtttatcttttcttttctgagattctccaactttccggaagttagtttactttctctctgaacttttttgtcttcaatctttgcttctacagatgacatccactgtatagtagcaccttcttcttgggaagcaatttctgaagtcatcgtcttcctttttttcttgctctgctccctcttcctttcagttaggctctcttcttttttctctccattttggggcttctgatgtgtttgtgatgctccacacacacctgggacagacttcttgtttccaaaaaagtccagtccctgaagcacctccgaagaatcaaagtcatatttcctttttcctatctggaatcgagctgcgtctgccgagaagcgtctcgtgtcgaatttggcccccgcgccgagccggcgaaagagatcgtggacgtccatctttacccagaaagcgccacagttct

SEQ ID NO: 12401 - RNA, 4353 nt, Homo sapiens
  source 1..4353: mol_type = other RNA
ctgggaggtcaaggctgcagtgggccatgattgtgccactaaactccaaattaggtaacagaccctgtttctcaaaaaaaaaaaaaaaaacaaaacaaaaaaactcataaagtaaaagttacagtaagctaaggttaatttattgaagaaaaaatatatatctaatatatataatacataatatatataatgtgtgtgtgtgtgtttattttcaagacagtcttgccctgtcgcccaggctggagtgcagtagcgcgatctcggcttactgcaacctccgcctcacaggttcaagctattctcctgcctcagactcctgagtagccgggactatgccaccacacccggctaactttttttggtattttttttagtagagatggggttttgccatgttgcccgggctggtctctaaactcctgagctcagacaacctgcccgcctaggcctcccgaagtgttaggattacaggcatgagccactacgcctggccaagaaaaatattttcaataaatttagtataggttaagtgtgcagtgtttatacaagtctacatgttccaactgtctatagcatgcaggacagtaacatgctatacgggtttgtagcctaggagcaacagactataccatatagcctaggtgtactggtaggctataccatctaggtttgtggaagtaaacaacatgatgtttacacaatgacaatatcacctaacgatgcatttctcagaacatatctctgtcattaagtgatgcgtgactctatttgctcctttatctctaacattacattgtaagggtaaggactgtgttatcaagcctgtattcctaacaaaatctatgtttaagaaatatttattgtgagtttactatgtatcaggtacagtgctaggtactcacaattggagacataattttatagatgagaacactgaaactctgagaaattaagaacttactcaaagtcacacagctggcaaatgggttgcaccagtatacctacctccagaatatatattgggtaaaggatctgtttgcatgaacaaacaaaaaaatcatattcttgtaagtatttttacaccctgtaccagtagatctttctttaaataaattccgaagatgaacaatttttgtcccatctaaaatattcaaagcaaagtccacctgttctgactctagaacaaaaagctacaaatagaggaaataaataagttgaattcaaatgctgctgagaaaaggcaatgtatattatagttctgtggtagtactgataacattcaagtcattcttaggcaccagtcttacgtatatgaagtcactttttcattccattgtacaaaactcatattttgagaaaaatctaatagctaatagtctccaacaccatatgatcataatcctttagcttaagtagagatctacttattaaatgaggcaccatcaacctaaggaaagataagctgtaagagaatgaagacagaggtatatcaagtaacaagaacattcttccttatcaggataaaatgtttatcagtattcaaataaaatatcttaaatggaaagagacaggaaagaacatggttaaatcacagaaaatgaagaaagggagaagctgatcatgatcttgtacaacattatgacagcactaaggtattacgtatccaatacaaggatacttaatagaccaaagaatttaaaatcccagggaactggaataaccagccacaaaagaggcctctctttgttgtggttcacaacacaaaaggccatcaacaaattaggaaatattaaaattaagagagcagcaggtttcttcttggtagacagctcatgctaccatccacaaagtgagcagtggaaggggtatttaatgtcaaggctttattttgaatttctgttccagatgcctctccacagcattcatcacaccttccttcacacttgaagggaaaagtccttaagagttcaccacattttggtgttatttttagcataaacatttgtttttctataagaagtatctctctggattcaaaccacagaaatgtcaatgaatgttatttccattgtataatcatttaaaagtcacctacagagctgggtgcagcagcttgtgcctgtaatctcagttactcaggaggctaaggcaggaggattgtgtgaggtcaggagttcaagaccagcctggacaacatggcaagaccctcatctctacaggaaaaaaaaaaggcacctacaaattgaaactgacttgatagtttaggatcatttatcaccagtcccatgtacttgtagttgatttcaaatgtttggtacaggtgactgtaagacttcaagtattccatgaaaataacattcatgctgggatcataaaattacatttctgggacagtatttttaaagtctgtttttaacttttgtcttcaagagctactttcttcttgctgttctgaccagtgacctttttctgtttatccttagctttttctaagaaacattttggagttgtactaatgctctccctttccaatggtttcttaatcatctttttcttttgtttgcttagtagtttctgaaaaccttttatgtattctggtacaggacacccagcctgctgtataacattagcaacgcttcttaataatggcttatcatcctcagtgaaaaatgtaattgcttttcccttattccctgctcttccagttcgacctatcctgtggatatattccactgagctagttggaaagtcatagttgatcaccaagttcacacctttaaaatcaatccctcttgctagcaaggctgtacaaatcagaacccagatttttcctgctctgaaactgtggactgtgttatctctctgttgttgtgttctctctgcatgaataacatccacattaataccttcatatatgagctcatgaaaaagttctttagccctttcaatggactgaacaaaaacaagaacaggtggattgaaaccctttttaacaagttctctcacggccagaagttttccggtctcagatccaacaaagagaagctcttgttctacagtttctactgcagaattccttgctccaatggacacactgatgacattgtccaggttgagtttgcaccactgttcaacatcatatgcaaaagttgcactgaacatagctcttcggaccttgtgggatgtgcaggccaggaaaatggaagccagctggtctctgaacccagttttgccatcttcaaacagtttatctgattcgtctactacaagccactcaacacttgctaggtcgattccggggggatcttgctttaataaatagattagtcgatttggagtagtcacaagaatatcaaactttttagatgatttaggtccaaatttcttggctgccactgctgctttgtggatcatgtgtattctgaatcctgttccctcagaaatttttattaactctctgtgaatctggctggcaagttctcgtgttggtgatataatcagggctctgaagcctttatttgcgggttgtttcagctgcattaaaataggaatgctaaaagctaatgtttttccagatccagttggagcagaagccagaagttcccgaccatgcagcataactgggatggcttgcatttggattggcgtaggcatttggaaacctgcatctagaatgttctgaagtagtcgagaattgattttatattcctggtcaagttgctgaaatgtagcaattgggtcaggaagatcggttccttggacgtgaattttgtgtttattccgcaagaagtttatcttttcttttctgagattctccaactttccggaagttagtttactttctctctgaacttttttgtcttcaatctttgcttctacagatgacatccactgtatagtagcaccttcttcttgggaagcaatttctggctgggcgtggtggctcacatctgtaatcccagcactttgggagcccaaggtgggtgaatcacgaggtcaggagatcgagaccatactggctaacatggtgaaaccctgtctctgaagtcatcgtcttcctttttttcttgctctgctccctcttcctttcagttaggctctcttcttttttctctccattttggggcttctgatgtgtttgtgatgctccacacacacctgggacagacttcttgtttccaaaaaagtccagtccctgaagcacctccgaagaatcaaagtcatatttcctttttcctatctggaatcgagctgcgtctgccgagaagcgtctcgtgtcgaatttggcccccgcgccgagccggcgaaagagatcgtggacgtccatctttacccagaaagcgccacagttct

SEQ ID NO: 12402 - RNA, 5049 nt, Homo sapiens
  source 1..5049: mol_type = other RNA
ctgggaggtcaaggctgcagtgggctaagatcgcaccactgcactccagcctgggcaacagagtaagaccctgtctcaaaaaaaaaaaaaaaagattaaatgcaaaggcttattcggggaactctgtatgtaagttggcaaagaccaaaatagtgccaacatatgaagcactgaaaaagaaaaagttaaaatatcttagcctcaacactcgaaatatagcaagcccacatatttgaagaccaaacacatcaagactcatctttcccttaaaagaattttcagctgggcacagtggctcgtgcctgtaatcccagcactttgggaggctgaggcgggtggattactttagaccaggagtttgggaccagcctggccaaaatgtgaaacccccgtctctactaaaaatataaaaattagccgagactggtggtgcacacctgtagtcccagctattcaggagactgagacaagactcgcttgaacccaggaggtggaggctgcagtgagccaacattgcaccactgcactccagcctagacaacagagtgagactttgtcacaaaaaaaaaaaagagagaatttttctttgtcagatgtagaatataacttaagagaaatttattaacatttaagctccttagtatagaaaactggaggaaaataactttagtacacacttaatttgctatactaaatttttttaataaagaccttcaaaaggaaaatttagattataagtagcatggcacatatagaatatgaacacagaaagttcatatctaagccctaagccacttatgataaacacctataaaaggaacaaaaactaaacttccacattattttacccagtaaaagatgtaggctattagtagaaagttggttaagtaaattcaaaaaataaaaatataaaaaagaaataatgagaaaatttttgaaaaatattaataaaataaagatgtaggctacatagctgaggctattattcacaccatatagaaattaggttctcgggccaagcagaaactataacataatcagaaagaatacctaaagaaataaagtatgacttcctaaattttttattttaaaaatgcccagtttatttatttgctttgcctaagatagctgcattcattattacagggtcaggggacttgtaaaaacaaatatcaattattataaataatcacagaaaacaaataaactggaaaataaacagcggttactaatttaaggttttaacccttaccccaaccacccaaaaaaagtagccatttttaaaataaagattaagagttggtggaatttaagggaaatgccatccggtaatgttacctaaatactagaaaggaatcagcacaaggaaacaggaacaaagcagtgcagtacttcggtattacagcgccacccactggctagaagtcctcatagcacatatgagatgtagccataaaatagatgaattcttgaaataaggaatataacactgactattctgattcagtagaacataaaaaatgtctaacaaaacagaaccagacacattatattatttctacaagtaaacagaatatctattagatatgttcacaagggttttatcaattttgaaatccaagtgtataatccccaaatgctgtaaggacttaaattttatagccaaaacaattaacacataaaatgctatttcatctctgtagctgaatacataaatagtatctttaagtaaaagatgcatacttgcatttcattgctaagcaattcataatatatttaaatgctggtaaaacctacaatggcatctgcttcacttctacctttactagagaagtaacaaaatacactgagcaaaggatatgtccaaaaaactaaactgaaaaacagtttctaaataaagtccacagaccattcagataaactagtaaaaatagtttttctttaaagtaccacagcacctttgtagttcaaaatatatttaccataggctgggcgtggtggctcacgcctgtaatcccagcactttgggaagctgaggcaggcagatcacaaggtcaggagatcgagaccatcctgtgaatggtgaaaccctgtctctactaaaaatataaaaaaaattagcccggcatggtggcgggcacctgtagtcccagctactcaggaggctgaggcaggagaatggtgtgaacccaggaggcagagcttgcagtgagccgagattgcaccactgcactccagcctgggcgacagagcaagactctgtctcaaaaaaaaaaaaaaaaaaaaaaaaaaaaatatatatatatatatatatatatatatatatatatatcgtaatatatctctttattatcctagtgacatctgttgtgattttccaaatcactatttattttcttaaataccaacattcttaaaatcttggcatgaaatatttgagagttacttctcctgaagtacaatctttcctttaagacccagaattacatatagggcatgacattaatttatagtctatatgaccctcttgaatgttgttctctaaaggctggacttcagaattcctctacagacatgaccccagtcttccaagtgagaattcacaaatatgctccaggcagtcaggacaggcttcaagtttctttggtttgatgataattatcacttggcctgcaaaagccaaggtctttgcttgctcatagatggttgattgcagataaaaatatgatgagaaaagtaacattcccacagacataaattgccaacactgcctttttaaaagcatgaccctctgtttccactgcagtaaatgactgaaggatctgaattctgtcatcatccaatatttcaactccagaacaacctcagtcccaacatgccaggctacgaatccggtcattgcataggttttccatgaatcaggaagattcagtcctggtaaatccattcccaggaacatcgctgccactgctattattctagcagctgttcccatactccaatgagtccagttaaacatttgccttcttgggtcatgtaaaggtggcctgaagactgccagaagaggctgaagaactgccaaagtcatcactatacagccgaggtatgggtggtaacctgcatgcctactccagcctcccctgtatataaacggcataacaaaagcaatgcaggtgaggacagttgtggtgaacatgagcatccgatgcacctgaaaccaagctgcttcaccaagcaagaaagcttttgaccaaactggcttgaagaaccgggcaaccagtacacctatgctaacagtagtcatccatgccacaaacattaaggcaccatgaaccttcagaaggagtacagaatgggatcctcctatgttctttggagagtctgtcacatcatatttttcataggtaatcaaaggttgctgagagtgcttgtaaattcgaccatcattagctgcaccatctgctagaaatatgtaatagcttgtgtttagatcaaatctattcttaactccaggaagggtaatgtttcttctgaaagaacactgcataacaccgtccgccaacctccaagccatatcctcaagggtatccctggagtccattacagggtgacttcgccccgttaaatgggaaggctggatgtacacagtctgatcttcatgaatacacagataagcatcatcatcacccatccactgatcatgagacaatgcaaaggataaatagcctttactggggccgctcatttcaaccatcaccgattggtcatctcttgtgaaggacaagaagacacaggaagcctccttctctgggtcacagttcaaaggactcctaatacagaacttcttgttcccacaatctgaggcactgaatggtttggttaagtgggaaacgggaggtaacgttggcaaaggtactactgtagctttaggtgttgtaaaaggaaatgcatttggttgtgaaattataggaccaggaatcttcacccagtagattttatacttctcaacaactgtgactagaaactgtgtgtgatttggagcactgcttggagcattccagtagactttaatttctgtttttttagatgcacttctgtgactcactgctgatccctgtatatcttcacaggtcaaaagttgtgacacttcactgtcaatcaatgtgaaggagccaataggagggccattcagatcctcagcattacgcgcttctaggagaaagcctttaaatggatgccctgacaaagtaacttcaatctgatctcctggcctgaatgtcatctgactcacgtaaatgtcatgaacaggaacagactgtggactatgaccatgttcaggaatcattccatggcatgactgtgttacttttccattgggataattagccacataactaatgtgcaacagaagtatgcaggtaccaagagtaaatccagaaactgccatctgataaaaagaatgtgatatgtgaagtttcacccgaatttcaatctcagctctacaaattactgtgagactttgggcaaatcatttaatcctccacttccttaccacttttttaaaaatacagaagtggctgggcgcggtggctcacgcctgtaatcccagcactttgggaggccgaggcaggcagatgacctgacgctgggagttcgaaaccagactgaccaacatggagaaaccccgtttctactaaaaatacaaaattagccgggtgtggtggtgcctgcctgtaatcccagctactcaggaggctgaggcaggagaattgcttgaacccgggaggcagaggttgcagtgagccgaaatcccgccgttgcactccagcctgggccacaagagcaacactccgtctcgaaaataataaataaataggccagacgcggtggctcaagcctgtaatcccagcactttgggaggcggaggcgggcatatcacgaggtcaggagatagagaccatccttgccaacacagtgaaaccccgtctctactaaaaatacaaaaaattagccgggcgtggtggcgggcgcctgtaatcccagcagtat

SEQ ID NO: 12403 - RNA, 4609 nt, Homo sapiens
  source 1..4609: mol_type = other RNA
ctgggaggtcaaggctgcagtgggctaagatcgcaccactgcactccagcctgggcaacagagtaagaccctgtctcaaaaaaaaaaaaaaaagattaaatgcaaaggcttattcggggaactctgtatgtaagttggcaaagaccaaaatagtgccaacatatgaagcactgaaaaagaaaaagttaaaatatcttagcctcaacactcgaaatatagcaagcccacatatttgaagaccaaacacatcaagactcatctttcccttaaaagaattttcagctgggcacagtggctcgtgcctgtaatcccagcactttgggaggctgaggcgggtggattactttagaccaggagtttgggaccagcctggccaaaatgtgaaacccccgtctctactaaaaatataaaaattagccgagactggtggtgcacacctgtagtcccagctattcaggagactgagacaagactcgcttgaacccaggaggtggaggctgcagtgagccaacattgcaccactgcactccagcctagacaacagagtgagactttgtcacaaaaaaaaaaaagagagaatttttctttgtcagatgtagaatataacttaagagaaatttattaacatttaagctccttagtatagaaaactggaggaaaataactttagtacacacttaatttgctatactaaatttttttaataaagaccttcaaaaggaaaatttagattataagtagcatggcacatatagaatatgaacacagaaagttcatatctaagccctaagccacttatgataaacacctataaaaggaacaaaaactaaacttccacattattttacccagtaaaagatgtaggctattagtagaaagttggttaagtaaattcaaaaaataaaaatataaaaaagaaataatgagaaaatttttgaaaaatattaataaaataaagatgtaggctacatagctgaggctattattcacaccatatagaaattaggttctcgggccaagcagaaactataacataatcagaaagaatacctaaagaaataaagtatgacttcctaaattttttattttaaaaatgcccagtttatttatttgctttgcctaagatagctgcattcattattacagggtcaggggacttgtaaaaacaaatatcaattattataaataatcacagaaaacaaataaactggaaaataaacagcggttactaatttaaggttttaacccttaccccaaccacccaaaaaaagtagccatttttaaaataaagattaagagttggtggaatttaagggaaatgccatccggtaatgttacctaaatactagaaaggaatcagcacaaggaaacaggaacaaagcagtgcagtacttcggtattacagcgccacccactggctagaagtcctcatagcacatatgagatgtagccataaaatagatgaattcttgaaataaggaatataacactgactattctgattcagtagaacataaaaaatgtctaacaaaacagaaccagacacattatattatttctacaagtaaacagaatatctattagatatgttcacaagggttttatcaattttgaaatccaagtgtataatccccaaatgctgtaaggacttaaattttatagccaaaacaattaacacataaaatgctatttcatctctgtagctgaatacataaatagtatctttaagtaaaagatgcatacttgcatttcattgctaagcaattcataatatatttaaatgctggtaaaacctacaatggcatctgcttcacttctacctttactagagaagtaacaaaatacactgagcaaaggatatgtccaaaaaactaaactgaaaaacagtttctaaataaagtccacagaccattcagataaactagtaaaaatagtttttctttaaagtaccacagcacctttgtagttcaaaatatatttaccataggctgggcgtggtggctcacgcctgtaatcccagcactttgggaagctgaggcaggcagatcacaaggtcaggagatcgagaccatcctgtgaatggtgaaaccctgtctctactaaaaatataaaaaaaattagcccggcatggtggcgggcacctgtagtcccagctactcaggaggctgaggcaggagaatggtgtgaacccaggaggcagagcttgcagtgagccgagattgcaccactgcactccagcctgggcgacagagcaagactctgtctcaaaaaaaaaaaaaaaaaaaaaaaaaaaaatatatatatatatatatatatatatatatatatatatcgtaatatatctctttattatcctagtgacatctgttgtgattttccaaatcactatttattttcttaaataccaacattcttaaaatcttggcatgaaatatttgagagttacttctcctgaagtacaatctttcctttaagacccagaattacatatagggcatgacattaatttatagtctatatgaccctcttgaatgttgttctctaaaggctggacttcagaattcctctacagacatgaccccagtcttccaagtgagaattcacaaatatgctccaggcagtcaggacaggcttcaagtttctttggtttgatgataattatcacttggcctgcaaaagccaaggtctttgcttgctcatagatggttgattgcagataaaaatatgatgagaaaagtaacattcccacagacataaattgccaacactgcctttttaaaagcatgaccctctgtttccactgcagtaaatgactgaaggatctgaattctgtcatcatccaatatttcaactttgcgagagagccgataagcatgtacctccagaacaacctcagtcccaacatgccaggctacgaatccggtcattgcataggttttccatgaatcaggaagattcagtcctggtaaatccattcccaggaacatcgctgccactgctattattctagcagctgttcccatactccaatgagtccagttaaacatttgccttcttgggtcatgtaaaggtggcctgaagactgccagaagaggctgaagaactgccaaagtcatcactatacagccgaggtatgggtggtaacctgcatgcctactccagcctcccctgtatataaacggcataacaaaagcaatgcaggtgaggacagttgtggtgaacatgagcatccgatgcacctgaaaccaagctgcttcaccaagcaagaaagcttttgaccaaactggcttgaagaaccgggcaaccagtacacctatgctaacagtagtcatccatgccacaaacattaaggcaccatgaaccttcagaaggagtacagaatgggatcctcctatgttctttggagagtctgtcacatcatatttttcataggtaatcaaaggttgctgagagtgcttgtaaattcgaccatcattagctgcaccatctgctagaaatatgtaatagcttgtgtttagatcaaatctattcttaactccaggaagggtaatgtttcttctgaaagaacactgcataacaccgtccgccaacctccaagccatatcctcaagggtatccctggagtccattacagggtgacttcgccccgttaaatgggaaggctggatgtacacagtctgatcttcatgaatacacagataagcatcatcatcacccatccactgatcatgagacaatgcaaaggataaatagcctttactggggccgctcatttcaaccatcaccgattggtcatctcttgtgaaggacaagaagacacaggaagcctccttctctgggtcacagttcaaaggactcctaatacagaacttcttgttcccacaatctgaggcactgaatggtttggttaagtgggaaacgggaggtaacgttggcaaaggtactactgtagctttaggtgttgtaaaaggaaatgcatttggttgtgaaattataggaccaggaatcttcacccagtagattttatacttctcaacaactgtgactagaaactgtgtgtgatttggagcactgcttggagcattccagtagactttaatttctgtttttttagatgcacttctgtgactcactgctgatccctgtatatcttcacaggtcaaaagttgtgacacttcactgtcaatcaatgtgaaggagccaataggagggccattcagatcctcagcattacgcgcttctaggagaaagcctttaaatggatgccctgacaaagtaacttcaatctgatctcctggcctgaatgtcatctgactcacgtaaatgtcatgaacaggaacagactgtggactatgaccatgttcaggaatcattccatggcatgactgtgttacttttccattgggataattagccacataactaatgtgcaacagaagtatgcaggtaccaagagtaaatccagaaactgccatctgataaaaagaatgtgatatgtgaagtttcacccgaatttcaatctcagctctacaaattactgtgagactttgggcaaatcatttaatcctccacttccttaccttgagaagcgaaggcagcctaaccaact

SEQ ID NO: 12404 - RNA, 68 nt, Homo sapiens
  source 1..68: mol_type = other RNA
ctgggaggtcaaggctgcagtgggctatgatcacaccactgcactccagcctgtgcgacagagcaaga

SEQ ID NO: 12405 - RNA, 335 nt, Homo sapiens
  source 1..335: mol_type = other RNA
ctgggaggtcaaggctgcagttatctgaaggcttgactgggcgtggagggtgtgttttgaaggtaactcattcttacggttctaagttgacacttgctgttgttgaaaggcttcagttccacactacatgggcctttctagacagctcaagtgaaaaggcagttggttttccccttcaggcgtttgatcatctcgtccgtggtgatcttgtcggtgatctcttttacccccggagggtaagcgatcttcccgtcggcactcacgacgccacagagggcagtggcaggcttgggctgcgcggtgaagtccatcctgggggacaacttttggttcac

SEQ ID NO: 12406 - RNA, 3302 nt, Homo sapiens
  source 1..3302: mol_type = other RNA
ctgggaggtgtgatatcgtggtatctacccaaagtgttcacagcagtgaaataacacaatgtatgggattttaagatacttaagcaaacaaaaaaatgacaaatgaagcaaacatggtaagatagtgataagtgtcagatctggatgttgagtaccaatgcactattctagttttgtgtaatttttaaatttcttcattaaaaattgttttacagactccctcctagacacagcatgccagagtctccaaaggcctagctcaggaatctattcttaagctcccaacaagaatcttacatagtcaggcaggcaatgatcattatttgaggaccattagaaatgatctaatacataccctccaaacttcacatttttagtattctcattttctactcagtaagctcaatttcacagtttcttatattcaccatggcattctgccaaggaactacaactcgtgttctctaaacccatctgttctaagaatgctggactggttatcaacttctaatgcaccctgcttaaactttcctctctcaatttgtccctgactgaactgcagacgacagaacaactgtactaaccatctctttctgcatattccatgtctccacagaggtcactgtgtcttcacaaagctaactgccacaattttcacaggttgtatttttccttcatgattttccattttctacttgagcattaaaatatcagggagaaaaagaagataaccatatagataatcatattgttggtaaaataagatatgtgccccagcatagtatatgctaagtattcagaatctatagttatattagctaacaggtcaagaatgccaaagaagtaatttctcaagatttaaaaaaattaactgtcttaggtgatattcaaaaatgcacatcaacccaattaaaaccacattttctacagctggatgtaacaatcttattccaaatcatccacttaagttgtttaacttacttaaagtaaggctctagacatttgcttcttcaaaagtatcttgcaaggccgttatgaggtagaagacaagtttaaatggaccatatttttctactccattgtaactaaaattactactcacaggaagtatatagcttatgcattttggtccatcacactttccaccatcatgagtatactcttaaggttctcactttaccatcagcataatatattttgcttccagaatgcccagtaaagctgacgtttttcatttaaagtgattaaaaaaaaattccccaaatatctatttaacaatcttagatctgagttttggcaagacagtttaatgcatacaaaatgaaacactacatttctcactctctctcacacacaaacacgcacacacagattaaaatcccaaagttttcactatttttcctctaccttacacagctcaatttttaacatgcagcttacttgtaatctaaaaataattttaaacatgattgtcataaaaatattttaaaacagagatgaaatgtataaaggcacacatagattgtcaatggttacatcagttacatcacatttcttcagaaacaacagacctgtttctgctcctgtaaacaaacttttttctcacacttttaaagtgaggttagtgctgacataaaattattgctctactcacagtcttgagtgttggcactgtttgaggtacattttctccatctacacacccctaccactcttgagagtatgagtcaacagaagtctgcaggttaaacccattcaatagtattttcatcaatactggaatgatagcaagtaacattacaaaacatcagagataaaaaatgttcaatgttgaggcccaagattttaacttattcttcattacctgaaaatactgcttacttaacttctttaggaaaaaaaaaattattctggagatgagtaattccttcctgaatacttcatccaagacgattccttcacacttatcttctgattctttgttttcatccatttgattaagcagtcaccaagaatcacttttcctttggtgatctggcataacgatctcttacactttttgctagttgtttgataaatattttgtaaatttttccacagtatgtatgcactgttttttgtagttccagttctaaaggttttaataaggaacggatgttgtcatcttcaaaagaacaatttctcagtgcttcataaacagctctaaatgctggttgcttatcgtcatggtaaacacctctgttcccatgaagaataaagattcctccttcttctgcttcttggcaattgcttccatatatacaatgatctggtcgataattccattgacacggaaaaacaaaaaggctttctggattatgaaaaaacacgatattcaatagatcttgatcaccccatgtgatgtttagtttgtattttttaagcaatggcataagtatatctccccattgtagtcgtacagttgtcatatcattcttgaaatacttccttctcattcgagtcatgttcatcaacataactccagagtttactccagtttttccataatatggatgcctagcaaagcgattataccatcctattcgaggttcctcatgttctggtgccattgcagcaatttgtgtggaattaaatttctttagtaaagaccaaatatcatcaactggtcgtaaaaaaaggatatcagtgtcgacatacaatagtgagtcaacttctttcaggattaacggcaagaacaatctctgcgaagcacatggtttaaagagttttttccactctgctgcattctcacttggaaaggttatggggtataacgtataattaaatgtttgtagaaatgaccagttgtcaagtctgcctttaaagctatgatgtagctgatcttcagcaaaaatatggaattgaagaggtttgatgctgaaaatgatagctgacttcaacatggtcatagtttcttccagtctttcaccacaggcaactacagctagatgcattttctcaacaggctgtattttcagactgtacaatgcagttcttacagagaggagaatggtggttaccaggcactggaggtgaaggggtgggagagagtatgtgatggaaagatgttgaccaaagaatacaatacaaacttccagtcagaaggaataagttctcaagatctactgcacagcaaggtgtctacagataattatgtttatttcaaaactaaaagccgcttcccaaaagcagttcattccacaaacatcagagggcagcatccaatagggattccagtaacacagagagaaatctttacacct

SEQ ID NO: 12407 - RNA, 3566 nt, Homo sapiens
  source 1..3566: mol_type = other RNA
ctgggaggtgtgatatcgtggtatctacccaaagtgttcacagcagtgaaataacacaatgtatgggattttaagatacttaagcaaacaaaaaaatgacaaatgaagcaaacatggtaagatagtgataagtgtcagatctggatgttgagtaccaatgcactattctagttttgtgtaatttttaaatttcttcattaaaaattgttttacagactccctcctagacacagcatgccagagtctccaaaggcctagctcaggaatctattcttaagctcccaacaagaatcttacatagtcaggcaggcaatgatcattatttgaggaccattagaaatgatctaatacataccctccaaacttcacatttttagtattctcattttctactcagtaagctcaatttcacagtttcttatattcaccatggcattctgccaaggaactacaactcgtgttctctaaacccatctgttctaagaatgctggactggttatcaacttctaatgcaccctgcttaaactttcctctctcaatttgtccctgactgaactgcagacgacagaacaactgtactaaccatctctttctgcatattccatgtctccacagaggtcactgtgtcttcacaaagctaactgccacaattttcacaggttgtatttttccttcatgattttccattttctacttgagcattaaaatatcagggagaaaaagaagataaccatatagataatcatattgttggtaaaataagatatgtgccccagcatagtatatgctaagtattcagaatctatagttatattagctaacaggtcaagaatgccaaagaagtaatttctcaagatttaaaaaaattaactgtcttaggtgatattcaaaaatgcacatcaacccaattaaaaccacattttctacagctggatgtaacaatcttattccaaatcatccacttaagttgtttaacttacttaaagtaaggctctagacatttgcttcttcaaaagtatcttgcaaggccgttatgaggtagaagacaagtttaaatggaccatatttttctactccattgtaactaaaattactactcacaggaagtatatagcttatgcattttggtccatcacactttccaccatcatgagtatactcttaaggttctcactttaccatcagcataatatattttgcttccagaatgcccagtaaagctgacgtttttcatttaaagtgattaaaaaaaaattccccaaatatctatttaacaatcttagatctgagttttggcaagacagtttaatgcatacaaaatgaaacactacatttctcactctctctcacacacaaacacgcacacacagattaaaatcccaaagttttcactatttttcctctaccttacacagctcaatttttaacatgcagcttacttgtaatctaaaaataattttaaacatgattgtcataaaaatattttaaaacagagatgaaatgtataaaggcacacatagattgtcaatggttacatcagttacatcacatttcttcagaaacaacagacctgtttctgctcctgtaaacaaacttttttctcacacttttaaagtgaggttagtgctgacataaaattattgctctactcacagtcttgagtgttggcactgtttgaggtacattttctccatctacacacccctaccactcttgagagtatgagtcaacagaagtctgcaggttaaacccattcaatagtattttcatcaatactggaatgatagcaagtaacattacaaaacatcagagataaaaaatgttcaatgttgaggcccaagattttaacttattcttcattacctgaaaatactgcttacttaacttctttaggaaaaaaaaaattattctggagatgagtaattccttcctgaatacttcatccaagacgattccttcacacttatcttctgattctttgttttcatccatttgattaagcagtcaccaagaatcacttttcctttggtgatctggcataacgatctcttacactttttgctagttgtttgataaatattttgtaaatttttccacagtatgtatgcactgttttttgtagttccagttctaaaggttttaataaggaacggatgttgtcatcttcaaaagaacaatttctcagtgcttcataaacagctctaaatgctggttgcttatcgtcatggtaaacacctctgttcccatgaagaataaagattcctccttcttctgcttcttggcaattgcttccatatatacaatgatctggtcgataattccattgacacggaaaaacaaaaaggctttctggattatgaaaaaacacgatattcaatagatcttgatcaccccatgtgatgtttagtttgtattttttaagcaatggcataagtatatctccccattgtagtcgtacagttgtcatatcattcttgaaatacttccttctcattcgagtcatgttcatcaacataactccagagtttactccagtttttccataatatggatgcctagcaaagcgattataccatcctattcgaggttcctcatgttctggtgccattgcagcaatttgtgtggaattaaatttctttagtaaagaccaaatatcatcaactggtcgtaaaaaaaggatatcagtgtcgacatacaatagtgagtcaacttctttcaggattaacggcaagaacaatctctgcgaagcacatggtttaaagagttttttccactctgctgcattctcacttggaaaggttatggggtataacgtataattaaatgtttgtagaaatgaccagttgtcaagtctgcctttaaagctatgatgtagctgatcttcagcaaaaatatggaattgaagaggtttgatgctgaaaatgatagctgacttcaacatggtcatagtttcttccagtctttcaccacaggcaactacagctagatgcattttctcaacaggctgtattttcagactgtacctaaaagccgcttcccaaaagcagttcattccacaaacatcagagggcagcatccaatagggattccagtaacacagagagaaatctttacacctgtccgacacgccgggatgcgctgcggggcccgcgacgccggcgcctctcacggcgccgcgtccgccgcccgcgagccaggaagccaccgcggcctgcggcttcccgccaccgccgcccgttccttcttccagggacacggcgagctggctgaaagcgtaaaggagcgagcagaagccgcaggccacacacagcaccacgacgcgcaggtagcgccgcatcgccccggccgcgctcctccttcgccgccgccgccgcgcccgccccgacgaactggagcggagggaggggcaccgcgcagccgcgggcgcaacaagttcctcacccgcagccgccgccgccgccttgcgcccgctcccttccttccctccccgcccaccacctaggcgagcgcagtcgcggctccggagccgaaggactacccgcccggaagcctggacaccgcctct

SEQ ID NO: 12408 - RNA, 3473 nt, Homo sapiens
  source 1..3473: mol_type = other RNA
ctgggaggtgtgatatcgtggtatctacccaaagtgttcacagcagtgaaataacacaatgtatgggattttaagatacttaagcaaacaaaaaaatgacaaatgaagcaaacatggtaagatagtgataagtgtcagatctggatgttgagtaccaatgcactattctagttttgtgtaatttttaaatttcttcattaaaaattgttttacagactccctcctagacacagcatgccagagtctccaaaggcctagctcaggaatctattcttaagctcccaacaagaatcttacatagtcaggcaggcaatgatcattatttgaggaccattagaaatgatctaatacataccctccaaacttcacatttttagtattctcattttctactcagtaagctcaatttcacagtttcttatattcaccatggcattctgccaaggaactacaactcgtgttctctaaacccatctgttctaagaatgctggactggttatcaacttctaatgcaccctgcttaaactttcctctctcaatttgtccctgactgaactgcagacgacagaacaactgtactaaccatctctttctgcatattccatgtctccacagaggtcactgtgtcttcacaaagctaactgccacaattttcacaggttgtatttttccttcatgattttccattttctacttgagcattaaaatatcagggagaaaaagaagataaccatatagataatcatattgttggtaaaataagatatgtgccccagcatagtatatgctaagtattcagaatctatagttatattagctaacaggtcaagaatgccaaagaagtaatttctcaagatttaaaaaaattaactgtcttaggtgatattcaaaaatgcacatcaacccaattaaaaccacattttctacagctggatgtaacaatcttattccaaatcatccacttaagttgtttaacttacttaaagtaaggctctagacatttgcttcttcaaaagtatcttgcaaggccgttatgaggtagaagacaagtttaaatggaccatatttttctactccattgtaactaaaattactactcacaggaagtatatagcttatgcattttggtccatcacactttccaccatcatgagtatactcttaaggttctcactttaccatcagcataatatattttgcttccagaatgcccagtaaagctgacgtttttcatttaaagtgattaaaaaaaaattccccaaatatctatttaacaatcttagatctgagttttggcaagacagtttaatgcatacaaaatgaaacactacatttctcactctctctcacacacaaacacgcacacacagattaaaatcccaaagttttcactatttttcctctaccttacacagctcaatttttaacatgcagcttacttgtaatctaaaaataattttaaacatgattgtcataaaaatattttaaaacagagatgaaatgtataaaggcacacatagattgtcaatggttacatcagttacatcacatttcttcagaaacaacagacctgtttctgctcctgtaaacaaacttttttctcacacttttaaagtgaggttagtgctgacataaaattattgctctactcacagtcttgagtgttggcactgtttgaggtacattttctccatctacacacccctaccactcttgagagtatgagtcaacagaagtctgcaggttaaacccattcaatagtattttcatcaatactggaatgatagcaagtaacattacaaaacatcagagataaaaaatgttcaatgttgaggcccaagattttaacttattcttcattacctgaaaatactgcttacttaacttctttaggaaaaaaaaaattattctggagatgagtaattccttcctgaatacttcatccaagacgattccttcacacttatcttctgattctttgttttcatccatttgattaagcagtcaccaagaatcacttttcctttggtgatctggcataacgatctcttacactttttgctagttgtttgataaatattttgtaaatttttccacagtatgtatgcactgttttttgtagttccagttctaaaggttttaataaggaacggatgttgtcatcttcaaaagaacaatttctcagtgcttcataaacagctctaaatgctggttgcttatcgtcatggtaaacacctctgttcccatgaagaataaagattcctccttcttctgcttcttggcaattgcttccatatatacaatgatctggtcgataattccattgacacggaaaaacaaaaaggctttctggattatgaaaaaacacgatattcaatagatcttgatcaccccatgtgatgtttagtttgtattttttaagcaatggcataagtatatctccccattgtagtcgtacagttgtcatatcattcttgaaatacttccttctcattcgagtcatgttcatcaacataactccagagtttactccagtttttccataatatggatgcctagcaaagcgattataccatcctattcgaggttcctcatgttctggtgccattgcagcaatttgtgtggaattaaatttctttagtaaagaccaaatatcatcaactggtcgtaaaaaaaggatatcagtgtcgacatacaatagtgagtcaacttctttcaggattaacggcaagaacaatctctgcgaagcacatggtttaaagagttttttccactctgctgcattctcacttggaaaggttatggggtataacgtataattaaatgtttgtagaaatgaccagttgtcaagtctgcctttaaagctatgatgtagctgatcttcagcaaaaatatggaattgaagaggtttgatgctgaaaatgatagctgacttcaacatggtcatagtttcttccagtctttcaccacaggcaactacagctagatgcattttctcaacaggctgtattttcagactgtacctgtccgacacgccgggatgcgctgcggggcccgcgacgccggcgcctctcacggcgccgcgtccgccgcccgcgagccaggaagccaccgcggcctgcggcttcccgccaccgccgcccgttccttcttccagggacacggcgagctggctgaaagcgtaaaggagcgagcagaagccgcaggccacacacagcaccacgacgcgcaggtagcgccgcatcgccccggccgcgctcctccttcgccgccgccgccgcgcccgccccgacgaactggagcggagggaggggcaccgcgcagccgcgggcgcaacaagttcctcacccgcagccgccgccgccgccttgcgcccgctcccttccttccctccccgcccaccacctaggcgagcgcagtcgcggctccggagccgaaggactacccgcccggaagcctggacaccgcctct

SEQ ID NO: 12409 - RNA, 579 nt, Homo sapiens
  source 1..579: mol_type = other RNA
ctgggcccgcggcgggcgtggggaaggactcggccgagaccggcgagcccaggttgaagctgcgttcgaagtacttgtgcttctcgtgctcgcggctcacgggccgcgtgggactgtagagcggcgcggggtgcgcagcctcggggttgccgaagtgcgcggcccgcgggccctgcgggggtggctgcggcccaggcgcgcaggcaagcgcggcggcgagcgctgcatgggcgcgctccgcgggcggcggcggcggcagcggcccggggaccgggctcggcgccgggggctcggcgcgggcgcccccgcagctgggcgagagcagcagtgcgcggtcgccgtcctcgccgccgcggacccggtaggaaacgggcgtggacttcttgctgcgcttcaccaggaagccgcggggcatgttggcgcggcccgagggcacggcactggctcggtcccccctccgcgctcggccccggcggccctcagtgcccccggcccattgcccgggcgcggcggctgcgggactcgcgtggcgccggcgacggctcggcccagctctgcgccctgcacgcgcgtccctgt

SEQ ID NO: 12410 - RNA, 524 nt, Homo sapiens
  source 1..524: mol_type = other RNA
ctgggctcccggacgaggcgggggaccttgggactggtttcctccttgtgggggtggtccttctggctttcccggacgaggcgggggaccttgggactggtttcctccttgtgggggtggtccttctggctttcccggacgaggtgggggaccttgggactggtttcctccttgtgggggttgtccttctggctttcccggacgaggtgggggaccttgggactggtttcctccttgtgggggtggtccttctggctttcctggacgaggtgggggaccttgggactggttgcctccttgtgggggtcgtccttctggctttcctggaggaggtggggtacgttggggctggtttcctccttgtgggcgtcgtccttctggctttcctgatattacggagggagattcttcctggctgacatcttcatttaagctctgagctgagctcagggccagcagggccaccgacagcagaatcagtagcatcttgctggaggctctggagtcactcccaactctgtgct

SEQ ID NO: 12411 - RNA, 461 nt, Homo sapiens
  source 1..461: mol_type = other RNA
ctgggctcccggacgaggcgggggaccttgggactggtttcctccttgtgggggtggtccttctggctttcccggacgaggtgggggaccttgggactggtttcctccttgtgggggttgtccttctggctttcccggacgaggtgggggaccttgggactggtttcctccttgtgggggtggtccttctggctttcctggacgaggtgggggaccttgggactggttgcctccttgtgggggtcgtccttctggctttcctggaggaggtggggtacgttggggctggtttcctccttgtgggcgtcgtccttctggctttcctgatattacggagggagattcttcctggctgacatcttcatttaagctctgagctgagctcagggccagcagggccaccgacagcagaatcagtagcatcttgctggaggctctggagtcactcccaactctgtgct

SEQ ID NO: 12412 - RNA, 35 nt, Homo sapiens
  source 1..35: mol_type = other RNA
ctggggagatcctcgaggttggcctgctttccctc

SEQ ID NO: 12413 - RNA, 221 nt, Homo sapiens
  source 1..221: mol_type = other RNA
ctggggagatcctcgaggttggcctgctttccctccttttcttacaacttctggagaagcgtcagccctctgcagggaggcggccaagctggcaggcgagtcggcgagggtgtcattgcttatatggctgcggggaccgaagctaggaatagacgcgctgagggctaggagggctccgaccggacggaaggatgccgcatcgcgggtcgctgcccggagct

SEQ ID NO: 12414 - RNA, 5718 nt, Homo sapiens
  source 1..5718: mol_type = other RNA
ctggggagtggctggggagacccgcctgtctccacgcggtgccatgtgctgtgcccaccgctggagctccagctcccattcctttcttacggtgccactaacacattgcattctctcgcatctccaggccttttcatgcgctgctccctccctcccttctctatcaggctaagtcctactcgcccttcaagactactccactaaaaggagcggctccagaaaatggtgcctgaccccacccacacaccccaagttgggttttcccctcctctgtgttcccacatacccagggcttccttctgggcctgcacttattttatcatcttcacattatccccaccaggctctgtccactcctgaaactcttatcctacactgtctgacgtggcagctacttacccacatgtgcttatttatttacatttacattgaataaaatgaaaagtgcagttccttagttgcactagccatgtttcgagtgctcagtagccacatgtggctagtggttaccgtactgaacagcacaggtatgggacattttgcttatcacagacagacctattggacagcactagagaacaaacataagaactctgagatgctaggacctttgtcctttgtttttgtttgtttgtttgtttttgagacagagtcttgctctgtcacccaggctggagtgcagtggcgcgagctcgctcagctcactgcaacctccgcctctcgggttcaagcagttctgttctttgttatgtgttgtctgtccccatctgcatccccagagggattggcagcagcacctttgatgtaagaatagtcagtgggcttgctgtctttgggtcctcagagaaatggggaggtgaggagatgaactaccccctccacagtctggacagtgcatttctggaggggtggagggagtgaggagcatggacagcccagcgctgggactgcaatgaggactggaggagaagaacgtaggaaacagttgaaggaagcatgaggagctcccagaggggcccggaaacttggtacacaggttgcatcaatcaataaatcaaccaatgcaaagatatctaactctgagacttagaaccattcattcattcattcatttgatcaacaaaattttagtgccatctgtgctgtgccaggcactatatggggcaatgttctggatggagatgattcagaccagtgtcactcccaagccacttaaggcctggtggggaaggatctcagagtatgtgatgaagggcacattttgtgaaggatgggttcttcaagcccatcttgcaagggttgggaaaaccttcatcagggatgttggggggagtattgtggcaggggggaaagccacaagtaaaatgctgagtttggaaagtacacagaggcatttttggggaatagtaagtggatggccaatgtgtgggtgaggaatgagagttaggaccacagagattggctgggccaccttgtggaacacctcccatgtcaagataaggggtttctgtaggtggcttactgtgtgtctggcatgaggtaggcacttcacatgcatctgttaactgtcctgcaaggttgttatccccatcttacaggtggaaggccaggctctgaagggctaggtgacttgccaaatgcagcacaggcaagtcaccgagccaggatttgagcgctaaaagctgagctttggaaaaatgcaaccagaatcaagttgaaggtggggaaatgatcgtgcagcttggtccagcagggaagaaaactaaaaaatgttgattggacttgattcaggaccctgtgggtctaagctcttcaaaccctcaagtctggtccatgaggcggcatcaaatgcgtaggtggccccagctgctgcttttgctagttgtcttccctgggacacttcgatggtgctgtccagcgatcccacgctgttacgccgcccccgcttccctgcatcagagaggtctcgcagggaactgctgagtgcgccccgtttgagcccatcgcctgccccgtaagtgtcctccaggctactgcgggccatcgtcccattcactgagtccttggcccctccaggctgtgaggcgttaggccgcatcatacctttctgcttctccagctccgactccacacggtatttctccatctcctgcacctccgcaatggactcgcgcaggtcggatgtaaagcgcagccggtcctggaggctgggggcattgaagatgatgaggacttttcgctccccaccaggtactgcagacagcaacttgatcccaaactggtaatatgaattctggaagagctgcatgtgcatttccacgagggggaaagactgacggaaactgtacgtcaccaagatcttcttcttctggaaaattttggtgaccacaaggagatcattgaagaggaagacctcccgctgatgcaaccctagcctctgggggcggtttggatctggcacctcgtagagctggcagcagcaaaccagtcgacggtgagggagagacaggactggtttctttccaacaatcatgcgctccacagcctgcacctgggacacatggtcatcgttggtccgcagttcacgcccctggatgcgctggtagatgcccaccaggaggtctcgggggatgtcttcaccattgtcaacccctctcaggttcttgatgaagtcatctagtttcatctttcgttcagctttgacgctgggactgtacatgtcggtattgaggaggatgatggcaaaagcaaggatgaagatggtgtctgggttccggaactggcgcacgagggctgggttacagacacagtaccgctggctgaaggcttcgatgagtcgctccactttctgggcctcaccctgaacccggatatgggactggaacttccggagcgcatcatccagatccatggaggagaagtccatctcatccaccacacagtccaacacgtctctgttgaactgcttctgccggttccctaggaattcccctatcatctgccggctgaggcctttccgctccaggatgaagtgagccactcccaccggtgtgtctgacaggaagccccgctcgatcagatactggatacccttctctggcttcttgttgaagaggttgaggccgattcggtagtgccgcctctggaccacatcattgttgaaagctggcgagtcccagctatgccttgtctcccgctggtaagtctgcttgcacaggccggtagccggaggctcccttagactgtcccgagaagaggagccggagctgcagttgatggtctcattggaattgctggagctctcaaggctctcgttatctccaccatcagagttctcgcctgctgcctcgcacttccccaacctccgacccccagccacaccactgggcccagtgccactgttgggggctggtggcaggggccctggtggggctggggctgggccttcaggggctgggtagtggcggtgtgggatcggggccctgcctggtggccccttgtgcttcagggtcccatgggggctgcagccatcagcctcatacaccagctggcggtggacagagccgcgatctgagcggtcactcaggtccacggagctgtcactaggaggctcaatggtaagcaggggaaggtgggcagcccgcagccggaaatcccggcactccaagcacccgggacccctgcgagtgccttcctcacggctaccgtcttcccgggttcctgatggcactggtggaggaactggcgggagaggggctggcgcccagaactcgggccggccctggggtgggggttctgtgctgggcagtcgctcaggggattgttggggaactgtgtcatccaggtagaggggaagatcactgaaggatgtggctgagctgtcctcttgctgttcctttgactcccgcttctccagctgggctgaccctggctcctcagacatgggccctgacgggtggcagttcagggcttcgtcgatggattcagccagagactttacctgtttggagaaggagtcctcaagttctgtgatgtcattagaaaactctccagatgtggtgacggagcttccaccaccatcgatgcccccaccacaggagcctccatatgggagcccccgttcaagccggtggctccgggcaccagccatggcaccctcgtccagcgaggcaggcttgccctcgaagtacgcggggttctgtgccttctcatactcctcaaaggagaactgcatccgcatgttggaaaggatgatgcggcgggacatgcggctctctgaggctgagctgcgtagccgctcaaagttcttgttcatgcggtactggcggaaggctgtctggatggtcctggcagccctgcggctcaggaaggagcccccatacttcctctccagcatttccaccttcttgtcctgcaggtctgtggagagttcatagctgtccgatagggccttggagcgctttatctcctcctcctcctgcttcctcagggcgacactggctggctggaggcgtgcccgctgagcccagggaaggcccactccagcaggggggccccccatgtggctgctggaggggggcagctggctcagccggtaggggggttggctcccaggactatcaaccgctgtgctcaggtcactgcctggggcatcaccctccacactgctctctgccagcctgcctgagggggtaagcttcatggagtcaaggacctgagtaggacagcaatactggtgtagagtatgagacgctgtggacctgactgttctggaattctcaccatcagattttctctggagggtcgtggccgggctggtgctggtactggtgctgtggcctccgccggcgccgggactggagctcctggatgcgccacggctcagctggccccgctcccgcggtggccgcggccccacgcccaccgccgccgaatagcccgcttccttctcgcggcccgggtgcgccggcccggcctcccgcccgccacgctcgcgacccagggctgggttctcgtggtgcaggtggcactgggccacgtcacgctcgcgggctgtgtaaccggtagtgtcctggagcgggtaggaggcgtcccgctccttgtcccgatacacagcctcccgattctggtaggcgccttcccggttcgggtagcccacgtcccgggccgcctggtggaactggctctcccgcagctcgcggtggtggaactgggtctcgcgcaggttctggtactggctctcgcggcccgggctatcccgcgcgccgtgggggtcccggtgcagctccccgcggtgcagctggctctcctctcgcaggtcgcggttctcctgggtgagctggtccagctggccctccagctcctcgatgcgccgccgctgggtttccagcagctgctgctggctctcgatgatgttgttcagctccagcaggtactccacggcccgatttgggctctcggatcccgggccgcccgggggccccgaccccgcctccatcctggcggcccaggggcaggggaacgggcaggagagccctgtccccgctctctcacggcgccaccctcccccgggcccagccgggggagggggccggcgggacgcgagggcgcgcaccgggcttgagggcccgggggccctagggggcccgggagacagcgctggggccggcggcacggggagcaggagctgaggctgccgccgccaccaccaccaccaca

SEQ ID NO: 12415 - RNA, 2342 nt, Homo sapiens
  source 1..2342: mol_type = other RNA
ctggggagtggctggggaggaactgggctatgtggaaagactgggctgcgcccgtctacggatgccttctctcttgatttcaatgattgatagcatgtggctttcagacctaaggaagagttagagctttggagaatcacaatgcctgtgattgaaatcaggatttaaaaaagggttagaggcataggggaaggctaccattacaggaagtagttggatcttaattttcacatgtatagggctagacagcttcatctgtaaagttctgtatttccataattgttttatctttaggaagtccagtgtaaagatcttacagtttcactcataaaaatatcctgggctcagacagtgagcctgtggacaaacggaggctactgcagcattctggcattagcactctgattttatctggagagccctttcatatggttctcagggcctggcttacccgctggagccaggctagaaacatgacttagggctggatgagaatcatcctgagaattccgtgggggccagactggaaagtcctggaaaatcatggagctgctggaggccctaaaagtcaacacaaaaagagctaaactcactcaagaagctaagaaaatggcccaggaacactggtagaactgctagatgacagggtttcaggcatgggaaccagatcaatctgtacttcttgctgtgaactactctgtattgggtttcaggtactggctgatcttgctggttctgttcatggtttaacatcaagatattactgccccaaacatgtcagtcttacagatttgttttcagaaacttcaagtactctttgaggtaagaataggaaaagagatcctcaagcacgtgcagatgcttgcgggatggacctgaattttcattagtctcctagccttggtgtagtgaatggagtcaaccgttttccttacttaaaagctggttcagcctcagtaaatagatgaactgaaaactagtagaggattctatcgaaccctaccctagttggattcaactaccctagataaattttgcatagtaaaaattcaattagaagaggccaaaaagccttttttttctttttaacgctgttttaaacactaacggagtacatggttatttgcatacccagcttagaattttatattgggggttgagagtggaaatgacctaattgagaactcaggtctatttctctatacaaatacccctgtctaccagactggactagaaaagtaactgagctgtagttaactgctgttgagctttaaaaaaattggagtaaacatacttgcatttatattctttgttaattttagctggagttataacaaatttaaaggaaggtcacaacctacctgtaattacaattccataccaccaccacatctgttctgtgcttttattttacgaaaaagctaatggcaaatctacattaaactaagttgaatacaaagtcttagtgaagaaggcctggtggtctcgtttacaaaaatggccagtgtcatatttgggcttaaaatttcaagaagggcacttcaaatggctttgcatttgcatgtttcagtgctagagcgtaggaatagaccctggcgtccactgtgagatgttcttcagctaccagagcatcaagtctctgcagcaggtcattcttgggtaaagaaatgacttccacaaactctccatcccctggctttggcttcggccttgcgttttcggcatcatctccgttaatggtgactgtcacgatgtgtatagtacagtttgacaagcctgggtccatacagaccgctggagaacattcggcaatgtcccctttgtagccagtttcttcttcaagctcccggagagcagctgcttctggggtttcaccatcatctatgagacctgcagggaactctatgcagtagccccccattggtggtcggaactgtttcaccagaacgatacactcatagtgaagtgttctctgcagcacggggatgaccgcgacaccatccgcagtctgctctttcctggttgtacgtttcactgattcccaagttctagttttaccagtaggatccatgtacgttgttttttcaagcttgacccattttccttctgaaattaactcctctgaaatgatatactgtttgccattctgagaagattccgttggttcttggctctccattttcaaacgagtctttacagccctcaggtgagaagttcacctccaaggtgtaggggtgaagaacggaagaggacgaaataactagctggaggcagcagtgtcagccgatgccggtgccacggctcgaaacaccggcgcctctcgcggtgctaaaaggatgggc

SEQ ID NO: 12416 - RNA, 2437 nt, Homo sapiens
  source 1..2437: mol_type = other RNA
ctggggagtggctggggaggaactgggctatgtggaaagactgggctgcgcccgtctacggatgccttctctcttgatttcaatgattgatagcatgtggctttcagacctaaggaagagttagagctttggagaatcacaatgcctgtgattgaaatcaggatttaaaaaagggttagaggcataggggaaggctaccattacaggaagtagttggatcttaattttcacatgtatagggctagacagcttcatctgtaaagttctgtatttccataattgttttatctttaggaagtccagtgtaaagatcttacagtttcactcataaaaatatcctgggctcagacagtgagcctgtggacaaacggaggctactgcagcattctggcattagcactctgattttatctggagagccctttcatatggttctcagggcctggcttacccgctggagccaggctagaaacatgacttagggctggatgagaatcatcctgagaattccgtgggggccagactggaaagtcctggaaaatcatggagctgctggaggccctaaaagtcaacacaaaaagagctaaactcactcaagaagctaagaaaatggcccaggaacactggtagaactgctagatgacagggtttcaggcatgggaaccagatcaatctgtacttcttgctgtgaactactctgtattgggtttcaggtactggctgatcttgctggttctgttcatggtttaacatcaagatattactgccccaaacatgtcagtcttacagatttgttttcagaaacttcaagtactctttgaggtaagaataggaaaagagatcctcaagcacgtgcagatgcttgcgggatggacctgaattttcattagtctcctagccttggtgtagtgaatggagtcaaccgttttccttacttaaaagctggttcagcctcagtaaatagatgaactgaaaactagtagaggattctatcgaaccctaccctagttggattcaactaccctagataaattttgcatagtaaaaattcaattagaagaggccaaaaagccttttttttctttttaacgctgttttaaacactaacggagtacatggttatttgcatacccagcttagaattttatattgggggttgagagtggaaatgacctaattgagaactcaggtctatttctctatacaaatacccctgtctaccagactggactagaaaagtaactgagctgtagttaactgctgttgagctttaaaaaaattggagtaaacatacttgcatttatattctttgttaattttagctggagttataacaaatttaaaggaaggtcacaacctacctgtaattacaattccataccaccaccacatctgttctgtgcttttattttacgaaaaagctaatggcaaatctacattaaactaagttgaatacaaagtcttagtgaagaaggcctggtggtctcgtttacaaaaatggccagtgtcatatttgggcttaaaatttcaagaagggcacttcaaatggctttgcatttgcatgtttcagtgctagagcgtaggaatagaccctggcgtccactgtgagatgttcttcagctaccagagcatcaagtctctgcagcaggtcattcttgggtaaagaaatgacttccacaaactctccatcccctggctttggcttcggccttgcgttttcggcatcatctccgttaatggtgactgtcacgatgtgtatagtacagtttgacaagcctgggtccatacagaccgctggagaacattcggcaatgtcccctttgtagccagtttcttcttcaagctcccggagagcagctgcttctggggtttcaccatcatctatgagacctgcagggaactctatgcagtagccccccattggtggtcggaactgtttcaccagaacgatacactcatagtgaagtgttctctgcagcacggggatgaccgcgacaccatccgcagtctgctctttcctggttgtacgtttcactgattcccaagttcttttggcatagctctctctgctgcctcctaaggttagtcctaaagactgaagaagacagtgctgggaaaagcactgaaggtcccatcccaaacactagttttaccagtaggatccatgtacgttgttttttcaagcttgacccattttccttctgaaattaactcctctgaaatgatatactgtttgccattctgagaagattccgttggttcttggctctccattttcaaacgagtctttacagccctcaggtgagaagttcacctccaaggtgtaggggtgaagaacggaagaggacgaaataactagctggaggcagcagtgtcagccgatgccggtgccacggctcgaaacaccggcgcctctcgcggtgctaaaaggatgggc

SEQ ID NO: 12417 - RNA, 2333 nt, Homo sapiens
  source 1..2333: mol_type = other RNA
ctggggagtggctggggaggaactgggctatgtggaaagactgggctgcgcccgtctacggatgccttctctcttgatttcaatgattgatagcatgtggctttcagacctaaggaagagttagagctttggagaatcacaatgcctgtgattgaaatcaggatttaaaaaagggttagaggcataggggaaggctaccattacaggaagtagttggatcttaattttcacatgtatagggctagacagcttcatctgtaaagttctgtatttccataattgttttatctttaggaagtccagtgtaaagatcttacagtttcactcataaaaatatcctgggctcagacagtgagcctgtggacaaacggaggctactgcagcattctggcattagcactctgattttatctggagagccctttcatatggttctcagggcctggcttacccgctggagccaggctagaaacatgacttagggctggatgagaatcatcctgagaattccgtgggggccagactggaaagtcctggaaaatcatggagctgctggaggccctaaaagtcaacacaaaaagagctaaactcactcaagaagctaagaaaatggcccaggaacactggtagaactgctagatgacagggtttcaggcatgggaaccagatcaatctgtacttcttgctgtgaactactctgtattgggtttcaggtactggctgatcttgctggttctgttcatggtttaacatcaagatattactgccccaaacatgtcagtcttacagatttgttttcagaaacttcaagtactctttgaggtaagaataggaaaagagatcctcaagcacgtgcagatgcttgcgggatggacctgaattttcattagtctcctagccttggtgtagtgaatggagtcaaccgttttccttacttaaaagctggttcagcctcagtaaatagatgaactgaaaactagtagaggattctatcgaaccctaccctagttggattcaactaccctagataaattttgcatagtaaaaattcaattagaagaggccaaaaagccttttttttctttttaacgctgttttaaacactaacggagtacatggttatttgcatacccagcttagaattttatattgggggttgagagtggaaatgacctaattgagaactcaggtctatttctctatacaaatacccctgtctaccagactggactagaaaagtaactgagctgtagttaactgctgttgagctttaaaaaaattggagtaaacatacttgcatttatattctttgttaattttagctggagttataacaaatttaaaggaaggtcacaacctacctgtaattacaattccataccaccaccacatctgttctgtgcttttattttacgaaaaagctaatggcaaatctacattaaactaagttgaatacaaagtcttagtgaagaaggcctggtggtctcgtttacaaaaatggccagtgtcatatttgggcttaaaatttcaagaagggcacttcaaatggctttgcatttgcatgtttcagtgctagagcgtaggaatagaccctggcgtccactgtgagatgttcttcagctaccagagcatcaagtctctgcagcaggtcattcttgggtaaagaaatgacttccacaaactctggctttggcttcggccttgcgttttcggcatcatctccgttaatggtgactgtcacgatgtgtatagtacagtttgacaagcctgggtccatacagaccgctggagaacattcggcaatgtcccctttgtagccagtttcttcttcaagctcccggagagcagctgcttctggggtttcaccatcatctatgagacctgcagggaactctatgcagtagccccccattggtggtcggaactgtttcaccagaacgatacactcatagtgaagtgttctctgcagcacggggatgaccgcgacaccatccgcagtctgctctttcctggttgtacgtttcactgattcccaagttctagttttaccagtaggatccatgtacgttgttttttcaagcttgacccattttccttctgaaattaactcctctgaaatgatatactgtttgccattctgagaagattccgttggttcttggctctccattttcaaacgagtctttacagccctcaggtgagaagttcacctccaaggtgtaggggtgaagaacggaagaggacgaaataactagctggaggcagcagtgtcagccgatgccggtgccacggctcgaaacaccggcgcctctcgcggtgctaaaaggatgggc

SEQ ID NO: 12418 - RNA, 1365 nt, Homo sapiens
  source 1..1365: mol_type = other RNA
ctggggagtggctggggaggcaaagcccattaaagttggcagttgtgctttgtcaaccatttagtgtggttgaagcaaaggtaaagtagcaaggattgttcctgcaggaaaacatatttaagcttataggccaggttttacaagtaagagtgcaaggacaagaaaagtagaggttttatttcagggcaaaataagaaatgcgcaggatatggtccttctggttcaacaaagtctccaagatgctttcaagttgaacatgtttctgagcattgcaaggatagctcataaatggttattcttaagctgttgcttattaaatcaaatctgaatctggcaaagtaacagcagaagccaggggaaagccagtagatgatgcattaatgcggccttgaaaattattttcaagtcttactcagcaacacaatttggttacatcctgcttcatgtggaatgatttcattcctttgttggtttttttttaacagtcggccttctacaatagctatttaaattaagcattaaatttatcaaaagtgtattctttactgtaattaattctaaaagatagaagaataccatcttcttctgcaaatacagagtgagcacctatggaattcaacaatatttatgaagaaagaaattgtatttatacaggaggggaaaaaaaagcagtagactgaggcagatctatgtttaaaacacagctcatttactagctgtgtggctttggatggatccattaacctctccgaatttctttccttaattataacaggcactaataatgcctgcatacatgagagttatgaattaaaaataatatgtgtaaagtgtttcacacacaataatagcgacaatctaatgaggcctattaagatatcctgaggctcataaaggagaattgctgagacctcttgaataacatttctgaaaatgtgttgggaaaacattagtccctactgatgggtctgctattatcaaatctgggaaatgtgttttataggcttctattagaaattagtaaagactctgagaagctctgcaactaagaaatctgcttcagttcaacactgagttttccaggcctaagaattctgcaaccttttattaggcatcaacaggaattccagtcttgggtgaactttgcccctgacatcaaaaaagaaagccgattcgttacagtttgttcagctgaggatgtgtttcttactatgttattttgacattgttacctttctttttcactgattttttaacctccagttttaactcatgaaaagaaatttggaggaaatgtcatttattaaaagtataccctttgtcagatagatagattgcaaaaattttctcccattctgtaggttg

SEQ ID NO: 12419 - RNA, 648 nt, Homo sapiens
  source 1..648: mol_type = other RNA
ctgggggacgcgtgagcgcgagccgcttcctcacggctcggccgcggcgcgtagcccccgccacatcgggcctggctctcctcagccgccggctcggctcggtgcgcgcgggggtcttgagctcaccgccggcggggcggggttacatggcgcgcgaggaggggggagagaagaggagagcctaggtgccctcctctcccctcccccccggcggcggcgcgcgcacggccctcgccggcctcacccctccgcaccccgcccgcctgctcttcaccggccaggccctgccgggtcgccgcggcctcggcgccccaccccctcccgggccagcggggggctgggagggggcgaggaggaagggggttctcctctcccctccccggagggggccgcagcggcggctccggctcctcctctccctcacaccccctcccgcccccctctacctgcgggggacacgggcagaaggaggcggtgcacggacggggcccggcgacaactgtcagttagaagccccgctgggcggtgaggggggagaaaggggaggggcagggagagaagggggagggcactcagccccccggctgggaagagctgtggagagaagcaaagaaagaggccctgtcgccatccccggtgcgcatgcgt

SEQ ID NO: 12420 - RNA, 654 nt, Homo sapiens
  source 1..654: mol_type = other RNA
ctgggggacgcgtgagcgcgagccgcttcctcacggctcggccgcggcgcgtagcccccgccacatcgggcctggctctcctcagccgccggctcggctcggtgcgcgcgggggtcttgagctcaccgccggcggggcggggttacatggcgcgcgaggaggggggagagaagaggagagcctaggtgccctcctctcccctcccccccggcggcggcgcgcgcacggccctcgccggcctcacccctccgcaccccgcccgcctgctcttcaccggccaggccctgccgggtcgccgcggcctcggcgccccaccccctcccgggccagcggggggctgggagggggcgaggaggaagggggttctcctctcccctccccggagggggccgcagcggcggctccggctcctcctctccctcacaccccctcccgcccccctctacctgcgggggacacgggcagaaggaggcggtgcacggacggggcccggcgacaactgtcagttagaagccccgctgggcggtgaggggggagaaaggggaggggcagggagagaagggggagggcactcagccccccggctgggaagagctgtggagagaagcaaagaaagaggccctgtcgccatccccggtgcgcatgcgtagtaga

SEQ ID NO: 12421 - RNA, 655 nt, Homo sapiens
  source 1..655: mol_type = other RNA
ctgggggacgcgtgagcgcgagccgcttcctcacggctcggccgcggcgcgtagcccccgccacatcgggcctggctctcctcagccgccggctcggctcggtgcgcgcgggggtcttgagctcaccgccggcggggcggggttacatggcgcgcgaggaggggggagagaagaggagagcctaggtgccctcctctcccctcccccccggcggcggcgcgcgcacggccctcgccggcctcacccctccgcaccccgcccgcctgctcttcaccggccaggccctgccgggtcgccgcggcctcggcgccccaccccctcccgggccagcggggggctgggagggggcgaggaggaagggggttctcctctcccctccccggagggggccgcagcggcggctccggctcctcctctccctcacaccccctcccgcccccctctacctgcgggggacacgggcagaaggaggcggtgcacggacggggcccggcgacaactgtcagttagaagccccgctgggcggtgaggggggagaaaggggaggggcagggagagaagggggagggcactcagccccccggctgggaagagctgtggagagaagcaaagaaagaggccctgtcgccatccccggtgcgcatgcgtagtagaa

SEQ ID NO: 12422 - RNA, 739 nt, Homo sapiens
  source 1..739: mol_type = other RNA
ctggggttctgagacagacagtcggtagactccaagcagaaactgtgcaaaagtctcttgccggtgctccggaaattgccaggggttccaggccgcaaggcgagacggctaagttgcttatgagtgcccttctgctcaggagacgatgcgctttccggatctgtctacgtcatcgcgtatctcattgctccaacagccatggatccctctttgcagtcttcacagttgatagacacttagaggccaccacttcccaccccatgaagcgcactatggtgacccatgtggtttcagggcctcagaagactggatcctgcacccagtgctcaattcctggacatggtcttctaattcctacagggtggcacagcttcatcccggtgatccatgcaggtgggaacaatccagttaacttttcccatccgagtgattctctttctcttcttcattcataaatgccataactctcccggtcctcctttccaaggctcgtgcacttgatttcaaggcttgcctgccacccagggtgccaccagagtcccagtgcctgggttgggggctggagcgcaccctttgggatcccccagcctgtcctccgcctcacggctgcctcgcttctgagctgccaccctcagctgactcactcagatgagatttgggagggaggggggcaggaggaggagttgcgagaaggaggaaaacccgcctggtcgggtccacactttgcctagatgcgttt

SEQ ID NO: 12423 - RNA, 1854 nt, Homo sapiens
  source 1..1854: mol_type = other RNA
ctgggttgggctgggctgggagtccctccctcccctccccccgccccgccccccatgcacacagcaaaacatgaaaaagaaaacatctcgaaactgcaaaaaacaccatggccctcccccctccccatagatcccccaaaaaaataaaacacgacgctccctcacagcggccccctccctcccctgccccctccctcggggtccctgcttcggagggggaggggggcggggagggtgggcgtggggcgggcccagcagtctccagcgcgctcacgggggaaagcgggggcgcccccgaccccggcagcctcgatgcacgcgcgcccgcgcacgcgccccggacacgcccctcggctcccccgccgcgcccctacacaggcgtggttttcctgttgagcgtgttggtgttggaggcggcggcctccttggccagggtcccgggggcgggcgcagagggcgcgggtggcgcgggcgcgggcggggcgggcggcccggtgaccgtgaccgtgacgccgccgcccgcctccttggggaaggcgttgtgcagcgtgaggaagccggacgcccccccgcggtcccgctcggcacccgccccgccgccgcctccgccgccgcccccggcgcccccggccgcgccgccgaacgcccccacggcgccgccgccgccgccgccggcccccgccagccccgcggccacgctgcccttggaggggtcgcggctgagcgtgtacatggagatgtccgtggaggcaaagcccgggcccccggggccgccgggagacgcgtcccgcgacggcgacggctcgctggagcgggagctagagcgggagcggcggcggtagcggaagcggtaactgggcagacggaggatggccgaggggccgctcccgccactgccgcccgcgcccccgccggccttgagcaggtccgagcgagactggcagtgcgcctcgcggctgcgctcgatgtagatgttgacggccagcacgcctatcacctcggccaggatgaacgacagcccgccgaagtagaaggaccagccgtacgagtagtggtttttcttctcctcgtcccgcttcgggcccggctcgcccgcgttggcggagatgtacacgatcacgccgatgatgttgctcaggcctgctgccacgaacaggatccctgcgcccagaatgatgttcctcttggacttgtagacgcgggaggccgccacgcacacacccccgagcagcagcaggatggcgctaaggatggggaagatgctggaggcccggacaactcggagtagatactccgcgctgtcgtggtcgtagtccgtgtcctccgggaaatgattgatcttcacgcagacgcctcttttcaacccttccaggcagcagatcctccagaggcccgagtgcgtgaggccgccggggtccttcttctccgaggcgccgccgcccccgcggtggggggtcccgtcgtcgccgccggccgtgaggttggtggtgttgcagatgagggcgcgcgtgtagagccagtagtcagtgctgatggcgatggtcatgaggccgaaggcggcgaaggcgcccaccgtcgtcagcagcacctgcacccccttctcgcaccagaggccccgctcttcgttccagcgcttcagcgactccagtttgaccacgggcagccggggggccgtgggccaccaccggggcagcgggggcggggccgtgccggcggctgggggggggttcacagcgcaggcagaagcggggggcccggggccggcggggctggggaggggggcggcgaggaggaggctgcggccggggagggggtcagagcgcggccatggtcggcggctggtggagggcaagg

SEQ ID NO: 12424 - RNA, 759 nt, Homo sapiens
  source 1..759: mol_type = other RNA
ctgggttgggctgggctgggcagccagcaggtcaatggcaatgacaagagtgggatggaggaggaagccagacggggtaggtggccttggggtgtgtgggtgagtcagccccatgccagccactggtggtgtcaggtggcagccgcactcttgttgccatgacaactcctcccccggaagacagggaggccgttggacgagtttccgctcagagcggagagcccaggccctgggctgcagggaagagtaggagccaaggcaggcagagagcacaccagggagaatgggcggctgcagaaaccagcagcagcgggtggagggaacctgcttcagggaacaggcagatgagataatgggagtaacaggtggcaggtggaaggaacaggtggagagggagcagaggggaataatagactgggaacaggtgtgggaaatgacagtggaaatcaaagaagacacaacaagggcatgacaggtaagggagaggtaggcggagaaaggagtggcaagagcgagagtgccgaaggatgaagggacatgacccgggggctgaggccagagagggaagctgttttagtcagctcagccagtccaggggccagtgaagcgtctctatgcttggggggaagagctggggaaagttctgaatggcctggagcctattcttgaggctggatgtggggaccagggaattgatagagtgctctgggtctcccacttagaaagaaaagtcagtcttcccataaagttaaagggctc

SEQ ID NO: 12425 - RNA, 769 nt, Homo sapiens
  source 1..769: mol_type = other RNA
ctgggttgggctgggctgggcagccagcaggtcaatggcaatgacaagagtgggatggaggaggaagccagacggggtaggtggccttggggtgtgtgggtgagtcagccccatgccagccactggtggtgtcaggtggcagccgcactcttgttgccatgacaactcctcccccggaagacagggaggccgttggacgagtttccgctcagagcggagagcccaggccctgggctgcagggaagagtaggagccaaggcaggcagagagcacaccagggagaatgggcggctgcagaaaccagcagcagcgggtggagggaacctgcttcagggaacaggcagatgagataatgggagtaacaggtggcaggtggaaggaacaggtggagagggagcagaggggaataatagactgggaacaggtgtgggaaatgacagtggaaatcaaagaagacacaacaagggcatgacaggtaagggagaggtaggcggagaaaggagtggcaagagcgagagtgccgaaggatgaagggacatgacccgggggctgaggccagagagggaagctgttttagtcagctcagccagtccaggggccagtgaagcgtctctatgcttggggggaagagctggggaaagttctgaatggcctggagcctattcttgaggctggatgtggggaccagggaattgatagagtgctctgggtctcccacttagaaagaaaagtcagtcttcccataaagttaaagggctcttcatgacga

SEQ ID NO: 12426 - RNA, 2303 nt, Homo sapiens
  source 1..2303: mol_type = other RNA
ctgggttgggctgggctgggctgtgcagacccacggccgctgcgggaggcggcctgctgcgtccctcggggaactggtgccgtgcaggggctacggaggaggctgtcccaagggcggggacttcctgggcccttctgtgaggagccttggtctcagcttccggctgtcctgcccccagtctgcctggcacgctgaggggcaaacaaggcaggagaggcggggagagccccacagtgcccagactgctgttgagggtttctgccagccagggcatggagggcactgagtcccctgggctcaaggctgcccacctgggcagacacggggtcccaggcacgggcctgagatgaggacacatcggctggcagaaaggagaaaggatggagcctccacaccccgggacctgtgacttcaccctggttcgcagatgcaccccacaggctagggggtggcgacctttcgggctcttgcaggcccggcccccacccctgcctgctctgctctgcaccgcaccctggcgaggcctggctgcgcacgcgtgtaataggccgagggggagccgtggccgaggcgtcttgttccggaccgagagggtgggcctcttctgggctggtcgccaccttctctgtcacagtctgtggttcctaaccagctcagctcacaggggcgacagaggatctcctgttcccgcagcgcccagaaggctctgccacgggactcacggccctggccaccgcagcccagatctgcagcaggaaagccggtgcggccctggcttcccgcccctagggcaggtccagcagggagtgctcggcgtagagcttctgggagacgttgtagacacgctggatgaaggggagggcctcgcctagcatctgcacggcctgctccgggggccccacgttcatggcctccaggaagacctcgcgtgtgggcagcgtgcagaaggccacggtgacggcgcggcgcacgacccaggggtggtaggcggccagcgaggcgttgtaggagtcggcgcagagcgcggaggtgcgtgcgtcctcggggctggtacgcaggccctccaggaacagctgcagccagtgcagggcgcggtgcaggcgcagcaccgtccggcagccagactccgggtggtgggagcggcgctccaggtccaccagccggttgctcagctcgtgggccaccatggcctgcaggctgcggtagtgctcgctctgcgggccgcccctgaggcgctccatgatccgcagcttggagaccacgtccttggagatgaatgagaagatggtgcccaggctgttcagaaacctgaccaggcccttccagctggcaatgtaggggtccagcaagacctcttccttctcatcgagacactgcttgaaactgaccaggacgactttcagattgaaacctgtctccgagtcatccattttttgataggaacggaaatacagtagggctggggggctgtgtcgctggggtcagcttgctctgtggctcattttcgggcttcaggtgtgggggatggctgctcctgggcctcagaaagatgcagtcccatagacttccagcacgcccctcccctcctcgggccttaattttgtccactgagaagatggtctctgaggctctggggtttccttcttggtcaccagatattctgcgggccttgccttcctgcccagattcgagccagtggcaaacagaagctgccaggagcttctcagagctgtggctggtggctcggtaacaacaggaagggcagtggctgtgcaggaggcaggcagcttgccagcccaggaaggtgacccaggacacctccaggcctttcccagggcagcccaacggcccaaggtcagggccgggcgcgagggcggcctgagcacagagcacgggggctgacagcaggctggggggccagcaggagacggggccccacggcgccccaggccttgtgggtgggaccagaccctgtcgagcgagcgctacgagtctcacctgggaagggggcttcagatggcaccggactggatgggcaccggttcgggtccctgctccaccgagaggcccaggaaggggcggaggcccggggtggtgttggggaggggccgacctgagccacggctccgtcctgcgcgggagccgggtcctcggccgcccgcccgctccggccctctaggacgacgtcccctcccgctcccggcccctcggcgacttccggaccgtgcgggttgggttgggcaggtgcggccgccgagtccgagccgctcacctaggccgtagccgccgtgcgggccccgtcc

SEQ ID NO: 12427 - RNA, 1854 nt, Homo sapiens
  source 1..1854: mol_type = other RNA
ctgggttgggctgggctgggctgtgcagacccacggccgctgcgggaggcggcctgctgcgtccctcggggaactggtgccgtgcaggggctacggaggaggctgtcccaagggcggggacttcctgggcccttctgtgaggagccttggtctcagcttccggctgtcctgcccccagtctgcctggcacgctgaggggcaaacaaggcaggagaggcggggagagccccacagtgcccagactgctgttgagggtttctgccagccagggcatggagggcactgagtcccctgggctcaaggctgcccacctgggcagacacggggtcccaggcacgggcctgagatgaggacacatcggctggcagaaaggagaaaggatggagcctccacaccccgggacctgtgacttcaccctggttcgcagatgcaccccacaggctagggggtggcgacctttcgggctcttgcaggcccggcccccacccctgcctgctctgctctgcaccgcaccctggcgaggcctggctgcgcacgcgtgtaataggccgagggggagccgtggccgaggcgtcttgttccggaccgagagggtgggcctcttctgggctggtcgccaccttctctgtcacagtctgtggttcctaaccagctcagctcacaggggcgacagaggatctcctgttcccgcagcgcccagaaggctctgccacgggactcacggccctggccaccgcagcccagatctgcagcaggaaagccggtgcggccctggcttcccgcccctagggcaggtccagcagggagtgctcggcgtagagcttctgggagacgttgtagacacgctggatgaaggggagggcctcgcctagcatctgcacggcctgctccgggggccccacgttcatggcctccaggaagacctcgcgtgtgggcagcgtgcagaaggccacggtgacggcgcggcgcacgacccaggggtggtaggcggccagcgaggcgttgtaggagtcggcgcagagcgcggaggtgcgtgcgtcctcggggctggtacgcaggccctccaggaacagctgcagccagtgcagggcgcggtgcaggcgcagcaccgtccggcagccagactccgggtggtgggagcggcgctccaggtccaccagccggttgctcagctcgtgggccaccatggcctgcaggctgcggtagtgctcgctctgcgggccgcccctgaggcgctccatgatccgcagcttggagaccacgtccttggagatgaatgagaagatggtgcccaggctgttcagaaacctgaccaggcccttccagctggcaatgtaggggtccagcaagacctcttccttctcatcgagacactgcttgaaactgaccaggacgactttcagattgaaacctgtctccgagtcatccattttttgataggaacggaaatacagtagggctggggggctgtgtcgctggggtcagcttgctctgtggctcattttctgctctggggaacctgagagtcagctgcattccacctcgaccaggaagagggcctgggggttcctaggccggttggtgctgggagccctgtcctggcctccctggctgcagggactccatcggtgggggagggggaagggcacccagccgtggtgagagctcctggccaggagcaggtgggcaggttgctcagcaccctaggactgggcccttcatcactagggatcatgggctgcaagccctgcccagcccgtggcccaggctgctggagcactggtgcctgcagggtgctgaagcctggcgttgcaggccccacaggttgggttgcatgcttggcaccaggcggag

SEQ ID NO: 12428 - RNA, 1806 nt, Homo sapiens
  source 1..1806: mol_type = other RNA
ctgggttgggctgggctgggctgtgcagacccacggccgctgcgggaggcggcctgctgcgtccctcggggaactggtgccgtgcaggggctacggaggaggctgtcccaagggcggggacttcctgggcccttctgtgaggagccttggtctcagcttccggctgtcctgcccccagtctgcctggcacgctgaggggcaaacaaggcaggagaggcggggagagccccacagtgcccagactgctgttgagggtttctgccagccagggcatggagggcactgagtcccctgggctcaaggctgcccacctgggcagacacggggtcccaggcacgggcctgagatgaggacacatcggctggcagaaaggagaaaggatggagcctccacaccccgggacctgtgacttcaccctggttcgcagatgcaccccacaggctagggggtggcgacctttcgggctcttgcaggcccggcccccacccctgcctgctctgctctgcaccgcaccctggcgaggcctggctgcgcacgcgtgtaataggccgagggggagccgtggccgaggcgtcttgttccggaccgagagggtgggcctcttctgggctggtcgccaccttctctgtcacagtctgtggttcctaaccagctcagctcacaggggcgacagaggatctcctgttcccgcagcgcccagaaggctctgccacgggactcacggccctggccaccgcagcccagatctgcagcaggaaagccggtgcggccctggcttcccgcccctagggcaggtccagcagggagtgctcggcgtagagcttctgggagacgttgtagacacgctggatgaaggggagggcctcgcctagcatctgcacggcctgctccgggggccccacgttcatggcctccaggaagacctcgcgtgtgggcagcgtgcagaaggccacggtgacggcgcggcgcacgacccaggggtggtaggcggccagcgaggcgttgtaggagtcggcgcagagcgcggaggtgcgtgcgtcctcggggctggtacgcaggccctccaggaacagctgcagccagtgcagggcgcggtgcaggcgcagcaccgtccggcagccagactccgggtggtgggagcggcgctccaggtccaccagccggttgctcagctcgtgggccaccatggcctgcaggctgcggtagtgctcgctctgcgggccgcccctgaggcgctccatgatccgcagcttggagaccacgtccttggagatgaatgagaagatggtgcccaggctgttcagaaacctgaccaggcccttccagctggcaatgtaggggtccagcaagacctcttccttctcatcgagacactgcttgaaactgaccaggacgactttcagattgaaacctgtctccgagtcatccattttttgataggaacggaaatacagtagggctggggggctgtgtcgctggggtcagcttgctctgtggctcattttctgggaagggggcttcagatggcaccggactggatgggcaccggttcgggtccctgctccaccgagaggcccaggaaggggcggaggcccggggtggtgttggggaggggccgacctgagccacggctccgtcctgcgcgggagccgggtcctcggccgcccgcccgctccggccctctaggacgacgtcccctcccgctcccggcccctcggcgacttccggaccgtgcgggttgggttgggcaggtgcggccgccgagtccgagccgctcacctaggccgtagccgccgtgcgggcccc

SEQ ID NO: 12429 - RNA, 1654 nt, Homo sapiens
  source 1..1654: mol_type = other RNA
ctgggttgggctgggctgggctgtgcagacccacggccgctgcgggaggcggcctgctgcgtccctcggggaactggtgccgtgcaggggctacggaggaggctgtcccaagggcggggacttcctgggcccttctgtgaggagccttggtctcagcttccggctgtcctgcccccagtctgcctggcacgctgaggggcaaacaaggcaggagaggcggggagagccccacagtgcccagactgctgttgagggtttctgccagccagggcatggagggcactgagtcccctgggctcaaggctgcccacctgggcagacacggggtcccaggcacgggcctgagatgaggacacatcggctggcagaaaggagaaaggatggagcctccacaccccgggacctgtgacttcaccctggttcgcagatgcaccccacaggctagggggtggcgacctttcgggctcttgcaggcccggcccccacccctgcctgctctgctctgcaccgcaccctggcgaggcctggctgcgcacgcgtgtaataggccgagggggagccgtggccgaggcgtcttgttccggaccgagagggtgggcctcttctgggctggtcgccaccttctctgtcacagtctgtggttcctaaccagctcagctcacaggggcgacagaggatctcctgttcccgcagcgcccagaaggctctgccacgggactcacggccctggccaccgcagcccagatctgcagcaggaaagccggtgcggccctggcttcccgcccctagggcaggtccagcagggagtgctcggcgtagagcttctgggagacgttgtagacacgctggatgaaggggagggcctcgcctagcatctgcacggcctgctccgggggccccacgttcatggcctccaggaagacctcgcgtgtgggcagcgtgcagaaggccacggtgacggcgcggcgcacgacccaggggtggtaggcggccagcgaggcgttgtaggagtcggcgcagagcgcggaggtgcgtgcgtcctcggggctggtacgcaggccctccaggaacagctgcagccagtgcagggcgcggtgcaggcgcagcaccgtccggcagccagactccgggtggtgggagcggcgctccaggtccaccagccggttgctcagctcgtgggccaccatggcctgcaggctgcggtagtgctcgctctgcgggccgcccctgaggcgctccatgatccgcagcttggagaccacgtccttggagatgaatgagaagatggtgcccaggctgttcagaaacctgggaagggggcttcagatggcaccggactggatgggcaccggttcgggtccctgctccaccgagaggcccaggaaggggcggaggcccggggtggtgttggggaggggccgacctgagccacggctccgtcctgcgcgggagccgggtcctcggccgcccgcccgctccggccctctaggacgacgtcccctcccgctcccggcccctcggcgacttccggaccgtgcgggttgggttgggcaggtgcggccgccgagtccgagccgctcacctaggccgtagccgccgtgcgggccccgtccccgcccaccgccccgccctcgccccgccctcgcccgccgcc

SEQ ID NO: 12430 - RNA, 2712 nt, Homo sapiens
  source 1..2712: mol_type = other RNA
ctggtacaggcctgggggacagtcacagcggaaggacccttcactgttgatgcagtgcccattcatgcagattcctggggtctggcattcatcaacatcagtacagtaacgcccatttggagccaagacaaatcctggtttgcagatgcacttgaagctgccatcttcattgatgcacattccattcaaacacatgttggtagttgtacattcatcatgatcaacacagttttttccatctgtagttaattcaaagccggcattgcaaatgcactggaaacttccatctgtgttcacgcatcgaccgtttttacaaagaaccccattctggatgcactcatcaatatcaatgcatgcttgcttggtaggagtcctctggaatccagcatgacatttacaataataggaaccaggtgtgttaacacaatctccattagtgcagggatttgatgtgcattcatcaacatctatacaatctccatttgcatcctgcttataacccatgttgcattcacatcggtagcttgagacagttggtatacagcgtccatttaaacaaaggttagcatgatgcttacagatatctattgtctggttcagaattgttagtccagtgatgataggtccctgtcccccggcccccacaccggctcccccaacgccaggagaaaagccattgcctccagggatggggatgaagcctgtccctcctgggccatagccattgccattgccacttggggcaaagccatttcccccagtgcctccaggtctggaaccagcactccctggaattcctcccattggaagtccatccatgcaaagtctgcgatattcctcagaacctctgacaggacaggcttcaggaatggttccgatgccccagcagcggccaggctcacagcagcactgcattttcgtcattctccccgggagctcttgtgcacagcggccattcaccaggcccgagaaacacatgcctgttctctgatcgatgcatcgagagccatctgttgaggttacatatccacgtggacaaacacaaaaatagcttcccacggtgttggaacattcaccagtttcacatatcccaggaatgatgctgcactcatcaatgtcttcacatttctgagtagtttcactctgtttgtgaccagcagggcatctgcattcaaaagagcccactgtattgatacagtttcctccttggcatatccctgggatagcctggcattcatcaacatcttggcaagctccagtgcggatgttggggatgaaaccccgtcggcagggctgaggctgggctggacacatctcacagggatggccccacgcccgtccaatggtggcacagcacagagtcttcgtgcagacaatgcctgtcagctgcccttggcacatctggttgttgacctgagtgaaacacgggcctgtcctgtaatctctttcacactgtggaccagtgaacccataaacacaagcacagcggttgggtccgatgcaacgtccaccattctgacatccattttcacagacaggttgtccacaataagttccaatatatcctttctggcactggcagtggtcatctgcacaggtcccaccattcatgcatctcacactgcactgctgaattgattttgatccacaggttgatgatatttgcccactggaacaagtacacatgttaggacgggaacaaaatccatctccacaactatttctacaaatcgggacaatgcactggtttcctccagggagcgtcttccatccagggcagcagtaggagtggaatctggagccgcacacgttgggccctcggagcacgtcctgctgtcctcgccggcggacgcggctggccactgcggcaccctcctcgcgatactcgggcgctagaaacccgccttcagagcctgctgtagcggaccgaacctgttgcggcggcggctggggccggggcggcttgggcggaggaggctgaggctggccggccgtgccctgcgcccagagcaccacacagcccagccacaggaagtagagctggagacacagcctccgtcttctccccatcgccggcgccgaaagcgcgcggccgtagacccgcggagagggagtgatcaaagacaaaatctgcgcgcctcagaaaagagtcagggtctaataagcccttcgtcggctccggggactccctcgggctcgggctccctgctctagctggagacctcgacagagcgccggccccctgactgcccgcgaagcgagacgcggggcgccgggtctagcgcagtgagcggcgaggcgcggcggaggtgcagccggcagccccgagcggtacacgttgcataaccggcctaaagccccgagcgactccaggaccgtcagcgggcgggggaggaaattacaaaagccctggcgtaaaatttcaaaaaatgtgaacctcaaaagaaaaaagggcctgcacgcagagctcggcggattcccgtgcgctccgaagacggatattggaaagctgcaaaagtcaccagaaagaaacaggcaagcaaacaaaagtcgcccccagaagaagaggagggttccctccgggctcgctcggagtcccacagggcaacgaagcgcgggtagcggctgcggagccgggcggaggtgcgcggggccggggcgtgcggccagcaagagagagggcgggaggctgggcgctggagaagatgcggc

SEQ ID NO: 12431 - RNA, 2191 nt, Homo sapiens
  source 1..2191: mol_type = other RNA
ctggtacaggcctgggggacagtcacagcggaaggacccttcactgttgatgcagtgcccattcatgcagattcctggggtctggcattcatcaacatcagtacagtaacgcccatttggagccaagacaaatcctggtttgcagatgcacttgaagctgccatcttcattgatgcacattccattcaaacacatgttggtagttgtacattcatcatgatcaacacagttttttccatctgtagttaattcaaagccggcattgcaaatgcactggaaacttccatctgtgttcacgcatcgaccgtttttacaaagaaccccattctggatgcactcatcaatatcaatgcatgcttgcttggtaggagtcctctggaatccagcatgacatttacaataataggaaccaggtgtgttaacacaatctccattagtgcagggatttgatgtgcattcatcaacatctatacaatctccatttgcatcctgcttataacccatgttgcattcacatcggtagcttgagacagttggtatacagcgtccatttaaacaaaggttagcatgatgcttacagatatctattgtctggttcagaattgttagtccagtgatgataggtccctgtcccccggcccccacaccggctcccccaacgccaggagaaaagccattgcctccagggatggggatgaagcctgtccctcctgggccatagccattgccattgccacttggggcaaagccatttcccccagtgcctccaggtctggaaccagcactccctggaattcctcccattggaagtccatccatgcaaagtctgcgatattcctcgatgcatcgagagccatctgttgaggttacatatccacgtggacaaacacaaaaatagcttcccacggtgttggaacattcaccagtttcacatatcccaggaatgatgctgcactcatcaatgtcttcacatttctgagtagtttcactctgtttgtgaccagcagggcatctgcattcaaaagagcccactgtattgatacagtttcctccttggcatatccctgggatagcctggcattcatcaacatcttggcaagctccagtgcggatgttggggatgaaaccccgtcggcagggctgaggctgggctggacacatctcacagggatggccccacgcccgtccaatggtggcacagcacagagtcttcgtgcagacaatgcctgtcagctgcccttggcacatctggttgttgacctgagtgaaacacgggcctgtcctgtaatctctttcacactgtggaccagtgaacccataaacacaagcacagcggttgggtccgatgcaacgtccaccattctgacatccattttcacagacaggttgtccacaataagttccaatatatcctttctggcactggcagtggtcatctgcacaggtcccaccattcatgcatctcacactgcactgctgaattgattttgatccacaggttgatgatatttgcccactggaacaagtacacatgttaggacgggaacaaaatccatctccacaactatttctacaaatcgggacaatgcactggtttcctccagggagcgtcttccatccagggcagcagtaggagtggaatctggagccgcacacgttgggccctcggagcacgtcctgctgtcctcgccggcggacgcggctggccactgcggcaccctcctcgcgatactcgggcgctagaaacccgccttcagagcctgctgtagcggaccgaacctgttgcggcggcggctggggccggggcggcttgggcggaggaggctgaggctggccggccgtgccctgcgcccagagcaccacacagcccagccacaggaagtagagctggagacacagcctccgtcttctccccatcgccggcgccgaaagcgcgcggccgtagacccgcggagagggagtgatcaaagacaaaatctgcgcgcctcagaaaagagtcagggtctaataagcccttcgtcggctccggggactccctcgggctcgggctccctgctctagctggagacctcgacagagcgccggccccctgactgcccgcgaagcgagacgcggggcgccgggtctagcgcagtgagcggcgaggcgcggcggaggtgcagccggcagccccgagcggtacacgttgcat

SEQ ID NO: 12432 - RNA, 739 nt, Homo sapiens
  source 1..739: mol_type = other RNA
ctggtacaggcctgggggacagtgctcgcatgtagcagggccctggcaggggccccacagcaaactcggtgacattgggatgctcctggtcaccaaagaagatgacggcacgggcttcccgcacaggatgcctttcacctttatccagaaacctcagcacatggtacttcttgggcagcagcatctcgatgagaaacacggtgttcttggccatggtggtggtactggagggctgcagcctcagctccttcttggaccagaggaagctgtgcactgccttcagctcttggttgcttaggtctgaaaacacccctgccttcctgggcagagtccccggggagggctccgccatggccgtctgcagcatcaggatggcagccacggcccagcccagggccggcatctctcgctccacggctctgaagctgacagatggaccagggcaggggctgatagaggctggcacccacagcaaaacagagaattcaaccgctcttgatttgaatgcaggtcattcgaagagaagttagggctttagtcctttacaattcagctttagtcaaaggggttcctctctctgtgtttgcctcatcattggtagtaggggacaaacctggaggttctctcatcaacaggtacagatttgaaagcaggcagggtggaggagcttgttctttctgcagcctgacccaggagaggaggtaaagcagagggctcccagaggccgcccttgtaggtc

SEQ ID NO: 12433 - RNA, 709 nt, Homo sapiens
  source 1..709: mol_type = other RNA
ctggtacaggcctgggggacagtgctcgcatgtagcagggccctggcaggggccccacagcaaactcggtgacattgggatgctcctggtcaccaaagaagatgacggcacgggcttcccgcacaggatgcctttcacctttatccagaaacctcagcacatggtacttcttgggcagcagcatctcgatgagaaacacggtgttcttggccatggtggtggtactggagggctgcagcctcagctccttcttggaccagaggaagctgtgcactgccttcagctcttggttgcttaggtctgaaaacacccctgccttcctgggcagagtccccggggagggctccgccatggccgtctgcagcatcaggatggcagccacggcccagcccagggccggcatctctcgctccacggctctgaagctgacagatggaccagggcaggggctgatagaggctggcacccacagcaaaacagagaattcaaccgctcttgatttgaatgcaggtcattcgaagagaagttagggctttagtcctttacaattcagctttagtcaaaggggttcctctctctgtgtttgcctcatcattggtagtaggggacaaacctggaggttctctcatcaacaggtacagatttgaaagctaaattcctgcagtagactcctactggctttcctgctcccaaacttgtctcctccaaa

SEQ ID NO: 12434 - RNA, 479 nt, Homo sapiens
  source 1..479: mol_type = other RNA
ctggtacaggcctgggggacagtgctcgcatgtagcagggccctggcaggggccccacagcaaactcggtgacattgggatgctcctggtcaccaaagaagatgacggcacgggcttcccgcacaggatgcctttcacctttatccagaaacctcagcacatggtacttcttgggcagcagcatctcgatgagaaacacggtgttcttggccatggtggtggtactggagggctgcagcctcagctccttcttggaccagaggaagctgtgcactgccttcagctcttggttgcttaggtctgaaaacacccctgccttcctgggcagagtccccggggagggctccgccatggccgtctgcagcatcaggatggcagccacggcccagcccagggccggcatctctcgctccacggctctggagggagcaggtgaggcaggggctgcaggcggaacccagagccagcaggaaggatat

SEQ ID NO: 12435 - RNA, 461 nt, Homo sapiens
  source 1..461: mol_type = other RNA
ctggtacaggcctgggggacagtgctcgcatgtagcagggccctggcaggggccccacagcaaactcggtgacattgggatgctcctggtcaccaaagaagatgacggcacgggcttcccgcacaggatgcctttcacctttatccagaaacctcagcacatggtacttcttgggcagcagcatctcgatgagaaacacggtgttcttggccatggtggtggtactggagggctgcagcctcagctccttcttggaccagaggaagctgtgcactgccttcagctcttggttgcttaggtctgaaaacacccctgccttcctgggcagagtccccggggagggctccgccatggccgtctgcagcatcaggatggcagccacggcccagcccagggccggcatctctcgctccacggctctgtgtgctctgctcccagttcgctctgcttccagcctttgc

SEQ ID NO: 12436 - RNA, 421 nt, Homo sapiens
  source 1..421: mol_type = other RNA
ctggtacaggcctgggggacagtttcgagtctcagctccaacacttcctgcatgccaaaactgcgtcagcctttgcttgttcttaactttagcaggaaagcctctagtgttccaccattgagatcttcctttaaaatcctttttgtaaaatttgggctgtgctatccattctatctgatgttccacagcacttcattctacacaaaaaatgaaaggagacttgcagaattgaggggacctgccccaagtaacctaaggagcaggtgggagctctcatttccttttctgcagttcaggggtcttctgctatgtggaaaagctcagggcccaggataagtccactgacattaaaaattaaaaaaactgaattcaaggctgggtgcagtggctactgcctgtaatcatagcactttgggaggcc

SEQ ID NO: 12437 - RNA, 282 nt, Homo sapiens
  source 1..282: mol_type = other RNA
ctggtacaggcctgggggacagtttcgagtctcagctccaacacttcctgcatgccaaaactgcgtcagcctttgcttgttcttaactttagcaggaaagcctctagtgttccaccattgagatcttcctttaaaatcctttttgtaaaatttgggctgtgctatccattctatctgatgttccacagcacttccccagctcaaaaacacttcggcttgggggcggtgccaaggctgtgagtgcttccaacacttcggcttgggggcggtgccaaggctgtg

SEQ ID NO: 12438 - RNA, 283 nt, Homo sapiens
  source 1..283: mol_type = other RNA
ctggtacaggcctgggggacagtttcgagtctcagctccaacacttcctgcatgccaaaactgcgtcagcctttgcttgttcttaactttagcaggaaagcctctagtgttccaccattgagatcttcctttaaaatcctttttgtaaaatttgggctgtgctatccattctatctgatgttccacagcacttcctccaaagatgatgatgggttgtggggagtcagagctgaagtcggcggacggggaagaagccgcggcggtcccggggccacccccggag

SEQ ID NO: 12439 - RNA, 479 nt, Homo sapiens
  source 1..479: mol_type = other RNA
ctggtacaggcctgggggacagtttcgagtctcagctccaacacttcctgcatgccaaaactgcgtcagcctttgcttgttcttaactttagcaggaaagcctctagtgttccaccattgagatcttcctttaaaatcctttttgtaaaatttgggctgtgctatccattctatctgatgttccacagcacttcctccgtccccgctgcgctctcagggctgaacgtgccgcgctccaagcggctcttccgggacctggtgagcctgcaggtgccggaggaacaggttctgaatgccgcgctcagggagaaattggctctcctgccgccacaggctcgagccccgcacccaaaggtgatggggtctgggcgtggggcttcctccatgtacccccttacccggatccttcctcccaaagtgtaaccttgctttgggcccaacctcccaacaggagccacctgggcctgggccagacatga

SEQ ID NO: 12440 - RNA, 317 nt, Homo sapiens
  source 1..317: mol_type = other RNA
ctggtacaggcctgggggacagtttcgagtctcagctccaacacttcctgcatgccaaaactgcgtcagcctttgcttgttcttaactttagcaggaaagcctctagtgttccaccattgagatcttcctttaaaatcctttttgtaaaatttgggctgtgctatccattctatctgatgttccacagcacttcctggtcactgccctgccctctgctcccaggtccgcttccgcctgacgccgccctccccggtgcggtccgagccgcagcctgcggtgccgcaggagctggagatgcccgtgctgaagagcagcc

SEQ ID NO: 12441 - RNA, 286 nt, Homo sapiens
  source 1..286: mol_type = other RNA
ctggtacaggcctgggggacagtttcgagtctcagctccaacacttcctgcatgccaaaactgcgtcagcctttgcttgttcttaactttagcaggaaagcctctagtgttccaccattgagatcttcctttaaaatcctttttgtaaaatttgggctgtgctatccattctatctgatgttccacagcacttccttaaagctgccccatttatggccaggtgcggtggctcatgcctgtaatcccagcactttgggaggccgaggtgggcggatcacgaggtcag

SEQ ID NO: 12442 - RNA, 3190 nt, Homo sapiens
  source 1..3190: mol_type = other RNA
ctgtaatataaatttaatttattttattaaaataacataattgagggaccatcagataactgtattttgtcaggtgcaataaaaacaaaattaaaacccaaatcatcaagaaaacctgtattcctggcttccttgtatacacatgatgtgactagagaaacaaggctgtttgtttgtttgtttgttagagaaacaaggctggccctgcggccccgccccataggggcagctcctggaagacaaaattcagcatgatggaagactgctccctgagagggctgagatgcggattggccgagtgccttgcctggaaaaccatcccaatgcactggacaccttagaagctgtgaaaggaggacgtgtcccctaagaaaagttccatagtaccaaagcaggctccttcgggcggccagagtctcggcagtcctgggctgtttggtgccttatgtgcaaaatgtctggcgctgcaccactctctgaagaaagtcccgcctgtgacatgcattcctccagaagctgatttccaaaatcccatgtgtctccacatcagggctggactgcctgctaccttacttcctctaaatactcatgtagccaacagctggggctgggcccctgctttttgtactaccatcaacatccacttgcgcatctacagaaggctgggccttgagcatggggaatgtggggagggagcaggacacaccagcactgcaaatggcttccttctcccagggcccaaagggatagaaaagaaggcaacatgaagttaaggccctgtgagcagtctagaaggtccttagcagcagcttctctgaaaacatgtgttctgcctctggagaaagggagcagaaaagtggtgcctgctggcttctcctcctcccctggcagcctgaagacaggtgcaaagtcaactagaagacaggcagcctcggggacgtggtcagcgtgcaagcattgatatcctcagtgtgggctgcccgatgcaaggatggctcggaagcgctccggttgatcttcggtagagagtgttggagcagctcaatggaagacaggatctggggaaaaagaggcctctcttcctttactttcttcacacagtcagctaccagcctcttcattgctttggggcagttcttatatagcttactaagatctggggaggcatatcctcggcccaccatgaagatgatctgatctcggttgttgatgtgagaataaggaagctcccccgtcatcagttcatacaatacgatgccataggagtagacatccgactggaaactgaatgggttgttatcctgcattcggatcacctctggggccatccagaggacagagccagtaggttgttcaacctgctgagaaccactccagcgtgactttactgttgccaaaccaaaatctccaattttcactgttaagccttcatggagaaatatattgttggatttcatgtctctatggatgatgttctttgcatgcaaatagtccattccctgagccgtctgccgggcaatgtcaattagctggaacatctgaaacttggtctcctggacatgcaggtgtttgtagaggctgctgccctcgcaccactgggtcacaattgccaggttgtcctttgtcatgtaccccatgaaaagcagaatgttcacatgccgtgttttgcgcagaacagccacctcattcctgaaggcctggaattgctctggggttgggtcgacaacctttaggatctttactgcaacatctccgtgccatttacccttataaacagttccaaaagagcctgacccaatccgagtggacagcatcacttcactggcttctatttcccaataatagcttgaatctctctgtccacgaggcaattttgtttttctcctgggtcccagatactggtgcccgctctctttgtgctggcacgggggttttcggctgtgaccagcctgttgggctcagattgttggggctactggacagggctgaaggtgaggctgattcgctgtgacttcgaattgcatcctcaatcatcctgctgtccacaggcagggtggtgctgaccatgtggacattaggtgtggatgtcgacctctgcctctgggagagggaaccttcagatgagggactggaggtgttaaaggtgaaggcgtgaggtgtagaatatctgtgctgagaactaacaggcatcctggaaacagactctcgcatacgacgcatagtcaaagaaggtagtgctgggactccactatcaccaatagtggaatttggaaacaataagagttgtctgatgttactccagtccacacacatagtaggtactttggtgctacagtgctcatgaaatttgtagccacaagtctgacatcgaaatccattgagcaggaatttctgacagatgtcacagaaggcaagcttcaggaacgtcttccgagcaaagttgtgtgttgtgaggggaacatgatccaggaaatctacttgaagttcttctccaatcaaagacgcagcatcagtattccaatctaagcgtgcttttttacctttgtgttcgtggagaagtctgaacactgcacagcactctggttgcaggcccctcaccttgagtgctttcataaggcagtcatgcaagctcattccatttcgcacattgaccactgttctttgcttgttcggcaagaaaacacggatagtgttgcttgtcttagaaggatctgtgagtttgccatcatctgatgcccggcgctgatagccaaactgctgaactattgtaggagagatgcagctggagccatcaaacacggcatctttgaatccaaaaccattgctgatcgtcttccaagctccctgtatgtgctccattgatgcagcttaaacaattcttaaacctgagggagccaggccgccccaacgtcctgtcgttcggcggcagcttctcgcccgctcctcctccccgcggcgggtgagggagcgggaggcggtcacattcggcgcgtccccagcccaggggacggagccccgagcagcccccgcatcgtagcaaacgcgctccgcgcctcagggcacgcgccccaaagcccggccagctgacccttttcggggcccaaaaaaggcagcagaaagccgttcccgcctcacaatcgttttcctcttactcccgccatctaagatggcggcccaagcgcccgcgatt

SEQ ID NO: 12443 - RNA, 2980 nt, Homo sapiens
  source 1..2980: mol_type = other RNA
ctgtaatataaatttaatttattttattaaaataacataattgagggaccatcagataactgtattttgtcaggtgcaataaaaacaaaattaaaacccaaatcatcaagaaaacctgtattcctggcttccttgtatacacatgatgtgactagagaaacaaggctgtttgtttgtttgtttgttagagaaacaaggctggccctgcggccccgccccataggggcagctcctggaagacaaaattcagcatgatggaagactgctccctgagagggctgagatgcggattggccgagtgccttgcctggaaaaccatcccaatgcactggacaccttagaagctgtgaaaggaggacgtgtcccctaagaaaagttccatagtaccaaagcaggctccttcgggcggccagagtctcggcagtcctgggctgtttggtgccttatgtgcaaaatgtctggcgctgcaccactctctgaagaaagtcccgcctgtgacatgcattcctccagaagctgatttccaaaatcccatgtgtctccacatcagggctggactgcctgctaccttacttcctctaaatactcatgtagccaacagctggggctgggcccctgctttttgtactaccatcaacatccacttgcgcatctacagaaggctgggccttgagcatggggaatgtggggagggagcaggacacaccagcactgcaaatggcttccttctcccagggcccaaagggatagaaaagaaggcaacatgaagttaaggccctgtgagcagtctagaaggtccttagcagcagcttctctgaaaacatgtgttctgcctctggagaaagggagcagaaaagtggtgcctgctggcttctcctcctcccctggcagcctgaagacaggtgcaaagtcaactagaagacaggcagcctcggggacgtggtcagcgtgcaagcattgatatcctcagtgtgggctgcccgatgcaaggatggctcggaagcgctccggttgatcttcggtagagagtgttggagcagctcaatggaagacaggatctggggaaaaagaggcctctcttcctttactttcttcacacagtcagctaccagcctcttcattgctttggggcagttcttatatagcttactaagatctggggaggcatatcctcggcccaccatgaagatgatctgatctcggttgttgatgtgagaataaggaagctcccccgtcatcagttcatacaatacgatgccataggagtagacatccgactggaaactgaatgggttgttatcctgcattcggatcacctctggggccatccagaggacagagccagtaggttgttcaacctgctgagaaccactccagcgtgactttactgttgccaaaccaaaatctccaattttcactgttaagccttcatggagaaatatattgttggatttcatgtctctatggatgatgttctttgcatgcaaatagtccattccctgagccgtctgccgggcaatgtcaattagctggaacatctgaaacttggtctcctggacatgcaggtgtttgtagaggctgctgccctcgcaccactgggtcacaattgccaggttgtcctttgtcatgtaccccatgaaaagcagaatgttcacatgccgtgttttgcgcagaacagccacctcattcctgaaggcctggaattgctctggggttgggtcgacaacctttaggatctttactgcaacatctccgtgccatttacccttataaacagttccaaaagagcctgacccaatccgagtggacagcatcacttcactggcttctatttcccaataatagcttgaatctctctgtccacgaggcctaattttgtttttctcctgggtcccagatactggtgcccgctctctttgtgctggcacgggggttttcggctgtgaccagcctgttgggctcagattgttggggctactggacagggctgaaggtgaggctgattcgctgtgacttcgaattgcatcctcaatcatcctgctgtccacaggcagggtggtgctgaccatgtggacattaggtgtggatgtcgacctctgcctctgggagagggaaccttcagatgagggactggaggtgttaaaggtgaaggcgtgaggtgtagaatatctgtgctgagaaaagagttgtctgatgttactccagtccacacacatagtaggtactttggtgctacagtgctcatgaaatttgtagccacaagtctgacatcgaaatccattgagcaggaatttctgacagatgtcacagaaggcaagcttcaggaacgtcttccgagcaaagttgtgtgttgtgaggggaacatgatccaggaaatctacttgaagttcttctccaatcaaagacgcagcatcagtattccaatctaagcgtgcttttttacactgttctttgcttgttcggcaagaaaacacggatagtgttgcttgtcttagaaggatctgtgagtttgccatcatctgatgcccggcgctgatagccaaactgctgaactattgtaggagagatgcagctggagccatcaaacacggcatctttgaatccaaaaccattgctgatcgtcttccaagctccctgtatgtgctccattgatgcagcttaaacaattcttaaacctgagggagccaggccgccccaacgtcctgtcgttcggcggcagcttctcgcccgctcctcctccccgcggcgggtgagggagcgggaggcggtcacattcggcgcgtccccagcccaggggacggagccccgagcagcccccgcatcgtagcaaacgcgctccgcgcctcagggcacgcgccccaaagcccggccagctgacccttttcggggcccaaaaaaggcagcagaaagccgttcccgcctcacaatcgttttcctcttactcccgccatctaagatggcggcccaagcgcccgcgatt

SEQ ID NO: 12444 - RNA, 3093 nt, Homo sapiens
  source 1..3093: mol_type = other RNA
ctgtaatataaatttaatttattttattaaaataacataattgagggaccatcagataactgtattttgtcaggtgcaataaaaacaaaattaaaacccaaatcatcaagaaaacctgtattcctggcttccttgtatacacatgatgtgactagagaaacaaggctgtttgtttgtttgtttgttagagaaacaaggctggccctgcggccccgccccataggggcagctcctggaagacaaaattcagcatgatggaagactgctccctgagagggctgagatgcggattggccgagtgccttgcctggaaaaccatcccaatgcactggacaccttagaagctgtgaaaggaggacgtgtcccctaagaaaagttccatagtaccaaagcaggctccttcgggcggccagagtctcggcagtcctgggctgtttggtgccttatgtgcaaaatgtctggcgctgcaccactctctgaagaaagtcccgcctgtgacatgcattcctccagaagctgatttccaaaatcccatgtgtctccacatcagggctggactgcctgctaccttacttcctctaaatactcatgtagccaacagctggggctgggcccctgctttttgtactaccatcaacatccacttgcgcatctacagaaggctgggccttgagcatggggaatgtggggagggagcaggacacaccagcactgcaaatggcttccttctcccagggcccaaagggatagaaaagaaggcaacatgaagttaaggccctgtgagcagtctagaaggtccttagcagcagcttctctgaaaacatgtgttctgcctctggagaaagggagcagaaaagtggtgcctgctggcttctcctcctcccctggcagcctgaagacaggtgcaaagtcaactagaagacaggcagcctcggggacgtggtcagcgtgcaagcattgatatcctcagtgtgggctgcccgatgcaaggatggctcggaagcgctccggttgatcttcggtagagagtgttggagcagctcaatggaagacaggatctggggaaaaagaggcctctcttcctttactttcttcacacagtcagctaccagcctcttcattgctttggggcagttcttatatagcttactaagatctggggaggcatatcctcggcccaccatgaagatgatctgatctcggttgttgatgtgagaataaggaagctcccccgtcatcagttcatacaatacgatgccataggagtagacatccgactggaaactgaatgggttgttatcctgcattcggatcacctctggggccatccagaggacagagccagtaggttgttcaacctgctgagaaccactccagcgtgactttactgttgccaaaccaaaatctccaattttcactgttaagccttcatggagaaatatattgttggatttcatgtctctatggatgatgttctttgcatgcaaatagtccattccctgagccgtctgccgggcaatgtcaattagctggaacatctgaaacttggtctcctggacatgcaggtgtttgtagaggctgctgccctcgcaccactgggtcacaattgccaggttgtcctttgtcatgtaccccatgaaaagcagaatgttcacatgccgtgttttgcgcagaacagccacctcattcctgaaggcctggaattgctctggggttgggtcgacaacctttaggatctttactgcaacatctccgtgccatttacccttataaacagttccaaaagagcctgacccaatccgagtggacagcatcacttcactggcttctatttcccaataatagcttgaatctctctgtccacgaggcctaattttgtttttctcctgggtcccagatactggtgcccgctctctttgtgctggcacgggggttttcggctgtgaccagcctgttgggctcagattgttggggctactggacagggctgaaggtgaggctgattcgctgtgacttcgaattgcatcctcaatcatcctgctgtccacaggcagggtggtgctgaccatgtggacattaggtgtggatgtcgacctctgcctctgggagagggaaccttcagatgagggactggaggtgttaaaggtgaaggcgtgaggtgtagaatatctgtgctgagaaaagagttgtctgatgttactccagtccacacacatagtaggtactttggtgctacagtgctcatgaaatttgtagccacaagtctgacatcgaaatccattgagcaggaatttctgacagatgtcacagaaggcaagcttcaggaacgtcttccgagcaaagttgtgtgttgtgaggggaacatgatccaggaaatctacttgaagttcttctccaatcaaagacgcagcatcagtattccaatctaagcgtgcttttttacctttgtgttcgtggagaagtctgaacactgcacagcactctggttgcaggcccctcaccttgagtgctttcataaggcagtcatgcaagctcattccatttcgcacattgaccactgttctttgcttgttcggcaagaaaacacggatagtgttgcttgtcttagaaggatctgtgagtttgccatcatctgatgcccggcgctgatagccaaactgctgaactattgtaggagagatgcagctggagccatcaaacacggcatctttgaatccaaaaccattgctgatcgtcttccaagctccctgtatgtgctccattgatgcagcttaaacaattcttaaacctgagggagccaggccgccccaacgtcctgtcgttcggcggcagcttctcgcccgctcctcctccccgcggcgggtgagggagcgggaggcggtcacattcggcgcgtccccagcccaggggacggagccccgagcagcccccgcatcgtagcaaacgcgctccgcgcctcagggcacgcgccccaaagcccggccagctgacccttttcggggcccaaaaaaggcagcagaaagccgttcccgcctcacaatcgttttcctcttactcccgccatctaagatggcggcccaagcgcccgcgatt

SEQ ID NO: 12445 - RNA, 2881 nt, Homo sapiens
  source 1..2881: mol_type = other RNA
ctgtaatataaatttaatttattttattaaaataacataattgagggaccatcagataactgtattttgtcaggtgcaataaaaacaaaattaaaacccaaatcatcaagaaaacctgtattcctggcttccttgtatacacatgatgtgactagagaaacaaggctgtttgtttgtttgtttgttagagaaacaaggctggccctgcggccccgccccataggggcagctcctggaagacaaaattcagcatgatggaagactgctccctgagagggctgagatgcggattggccgagtgccttgcctggaaaaccatcccaatgcactggacaccttagaagctgtgaaaggaggacgtgtcccctaagaaaagttccatagtaccaaagcaggctccttcgggcggccagagtctcggcagtcctgggctgtttggtgccttatgtgcaaaatgtctggcgctgcaccactctctgaagaaagtcccgcctgtgacatgcattcctccagaagctgatttccaaaatcccatgtgtctccacatcagggctggactgcctgctaccttacttcctctaaatactcatgtagccaacagctggggctgggcccctgctttttgtactaccatcaacatccacttgcgcatctacagaaggctgggccttgagcatggggaatgtggggagggagcaggacacaccagcactgcaaatggcttccttctcccagggcccaaagggatagaaaagaaggcaacatgaagttaaggccctgtgagcagtctagaaggtccttagcagcagcttctctgaaaacatgtgttctgcctctggagaaagggagcagaaaagtggtgcctgctggcttctcctcctcccctggcagcctgaagacaggtgcaaagtcaactagaagacaggcagcctcggggacgtggtcagcgtgcaagcattgatatcctcagtgtgggctgcccgatgcaaggatggctcggaagcgctccggttgatcttcggtagagagtgttggagcagctcaatggaagacaggatctggggaaaaagaggcctctcttcctttactttcttcacacagtcagctaccagcctcttcattgctttggggcagttcttatatagcttactaagatctggggaggcatatcctcggcccaccatgaagatgatctgatctcggttgttgatgtgagaataaggaagctcccccgtcatcagttcatacaatacgatgccataggagtagacatccgactggaaactgaatgggttgttatcctgcattcggatcacctctggggccatccagaggacagagccagtaggttgttcaacctgctgagaaccactccagcgtgactttactgttgccaaaccaaaatctccaattttcactgttaagccttcatggagaaatatattgttggatttcatgtctctatggatgatgttctttgcatgcaaatagtccattccctgagccgtctgccgggcaatgtcaattagctggaacatctgaaacttggtctcctggacatgcaggtgtttgtagaggctgctgccctcgcaccactgggtcacaattgccaggttgtcctttgtcatgtaccccatgaaaagcagaatgttcacatgccgtgttttgcgcagaacagccacctcattcctgaaggcctggaattgctctggggttgggtcgacaacctttaggatctttactgcaacatctccgtgccatttacccttataaacagttccaaaagagcctgacccaatccgagtggacagcatcacttcactggcttctatttcccaataatagcttgaatctctctgtccacgaggcctaattttgtttttctcctgggtcccagatactggtgcccgctctctttgtgctggcacgggggttttcggctgtgaccagcctgttgggctcagattgttggggctactggacagggctgaaggtgaggctgattcgctgtgacttcgaattgcatcctcaatcatcctgctgtccacaggcagggtggtgctgaccatgtggacattaggtgtggatgtcgacctctgcctctgggagagggaaccttcagatgagggactggaggtgttaaaggtgaaggcgtgaggtgtagaatatctgtgctgagaaaagagttgtctgatgttactccagtccacacacatagtaggtactttggtgctacagtgctcatgaaatttgtagccacaagtctgacatcgaaatccattgagcaggaatttctgacagatgtcacagaaggcaagcttcaggaacgtcttccgagcaaagttgtgtgttgtgaggggaacatgatccaggaaatctacttgaagttcttctccaatcaaagacgcagcatcagtattccaatctaagcgtgcttttttacctttgtgttcgtggagaagtctgaacactgcacagcactctggttgcaggcccctcaccttgagtgctttcataaggcagtcatgcaagctcattccatttcgcacattgaccactgttctttgcttgttcggcaagaaaacacggatagtgttgcttgtcttagaaggatctgtgagtttgccatcatctgatgcccggcgctgatagccaaactgctgaactattgtaggagagatgcagctggagccatcaaacacggcatctttgaatccaaaaccattgctgatcgtcttccaagctccctgtatgtgctccattgatgcagcttaaacaattcttaaacctgtaatcccagcactttgggaggcccagatgggaggacagcttgaggccaagagttcaagaccagcctggtcaacacagcaagaccccattt

SEQ ID NO: 12446 - RNA, 3079 nt, Homo sapiens
  source 1..3079: mol_type = other RNA
ctgtaatataaatttaatttattttattaaaataacataattgagggaccatcagataactgtattttgtcaggtgcaataaaaacaaaattaaaacccaaatcatcaagaaaacctgtattcctggcttccttgtatacacatgatgtgactagagaaacaaggctgtttgtttgtttgtttgttagagaaacaaggctggccctgcggccccgccccataggggcagctcctggaagacaaaattcagcatgatggaagactgctccctgagagggctgagatgcggattggccgagtgccttgcctggaaaaccatcccaatgcactggacaccttagaagctgtgaaaggaggacgtgtcccctaagaaaagttccatagtaccaaagcaggctccttcgggcggccagagtctcggcagtcctgggctgtttggtgccttatgtgcaaaatgtctggcgctgcaccactctctgaagaaagtcccgcctgtgacatgcattcctccagaagctgatttccaaaatcccatgtgtctccacatcagggctggactgcctgctaccttacttcctctaaatactcatgtagccaacagctggggctgggcccctgctttttgtactaccatcaacatccacttgcgcatctacagaaggctgggccttgagcatggggaatgtggggagggagcaggacacaccagcactgcaaatggcttccttctcccagggcccaaagggatagaaaagaaggcaacatgaagttaaggccctgtgagcagtctagaaggtccttagcagcagcttctctgaaaacatgtgttctgcctctggagaaagggagcagaaaagtggtgcctgctggcttctcctcctcccctggcagcctgaagacaggtgcaaagtcaactagaagacaggcagcctcggggacgtggtcagcgtgcaagcattgatatcctcagtgtgggctgcccgatgcaaggatggctcggaagcgctccggttgatcttcggtagagagtgttggagcagctcaatggaagacaggatctggggaaaaagaggcctctcttcctttactttcttcacacagtcagctaccagcctcttcattgctttggggcagttcttatatagcttactaagatctggggaggcatatcctcggcccaccatgaagatgatctgatctcggttgttgatgtgagaataaggaagctcccccgtcatcagttcatacaatacgatgccataggagtagacatccgactggaaactgaatgggttgttatcctgcattcggatcacctctggggccatccagaggacagagccagtaggttgttcaacctgctgagaaccactccagcgtgactttactgttgccaaaccaaaatctccaattttcactgttaagccttcatggagaaatatattgttggatttcatgtctctatggatgatgttctttgcatgcaaatagtccattccctgagccgtctgccgggcaatgtcaattagctggaacatctgaaacttggtctcctggacatgcaggtgtttgtagaggctgctgccctcgcaccactgggtcacaattgccaggttgtcctttgtcatgtaccccatgaaaagcagaatgttcacatgccgtgttttgcgcagaacagccacctcattcctgaaggcctggaattgctctggggttgggtcgacaacctttaggatctttactgcaacatctccgtgccatttacccttataaacagttccaaaagagcctgacccaatccgagtggacagcatcacttcactggcttctatttcccaataatagcttgaatctctctgtccacgaggcctaattttgtttttctcctgggtcccagatactggtgcccgctctctttgtgctggcacgggggttttcggctgtgaccagcctgttgggctcagattgttggggctactggacagggctgaaggtgaggctgattcgctgtgacttcgaattgcatcctcaatcatcctgctgtccacaggcagggtggtgctgaccatgtggacattaggtgtggatgtcgacctctgcctctgggagagggaaccttcagatgagggactggaggtgttaaaggtgaaggcgtgaggtgtagaatatctgtgctgagaactaacaggcatcctggaaacagactctcgcatacgacgcatagtcaaagaaggtagtgctgggactccactatcaccaatagtggaatttggaaacaataagagttgtctgatgttactccagtccacacacatagtaggtactttggtgctacagtgctcatgaaatttgtagccacaagtctgacatcgaaatccattgagcaggaatttctgacagatgtcacagaaggcaagcttcaggaacgtcttccgagcaaagttgtgtgttgtgaggggaacatgatccaggaaatctacttgaagttcttctccaatcaaagacgcagcatcagtattccaatctaagcgtgcttttttacactgttctttgcttgttcggcaagaaaacacggatagtgttgcttgtcttagaaggatctgtgagtttgccatcatctgatgcccggcgctgatagccaaactgctgaactattgtaggagagatgcagctggagccatcaaacacggcatctttgaatccaaaaccattgctgatcgtcttccaagctccctgtatgtgctccattgatgcagcttaaacaattcttaaacctgagggagccaggccgccccaacgtcctgtcgttcggcggcagcttctcgcccgctcctcctccccgcggcgggtgagggagcgggaggcggtcacattcggcgcgtccccagcccaggggacggagccccgagcagcccccgcatcgtagcaaacgcgctccgcgcctcagggcacgcgccccaaagcccggccagctgacccttttcggggcccaaaaaaggcagcagaaagccgttcccgcctcacaatcgttttcctcttactcccgccatctaagatggcggcccaagcgcccgcgatt

SEQ ID NO: 12447 - RNA, 3172 nt, Homo sapiens
  source 1..3172: mol_type = other RNA
ctgtaatataaatttaatttattttattaaaataacataattgagggaccatcagataactgtattttgtcaggtgcaataaaaacaaaattaaaacccaaatcatcaagaaaacctgtattcctggcttccttgtatacacatgatgtgactagagaaacaaggctgtttgtttgtttgtttgttagagaaacaaggctggccctgcggccccgccccataggggcagctcctggaagacaaaattcagcatgatggaagactgctccctgagagggctgagatgcggattggccgagtgccttgcctggaaaaccatcccaatgcactggacaccttagaagctgtgaaaggaggacgtgtcccctaagaaaagttccatagtaccaaagcaggctccttcgggcggccagagtctcggcagtcctgggctgtttggtgccttatgtgcaaaatgtctggcgctgcaccactctctgaagaaagtcccgcctgtgacatgcattcctccagaagctgatttccaaaatcccatgtgtctccacatcagggctggactgcctgctaccttacttcctctaaatactcatgtagccaacagctggggctgggcccctgctttttgtactaccatcaacatccacttgcgcatctacagaaggctgggccttgagcatggggaatgtggggagggagcaggacacaccagcactgcaaatggcttccttctcccagggcccaaagggatagaaaagaaggcaacatgaagttaaggccctgtgagcagtctagaaggtccttagcagcagcttctctgaaaacatgtgttctgcctctggagaaagggagcagaaaagtggtgcctgctggcttctcctcctcccctggcagcctgaagacaggtgcaaagtcaactagaagacaggcagcctcggggacgtggtcagcgtgcaagcattgatatcctcagtgtgggctgcccgatgcaaggatggctcggaagcgctccggttgatcttcggtagagagtgttggagcagctcaatggaagacaggatctggggaaaaagaggcctctcttcctttactttcttcacacagtcagctaccagcctcttcattgctttggggcagttcttatatagcttactaagatctggggaggcatatcctcggcccaccatgaagatgatctgatctcggttgttgatgtgagaataaggaagctcccccgtcatcagttcatacaatacgatgccataggagtagacatccgactggaaactgaatgggttgttatcctgcattcggatcacctctggggccatccagaggacagagccagtaggttgttcaacctgctgagaaccactccagcgtgactttactgttgccaaaccaaaatctccaattttcactgttaagccttcatggagaaatatattgttggatttcatgtctctatggatgatgttctttgcatgcaaatagtccattccctgagccgtctgccgggcaatgtcaattagctggaacatctgaaacttggtctcctggacatgcaggtgtttgtagaggctgctgccctcgcaccactgggtcacaattgccaggttgtcctttgtcatgtaccccatgaaaagcagaatgttcacatgccgtgttttgcgcagaacagccacctcattcctgaaggcctggaattgctctggggttgggtcgacaacctttaggatctttactgcaacatctccgtgccatttacccttataaacagttccaaaagagcctgacccaatccgagtggacagcatcacttcactggcttctatttcccaataatagcttgaatctctctgtccacgaggcctaattttgtttttctcctgggtcccagatactggtgcccgctctctttgtgctggcacgggggttttcggctgtgaccagcctgttgggctcagattgttggggctactggacagggctgaaggtgaggctgattcgctgtgacttcgaattgcatcctcaatcatcctgctgtccacaggcagggtggtgctgaccatgtggacattaggtgtggatgtcgacctctgcctctgggagagggaaccttcagatgagggactggaggtgttaaaggtgaaggcgtgaggtgtagaatatctgtgctgagaactaacaggcatcctggaaacagactctcgcatacgacgcatagtcaaagaaggtagtgctgggactccactatcaccaatagtggaatttggaaacaataagagttgtctgatgttactccagtccacacacatagtaggtactttggtgctacagtgctcatgaaatttgtagccacaagtctgacatcgaaatccattgagcaggaatttctgacagatgtcacagaaggcaagcttcaggaacgtcttccgagcaaagttgtgtgttgtgaggggaacatgatccaggaaatctacttgaagttcttctccaatcaaagacgcagcatcagtattccaatctaagcgtgcttttttacactgttctttgcttgttcggcaagaaaacacggatagtgttgcttgtcttagaaggatctgtgagtttgccatcatctgatgcccggcgctgatagccaaactgctgaactattgtaggagagatgcagctggagccatcaaacacggcatctttgaatccaaaaccattgctgatcgtcttccaagctccctgtatgtgctccattgatgcagcttaaacaattcttaaacctgcaaatcccaggactctggaaggctgagatgggaggactacttgagcccaggagtttaacaccagctctgggaaacataccaagaccccgtctgagggagccaggccgccccaacgtcctgtcgttcggcggcagcttctcgcccgctcctcctccccgcggcgggtgagggagcgggaggcggtcacattcggcgcgtccccagcccaggggacggagccccgagcagcccccgcatcgtagcaaacgcgctccgcgcctcagggcacgcgccccaaagcccggccagctgacccttttcggggcccaaaaaaggcagcagaaagccgttcccgcctcacaatcgttttcctcttactcccgccatctaagatggcggcccaagcgcccgcgatt

SEQ ID NO: 12448 - RNA, 3027 nt, Homo sapiens
  source 1..3027: mol_type = other RNA
ctgtaatataaatttaatttattttattaaaataacataattgagggaccatcagataactgtattttgtcaggtgcaataaaaacaaaattaaaacccaaatcatcaagaaaacctgtattcctggcttccttgtatacacatgatgtgactagagaaacaaggctgtttgtttgtttgtttgttagagaaacaaggctggccctgcggccccgccccataggggcagctcctggaagacaaaattcagcatgatggaagactgctccctgagagggctgagatgcggattggccgagtgccttgcctggaaaaccatcccaatgcactggacaccttagaagctgtgaaaggaggacgtgtcccctaagaaaagttccatagtaccaaagcaggctccttcgggcggccagagtctcggcagtcctgggctgtttggtgccttatgtgcaaaatgtctggcgctgcaccactctctgaagaaagtcccgcctgtgacatgcattcctccagaagctgatttccaaaatcccatgtgtctccacatcagggctggactgcctgctaccttacttcctctaaatactcatgtagccaacagctggggctgggcccctgctttttgtactaccatcaacatccacttgcgcatctacagaaggctgggccttgagcatggggaatgtggggagggagcaggacacaccagcactgcaaatggcttccttctcccagggcccaaagggatagaaaagaaggcaacatgaagttaaggccctgtgagcagtctagaaggtccttagcagcagcttctctgaaaacatgtgttctgcctctggagaaagggagcagaaaagtggtgcctgctggcttctcctcctcccctggcagcctgaagacaggtgcaaagtcaactagaagacaggcagcctcggggacgtggtcagcgtgcaagcattgatatcctcagtgtgggctgcccgatgcaaggatggctcggaagcgctccggttgatcttcggtagagagtgttggagcagctcaatggaagacaggatctggggaaaaagaggcctctcttcctttactttcttcacacagtcagctaccagcctcttcattgctttggggcagttcttatatagcttactaagatctggggaggcatatcctcggcccaccatgaagatgatctgatctcggttgttgatgtgagaataaggaagctcccccgtcatcagttcatacaatacgatgccataggagtagacatccgactggaaactgaatgggttgttatcctgcattcggatcacctctggggccatccagaggacagagccagtaggttgttcaacctgctgagaaccactccagcgtgactttactgttgccaaaccaaaatctccaattttcactgttaagccttcatggagaaatatattgttggatttcatgtctctatggatgatgttctttgcatgcaaatagtccattccctgagccgtctgccgggcaatgtcaattagctggaacatctgaaacttggtctcctggacatgcaggtgtttgtagaggctgctgccctcgcaccactgggtcacaattgccaggttgtcctttgtcatgtaccccatgaaaagcagaatgttcacatgccgtgttttgcgcagaacagccacctcattcctgaaggcctggaattgctctggggttgggtcgacaacctttaggatctttactgcaacatctccgtgccatttacccttataaacagttccaaaagagcctgacccaatccgagtggacagcatcacttcactggcttctatttcccaataatagcttgaatctctctgtccacgaggcctaattttgtttttctcctgggtcccagatactggtgcccgctctctttgtgctggcacgggggttttcggctgtgaccagcctgttgggctcagattgttggggctactggacagggctgaaggtgaggctgattcgctgtgacttcgaattgcatcctcaatcatcctgctgtccacaggcagggtggtgctgaccatgtggacattaggtgtggatgtcgacctctgcctctgggagagggaaccttcagatgagggactggaggtgttaaaggtgaaggcgtgaggtgtagaatatctgtgctgagaactaacaggcatcctggaaacagactctcgcatacgacgcatagtcaaagaaggtagtgctgggactccactatcaccaatagtggaatttggaaacaataagagttgtctgatgttactccagtccacacacatagtaggtactttggtgctacagtgctcatgaaatttgtagccacaagtctgacatcgaaatccattgagcaggaatttctgacagatgtcacagaaggcaagcttcaggaacgtcttccgagcaaagttgtgtgttgtgaggggaacatgatccaggaaatctacttgaagttcttctccaatcaaagacgcagcatcagtattccaatctaagcgtgcttttttacctttgtgttcgtggagaagtctgaacactgcacagcactctggttgcaggcccctcaccttgagtgctttcataaggcagtcatgcaagctcattccatttcgcacattgaccactgttctttgcttgttcggcaagaaaacacggatagtgttgcttgtcttagaaggatctgtgagtttgccatcatctgatgcccggcgctgatagccaaactgctgaactattgtaggagagatgcagctggagccatcaaacacggcatctttgaatccaaaaccattgctgatcgtcttccaagctccctgtatgtgctccattgatgcagcttaaacaattcttaaacccgattcctcacgtcgtctctaaaagggtgtcacttgactgaagtaccctgagaaagggtgcaagcccgggtcccacattcggcggcccaagagaaaaggaattggcccatccaagtgacaacagatatggggcagctct

SEQ ID NO: 12449 - RNA, 3192 nt, Homo sapiens
  source 1..3192: mol_type = other RNA
ctgtaatataaatttaatttattttattaaaataacataattgagggaccatcagataactgtattttgtcaggtgcaataaaaacaaaattaaaacccaaatcatcaagaaaacctgtattcctggcttccttgtatacacatgatgtgactagagaaacaaggctgtttgtttgtttgtttgttagagaaacaaggctggccctgcggccccgccccataggggcagctcctggaagacaaaattcagcatgatggaagactgctccctgagagggctgagatgcggattggccgagtgccttgcctggaaaaccatcccaatgcactggacaccttagaagctgtgaaaggaggacgtgtcccctaagaaaagttccatagtaccaaagcaggctccttcgggcggccagagtctcggcagtcctgggctgtttggtgccttatgtgcaaaatgtctggcgctgcaccactctctgaagaaagtcccgcctgtgacatgcattcctccagaagctgatttccaaaatcccatgtgtctccacatcagggctggactgcctgctaccttacttcctctaaatactcatgtagccaacagctggggctgggcccctgctttttgtactaccatcaacatccacttgcgcatctacagaaggctgggccttgagcatggggaatgtggggagggagcaggacacaccagcactgcaaatggcttccttctcccagggcccaaagggatagaaaagaaggcaacatgaagttaaggccctgtgagcagtctagaaggtccttagcagcagcttctctgaaaacatgtgttctgcctctggagaaagggagcagaaaagtggtgcctgctggcttctcctcctcccctggcagcctgaagacaggtgcaaagtcaactagaagacaggcagcctcggggacgtggtcagcgtgcaagcattgatatcctcagtgtgggctgcccgatgcaaggatggctcggaagcgctccggttgatcttcggtagagagtgttggagcagctcaatggaagacaggatctggggaaaaagaggcctctcttcctttactttcttcacacagtcagctaccagcctcttcattgctttggggcagttcttatatagcttactaagatctggggaggcatatcctcggcccaccatgaagatgatctgatctcggttgttgatgtgagaataaggaagctcccccgtcatcagttcatacaatacgatgccataggagtagacatccgactggaaactgaatgggttgttatcctgcattcggatcacctctggggccatccagaggacagagccagtaggttgttcaacctgctgagaaccactccagcgtgactttactgttgccaaaccaaaatctccaattttcactgttaagccttcatggagaaatatattgttggatttcatgtctctatggatgatgttctttgcatgcaaatagtccattccctgagccgtctgccgggcaatgtcaattagctggaacatctgaaacttggtctcctggacatgcaggtgtttgtagaggctgctgccctcgcaccactgggtcacaattgccaggttgtcctttgtcatgtaccccatgaaaagcagaatgttcacatgccgtgttttgcgcagaacagccacctcattcctgaaggcctggaattgctctggggttgggtcgacaacctttaggatctttactgcaacatctccgtgccatttacccttataaacagttccaaaagagcctgacccaatccgagtggacagcatcacttcactggcttctatttcccaataatagcttgaatctctctgtccacgaggcctaattttgtttttctcctgggtcccagatactggtgcccgctctctttgtgctggcacgggggttttcggctgtgaccagcctgttgggctcagattgttggggctactggacagggctgaaggtgaggctgattcgctgtgacttcgaattgcatcctcaatcatcctgctgtccacaggcagggtggtgctgaccatgtggacattaggtgtggatgtcgacctctgcctctgggagagggaaccttcagatgagggactggaggtgttaaaggtgaaggcgtgaggtgtagaatatctgtgctgagaactaacaggcatcctggaaacagactctcgcatacgacgcatagtcaaagaaggtagtgctgggactccactatcaccaatagtggaatttggaaacaataagagttgtctgatgttactccagtccacacacatagtaggtactttggtgctacagtgctcatgaaatttgtagccacaagtctgacatcgaaatccattgagcaggaatttctgacagatgtcacagaaggcaagcttcaggaacgtcttccgagcaaagttgtgtgttgtgaggggaacatgatccaggaaatctacttgaagttcttctccaatcaaagacgcagcatcagtattccaatctaagcgtgcttttttacctttgtgttcgtggagaagtctgaacactgcacagcactctggttgcaggcccctcaccttgagtgctttcataaggcagtcatgcaagctcattccatttcgcacattgaccactgttctttgcttgttcggcaagaaaacacggatagtgttgcttgtcttagaaggatctgtgagtttgccatcatctgatgcccggcgctgatagccaaactgctgaactattgtaggagagatgcagctggagccatcaaacacggcatctttgaatccaaaaccattgctgatcgtcttccaagctccctgtatgtgctccattgatgcagcttaaacaattcttaaacctgagggagccaggccgccccaacgtcctgtcgttcggcggcagcttctcgcccgctcctcctccccgcggcgggtgagggagcgggaggcggtcacattcggcgcgtccccagcccaggggacggagccccgagcagcccccgcatcgtagcaaacgcgctccgcgcctcagggcacgcgccccaaagcccggccagctgacccttttcggggcccaaaaaaggcagcagaaagccgttcccgcctcacaatcgttttcctcttactcccgccatctaagatggcggcccaagcgcccgcgatt

SEQ ID NO: 12450 - RNA, 3285 nt, Homo sapiens
  source 1..3285: mol_type = other RNA
ctgtaatataaatttaatttattttattaaaataacataattgagggaccatcagataactgtattttgtcaggtgcaataaaaacaaaattaaaacccaaatcatcaagaaaacctgtattcctggcttccttgtatacacatgatgtgactagagaaacaaggctgtttgtttgtttgtttgttagagaaacaaggctggccctgcggccccgccccataggggcagctcctggaagacaaaattcagcatgatggaagactgctccctgagagggctgagatgcggattggccgagtgccttgcctggaaaaccatcccaatgcactggacaccttagaagctgtgaaaggaggacgtgtcccctaagaaaagttccatagtaccaaagcaggctccttcgggcggccagagtctcggcagtcctgggctgtttggtgccttatgtgcaaaatgtctggcgctgcaccactctctgaagaaagtcccgcctgtgacatgcattcctccagaagctgatttccaaaatcccatgtgtctccacatcagggctggactgcctgctaccttacttcctctaaatactcatgtagccaacagctggggctgggcccctgctttttgtactaccatcaacatccacttgcgcatctacagaaggctgggccttgagcatggggaatgtggggagggagcaggacacaccagcactgcaaatggcttccttctcccagggcccaaagggatagaaaagaaggcaacatgaagttaaggccctgtgagcagtctagaaggtccttagcagcagcttctctgaaaacatgtgttctgcctctggagaaagggagcagaaaagtggtgcctgctggcttctcctcctcccctggcagcctgaagacaggtgcaaagtcaactagaagacaggcagcctcggggacgtggtcagcgtgcaagcattgatatcctcagtgtgggctgcccgatgcaaggatggctcggaagcgctccggttgatcttcggtagagagtgttggagcagctcaatggaagacaggatctggggaaaaagaggcctctcttcctttactttcttcacacagtcagctaccagcctcttcattgctttggggcagttcttatatagcttactaagatctggggaggcatatcctcggcccaccatgaagatgatctgatctcggttgttgatgtgagaataaggaagctcccccgtcatcagttcatacaatacgatgccataggagtagacatccgactggaaactgaatgggttgttatcctgcattcggatcacctctggggccatccagaggacagagccagtaggttgttcaacctgctgagaaccactccagcgtgactttactgttgccaaaccaaaatctccaattttcactgttaagccttcatggagaaatatattgttggatttcatgtctctatggatgatgttctttgcatgcaaatagtccattccctgagccgtctgccgggcaatgtcaattagctggaacatctgaaacttggtctcctggacatgcaggtgtttgtagaggctgctgccctcgcaccactgggtcacaattgccaggttgtcctttgtcatgtaccccatgaaaagcagaatgttcacatgccgtgttttgcgcagaacagccacctcattcctgaaggcctggaattgctctggggttgggtcgacaacctttaggatctttactgcaacatctccgtgccatttacccttataaacagttccaaaagagcctgacccaatccgagtggacagcatcacttcactggcttctatttcccaataatagcttgaatctctctgtccacgaggcctaattttgtttttctcctgggtcccagatactggtgcccgctctctttgtgctggcacgggggttttcggctgtgaccagcctgttgggctcagattgttggggctactggacagggctgaaggtgaggctgattcgctgtgacttcgaattgcatcctcaatcatcctgctgtccacaggcagggtggtgctgaccatgtggacattaggtgtggatgtcgacctctgcctctgggagagggaaccttcagatgagggactggaggtgttaaaggtgaaggcgtgaggtgtagaatatctgtgctgagaactaacaggcatcctggaaacagactctcgcatacgacgcatagtcaaagaaggtagtgctgggactccactatcaccaatagtggaatttggaaacaataagagttgtctgatgttactccagtccacacacatagtaggtactttggtgctacagtgctcatgaaatttgtagccacaagtctgacatcgaaatccattgagcaggaatttctgacagatgtcacagaaggcaagcttcaggaacgtcttccgagcaaagttgtgtgttgtgaggggaacatgatccaggaaatctacttgaagttcttctccaatcaaagacgcagcatcagtattccaatctaagcgtgcttttttacctttgtgttcgtggagaagtctgaacactgcacagcactctggttgcaggcccctcaccttgagtgctttcataaggcagtcatgcaagctcattccatttcgcacattgaccactgttctttgcttgttcggcaagaaaacacggatagtgttgcttgtcttagaaggatctgtgagtttgccatcatctgatgcccggcgctgatagccaaactgctgaactattgtaggagagatgcagctggagccatcaaacacggcatctttgaatccaaaaccattgctgatcgtcttccaagctccctgtatgtgctccattgatgcagcttaaacaattcttaaacctgcaaatcccaggactctggaaggctgagatgggaggactacttgagcccaggagtttaacaccagctctgggaaacataccaagaccccgtctgagggagccaggccgccccaacgtcctgtcgttcggcggcagcttctcgcccgctcctcctccccgcggcgggtgagggagcgggaggcggtcacattcggcgcgtccccagcccaggggacggagccccgagcagcccccgcatcgtagcaaacgcgctccgcgcctcagggcacgcgccccaaagcccggccagctgacccttttcggggcccaaaaaaggcagcagaaagccgttcccgcctcacaatcgttttcctcttactcccgccatctaagatggcggcccaagcgcccgcgatt

SEQ ID NO: 12451 - RNA, 3139 nt, Homo sapiens
  source 1..3139: mol_type = other RNA
ctgtaatataaatttaatttattttattaaaataacataattgagggaccatcagataactgtattttgtcaggtgcaataaaaacaaaattaaaacccaaatcatcaagaaaacctgtattcctggcttccttgtatacacatgatgtgactagagaaacaaggctgtttgtttgtttgtttgttagagaaacaaggctggccctgcggccccgccccataggggcagctcctggaagacaaaattcagcatgatggaagactgctccctgagagggctgagatgcggattggccgagtgccttgcctggaaaaccatcccaatgcactggacaccttagaagctgtgaaaggaggacgtgtcccctaagaaaagttccatagtaccaaagcaggctccttcgggcggccagagtctcggcagtcctgggctgtttggtgccttatgtgcaaaatgtctggcgctgcaccactctctgaagaaagtcccgcctgtgacatgcattcctccagaagctgatttccaaaatcccatgtgtctccacatcagggctggactgcctgctaccttacttcctctaaatactcatgtagccaacagctggggctgggcccctgctttttgtactaccatcaacatccacttgcgcatctacagaaggctgggccttgagcatggggaatgtggggagggagcaggacacaccagcactgcaaatggcttccttctcccagggcccaaagggatagaaaagaaggcaacatgaagttaaggccctgtgagcagtctagaaggtccttagcagcagcttctctgaaaacatgtgttctgcctctggagaaagggagcagaaaagtggtgcctgctggcttctcctcctcccctggcagcctgaagacaggtgcaaagtcaactagaagacaggcagcctcggggacgtggtcagcgtgcaagcattgatatcctcagtgtgggctgcccgatgcaaggatggctcggaagcgctccggttgatcttcggtagagagtgttggagcagctcaatggaagacaggatctggggaaaaagaggcctctcttcctttactttcttcacacagtcagctaccagcctcttcattgctttggggcagttcttatatagcttactaagatctggggaggcatatcctcggcccaccatgaagatgatctgatctcggttgttgatgtgagaataaggaagctcccccgtcatcagttcatacaatacgatgccataggagtagacatccgactggaaactgaatgggttgttatcctgcattcggatcacctctggggccatccagaggacagagccagtaggttgttcaacctgctgagaaccactccagcgtgactttactgttgccaaaccaaaatctccaattttcactgttaagccttcatggagaaatatattgttggatttcatgtctctatggatgatgttctttgcatgcaaatagtccattccctgagccgtctgccgggcaatgtcaattagctggaacatctgaaacttggtctcctggacatgcaggtgtttgtagaggctgctgccctcgcaccactgggtcacaattgccaggttgtcctttgtcatgtaccccatgaaaagcagaatgttcacatgccgtgttttgcgcagaacagccacctcattcctgaaggcctggaattgctctggggttgggtcgacaacctttaggatctttactgcaacatctccgtgccatttacccttataaacagttccaaaagagcctgacccaatccgagtggacagcatcacttcactggcttctatttcccaataatagcttgaatctctctgtccacgaggcctaattttgtttttctcctgggtcccagatactggtgcccgctctctttgtgctggcacgggggttttcggctgtgaccagcctgttgggctcagattgttggggctactggacagggctgaaggtgaggctgattcgctgtgacttcgaattgcatctcttcccctcaaacaaaatcgtctggaccacgccctgggagaagcactcaggttgttattctcaatcatcctgctgtccacaggcagggtggtgctgaccatgtggacattaggtgtggatgtcgacctctgcctctgggagagggaaccttcagatgagggactggaggtgttaaaggtgaaggcgtgaggtgtagaatatctgtgctgagaactaacaggcatcctggaaacagactctcgcatacgacgcatagtcaaagaaggtagtgctgggactccactatcaccaatagtggaatttggaaacaataagagttgtctgatgttactccagtccacacacatagtaggtactttggtgctacagtgctcatgaaatttgtagccacaagtctgacatcgaaatccattgagcaggaatttctgacagatgtcacagaaggcaagcttcaggaacgtcttccgagcaaagttgtgtgttgtgaggggaacatgatccaggaaatctacttgaagttcttctccaatcaaagacgcagcatcagtattccaatctaagcgtgcttttttacactgttctttgcttgttcggcaagaaaacacggatagtgttgcttgtcttagaaggatctgtgagtttgccatcatctgatgcccggcgctgatagccaaactgctgaactattgtaggagagatgcagctggagccatcaaacacggcatctttgaatccaaaaccattgctgatcgtcttccaagctccctgtatgtgctccattgatgcagcttaaacaattcttaaacctgagggagccaggccgccccaacgtcctgtcgttcggcggcagcttctcgcccgctcctcctccccgcggcgggtgagggagcgggaggcggtcacattcggcgcgtccccagcccaggggacggagccccgagcagcccccgcatcgtagcaaacgcgctccgcgcctcagggcacgcgccccaaagcccggccagctgacccttttcggggcccaaaaaaggcagcagaaagccgttcccgcctcacaatcgttttcctcttactcccgccatctaagatggcggcccaagcgcccgcgatt

SEQ ID NO: 12452 - RNA, 3252 nt, Homo sapiens
  source 1..3252: mol_type = other RNA
ctgtaatataaatttaatttattttattaaaataacataattgagggaccatcagataactgtattttgtcaggtgcaataaaaacaaaattaaaacccaaatcatcaagaaaacctgtattcctggcttccttgtatacacatgatgtgactagagaaacaaggctgtttgtttgtttgtttgttagagaaacaaggctggccctgcggccccgccccataggggcagctcctggaagacaaaattcagcatgatggaagactgctccctgagagggctgagatgcggattggccgagtgccttgcctggaaaaccatcccaatgcactggacaccttagaagctgtgaaaggaggacgtgtcccctaagaaaagttccatagtaccaaagcaggctccttcgggcggccagagtctcggcagtcctgggctgtttggtgccttatgtgcaaaatgtctggcgctgcaccactctctgaagaaagtcccgcctgtgacatgcattcctccagaagctgatttccaaaatcccatgtgtctccacatcagggctggactgcctgctaccttacttcctctaaatactcatgtagccaacagctggggctgggcccctgctttttgtactaccatcaacatccacttgcgcatctacagaaggctgggccttgagcatggggaatgtggggagggagcaggacacaccagcactgcaaatggcttccttctcccagggcccaaagggatagaaaagaaggcaacatgaagttaaggccctgtgagcagtctagaaggtccttagcagcagcttctctgaaaacatgtgttctgcctctggagaaagggagcagaaaagtggtgcctgctggcttctcctcctcccctggcagcctgaagacaggtgcaaagtcaactagaagacaggcagcctcggggacgtggtcagcgtgcaagcattgatatcctcagtgtgggctgcccgatgcaaggatggctcggaagcgctccggttgatcttcggtagagagtgttggagcagctcaatggaagacaggatctggggaaaaagaggcctctcttcctttactttcttcacacagtcagctaccagcctcttcattgctttggggcagttcttatatagcttactaagatctggggaggcatatcctcggcccaccatgaagatgatctgatctcggttgttgatgtgagaataaggaagctcccccgtcatcagttcatacaatacgatgccataggagtagacatccgactggaaactgaatgggttgttatcctgcattcggatcacctctggggccatccagaggacagagccagtaggttgttcaacctgctgagaaccactccagcgtgactttactgttgccaaaccaaaatctccaattttcactgttaagccttcatggagaaatatattgttggatttcatgtctctatggatgatgttctttgcatgcaaatagtccattccctgagccgtctgccgggcaatgtcaattagctggaacatctgaaacttggtctcctggacatgcaggtgtttgtagaggctgctgccctcgcaccactgggtcacaattgccaggttgtcctttgtcatgtaccccatgaaaagcagaatgttcacatgccgtgttttgcgcagaacagccacctcattcctgaaggcctggaattgctctggggttgggtcgacaacctttaggatctttactgcaacatctccgtgccatttacccttataaacagttccaaaagagcctgacccaatccgagtggacagcatcacttcactggcttctatttcccaataatagcttgaatctctctgtccacgaggcctaattttgtttttctcctgggtcccagatactggtgcccgctctctttgtgctggcacgggggttttcggctgtgaccagcctgttgggctcagattgttggggctactggacagggctgaaggtgaggctgattcgctgtgacttcgaattgcatctcttcccctcaaacaaaatcgtctggaccacgccctgggagaagcactcaggttgttattctcaatcatcctgctgtccacaggcagggtggtgctgaccatgtggacattaggtgtggatgtcgacctctgcctctgggagagggaaccttcagatgagggactggaggtgttaaaggtgaaggcgtgaggtgtagaatatctgtgctgagaactaacaggcatcctggaaacagactctcgcatacgacgcatagtcaaagaaggtagtgctgggactccactatcaccaatagtggaatttggaaacaataagagttgtctgatgttactccagtccacacacatagtaggtactttggtgctacagtgctcatgaaatttgtagccacaagtctgacatcgaaatccattgagcaggaatttctgacagatgtcacagaaggcaagcttcaggaacgtcttccgagcaaagttgtgtgttgtgaggggaacatgatccaggaaatctacttgaagttcttctccaatcaaagacgcagcatcagtattccaatctaagcgtgcttttttacctttgtgttcgtggagaagtctgaacactgcacagcactctggttgcaggcccctcaccttgagtgctttcataaggcagtcatgcaagctcattccatttcgcacattgaccactgttctttgcttgttcggcaagaaaacacggatagtgttgcttgtcttagaaggatctgtgagtttgccatcatctgatgcccggcgctgatagccaaactgctgaactattgtaggagagatgcagctggagccatcaaacacggcatctttgaatccaaaaccattgctgatcgtcttccaagctccctgtatgtgctccattgatgcagcttaaacaattcttaaacctgagggagccaggccgccccaacgtcctgtcgttcggcggcagcttctcgcccgctcctcctccccgcggcgggtgagggagcgggaggcggtcacattcggcgcgtccccagcccaggggacggagccccgagcagcccccgcatcgtagcaaacgcgctccgcgcctcagggcacgcgccccaaagcccggccagctgacccttttcggggcccaaaaaaggcagcagaaagccgttcccgcctcacaatcgttttcctcttactcccgccatctaagatggcggcccaagcgcccgcgatt

SEQ ID NO: 12453 - RNA, 3251 nt, Homo sapiens
  source 1..3251: mol_type = other RNA
ctgtaatataaatttaatttattttattaaaataacataattgagggaccatcagataactgtattttgtcaggtgcaataaaaacaaaattaaaacccaaatcatcaagaaaacctgtattcctggcttccttgtatacacatgatgtgactagagaaacaaggctgtttgtttgtttgtttgttagagaaacaaggctggccctgcggccccgccccataggggcagctcctggaagacaaaattcagcatgatggaagactgctccctgagagggctgagatgcggattggccgagtgccttgcctggaaaaccatcccaatgcactggacaccttagaagctgtgaaaggaggacgtgtcccctaagaaaagttccatagtaccaaagcaggctccttcgggcggccagagtctcggcagtcctgggctgtttggtgccttatgtgcaaaatgtctggcgctgcaccactctctgaagaaagtcccgcctgtgacatgcattcctccagaagctgatttccaaaatcccatgtgtctccacatcagggctggactgcctgctaccttacttcctctaaatactcatgtagccaacagctggggctgggcccctgctttttgtactaccatcaacatccacttgcgcatctacagaaggctgggccttgagcatggggaatgtggggagggagcaggacacaccagcactgcaaatggcttccttctcccagggcccaaagggatagaaaagaaggcaacatgaagttaaggccctgtgagcagtctagaaggtccttagcagcagcttctctgaaaacatgtgttctgcctctggagaaagggagcagaaaagtggtgcctgctggcttctcctcctcccctggcagcctgaagacaggtgcaaagtcaactagaagacaggcagcctcggggacgtggtcagcgtgcaagcattgatatcctcagtgtgggctgcccgatgcaaggatggctcggaagcgctccggttgatcttcggtagagagtgttggagcagctcaatggaagacaggatctggggaaaaagaggcctctcttcctttactttcttcacacagtcagctaccagcctcttcattgctttggggcagttcttatatagcttactaagatctggggaggcatatcctcggcccaccatgaagatgatctgatctcggttgttgatgtgagaataaggaagctcccccgtcatcagttcatacaatacgatgccataggagtagacatccgactggaaactgaatgggttgttatcctgcattcggatcacctctggggccatccagaggacagagccagtaggttgttcaacctgctgagaaccactccagcgtgactttactgttgccaaaccaaaatctccaattttcactgttaagccttcatggagaaatatattgttggatttcatgtctctatggatgatgttctttgcatgcaaatagtccattccctgagccgtctgccgggcaatgtcaattagctggaacatctgaaacttggtctcctggacatgcaggtgtttgtagaggctgctgccctcgcaccactgggtcacaattgccaggttgtcctttgtcatgtaccccatgaaaagcagaatgttcacatgccgtgttttgcgcagaacagccacctcattcctgaaggcctggaattgctctggggttgggtcgacaacctttaggatctttactgcaacatctcctgcaaaattagttggcagtcagtgcaatcagttgaatgatctcagtctttcaaataaccgtgccatttacccttataaacagttccaaaagagcctgacccaatccgagtggacagcatcacttcactggcttctatttcccaataatagcttgaatctctctgtccacgaggcctaattttgtttttctcctgggtcccagatactggtgcccgctctctttgtgctggcacgggggttttcggctgtgaccagcctgttgggctcagattgttggggctactggacagggctgaaggtgaggctgattcgctgtgacttcgaattgcatcctcaatcatcctgctgtccacaggcagggtggtgctgaccatgtggacattaggtgtggatgtcgacctctgcctctgggagagggaaccttcagatgagggactggaggtgttaaaggtgaaggcgtgaggtgtagaatatctgtgctgagaactaacaggcatcctggaaacagactctcgcatacgacgcatagtcaaagaaggtagtgctgggactccactatcaccaatagtggaatttggaaacaataagagttgtctgatgttactccagtccacacacatagtaggtactttggtgctacagtgctcatgaaatttgtagccacaagtctgacatcgaaatccattgagcaggaatttctgacagatgtcacagaaggcaagcttcaggaacgtcttccgagcaaagttgtgtgttgtgaggggaacatgatccaggaaatctacttgaagttcttctccaatcaaagacgcagcatcagtattccaatctaagcgtgcttttttacctttgtgttcgtggagaagtctgaacactgcacagcactctggttgcaggcccctcaccttgagtgctttcataaggcagtcatgcaagctcattccatttcgcacattgaccactgttctttgcttgttcggcaagaaaacacggatagtgttgcttgtcttagaaggatctgtgagtttgccatcatctgatgcccggcgctgatagccaaactgctgaactattgtaggagagatgcagctggagccatcaaacacggcatctttgaatccaaaaccattgctgatcgtcttccaagctccctgtatgtgctccattgatgcagcttaaacaattcttaaacctgagggagccaggccgccccaacgtcctgtcgttcggcggcagcttctcgcccgctcctcctccccgcggcgggtgagggagcgggaggcggtcacattcggcgcgtccccagcccaggggacggagccccgagcagcccccgcatcgtagcaaacgcgctccgcgcctcagggcacgcgccccaaagcccggccagctgacccttttcggggcccaaaaaaggcagcagaaagccgttcccgcctcacaatcgttttcctcttactcccgccatctaagatggcggcccaagcgcccgcgatt

SEQ ID NO: 12454 - RNA, 3305 nt, Homo sapiens
  source 1..3305: mol_type = other RNA
ctgtaatataaatttaatttattttattaaaataacataattgagggaccatcagataactgtattttgtcaggtgcaataaaaacaaaattaaaacccaaatcatcaagaaaacctgtattcctggcttccttgtatacacatgatgtgactagagaaacaaggctgtttgtttgtttgtttgttagagaaacaaggctggccctgcggccccgccccataggggcagctcctggaagacaaaattcagcatgatggaagactgctccctgagagggctgagatgcggattggccgagtgccttgcctggaaaaccatcccaatgcactggacaccttagaagctgtgaaaggaggacgtgtcccctaagaaaagttccatagtaccaaagcaggctccttcgggcggccagagtctcggcagtcctgggctgtttggtgccttatgtgcaaaatgtctggcgctgcaccactctctgaagaaagtcccgcctgtgacatgcattcctccagaagctgatttccaaaatcccatgtgtctccacatcagggctggactgcctgctaccttacttcctctaaatactcatgtagccaacagctggggctgggcccctgctttttgtactaccatcaacatccacttgcgcatctacagaaggctgggccttgagcatggggaatgtggggagggagcaggacacaccagcactgcaaatggcttccttctcccagggcccaaagggatagaaaagaaggcaacatgaagttaaggccctgtgagcagtctagaaggtccttagcagcagcttctctgaaaacatgtgttctgcctctggagaaagggagcagaaaagtggtgcctgctggcttctcctcctcccctggcagcctgaagacaggtgcaaagtcaactagaagacaggcagcctcggggacgtggtcagcgtgcaagcattgatatcctcagtgtgggctgcccgatgcaaggatggctcggaagcgctccggttgatcttcggtagagagtgttggagcagctcaatggaagacaggatctggggaaaaagaggcctctcttcctttactttcttcacacagtcagctaccagcctcttcattgctttggggcagttcttatatagcttactaagatctggggaggcatatcctcggcccaccatgaagatgatctgatctcggttgttgatgtgagaataaggaagctcccccgtcatcagttcatacaatacgatgccataggagtagacatccgactggaaactgaatgggttgttatcctgcattcggatcacctctggggccatccagaggacagagccagtaggttgttcaacctgctgagaaccactccagcgtgactttactgttgccaaaccaaaatctccaattttcactgttaagccttcatggagaaatatattgttggatttcatgtctctatggatgatgttctttgcatgcaaatagtccattccctgagccgtctgccgggcaatgtcaattagctggaacatctgaaacttggtctcctggacatgcaggtgtttgtagaggctgctgccctcgcaccactgggtcacaattgccaggttgtcctttgtcatgtaccccatgaaaagcagaatgttcacatgccgtgttttgcgcagaacagccacctcattcctgaaggcctggaattgctctggggttgggtcgacaacctttaggatctttactgcaacatctcctttcttccaagtgacaaagtgtttccattaaaatcagaacattaatattccacatagattcaagaattaagtcaatgccttccctgtttgatagggacacccacagctaatccgtgccatttacccttataaacagttccaaaagagcctgacccaatccgagtggacagcatcacttcactggcttctatttcccaataatagcttgaatctctctgtccacgaggcctaattttgtttttctcctgggtcccagatactggtgcccgctctctttgtgctggcacgggggttttcggctgtgaccagcctgttgggctcagattgttggggctactggacagggctgaaggtgaggctgattcgctgtgacttcgaattgcatcctcaatcatcctgctgtccacaggcagggtggtgctgaccatgtggacattaggtgtggatgtcgacctctgcctctgggagagggaaccttcagatgagggactggaggtgttaaaggtgaaggcgtgaggtgtagaatatctgtgctgagaactaacaggcatcctggaaacagactctcgcatacgacgcatagtcaaagaaggtagtgctgggactccactatcaccaatagtggaatttggaaacaataagagttgtctgatgttactccagtccacacacatagtaggtactttggtgctacagtgctcatgaaatttgtagccacaagtctgacatcgaaatccattgagcaggaatttctgacagatgtcacagaaggcaagcttcaggaacgtcttccgagcaaagttgtgtgttgtgaggggaacatgatccaggaaatctacttgaagttcttctccaatcaaagacgcagcatcagtattccaatctaagcgtgcttttttacctttgtgttcgtggagaagtctgaacactgcacagcactctggttgcaggcccctcaccttgagtgctttcataaggcagtcatgcaagctcattccatttcgcacattgaccactgttctttgcttgttcggcaagaaaacacggatagtgttgcttgtcttagaaggatctgtgagtttgccatcatctgatgcccggcgctgatagccaaactgctgaactattgtaggagagatgcagctggagccatcaaacacggcatctttgaatccaaaaccattgctgatcgtcttccaagctccctgtatgtgctccattgatgcagcttaaacaattcttaaacctgagggagccaggccgccccaacgtcctgtcgttcggcggcagcttctcgcccgctcctcctccccgcggcgggtgagggagcgggaggcggtcacattcggcgcgtccccagcccaggggacggagccccgagcagcccccgcatcgtagcaaacgcgctccgcgcctcagggcacgcgccccaaagcccggccagctgacccttttcggggcccaaaaaaggcagcagaaagccgttcccgcctcacaatcgttttcctcttactcccgccatctaagatggcggcccaagcgcccgcgatt

SEQ ID NO: 12455 - RNA, 619 nt, Homo sapiens
  source 1..619: mol_type = other RNA
ctgtacagcctcctagctttccccaggctgcgccctgcacgggacggggcccggcggggacccccagccccactcagggacccttagccccactgggctgccccagggaccctgggaggaagagccgggctcttttctgtccttgtccctgcatcccctccttcccctgaaatctgttttccttccctgtctgtctccatctctgctgtgtctctgtggcttctgtgtctctttcacagtggatcctctgactccctcttattctggctttctaggtctctgcccctcccgatatctctctgtgtctctatttctgtcgtttttggtctttctgtctctggctctcagaatgtctctgtgcctatctccatctctgacccccaccccagggtctaccgggccaccgcacaccatgttgccagtctctaggtccctgagaccctttaacctgtgaggacatccagggtcacaggtgaggttcttgggagcctggcgtctggcccaaccacacacctggggaattgctggcctgacttctgacccctgactcctcatacccttcctccagagcatgacatttgaccaccaactgaaacctgacctctgaccccagaccact

SEQ ID NO: 12456 - RNA, 1236 nt, Homo sapiens
  source 1..1236: mol_type = other RNA
ctgtgggctcagctctgggtgggaaggcattgagaatggacattgtcaactgggccaaaggaggccaaggagaagtgctgggggcatgggaactgaaaaagagaggaggctcagcacgtctttgagctgggagagggacagcagcagcggcttttccaaaggaagcaacagctgagagaggtctcagagagttgttctcagcccagtggagggtgttcaggcagagggaacagcgtgtgcaaaagcccagaggctgggaaagaagcagaaagaggactgtggggctggagcatggtgggcaaggggaggaaggtgtggtgggcagacagattgcctgggacccagccgtgcaggggcagaggagatacgggatccttgcaggcccccagccggggctcaggcacagagacagtgcaggtgggcaaagggaggagacgtggagaaatattttggaggcatgccctgatgaatgagcccaggatgcacccttagtgtcagtgtggagctccttccttgactgtgtgatgagctgaactcgggggtattttctggacattgaggtgctacaccaagagcccaggacaggctaagtgagcactagcagctcctggcccacctcaaaagcaggagagacaggggagactgaggaggccggggcggaaggggaagccaggaaggtaggagaggccagggaagcagaggaggcccgggaggcaatggaggcaggagaggctggggaggttatgtcctttccatgattctgccctcgatcctaggcccctgaactccctgagcttccccaccccaagcgctggaaccatgttgcacaatggtctccccactaagctcctgatggcagcccctaccctgctgtgctccctgtttcaaccctaacagctctcacagtgggcagcacatagtaggtgctgaggaaacactggtgggagagcacgtgggtctgctcagcaccttcctctctcctccagctctcccctgtcacgaaataattctgataacgacacatggactttgagaccctcttctattactttccatatgctaatccatctatacctcacagcagccctgggggtgggtgcaatgaggatgcccattttatagaggaggagactgaggtataaagagggtaagtgacatacgcacactacaggggctggggtcaagtgatcagagcactcaatccccaaaggcaaggtggatgcagttaccataaaa

SEQ ID NO: 12457 - RNA, 30 nt, Homo sapiens
  source 1..30: mol_type = other RNA
cttagcaggttgtattatcattgtccgtgt

SEQ ID NO: 12458 - RNA, 8747 nt, Homo sapiens
  source 1..8747: mol_type = other RNA
cttagcaggttgtattatcatttataatcaaccaggacttaaaaaattcacacacacacgagaagtaccccaagagattattaaaaaggaaattttcaggtggttttcatagagattccaattctgtgtatcttggatggggtctgggaatatgtttttaacaaaaattaggttaattctgatacaggtcgtccatacactatttttttcagaaattgataagttaaatcagggcttattttttcctaaggataatcacagtcaaacaaataatattgttcttttaagttggtagacactctagcattctgagtgcatttttatttattatatagtacatccaaaaatcatttttctaaactttggaaatattttcagcaaatgaatgcataaaatgagatactgtgtgttttactagttttcctggtatttgaggacaaaagtcgtagttatcccttctcctgttttctccacctctctaagtatagaagtggggggaggagtaggaggagtaggaggaggaggaggaagaggagggaagaggaggaggaggaggttgtcagagcattaagaagcaagagagtagaatgttacagggggtgctacaatcacccagataatagcaggaagtagggtggagaggcatgttataaatcagaaagaagaatcttcggagaaggctgggaagcaggtgatttttagagttgaggaagcgggcacacctgcaaaacagaagagatttttggatgaaggttatagaacagcagtctagaggcagcagtgggagccagtttctgtccctagatactagagctccaagagcctgggagaatgactcatctctgcagaaagaggtgggaaggaatgtcgttgccaggggacccagtggctacgacagaaagatgccaaaaaaaggtactggatttctcccaacatctttgtcattggtcaaaagagacttccccaaacaatgaaatactgtttggagatcccactggatataggaccaaagggcaagcagcactgtgagcaaggatatggaaacccggaatgggataacctcactacctgcacaacacaaatagggtcaaggataatgttcaggagttgatttcctttggaagcttggcgggggaaggaatacactcttcagagcaggacttgaaaagtgagatgcttaggggccaggcaagtaaggtgaatgagtgatggtggattagtgaagagtgtgaacaactagagatctccaacctcatctaaagggactgaccttgcctctgtccaactattttcaggtgggcatatagaatgtagggtaacaaatcccctgtcattaatgaggcccaatgttggcagctaattcagatgttaaataaaatgcactgtcagccaaaccaaacatatctgtagccagatctaccccgtgggctgccaatgtatggtctcagctttggagccagagagactgttattaaacctctttgatactcagttttctcattcatgaaatgataggtggaaaaatactcgactttgatttttttgaaagctacttttggaaacggttagacttactcttcatgtcattaaatgaatgtatgcaaagtatttttcccgtgtctgctactgagtagatcctcagtaaatggctcttatgttgaccagaatcatgcatttttctcaaaattttcttccccaaacaatcaagcaactgctatttcttagaaatgtaaaagatttctgtgtctgcaactatccttcaggtcaagggatgactattagtgtagaaaaggtgtgtggctcagctcccttccctcagctgccctgctctagcaccttcctttcagatcctctggtcctatagatgcctgaaggtcacaggcagaaatatacgaattctacactaaaagaagttgtacaggaacctttaaacaacagcatcaaaagcatctgttaaagtaacgctttccactgagtgccttgctagacatggtacaaagtgcattcaacagacacagttcctttcctcttggaagacctaagacattccaatgacaacaacagatattttatattcataaaaagtgagataaatagcacatgaacaaataaattaacgaacctccctgacaaaaaaaatcgaggaaaggaatgcctgcatttattggtaagagaataatctgatgcatgttacaccaggggaaaactctgctgtctttttctgcctatcagggagctcataaagagatgagattttgaaattgaataatctcaagagattccttggtgagttaacaagaaatgaatgtccagatatatagagaggggagcattccaaatatagtgtgagacttgaggagaggtttagggatggaaaaagatgactgcttaaatggatttaaatacttttgcctggaagcatatgatcctggtgaaaaactaagatgtgactgactaggaaattctgagaatgaaatgatatgaggcaatgttctgttgaactccccagacctggccttcctcaggtaatgatcacaggcctgggaaatgtctgccatcttctagcaagagcttatttattttcacctggtttcatggtgttttttcagtcggtttaagtcagcttgctcctctattcttttctgcagtcttcccgtgtaggctcagggtaatctgactacaaactagtactagggaaggagactcaggaagaaggggataatgcacagttgctctgtttctagcaggagtggttctcactgtgtgtgactagcttgctgaaccgtgaccatctgcagtggctgtcaggggcctatgtgtggaaagttcgcctgaactttcttcctcttagattctgcttatccttgactggtcttgtagctgtctggaatttcttgtcaaagaaatgatattttgttttcacaaggctaaatttgttccagggactattttttcttcttaaaaacattgtttccatgattaactaaggattacaaaaaagttgtggggaggaaacctaatttcttccaaagtctttgaacctgtcagtttaactcagcaggaataaagaaataagctgatttgaaatgtgataactaactagctaaatacacacacacacacacacacacacacacacacacacacagacacccatatttgtatggaaaaaatttcaggattccaatatattgtttttgcctctacctatcctgaatagaggtaacggaaagcaaaagtaaatattggtttgtaatattctaagcaaagagtttggtagtggtatttgctgcttggcttcatcctggcttctgacctacttatcatctctgtctccttaggcaagttactcagctatagtctgctttactttcctttatgatagatggaaagggagagggctacataatattacctatgttagactggctatggagattaaattaatgcatgtaaactacttgaagagtgcctgacacccagtaagtattgaataaatgttagctaggatcatgcatacgattactgtataatgatcatgattgagattgagaaggtatgagcctaaatgtaggactaaattgaattagccttggcctaaggttctcaggtagttgagctataattaaacgcctttggccaatcctttttcaagtatcagagcatcttgggagggttagccctgggcaaaacatctgcttcaccacgccccatgaaggcctagaggctgggatgccctgagaggccacatgagaatgcacaggagggagacgtttactgtagtcctagcctaatcccaagttctattaattcagcaagtgattttttcaaagggcactctaatattcaaaattctctgcatcttcttatatataccttctgctaaatactatacattttaggagataagaataataatacatcaataaaatgtaaaagtatttttcctctttctaattaaaaatgacatacaagtagttcttgaattagaactactaattccctaatgataataatattattattttctgttacagaatgttttatagacatctagcaagtggcatcacatttccattgaattaatggatatttccaaatgtttgagaaaatccgaaaactggatgtcctgtacatacatttccattgaagtttatggcagtttctgggcacaatcacatcaatattgcacatctatagatagtttacaggttacataactgtggttttggatttaattgccaacttgttaccctgatagtaattccagacaggggaataacagagcgaaggggtctgcccattgtgttactgctgcctataaaaacaaataggatccttagggtttaattggaggacttataattgcacctaatgttaaaatgggaactttggacatctggaagatgagtctggatttggtcacttgcctttaggaattaaattcatgaaattgtgatggtcctaaagaacagtggtgttcccacctggatttatgcacaggcagaaatgacaaaggtgaatgtgagctggtctgcaaggccaaataagtcaggagagaaaaatggagtttggctttaaactcacaagtaatccaggatgatgactggcttctttggtcctaacatgaaaataagccatctaaaatgaagagcaggtacataaaaagtttgttcttacttggcaaagacatgcatggcttttggaacttgcaactacacagggtgtcacttggcatcatagagcccatttaggaaaagaatgacccatggtgacacgggctcgttggaaagggtcaggaaaggaacatatacagcaaaaggtacaatacagctttccgtagagaacactgggtatcattttcttccactcatccctcctctccaccatcaaagccaaacatttatataggtatgcattccaccctgcccaatgcattacaaatgccaataagagaggtaggactgttgtttccatttttttccttctaaagctattgaaagttctttgtctgttccttatatagttttaggaatacttttgaggaaattgcctttattctttatagtggatttcatataaagcaagttttgtgtttcttaggaataaaatttcaggcttctggaatattttttattttctctctccataaaaagataatttcaatttccctaaattactaggaatctactctacatggtgcagcaaaattttaaattatgtaatttagattactccagagtaaaacgtcttaaaaactgagagcacagcttaagtgtatggtctagaggcaagagttaatggcatggaaaagtagtaaaaggttggattagaaggtttaatacttttgatctctcagcccattgcagtttacttactccttaggagacacagatgggacacggcaggtgtgtgtaaggagcgaagcaattcatgaatactcagccatgaaatagaaaatcaaaatgaaataagtatgactgcaactatcttggtctattaacattcaactattaatacctactgttctttgaaagccattactgaatatttactgataagaaaaaaatgatagcttaggaagaggaagatgttcaggaaaagcatttaagcagggtttgaaagacttgtgattttcttaactcggggtaaaagtcgaccaattaaagtaggtttcccatccaaatgtttcccatccaaaatgatccctttttttttccccaagggatctaatttaggatcccttggaaaaaaattccaaaatgcattacaactattcataagggtgacacatggacctatttttctaaggactttgatttaatatttgaatgcaatggtatctgactttgttagtatagaatatttaaacttaaaaagaaaataccttaatttacttatgcataagcctattaaacacatttctaggggctctttttatgtttattctctagaacataacctatctttgaagtggtatattagtttttaaaaagtcattcctaagctgaataattaaactgaaaacaaaagctattcttagggtgtattccacatataaagctatgcacatgatgctttgattcaaataatatacttataaaactttgttattgtttgagttccatattcagaatggcaacttttgtttttgatgattattccatcctgaaacaatttcccccctgctcaattaaaccagaattaggagcacatttatatctgatgagacttaagcttctcaactgcctgcttcagaaatgtagacctttagtgcttgtgttcattttgtctctttgtggaaggctcaaaagaaaacagaatcaattcccttaagtttttctggaagaagaaggttggttttgttgctttgatcttagcatgttgtgcattttttattggctgttgaatataaaaagccacagcctcatctggtttttctgctatattctcatattgtaaatcacataatgccttccaatctaaagtaaaatgcctaagtccaaaatatcacttcaaaatggatttatcattatagttgatagaaagatttccagggtgtaagaaaacaattcaacagtttgattaatatgccacagactgctaaaaatatattcatgcattttagacaataaatttcaggatatagacatacactcatgctatttgagatccttttttcctaccattgcaagaggctgctttagctaatgcaacagctggctaggttattgcttcaacaatataattcataatgcaaaagcagctcttttccaaacattttagagcaactcaagttgtttacatctcctgtaggtgattttcctataactttgtgccaattggtgtcatactatttggtaaaaatctacattaaatcaagacaactgcacttggttaaatttctgtcatacagagaattatagaaaaattacagctgatttgaacttatcatcattaagtatatacagggttttagaaaatgaatgcaaactacaaaaatggagttgtataattaaacattaaatagtccaagtaataaaagtcatagattaattgtctctcagttctagtcagatcctttaaatactgtctcacgacttgagcattggttctttcatcggaagagtgcctatccttaaagttgggaaatttcagctcctttggagcaccgatcatctgtaaaaagtaattggcatcttcttccaaagtctcaaatttccctacaaaatcatagttgatcaaacacggatagcagagtttgctgaccttttcccagtgaatgtccattcctactggacggtgggaatccagcaagtagtggataaactctttgaacttgactccagatccattaattaatgcttcttcacaggcatttggtcgatatttcttgataattgcctttccgaatactggatggtaataactattggggtgttcaaatttgtccctaaaggctgatactaatctttccatgggatcacgaacaaacacagctttggtgtaagtatttaagcgggtatatatcccttttaggtcaaagctatctagcttcttcaaatgcttcccgtagtggacagcattgtgggagatgttgtatgcagaggaagccaatccatttagtaccatcagaattcttttccaattggaacagccagccttaggtacctcacaatataagattttgtgtttatcttctacatagattctggatactgtatgaaaaagatgtgactgatgatgactcaccccaccgtatttcttgcaaaactcctgaaggaaagaccttcgtttctcttgggtctcctcagttttcttccatttattatctttgactaaacttttgtttaaagggtgaatgtccactggccaattcatgttgctgaacttgttaaaaacagtcttagctccttgacgtttttcaatcaacttctctgttggtgaccctgtggacttacttaaagcttgatcccctccttgtgaatgactggtctttgttaagagcctagtagatctctcagaattgagtagaagattttcctttttttctcgtacatcctcaggcatgtgaaacttggggttctggttggtgatatgttcctggattttttctgtactcacagcctcgtaaccagagggaagaaacttcatctaagtcttagtttcttcaactgtaaaatgagaaaaaataatatcggtccttcctacctcacagggtgattctgggtacaggccgcaagtacttcactggtccccatcctgaagttactttttgttctcttctcttctccactctccctgtatgttgttcttcaatccagacttgcaaatacatgaagaggagtagcccagctactccaaatatcagcacagagaggaagacttgtttggggttcatgaccatttcagatggctgcatttctccttatttcagaatctgaagaccacatgatttgttttcccgtaaaacttcagtcttttcttgttctctaagagcccaattccataaagtaacctcgcgggccgctgccgggcgcttgcaggtgctgctgttccaggagcgcagcttcggaggaaacttccccgcgctccggggcaaactcccgcgcactcctggcagccgtgaggtggctgagagcggagcgccgcgccgggagcggggacagctcggagtcgggcgctcaccctggccctgaccctcccgcgtccggcccggctggggctgcggcgccgcctccgcgccc

SEQ ID NO: 12459 - RNA, 8523 nt, Homo sapiens
  source 1..8523: mol_type = other RNA
cttagcaggttgtattatcatttataatcaaccaggacttaaaaaattcacacacacacgagaagtaccccaagagattattaaaaaggaaattttcaggtggttttcatagagattccaattctgtgtatcttggatggggtctgggaatatgtttttaacaaaaattaggttaattctgatacaggtcgtccatacactatttttttcagaaattgataagttaaatcagggcttattttttcctaaggataatcacagtcaaacaaataatattgttcttttaagttggtagacactctagcattctgagtgcatttttatttattatatagtacatccaaaaatcatttttctaaactttggaaatattttcagcaaatgaatgcataaaatgagatactgtgtgttttactagttttcctggtatttgaggacaaaagtcgtagttatcccttctcctgttttctccacctctctaagtatagaagtggggggaggagtaggaggagtaggaggaggaggaggaagaggagggaagaggaggaggaggaggttgtcagagcattaagaagcaagagagtagaatgttacagggggtgctacaatcacccagataatagcaggaagtagggtggagaggcatgttataaatcagaaagaagaatcttcggagaaggctgggaagcaggtgatttttagagttgaggaagcgggcacacctgcaaaacagaagagatttttggatgaaggttatagaacagcagtctagaggcagcagtgggagccagtttctgtccctagatactagagctccaagagcctgggagaatgactcatctctgcagaaagaggtgggaaggaatgtcgttgccaggggacccagtggctacgacagaaagatgccaaaaaaaggtactggatttctcccaacatctttgtcattggtcaaaagagacttccccaaacaatgaaatactgtttggagatcccactggatataggaccaaagggcaagcagcactgtgagcaaggatatggaaacccggaatgggataacctcactacctgcacaacacaaatagggtcaaggataatgttcaggagttgatttcctttggaagcttggcgggggaaggaatacactcttcagagcaggacttgaaaagtgagatgcttaggggccaggcaagtaaggtgaatgagtgatggtggattagtgaagagtgtgaacaactagagatctccaacctcatctaaagggactgaccttgcctctgtccaactattttcaggtgggcatatagaatgtagggtaacaaatcccctgtcattaatgaggcccaatgttggcagctaattcagatgttaaataaaatgcactgtcagccaaaccaaacatatctgtagccagatctaccccgtgggctgccaatgtatggtctcagctttggagccagagagactgttattaaacctctttgatactcagttttctcattcatgaaatgataggtggaaaaatactcgactttgatttttttgaaagctacttttggaaacggttagacttactcttcatgtcattaaatgaatgtatgcaaagtatttttcccgtgtctgctactgagtagatcctcagtaaatggctcttatgttgaccagaatcatgcatttttctcaaaattttcttccccaaacaatcaagcaactgctatttcttagaaatgtaaaagatttctgtgtctgcaactatccttcaggtcaagggatgactattagtgtagaaaaggtgtgtggctcagctcccttccctcagctgccctgctctagcaccttcctttcagatcctctggtcctatagatgcctgaaggtcacaggcagaaatatacgaattctacactaaaagaagttgtacaggaacctttaaacaacagcatcaaaagcatctgttaaagtaacgctttccactgagtgccttgctagacatggtacaaagtgcattcaacagacacagttcctttcctcttggaagacctaagacattccaatgacaacaacagatattttatattcataaaaagtgagataaatagcacatgaacaaataaattaacgaacctccctgacaaaaaaaatcgaggaaaggaatgcctgcatttattggtaagagaataatctgatgcatgttacaccaggggaaaactctgctgtctttttctgcctatcagggagctcataaagagatgagattttgaaattgaataatctcaagagattccttggtgagttaacaagaaatgaatgtccagatatatagagaggggagcattccaaatatagtgtgagacttgaggagaggtttagggatggaaaaagatgactgcttaaatggatttaaatacttttgcctggaagcatatgatcctggtgaaaaactaagatgtgactgactaggaaattctgagaatgaaatgatatgaggcaatgttctgttgaactccccagacctggccttcctcaggtaatgatcacaggcctgggaaatgtctgccatcttctagcaagagcttatttattttcacctggtttcatggtgttttttcagtcggtttaagtcagcttgctcctctattcttttctgcagtcttcccgtgtaggctcagggtaatctgactacaaactagtactagggaaggagactcaggaagaaggggataatgcacagttgctctgtttctagcaggagtggttctcactgtgtgtgactagcttgctgaaccgtgaccatctgcagtggctgtcaggggcctatgtgtggaaagttcgcctgaactttcttcctcttagattctgcttatccttgactggtcttgtagctgtctggaatttcttgtcaaagaaatgatattttgttttcacaaggctaaatttgttccagggactattttttcttcttaaaaacattgtttccatgattaactaaggattacaaaaaagttgtggggaggaaacctaatttcttccaaagtctttgaacctgtcagtttaactcagcaggaataaagaaataagctgatttgaaatgtgataactaactagctaaatacacacacacacacacacacacacacacacacacacacagacacccatatttgtatggaaaaaatttcaggattccaatatattgtttttgcctctacctatcctgaatagaggtaacggaaagcaaaagtaaatattggtttgtaatattctaagcaaagagtttggtagtggtatttgctgcttggcttcatcctggcttctgacctacttatcatctctgtctccttaggcaagttactcagctatagtctgctttactttcctttatgatagatggaaagggagagggctacataatattacctatgttagactggctatggagattaaattaatgcatgtaaactacttgaagagtgcctgacacccagtaagtattgaataaatgttagctaggatcatgcatacgattactgtataatgatcatgattgagattgagaaggtatgagcctaaatgtaggactaaattgaattagccttggcctaaggttctcaggtagttgagctataattaaacgcctttggccaatcctttttcaagtatcagagcatcttgggagggttagccctgggcaaaacatctgcttcaccacgccccatgaaggcctagaggctgggatgccctgagaggccacatgagaatgcacaggagggagacgtttactgtagtcctagcctaatcccaagttctattaattcagcaagtgattttttcaaagggcactctaatattcaaaattctctgcatcttcttatatataccttctgctaaatactatacattttaggagataagaataataatacatcaataaaatgtaaaagtatttttcctctttctaattaaaaatgacatacaagtagttcttgaattagaactactaattccctaatgataataatattattattttctgttacagaatgttttatagacatctagcaagtggcatcacatttccattgaattaatggatatttccaaatgtttgagaaaatccgaaaactggatgtcctgtacatacatttccattgaagtttatggcagtttctgggcacaatcacatcaatattgcacatctatagatagtttacaggttacataactgtggttttggatttaattgccaacttgttaccctgatagtaattccagacaggggaataacagagcgaaggggtctgcccattgtgttactgctgcctataaaaacaaataggatccttagggtttaattggaggacttataattgcacctaatgttaaaatgggaactttggacatctggaagatgagtctggatttggtcacttgcctttaggaattaaattcatgaaattgtgatggtcctaaagaacagtggtgttcccacctggatttatgcacaggcagaaatgacaaaggtgaatgtgagctggtctgcaaggccaaataagtcaggagagaaaaatggagtttggctttaaactcacaagtaatccaggatgatgactggcttctttggtcctaacatgaaaataagccatctaaaatgaagagcaggtacataaaaagtttgttcttacttggcaaagacatgcatggcttttggaacttgcaactacacagggtgtcacttggcatcatagagcccatttaggaaaagaatgacccatggtgacacgggctcgttggaaagggtcaggaaaggaacatatacagcaaaaggtacaatacagctttccgtagagaacactgggtatcattttcttccactcatccctcctctccaccatcaaagccaaacatttatataggtatgcattccaccctgcccaatgcattacaaatgccaataagagaggtaggactgttgtttccatttttttccttctaaagctattgaaagttctttgtctgttccttatatagttttaggaatacttttgaggaaattgcctttattctttatagtggatttcatataaagcaagttttgtgtttcttaggaataaaatttcaggcttctggaatattttttattttctctctccataaaaagataatttcaatttccctaaattactaggaatctactctacatggtgcagcaaaattttaaattatgtaatttagattactccagagtaaaacgtcttaaaaactgagagcacagcttaagtgtatggtctagaggcaagagttaatggcatggaaaagtagtaaaaggttggattagaaggtttaatacttttgatctctcagcccattgcagtttacttactccttaggagacacagatgggacacggcaggtgtgtgtaaggagcgaagcaattcatgaatactcagccatgaaatagaaaatcaaaatgaaataagtatgactgcaactatcttggtctattaacattcaactattaatacctactgttctttgaaagccattactgaatatttactgataagaaaaaaatgatagcttaggaagaggaagatgttcaggaaaagcatttaagcagggtttgaaagacttgtgattttcttaactcggggtaaaagtcgaccaattaaagtaggtttcccatccaaatgtttcccatccaaaatgatccctttttttttccccaagggatctaatttaggatcccttggaaaaaaattccaaaatgcattacaactattcataagggtgacacatggacctatttttctaaggactttgatttaatatttgaatgcaatggtatctgactttgttagtatagaatatttaaacttaaaaagaaaataccttaatttacttatgcataagcctattaaacacatttctaggggctctttttatgtttattctctagaacataacctatctttgaagtggtatattagtttttaaaaagtcattcctaagctgaataattaaactgaaaacaaaagctattcttagggtgtattccacatataaagctatgcacatgatgctttgattcaaataatatacttataaaactttgttattgtttgagttccatattcagaatggcaacttttgtttttgatgattattccatcctgaaacaatttcccccctgctcaattaaaccagaattaggagcacatttatatctgatgagacttaagcttctcaactgcctgcttcagaaatgtagacctttagtgcttgtgttcattttgtctctttgtggaaggctcaaaagaaaacagaatcaattcccttaagtttttctggaagaagaaggttggttttgttgctttgatcttagcatgttgtgcattttttattggctgttgaatataaaaagccacagcctcatctggtttttctgctatattctcatattgtaaatcacataatgccttccaatctaaagtaaaatgcctaagtccaaaatatcacttcaaaatggatttatcattatagttgatagaaagatttccagggtgtaagaaaacaattcaacagtttgattaatatgccacagactgctaaaaatatattcatgcattttagacaataaatttcaggatatagacatacactcatgctatttgagatccttttttcctaccattgcaagaggctgctttagctaatgcaacagctggctaggttattgcttcaacaatataattcataatgcaaaagcagctcttttccaaacattttagagcaactcaagttgtttacatctcctgtaggtgattttcctataactttgtgccaattggtgtcatactatttggtaaaaatctacattaaatcaagacaactgcacttggttaaatttctgtcatacagagaattatagaaaaattacagctgatttgaacttatcatcattaagtatatacagggttttagaaaatgaatgcaaactacaaaaatggagttgtataattaaacattaaatagtccaagtaataaaagtcatagattaattgtctctcagttctagtcagatcctttaaatactgtctcacgacttgagcattggttctttcatcggaagagtgcctatccttaaagttgggaaatttcagctcctttggagcaccgatcatctgtaaaaagtaattggcatcttcttccaaagtctcaaatttccctacaaaatcatagttgatcaaacacggatagcagagtttgctgaccttttcccagtgaatgtccattcctactggacggtgggaatccagcaagtagtggataaactctttgaacttgactccagatccattaattaatgcttcttcacaggcatttggtcgatatttcttgataattgcctttccgaatactggatggtaataactattggggtgttcaaatttgtccctaaaggctgatactaatctttccatgggatcacgaacaaacacagctttggtgtaagtatttaagcgggtatatatcccttttaggtcaaagctatctagcttcttcaaatgcttcccgtagtggacagcattgtgggagatgttgtatgcagaggaagccaatccatttagtaccatcagaattcttttccaattggaacagccagccttaggtacctcacaatataagattttgtgtttatcttctacatagattctggatactgtatgaaaaagatgtgactgatgatgactcaccccaccgtatttcttgcaaaactcctgaaggaaagaccttcgtttctcttgggtctcctcagttttcttccatttattatctttgactaaacttttgtttaaagggtgaatgtccactggccaattcatgttgctgaacttgttaaaaacagtcttagctccttgacgtttttcaatcaacttctctgttggtgaccctgtggacttacttaaagcttgatcccctccttgtgaatgactggtctttgttaagagcctagtagatctctcagaattgagtagaagattttcctttttttctcgtacatcctcaggcatgtgaaacttggggttctggttggtgatatgttcctggattttttctgtactcatgattctgggtacaggccgcaagtacttcactggtccccatcctgaagttactttttgttctcttctcttctccactctccctgtatgttgttcttcaatccagacttgcaaatacatgaagaggagtagcccagctactccaaatatcagcacagagaggaagacttgtttggggttcatgaccatttcagatggctgcatttctccttatttcagaatctgaagaccacatgatttgttttcccgtaaaacttcagtcttttcttgttctctaagagcccaattccataaagtaacctagaattttaaaaagaaatctacattgtacatttctgctaatattaattctcaaatacggcataaatattcactatctcaacaaggctgaagacttaatgt

SEQ ID NO: 12460 - RNA, 8594 nt, Homo sapiens
  source 1..8594: mol_type = other RNA
cttagcaggttgtattatcatttataatcaaccaggacttaaaaaattcacacacacacgagaagtaccccaagagattattaaaaaggaaattttcaggtggttttcatagagattccaattctgtgtatcttggatggggtctgggaatatgtttttaacaaaaattaggttaattctgatacaggtcgtccatacactatttttttcagaaattgataagttaaatcagggcttattttttcctaaggataatcacagtcaaacaaataatattgttcttttaagttggtagacactctagcattctgagtgcatttttatttattatatagtacatccaaaaatcatttttctaaactttggaaatattttcagcaaatgaatgcataaaatgagatactgtgtgttttactagttttcctggtatttgaggacaaaagtcgtagttatcccttctcctgttttctccacctctctaagtatagaagtggggggaggagtaggaggagtaggaggaggaggaggaagaggagggaagaggaggaggaggaggttgtcagagcattaagaagcaagagagtagaatgttacagggggtgctacaatcacccagataatagcaggaagtagggtggagaggcatgttataaatcagaaagaagaatcttcggagaaggctgggaagcaggtgatttttagagttgaggaagcgggcacacctgcaaaacagaagagatttttggatgaaggttatagaacagcagtctagaggcagcagtgggagccagtttctgtccctagatactagagctccaagagcctgggagaatgactcatctctgcagaaagaggtgggaaggaatgtcgttgccaggggacccagtggctacgacagaaagatgccaaaaaaaggtactggatttctcccaacatctttgtcattggtcaaaagagacttccccaaacaatgaaatactgtttggagatcccactggatataggaccaaagggcaagcagcactgtgagcaaggatatggaaacccggaatgggataacctcactacctgcacaacacaaatagggtcaaggataatgttcaggagttgatttcctttggaagcttggcgggggaaggaatacactcttcagagcaggacttgaaaagtgagatgcttaggggccaggcaagtaaggtgaatgagtgatggtggattagtgaagagtgtgaacaactagagatctccaacctcatctaaagggactgaccttgcctctgtccaactattttcaggtgggcatatagaatgtagggtaacaaatcccctgtcattaatgaggcccaatgttggcagctaattcagatgttaaataaaatgcactgtcagccaaaccaaacatatctgtagccagatctaccccgtgggctgccaatgtatggtctcagctttggagccagagagactgttattaaacctctttgatactcagttttctcattcatgaaatgataggtggaaaaatactcgactttgatttttttgaaagctacttttggaaacggttagacttactcttcatgtcattaaatgaatgtatgcaaagtatttttcccgtgtctgctactgagtagatcctcagtaaatggctcttatgttgaccagaatcatgcatttttctcaaaattttcttccccaaacaatcaagcaactgctatttcttagaaatgtaaaagatttctgtgtctgcaactatccttcaggtcaagggatgactattagtgtagaaaaggtgtgtggctcagctcccttccctcagctgccctgctctagcaccttcctttcagatcctctggtcctatagatgcctgaaggtcacaggcagaaatatacgaattctacactaaaagaagttgtacaggaacctttaaacaacagcatcaaaagcatctgttaaagtaacgctttccactgagtgccttgctagacatggtacaaagtgcattcaacagacacagttcctttcctcttggaagacctaagacattccaatgacaacaacagatattttatattcataaaaagtgagataaatagcacatgaacaaataaattaacgaacctccctgacaaaaaaaatcgaggaaaggaatgcctgcatttattggtaagagaataatctgatgcatgttacaccaggggaaaactctgctgtctttttctgcctatcagggagctcataaagagatgagattttgaaattgaataatctcaagagattccttggtgagttaacaagaaatgaatgtccagatatatagagaggggagcattccaaatatagtgtgagacttgaggagaggtttagggatggaaaaagatgactgcttaaatggatttaaatacttttgcctggaagcatatgatcctggtgaaaaactaagatgtgactgactaggaaattctgagaatgaaatgatatgaggcaatgttctgttgaactccccagacctggccttcctcaggtaatgatcacaggcctgggaaatgtctgccatcttctagcaagagcttatttattttcacctggtttcatggtgttttttcagtcggtttaagtcagcttgctcctctattcttttctgcagtcttcccgtgtaggctcagggtaatctgactacaaactagtactagggaaggagactcaggaagaaggggataatgcacagttgctctgtttctagcaggagtggttctcactgtgtgtgactagcttgctgaaccgtgaccatctgcagtggctgtcaggggcctatgtgtggaaagttcgcctgaactttcttcctcttagattctgcttatccttgactggtcttgtagctgtctggaatttcttgtcaaagaaatgatattttgttttcacaaggctaaatttgttccagggactattttttcttcttaaaaacattgtttccatgattaactaaggattacaaaaaagttgtggggaggaaacctaatttcttccaaagtctttgaacctgtcagtttaactcagcaggaataaagaaataagctgatttgaaatgtgataactaactagctaaatacacacacacacacacacacacacacacacacacacacagacacccatatttgtatggaaaaaatttcaggattccaatatattgtttttgcctctacctatcctgaatagaggtaacggaaagcaaaagtaaatattggtttgtaatattctaagcaaagagtttggtagtggtatttgctgcttggcttcatcctggcttctgacctacttatcatctctgtctccttaggcaagttactcagctatagtctgctttactttcctttatgatagatggaaagggagagggctacataatattacctatgttagactggctatggagattaaattaatgcatgtaaactacttgaagagtgcctgacacccagtaagtattgaataaatgttagctaggatcatgcatacgattactgtataatgatcatgattgagattgagaaggtatgagcctaaatgtaggactaaattgaattagccttggcctaaggttctcaggtagttgagctataattaaacgcctttggccaatcctttttcaagtatcagagcatcttgggagggttagccctgggcaaaacatctgcttcaccacgccccatgaaggcctagaggctgggatgccctgagaggccacatgagaatgcacaggagggagacgtttactgtagtcctagcctaatcccaagttctattaattcagcaagtgattttttcaaagggcactctaatattcaaaattctctgcatcttcttatatataccttctgctaaatactatacattttaggagataagaataataatacatcaataaaatgtaaaagtatttttcctctttctaattaaaaatgacatacaagtagttcttgaattagaactactaattccctaatgataataatattattattttctgttacagaatgttttatagacatctagcaagtggcatcacatttccattgaattaatggatatttccaaatgtttgagaaaatccgaaaactggatgtcctgtacatacatttccattgaagtttatggcagtttctgggcacaatcacatcaatattgcacatctatagatagtttacaggttacataactgtggttttggatttaattgccaacttgttaccctgatagtaattccagacaggggaataacagagcgaaggggtctgcccattgtgttactgctgcctataaaaacaaataggatccttagggtttaattggaggacttataattgcacctaatgttaaaatgggaactttggacatctggaagatgagtctggatttggtcacttgcctttaggaattaaattcatgaaattgtgatggtcctaaagaacagtggtgttcccacctggatttatgcacaggcagaaatgacaaaggtgaatgtgagctggtctgcaaggccaaataagtcaggagagaaaaatggagtttggctttaaactcacaagtaatccaggatgatgactggcttctttggtcctaacatgaaaataagccatctaaaatgaagagcaggtacataaaaagtttgttcttacttggcaaagacatgcatggcttttggaacttgcaactacacagggtgtcacttggcatcatagagcccatttaggaaaagaatgacccatggtgacacgggctcgttggaaagggtcaggaaaggaacatatacagcaaaaggtacaatacagctttccgtagagaacactgggtatcattttcttccactcatccctcctctccaccatcaaagccaaacatttatataggtatgcattccaccctgcccaatgcattacaaatgccaataagagaggtaggactgttgtttccatttttttccttctaaagctattgaaagttctttgtctgttccttatatagttttaggaatacttttgaggaaattgcctttattctttatagtggatttcatataaagcaagttttgtgtttcttaggaataaaatttcaggcttctggaatattttttattttctctctccataaaaagataatttcaatttccctaaattactaggaatctactctacatggtgcagcaaaattttaaattatgtaatttagattactccagagtaaaacgtcttaaaaactgagagcacagcttaagtgtatggtctagaggcaagagttaatggcatggaaaagtagtaaaaggttggattagaaggtttaatacttttgatctctcagcccattgcagtttacttactccttaggagacacagatgggacacggcaggtgtgtgtaaggagcgaagcaattcatgaatactcagccatgaaatagaaaatcaaaatgaaataagtatgactgcaactatcttggtctattaacattcaactattaatacctactgttctttgaaagccattactgaatatttactgataagaaaaaaatgatagcttaggaagaggaagatgttcaggaaaagcatttaagcagggtttgaaagacttgtgattttcttaactcggggtaaaagtcgaccaattaaagtaggtttcccatccaaatgtttcccatccaaaatgatccctttttttttccccaagggatctaatttaggatcccttggaaaaaaattccaaaatgcattacaactattcataagggtgacacatggacctatttttctaaggactttgatttaatatttgaatgcaatggtatctgactttgttagtatagaatatttaaacttaaaaagaaaataccttaatttacttatgcataagcctattaaacacatttctaggggctctttttatgtttattctctagaacataacctatctttgaagtggtatattagtttttaaaaagtcattcctaagctgaataattaaactgaaaacaaaagctattcttagggtgtattccacatataaagctatgcacatgatgctttgattcaaataatatacttataaaactttgttattgtttgagttccatattcagaatggcaacttttgtttttgatgattattccatcctgaaacaatttcccccctgctcaattaaaccagaattaggagcacatttatatctgatgagacttaagcttctcaactgcctgcttcagaaatgtagacctttagtgcttgtgttcattttgtctctttgtggaaggctcaaaagaaaacagaatcaattcccttaagtttttctggaagaagaaggttggttttgttgctttgatcttagcatgttgtgcattttttattggctgttgaatataaaaagccacagcctcatctggtttttctgctatattctcatattgtaaatcacataatgccttccaatctaaagtaaaatgcctaagtccaaaatatcacttcaaaatggatttatcattatagttgatagaaagatttccagggtgtaagaaaacaattcaacagtttgattaatatgccacagactgctaaaaatatattcatgcattttagacaataaatttcaggatatagacatacactcatgctatttgagatccttttttcctaccattgcaagaggctgctttagctaatgcaacagctggctaggttattgcttcaacaatataattcataatgcaaaagcagctcttttccaaacattttagagcaactcaagttgtttacatctcctgtaggtgattttcctataactttgtgccaattggtgtcatactatttggtaaaaatctacattaaatcaagacaactgcacttggttaaatttctgtcatacagagaattatagaaaaattacagctgatttgaacttatcatcattaagtatatacagggttttagaaaatgaatgcaaactacaaaaatggagttgtataattaaacattaaatagtccaagtaataaaagtcatagattaattgtctctcagttctagtcagatcctttaaatactgtctcacgacttgagcattggttctttcatcggaagagtgcctatccttaaagttgggaaatttcagctcctttggagcaccgatcatctgtaaaaagtaattggcatcttcttccaaagtctcaaatttccctacaaaatcatagttgatcaaacacggatagcagagtttgctgaccttttcccagtgaatgtccattcctactggacggtgggaatccagcaagtagtggataaactctttgaacttgactccagatccattaattaatgcttcttcacaggcatttggtcgatatttcttgataattgcctttccgaatactggatggtaataactattggggtgttcaaatttgtccctaaaggctgatactaatctttccatgggatcacgaacaaacacagctttggtgtaagtatttaagcgggtatatatcccttttaggtcaaagctatctagcttcttcaaatgcttcccgtagtggacagcattgtgggagatgttgtatgcagaggaagccaatccatttagtaccatcagaattcttttccaattggaacagccagccttaggtacctcacaatataagattttgtgtttatcttctacatagattctggatactgtatgaaaaagatgtgactgatgatgactcaccccaccgtatttcttgcaaaactcctgaaggaaagaccttcgtttctcttgggtctcctcagttttcttccatttattatctttgactaaacttttgtttaaagggtgaatgtccactggccaattcatgttgctgaacttgttaaaaacagtcttagctccttgacgtttttcaatcaacttctctgttggtgaccctgtggacttacttaaagcttgatcccctccttgtgaatgactggtctttgttaagagcctagtagatctctcagaattgagtagaagattttcctttttttctcgtacatcctcaggcatgtgaaacttggggttctggttggtgatatgttcctggattttttctgtactcatgattctgggtacaggccgcaagtacttcactggtccccatcctgaagttactttttgttctcttctcttctccactctccctgtatgttgttcttcaatccagacttgcaaatacatgaagaggagtagcccagctactccaaatatcagcacagagaggaagacttgtttggggttcatgaccatttcagatggctgcatttctccttatttcagaatctgaagaccacatgatttgttttcccgtaaaacttcagtcttttcttgttctctaagagcccaattccataaagtaacctcgcgggccgctgccgggcgcttgcaggtgctgctgttccaggagcgcagcttcggaggaaacttccccgcgctccggggcaaactcccgcgcactcctggcagccgtgaggtggctgagagcggagcgccgcgccgggagcggggacagctcggagtcgggcgctcaccct

SEQ ID NO: 12461 - RNA, 8308 nt, Homo sapiens
  source 1..8308: mol_type = other RNA
cttagcaggttgtattatcatttataatcaaccaggacttaaaaaattcacacacacacgagaagtaccccaagagattattaaaaaggaaattttcaggtggttttcatagagattccaattctgtgtatcttggatggggtctgggaatatgtttttaacaaaaattaggttaattctgatacaggtcgtccatacactatttttttcagaaattgataagttaaatcagggcttattttttcctaaggataatcacagtcaaacaaataatattgttcttttaagttggtagacactctagcattctgagtgcatttttatttattatatagtacatccaaaaatcatttttctaaactttggaaatattttcagcaaatgaatgcataaaatgagatactgtgtgttttactagttttcctggtatttgaggacaaaagtcgtagttatcccttctcctgttttctccacctctctaagtatagaagtggggggaggagtaggaggagtaggaggaggaggaggaagaggagggaagaggaggaggaggaggttgtcagagcattaagaagcaagagagtagaatgttacagggggtgctacaatcacccagataatagcaggaagtagggtggagaggcatgttataaatcagaaagaagaatcttcggagaaggctgggaagcaggtgatttttagagttgaggaagcgggcacacctgcaaaacagaagagatttttggatgaaggttatagaacagcagtctagaggcagcagtgggagccagtttctgtccctagatactagagctccaagagcctgggagaatgactcatctctgcagaaagaggtgggaaggaatgtcgttgccaggggacccagtggctacgacagaaagatgccaaaaaaaggtactggatttctcccaacatctttgtcattggtcaaaagagacttccccaaacaatgaaatactgtttggagatcccactggatataggaccaaagggcaagcagcactgtgagcaaggatatggaaacccggaatgggataacctcactacctgcacaacacaaatagggtcaaggataatgttcaggagttgatttcctttggaagcttggcgggggaaggaatacactcttcagagcaggacttgaaaagtgagatgcttaggggccaggcaagtaaggtgaatgagtgatggtggattagtgaagagtgtgaacaactagagatctccaacctcatctaaagggactgaccttgcctctgtccaactattttcaggtgggcatatagaatgtagggtaacaaatcccctgtcattaatgaggcccaatgttggcagctaattcagatgttaaataaaatgcactgtcagccaaaccaaacatatctgtagccagatctaccccgtgggctgccaatgtatggtctcagctttggagccagagagactgttattaaacctctttgatactcagttttctcattcatgaaatgataggtggaaaaatactcgactttgatttttttgaaagctacttttggaaacggttagacttactcttcatgtcattaaatgaatgtatgcaaagtatttttcccgtgtctgctactgagtagatcctcagtaaatggctcttatgttgaccagaatcatgcatttttctcaaaattttcttccccaaacaatcaagcaactgctatttcttagaaatgtaaaagatttctgtgtctgcaactatccttcaggtcaagggatgactattagtgtagaaaaggtgtgtggctcagctcccttccctcagctgccctgctctagcaccttcctttcagatcctctggtcctatagatgcctgaaggtcacaggcagaaatatacgaattctacactaaaagaagttgtacaggaacctttaaacaacagcatcaaaagcatctgttaaagtaacgctttccactgagtgccttgctagacatggtacaaagtgcattcaacagacacagttcctttcctcttggaagacctaagacattccaatgacaacaacagatattttatattcataaaaagtgagataaatagcacatgaacaaataaattaacgaacctccctgacaaaaaaaatcgaggaaaggaatgcctgcatttattggtaagagaataatctgatgcatgttacaccaggggaaaactctgctgtctttttctgcctatcagggagctcataaagagatgagattttgaaattgaataatctcaagagattccttggtgagttaacaagaaatgaatgtccagatatatagagaggggagcattccaaatatagtgtgagacttgaggagaggtttagggatggaaaaagatgactgcttaaatggatttaaatacttttgcctggaagcatatgatcctggtgaaaaactaagatgtgactgactaggaaattctgagaatgaaatgatatgaggcaatgttctgttgaactccccagacctggccttcctcaggtaatgatcacaggcctgggaaatgtctgccatcttctagcaagagcttatttattttcacctggtttcatggtgttttttcagtcggtttaagtcagcttgctcctctattcttttctgcagtcttcccgtgtaggctcagggtaatctgactacaaactagtactagggaaggagactcaggaagaaggggataatgcacagttgctctgtttctagcaggagtggttctcactgtgtgtgactagcttgctgaaccgtgaccatctgcagtggctgtcaggggcctatgtgtggaaagttcgcctgaactttcttcctcttagattctgcttatccttgactggtcttgtagctgtctggaatttcttgtcaaagaaatgatattttgttttcacaaggctaaatttgttccagggactattttttcttcttaaaaacattgtttccatgattaactaaggattacaaaaaagttgtggggaggaaacctaatttcttccaaagtctttgaacctgtcagtttaactcagcaggaataaagaaataagctgatttgaaatgtgataactaactagctaaatacacacacacacacacacacacacacacacacacacacagacacccatatttgtatggaaaaaatttcaggattccaatatattgtttttgcctctacctatcctgaatagaggtaacggaaagcaaaagtaaatattggtttgtaatattctaagcaaagagtttggtagtggtatttgctgcttggcttcatcctggcttctgacctacttatcatctctgtctccttaggcaagttactcagctatagtctgctttactttcctttatgatagatggaaagggagagggctacataatattacctatgttagactggctatggagattaaattaatgcatgtaaactacttgaagagtgcctgacacccagtaagtattgaataaatgttagctaggatcatgcatacgattactgtataatgatcatgattgagattgagaaggtatgagcctaaatgtaggactaaattgaattagccttggcctaaggttctcaggtagttgagctataattaaacgcctttggccaatcctttttcaagtatcagagcatcttgggagggttagccctgggcaaaacatctgcttcaccacgccccatgaaggcctagaggctgggatgccctgagaggccacatgagaatgcacaggagggagacgtttactgtagtcctagcctaatcccaagttctattaattcagcaagtgattttttcaaagggcactctaatattcaaaattctctgcatcttcttatatataccttctgctaaatactatacattttaggagataagaataataatacatcaataaaatgtaaaagtatttttcctctttctaattaaaaatgacatacaagtagttcttgaattagaactactaattccctaatgataataatattattattttctgttacagaatgttttatagacatctagcaagtggcatcacatttccattgaattaatggatatttccaaatgtttgagaaaatccgaaaactggatgtcctgtacatacatttccattgaagtttatggcagtttctgggcacaatcacatcaatattgcacatctatagatagtttacaggttacataactgtggttttggatttaattgccaacttgttaccctgatagtaattccagacaggggaataacagagcgaaggggtctgcccattgtgttactgctgcctataaaaacaaataggatccttagggtttaattggaggacttataattgcacctaatgttaaaatgggaactttggacatctggaagatgagtctggatttggtcacttgcctttaggaattaaattcatgaaattgtgatggtcctaaagaacagtggtgttcccacctggatttatgcacaggcagaaatgacaaaggtgaatgtgagctggtctgcaaggccaaataagtcaggagagaaaaatggagtttggctttaaactcacaagtaatccaggatgatgactggcttctttggtcctaacatgaaaataagccatctaaaatgaagagcaggtacataaaaagtttgttcttacttggcaaagacatgcatggcttttggaacttgcaactacacagggtgtcacttggcatcatagagcccatttaggaaaagaatgacccatggtgacacgggctcgttggaaagggtcaggaaaggaacatatacagcaaaaggtacaatacagctttccgtagagaacactgggtatcattttcttccactcatccctcctctccaccatcaaagccaaacatttatataggtatgcattccaccctgcccaatgcattacaaatgccaataagagaggtaggactgttgtttccatttttttccttctaaagctattgaaagttctttgtctgttccttatatagttttaggaatacttttgaggaaattgcctttattctttatagtggatttcatataaagcaagttttgtgtttcttaggaataaaatttcaggcttctggaatattttttattttctctctccataaaaagataatttcaatttccctaaattactaggaatctactctacatggtgcagcaaaattttaaattatgtaatttagattactccagagtaaaacgtcttaaaaactgagagcacagcttaagtgtatggtctagaggcaagagttaatggcatggaaaagtagtaaaaggttggattagaaggtttaatacttttgatctctcagcccattgcagtttacttactccttaggagacacagatgggacacggcaggtgtgtgtaaggagcgaagcaattcatgaatactcagccatgaaatagaaaatcaaaatgaaataagtatgactgcaactatcttggtctattaacattcaactattaatacctactgttctttgaaagccattactgaatatttactgataagaaaaaaatgatagcttaggaagaggaagatgttcaggaaaagcatttaagcagggtttgaaagacttgtgattttcttaactcggggtaaaagtcgaccaattaaagtaggtttcccatccaaatgtttcccatccaaaatgatccctttttttttccccaagggatctaatttaggatcccttggaaaaaaattccaaaatgcattacaactattcataagggtgacacatggacctatttttctaaggactttgatttaatatttgaatgcaatggtatctgactttgttagtatagaatatttaaacttaaaaagaaaataccttaatttacttatgcataagcctattaaacacatttctaggggctctttttatgtttattctctagaacataacctatctttgaagtggtatattagtttttaaaaagtcattcctaagctgaataattaaactgaaaacaaaagctattcttagggtgtattccacatataaagctatgcacatgatgctttgattcaaataatatacttataaaactttgttattgtttgagttccatattcagaatggcaacttttgtttttgatgattattccatcctgaaacaatttcccccctgctcaattaaaccagaattaggagcacatttatatctgatgagacttaagcttctcaactgcctgcttcagaaatgtagacctttagtgcttgtgttcattttgtctctttgtggaaggctcaaaagaaaacagaatcaattcccttaagtttttctggaagaagaaggttggttttgttgctttgatcttagcatgttgtgcattttttattggctgttgaatataaaaagccacagcctcatctggtttttctgctatattctcatattgtaaatcacataatgccttccaatctaaagtaaaatgcctaagtccaaaatatcacttcaaaatggatttatcattatagttgatagaaagatttccagggtgtaagaaaacaattcaacagtttgattaatatgccacagactgctaaaaatatattcatgcattttagacaataaatttcaggatatagacatacactcatgctatttgagatccttttttcctaccattgcaagaggctgctttagctaatgcaacagctggctaggttattgcttcaacaatataattcataatgcaaaagcagctcttttccaaacattttagagcaactcaagttgtttacatctcctgtaggtgattttcctataactttgtgccaattggtgtcatactatttggtaaaaatctacattaaatcaagacaactgcacttggttaaatttctgtcatacagagaattatagaaaaattacagctgatttgaacttatcatcattaagtatatacagggttttagaaaatgaatgcaaactacaaaaatggagttgtataattaaacattaaatagtccaagtaataaaagtcatagattaattgtctctcagttctagtcagatcctttaaatactgtctcacgacttgagcattggttctttcatcggaagagtgcctatccttaaagttgggaaatttcagctcctttggagcaccgatcatctgtaaaaagtaattggcatcttcttccaaagtctcaaatttccctacaaaatcatagttgatcaaacacggatagcagagtttgctgaccttttcccagtgaatgtccattcctactggacggtgggaatccagcaagtagtggataaactctttgaacttgactccagatccattaattaatgcttcttcacaggcatttggtcgatatttcttgataattgcctttccgaatactggatggtaataactattggggtgttcaaatttgtccctaaaggctgatactaatctttccatgggatcacgaacaaacacagctttggtgtaagtatttaagcgggtatatatcccttttaggtcaaagctatctagcttcttcaaatgcttcccgtagtggacagcattgtgggagatgttgtatgcagaggaagccaatccatttagtaccatcagaattcttttccaattggaacagccagccttaggtacctcacaatataagattttgtgtttatcttctacatagattctggatactgtatgaaaaagatgtgactgatgatgactcaccccaccgtatttcttgcaaaactcctgaaggaaagaccttcgtttctcttgggtctcctcagttttcttccatttattatctttgactaaacttttgtttaaagggtgaatgtccactggccaattcatgttgctgaacttgttaaaaacagtcttagctccttgacgtttttcaatcaacttctctgttggtgaccctgtggacttacttaaagcttgatcccctccttgtgaatgactggtctttgttaagagcctagtagatctctcagaattgagtagaagattttcctttttttctcgtacatcctcaggcatgtgaaacttggggttcttgaatctagatagaagtgcagttatatttcttcacaccatcaaggagacctaattgtctccagtcattgataagataaatgatgggagagggtggggtgctcaaaagtcagtcttttctggggacacaggtcagtgtgtctctcctgggtccctctgtgccacagctactcctcttaaatcttgattccagggcttcagaagctgatggcatagttatgag

SEQ ID NO: 12462 - RNA, 8556 nt, Homo sapiens
  source 1..8556: mol_type = other RNA
cttagcaggttgtattatcatttataatcaaccaggacttaaaaaattcacacacacacgagaagtaccccaagagattattaaaaaggaaattttcaggtggttttcatagagattccaattctgtgtatcttggatggggtctgggaatatgtttttaacaaaaattaggttaattctgatacaggtcgtccatacactatttttttcagaaattgataagttaaatcagggcttattttttcctaaggataatcacagtcaaacaaataatattgttcttttaagttggtagacactctagcattctgagtgcatttttatttattatatagtacatccaaaaatcatttttctaaactttggaaatattttcagcaaatgaatgcataaaatgagatactgtgtgttttactagttttcctggtatttgaggacaaaagtcgtagttatcccttctcctgttttctccacctctctaagtatagaagtggggggaggagtaggaggagtaggaggaggaggaggaagaggagggaagaggaggaggaggaggttgtcagagcattaagaagcaagagagtagaatgttacagggggtgctacaatcacccagataatagcaggaagtagggtggagaggcatgttataaatcagaaagaagaatcttcggagaaggctgggaagcaggtgatttttagagttgaggaagcgggcacacctgcaaaacagaagagatttttggatgaaggttatagaacagcagtctagaggcagcagtgggagccagtttctgtccctagatactagagctccaagagcctgggagaatgactcatctctgcagaaagaggtgggaaggaatgtcgttgccaggggacccagtggctacgacagaaagatgccaaaaaaaggtactggatttctcccaacatctttgtcattggtcaaaagagacttccccaaacaatgaaatactgtttggagatcccactggatataggaccaaagggcaagcagcactgtgagcaaggatatggaaacccggaatgggataacctcactacctgcacaacacaaatagggtcaaggataatgttcaggagttgatttcctttggaagcttggcgggggaaggaatacactcttcagagcaggacttgaaaagtgagatgcttaggggccaggcaagtaaggtgaatgagtgatggtggattagtgaagagtgtgaacaactagagatctccaacctcatctaaagggactgaccttgcctctgtccaactattttcaggtgggcatatagaatgtagggtaacaaatcccctgtcattaatgaggcccaatgttggcagctaattcagatgttaaataaaatgcactgtcagccaaaccaaacatatctgtagccagatctaccccgtgggctgccaatgtatggtctcagctttggagccagagagactgttattaaacctctttgatactcagttttctcattcatgaaatgataggtggaaaaatactcgactttgatttttttgaaagctacttttggaaacggttagacttactcttcatgtcattaaatgaatgtatgcaaagtatttttcccgtgtctgctactgagtagatcctcagtaaatggctcttatgttgaccagaatcatgcatttttctcaaaattttcttccccaaacaatcaagcaactgctatttcttagaaatgtaaaagatttctgtgtctgcaactatccttcaggtcaagggatgactattagtgtagaaaaggtgtgtggctcagctcccttccctcagctgccctgctctagcaccttcctttcagatcctctggtcctatagatgcctgaaggtcacaggcagaaatatacgaattctacactaaaagaagttgtacaggaacctttaaacaacagcatcaaaagcatctgttaaagtaacgctttccactgagtgccttgctagacatggtacaaagtgcattcaacagacacagttcctttcctcttggaagacctaagacattccaatgacaacaacagatattttatattcataaaaagtgagataaatagcacatgaacaaataaattaacgaacctccctgacaaaaaaaatcgaggaaaggaatgcctgcatttattggtaagagaataatctgatgcatgttacaccaggggaaaactctgctgtctttttctgcctatcagggagctcataaagagatgagattttgaaattgaataatctcaagagattccttggtgagttaacaagaaatgaatgtccagatatatagagaggggagcattccaaatatagtgtgagacttgaggagaggtttagggatggaaaaagatgactgcttaaatggatttaaatacttttgcctggaagcatatgatcctggtgaaaaactaagatgtgactgactaggaaattctgagaatgaaatgatatgaggcaatgttctgttgaactccccagacctggccttcctcaggtaatgatcacaggcctgggaaatgtctgccatcttctagcaagagcttatttattttcacctggtttcatggtgttttttcagtcggtttaagtcagcttgctcctctattcttttctgcagtcttcccgtgtaggctcagggtaatctgactacaaactagtactagggaaggagactcaggaagaaggggataatgcacagttgctctgtttctagcaggagtggttctcactgtgtgtgactagcttgctgaaccgtgaccatctgcagtggctgtcaggggcctatgtgtggaaagttcgcctgaactttcttcctcttagattctgcttatccttgactggtcttgtagctgtctggaatttcttgtcaaagaaatgatattttgttttcacaaggctaaatttgttccagggactattttttcttcttaaaaacattgtttccatgattaactaaggattacaaaaaagttgtggggaggaaacctaatttcttccaaagtctttgaacctgtcagtttaactcagcaggaataaagaaataagctgatttgaaatgtgataactaactagctaaatacacacacacacacacacacacacacacacacacacacagacacccatatttgtatggaaaaaatttcaggattccaatatattgtttttgcctctacctatcctgaatagaggtaacggaaagcaaaagtaaatattggtttgtaatattctaagcaaagagtttggtagtggtatttgctgcttggcttcatcctggcttctgacctacttatcatctctgtctccttaggcaagttactcagctatagtctgctttactttcctttatgatagatggaaagggagagggctacataatattacctatgttagactggctatggagattaaattaatgcatgtaaactacttgaagagtgcctgacacccagtaagtattgaataaatgttagctaggatcatgcatacgattactgtataatgatcatgattgagattgagaaggtatgagcctaaatgtaggactaaattgaattagccttggcctaaggttctcaggtagttgagctataattaaacgcctttggccaatcctttttcaagtatcagagcatcttgggagggttagccctgggcaaaacatctgcttcaccacgccccatgaaggcctagaggctgggatgccctgagaggccacatgagaatgcacaggagggagacgtttactgtagtcctagcctaatcccaagttctattaattcagcaagtgattttttcaaagggcactctaatattcaaaattctctgcatcttcttatatataccttctgctaaatactatacattttaggagataagaataataatacatcaataaaatgtaaaagtatttttcctctttctaattaaaaatgacatacaagtagttcttgaattagaactactaattccctaatgataataatattattattttctgttacagaatgttttatagacatctagcaagtggcatcacatttccattgaattaatggatatttccaaatgtttgagaaaatccgaaaactggatgtcctgtacatacatttccattgaagtttatggcagtttctgggcacaatcacatcaatattgcacatctatagatagtttacaggttacataactgtggttttggatttaattgccaacttgttaccctgatagtaattccagacaggggaataacagagcgaaggggtctgcccattgtgttactgctgcctataaaaacaaataggatccttagggtttaattggaggacttataattgcacctaatgttaaaatgggaactttggacatctggaagatgagtctggatttggtcacttgcctttaggaattaaattcatgaaattgtgatggtcctaaagaacagtggtgttcccacctggatttatgcacaggcagaaatgacaaaggtgaatgtgagctggtctgcaaggccaaataagtcaggagagaaaaatggagtttggctttaaactcacaagtaatccaggatgatgactggcttctttggtcctaacatgaaaataagccatctaaaatgaagagcaggtacataaaaagtttgttcttacttggcaaagacatgcatggcttttggaacttgcaactacacagggtgtcacttggcatcatagagcccatttaggaaaagaatgacccatggtgacacgggctcgttggaaagggtcaggaaaggaacatatacagcaaaaggtacaatacagctttccgtagagaacactgggtatcattttcttccactcatccctcctctccaccatcaaagccaaacatttatataggtatgcattccaccctgcccaatgcattacaaatgccaataagagaggtaggactgttgtttccatttttttccttctaaagctattgaaagttctttgtctgttccttatatagttttaggaatacttttgaggaaattgcctttattctttatagtggatttcatataaagcaagttttgtgtttcttaggaataaaatttcaggcttctggaatattttttattttctctctccataaaaagataatttcaatttccctaaattactaggaatctactctacatggtgcagcaaaattttaaattatgtaatttagattactccagagtaaaacgtcttaaaaactgagagcacagcttaagtgtatggtctagaggcaagagttaatggcatggaaaagtagtaaaaggttggattagaaggtttaatacttttgatctctcagcccattgcagtttacttactccttaggagacacagatgggacacggcaggtgtgtgtaaggagcgaagcaattcatgaatactcagccatgaaatagaaaatcaaaatgaaataagtatgactgcaactatcttggtctattaacattcaactattaatacctactgttctttgaaagccattactgaatatttactgataagaaaaaaatgatagcttaggaagaggaagatgttcaggaaaagcatttaagcagggtttgaaagacttgtgattttcttaactcggggtaaaagtcgaccaattaaagtaggtttcccatccaaatgtttcccatccaaaatgatccctttttttttccccaagggatctaatttaggatcccttggaaaaaaattccaaaatgcattacaactattcataagggtgacacatggacctatttttctaaggactttgatttaatatttgaatgcaatggtatctgactttgttagtatagaatatttaaacttaaaaagaaaataccttaatttacttatgcataagcctattaaacacatttctaggggctctttttatgtttattctctagaacataacctatctttgaagtggtatattagtttttaaaaagtcattcctaagctgaataattaaactgaaaacaaaagctattcttagggtgtattccacatataaagctatgcacatgatgctttgattcaaataatatacttataaaactttgttattgtttgagttccatattcagaatggcaacttttgtttttgatgattattccatcctgaaacaatttcccccctgctcaattaaaccagaattaggagcacatttatatctgatgagacttaagcttctcaactgcctgcttcagaaatgtagacctttagtgcttgtgttcattttgtctctttgtggaaggctcaaaagaaaacagaatcaattcccttaagtttttctggaagaagaaggttggttttgttgctttgatcttagcatgttgtgcattttttattggctgttgaatataaaaagccacagcctcatctggtttttctgctatattctcatattgtaaatcacataatgccttccaatctaaagtaaaatgcctaagtccaaaatatcacttcaaaatggatttatcattatagttgatagaaagatttccagggtgtaagaaaacaattcaacagtttgattaatatgccacagactgctaaaaatatattcatgcattttagacaataaatttcaggatatagacatacactcatgctatttgagatccttttttcctaccattgcaagaggctgctttagctaatgcaacagctggctaggttattgcttcaacaatataattcataatgcaaaagcagctcttttccaaacattttagagcaactcaagttgtttacatctcctgtaggtgattttcctataactttgtgccaattggtgtcatactatttggtaaaaatctacattaaatcaagacaactgcacttggttaaatttctgtcatacagagaattatagaaaaattacagctgatttgaacttatcatcattaagtatatacagggttttagaaaatgaatgcaaactacaaaaatggagttgtataattaaacattaaatagtccaagtaataaaagtcatagattaattgtctctcagttctagtcagatcctttaaatactgtctcacgacttgagcattggttctttcatcggaagagtgcctatccttaaagttgggaaatttcagctcctttggagcaccgatcatctgtaaaaagtaattggcatcttcttccaaagtctcaaatttccctacaaaatcatagttgatcaaacacggatagcagagtttgctgaccttttcccagtgaatgtccattcctactggacggtgggaatccagcaagtagtggataaactctttgaacttgactccagatccattaattaatgcttcttcacaggcatttggtcgatatttcttgataattgcctttccgaatactggatggtaataactattggggtgttcaaatttgtccctaaaggctgatactaatctttccatgggatcacgaacaaacacagctttggtgtaagtatttaagcgggtatatatcccttttaggtcaaagctatctagcttcttcaaatgcttcccgtagtggacagcattgtgggagatgttgtatgcagaggaagccaatccatttagtaccatcagaattcttttccaattggaacagccagccttaggtacctcacaatataagattttgtgtttatcttctacatagattctggatactgtatgaaaaagatgtgactgatgatgactcaccccaccgtatttcttgcaaaactcctgaaggaaagaccttcgtttctcttgggtctcctcagttttcttccatttattatctttgactaaacttttgtttaaagggtgaatgtccactggccaattcatgttgctgaacttgttaaaaacagtcttagctccttgacgtttttcaatcaacttctctgttggtgaccctgtggacttacttaaagcttgatcccctccttgtgaatgactggtctttgttaagagcctagtagatctctcagaattgagtagaagattttcctttttttctcgtacatcctcaggcatgtgaaacttggggtttgattctgggtacaggccgcaagtacttcactggtccccatcctgaagttactttttgttctcttctcttctccactctccctgtatgttgttcttcaatccagacttgcaaatacatgaagaggagtagcccagctactccaaatatcagcacagagaggaagacttgtttggggttcatgaccatttcagatggctgcatttctccttatttcagaatctgaagaccacatgatttgttttcccgtaaaacttcagtcttttcttgttctctaagagcccaattccataaagtaacctcgcgggccgctgccgggcgcttgcaggtgctgctgttccaggagcgcagcttcggaggaaacttccccgcgctccggggcaaactcccgcgcactcctggcagccgtgaggtggctgagagcggagcgccgcgccgggagcggggacagctcggagtcgggcgctcaccct

SEQ ID NO: 12463 - RNA, 31 nt, Homo sapiens
  source 1..31: mol_type = other RNA
cttctcttctctccttcccagacacaaccgc

SEQ ID NO: 12464 - RNA, 32 nt, Homo sapiens
  source 1..32: mol_type = other RNA
cttctcttctctccttcccagacacaaccgcg

SEQ ID NO: 12465 - RNA, 465 nt, Homo sapiens
  source 1..465: mol_type = other RNA
cttctcttctctccttcccaggtgaccatgcttctctgtcccagagggtgcagcctgtttatttcaacaaattccctttgcacacagttctgttttgcagtccagtctcctttatgctgacattgatctaaatgctttttaggcactagtagggacataagtgactttattttaaatgctaatctgctgactaaccccaagtctgggaatgcctccaaaatgtctaggtgatgtattactgtttatgtaggaacagttattcattgtaagtttccctcaaaacaacccttgataatgttgtagaaatcataggctgtgatgcttatagccacctacatattccttccagagtatagatactttttcctcaagatacacatcctgggtctgggcgattgcagtgcagagatttacctgtcttgtagccagctgcctaagaccaagcttctgtttgtaagttccccc

SEQ ID NO: 12466 - RNA, 27 nt, Homo sapiens
  source 1..27: mol_type = other RNA
cttgccatcctggtccactgcatatag

SEQ ID NO: 12467 - RNA, 25598 nt, Homo sapiens
  source 1..25598: mol_type = other RNA
cttggattttcctgggcctcagtgtcccatctatgggataaagagggagaactagcaggtgttttaaatacctcctgctagtctcaccttctgggatctaatctgtggctaggctttacttaatttggcttaaagcacatgctgtataaaacatgtcctgttaaaagcattttgagtacagtattttttgttactttgcttcattcgtttgtttgtttttcaaattgccacttaccatttttagtacaaattccttttgaaaagctcccactctctccatctctctgaagaggggcacctgggtgtcatgaatacacctgtggcctaagatatggtaatggagggaacagaccaggttctgagtggatgaaaatagctcaaaaggagatagcaaggagcaccaagaaaaaatttgctgggaataggagcatcttgttagatgcatgctgaacccccgaactcagtttatccaggtggaggtcccaagaaaccaaatgcagctcccttttttacagttctgcatatgtgggagctgaattgcatactgatttcatcttgctgaagtgcacattccccttccagtaacagcaatctagcttcctattttggggtttccttccccctaccccgcaccccattagcccctgtctgtgttctctagccctgaattcagatgtcccagactggtcaaataatggtattctacttccctgtcacaaatggccatcatgtccagagcttttgtccaaagtgctagggaataagacactcttttttctgttccagtcaaacacaggggagagggaagataagatgtaaacttctggtcaccaccctgaaactgcatgaagcttaggaatgaacagggaaagcacatccaagagatggtgacatctttgaggtactatcaacctgctcctggaaccagtgtggtttttaagtcacttgaaccaatacatttttttaaaattacttaagccagtttgagtttcaccttctgtttctcaaagtgaaaagaacctgcatacaacttcttgtacatgaatattgatatcacttcccagatttgggacgttttcagctattatttctttagataggctttgtgtccctttatctctctcttctctttctgaaattgcattatgtaaatattagttctcttgatggtttcccatagatcccatagacttcttttattcttttttctttttgttccttcgactggataatttcaagtgtcctgtctttgagttcacttattctttcttctgcttaattgaacctactgttgaagctttctattgaatttttcagtttattcattatacattataaatatatacaattattatttatcaattaaaaatacattttaaaaggaacaaatgccatataaataccaactccacttgacttatagtgacttcctgaagaactatattgggaaaaaccctggggccttgtctgggctcatgactcatgaggaaggtatgcaggaagagggaaaaggtgaaaattgagcattccttgactaagtcgaaacccctgactcagtcttctgcctcactctggactaggcaatgcttcatatatctccaaggttggtctttcaggttggcatataggaaggaatttgtcagcatgtatccctgaagggtaaatgtccacatttgcttagatgtttagtgggtattccaaccctcaaagagctgtgcttggtgctgtaaacaaatttgttcccagtatctgacctaagagaacttatactcagaaggaggcatctgcttcctgcttcaccttgaaggttatgtactccactcacttctttgacctcaaataatttgtaatctgcaaatagtcaaagtgagcaatgatgccaaaaagcataatgggttatagaggtaccatttacaaagtgtataaaacaggacaggaagtgaatcctagggatggaagcaatggaagattactcccattatttttaatctggttttcatggttccaccaacctgggcaagctaatctggttaactgagactcttcttgatagaacttttattggttctgactccacttgacatcctcagaaaacaaacactgaataagaatgagctacttttctggaaaaaaaaaaaactattcactcaaagcacttaaaatcaaaacacacgcaaaaatatattactactcatttgagggtaccctgttatgaaggtataatttatatataataaaattcattattttttagttacagagttctatgagttttggcaaatgcattcaatgccatcactactacaatcaagatatagaacagctccatcacttcaaacaattttcttgtgtcttttttcatcaattcttcctccaactcacagcacagatctgtttgctgatcctgtagtttttaaaatgccatatggattatatacagtatgtagcattttaagtctgacttcctctaattagcataatgcatttgatgtaactccaagttgttgcatgtattgggtgctcatttctttttattactgagtagtattccactgtatgaatacaccatagtttgtttatccatttcccagtttgaagacattgggttgttccaatttctggcaactatgaataaatccactctaaacatttgtgtataggcttttgtatacataagttttcatttctttgatataaatacctaggagtagcaattctggatcactttgtaagtgtatgtttaatttataagaaactatcaaagcattttccaaaacagctgtttcattttgcattcccagcagcaatagccacttttatttttcaatgtgtggaatgtcatttttatatagatttggcccactatcatatctccattagggctcaaaagacttcatgtctgtgctgggagcaaagtaacctatagataccactcgatcatttttctgacatgagacttacagagtatcatctctagggtgatttttgaaaaacacataaatgcagaatcttggtgtttaaaaggaaattagaactcattagttcaacttctttaagtaaggctgttttgatccaattataatcaattttcactcactaaggccctgcttaatagcctattttactgcccgtgtgaacttgggtatgttacataactgccttaaaccacagcttcttcatctctgcagggtttttgtaagaacaagagaaaaaaaatgtatctgaaatcagaaagcaattaaatattgtgctaattaaaaaacagacattgctagtgactgttctaaaaacctaatagcacaaatcatgtgattactaaatgttagaactaaaagaaccttagagatcttccattaggtcccagctctaaatgatagacttagtgagaaaacggaagccctggaaagccaaggtaaccccactcactccctattacatctccttgtcttacttttatcatagcactcatttttctgctgtttctctgaccctttgtgagttaagatctgccagggtagcaacctccatcaactacattgcttagaatgcagtaagttcttaataaatgcttgttgaattatcattttaaaagtgaacttcaattagattattcatacacaacaggtttgagtacatgacagataccttttttgacaaattattaagccacttgttagggtgacttgtaggcatcataataagccaaatcagagcataagaattgctcagtcaaccaaatgtgacgagcctaaatcccattcccatgctgtaatctcccagtcctgttctgtcttgctcctccaagggacacgttgtataaacagcatcaagtgttaacttgttaaaacagttacacccaaaaaatgctgagattatttaacaatgcaataatatgaggtcatatcaagaattccaaggagaggcagagttttcaaagactccagttcaatgccagggagctattgtttctaaaatgatttttggaaaatgaaatattaattccccagctaatgtatttcatggtagttcattgtgcttaattctctaatctgaaattctttattttagatccattccaaaatcatcttattagtctcacactttagaagaaatgtgtaaatcaaatgcttctaaatttaatttgatttaaattattttaaccactgtaacccctctgtggggagaggagaaaaagcacatttttgccaatggtctttgttctgaacaaagattggttctatctgtcaccattgggaatgttcaggaatattctcattggattgcaagtgccaagaggacaagaactttataagtttttttcattgatctattgctacagcctggggcagtgccaggcacatagaaggaatctaacaactatttattgagtatgtaagtaaacttgaggagataaggtgttgaaactctcccaggccttattcatgagagatcaggctgagcttccagctaacatttctatcccacagcagacctgcatggtctttacatctatagtcttgggcatattccataagacttccacatatttggctgggtttctcacctatagcattttcaaagagtctcactatatataaacactgaaataactaagtgccaggaatgactacagaaacaaagggaaaccttataacgagtgtggtggagtgattcagtgaagatcatcagattaagactgagaagaacaaagctgtggtcactctcccaccacttaacaagcatgggaagctcaccaagtcatgtcctcactcgaggcctcattcaaaatctgtgtgtgtgtgtgtgtgtgtgtgtgtgtgtgtgtgtgtgtgtgtgttctttagatcatgaaacttctcatctgaaaatctccactctgtggcccagagtaagcttacatagtgagtgcacctaaaggtgagccatctccactttggccacttctccagatacccacaaggaagtgccgagaatgctgttgcacctcctctggccaaggacagagagtcatatcatctgcccacttggagacagagaaggtgacttacctaatatttttcctgcatgtcttaaggacaaggctgggttcttttggccttactgggtaataaaaactctatgcacacaggctagaagttgagtggtggaagattcaagagaacaagctagattttatgaaaagtgggtaacaaagcatctttactccttctcccatggacatgaaaatcattatcaaaaatcctaccccagatgggaatgttatctggtcttgtaaagctgccttactatctagtccccaagatagccccaagtgaaccaggcttcccagtgctcatgccattgagtaatcccctcctataccagctctaggctggctttgtataaccaataaaatatagcagatgtgacactgtgtgacttctgaggccaggtcataggaagctttgcagctccccgtttaatctcctggaatgctagctcttggaatgcactctcttggaaccagccaccatgctgtaagacggccaagccacatggagtcgacatggctcacggctccagttgatcacagccccagctgagctcccaaccaactgcaagcatcaactgttagccccgtgaggaagccatcttcgatgcccagcccagaggagcctttgatgactccagctctggccactattggactgcaacaacagtagagaacccaagcgagaattgcccgggtgagcccagtcaatccatcagaccaacagatgatgataagctgttttaaatcagaaacttttggggtggtttgttatgtcacttgttccacctcatggttcaaaaacacgatccccataactttaatgtttaagggttatcactttgctttcttctttggatttgagatgtcatttgcaagcaaccttctctctcactcaaaatgtttcccttatctggtctagttgtgccctactgagcccagacatgaaggaaataaaaaaacaaccaccaaccacacactcatataacacacacaacacacacaaaacaatgtcttggattgtggaagaatttgctattgtcattgttttttaacgtattttctttatatttccttgagttccttttggagtcattgaattccctttttgagtcttttttccaagattacaggctcaagtcatgggttttaaaaatagccataatctattaacgacctattacattccagccaccatgctaactgctttagacatattaattcattaattttacaataactttgctatataggtatttattatccccattttacagttgaaagagccatagctcagaaagataaagtgatttgttaatgctacacagatactaagcactttgagacaagatttgaacctaggtctaccttaaccagcataaatatggctgaggaatatctgaattcattcacatccagaaatcacattgtagttgttgaatcctttggcaggagctataccttggtcagcagaactgtgtaccttggaaaatcactctgaaggaaggacttacatgtgagttttggggattgcaaagtgttgacattttcagaccacctatgtatattgctgcagatgttggtacaattctgtattgtccggtttgcactgataataaaacagtctgataaaatcttatgccattcttccagaacatgaatactggaaccactcattcaaggggatctggagagtgacccaggatagagtgagtcacagggacccaagagcttcaacaatctggtattcagaagcagctggaatgaacggagagagaagaactatatagcaaccaggacatttgggaaatgtccctatgaatcaatccacctgcactggggaaaaatgagatacataacagaaaagaatgagttcttggggtgtggggatacacaagtgtgtgcatgtttgtgtgtatgtgtgtgtgtttgatggggtgggggctgcttcttttctaggagtcatttccaagcaacctctcctctcactcaaaatatagctcccttaagccagttttccctgctttctctcatgggtgaaccatcctggggaaactgagatagccccaaagtaggtttcatgatggtatgctctgggtgcgctaggctactctgttttgttctttctctgatttattcctgtctctgcttgcacttgcagttcctttctcctactaggacattggtcatttaaaatatattcatagtaagatgacaaactgttcctctttagaagtacagatatatgcctctctgagccttagtttccttagtttgctgtaaatgttcacacctcccatcataagcaagctggcctttgtcaacaaacacacatacccacacaatgttgtgctgccaagtggttcacaggagaggatttgaggggaagaccaggttaacctaaagacaaccatgctgatgaagccaagtcaggagcaaaaggagatcagagcagcttggtggcgaacagcatgggcccttggaccagatcaattgaatgcaaattctgcccctgctactcacaagctattggacctcaaacaagttactgaacttctccaagaccttgtttcctcacctataaaatgggcatgttaataataccacccttgaggttgttgtgaacacagaaaatgaaatcatgcattcaaagaatttaatccaatgctttatacaccataaatgctcagtaaacattagctgtgttatttattatagagtatacaggatacaaaatataatagcaattatatattaaatatttgcaataagcaaggccctgagttaagtattctaagtacattatctcttttaattttcacagcaattctataaggcaagttctgggataacccatttgacaggtgagaaaactgagacccagagaggttaagtcatgtctccaaggtcccaaagctatctgactccaagccctgaggtcccagccaagttcacaaacttcatttcccaaaacccagaattagatcacttgttgaacatctgttgacactttccaggggactttcaaaaccccaatccctcagaagccccaaaacgtttaatatgaccctttaaaacaccaggaacattcacagcaaaagaccaataactacacatggggtagaaattaacatatgtagaggactttttcttctctatacaaaagcttttacccatataccacattggatgtgagagtgaatatactgcaagaatgtacttcctgcagctgaaaccagcagggcaaagaaggtgctttcactagggtaatgtgtaccccttgctgtgctctgaagaagagggtcaatttctttgtggggagtagcaacacaaaccatccagccagcaattaaatctacagttccctcaacaacaaagctaactttagccatatgggctcatcctgtatttcccaggacccaggagtctttggaagtttcttgagtgggcttccaccttagcttttgctttctgtcagataatacagtggttatatctgaagggtttcccccaggagctccagttcttttagtggtagtaacatcaagtagtctccagacattgcagctgggtggttgaaatgcttgctctgggaggggtggccagtcagctggggtcacaaaagccttgtaattagaatcagtgtgactaatttccaggtagaatgagaggctcttgcaaactgcttttgtagaaattatactcactggtgtccaacctgccctgaatcactctatactcacaacagaaacagctggtgtcagagaactctacaaatatggcagatcatcacatgggactttatccatggaggtgagcctcctcttgcactggaagctggtatgctgatgatgtcatggtggctcaactttcctggtgtctaaggggagtgtcagagagcaaccctaacatgtgttgggtgaccatgggtaaggctttcccttttctggttcacttttcatataataacaacagagctgagctagagggtctccaaagcccaccagctgccactttgtatgacataaaattatcagaacatgaattcaatcactaggtaataagaggtaacaattgaacatttagctgtttcatccaacagccctatgaagttgatatcattaatacttccatattacagatgcagaaatggaggcccagaatggttaagtgccttgcccaaggtcatgcacacagtggggatttttacccaggtagcataatcccaaggtttatgctcttaaccattcataatattaatgaaaacactaagaaaccaacaatgcatacaaagggttccagatcctgcttttctggatgtctccatttttatccataagcagtatgtatgtcagttctcaggcatcacctggaggatacatatataacacctacctaagccctagcatgtcaaccctggacaggtcctgacagattaccgagactgaggtttttaactcatcatccttgggcgtgcattaaagggtccatgaggcctttgaaagtatgtgtatgggtgtgtatacataattccaagaagagatttcattggttttttttttttttttttttttcagattttcgaaggggtctatgaacttttagggcaatcttttgacagttggtaaaactgagacctcaggtgggagatggacttgtcccagtatacacaaggagtgacagaactaggttcagaccccagatcacctgaccccaatcccactgctctttaactacatcacactgagctaactcatccctgcaacatgcaccaagagtcttccaggattaaactgctgggtataacatgcacagctcatagggtttgggtatggcttggaaaatcatcatgcttcacatatatcattgactttaactttggtcctctgtatctcatcatttccttgaagtttgtatcattgatagttacctctgatctgccactctgcccatcttctgtgaatgaaaacttagcccacagcgtttcatttagatctggtctgggctgcctttacctggcctcactcctggcttccatagacgcttaaggtgattaggcatttgtccctcaccgtttcgattgaaataatcagttcaaaataaaactgacaacagctaacctacacaaagaatgtgttaatgagcaaacattcacaggggaatcaaattatcccaataaaattcaaatcaatcaaatttaaaccaggaaaatttgacttagtagaaataaaactacgatggaaaattcagtggcagaagctaaaatttgacctaaataaattattgtcaataaattataagccatcattgtaaaattccaaatgcaaaagaattcatctccataaaatgattttgataaaatagaagatggaaaaaggtagaaattgtttaactgctctgtattgaacatttatcttggagtaaaaatgattgagtaagcattaattaagaaaatactttcttgataaaaattcagccattattggtgtttttaatgttgtagttataagcatggagtcaaaacaccctcagcaatatatcacggaggtcaaaacgtctgccagactaaacataggttcaaaatgacagttccaataaagggaggtcacaacttcctgtgactgtgcttggtaagtgatggaggcaatcatttacagatgatgctctgacaagggaggcagactgagaccatcactgtcacatgctcacttgaatagccaagcatctagcccagattacattcctctaagcatgccttaaccccacaggttcaacaaagaagtgttcattaacttcttcgcccaaacaagtactcttctgaaatgtctgtcaacacaataacaataatagccaacacttatataacatgggccaggcactttacatatattcacacatttgatccacacaacaatcccatgagataagtactattatcatctccatttgccaatgataaacatgaagcaccaagagcttaacaacttgcctgaggtcacacatttcataagcagtggagctgttcagtctactaccatgcatcccagacaggatgttcaggtgaacaagatctatctagcttaagttccataaaatttatcaaaatttcagctgaggttttatgcaatacttgcaatatagataaggcttggactggtgtcctgaagctgccactctctatctacaggactttgggtaagattaatctcttaacctctttgaactcatttcttcacatgtgttatgtgaataactatacaatgcaattacttcttgcaggtaggagaaattaagagaagtcaatgatataataagagtataacctttagtacagtgtttgaggtaaaagtgctcaaatctaagctgtgatggtaagaataataggtaagtttatcagaggactctgacttgccctggagcccataggacttatgaagacagggactgtcattatcttgctcactggattgtgagtttagcacatgagaggtgttgaatattggttagttggttgtttcattggttgggtatgtgggtggttgggtggttagatggttggttggttggttggttggttggttggttggttggttggttggttggttggttggttaattggctggttggataaatgaatggatggatggaaggatggatggatggatggatggatggatggatggatggatgaatagatggatgaatagatggatgaatagatggataaccgtctgcatcctctgtcccaaaggagctaaactcagacttttcttcctagtcctttgcatatatgcatccaatctcccccaaacagactgacagatactcaagggcaaggatgaggtttttatccacatcccacaataccatgaacttatgatttcccaaggaaagagacttgggattatgaaacaatactctggaccactcaggcctcaaaataccttaaaggtactgcctatcccctggatctttattccatagaacattcatcactgaagggatttcctgtggtatttggtgcaataaggcttatataagccaaggtccctgctccctagattttctatcatccctcctccttaagacaaagggaaacattcaaatgttcaaaagagaaatatttatcttgaagatcctaagttctgaaagagaaaacgtgtatcagaattacataattatataaagcactgattttccaggtcagacaaaagtgattttgaatctctgcaaacatctgaaatactttaaaccttgattctatcacctgaaaaggggagataaggtcaccttctttggaggatcatttggaggatcaaatcctatactgtgggtaaattacttagcacaaccatcattacagcttcagtaaaagaccatgattatccctggtcaaactactatctgtttgaaaattaagaaaagacctaccacagctatagcaacttattctaaacaaacaaaaattatgcttattattctcaataaacttttgctgaatacctgctatatatgtgagcagccctatcacctgatttctcaatcactcatgagcaataagtagttatattatagttttaaaactttctccctgaaggtcaaaacccaagtccaacatttcattcctttatttttttattcacccattcaacaaatctttattgagagcctgccatgcatcagacactgggctgggctccagaaatacagagctgagtgacccaaataagattcctgttttcatggaacttctaatctaggtggtgcacatggattattaaaataaaaaaactcacataaagtacacttttaaactatgataagtgctttgaaggaaaagtacagggacaaatgagcacaagcaaaagggagatgctaaggacatgaggaaaaagaaaaaagagaccaactggccgggtgccatggctcacacctgttaccccagcactttggaaggctgaggtgggtggatgatttgagcccaggagtttgagactagcatgggcaacatggtggaaacccatctctacaaaaactaccaaaaaaaaaaaaaattagctgggagtggttgtacatgcctgtagtcccagctactcgggaggctgaagtgggaggatcacccaagcacctgagtctagaaggtcgaggtagcagtgaaccatggccaccccactgcactccagcctgggcaacagagtgagaccctgcctaaataagagagaaagagagagagagagagaaacagacagatggactttatacaacttggaaagaaagaaaagaatgccacaggacttggaagaggatcagaatatcagtttatataagctcttaggactgtaaaacaaccggaaatgaaaatcctccaagtaatctttctgtttgctatcctttccctccacccactacagccccaaagctacatgttctagaacagacaaaagttagttttgttttgttttatgaataagtagctttttggtcaccaggattaccacgcagctgttatttcagcctagcccgtggcagctcccctgaggaggaaagcagatgtagccattgtcactgcttgctgtctggtacaatgttcaaagaattcaggggcattcctatgaatgtctctatgaagtagatgtcagatatatccccagatgaacaaacatcagaagttctctatgtgcaagaaagttcaataaccaaaaaagtcaccttcacacatatttggcccgtgcaaggaagatcaagtagctgagagtcatacagatcatgtttaactatggtccgctagatttggaaggttaaaataaaagacagaagcgaggtatctattttcaaaatccttttcatagataacagtaaaatgtgtgaccctaaataaaaatacagtaaaatggaaggttagggaagtagataattaagcattcctgaatactaagtgagtaaaaaaagtgctactaccaacatttatgcataagaaacaaagcatctgtacatgaacatgggctcttcccaggctatttgttttgcaacacatatttggatgagaaggatgttcctaatagctttttccatgatgtcaaaagtaggctattctctcatgttcatgatcttccttctgctaccaccattggagctacgggtactatgatgggtgagacccacgaaactccacctggctgcttcccttcctcagatgtccatagtcttctacgattggctctggagtctcttgcaagtttccctcattcacctcactcccaacctggaatcttcttcaaaacataacttactgatcttataatttgttttgaccaatcactactataggtcaaagctttctgttcctccttctattttccatttgggaaatgcagtctctctttttttctaggctaagttacctgactgtggtcaacaataacaccagtatttctttttcaagacctcctggaaagtcagttctctccaatcctgttctaaagtaaccaattttgattgattcaattacaccagaatgattgtgttgatttcagcccagtatttcaggctgatgaaacaagttttaatctaatgcttctattcatgatcatattagtgatagcatttctctcagagatgtgtcacctgacagaaacacaatataatataatggtttcatttcctagctccagcatcagaggacatgacttcaaatttcacctcgatcaccactaactgtggacttagacaagccacatcaattctctaaacctcagtggagataaaaataatagtaactacaccaaaatgttgtgtgattacatgagagtcatcacaaaggttttgcatgagacttaatgcataaaacacattaacctcaactgttatttttattttgagatgtacacactctctggtctcaaaaagaagtaagatatccatcaaataatacatagaaaagaacaaaggctggagccctcctgcacttttttagagaccaccctccaggtcagcacttttcaaactacaggttaatgagtgagaaattcatttggtgagtcataaatttgatattttttaactagaatagaatgtttttaaaaatgaatagaacaaaacagaatgtatgagtgcatttctctatgttgttgcatatgcacaaacatatgcacacgaggataaaccataaaatgcatttcttactgtgggccacaacaacaacaacataacaacaaaaaaggatttgacagccactaccctagtctgattcagaactattaatattaaatacgttctttaccaatgatacactatttaggaagacatcactgccccctactggaactcttggatttctcacagaaaaggacagcaatggattagcctgtcttctcattagccatgtgacttcaaccatcctctcacctaccctgtctggaagttcatctcaaagagcctcatccctcaagctagtgtgatgccctggataaggagtcaaaggcagcactagaagtggcagctgggttctcacctttgaaatcgttttgaaagcacagcatccttccctctcacctgcctcgcagtctgtactgggaagccaagccaagcagccccactgtgcagtcctggccacgcaagttattcttgatcctgcaccatggcagctggggagaatccccaccccctaagcagtcacttgtctctgcttctctggggagaagacaccccttagaggagggtgaacgaagtgcacattcccagagccagcacttccagcagcctccatcctcaagtcccctgagttctggaataatcagacagagttgggagagtgagggggtacatatcaggaaatatatgctgtcccaccgaagagggaagaccgccaagtgagaggcccagtagcaaagagcacccctaacatacacaccctcccgcttaacggtgtgggacccaggaatagatgtgcttattaagaatctactcagttctgcttcattgtgacagctaccaccaattgacattcataccaagccatccatacatctcgtctcaattaaaagtctgagcagaggaataattgaagcttaaagaggtaaagtaagttgctcaggtcactcagtgatgaaaaggagaaagagcttcagacccaagtgtccctgaatgcaggaccagggtgcctggccacacctccaggtttggctgcacttctcaatgtcaaggcttacatgcctccaaagatggatttcctttttagccatttccttgtctatgacataagtaagtctgatataattctgacagccctgggctcagggaagttaattaatttgcagaaggtcacacagctagtaagaaacagattctaacctaagtatgcccaactccaaaacacattacattgcccccacctgagctgccacctgagtgagtgcagagcccattcccttgaatttcttccttctttgccgcttgtccacacatctcaatgggagcaattaaaagaggaaaagagaccaaaactgacaaggtcatgaaaaacaaggaaaggcagaaaccgtcatagaccagagatgcatagggaaatatggcaactaaatccaatgtgggatcagaagaacattagtggggaaaactgttgatatctgaatcaaggctggagtgttgtgttgcaatcgccaagtcctaatgtgttttctaccttctccactgctgccctaatctagtctcatgctgcttctagaatcatctttccaaagcacaaatctgaccatgtttctttcaactgcttataatccttctataccttcccctcaacctccaggtagaatccaaaccctctttgcttccctgaatctgctccagcctcactgcactcagagtgacctgttctcagaaaacatcaccccctgtccaccctctggacctttgcttgacacatgcactgtctgtcaataccaacctgctggtctgcagttagaattaagtaagtgtccctttcagaactcagtttggatatcacgtcctccagaaagcccttcctgatgcccgtaaccctgtctgggtaaaatcccttccccgcagtgcctgtaacatcctgtaactaacaccaatcacaatgcttctgatactgaatcatattacataatatatcatttgcccctttcctgtcacccagctgaatccccacttccctgaaatgtgtgcccaaacctggcattgaatgacactgaccctcctcagaaggagctcagtcctcttccctgcttactccatttctctgagtgtgcaaggaaaaagtggttgttgctagtctgtcatctacactctctgccacttattaatctctctgttttcaaacaatgccagataaggcctaggctgggtgcttgcaatgagcaacaggacctagcttgaagttaatgcattattttattttcattgtatttgccattatttacataattctgtttatggaaaacaatacaagtttttcttctatatagactagtcatcccttataaaaataagttaatatgagtaaaagaagtaaatcaatttagaaaatgttttgtaaaggctctttggtgcatatcgtgataaatgcatgcatacatacacacacgtgtacatatacacacacaactgtgaaggaagccctgaacagcagaaatcctgtcatttgtgcaactaagtccttgagtcatgagacccccgcctcaagtaccactgtctttgccactaactaccaatgtgtctgggagaaagttacccttctgttcctcagtttactcacctgtaaaaagaagataatataattgagctataaaaatatattatttcatctctccaatactatttctcatcctattcatacagtataaaaatagcactgctgaaaaacccagaggtgaggttcttttatcagaggacaaatatctgagatgtgtagaggttaagtgacttgcccaaggtcgcactgcaatttaatatcaaaatcaagaccaaaatacaggttccctttagtgataggcttcctgatccctcatcctaacaccctccattcctgcatattcccttccccaaataaacttctgccaaatgaggtgcattatatttacaaagaggaagaaaatgaacacacacacacacacatacatatatatacacatgcacaatataaaggcatcttaaaataatggaaaagcaaataagaaaaggacaaaagcaatattggatttcagaatgttaatactgttggacagggaactagtatacctgaaagctgagaaaacatgttacagggttttccacaatgttgcaatgcccttcttgttctttatttagattagatgtaaggagccagcagtcacacagcccatataagatttgagggaacaattagaataaagagggtaactagatcatgtttggctatgatacacttatttttttaaatgtttaagtagagaccaaatccaatcaccactttactctctgtggatcatgaaaaaaagacagcatcaacatgtttccaaagggaatagctggcccacatttcaaaaatgaaaattttaaacactttttaaaagagttttagcaagcggtttacatatagaatgtagtaattgcaattatatagcacaatgtttttcttattttaaaaaaatagtcttacccttgtctttggaaacatgctaaacatttttataactgacctggttatgggtaaattcatcagatttataggtaaatcaaagtgcacagaattgggaaattttagctaaaatttccaaggagatgtaacatggatagaaacaacgctcttcacgtatgtgtgtgtatgtgtatgcatatgcaaatgcatgtgcatatttgcagcaattgagaaagatctgtccaaacagaagttcaagtcagaagacacagaagtttcaactgattataaagctcaatggaagccaaggacagatgtggctgctggggagaggaagaatcaaattaagtatagtaacatccctctgtactcttcacccaccggccaatatcaaaagcctcatgcagttgtgggaactgctctttcagagaaacagaaacaaatctggccagaggagagtgagtggtcagtgggaaaagggaggggatctgtaacctgagtcagatggggaatggccagtggcatggtttccagggctgtgtgagccttcttcaaatacacgatatgtaactgttctggaatgtgtgtgcccctgactgtctcccaggaatgttgttgaaaggactatgcacgggagattagactgaatagcctcaaccgcaacgtccctcccagcttggggcttttacagcttgtggtgggggcaaaaccacatctattctccatggtagtagattagataactttactaattagacaactggaagcttctccttcctggagaatactctctagagtagacagccttttgacaaccaaccacatctctaagagaaaatgtgtgccaattagtagacaaccttgatgactagaagatgcaatggcggctcaactcaccactcccatctcaccctttcatacaaccaatcatctggtcagcccaagaagctagaaattaagggcagatggtctgataataaaagctaagctgatgggcatcagatgcagggaattatggctggtatccttgtggttcacagaaaaggagcaagggtgaaccacctgcatcaggcttgcttgagttgctttctaaaaatgcatgttcctgggatacatcccagatctactgaatcagaattattagagatagaaaccaagaagttcatgttccacaacctcaccaggtaatagttatgcacactatctgagggctcttgccctgcagtggtgcttcccatactttagggtgcattaaaatcaccaggaaagcttggacgagtcagcgttctgggatccagagattctgattcagagatcataggtggggccacagattttcatttcaaacaatctcacaggtgatgctgatgctgctggttagtggaccatattttcagtttgctgaaattagagaattcccaatttcattatcaaagaactcagatactgtggtaggtcacttctgaaatgatccccaatgattcctcaccatctggtattcaagctgttggtaaacactcccctcttgtgggagctagacctagtgactcatttattatgaattgaataggcaagactaaggagatgtcacttctgtgatcaggttatagaaagagtcactcccttttctcctgctcactctggttcttgctcctcttgtttgctccctctagtgaagcatggtgccatgttgtgactgccctgtggagaggcccacgtggcaagtggctgcaggaagcctctggccaacagctagcaaaaaactgactcctaacaacagctgtgtgggtgagcttggaagcccatccttctctagttgaagttgagataactgcagccccagctgattgcagcctgtgaaccaccctaagctggtgggctcagctaagtcatgcttggattcctgcccttcagaaaccatgagattataagtgttttaggccactcagtgtgctatgcagtgatgttattaatagagatgctttgtaaagcagctgccctgaaatcaataagatgccttgtagttgggtatggcacatgcctgtagttccagctactcaggaggttgacactggaggatcacttgagccccggagtctgaggtcgcaggaagccctgactgtaccactgaactccagcctgggcaacagaggagaaactgtctcaaaaaaaaaaaaaaaaaaaaaagacatgtattggtattctctcccatccatcaagtcctccatctcatctgcccccattgtggatgagacaaaatgtgtgtgtaaatgtaactggacaatatttaatcatatacactatttacatgtaatttatgtcataattttcttaacattcaatttccaagcctttgctcttggaaagcttccctggagcttctgggaggttatgtgggagcacagccttatggcaggaggaagatggtgaatccaagtcaggtttcgtgcaatccatctggccattctgaggctgtgtcttttgagctaagatcctggtgaattctctcctgtcaatccctgtgagcatgaggagtgatacatactttggttctgaagaaagaaatggaaaaaactacaggttcctctgctggcaaggggaaggggtctttccctgagaaaatcggtgaagagcacaaattccaatctgcttgcctttgcaccagtgcagtgactgatttcctcattgggggaggaaggaaggctcctggagggcaagatccctcatcttctccagaattatgtatggagaaagtgcttttcagaggctgtttgtgtggaaggcaacagtcaaccggtaaaggctccagatgcaaagcctggaaccaggaattctcatcgctgcaccatcaaatctttctgtggcctgcaatgagcccttctcctcctggacttcattcttcttcttgtgaaatgagggggctaggccaggtaaggactcggaccctcccaatgagtatttaagagcctagggcagtggggtcagagtctggccatgccaaatgtccagagacaggacagctttcctcagagggccaggccaccaccactcagccaccgcgccctctctgaggagcacccggagggcctgctgtgccacagggggctctggcagatgttgtccagcctgctcctaatggtgtcctgaagctcctcatcacccagcaggaccgctgctgccagggccagaaggaagtactcagtggcatcatgggcatccttcagctggcagaaggtgagtctgcccaggcgataatacaccttggcatagtacagggcctccttgggactctgcagccatggtggacagagggacagggtcttcaggtagcagtcctcagccatctcatacatgtgcagggagtagtacactgtagccaggcggtgaaaggccaccagctcttgcctctgatctcctgtgactgtgctgagcctggcggccagggtggcaaattccaaagccttctcatagccttcgaggctaatctgcagctctgtcagcttattgaaaatccggagctcagttctcaccgccttcaacctccttgctaaaggaacagctccagctcggtagtactccactgcatgatgcctgtggcgggtcccattgaagaacacatcacctgcttcttcataaagtttgagagccagcaaaggctcctctgacttcagggctgtctggatggctgcctgcaggcacagctccaccagctcgtcttcctgcatgaggtagtggagtcgccccgccccaagccaggcctcagcagccttgtctgtctcccccaggtcaatgaagatacgcaggctctccttgatgcatgtgagtgacctcctgagggacctggcggtatttaggttccgataaagctgccccagggactccagcagcctcccttccatctcccggtccctgagttgctgagccagggccagccagtgctcatggtaggtgatgcatgcctcagggtttggggacacagagctgtagaaatggcagagggatttggtggcctgaagctgactctttagatgtcgatgccttaagccaaacagcaatgccatttcataacaaagaaggccatgggtcagctggtgtccagacaccagaacttgggccaaccagagaaacacctgtactaattccatgtctgtctccttactggcctgaagttcacaatagagtcgtacagcctgcaggagatagtttctggctggatgctgagcccaggacttaaggctcaggtggccaagattggccatagccactgcctggttatgcacatctcccacctcctgggctctgttcaaggcccgaagatagctcttggctgccctgttcacccggccttcaccttggagtgcaagtcccaggaggttatagatgactcccctttgagtgagactctctgtctccttcagggagcatagcagtggctcaagcacatccaaagccttcttggcctggctggctaagagataggcccatgccaggcagagagaagactcaaaggattcctgctcacccagcagctgccctagcaccaaggcctggctcaggtagtggatggcaccgtcaggagacctgtgctcgaggtacactttggaaaggatgagacacagggccctctgggtgctccggtctgctagttcctcacaggcagccagggcctgtctgagcattgggcaggccaaggcagaaacttcaccccagcctggggaaggaaagccaaggagcttggttgtgttctggaggacaaggtggacctgccaaataggaagagacatcccttgggcactctggataccatgttgctggacagaggccactgcaaggtgtggaagatatttcttgtcatacagaaaactcaaaacactggccacagcctcagaggcaggagggtgtccagagaggagctgcaggcgctcggcaaagggcaggacctcctcgtgccggcctaggctcaggagcaagcggatggccagaaagcaggccctggcctccagcgggctgctgcccaccacaatcccctggcgcagcacgtaggccaccacgtcgagttcatgcttggcactagactcacggtcaggcaggcaggccagcagggcacctgccttttccaacagggcggagcctttatgtctcagcctctgtttcaggtagatggcagccaaattgatgtacagagtggccaccaaggataggtcctcaaatgctccattgagaatgtggatggcctcctcgaagtacaccctggcctgagagagtttgaccttcctgatgctcagccggcccaggaggaagcagagacgggcatgggcccaggtcatgtggctcttcttggcccactttcttgatgcctccaggtaggccacaaactcatcctcctcagagaagctataaaaggaagaagtgaggaaagagaaggagaagtcatagagactcttaaagtggtcagcataaccctcatgatccagaaaagccaatatgggggcgaagttctcagcctcctcctcctgaccagtgcttaggtccatgagcagttccgggtcatcaaggtcatcaggctccggcaggcgatagctgtctgaggtggccgagaggagctcctcctccaggctggagtcctcagagctgctggactgtctggaccccacggcctgatgctcctcccaggctctgccaggcctgacctccttgaaaccttcaggctgggatgcactcagatcatttggaggattctggatggattcaaacccactgagccggtagacagatgtgatgtcagtgcgagcaagagtgtggaggaagctggaacactcagtctgcttatcacttcccagggccaacagggagcatctctcctcatcactgagaaaggcagagttcctgctcattggggaataagaatcaggatctatgttcctggtggggacaaagcccacttgtcctgaacttgtcgactttccaatgaaccactgaagcccaggtatgacaaagccgatgatctcaatgctttctccctggtagaaattcagttcatccttttctcctggctcataacccgtcaaggccttacagcgtcctctgccaatctgataggagcctgtccaatccctcttcctggaaaggccacagcttcctggataattctttaggaaccactggtggaaagggagaggcagaggctccaaggctgacaccagtaccaggccccgctgacctgtcaccaaagacacgccttccaactcggagccagcttctgccatcttcactgagattaactcattcttgcaaagtgtcaagcattccccttccttctcggctggtggagtcacggagcacagggctctgcagaagaagtggccttcctgtatcaggagtcccaggtatattgtttccaggtgtttatcatctacagacacttggatctctgtatcctccaccaatatgcagttgagccagtacttgtggtcaaagaggagatgttctagacacatggatacgtagcctaaattaaggtaggtggagaacttccagatttcctccatggtcttgaaggtgatgagaaactgggccctctgagactggatactgaccaaccttgctgagaggtccttaaacagcatgcgcacctcctggtcctcattctccagtgcccagagccgcctccgagcagcttcctgtaggggtccatttacacacctcctggagcggctctttacacagaaggagagtgtcaggtctggattaatgttctgtggcagaaaacatttttccttgtattcagatgaggctatacactcactcgatacagttggatccttggaaggagtttctttacctgggccccgggtcagactccgctccctggggatgcagaagcagccacccatgtgtgtaccatcctaccctggccgaggcccttgggaacac

SEQ ID NO: 12468 - RNA, 4415 nt, Homo sapiens
  source 1..4415: mol_type = other RNA
cttggcaccattaaaaagtacaaggcctgtgagataatcgtatatatttttccaagaacaaaccagtcagatttgttttctctccccattttgcttatcattacagcctcacagtctacctaaacacctctggagggagctctgtaccttttaggacattatcgtttgaagacaatctgtaacttggctacagtcttgagtagcaagatgctacaaccctgaaaaggtcaaagatgctgttcctctggtttacttatagataggacaacttgtttacagcaattaaaaaatccaaaataagctaatcataagctagtaatttccactgttgtgccttaaggttcatagttaagcatgtataaagctttgatgacaattgcaaagaagctgtgtttgtgaaagtttactgaagtgccaggagagctgcacataacaggcagtgcagtaaagtaggagtgtggaattggaagatggactgcctcaggatgaaacctaactgccacttcctggtgttgtgaacttgggcaagttctgagttcttcatctctaaaatacagattcaggaaataatcgtacctttctcattacaggtgctgggagaatcaaacagtttaatatatgtaaaatgcttaggtaagtacctggctatttggtatttattatacatatcgtatatatatgtataatattacttattcatatattttattatataaatgtatataaaatatttaatatatatttactctcatataaaatatattatcatatatttattatagcttatattaaatagtataagagttatagcaattatcatcactttttatttgcttcatttttatgatcattctatggttctctttatttcctatcctatcttatatccagtttcaatgctgcccaattactactgactccattactcttatccctaaaaccttaattctaaagttagacattacctaaatataaactgttataacattcttaaacattgtaataccagtttaaatcattcattaattcactgctttactgaaacacagataaaaatgtctcattttatcattttatcttctttttgaccagtagatttggaccttaatactaatttactacaccattcactctgatatagactgaaacccaggataattaaagtatcatatacttggtggaagttaaatgtttatataaaatggataccaaatggaaataaaatgtttctccattttgtgcattcacagtgatcccaacatcttgcatcttcttttataataaatatatttcctaggctaattttcagaccttgaagccttggagaccactgaaattaataaatttgttgtagctccaaaagtctcttagctgatcattacgttggctggctgcaatagggaaagggccattgctgatacttgtgtatttaccaatcttgtttaatcacaatgaaagaagatgaaggtgtcatggaaagtggattttgtgtaatgctatatcaactgaagtgacttccataagccttcacaggtgttcacaggaatcagacattagaaaaatccctcctaatccaagatttggaatatacttcttgtattcaactggtacttgttgtgaagtaaattattggccctaataattacctacctacatccatgctcattgccctgtaactgcaagttctcccactcaagtctactcccctgtcagtcacttttctttgggcttgaccatttgatgtactttgacaatgcatgtggatggaagtgctaatgtgacatttctcagcctagcctttcgtcttgctcaattgccactgccatgagaggagcttccactgagaagctactatcccccaagtctggttctcagaatatgcacatgtggaagagaagaaagcctgacttttagcaagaagcctattcctgtggtatgtgcaacctcagcagagcttttcattaaagtcaagtccagtccaaatcagctgatccttgagtgacctgcatatatctgagaaatattattgttgtatgccactgatagatattttgtgattgattatctatctgtcacataacaaaagctgactgacatacatgtagtttcaggattatcaaaaaggcattatcttttcaaaaatgctagaaataattccaaagataattgtttgtgccagatgacataattgtatatacattgtagatggaattatcaagattacttttaatgccaacgacatttaggaatgctaattaacttatgaaacaccatcacatatcattaataaaggaaatttatattttgtgttccctaaatggcactataggaaatgtaacatatgctcattaagtttgcggttatgattttaatcattgaaatgaagtcaatgaaattgtataactgaaaaattccaccaaataactataaatttcacttttagatggatattagaatttataaaatatgtctagtgacttaattgtatactatttaacaattacaagactattataacatatttaattaacagaattgaaacaagtatttgttgaaaaacaaagaacattttaaacaactaattaatagtattttcaaaagagctcgacaaatgtattagccatatgaaattgaaataaataaaaagcaattaagtttccaaatgttaaaaaagttctacttctatatgattctcgtctaaggtgaaagcaatgatataagttcaactatgtaagaaaaagttttaaaaattgcatttatgaccacttcttatattccaacactttgtgttgataatgcaactaaacttctttaaaaatctctttctttgattaccatttagcatcaattatatggaaatcttttacaacttcaatatcttttaagggacagacaattaatggtccattttacagaataatagagctaaactatattgagtgaaataagatacagttacatgggaataaggatggcattaccaaccgaaactggctgattttagtatagaaatatgactcataaaatttcatacaatttaagactaaccattaagttgaattgataattatatttagagatcaattctaaaatgctaattaaaatactattgaaaatcttttcagtatgagattttcatatattctactttattatgcttcaaacgtggtaaattgctaaggaatggagttattttctaagagtttctatctgtgctgagctcaaaagaatgcccactctccataaataaaaagtaaacaaaggaaatgcatcagaaagttggaaaatagtttcatcatgcttctgaagaaatttcttgatttcttggtcatcatgacctatacttgaagtgttgccttcttcggtttccttttgaagaagctgctccagaacccagaacaggtagaaaatgttttcatagcgtgacacatcataactggcttgctcctgattgatggctcccagatcatcagcaaagccatttacttctgatagaagcagagatataatagattttctcaacaagctgcaatttcccaaggtaaccagactctgagagacataatgctgcacctgaaactgatttatatgattgtttcctaaaatagcatgtagtagggttttctcaaattcttccaacttcttggaacactttttaagaatatgactagataagttatagtcactgatcagactagctaaagtaccaacagcttctgtccaaaatcttgaaaaaggaagtttgggattacggtaaaaagtgatcaggccatccagcaattgaaaaacagaatcagagactgtggaagagtctttttcaaagtgggttaagtctcttttaagattacctgattctgtcaagttctttaattcaagtagatattgcaagaattgcatgtgagaagacaaaggattttgcaggatagcacaaggtcttttcacaagaggcagtggtggaaagtgagtgggggtacagctttccacaaagtgctgggacaggtctgaggattcagttctctgctcattcgacaaatcacatccagaatcttccatcgaagttaatgtactttcagaactcttaggttcctgagcctccaactgggaggaaacgtatccactcttaaaggatcctgaacaaagcctgctcacaagaagtttttgacgtaattgcataacttcagcttccaagatttcaacttttgatctccattttgactgctcctcagacagcaacatagcaaggtgctctgtgtattctctgctgcttttgtctgctggttttgagcggataattgccaaggccagagccagctttgaagttctcaaataccatttttgaacatccatcctggcttttgtcccagtaaacagagaagcagaaatgagatgataacagggcaagagaacgcctcatc

SEQ ID NO: 12469 - RNA, 4795 nt, Homo sapiens
  source 1..4795: mol_type = other RNA
cttggcaccattaaaaagtacaaggcctgtgagataatcgtatatatttttccaagaacaaaccagtcagatttgttttctctccccattttgcttatcattacagcctcacagtctacctaaacacctctggagggagctctgtaccttttaggacattatcgtttgaagacaatctgtaacttggctacagtcttgagtagcaagatgctacaaccctgaaaaggtcaaagatgctgttcctctggtttacttatagataggacaacttgtttacagcaattaaaaaatccaaaataagctaatcataagctagtaatttccactgttgtgccttaaggttcatagttaagcatgtataaagctttgatgacaattgcaaagaagctgtgtttgtgaaagtttactgaagtgccaggagagctgcacataacaggcagtgcagtaaagtaggagtgtggaattggaagatggactgcctcaggatgaaacctaactgccacttcctggtgttgtgaacttgggcaagttctgagttcttcatctctaaaatacagattcaggaaataatcgtacctttctcattacaggtgctgggagaatcaaacagtttaatatatgtaaaatgcttaggtaagtacctggctatttggtatttattatacatatcgtatatatatgtataatattacttattcatatattttattatataaatgtatataaaatatttaatatatatttactctcatataaaatatattatcatatatttattatagcttatattaaatagtataagagttatagcaattatcatcactttttatttgcttcatttttatgatcattctatggttctctttatttcctatcctatcttatatccagtttcaatgctgcccaattactactgactccattactcttatccctaaaaccttaattctaaagttagacattacctaaatataaactgttataacattcttaaacattgtaataccagtttaaatcattcattaattcactgctttactgaaacacagataaaaatgtctcattttatcattttatcttctttttgaccagtagatttggaccttaatactaatttactacaccattcactctgatatagactgaaacccaggataattaaagtatcatatacttggtggaagttaaatgtttatataaaatggataccaaatggaaataaaatgtttctccattttgtgcattcacagtgatcccaacatcttgcatcttcttttataataaatatatttcctaggctaattttcagaccttgaagccttggagaccactgaaattaataaatttgttgtagctccaaaagtctcttagctgatcattacgttggctggctgcaatagggaaagggccattgctgatacttgtgtatttaccaatcttgtttaatcacaatgaaagaagatgaaggtgtcatggaaagtggattttgtgtaatgctatatcaactgaagtgacttccataagccttcacaggtgttcacaggaatcagacattagaaaaatccctcctaatccaagatttggaatatacttcttgtattcaactggtacttgttgtgaagtaaattattggccctaataattacctacctacatccatgctcattgccctgtaactgcaagttctcccactcaagtctactcccctgtcagtcacttttctttgggcttgaccatttgatgtactttgacaatgcatgtggatggaagtgctaatgtgacatttctcagcctagcctttcgtcttgctcaattgccactgccatgagaggagcttccactgagaagctactatcccccaagtctggttctcagaatatgcacatgtggaagagaagaaagcctgacttttagcaagaagcctattcctgtggtatgtgcaacctcagcagagcttttcattaaagtcaagtccagtccaaatcagctgatccttgagtgacctgcatatatctgagaaatattattgttgtatgccactgatagatattttgtgattgattatctatctgtcacataacaaaagctgactgacatacatgtagtttcaggattatcaaaaaggcattatcttttcaaaaatgctagaaataattccaaagataattgtttgtgccagatgacataattgtatatacattgtagatggaattatcaagattacttttaatgccaacgacatttaggaatgctaattaacttatgaaacaccatcacatatcattaataaaggaaatttatattttgtgttccctaaatggcactataggaaatgtaacatatgctcattaagtttgcggttatgattttaatcattgaaatgaagtcaatgaaattgtataactgaaaaattccaccaaataactataaatttcacttttagatggatattagaatttataaaatatgtctagtgacttaattgtatactatttaacaattacaagactattataacatatttaattaacagaattgaaacaagtatttgttgaaaaacaaagaacattttaaacaactaattaatagtattttcaaaagagctcgacaaatgtattagccatatgaaattgaaataaataaaaagcaattaagtttccaaatgttaaaaaagttctacttctatatgattctcgtctaaggtgaaagcaatgatataagttcaactatgtaagaaaaagttttaaaaattgcatttatgaccacttcttatattccaacactttgtgttgataatgcaactaaacttctttaaaaatctctttctttgattaccatttagcatcaattatatggaaatcttttacaacttcaatatcttttaagggacagacaattaatggtccattttacagaataatagagctaaactatattgagtgaaataagatacagttacatgggaataaggatggcattaccaaccgaaactggctgattttagtatagaaatatgactcataaaatttcatacaatttaagactaaccattaagttgaattgataattatatttagagatcaattctaaaatgctaattaaaatactattgaaaatcttttcagtatgagattttcatatattctactttattatgcttcaaacgtggtaaattgctaaggaatggagttattttctaagagtttctatctgtgctgagctcaaaagaatgcccactctccataaataaaaagtaaacaaaggaaatgcatcagaaagttggaaaatagtttcatcatgcttctgaagaaatttcttgatttcttggtcatcatgacctatacttgaagtgttgccttcttcggtttccttttgaagaagctgctccagaacccagaacaggtagaaaatgttttcatagcgtgacacatcataactggcttgctcctgattgatggctcccagatcatcagcaaagccatttacttctgatagaagcagagatataatagattttctcaacaagctgcaatttcccaaggtaaccagactctgagagacataatgctgcacctgaaactgatttatatgattgtttcctaaaatagcatgtagtagggttttctcaaattcttccaacttcttggaacactttttaagaatatgactagataagttatagtcactgatcagactagctaaagtaccaacagcttctgtccaaaatcttgaaaaaggaagtttgggattacggtaaaaagtgatcaggccatccagcaattgaaaaacagaatcagagactgtggaagagtctttttcaaagtgggttaagtctcttttaagattacctgattctgtcaagttctttaattcaagtagatattgcaagaattgcatgtgagaagacaaaggattttgcaggatagcacaaggtcttttcacaagaggcagtggtggaaagtgagtgggggtacagctttccacaaagtgctgggacaggtctgaggattcagttctctgctcattcgacaaatcacatccagaatcttccatcgaagttaatgtactttcagaactcttaggttcctgagcctccaactgggaggaaacgtatccactcttaaaggatcctgaacaaagcctgctcacaagaagtttttgacgtaattgcataacttcagcttccaagatttcaacttttgatctccattttgactgctcctcagacagcaacatagcaaggtgctctgtgtattctctgctgcttttgtctgctggttttgagcggataattgccaaggccagagccagctttgaagttctcaaataccatttttgaacatccatcctggcttttgtccctgaaaatattgcgagctcaggtccaaacccagggcacgtgaaagggacgagtggtccacaggcacagaaagccaggcctcgcgctgagggagggcgtcctggaaagctgtgcagggcccgccccgcctaccttctgggttcctgtagcgggggagggcgccctcaagcgggcacgggagccctggagcaggcgctctgcgccatccccaggggcggggttccacgtgctgccccgcaggtggtcaccagagccagcggggaaacgctggccagcgcccagggccttccactcgtgggggaagtgagggagcaggtcccggagaccacaagccccagaagaccctgcggccgactcgaccccttctgcccctcttggcgggctgttccgaggaggagacgagtgctccacaaccagtccagagaaaataactcc

SEQ ID NO: 12470 - RNA, 4172 nt, Homo sapiens
  source 1..4172: mol_type = other RNA
cttggcaccattaaaaagtacaaggcctgtgagataatcgtatatatttttccaagaacaaaccagtcagatttgttttctctccccattttgcttatcattacagcctcacagtctacctaaacacctctggagggagctctgtaccttttaggacattatcgtttgaagacaatctgtaacttggctacagtcttgagtagcaagatgctacaaccctgaaaaggtcaaagatgctgttcctctggtttacttatagataggacaacttgtttacagcaattaaaaaatccaaaataagctaatcataagctagtaatttccactgttgtgccttaaggttcatagttaagcatgtataaagctttgatgacaattgcaaagaagctgtgtttgtgaaagtttactgaagtgccaggagagctgcacataacaggcagtgcagtaaagtaggagtgtggaattggaagatggactgcctcaggatgaaacctaactgccacttcctggtgttgtgaacttgggcaagttctgagttcttcatctctaaaatacagattcaggaaataatcgtacctttctcattacaggtgctgggagaatcaaacagtttaatatatgtaaaatgcttaggtaagtacctggctatttggtatttattatacatatcgtatatatatgtataatattacttattcatatattttattatataaatgtatataaaatatttaatatatatttactctcatataaaatatattatcatatatttattatagcttatattaaatagtataagagttatagcaattatcatcactttttatttgcttcatttttatgatcattctatggttctctttatttcctatcctatcttatatccagtttcaatgctgcccaattactactgactccattactcttatccctaaaaccttaattctaaagttagacattacctaaatataaactgttataacattcttaaacattgtaataccagtttaaatcattcattaattcactgctttactgaaacacagataaaaatgtctcattttatcattttatcttctttttgaccagtagatttggaccttaatactaatttactacaccattcactctgatatagactgaaacccaggataattaaagtatcatatacttggtggaagttaaatgtttatataaaatggataccaaatggaaataaaatgtttctccattttgtgcattcacagtgatcccaacatcttgcatcttcttttataataaatatatttcctaggctaattttcagaccttgaagccttggagaccactgaaattaataaatttgttgtagctccaaaagtctcttagctgatcattacgttggctggctgcaatagggaaagggccattgctgatacttgtgtatttaccaatcttgtttaatcacaatgaaagaagatgaaggtgtcatggaaagtggattttgtgtaatgctatatcaactgaagtgacttccataagccttcacaggtgttcacaggaatcagacattagaaaaatccctcctaatccaagatttggaatatacttcttgtattcaactggtacttgttgtgaagtaaattattggccctaataattacctacctacatccatgctcattgccctgtaactgcaagttctcccactcaagtctactcccctgtcagtcacttttctttgggcttgaccatttgatgtactttgacaatgcatgtggatggaagtgctaatgtgacatttctcagcctagcctttcgtcttgctcaattgccactgccatgagaggagcttccactgagaagctactatcccccaagtctggttctcagaatatgcacatgtggaagagaagaaagcctgacttttagcaagaagcctattcctgtggtatgtgcaacctcagcagagcttttcattaaagtcaagtccagtccaaatcagctgatccttgagtgacctgcatatatctgagaaatattattgttgtatgccactgatagatattttgtgattgattatctatctgtcacataacaaaagctgactgacatacatgtagtttcaggattatcaaaaaggcattatcttttcaaaaatgctagaaataattccaaagataattgtttgtgccagatgacataattgtatatacattgtagatggaattatcaagattacttttaatgccaacgacatttaggaatgctaattaacttatgaaacaccatcacatatcattaataaaggaaatttatattttgtgttccctaaatggcactataggaaatgtaacatatgctcattaagtttgcggttatgattttaatcattgaaatgaagtcaatgaaattgtataactgaaaaattccaccaaataactataaatttcacttttagatggatattagaatttataaaatatgtctagtgacttaattgtatactatttaacaattacaagactattataacatatttaattaacagaattgaaacaagtatttgttgaaaaacaaagaacattttaaacaactaattaatagtattttcaaaagagctcgacaaatgtattagccatatgaaattgaaataaataaaaagcaattaagtttccaaatgttaaaaaagttctacttctatatgattctcgtctaaggtgaaagcaatgatataagttcaactatgtaagaaaaagttttaaaaattgcatttatgaccacttcttatattccaacactttgtgttgataatgcaactaaacttctttaaaaatctctttctttgattaccatttagcatcaattatatggaaatcttttacaacttcaatatcttttaagggacagacaattaatggtccattttacagaataatagagctaaactatattgagtgaaataagatacagttacatgggaataaggatggcattaccaaccgaaactggctgattttagtatagaaatatgactcataaaatttcatacaatttaagactaaccattaagttgaattgataattatatttagagatcaattctaaaatgctaattaaaatactattgaaaatcttttcagtatgagattttcatatattctactttattatgcttcaaacgtggtaaattgctaaggaatggagttattttctaagagtttctatctgtgctgagctcaaaagaatgcccactctccataaataaaaagtaaacaaaggaaatgcatcagaaagttggaaaatagtttcatcatgcttctgaagaaatttcttgatttcttggtcatcatgacctatacttgaagtgttgccttcttcggtttccttttgaagaagctgctccagaacccagaacaggtagaaaatgttttcatagcgtgacacatcataactggcttgctcctgattgatggctcccagatcatcagcaaagccatttacttctgatagaagcagagatataatagattttctcaacaagctgcaatttcccaaggtaaccagactctgagagacataatgctgcacctgaaactgatttatatgattgtttcctaaaatagcatgtagtagggttttctcaaattcttccaacttcttggaacactttttaagaatatgactagataagttatagtcactgatcagactagctaaagtaccaacagcttctgtccaaaatcttgaaaaaggaagtttgggattacggtaaaaagtgatcaggccatccagcaattgaaaaacagaatcagagactgtggaagagtctttttcaaagtgggttaagtctcttttaagattacctgattctgtcaagttctttaattcaagtagatattgcaagaattgcatgtgagaagacaaaggattttgcaggatagcacaaggtcttttcacaagaggcagtggtggaaagtgagtgggggtacagctttccacaaagtgctgggacaggtctgaggattcagttctctgctcattcgacaaatcacatccagaatcttccatcgaagttaatgtactttcagaactcttaggttcctgagcctccaactgggaggaaacgtatccttgcttgacatctcatctgtttcctcattctgaaaatattctccttgttcaacttc

SEQ ID NO: 12471 - RNA, 4469 nt, Homo sapiens
  source 1..4469: mol_type = other RNA
cttggcaccattaaaaagtacaaggcctgtgagataatcgtatatatttttccaagaacaaaccagtcagatttgttttctctccccattttgcttatcattacagcctcacagtctacctaaacacctctggagggagctctgtaccttttaggacattatcgtttgaagacaatctgtaacttggctacagtcttgagtagcaagatgctacaaccctgaaaaggtcaaagatgctgttcctctggtttacttatagataggacaacttgtttacagcaattaaaaaatccaaaataagctaatcataagctagtaatttccactgttgtgccttaaggttcatagttaagcatgtataaagctttgatgacaattgcaaagaagctgtgtttgtgaaagtttactgaagtgccaggagagctgcacataacaggcagtgcagtaaagtaggagtgtggaattggaagatggactgcctcaggatgaaacctaactgccacttcctggtgttgtgaacttgggcaagttctgagttcttcatctctaaaatacagattcaggaaataatcgtacctttctcattacaggtgctgggagaatcaaacagtttaatatatgtaaaatgcttaggtaagtacctggctatttggtatttattatacatatcgtatatatatgtataatattacttattcatatattttattatataaatgtatataaaatatttaatatatatttactctcatataaaatatattatcatatatttattatagcttatattaaatagtataagagttatagcaattatcatcactttttatttgcttcatttttatgatcattctatggttctctttatttcctatcctatcttatatccagtttcaatgctgcccaattactactgactccattactcttatccctaaaaccttaattctaaagttagacattacctaaatataaactgttataacattcttaaacattgtaataccagtttaaatcattcattaattcactgctttactgaaacacagataaaaatgtctcattttatcattttatcttctttttgaccagtagatttggaccttaatactaatttactacaccattcactctgatatagactgaaacccaggataattaaagtatcatatacttggtggaagttaaatgtttatataaaatggataccaaatggaaataaaatgtttctccattttgtgcattcacagtgatcccaacatcttgcatcttcttttataataaatatatttcctaggctaattttcagaccttgaagccttggagaccactgaaattaataaatttgttgtagctccaaaagtctcttagctgatcattacgttggctggctgcaatagggaaagggccattgctgatacttgtgtatttaccaatcttgtttaatcacaatgaaagaagatgaaggtgtcatggaaagtggattttgtgtaatgctatatcaactgaagtgacttccataagccttcacaggtgttcacaggaatcagacattagaaaaatccctcctaatccaagatttggaatatacttcttgtattcaactggtacttgttgtgaagtaaattattggccctaataattacctacctacatccatgctcattgccctgtaactgcaagttctcccactcaagtctactcccctgtcagtcacttttctttgggcttgaccatttgatgtactttgacaatgcatgtggatggaagtgctaatgtgacatttctcagcctagcctttcgtcttgctcaattgccactgccatgagaggagcttccactgagaagctactatcccccaagtctggttctcagaatatgcacatgtggaagagaagaaagcctgacttttagcaagaagcctattcctgtggtatgtgcaacctcagcagagcttttcattaaagtcaagtccagtccaaatcagctgatccttgagtgacctgcatatatctgagaaatattattgttgtatgccactgatagatattttgtgattgattatctatctgtcacataacaaaagctgactgacatacatgtagtttcaggattatcaaaaaggcattatcttttcaaaaatgctagaaataattccaaagataattgtttgtgccagatgacataattgtatatacattgtagatggaattatcaagattacttttaatgccaacgacatttaggaatgctaattaacttatgaaacaccatcacatatcattaataaaggaaatttatattttgtgttccctaaatggcactataggaaatgtaacatatgctcattaagtttgcggttatgattttaatcattgaaatgaagtcaatgaaattgtataactgaaaaattccaccaaataactataaatttcacttttagatggatattagaatttataaaatatgtctagtgacttaattgtatactatttaacaattacaagactattataacatatttaattaacagaattgaaacaagtatttgttgaaaaacaaagaacattttaaacaactaattaatagtattttcaaaagagctcgacaaatgtattagccatatgaaattgaaataaataaaaagcaattaagtttccaaatgttaaaaaagttctacttctatatgattctcgtctaaggtgaaagcaatgatataagttcaactatgtaagaaaaagttttaaaaattgcatttatgaccacttcttatattccaacactttgtgttgataatgcaactaaacttctttaaaaatctctttctttgattaccatttagcatcaattatatggaaatcttttacaacttcaatatcttttaagggacagacaattaatggtccattttacagaataatagagctaaactatattgagtgaaataagatacagttacatgggaataaggatggcattaccaaccgaaactggctgattttagtatagaaatatgactcataaaatttcatacaatttaagactaaccattaagttgaattgataattatatttagagatcaattctaaaatgctaattaaaatactattgaaaatcttttcagtatgagattttcatatattctactttattatgcttcaaacgtggtaaattgctaaggaatggagttattttctaagagtttctatctgtgctgagctcaaaagaatgcccactctccataaataaaaagtaaacaaaggaaatgcatcagaaagttggaaaatagtttcatcatgcttctgaagaaatttcttgatttcttggtcatcatgacctatacttgaagtgttgccttcttcggtttccttttgaagaagctgctccagaacccagaacaggtagaaaatgttttcatagcgtgacacatcataactggcttgctcctgattgatggctcccagatcatcagcaaagccatttacttctgatagaagcagagatataatagattttctcaacaagctgcaatttcccaaggtaaccagactctgagagacataatgctgcacctgatttatatgattgtttcctaaaatagcatgtagtagggttttctcaaattcttccaacttcttggaacactttttaagaatatgactagataagttatagtcactgatcagactagctaaagtaccaacagcttctgtccaaaatcttgaaaaaggaagtttgggattacggtaaaaagtgatcaggccatccagcaattgaaaaacagaatcagagactgtggaagagtctttttcaaagtgggttaagtctcttttaagattacctgattctgtcaagttctttaattcaagtagatattgcaagaattgcatgtgagaagacaaaggattttgcaggatagcacaaggtcttttcacaagaggcagtggtggaaagtgagtgggggtacagctttccacaaagtgctgggacaggtctgaggattcagttctctgctcattcgacaaatcacatccagaatcttccatcgaagttaatgtactttcagaactcttaggttcctgagcctccaactgggaggaaacgtatccactcttaaaggatcctgaacaaagcctgctcacaagaagtttttgacgtaattgcataacttcagcttccaagatttcaacttttgatctccattttgactgctcctcagacagcaacatagcaaggtgctctgtgtattctctgctgcttttgtctgctggttttgagcggataattgccaaggccagagccagctttgaagttctcaaataccatttttgaacatccatcctggcttttgtcccagtaaacagagaagcagaaatgagatgataacagggcaagagaacgcctcatcaggggtgggagggctgacttggtaacaagagagacctctcttaggaaccagcttaaacat

SEQ ID NO: 12472 - RNA, 26 nt, Homo sapiens
  source 1..26: mol_type = other RNA
cttggcaccattaaaaagtacacttc

SEQ ID NO: 12473 - RNA, 131 nt, Homo sapiens
  source 1..131: mol_type = other RNA
ctttgcttcctgctcccctagtccaaggtgagcccgggaatcccgcagcccccgcccccgccccccaactcggagtcgctttcctggtcgccgccgagctccttccaccccgcggcgccgggagctgcggt

SEQ ID NO: 12474 - RNA, 1464 nt, Homo sapiens
  source 1..1464: mol_type = other RNA
gaaaatcctttttgtttttccagagtcttcaggcagttgcttttggtattttgtcttgagtttctcactctaataaacatggtgacattctcttctgggttggttgtaagccttgatgaacaagtgatggacactggttgcccaaatgggatggctcttttcatctatccagggcctctcatctatcttcaccactgataactatatatggaaagcagggctgcagccaaccttaaaagagtcacattctagggatgcagtgattaaggtctagacaattcaagagaggacatggttgagagatatgccattctatgttaatgcagtaagttctataaataaatgctattaatacattccaaacaataaatttaacatgaccacagtatgaataattgtttgcattttcctgcattctctgtgtgagacctgtgtttgtggtcatcatgaacaaatacactaacaccatttgagtcattagtatccagtgttcacaggcagtacaatggatgttgaagcaatatgagtaatgctgtaatcagcattaaataaatggcattatggaactgcagaggcaaaaagatctatacggttccaattataataggacctgaagagccattgcattgtgaatgataatagtgttactaccttttccttgcagtggtagatatgaaattgaacaggaatggtttctttagtaataattaatacaaataggtgactccaagaaactagaaaaaatttttatgttcaccgattggacaataagtagctatgtttccttaccttgactctcttcagcttttccttaccttgactctttaacagcaaatcactccatctcacatgggtccatgacttttataattatttttgtaatcagatgattgctatagatagattctctctctcctcgaacatttcctcagggcttttaatatctacaggcaaccccactcaacaggtacaggactagatattgcagctataaagaagattatgtcacagtctctttgtttaaggagcgcacagagtgccgatgcatatggatgtgtaaatagtgagaaaactgtgttgtaagtatagtataggtataatcagaggatattatgggtgttcccaggaagaatgactccctcagttcatgggtggggaagggaaatgcattaaggatacttcatcacaagtaacagaaaccaaagctggttaaactttatccttaaaggactgggataagagcgaggcaaataacacaaacagggcatgacatttaaggaggcagtctcaggtgctgagcctggagttatcacttgagaatgagcgcctccttaaatgttgaaccctaggcatctggctcaccctagtccccatcctgttattccttcagtcttaccttcttcaaaaactctcatcccccacagtgaaaaacagttgaaaaactgtttacatcctagtgtaaat

SEQ ID NO: 12475 - RNA, 2661 nt, Homo sapiens
  source 1..2661: mol_type = other RNA
gaaaatcctttttgtttttccagcaggtagcatagggaattgactccataacagttcgtaaacatttttcagcagtcctgacttctgctttgcaggcaaggccacatcatcaccaccttaaggactcgggtcaaatgcagcgtttgtaaaaactccatatgttcctaggtggctgtgaggattcaaggggcatttcccatcatctttttgtctgaaacgctttcttagcaaagccaggagcgtcccacccattatcagacctatcgtagaagccaccgctccaccaaagtaagtcagggcttcctggatagtcaatggtcctgcttggcaggttggcacggtagttgaccagtggccattctcttggcatgctgtttgtgcagagccattaagtaactggccctctagacaatggaaagagcagattgatccataactgaagtttccccagaggttggagcagttcatcgctattggcttattaacatgtagttctgagcatttcacagctctgcatgctggagttactgctgtccattgtcctgaaggtctgcagctgagagtgctgtctcctatgagtgtgaatccagcgttgcagccaaagtaacaagtggtattaaaaccaaaggttcccggatgatgcctacagtacatggttccctgcccaggagtggtgagggctggacattgcacccctggagtaggaagtgatgctatgcctttgcaggttggtggagtagctgaccatcttccagaagttgtgcattccacattattgggcccctccagcttaaagccgttgtcacaagagaaatggcaggtggagccaacattgaattctccacgagtgtcagaacaatccaggctgccctgctctggggcaaagagttctgggcacttgatggcttcacacattggtggggagtctgtccagcgtcccgatcgagtacaatccaatctttctggtccagacaaagaatatccctcgtcacagatgaattgacatgtggatttataactggaacttccaagaggttgaacacaggtcattgttccattctgagggcttagcaaaggtgtgcagggaatggcttggcattctggaggaacagaattccagtttccagtagccaagcactgtagcacacttgctcccaccaggagcaagccttcattgcaggtgaagctgcagactgactggtacctaaaggcaccgaaggggtgggagcagttcacccgggcctcatttggaactgggagatcctggcactgcaaagcttgacagactggggctggtgctgtccactgtcccaagttatcacaccgaactatatcggctcctctcagcatgaaaccttcagcacagcggaagctacagttggtgtcatactgaaacgctctcaaggatggagagcaatccatgcttccgtggacaggactctccagcggctcacacgaaatagcctcacaggttggcaagggtgcagaccagtgtccagagtcaatgcagcggagcatgtccaagcccctcactctgtagccgggctggcactcaaatttacagctggagccataggcaaaagcagtgagcggatgaacacagtccatggttccttcactgggggcttccaggtgctgacactgcacagctttacacactggggctggggctgtccatacccccgaggctgtgcattgcaccacttccggtccaactaatgcaaatccctcttcacaactgaagctgcagctagactgatgctggaatgcttttgcagaatgaaggcaggtcatgtttcctcgttcaggaatcttcaggggtgggcactgggcagctaaacactgtggaggcttatttgtccagattccagaagccaagcattccagcttgctgggcccatttacttggtacccgtcagtgcagtggaagctgcactgcgagttaaaagagaagtttcccagagggtggctgcagttcatgagcacgtgttgagggagctcaagttctccacactctctcacgtattcacattctggcccatagaatccagggtaacaggagcaggtgtagttcccgatggtctcgaggcactctccttgtttgctgcaggacatgtcctggcaggaggctgtgtaacacaatgcgtgctttttcttcaagcagtgctcatcattccacttgccaggggctgacggactcttgatgtatatctccacgcagtcctcgttgttccttttgttgttaggttcattatcagcccagttctcagcctcgttggtgagagcctttttggttcccacccatgtccatgtcttattgttctttcggatcccaatccagtagtaggagctgtagtagggtaggaccttattgaggtaatcaatttcatttttattctggatggccactaagtctgtgtagcgattctggcagtatttacgggaaatattccatgagtatgcttttgtgctgtaatgataagtccatgctgccacttctttctggtttgttagttcagagatcagggcactgaagcaaaggagttgggaaattccaaagaccactctctggaatctctggtacaagatggctatttggcagttggccatctcctctgtgactctgctggttttctgccttctgcccaacccagactgctt

SEQ ID NO: 12476 - RNA, 7014 nt, Homo sapiens
  source 1..7014: mol_type = other RNA
gaaaatcctttttgtttttccaggagcttttaaatcttgaccaaagacatataggtggggtgtaaatagccaaatagatattgatctgtttatttatataataggcttatatcaatgcatatgtgcatagcaggcatgggttctgcaatactcaggttctgtgcgaggtgccaggaattcagtgatgagtgaggcaaacatgatcctgctcttgtggaatttacagtccagttggggtggggagggagaaagaaattttaaagagaaattaaacattaactatatacttacaatttaatgagaaaaaaataaaatccaaggttctttgaaagcatttatttaacaggcagatctaacatgacctgggccaccaaaggaggccatctggaggagatgacatttaataaaggctgaagagaaatgaggcttgaaagtgtgcagaggtcttgagaaaggagcagtccatttgagtagctcaatggcaggcgggttggagtgtgatgagcaaaggggtggggcagtgagagcttcaggtgaggaggctgagggaacagtgagagcccaaaggacatcctaggtcacgcgaaggagtctacactttatctgaagtgccaacgtaagtctttgaagaattccaagcaagcatgagtgatgcaatcactacttcatgtgtaaaagatcaccctggctattgtataaggagtggaccaacagactggagtatttgctgattaagtgacttctaggatttctttcaaattaatccaggagttgtggggagaaacagatgaaacaatattgggcatgtgtcagtaaccatcaaggctgagtgatgagtacatgagggtctgtgttactgtcgtctaaaatttccacatggaaaagttgttaaaaccaccatataaatgaatatcttttataaacaagctcagcgtgtgtgtatgaagaaacatttctagcctgtatagaaaaagtgatctccatcttcacaaatgaagggaaatggtttacaatacaaatatacagaaagagctaatgatgtgagccacatacaagctcccctgtggatcctggccacatctcttaaatccagtctcgggttcctggcctgggagtctatgtcaccctcatgattttttgccacagacaaaattaaccagtggttttagcacaactcatttcttcagcatacctgaagagtatctatgccttctcaagaagtgtccttcaacctccagggtagtaatgaagggtaccccaaagaagcatttttaacagaaaagagaccagagaaggagagaatcctcactgttggactttgccccatgctgcctccttgggaccctgggagatcctttcccggcctgctggatctgccctttccccctgagaggcaggaagagctgagatctccaagccagaccttcacagtgcctctctctacagtcttagtgtgggaggggcatctttccatggcttcctgagatggagatttatttaagaaggaaagcttgttgaattccctcttacctttttaaatgaaaggtattattattattctatatctggggaaactggtcagacacctgtttatgttacatgccatagagttacagatgttaaagacctcagggcttcatctggcgtgatgtcagcgagggcctacattcagggttggggagggtgtgtactgtccagcattcctctaaaagtgtgtgactggcaaggcaggctccagcatcttctgaccactaatctaatattactgtccccacaggccctccctgtcatcacctttaccactgccctctccacccgcaacacccccgaggttgtggacttgtgagttctttgtgtatagctgttcaaacatttcctatagacgtgggtagtggacaaaggacttgcttgtgagaacttttcccatggagtgcagaatcagtgggtgcgggggtagcttgagcacacttagtttttagcccaggatttctacttgaaaagaattccccaaatcattaaccagtaatcgcacatctaaaagtaactttatatgcacccaaataggcacactgggaagactatttttcttgcttccccttctgtctttctcatctttgcttcaaatgtttctgctcaatacttaacgtgtgcttgcctcaaaagcagcctgacctgcgactcgcagagaatggagtattcacactggcaggatcctcagaaattaacacaaaaaaggcatatgacgatgacacacacatttgtgtaaagaaaaaataaaaggcattccagctgttatttcttaattttttttaacttggtttgggaatatatactacctgttttctggtgtcaacatgccatcaggtttcttaggctgactaaatcatcccaaaatgctgataatgatgagacaaaagaaagtctatcatttttttagggcttctgaggttccactgagttttgccctcatctaggtccagaagggcttagggaagtcccaggcgagtcagcagagctcaggaagctgaagccttgtctcagaggttagtgctcctttgctgaatcatctccagcaagaaatcacgtgactcagggtctactcaggtgaagtcggcacccttgtctttgagctcacacaggtggctgagctaaataagtgctgaaaggagctgggtgcactctcctgagtcacctttgttgactctggaagcactgtaaacttggcatcagaaggagattataaagtgcttttgttcctaagctttataaagtgtgtgtgtatgcatgtgggtttctctgtcatccagcctctcagatttcatcatccgagcattgtctgcaggaatcctgtttgcctggaaaaaagtagttcgtatagcttgggcatgtagggtagcagcagctttttcttaacacttggaagtcattggagagcattgaaatccgccccatcagtcagagctgcttgagactggtttgtcaggaatagaagcatgttgtctaacaacgggcattggcacaactgcatgaccttgggtttccatctccgagacttgcctctaacctttacctggctgtagaggaacagggagagccagatgagcctcagggtcaaggctgacctcagagtgtagtctctcagcagctttctatctgtgcccctgccttttagtagaacaggatggacttacaagtttggcatttgggtcccattagggacataagcaaataatggaagtattctgcaaaagaattatgctgccactgttcacagcggtgggaacagagtgtttagggacagtctattcgagcctaggacggcaacaagatgttcactaatactatcatttcttgagggctttctttatgccaggcgctttacgttaattctctcattgactcatcataactttttaaaatataggaaaatcttcatgttagagttgagaaatctaaggctcagagaagttaagaaatttgtccacagtcacacagtaactcagtggtgaaagaatgatacaaacacaagcagtgacactgcagagcctgaccagccctccatgtcagagaagctgttagttctttcagccttccctggcttgcaggaggcctcccaggacattcctatacaaacttggcccaaatcctttacatgtccccttagaactagcgtcaggagggagcatgcctgcttgctttcccctgcagccacacctcctctgtagtctgggaaaaaaactgttaagtgtctcattctcggggccaggtgtgcctctgattccttgagtatcctctagttcagttccactgtaatgagggccacagcaggaaggggaacataaaatgagtccctgagttcttgacccttctctttcccctgctctccagtcagtttgagacttacacttggggtagaatccagattttccaccctggtcccctcactcactctgtgcagcttataaagtgcttttcttggccctagaaaacattctgcttcctttagtaaatgtgtgcagaatatttcatgaagtcacattattttcctctttggccgactttccctcttggatcacagtcagggagaaagtcagctgaggtgaggcaacttttcagtgtgaccttaaatgtggatgaaagtgatggccccgaggagcacaattgttaacttactggcatttgggtcccattagggacataagcaaataatgaaagttttctgcaaaaggattatgctgtcaccattcacagcagtaggaacagagagtttagggaaaggcctgtgcccagcctaggatggcaagctatccacctccaactccacaccatctgcaccaacgtgaactgtgaaagatttcaggcctgggactaatgttaaatgttcccttaactcctcatctccacatcactggacgggggtagtggtagaagggccaccccaccaccaccacaacacacaaagcttctacccccttagtatcaccccggaccctccttctcccggtcctggtttctgtttcatggtattcatcctcctctggcctcttcatggcatcctccagctgccactctggctgcttctcaccctacaccaggggtcaggagccatgaaagtccgtgagtgataccagccaggtgggaggtgatagggagtggtggggcatgtgactgactgggcatctggtgccccatgaaaagcagaagcccctgctcaactccaggccgtttctatgagaggagtgcaggcccagtgttcccgagtatctcattttccacgagaagttggaaaacctgacttttcatgtgatgtgacatttcctagcgtttaaatatttgagaagtaattaaaattatttcaaaacacactaggtaggccaaataaaatgtgtctgagacctagggctggtatcagttctagtctgtctctgtcactttccacaatctaacctgccctcccagcttcagtggttactcaaatttcaatgtctctgagcgttagatggccagccctggcctgcaccccagatttaccctagaattcatctgcatgtgggtgcccacacacctccaatgcaaagcggagcccatcagcctcccagatttggcagactgtaggatctcagtaagtgtgagctatttttgtctttgttccactaacaaaaatactactactactaacactgctactaatactcatgctacaaagaataatctcttgcccctcttttgttccatttctgttactcaacaccactgccccatcaggcagccagggaggaccctgtgatcttggactcttcactcccattcccggcagttagtggattgtgtttattcttccacggccctctagaatgtgcttccaactcttccttccaattaactagaaactctcctagttgctgaacttgtcatgtgttctcagctattgtctcagcctctaactgctcaccaccaggcgctacctctgcatttaagatttattcatcacgctgtggctagtgtcatcccctaaattgccgtgcagctctcatcactcacctcggatggatcccaccggctgcccccgcagttcctcagccatccctgcatgccagctgtaccaggcacttgtatgcctctgcatttgtgctggctgtgtcctcaggcgcattttcttccttcatgcctactatgttaattctgttcgtcctcatctctggtcaaatgccacctcttccacgaggctgtcacttgccttcccaccaccagccccagtgttatttgccccgtgcctcttccaagctctcacagcacttgatctaagtctcttttcatttcatccggctgtgtattatgaagtttgcttgattcttcccccttctcttgattagctcctggatgaagagacactgtctttgtcatctgcgtatccccaagaaacccctagtgtgctgccttacatgtagtagacaccttgaaaacctttgtcaattgaatcaaagtttgtttgtgtgtgtgtgtgttttgttttttcttttggtttgttttttttgtaagttgaggatggctgcatctaaagggctcaggccaaggtattaaaaacaaaactgcttggttattcaaaaggatttatcagaaccccaagaggctaagtatcaagctagtgaaagggttattctgcctgtccccaattccaagggtgcagtttttagaggacggacggtcgtgtttggtctacttgtcgtcaggcaaggcctcttccacagtgccccatggaagcttgggttcagtgccaggggcagggaggaatgggcaagcctcttggacactggggcttcagccaccctggcatatagagtcctgcactgtttgtcttgcccagaagaacaggctgtacccacccattcacaagatgtcctctctcacatcattggcaggcctgggaatttcccacaggccatctgggtgtgttctgccgtcctgtctcccaagttttttgcagcattgtttcttgttaattagctcttagaatagcaactgctcttccatcaggaattgtatcccgttgactttcctaaggcaagaatctactcatttcttttttgtaagcattttctcccttcctgcctgcattgcacaggcttacttagtgagagcccaagcagtgtgaactaactcctagctcttacagaactgagttacttataatatgcatctcctgaatcctgggtgaccactgtaagtgcctgaagtggcagctgctctgactgggcctgtgcagctctgaatgctgcatttacttttgggtcctgcctccaacccagaaccacctgtggcctttaattcctgttactaggagagaggagaagcgattaaaccctgtcagtatattcatttattagctgccctttgaagcttttttgaaagcattttacaaggtatatcccgtcaggttgcttaggaacttttgcagcctccttcttcaacattatcattttcatttgaatcaacactggcagcttgacacctctg

SEQ ID NO: 12477 - RNA, 6799 nt, Homo sapiens
  source 1..6799: mol_type = other RNA
gaaaatcctttttgtttttccaggagcttttaaatcttgaccaaagacatataggtggggtgtaaatagccaaatagatattgatctgtttatttatataataggcttatatcaatgcatatgtgcatagcaggcatgggttctgcaatactcaggttctgtgcgaggtgccaggaattcagtgatgagtgaggcaaacatgatcctgctcttgtggaatttacagtccagttggggtggggagggagaaagaaattttaaagagaaattaaacattaactatatacttacaatttaatgagaaaaaaataaaatccaaggttctttgaaagcatttatttaacaggcagatctaacatgacctgggccaccaaaggaggccatctggaggagatgacatttaataaaggctgaagagaaatgaggcttgaaagtgtgcagaggtcttgagaaaggagcagtccatttgagtagctcaatggcaggcgggttggagtgtgatgagcaaaggggtggggcagtgagagcttcaggtgaggaggctgagggaacagtgagagcccaaaggacatcctaggtcacgcgaaggagtctacactttatctgaagtgccaacgtaagtctttgaagaattccaagcaagcatgagtgatgcaatcactacttcatgtgtaaaagatcaccctggctattgtataaggagtggaccaacagactggagtatttgctgattaagtgacttctaggatttctttcaaattaatccaggagttgtggggagaaacagatgaaacaatattgggcatgtgtcagtaaccatcaaggctgagtgatgagtacatgagggtctgtgttactgtcgtctaaaatttccacatggaaaagttgttaaaaccaccatataaatgaatatcttttataaacaagctcagcgtgtgtgtatgaagaaacatttctagcctgtatagaaaaagtgatctccatcttcacaaatgaagggaaatggtttacaatacaaatatacagaaagagctaatgatgtgagccacatacaagctcccctgtggatcctggccacatctcttaaatccagtctcgggttcctggcctgggagtctatgtcaccctcatgattttttgccacagacaaaattaaccagtggttttagcacaactcatttcttcagcatacctgaagagtatctatgccttctcaagaagtgtccttcaacctccagggtagtaatgaagggtaccccaaagaagcatttttaacagaaaagagaccagagaaggagagaatcctcactgttggactttgccccatgctgcctccttgggaccctgggagatcctttcccggcctgctggatctgccctttccccctgagaggcaggaagagctgagatctccaagccagaccttcacagtgcctctctctacagtcttagtgtgggaggggcatctttccatggcttcctgagatggagatttatttaagaaggaaagcttgttgaattccctcttacctttttaaatgaaaggtattattattattctatatctggggaaactggtcagacacctgtttatgttacatgccatagagttacagatgttaaagacctcagggcttcatctggcgtgatgtcagcgagggcctacattcagggttggggagggtgtgtactgtccagcattcctctaaaagtgtgtgactggcaaggcaggctccagcatcttctgaccactaatctaatattactgtccccacaggccctccctgtcatcacctttaccactgccctctccacccgcaacacccccgaggttgtggacttgtgagttctttgtgtatagctgttcaaacatttcctatagacgtgggtagtggacaaaggacttgcttgtgagaacttttcccatggagtgcagaatcagtgggtgcgggggtagcttgagcacacttagtttttagcccaggatttctacttgaaaagaattccccaaatcattaaccagtaatcgcacatctaaaagtaactttatatgcacccaaataggcacactgggaagactatttttcttgcttccccttctgtctttctcatctttgcttcaaatgtttctgctcaatacttaacgtgtgcttgcctcaaaagcagcctgacctgcgactcgcagagaatggagtattcacactggcaggatcctcagaaattaacacaaaaaaggcatatgacgatgacacacacatttgtgtaaagaaaaaataaaaggcattccagctgttatttcttaattttttttaacttggtttgggaatatatactacctgttttctggtgtcaacatgccatcaggtttcttaggctgactaaatcatcccaaaatgctgataatgatgagacaaaagaaagtctatcatttttttagggcttctgaggttccactgagttttgccctcatctaggtccagaagggcttagggaagtcccaggcgagtcagcagagctcaggaagctgaagccttgtctcagaggttagtgctcctttgctgaatcatctccagcaagaaatcacgtgactcagggtctactcaggtgaagtcggcacccttgtctttgagctcacacaggtggctgagctaaataagtgctgaaaggagctgggtgcactctcctgagtcacctttgttgactctggaagcactgtaaacttggcatcagaaggagattataaagtgcttttgttcctaagctttataaagtgtgtgtgtatgcatgtgggtttctctgtcatccagcctctcagatttcatcatccgagcattgtctgcaggaatcctgtttgcctggctgtagaggaacagggagagccagatgagcctcagggtcaaggctgacctcagagtgtagtctctcagcagctttctatctgtgcccctgccttttagtagaacaggatggacttacaagtttggcatttgggtcccattagggacataagcaaataatggaagtattctgcaaaagaattatgctgccactgttcacagcggtgggaacagagtgtttagggacagtctattcgagcctaggacggcaacaagatgttcactaatactatcatttcttgagggctttctttatgccaggcgctttacgttaattctctcattgactcatcataactttttaaaatataggaaaatcttcatgttagagttgagaaatctaaggctcagagaagttaagaaatttgtccacagtcacacagtaactcagtggtgaaagaatgatacaaacacaagcagtgacactgcagagcctgaccagccctccatgtcagagaagctgttagttctttcagccttccctggcttgcaggaggcctcccaggacattcctatacaaacttggcccaaatcctttacatgtccccttagaactagcgtcaggagggagcatgcctgcttgctttcccctgcagccacacctcctctgtagtctgggaaaaaaactgttaagtgtctcattctcggggccaggtgtgcctctgattccttgagtatcctctagttcagttccactgtaatgagggccacagcaggaaggggaacataaaatgagtccctgagttcttgacccttctctttcccctgctctccagtcagtttgagacttacacttggggtagaatccagattttccaccctggtcccctcactcactctgtgcagcttataaagtgcttttcttggccctagaaaacattctgcttcctttagtaaatgtgtgcagaatatttcatgaagtcacattattttcctctttggccgactttccctcttggatcacagtcagggagaaagtcagctgaggtgaggcaacttttcagtgtgaccttaaatgtggatgaaagtgatggccccgaggagcacaattgttaacttactggcatttgggtcccattagggacataagcaaataatgaaagttttctgcaaaaggattatgctgtcaccattcacagcagtaggaacagagagtttagggaaaggcctgtgcccagcctaggatggcaagctatccacctccaactccacaccatctgcaccaacgtgaactgtgaaagatttcaggcctgggactaatgttaaatgttcccttaactcctcatctccacatcactggacgggggtagtggtagaagggccaccccaccaccaccacaacacacaaagcttctacccccttagtatcaccccggaccctccttctcccggtcctggtttctgtttcatggtattcatcctcctctggcctcttcatggcatcctccagctgccactctggctgcttctcaccctacaccaggggtcaggagccatgaaagtccgtgagtgataccagccaggtgggaggtgatagggagtggtggggcatgtgactgactgggcatctggtgccccatgaaaagcagaagcccctgctcaactccaggccgtttctatgagaggagtgcaggcccagtgttcccgagtatctcattttccacgagaagttggaaaacctgacttttcatgtgatgtgacatttcctagcgtttaaatatttgagaagtaattaaaattatttcaaaacacactaggtaggccaaataaaatgtgtctgagacctagggctggtatcagttctagtctgtctctgtcactttccacaatctaacctgccctcccagcttcagtggttactcaaatttcaatgtctctgagcgttagatggccagccctggcctgcaccccagatttaccctagaattcatctgcatgtgggtgcccacacacctccaatgcaaagcggagcccatcagcctcccagatttggcagactgtaggatctcagtaagtgtgagctatttttgtctttgttccactaacaaaaatactactactactaacactgctactaatactcatgctacaaagaataatctcttgcccctcttttgttccatttctgttactcaacaccactgccccatcaggcagccagggaggaccctgtgatcttggactcttcactcccattcccggcagttagtggattgtgtttattcttccacggccctctagaatgtgcttccaactcttccttccaattaactagaaactctcctagttgctgaacttgtcatgtgttctcagctattgtctcagcctctaactgctcaccaccaggcgctacctctgcatttaagatttattcatcacgctgtggctagtgtcatcccctaaattgccgtgcagctctcatcactcacctcggatggatcccaccggctgcccccgcagttcctcagccatccctgcatgccagctgtaccaggcacttgtatgcctctgcatttgtgctggctgtgtcctcaggcgcattttcttccttcatgcctactatgttaattctgttcgtcctcatctctggtcaaatgccacctcttccacgaggctgtcacttgccttcccaccaccagccccagtgttatttgccccgtgcctcttccaagctctcacagcacttgatctaagtctcttttcatttcatccggctgtgtattatgaagtttgcttgattcttcccccttctcttgattagctcctggatgaagagacactgtctttgtcatctgcgtatccccaagaaacccctagtgtgctgccttacatgtagtagacaccttgaaaacctttgtcaattgaatcaaagtttgtttgtgtgtgtgtgtgttttgttttttcttttggtttgttttttttgtaagttgaggatggctgcatctaaagggctcaggccaaggtattaaaaacaaaactgcttggttattcaaaaggatttatcagaaccccaagaggctaagtatcaagctagtgaaagggttattctgcctgtccccaattccaagggtgcagtttttagaggacggacggtcgtgtttggtctacttgtcgtcaggcaaggcctcttccacagtgccccatggaagcttgggttcagtgccaggggcagggaggaatgggcaagcctcttggacactggggcttcagccaccctggcatatagagtcctgcactgtttgtcttgcccagaagaacaggctgtacccacccattcacaagatgtcctctctcacatcattggcaggcctgggaatttcccacaggccatctgggtgtgttctgccgtcctgtctcccaagttttttgcagcattgtttcttgttaattagctcttagaatagcaactgctcttccatcaggaattgtatcccgttgactttcctaaggcaagaatctactcatttcttttttgtaagcattttctcccttcctgcctgcattgcacaggcttacttagtgagagcccaagcagtgtgaactaactcctagctcttacagaactgagttacttataatatgcatctcctgaatcctgggtgaccactgtaagtgcctgaagtggcagctgctctgactgggcctgtgcagctctgaatgctgcatttacttttgggtcctgcctccaacccagaaccacctgtggcctttaattcctgttactaggagagaggagaagcgattaaaccctgtcagtatattcatttattagctgccctttgaagcttttttgaaagcattttacaaggtatatcccgtcaggttgcttaggaacttttgcagcctccttcttcaacattatcattttcatttgaatcaacactggcagcttgacacctctg

SEQ ID NO: 12478 - RNA, 361 nt, Homo sapiens
  source 1..361: mol_type = other RNA
gaaaatcctttttgtttttccagtataggcataatcgagaaatgcttttactgccttggaggacaaattagtaatggtaacacttccatcatctctttctttcatgtttacttcaaacatagcccgctggcctttggctgatatttccgggcagtcagaggaagaaggaaatcggctgaatcccgcagtaccgcactttaatcgacctccaggtagtcatttacagtcatctgcagagaccaacttttccctggaccaaaacctgcagggcacttggatcgcgtgggctttcatacgagagtcaacaacagcctacacggaacaactgcaactgcagtctccgaagtctccaccccagtct

SEQ ID NO: 12479 - RNA, 641 nt, Homo sapiens
  source 1..641: mol_type = other RNA
gaaaatcctttttgtttttccagtataggcataatcgagaaatgcttttactgccttggaggacaaattagtaatggtaacacttccatcatctctttctttcatgtttacttcaaacatagccctgaaaaagtcactgcatgctgctaacacacaacgatgacacgggattatttcatctttcataattattttgaaatcataaaagacattttgttctctaaaattctgtagtacacttaagattttttgtccatgatcttctgatacaaggaagttgtttttcttctcagatggaattccattacatgtgcttcgttgattgaaagcatatgaattatccatagccaattccatatgtccttagaacagattgtaagctccctgcagctggtaagcagattttcaacatggcagctgacacaggcttttggttagctaagatgatatattaagccaataattcgttttactgtcctttggggatctgaatttgtgtgtgtgtgtgctcagaatcccatctactttcgagggattcggggggcttatgatatcacgaaaagttaatgaagacaagtatagataaaaacataatagaacccatcttaaataggacagaaatcataggcaggtaattgtgt

SEQ ID NO: 12480 - RNA, 606 nt, Homo sapiens
  source 1..606: mol_type = other RNA
gaaaatcctttttgtttttccagtataggcataatcgagaaatgcttttactgccttggaggacaaattagtaatggtaacacttccatcatctctttctttcatgtttacttcaaacatagccctgaaaaagtcactgcatgctgctaacacacaacgatgacacgggattatttcatctttcataattattttgaaatcataaaagacattttgttctctaaaattctgtagtacacttaagattttttgtccatgatcttctgatacaaggaagttgtttttcttctcagatggaattccattacatgtgcttcgttgattgaaagcatatgaattatccatagccaattccatatgtccttagaacgctggcctttggctgatatttccgggcagtcagaggaagaaggaaatcggctgaatcccgcagtaccgcactttaatcgacctccaggtagtcatttacagtcatctgcagagaccaacttttccctggaccaaaacctgcagggcacttggatcgcgtgggctttcatacgagagtcaacaacagcctacacggaacaactgcaactgcagtctccgaagtctccaccccagtct

SEQ ID NO: 12481 - RNA, 405 nt, Homo sapiens
  source 1..405: mol_type = other RNA
gaaaatcctttttgtttttccagtataggcataatcgagaaatgcttttactgccttggaggacaaattagtaatggtaacacttccatcatctctttctttcatgtttacttcaaacatagccctgaaaaagtcactgcatgctgctaacacacaacgatgacacgggattatttcatctttcataattattttgaaatcataaaagacattttgttctctaaaattctgtagtacacttaagattttttgtccatgatcttctgatacaaggaagttgtttttcttctcagatggaattccattacatgtgcttcgttgattgaaagcatatgaattatccatagccaattccatatgtccttagaactgcaactgcagtctccgaagtctccaccccagtct

SEQ ID NO: 12482 - RNA, 1027 nt, Homo sapiens
  source 1..1027: mol_type = other RNA
gaaaatcctttttgtttttccagtataggcataatcgagaaatgcttttactgccttggaggacaaattagtaatggtaacacttccatcatctctttctttcatgtttacttcaaacatagccctgaaaaagtcactgcatgctgctaacacacaacgatgacacgggattatttcatctttcataattattttgaaatcataaaagacattttgttctctaaaattctgtagtacacttaagattttttgtccatgatcttctgatacaaggaagttgtttttcttctcagatggaattccattacatgtgcttcgttgattgaaagcatatgaattatccatagccaattccatatgtccttagaataccgctggcctttggctgatatttccgggcagtcagaggaagaaggaaatcggctgaatcccgcagtaccgcactttaatcgacctccaggtagtcatttacagtcatctgcagagaccaacttttccctggaccaaaacctgcagggcacttggatcgcgtgggctttcatacgagagtcaacaacagcctacacggaacaactgcaactgcagtctccgaagtctccaccccagtctccctgcctccagaggactggttgcgattggcctgcaccgctgtcccgttaactcttccgcaagtgtgagtggcgtaactgtcgggctcttggccttggtcccgcccttcgctcgcctccgaagcctcgcctacttgacgtcatacaatgccgcaaagcgcagggctgatctccgtctccgcccccagctgctttctccgagaggaggtggctgagtcgggggcgggctgggagggctgtcggtgggccagtctgcgtagcgacggcccgtcccctgcgcacggacgccgggaagaagggggtggggccacgtttgcgtccgcgccatcaggcccgagatagcggcgaggtccgctttcagtgtatggttttccctgccaaacggttctgcttggtgccatccatggagggcgtgcgct

SEQ ID NO: 12483 - RNA, 630 nt, Homo sapiens
  source 1..630: mol_type = other RNA
gaaagagagctgagtgtgcaggagggatcaatgtttacctccgcctctggacagcagctccctagccacacggaggagctcacggtggctggggggtccagcaggactttggggcctgatctgctctgggactctggacaccatgccctcaggcctcatgcggcaaggtcatgggtcactgagtggatgcagggcctagggccctgcccatgacagcctccacgtacctggtctacacacagcccagccgcacgaagattatccagaaaagtctcccgccaggtcctgtgcatgtctgttctgtcccgggcggcactgtcctgctgcctgtctagcttcaggtcctcctcccaaacgaggacgaagtcgatccggggcttggcaggactcccagctctgcaggcggccgcttgctgtccacctggctccgaggcgtgggctgtgctcccgtaagagcccctcttctctgcctcaggggggctcacatcgatcaggacggtgctgtcctcttcctgggcccgtcgccgcagcatcctgctcctggcacagtggcttccggaagaggtctcggaggtcatggcccacctctcagcgtgagcctggtctcggcagtagagtcccgtcctcact

SEQ ID NO: 12484 - RNA, 5162 nt, Homo sapiens
  source 1..5162: mol_type = other RNA
gaaagtgcttccttttagaggctgaataatattccactgtatgaatataccacattttgttgatcattcacccactgatgggcacatattgcttccatctcttagctactgtgaataatggtgccgtgagtatgggcatacaaaaactaccactaatattttacagtgcttgcttcatatctgtccatgtgtccgtcactccacccatcatattttttatgtatttcataagttacagaccacagtaacttccctcaaacatgtcagtatacatatcaatgaccagcgttcattgtttttttccaagtcattttgaactgccgtagcaatgagtaatatagcctcaaacgcacacatacacacacaacacgtgcgtcactacagaaaacttttcctggcagacaggaaagggcccattgttggtgatgtcattttaattaagataaaaccaccaccaccatttagtaatagcctggggtaacaagggctgcgtcacggactgccacttttgccatcctgctcagagcagggccatgcctaacccgtatctggggattgcttcagatattatgaatcgcttcaatattatgaattactacaattcataataattgcttcagatattatgaattacaatatggttcaaaggtgctttagcagatgaagacacaaatgtgtaaacacatatgaattacaatgcagactgcccagatgtgtagcaagtcctctgaatgtttactaaacagtaaggtgattccagaggaagatgcttgaggacaatttgggaaaactgacaacttgaaaactcagtctctctaggcaaggcctacttgcagataaccttgggagttctgtgctgggaggaaagctaaaggactaagttaggcctctgaatctgctctggaagcctgcatgcacttgggtcagaacaagcccatgtgtcaatgtgggtaaagattcctcagctgataagcaggaaaatgggcagggcattttggtctttgaggttcaaagctcagatgctcactgccttggtatacacgcacacacaccccaccccccagctgacggcacaagagtatacagatgcaatagtctaaagtacattgtccaaatatggatggccatgagccacatgtggctatgaagcacttaaatgtggctagtctgaactgagatgggccctataaaatatttcagtaacaggtttttatactgattataggttgacataataatattttggatataccgtattaaaggaaatatgtcattaaatttcacctgtttcctttattatgtggctacttgaaaattttaaaattacatatgtagctcacactataaaacacagattagaaatattgtatagcactgacctagaaacctccatttaggtaaaacatcttaacccctttggaagcaaaatatgttaaataacagcataaactcccaccaagaaaatcctcaccttcctcctttcaacacatttattatatacagctgtcactgcattgtcaatctgccaaatggctctatgttccaacagggctggagtagtcccctgctcacaccagccttcacaatacttcccatgtcttccctgttaacctctctccacccagcacccaggctcccaactctcctggctgcctccagccctcagctggcaccactgacatgctgtttccagtacccttttcttctttctgcatcctccctgggggacatatatccctcatctcgtgacttcagctgtcacataaattcaaatgtttcagaactctattttttacctcctacatctgtcagtttaaatgtcaggatattttactttcagtaaagccctaaaaagacaaatctatgtacttttaaagaataaaagaaatgactggctgcagctcaaacctacaactgcttgcgaaactctacaatgtctggcagatgctagaaagaaggggatcaagacagagcacacttggcgtggtatgctatctatagaaaatgttaaaataaaattaagtaatctaggtttcctctctttattttctacatctactctctgaagagggcaataaataaggaaatgtcccaaagagggacaaattaagtcccaaaataacacaaaattgggcaaatccagtcatgaagaaagaacagaggttcttaaattgggacacacagaggcaggtctgcaggtctaggaatctctgaacatatgtgcaaaattctgggtatgtgtgcatatgttatataacaaagcgaagggtccatatagctttcatcgcatttcaaagggtctagcactgaaataaggactactgctatgtgacttaaaaaatgaaactcaggctgggcgcagtggctcacgcctgtaatcccagcactttgggaggccgaggcaagcagatcacctgagacgaggagtttgagacccgcctggccaacggtgaaacccagtctctactaaaaatacaaaaattagccggaattggtggtgtgcctctagtcccagctactcaggaggctgaagaaagagaatcgcttgaacctgggaggtggaggttgtgacaaagcaagactccatctcaaaaaaaaaaaaaacccagaaactcaattcagttatgaaggtaaagatgacctgtttacatgataatattttaagataccagtgactgcaagcatgtagttattaagtccattacagtgcacatttattgactctgtgtatcttcacagtgtgatcttcaccacagcttgcaaagtgtaaccactcagcaccttctgcttccttctgttcagtttttccactgcaattcttccagcataattttctgatagccagtgtatgactttggctttgacttgtttctacacagtgggtccagtcatttatttctggaacttgatcagtctttttccaggtatataagcaaatctttccacactccaatcctactgcaaccacgtatcgttgagaagggtggagcactgggcagacgctgacagctgtcacagccccacccacgtccaggactgaggagcaggggccaatgttgtgctcaatacagtcatcagtggagtcgcactcaccccagacaaccacctttttgtctcgactcccagtgaagaaatacttgctgtcaggactccaatcacaagaccaaataattcgaactcaggtgagattgtatcctgctttttccacaatgaccaggttcgatctctggaaacagctagtaagaacttctcattaggtgagaaggccatctgcgtgactgtcaaactgtggaaaactaaattctgcacctgtttccaagatgtagtgttccaaagaatgatagctgcatgctctttcttagctgccttacaagctgaggcaagcagagtctttgaactgttacaagtaacacaaaatatttcataaccgtgcccatatagtttttgaacttcaggccacaaagtattctgcagaagatgatcctcagtgggaggctcagtaagtatggagggctgaaaggccacctgctgatactcaaaaccagtactagttaacagctcctcttcatcagaaggctgagaagctatatctccctgaaagacagctttatttgataatcccaatgcagggacagtggctccttctggaagatcactatcttgattacagagcacatgattcagtgattgtcctgtaatggcacaaaaattttccacaaaattccgaggtgcagaaaaaacccgaagaactttttcatctgctccagatacaaactgaaaccgattaatcattgccaaacatttcaggtcatacccatgtatctgaggccttgcaatttcatgccaagtcacctgtgattggtcttttctcttccatggagcaaaaagtctagttgtctgatcagtaccaacagtgataataaattctccttctggatcccagactaggtcttggacaccatcaaagtgtcctgaaatgacaatctctggagtccactctcttgggttaactgtattctgtttccaaaggtgcaacgctccgtggaaagcatgagcaatgatcatggagccatcttcattgaactggcaatcataaaatcccaaagtattcccacctacttcacctactcgaacctgttctagccaaactcctgactcttcatctggagcccagagaatcatggttttatccatggaagcagataataatctcactggctgctgtaggacaccatctttgtaaaacacaggttgccagtgaactgcatttacccagttttcatgaccggctagcactgtctccagagtaacagcaaatgctattttaacactttcattttctatggtaaaagtattttctttcagtcttatgttatcgtcatcctgagtttctaaagatgttgactttatatacagcttccatattcttatcaggcaatcttgtgaacagcttgctaggaaaagatctctaccaaaggctgcccattccactcctctaatccaatcctcatgtccacagagagaaagcactttctgaaactgatcattttgttgagcaaatatgtgaattctgcaatcatcattgccacatgctaatattggtacatcagtatttggcaaaaaagataagcagagagccaaagcaaatccatttccaaagtttaaagtctgaaggcacattacttctggaccctttttagaccagagtcgaacagcagaatctgcagctgcagaaacgatcagtgtacataatgcaggatctgatgtcctcctctggtaaacagcatgcaccgcataaacaggtccttcatggccttgaagatgcactgcttttaaaagctgattatcctctatttcccagtgaatcacttgattatcagatcctccagaaactaattcagtagaaggggagccatcctgtttacaaatccactgtatgcaattgactcgggcggtgtgaccattcaagttggtaacaacaacccttttcagggggtcatagagcaccacggagcaggacgtgccaaaggccagaagtcctctgggcccagagctccagttcaggactccccgcacccggtttgggcagcaaaacacgtgagaagtctccagcacgggtgccaccatgtcgccaactggtcagccgcacaaacaagagacgc

SEQ ID NO: 12485 - RNA, 5165 nt, Homo sapiens
  source 1..5165: mol_type = other RNA
gaaagtgcttccttttagaggctgaataatattccactgtatgaatataccacattttgttgatcattcacccactgatgggcacatattgcttccatctcttagctactgtgaataatggtgccgtgagtatgggcatacaaaaactaccactaatattttacagtgcttgcttcatatctgtccatgtgtccgtcactccacccatcatattttttatgtatttcataagttacagaccacagtaacttccctcaaacatgtcagtatacatatcaatgaccagcgttcattgtttttttccaagtcattttgaactgccgtagcaatgagtaatatagcctcaaacgcacacatacacacacaacacgtgcgtcactacagaaaacttttcctggcagacaggaaagggcccattgttggtgatgtcattttaattaagataaaaccaccaccaccatttagtaatagcctggggtaacaagggctgcgtcacggactgccacttttgccatcctgctcagagcagggccatgcctaacccgtatctggggattgcttcagatattatgaatcgcttcaatattatgaattactacaattcataataattgcttcagatattatgaattacaatatggttcaaaggtgctttagcagatgaagacacaaatgtgtaaacacatatgaattacaatgcagactgcccagatgtgtagcaagtcctctgaatgtttactaaacagtaaggtgattccagaggaagatgcttgaggacaatttgggaaaactgacaacttgaaaactcagtctctctaggcaaggcctacttgcagataaccttgggagttctgtgctgggaggaaagctaaaggactaagttaggcctctgaatctgctctggaagcctgcatgcacttgggtcagaacaagcccatgtgtcaatgtgggtaaagattcctcagctgataagcaggaaaatgggcagggcattttggtctttgaggttcaaagctcagatgctcactgccttggtatacacgcacacacaccccaccccccagctgacggcacaagagtatacagatgcaatagtctaaagtacattgtccaaatatggatggccatgagccacatgtggctatgaagcacttaaatgtggctagtctgaactgagatgggccctataaaatatttcagtaacaggtttttatactgattataggttgacataataatattttggatataccgtattaaaggaaatatgtcattaaatttcacctgtttcctttattatgtggctacttgaaaattttaaaattacatatgtagctcacactataaaacacagattagaaatattgtatagcactgacctagaaacctccatttaggtaaaacatcttaacccctttggaagcaaaatatgttaaataacagcataaactcccaccaagaaaatcctcaccttcctcctttcaacacatttattatatacagctgtcactgcattgtcaatctgccaaatggctctatgttccaacagggctggagtagtcccctgctcacaccagccttcacaatacttcccatgtcttccctgttaacctctctccacccagcacccaggctcccaactctcctggctgcctccagccctcagctggcaccactgacatgctgtttccagtacccttttcttctttctgcatcctccctgggggacatatatccctcatctcgtgacttcagctgtcacataaattcaaatgtttcagaactctattttttacctcctacatctgtcagtttaaatgtcaggatattttactttcagtaaagccctaaaaagacaaatctatgtacttttaaagaataaaagaaatgactggctgcagctcaaacctacaactgcttgcgaaactctacaatgtctggcagatgctagaaagaaggggatcaagacagagcacacttggcgtggtatgctatctatagaaaatgttaaaataaaattaagtaatctaggtttcctctctttattttctacatctactctctgaagagggcaataaataaggaaatgtcccaaagagggacaaattaagtcccaaaataacacaaaattgggcaaatccagtcatgaagaaagaacagaggttcttaaattgggacacacagaggcaggtctgcaggtctaggaatctctgaacatatgtgcaaaattctgggtatgtgtgcatatgttatataacaaagcgaagggtccatatagctttcatcgcatttcaaagggtctagcactgaaataaggactactgctatgtgacttaaaaaatgaaactcaggctgggcgcagtggctcacgcctgtaatcccagcactttgggaggccgaggcaagcagatcacctgagacgaggagtttgagacccgcctggccaacggtgaaacccagtctctactaaaaatacaaaaattagccggaattggtggtgtgcctctagtcccagctactcaggaggctgaagaaagagaatcgcttgaacctgggaggtggaggttgtgacaaagcaagactccatctcaaaaaaaaaaaaaacccagaaactcaattcagttatgaaggtaaagatgacctgtttacatgataatattttaagataccagtgactgcaagcatgtagttattaagtccattacagtgcacatttattgactctgtgtatcttcacagtgtgatcttcaccacagcttgcaaagtgtaaccactcagcaccttctgcttccttctgttcagtttttccactgcaattcttccagcataattttctgatagccagtgtatgactttggctttgacttgtttctacacagtgggtccagtcatttatttctggaacttgatcagtctttttccaggtatataagcaaatctttccacactccaatcctactgcaaccacgtatcgttgagaagggtggagcactgggcagacgctgacagctgtcacagccccacccacgtccaggactgaggagcaggggccaatgttgtgctcaatacagtcatcagtggagtcgcactcaccccagacaaccacctttttgtctcgactcccagtgaagaaatacttgctgtcaggactccaatcacaagaccaaataattctacgaactcaggtgagattgtatcctgctttttccacaatgaccaggttcgatctctggaaacagctagtaagaacttctcattaggtgagaaggccatctgcgtgactgtcaaactgtggaaaactaaattctgcacctgtttccaagatgtagtgttccaaagaatgatagctgcatgctctttcttagctgccttacaagctgaggcaagcagagtctttgaactgttacaagtaacacaaaatatttcataaccgtgcccatatagtttttgaacttcaggccacaaagtattctgcagaagatgatcctcagtgggaggctcagtaagtatggagggctgaaaggccacctgctgatactcaaaaccagtactagttaacagctcctcttcatcagaaggctgagaagctatatctccctgaaagacagctttatttgataatcccaatgcagggacagtggctccttctggaagatcactatcttgattacagagcacatgattcagtgattgtcctgtaatggcacaaaaattttccacaaaattccgaggtgcagaaaaaacccgaagaactttttcatctgctccagatacaaactgaaaccgattaatcattgccaaacatttcaggtcatacccatgtatctgaggccttgcaatttcatgccaagtcacctgtgattggtcttttctcttccatggagcaaaaagtctagttgtctgatcagtaccaacagtgataataaattctccttctggatcccagactaggtcttggacaccatcaaagtgtcctgaaatgacaatctctggagtccactctcttgggttaactgtattctgtttccaaaggtgcaacgctccgtggaaagcatgagcaatgatcatggagccatcttcattgaactggcaatcataaaatcccaaagtattcccacctacttcacctactcgaacctgttctagccaaactcctgactcttcatctggagcccagagaatcatggttttatccatggaagcagataataatctcactggctgctgtaggacaccatctttgtaaaacacaggttgccagtgaactgcatttacccagttttcatgaccggctagcactgtctccagagtaacagcaaatgctattttaacactttcattttctatggtaaaagtattttctttcagtcttatgttatcgtcatcctgagtttctaaagatgttgactttatatacagcttccatattcttatcaggcaatcttgtgaacagcttgctaggaaaagatctctaccaaaggctgcccattccactcctctaatccaatcctcatgtccacagagagaaagcactttctgaaactgatcattttgttgagcaaatatgtgaattctgcaatcatcattgccacatgctaatattggtacatcagtatttggcaaaaaagataagcagagagccaaagcaaatccatttccaaagtttaaagtctgaaggcacattacttctggaccctttttagaccagagtcgaacagcagaatctgcagctgcagaaacgatcagtgtacataatgcaggatctgatgtcctcctctggtaaacagcatgcaccgcataaacaggtccttcatggccttgaagatgcactgcttttaaaagctgattatcctctatttcccagtgaatcacttgattatcagatcctccagaaactaattcagtagaaggggagccatcctgtttacaaatccactgtatgcaattgactcgggcggtgtgaccattcaagttggtaacaacaacccttttcagggggtcatagagcaccacggagcaggacgtgccaaaggccagaagtcctctgggcccagagctccagttcaggactccccgcacccggtttgggcagcaaaacacgtgagaagtctccagcacgggtgccaccatgtcgccaactggtcagccgcacaaacaagagacgc

SEQ ID NO: 12486 - RNA, 5098 nt, Homo sapiens
  source 1..5098: mol_type = other RNA
gaaagtgcttccttttagaggctgaataatattccactgtatgaatataccacattttgttgatcattcacccactgatgggcacatattgcttccatctcttagctactgtgaataatggtgccgtgagtatgggcatacaaaaactaccactaatattttacagtgcttgcttcatatctgtccatgtgtccgtcactccacccatcatattttttatgtatttcataagttacagaccacagtaacttccctcaaacatgtcagtatacatatcaatgaccagcgttcattgtttttttccaagtcattttgaactgccgtagcaatgagtaatatagcctcaaacgcacacatacacacacaacacgtgcgtcactacagaaaacttttcctggcagacaggaaagggcccattgttggtgatgtcattttaattaagataaaaccaccaccaccatttagtaatagcctggggtaacaagggctgcgtcacggactgccacttttgccatcctgctcagagcagggccatgcctaacccgtatctggggattgcttcagatattatgaatcgcttcaatattatgaattactacaattcataataattgcttcagatattatgaattacaatatggttcaaaggtgctttagcagatgaagacacaaatgtgtaaacacatatgaattacaatgcagactgcccagatgtgtagcaagtcctctgaatgtttactaaacagtaaggtgattccagaggaagatgcttgaggacaatttgggaaaactgacaacttgaaaactcagtctctctaggcaaggcctacttgcagataaccttgggagttctgtgctgggaggaaagctaaaggactaagttaggcctctgaatctgctctggaagcctgcatgcacttgggtcagaacaagcccatgtgtcaatgtgggtaaagattcctcagctgataagcaggaaaatgggcagggcattttggtctttgaggttcaaagctcagatgctcactgccttggtatacacgcacacacaccccaccccccagctgacggcacaagagtatacagatgcaatagtctaaagtacattgtccaaatatggatggccatgagccacatgtggctatgaagcacttaaatgtggctagtctgaactgagatgggccctataaaatatttcagtaacaggtttttatactgattataggttgacataataatattttggatataccgtattaaaggaaatatgtcattaaatttcacctgtttcctttattatgtggctacttgaaaattttaaaattacatatgtagctcacactataaaacacagattagaaatattgtatagcactgacctagaaacctccatttaggtaaaacatcttaacccctttggaagcaaaatatgttaaataacagcataaactcccaccaagaaaatcctcaccttcctcctttcaacacatttattatatacagctgtcactgcattgtcaatctgccaaatggctctatgttccaacagggctggagtagtcccctgctcacaccagccttcacaatacttcccatgtcttccctgttaacctctctccacccagcacccaggctcccaactctcctggctgcctccagccctcagctggcaccactgacatgctgtttccagtacccttttcttctttctgcatcctccctgggggacatatatccctcatctcgtgacttcagctgtcacataaattcaaatgtttcagaactctattttttacctcctacatctgtcagtttaaatgtcaggatattttactttcagtaaagccctaaaaagacaaatctatgtacttttaaagaataaaagaaatgactggctgcagctcaaacctacaactgcttgcgaaactctacaatgtctggcagatgctagaaagaaggggatcaagacagagcacacttggcgtggtatgctatctatagaaaatgttaaaataaaattaagtaatctaggtttcctctctttattttctacatctactctctgaagagggcaataaataaggaaatgtcccaaagagggacaaattaagtcccaaaataacacaaaattgggcaaatccagtcatgaagaaagaacagaggttcttaaattgggacacacagaggcaggtctgcaggtctaggaatctctgaacatatgtgcaaaattctgggtatgtgtgcatatgttatataacaaagcgaagggtccatatagctttcatcgcatttcaaagggtctagcactgaaataaggactactgctatgtgacttaaaaaatgaaactcaggctgggcgcagtggctcacgcctgtaatcccagcactttgggaggccgaggcaagcagatcacctgagacgaggagtttgagacccgcctggccaacggtgaaacccagtctctactaaaaatacaaaaattagccggaattggtggtgtgcctctagtcccagctactcaggaggctgaagaaagagaatcgcttgaacctgggaggtggaggttgtgacaaagcaagactccatctcaaaaaaaaaaaaaacccagaaactcaattcagttatgaaggtaaagatgacctgtttacatgataatattttaagataccagtgactgcaagcatgtagttattaagtccattacagtgcacatttattgactctgtgtatcttcacagtgtgatcttcaccacagcttgcaaagtgtaaccactcagcaccttctgcttccttctgttcagtttttccactgcaattcttccagcataattttctgatagccagtgtatgactttggctttgacttgtttctacacagtgggtccagtcatttatttctggaacttgatcagtctttttccaggtatataagcaaatctttccacactccaatcctactgcaaccacgtatcgttgagaagggtggagcactgggcagacgctgacagctgtcacagccccacccacgtccaggactgaggagcaggggccaatgttgtgctcaatacagtcatcagtggagtcgcactcaccccagacaaccacctttttgtctcgactcccagtgaagaaatacttgctgtcaggactccaatcacaagaccaaataattctacgaactcaggtgagattgtatcctgctttttccacaatgaccaggttcgatctctggaaacagctagtaagaacttctcattaggtgagaaggccatctgcgtgactgtcaaactgtggaaaactaaattctgcacctgtttccaagatgtagtgttccaaagaatgatagctgcatgctctttcttagctgccttacaagctgaggcaagcagagtctttgaactgttacaagtaacacaaaatatttcataaccgtgcccatatagtttttgaacttcaggccacaaagtattctgcagaagatgatcctcagtgggaggctcagtaagtatggagggctgaaaggccacctgctgatactcaaaaccagtactagttaacagctcctcttcatcagaaggctgagaagctatatctccctgaaagacagctttatttgataatcccaatgcagggacagtggctccttctggaagatcactatcttgattacagagcacatgattcagtgattgtcctgtaatggcacaaaaattttccacaaaattccgaggtgcagaaaaaacccgaagaactttttcatctgctccagatacaaactgaaaccgattaatcattgccaaacatttcaggtcatacccatgtatctgaggccttgcaatttcatgccaagtcacctgtgattggtcttttctcttccatggagcaaaaagtctagttgtctgatcagtaccaacagtgataataaattctccttctggatcccagactaggtcttggacaccatcaaagtgtcctgaaatgacaatctctggagtccactctcttgggttaactgtattctgtttccaaaggtgcaacgctccgtggaaagcatgagcaatgatcatggagccatcttcattgaactggcaatcataaaatcccaaagtattcccacctacttcacctactcgaacctgttctagccaaactcctgactcttcatctggagcccagagaatcatggttttatccatggaagcagataataatctcactggctgctgtaggacaccatctttgtaaaacacaggttgccagtgaactgcatttacccagttttcatgaccggctagcactgtctccagagtaacagcaaatgctattttaacactttcattttctatggtaaaagtattttctttcagtcttatgttatcgtcatcctgagtttctaaagatgttgactttatatacagcttccatattcttatcaggcaatcttgtgaacagcttgctaggaaaagatctctacctgatcattttgttgagcaaatatgtgaattctgcaatcatcattgccacatgctaatattggtacatcagtatttggcaaaaaagataagcagagagccaaagcaaatccatttccaaagtttaaagtctgaaggcacattacttctggaccctttttagaccagagtcgaacagcagaatctgcagctgcagaaacgatcagtgtacataatgcaggatctgatgtcctcctctggtaaacagcatgcaccgcataaacaggtccttcatggccttgaagatgcactgcttttaaaagctgattatcctctatttcccagtgaatcacttgattatcagatcctccagaaactaattcagtagaaggggagccatcctgtttacaaatccactgtatgcaattgactcgggcggtgtgaccattcaagttggtaacaacaacccttttcagggggtcatagagcaccacggagcaggacgtgccaaaggccagaagtcctctgggcccagagctccagttcaggactccccgcacccggtttgggcagcaaaacacgtgagaagtctccagcacgggtgccaccatgtcgccaactggtcagccgcacaaacaagagacgc

SEQ ID NO: 12487 - RNA, 5085 nt, Homo sapiens
  source 1..5085: mol_type = other RNA
gaaagtgcttccttttagaggctgaataatattccactgtatgaatataccacattttgttgatcattcacccactgatgggcacatattgcttccatctcttagctactgtgaataatggtgccgtgagtatgggcatacaaaaactaccactaatattttacagtgcttgcttcatatctgtccatgtgtccgtcactccacccatcatattttttatgtatttcataagttacagaccacagtaacttccctcaaacatgtcagtatacatatcaatgaccagcgttcattgtttttttccaagtcattttgaactgccgtagcaatgagtaatatagcctcaaacgcacacatacacacacaacacgtgcgtcactacagaaaacttttcctggcagacaggaaagggcccattgttggtgatgtcattttaattaagataaaaccaccaccaccatttagtaatagcctggggtaacaagggctgcgtcacggactgccacttttgccatcctgctcagagcagggccatgcctaacccgtatctggggattgcttcagatattatgaatcgcttcaatattatgaattactacaattcataataattgcttcagatattatgaattacaatatggttcaaaggtgctttagcagatgaagacacaaatgtgtaaacacatatgaattacaatgcagactgcccagatgtgtagcaagtcctctgaatgtttactaaacagtaaggtgattccagaggaagatgcttgaggacaatttgggaaaactgacaacttgaaaactcagtctctctaggcaaggcctacttgcagataaccttgggagttctgtgctgggaggaaagctaaaggactaagttaggcctctgaatctgctctggaagcctgcatgcacttgggtcagaacaagcccatgtgtcaatgtgggtaaagattcctcagctgataagcaggaaaatgggcagggcattttggtctttgaggttcaaagctcagatgctcactgccttggtatacacgcacacacaccccaccccccagctgacggcacaagagtatacagatgcaatagtctaaagtacattgtccaaatatggatggccatgagccacatgtggctatgaagcacttaaatgtggctagtctgaactgagatgggccctataaaatatttcagtaacaggtttttatactgattataggttgacataataatattttggatataccgtattaaaggaaatatgtcattaaatttcacctgtttcctttattatgtggctacttgaaaattttaaaattacatatgtagctcacactataaaacacagattagaaatattgtatagcactgacctagaaacctccatttaggtaaaacatcttaacccctttggaagcaaaatatgttaaataacagcataaactcccaccaagaaaatcctcaccttcctcctttcaacacatttattatatacagctgtcactgcattgtcaatctgccaaatggctctatgttccaacagggctggagtagtcccctgctcacaccagccttcacaatacttcccatgtcttccctgttaacctctctccacccagcacccaggctcccaactctcctggctgcctccagccctcagctggcaccactgacatgctgtttccagtacccttttcttctttctgcatcctccctgggggacatatatccctcatctcgtgacttcagctgtcacataaattcaaatgtttcagaactctattttttacctcctacatctgtcagtttaaatgtcaggatattttactttcagtaaagccctaaaaagacaaatctatgtacttttaaagaataaaagaaatgactggctgcagctcaaacctacaactgcttgcgaaactctacaatgtctggcagatgctagaaagaaggggatcaagacagagcacacttggcgtggtatgctatctatagaaaatgttaaaataaaattaagtaatctaggtttcctctctttattttctacatctactctctgaagagggcaataaataaggaaatgtcccaaagagggacaaattaagtcccaaaataacacaaaattgggcaaatccagtcatgaagaaagaacagaggttcttaaattgggacacacagaggcaggtctgcaggtctaggaatctctgaacatatgtgcaaaattctgggtatgtgtgcatatgttatataacaaagcgaagggtccatatagctttcatcgcatttcaaagggtctagcactgaaataaggactactgctatgtgacttaaaaaatgaaactcaggctgggcgcagtggctcacgcctgtaatcccagcactttgggaggccgaggcaagcagatcacctgagacgaggagtttgagacccgcctggccaacggtgaaacccagtctctactaaaaatacaaaaattagccggaattggtggtgtgcctctagtcccagctactcaggaggctgaagaaagagaatcgcttgaacctgggaggtggaggttgtgacaaagcaagactccatctcaaaaaaaaaaaaaacccagaaactcaattcagttatgaaggtaaagatgacctgtttacatgataatattttaagataccagtgactgcaagcatgtagttattaagtccattacagtgcacatttattgactctgtgtatcttcacagtgtgatcttcaccacagcttgcaaagtgtaaccactcagcaccttctgcttccttctgttcagtttttccactgcaattcttccagcataattttctgatagccagtgtatgactttggctttgacttgtttctacacagtgggtccagtcatttatttctggaacttgatcagtctttttccaggtatataagcaaatctttccacactccaatcctactgcaaccacgtatcgttgagaagggtggagcactgggcagacgctgacagctgtcacagccccacccacgtccaggactgaggagcaggggccaatgttgtgctcaatacagtcatcagtggagtcgcactcaccccagacaaccacctttttgtctcgactcccagtgaagaaatacttgctgtcaggactccaatcacaagaccaaataattctactgtgcacagaagtaattttgttggtgaaggcaaaaagactaaaaactggctcgaactcaggtgagattgtatcctgctttttccacaatgaccaggttcgatctctggaaacagctagtaagaacttctcattaggtgagaaggccatctgcgtgactgtcaaactgtggaaaactaaattctgcacctgtttccaagatgtagtgttccaaagaatgatagctgcatgctctttcttagctgccttacaagctgaggcaagcagagtctttgaactgttacaagtaacacaaaatatttcataaccgtgcccatatagtttttgaacttcaggccacaaagtattctgcagaagatgatcctcagtgggaggctcagtaagtatggagggctgaaaggccacctgctgatactcaaaaccagtactagttaacagctcctcttcatcagaaggctgagaagctatatctccctgaaagacagctttatttgataatcccaatgcagggacagtggctccttctggaagatcactatcttgattacagagcacatgattcagtgattgtcctgtaatggcacaaaaattttccacaaaattccgaggtgcagaaaaaacccgaagaactttttcatctgctccagatacaaactgaaaccgattaatcattgccaaacatttcaggtcatacccatgtatctgaggccttgcaatttcatgccaagtcacctgtgattggtcttttctcttccatggagcaaaaagtctagttgtctgatcagtaccaacagtgataataaattctccttctggatcccagactaggtcttggacaccatcaaagtgtcctgaaatgacaatctctggagtccactctctctgttctagccaaactcctgactcttcatctggagcccagagaatcatggttttatccatggaagcagataataatctcactggctgctgtaggacaccatctttgtaaaacacaggttgccagtgaactgcatttacccagttttcatgaccggctagcactgtctccagagtaacagcaaatgctattttaacactttcattttctatggtaaaagtattttctttcagtcttatgttatcgtcatcctgagtttctaaagatgttgactttatatacagcttccatattcttatcaggcaatcttgtgaacagcttgctaggaaaagatctctaccaaaggctgcccattccactcctctaatccaatcctcatgtccacagagagaaagcactttctgaaactgatcattttgttgagcaaatatgtgaattctgcaatcatcattgccacatgctaatattggtacatcagtatttggcaaaaaagataagcagagagccaaagcaaatccatttccaaagtttaaagtctgaaggcacattacttctggaccctttttagaccagagtcgaacagcagaatctgcagctgcagaaacgatcagtgtacataatgcaggatctgatgtcctcctctggtaaacagcatgcaccgcataaacaggtccttcatggccttgaagatgcactgcttttaaaagctgattatcctctatttcccagtgaatcacttgattatcagatcctccagaaactaattcagtagaaggggagccatcctgtttacaaatccactgtatgcaattgactcgggcggtgtgaccattcaagttggtaacaacaacccttttcagggggtcatagagcaccacggagcaggacgtgccaaaggccagaagtcctctgggcccagagctccagttcaggactccccgcacccggtttgggcagcaaaacacgtgagaagtctccagcacgggtgccaccatgtcgccaactggtcagccgcacaaacaagagacgc

SEQ ID NO: 12488 - RNA, 5007 nt, Homo sapiens
  source 1..5007: mol_type = other RNA
gaaagtgcttccttttagaggctgaataatattccactgtatgaatataccacattttgttgatcattcacccactgatgggcacatattgcttccatctcttagctactgtgaataatggtgccgtgagtatgggcatacaaaaactaccactaatattttacagtgcttgcttcatatctgtccatgtgtccgtcactccacccatcatattttttatgtatttcataagttacagaccacagtaacttccctcaaacatgtcagtatacatatcaatgaccagcgttcattgtttttttccaagtcattttgaactgccgtagcaatgagtaatatagcctcaaacgcacacatacacacacaacacgtgcgtcactacagaaaacttttcctggcagacaggaaagggcccattgttggtgatgtcattttaattaagataaaaccaccaccaccatttagtaatagcctggggtaacaagggctgcgtcacggactgccacttttgccatcctgctcagagcagggccatgcctaacccgtatctggggattgcttcagatattatgaatcgcttcaatattatgaattactacaattcataataattgcttcagatattatgaattacaatatggttcaaaggtgctttagcagatgaagacacaaatgtgtaaacacatatgaattacaatgcagactgcccagatgtgtagcaagtcctctgaatgtttactaaacagtaaggtgattccagaggaagatgcttgaggacaatttgggaaaactgacaacttgaaaactcagtctctctaggcaaggcctacttgcagataaccttgggagttctgtgctgggaggaaagctaaaggactaagttaggcctctgaatctgctctggaagcctgcatgcacttgggtcagaacaagcccatgtgtcaatgtgggtaaagattcctcagctgataagcaggaaaatgggcagggcattttggtctttgaggttcaaagctcagatgctcactgccttggtatacacgcacacacaccccaccccccagctgacggcacaagagtatacagatgcaatagtctaaagtacattgtccaaatatggatggccatgagccacatgtggctatgaagcacttaaatgtggctagtctgaactgagatgggccctataaaatatttcagtaacaggtttttatactgattataggttgacataataatattttggatataccgtattaaaggaaatatgtcattaaatttcacctgtttcctttattatgtggctacttgaaaattttaaaattacatatgtagctcacactataaaacacagattagaaatattgtatagcactgacctagaaacctccatttaggtaaaacatcttaacccctttggaagcaaaatatgttaaataacagcataaactcccaccaagaaaatcctcaccttcctcctttcaacacatttattatatacagctgtcactgcattgtcaatctgccaaatggctctatgttccaacagggctggagtagtcccctgctcacaccagccttcacaatacttcccatgtcttccctgttaacctctctccacccagcacccaggctcccaactctcctggctgcctccagccctcagctggcaccactgacatgctgtttccagtacccttttcttctttctgcatcctccctgggggacatatatccctcatctcgtgacttcagctgtcacataaattcaaatgtttcagaactctattttttacctcctacatctgtcagtttaaatgtcaggatattttactttcagtaaagccctaaaaagacaaatctatgtacttttaaagaataaaagaaatgactggctgcagctcaaacctacaactgcttgcgaaactctacaatgtctggcagatgctagaaagaaggggatcaagacagagcacacttggcgtggtatgctatctatagaaaatgttaaaataaaattaagtaatctaggtttcctctctttattttctacatctactctctgaagagggcaataaataaggaaatgtcccaaagagggacaaattaagtcccaaaataacacaaaattgggcaaatccagtcatgaagaaagaacagaggttcttaaattgggacacacagaggcaggtctgcaggtctaggaatctctgaacatatgtgcaaaattctgggtatgtgtgcatatgttatataacaaagcgaagggtccatatagctttcatcgcatttcaaagggtctagcactgaaataaggactactgctatgtgacttaaaaaatgaaactcaggctgggcgcagtggctcacgcctgtaatcccagcactttgggaggccgaggcaagcagatcacctgagacgaggagtttgagacccgcctggccaacggtgaaacccagtctctactaaaaatacaaaaattagccggaattggtggtgtgcctctagtcccagctactcaggaggctgaagaaagagaatcgcttgaacctgggaggtggaggttgtgacaaagcaagactccatctcaaaaaaaaaaaaaacccagaaactcaattcagttatgaaggtaaagatgacctgtttacatgataatattttaagataccagtgactgcaagcatgtagttattaagtccattacagtgcacatttattgactctgtgtatcttcacagtgtgatcttcaccacagcttgcaaagtgtaaccactcagcaccttctgcttccttctgttcagtttttccactgcaattcttccagcataattttctgatagccagtgtatgactttggctttgacttgtttctacacagtgggtccagtcatttatttctggaacttgatcagtctttttccaggtatataagcaaatctttccacactccaatcctactgcaaccacgtatcgttgagaagggtggagcactgggcagacgctgacagctgtcacagccccacccacgtccaggactgaggagcaggggccaatgttgtgctcaatacagtcatcagtggagtcgcactcaccccagacaaccacctttttgtctcgactcccagtgaagaaatacttgctgtcaggactccaatcacaagaccaaataattctactgtgcacagaagtaattttgttggtgaaggcaaaaagactaaaaactggctcgaactcaggtgagattgtatcctgctttttccacaatgaccaggttcgatctctggaaacagctagtaagaacttctcattaggtgagaaggccatctgcgtgactgtcaaactgtggaaaactaaattctgcacctgtttccaagatgtagtgttccaaagaatgatagctgcatgctctttcttagctgccttacaagctgaggcaagcagagtctttgaactgttacaagtaacacaaaatatttcataaccgtgcccatatagtttttgaacttcaggccacaaagtattctgcagaagatgatcctcagtgggaggctcagtaagtatggagggctgaaaggccacctgctgatactcaaaaccagtactagttaacagctcctcttcatcagaaggctgagaagctatatctccctgaaagacagctttatttgataatcccaatgcagggacagtggctccttctggaagatcactatcttgattacagagcacatgattcagtgattgtcctgtaatggcacaaaaattttccacaaaattccgaggtgcagaaaaaacccgaagaactttttcatctgctccagatacaaactgaaaccgattaatcattgccaaacatttcaggtcatacccatgtatctgaggccttgcaatttcatgccaagtcacctgtgattggtcttttctcttccatggagcaaaaagtctagttgtctgatcagtaccaacagtgataataaattctccttctggatcccagactaggtcttggacaccatcaaagtgtcctgaaatgacaatctctggagtccactctctctgttctagccaaactcctgactcttcatctggagcccagagaatcatggttttatccatggaagcagataataatctcactggctgctgtaggacaccatctttgtaaaacacaggttgccagtgaactgcatttacccagttttcatgaccggctagcactgtctccagagtaacagcaaatgctattttaacactttcattttctatggtaaaagtattttctttcagtcttatgttatcgtcatcctgagtttctaaagatgttgactttatatacagcttccatattcttatcaggcaatcttgtgaacagcttgctaggaaaagatctctaccaaaggctgcccattccactcctctaatccaatcctcatgtccacagagagaaagcactttctgaaactgatcattttgttgagcaaatatgtgaattctgcaatcatcattgccacatgctaatattggtacttctggaccctttttagaccagagtcgaacagcagaatctgcagctgcagaaacgatcagtgtacataatgcaggatctgatgtcctcctctggtaaacagcatgcaccgcataaacaggtccttcatggccttgaagatgcactgcttttaaaagctgattatcctctatttcccagtgaatcacttgattatcagatcctccagaaactaattcagtagaaggggagccatcctgtttacaaatccactgtatgcaattgactcgggcggtgtgaccattcaagttggtaacaacaacccttttcagggggtcatagagcaccacggagcaggacgtgccaaaggccagaagtcctctgggcccagagctccagttcaggactccccgcacccggtttgggcagcaaaacacgtgagaagtctccagcacgggtgccaccatgtcgccaactggtcagccgcacaaacaagagacgc

SEQ ID NO: 12489 - RNA, 5202 nt, Homo sapiens
  source 1..5202: mol_type = other RNA
gaaagtgcttccttttagaggctgaataatattccactgtatgaatataccacattttgttgatcattcacccactgatgggcacatattgcttccatctcttagctactgtgaataatggtgccgtgagtatgggcatacaaaaactaccactaatattttacagtgcttgcttcatatctgtccatgtgtccgtcactccacccatcatattttttatgtatttcataagttacagaccacagtaacttccctcaaacatgtcagtatacatatcaatgaccagcgttcattgtttttttccaagtcattttgaactgccgtagcaatgagtaatatagcctcaaacgcacacatacacacacaacacgtgcgtcactacagaaaacttttcctggcagacaggaaagggcccattgttggtgatgtcattttaattaagataaaaccaccaccaccatttagtaatagcctggggtaacaagggctgcgtcacggactgccacttttgccatcctgctcagagcagggccatgcctaacccgtatctggggattgcttcagatattatgaatcgcttcaatattatgaattactacaattcataataattgcttcagatattatgaattacaatatggttcaaaggtgctttagcagatgaagacacaaatgtgtaaacacatatgaattacaatgcagactgcccagatgtgtagcaagtcctctgaatgtttactaaacagtaaggtgattccagaggaagatgcttgaggacaatttgggaaaactgacaacttgaaaactcagtctctctaggcaaggcctacttgcagataaccttgggagttctgtgctgggaggaaagctaaaggactaagttaggcctctgaatctgctctggaagcctgcatgcacttgggtcagaacaagcccatgtgtcaatgtgggtaaagattcctcagctgataagcaggaaaatgggcagggcattttggtctttgaggttcaaagctcagatgctcactgccttggtatacacgcacacacaccccaccccccagctgacggcacaagagtatacagatgcaatagtctaaagtacattgtccaaatatggatggccatgagccacatgtggctatgaagcacttaaatgtggctagtctgaactgagatgggccctataaaatatttcagtaacaggtttttatactgattataggttgacataataatattttggatataccgtattaaaggaaatatgtcattaaatttcacctgtttcctttattatgtggctacttgaaaattttaaaattacatatgtagctcacactataaaacacagattagaaatattgtatagcactgacctagaaacctccatttaggtaaaacatcttaacccctttggaagcaaaatatgttaaataacagcataaactcccaccaagaaaatcctcaccttcctcctttcaacacatttattatatacagctgtcactgcattgtcaatctgccaaatggctctatgttccaacagggctggagtagtcccctgctcacaccagccttcacaatacttcccatgtcttccctgttaacctctctccacccagcacccaggctcccaactctcctggctgcctccagccctcagctggcaccactgacatgctgtttccagtacccttttcttctttctgcatcctccctgggggacatatatccctcatctcgtgacttcagctgtcacataaattcaaatgtttcagaactctattttttacctcctacatctgtcagtttaaatgtcaggatattttactttcagtaaagccctaaaaagacaaatctatgtacttttaaagaataaaagaaatgactggctgcagctcaaacctacaactgcttgcgaaactctacaatgtctggcagatgctagaaagaaggggatcaagacagagcacacttggcgtggtatgctatctatagaaaatgttaaaataaaattaagtaatctaggtttcctctctttattttctacatctactctctgaagagggcaataaataaggaaatgtcccaaagagggacaaattaagtcccaaaataacacaaaattgggcaaatccagtcatgaagaaagaacagaggttcttaaattgggacacacagaggcaggtctgcaggtctaggaatctctgaacatatgtgcaaaattctgggtatgtgtgcatatgttatataacaaagcgaagggtccatatagctttcatcgcatttcaaagggtctagcactgaaataaggactactgctatgtgacttaaaaaatgaaactcaggctgggcgcagtggctcacgcctgtaatcccagcactttgggaggccgaggcaagcagatcacctgagacgaggagtttgagacccgcctggccaacggtgaaacccagtctctactaaaaatacaaaaattagccggaattggtggtgtgcctctagtcccagctactcaggaggctgaagaaagagaatcgcttgaacctgggaggtggaggttgtgacaaagcaagactccatctcaaaaaaaaaaaaaacccagaaactcaattcagttatgaaggtaaagatgacctgtttacatgataatattttaagataccagtgactgcaagcatgtagttattaagtccattacagtgcacatttattgactctgtgtatcttcacagtgtgatcttcaccacagcttgcaaagtgtaaccactcagcaccttctgcttccttctgttcagtttttccactgcaattcttccagcataattttctgatagccagtgtatgactttggctttgacttgtttctacacagtgggtccagtcatttatttctggaacttgatcagtctttttccaggtatataagcaaatctttccacactccaatcctactgcaaccacgtatcgttgagaagggtggagcactgggcagacgctgacagctgtcacagccccacccacgtccaggactgaggagcaggggccaatgttgtgctcaatacagtcatcagtggagtcgcactcaccccagacaaccacctttttgtctcgactcccagtgaagaaatacttgctgtcaggactccaatcacaagaccaaataattctactgtgcacagaagtaattttgttggtgaaggcaaaaagactaaaaactggctcgaactcaggtgagattgtatcctgctttttccacaatgaccaggttcgatctctggaaacagctagtaagaacttctcattaggtgagaaggccatctgcgtgactgtcaaactgtggaaaactaaattctgcacctgtttccaagatgtagtgttccaaagaatgatagctgcatgctctttcttagctgccttacaagctgaggcaagcagagtctttgaactgttacaagtaacacaaaatatttcataaccgtgcccatatagtttttgaacttcaggccacaaagtattctgcagaagatgatcctcagtgggaggctcagtaagtatggagggctgaaaggccacctgctgatactcaaaaccagtactagttaacagctcctcttcatcagaaggctgagaagctatatctccctgaaagacagctttatttgataatcccaatgcagggacagtggctccttctggaagatcactatcttgattacagagcacatgattcagtgattgtcctgtaatggcacaaaaattttccacaaaattccgaggtgcagaaaaaacccgaagaactttttcatctgctccagatacaaactgaaaccgattaatcattgccaaacatttcaggtcatacccatgtatctgaggccttgcaatttcatgccaagtcacctgtgattggtcttttctcttccatggagcaaaaagtctagttgtctgatcagtaccaacagtgataataaattctccttctggatcccagactaggtcttggacaccatcaaagtgtcctgaaatgacaatctctggagtccactctctctgttctagccaaactcctgactcttcatctggagcccagagaatcatggttttatccatggaagcagataataatctcactggctgctgtaggacaccatctttgtaaaacacaggttgccagtgaactgcatttacccagttttcatgaccggctagcactgtctccagagtaacagcaaatgctattttaacactttcattttctatggtaaaagtattttctttcagtcttatgttatcgtcatcctgagtttctaaagatgttgactttatatacagcttccatattcttatcaggcaatcttgtgaacagcttgctaggaaaagatctctaccaaaggctgcccattccactcctctaatccaatcctcatgtccacagagagaaagcactttctgaaactgatcattttgttgagcaaatatgtgaattctgcaatcatcattgccacatgctaatattggtattggcctgaatgcagatggaagaaatgaaattctgttatgatgccagaatgtgtgcagcttctccttccacagagccttgcacagaatggaagcgtaacatgaaaccatagagtcgcagctcctgctacagagggcgagagaggctggtggcttccaggccctgcctcgttccacctggccagtcttccaggtaacttctggaccctttttagaccagagtcgaacagcagaatctgcagctgcagaaacgatcagtgtacataatgcaggatctgatgtcctcctctggtaaacagcatgcaccgcataaacaggtccttcatggccttgaagatgcactgcttttaaaagctgattatcctctatttcccagtgaatcacttgattatcagatcctccagaaactaattcagtagaaggggagccatcctgtttacaaatccactgtatgcaattgactcgggcggtgtgaccattcaagttggtaacaacaacccttttcagggggtcatagagcaccacggagcaggacgtgccaaaggccagaagtcctctgggcccagagctccagttcaggactccccgcacccggtttgggcagcaaaacacgtgagaagtctccagcacgggtgccaccatgtcgccaactggtcagccgcacaaacaagagacgc

SEQ ID NO: 12490 - RNA, 5217 nt, Homo sapiens
  source 1..5217: mol_type = other RNA
gaaagtgcttccttttagaggctgaataatattccactgtatgaatataccacattttgttgatcattcacccactgatgggcacatattgcttccatctcttagctactgtgaataatggtgccgtgagtatgggcatacaaaaactaccactaatattttacagtgcttgcttcatatctgtccatgtgtccgtcactccacccatcatattttttatgtatttcataagttacagaccacagtaacttccctcaaacatgtcagtatacatatcaatgaccagcgttcattgtttttttccaagtcattttgaactgccgtagcaatgagtaatatagcctcaaacgcacacatacacacacaacacgtgcgtcactacagaaaacttttcctggcagacaggaaagggcccattgttggtgatgtcattttaattaagataaaaccaccaccaccatttagtaatagcctggggtaacaagggctgcgtcacggactgccacttttgccatcctgctcagagcagggccatgcctaacccgtatctggggattgcttcagatattatgaatcgcttcaatattatgaattactacaattcataataattgcttcagatattatgaattacaatatggttcaaaggtgctttagcagatgaagacacaaatgtgtaaacacatatgaattacaatgcagactgcccagatgtgtagcaagtcctctgaatgtttactaaacagtaaggtgattccagaggaagatgcttgaggacaatttgggaaaactgacaacttgaaaactcagtctctctaggcaaggcctacttgcagataaccttgggagttctgtgctgggaggaaagctaaaggactaagttaggcctctgaatctgctctggaagcctgcatgcacttgggtcagaacaagcccatgtgtcaatgtgggtaaagattcctcagctgataagcaggaaaatgggcagggcattttggtctttgaggttcaaagctcagatgctcactgccttggtatacacgcacacacaccccaccccccagctgacggcacaagagtatacagatgcaatagtctaaagtacattgtccaaatatggatggccatgagccacatgtggctatgaagcacttaaatgtggctagtctgaactgagatgggccctataaaatatttcagtaacaggtttttatactgattataggttgacataataatattttggatataccgtattaaaggaaatatgtcattaaatttcacctgtttcctttattatgtggctacttgaaaattttaaaattacatatgtagctcacactataaaacacagattagaaatattgtatagcactgacctagaaacctccatttaggtaaaacatcttaacccctttggaagcaaaatatgttaaataacagcataaactcccaccaagaaaatcctcaccttcctcctttcaacacatttattatatacagctgtcactgcattgtcaatctgccaaatggctctatgttccaacagggctggagtagtcccctgctcacaccagccttcacaatacttcccatgtcttccctgttaacctctctccacccagcacccaggctcccaactctcctggctgcctccagccctcagctggcaccactgacatgctgtttccagtacccttttcttctttctgcatcctccctgggggacatatatccctcatctcgtgacttcagctgtcacataaattcaaatgtttcagaactctattttttacctcctacatctgtcagtttaaatgtcaggatattttactttcagtaaagccctaaaaagacaaatctatgtacttttaaagaataaaagaaatgactggctgcagctcaaacctacaactgcttgcgaaactctacaatgtctggcagatgctagaaagaaggggatcaagacagagcacacttggcgtggtatgctatctatagaaaatgttaaaataaaattaagtaatctaggtttcctctctttattttctacatctactctctgaagagggcaataaataaggaaatgtcccaaagagggacaaattaagtcccaaaataacacaaaattgggcaaatccagtcatgaagaaagaacagaggttcttaaattgggacacacagaggcaggtctgcaggtctaggaatctctgaacatatgtgcaaaattctgggtatgtgtgcatatgttatataacaaagcgaagggtccatatagctttcatcgcatttcaaagggtctagcactgaaataaggactactgctatgtgacttaaaaaatgaaactcaggctgggcgcagtggctcacgcctgtaatcccagcactttgggaggccgaggcaagcagatcacctgagacgaggagtttgagacccgcctggccaacggtgaaacccagtctctactaaaaatacaaaaattagccggaattggtggtgtgcctctagtcccagctactcaggaggctgaagaaagagaatcgcttgaacctgggaggtggaggttgtgacaaagcaagactccatctcaaaaaaaaaaaaaacccagaaactcaattcagttatgaaggtaaagatgacctgtttacatgataatattttaagataccagtgactgcaagcatgtagttattaagtccattacagtgcacatttattgactctgtgtatcttcacagtgtgatcttcaccacagcttgcaaagtgtaaccactcagcaccttctgcttccttctgttcagtttttccactgcaattcttccagcataattttctgatagccagtgtatgactttggctttgacttgtttctacacagtgggtccagtcatttatttctggaacttgatcagtctttttccaggtatataagcaaatctttccacactccaatcctactgcaaccacgtatcgttgagaagggtggagcactgggcagacgctgacagctgtcacagccccacccacgtccaggactgaggagcaggggccaatgttgtgctcaatacagtcatcagtggagtcgcactcaccccagacaaccacctttttgtctcgactcccagtgaagaaatacttgctgtcaggactccaatcacaagaccaaataattctactgtgcacagaagtaattttgttggtgaaggcaaaaagactaaaaactggctcgaactcaggtgagattgtatcctgctttttccacaatgaccaggttcgatctctggaaacagctagtaagaacttctcattaggtgagaaggccatctgcgtgactgtcaaactgtggaaaactaaattctgcacctgtttccaagatgtagtgttccaaagaatgatagctgcatgctctttcttagctgccttacaagctgaggcaagcagagtctttgaactgttacaagtaacacaaaatatttcataaccgtgcccatatagtttttgaacttcaggccacaaagtattctgcagaagatgatcctcagtgggaggctcagtaagtatggagggctgaaaggccacctgctgatactcaaaaccagtactagttaacagctcctcttcatcagaaggctgagaagctatatctccctgaaagacagctttatttgataatcccaatgcagggacagtggctccttctggaagatcactatcttgattacagagcacatgattcagtgattgtcctgtaatggcacaaaaattttccacaaaattccgaggtgcagaaaaaacccgaagaactttttcatctgctccagatacaaactgaaaccgattaatcattgccaaacatttcaggtcatacccatgtatctgaggccttgcaatttcatgccaagtcacctgtgattggtcttttctcttccatggagcaaaaagtctagttgtctgatcagtaccaacagtgataataaattctccttctggatcccagactaggtcttggacaccatcaaagtgtcctgaaatgacaatctctggagtccactctcttgggttaactgtattctgtttccaaaggtgcaacgctccgtggaaagcatgagcaatgatcatggagccatcttcattgaactggcaatcataaaatcccaaagtattcccacctacttcacctactcgaacctgttctagccaaactcctgactcttcatctggagcccagagaatcatggttttatccatggaagcagataataatctcactggctgctgtaggacaccatctttgtaaaacacaggttgccagtgaactgcatttacccagttttcatgaccggctagcactgtctccagagtaacagcaaatgctattttaacactttcattttctatggtaaaagtattttctttcagtcttatgttatcgtcatcctgagtttctaaagatgttgactttatatacagcttccatattcttatcaggcaatcttgtgaacagcttgctaggaaaagatctctaccaaaggctgcccattccactcctctaatccaatcctcatgtccacagagagaaagcactttctgaaactgatcattttgttgagcaaatatgtgaattctgcaatcatcattgccacatgctaatattggtacatcagtatttggcaaaaaagataagcagagagccaaagcaaatccatttccaaagtttaaagtctgaaggcacattacttctggaccctttttagaccagagtcgaacagcagaatctgcagctgcagaaacgatcagtgtacataatgcaggatctgatgtcctcctctggtaaacagcatgcaccgcataaacaggtccttcatggccttgaagatgcactgcttttaaaagctgattatcctctatttcccagtgaatcacttgattatcagatcctccagaaactaattcagtagaaggggagccatcctgtttacaaatccactgtatgcaattgactcgggcggtgtgaccattcaagttggtaacaacaacccttttcagggggtcatagagcaccacggagcaggacgtgccaaaggccagaagtcctctgggcccagagctccagttcaggactccccgcacccggtttgggcagcaaaacacgtgagaagtctccagcacgggtgccaccatgtcgccaactggtcagccgcacaaacaagagacgc

SEQ ID NO: 12491 - RNA, 5138 nt, Homo sapiens
  source 1..5138: mol_type = other RNA
gaaagtgcttccttttagaggctgaataatattccactgtatgaatataccacattttgttgatcattcacccactgatgggcacatattgcttccatctcttagctactgtgaataatggtgccgtgagtatgggcatacaaaaactaccactaatattttacagtgcttgcttcatatctgtccatgtgtccgtcactccacccatcatattttttatgtatttcataagttacagaccacagtaacttccctcaaacatgtcagtatacatatcaatgaccagcgttcattgtttttttccaagtcattttgaactgccgtagcaatgagtaatatagcctcaaacgcacacatacacacacaacacgtgcgtcactacagaaaacttttcctggcagacaggaaagggcccattgttggtgatgtcattttaattaagataaaaccaccaccaccatttagtaatagcctggggtaacaagggctgcgtcacggactgccacttttgccatcctgctcagagcagggccatgcctaacccgtatctggggattgcttcagatattatgaatcgcttcaatattatgaattactacaattcataataattgcttcagatattatgaattacaatatggttcaaaggtgctttagcagatgaagacacaaatgtgtaaacacatatgaattacaatgcagactgcccagatgtgtagcaagtcctctgaatgtttactaaacagtaaggtgattccagaggaagatgcttgaggacaatttgggaaaactgacaacttgaaaactcagtctctctaggcaaggcctacttgcagataaccttgggagttctgtgctgggaggaaagctaaaggactaagttaggcctctgaatctgctctggaagcctgcatgcacttgggtcagaacaagcccatgtgtcaatgtgggtaaagattcctcagctgataagcaggaaaatgggcagggcattttggtctttgaggttcaaagctcagatgctcactgccttggtatacacgcacacacaccccaccccccagctgacggcacaagagtatacagatgcaatagtctaaagtacattgtccaaatatggatggccatgagccacatgtggctatgaagcacttaaatgtggctagtctgaactgagatgggccctataaaatatttcagtaacaggtttttatactgattataggttgacataataatattttggatataccgtattaaaggaaatatgtcattaaatttcacctgtttcctttattatgtggctacttgaaaattttaaaattacatatgtagctcacactataaaacacagattagaaatattgtatagcactgacctagaaacctccatttaggtaaaacatcttaacccctttggaagcaaaatatgttaaataacagcataaactcccaccaagaaaatcctcaccttcctcctttcaacacatttattatatacagctgtcactgcattgtcaatctgccaaatggctctatgttccaacagggctggagtagtcccctgctcacaccagccttcacaatacttcccatgtcttccctgttaacctctctccacccagcacccaggctcccaactctcctggctgcctccagccctcagctggcaccactgacatgctgtttccagtacccttttcttctttctgcatcctccctgggggacatatatccctcatctcgtgacttcagctgtcacataaattcaaatgtttcagaactctattttttacctcctacatctgtcagtttaaatgtcaggatattttactttcagtaaagccctaaaaagacaaatctatgtacttttaaagaataaaagaaatgactggctgcagctcaaacctacaactgcttgcgaaactctacaatgtctggcagatgctagaaagaaggggatcaagacagagcacacttggcgtggtatgctatctatagaaaatgttaaaataaaattaagtaatctaggtttcctctctttattttctacatctactctctgaagagggcaataaataaggaaatgtcccaaagagggacaaattaagtcccaaaataacacaaaattgggcaaatccagtcatgaagaaagaacagaggttcttaaattgggacacacagaggcaggtctgcaggtctaggaatctctgaacatatgtgcaaaattctgggtatgtgtgcatatgttatataacaaagcgaagggtccatatagctttcatcgcatttcaaagggtctagcactgaaataaggactactgctatgtgacttaaaaaatgaaactcaggctgggcgcagtggctcacgcctgtaatcccagcactttgggaggccgaggcaagcagatcacctgagacgaggagtttgagacccgcctggccaacggtgaaacccagtctctactaaaaatacaaaaattagccggaattggtggtgtgcctctagtcccagctactcaggaggctgaagaaagagaatcgcttgaacctgggaggtggaggttgtgacaaagcaagactccatctcaaaaaaaaaaaaaacccagaaactcaattcagttatgaaggtaaagatgacctgtttacatgataatattttaagataccagtgactgcaagcatgtagttattaagtccattacagtgcacatttattgactctgtgtatcttcacagtgtgatcttcaccacagcttgcaaagtgtaaccactcagcaccttctgcttccttctgttcagtttttccactgcaattcttccagcataattttctgatagccagtgtatgactttggctttgacttgtttctacacagtgggtccagtcatttatttctggaacttgatcagtctttttccaggtatataagcaaatctttccacactccaatcctactgcaaccacgtatcgttgagaagggtggagcactgggcagacgctgacagctgtcacagccccacccacgtccaggactgaggagcaggggccaatgttgtgctcaatacagtcatcagtggagtcgcactcaccccagacaaccacctttttgtctcgactcccagtgaagaaatacttgctgtcaggactccaatcacaagaccaaataattctactgtgcacagaagtaattttgttggtgaaggcaaaaagactaaaaactggctcgaactcaggtgagattgtatcctgctttttccacaatgaccaggttcgatctctggaaacagctagtaagaacttctcattaggtgagaaggccatctgcgtgactgtcaaactgtggaaaactaaattctgcacctgtttccaagatgtagtgttccaaagaatgatagctgcatgctctttcttagctgccttacaagctgaggcaagcagagtctttgaactgttacaagtaacacaaaatatttcataaccgtgcccatatagtttttgaacttcaggccacaaagtattctgcagaagatgatcctcagtgggaggctcagtaagtatggagggctgaaaggccacctgctgatactcaaaaccagtactagttaacagctcctcttcatcagaaggctgagaagctatatctccctgaaagacagctttatttgataatcccaatgcagggacagtggctccttctggaagatcactatcttgattacagagcacatgattcagtgattgtcctgtaatggcacaaaaattttccacaaaattccgaggtgcagaaaaaacccgaagaactttttcatctgctccagatacaaactgaaaccgattaatcattgccaaacatttcaggtcatacccatgtatctgaggccttgcaatttcatgccaagtcacctgtgattggtcttttctcttccatggagcaaaaagtctagttgtctgatcagtaccaacagtgataataaattctccttctggatcccagactaggtcttggacaccatcaaagtgtcctgaaatgacaatctctggagtccactctcttgggttaactgtattctgtttccaaaggtgcaacgctccgtggaaagcatgagcaatgatcatggagccatcttcattgaactggcaatcataaaatcccaaagtattcccacctacttcacctactcgaacctgttctagccaaactcctgactcttcatctggagcccagagaatcatggttttatccatggaagcagataataatctcactggctgctgtaggacaccatctttgtaaaacacaggttgccagtgaactgcatttacccagttttcatgaccggctagcactgtctccagagtaacagcaaatgctattttaacactttcattttctatggtaaaagtattttctttcagtcttatgttatcgtcatcctgagtttctaaagatgttgactttatatacagcttccatattcttatcaggcaatcttgtgaacagcttgctaggaaaagatctctaccaaaggctgcccattccactcctctaatccaatcctcatgtccacagagagaaagcactttctgaaactgatcattttgttgagcaaatatgtgaattctgcaatcatcattgccacatgctaatattggtacatcagtatttggcaaaaaagataagcagagagccaaagcaaatccatttccaaagtttaaagtctgaaggcacattacttctggaccctttttagaccagagtcgaacagcagaatctgcagctgcagaaacgatcagtgtacataatgcaggatctgatgtcctcctctggtaaacagcatgcaccgcataaacaggtccttcatggccttgaagatgcactgcttttaaaagctgattatcctctatttcccagtgaatcacttgattatcagatcctccagaaactaattcagtagaaggggcagggggtcatagagcaccacggagcaggacgtgccaaaggccagaagtcctctgggcccagagctccagttcaggactccccgcacccggtttgggcagcaaaacacgtgagaagtctccagcacgggtgccaccatgtcgccaactggtcagccgcacaaacaagagacgc

SEQ ID NO: 12492 - RNA, 5139 nt, Homo sapiens
  source 1..5139: mol_type = other RNA
gaaagtgcttccttttagaggctgaataatattccactgtatgaatataccacattttgttgatcattcacccactgatgggcacatattgcttccatctcttagctactgtgaataatggtgccgtgagtatgggcatacaaaaactaccactaatattttacagtgcttgcttcatatctgtccatgtgtccgtcactccacccatcatattttttatgtatttcataagttacagaccacagtaacttccctcaaacatgtcagtatacatatcaatgaccagcgttcattgtttttttccaagtcattttgaactgccgtagcaatgagtaatatagcctcaaacgcacacatacacacacaacacgtgcgtcactacagaaaacttttcctggcagacaggaaagggcccattgttggtgatgtcattttaattaagataaaaccaccaccaccatttagtaatagcctggggtaacaagggctgcgtcacggactgccacttttgccatcctgctcagagcagggccatgcctaacccgtatctggggattgcttcagatattatgaatcgcttcaatattatgaattactacaattcataataattgcttcagatattatgaattacaatatggttcaaaggtgctttagcagatgaagacacaaatgtgtaaacacatatgaattacaatgcagactgcccagatgtgtagcaagtcctctgaatgtttactaaacagtaaggtgattccagaggaagatgcttgaggacaatttgggaaaactgacaacttgaaaactcagtctctctaggcaaggcctacttgcagataaccttgggagttctgtgctgggaggaaagctaaaggactaagttaggcctctgaatctgctctggaagcctgcatgcacttgggtcagaacaagcccatgtgtcaatgtgggtaaagattcctcagctgataagcaggaaaatgggcagggcattttggtctttgaggttcaaagctcagatgctcactgccttggtatacacgcacacacaccccaccccccagctgacggcacaagagtatacagatgcaatagtctaaagtacattgtccaaatatggatggccatgagccacatgtggctatgaagcacttaaatgtggctagtctgaactgagatgggccctataaaatatttcagtaacaggtttttatactgattataggttgacataataatattttggatataccgtattaaaggaaatatgtcattaaatttcacctgtttcctttattatgtggctacttgaaaattttaaaattacatatgtagctcacactataaaacacagattagaaatattgtatagcactgacctagaaacctccatttaggtaaaacatcttaacccctttggaagcaaaatatgttaaataacagcataaactcccaccaagaaaatcctcaccttcctcctttcaacacatttattatatacagctgtcactgcattgtcaatctgccaaatggctctatgttccaacagggctggagtagtcccctgctcacaccagccttcacaatacttcccatgtcttccctgttaacctctctccacccagcacccaggctcccaactctcctggctgcctccagccctcagctggcaccactgacatgctgtttccagtacccttttcttctttctgcatcctccctgggggacatatatccctcatctcgtgacttcagctgtcacataaattcaaatgtttcagaactctattttttacctcctacatctgtcagtttaaatgtcaggatattttactttcagtaaagccctaaaaagacaaatctatgtacttttaaagaataaaagaaatgactggctgcagctcaaacctacaactgcttgcgaaactctacaatgtctggcagatgctagaaagaaggggatcaagacagagcacacttggcgtggtatgctatctatagaaaatgttaaaataaaattaagtaatctaggtttcctctctttattttctacatctactctctgaagagggcaataaataaggaaatgtcccaaagagggacaaattaagtcccaaaataacacaaaattgggcaaatccagtcatgaagaaagaacagaggttcttaaattgggacacacagaggcaggtctgcaggtctaggaatctctgaacatatgtgcaaaattctgggtatgtgtgcatatgttatataacaaagcgaagggtccatatagctttcatcgcatttcaaagggtctagcactgaaataaggactactgctatgtgacttaaaaaatgaaactcaggctgggcgcagtggctcacgcctgtaatcccagcactttgggaggccgaggcaagcagatcacctgagacgaggagtttgagacccgcctggccaacggtgaaacccagtctctactaaaaatacaaaaattagccggaattggtggtgtgcctctagtcccagctactcaggaggctgaagaaagagaatcgcttgaacctgggaggtggaggttgtgacaaagcaagactccatctcaaaaaaaaaaaaaacccagaaactcaattcagttatgaaggtaaagatgacctgtttacatgataatattttaagataccagtgactgcaagcatgtagttattaagtccattacagtgcacatttattgactctgtgtatcttcacagtgtgatcttcaccacagcttgcaaagtgtaaccactcagcaccttctgcttccttctgttcagtttttccactgcaattcttccagcataattttctgatagccagtgtatgactttggctttgacttgtttctacacagtgggtccagtcatttatttctggaacttgatcagtctttttccaggtatataagcaaatctttccacactccaatcctactgcaaccacgtatcgttgagaagggtggagcactgggcagacgctgacagctgtcacagccccacccacgtccaggactgaggagcaggggccaatgttgtgctcaatacagtcatcagtggagtcgcactcaccccagacaaccacctttttgtctcgactcccagtgaagaaatacttgctgtcaggactccaatcacaagaccaaataattctactgtgcacagaagtaattttgttggtgaaggcaaaaagactaaaaactggctcgaactcaggtgagattgtatcctgctttttccacaatgaccaggttcgatctctggaaacagctagtaagaacttctcattaggtgagaaggccatctgcgtgactgtcaaactgtggaaaactaaattctgcacctgtttccaagatgtagtgttccaaagaatgatagctgcatgctctttcttagctgccttacaagctgaggcaagcagagtctttgaactgttacaagtaacacaaaatatttcataaccgtgcccatatagtttttgaacttcaggccacaaagtattctgcagaagatgatcctcagtgggaggctcagtaagtatggagggctgaaaggccacctgctgatactcaaaaccagtactagttaacagctcctcttcatcagaaggctgagaagctatatctccctgaaagacagctttatttgataatcccaatgcagggacagtggctccttctggaagatcactatcttgattacagagcacatgattcagtgattgtcctgtaatggcacaaaaattttccacaaaattccgaggtgcagaaaaaacccgaagaactttttcatctgctccagatacaaactgaaaccgattaatcattgccaaacatttcaggtcatacccatgtatctgaggccttgcaatttcatgccaagtcacctgtgattggtcttttctcttccatggagcaaaaagtctagttgtctgatcagtaccaacagtgataataaattctccttctggatcccagactaggtcttggacaccatcaaagtgtcctgaaatgacaatctctggagtccactctcttgggttaactgtattctgtttccaaaggtgcaacgctccgtggaaagcatgagcaatgatcatggagccatcttcattgaactggcaatcataaaatcccaaagtattcccacctacttcacctactcgaacctgttctagccaaactcctgactcttcatctggagcccagagaatcatggttttatccatggaagcagataataatctcactggctgctgtaggacaccatctttgtaaaacacaggttgccagtgaactgcatttacccagttttcatgaccggctagcactgtctccagagtaacagcaaatgctattttaacactttcattttctatggtaaaagtattttctttcagtcttatgttatcgtcatcctgagtttctaaagatgttgactttatatacagcttccatattcttatcaggcaatcttgtgaacagcttgctaggaaaagatctctaccaaaggctgcccattccactcctctaatccaatcctcatgtccacagagagaaagcactttctgaaactgatcattttgttgagcaaatatgtgaattctgcaatcatcattgccacatgctaatattggtacttctggaccctttttagaccagagtcgaacagcagaatctgcagctgcagaaacgatcagtgtacataatgcaggatctgatgtcctcctctggtaaacagcatgcaccgcataaacaggtccttcatggccttgaagatgcactgcttttaaaagctgattatcctctatttcccagtgaatcacttgattatcagatcctccagaaactaattcagtagaaggggagccatcctgtttacaaatccactgtatgcaattgactcgggcggtgtgaccattcaagttggtaacaacaacccttttcagggggtcatagagcaccacggagcaggacgtgccaaaggccagaagtcctctgggcccagagctccagttcaggactccccgcacccggtttgggcagcaaaacacgtgagaagtctccagcacgggtgccaccatgtcgccaactggtcagccgcacaaacaagagacgc

SEQ ID NO: 12493 - RNA, 5412 nt, Homo sapiens
  source 1..5412: mol_type = other RNA
gaaagtgcttccttttagaggctgaataatattccactgtatgaatataccacattttgttgatcattcacccactgatgggcacatattgcttccatctcttagctactgtgaataatggtgccgtgagtatgggcatacaaaaactaccactaatattttacagtgcttgcttcatatctgtccatgtgtccgtcactccacccatcatattttttatgtatttcataagttacagaccacagtaacttccctcaaacatgtcagtatacatatcaatgaccagcgttcattgtttttttccaagtcattttgaactgccgtagcaatgagtaatatagcctcaaacgcacacatacacacacaacacgtgcgtcactacagaaaacttttcctggcagacaggaaagggcccattgttggtgatgtcattttaattaagataaaaccaccaccaccatttagtaatagcctggggtaacaagggctgcgtcacggactgccacttttgccatcctgctcagagcagggccatgcctaacccgtatctggggattgcttcagatattatgaatcgcttcaatattatgaattactacaattcataataattgcttcagatattatgaattacaatatggttcaaaggtgctttagcagatgaagacacaaatgtgtaaacacatatgaattacaatgcagactgcccagatgtgtagcaagtcctctgaatgtttactaaacagtaaggtgattccagaggaagatgcttgaggacaatttgggaaaactgacaacttgaaaactcagtctctctaggcaaggcctacttgcagataaccttgggagttctgtgctgggaggaaagctaaaggactaagttaggcctctgaatctgctctggaagcctgcatgcacttgggtcagaacaagcccatgtgtcaatgtgggtaaagattcctcagctgataagcaggaaaatgggcagggcattttggtctttgaggttcaaagctcagatgctcactgccttggtatacacgcacacacaccccaccccccagctgacggcacaagagtatacagatgcaatagtctaaagtacattgtccaaatatggatggccatgagccacatgtggctatgaagcacttaaatgtggctagtctgaactgagatgggccctataaaatatttcagtaacaggtttttatactgattataggttgacataataatattttggatataccgtattaaaggaaatatgtcattaaatttcacctgtttcctttattatgtggctacttgaaaattttaaaattacatatgtagctcacactataaaacacagattagaaatattgtatagcactgacctagaaacctccatttaggtaaaacatcttaacccctttggaagcaaaatatgttaaataacagcataaactcccaccaagaaaatcctcaccttcctcctttcaacacatttattatatacagctgtcactgcattgtcaatctgccaaatggctctatgttccaacagggctggagtagtcccctgctcacaccagccttcacaatacttcccatgtcttccctgttaacctctctccacccagcacccaggctcccaactctcctggctgcctccagccctcagctggcaccactgacatgctgtttccagtacccttttcttctttctgcatcctccctgggggacatatatccctcatctcgtgacttcagctgtcacataaattcaaatgtttcagaactctattttttacctcctacatctgtcagtttaaatgtcaggatattttactttcagtaaagccctaaaaagacaaatctatgtacttttaaagaataaaagaaatgactggctgcagctcaaacctacaactgcttgcgaaactctacaatgtctggcagatgctagaaagaaggggatcaagacagagcacacttggcgtggtatgctatctatagaaaatgttaaaataaaattaagtaatctaggtttcctctctttattttctacatctactctctgaagagggcaataaataaggaaatgtcccaaagagggacaaattaagtcccaaaataacacaaaattgggcaaatccagtcatgaagaaagaacagaggttcttaaattgggacacacagaggcaggtctgcaggtctaggaatctctgaacatatgtgcaaaattctgggtatgtgtgcatatgttatataacaaagcgaagggtccatatagctttcatcgcatttcaaagggtctagcactgaaataaggactactgctatgtgacttaaaaaatgaaactcaggctgggcgcagtggctcacgcctgtaatcccagcactttgggaggccgaggcaagcagatcacctgagacgaggagtttgagacccgcctggccaacggtgaaacccagtctctactaaaaatacaaaaattagccggaattggtggtgtgcctctagtcccagctactcaggaggctgaagaaagagaatcgcttgaacctgggaggtggaggttgtgacaaagcaagactccatctcaaaaaaaaaaaaaacccagaaactcaattcagttatgaaggtaaagatgacctgtttacatgataatattttaagataccagtgactgcaagcatgtagttattaagtccattacagtgcacatttattgactctgtgtatcttcacagtgtgatcttcaccacagcttgcaaagtgtaaccactcagcaccttctgcttccttctgttcagtttttccactgcaattcttccagcataattttctgatagccagtgtatgactttggctttgacttgtttctacacagtgggtccagtcatttatttctggaacttgatcagtctttttccaggtatataagcaaatctttccacactccaatcctactgcaaccacgtatcgttgagaagggtggagcactgggcagacgctgacagctgtcacagccccacccacgtccaggactgaggagcaggggccaatgttgtgctcaatacagtcatcagtggagtcgcactcaccccagacaaccacctttttgtctcgactcccagtgaagaaatacttgctgtcaggactccaatcacaagaccaaataattctactgtgcacagaagtaattttgttggtgaaggcaaaaagactaaaaactggctcgaactcaggtgagattgtatcctgctttttccacaatgaccaggttcgatctctggaaacagctagtaagaacttctcattaggtgagaaggccatctgcgtgactgtcaaactgtggaaaactaaattctgcacctgtttccaagatgtagtgttccaaagaatgatagctgcatgctctttcttagctgccttacaagctgaggcaagcagagtctttgaactgttacaagtaacacaaaatatttcataaccgtgcccatatagtttttgaacttcaggccacaaagtattctgcagaagatgatcctcagtgggaggctcagtaagtatggagggctgaaaggccacctgctgatactcaaaaccagtactagttaacagctcctcttcatcagaaggctgagaagctatatctccctgaaagacagctttatttgataatcccaatgcagggacagtggctccttctggaagatcactatcttgattacagagcacatgattcagtgattgtcctgtaatggcacaaaaattttccacaaaattccgaggtgcagaaaaaacccgaagaactttttcatctgctccagatacaaactgaaaccgattaatcattgccaaacatttcaggtcatacccatgtatctgaggccttgcaatttcatgccaagtcacctgtgattggtcttttctcttccatggagcaaaaagtctagttgtctgatcagtaccaacagtgataataaattctccttctggatcccagactaggtcttggacaccatcaaagtgtcctgaaatgacaatctctggagtccactctcttgggttaactgtattctgtttccaaaggtgcaacgctccgtggaaagcatgagcaatgatcatggagccatcttcattgaactggcaatcataaaatcccaaagtattcccacctacttcacctactcgaacctgttctagccaaactcctgactcttcatctggagcccagagaatcatggttttatccatggaagcagataataatctcactggctgctgtaggacaccatctttgtaaaacacaggttgccagtgaactgcatttacccagttttcatgaccggctagcactgtctccagagtaacagcaaatgctattttaacactttcattttctatggtaaaagtattttctttcagtcttatgttatcgtcatcctgagtttctaaagatgttgactttatatacagcttccatattcttatcaggcaatcttgtgaacagcttgctaggaaaagatctctaccaaaggctgcccattccactcctctaatccaatcctcatgtccacagagagaaagcactttctgaaactgatcattttgttgagcaaatatgtgaattctgcaatcatcattgccacatgctaatattggtattggcctgaatgcagatggaagaaatgaaattctgttatgatgccagaatgtgtgcagcttctccttccacagagccttgcacagaatggaagcgtaacatgaaaccatagagtcgcagctcctgctacagagggcgagagaggctggtggcttccaggccctgcctcgttccacctggccagtcttccaggtaacatcagtatttggcaaaaaagataagcagagagccaaagcaaatccatttccaaagtttaaagtctgaaggcacattacttctggaccctttttagaccagagtcgaacagcagaatctgcagctgcagaaacgatcagtgtacataatgcaggatctgatgtcctcctctggtaaacagcatgcaccgcataaacaggtccttcatggccttgaagatgcactgcttttaaaagctgattatcctctatttcccagtgaatcacttgattatcagatcctccagaaactaattcagtagaaggggagccatcctgtttacaaatccactgtatgcaattgactcgggcggtgtgaccattcaagttggtaacaacaacccttttcagggggtcatagagcaccacggagcaggacgtgccaaaggccagaagtcctctgggcccagagctccagttcaggactccccgcacccggtttgggcagcaaaacacgtgagaagtctccagcacgggtgccaccatgtcgccaactggtcagccgcacaaacaagagacgc

SEQ ID NO: 12494 - RNA, 5334 nt, Homo sapiens
  source 1..5334: mol_type = other RNA
gaaagtgcttccttttagaggctgaataatattccactgtatgaatataccacattttgttgatcattcacccactgatgggcacatattgcttccatctcttagctactgtgaataatggtgccgtgagtatgggcatacaaaaactaccactaatattttacagtgcttgcttcatatctgtccatgtgtccgtcactccacccatcatattttttatgtatttcataagttacagaccacagtaacttccctcaaacatgtcagtatacatatcaatgaccagcgttcattgtttttttccaagtcattttgaactgccgtagcaatgagtaatatagcctcaaacgcacacatacacacacaacacgtgcgtcactacagaaaacttttcctggcagacaggaaagggcccattgttggtgatgtcattttaattaagataaaaccaccaccaccatttagtaatagcctggggtaacaagggctgcgtcacggactgccacttttgccatcctgctcagagcagggccatgcctaacccgtatctggggattgcttcagatattatgaatcgcttcaatattatgaattactacaattcataataattgcttcagatattatgaattacaatatggttcaaaggtgctttagcagatgaagacacaaatgtgtaaacacatatgaattacaatgcagactgcccagatgtgtagcaagtcctctgaatgtttactaaacagtaaggtgattccagaggaagatgcttgaggacaatttgggaaaactgacaacttgaaaactcagtctctctaggcaaggcctacttgcagataaccttgggagttctgtgctgggaggaaagctaaaggactaagttaggcctctgaatctgctctggaagcctgcatgcacttgggtcagaacaagcccatgtgtcaatgtgggtaaagattcctcagctgataagcaggaaaatgggcagggcattttggtctttgaggttcaaagctcagatgctcactgccttggtatacacgcacacacaccccaccccccagctgacggcacaagagtatacagatgcaatagtctaaagtacattgtccaaatatggatggccatgagccacatgtggctatgaagcacttaaatgtggctagtctgaactgagatgggccctataaaatatttcagtaacaggtttttatactgattataggttgacataataatattttggatataccgtattaaaggaaatatgtcattaaatttcacctgtttcctttattatgtggctacttgaaaattttaaaattacatatgtagctcacactataaaacacagattagaaatattgtatagcactgacctagaaacctccatttaggtaaaacatcttaacccctttggaagcaaaatatgttaaataacagcataaactcccaccaagaaaatcctcaccttcctcctttcaacacatttattatatacagctgtcactgcattgtcaatctgccaaatggctctatgttccaacagggctggagtagtcccctgctcacaccagccttcacaatacttcccatgtcttccctgttaacctctctccacccagcacccaggctcccaactctcctggctgcctccagccctcagctggcaccactgacatgctgtttccagtacccttttcttctttctgcatcctccctgggggacatatatccctcatctcgtgacttcagctgtcacataaattcaaatgtttcagaactctattttttacctcctacatctgtcagtttaaatgtcaggatattttactttcagtaaagccctaaaaagacaaatctatgtacttttaaagaataaaagaaatgactggctgcagctcaaacctacaactgcttgcgaaactctacaatgtctggcagatgctagaaagaaggggatcaagacagagcacacttggcgtggtatgctatctatagaaaatgttaaaataaaattaagtaatctaggtttcctctctttattttctacatctactctctgaagagggcaataaataaggaaatgtcccaaagagggacaaattaagtcccaaaataacacaaaattgggcaaatccagtcatgaagaaagaacagaggttcttaaattgggacacacagaggcaggtctgcaggtctaggaatctctgaacatatgtgcaaaattctgggtatgtgtgcatatgttatataacaaagcgaagggtccatatagctttcatcgcatttcaaagggtctagcactgaaataaggactactgctatgtgacttaaaaaatgaaactcaggctgggcgcagtggctcacgcctgtaatcccagcactttgggaggccgaggcaagcagatcacctgagacgaggagtttgagacccgcctggccaacggtgaaacccagtctctactaaaaatacaaaaattagccggaattggtggtgtgcctctagtcccagctactcaggaggctgaagaaagagaatcgcttgaacctgggaggtggaggttgtgacaaagcaagactccatctcaaaaaaaaaaaaaacccagaaactcaattcagttatgaaggtaaagatgacctgtttacatgataatattttaagataccagtgactgcaagcatgtagttattaagtccattacagtgcacatttattgactctgtgtatcttcacagtgtgatcttcaccacagcttgcaaagtgtaaccactcagcaccttctgcttccttctgttcagtttttccactgcaattcttccagcataattttctgatagccagtgtatgactttggctttgacttgtttctacacagtgggtccagtcatttatttctggaacttgatcagtctttttccaggtatataagcaaatctttccacactccaatcctactgcaaccacgtatcgttgagaagggtggagcactgggcagacgctgacagctgtcacagccccacccacgtccaggactgaggagcaggggccaatgttgtgctcaatacagtcatcagtggagtcgcactcaccccagacaaccacctttttgtctcgactcccagtgaagaaatacttgctgtcaggactccaatcacaagaccaaataattctactgtgcacagaagtaattttgttggtgaaggcaaaaagactaaaaactggctcgaactcaggtgagattgtatcctgctttttccacaatgaccaggttcgatctctggaaacagctagtaagaacttctcattaggtgagaaggccatctgcgtgactgtcaaactgtggaaaactaaattctgcacctgtttccaagatgtagtgttccaaagaatgatagctgcatgctctttcttagctgccttacaagctgaggcaagcagagtctttgaactgttacaagtaacacaaaatatttcataaccgtgcccatatagtttttgaacttcaggccacaaagtattctgcagaagatgatcctcagtgggaggctcagtaagtatggagggctgaaaggccacctgctgatactcaaaaccagtactagttaacagctcctcttcatcagaaggctgagaagctatatctccctgaaagacagctttatttgataatcccaatgcagggacagtggctccttctggaagatcactatcttgattacagagcacatgattcagtgattgtcctgtaatggcacaaaaattttccacaaaattccgaggtgcagaaaaaacccgaagaactttttcatctgctccagatacaaactgaaaccgattaatcattgccaaacatttcaggtcatacccatgtatctgaggccttgcaatttcatgccaagtcacctgtgattggtcttttctcttccatggagcaaaaagtctagttgtctgatcagtaccaacagtgataataaattctccttctggatcccagactaggtcttggacaccatcaaagtgtcctgaaatgacaatctctggagtccactctcttgggttaactgtattctgtttccaaaggtgcaacgctccgtggaaagcatgagcaatgatcatggagccatcttcattgaactggcaatcataaaatcccaaagtattcccacctacttcacctactcgaacctgttctagccaaactcctgactcttcatctggagcccagagaatcatggttttatccatggaagcagataataatctcactggctgctgtaggacaccatctttgtaaaacacaggttgccagtgaactgcatttacccagttttcatgaccggctagcactgtctccagagtaacagcaaatgctattttaacactttcattttctatggtaaaagtattttctttcagtcttatgttatcgtcatcctgagtttctaaagatgttgactttatatacagcttccatattcttatcaggcaatcttgtgaacagcttgctaggaaaagatctctaccaaaggctgcccattccactcctctaatccaatcctcatgtccacagagagaaagcactttctgaaactgatcattttgttgagcaaatatgtgaattctgcaatcatcattgccacatgctaatattggtattggcctgaatgcagatggaagaaatgaaattctgttatgatgccagaatgtgtgcagcttctccttccacagagccttgcacagaatggaagcgtaacatgaaaccatagagtcgcagctcctgctacagagggcgagagaggctggtggcttccaggccctgcctcgttccacctggccagtcttccaggtaacttctggaccctttttagaccagagtcgaacagcagaatctgcagctgcagaaacgatcagtgtacataatgcaggatctgatgtcctcctctggtaaacagcatgcaccgcataaacaggtccttcatggccttgaagatgcactgcttttaaaagctgattatcctctatttcccagtgaatcacttgattatcagatcctccagaaactaattcagtagaaggggagccatcctgtttacaaatccactgtatgcaattgactcgggcggtgtgaccattcaagttggtaacaacaacccttttcagggggtcatagagcaccacggagcaggacgtgccaaaggccagaagtcctctgggcccagagctccagttcaggactccccgcacccggtttgggcagcaaaacacgtgagaagtctccagcacgggtgccaccatgtcgccaactggtcagccgcacaaacaagagacgc

SEQ ID NO: 12495 - RNA, 5007 nt, Homo sapiens
  source 1..5007: mol_type = other RNA
gaaagtgcttccttttagaggctgaataatattccactgtatgaatataccacattttgttgatcattcacccactgatgggcacatattgcttccatctcttagctactgtgaataatggtgccgtgagtatgggcatacaaaaactaccactaatattttacagtgcttgcttcatatctgtccatgtgtccgtcactccacccatcatattttttatgtatttcataagttacagaccacagtaacttccctcaaacatgtcagtatacatatcaatgaccagcgttcattgtttttttccaagtcattttgaactgccgtagcaatgagtaatatagcctcaaacgcacacatacacacacaacacgtgcgtcactacagaaaacttttcctggcagacaggaaagggcccattgttggtgatgtcattttaattaagataaaaccaccaccaccatttagtaatagcctggggtaacaagggctgcgtcacggactgccacttttgccatcctgctcagagcagggccatgcctaacccgtatctggggattgcttcagatattatgaatcgcttcaatattatgaattactacaattcataataattgcttcagatattatgaattacaatatggttcaaaggtgctttagcagatgaagacacaaatgtgtaaacacatatgaattacaatgcagactgcccagatgtgtagcaagtcctctgaatgtttactaaacagtaaggtgattccagaggaagatgcttgaggacaatttgggaaaactgacaacttgaaaactcagtctctctaggcaaggcctacttgcagataaccttgggagttctgtgctgggaggaaagctaaaggactaagttaggcctctgaatctgctctggaagcctgcatgcacttgggtcagaacaagcccatgtgtcaatgtgggtaaagattcctcagctgataagcaggaaaatgggcagggcattttggtctttgaggttcaaagctcagatgctcactgccttggtatacacgcacacacaccccaccccccagctgacggcacaagagtatacagatgcaatagtctaaagtacattgtccaaatatggatggccatgagccacatgtggctatgaagcacttaaatgtggctagtctgaactgagatgggccctataaaatatttcagtaacaggtttttatactgattataggttgacataataatattttggatataccgtattaaaggaaatatgtcattaaatttcacctgtttcctttattatgtggctacttgaaaattttaaaattacatatgtagctcacactataaaacacagattagaaatattgtatagcactgacctagaaacctccatttaggtaaaacatcttaacccctttggaagcaaaatatgttaaataacagcataaactcccaccaagaaaatcctcaccttcctcctttcaacacatttattatatacagctgtcactgcattgtcaatctgccaaatggctctatgttccaacagggctggagtagtcccctgctcacaccagccttcacaatacttcccatgtcttccctgttaacctctctccacccagcacccaggctcccaactctcctggctgcctccagccctcagctggcaccactgacatgctgtttccagtacccttttcttctttctgcatcctccctgggggacatatatccctcatctcgtgacttcagctgtcacataaattcaaatgtttcagaactctattttttacctcctacatctgtcagtttaaatgtcaggatattttactttcagtaaagccctaaaaagacaaatctatgtacttttaaagaataaaagaaatgactggctgcagctcaaacctacaactgcttgcgaaactctacaatgtctggcagatgctagaaagaaggggatcaagacagagcacacttggcgtggtatgctatctatagaaaatgttaaaataaaattaagtaatctaggtttcctctctttattttctacatctactctctgaagagggcaataaataaggaaatgtcccaaagagggacaaattaagtcccaaaataacacaaaattgggcaaatccagtcatgaagaaagaacagaggttcttaaattgggacacacagaggcaggtctgcaggtctaggaatctctgaacatatgtgcaaaattctgggtatgtgtgcatatgttatataacaaagcgaagggtccatatagctttcatcgcatttcaaagggtctagcactgaaataaggactactgctatgtgacttaaaaaatgaaactcaggctgggcgcagtggctcacgcctgtaatcccagcactttgggaggccgaggcaagcagatcacctgagacgaggagtttgagacccgcctggccaacggtgaaacccagtctctactaaaaatacaaaaattagccggaattggtggtgtgcctctagtcccagctactcaggaggctgaagaaagagaatcgcttgaacctgggaggtggaggttgtgacaaagcaagactccatctcaaaaaaaaaaaaaacccagaaactcaattcagttatgaaggtaaagatgacctgtttacatgataatattttaagataccagtgactgcaagcatgtagttattaagtccattacagtgcacatttattgactctgtgtatcttcacagtgtgatcttcaccacagcttgcaaagtgtaaccactcagcaccttctgcttccttctgttcagtttttccactgcaattcttccagcataattttctgatagccagtgtatgactttggctttgacttgtttctacacagtgggtccagtcatttatttctggaacttgatcagtctttttccaggtatataagcaaatctttccacactccaatcctactgcaaccacgtatcgttgagaagggtggagcactgggcagacgctgacagctgtcacagccccacccacgtccaggactgaggagcaggggccaatgttgtgctcaatacagtcatcagtggagtcgcactcaccccagacaaccacctttttgtctcgactcccagtgaagaaatacttgctgtcaggactccaatcacaagaccaaataattctactgtgcacagaagtaattttgttggtgaaggcaaaaagactaaaaactggctcgaactcaggtgagattgtatcctgctttttccacaatgaccaggttcgatctctggaaacagctagtaagaacttctcattaggtgagaaggccatctgcgtgactgtcaaactgtggaaaactaaattctgcacctgtttccaagatgtagtgttccaaagaatgatagctgcatgctctttcttagctgccttacaagctgaggcaagcagagtctttgaactgttacaagtaacacaaaatatttcataaccgtgcccatatagtttttgaacttcaggccacaaagtattctgcagaagatgatcctcagtgggaggctcagtaagtatggagggctgaaaggccacctgctgatactcaaaaccagtactagttaacagctcctcttcatcagaaggctgagaagctatatctccctgaaagacagctttatttgataatcccaatgcagggacagtggctccttctggaagatcactatcttgattacagagcacatgattcagtgattgtcctgtaatggcacaaaaattttccacaaaattccgaggtgcagaaaaaacccgaagaactttttcatctgctccagatacaaactgaaaccgattaatcattgccaaacatttcaggtcatacccatgtatctgaggccttgcaatttcatgccaagtcacctgtgattggtcttttctcttccatggagcaaaaagtctagttgtctgatcagtaccaacagtgataataaattctccttctggatcccagactaggtcttggacaccatcaaagtgtcctgaaatgacaatctctggagtccactctcttgggttaactgtattctgtttccaaaggtgcaacgctccgtggaaagcatgagcaatgatcatggagccatcttcattgaactggcaatcataaaatcccaaagtattcccacctacttcacctactcgaacctgttctagccaaactcctgactcttcatctggagcccagagaatcatggttttatccatggaagcagataataatctcactggctgctgtaggacaccatctttgtaaaacacaggttgccagtgaactgcatttacccagttttcatgaccggctagcactgtctccagagtaacagcaaatgctattttaacactttcattttctatggtaaaagtattttctttcagtcttatgttatcgtcatcctgagtttctaaagatgttgactttatatacagcttccatattcttatcaggcaatcttgtgaacagcttgctaggaaaagatctctaccttctggaccctttttagaccagagtcgaacagcagaatctgcagctgcagaaacgatcagtgtacataatgcaggatctgatgtcctcctctggtaaacagcatgcaccgcataaacaggtccttcatggccttgaagatgcactgcttttaaaagctgattatcctctatttcccagtgaatcacttgattatcagatcctccagaaactaattcagtagaaggggagccatcctgtttacaaatccactgtatgcaattgactcgggcggtgtgaccattcaagttggtaacaacaacccttttcagggggtcatagagcaccacggagcaggacgtgccaaaggccagaagtcctctgggcccagagctccagttcaggactccccgcacccggtttgggcagcaaaacacgtgagaagtctccagcacgggtgccaccatgtcgccaactggtcagccgcacaaacaagagacgc

SEQ ID NO: 12496 - RNA, 5067 nt, Homo sapiens
  source 1..5067: mol_type = other RNA
gaaagtgcttccttttagaggctgaataatattccactgtatgaatataccacattttgttgatcattcacccactgatgggcacatattgcttccatctcttagctactgtgaataatggtgccgtgagtatgggcatacaaaaactaccactaatattttacagtgcttgcttcatatctgtccatgtgtccgtcactccacccatcatattttttatgtatttcataagttacagaccacagtaacttccctcaaacatgtcagtatacatatcaatgaccagcgttcattgtttttttccaagtcattttgaactgccgtagcaatgagtaatatagcctcaaacgcacacatacacacacaacacgtgcgtcactacagaaaacttttcctggcagacaggaaagggcccattgttggtgatgtcattttaattaagataaaaccaccaccaccatttagtaatagcctggggtaacaagggctgcgtcacggactgccacttttgccatcctgctcagagcagggccatgcctaacccgtatctggggattgcttcagatattatgaatcgcttcaatattatgaattactacaattcataataattgcttcagatattatgaattacaatatggttcaaaggtgctttagcagatgaagacacaaatgtgtaaacacatatgaattacaatgcagactgcccagatgtgtagcaagtcctctgaatgtttactaaacagtaaggtgattccagaggaagatgcttgaggacaatttgggaaaactgacaacttgaaaactcagtctctctaggcaaggcctacttgcagataaccttgggagttctgtgctgggaggaaagctaaaggactaagttaggcctctgaatctgctctggaagcctgcatgcacttgggtcagaacaagcccatgtgtcaatgtgggtaaagattcctcagctgataagcaggaaaatgggcagggcattttggtctttgaggttcaaagctcagatgctcactgccttggtatacacgcacacacaccccaccccccagctgacggcacaagagtatacagatgcaatagtctaaagtacattgtccaaatatggatggccatgagccacatgtggctatgaagcacttaaatgtggctagtctgaactgagatgggccctataaaatatttcagtaacaggtttttatactgattataggttgacataataatattttggatataccgtattaaaggaaatatgtcattaaatttcacctgtttcctttattatgtggctacttgaaaattttaaaattacatatgtagctcacactataaaacacagattagaaatattgtatagcactgacctagaaacctccatttaggtaaaacatcttaacccctttggaagcaaaatatgttaaataacagcataaactcccaccaagaaaatcctcaccttcctcctttcaacacatttattatatacagctgtcactgcattgtcaatctgccaaatggctctatgttccaacagggctggagtagtcccctgctcacaccagccttcacaatacttcccatgtcttccctgttaacctctctccacccagcacccaggctcccaactctcctggctgcctccagccctcagctggcaccactgacatgctgtttccagtacccttttcttctttctgcatcctccctgggggacatatatccctcatctcgtgacttcagctgtcacataaattcaaatgtttcagaactctattttttacctcctacatctgtcagtttaaatgtcaggatattttactttcagtaaagccctaaaaagacaaatctatgtacttttaaagaataaaagaaatgactggctgcagctcaaacctacaactgcttgcgaaactctacaatgtctggcagatgctagaaagaaggggatcaagacagagcacacttggcgtggtatgctatctatagaaaatgttaaaataaaattaagtaatctaggtttcctctctttattttctacatctactctctgaagagggcaataaataaggaaatgtcccaaagagggacaaattaagtcccaaaataacacaaaattgggcaaatccagtcatgaagaaagaacagaggttcttaaattgggacacacagaggcaggtctgcaggtctaggaatctctgaacatatgtgcaaaattctgggtatgtgtgcatatgttatataacaaagcgaagggtccatatagctttcatcgcatttcaaagggtctagcactgaaataaggactactgctatgtgacttaaaaaatgaaactcaggctgggcgcagtggctcacgcctgtaatcccagcactttgggaggccgaggcaagcagatcacctgagacgaggagtttgagacccgcctggccaacggtgaaacccagtctctactaaaaatacaaaaattagccggaattggtggtgtgcctctagtcccagctactcaggaggctgaagaaagagaatcgcttgaacctgggaggtggaggttgtgacaaagcaagactccatctcaaaaaaaaaaaaaacccagaaactcaattcagttatgaaggtaaagatgacctgtttacatgataatattttaagataccagtgactgcaagcatgtagttattaagtccattacagtgcacatttattgactctgtgtatcttcacagtgtgatcttcaccacagcttgcaaagtgtaaccactcagcaccttctgcttccttctgttcagtttttccactgcaattcttccagcataattttctgatagccagtgtatgactttggctttgacttgtttctacacagtgggtccagtcatttatttctggaacttgatcagtctttttccaggtatataagcaaatctttccacactccaatcctactgcaaccacgtatcgttgagaagggtggagcactgggcagacgctgacagctgtcacagccccacccacgtccaggactgaggagcaggggccaatgttgtgctcaatacagtcatcagtggagtcgcactcaccccagacaaccacctttttgtctcgactcccagtgaagaaatacttgctgtcaggactccaatcacaagaccaaataattctactgtgcacagaagtaattttgttggtgaaggcaaaaagactaaaaactggctcgaactcaggtgagattgtatcctgctttttccacaatgaccaggttcgatctctggaaacagctagtaagaacttctcattaggtgagaaggccatctgcgtgactgtcaaactgtggaaaactaaattctgcacctgtttccaagatgtagtgttccaaagaatgatagctgcatgctctttcttagctgccttacaagctgaggcaagcagagtctttgaactgttacaagtaacacaaaatatttcataaccgtgcccatatagtttttgaacttcaggccacaaagtattctgcagaagatgatcctcagtgggaggctcagtaagtatggagggctgaaaggccacctgctgatactcaaaaccagtactagttaacagctcctcttcatcagaaggctgagaagctatatctccctgaaagacagctttatttgataatcccaatgcagggacagtggctccttctggaagatcactatcttgattacagagcacatgattcagtgattgtcctgtaatggcacaaaaattttccacaaaattccgaggtgcagaaaaaacccgaagaactttttcatctgctccagatacaaactgaaaccgattaatcattgccaaacatttcaggtcatacccatgtatctgaggccttgcaatttcatgccaagtcactgggttaactgtattctgtttccaaaggtgcaacgctccgtggaaagcatgagcaatgatcatggagccatcttcattgaactggcaatcataaaatcccaaagtattcccacctacttcacctactcgaacctgttctagccaaactcctgactcttcatctggagcccagagaatcatggttttatccatggaagcagataataatctcactggctgctgtaggacaccatctttgtaaaacacaggttgccagtgaactgcatttacccagttttcatgaccggctagcactgtctccagagtaacagcaaatgctattttaacactttcattttctatggtaaaagtattttctttcagtcttatgttatcgtcatcctgagtttctaaagatgttgactttatatacagcttccatattcttatcaggcaatcttgtgaacagcttgctaggaaaagatctctaccaaaggctgcccattccactcctctaatccaatcctcatgtccacagagagaaagcactttctgaaactgatcattttgttgagcaaatatgtgaattctgcaatcatcattgccacatgctaatattggtacatcagtatttggcaaaaaagataagcagagagccaaagcaaatccatttccaaagtttaaagtctgaaggcacattacttctggaccctttttagaccagagtcgaacagcagaatctgcagctgcagaaacgatcagtgtacataatgcaggatctgatgtcctcctctggtaaacagcatgcaccgcataaacaggtccttcatggccttgaagatgcactgcttttaaaagctgattatcctctatttcccagtgaatcacttgattatcagatcctccagaaactaattcagtagaaggggagccatcctgtttacaaatccactgtatgcaattgactcgggcggtgtgaccattcaagttggtaacaacaacccttttcagggggtcatagagcaccacggagcaggacgtgccaaaggccagaagtcctctgggcccagagctccagttcaggactccccgcacccggtttgggcagcaaaacacgtgagaagtctccagcacgggtgccaccatgtcgccaactggtcagccgcacaaacaagagacgc

SEQ ID NO: 12497 - RNA, 5083 nt, Homo sapiens
  source 1..5083: mol_type = other RNA
gaaagtgcttccttttagaggctgaataatattccactgtatgaatataccacattttgttgatcattcacccactgatgggcacatattgcttccatctcttagctactgtgaataatggtgccgtgagtatgggcatacaaaaactaccactaatattttacagtgcttgcttcatatctgtccatgtgtccgtcactccacccatcatattttttatgtatttcataagttacagaccacagtaacttccctcaaacatgtcagtatacatatcaatgaccagcgttcattgtttttttccaagtcattttgaactgccgtagcaatgagtaatatagcctcaaacgcacacatacacacacaacacgtgcgtcactacagaaaacttttcctggcagacaggaaagggcccattgttggtgatgtcattttaattaagataaaaccaccaccaccatttagtaatagcctggggtaacaagggctgcgtcacggactgccacttttgccatcctgctcagagcagggccatgcctaacccgtatctggggattgcttcagatattatgaatcgcttcaatattatgaattactacaattcataataattgcttcagatattatgaattacaatatggttcaaaggtgctttagcagatgaagacacaaatgtgtaaacacatatgaattacaatgcagactgcccagatgtgtagcaagtcctctgaatgtttactaaacagtaaggtgattccagaggaagatgcttgaggacaatttgggaaaactgacaacttgaaaactcagtctctctaggcaaggcctacttgcagataaccttgggagttctgtgctgggaggaaagctaaaggactaagttaggcctctgaatctgctctggaagcctgcatgcacttgggtcagaacaagcccatgtgtcaatgtgggtaaagattcctcagctgataagcaggaaaatgggcagggcattttggtctttgaggttcaaagctcagatgctcactgccttggtatacacgcacacacaccccaccccccagctgacggcacaagagtatacagatgcaatagtctaaagtacattgtccaaatatggatggccatgagccacatgtggctatgaagcacttaaatgtggctagtctgaactgagatgggccctataaaatatttcagtaacaggtttttatactgattataggttgacataataatattttggatataccgtattaaaggaaatatgtcattaaatttcacctgtttcctttattatgtggctacttgaaaattttaaaattacatatgtagctcacactataaaacacagattagaaatattgtatagcactgacctagaaacctccatttaggtaaaacatcttaacccctttggaagcaaaatatgttaaataacagcataaactcccaccaagaaaatcctcaccttcctcctttcaacacatttattatatacagctgtcactgcattgtcaatctgccaaatggctctatgttccaacagggctggagtagtcccctgctcacaccagccttcacaatacttcccatgtcttccctgttaacctctctccacccagcacccaggctcccaactctcctggctgcctccagccctcagctggcaccactgacatgctgtttccagtacccttttcttctttctgcatcctccctgggggacatatatccctcatctcgtgacttcagctgtcacataaattcaaatgtttcagaactctattttttacctcctacatctgtcagtttaaatgtcaggatattttactttcagtaaagccctaaaaagacaaatctatgtacttttaaagaataaaagaaatgactggctgcagctcaaacctacaactgcttgcgaaactctacaatgtctggcagatgctagaaagaaggggatcaagacagagcacacttggcgtggtatgctatctatagaaaatgttaaaataaaattaagtaatctaggtttcctctctttattttctacatctactctctgaagagggcaataaataaggaaatgtcccaaagagggacaaattaagtcccaaaataacacaaaattgggcaaatccagtcatgaagaaagaacagaggttcttaaattgggacacacagaggcaggtctgcaggtctaggaatctctgaacatatgtgcaaaattctgggtatgtgtgcatatgttatataacaaagcgaagggtccatatagctttcatcgcatttcaaagggtctagcactgaaataaggactactgctatgtgacttaaaaaatgaaactcaggctgggcgcagtggctcacgcctgtaatcccagcactttgggaggccgaggcaagcagatcacctgagacgaggagtttgagacccgcctggccaacggtgaaacccagtctctactaaaaatacaaaaattagccggaattggtggtgtgcctctagtcccagctactcaggaggctgaagaaagagaatcgcttgaacctgggaggtggaggttgtgacaaagcaagactccatctcaaaaaaaaaaaaaacccagaaactcaattcagttatgaaggtaaagatgacctgtttacatgataatattttaagataccagtgactgcaagcatgtagttattaagtccattacagtgcacatttattgactctgtgtatcttcacagtgtgatcttcaccacagcttgcaaagtgtaaccactcagcaccttctgcttccttctgttcagtttttccactgcaattcttccagcataattttctgatagccagtgtatgactttggctttgacttgtttctacacagtgggtccagtcatttatttctggaacttgatcagtctttttccaggtatataagcaaatctttccacactccaatcctactgcaaccacgtatctttttgtctcgactcccagtgaagaaatacttgctgtcaggactccaatcacaagaccaaataattctactgtgcacagaagtaattttgttggtgaaggcaaaaagactaaaaactggctcgaactcaggtgagattgtatcctgctttttccacaatgaccaggttcgatctctggaaacagctagtaagaacttctcattaggtgagaaggccatctgcgtgactgtcaaactgtggaaaactaaattctgcacctgtttccaagatgtagtgttccaaagaatgatagctgcatgctctttcttagctgccttacaagctgaggcaagcagagtctttgaactgttacaagtaacacaaaatatttcataaccgtgcccatatagtttttgaacttcaggccacaaagtattctgcagaagatgatcctcagtgggaggctcagtaagtatggagggctgaaaggccacctgctgatactcaaaaccagtactagttaacagctcctcttcatcagaaggctgagaagctatatctccctgaaagacagctttatttgataatcccaatgcagggacagtggctccttctggaagatcactatcttgattacagagcacatgattcagtgattgtcctgtaatggcacaaaaattttccacaaaattccgaggtgcagaaaaaacccgaagaactttttcatctgctccagatacaaactgaaaccgattaatcattgccaaacatttcaggtcatacccatgtatctgaggccttgcaatttcatgccaagtcacctgtgattggtcttttctcttccatggagcaaaaagtctagttgtctgatcagtaccaacagtgataataaattctccttctggatcccagactaggtcttggacaccatcaaagtgtcctgaaatgacaatctctggagtccactctcttgggttaactgtattctgtttccaaaggtgcaacgctccgtggaaagcatgagcaatgatcatggagccatcttcattgaactggcaatcataaaatcccaaagtattcccacctacttcacctactcgaacctgttctagccaaactcctgactcttcatctggagcccagagaatcatggttttatccatggaagcagataataatctcactggctgctgtaggacaccatctttgtaaaacacaggttgccagtgaactgcatttacccagttttcatgaccggctagcactgtctccagagtaacagcaaatgctattttaacactttcattttctatggtaaaagtattttctttcagtcttatgttatcgtcatcctgagtttctaaagatgttgactttatatacagcttccatattcttatcaggcaatcttgtgaacagcttgctaggaaaagatctctaccaaaggctgcccattccactcctctaatccaatcctcatgtccacagagagaaagcactttctgaaactgatcattttgttgagcaaatatgtgaattctgcaatcatcattgccacatgctaatattggtacatcagtatttggcaaaaaagataagcagagagccaaagcaaatccatttccaaagtttaaagtctgaaggcacattacttctggaccctttttagaccagagtcgaacagcagaatctgcagctgcagaaacgatcagtgtacataatgcaggatctgatgtcctcctctggtaaacagcatgcaccgcataaacaggtccttcatggccttgaagatgcactgcttttaaaagctgattatcctctatttcccagtgaatcacttgattatcagatcctccagaaactaattcagtagaaggggagccatcctgtttacaaatccactgtatgcaattgactcgggcggtgtgaccattcaagttggtaacaacaacccttttcagggggtcatagagcaccacggagcaggacgtgccaaaggccagaagtcctctgggcccagagctccagttcaggactccccgcacccggtttgggcagcaaaacacgtgagaagtctccagcacgggtgccaccatgtcgccaactggtcagccgcacaaacaagagacgc

SEQ ID NO: 12498 - RNA, 5278 nt, Homo sapiens
  source 1..5278: mol_type = other RNA
gaaagtgcttccttttagaggctgaataatattccactgtatgaatataccacattttgttgatcattcacccactgatgggcacatattgcttccatctcttagctactgtgaataatggtgccgtgagtatgggcatacaaaaactaccactaatattttacagtgcttgcttcatatctgtccatgtgtccgtcactccacccatcatattttttatgtatttcataagttacagaccacagtaacttccctcaaacatgtcagtatacatatcaatgaccagcgttcattgtttttttccaagtcattttgaactgccgtagcaatgagtaatatagcctcaaacgcacacatacacacacaacacgtgcgtcactacagaaaacttttcctggcagacaggaaagggcccattgttggtgatgtcattttaattaagataaaaccaccaccaccatttagtaatagcctggggtaacaagggctgcgtcacggactgccacttttgccatcctgctcagagcagggccatgcctaacccgtatctggggattgcttcagatattatgaatcgcttcaatattatgaattactacaattcataataattgcttcagatattatgaattacaatatggttcaaaggtgctttagcagatgaagacacaaatgtgtaaacacatatgaattacaatgcagactgcccagatgtgtagcaagtcctctgaatgtttactaaacagtaaggtgattccagaggaagatgcttgaggacaatttgggaaaactgacaacttgaaaactcagtctctctaggcaaggcctacttgcagataaccttgggagttctgtgctgggaggaaagctaaaggactaagttaggcctctgaatctgctctggaagcctgcatgcacttgggtcagaacaagcccatgtgtcaatgtgggtaaagattcctcagctgataagcaggaaaatgggcagggcattttggtctttgaggttcaaagctcagatgctcactgccttggtatacacgcacacacaccccaccccccagctgacggcacaagagtatacagatgcaatagtctaaagtacattgtccaaatatggatggccatgagccacatgtggctatgaagcacttaaatgtggctagtctgaactgagatgggccctataaaatatttcagtaacaggtttttatactgattataggttgacataataatattttggatataccgtattaaaggaaatatgtcattaaatttcacctgtttcctttattatgtggctacttgaaaattttaaaattacatatgtagctcacactataaaacacagattagaaatattgtatagcactgacctagaaacctccatttaggtaaaacatcttaacccctttggaagcaaaatatgttaaataacagcataaactcccaccaagaaaatcctcaccttcctcctttcaacacatttattatatacagctgtcactgcattgtcaatctgccaaatggctctatgttccaacagggctggagtagtcccctgctcacaccagccttcacaatacttcccatgtcttccctgttaacctctctccacccagcacccaggctcccaactctcctggctgcctccagccctcagctggcaccactgacatgctgtttccagtacccttttcttctttctgcatcctccctgggggacatatatccctcatctcgtgacttcagctgtcacataaattcaaatgtttcagaactctattttttacctcctacatctgtcagtttaaatgtcaggatattttactttcagtaaagccctaaaaagacaaatctatgtacttttaaagaataaaagaaatgactggctgcagctcaaacctacaactgcttgcgaaactctacaatgtctggcagatgctagaaagaaggggatcaagacagagcacacttggcgtggtatgctatctatagaaaatgttaaaataaaattaagtaatctaggtttcctctctttattttctacatctactctctgaagagggcaataaataaggaaatgtcccaaagagggacaaattaagtcccaaaataacacaaaattgggcaaatccagtcatgaagaaagaacagaggttcttaaattgggacacacagaggcaggtctgcaggtctaggaatctctgaacatatgtgcaaaattctgggtatgtgtgcatatgttatataacaaagcgaagggtccatatagctttcatcgcatttcaaagggtctagcactgaaataaggactactgctatgtgacttaaaaaatgaaactcaggctgggcgcagtggctcacgcctgtaatcccagcactttgggaggccgaggcaagcagatcacctgagacgaggagtttgagacccgcctggccaacggtgaaacccagtctctactaaaaatacaaaaattagccggaattggtggtgtgcctctagtcccagctactcaggaggctgaagaaagagaatcgcttgaacctgggaggtggaggttgtgacaaagcaagactccatctcaaaaaaaaaaaaaacccagaaactcaattcagttatgaaggtaaagatgacctgtttacatgataatattttaagataccagtgactgcaagcatgtagttattaagtccattacagtgcacatttattgactctgtgtatcttcacagtgtgatcttcaccacagcttgcaaagtgtaaccactcagcaccttctgcttccttctgttcagtttttccactgcaattcttccagcataattttctgatagccagtgtatgactttggctttgacttgtttctacacagtgggtccagtcatttatttctggaacttgatcagtctttttccaggtatataagcaaatctttccacactccaatcctactgcaaccacgtatctttttgtctcgactcccagtgaagaaatacttgctgtcaggactccaatcacaagaccaaataattctactgtgcacagaagtaattttgttggtgaaggcaaaaagactaaaaactggctcgaactcaggtgagattgtatcctgctttttccacaatgaccaggttcgatctctggaaacagctagtaagaacttctcattaggtgagaaggccatctgcgtgactgtcaaactgtggaaaactaaattctgcacctgtttccaagatgtagtgttccaaagaatgatagctgcatgctctttcttagctgccttacaagctgaggcaagcagagtctttgaactgttacaagtaacacaaaatatttcataaccgtgcccatatagtttttgaacttcaggccacaaagtattctgcagaagatgatcctcagtgggaggctcagtaagtatggagggctgaaaggccacctgctgatactcaaaaccagtactagttaacagctcctcttcatcagaaggctgagaagctatatctccctgaaagacagctttatttgataatcccaatgcagggacagtggctccttctggaagatcactatcttgattacagagcacatgattcagtgattgtcctgtaatggcacaaaaattttccacaaaattccgaggtgcagaaaaaacccgaagaactttttcatctgctccagatacaaactgaaaccgattaatcattgccaaacatttcaggtcatacccatgtatctgaggccttgcaatttcatgccaagtcacctgtgattggtcttttctcttccatggagcaaaaagtctagttgtctgatcagtaccaacagtgataataaattctccttctggatcccagactaggtcttggacaccatcaaagtgtcctgaaatgacaatctctggagtccactctcttgggttaactgtattctgtttccaaaggtgcaacgctccgtggaaagcatgagcaatgatcatggagccatcttcattgaactggcaatcataaaatcccaaagtattcccacctacttcacctactcgaacctgttctagccaaactcctgactcttcatctggagcccagagaatcatggttttatccatggaagcagataataatctcactggctgctgtaggacaccatctttgtaaaacacaggttgccagtgaactgcatttacccagttttcatgaccggctagcactgtctccagagtaacagcaaatgctattttaacactttcattttctatggtaaaagtattttctttcagtcttatgttatcgtcatcctgagtttctaaagatgttgactttatatacagcttccatattcttatcaggcaatcttgtgaacagcttgctaggaaaagatctctaccaaaggctgcccattccactcctctaatccaatcctcatgtccacagagagaaagcactttctgaaactgatcattttgttgagcaaatatgtgaattctgcaatcatcattgccacatgctaatattggtattggcctgaatgcagatggaagaaatgaaattctgttatgatgccagaatgtgtgcagcttctccttccacagagccttgcacagaatggaagcgtaacatgaaaccatagagtcgcagctcctgctacagagggcgagagaggctggtggcttccaggccctgcctcgttccacctggccagtcttccaggtaacatcagtatttggcaaaaaagataagcagagagccaaagcaaatccatttccaaagtttaaagtctgaaggcacattacttctggaccctttttagaccagagtcgaacagcagaatctgcagctgcagaaacgatcagtgtacataatgcaggatctgatgtcctcctctggtaaacagcatgcaccgcataaacaggtccttcatggccttgaagatgcactgcttttaaaagctgattatcctctatttcccagtgaatcacttgattatcagatcctccagaaactaattcagtagaaggggagccatcctgtttacaaatccactgtatgcaattgactcgggcggtgtgaccattcaagttggtaacaacaacccttttcagggggtcatagagcaccacggagcaggacgtgccaaaggccagaagtcctctgggcccagagctccagttcaggactccccgcacccggtttgggcagcaaaacacgtgagaagtctccagcacgggtgccaccatgtcgccaactggtcagccgcacaaacaagagacgc

SEQ ID NO: 12499 - RNA, 95 nt, Homo sapiens
  source 1..95: mol_type = other RNA
gaacgcctgttcttgccaggtggcccctctcctacagctaagctaccactgcagctctcagaagtttccagtaacagccccttccttgccccttt

SEQ ID NO: 12500 - RNA, 5747 nt, Homo sapiens
  source 1..5747: mol_type = other RNA
gaactcaccctctgctcccagaaaccctcctggctcctccagaccctccggggctctggcccgcagctcccctctccctccggcggcgggggtcggctgtgactcaccagagggccagcggccggggttggggtgggggggccggaatgctctcacttcctctccgcgcacctgccccgaggctggagcgccgcccggccgggcctccggcggatgttttccttgttcccaagcgtgtagtgcgcgccagccgccccctccgggacctgcgcgccagccaccgcgcccccaggacccagcgggcctggtcctcaccactcaccccctccccagcaggcacgcatgcgggctcgacccacacctctgcaccgccccccaacttctgggagaggactcctggctcagcccagcctctagctttccagaagcccctatatgcctacctcatcttcgttataggcgatgaaccttcacttctgtccccgtttccgcacacgcaccaatccccactggcgatcccttccccttcggcatcacccccaccttcatgcgccccagctccccactcacatccgccccctattgggctggctctagcttgcaagagcagaaggtggcccagggcccagccttccaggatgtcccctggaccccctctctgggaaaggcggcagagctactggccactgacaagacctttgggccctcgtgctagacaggccttcgaatccacctgctccagcccagagagcaggcccaggccgtgcctcccacaccgcagccgacctcagagcaccctgcctcaactgtgagttttttcttggcaatcctctgaaacggaaagggtatcagtcctgactagggcgaacgtgaggtccattctgcatctccatccaccttagctgtctccttggaaaaggacagcaagggagtttgaggtgcactgacacagtcatttctgaacagtgaagagatgacaggtagggtggtcccccttgaaaagtcagccagaagtagctgtatctgatgcactaggtggcagggagtgagtcttggagtaaatgggactgaaaacgtagaaaaaccaaataaatgccaaagagactatccctatggagaatacctagaacatgggtctttgaagtgtggaaaaatgaaagaaatccaatttgaccagggcctttagtgccaaagagatggctagcaggagagtggtgagaaaggagaactggagagttcacatgagcggaaataggaagaaatggatccaaatccaagtgagaaaaagcaggagacttaaagttagcctggcaggatgatgagaaaaggacatcttgtcctagggtagaggcgagggtgcagatctgggggaagaaggcttattgggaacagtttctcaaactagacattcagaagtcaatacaagggccaaaaccaaaatgttcctggaggtacctgtttttgaaagaggtgggaaaggtgacatggattaggggtctccatcccccaggccacaggccagtaccagtctgtggcctgttaggaagcgggagcacaaagcaggaggtgggcggcaggcgagtgagcattaccgcctgagctcctcctcctggcagatcagcagaggcattagattctcacaggagtgcaaaccccactgtgaactccgcatgcaagggatctagattgcacactccttatgagaatctaatgcctgatgatctgagatgaaacagtttcatcccaaaatcatctccccgctgctatccccctccatccactggtggaaaaattgttttccacaaaaccggtccctggtaccaaaaaggttggggactgctgacaaggagtatgagtgtgaaaggtgcagaggtctatgccaggagacagccatccccaatagaagccctcagctatgcacaaactgcttaatgtcattcaaagaaaataatgtcgcccattttgcctcagagctttagccccaatcacagcaactgctatttcctgacgcttacgcaccagagatggtgataagagcactgcacgcattatctcagtaatcctcataacagcccaatgagttggcattactatccccaatttatagatgaggaaacaggctcagagaggtgaagtaatctgaccaggttacatagctaagtggagtcaggatctgaatccaagaagactgtctctacagcccatgctctcaataatccatcctgggctcctccagaacctgtgggaaactcagaggatgccaaatgataaattcctaaaaacctcactccattatatatgggaggaaagagaggacacctctgtgaacctggagtgattcatcccatcagggcacttagagatgctcctctttgaaaggggaaagaaccatccccagatgtggggtgatcccacatctgctgtatgtttgaaggtgataagcaatggacagttcacctctggaatgcctgaggaaaagagaccctccccaccatctctgaggggcagccctatttcttggatacattagggaaaccctgccctaggatctgagggaaacacagtctccactccaggtgcctgctcactctcctggagcttctggccgtcgcaccctattgcagctcctgggtttggctggggcacaggattaaccatccccaggaaatgcctccctccggtccaggcagggatcccagcatacacacccctggtggtggcagtgggggagaaagggggaaggtggaatgcttccttctctccaggtcagggaagagatctggggaccacctgggggccctcgcccctcctgcctccttgctggggaagtgcccagtccagtgccccctccatggccacctccctccctctagctgtgccggggcatgaatcagctctcacagcttgttaaagctagacctcttgttttcatgccctcacctcaggaaacagagttacaacttttccagctctactcagcagggggccagggtcctcactttataaacatccccagcctgtgagagcagagggcagggagatagtgtgagacaggagcccaggggagaaagacagaaactaagactcaaggagcaacgcaaagcaaagtcaaggagtcaagaccagagtagctgagcagaggccaagaagggtctgagagggctgtgcagcagcaatggccctaaggatgctctgggctggacaggccaaggggatcctaggaggctgggggatcatctgcttggtgatgtctctactcctccagcacccaggagtctacagcaagtgctacttccaagctcaaggtaaagtggggtgaagcgttaggaatggaggagcagcagagagggcacagggaggatggggccttacagatgatcccgtgtcaaaatacccaggcttcctccagctgtgaaacaggaaagacaaactaaatacggggatagtgcgtacttactgtctccaccccagaccagaagagcctctgcctctcatcagcactcctacacctactaacatttcccgttcttccctagccccctgtcactatgaggggaaatattttaccctgggtgagtcttggctccgcaaggactgtttccattgcacctgtctgcatcctgttggcgtgggctgctgtgacacgtgagtgaccaaagatggccagagagaatgactctgatatgagtgactgagggatgaccagggagtgactagattgctgtgatgtaagaatgaacagaagagcaatacaagatgggccaaacctgaagggaccaacactagtgtgaaagataaggcttcaggctataaatcaggggaggttggggtggacctggagagaaaatactcctgttataaaacaaaaaggcccacatatggtaggtgacagcttagttaggaggaccaaggggccactgaaaggggctctgtggggggaaaactgtgagagagggaacatgtgggcagggataaaggcagcctttcactgtgctgactccttcccctatccttggttccccaggtcccagcatcccatcgacttcccggctgggtgtgaggtacgtcaggaggcaggaacctgccagttctccttggtgcaaaaatctgaccctcggctgccctgcaaagggggagggcctgacccagaatggggctcagccaacacccctgttcctggggctcctgctccccactccagctaaactcaactgatcatccatctgctgactgctcactgctgctgccacttccagggaaaccactagcagctgccaatgtattctgaacaaataaattaatgctatagctgaaagcccgactctcactgtccacgacattggaccccaggtggaaaaagtgggtcccattagagtccaggtgctgagttctcagtatccggaaggaactagcaccagggtgggccagtttcagatggttatggtgctggtgctggggcctggggcagcatatgaggccagggtggggctagtaggcagcaccttgatgggcaggtcccagctgaaggtgtctacaggtacttgctcaggtcctgtccaggtggtaggttcgggctgttccacagggggtaggagtaccaatcctggttctcgggacgttacaaattcaaaatgcaatctccacttcaaggacacaatggctgtacagaagcctggggtggagctgagagggattgggagggagaagctggttctagttgtatgtaggcaggattcctggtgccgggcgtgagtcacatgtgacacagaggggacaccccctgccccacgtcgccgctggtactcaggctgtacacgctcctcggtctgtaagctgactgaaaactgcaaacaagctacggttccttcccctaagtttaaggtccccaccacgtcctcgccaagtctgtacacagatttgaagatgccaaacgtcccaactttccctcggccatcactgatattgtatagatggaggctgcggcaggatgtggcagccattaggcgttccccagccagctcagctagccatgaatctttcttcccaccttcatcctcctccaagaatggactggatggggctacagcctcatcctggggaaaccggacatcctgaaggccagtcagcacaagaaccctcagagggactctgagtaaagtgataggggagttgacacgctggcagccaatggtcagtttgtagacgtacttgactgactgaccccgaaaggagggtggtccctctatgggcagcacttcactgtaggagtatgatttggactctccaggatcaagcctcaggtcacagaatagaattttcggtggagtagaaaggatacactggcccctctcacctcggtgtggcagaaagacagtctggctgtcgggctggacatctggctgactagagtcaggaggaggcagtgctactcgactctcactggcatggaactggcagtggatttgggcactggcccaggccagggcctcactggatgcagaagtggccgtgggcggaagggggttggtgacggtcactacacactccagcgcctccccagccaaaaatacaggaccccggctgagctctgctaccacttcaatcatggcagctccggaatcagatctcgcatagtcgacactagggatcggcacccctaggcctcatctgcccgcccctcagggacctggctaggtacgcggcggcggcggcggcggcggcgtccgctgggcggtagaggcgggact

SEQ ID NO: 12501 - RNA, 5653 nt, Homo sapiens
  source 1..5653: mol_type = other RNA
gaagaataggagggactttgtttaatctgtgtgtgagggagaatgtgaataggatatcactgagaggggcttacatttcttagcagctccttgtagatctcagcttgccactcagcctccctcttggacttcatttcattccaaaggtttcagagaattccacatagtatttcaattaataataactatgtatttccctgaatagcaaaatattggacattcccagagagaggcaaaagggccagagtcccaccacctcagttatgagcagctgatctcattgttagactcatgtgtggcattaaattgtagatttgtggtcactttctgtgttaataggacactttccaaaagccttgtcttcttttgacagccaaggtgattggcttcagtgttttcagaaatgcagtgggacacaatgaagagatgtagaagggtgacaggaaccaagggctggagctgccaggcttctgtggtgccgtccttggcaggaaaaagtgtaggagtcatcccctgaggaaaaggcaccaggtagatcctgggaggggattcagctgactgggtgcccaccattagttactgtgaagataaatttaaggagtaaggatcatggcaaggagagtggtggagaagggctccaggcacaggtggtatagaaacagtaggcctgggtacaagctgctggcagtaacttgacaggctcacatatgtttagaaaacctcttatatttgtggttctttcccagaaacttcagtgctcaacaccctgcccttcatcacactaagggcaagcagaactaagctcagtgatccctcccaaagcacttgggccttgggtttgcctcctggctctaggctcattttagcaccaagcaaactgtcttttctctattctcatgtcctggtcaggcatgagaatcaacttttgtcacaggtactctgacctccaactacgtgaccctgctccctaccaatccctgggcctgtgggacaggcccttctccattttctactgtcatctcattccaggaggctttcatttcatgcaactgagaggcagtggaggcagtaaacaggcagcaggattacagcaggctccaagatggattttctagaaagatcttcccagtataaacagggagaagtcagaggagagtctatcatctggatctgacatctgtcttattagatattgtgttttgataaacacaaaagcacctcctcaaggagggaatactgtggcactcctctaaaatgaaccatctgaattgtgggttaaagctccttccctagacaggaaggtctttttagcctccctcacaccttcccttaacacaatacagtggagataaggagcagatgggcaacgtattgctgaaacatatagagtgcatttctagtggcaccctgccccaccagcatatttatggaaatgaaaatactggtcctctggagggctgcagcagttggggagcctataaactctttttcatggctctgtgtgttctccttgagcagaccaatgtttctatctgaactgagggttaggagctagggtgggtgccctggttggggggcacaagccactcaaggacagtgacgaggacagtggtgggggtggcctggggttgaggcagagccaggttgtctggagtgtaaccgaagcttattgtctagggactggggaccatccaagaaagctgggcccatcagcttctgagcacgatgagattgggccttggagcaccctgtcggcttctctgtcttacttctccccacagggctcttggctggagccaggctctttgcaacattttcttttctggttttggccaccttcacagtggcagagaacatggaatccttgtgccctttgccttttgtcttggggttaatacactccagaaaacatttaattttatttctgaagctagactctgtaaggctgggcttcttttgagtatgggctggcatcaccagcccatgtaaaacttggcattgcaaagtttggccctgcaaaggcttagcctgagttggttggctcaggaaaggctgaccctgtgaagctggggcaccacagtctgggtattctcaggaattgttgctggttcaaggatgacagttagcttggtttgactgtcttgcaggtccttctcagactctttctccccagggactcgtggaggtagctgtgggagcttaaactgagggtgatgctgggggctgtgttgacagggatcagcaagatgaaagctacggctccatcgccaggaccctcggggtgtcttgtttggaagcatccctgctggcctctggtcttcagcagggcgtctctcttctctggttgaggagcgcccaaaccccgcatccccttctctgtagtccctggctgctttggtttcctctgggtcctctctgtttcctgctagcatggggacatgggctgggtccttgctcttgctagggctttgaggctcagggccacagggttcctccaggctggggttgttcacactggcctctacctgaacacaaggcatgtgggcctctgtcatgtccccactgggttgtgagatcttggagaccgagtgggcagaaccctggggtactgctttggaattggattgcttttggttctgctgcactgccttcaagtcattggccagctgttctttaaggtgaaccccttctggattaggggcaggaagagtgtctggtgggatgggcagttcctggagcaatgtctccccttggtggtttagactttcaagagacttctgtgtggatatgttctctggtgctgcagcagtttgttccctggacttccttgccctaatgggaattccccattgtatctctaggaccttttttctcaggtggaagtttagtttggtcaagatatgtgtctggagtgagtgggggctagtaggatgcgtctggctttctagaggcagcgtctccattgttccttttactggcactgcaggctggaactcttttgcaacgtctgtacaactctcattgttgccttgagggcatggcccaagacttatacactgttcttcaaatgaaaccatctaaatcagaggctctgctgggatttccacgggactaggctccatctctgtgatgacagattggctagtgactgccggggccagggccctggggagcgccacataatacagagcaggcagccccgacaggaaggccagatgcttgtgccgtaaagttgtctccagtttctcaatggcttccacagacaagactcggagcagcttagggtgttcagtgacagtacctggtaaggcctgttgctgctgatcaagggccgttggcatccagggcataactttgtgatgtaggtctgggtcacttgctgtctgcagtaccaggaactggctttctggaatgcagggaaaaggagccactgccaggaccccagaaattctgcagtcccaggacctgtgtacacaggcggggatcttgccctggtggatttgtccacatttggagtcgatgtggctctgcagtattgccttgacctgagttaacaagtgtggcctggggatggacactggggccgcaatgggtgacagcacatcgcaagccccgttggcctctagggctacaggctgggggatgctcacgttggctagggctgtgctgctgctggacacagtctgctggtcagtggaggtaaggagcaactggatggactgctggatcttctgaggcaggccccagcgatggcgaatcgactgtttctggatgtggaattccagcagcttccgggcatgctccgggaagaagagtagttccctggtgagcactgagatggacttccctgtctgggaagctgtcgtggtctcaggagactgagctttgccacagggctcatgctgcatgaggcactgggtgtgctgagacctctggagggcagctggccagccccactgaagctggagttgcctctgtagcaggtgccactccaaggcttcatactcagccagagtcagaaatgggacattgatctgagctcgttgatggtcagatggagacacccaatttggcgaaagtggggaagagggtggggctgactggggtgaagttttagggagcagttgggggaaggagagatcattgaagagaaaaggatccttcaaggggggcttgggcacattttcaatcttgggaaggccttgagatcccatgaaagtggcaaccagggactcactgtgcagagaagggagcccacagaatagctggctgtatttctgctggagatcactccctgagtcattatcttgtcccccagactgtggatgggggccacttagggctttaagggctggagagggcaaggctagagccatagggtttggagtttgctgacagtggtgtctttgttctgggttcattgtggaccattcagaaacccagaaggtctggatgggctggccagccacacatgaacaccaggtctggagggaaatggtctcagatctgtgaagagagacctgagaagtattattcaggttgaaagaaactggctggtcatttccaggttggtaatacaatggtgggtttggcataagctgcctcagggactcctccacacgtcttgggagcccccacctctggaaatgcatccattttttaacatgtacctcaagaagcctcagcacttcaggactgagaaatggcaggtgggcagggaggaccatatgcaaggccatcggatgcatccggttcagggtttctgggttcagggacagcaaggagacctggaaattcaagtgatgctggccttggtttccctggacaaggctggggttgctctgctcatctcctcctggttcagtggagcccttggcttgtcaagccttgaagaagctatggtgtttgggccccggagcacagctggcacttgaaattccggccctagctggaggtgatcagcccagtaatcttgtatgccatctgcatacgttgactgggcagctgactgggttaaagatttctgatctgttaattgtgacagtgttgggtttatagatgccagtgaaagctctctgatatttctggaatggagctctatactctgctcaaaggatacactagacagagacaagatctctaggcaagaggagacctgtgatggactcctcgacaaagttggggagatctagtcattctcatccgccagcaactgctgaatctccagagccatagcattgcaaatttggcaacagggatctgtacataggattcgccgcacacttccctctgggggaagccagccctggcttttcatgacagagaacagctcttgtggcttctgatcttcttcctgagaaagtctcctagctgttgatgctgcatctctagctctttgcctgactttttggtgacgccagcagcagctcctttcaacttccaagttcaattcatggtggctccttttcacttgccagataattacaataacgatgaagatggagccataggtgtataagggatatccaacatcccacagaacaaaagtagggctcaacatggtctaaacctcattagcatgagatcagccatccctctatctcggcattcagggttctggtgcctaatgactcccagtgctaggccttgtcat

SEQ ID NO: 12502 - RNA, 4589 nt, Homo sapiens
  source 1..4589: mol_type = other RNA
gaagctctcccctccccgcagcccgagctgggggaggacagagatggccccacttctacaggcagccgtggcccacagtccagcacagtgctctgtgctcccaggctgagcgctgactgggacgtgtggccaggggggctctgttggggcctgggtgtgttgggctcagcttctggtgagagagcccccagcaccatgtggggcggagggatgggtacatgggtgttccaccgtggccgggtggaaaccacatccgacacaggctcccccaagctgatgctggcgtcggacacgtgtccatgggtgttgcaccgtgaccggatgggagccacgtccgatacgttctccccaaccctgatgctggtgtcagacacatgtccgtgggtgttccaccgtggccgggtgggagccatgtctgacacagactcccccaagctgatgctggcatcagacacgtgtccatgggtgttccaccgtggccgggcgggagccatgtctgacacagactcccccaagctgatgctggcatcggacacgtgtccatgggtgttccaccgtggccgggtgggagccacgtccgacacgttctccccaaccctgatgctggcgttggacacgtgcccgtgggtattccaccgtggcctggtgggagccacatctgacacattctccccgaccctgatgctggcgttggacacatgtccatggatgttccaccgtggccgagtgggagccacatctgacacagactcccctaagctgatgctggcattggatacgtgtccgtgggtgttccaccgtggctgggtgggagccacatctgacacattctccccgaccctgatgctggcgtcagacacgtgcccgtgggtgttccaccgtggccgggtgggagctatttcagaagcgtagtcccctgtgggaagaccaccccctgacacctgcccaaagagccgctctgtgggctggctgctcccctcctccagagcagcacgcctgggtgggtgtgaggggagcagagtctcccgcgaggcggagccacaggcatccatcttcccacaactgtcctcccacagctgtagccctgagctgcccaagctgcactctgcagcctgcaggggccctggtgcaggtgaggtggccacagctggcctcaggacagtactaaagtcgtactcctgtggcctggagggctgagtgctggctgctgcgggtgcctccccaggagctgaggggggcaggtccaagttaatggtctgcagcgccacctccaggagagggaccatgccagtctgcacggacggctcagcccctgggcccacaggtaggaagtctccaatgctgaggctgtcagagaagggtctggccccctccgcctgctgcagccccctgccaccagcccccactgctagaggcttaaggggctgtggggtcagcaggcctggcctgttccagccatcccaggcaggcgagtgttgctctgcagacccagaatcacagccttggcctccctctgggtgctcagggcccggagacgtgacctgggggtgcacgctcaagaggacgtctggcggctcctggggctggtgagcctcagacactgctttcagcatctcctgaatgtgtttctcatcttctaagagaaaacgaagccgtgcactctccagtcggtgcctctggattctccacagtgccttctgctcccgacgagctgcctctgcagagagcttgctgtagtggtcgaccagtgcctgcctcgccttcctctccagctcctcctccagggacttcagccttctctccctgtctcggagttcacgggcgtagctgaagtcatcatccagctcctcctgcctggccgcctggcgtcgctcctggtccttcacaaattgttctttcagcctctgaaactgctcacgcttccgggcatccaaggccatccgttctgacatctgccggtcactcagtgcactcaggaccctggatgctgcttcccgggcatgagcgattaattcttgttttgcaatttccatacgtaattccttctcctccttgctgacagagctgtggcgggccaccctctccatgcgcccaacgtagacggcacagtccttctcaatctccttcaactcctcaagggagaaaatcaccgagatccgggggacagggacgtcggaccaacagaggtaatgccgggggcagcagagcttcagcaggttaatggtctttccgcagacgtatatgtcgtgggcaatgtgcttcagaaacacgggaacacagtcctccacctctttggagatgagcacgtagccatgtgtccagtacaacttatctcggaagctgaggtactcgtggttcacctgaatcatgaactcgccataagcgtctctgaacaccccgctgtacacccagtcgtggatgaaccgggtgtagggctcgcagctggtcttcagcagggacagcagtacagggtagtgctcgttgctgcagttgtgcagagcctcctggtagaggtaggacagcagcttcacgccggtgggaaacgcggccctggggcctcctccacaggtgcccgggagcacagcgccaacgccacagagctcggccaggtacctgagctgccggccaagtttcttgaagagaaaaccaatggtgaggaggctcagggtgggcggagtggaaaggacgcaggcccggtaatactgcaggtacctcctcaggccactggtgaaggcctggaacacgaggcccttgctgtacaaagagtccaggacgggctgcagagagaaatgactcaggcgcgtgtagcaggtcccatactcggccacttccgagagcaggctgctgatgctctcgggagacgctcctgacacgtggacgccccgcttcaccacaaaggcctgggccggctggcagagcgaaaacgtggcagacacgaccccaatcaagacgttcagcacgtctttcaccagctcgcactccttcaccagcacgggctgcggggcctgtaggacgcccccagcaagcagctggagctccccttggtggagcctgcagaacttgtcgaaagcgtcccttcccgcctccgtcaggtaaggctcctctctgtggccaggggggcagccaactcgctcccagcacctccgcttgctggcctcataggtaagtgcggcttcccacaggtccacgtctggggtcacgctgggctcagactgggaatcaggagtcaagttggacgctgactggaatccttcgtcttcccactgatccacactcggtgggaccttaatagccagcccagagaggtccgcattgtctggcacggggggcaggcccagtcggacgtccatgtcataagtgcggctgtgcacaagggccccgaagagcgagacccgggtgtctctctcgaacctgtcaccacaagggtcaccaaatgagaagagcccgacggtgggcaggccagtgcctggagcagcctccataacctgaagtgtttcctggatcatgctgtgacacaaacactcttctctggagatcagagactgaacgtccatctcaaacacactcaggtcgtcgcaatcatagccgctgtacggaacgtttctccccacatgcttgttgttaaggaagtagtctcgttttctcggcagaacttgagggggaccactccctgccagctgaaccaggaggtccaaaacagaccccacctccaaaagcggacagcaaggggctgcttccagctcctccacaagctcctccaaacggtcggccttggggcccaggccacccactctcaagtcaaaggacaacatgaggatcttgtttctcgctggtagttttgacatgtcaggctgcagctgttgagtctcatcttgaaaaagatttgtgaaaagagcattgtaggccaccttcttgaggctccgctttgccctcttccggttcacactgcgctggcccaggtgagtcttggcagccggcaggagggcctcacacaggtcgtcgaacagctgcgtgatgctggccatgccccttctcagctccgggcccccggcgtgtgggaaaacacctcacccgggcttcactcacgctccggaagacagggagtgagagagggtccgaagaggctgaatgacaggcggcctctccaatgccgaagctcagaactggtattttttaaaggaggtcttgcggttgctctactcagagtaaacacgccctgccctccccagtccaagcacgctgcccggcgcccggcagcccaccagaagccagctcggcgtttcttctaattcagtagccctcaacctttagggagtcacagaaccgtggcaaaaccgaagaacgaaacgcgcgcccgcgcagtacagcggacgaactcggctttgcacccgttcttcgggacccacgagaggagacggccaggagagggtgccactccgagggtcgtgggcagcggagagtctgggggctcagccgggtgggtcccgggttctggcctgcacgtccacccgttctccaggcctcacccgtggaaagtgcccacggctgccgctctcgccgcctccgtcgcgtcacagccgcgccagtgt

SEQ ID NO: 12503 - RNA, 4594 nt, Homo sapiens
  source 1..4594: mol_type = other RNA
gaagctctcccctccccgcagcccgagctgggggaggacagagatggccccacttctacaggcagccgtggcccacagtccagcacagtgctctgtgctcccaggctgagcgctgactgggacgtgtggccaggggggctctgttggggcctgggtgtgttgggctcagcttctggtgagagagcccccagcaccatgtggggcggagggatgggtacatgggtgttccaccgtggccgggtggaaaccacatccgacacaggctcccccaagctgatgctggcgtcggacacgtgtccatgggtgttgcaccgtgaccggatgggagccacgtccgatacgttctccccaaccctgatgctggtgtcagacacatgtccgtgggtgttccaccgtggccgggtgggagccatgtctgacacagactcccccaagctgatgctggcatcagacacgtgtccatgggtgttccaccgtggccgggcgggagccatgtctgacacagactcccccaagctgatgctggcatcggacacgtgtccatgggtgttccaccgtggccgggtgggagccacgtccgacacgttctccccaaccctgatgctggcgttggacacgtgcccgtgggtattccaccgtggcctggtgggagccacatctgacacattctccccgaccctgatgctggcgttggacacatgtccatggatgttccaccgtggccgagtgggagccacatctgacacagactcccctaagctgatgctggcattggatacgtgtccgtgggtgttccaccgtggctgggtgggagccacatctgacacattctccccgaccctgatgctggcgtcagacacgtgcccgtgggtgttccaccgtggccgggtgggagctatttcagaagcgtagtcccctgtgggaagaccaccccctgacacctgcccaaagagccgctctgtgggctggctgctcccctcctccagagcagcacgcctgggtgggtgtgaggggagcagagtctcccgcgaggcggagccacaggcatccatcttcccacaactgtcctcccacagctgtagccctgagctgcccaagctgcactctgcagcctgcaggggccctggtgcaggtgaggtggccacagctggcctcaggacagtactaaagtcgtactcctgtggcctggagggctgagtgctggctgctgcgggtgcctccccaggagctgaggggggcaggtccaagttaatggtctgcagcgccacctccaggagagggaccatgccagtctgcacggacggctcagcccctgggcccacaggtaggaagtctccaatgctgaggctgtcagagaagggtctggccccctccgcctgctgcagccccctgccaccagcccccactgctagaggcttaaggggctgtggggtcagcaggcctggcctgttccagccatcccaggcaggcgagtgttgctctgcagacccagaatcacagccttggcctccctctgggtgctcagggcccggagacgtgacctgggggtgcacgctcaagaggacgtctggcggctcctggggctggtgagcctcagacactgctttcagcatctcctgaatgtgtttctcatcttctaagagaaaacgaagccgtgcactctccagtcggtgcctctggattctccacagtgccttctgctcccgacgagctgcctctgcagagagcttgctgtagtggtcgaccagtgcctgcctcgccttcctctccagctcctcctccagggacttcagccttctctccctgtctcggagttcacgggcgtagctgaagtcatcatccagctcctcctgcctggccgcctggcgtcgctcctggtccttcacaaattgttctttcagcctctgaaactgctcacgcttccgggcatccaaggccatccgttctgacatctgccggtcactcagtgcactcaggaccctggatgctgcttcccgggcatgagcgattaattcttgttttgcaatttccatacgtaattccttctcctccttgctgacagagctgtggcgggccaccctctccatgcgcccaacgtagacggcacagtccttctcaatctccttcaactcctcaagggagaaaatcaccgagatccgggggacagggacgtcggaccaacagaggtaatgccgggggcagcagagcttcagcaggttaatggtctttccgcagacgtatatgtcgtgggcaatgtgcttcagaaacacgggaacacagtcctccacctctttggagatgagcacgtagccatgtgtccagtacaacttatctcggaagctgaggtactcgtggttcacctgaatcatgaactcgccataagcgtctctgaacaccccgctgtacacccagtcgtggatgaaccgggtgtagggctcgcagctggtcttcagcagggacagcagtacagggtagtgctcgttgctgcagttgtgcagagcctcctggtagaggtaggacagcagcttcacgccggtgggaaacgcggccctggggcctcctccacaggtgcccgggagcacagcgccaacgccacagagctcggccaggtacctgagctgccggccaagtttcttgaagagaaaaccaatggtgaggaggctcagggtgggcggagtggaaaggacgcaggcccggtaatactgcaggtacctcctcaggccactggtgaaggcctggaacacgaggcccttgctgtacaaagagtccaggacgggctgcagagagaaatgactcaggcgcgtgtagcaggtcccatactcggccacttccgagagcaggctgctgatgctctcgggagacgctcctgacacgtggacgccccgcttcaccacaaaggcctgggccggctggcagagcgaaaacgtggcagacacgaccccaatcaagacgttcagcacgtctttcaccagctcgcactccttcaccagcacgggctgcggggcctgtaggacgcccccagcaagcagctggagctccccttggtggagcctgcagaacttgtcgaaagcgtcccttcccgcctccgtcaggtaaggctcctctctgtggccaggggggcagccaactcgctcccagcacctccgcttgctggcctcataggtaagtgcggcttcccacaggtccacgtctggggtcacgctgggctcagactgggaatcaggagtcaagttggacgctgactggaatccttcgtcttcccactgatccacactcggtgggaccttaatagccagcccagagaggtccgcattgtctggcacggggggcaggcccagtcggacgtccatgtcataagtgcggctgtgcacaagggccccgaagagcgagacccgggtgtctctctcgaacctgtcaccacaagggtcaccaaatgagaagagcccgacggtgggcaggccagtgcctggagcagcctccataacctgaagtgtttcctggatcatgctgtgacacaaacactcttctctggagatcagagactgaacgtccatctcaaacacactcaggtcgtcgcaatcatagccgctgtacggaacgtttctccccacatgcttgttgttaaggaagtagtctcgttttctcggcagaacttgagggggaccactccctgccagctgaaccaggaggtccaaaacagaccccacctccaaaagcggacagcaaggggctgcttccagctcctccacaagctcctccaaacggtcggccttggggcccaggccacccactctcaagtcaaaggacaacatgaggatcttgtttctcgctggtagttttgacatgtcaggctgcagctgttgagtctcatcttgaaaaagatttgtgaaaagagcattgtaggccaccttcttgaggctccgctttgccctcttccggttcacactgcgctggcccaggtgagtcttggcagccggcaggagggcctcacacaggtcgtcgaacagctgcgtgatgctggccatgccccttctcagctccgggcccccggcgtgtgggaaaacacctcacccgggcttcactcacgctccggaagacagggagtgagagagggtccgaagaggctgaatgacaggcggcctctccaatgccgaagctcagaactggtattttttaaaggaggtcttgcggttgctctactcagagtaaacacgccctgccctccccagtccaagcacgctgcccggcgcccggcagcccaccagaagccagctcggcgtttcttctaattcagtagccctcaacctttagggagtcacagaaccgtggcaaaaccgaagaacgaaacgcgcgcccgcgcagtacagcggacgaactcggctttgcacccgttcttcgggacccacgagaggagacggccaggagagggtgccactccgagggtcgtgggcagcggagagtctgggggctcagccgggtgggtcccgggttctggcctgcacgtccacccgttctccaggcctcacccgtggaaagtgcccacggctgccgctctcgccgcctccgtcgcgtcacagccgcgccagtgtgaaga

SEQ ID NO: 12504 - RNA, 349 nt, Homo sapiens
  source 1..349: mol_type = other RNA
gaagctctcccctccccgcagctggcggccttcgcgggccgaggaattttgaggtcgtccgcacctacggcccggtggagctggcaggcaggggcgggggcgggagaaggacggcgggcaggccggggtggggtggggctgggggcgcttgtgacggtggccgtgaccgcggcattaggtgatgcgtccttgaggggctgggggcttccgggcggcgagcggggcgcagtaggaggctcttagagacctcggaggaaaccagcccagcgctacgggactggcaagaatgcgaagaggaaccgagagtgaacggagtgcgaggcgccgggtcggaggcgagaggggctct

SEQ ID NO: 12505 - RNA, 889 nt, Homo sapiens
  source 1..889: mol_type = other RNA
gaagtggagcacatcagtgaagaggaagaacatgcggggccgaggctccccatggggaggcaccactaacagccagccctggcgtaggaaccagcgccctgaggtcagcccctttgcctggcgtccactgagcagagcctggacacgccgaaggtgctggtcattcttctgtttctgaccaatagtatggactctctgggcagtctcacttatcagtcgggcagccccagacattgttggaggtcagaatcagaaaggaatacaggagaggaagcctccagcctgcgttgccgaggagcaagaacctacgtgtgagctgttgatggtcagggctgttgggacctgtgttttcagccaaagctacgacgagattctcatactgctggagccgttgcagaggcagagggagcaggtcctggagctgaaggcccccaaactcagggcggccttcctgaagccgtacaaacctccggaaacctttatttttctttagctgctcctgcagggtggtctgggacctctctgagttggcagcaaattggttatagagctccaagtggcggcagaagccctccagcccttggccccagcatcctccttccaggtagggaagcagctcctggctggcgccgtagatgagctcccaggagccaaacagggcctggcgctcaggtggtcgcagggtccccttggctttcaggatccccaaaaagtacgtggccaccagccccagctgttcttggtagcgccgctcggtctctagcagctcccgggcggtgcaggcgcgtttccgctcccagcgggcacgctgctcttgcaccgggcaccgcgaaccggggcaggagagctccatgccctggctgagggatcgacacttccggctgcagtc

SEQ ID NO: 12506 - RNA, 797 nt, Homo sapiens
  source 1..797: mol_type = other RNA
gaagtggagcacatcagtgaagaggaagaacatgcggggccgaggctccccatggggaggcaccactaacagccagccctggcgtaggaaccagcgccctgaggtcagcccctttgcctggcgtccactgagcagagcctggacacgccgaaggtgctggtcattcttctgtttctgaccaatagtatggactctctgggcagtctcacttatcagtcgggcagcccgtgtgagctgttgatggtcagggctgttgggacctgtgttttcagccaaagctacgacgagattctcatactgctggagccgttgcagaggcagagggagcaggtcctggagctgaaggcccccaaactcagggcggccttcctgaagccgtacaaacctccggaaacctttatttttctttagctgctcctgcagggtggtctgggacctctctgagttggcagcaaattggttatagagctccaagtggcggcagaagccctccagcccttggccccagcatcctccttccaggtagggaagcagctcctggctggcgccgtagatgagctcccaggagccaaacagggcctggcgctcaggtggtcgcagggtccccttggctttcaggatccccaaaaagtacgtggccaccagccccagctgttcttggtagcgccgctcggtctctagcagctcccgggcggtgcaggcgcgtttccgctcccagcgggcacgctgctcttgcaccgggcaccgcgaaccggggcaggagagctccatgccctggctgagggatcgacacttcc

SEQ ID NO: 12507 - RNA, 807 nt, Homo sapiens
  source 1..807: mol_type = other RNA
gaagtggagcacatcagtgaagaggaagaacatgcggggccgaggctccccatggggaggcaccactaacagccagccctggcgtaggaaccagcgccctgaggtcagcccctttgcctggcgtccactgagcagagcctggacacgccgaaggtgctggtcattcttctgtttctgaccaatagtatggactctctgggcagtctcacttatcagtcgggcagcccgtgtgagctgttgatggtcagggctgttgggacctgtgttttcagccaaagctacgacgagattctcatactgctggagccgttgcagaggcagagggagcaggtcctggagctgaaggcccccaaactcagggcggccttcctgaagccgtacaaacctccggaaacctttatttttctttagctgctcctgcagggtggtctgggacctctctgagttggcagcaaattggttatagagctccaagtggcggcagaagccctccagcccttggccccagcatcctccttccaggtagggaagcagctcctggctggcgccgtagatgagctcccaggagccaaacagggcctggcgctcaggtggtcgcagggtccccttggctttcaggatccccaaaaagtacgtggccaccagccccagctgttcttggtagcgccgctcggtctctagcagctcccgggcggtgcaggcgcgtttccgctcccagcgggcacgctgctcttgcaccgggcaccgcgaaccggggcaggagagctccatgccctggctgagggatcgacacttccggctgcagtc

SEQ ID NO: 12508 - RNA, 840 nt, Homo sapiens
  source 1..840: mol_type = other RNA
gaagtggagcacatcagtgaagaggaagaacatgcggggccgaggctccccatggggaggcaccactaacagccagccctggcgtaggaaccagcgccctgggggatgggagcgctgttattctggtgcagctgaggtcagcccctttgcctggcgtccactgagcagagcctggacacgccgaaggtgctggtcattcttctgtttctgaccaatagtatggactctctgggcagtctcacttatcagtcgggcagcccgtgtgagctgttgatggtcagggctgttgggacctgtgttttcagccaaagctacgacgagattctcatactgctggagccgttgcagaggcagagggagcaggtcctggagctgaaggcccccaaactcagggcggccttcctgaagccgtacaaacctccggaaacctttatttttctttagctgctcctgcagggtggtctgggacctctctgagttggcagcaaattggttatagagctccaagtggcggcagaagccctccagcccttggccccagcatcctccttccaggtagggaagcagctcctggctggcgccgtagatgagctcccaggagccaaacagggcctggcgctcaggtggtcgcagggtccccttggctttcaggatccccaaaaagtacgtggccaccagccccagctgttcttggtagcgccgctcggtctctagcagctcccgggcggtgcaggcgcgtttccgctcccagcgggcacgctgctcttgcaccgggcaccgcgaaccggggcaggagagctccatgccctggctgagggatcgacacttccggctgcagtc

SEQ ID NO: 12509 - RNA, 678 nt, Homo sapiens
  source 1..678: mol_type = other RNA
gaagtggagcacatcagtgaagaggaagaacatgcggggccgaggctccccatggggaggcaccactaacagccagccctggcgtaggaaccagcgccgtgtgagctgttgatggtcagggctgttgggacctgtgttttcagccaaagctacgacgagattctcatactgctggagccgttgcagaggcagagggagcaggtcctggagctgaaggcccccaaactcagggcggccttcctgaagccgtacaaacctccggaaacctttatttttctttagctgctcctgcagggtggtctgggacctctctgagttggcagcaaattggttatagagctccaagtggcggcagaagccctccagcccttggccccagcatcctccttccaggtagggaagcagctcctggctggcgccgtagatgagctcccaggagccaaacagggcctggcgctcaggtggtcgcagggtccccttggctttcaggatccccaaaaagtacgtggccaccagccccagctgttcttggtagcgccgctcggtctctagcagctcccgggcggtgcaggcgcgtttccgctcccagcgggcacgctgctcttgcaccgggcaccgcgaaccggggcaggagagctccatgccctggctgagggatcgacacttccggctgcagtc

SEQ ID NO: 12510 - RNA, 336 nt, Homo sapiens
  source 1..336: mol_type = other RNA
gaatcggaaaggaggcgccggctgtggcggcggcgggagctgctcggaagctacacctcgcaagggctcccccctttccccaccccctcccccgacccttttcccctccccgggccacccagcccgcccaactcccagcggagagcaaggtaagagactcggccgaccccttcttttcctccagctccctccccccaccctttccccgccgctctgccgtcggggagccggactcctgggggcgggagggcgagggagaaggcagccctcgccgcgcccacgcgtgctgccaccctcccggcgcccaagcggcggcgccacccgcccagccccctt

SEQ ID NO: 12511 - RNA, 1571 nt, Homo sapiens
  source 1..1571: mol_type = other RNA
gacaattgttgatcttgggcctccatcgcctaggggaagcctggggcacacaaacatctcccgcgtttcccaagcgatcccccgggctggtgccctctggcgccgatgatacccctgcgctctccactgcggtggaggccagccgggcctcgcccaccccggggcccgccctcggcgcccaacccttcaccctccgcttcagcttcccccaggacacctggctgacatactcccgccacctgtccgctttggacagctgaggccccaggttgtcctcaaacatgggcactggcaggttgacgcggcggcgggcaggcggcgcgctgggctgcttctcctgtcgccggaggaaggcctcgaccagttcctcatcatcctcactctccaggtcgcttcccaggaacttgctgcccaggtagctgacgggcattttgcgcaccttcttgccccgccgcgggccctggcggctcttgtctctggaggtctcgaagtcgctgaactcgctgtcgctggcgttgctgctgtcgtacgtgcccacgaccagccggggcggaggagtcaccatctgctgcactctcctcctcactcggggctccttgggctttttggggggctggggcgggtgcggggtgctcttctccatgatgcgggccacgtcctccagggtgcggccctcttcttccaggaactgggtcagccgctcccgaaattctgcttccttggtggcgggcttagagatgactctccagacgcccccagccagcctgacctcccgggggatgagcaaatagtcgacgtcctccccgatctgcagcatccccaccgtggagtcctcctccttgcggaacaccttgccgatcttcttaaatgtccccacgggctttagggcttccacgaggacgtccaaatccacatctttgcagacatcggggacgctccaaagaatgaggcagtcgggggacggcaggaagccccaggggaaccagccccccacgtggcttttctcgagagtctttaagatctccagggtgatatctggggtgagggggcaatgagccccaacaaactactgtagcccttagtcttgagggagggactggatggggggagttccagcaacgctgaccggagagtctcacctccctagccagggacgagccaaacgcctccaatctcttcgcctgcaacaagtacagtcttgaccaagtccggctcccccaccaaggacttgggggaatcaatttccaggatgcctacgtgagccgggggcgaggtcagtcccaaggctcaaggcccactccaagctggaaacgtggtgtcccagctccaagttggggcgcgcgggctgccagcgactcttcctgccccaggccccagggacgcggctggaacttgggacaggacttcgcagacaaagacggtccagtcgaagctattcaatatggccgaggcgctgggaggccccagcccgggcctccagtagggtcccccgcccccaggcaggccgccacccagctccaggctgaccttgacgcgccgcagcctgccagcccgcgcgcttagagctctgc

SEQ ID NO: 12512 - RNA, 1911 nt, Homo sapiens
  source 1..1911: mol_type = other RNA
gacaattgttgatcttgggcctgttccactgttaacataacttttttctgcttctgtcctctataactgtatactgcctctgtcagtataggaaatcaacaactcttagtactgcgtggactaacacatcaggttgaaggtgctccaattctacaaagtctatactgttcaccctctgaggctgtctcggaggaagatctctgaggtaggaatgttttgaggacacatatgccagtaagtcttgaagtacaacgtcactaactacactggaatattcttcaggctgaatagatgaataactcccaagatttaataactgactgctaaatgttgattgtagtactgtctcaccaatccattggtcctcatgaataacaacatccgtgagtaaaattatatctccaagaaacactgtaaatgcccaaaatgctgcagtcctccacagaaaaaccttcttcttagtttctgattgatcacttactgtaactgttgctaaaggcactttagagccagaatttggtccgaattttatgtttatttccttcacatggcatggagatagcaccatgactaaacaattatacttctggcttttagaatcacagttttttattaatgatttttttaatactcttaaattcagacacatttctccgatccatttctacagcagaatctcctccattagaaatcaacttcattttcttagctacttgaaggactctagatagagcttcagactgggccactttatcttcagaggtacagcttcttttaatagcacttttgtggaaggtatttagttgggaacacagtattcctgagctacacaactcaatacgtatctcatttggtggcagttcatcttcagaactgaaaagttcttgagatcctgtatgttcttcaagacctttatcagagtttatgtgaatgcggctattttctgttttaggacaaacaggactaaaaagttcaagggaatatgcttggttttgtccactttcatatgcttctgtaaaaccatcaagctgaatcgaattctcttcaggtattcttatctccccgtaacttgcctttggttcagtctccatgtttacattccctttatttacaggactccgccttttatctttcttttgagctaaaaaaagcaacctggctggaggtaattatactgagaaattctttatcagttgatattttaaggtctgagaccttcttaactgctgcttcagaccttgacttatctactgagttcgaggaaaataatcccaaacgctggttttgtatttcatgatattctgttggcacacactctctttgtaccacttcaggccctatattaattttttcagtactacaaaccaaatccaacacagctgcacatttatggcccaactgaaacaaatttgtgttaaagttctgaccacatatatctggctgatgtttaggctgttcatctctaattttattttcactgagaagctttgatacttttcttcttcggttaaatgcggaactgtgcttttaaatccacatatttgcatattagagctagttatgccactcagtctagaggagtgaatcttctgggattctatattctgtgtttcagaaacagaacgtacaaagtcatctttcacatgaacatgtctattcatacagtttgctaagaaatgaccacaaagatctggagaaccaatagaatctgggacttcatagttttcaagatttttgtgctgtttttcatccttcagatataaagaatgttgactgtataaaagctgaatttttttccaggggtcagcaacagacattaaagaagctgtgtcttctgatactgtcattttcagtggagcaactggagcaccccaaaaaatgtggacttgagatcctccactcatgatttct

SEQ ID NO: 12513 - RNA, 945 nt, Homo sapiens
  source 1..945: mol_type = other RNA
gacaattgttgatcttgggcctgttccactgttaacataacttttttctgcttctgtcctctataactgtatactgcctctgtcagtataggaaatcaacaactcttagtactgcgtggactaacacatcaggttgaaggtgctccaattctacaaagtctatactgttcaccctctgaggctgtctcggaggaagatctctgaggtaggaatgttttgaggacacatatgccagtaagtcttgaagtacaacgtcactaactacactggaatcttgtgaagctgcccccgtccattttttctgcctccaaaatcatccttcgaaaaacatcaacagcagtctgattttctttagcagaagattccaaaaaagctgcattccaagattctgccaaagctttcccttcttcataactgatcaccctttccatatgcaggtctttcttatttccaaccaacataataggtatttgtactttccccaccatatccaacaatttgccatggataactttaatcacttcaaaacttttgattgatgtaacagaatacacaagaatatagccattaatatctatggagtatgtctgaggaaagatagaatattcatcttgcccggctgtgtctacaagttaaagatgatattcttgtccatttactgtgatcaactttgtaaaagtgttttctatggttggatcgtaggagtccacaaattggccttcaacaaattgaatcgtcaatgaggatttccccacagaccggtagcccaggatcgcgatcttccgggactttgactgcggcatcttggcggcctcctcagccccggcccaaccacatcaaccgcggcggcggcggctcctgctgctgtgatcggcggcggccgcgccgggagagagcggcatacagagcaggggcggcggcgggcgcggctgcctctcgctcgct

SEQ ID NO: 12514 - RNA, 1911 nt, Homo sapiens
  source 1..1911: mol_type = other RNA
gacaattgttgatcttgggcctgttccactgttaacataacttttttctgcttctgtcctctataactgtatactgcctctgtcagtataggaaatcaacaactcttagtactgcgtggactaacacatcaggttgaaggtgctccaattctacaaagtctatactgttcaccctctgaggctgtctcggaggaagatctctgaggtaggaatgttttgaggacacatatgccagtaagtcttgaagtacaacgtcactaactacgctggaatattcttcaggctgaatagatgaataactcccaagatttaataactgactgctaaatgttgattgtagtactgtctcaccaatccattggtcctcatgaataacaacatccgtgagtaaaattatatctccaagaaacactgtaaatgcccaaaatgctgcagtcctccacagaaaaaccttcttcttagtttctgattgatcacttactgtaactgttgctaaaggcactttagagccagaatttggtccgaattttgtttatttccttcacatggcatggagatagcaccatgactaaacaattatacttctggcttttagaatcacagttttttattaatgatgtttttttaatactcttaaattcagacacatttctccgatccatttctacagcagaatctcctccattagaaatcaacttcattttcttagctacttgaaggactccagatagagcttcagactggcccactttatcttcagaggtacagcttcttttaatagcacttttgtggaaggtatttagttgggaacacagtattcctgagctacacaactcaatatgtatctcatttggtggcagttcatcttcagaactgaaaagttcttgagatcctgtatgttcttcaagacctttatcagagtttatgtgaatgcggctattttctgttttaggacaaacaggactaaaaagttcaagggaatatgcttggttttgtccactttcatatgcttctgtaaaaccatcaagctgaatcgaattctcttcaggtattcttatctccccgtaacttgcctttggttcagtctccatgtttacattccctttatttacaggactccgccttttatctttcttttgagctaaaaaaagcaacctggctggaggtaattatactgagaaattctttatcagttgatattttaaggtctgagaccttcttaactgctgcttcagaccttgacttatctactgagttcgaggaaaataatcccaaacactggttttgtatttcatgatattctgttggcacacactctctttgtaccacttcaggccctatattaattttttcagtactacaaaccaaatccaacacagctgcacatttatggcccaactgaaacaaatttgtgttaaagttctgaccacatatatctggctgatgtttaggctgttcatctctaattttattttcactgagaagctttgatacttttcttcttcggttaaatgcggaactgtgcttttaaatccacatatttgcatattagagctagttatgtcactcagtctagaggagtgaatcttctgggattctatattctgtgtttcagaaacagaatgtacaaagtcatctttcacatgaacatgtctattcatacagtttgctaagaaatgaccacaaagatctggagaaccaatagaatctgggacttcatagttttcaagatttttgtgctgtttttcatccttcagatataaagaatgttgactgtataaaagctgaatttttttccaggggtcagcaacagacattaaagaagctgtgtcttctgatactgtcattttcagtgaagcaactggagcaccccaaaaaatgtggacttgagatcctccactcatgatttct

SEQ ID NO: 12515 - RNA, 1012 nt, Homo sapiens
  source 1..1012: mol_type = other RNA
gacaattgttgatcttgggcctgttccactgttaacataacttttttctgcttctgtcctctataactgtatactgcctctgtcagtatagtgaaatcaacaactcttagtactgcgtggactaatacatcaggttgaaggtgctccaattctacaaagtctatactgttcaccctctgaggctgcctcggaggaagatctctgaggtaggaatgttttgaggacacatatgccagtaagtcttgaagtacaacttcactaactacactggaatattcttcaggctgaatagatgaataactcccaagatttaataactgactgctaaatgttgattgtagtactgtctcgccaatccattggtcctcatgaataacaacatcacatatatctggctgatgtttaggctgttcatctctaattttattttcactgagaagcttttgatacttttcttcttcggtgaaatgcggaactgtgcttttaaatccacatatttgcatattagagctagttatatcactcagtctagaggagtgaatcttctgggattctatattctgtgtttcagaaacagaacgtacaaagtcatctttcacatgaacatgtctattcatacagtttgctaagaaatgaccactaagatctggagaaccaatagattctgggactttatagttttcaagatttttgtgctgtttttcatccttcagatataaagaatgttgactgtataaaagctgaatttttttccaggggtcagcaacagacattaaagaagctgtgtcttctgatactgtgattttcagtggagcaattggagcaccccaaaaaatgtggacttgagatcctccactcatgatttctgtaatcccagctactcaggaggctggagcaggagaattgcttgaaccttaatcttttgaccatcaaggaaaattcaggattcaggtcagagtacatttttcactgagagccccgccggaggcgggtgcggcctccgggcaaatcc

SEQ ID NO: 12516 - RNA, 1080 nt, Homo sapiens
  source 1..1080: mol_type = other RNA
gacaattgttgatcttgggcctgttccactgttaacataacttttttctgcttctgtcctctataactgtatactgcctctgtcagtatagtgaaatcaacaactcttagtactgcgtggactaatacatcaggttgaaggtgctccaattctacaaagtctatactgttcaccctctgaggctgcctcggaggaagatctctgaggtaggaatgttttgaggacacatatgccagtaagtcttgaagtacaacttcactaactacactggaatattcttcaggctgaatagatgaataactcccaagatttaataactgactgctaaatgttgattgtagtactgtctcgccaatccattggtcctcatgaataacaacatcacatatatctggctgatgtttaggctgttcatctctaattttattttcactgagaagcttttgatacttttcttcttcggtgaaatgcggaactgtgcttttaaatccacatatttgcatattagagctagttatatcactcagtctagaggagtgaatcttctgggattctatattctgtgtttcagaaacagaacgtacaaagtcatctttcacatgaacatgtctattcatacagtttgctaagaaatgaccactaagatctggagaaccaatagattctgggactttatagttttcaagatttttgtgctgtttttcatccttcagatataaagaatgttgactgtataaaagctgaatttttttccaggggtcagcaacagacattaaagaagctgtgtcttctgatactgtgattttcagtggagcaattggagcaccccaaaaaatgtggacttgagatcctccactcatgatttctgtgatcccagctacttgggaggctgaggtggaagaatcgcttgaacctaggaggcggaggatgcagtgagccgagatcacaccactgtactccagtctggccatcaggacgagacttaatcttttgaccatcaaggaaaattcaggattcaggtcagagtacatttttcactgagagccccgccggaggcgggtgcggcctccgggcaaatcc

SEQ ID NO: 12517 - RNA, 964 nt, Homo sapiens
  source 1..964: mol_type = other RNA
gacaattgttgatcttgggcctgttccactgttaacataacttttttctgcttctgtcctctataactgtatactgcctctgtcagtatagtgaaatcaacaactcttagtactgcgtggactaatacatcaggttgaaggtgctccaattctacaaagtctatactgttcaccctctgaggctgcctcggaggaagatctctgaggtaggaatgttttgaggacacatatgccagtaagtcttgaagtacaacttcactaactacactggaatattcttcaggctgaatagatgaataactcccaagatttaataactgactgctaaatgttgattgtagtactgtctcgccaatccattggtcctcatgaataacaacatcacatatatctggctgatgtttaggctgttcatctctaattttattttcactgagaagcttttgatacttttcttcttcggtgaaatgcggaactgtgcttttaaatccacatatttgcatattagagctagttatatcactcagtctagaggagtgaatcttctgggattctatattctgtgtttcagaaacagaacgtacaaagtcatctttcacatgaacatgtctattcatacagtttgctaagaaatgaccactaagatctggagaaccaatagattctgggactttatagttttcaagatttttgtgctgtttttcatccttcagatataaagaatgttgactgtataaaagctgaatttttttccaggggtcagcaacagacattaaagaagctgtgtcttctgatactgtgattttcagtggagcaattggagcaccccaaaaaatgtggacttgagatcctccactcatgatttcttaatcttttgaccatcaaggaaaattcaggattcaggtcagagtacatttttcactgagagccccgccggaggcgggtgcggcctccgggcaaatcc

SEQ ID NO: 12518 - RNA, 659 nt, Homo sapiens
  source 1..659: mol_type = other RNA
gacaattgttgatcttgggcctgttccactgttaacataacttttttctgcttctgtcctctataactgtatactgcctctgtcagtatagtgaaatcaacaactcttagtactgcgtggactaatacatcaggttgaaggtgctccaattctacaaagtctatactgttcaccctctgaggctgcctcggaggaagatctctgaggtaggaatgttttgaggacacatatgccagtaagtcttgaagtacaacttcactaactacactggaatattcttcaggctgaatagatgaataactcccaagatttaataactgactgctaaatgttgattgtagtactgtctcgccaatccattggtcctcatgaataacaacatcacatatatctggctgatgtttaggctgttcatctctaattttattttcactgagaagcttttgatacttttcttcttcggtgaaatgcggaactgtgcttttaaatccacatatttgcatattagagctagttatatcactcagtctagaggagtgaatcttctgggattctatattcttaatcttttgaccatcaaggaaaattcaggattcaggtcagagtacatttttcactgagagccccgccggaggcgggtgcggcctccgggcaaatcc

SEQ ID NO: 12519 - RNA, 1955 nt, Homo sapiens
  source 1..1955: mol_type = other RNA
gacaattgttgatcttgggcctgttccactgttaacataacttttttctgcttctgtcctctataactgtatactgcctctgtcagtatagtgaaatcaacaactcttagtactgcgtggactaatacatcaggttgaaggtgctccaattctacaaagtctatactgttcaccctctgaggctgcctcggaggaagatctctgaggtaggaatgttttgaggacacatatgccagtaagtcttgaagtacaacttcactaactacactggaatattcttcaggctgaatagatgaataactcccaagatttaataactgactgctaaatgttgattgtagtactgtctcgccaatccattggtcctcatgaataacaacatctgtgagtaaaattatatctccaagaaacactgtaaatgcccaaaatgctgcagtcctccacagaaaaaccttcttcttagtttctgattgatcaattactgtaactgttgctaaaggcactttagagccagaatttggtccgaattttatgtttatttccttcacatggcatggagatagcaccatgactaaacaattatacttctggcttttagaatcacagttttttattaatgatgtttttttaatactcttaaattcagacacatttctccgatccatttctacagcagaatctcctccattagaaatcaacttcattttcttagctacttgaaggactctagatagagcttcagactggcccactttatcttcagaggtacagcttcttttaatagcacttttgtggaaggtatttagttgggaacacagtattcctgagctacacaactcaatacgtatctcatttggtggcagttcatcttcagaactgaaaagttcttgagatcctgtatgttcttcaagacctttatcagagtttatgtgaatgcggctattttctgttttaggacaaacaggactaaaaagttcaagggaatatgcttggttttgtccactttcatatgcttctgtaaaaccatcaagctgaatcgaattctcttcaggtattcttatctccccgtaacttgcctttggttcagtctccatgtttacattccctttatttacaggactccgccttttatctttcttttgagctaaaaaagcaacctggctggaggtaattatactgagaaattctgtatcagttgatattttaaggtctgagaccttcctaactgctgcttcagaccttgacttatctactgcgttcgaggaaaataatcccaaacactggttttgtatttcatgatattctgttggcacacactctctttgtaccacttcaggccctatattaattttttcagtactacaaaccaaatccaacacagctgcacatttatggcccaactgaaacaaatttgtgttaaagttcttaccacatatatctggctgatgtttaggctgttcatctctaattttattttcactgagaagcttttgatacttttcttcttcggtgaaatgcggaactgtgcttttaaatccacatatttgcatattagagctagttatatcactcagtctagaggagtgaatcttctgggattctatattctgtgtttcagaaacagaacgtacaaagtcatctttcacatgaacatgtctattcatacagtttgctaagaaatgaccactaagatctggagaaccaatagattctgggactttatagttttcaagatttttgtgctgtttttcatccttcagatataaagaatgttgactgtataaaagctgaatttttttccaggggtcagcaacagacattaaagaagctgtgtcttctgatactgtgattttcagtggagcaattggagcaccccaaaaaatgtggacttgagatcctccactcatgatttctgagagccccgccggaggcgggtgcggcctccgggcaaatcc

SEQ ID NO: 12520 - RNA, 2127 nt, Homo sapiens
  source 1..2127: mol_type = other RNA
gacaattgttgatcttgggcctgttccactgttaacataacttttttctgcttctgtcctctataactgtatactgcctctgtcagtatagtgaaatcaacaactcttagtactgcgtggactaatacatcaggttgaaggtgctccaattctacaaagtctatactgttcaccctctgaggctgcctcggaggaagatctctgaggtaggaatgttttgaggacacatatgccagtaagtcttgaagtacaacttcactaactacactggaatattcttcaggctgaatagatgaataactcccaagatttaataactgactgctaaatgttgattgtagtactgtctcgccaatccattggtcctcatgaataacaacatctgtgagtaaaattatatctccaagaaacactgtaaatgcccaaaatgctgcagtcctccacagaaaaaccttcttcttagtttctgattgatcaattactgtaactgttgctaaaggcactttagagccagaatttggtccgaattttatgtttatttccttcacatggcatggagatagcaccatgactaaacaattatacttctggcttttagaatcacagttttttattaatgatgtttttttaatactcttaaattcagacacatttctccgatccatttctacagcagaatctcctccattagaaatcaacttcattttcttagctacttgaaggactctagatagagcttcagactggcccactttatcttcagaggtacagcttcttttaatagcacttttgtggaaggtatttagttgggaacacagtattcctgagctacacaactcaatacgtatctcatttggtggcagttcatcttcagaactgaaaagttcttgagatcctgtatgttcttcaagacctttatcagagtttatgtgaatgcggctattttctgttttaggacaaacaggactaaaaagttcaagggaatatgcttggttttgtccactttcatatgcttctgtaaaaccatcaagctgaatcgaattctcttcaggtattcttatctccccgtaacttgcctttggttcagtctccatgtttacattccctttatttacaggactccgccttttatctttcttttgagctaaaaaagcaacctggctggaggtaattatactgagaaattctgtatcagttgatattttaaggtctgagaccttcctaactgctgcttcagaccttgacttatctactgcgttcgaggaaaataatcccaaacactggttttgtatttcatgatattctgttggcacacactctctttgtaccacttcaggccctatattaattttttcagtactacaaaccaaatccaacacagctgcacatttatggcccaactgaaacaaatttgtgttaaagttcttaccacatatatctggctgatgtttaggctgttcatctctaattttattttcactgagaagcttttgatacttttcttcttcggtgaaatgcggaactgtgcttttaaatccacatatttgcatattagagctagttatatcactcagtctagaggagtgaatcttctgggattctatattctgtgtttcagaaacagaacgtacaaagtcatctttcacatgaacatgtctattcatacagtttgctaagaaatgaccactaagatctggagaaccaatagattctgggactttatagttttcaagatttttgtgctgtttttcatccttcagatataaagaatgttgactgtataaaagctgaatttttttccaggggtcagcaacagacattaaagaagctgtgtcttctgatactgtgattttcagtggagcaattggagcaccccaaaaaatgtggacttgagatcctccactcatgatttctgtgatcccagctacttgggaggctgaggtggaagaatcgcttgaacctaggaggcggaggatgcagtgagccgagatcacaccactgtactccagtctggccatcaggacgagacttaatcttttgaccatcaaggaaaattcaggattcaggtcagagtacatttttcactgagagccccgccggaggcgggtgcggcctccgggcaaatcc

SEQ ID NO: 12521 - RNA, 2011 nt, Homo sapiens
  source 1..2011: mol_type = other RNA
gacaattgttgatcttgggcctgttccactgttaacataacttttttctgcttctgtcctctataactgtatactgcctctgtcagtatagtgaaatcaacaactcttagtactgcgtggactaatacatcaggttgaaggtgctccaattctacaaagtctatactgttcaccctctgaggctgcctcggaggaagatctctgaggtaggaatgttttgaggacacatatgccagtaagtcttgaagtacaacttcactaactacactggaatattcttcaggctgaatagatgaataactcccaagatttaataactgactgctaaatgttgattgtagtactgtctcgccaatccattggtcctcatgaataacaacatctgtgagtaaaattatatctccaagaaacactgtaaatgcccaaaatgctgcagtcctccacagaaaaaccttcttcttagtttctgattgatcaattactgtaactgttgctaaaggcactttagagccagaatttggtccgaattttatgtttatttccttcacatggcatggagatagcaccatgactaaacaattatacttctggcttttagaatcacagttttttattaatgatgtttttttaatactcttaaattcagacacatttctccgatccatttctacagcagaatctcctccattagaaatcaacttcattttcttagctacttgaaggactctagatagagcttcagactggcccactttatcttcagaggtacagcttcttttaatagcacttttgtggaaggtatttagttgggaacacagtattcctgagctacacaactcaatacgtatctcatttggtggcagttcatcttcagaactgaaaagttcttgagatcctgtatgttcttcaagacctttatcagagtttatgtgaatgcggctattttctgttttaggacaaacaggactaaaaagttcaagggaatatgcttggttttgtccactttcatatgcttctgtaaaaccatcaagctgaatcgaattctcttcaggtattcttatctccccgtaacttgcctttggttcagtctccatgtttacattccctttatttacaggactccgccttttatctttcttttgagctaaaaaagcaacctggctggaggtaattatactgagaaattctgtatcagttgatattttaaggtctgagaccttcctaactgctgcttcagaccttgacttatctactgcgttcgaggaaaataatcccaaacactggttttgtatttcatgatattctgttggcacacactctctttgtaccacttcaggccctatattaattttttcagtactacaaaccaaatccaacacagctgcacatttatggcccaactgaaacaaatttgtgttaaagttcttaccacatatatctggctgatgtttaggctgttcatctctaattttattttcactgagaagcttttgatacttttcttcttcggtgaaatgcggaactgtgcttttaaatccacatatttgcatattagagctagttatatcactcagtctagaggagtgaatcttctgggattctatattctgtgtttcagaaacagaacgtacaaagtcatctttcacatgaacatgtctattcatacagtttgctaagaaatgaccactaagatctggagaaccaatagattctgggactttatagttttcaagatttttgtgctgtttttcatccttcagatataaagaatgttgactgtataaaagctgaatttttttccaggggtcagcaacagacattaaagaagctgtgtcttctgatactgtgattttcagtggagcaattggagcaccccaaaaaatgtggacttgagatcctccactcatgatttcttaatcttttgaccatcaaggaaaattcaggattcaggtcagagtacatttttcactgagagccccgccggaggcgggtgcggcctccgggcaaatcc

SEQ ID NO: 12522 - RNA, 481 nt, Homo sapiens
  source 1..481: mol_type = other RNA
gacaattgttgatcttgggcctgttccactgttaacataacttttttctgcttctgtcctctataactgtatactgcctctgtcagtatagtgaaatcaacaactcttagtactgcgtggactaatacatcaggttgaaggtgctccaattctacaaagtctatactgttcaccctctgaggctgcctcggaggaagatctctgaggtaggaatgttttgaggacacatatgccagtaagtcttgaagtacaacttcactaactacactggaatattcttcaggctgaatagatgaataactcccaagatttaataactgactgctaaatgttgattgtagtactgtctcgccaatccattggtcctcatgaataacaacatcttaatcttttgaccatcaaggaaaattcaggattcaggtcagagtacatttttcactgagagccccgccggaggcgggtgcggcctccgggcaaatcc

SEQ ID NO: 12523 - RNA, 762 nt, Homo sapiens
  source 1..762: mol_type = other RNA
gacaattgttgatcttgggcctgttccactgttaacataacttttttctgcttctgtcctctataactgtatactgcctctgtcagtatagtgaaatcaacaactcttagtactgcgtggactaatacatcaggttgaaggtgctccaattctacaaagtctatactgttcaccctctgaggctgcctcggaggaagatctctgaggtaggaatgttttgaggacacatatgccagtaagtcttgaagtacaacttcactaactacactggaatattcttcaggctgaatagatgaataactcccaagatttaataactgactgctaaatgttgattgtagtactgtctcgccaatccattggtcctcatgaataacaacatcttagtggctgggtgtggtggctcacacctataatcccaacactgggaggcggaggcaggcggatcacaaggtcaggagttcaagagcagcctggccaacatggtgaaacctcatctctactgaaagtacaaaaattaggcgggcgtggtggcaggcacctgtaatcccagctactcgggaggctgaagcaggagaatcacttgaacccgggaagtggaggttgcagcgagccgagattgtgccactcctctccagcctgggcgacagagcaagactccgtcttaatcttttgaccatcaaggaaaattcaggattcaggtcagagtacatttttcactgagagccccgccggaggcgggtgcggcctccgggcaaatcc

SEQ ID NO: 12524 - RNA, 2220 nt, Homo sapiens
  source 1..2220: mol_type = other RNA
gacaattgttgatcttgggcctgttccactgttaacataacttttttctgcttctgtcctctataactgtatactgcctctgtcagtatagtgaaatcaacaactcttagtactgcgtggactaatacatcaggttgaaggtgctccaattctacaaagtctatactgttcaccctctgaggctgcctcggaggaagatctctgaggtaggaatgttttgaggacacatatgccagtaagtcttgaagtacaacttcactaactacactggaatattcttcaggctgaatagatgaataactcccaagatttaataactgactgctaaatgttgattgtagtactgtctcgccaatccattggtcctcatgaataacaacattaaaaaacagtggttccccactgcctagccaggaagagctagtacagcattcaagacttttcatgatccaacattcaggatgcatgttcttcagaaaaaaggaacagacgagaaatttcaaggagagcattctgaaagctaggactgtgagtaaaattatatctccaagaaacactgtaaatgcccaaaatgctgcagtcctccacagaaaaaccttcttcttagtttctgattgatcaattactgtaactgttgctaaaggcactttagagccagaatttggtccgaattttatgtttatttccttcacatggcatggagatagcaccatgactaaacaattatacttctggcttttagaatcacagttttttattaatgatgtttttttaatactcttaaattcagacacatttctccgatccatttctacagcagaatctcctccattagaaatcaacttcattttcttagctacttgaaggactctagatagagcttcagactggcccactttatcttcagaggtacagcttcttttaatagcacttttgtggaaggtatttagttgggaacacagtattcctgagctacacaactcaatacgtatctcatttggtggcagttcatcttcagaactgaaaagttcttgagatcctgtatgttcttcaagacctttatcagagtttatgtgaatgcggctattttctgttttaggacaaacaggactaaaaagttcaagggaatatgcttggttttgtccactttcatatgcttctgtaaaaccatcaagctgaatcgaattctcttcaggtattcttatctccccgtaacttgcctttggttcagtctccatgtttacattccctttatttacaggactccgccttttatctttcttttgagctaaaaaagcaacctggctggaggtaattatactgagaaattctgtatcagttgatattttaaggtctgagaccttcctaactgctgcttcagaccttgacttatctactgcgttcgaggaaaataatcccaaacactggttttgtatttcatgatattctgttggcacacactctctttgtaccacttcaggccctatattaattttttcagtactacaaaccaaatccaacacagctgcacatttatggcccaactgaaacaaatttgtgttaaagttcttaccacatatatctggctgatgtttaggctgttcatctctaattttattttcactgagaagcttttgatacttttcttcttcggtgaaatgcggaactgtgcttttaaatccacatatttgcatattagagctagttatatcactcagtctagaggagtgaatcttctgggattctatattctgtgtttcagaaacagaacgtacaaagtcatctttcacatgaacatgtctattcatacagtttgctaagaaatgaccactaagatctggagaaccaatagattctgggactttatagttttcaagatttttgtgctgtttttcatccttcagatataaagaatgttgactgtataaaagctgaatttttttccaggggtcagcaacagacattaaagaagctgtgtcttctgatactgtgattttcagtggagcaattggagcaccccaaaaaatgtggacttgagatcctccactcatgatttcctgaagattacaggtccttttctttgacacagtttctgttattgttttttgttaaagcatgctcacttaatcttttgaccatcaaggaaaattcaggattcaggtcagagtacatttttcactgagagccccgccggaggcgggtgcggcctccgggcaaatc

SEQ ID NO: 12525 - RNA, 2064 nt, Homo sapiens
  source 1..2064: mol_type = other RNA
gacaattgttgatcttgggcctgttccactgttaacataacttttttctgcttctgtcctctataactgtatactgcctctgtcagtatagtgaaatcaacaactcttagtactgcgtggactaatacatcaggttgaaggtgctccaattctacaaagtctatactgttcaccctctgaggctgcctcggaggaagatctctgaggtaggaatgttttgaggacacatatgccagtaagtcttgaagtacaacttcactaactacactggaatattcttcaggctgaatagatgaataactcccaagatttaataactgactgctaaatgttgattgtagtactgtctcgccaatccattggtcctcatgaataacaacattaaaaaacagtggttccccactgcctagccaggaagagctagtacagcattcaagacttttcatgatccaacattcaggatgcatgttcttcagaaaaaaggaacagacgagaaatttcaaggagagcattctgaaagctaggactgtgagtaaaattatatctccaagaaacactgtaaatgcccaaaatgctgcagtcctccacagaaaaaccttcttcttagtttctgattgatcaattactgtaactgttgctaaaggcactttagagccagaatttggtccgaattttatgtttatttccttcacatggcatggagatagcaccatgactaaacaattatacttctggcttttagaatcacagttttttattaatgatgtttttttaatactcttaaattcagacacatttctccgatccatttctacagcagaatctcctccattagaaatcaacttcattttcttagctacttgaaggactctagatagagcttcagactggcccactttatcttcagaggtacagcttcttttaatagcacttttgtggaaggtatttagttgggaacacagtattcctgagctacacaactcaatacgtatctcatttggtggcagttcatcttcagaactgaaaagttcttgagatcctgtatgttcttcaagacctttatcagagtttatgtgaatgcggctattttctgttttaggacaaacaggactaaaaagttcaagggaatatgcttggttttgtccactttcatatgcttctgtaaaaccatcaagctgaatcgaattctcttcaggtattcttatctccccgtaacttgcctttggttcagtctccatgtttacattccctttatttacaggactccgccttttatctttcttttgagctaaaaaagcaacctggctggaggtaattatactgagaaattctgtatcagttgatattttaaggtctgagaccttcctaactgctgcttcagaccttgacttatctactgcgttcgaggaaaataatcccaaacactggttttgtatttcatgatattctgttggcacacactctctttgtaccacttcaggccctatattaattttttcagtactacaaaccaaatccaacacagctgcacatttatggcccaactgaaacaaatttgtgttaaagttcttaccacatatatctggctgatgtttaggctgttcatctctaattttattttcactgagaagcttttgatacttttcttcttcggtgaaatgcggaactgtgcttttaaatccacatatttgcatattagagctagttatatcactcagtctagaggagtgaatcttctgggattctatattctgtgtttcagaaacagaacgtacaaagtcatctttcacatgaacatgtctattcatacagtttgctaagaaatgaccactaagatctggagaaccaatagattctgggactttatagttttcaagatttttgtgctgtttttcatccttcagatataaagaatgttgactgtataaaagctgaatttttttccaggggtcagcaacagacattaaagaagctgtgtcttctgatactgtgattttcagtggagcaattggagcaccccaaaaaatgtggacttgagatcctccactcatgatttctgtaatc

SEQ ID NO: 12526 - RNA, 2078 nt, Homo sapiens
  source 1..2078: mol_type = other RNA
gacaattgttgatcttgggcctgttccactgttaacataacttttttctgcttctgtcctctataactgtatactgcctctgtcagtatagtgaaatcaacaactcttagtactgcgtggactaatacatcaggttgaaggtgctccaattctacaaagtctatactgttcaccctctgaggctgcctcggaggaagatctctgaggtaggaatgttttgaggacacatatgccagtaagtcttgaagtacaacttcactaactacactggaatattcttcaggctgaatagatgaataactcccaagatttaataactgactgctaaatgttgattgtagtactgtctcgccaatccattggtcctcatgaataacaacattaaaaaacagtggttccccactgcctagccaggaagagctagtacagcattcaagacttttcatgatccaacattcaggatgcatgttcttcagaaaaaaggaacagacgagaaatttcaaggagagcattctgaaagctaggactgtgagtaaaattatatctccaagaaacactgtaaatgcccaaaatgctgcagtcctccacagaaaaaccttcttcttagtttctgattgatcaattactgtaactgttgctaaaggcactttagagccagaatttggtccgaattttatgtttatttccttcacatggcatggagatagcaccatgactaaacaattatacttctggcttttagaatcacagttttttattaatgatgtttttttaatactcttaaattcagacacatttctccgatccatttctacagcagaatctcctccattagaaatcaacttcattttcttagctacttgaaggactctagatagagcttcagactggcccactttatcttcagaggtacagcttcttttaatagcacttttgtggaaggtatttagttgggaacacagtattcctgagctacacaactcaatacgtatctcatttggtggcagttcatcttcagaactgaaaagttcttgagatcctgtatgttcttcaagacctttatcagagtttatgtgaatgcggctattttctgttttaggacaaacaggactaaaaagttcaagggaatatgcttggttttgtccactttcatatgcttctgtaaaaccatcaagctgaatcgaattctcttcaggtattcttatctccccgtaacttgcctttggttcagtctccatgtttacattccctttatttacaggactccgccttttatctttcttttgagctaaaaaagcaacctggctggaggtaattatactgagaaattctgtatcagttgatattttaaggtctgagaccttcctaactgctgcttcagaccttgacttatctactgcgttcgaggaaaataatcccaaacactggttttgtatttcatgatattctgttggcacacactctctttgtaccacttcaggccctatattaattttttcagtactacaaaccaaatccaacacagctgcacatttatggcccaactgaaacaaatttgtgttaaagttcttaccacatatatctggctgatgtttaggctgttcatctctaattttattttcactgagaagcttttgatacttttcttcttcggtgaaatgcggaactgtgcttttaaatccacatatttgcatattagagctagttatatcactcagtctagaggagtgaatcttctgggattctatattctgtgtttcagaaacagaacgtacaaagtcatctttcacatgaacatgtctattcatacagtttgctaagaaatgaccactaagatctggagaaccaatagattctgggactttatagttttcaagatttttgtgctgtttttcatccttcagatataaagaatgttgactgtataaaagctgaatttttttccaggggtcagcaacagacattaaagaagctgtgtcttctgatactgtgattttcagtggagcaattggagcaccccaaaaaatgtggacttgagatcctccactcatgatttctgtaatcccagctactcagga

SEQ ID NO: 12527 - RNA, 2423 nt, Homo sapiens
  source 1..2423: mol_type = other RNA
gacaattgttgatcttgggcctgttccactgttaacataacttttttctgcttctgtcctctataactgtatactgcctctgtcagtatagtgaaatcaacaactcttagtactgcgtggactaatacatcaggttgaaggtgctccaattctacaaagtctatactgttcaccctctgaggctgcctcggaggaagatctctgaggtaggaatgttttgaggacacatatgccagtaagtcttgaagtacaacttcactaactacactggaatattcttcaggctgaatagatgaataactcccaagatttaataactgactgctaaatgttgattgtagtactgtctcgccaatccattggtcctcatgaataacaacattaaaaaacagtggttccccactgcctagccaggaagagctagtacagcattcaagacttttcatgatccaacattcaggatgcatgttcttcagaaaaaaggaacagacgagaaatttcaaggagagcattctgaaagctaggactgtgagtaaaattatatctccaagaaacactgtaaatgcccaaaatgctgcagtcctccacagaaaaaccttcttcttagtttctgattgatcaattactgtaactgttgctaaaggcactttagagccagaatttggtccgaattttatgtttatttccttcacatggcatggagatagcaccatgactaaacaattatacttctggcttttagaatcacagttttttattaatgatgtttttttaatactcttaaattcagacacatttctccgatccatttctacagcagaatctcctccattagaaatcaacttcattttcttagctacttgaaggactctagatagagcttcagactggcccactttatcttcagaggtacagcttcttttaatagcacttttgtggaaggtatttagttgggaacacagtattcctgagctacacaactcaatacgtatctcatttggtggcagttcatcttcagaactgaaaagttcttgagatcctgtatgttcttcaagacctttatcagagtttatgtgaatgcggctattttctgttttaggacaaacaggactaaaaagttcaagggaatatgcttggttttgtccactttcatatgcttctgtaaaaccatcaagctgaatcgaattctcttcaggtattcttatctccccgtaacttgcctttggttcagtctccatgtttacattccctttatttacaggactccgccttttatctttcttttgagctaaaaaagcaacctggctggaggtaattatactgagaaattctgtatcagttgatattttaaggtctgagaccttcctaactgctgcttcagaccttgacttatctactgcgttcgaggaaaataatcccaaacactggttttgtatttcatgatattctgttggcacacactctctttgtaccacttcaggccctatattaattttttcagtactacaaaccaaatccaacacagctgcacatttatggcccaactgaaacaaatttgtgttaaagttcttaccacatatatctggctgatgtttaggctgttcatctctaattttattttcactgagaagcttttgatacttttcttcttcggtgaaatgcggaactgtgcttttaaatccacatatttgcatattagagctagttatatcactcagtctagaggagtgaatcttctgggattctatattctgtgtttcagaaacagaacgtacaaagtcatctttcacatgaacatgtctattcatacagtttgctaagaaatgaccactaagatctggagaaccaatagattctgggactttatagttttcaagatttttgtgctgtttttcatccttcagatataaagaatgttgactgtataaaagctgaatttttttccaggggtcagcaacagacattaaagaagctgtgtcttctgatactgtgattttcagtggagcaattggagcaccccaaaaaatgtggacttgagatcctccactcatgatttcttaatcttttgaccatcaaggaaaattcaggattcaggtcagagtacatttttcactcccctccgcttgtggccatgtaccgctacctgggcgaagcgctgttgctgtcccgggccgggcccgctgccctgggctcggcgtccgccgactcggccgcgttgctgggctgggcccggggacagcccgccgccgccccgcagccggggctggcattggccgcccggcgccactacagcgaggcggtggccgaccgcgaggacgaccccaacttcttcaagatggtggagggcttcttcgatcgcggcgccagcatcgtggaggacaagctggtggaggacctgaggacccgggagagcgaggagcaga

SEQ ID NO: 12528 - RNA, 2155 nt, Homo sapiens
  source 1..2155: mol_type = other RNA
gacaattgttgatcttgggcctgttccactgttaacataacttttttctgcttctgtcctctataactgtatactgcctctgtcagtatagtgaaatcaacaactcttagtactgcgtggactaatacatcaggttgaaggtgctccaattctacaaagtctatactgttcaccctctgaggctgcctcggaggaagatctctgaggtaggaatgttttgaggacacatatgccagtaagtcttgaagtacaacttcactaactacactggaatattcttcaggctgaatagatgaataactcccaagatttaataactgactgctaaatgttgattgtagtactgtctcgccaatccattggtcctcatgaataacaacattaaaaaacagtggttccccactgcctagccaggaagagctagtacagcattcaagacttttcatgatccaacattcaggatgcatgttcttcagaaaaaaggaacagacgagaaatttcaaggagagcattctgaaagctaggactgtgagtaaaattatatctccaagaaacactgtaaatgcccaaaatgctgcagtcctccacagaaaaaccttcttcttagtttctgattgatcaattactgtaactgttgctaaaggcactttagagccagaatttggtccgaattttatgtttatttccttcacatggcatggagatagcaccatgactaaacaattatacttctggcttttagaatcacagttttttattaatgatgtttttttaatactcttaaattcagacacatttctccgatccatttctacagcagaatctcctccattagaaatcaacttcattttcttagctacttgaaggactctagatagagcttcagactggcccactttatcttcagaggtacagcttcttttaatagcacttttgtggaaggtatttagttgggaacacagtattcctgagctacacaactcaatacgtatctcatttggtggcagttcatcttcagaactgaaaagttcttgagatcctgtatgttcttcaagacctttatcagagtttatgtgaatgcggctattttctgttttaggacaaacaggactaaaaagttcaagggaatatgcttggttttgtccactttcatatgcttctgtaaaaccatcaagctgaatcgaattctcttcaggtattcttatctccccgtaacttgcctttggttcagtctccatgtttacattccctttatttacaggactccgccttttatctttcttttgagctaaaaaagcaacctggctggaggtaattatactgagaaattctgtatcagttgatattttaaggtctgagaccttcctaactgctgcttcagaccttgacttatctactgcgttcgaggaaaataatcccaaacactggttttgtatttcatgatattctgttggcacacactctctttgtaccacttcaggccctatattaattttttcagtactacaaaccaaatccaacacagctgcacatttatggcccaactgaaacaaatttgtgttaaagttcttaccacatatatctggctgatgtttaggctgttcatctctaattttattttcactgagaagcttttgatacttttcttcttcggtgaaatgcggaactgtgcttttaaatccacatatttgcatattagagctagttatatcactcagtctagaggagtgaatcttctgggattctatattctgtgtttcagaaacagaacgtacaaagtcatctttcacatgaacatgtctattcatacagtttgctaagaaatgaccactaagatctggagaaccaatagattctgggactttatagttttcaagatttttgtgctgtttttcatccttcagatataaagaatgttgactgtataaaagctgaatttttttccaggggtcagcaacagacattaaagaagctgtgtcttctgatactgtgattttcagtggagcaattggagcaccccaaaaaatgtggacttgagatcctccactcatgatttcttaatcttttgaccatcaaggaaaattcaggattcaggtcagagtacatttttcactgagagccccgccggaggcgggtgcggcctccgggcaaatcc

SEQ ID NO: 12529 - RNA, 2164 nt, Homo sapiens
  source 1..2164: mol_type = other RNA
gacaattgttgatcttgggcctgttccactgttaacataacttttttctgcttctgtcctctataactgtatactgcctctgtcagtatagtgaaatcaacaactcttagtactgcgtggactaatacatcaggttgaaggtgctccaattctacaaagtctatactgttcaccctctgaggctgcctcggaggaagatctctgaggtaggaatgttttgaggacacatatgccagtaagtcttgaagtacaacttcactaactacactggaatattcttcaggctgaatagatgaataactcccaagatttaataactgactgctaaatgttgattgtagtactgtctcgccaatccattggtcctcatgaataacaacattaaaaaacagtggttccccactgcctagccaggaagagctagtacagcattcaagacttttcatgatccaacattcaggatgcatgttcttcagaaaaaaggaacagacgagaaatttcaaggagagcattctgaaagctaggactgtgagtaaaattatatctccaagaaacactgtaaatgcccaaaatgctgcagtcctccacagaaaaaccttcttcttagtttctgattgatcaattactgtaactgttgctaaaggcactttagagccagaatttggtccgaattttatgtttatttccttcacatggcatggagatagcaccatgactaaacaattatacttctggcttttagaatcacagttttttattaatgatgtttttttaatactcttaaattcagacacatttctccgatccatttctacagcagaatctcctccattagaaatcaacttcattttcttagctacttgaaggactctagatagagcttcagactggcccactttatcttcagaggtacagcttcttttaatagcacttttgtggaaggtatttagttgggaacacagtattcctgagctacacaactcaatacgtatctcatttggtggcagttcatcttcagaactgaaaagttcttgagatcctgtatgttcttcaagacctttatcagagtttatgtgaatgcggctattttctgttttaggacaaacaggactaaaaagttcaagggaatatgcttggttttgtccactttcatatgcttctgtaaaaccatcaagctgaatcgaattctcttcaggtattcttatctccccgtaacttgcctttggttcagtctccatgtttacattccctttatttacaggactccgccttttatctttcttttgagctaaaaaagcaacctggctggaggtaattatactgagaaattctgtatcagttgatattttaaggtctgagaccttcctaactgctgcttcagaccttgacttatctactgcgttcgaggaaaataatcccaaacactggttttgtatttcatgatattctgttggcacacactctctttgtaccacttcaggccctatattaattttttcagtactacaaaccaaatccaacacagctgcacatttatggcccaactgaaacaaatttgtgttaaagttcttaccacatatatctggctgatgtttaggctgttcatctctaattttattttcactgagaagcttttgatacttttcttcttcggtgaaatgcggaactgtgcttttaaatccacatatttgcatattagagctagttatatcactcagtctagaggagtgaatcttctgggattctatattctgtgtttcagaaacagaacgtacaaagtcatctttcacatgaacatgtctattcatacagtttgctaagaaatgaccactaagatctggagaaccaatagattctgggactttatagttttcaagatttttgtgctgtttttcatccttcagatataaagaatgttgactgtataaaagctgaatttttttccaggggtcagcaacagacattaaagaagctgtgtcttctgatactgtgattttcagtggagcaattggagcaccccaaaaaatgtggacttgagatcctccactcatgatttcttaatcttttgaccatcaaggaaaattcaggattcaggtcagagtacatttttcactgagagccccgccggaggcgggtgcggcctccgggcaaatccggccgcccg

SEQ ID NO: 12530 - RNA, 2464 nt, Homo sapiens
  source 1..2464: mol_type = other RNA
gacaattgttgatcttgggcctgttccactgttaacataacttttttctgcttctgtcctctataactgtatactgcctctgtcagtatagtgaaatcaacaactcttagtactgcgtggactaatacatcaggttgaaggtgctccaattctacaaagtctatactgttcaccctctgaggctgcctcggaggaagatctctgaggtaggaatgttttgaggacacatatgccagtaagtcttgaagtacaacttcactaactacactggaatattcttcaggctgaatagatgaataactcccaagatttaataactgactgctaaatgttgattgtagtactgtctcgccaatccattggtcctcatgaataacaacattaaaaaacagtggttccccactgcctagccaggaagagctagtacagcattcaagacttttcatgatccaacattcaggatgcatgttcttcagaaaaaaggaacagacgagaaatttcaaggagagcattctgaaagctaggactgtgagtaaaattatatctccaagaaacactgtaaatgcccaaaatgctgcagtcctccacagaaaaaccttcttcttagtttctgattgatcaattactgtaactgttgctaaaggcactttagagccagaatttggtccgaattttatgtttatttccttcacatggcatggagatagcaccatgactaaacaattatacttctggcttttagaatcacagttttttattaatgatgtttttttaatactcttaaattcagacacatttctccgatccatttctacagcagaatctcctccattagaaatcaacttcattttcttagctacttgaaggactctagatagagcttcagactggcccactttatcttcagaggtacagcttcttttaatagcacttttgtggaaggtatttagttgggaacacagtattcctgagctacacaactcaatacgtatctcatttggtggcagttcatcttcagaactgaaaagttcttgagatcctgtatgttcttcaagacctttatcagagtttatgtgaatgcggctattttctgttttaggacaaacaggactaaaaagttcaagggaatatgcttggttttgtccactttcatatgcttctgtaaaaccatcaagctgaatcgaattctcttcaggtattcttatctccccgtaacttgcctttggttcagtctccatgtttacattccctttatttacaggactccgccttttatctttcttttgagctaaaaaagcaacctggctggaggtaattatactgagaaattctgtatcagttgatattttaaggtctgagaccttcctaactgctgcttcagaccttgacttatctactgcgttcgaggaaaataatcccaaacactggttttgtatttcatgatattctgttggcacacactctctttgtaccacttcaggccctatattaattttttcagtactacaaaccaaatccaacacagctgcacatttatggcccaactgaaacaaatttgtgttaaagttcttaccacatatatctggctgatgtttaggctgttcatctctaattttattttcactgagaagcttttgatacttttcttcttcggtgaaatgcggaactgtgcttttaaatccacatatttgcatattagagctagttatatcactcagtctagaggagtgaatcttctgggattctatattctgtgtttcagaaacagaacgtacaaagtcatctttcacatgaacatgtctattcatacagtttgctaagaaatgaccactaagatctggagaaccaatagattctgggactttatagttttcaagatttttgtgctgtttttcatccttcagatataaagaatgttgactgtataaaagctgaatttttttccaggggtcagcaacagacattaaagaagctgtgtcttctgatactgtgattttcagtggagcaattggagcaccccaaaaaatgtggacttgagatcctccactcatgatttcttcgtccacagaatcctcaaaaggctcaggaactggtaacagatagcgcttgcacgacatcataactccagccaaatgcatgacactgacggcagaaatccttgggtttctgtgcttctgctccctggtctgtcaagtgggtgtaataaccacagcattcctctcttaggactgttgtaaagctgtgatcccagctacttgggaggctgaggtggaagaatcgcttgaacctaggaggcggaggatgcagtgagccgagatcacaccactgtactccagtctggccatcaggacgagacttaatcttttgaccatcaaggaaaattcaggattcaggtcagagtacatttttcactgagagccccgccggaggcgggtgcggcctccgggcaaatccggccgcccgt

SEQ ID NO: 12531 - RNA, 2078 nt, Homo sapiens
  source 1..2078: mol_type = other RNA
gacaattgttgatcttgggcctgttccactgttaacataacttttttctgcttctgtcctctataactgtatactgcctctgtcagtatagtgaaatcaacaactcttagtactgcgtggactaatacatcaggttgaaggtgctccaattctacaaagtctatactgttcaccctctgaggctgcctcggaggaagatctctgaggtaggaatgttttgaggacacatatgccagtaagtcttgaagtacaacttcactaactacactggaatattcttcaggctgaatagatgaataactcccaagatttaataactgactgctaaatgttgattgtagtactgtctcgccaatccattggtcctcatgaataacaacattaaaaaacagtggttccccactgcctagccaggaagagctagtacagcattcaagacttttcatgatccaacattcaggatgcatgttcttcagaaaaaaggaacagacgagaaatttcaaggagagcattctgaaagctaggactgtgagtaaaattatatctccaagaaacactgtaaatgcccaaaatgctgcagtcctccacagaaaaaccttcttcttagtttctgattgatcaattactgtaactgttgctaaaggcactttagagccagaatttggtccgaattttatgtttatttccttcacatggcatggagatagcaccatgactaaacaattatacttctggcttttagaatcacagttttttattaatgatgtttttttaatactcttaaattcagacacatttctccgatccatttctacagcagaatctcctccattagaaatcaacttcattttcttagctacttgaaggactctagatagagcttcagactggcccactttatcttcagaggtacagcttcttttaatagcacttttgtggaaggtatttagttgggaacacagtattcctgagctacacaactcaatacgtatctcatttggtggcagttcatcttcagaactgaaaagttcttgagatcctgtatgttcttcaagacctttatcagagtttatgtgaatgcggctattttctgttttaggacaaacaggactaaaaagttcaagggaatatgcttggttttgtccactttcatatgcttctgtaaaaccatcaagctgaatcgaattctcttcaggtattcttatctccccgtaacttgcctttggttcagtctccatgtttacattccctttatttacaggactccgccttttatctttcttttgagctaaaaaagcaacctggctggaggtaattatactgagaaattctgtatcagttgatattttaaggtctgagaccttcctaactgctgcttcagaccttgacttatctactgcgttcgaggaaaataatcccaaacactggttttgtatttcatgatattctgttggcacacactctctttgtaccacttcaggccctatattaattttttcagtactacaaaccaaatccaacacagctgcacatttatggcccaactgaaacaaatttgtgttaaagttcttaccacatatatctggctgatgtttaggctgttcatctctaattttattttcactgagaagcttttgatacttttcttcttcggtgaaatgcggaactgtgcttttaaatccacatatttgcatattagagctagttatatcactcagtctagaggagtgaatcttctgggattctatattctgtgtttcagaaacagaacgtacaaagtcatctttcacatgaacatgtctattcatacagtttgctaagaaatgaccactaagatctggagaaccaatagattctgggactttatagttttcaagatttttgtgctgtttttcatccttcagatataaagaatgttgactgtataaaagctgaatttttttccaggggtcagcaacagacattaaagaagctgtgtcttctgatactgtgattttcagtggagcaattggagcaccccaaaaaatgtggacttgagatcctccactcatgattttttaggccgggcgcagtggctc

SEQ ID NO: 12532 - RNA, 1847 nt, Homo sapiens
  source 1..1847: mol_type = other RNA
gacaattgttgatcttgggcctgttccactgttaacataacttttttctgcttctgtcctctataactgtatactgcctctgtcagtatagtgaaatcaacaactcttagtactgcgtggactaatacatcaggttgaaggtgctccaattctacaaagtctatactgttcaccctctgaggctgcctcggaggaagatctctgaggtaggaatgttttgaggacacatatgccagtaagtcttgaagtacaacttcactaactacactggaatctgtgagtaaaattatatctccaagaaacactgtaaatgcccaaaatgctgcagtcctccacagaaaaaccttcttcttagtttctgattgatcaattactgtaactgttgctaaaggcactttagagccagaatttggtccgaattttatgtttatttccttcacatggcatggagatagcaccatgactaaacaattatacttctggcttttagaatcacagttttttattaatgatgtttttttaatactcttaaattcagacacatttctccgatccatttctacagcagaatctcctccattagaaatcaacttcattttcttagctacttgaaggactctagatagagcttcagactggcccactttatcttcagaggtacagcttcttttaatagcacttttgtggaaggtatttagttgggaacacagtattcctgagctacacaactcaatacgtatctcatttggtggcagttcatcttcagaactgaaaagttcttgagatcctgtatgttcttcaagacctttatcagagtttatgtgaatgcggctattttctgttttaggacaaacaggactaaaaagttcaagggaatatgcttggttttgtccactttcatatgcttctgtaaaaccatcaagctgaatcgaattctcttcaggtattcttatctccccgtaacttgcctttggttcagtctccatgtttacattccctttatttacaggactccgccttttatctttcttttgagctaaaaaagcaacctggctggaggtaattatactgagaaattctgtatcagttgatattttaaggtctgagaccttcctaactgctgcttcagaccttgacttatctactgcgttcgaggaaaataatcccaaacactggttttgtatttcatgatattctgttggcacacactctctttgtaccacttcaggccctatattaattttttcagtactacaaaccaaatccaacacagctgcacatttatggcccaactgaaacaaatttgtgttaaagttcttaccacatatatctggctgatgtttaggctgttcatctctaattttattttcactgagaagcttttgatacttttcttcttcggtgaaatgcggaactgtgcttttaaatccacatatttgcatattagagctagttatatcactcagtctagaggagtgaatcttctgggattctatattctgtgtttcagaaacagaacgtacaaagtcatctttcacatgaacatgtctattcatacagtttgctaagaaatgaccactaagatctggagaaccaatagattctgggactttatagttttcaagatttttgtgctgtttttcatccttcagatataaagaatgttgactgtataaaagctgaatttttttccaggggtcagcaacagacattaaagaagctgtgtcttctgatactgtgattttcagtggagcaattggagcaccccaaaaaatgtggacttgagatcctccactcatgatttctgagagccccgccggaggcgggtgcggcctccgggcaaatcc

SEQ ID NO: 12533 - RNA, 1903 nt, Homo sapiens
  source 1..1903: mol_type = other RNA
gacaattgttgatcttgggcctgttccactgttaacataacttttttctgcttctgtcctctataactgtatactgcctctgtcagtatagtgaaatcaacaactcttagtactgcgtggactaatacatcaggttgaaggtgctccaattctacaaagtctatactgttcaccctctgaggctgcctcggaggaagatctctgaggtaggaatgttttgaggacacatatgccagtaagtcttgaagtacaacttcactaactacactggaatctgtgagtaaaattatatctccaagaaacactgtaaatgcccaaaatgctgcagtcctccacagaaaaaccttcttcttagtttctgattgatcaattactgtaactgttgctaaaggcactttagagccagaatttggtccgaattttatgtttatttccttcacatggcatggagatagcaccatgactaaacaattatacttctggcttttagaatcacagttttttattaatgatgtttttttaatactcttaaattcagacacatttctccgatccatttctacagcagaatctcctccattagaaatcaacttcattttcttagctacttgaaggactctagatagagcttcagactggcccactttatcttcagaggtacagcttcttttaatagcacttttgtggaaggtatttagttgggaacacagtattcctgagctacacaactcaatacgtatctcatttggtggcagttcatcttcagaactgaaaagttcttgagatcctgtatgttcttcaagacctttatcagagtttatgtgaatgcggctattttctgttttaggacaaacaggactaaaaagttcaagggaatatgcttggttttgtccactttcatatgcttctgtaaaaccatcaagctgaatcgaattctcttcaggtattcttatctccccgtaacttgcctttggttcagtctccatgtttacattccctttatttacaggactccgccttttatctttcttttgagctaaaaaagcaacctggctggaggtaattatactgagaaattctgtatcagttgatattttaaggtctgagaccttcctaactgctgcttcagaccttgacttatctactgcgttcgaggaaaataatcccaaacactggttttgtatttcatgatattctgttggcacacactctctttgtaccacttcaggccctatattaattttttcagtactacaaaccaaatccaacacagctgcacatttatggcccaactgaaacaaatttgtgttaaagttcttaccacatatatctggctgatgtttaggctgttcatctctaattttattttcactgagaagcttttgatacttttcttcttcggtgaaatgcggaactgtgcttttaaatccacatatttgcatattagagctagttatatcactcagtctagaggagtgaatcttctgggattctatattctgtgtttcagaaacagaacgtacaaagtcatctttcacatgaacatgtctattcatacagtttgctaagaaatgaccactaagatctggagaaccaatagattctgggactttatagttttcaagatttttgtgctgtttttcatccttcagatataaagaatgttgactgtataaaagctgaatttttttccaggggtcagcaacagacattaaagaagctgtgtcttctgatactgtgattttcagtggagcaattggagcaccccaaaaaatgtggacttgagatcctccactcatgatttcttaatcttttgaccatcaaggaaaattcaggattcaggtcagagtacatttttcactgagagccccgccggaggcgggtgcggcctccgggcaaatcc

SEQ ID NO: 12534 - RNA, 3667 nt, Homo sapiens
  source 1..3667: mol_type = other RNA
gacctggacatgtttgtgcccagtccctggatctgtggcctggacactaattcctcacactggtctctgagtgggctgctctggatttcaaattcaaggggtgatgcaagatcgaagagcaggggaagccttgtgaacagaggccatcggcaagtggcacagttagagaccgagcctcaccacgagcttcggagagctgtcagcccaggagcctgagctcatgagagaaagcacctgcatgtctcctgtggagcacagaggtgcgcagagtcctggagggaaggccgtgtgcaggtgctgggttcccagcatccgttcaactctgggcagggtcagagacattcctgaagacacagtcttccaggagacaaagagcaggaagtaccttcagaaaccccatcagcaacgttcctgtcacataaagaggacgttacccaaccaagctctgtggctacggccatcttggtggacaggtgcggcgataaagctgtattctgtcccctacagcagatccggagagtctctggctaaaacagtctgcgtggtaagatggtggactcctgacccggctctgccatctgctacctgtgtgaacttcgggaaattatgtagtctcttggacctcagttgccccatccaacctcagagattgatttgctgttcttcacagccagggcgagatacttccctccttcacttgttattttgttttttcccagtttaagatgcgtgaggcctttgcattcatccaggattttggtgacgtacctggctccgacatcggtgatctggttgttgtataaacccaaataggtcacaattttgtatttggtcagctcttcgcttagcacctttaccccaccgtcagtgatctggtttacgctgagtctgagaacagtgaggcggctgaagcagggctgcagctcccgcacgccgtagtcgttgagattgttgttgtctaggtctagggccagccgcttggggaagtgatgcaggacgaaggagagggcgctgcagtcggccgagcaggcgttgcagtaggtcagcttgaggtagttggcgcagatgcccctggccgccagctgccccaccttctggctctgtgtctcgtagatgcagcgcagcatccagatgaacgtgggcatggcctgcacctggttgaagctttcgacctgaacgcggggcaggctcttcaggtagccccgcaggctggaaaacaggtgtgcccacagggccttgcgctttctcctcagggctgccgcgggcaccagatgccgcaggagtttctgtttggctttggacaacagcccgcacaggaagaggttggtgaactggaagtgatccttgttcttgaagaggtcttcccgcgccggaccactgccctgcaggcactggaacgggaggaagggaggatagcaggacgtggtcgctgcccccgcagggggcatccactcctggaagaacctgagcagctcctgagtgcccaccctgtcgtccagcacgaggaagaaggctgtaaagaaggcctggagggtgaggtggaaaaactcataggactgctggtcacccccggggcccagctccggcaaagcccgcaggaagcccagctgcatgtctctctcctgcagcccggaggcctgcacctcctcctgggtgaagacaaagaggctcttctccatgccccggtgggccacctgccccagcgagcacagagtgtcccggccggcgtggagggtctccactgggctgcgtgtgttccgctgcaccaggctgctgggctgcatcctgttcagatggacctcagtgaccaggaggaagacatctgtcagggtcatcgtgcagtcgggcagctgtggtgagccttcaaaggcagcacggaagtgctggaagcaccggaagatgatccagcagaagaggggcacagagcacaggctgcagaggttggggttggcctccagctggctcagcaggcggtcctgcagggcccgctcggggaacatcctcctggcataggcgcgcaggtggctgggggagaagccccggagaagcaccttcttccgcaggaactggcgcgggacctcgatgcctgtgcgggctgtgagcagcttgctagcccccttgagcagcttcccactgagcaggttggccagcaagaccagggggtgggcaggctcccaggggcaggagctgtcaggcacgcggctcaggtccaagtccgagtgcagctcgtccaggccatcgaaggtgaagagggccacgtgggggaagcgcagcaggaaggcaaacacctcctcggggtcccgctctgggtagcagtagtgcttgaagagcaggtcctgcagacacagcctgtcactttccttgaagcagctgaacatgcggcagcgaaagtggaagaagaatttgacccctgcgtctagccggcccgtggcccagaggctctgcagccgctgtagcagcatggacttgcccaccccagcatcacccaggatgaagatggtctcaccctgctcattgaggatgccggtggtgtggtccaggaggcaggccaggctgttcaggctgcccaggctctcattgctgaagccaaccagctccatgatggtgtccatgtagatctcctccagcagcagctcctccttctgggcatagcacagcacgaacttggagtcacggcccagatggtgtcgcagctgctgggtatacctgctcactgggtcagtgttgaccacgactttgctctgagtgagcagggaaggggagaagccgatctccagcagccaaggcctgaggtccacgtaggcatctgcgagttgctggagcaagtagaggaagaactcggacacctcctcgcccttgctctgtaccaggtccagaattttgcggaccttgtcaggctgggtggggcaggcacacacaatctccgcatcttcggccgagaagtagtcattcttcagcaagttgtccaccagacactgagtattgcggatgtgagtgaccagaagttcccgattgcttttcagtaattgaatgtgggggtgagactctgatgggattatttccatctcactgtggccctgctcttccatagttaaagtagcaagcggctacttttcccaaattcatcttcagctgcgtgtgtcctctcagcagaagggcaatcaggattcaggccgcgccctccagggcccctgctactctgcgcagcccctttttaagtttctggcatcattctttgaagttagaatattttaaaacaacattgtttaaatcttcaatttccaatttatttctggaattgcttctgtctcttccaagcctgcgattcccataaaaacagcaacttgtcttcccagatgttttctgtaatcgccgccacaatctccacctcttgccatcaaaggcagaaaccgaaggaaagtctcctgacttacaatcactcagtgtcactttcaccgcaggcttctttctttccttgcactgtcccaggggaccttgagcggagatgtgcatttcttataactgagatgttggccaccaggtttacagacttcgcagccgctgagagctagagaagagcccggagagcgccatggtccggggacgccggggccgggaagcgccgtggcccgggaggacgctgctcccgcagtagcgcgagggaggg

SEQ ID NO: 12535 - RNA, 34 nt, Homo sapiens
  source 1..34: mol_type = other RNA
gactatagaactttccccctcatccctctaccct

SEQ ID NO: 12536 - RNA, 26 nt, Homo sapiens
  source 1..26: mol_type = other RNA
gagacaggttcatgctgctatcgttc

SEQ ID NO: 12537 - RNA, 4096 nt, Homo sapiens
  source 1..4096: mol_type = other RNA
gagagatcagaggcgcagagtggccccactcttgtccacctccatcacccgccccgattcccatagccccagcagatctccgagggaccagtgggagggcccaggccttctccgccaggcaccctgccctgaggcagccaccaggctcctccgggtcccctgctgggcaaagctgacctcttgttggcccctgcagccggcccggggtccctgcagggaggctagcgtgggcaggacagaggctctggatgctctggaggtctgggtgcccctgcagcagcggcagcggcctcatgagacgcagtgagacctgcctgcagcgtggccccaccttcctgggggttcctggcccgggtgggttggggctgcccctggcaccacgtcacaggccggccttgtcgctgtagaagggcgtgacatggaacatgtagcagtgggtgcacactcggaccggcttcacctgcccgtagcggggcagcggtgctgagtgcgaggagcagcgcgagcagaagatctggaatggggttggggcagtgagggtctgcggcagaccagccccacccaccctggctcctcgccctcccacacacctacccacccagctcaggccgcattggtgggtggggactgcccagccccagctgccaggggttgtgaccttcaggaggctggactctatgaggggtccacgtcctgcaccaaggctgctgcaggctcctgttcacactcgctgtcccctctctgtggctggctctgcagcagccgggactggacatgggcaccatccaggttcccgtggtcaaatgcctggagtcagaacagggcccgggacctccaggggcctctgcacaagaccccacaggcctcgctggcctccctgggcatcggttctgacttccagacctcaggctctgtccgtggacgcccttggatgctgagggaccctccgtgcaaggggtctcacccaccttcccacagctgcggcagtggtgcttccggcggatgacggtgaagggtgctttgcacgccgtgcagaagccacaggcctcgtctggcacccactccggggggtcttcaaagtccccatcgcgggtcttggctgccagttcagaggatgacagggtctcctggcacagtgcacagtcctccaaggccgcactccgcagagtctgggtgactgccgtctctgaatcatgatttccagaaggcagtcctgccaacctccctggtagaatgcagcctggcggtgtggattcggcagggcagagctgggtcggcacatgggctcctccctgctggcaagggtatgccctgctgggccagggctccaggaccaggcgggctgccccatgtgcccggacgccccatgaacagaagcctctgtggtgagggatggctccttccttaacttttccttgtcgtctgtttcaggcttggtggccatgacctcaaacagtgttttaagaatacttctcaggtcactggcatagttcgtctgcagctggtcagccacacctgaaatgcagacgaacaggcggtggatgaggtcgtggctgccgtggaacctggaccggatcttctctcttgtggcctgtggggcagcatgcgtggctgctggggccgcctctggccccatcttgtctgaggagcaggacccagctgtggagctgctggagcccgacagggcctgaggcgcctcgtgagccgaggggctcccagcatgcagctctctggcctctggctcctgctgacctgcaaccccagcctctccttgcagcccactcgctgtgtccacctgggaacctgaggtgtgaggcaggcacttgtcggaagtgggggctttgggctcccgcccgttggaggcatcttctgagggtgggggcgcctcctcctgtctctcaggggccctgtcgctggccttggctaagccggcagcgtacgaggcaccaatgacgcctcccgggctgcacttctcccgcagacgctccaccacgtcctccctgctgtccccgcagctcccacagcacacgcaggaatgcagaaggcagttggtggccccagtgctaagcttgtgggggccgccatccatcccctcggccacgggctccgaggcggcctcctgggtggcgaccgcagagtccagggaagtgggcgatttggggttgaagatgaccgtggctgagagcttcatgccccctgtccggtgggcgatcatctcagccgtctctgcgtcatccgcacccacctcccagccgtccaggtgcagccgcgagtccaggcagctgcaggagctggtgcccgcgaggctggccccatctgtgccctcggcctcgagattgttgttgctcaagtcctcctccttttccgaggcgggcaagctgatccccgccgctccgcctggcccaccctgccctttctcctgggggtcggcccaggtactgcctgcccacccaaatgggccagctggggactcgggcctggccagggcttctgccgtcccctccacgtcatccatgaagaacacgcgctcctcctcgtcactgcctgaccgcaggcgcggtctacctggagaggcctccccgcctgggctgccctccgctcctggcctgtgagctggggactggcaggcaatgggcggtgaaagcaaagaggacatctcgtcccccgccctgtggaccatgcggctgagctgctccagctcctggtcgtcgtactgcatggagcaggccagctctgcatccgggtctttggccttagctgagagtggcccctcaggggggagaggggcagagagggcaggcgccagggcagcgggtccctgcacgtctgcgcggatggggaactccacgtcttgggaaatgcagaggttccgttccagcgtgtgcagctcctcctccgtcagcgtctgcagcaaatcccttattttccgcagcaacgtgtggaagggccggaacagctcggacatgtcttccaccttgcggtccaagttcagaggtccgtccgcatagaccacgaggccacacacgatggccagcctggggatgctgaacatgagggccggctcgtagtcatcaatcatgtcctgagtcaggtacccgaagtccagggccctctccaccgtctcgcagaagagcacgatgacctcctgctgcacgtagtactccctgggggacttcacaggcaccatggccgagacgtagctgagctcaaactctgcgaacaggacgtcgaagtgcctcagcgcttccctcatcttctctgtgtaggtgttcaggtcccgcagcgcctggtcacggagggcgccccgcacgtcctccaggctgcgcgtcagctccttggccagcgggcgcatggccatgctctccagctcccggttcatgatgatggagccggcggccaggcactcggcaccgaaccacagctggccggccaggttgtcgtgccggatctcctcagggaacttgacgcagaaatctctgggggcgcggtcctgggggatgcactcatccatgatctggttaatgatgttcaacacattgtcctgacaggagcggaactggctgaccagcagcgtgcaccgctgggggtccttccgcccatccaggctgtccagctccgcggccacctggttcagctcctcgtcggcatagtagaaccgggcaagcagctgcggatccgacctcttgggtttgtagagccactttcggaacctgttcatcatcgccgcgccggccctggccggactccgggcggccctcgccctccgcagcgctgcgcccgggcccggctgaggcgcggggcggacgcggaggcacggccggagcccccgcgctgtcgcagggaggctggctagcgaagcccggagcgccgagcgggcggcgggcaggtgcgcggggcaggtgcgcggccctgagtatgctctgcaagcggcgcgccgggcagacctcagacccgggagtgggcgctcgggcgcacggacagacgcgggcacgggggcgcgcggctcctcgctgctcactgacacccagcgctccgctggtcacggccgccccgcgccgcacatgcgcctagggcgccgcgagccccgggcccaccg

SEQ ID NO: 12538 - RNA, 4099 nt, Homo sapiens
  source 1..4099: mol_type = other RNA
gagagatcagaggcgcagagtggccccactcttgtccacctccatcacccgccccgattcccatagccccagcagatctccgagggaccagtgggagggcccaggccttctccgccaggcaccctgccctgaggcagccaccaggctcctccgggtcccctgctgggcaaagctgacctcttgttggcccctgcagccggcccggggtccctgcagggaggctagcgtgggcaggacagaggctctggatgctctggaggtctgggtgcccctgcagcagcggcagcggcctcatgagacgcagtgagacctgcctgcagcgtggccccaccttcctgggggttcctggcccgggtgggttggggctgcccctggcaccacgtcacaggccggccttgtcgctgtagaagggcgtgacatggaacatgtagcagtgggtgcacactcggaccggcttcacctgcccgtagcggggcagcggtgctgagtgcgaggagcagcgcgagcagaagatctggaatggggttggggcagtgagggtctgcggcagaccagccccacccaccctggctcctcgccctcccacacacctacccacccagctcaggccgcattggtgggtggggactgcccagccccagctgccaggggttgtgaccttcaggaggctggactctatgaggggtccacgtcctgcaccaaggctgctgcaggctcctgttcacactcgctgtcccctctctgtggctggctctgcagcagccgggactggacatgggcaccatccaggttcccgtggtcaaatgcctggagtcagaacagggcccgggacctccaggggcctctgcacaagaccccacaggcctcgctggcctccctgggcatcggttctgacttccagacctcaggctctgtccgtggacgcccttggatgctgagggaccctccgtgcaaggggtctcacccaccttcccacagctgcggcagtggtgcttccggcggatgacggtgaagggtgctttgcacgccgtgcagaagccacaggcctcgtctggcacccactccggggggtcttcaaagtccccatcgcgggtcttggctgccagttcagaggatgacagggtctcctggcacagtgcacagtcctccaaggccgcactccgcagagtctgggtgactgccgtctctgaatcatgatttccagaaggcagtcctgccaacctccctggtagaatgcagcctggcggtgtggattcggcagggcagagctgggtcggcacatgggctcctccctgctggcaagggtatgccctgctgggccagggctccaggaccaggcgggctgccccatgtgcccggacgccccatgaacagaagcctctgtggtgagggatggctctgccttccttaacttttccttgtcgtctgtttcaggcttggtggccatgacctcaaacagtgttttaagaatacttctcaggtcactggcatagttcgtctgcagctggtcagccacacctgaaatgcagacgaacaggcggtggatgaggtcgtggctgccgtggaacctggaccggatcttctctcttgtggcctgtggggcagcatgcgtggctgctggggccgcctctggccccatcttgtctgaggagcaggacccagctgtggagctgctggagcccgacagggcctgaggcgcctcgtgagccgaggggctcccagcatgcagctctctggcctctggctcctgctgacctgcaaccccagcctctccttgcagcccactcgctgtgtccacctgggaacctgaggtgtgaggcaggcacttgtcggaagtgggggctttgggctcccgcccgttggaggcatcttctgagggtgggggcgcctcctcctgtctctcaggggccctgtcgctggccttggctaagccggcagcgtacgaggcaccaatgacgcctcccgggctgcacttctcccgcagacgctccaccacgtcctccctgctgtccccgcagctcccacagcacacgcaggaatgcagaaggcagttggtggccccagtgctaagcttgtgggggccgccatccatcccctcggccacgggctccgaggcggcctcctgggtggcgaccgcagagtccagggaagtgggcgatttggggttgaagatgaccgtggctgagagcttcatgccccctgtccggtgggcgatcatctcagccgtctctgcgtcatccgcacccacctcccagccgtccaggtgcagccgcgagtccaggcagctgcaggagctggtgcccgcgaggctggccccatctgtgccctcggcctcgagattgttgttgctcaagtcctcctccttttccgaggcgggcaagctgatccccgccgctccgcctggcccaccctgccctttctcctgggggtcggcccaggtactgcctgcccacccaaatgggccagctggggactcgggcctggccagggcttctgccgtcccctccacgtcatccatgaagaacacgcgctcctcctcgtcactgcctgaccgcaggcgcggtctacctggagaggcctccccgcctgggctgccctccgctcctggcctgtgagctggggactggcaggcaatgggcggtgaaagcaaagaggacatctcgtcccccgccctgtggaccatgcggctgagctgctccagctcctggtcgtcgtactgcatggagcaggccagctctgcatccgggtctttggccttagctgagagtggcccctcaggggggagaggggcagagagggcaggcgccagggcagcgggtccctgcacgtctgcgcggatggggaactccacgtcttgggaaatgcagaggttccgttccagcgtgtgcagctcctcctccgtcagcgtctgcagcaaatcccttattttccgcagcaacgtgtggaagggccggaacagctcggacatgtcttccaccttgcggtccaagttcagaggtccgtccgcatagaccacgaggccacacacgatggccagcctggggatgctgaacatgagggccggctcgtagtcatcaatcatgtcctgagtcaggtacccgaagtccagggccctctccaccgtctcgcagaagagcacgatgacctcctgctgcacgtagtactccctgggggacttcacaggcaccatggccgagacgtagctgagctcaaactctgcgaacaggacgtcgaagtgcctcagcgcttccctcatcttctctgtgtaggtgttcaggtcccgcagcgcctggtcacggagggcgccccgcacgtcctccaggctgcgcgtcagctccttggccagcgggcgcatggccatgctctccagctcccggttcatgatgatggagccggcggccaggcactcggcaccgaaccacagctggccggccaggttgtcgtgccggatctcctcagggaacttgacgcagaaatctctgggggcgcggtcctgggggatgcactcatccatgatctggttaatgatgttcaacacattgtcctgacaggagcggaactggctgaccagcagcgtgcaccgctgggggtccttccgcccatccaggctgtccagctccgcggccacctggttcagctcctcgtcggcatagtagaaccgggcaagcagctgcggatccgacctcttgggtttgtagagccactttcggaacctgttcatcatcgccgcgccggccctggccggactccgggcggccctcgccctccgcagcgctgcgcccgggcccggctgaggcgcggggcggacgcggaggcacggccggagcccccgcgctgtcgcagggaggctggctagcgaagcccggagcgccgagcgggcggcgggcaggtgcgcggggcaggtgcgcggccctgagtatgctctgcaagcggcgcgccgggcagacctcagacccgggagtgggcgctcgggcgcacggacagacgcgggcacgggggcgcgcggctcctcgctgctcactgacacccagcgctccgctggtcacggccgccccgcgccgcacatgcgcctagggcgccgcgagccccgggcccaccg

SEQ ID NO: 12539 - RNA, 5169 nt, Homo sapiens
  source 1..5169: mol_type = other RNA
gagagatcagaggcgcagagtggccccactcttgtccacctccatcacccgccccgattcccatagccccagcagatctccgagggaccagtgggagggcccaggccttctccgccaggcaccctgccctgaggcagccaccaggctcctccgggtcccctgctgggcaaagctgacctcttgttggcccctgcagccggcccggggtccctgcagggaggctagcgtgggcaggacagaggctctggatgctctggaggtctgggtgcccctgcagcagcggcagcggcctcatgagacgcagtgagacctgcctgcagcgtggccccaccttcctgggggttcctggcccgggtgggttggggctgcccctggcaccacgtcacaggccggccttgtcgctgtagaagggcgtgacatggaacatgtagcagtgggtgcacactcggaccggcttcacctgcccgtagcggggcagcggtgctgagtgcgaggagcagcgcgagcagaagatcttcaggaggctggactctatgaggggtccacgtcctgcaccaaggctgctgcaggctcctgttcacactcgctgtcccctctctgtggctggctctgcagcagccgggactggacatgggcaccatccaggttcccgtggtcaaatgcctggagtcagaacagggcccgggacctccaggggcctctgcacaagaccccacaggcctcgctggcctccctgggcatcggttctgacttccagacctcaggctctgtccgtggacgcccttggatgctgagggaccctccgtgcaaggggtctcacccaccttcccacagctgcggcagtggtgcttccggcggatgacggtgaagggtgctttgcacgccgtgcagaagccacaggcctcgtctggcacccactccggggggtcttcaaagtccccatcgcgggtcttggctgccagttcagaggatgacagggtctcctggcacagtgcacagtcctccaaggccgcactccgcagagtctgggtgaccttccttaacttttccttgtcgtctgtttcaggcttggtggccatgacctcaaacagtgttttaagaatacttctcaggtcactggcatagttcgtctgcagctggtcagccacacctgaaatgcagacgaacaggcggtggatgaggtcgtggctgccgtggaacctggaccggatcttctctcttgtggcctgtggggcagcatgcgtggctgctggggccgcctctggccccatcttgtctgaggagcaggacccagctgtggagctgctggagcccgacagggcctgaggcgcctcgtgagccgaggggctcccagcatgcagctctctggcctctggctcctgctgacctgcaaccccagcctctccttgcagcccactcgctgtgtccacctgggaacctgaggtgtgaggcaggcacttgtcggaagtgggggctttgggctcccgcccgttggaggcatcttctgagggtgggggcgcctcctcctgtctctcaggggccctgtcgctggccttggctaagccggcagcgtacgaggcaccaatgacgcctcccgggctgcacttctcccgcagacgctccaccacgtcctccctgctgtccccgcagctcccacagcacacgcaggaatgcagaaggcagttggtggccccagtgctaagcttgtgggggccgccatccatcccctcggccacgggctccgaggcggcctcctgggtggcgaccgcagagtccagggaagtgggcgatttggggttgaagatgaccgtggctgagagcttcatgccccctgtccggtgggcgatcatctcagccgtctctgcgtcatccgcacccacctcccagccgtccaggtgcagccgcgagtccaggcagctgcaggagctggtgcccgcgaggctggccccatctgtgccctcggcctcgagattgttgttgctcaagtcctcctccttttccgaggcgggcaagctgatccccgccgctccgcctggcccaccctgccctttctcctgggggtcggcccaggtactgcctgcccacccaaatgggccagctggggactcgggcctggccagggcttctgccgtcccctccacgtcatccatgaagaacacgcgctcctcctcgtcactgcctgaccgcaggcgcggtctacctggagaggcctccccgcctgggctgccctccgctcctggcctgtgagctggggactggcaggcaatgggcggtgaaagcaaagaggacatctcgtcccccgccctgtggaccatgcggctgagctgctccagctcctggtcgtcgtactgcatggagcaggccagctctgcatccgggtctttggccttagctgagagtggcccctcaggggggagaggggcagagagggcaggcgccagggcagcgggtccctgcacgtctgcgcggatggggaactccacgtcttgggaaatgcagaggttccgttccagcgtgtgcagctcctcctccgtcagcgtctgcagcaaatcccttattttccgcagcaacgtgtggaagggccggaacagctcggacatgtcttccaccttgcggtccaagttcagaggtccgtccgcatagaccacgaggccacacacgatggccagcctggggatgctgaacatgagggccggctcgtagtcatcaatcatgtcctgagtcaggtacccgaagtccagggccctctccaccgtctcgcagaagagcacgatgacctcctgctgcacgtagtactccctgggggacttcacaggcaccatggccgagacgtagctgagctcaaactctgcgaacaggacgtcgaagtgcctcagcgcttccctcatcttctctgtgtaggtgttcaggtcccgcagcgcctggtcacggagggcgccccgcacgtcctccaggctgcgcgtcagctccttggccagcgggcgcatggccatgctctccagctcccggttcatgatgatggagccggcggccaggcacccacagcacaggccagctcgtgttcccggtccccgcaggaggtttttcttacattcagagcaatcgtgagggcgataaccgatgtcccccaatgtgacccacggggtcctcacagggccccaggagcagggagggcagggcatggcagggcaggtaagggcaggggaggggagggcaggggaggggaggggaggggaaggtggactgaggcccttgggtctgggggctccctgcaggaggaaccctggtcatgtgactcttttccgctccccgtccaggccacagggatgaagttcaaggagcttggagcttccaggctccacaatcaggtctgtgctcccagggatgaagcagccgggctgatccgggcccgaggtccccagcctatctagggagccacagacaccacctgtcaagttgctcactgccagagaaacgcaaccttccccggaacgcagactcatcagtgtgagagtccctgggctcctgggcaggtaaggagggctcctccgcacccacaaatccacccatgtctgccctgggtgctgcgaggcagctccccagcgtgcgctcagcaactgggaatttcaccaagctgccctctggcacaggggctgagtccaggccctggtagacctgttgtcacagggaggcttgtctagaggccggggcctcgccaggtttaggatagaaccaatccacctgctgtcccctcagggatgatcaagtgatgcaggacaagaagccatttcccaggtgacagaatgagacggcgctgatcgcccaggcccaagctgcaggtgggcacagagcttggggcaccaggaccacacaaggagctgtgcccacccctgtgcatgcatgcccctgccaggccagccgggcacagaacacgctccatctcatgactgccccaggacccactccacggaggtggaaactgaggctggggaggagggagaacctgcccgcgggcccctgtaactaacccaagcctcggcagaggacaccccaaccaggtggctcagaaggtggggtgggcagggtggacacagggacggggcagcgtgggatgaagactccgcaccccagggattcctagaaaggggaggcgggcaggatggggacggcacaatagagagggtggcggtgtcggggctgaggtcaggctcgggagcacggcaaggggaggaggctggggagtccgcatggtgggggcctgggggagactgttcccgccaccttgaagggcaccttcctctcggtgcctcagtttcctgattgggagatgaagatgaagatgacaggctattgccacatgtggcctgcgtggggctgcagcacggctccccagcccctgctgctgcccatgctgcagggccggaggggaacacttgttcctgatgtgggcattactgccattaaaaaccacttttaggtcctggctgtctgggggcctgtgaacctcataaaaaccacatgggaaatttcatttgtatgtatagttttgggggcaccagttcatggctttcccagatcctccaggggtgcacggcctaccaggctcagaccacaccacgtaacccagagtggacggagctcttggaggagacaccaggtcccggcacctgcaggcgcccatgcacaaggttcgcagggacttggctagacgccaccccacatcaggacctccgaacccgggtggccacccgctacctcggcaccgaaccacagctggccggccaggttgtcgtgccggatctcctcagggaacttgacgcagaaatctctgggggcgcggtcctgggggatgcactcatccatgatctggttaatgatgttcaacacattgtcctgacaggagcggaactggctgaccagcagcgtgcaccgctgggggtccttccgcccatccaggctgtccagctccgcggccacctggttcagctcctcgtcggcatagtagaaccgggcaagcagctgcggatccgacctctcgcgtctcgccgtcaggggtgacagtggtggacgcaggtgatgagcataacgttgtgcattcccgccgccgcgccctcgtcaaggcgcccacggcctccgagcgggtgactgggaatggcgggggctgtgttc

SEQ ID NO: 12540 - RNA, 3730 nt, Homo sapiens
  source 1..3730: mol_type = other RNA
gagagatcagaggcgcagagtggccccactcttgtccacctccatcacccgccccgattcccatagccccagcagatctccgagggaccagtgggagggcccaggccttctccgccaggcaccctgccctgaggcagccaccaggctcctccgggtcccctgctgggcaaagctgacctcttgttggcccctgcagccggcccggggtccctgcagggaggctagcgtgggcaggacagaggctctggatgctctggaggtctgggtgcccctgcagcagcggcagcggcctcatgagacgcagtgagacctgcctgcagcgtggccccaccttcctgggggttcctggcccgggtgggttggggctgcccctggcaccacgtcacaggccggccttgtcgctgtagaagggcgtgacatggaacatgtagcagtgggtgcacactcggaccggcttcacctgcccgtagcggggcagcggtgctgagtgcgaggagcagcgcgagcagaagatcttcaggaggctggactctatgaggggtccacgtcctgcaccaaggctgctgcaggctcctgttcacactcgctgtcccctctctgtggctggctctgcagcagccgggactggacatgggcaccatccaggttcccgtggtcaaatgcctggagtcagaacagggcccgggacctccaggggcctctgcacaagaccccacaggcctcgctggcctccctgggcatcggttctgacttccagacctcaggctctgtccgtggacgcccttggatgctgagggaccctccgtgcaaggggtctcacccaccttcccacagctgcggcagtggtgcttccggcggatgacggtgaagggtgctttgcacgccgtgcagaagccacaggcctcgtctggcacccactccggggggtcttcaaagtccccatcgcgggtcttggctgccagttcagaggatgacagggtctcctggcacagtgcacagtcctccaaggccgcactccgcagagtctgggtgaccttccttaacttttccttgtcgtctgtttcaggcttggtggccatgacctcaaacagtgttttaagaatacttctcaggtcactggcatagttcgtctgcagctggtcagccacacctgaaatgcagacgaacaggcggtggatgaggtcgtggctgccgtggaacctggaccggatcttctctcttgtggcctgtggggcagcatgcgtggctgctggggccgcctctggccccatcttgtctgaggagcaggacccagctgtggagctgctggagcccgacagggcctgaggcgcctcgtgagccgaggggctcccagcatgcagctctctggcctctggctcctgctgacctgcaaccccagcctctccttgcagcccactcgctgtgtccacctgggaacctgaggtgtgaggcaggcacttgtcggaagtgggggctttgggctcccgcccgttggaggcatcttctgagggtgggggcgcctcctcctgtctctcaggggccctgtcgctggccttggctaagccggcagcgtacgaggcaccaatgacgcctcccgggctgcacttctcccgcagacgctccaccacgtcctccctgctgtccccgcagctcccacagcacacgcaggaatgcagaaggcagttggtggccccagtgctaagcttgtgggggccgccatccatcccctcggccacgggctccgaggcggcctcctgggtggcgaccgcagagtccagggaagtgggcgatttggggttgaagatgaccgtggctgagagcttcatgccccctgtccggtgggcgatcatctcagccgtctctgcgtcatccgcacccacctcccagccgtccaggtgcagccgcgagtccaggcagctgcaggagctggtgcccgcgaggctggccccatctgtgccctcggcctcgagattgttgttgctcaagtcctcctccttttccgaggcgggcaagctgatccccgccgctccgcctggcccaccctgccctttctcctgggggtcggcccaggtactgcctgcccacccaaatgggccagctggggactcgggcctggccagggcttctgccgtcccctccacgtcatccatgaagaacacgcgctcctcctcgtcactgcctgaccgcaggcgcggtctacctggagaggcctccccgcctgggctgccctccgctcctggcctgtgagctggggactggcaggcaatgggcggtgaaagcaaagaggacatctcgtcccccgccctgtggaccatgcggctgagctgctccagctcctggtcgtcgtactgcatggagcaggccagctctgcatccgggtctttggccttagctgagagtggcccctcaggggggagaggggcagagagggcaggcgccagggcagcgggtccctgcacgtctgcgcggatggggaactccacgtcttgggaaatgcagaggttccgttccagcgtgtgcagctcctcctccgtcagcgtctgcagcaaatcccttattttccgcagcaacgtgtggaagggccggaacagctcggacatgtcttccaccttgcggtccaagttcagaggtccgtccgcatagaccacgaggccacacacgatggccagcctggggatgctgaacatgagggccggctcgtagtcatcaatcatgtcctgagtcaggtacccgaagtccagggccctctccaccgtctcgcagaagagcacgatgacctcctgctgcacgtagtactccctgggggacttcacaggcaccatggccgagacgtagctgagctcaaactctgcgaacaggacgtcgaagtgcctcagcgcttccctcatcttctctgtgtaggtgttcaggtcccgcagcgcctggtcacggagggcgccccgcacgtcctccaggctgcgcgtcagctccttggccagcgggcgcatggccatgctctccagctcccggttcatgatgatggagccggcggccaggcactcggcaccgaaccacagctggccggccaggttgtcgtgccggatctcctcagggaacttgacgcagaaatctctgggggcgcggtcctgggggatgcactcatccatgatctggttaatgatgttcaacacattgtcctgacaggagcggaactggctgaccagcagcgtgcaccgctgggggtccttccgcccatccaggctgtccagctccgcggccacctggttcagctcctcgtcggcatagtagaaccgggcaagcagctgcggatccgacctcttgggtttgtagagccactttcggaacctgttcatcatcgccgcgccggccctggccggactccgggcggccctcgccctccgcagcgctgcgcccgggcccggctgaggcgcggggcggacgcggaggcacggccggagcccccgcgctgtcgcagggaggctggctagcgaagcccggagcgccgagcgggcggcgggcaggtgcgcggggcaggtgcgcggccctgagtatgctctgcaagcggcgcgccgggcagacctcagacccgggagtgggcgctcgggcgcacggacagacgcgggcacgggggcgcgcggctcctcgctgctcactgacacccagcgctccgctggtcacggccgccccgcgccgcacatgcgcctagggcgccgcgagccccgggcccacc

SEQ ID NO: 12541 - RNA, 3144 nt, Homo sapiens
  source 1..3144: mol_type = other RNA
gagagatcagaggcgcagagtggccccactcttgtccacctccatcacccgccccgattcccatagccccagcagatctccgagggaccagtgggagggcccaggccttctccgccaggcaccctgccctgaggcagccaccaggctcctccgggtcccctgctgggcaaagctgacctcttgttggcccctgcagccggcccggggtccctgcagggaggctagcgtgggcaggacagaggctctggatgctctggaggtctgggtgcccctgcagcagcggcagcggcctcatgagacgcagtgagacctgcctgcagcgtggccccaccttcctgggggttcctggcccgggtgggttggggctgcccctggcaccacgtcacaggccggccttgtcgctgtagaagggcgtgacatggaacatgtagcagtgggtgcacactcggaccggcttcacctgcccgtagcggggcagcggtgctgagtgcgaggagcagcgcgagcagaagatcttcaggaggctggactctatgaggggtccacgtcctgcaccaaggctgctgcaggctcctgttcacactcgctgtcccctctctgtggctggctctgcagcagccgggactggacatgggcaccatccaggttcccgtggtcaaatgcctggagtcagaacagggcccgggacctccaggggcctctgcacaagaccccacaggcctcgctggcctccctgggcatcggttctgacttccagacctcaggctctgtccgtggacgcccttggatgctgagggaccctccgtgcaaggggtctcacccaccttcccacagctgcggcagtggtgcttccggcggatgacggtgaagggtgctttgcacgccgtgcagaagccacaggcctcgtctggcacccactccggggggtcttcaaagtccccatcgcgggtcttggctgccagttcagaggatgacagggtctcctggcacagtgcacagtcctccaaggccgcactccgcagagtctgggtgaccttccttaacttttccttgtcgtctgtttcaggcttggtggccatgacctcaaacagtgttttaagaatacttctcaggtcactggcatagttcgtctgcagctggtcagccacacctgaaatgcagacgaacaggcggtggatgaggtcgtggctgccgtggaacctggaccggatcttctctcttgtggcctgtggggcagcatgcgtggctgctggggccgcctctggccccatcttgtctgaggagcaggacccagctgtggagctgctggagcccgacagggcctgaggcgcctcgtgagccgaggggctcccagcatgcagctctctggcctctggctcctgctgacctgcaaccccagcctctccttgcagcccactcgctgtgtccacctgggaacctgaggtgtgaggcaggcacttgtcggaagtgggggctttgggctcccgcccgttggaggcatcttctgagggtgggggcgcctcctcctgtctctcaggggccctgtcgctggccttggctaagccggcagcgtacgaggcaccaatgacgcctcccgggctgcacttctcccgcagacgctccaccacgtcctccctgctgtccccgcagctcccacagcacacgcaggaatgcagaaggcagttggtggccccagtgctaagcttgtgggggccgccatccatcccctcggccacgggctccgaggcggcctcctgggtggcgaccgcagagtccagggaagtgggcgatttggggttgaagatgaccgtggctgagagcttcatgccccctgtccggtgggcgatcatctcagccgtctctgcgtcatccgcacccacctcccagccgtccaggtgcagccgcgagtccaggcagctgcaggagctggtgcccgcgaggctggccccatctgtgccctcggcctcgagattgttgttgctcaagtcctcctccttttccgaggcgggcaagctgatccccgccgctccgcctggcccaccctgccctttctcctgggggtcggcccaggtactgcctgcccacccaaatgggccagctggggactcgggcctggccagggcttctgccgtcccctccacgtcatccatgaagaacacgcgctcctcctcgtcactgcctgaccgcaggcgcggtctacctggagaggcctccccgcctgggctgccctccgctcctggcctgtgagctggggactggcaggcaatgggcggtgaaagcaaagaggacatctcgtcccccgccctgtggaccatgcggctgagctgctccagctcctggtcgtcgtactgcatggagcaggccagctctgcatccgggtctttggccttagctgagagtggcccctcaggggggagaggggcagagagggcaggcgccagggcagcgggtccctgcacgtctgcgcggatggggaactccacgtcttgggaaatgcagaggttccgttccagcgtgtgcagctcctcctccgtcagcgtctgcagcaaatcccttattttccgcagcaacgtgtggaagggccggaacagctcggacatgtcttccaccttgcggtccaagttcagaggtccgtccgcatagaccacgaggccacacacgatggccagcctggggatgctgaacatgagggccggctcgtagtcatcaatcatgtcctgagtcaggtacccgaagtccagggccctctccaccgtctcgcagaagagcacgatgacctcctgctgcacgtagtactccctgggggacttcacaggcaccatggccgagacgtagctgagctcaaactctgcgaacaggacgtcgaagtgcctcagcgcttccctcatcttctctgtgtaggtgttcaggtcccgcagcgcctggtcacggagggcgccccgcacgtcctccaggctgcgcgtcagctccttggccagcgggcgcatggccatgctctccagctcccggttcatgatgatggagccggcggccaggcactcggggcccctcttctcaccccacagcacaggccagctcgtgttcccggtccccgcaggaggtttttcttacattcagagcaatcgtgagggcgataaccgatgt

SEQ ID NO: 12542 - RNA, 3336 nt, Homo sapiens
  source 1..3336: mol_type = other RNA
gagagatcagaggcgcagagtggccccactcttgtccacctccatcacccgccccgattcccatagccccagcagatctccgagggaccagtgggagggcccaggccttctccgccaggcaccctgccctgaggcagccaccaggctcctccgggtcccctgctgggcaaagctgacctcttgttggcccctgcagccggcccggggtccctgcagggaggctagcgtgggcaggacagaggctctggatgctctggaggtctgggtgcccctgcagcagcggcagcggcctcatgagacgcagtgagacctgcctgcagcgtggccccaccttcctgggggttcctggcccgggtgggttggggctgcccctggcaccacgtcacaggccggccttgtcgctgtagaagggcgtgacatggaacatgtagcagtgggtgcacactcggaccggcttcacctgcccgtagcggggcagcggtgctgagtgcgaggagcagcgcgagcagaagatcttcccacagctgcggcagtggtgcttccggcggatgacggtgaagggtgctttgcacgccgtgcagaagccacaggcctcgtctggcacccactccggggggtcttcaaagtccccatcgcgggtcttggctgccagttcagaggatgacagggtctcctggcacagtgcacagtcctccaaggccgcactccgcagagtctgggtgaccttccttaacttttccttgtcgtctgtttcaggcttggtggccatgacctcaaacagtgttttaagaatacttctcaggtcactggcatagttcgtctgcagctggtcagccacacctgaaatgcagacgaacaggcggtggatgaggtcgtggctgccgtggaacctggaccggatcttctctcttgtggcctgtggggcagcatgcgtggctgctggggccgcctctggccccatcttgtctgaggagcaggacccagctgtggagctgctggagcccgacagggcctgaggcgcctcgtgagccgaggggctcccagcatgcagctctctggcctctggctcctgctgacctgcaaccccagcctctccttgcagcccactcgctgtgtccacctgggaacctgaggtgtgaggcaggcacttgtcggaagtgggggctttgggctcccgcccgttggaggcatcttctgagggtgggggcgcctcctcctgtctctcaggggccctgtcgctggccttggctaagccggcagcgtacgaggcaccaatgacgcctcccgggctgcacttctcccgcagacgctccaccacgtcctccctgctgtccccgcagctcccacagcacacgcaggaatgcagaaggcagttggtggccccagtgctaagcttgtgggggccgccatccatcccctcggccacgggctccgaggcggcctcctgggtggcgaccgcagagtccagggaagtgggcgatttggggttgaagatgaccgtggctgagagcttcatgccccctgtccggtgggcgatcatctcagccgtctctgcgtcatccgcacccacctcccagccgtccaggtgcagccgcgagtccaggcagctgcaggagctggtgcccgcgaggctggccccatctgtgccctcggcctcgagattgttgttgctcaagtcctcctccttttccgaggcgggcaagctgatccccgccgctccgcctggcccaccctgccctttctcctgggggtcggcccaggtactgcctgcccacccaaatgggccagctggggactcgggcctggccagggcttctgccgtcccctccacgtcatccatgaagaacacgcgctcctcctcgtcactgcctgaccgcaggcgcggtctacctggagaggcctccccgcctgggctgccctccgctcctggcctgtgagctggggactggcaggcaatgggcggtgaaagcaaagaggacatctcgtcccccgccctgtggaccatgcggctgagctgctccagctcctggtcgtcgtactgcatggagcaggccagctctgcatccgggtctttggccttagctgagagtggcccctcaggggggagaggggcagagagggcaggcgccagggcagcgggtccctgcacgtctgcgcggatggggaactccacgtcttgggaaatgcagaggttccgttccagcgtgtgcagctcctcctccgtcagcgtctgcagcaaatcccttattttccgcagcaacgtgtggaagggccggaacagctcggacatgtcttccaccttgcggtccaagttcagaggtccgtccgcatagaccacgaggccacacacgatggccagcctggggatgctgaacatgagggccggctcgtagtcatcaatcatgtcctgagtcaggtacccgaagtccagggccctctccaccgtctcgcagaagagcacgatgacctcctgctgcacgtagtactccctgggggacttcacaggcaccatggccgagacgtagctgagctcaaactctgcgaacaggacgtcgaagtgcctcagcgcttccctcatcttctctgtgtaggtgttcaggtcccgcagcgcctggtcacggagggcgccccgcacgtcctccaggctgcgcgtcagctccttggccagcgggcgcatggccatgctctccagctcccggttcatgatgatggagccggcggccaggcactcggcaccgaaccacagctggccggccaggttgtcgtgccggatctcctcagggaacttgacgcagaaatctctgggggcgcggtcctgggggatgcactcatccatgatctggttaatgatgttcaacacattgtcctgacaggagcggaactggctgaccagcagcgtgcaccgctgggggtccttccgcccatccaggctgtccagctccgcggccacctggttcagctcctcgtcggcatagtagaaccgggcaagcagctgcggatccgacctccagagggtggctgtgcctgtttagaggaatcctccacagcccagacgcaacaggagccacgtgggaagggaatttagacggtcggcactgggcacagacgcccgggtgggctccaggttcttggccgcctgtcccctctgattagcatctgcaaagtgggcttaaggacgcagagaacccgcttagcctggacaagcccttagcacctcgcgtctcgccgtcaggggtgacagtggtggacgcaggtgatgagcataacgttgtgcattcccgccgccgcgccctcgtcaaggcgcccacggcctccgagcgggtgactgggaatggc

SEQ ID NO: 12543 - RNA, 3368 nt, Homo sapiens
  source 1..3368: mol_type = other RNA
gagagatcagaggcgcagagtggccccactcttgtccacctccatcacccgccccgattcccatagccccagcagatctccgagggaccagtgggagggcccaggccttctccgccaggcaccctgccctgaggcagccaccaggctcctccgggtcccctgctgggcaaagctgacctcttgttggcccctgcagccggcccggggtccctgcagggaggctagcgtgggcaggacagaggctctggatgctctggaggtctgggtgcccctgcagcagcggcagcggcctcatgagacgcagtgagacctgcctgcagcgtggccccaccttcctgggggttcctggcccgggtgggttggggctgcccctggcaccacgtcacaggccggccttgtcgctgtagaagggcgtgacatggaacatgtagcagtgggtgcacactcggaccggcttcacctgcccgtagcggggcagcggtgctgagtgcgaggagcagcgcgagcagaagatcttcccacagctgcggcagtggtgcttccggcggatgacggtgaagggtgctttgcacgccgtgcagaagccacaggcctcgtctggcacccactccggggggtcttcaaagtccccatcgcgggtcttggctgccagttcagaggatgacagggtctcctggcacagtgcacagtcctccaaggccgcactccgcagagtctgggtgaccttccttaacttttccttgtcgtctgtttcaggcttggtggccatgacctcaaacagtgttttaagaatacttctcaggtcactggcatagttcgtctgcagctggtcagccacacctgaaatgcagacgaacaggcggtggatgaggtcgtggctgccgtggaacctggaccggatcttctctcttgtggcctgtggggcagcatgcgtggctgctggggccgcctctggccccatcttgtctgaggagcaggacccagctgtggagctgctggagcccgacagggcctgaggcgcctcgtgagccgaggggctcccagcatgcagctctctggcctctggctcctgctgacctgcaaccccagcctctccttgcagcccactcgctgtgtccacctgggaacctgaggtgtgaggcaggcacttgtcggaagtgggggctttgggctcccgcccgttggaggcatcttctgagggtgggggcgcctcctcctgtctctcaggggccctgtcgctggccttggctaagccggcagcgtacgaggcaccaatgacgcctcccgggctgcacttctcccgcagacgctccaccacgtcctccctgctgtccccgcagctcccacagcacacgcaggaatgcagaaggcagttggtggccccagtgctaagcttgtgggggccgccatccatcccctcggccacgggctccgaggcggcctcctgggtggcgaccgcagagtccagggaagtgggcgatttggggttgaagatgaccgtggctgagagcttcatgccccctgtccggtgggcgatcatctcagccgtctctgcgtcatccgcacccacctcccagccgtccaggtgcagccgcgagtccaggcagctgcaggagctggtgcccgcgaggctggccccatctgtgccctcggcctcgagattgttgttgctcaagtcctcctccttttccgaggcgggcaagctgatccccgccgctccgcctggcccaccctgccctttctcctgggggtcggcccaggtactgcctgcccacccaaatgggccagctggggactcgggcctggccagggcttctgccgtcccctccacgtcatccatgaagaacacgcgctcctcctcgtcactgcctgaccgcaggcgcggtctacctggagaggcctccccgcctgggctgccctccgctcctggcctgtgagctggggactggcaggcaatgggcggtgaaagcaaagaggacatctcgtcccccgccctgtggaccatgcggctgagctgctccagctcctggtcgtcgtactgcatggagcaggccagctctgcatccgggtctttggccttagctgagagtggcccctcaggggggagaggggcagagagggcaggcgccagggcagcgggtccctgcacgtctgcgcggatggggaactccacgtcttgggaaatgcagaggttccgttccagcgtgtgcagctcctcctccgtcagcgtctgcagcaaatcccttattttccgcagcaacgtgtggaagggccggaacagctcggacatgtcttccaccttgcggtccaagttcagaggtccgtccgcatagaccacgaggccacacacgatggccagcctggggatgctgaacatgagggccggctcgtagtcatcaatcatgtcctgagtcaggtacccgaagtccagggccctctccaccgtctcgcagaagagcacgatgacctcctgctgcacgtagtactccctgggggacttcacaggcaccatggccgagacgtagctgagctcaaactctgcgaacaggacgtcgaagtgcctcagcgcttccctcatcttctctgtgtaggtgttcaggtcccgcagcgcctggtcacggagggcgccccgcacgtcctccaggctgcgcgtcagctccttggccagcgggcgcatggccatgctctccagctcccggttcatgatgatggagccggcggccaggcactcggcaccgaaccacagctggccggccaggttgtcgtgccggatctcctcagggaacttgacgcagaaatctctgggggcgcggtcctgggggatgcactcatccatgatctggttaatgatgttcaacacattgtcctgacaggagcggaactggctgaccagcagcgtgcaccgctgggggtccttccgcccatccaggctgtccagctccgcggccacctggttcagctcctcgtcggcatagtagaaccgggcaagcagctgcggatccgacctcttgggtttgtagagccactttcggaacctgttcatcatcgccgcgccggccctggccggactccgggcggccctcgccctccgcagcgctgcgcccgggcccggctgaggcgcggggcggacgcggaggcacggccggagcccccgcgctgtcgcagggaggctggctagcgaagcccggagcgccgagcgggcggcgggcaggtgcgcggggcaggtgcgcggccctgagtatgctctgcaagcggcgcgccgggcagacctcagacccgggagtgggcgctcgggcgcacggacagacgcgggcacgggggcgcgcggctcctcgctgctcactgacacccagcgctccgctggtcac

SEQ ID NO: 12544 - RNA, 4964 nt, Homo sapiens
  source 1..4964: mol_type = other RNA
gagagatcagaggcgcagagtggccccactcttgtccacctccatcacccgccccgattcccatagccccagcagatctccgagggaccagtgggagggcccaggccttctccgccaggcaccctgccctgaggcagccaccaggctcctccgggtcccctgctgggcaaagctgacctcttgttggcccctgcagccggcccggggtccctgcagggaggctagcgtgggcaggacagaggctctggatgctctggaggtctgggtgcccctgcagcagcggcagcggcctcatgagacgcagtgagacctgcctgcagcgtggccccaccttcctgggggttcctggcccgggtgggttggggctgcccctggcaccacgtcacaggccggccttgtcgctgtagaagggcgtgacatggaacatgtagcagtgggtgcacactcggaccggcttcacctgcccgtagcggggcagcggtgctgagtgcgaggagcagcgcgagcagaagatcttcccacagctgcggcagtggtgcttccggcggatgacggtgaagggtgctttgcacgccgtgcagaagccacaggcctcgtctggcacccactccggggggtcttcaaagtccccatcgcgggtcttggctgccagttcagaggatgacagggtctcctggcacagtgcacagtcctccaaggccgcactccgcagagtctgggtgaccttccttaacttttccttgtcgtctgtttcaggcttggtggccatgacctcaaacagtgttttaagaatacttctcaggtcactggcatagttcgtctgcagctggtcagccacacctgaaatgcagacgaacaggcggtggatgaggtcgtggctgccgtggaacctggaccggatcttctctcttgtggcctgtggggcagcatgcgtggctgctggggccgcctctggccccatcttgtctgaggagcaggacccagctgtggagctgctggagcccgacagggcctgaggcgcctcgtgagccgaggggctcccagcatgcagctctctggcctctggctcctgctgacctgcaaccccagcctctccttgcagcccactcgctgtgtccacctgggaacctgaggtgtgaggcaggcacttgtcggaagtgggggctttgggctcccgcccgttggaggcatcttctgagggtgggggcgcctcctcctgtctctcaggggccctgtcgctggccttggctaagccggcagcgtacgaggcaccaatgacgcctcccgggctgcacttctcccgcagacgctccaccacgtcctccctgctgtccccgcagctcccacagcacacgcaggaatgcagaaggcagttggtggccccagtgctaagcttgtgggggccgccatccatcccctcggccacgggctccgaggcggcctcctgggtggcgaccgcagagtccagggaagtgggcgatttggggttgaagatgaccgtggctgagagcttcatgccccctgtccggtgggcgatcatctcagccgtctctgcgtcatccgcacccacctcccagccgtccaggtgcagccgcgagtccaggcagctgcaggagctggtgcccgcgaggctggccccatctgtgccctcggcctcgagattgttgttgctcaagtcctcctccttttccgaggcgggcaagctgatccccgccgctccgcctggcccaccctgccctttctcctgggggtcggcccaggtactgcctgcccacccaaatgggccagctggggactcgggcctggccagggcttctgccgtcccctccacgtcatccatgaagaacacgcgctcctcctcgtcactgcctgaccgcaggcgcggtctacctggagaggcctccccgcctgggctgccctccgctcctggcctgtgagctggggactggcaggcaatgggcggtgaaagcaaagaggacatctcgtcccccgccctgtggaccatgcggctgagctgctccagctcctggtcgtcgtactgcatggagcaggccagctctgcatccgggtctttggccttagctgagagtggcccctcaggggggagaggggcagagagggcaggcgccagggcagcgggtccctgcacgtctgcgcggatggggaactccacgtcttgggaaatgcagaggttccgttccagcgtgtgcagctcctcctccgtcagcgtctgcagcaaatcccttattttccgcagcaacgtgtggaagggccggaacagctcggacatgtcttccaccttgcggtccaagttcagaggtccgtccgcatagaccacgaggccacacacgatggccagcctggggatgctgaacatgagggccggctcgtagtcatcaatcatgtcctgagtcaggtacccgaagtccagggccctctccaccgtctcgcagaagagcacgatgacctcctgctgcacgtagtactccctgggggacttcacaggcaccatggccgagacgtagctgagctcaaactctgcgaacaggacgtcgaagtgcctcagcgcttccctcatcttctctgtgtaggtgttcaggtcccgcagcgcctggtcacggagggcgccccgcacgtcctccaggctgcgcgtcagctccttggccagcgggcgcatggccatgctctccagctcccggttcatgatgatggagccggcggccaggcactgcgggaggggacacactcagggaggggcccgggtgagggccaggctctcaggggtcgccgacccggggaacctgactgcgcacctcggggcccctcttctcaccccacagcacaggccagctcgtgttcccggtccccgcaggaggtttttcttacattcagagcaatcgtgagggcgataaccgatgtcccccaatgtgacccacggggtcctcacagggccccaggagcagggagggcagggcatggcagggcaggtaagggcaggggaggggagggcaggggaggggaggggaggggaaggtggactgaggcccttgggtctgggggctccctgcaggaggaaccctggtcatgtgactcttttccgctccccgtccaggccacagggatgaagttcaaggagcttggagcttccaggctccacaatcaggtctgtgctcccagggatgaagcagccgggctgatccgggcccgaggtccccagcctatctagggagccacagacaccacctgtcaagttgctcactgccagagaaacgcaaccttccccggaacgcagactcatcagtgtgagagtccctgggctcctgggcaggtaaggagggctcctccgcacccacaaatccacccatgtctgccctgggtgctgcgaggcagctccccagcgtgcgctcagcaactgggaatttcaccaagctgccctctggcacaggggctgagtccaggccctggtagacctgttgtcacagggaggcttgtctagaggccggggcctcgccaggtttaggatagaaccaatccacctgctgtcccctcagggatgatcaagtgatgcaggacaagaagccatttcccaggtgacagaatgagacggcgctgatcgcccaggcccaagctgcaggtgggcacagagcttggggcaccaggaccacacaaggagctgtgcccacccctgtgcatgcatgcccctgccaggccagccgggcacagaacacgctccatctcatgactgccccaggacccactccacggaggtggaaactgaggctggggaggagggagaacctgcccgcgggcccctgtaactaacccaagcctcggcagaggacaccccaaccaggtggctcagaaggtggggtgggcagggtggacacagggacggggcagcgtgggatgaagactccgcaccccagggattcctagaaaggggaggcgggcaggatggggacggcacaatagagagggtggcggtgtcggggctgaggtcaggctcgggagcacggcaaggggaggaggctggggagtccgcatggtgggggcctgggggagactgttcccgccaccttgaagggcaccttcctctcggtgcctcagtttcctgattgggagatgaagatgaagatgacaggctattgccacatgtggcctgcgtggggctgcagcacggctccccagcccctgctgctgcccatgctgcagggccggaggggaacacttgttcctgatgtgggcattactgccattaaaaaccacttttaggtcctggctgtctgggggcctgtgaacctcataaaaaccacatgggaaatttcatttgtatgtatagttttgggggcaccagttcatggctttcccagatcctccaggggtgcacggcctaccaggctcagaccacaccacgtaacccagagtggacggagctcttggaggagacaccaggtcccggcacctgcaggcgcccatgcacaaggttcgcagggacttggctagacgccaccccacatcaggacctccgaacccgggtggccacccgctacctcggcaccgaaccacagctggccggccaggttgtcgtgccggatctcctcagggaacttgacgcagaaatctctgggggcgcggtcctgggggatgcactcatccatgatctggttaatgatgttcaacacattgtcctgacaggagcggaactggctgaccagcagcgtgcaccgctgggggtccttccgcccatccaggctgtccagctccgcggccacctggttcagctcctcgtcggcatagtagaaccgggcaagcagctgcggatccgacctctcgcgtctcgccgtcaggggtgacagtggtggacgcaggtgatgagcataacgttgtgcattcccgccgccgcgccctcgtcaaggcgcccacggcctccgagcgggtgactgggaatggcgggggctgtgttc

SEQ ID NO: 12545 - RNA, 3278 nt, Homo sapiens
  source 1..3278: mol_type = other RNA
gagagatcagaggcgcagagtggccccactcttgtccacctccatcacccgccccgattcccatagccccagcagatctccgagggaccagtgggagggcccaggccttctccgccaggcaccctgccctgaggcagccaccaggctcctccgggtcccctgctgggcaaagctgacctcttgttggcccctgcagccggcccggggtccctgcagggaggctagcgtgggcaggacagaggctctggatgctctggaggtctgggtgcccctgcagcagcggcagcggcctcatgagacgcagtgagacctgcctgcagcgtggccccaccttcctgggggttcctggcccgggtgggttggggctgcccctggcaccacgtcacaggccggccttgtcgctgtagaagggcgtgacatggaacatgtagcagtgggtgcacactcggaccggcttcacctgcccgtagcggggcagcggtgctgagtgcgaggagcagcgcgagcagaagatcttcccacagctgcggcagtggtgcttccggcggatgacggtgaagggtgctttgcacgccgtgcagaagccacaggcctcgtctggcacccactccggggggtcttcaaagtccccatcgcgggtcttggctgccagttcagaggatgacagggtctcctggcacagtgcacagtcctccaaggccgcactccgcagagtctgggtgaccttccttaacttttccttgtcgtctgtttcaggcttggtggccatgacctcaaacagtgttttaagaatacttctcaggtcactggcatagttcgtctgcagctggtcagccacacctgaaatgcagacgaacaggcggtggatgaggtcgtggctgccgtggaacctggaccggatcttctctcttgtggcctgtggggcagcatgcgtggctgctggggccgcctctggccccatcttgtctgaggagcaggacccagctgtggagctgctggagcccgacagggcctgaggcgcctcgtgagccgaggggctcccagcatgcagctctctggcctctggctcctgctgacctgcaaccccagcctctccttgcagcccactcgctgtgtccacctgggaacctgaggtgtgaggcaggcacttgtcggaagtgggggctttgggctcccgcccgttggaggcatcttctgagggtgggggcgcctcctcctgtctctcaggggccctgtcgctggccttggctaagccggcagcgtacgaggcaccaatgacgcctcccgggctgcacttctcccgcagacgctccaccacgtcctccctgctgtccccgcagctcccacagcacacgcaggaatgcagaaggcagttggtggccccagtgctaagcttgtgggggccgccatccatcccctcggccacgggctccgaggcggcctcctgggtggcgaccgcagagtccagggaagtgggcgatttggggttgaagatgaccgtggctgagagcttcatgccccctgtccggtgggcgatcatctcagccgtctctgcgtcatccgcacccacctcccagccgtccaggtgcagccgcgagtccaggcagctgcaggagctggtgcccgcgaggctggccccatctgtgccctcggcctcgagattgttgttgctcaagtcctcctccttttccgaggcgggcaagctgatccccgccgctccgcctggcccaccctgccctttctcctgggggtcggcccaggtactgcctgcccacccaaatgggccagctggggactcgggcctggccagggcttctgccgtcccctccacgtcatccatgaagaacacgcgctcctcctcgtcactgcctgaccgcaggcgcggtctacctggagaggcctccccgcctgggctgccctccgctcctggcctgtgagctggggactggcaggcaatgggcggtgaaagcaaagaggacatctcgtcccccgccctgtggaccatgcggctgagctgctccagctcctggtcgtcgtactgcatggagcaggccagctctgcatccgggtctttggccttagctgagagtggcccctcaggggggagaggggcagagagggcaggcgccagggcagcgggtccctgcacgtctgcgcggatggggaactccacgtcttgggaaatgcagaggttccgttccagcgtgtgcagctcctcctccgtcagcgtctgcagcaaatcccttattttccgcagcaacgtgtggaagggccggaacagctcggacatgtcttccaccttgcggtccaagttcagaggtccgtccgcatagaccacgaggccactctccaccgtctcgcagaagagcacgatgacctcctgctgcacgtagtactccctgggggacttcacaggcaccatggccgagacgtagctgagctcaaactctgcgaacaggacgtcgaagtgcctcagcgcttccctcatcttctctgtgtaggtgttcaggtcccgcagcgcctggtcacggagggcgccccgcacgtcctccaggctgcgcgtcagctccttggccagcgggcgcatggccatgctctccagctcccggttcatgatgatggagccggcggccaggcactcggcaccgaaccacagctggccggccaggttgtcgtgccggatctcctcagggaacttgacgcagaaatctctgggggcgcggtcctgggggatgcactcatccatgatctggttaatgatgttcaacacattgtcctgacaggagcggaactggctgaccagcagcgtgcaccgctgggggtccttccgcccatccaggctgtccagctccgcggccacctggttcagctcctcgtcggcatagtagaaccgggcaagcagctgcggatccgacctcttgggtttgtagagccactttcggaacctgttcatcatcgccgcgccggccctggccggactccgggcggccctcgccctccgcagcgctgcgcccgggcccggctgaggcgcggggcggacgcggaggcacggccggagcccccgcgctgtcgcagggaggctggctagcgaagcccggagcgccgagcgggcggcgggcaggtgcgcggggcaggtgcgcggccctgagtatgctctgcaagcggcgcgccgggcagacctcagacccgggagtgggcgctcgggcgcacggacagacgcgggcacgggggcgcgcggctcctcgctgctcactgacacccagcgctccgctggtcac

SEQ ID NO: 12546 - RNA, 3644 nt, Homo sapiens
  source 1..3644: mol_type = other RNA
gagagatcagaggcgcagagtggccccactcttgtccacctccatcacccgccccgattcccatagccccagcagatctccgagggaccagtgggagggcccaggccttctccgccaggcaccctgccctgaggcagccaccaggctcctccgggtcccctgctgggcaaagctgacctcttgttggcccctgcagccggcccggggtccctgcagggaggctagcgtgggcaggacagaggctctggatgctctggaggtctgggtgcccctgcagcagcggcagcggcctcatgagacgcagtgagacctgcctgcagcgtggccccaccttcctgggggttcctggcccgggtgggttggggctgcccctggcaccacgtcacaggccggccttgtcgctgtagaagggcgtgacatggaacatgtagcagtgggtgcacactcggaccggcttcacctgcccgtagcggggcagcggtgctgagtgcgaggagcagcgcgagcagaagatcttcccacagctgcggcagtggtgcttccggcggatgacggtgaagggtgctttgcacgccgtgcagaagccacaggcctcgtctggcacccactccggggggtcttcaaagtccccatcgcgggtcttggctgccagttcagaggatgacagggtctcctggcacagtgcacagtcctccaaggccgcactccgcagagtctgggtgactgccgtctctgaatcatgatttccagaaggcagtcctgccaacctccctggtagaatgcagcctggcggtgtggattcggcagggcagagctgggtcggcacatgggctcctccctgctggcaagggtatgccctgctgggccagggctccaggaccaggcgggctgccccatgtgcccggacgccccatgaacagaagcctctgtggtgagggatggctctgccttccttaacttttccttgtcgtctgtttcaggcttggtggccatgacctcaaacagtgttttaagaatacttctcaggtcactggcatagttcgtctgcagctggtcagccacacctgaaatgcagacgaacaggcggtggatgaggtcgtggctgccgtggaacctggaccggatcttctctcttgtggcctgtggggcagcatgcgtggctgctggggccgcctctggccccatcttgtctgaggagcaggacccagctgtggagctgctggagcccgacagggcctgaggcgcctcgtgagccgaggggctcccagcatgcagctctctggcctctggctcctgctgacctgcaaccccagcctctccttgcagcccactcgctgtgtccacctgggaacctgaggtgtgaggcaggcacttgtcggaagtgggggctttgggctcccgcccgttggaggcatcttctgagggtgggggcgcctcctcctgtctctcaggggccctgtcgctggccttggctaagccggcagcgtacgaggcaccaatgacgcctcccgggctgcacttctcccgcagacgctccaccacgtcctccctgctgtccccgcagctcccacagcacacgcaggaatgcagaaggcagttggtggccccagtgctaagcttgtgggggccgccatccatcccctcggccacgggctccgaggcggcctcctgggtggcgaccgcagagtccagggaagtgggcgatttggggttgaagatgaccgtggctgagagcttcatgccccctgtccggtgggcgatcatctcagccgtctctgcgtcatccgcacccacctcccagccgtccaggtgcagccgcgagtccaggcagctgcaggagctggtgcccgcgaggctggccccatctgtgccctcggcctcgagattgttgttgctcaagtcctcctccttttccgaggcgggcaagctgatccccgccgctccgcctggcccaccctgccctttctcctgggggtcggcccaggtactgcctgcccacccaaatgggccagctggggactcgggcctggccagggcttctgccgtcccctccacgtcatccatgaagaacacgcgctcctcctcgtcactgcctgaccgcaggcgcggtctacctggagaggcctccccgcctgggctgccctccgctcctggcctgtgagctggggactggcaggcaatgggcggtgaaagcaaagaggacatctcgtcccccgccctgtggaccatgcggctgagctgctccagctcctggtcgtcgtactgcatggagcaggccagctctgcatccgggtctttggccttagctgagagtggcccctcaggggggagaggggcagagagggcaggcgccagggcagcgggtccctgcacgtctgcgcggatggggaactccacgtcttgggaaatgcagaggttccgttccagcgtgtgcagctcctcctccgtcagcgtctgcagcaaatcccttattttccgcagcaacgtgtggaagggccggaacagctcggacatgtcttccaccttgcggtccaagttcagaggtccgtccgcatagaccacgaggccacacacgatggccagcctggggatgctgaacatgagggccggctcgtagtcatcaatcatgtcctgagtcaggtacccgaagtccagggccctctccaccgtctcgcagaagagcacgatgacctcctgctgcacgtagtactccctgggggacttcacaggcaccatggccgagacgtagctgagctcaaactctgcgaacaggacgtcgaagtgcctcagcgcttccctcatcttctctgtgtaggtgttcaggtcccgcagcgcctggtcacggagggcgccccgcacgtcctccaggctgcgcgtcagctccttggccagcgggcgcatggccatgctctccagctcccggttcatgatgatggagccggcggccaggcactcggcaccgaaccacagctggccggccaggttgtcgtgccggatctcctcagggaacttgacgcagaaatctctgggggcgcggtcctgggggatgcactcatccatgatctggttaatgatgttcaacacattgtcctgacaggagcggaactggctgaccagcagcgtgcaccgctgggggtccttccgcccatccaggctgtccagctccgcggccacctggttcagctcctcgtcggcatagtagaaccgggcaagcagctgcggatccgacctcttgggtttgtagagccactttcggaacctgttcatcatcgccgcgccggccctggccggactccgggcggccctcgccctccgcagcgctgcgcccgggcccggctgaggcgcggggcggacgcggaggcacggccggagcccccgcgctgtcgcagggaggctggctagcgaagcccggagcgccgagcgggcggcgggcaggtgcgcggggcaggtgcgcggccctgagtatgctctgcaagcggcgcgccgggcagacctcagacccgggagtgggcgctcgggcgcacggacagacgcgggcacgggggcgcgcggctcctcgctgctcactgacacccagcgctccgctggtcacggccgccccgcgccgcacatgcgcctagggcgccgcgagccccgggcccacc

SEQ ID NO: 12547 - RNA, 504 nt, Homo sapiens
  source 1..504: mol_type = other RNA
gagcaggcgaggctgggctgaaatactgggacaggttggagacgtcaagtccaagaacatccaagagctcggtccagactttccacagtgtctccacgaacatatccactcccagcacaaatctctcagtcagcctggccaagaacttctgagcggcgcgcacgttgtcctcgccgaacaggctgctgacgctctgggagaaggtgttgaccgtgcggcggtagctgttcttctccgcgccgccgcggccccgcgccccctgcgcgcccggggccagcagcccgagcagcagcagcagcagcagcagcagcaggagcccggcccgggccaggggcccgcctgaggcgcgcgcgcccatgctcggccggcggggcgcggggtcgcgatgcggggtgagggccgtgcgctgggccgcagcgggctccggctagggcaaggttggcgcgctcgggggccgcgcgccgcgcctttacccacagccgccgccgccgctgctgcgccacc

SEQ ID NO: 12548 - RNA, 289 nt, Homo sapiens
  source 1..289: mol_type = other RNA
gagcccctctctgctctccagagcattggcagtcagatgcatggtcacaagcagccgtgagacaggtagatctccacacctcaatcccccaggcccagggcttctatcttggggaaagtatgcgtgctcccgaaagggccttcccaagtcgtttcgccgcctgcagtgcccgaccgggggccgcgcgtccccggcaaccacgcccgcccgcgcagctgcagaggccggaaaaggcccgctcgcccgcgctcggcaccacccagcccgcgctccgggcgataccaccctg

SEQ ID NO: 12549 - RNA, 513 nt, Homo sapiens
  source 1..513: mol_type = other RNA
gagcccctctctgctctccagctccctggccagccggactgacttctgctcctcatggctgatgctgccttcgcccgtgggcagggatgccttggagtgcttggtggcagcctctctttccctctttgccacctggaagagcttatcctggatagcagcatgctcctgttcatacctcttgacaccctccttcatccctgagggctgctggccaccactgctccccgacctgggcagtgtggattctttgtgaggggctctcaagttgccatcttgaaggccaaaggtagaagatgtgggagcagggggtggagagctgggctccttcatgcggttcaccacgttttcagacagccggacaccctgcagcacccggacccgctcctcctcgtccactccgaaggacaccctgcggccctcgctgctctccgtgctccccatggcgagatgccgcagggccggcagccaccagacccgagacccggctccagagcaaccgggccaacaacgctt

SEQ ID NO: 12550 - RNA, 514 nt, Homo sapiens
  source 1..514: mol_type = other RNA
gagcccctctctgctctccagctccctggccagccggactgacttctgctcctcatggctgatgctgccttcgcccgtgggcagggatgccttggagtgcttggtggcagcctctctttccctctttgccacctggaagagcttatcctggatagcagcatgctcctgttcatacctcttgacaccctccttcatccctgagggctgctggccaccactgctccccgacctgggcagtgtggattctttgtgaggggctctcaagttgccatcttgaaggccaaaggtagaagatgtgggagcagggggtggagagctgggctccttcatgcggttcaccacgttttcagacagccggacaccctgcagcacccggacccgctcctcctcgtccactccgaaggacaccctgcggccctcgctgctctccgtgctccccatggcgagatgccgcagggccggcagccaccagacccgagacccggctccagagcaaccgggccaacaacgcttt

SEQ ID NO: 12551 - RNA, 481 nt, Homo sapiens
  source 1..481: mol_type = other RNA
gagcccctctctgctctccagctccctggccagccggactgacttctgctcctcatggctgatgctgccttcgcccgtgggcagggatgccttggagtgcttggtggcagcctctctttccctctttgccacctggaagagcttatcctggatagcagcatgctcctgttcatacctcttgacaccctccttcatccctgagggctgctggccaccactgctccccgacctgggcagtgtggattctttgtgaggggctctcaagttgccatcttgaaggccaaaggtagaagatgtgggagcagggggtggagagctgggctccttcatgcggttcaccacgttttcagacagctgtacagttcttcactcctccttccctgaagcccatgtcgcgaagctccaaggctgccagcctcgggctcgcgtctcggctcagcctcttcctggcctgagcccccggagtctcccaagccccacg

SEQ ID NO: 12552 - RNA, 604 nt, Homo sapiens
  source 1..604: mol_type = other RNA
gagcccctctctgctctccagctccctggcccaaggcagggagccaggcggctggaagattggagtgatggagcctttttattggatacctttggacttttgaatcatgtcaatgtattatcagccggactgacttctgctcctcatggctgatgctgccttcgcccgtgggcagggatgccttggagtgcttggtggcagcctctctttccctctttgccacctggaagagcttatcctggatagcagcatgctcctgttcatacctcttgacaccctccttcatccctgagggctgctggccaccactgctccccgacctgggcagtgtggattctttgtgaggggctctcaagttgccatcttgaaggccaaaggtagaagatgtgggagcagggggtggagagctgggctccttcatgcggttcaccacgttttcagacagccggacaccctgcagcacccggacccgctcctcctcgtccactccgaaggacaccctgcggccctcgctgctctccgtgctccccatggcgagatgccgcagggccggcagccaccagacccgagacccggctccagagcaaccgggccaacaacgctt

SEQ ID NO: 12553 - RNA, 516 nt, Homo sapiens
  source 1..516: mol_type = other RNA
gagcccctctctgctctccagctccctggcctgcagccggactgacttctgctcctcatggctgatgctgccttcgcccgtgggcagggatgccttggagtgcttggtggcagcctctctttccctctttgccacctggaagagcttatcctggatagcagcatgctcctgttcatacctcttgacaccctccttcatccctgagggctgctggccaccactgctccccgacctgggcagtgtggattctttgtgaggggctctcaagttgccatcttgaaggccaaaggtagaagatgtgggagcagggggtggagagctgggctccttcatgcggttcaccacgttttcagacagccggacaccctgcagcacccggacccgctcctcctcgtccactccgaaggacaccctgcggccctcgctgctctccgtgctccccatggcgagatgccgcagggccggcagccaccagacccgagacccggctccagagcaaccgggccaacaacgctt

SEQ ID NO: 12554 - RNA, 517 nt, Homo sapiens
  source 1..517: mol_type = other RNA
gagcccctctctgctctccagctccctggcctgcagccggactgacttctgctcctcatggctgatgctgccttcgcccgtgggcagggatgccttggagtgcttggtggcagcctctctttccctctttgccacctggaagagcttatcctggatagcagcatgctcctgttcatacctcttgacaccctccttcatccctgagggctgctggccaccactgctccccgacctgggcagtgtggattctttgtgaggggctctcaagttgccatcttgaaggccaaaggtagaagatgtgggagcagggggtggagagctgggctccttcatgcggttcaccacgttttcagacagccggacaccctgcagcacccggacccgctcctcctcgtccactccgaaggacaccctgcggccctcgctgctctccgtgctccccatggcgagatgccgcagggccggcagccaccagacccgagacccggctccagagcaaccgggccaacaacgcttt

SEQ ID NO: 12555 - RNA, 474 nt, Homo sapiens
  source 1..474: mol_type = other RNA
gagcccctctctgctctccagctccctggcctgcagccggactgacttctgctcctcatggctgatgctgccttcgcccgtgggcagggatgccttggagtgcttggtggcagcctctctttccctctttgccacctggaagagcttatcctggatagcagcatgctcctgttcatacctcttgacaccctccttcatccctgagggctgctggccaccactgctccccgacctgggcagtgtggattctttgtgaggggctctcaagttgccatcttgaaggccaaaggtagaagatgtgggagcagggggtggagagctgggctccttcatgcggttcaccacgttttcagacagctgtacagttcttcactcctccttccctgaagcccatgtcgcgaagctccaaggctgccagcctcgggctcgcgtctcggctcagcctcttcctggcctgagcccccggagtctccc

SEQ ID NO: 12556 - RNA, 7696 nt, Homo sapiens
  source 1..7696: mol_type = other RNA
gagcttattcataaaagtgcagacaacataaccagacacagcaaaacagacttcaatcagtagtccttgcatacaagaggcaagtccgctaagtgtacagccaactcttcatcctttaagggatctgaggatgggaaatttccagttcttaaaaactaagagtgagtgagtctcttttaaaaggcaatgctacaacctggttgggggcactatcatgttagatgggggaaaacaaaatagataatttgtttttcttcaataatggtctgtattttggtaaacagctcaaagatgacagcccaagttttgacattgctcttggagaaggctcttttctatctaagacaagagaacctcttcttccatcattataggagattcacacttatataccttaaatatattattttttgatttgaatacagaagacacttcacattgtgagcacaggacaaaatgcaggaccatataaatctccaaggaaaaagttaatgtgttggggcaaatctctacttgaatagtagtggctcagaagtggtggaaggtgcacaaagaacttactattagcaagcaagaagaggcaggtaaagggagaaagcccctcacccaataccaaatccttctctcccagtggccatttcctgttgattttacagttcaggagaatcttagatgctttagcagtaattcctttcttggctgttttgatcctcagcaaagtatataattattagtattaatggagtaaaaaaagtaagaggatcaatggtatcactactaagaaatacatatagaaagcacataaagattgtgtgatttattggttctttttcttatcatctttgcagaggaatcaccatcagtgttcttactttccatggttcatttctctctgcattacttatctcttattgcatcacaacacaaactcacagaaacactaactggctccttccccagcaccattttactgcattgcaacttatgattccaaattttacttaatgtcctctccactcacagaagtgctaagaggggattaaaaaggaaaagactgcatctaatgaccaccttctcataaacatcaacgcagagtactcattcttaagaaacacatgcattcttgccttaactgaggactgaaataacaaaaccaaacaaaaataacagaacttttaagtgccctgatggaaatgtacagtatgagttacatccatccatctatacacacatacagacactcatatgtatatacaatatatacatacaaatgataatagctataccaaaaatgtgcatatttaatacagttttaaaaagccagtagatcatggtataatacaatttatttccactagtgaatggcacaaatggagaaatgcaaaggaggtgtttcaagtacaatgaagtcatttttcacaggtgaaaataaatagtattattccagtgtccaacataatgtattctacaaaagtttaaaatgccagacatttagtacttacagaaatagaaagttactaaagtctgctttatggtctcaaaaagacactcatagagttttcaatttttgaaaagggggtgagaaaaaaattggtggaagcaggagggagtgtccaggatagtttctttagtgtactgaatgtttacctgatgtctaggcaaccaaaaatcatgactatgctaaaatgttccatttaccaacaaatccttgacctagagtactaagcatattacaccagtgtgtgtggcttcaaatacaagactctctatctctaggtattgaaatggcgaataagaattgcagctctgaaaatataatataaacacatttttcagatagcattatacaaataaaaatacttttggatactagaatttggggttagagctgacttcaataaggggaggaaaaaatatgtgcaaagggaagggagctcaatttggaataatatatttcaaagtatgtggctttgcatttttaaaatgctaaccaaaaaaaatgtgagatagagtgaccccaaggaactttttacagccagcctctggataccagatatagcatttacaacttctgatatgctagacaaattttccatagttttaattttcttaaagacatatagtgagtgaacaccaacactgggaaggaggtagtgttaatttgatcaaatattgatatttccccactgattcagaaagtgcttgctctttctctaggatatctcaaaacccttccaatttttctgctacaagctttactctatgatggttcctactatgtatgagattcctcagaagctagatctcacaaacatatacaaaccaattaatttgaatcattttttgcaaactgtatatactttaaagttaacttaatgataaaatccaggtatagtcatgacctacatgtaaaactggtggccaaatacattagatacaaaaccctactggagatctgaatggactcagtaactctcaatttgactaatttaagtccacaattggactttaaaatgtaccaccaataatattttgggtttgaaagagtttttgtatgcaaaagtgatctgcttccctattccacccatccagtagtacagagcagccagatctatgaataatttttaagggtatcaaattgtatttttgacattttattaaattctaaagctctctcgtcattttacaccaaataagtaatttctcaatttgttggaaacgctataatacctgaatgcaaaaaagatactgagacgactaaaagcccctttcactgatattacaagtacatgtcatgtcatgtttacctaaaaaccggtgacctggagcatgggctgaaagaacaacacataagagtgcttcttgaaacactgcctaaaattttgtgtgaactctatggtgatcttggttttaaaaacatttacattaaaacattaattttcttccagtttccttaaaatgaatcccagaaactcctacaggtgaggattcatggcaactcgactgacatacctgggaaagacttaaaatttggttgagaaaaccaggacttcaacagtgatagattgattactgtttggtcattagtttggtctaggcaaagagtgccattgagagggacttagagagttctaccttggagccctctgactataggaaaagcaggatccagagttagcagcaaggattcttcaagacaacttggaagggagcaggacaataacttgtaagaaactctgatttgtcactgaaaaggatatttttcttcaagtcatactcacagcttcctacccacctccaacacaatttatatacaagaaatggaaaaccaagaaaataactgactttttagcattgggttcatccttcattgtacaacaaaacataacaaaacaaaacatgtgccccctgaaaaataagagttagctttcgtcaagagattccctgaccactataacttattttactttttttttttaattggccaaacttcctagttccttttcagtagtactttagcactgaggcttgagacttgtggaagtggtgtttcctattgtgtgatgttaacttgatgccaaatggtcactaagtctcaacgaactagaagtttgtaaagtactgcagcaacgaaaacagcaattaaaaatagaggacctgcacatgcagcaaaatctacagtggtgatgaagattagtcagcagctggtaaagtcattggctcagtgactcctggttcactgtggcaactaaacatttaaataattggctattctacttgtaaacagaaaatcacataagccaaaaggagataacaattatgtctatgtagtgtgacgagaatttcaatagatggcaatttgcaaatatggcatcaaacacctccggcatttgatttgtattggctatatgtctttgtttttgtacaaacaaagtaaaagtactgtttggggtcttgggcattatagagcttagctaggatgagatatcacagtataagcaacaaaacgtcaggacacgtaagcttcatctcctcactctgctgcgggacatacccaccatatgaactttcagggcccctctcacccttctggtcttccccattgaaggctcataggtttgttaatgcaatcctcacacaacttgtgatctccttaagtacccccatcttatcataatacaaagaaggcacaattgaatggacaaaaatcactcacaagcctatgacgcattcaggaaaaaagaaaaactaagttgttttctactctctgaaaaaatcaatgaagtcctttagtgttcatggatttctacacttgatcttagccaaaaggccgagaagcaatgtgttcatggatttctgctttctttttttagtccaaatgaggctgagaagtcagatcaatttaataacaaataaatacactggtgaggcaatgcaggtgtgtaccagtaataacttatttcaacatatgctgcctgctgtgagtggctcataagaatttgggatatgggataaaaaggctttagatcttttcagaaacttcttaggatacagacacccaaaagtgataactgaagccattttgctacgttctatttttgcagtgttcagaaaaatcccctatctagccaattcttttcaccacatgcataatatatgtgtatgtgtgtgtatatatatgtacacacatacacatttatttttaatatcaactccacttttcaaaatttccccaaaaacaaacaaacccggcagccaagtactatgacatcccaattagtaaacacaaaacagaacgctttacaaaaatgaataaaatataccatatgcactcagcttccacactgtagtacccaagtgaggaggctgctgtgatgatgtctgtaggcagtttcttttggcagacagctccagcggaattgccactctcaattattaagttatgtataagacatgtgtgacccattggatatttgtgaagtgacactcgtgcttctgctcatgccctgctccgtccgtcccccagaagctgtccgcctcagagcctgggggctattgcggactcccatactgctacctcgaggtaccccttgcattggccctgaagggtgaccccatggctggggtccaccttgcattggatggccccaagcttgtggtgggccacccatgggatgaccccagtgaggtcctggacccccagtagggttgtgtgaccaaccagaagctcccgggtagctgtggctgaatgcctcaggggagagattagaaaggaccatattactaaaacctagtctcatgctttcagagtcaaaagcttcaatctctctggcttgacgttccaacaggcttcgtattcgttctgtgcgctcattctgcaaagccaacatctcttcttcaatcttttgttctaagagtgccctccggagggagaccctctgttcaagctcgcgaagctctcgatcatgttgtgcctcagcttgcatcttgattttgctctgatacgcattcaacagctccagttcctgctgcagctgcatcttcaaaacctggcactctgcttcctgtgcttcatccaaacgcagggcttgtgtggagagcatttcattaatgctgtgatcatactgctcagccaagatagctaatttccgggtctgttcctccttgagccgtttcagaacagctttgtgctcactctttggtgtagtctccagcaggtgatttcttaatgctttgtactgtctggtttggattttgcaggtatcctgaaactgcttttttatttggagttctttagactctttaagctgctcttttcgaagtttatactctcttttctgggactcgagaaaactattcagttctttcttctgttgggcctgaatatgttgctgaaattttttctcttcattggacatcactttagcctctttctccatggcagcctggtgtttcttgataagtttctccatttctgcagcaaaattgttacgctgagtttcaagatctttgtctaatctgaggcgatgttcatccatctcagcctttagcttgttttccagagtcatcagttgcttttgatgttgtcgcctcattcgcttatagccagacatttgttctctaagctcagagtcctgctcatgttcttgcatttgcctcgtaaccagtgatgctgtccgtatagtagcaaagtgttctcgattacgatagtgtgatttgtgacgagatacttggggtggagattgtggatctgatgctcttgttctaggatctccctcttctctgtaattttcttcctctggttttaaatggataacagaactgttagacatcactgtgtggtctccctccatcatgtctagctcactcttgtcatctgagacatctggaagactgttaacactactgctttggctgctggcactgatggacatgctgggaatggattgattacttccaacactattaactgttcctgtccggccaacaccatgatcttgttcctcttcttcttcctgtgcttctactgctggtccattatgtgcctcctggaaaaggagtttcttcatctttcgatactgcagattgtccagctctcttactgcatcctttgtcctctgaatgagatctattaacacggtttcagggcgctcccgaagaacaaatatgtgctttaaaagttcctctgatgtaggtcgatcttgagggattttctggaggcaagaatctacaaagttgcgaaaataatcagaccattcattagactgtagtgtaggggattcattttgggctatgtgatataaggcactcattgcattcatattaaataaaggaggcttcctttccgctagttcaatacatgttattccaagagaccacacatctactttgccatcatattgtccttcatccatggctaaaattacttctggggccatccaatacggcgttcccacaaaggaattggcaggtgatgccatggaagcagagccaaagtcagcaagtttcacctggcctggttctgtcagaaggatatttcctgctttgatatctctatgaatcatagtatgagaatgtaagtaggctaatccctgaagagcaccatgtgtaattgctgctatttccacttcttgtaatggctttttgtgaacttctagtaaatccgaagcagatcctaaacaatattccattacaagccatgctgtgtgttcacgtaaataacagcctttgtattctatactgttgggatgttttattctttgtagaaacttgacttccttaataatatcctgccatttctcagtagactgctttccactataagacattttcttgatggccaccacttcattggtacgcacatctcgtgcaaaatacactgctccaaagcttccatggccaatttctctgagatctgtgaagagcttctctggatcttctttgaagaagagctctgcaatttcagggtccttcaggctgcctgctctgttagttgatggcatcctgctgagcagtcagctgtcttgattctaattttatactgctatcccgatccttggttcatctgtatgaatgaagtcacgttggcataaactacctttcgccgacaggtctggggcggagcaggcaggcgcagccccctgcagcgctccggtagccgctaccctggagggtgaggagtgaggaggaggagggg

SEQ ID NO: 12557 - RNA, 8702 nt, Homo sapiens
  source 1..8702: mol_type = other RNA
gagcttattcataaaagtgcagacaacataaccagacacagcaaaacagacttcaatcagtagtccttgcatacaagaggcaagtccgctaagtgtacagccaactcttcatcctttaagggatctgaggatgggaaatttccagttcttaaaaactaagagtgagtgagtctcttttaaaaggcaatgctacaacctggttgggggcactatcatgttagatgggggaaaacaaaatagataatttgtttttcttcaataatggtctgtattttggtaaacagctcaaagatgacagcccaagttttgacattgctcttggagaaggctcttttctatctaagacaagagaacctcttcttccatcattataggagattcacacttatataccttaaatatattattttttgatttgaatacagaagacacttcacattgtgagcacaggacaaaatgcaggaccatataaatctccaaggaaaaagttaatgtgttggggcaaatctctacttgaatagtagtggctcagaagtggtggaaggtgcacaaagaacttactattagcaagcaagaagaggcaggtaaagggagaaagcccctcacccaataccaaatccttctctcccagtggccatttcctgttgattttacagttcaggagaatcttagatgctttagcagtaattcctttcttggctgttttgatcctcagcaaagtatataattattagtattaatggagtaaaaaaagtaagaggatcaatggtatcactactaagaaatacatatagaaagcacataaagattgtgtgatttattggttctttttcttatcatctttgcagaggaatcaccatcagtgttcttactttccatggttcatttctctctgcattacttatctcttattgcatcacaacacaaactcacagaaacactaactggctccttccccagcaccattttactgcattgcaacttatgattccaaattttacttaatgtcctctccactcacagaagtgctaagaggggattaaaaaggaaaagactgcatctaatgaccaccttctcataaacatcaacgcagagtactcattcttaagaaacacatgcattcttgccttaactgaggactgaaataacaaaaccaaacaaaaataacagaacttttaagtgccctgatggaaatgtacagtatgagttacatccatccatctatacacacatacagacactcatatgtatatacaatatatacatacaaatgataatagctataccaaaaatgtgcatatttaatacagttttaaaaagccagtagatcatggtataatacaatttatttccactagtgaatggcacaaatggagaaatgcaaaggaggtgtttcaagtacaatgaagtcatttttcacaggtgaaaataaatagtattattccagtgtccaacataatgtattctacaaaagtttaaaatgccagacatttagtacttacagaaatagaaagttactaaagtctgctttatggtctcaaaaagacactcatagagttttcaatttttgaaaagggggtgagaaaaaaattggtggaagcaggagggagtgtccaggatagtttctttagtgtactgaatgtttacctgatgtctaggcaaccaaaaatcatgactatgctaaaatgttccatttaccaacaaatccttgacctagagtactaagcatattacaccagtgtgtgtggcttcaaatacaagactctctatctctaggtattgaaatggcgaataagaattgcagctctgaaaatataatataaacacatttttcagatagcattatacaaataaaaatacttttggatactagaatttggggttagagctgacttcaataaggggaggaaaaaatatgtgcaaagggaagggagctcaatttggaataatatatttcaaagtatgtggctttgcatttttaaaatgctaaccaaaaaaaatgtgagatagagtgaccccaaggaactttttacagccagcctctggataccagatatagcatttacaacttctgatatgctagacaaattttccatagttttaattttcttaaagacatatagtgagtgaacaccaacactgggaaggaggtagtgttaatttgatcaaatattgatatttccccactgattcagaaagtgcttgctctttctctaggatatctcaaaacccttccaatttttctgctacaagctttactctatgatggttcctactatgtatgagattcctcagaagctagatctcacaaacatatacaaaccaattaatttgaatcattttttgcaaactgtatatactttaaagttaacttaatgataaaatccaggtatagtcatgacctacatgtaaaactggtggccaaatacattagatacaaaaccctactggagatctgaatggactcagtaactctcaatttgactaatttaagtccacaattggactttaaaatgtaccaccaataatattttgggtttgaaagagtttttgtatgcaaaagtgatctgcttccctattccacccatccagtagtacagagcagccagatctatgaataatttttaagggtatcaaattgtatttttgacattttattaaattctaaagctctctcgtcattttacaccaaataagtaatttctcaatttgttggaaacgctataatacctgaatgcaaaaaagatactgagacgactaaaagcccctttcactgatattacaagtacatgtcatgtcatgtttacctaaaaaccggtgacctggagcatgggctgaaagaacaacacataagagtgcttcttgaaacactgcctaaaattttgtgtgaactctatggtgatcttggttttaaaaacatttacattaaaacattaattttcttccagtttccttaaaatgaatcccagaaactcctacaggtgaggattcatggcaactcgactgacatacctgggaaagacttaaaatttggttgagaaaaccaggacttcaacagtgatagattgattactgtttggtcattagtttggtctaggcaaagagtgccattgagagggacttagagagttctaccttggagccctctgactataggaaaagcaggatccagagttagcagcaaggattcttcaagacaacttggaagggagcaggacaataacttgtaagaaactctgatttgtcactgaaaaggatatttttcttcaagtcatactcacagcttcctacccacctccaacacaatttatatacaagaaatggaaaaccaagaaaataactgactttttagcattgggttcatccttcattgtacaacaaaacataacaaaacaaaacatgtgccccctgaaaaataagagttagctttcgtcaagagattccctgaccactataacttattttactttttttttttaattggccaaacttcctagttccttttcagtagtactttagcactgaggcttgagacttgtggaagtggtgtttcctattgtgtgatgttaacttgatgccaaatggtcactaagtctcaacgaactagaagtttgtaaagtactgcagcaacgaaaacagcaattaaaaatagaggacctgcacatgcagcaaaatctacagtggtgatgaagattagtcagcagctggtaaagtcattggctcagtgactcctggttcactgtggcaactaaacatttaaataattggctattctacttgtaaacagaaaatcacataagccaaaaggagataacaattatgtctatgtagtgtgacgagaatttcaatagatggcaatttgcaaatatggcatcaaacacctccggcatttgatttgtattggctatatgtctttgtttttgtacaaacaaagtaaaagtactgtttggggtcttgggcattatagagcttagctaggatgagatatcacagtataagcaacaaaacgtcaggacacgtaagcttcatctcctcactctgctgcgggacatacccaccatatgaactttcagggcccctctcacccttctggtcttccccattgaaggctcataggtttgttaatgcaatcctcacacaacttgtgatctccttaagtacccccatcttatcataatacaaagaaggcacaattgaatggacaaaaatcactcacaagcctatgacgcattcaggaaaaaagaaaaactaagttgttttctactctctgaaaaaatcaatgaagtcctttagtgttcatggatttctacacttgatcttagccaaaaggccgagaagcaatgtgttcatggatttctgctttctttttttagtccaaatgaggctgagaagtcagatcaatttaataacaaataaatacactggtgaggcaatgcaggtgtgtaccagtaataacttatttcaacatatgctgcctgctgtgagtggctcataagaatttgggatatgggataaaaaggctttagatcttttcagaaacttcttaggatacagacacccaaaagtgataactgaagccattttgctacgttctatttttgcagtgttcagaaaaatcccctatctagccaattcttttcaccacatgcataatatatgtgtatgtgtgtgtatatatatgtacacacatacacatttatttttaatatcaactccacttttcaaaatttccccaaaaacaaacaaacccggcagccaagtactatgacatcccaattagtaaacacaaaacagaacgctttacaaaaatgaataaaatataccatatgcactcagcttccacactgtagtacccaagtgaggaggctgctgtgatgatgtctgtaggcagtttcttttggcagacagctccagcggaattgccactctcaattattaagttatgtataagacatgtgtgacccattggatatttgtgaagtgacactcgtgcttctgctcatgccctgctccgtccgtcccccagaagctgtccgcctcagagcctgggggctattgcggactcccatactgctacctcgaggtaccccttgcattggccctgaagggtgaccccatggctggggtccaccttgcattggatggccccaagcttgtggtgggccacccatgggatgaccccagtgaggtcctggacccccagtagggttgtgtgaccaaccagaagctcccgggtagctgtggctgaatgcctcaggggagagattagaaaggaccatattactaaaacctagtctcatgctttcagagtcaaaagcttcaatctctctggcttgacgttccaacaggcttcgtattcgttctgtgcgctcattctgcaaagccaacatctcttcttcaatcttttgttctaagagtgccctccggagggagaccctctgttcaagctcgcgaagctctcgatcatgttgtgcctcagcttgcatcttgattttgctctgatacgcattcaacagctccagttcctgctgcagctgcatcttcaaaacctggcactctgcttcctgtgcttcatccaaacgcagggcttgtgtggagagcatttcattaatgctgtgatcatactgctcagccaagatagctaatttccgggtctgttcctccttgagccgtttcagaacagctttgtgctcactctttggtgtagtctccagcaggtgatttcttaatgctttgtactgtctggtttggattttgcaggtatcctgaaactgcttttttatttggagttctttagacttcaaactcttaggctgttgtcgaacttccatgacatgctttcgtcttagttctcgttctcttcgcttattatattccagctggttagtgagctcagtttgatgctgtaatctgatcaactcacagcgcatcttctgaattgtgttgaggtggcggaactccagttcttgcatagattcatgctgtcggagtagcatggcatgctctaagtccttctgagtctgtcttttgtttaactcctccctgacaaggtcctgctctaagttatgacgcccaagtaacattcttctcttgaagcgacggcattccagctctaggtattgtctttgacgtcgaagaaggttagcttcttcttctgcttggaaatgctgtatattctccttctgctttgaaagccactcctgtttttcttttttgggggtactctggttttcatttagctcctctttaagctgctcttttcgaagtttatactctcttttctgggactcgagaaaactattcagttctttcttctgttgggcctgaatatgttgctgaaattttttctcttcattggacatcactttagcctctttctccatggcagcctggtgtttcttgataagtttctccatttctgcagcaaaattgttacgctgagtttcaagatctttgtctaatctgaggcgatgttcatccatctcagcctttagcttgttttccagagtcatcagttgcttttgatgttgtcgcctcattcgcttatagccagacatttgttctctaagctcagagtcctgctcatgttcttgcatttgcctcgtaaccagtgatgctgtccgtatagtagcaaagtgttctcgattacgatagtgtgatttgtgacgagatacttggggtggagattgtggatctgatgctcttgttctaggatctccctcttctctgtaattttcttcctctggttttaaatggataacagaactgttagacatcactgtgtggtctccctccatcatgtctagctcactcttgtcatctgagacatctggaagactgttaacactactgctttggctgctggcactgatggacatgctgggaatggattgattacttccaacactattaactgttcctgtccggccaacaccatgatcttgttcctcttcttcttcctgtgcttctactgctggtccattatgtgcctcctggaaaaggagtttcttcatctttcgatactgcagattgtccagctctcttactgcatcctttgtcctctgaatgagatctattaacacggtttcagggcgctcccgaagaacaaatatgtgctttaaaagttcctctgatgtaggtcgatcttgagggattttctggaggcaagaatctacaaagttgcgaaaataatcagaccattcattagactgtagtgtaggggattcattttgggctatgtgatataaggcactcattgcattcatattaaataaaggaggcttcctttccgctagttcaatacatgttattccaagagaccacacatctactttgccatcatattgtccttcatccatggctaaaattacttctggggccatccaatacggcgttcccacaaaggaattggcaggtgatgccatggaagcagagccaaagtcagcaagtttcacctggcctggttctgtcagaaggatatttcctgctttgatatctctatgaatcatagtatgagaatgtaagtaggctaatccctgaagagcaccatgtgtaattgctgctatttccacttcttgtaatggctttttgtgaacttctagtaaatccgaagcagatcctaaacaatattccattacaagccatgctgtgtgttcacgtaaataacagcctttgtattctatactgttgggatgttttattctttgtagaaacttgacttccttaataatatcctgccatttctcagtagactgctttccactataagacattttcttgatggccaccacttcattggtacgcacatctcgtgcaaaatacactgctccaaagcttccatggccaatttctctgagatctgtgaagagcttctctggatcttctttgaagaagagctctgcaatttcagggtccttcaggctgcctgctctgttagttgatggcatcctgctgagcagtcagctgtcttgattctaattttatactgctatcccgatccttggttcatctgtatgaatgaagtcacgttggcataaactacctttcgccgacaggtctggggcggagcaggcaggcgcagccccctgcagcgctccggtagccgctaccctggagggtgaggagtgaggaggaggagggggcccggcgacagatcgccgccccccacccccgagccccagcaagccgcccagcccaagctctgcaacaaggggcggcggcggcggggggtgggggggggggcgaggggacgaccggggtcgaggaggcgccctcagcgcttgggctcagttaagatggcgcggggaagtgccgggagccgtctccgtcgccgcctcgggggaaccggcccgggcctcggccgcctctagtcctcacacagccgaggccctctcggtcccccgccgcggcccctcggcgggcgggcccacgcgcagccctccgccaccaacaccacccctggtaaggaggcgctcacaaagggaagagaggccgcgggccggccggcggacggcggggcggggtcccccggggccgggaggcctcagatgttcgcgagtgcctagtgctttcggcccgcgaagggcgcagggcgagcgggacccctcctctctcctcaggcaggcggcggcaccgactcagtctctttgccaccctccctctctctccccgagccctgaagccacagagcccggccgctgccc

SEQ ID NO: 12558 - RNA, 432 nt, Homo sapiens
  source 1..432: mol_type = other RNA
gagcttggatgagctgggctgagcacaaagcccagtccagaaccattgtcatttcagattccatccttccggccagacttctcgaatatcatgtggaaacacagaattcaaatcacagtgtcagagcagaaaacacccttataaatcaaccccttcgctgaagagatggaagacagagattccaagaggggacgggaccagcccaggtcactcaggaagttggtgacaagttaggactcgaacccaggtttctcgtcacgtaattcaggaaaccttccagatcagaggaatgcacagcgggagtctctggagtccacaggtcaatggcgcagcagcctctctccaggctttgggctgcaagccgggctgggtgctgggtgctcagggctctgccagctgccagccctcgctgcagcttccctgccgttctct

SEQ ID NO: 12559 - RNA, 442 nt, Homo sapiens
  source 1..442: mol_type = other RNA
gagcttggtctgtagcggtttccttcggggcaggtggggactgctcctttgggaggaaggaggaggcccaggccgcgtcttcaggcagctgcgcgcaccacccgaaggtgaggcatttggccccaaacagaccctcgaaaagccggactgatcgaggagttaccctacagcctgatctgcacctgctccagggagagagcgccccacccttcccgtggcgtggggtgagacccagcgttggataacgtgtggtcgggccgagcaaatgtttgatgaatgaatgaatgaatgaatgcctctctcacgtggcactcgtgaagctcagaggatatggtggaagtgcaagcgctttgtaaactgcagtgcattgtaaaaatgagttgtaatacattcctcccctccccctagccatgaaaggaaacaggggtgcggcttgagtaca

SEQ ID NO: 12560 - RNA, 1917 nt, Homo sapiens
  source 1..1917: mol_type = other RNA
gaggcagaagcaggatgacaaatggagctccgatctgaagggtccaggcaagcctccattgaaaccaaggcaggtccctgatactccaggtcttagtgggtgtagacaagcagggtcctaggcccaggaatgtcaagcattggacaggagtctataatttgctttccatctagcagaatagtcaataaatgagaaaactgtgctccagtcattcactcaagaggttggaaatggctttgtattagttgtctatttgctgcctaacaaattgcctcaacacttagtagcttaaaacaataataatttacctctcacagtttccatggctcataaattcagacagggcacatcacagtgaggatggcttgtccttgctccactatgtctggggtcatggctggaagaagcaaaggctggggctggcattatctgaagactcattcactcacacgcctgactgttgatgctgactacaggctgaaggcccagcagggacagttggccagacaccagcgtcagcctctccacgcagcctgggcttctgcagagtatggtggctgtccaagggccaggctccctgcatgagcattagtttcctcatcctgtaaacgtgaatgataatagcagccatggcatagggtttgcacgggagttaagtgagatcattcatgtactgtgcagtgccgacacttcgtgcattatcttcaaggtggttgttgctatctatcctgttaccagctgtcccccaactccaccgcctctaaagaagatgcgagccctgcctgttcagttgtcttcctctttctgaagcttggagagatccagccttgctaggggagtttctggagcttttcccaaacatggcggttactgctgccttcttgcccttgccccacatgttcctggcaacgtccgccacatatccccacatgcgtagaacgtcacagcgccctgcatttgcatattaaaaggctaggaagggagggccagctttttccctgctacgtgaataaaacatgcctggtcaaaccaatccgctaagccctgtgcaaatcagatcgcctcctccggcctctgcatgtatacctggctggcgtccaccacacttggggccctcctctttcggctttggagcccccctccctctgtctctgtaaggggaagcctctaagttctgccttctttcttgcctattaaactctccgctctttaaaaccactccacgtgtgtcagtgttgttttacctaattcaaggtaagacaagagccctggtgtccctccactcatgggagccgtatcagcagtgagccgagatcacgccactgcactaccgccttggtgacagagcgggactccgtctcaaggaaaaaaataaaagacactagctatcaagccatgacaagacatggaggcaccttaagtggggatattaaccaagtgaaagaagccaatctggcaagtccaccgcgccctgcctgccttcctcctttctggtcatcaaactgtttgcttctaacagtgcccagtgagtaggattctattgagtgccaggtgtaggaggagagatgccagcaggaaaaaggagaagcaatgctggctgcttcatggtacctgttagcttgaaaacacaaagatgctctccctgcgtcttgtttgacaagcgatcggcgggaggcgcgcttgttggcatgaacaggaaccactgcctgctttccttgacatggaagagcatgaacttctttgagcagatctgtgtggcaatgtcaccctgaaatgaaagtgcccggagggtcacaggacaccctgctgaggatagaagagccagtaatcccagggctatggaattgaacagcagagcagcccagcgataatggaggggaaatgtcacagaggccctgaaaagaaccctgtgccttt

SEQ ID NO: 12561 - RNA, 2413 nt, Homo sapiens
  source 1..2413: mol_type = other RNA
gaggcagaagcaggatgacaaatggagctccgatctgaagggtccaggcaagcctccattgaaaccaaggcaggtccctgatactccaggtcttagtgggtgtagacaagcagggtcctaggcccaggaatgtcaagcattggacaggagtctataatttgctttccatctagcagaatagtcaataaatgagaaaactgtgctccagtcattcactcaagaggttggaaatggctttgtattagttgtctatttgctgcctaacaaattgcctcaacacttagtagcttaaaacaataataatttacctctcacagtttccatggctcataaattcagacagggcacatcacagtgaggatggcttgtccttgctccactatgtctggggtcatggctggaagaagcaaaggctggggctggcattatctgaagactcattcactcacacgcctgactgttgatgctgactacaggctgaaggcccagcagggacagttggccagacaccagcgtcagcctctccacgcagcctgggcttctgcagagtatggtggctgtccaagggccaggctcctgaaagagggccaggcagaaacttcatgctttttataaccttgggagtcacagagtatcatttctgccccattatgtttgttataatacataacactaagtcctacccatatttaagagaaagagaaatagcttccatctttagatgggagaagggttaaagaatttgtggacctattttaaaaccaccataggcctcatagttacatggattttgacaaatagggacatttaagggtgacaaataagggcatttaaggttgctctcatattccgttttctttgcaaaactaagatgctgaaatttgaagaagatacagattgaaagaccttaagactttagcttttatgatgccatgccacctccagcctaggcacgtaagaaggaggtaagaggactcatttaggctcccgccagcagttcccaaagggctccctcccagagaggaattaaatatgctctgatgattatgatgtagggaagggaggctttcaccctgcatgagcattagtttcctcatcctgtaaacgtgaatgataatagcagccatggcatagggtttgcacgggagttaagtgagatcattcatgtactgtgcagtgccgacacttcgtgcattatcttcaaggtggttgttgctatctatcctgttaccagctgtcccccaactccaccgcctctaaagaagatgcgagccctgcctgttcagttgtcttcctctttctgaagcttggagagatccagccttgctaggggagtttctggagcttttcccaaacatggcggttactgctgccttcttgcccttgccccacatgttcctggcaacgtccgccacatatccccacatgcgtagaacgtcacagcgccctgcatttgcatattaaaaggctaggaagggagggccagctttttccctgctacgtgaataaaacatgcctggtcaaaccaatccgctaagccctgtgcaaatcagatcgcctcctccggcctctgcatgtatacctggctggcgtccaccacacttggggccctcctctttcggctttggagcccccctccctctgtctctgtaaggggaagcctctaagttctgccttctttcttgcctattaaactctccgctctttaaaaccactccacgtgtgtcagtgttgttttacctaattcaaggtaagacaagagccctggtgtccctccactcatgggagccgtatcagcagtgagccgagatcacgccactgcactaccgccttggtgacagagcgggactccgtctcaaggaaaaaaataaaagacactagctatcaagccatgacaagacatggaggcaccttaagtggggatattaaccaagtgaaagaagccaatctggcaagtccaccgcgccctgcctgccttcctcctttctggtcatcaaactgtttgcttctaacagtgcccagtgagtaggattctattgagtgccaggtgtaggaggagagatgccagcaggaaaaaggagaagcaatgctggctgcttcatggtacctgttagcttgaaaacacaaagatgctctccctgcgtcttgtttgacaagcgatcggcgggaggcgcgcttgttggcatgaacaggaaccactgcctgctttccttgacatggaagagcatgaacttctttgagcagatctgtgtggcaatgtcaccctgaaatgaaagtgcccggagggtcacaggacaccctgctgaggatagaagagccagtaatcccagggctatggaattgaacagcagagcagcccagcgataatggaggggaaatgtcacagaggccctgaaaagaaccctgtgccttt

SEQ ID NO: 12562 - RNA, 359 nt, Homo sapiens
  source 1..359: mol_type = other RNA
gaggctgagctgaggagtgaacgtaaaggcagtcttcactcccaggcttttgtccttctacccctctctcatcttcccctagctgcctccacctcttccactgccttccactctgagcctctaaaatggggcctctggccccactgtttctgaggaatctgggtgactggtgtgcagctgagaatctgtctccaaaggcaaagccagggtccaggctttgaggcctggagctgccactgactggctttgtgatactgggtgagattctcaacctctctgagtgctgttggatgggagccttcctgtgtagactctgaagaactgaagagatttgaggaggtctcctttacccgattaga

SEQ ID NO: 12563 - RNA, 6647 nt, Homo sapiens
  source 1..6647: mol_type = other RNA
gaggctgagctgaggagttcagaagctgtgatctgtcgtctaattccttggaaccacaggtgtttgttgctggtttcctgcttctcgatcaactctaagatgagctgcgctaccgtctgcagtgcccgtctggtgtgtgttctatacatcctcaccagctggagcttcttctcctctgtcacgtattcggaattcagtagtgcccacagtgttggtttctggcctctgaaccttcccactgtgatttccacttgctctgcctccagggcccttctcgtctcgtcatcgatgtgctcggagtcccgtgcagccttgttcactgggaacagcagccagcccgtgtcctcttgtgggcggcacctctcctgcagctctcggtacgagaccttctcttgcgtgttcgggtccacaaaccgtttcctcatgtgcttctggtcggaaatgagcgcatagatgtccttgtgcagacagccccgtctgtaggctgtttccagtgggagccggtggtggtgctgtgggtcgatgacaccccccgtggccacctgcacctccagcagcctcagtgcctccgccttctcgatgagctgcttctgcatggcctggaacagcgggatcgtgtctcctgtggccggatccctgtagcccgtggcagctctttcagccttcaggagcctctcccgcagctcctcgttcaccaggcccacatccacagcctcatccacagagagcttctggcgggtgcaggggtccaggaggaacccggtggcggcctgcgcctccagcagccaagtcgcaaatgctgcagggatgagctccttcctgctggcctcatggaggctcatgacctccctggtggagggcaccgtgacccccgcaatgcagccgctgccttccagatagggcttcacacactccagcgtgctgagtgcctgtcccccagtcctccccacacgaagtgtgtgcagggtcttctgatcgatgaccctggagttgaacaggtctgcagctgtcacctcccctctgatggccgccactttgatgccttggttttgcgtctctgtttcttcaattgtcgtggtgatgatttccagcaatttctccaggcccccactctgggctccatactcctggatgagctcccgcttcctgtcctctgtgaagtatggagaggacagcaggtcccagaaagagaccacctggtcagcaaacctccccacgcgcatttttgcagttctggattgcaacacgtgtctcgtggcctcattgatgtacacgtagttttctcctttctttatgatttgtagcaggtacaggcccgtctcggggtcctccacacagcgctccagaagctgcaggtacgtgaggttctcgtgcgtgttggggtcgaagaagcccttggtgtcgtcgctggggtccgccaggatgcggttcatctcctcgtcgaagtagccgcagcggtaggccacgtccacgggcacgcggtggctgtgcacggggtcgatgatgccgcccgtggcgatctgggcctccagcaggcggatgccgtgctcccggacgatgaggtccttctgcatggcctggaagagggagatctgctgcccggtataggggtcggtgtagccggtgacggcgcgctcggccgacagcagcttcacgtaggtttctttcccgaacattcctgctttgaacgcctcctccacggtcagcttccggttctccacggggtcgatgatgaagccggtagctgcctgtgcctccagcagcaccagggctgtgccaggccgcaggatgtgcctcctcagggcctctgggatgctcatcctctcctgggtgccctggataaggaccccggcaatgaagttgcctccctccagggaccgcttcacgctgtccatctccgccacctccttcacagtcgttgtcccctggctcagctcgtccagcgtcttcctgctgatcagctgcgccctgaacaggtccctggctgacacctgcttccggagccctctgaaggtggcctgcaggggctgcctctctgcagcctcgaccagggtggtgactgcgctgaccacctgccgcagggccgcagccctcccagaccgacagagtgccaccagctcccgccgcttgtcagcgccaacgtattcggagagcagcaggtcccagagtgacacgctacaccccttaaacctccctgtgctgacgggcaccttcatggccctcagagccaccgcggtgtggtcgtccacctcaagcactgtgtctgagggcagtggcaacagcaacaatccggtctcggagtcgcacacgcagcgctccctgagctgctggtaggtcacctggtcccgcgcactggggtcaaagaagaacttgttgtccttgtcaactgcagtcagcacctggctcgtctgtgtgtccagaaggccgagtctgcaggctgccgcctggggcaggtgcaccccgtggacagggtccaccacaccccctgtggccagctgcacctgcaggaggggcaagccctcgttctgtggcacgagccccttctccatggcctgccacagagagagggaggccctagagtagggatctgggtacccggccgccgccctctcggcctgcccgagctgctcactcagctccctgcccaccaggccgaccttaaccgcgtcctccactgacagtctctggttgttcagggggtcaacaaggaagccagatgccacctgggcttccagcagcctctggcccaggcctgtgggcaggaggccatccctcacggcctgggcgatgctggccttggccccagagggctgtagcagcacaccggccacgcagcctgtgccccacaggcaggccttcaccgccggctgctcggcgacctgggcgggcgactgcgtgccctgagccagggcctcaagggtctcctgggtgatgatgccagcatccagcagccagacagcgggtacctcaccccgtgggccgggcaccatgacgcgggcctgggccaggagcttggtctcctgtacccacctctgcacagaggctagcagctgtggcacagtggtcctcccctcctgcacgtcctccagcaggcccctccgttgctcctcggtgaagtggcaggagctgagcaggtcccagagggatgtgccatccttggcccccggcacggcctgcaggctcctctggacctgctcctcggtggggagggcaggagcactttctggcaggggcaggaggtgaaggccagaagtctcatccctggggcactcctccaggagctgggcatagctcgtgcgcccctggccgtccggtgtggggaaggtttcggaggagctggacaaggctgtctccatctcctggtcaacatagccacgctgaatggccactggcatggggaggtggtggtggctggtggggtcaatgatccctcctgtggccacttgagcctccaggaggcgggcagcttgctcccaagggatgagacctttcttcatggcctggaacacagacacctgcttcccagagaaggggtctctgaagccagcaatggcaccctcagcccgcttcagcctgccatacagctccggccccaccacacccctgcgcacggcctcatccaccgagaggctctctgggctgtgagggtccatgatggttccggtggccgcctgggcctccagcagggccagggccaccctgggccccagcagcttctgcctcatggcctggtagaggctgagccgctggccagagggcagcagccgcacaccgcccacagctcccaggccgcacaggtacctgcggacgccgtccatgagtaggagggcctccgggctgattgtcccggccagcacttggtccaacagctgctggtcaatgataccggcctccaggagctggtggacggtgacccggctccgcagtgcgggcagcatgatgtccgcctgtctctgcgtctccgcctccagcagctttgccacctgccccagcgtgacctcgcgctgccggtagcgacgcagcagctgcctcctgcggccctcgctgaagtactcagagttgatcagctcccacgcggagaccctctgcccctgaaaccgtccatacttcacggagagcagcaggttctggaaggcctgctgggtggcactgtccaccagcggggactgcgtgctgctgagtggcaggaggtacaggcccgtctcggggtcacgcacacagcgctccagaagctgcaggtacgtgaggttctcgtgcgtgttggggtcgaagaagcccttggtgtcgtcagaagggtccaacaggatcaagttcagcatctgatcgaagtagccgcgccggtaggccacgtccacgggcacgcggtggctgtgcacggggtcgatgacgccgcccgtggcgatctgggcctccagcaggcggatgccgtgctcccggacgatgaggcccttctgcatggcctggaagagggagatctgctgcccggtgtaggggtcagtgtagccagtgacagcgcgctcagccgacagcagcttcgcgaacacatcaggcccaatgacagcagccctcagtgcctcctcaacggagtgccccttgtttgcttttgggtcgatgatgaagcctgtggcagcttgtgcctccagaaggatgagggcagtgccgggccggaggagccccttgcatcgggcctcatagatgctcaggcgttcctgggagccagggagcagcaggccagcaatgcagcccgtaccctgcaggtacctctgcaccgaggccaggctgcccacatccttggctgtggcctgtccatgctccagccgctcgtacaggtcctggtcgatgatctcggctttcagcagctctcctggtgtcacggtgtccctcagcccagaaaaggtgaccctggcagtggctgcagcctgctcgagggtggcgctcagcttagcggccagcttctccacggagagggtcccttcctggtactgctgggccagcatcgccctctgctctgaggagatggcctcagagaagagcagctcccagagggacacgggccggccccggaacttccccacagagacggtggctgtggccgtgctcagggcctgccgagtgctgtacttgatgaatgggggtccctggggctcccctccccggggtccccctgagagtggcaggaaggcaagcccggtctctgggtcggtgacacagagggccagcagctgttcatagcgcaggccgccgtgcgtgccgtctgagaagctgccagcctgcgagagctgccgctgagtgtcttcatccaggcagccgcagcgcagggcggcctccaggggcagccggagcctgcgtgctggacagaccagcccgcctgtggccagctgggcatccaagagccgcagtgccagtggcctgtccactagccccttcttcatggcctggaaaagggggatttgggagccactgaaggggtcgtggtgccctgtcacggcctgctcggccaccaggagctgctcatggagctctgggctgaccaggcccgccctgactgcctcgtctacccacagccgctggcctgtgatggggtccaccagggtgtgggtggcagcctgggcctctaggagtggcagcgcggtgcccattgggagcaggtgctcggtggcagcctggaaaaagctcttcttgtggccttcgggcagcaggacaaccccggccacgctgccggtaccctccaggtagcgccgcacctcggcacgtgcactcacgtccactgcggccagcctgccctcccgcagaccctgcacagcctgctcgtccaggatgcccacctccagcagctcagctgcactcaccgccccgcccatggagcggaaggtgatcttgaggggcagcaaggctagccccgagccgggggcacgcacacacctttccagcagctggtggtatgtcagccgctccagcgtgttggggtcgaggaagcgcaggtcacctgtgccaggctcaagctctgacagcttgtgccatgtctcccggtccaggaggccctggtggcaggctggctcaggggccacgagcactccctgggcggggtccaccaggcccccagtggccagttggacctccagccagctctgccccagggccctgtccacaacctccttcccgatggcctgaaagagggccagcttctcaccgccgtaggggtcaggatagcccgtagtggcacgctcagcggccagcagcttctccttcagctccagccccaccagaccctgctgcagggccttggacacagggagcagctggccccgggcgaggtccaccaggcccccagtggctgcctgggcctctagcagagcctgcccgagcccagcaggcaggaggccctgctccatggcggcgtagacactctgggcctggcccgaggcctccacatacaccccagctatgctcctggcctggggcctggggggcgtgccggctcccagcgtggctgccatggctctgggtacactggcctgctctgtgctgttggtgcctgggacgggaagaggaggcaaggtgtggccactcatcacacacggctggttatgcagagcctgctgaggtccacctctgtcctgcccgctcgccgctcggtccgcagtgtc

SEQ ID NO: 12564 - RNA, 6676 nt, Homo sapiens
  source 1..6676: mol_type = other RNA
gaggctgagctgaggagttcagaagctgtgatctgtcgtctaattccttggaaccacaggtgtttgttgctggtttcctgcttctcgatcaactctaagatgagctgcgctaccgtctgcagtgcccgtctggtgtgtgttctatacatcctcaccagctggagcttcttctcctctgtcacgtattcggaattcagtagtgcccacagtgttggtttctggcctctgaaccttcccactgtgatttccacttgctctgcctccagggcccttctcgtctcgtcatcgatgtgctcggagtcccgtgcagccttgttcactgggaacagcagccagcccgtgtcctcttgtgggcggcacctctcctgcagctctcggtacgagaccttctcttgcgtgttcgggtccacaaaccgtttcctcatgtgcttctggtcggaaatgagcgcatagatgtccttgtgcagacagccccgtctgtaggctgtttccagtgggagccggtggtggtgctgtgggtcgatgacaccccccgtggccacctgcacctccagcagcctcagtgcctccgccttctcgatgagctgcttctgcatggcctggaacagcgggatcgtgtctcctgtggccggatccctgtagcccgtggcagctctttcagccttcaggagcctctcccgcagctcctcgttcaccaggcccacatccacagcctcatccacagagagcttctggcgggtgcaggggtccaggaggaacccggtggcggcctgcgcctccagcagccaagtcgcaaatgctgcagggatgagctccttcctgctggcctcatggaggctcatgacctccctggtggagggcaccgtgacccccgcaatgcagccgctgccttccagatagggcttcacacactccagcgtgctgagtgcctgtcccccagtcctccccacacgaagtgtgtgcagggtcttctgatcgatgaccctggagttgaacaggtctgcagctgtcacctcccctctgatggccgccactttgatgccttggttttgcgtctctgtttcttcaattgtcgtggtgatgatttccagcaatttctccaggcccccactctgggctccatactcctggatgagctcccgcttcctgtcctctgtgaagtatggagaggacagcaggtcccagaaagagaccacctggtcagcaaacctccccacgcgcatttttgcagttctggattgcaacacgtgtctcgtggcctcattgatgtacacgtagttttctcctttctttatgatttgtagcaggtacaggcccgtctcggggtcctccacacagcgctccagaagctgcaggtacgtgaggttctcgtgcgtgttggggtcgaagaagcccttggtgtcgtcgctggggtccgccaggatgcggttcatctcctcgtcgaagtagccgcagcggtaggccacgtccacgggcacgcggtggctgtgcacggggtcgatgatgccgcccgtggcgatctgggcctccagcaggcggatgccgtgctcccggacgatgaggtccttctgcatggcctggaagagggagatctgctgcccggtataggggtcggtgtagccggtgacggcgcgctcggccgacagcagcttcacgtaggtttctttcccgaacattcctgctttgaacgcctcctccacggtcagcttccggttctccacggggtcgatgatgaagccggtagctgcctgtgcctccagcagcaccagggctgtgccaggccgcaggatgtgcctcctcagggcctctgggatgctcatcctctcctgggtgccctggataaggaccccggcaatgaagttgcctccctccagggaccgcttcacgctgtccatctccgccacctccttcacagtcgttgtcccctggctcagctcgtccagcgtcttcctgctgatcagctgcgccctgaacaggtccctggctgacacctgcttccggagccctctgaaggtggcctgcaggggctgcctctctgcagcctcgaccagggtggtgactgcgctgaccacctgccgcagggccgcagccctcccagaccgacagagtgccaccagctcccgccgcttgtcagcgccaacgtattcggagagcagcaggtcccagagtgacacgctacaccccttaaacctccctgtgctgacgggcaccttcatggccctcagagccaccgcggtgtggtcgtccacctcaagcactgtgtctgagggcagtggcaacagcaacaatccggtctcggagtcgcacacgcagcgctccctgagctgctggtaggtcacctggtcccgcgcactggggtcaaagaagaacttgttgtccttgtcaactgcagtcagcacctggctcgtctgtgtgtccagaaggccgagtctgcaggctgccgcctggggcaggtgcaccccgtggacagggtccaccacaccccctgtggccagctgcacctgcaggaggggcaagccctcgttctgtggcacgagccccttctccatggcctgccacagagagagggaggccctagagtagggatctgggtacccggccgccgccctctcggcctgcccgagctgctcactcagctccctgcccaccaggccgaccttaaccgcgtcctccactgacagtctctggttgttcagggggtcaacaaggaagccagatgccacctgggcttccagcagcctctggcccaggcctgtgggcaggaggccatccctcacggcctgggcgatgctggccttggccccagagggctgtagcagcacaccggccacgcagcctgtgccccacaggcaggccttcaccgccggctgctcggcgacctgggcgggcgactgcgtgccctgagccagggcctcaagggtctcctgggtgatgatgccagcatccagcagccagacagcgggtacctcaccccgtgggccgggcaccatgacgcgggcctgggccaggagcttggtctcctgtacccacctctgcacagaggctagcagctgtggcacagtggtcctcccctcctgcacgtcctccagcaggcccctccgttgctcctcggtgaagtggcaggagctgagcaggtcccagagggatgtgccatccttggcccccggcacggcctgcaggctcctctggacctgctcctcggtggggagggcaggagcactttctggcaggggcaggaggtgaaggccagaagtctcatccctggggcactcctccaggagctgggcatagctcgtgcgcccctggccgtccggtgtggggaaggtttcggaggagctggacaaggctgtctccatctcctggtcaacatagccacgctgaatggccactggcatggggaggtggtggtggctggtggggtcaatgatccctcctgtggccacttgagcctccaggaggcgggcagcttgctcccaagggatgagacctttcttcatggcctggaacacagacacctgcttcccagagaaggggtctctgaagccagcaatggcaccctcagcccgcttcagcctgccatacagctccggccccaccacacccctgcgcacggcctcatccaccgagaggctctctgggctgtgagggtccatgatggttccggtggccgcctgggcctccagcagggccagggccaccctgggccccagcagcttctgcctcatggcctggtagaggctgagccgctggccagagggcagcagccgcacaccgcccacagctcccaggccgcacaggtacctgcggacgccgtccatgagtaggagggcctccgggctgattgtcccggccagcacttggtccaacagctgctggtcaatgataccggcctccaggagctggtggacggtgacccggctccgcagtgcgggcagcatgatgtccgcctgtctctgcgtctccgcctccagcagctttgccacctgccccagcgtgacctcgcgctgccggtagcgacgcagcagctgcctcctgcggccctcgctgaagtactcagagttgatcagctcccacgcggagaccctctgcccctgaaaccgtccatacttcacggagagcagcaggttctggaaggcctgctgggtggcactgtccaccagcggggactgcgtgctgctgagtggcaggaggtacaggcccgtctcggggtcacgcacacagcgctccagaagctgcaggtacgtgaggttctcgtgcgtgttggggtcgaagaagcccttggtgtcgtcagaagggtccaacaggatcaagttcagcatctgatcgaagtagccgcgccggtaggccacgtccacgggcacgcggtggctgtgcacggggtcgatgacgccgcccgtggcgatctgggcctccagcaggcggatgccgtgctcccggacgatgaggcccttctgcatggcctggaagagggagatctgctgcccggtgtaggggtcagtgtagccagtgacagcgcgctcagccgacagcagcttcgcgaacacatcaggcccaatgacagcagccctcagtgcctcctcaacggagtgccccttgtttgcttttgggtcgatgatgaagcctgtggcagcttgtgcctccagaaggatgagggcagtgccgggccggaggagccccttgcatcgggcctcatagatgctcaggcgttcctgggagccagggagcagcaggccagcaatgcagcccgtaccctgcaggtacctctgcaccgaggccaggctgcccacatccttggctgtggcctgtccatgctccagccgctcgtacaggtcctggtcgatgatctcggctttcagcagctctcctggtgtcacggtgtccctcagcccagaaaaggtgaccctggcagtggctgcagcctgctcgagggtggcgctcagcttagcggccagcttctccacggagagggtcccttcctggtactgctgggccagcatcgccctctgctctgaggagatggcctcagagaagagcagctcccagagggacacgggccggccccggaacttccccacagagacggtggctgtggccgtgctcagggcctgccgagtgctgtacttgatgaatgggggtccctggggctcccctccccggggtccccctgagagtggcaggaaggcaagcccggtctctgggtcggtgacacagagggccagcagctgttcatagcgcaggccgccgtgcgtgccgtctgagaagctgccagcctgcgagagctgccgctgagtgtcttcatccaggcagccgcagcgcagggcggcctccaggggcagccggagcctgcgtgctggacagaccagcccgcctgtggccagctgggcatccaagagccgcagtgccagtggcctgtccactagccccttcttcatggcctggaaaagggggatttgggagccactgaaggggtcgtggtgccctgtcacggcctgctcggccaccaggagctgctcatggagctctgggctgaccaggcccgccctgactgcctcgtctacccacagccgctggcctgtgatggggtccaccagggtgtgggtggcagcctgggcctctaggagtggcagcgcggtgcccattgggagcaggtgctcggtggcagcctggaaaaagctcttcttgtggccttcgggcagcaggacaaccccggccacgctgccggtaccctccaggtagcgccgcacctcggcacgtgcactcacgtccactgcggccagcctgccctcccgcagaccctgcacagcctgctcgtccaggatgcccacctccagcagctcagctgcactcaccgccccgcccatggagcggaaggtgatcttgaggggcagcaaggctagccccgagccgggggcacgcacacacctttccagcagctggtggtatgtcagccgctccagcgtgttggggtcgaggaagcgcaggtcacctgtgccaggctcaagctctgacagcttgtgccatgtctcccggtccaggaggccctggtggcaggctggctcaggggccacgagcactccctgggcggggtccaccaggcccccagtggccagttggacctccagccagctctgccccagggccctgtccacaacctccttcccgatggcctgaaagagggccagcttctcaccgccgtaggggtcaggatagcccgtagtggcacgctcagcggccagcagcttctccttcagctccagccccaccagaccctgctgcagggccttggacacagggagcagctggccccgggcgaggtccaccaggcccccagtggctgcctgggcctctagcagagcctgcccgagcccagcaggcaggaggccctgctccatggcggcgtagacactctgggcctggcccgaggcctccacatacaccccagctatgctcctggcctggggcctggggggcgtgccggctcccagcgtggctgccatggctctgggtacactggcctgctctgtgctgttggtgcctgggacgggaagaggaggcaaggtgtggccactcatcacacacggctggttatgcagagcctgctgaggtccacctctgtcctgcccgctcgccgctcggtccgcagtgtctccgcgcgcccgctccgcccgcatttcaa

SEQ ID NO: 12565 - RNA, 6815 nt, Homo sapiens
  source 1..6815: mol_type = other RNA
gaggctgagctgaggagttcagaagctgtgatctgtcgtctaattccttggaaccacaggtgtttgttgctggtttcctgcttctcgatcaactctaagatgagctgcgctaccgtctgcagtgcccgtctggtgtgtgttctatacatcctcaccagctggagcttcttctcctctgtcacgtattcggaattcagtagtgcccacagtgttggtttctggcctctgaaccttcccactgtgatttccacttgctctgcctccagggcccttctcgtctcgtcatcgatgtgctcggagtcccgtgcagccttgttcactgggaacagcagccagcccgtgtcctcttgtgggcggcacctctcctgcagctctcggtacgagaccttctcttgcgtgttcgggtccacaaaccgtttcctcatgtgcttctggtcggaaatgagcgcatagatgtccttgtgcagacagccccgtctgtaggctgtttccagtgggagccggtggtggtgctgtgggtcgatgacaccccccgtggccacctgcacctccagcagcctcagtgcctccgccttctcgatgagctgcttctgcatggcctggaacagcgggatcgtgtctcctgtggccggatccctgtagcccgtggcagctctttcagccttcaggagcctctcccgcagctcctcgttcaccaggcccacatccacagcctcatccacagagagcttctggcgggtgcaggggtccaggaggaacccggtggcggcctgcgcctccagcagccaagtcgcaaatgctgcagggatgagctccttcctgctggcctcatggaggctcatgacctccctggtggagggcaccgtgacccccgcaatgcagccgctgccttccagatagggcttcacacactccagcgtgctgagtgcctgtcccccagtcctccccacacgaagtgtgtgcagggtcttctgatcgatgaccctggagttgaacaggtctgcagctgtcacctcccctctgatggccgccactttgatgccttggttttgcgtctctgtttcttcaattgtcgtggtgatgatttccagcaatttctccaggcccccactctgggctccatactcctggatgagctcccgcttcctgtcctctgtgaagtatggagaggacagcaggtcccagaaagagaccacctggtcagcaaacctccccacgcgcatttttgcagttctggattgcaacacgtgtctcgtggcctcattgatgtacacgtagttttctcctttctttatgatttgtagcaggtacaggcccgtctcggggtcctccacacagcgctccagaagctgcaggtacgtgaggttctcgtgcgtgttggggtcgaagaagcccttggtgtcgtcgctggggtccgccaggatgcggttcatctcctcgtcgaagtagccgcagcggtaggccacgtccacgggcacgcggtggctgtgcacggggtcgatgatgccgcccgtggcgatctgggcctccagcaggcggatgccgtgctcccggacgatgaggtccttctgcatggcctggaagagggagatctgctgcccggtataggggtcggtgtagccggtgacggcgcgctcggccgacagcagcttcacgtaggtttctttcccgaacattcctgctttgaacgcctcctccacggtcagcttccggttctccacggggtcgatgatgaagccggtagctgcctgtgcctccagcagcaccagggctgtgccaggccgcaggatgtgcctcctcagggcctctgggatgctcatcctctcctgggtgccctggataaggaccccggcaatgaagttgcctccctccagggaccgcttcacgctgtccatctccgccacctccttcacagtcgttgtcccctggctcagctcgtccagcgtcttcctgctgatcagctgcgccctgaacaggtccctggctgacacctgcttccggagccctctgaaggtggcctgcaggggctgcctctctgcagcctcgaccagggtggtgactgcgctgaccacctgccgcagggccgcagccctcccagaccgacagagtgccaccagctcccgccgcttgtcagcgccaacgtattcggagagcagcaggtcccagagtgacacgctacaccccttaaacctccctgtgctgacgggcaccttcatggccctcagagccaccgcggtgtggtcgtccacctcaagcactgtgtctgagggcagtggcaacagcaacaatccggtctcggagtcgcacacgcagcgctccctgagctgctggtaggtcacctggtcccgcgcactggggtcaaagaagaacttgttgtccttgtcaactgcagtcagcacctggctcgtctgtgtgtccagaaggccgagtctgcaggctgccgcctggggcaggtgcaccccgtggacagggtccaccacaccccctgtggccagctgcacctgcaggaggggcaagccctcgttctgtggcacgagccccttctccatggcctgccacagagagagggaggccctagagtagggatctgggtacccggccgccgccctctcggcctgcccgagctgctcactcagctccctgcccaccaggccgaccttaaccgcgtcctccactgacagtctctggttgttcagggggtcaacaaggaagccagatgccacctgggcttccagcagcctctggcccaggcctgtgggcaggaggccatccctcacggcctgggcgatgctggccttggccccagagggctgtagcagcacaccggccacgcagcctgtgccccacaggcaggccttcaccgccggctgctcggcgacctgggcgggcgactgcgtgccctgagccagggcctcaagggtctcctgggtgatgatgccagcatccagcagccagacagcgggtacctcaccccgtgggccgggcaccatgacgcgggcctgggccaggagcttggtctcctgtacccacctctgcacagaggctagcagctgtggcacagtggtcctcccctcctgcacgtcctccagcaggcccctccgttgctcctcggtgaagtggcaggagctgagcaggtcccagagggatgtgccatccttggcccccggcacggcctgcaggctcctctggacctgctcctcggtggggagggcaggagcactttctggcaggggcaggaggtgaaggccagaagtctcatccctggggcactcctccaggagctgggcatagctcgtgcgcccctggccgtccggtgtggggaaggtttcggaggagctggacaaggctgtctccatctcctggtcaacatagccacgctgaatggccactggcatggggaggtggtggtggctggtggggtcaatgatccctcctgtggccacttgagcctccaggaggcgggcagcttgctcccaagggatgagacctttcttcatggcctggaacacagacacctgcttcccagagaaggggtctctgaagccagcaatggcaccctcagcccgcttcagcctgccatacagctccggccccaccacacccctgcgcacggcctcatccaccgagaggctctctgggctgtgagggtccatgatggttccggtggccgcctgggcctccagcagggccagggccaccctgggccccagcagcttctgcctcatggcctggtagaggctgagccgctggccagagggcagcagccgcacaccgcccacagctcccaggccgcacaggtacctgcggacgccgtccatgagtaggagggcctccgggctgattgtcccggccagcacttggtccaacagctgctggtcaatgataccggcctccaggagctggtggacggtgacccggctccgcagtgcgggcagcatgatgtccgcctgtctctgcgtctccgcctccagcagctttgccacctgccccagcgtgacctcgcgctgccggtagcgacgcagcagctgcctcctgcggccctcgctgaagtactcagagttgatcagctcccacgcggagaccctctgcccctgaaaccgtccatacttcacggagagcagcaggttctggaaggcctgctgggtggcactgtccaccagcggggactgcgtgctgctgagtggcaggaggtacaggcccgtctcggggtcacgcacacagcgctccagaagctgcaggtacgtgaggttctcgtgcgtgttggggtcgaagaagcccttggtgtcgtcagaagggtccaacaggatcaagttcagcatctgatcgaagtagccgcgccggtaggccacgtccacgggcacgcggtggctgtgcacggggtcgatgacgccgcccgtggcgatctgggcctccagcaggcggatgccgtgctcccggacgatgaggcccttctgcatggcctggaagagggagatctgctgcccggtgtaggggtcagtgtagccagtgacagcgcgctcagccgacagcagcttcgcgaacacatcaggcccaatgacagcagccctcagtgcctcctcaacggagtgccccttgtttgcttttgggtcgatgatgaagcctgtggcagcttgtgcctccagaaggatgagggcagtgccgggccggaggagccccttgcatcgggcctcatagatgctcaggcgttcctgggagccagggagcagcaggccagcaatgcagcccgtaccctgcaggtacctctgcaccgaggccaggctgcccacatccttggctgtggcctgtccatgctccagccgctcgtacaggtcctggtcgatgatctcggctttcagcagctctcctggtgtcacggtgtccctcagcccagaaaaggtgaccctggcagtggctgcagcctgctcgagggtggcgctcagcttagcggccagcttctccacggagagggtcccttcctggtactgctgggccagcatcgccctctgctctgaggagatggcctcagagaagagcagctcccagagggacacgggccggccccggaacttccccacagagacggtggctgtggccgtgctcagggcctgccgagtgctgtacttgatgaatgggggtccctggggctcccctccccggggtccccctgagagtggcaggaaggcaagcccggtctctgggtcggtgacacagagggccagcagctgttcatagcgcaggccgccgtgcgtgccgtctgagaagctgccagcctgcgagagctgccgctgagtgtcttcatccaggcagccgcagcgcagggcggcctccaggggcagccggagcctgcgtgctggacagaccagcccgcctgtggccagctgggcatccaagagccgcagtgccagtggcctgtccactagccccttcttcatggcctggaaaagggggatttgggagccactgaaggggtcgtggtgccctgtcacggcctgctcggccaccaggagctgctcatggagctctgggctgaccaggcccgccctgactgcctcgtctacccacagccgctggcctgtgatggggtccaccagggtgtgggtggcagcctgggcctctaggagtggcagcgcggtgcccattgggagcaggtgctcggtggcagcctggaaaaagctcttcttgtggccttcgggcagcaggacaaccccggccacgctgccggtaccctccaggtagcgccgcacctcggcacgtgcactcacgtccactgcggccagcctgccctcccgcagaccctgcacagcctgctcgtccaggatgcccacctccagcagctcagctgcactcaccgccccgcccatggagcggaaggtgatcttgaggggcagcaaggctagccccgagccgggggcacgcacacacctttccagcagctggtggtatgtcagccgctccagcgtgttggggtcgaggaagcgcaggtcacctgtgccaggctcaagctctgacagcttgtgccatgtctcccggtccaggaggccctggtggcaggctggctcaggggccacgagcactccctgggcggggtccaccaggcccccagtggccagttggacctccagccagctctgccccagggccctgtccacaacctccttcccgatggcctgaaagagggccagcttctcaccgccgtaggggtcaggatagcccgtagtggcacgctcagcggccagcagcttctccttcagctccagccccaccagaccctgctgcagggccttggacacagggagcagctggccccgggcgaggtccaccaggcccccagtggctgcctgggcctctagcagagcctgcccgagcccagcaggcaggaggccctgctccatggcggcgtagacactctgggcctggcccgaggcctccacatacaccccagctatgctcctggcctggggcctggggggcgtgccggctcccagcgtggctgccatggctctgggtacactggcctgctctgtgctgttggtgcctgggacgggaagaggaggcaaggtgtggccactcatcacacacggctggttatgcagagcctgctgaggtccacctctgtccttgtctgctcagcttcctggggacgctgcttcacgtcgtgtgtctgctgggtccaggggtcttcaaggctctccttggcaggcccccctgcccccatgacgttgtaagagctgggatgtcctgcctggagcagtgccaggcctcaccccccggtctggctcctccacctgggcacagagaatgttccctgtcaccct

SEQ ID NO: 12566 - RNA, 2033 nt, Homo sapiens
  source 1..2033: mol_type = other RNA
gagggcgggtggaggaggaagggtgtgggggcaggtggcgggaaccacacaggcctcagtggagccggtgccttcatctcagaggtcctcatggcagcactgttgccccaggaggtgtctggggacatgtgtgggggtcagggtcttgctacagggcaggggcaccatgggtgttcgccgtggggctgggaggcagagcctacacctgggcacagtcctgcagacctagcacccatgagccacggccgcctcgcctgccctcatgctggcctcaggtgcccctcacaggttgacacacccggcttactgtccccagcaccacactcctcggggatggctgcggctggcgtgggtactctctgcagctgtgctgaccccacaatggggttggctttgtgggagtcgagccccatgtacgtcatcaagggcttccatgccctgggctatgttgctgctggtgggactgagcccttgctcagactgtgggaagagccacttcaggcctcacccaagacagcccagaggctggagtggcctctccccaccaggtctgtgcaggtcggtgccccagaggccccgctcacacaggaacagggcggctgactccctgcacccctgggggccccgtgaggtgcttccttcgagggtcatggggtggagtgggcagagcacggctcccaggcgcaggcccgtgtgcctccctccagcccccaagtgctcctggaagttttcccggggtctccacacatctatttatgtctggcctgtttgaaacaggacccagcagggccgtgtccggcaccttgtttatctgcccagactcttcgggctgtgcatttgttgaagcgttggcatcatttgttccacagaacagcagttcttcacgtgtggtcctttgggtgttttcaggggggtctccaagaccagcacagtcatctcgggccccttgcctttttctctgtgttgacattcgcggcaatggcagagggctgatggtgggacacctgctggtgcctgggcccagatcaaggtggctttgagctcgtgaggcttctcgccaccatcgccagcagcattcggcagtgacgttccttgtgatggagctggaggtttgcgcacagtgctttgtgtgtgccatgtgggcgtctggcagccaagctgaaccaagctcctttattcttgcaacaccagtttccatggaacaaacagcgaacagccctgcatacccaggcttgggtgttttcctgaaaacaaccaagtaagcccatccctgtaaggaaaacagctgggagtatctggcaccaatgatacaatgttgagctttcaaatgacaagaggaatttttgaaaacttgtttctcgcattgtgagtgtgacagcttccgaataattctccacatgaccagcgtgtgattcctcaaaatcatgcataggtaaaagacccattcaaagagcaaagggggccagtggattttcatgaacaaaactcacgctcaatgaatgcagaaagttgtctccacacacaagcatttatgtgtttgtgaatgtgtgtctctgtgtacgtgtgtgtgcatgcctgtgtgtgcatgtctgtgtgtggtgtgagtgcatgtgcacgtgtgtgcgcatgtgtttgtgtctgtgtgtgcatgtttgtgcagtgtggtgtatgtgcgtgtctgtgtgcctgcatgcatgtgtacgtgtgtgactgcgtgtgtgtgcgtgtgtgtgcacgtgtatgtccatgtttgtgtgtgtgcatgtgtatgtgagtgcatgtctgtgtctgtgtggtgtgtgtacatgtgtgcatgcatgtttgcatttgcatgtgtgcatatgtgcatgtgtgcatatatgtgcacgtgtgtatgcgcatgcttgggtgtgtctgtacgtgtgagtgcatgtctgtgtggtgtgtgtacatgtgtgcatgcatgtttgcatgtgtacgcatgtgcacatgtgtgcatatacgtgtgcatatctgcatatgtgcatgtatatacacatgtgtgtaggtgcata

SEQ ID NO: 12567 - RNA, 288 nt, Homo sapiens
  source 1..288: mol_type = other RNA
gagggcgggtggaggaggacgcgggacgctcgggctcccaggcgctgccgctgcgggtcccatggcgcacgcaggtgcctgctcggccacctgcgccaacagcatccacagcgccgccaagccccgccatccgcgcgcgcggggcttcatccaggagcgctccgaggggctaggggccaccggagggtccccggccggcagcgtgcgagcgggcagggaggacccgacccaggcagagcgcgggaggattccccacagcgactccgccgccgcgccggggttattact

SEQ ID NO: 12568 - RNA, 1764 nt, Homo sapiens
  source 1..1764: mol_type = other RNA
gaggttttctgggtttctgtttcatctgtactgattgactatatcattttccctctctgagtcaattttctcatcagttacatgtaaataataataataataatgccacccaccttcctatctcactgagttcttttaaggaccaagtgaggtcatttgtcagacatgagtgcttggtaagtgaaaaatcaatgcaaacgaaaggcaatattattttctctatgcattgtaaatccctgcttctgtagcaggaaagcaccatgctgacttagttattcctaattaactcaaatattacccaagatctacagtccataaggtatgtaggcagaaagtgagatatgaacaaatccttcatcacaaatcaattctcaagcatttccccagggccagccatcctccctctgcagaaggggaccctgaggggtactcactctctaattgttttaacagcttggctgccctgccagagccctcccagaaaaccagattggtgaggggaggtgcagaatgaagaattaactggcacctcagcaattctggattctgtggaggggctggaaggctatactacagacacacacccctgcaggataattctagctggaggccgcagcagggtggatgagaacatgcttctgcaaacctcttgggatgcatcactgactggattctggcgattagagcttccagcctgccagaaattcctcagtgcatgatctgctgagcagctctgacagggattcactggtgtcctggtagaatgtggagcccaggccctcagagctcccactctccagctggaagctgcccaccagctcctgaatccactgcaggtctgcggagagctcctgcctcagaatctcaaactgggcttgcagatggtccagtttcctggccatgcttccgaggctacatcccgtggcctggatgtcttctcgcagcagcttcttcaatgactccaccttgcggaactcatacctgagctgggacaggtcatgccgggcgctctcattctcctctcggtaccaagcttccttctcattgaagatggagaccagggcctccacatcgtcctggatggtatcgtgggcctccaccagggcacggcatcccaggtcgacccgagccacgtcttccaccacacaggcaaaacgctcgaagttgacataggagttgttgggaggcatgcttgagtggcatttgagagtgtactctctcaggtgcttggtcttcagctgggtgggctctgtcttccgctgttcaggggctctgccttctccttttgacgtgatccaggggtgtctgagagcctcttggattgtgagccgtttccgggtctctttaaccagaagcttccgaataaagtccttggccagctcgctcgtctggctgaagaattcctcatcaaagtcgtaactcactgctgtgatatttgccagtgtttcctgcttcgtgtctcccaggaaaggggatgctccacttaagaggatgtaggtgatgacgcctatgctccacatgtcagcctccagacccaggggctcgtagttcacaatttctggagcaacaaattccggcgtcccaaaaatattcttaaattcaactccatcttctatttcgtgagccagaccaaagtcaatcagcttgatgtgtggaatgggaatattcttgtctaacaacataatgttttctggagctcaaggatgagcaccacgtcggtgcggttctcatagacgtcgtgcagcgtgatgacattgtggtgca

SEQ ID NO: 12569 - RNA, 1922 nt, Homo sapiens
  source 1..1922: mol_type = other RNA
gaggttttctgggtttctgtttcatctgtactgattgactatatcattttccctctctgagtcaattttctcatcagttacatgtaaataataataataataatgccacccaccttcctatctcactgagttcttttaaggaccaagtgaggtcatttgtcagacatgagtgcttggtaagtgaaaaatcaatgcaaacgaaaggcaatattattttctctatgcattgtaaatccctgcttctgtagcaggaaagcaccatgctgacttagttattcctaattaactcaaatattacccaagatctacagtccataaggtatgtaggcagaaagtgagatatgaacaaatccttcatcacaaatcaattctcaagcatttccccagggccagccatcctccctctgcagaaggggaccctgaggggtactcactctctaattgttttaacagcttggctgccctgccagagccctcccagaaaaccagattggtgaggggaggtgcagaatgaagaattaactggcacctcagcaattctggattctgtggaggggctggaaggctatactacagacacacacccctgcaggataattctagctggaggccgcagcagggtggatgagaacatgcttctgcaaacctcttgggatgcatcactgactggattctggcgattagagcttccagcctgccagaaattcctcagtgcatgatctgctgagcagctctgacagggattcactggtgtcctggtagaatgtggagcccaggccctcagagctcccactctccagctggaagctgcccaccagctcctgaatccactgcaggtctgcggagagctcctgcctcagaatctcaaactgggcttgcagatggtccagtttcctggccatgcttccgaggctacatcccgtggcctggatgtcttctcgcagcagcttcttcaatgactccaccttgcggaactcatacctgagctgggacaggtcatgccgggcgctctcattctcctctcggtaccaagcttccttctcattgaagatggagaccagggcctccacatcgtcctggatggtatcgtgggcctccaccagggcacggcatcccaggtcgacccgagccacgtcttccaccacacaggcaaaacgctcgaagttgacataggagttgttgggaggcatgcttgagtggcatttgagagtgtactctctcaggtgcttggtcttcagctgggtgggctctgtcttccgctgttcaggggctctgccttctccttttgacgtgatccaggggtgtctgagagcctcttggattgtgagccgtttccgggtctctttaaccagaagcttccgaataaagtccttggccagctcgctcgtctggctgaagaattcctcatcaaagtcgtaactcactgctgtgatatttgccagtgtttcctgcttcgtgtctcccaggaaaggggatgctccacttaagaggatgtaggtgatgacgcctatgctccacatgtcagcctccagacccaggggctcgtagttcacaatttctggagcaacaaattccggcgtcccaaaaatattcttaaattcaactccatcttctatttcgtgagccagaccaaagtcaatcagcttgatgtgtggaatgggaatattcttgtctaacaacataatgttttctggctcccgctcgatctcctcccggctcacaccgcgccggctcgcccggctctgccgcttcttgatgaacttggctgcatactcaagccccgtgctcttctcccggcacttcttcacgatggcaaactggccactccccagctcctctccgatgtcataaaagtcctccaccttctgctgcttgaatggctccatgtttggactcctcattgaggcctggaacatacaatc

SEQ ID NO: 12570 - RNA, 2341 nt, Homo sapiens
  source 1..2341: mol_type = other RNA
gaggttttctgggtttctgtttcatctgtactgattgactatatcattttccctctctgagtcaattttctcatcagttacatgtaaataataataataataatgccacccaccttcctatctcactgagttcttttaaggaccaagtgaggtcatttgtcagacatgagtgcttggtaagtgaaaaatcaatgcaaacgaaaggcaatattattttctctatgcattgtaaatccctgcttctgtagcaggaaagcaccatgctgacttagttattcctaattaactcaaatattacccaagatctacagtccataaggtatgtaggcagaaagtgagatatgaacaaatccttcatcacaaatcaattctcaagcatttccccagggccagccatcctccctctgcagaaggggaccctgaggggtactcactctctaattgttttaacagcttggctgccctgccagagccctcccagaaaaccagattggtgaggggaggtgcagaatgaagaattaactggcacctcagcaattctggattctgtggaggggctggaaggctatactacagacacacacccctgcaggataattctagctggaggccgcagcagggtggatgagaacatgcttctgcaaacctcttgggatgcatcactgactggattctggcgattagagcttccagcctgccagaaattcctcagtgcatgatctgctgagcagctctgacagggattcactggtgtcctggtagaatgtggagcccaggccctcagagctcccactctccagctggaagctgcccaccagctcctgaatccactgcaggtctgcggagagctcctgcctcagaatctcaaactgggcttgcagatggtccagtttcctggccatgcttccgaggctacatcccgtggcctggatgtcttctcgcagcagcttcttcaatgactccaccttgcggaactcatacctgagctgggacaggtcatgccgggcgctctcattctcctctcggtaccaagcttccttctcattgaagatggagaccagggcctccacatcgtcctggatggtatcgtgggcctccaccagggcacggcatcccaggtcgacccgagccacgtcttccaccacacaggcaaaacgctcgaagttgacataggagttgttgggaggcatgcttgagtggcatttgagagtgtactctctcaggtgcttggtcttcagctgggtgggctctgtcttccgctgttcaggggctctgccttctccttttgacgtgatccaggggtgtctgagagcctcttggattgtgagccgtttccgggtctctttaaccagaagcttccgaataaagtccttggccagctcgctcgtctggctgaagaattcctcatcaaagtcgtaactcactgctgtgatatttgccagtgtttcctgcttcgtgtctcccaggaaaggggatgctccacttaagaggatgtaggtgatgacgcctatgctccacatgtcagcctccagacccaggggctcgtagttcacaatttctggagcaacaaattccggcgtcccaaaaatattcttaaattcaactccatcttctatttcgtgagccagaccaaagtcaatcagcttgatgtgtggaatgggaatattcttgtctaacaacataatgttttctggcttgagatcaaagtgagcaattttctttgtgtgaaggtagttcaccccatccaggatctgcttaatgaagctggtggcctcctcctcactcagtgactccttctgggccaggaaatcgaagagctctcctccagacactagctcaaggatgagcaccacgtcggtgcggttctcatagacgtcgtgcagcgtgatgacattgtggtgcagcacctgccgcaggatgctcacctcccgctcgatctcctcccggctcacaccgcgccggctcgcccggctctgccgcttcttgatgaacttggctgcatactcaagccccgtgctcttctcccggcacttcttcacgatggcaaactggccactccccagctcctctccgatgtcataaaagtcctccaccttctgctgcttgaatggctccatgtttggactcctcattgaggcctggaacatacaatcggcgggaggctgagctgccgcggtcgcggccgcggcaggcgcggcgggagcggcgggcgcggcgggcgcggcgggcgcggcgggcgcggcgggaacgggggacgcggcggggtgcgctgggctcggccctgcagtcctctcctcccagagcgcccggcacccgcccgccgagcagcctaggagccgag

SEQ ID NO: 12571 - RNA, 1963 nt, Homo sapiens
  source 1..1963: mol_type = other RNA
gaggttttctgggtttctgtttcatctgtactgattgactatatcattttccctctctgagtcaattttctcatcagttacatgtaaataataataataataatgccacccaccttcctatctcactgagttcttttaaggaccaagtgaggtcatttgtcagacatgagtgcttggtaagtgaaaaatcaatgcaaacgaaaggcaatattattttctctatgcattgtaaatccctgcttctgtagcaggaaagcaccatgctgacttagttattcctaattaactcaaatattacccaagatctacagtccataaggtatgtaggcagaaagtgagatatgaacaaatccttcatcacaaatcaattctcaagcatttccccagggccagccatcctccctctgcagaaggggaccctgaggggtactcactctctaattgttttaacagcttggctgccctgccagagccctcccagaaaaccagattggtgaggggaggtgcagaatgaagaattaactggcacctcagcaattctggattctgtggaggggctggaaggctatactacagacacacacccctgcaggataattctagctggaggccgcagcagggtggatgagaacatgcttctgcaaacctcttgggatgcatcactgactggattctggcgattagagcttccagcctgccagaaattcctcagtgcatgatctgctgagcagctctgacagggattcactggtgtcctggtagaatgtggagcccaggccctcagagctcccactctccagctggaagctgcccaccagctcctgaatccactgcaggtctgcggagagctcctgcctcagaatctcaaactgggcttgcagatggtccagtttcctggccatgcttccgaggctacatcccgtggcctggatgtcttctcgcagcagcttcttcaatgactccaccttgcggaactcatacctgagctgggacaggtcatgccgggcgctctcattctcctctcggtaccaagcttccttctcattgaagatggagaccagggcctccacatcgtcctggatggtatcgtgggcctccaccagggcacggcatcccaggtcgacccgagccacgtcttccaccacacaggcaaaacgctcgaagttgacataggagttgttgggaggcatgcttgagtggcatttgagagtgtactctctcaggtgcttggtcttcagctgggtgggctctgtcttccgctgttcaggggctctgccttctccttttgacgtgatccaggggtgtctgagagcctcttggattgtgagccgtttccgggtctctttaaccagaagcttccgaataaagtccttggccagctcgctcgtctggctgaagaattcctcatcaaagtcgtaactcactgctgtgatatttgccagtgtttcctgcttcgtgtctcccaggaaaggggatgctccacttaagaggatgtaggtgatgacgcctatgctccacatgtcagcctccagacccaggggctcgtagttcacaatttctggagcaacaaattccggcgtcccaaaaatattcttaaattcaactccatcttctatttcgtgagccagaccaaagtcaatcagcttgatgtgtggaatgggaatattcttgtctaacaacataatgttttctggcttgagatcaaagtgagcaattttctttgtgtgaaggtagttcaccccatccaggatctgcttaatgaagctggtggcctcctcctcactcagtgactccttctgggccaggaaatcgaagagctctcctccagacactctcccgctcgatctcctcccggctcacaccgcgccggctcgcccggctctgccgcttcttgatgaacttggctgcatactcaagccccgtgctcttctcccggcacttcttcacgatggcaaactggcca

SEQ ID NO: 12572 - RNA, 1913 nt, Homo sapiens
  source 1..1913: mol_type = other RNA
gaggttttctgggtttctgtttcatctgtactgattgactatatcattttccctctctgagtcaattttctcatcagttacatgtaaataataataataataatgccacccaccttcctatctcactgagttcttttaaggaccaagtgaggtcatttgtcagacatgagtgcttggtaagtgaaaaatcaatgcaaacgaaaggcaatattattttctctatgcattgtaaatccctgcttctgtagcaggaaagcaccatgctgacttagttattcctaattaactcaaatattacccaagatctacagtccataaggtatgtaggcagaaagtgagatatgaacaaatccttcatcacaaatcaattctcaagcatttccccagggccagccatcctccctctgcagaaggggaccctgaggggtactcactctctaattgttttaacagcttggctgccctgccagagccctcccagaaaaccagattggtgaggggaggtgcagaatgaagaattaactggcacctcagcaattctggattctgtggaggggctggaaggctatactacagacacacacccctgcaggataattctagctggaggccgcagcagggtggatgagaacatgcttctgcaaacctcttgggatgcatcactgactggattctggcgattagagcttccagcctgccagaaattcctcagtgcatgatctgctgagcagctctgacagggattcactggtgtcctggtagaatgtggagcccaggccctcagagctcccactctccagctggaagctgcccaccagctcctgaatccactgcaggtctgcggagagctcctgcctcagaatctcaaactgggcttgcagatggtccagtttcctggccatgcttccgaggctacatcccgtggcctggatgtcttctcgcagcagcttcttcaatgactccaccttgcggaactcatacctgagctgggacaggtcatgccgggcgctctcattctcctctcggtaccaagcttccttctcattgaagatggagaccagggcctccacatcgtcctggatggtatcgtgggcctccaccagggcacggcatcccaggtcgacccgagccacgtcttccaccacacaggcaaaacgctcgaagttgacataggagttgttgggaggcatgcttgagtggcatttgagagtgtactctctcaggtgcttggtcttcagctgggtgggctctgtcttccgctgttcaggggctctgccttctccttttgacgtgatccaggggtgtctgagagcctcttggattgtgagccgtttccgggtctctttaaccagaagcttccgaataaagtccttggccagctcgctcgtctggctgaagaattcctcatcaaagtcgtaactcactgctgtgatatttgccagtgtttcctgcttcgtgtctcccaggaaaggggatgctccacttaagaggatgtaggtgatgacgcctatgctccacatgtcagcctccagacccaggggctcgtagttcacaatttctggagcaacaaattccggcgtcccaaaaatattcttaaattcaactccatcttctatttcgtgagccagaccaaagtcaatcagcttgatgtgtggaatgggaatattcttgtctaacaacataatgttttctggtctgatgagcttgtctgcttgtctccctctactgggttgcccaagggttttgttcctgtcatctccccagaggttgggatagagcctgatatccagcagctgctcaatatatgtgccccaagtgaagacaggtgccactgattaagcccctgcaatatacaggacccagtgctaagcaaacatgcgacatactttacacttcattgaactctcaactac

SEQ ID NO: 12573 - RNA, 1959 nt, Homo sapiens
  source 1..1959: mol_type = other RNA
gaggttttctgggtttctgtttcatctgtactgattgactatatcattttccctctctgagtcaattttctcatcagttacatgtaaataataataataataatgccacccaccttcctatctcactgagttcttttaaggaccaagtgaggtcatttgtcagacatgagtgcttggtaagtgaaaaatcaatgcaaacgaaaggcaatattattttctctatgcattgtaaatccctgcttctgtagcaggaaagcaccatgctgacttagttattcctaattaactcaaatattacccaagatctacagtccataaggtatgtaggcagaaagtgagatatgaacaaatccttcatcacaaatcaattctcaagcatttccccagggccagccatcctccctctgcagaaggggaccctgaggggtactcactctctaattgttttaacagcttggctgccctgccagagccctcccagaaaaccagattggtgaggggaggtgcagaatgaagaattaactggcacctcagcaattctggattctgtggaggggctggaaggctatactacagacacacacccctgcaggataattctagctggaggccgcagcagggtggatgagaacatgcttctgcaaacctcttgggatgcatcactgactggattctggcgattagagcttccagcctgccagaaattcctcagtgcatgatctgctgagcagctctgacagggattcactggtgtcctggtagaatgtggagcccaggccctcagagctcccactctccagctggaagctgcccaccagctcctgaatccactgcaggtctgcggagagctcctgcctcagaatctcaaactgggcttgcagatggtccagtttcctggccatgcttccgaggctacatcccgtggcctggatgtcttctcgcagcagcttcttcaatgactccaccttgcggaactcatacctgagctgggacaggtcatgccgggcgctctcattctcctctcggtaccaagcttccttctcattgaagatggagaccagggcctccacatcgtcctggatggtatcgtgggcctccaccagggcacggcatcccaggtcgacccgagccacgtcttccaccacacaggcaaaacgctcgaagttgacataggagttgttgggaggcatgcttgagtggcatttgagagtgtactctctcaggtgcttggtcttcagctgggtgggctctgtcttccgctgttcaggggctctgccttctccttttgacgtgatccaggggtgtctgagagcctcttggattgtgagccgtttccgggtctctttaaccagaagcttccgaataaagtccttggccagctcgctcgtctggctgaagaattcctcatcaaagtcgtaactcactgctgtgatatttgccagtgtttcctgcttcgtgtctcccaggaaaggggatgctccacttaagaggatgtaggtgatgacgcctatgctccacatgtcagcctccagacccaggggctcgtagttcacaatttctggagcaacaaattccggcgtcccaaaaatattcttaaattcaactccatcttctatttcgtgagccagaccaaagtcaatcagcttgatgtgtggaatgggaatattcttgtctaacaacataatgttttcttgagatcaaagtgagcaattttctttgtgtgaaggtagttcaccccatccaggatctgcttaatgaagctggtggcctcctcctcactcagtgactccttctgggccaggaaatcgaagagctctcctccagacactctcccgctcgatctcctcccggctcacaccgcgccggctcgcccggctctgccgcttcttgatgaacttggctgcatactcaagccccgtgctcttctcccggcacttcttcacgatggcaaactggcca

SEQ ID NO: 12574 - RNA, 1910 nt, Homo sapiens
  source 1..1910: mol_type = other RNA
gaggttttctgggtttctgtttcatctgtactgattgactatatcattttccctctctgagtcaattttctcatcagttacatgtaaataataataataataatgccacccaccttcctatctcactgagttcttttaaggaccaagtgaggtcatttgtcagacatgagtgcttggtaagtgaaaaatcaatgcaaacgaaaggcaatattattttctctatgcattgtaaatccctgcttctgtagcaggaaagcaccatgctgacttagttattcctaattaactcaaatattacccaagatctacagtccataaggtatgtaggcagaaagtgagatatgaacaaatccttcatcacaaatcaattctcaagcatttccccagggccagccatcctccctctgcagaaggggaccctgaggggtactcactctctaattgttttaacagcttggctgccctgccagagccctcccagaaaaccagattggtgaggggaggtgcagaatgaagaattaactggcacctcagcaattctggattctgtggaggggctggaaggctatactacagacacacacccctgcaggataattctagctggaggccgcagcagggtggatgagaacatgcttctgcaaacctcttgggatgcatcactgactggattctggcgattagagcttccagcctgccagaaattcctcagtgcatgatctgctgagcagctctgacagggattcactggtgtcctggtagaatgtggagcccaggccctcagagctcccactctccagctggaagctgcccaccagctcctgaatccactgcaggtctgcggagagctcctgcctcagaatctcaaactgggcttgcagatggtccagtttcctggccatgcttccgaggctacatcccgtggcctggatgtcttctcgcagcagcttcttcaatgactccaccttgcggaactcatacctgagctgggacaggtcatgccgggcgctctcattctcctctcggtaccaagcttccttctcattgaagatggagaccagggcctccacatcgtcctggatggtatcgtgggcctccaccagggcacggcatcccaggtcgacccgagccacgtcttccaccacacaggcaaaacgctcgaagttgacataggagttgttgggaggcatgcttgagtggcatttgagagtgtactctctcaggtgcttggtcttcagctgggtgggctctgtcttccgctgttcaggggctctgccttctccttttgacgtgatccaggggtgtctgagagcctcttggattgtgagccgtttccgggtctctttaaccagaagcttccgaataaagtccttggccagctcgctcgtctggctgaagaattcctcatcaaagtcgtaactcactgctgtgatatttgccagtgtttcctgcttcgtgtctcccaggaaaggggatgctccacttaagaggatgtaggtgatgacgcctatgctccacatgtcagcctccagacccaggggctcgtagttcacaatttctggagcaacaaattccggcgtcccaaaaatattcttaaattcaactccatcttctatttcgtgagccagaccaaagtcaatcagcttgatgtgtggaatgggaatattcttgtctaacaacataatgtttttctgatgagcttgtctgcttgtctccctctactgggttgcccaagggttttgttcctgtcatctccccagaggttgggatagagcctgatatccagcagctgctcaatatatgtgccccaagtgaagacaggtgccactgattaagcccctgcaatatacaggacccagtgctaagcaaacatgcgacatactttacacttcattgaactctcaactacc

SEQ ID NO: 12575 - RNA, 2446 nt, Homo sapiens
  source 1..2446: mol_type = other RNA
gaggttttctgggtttctgtttcatctgtactgattgactatatcattttccctctctgagtcaattttctcatcagttacatgtaaataataataataataatgccacccaccttcctatctcactgagttcttttaaggaccaagtgaggtcatttgtcagacatgagtgcttggtaagtgaaaaatcaatgcaaacgaaaggcaatattattttctctatgcattgtaaatccctgcttctgtagcaggaaagcaccatgctgacttagttattcctaattaactcaaatattacccaagatctacagtccataaggtatgtaggcagaaagtgagatatgaacaaatccttcatcacaaatcaattctcaagcatttccccagggccagccatcctccctctgcagaaggggaccctgaggggtactcactctctaattgttttaacagcttggctgccctgccagagccctcccagaaaaccagattggtgaggggaggtgcagaatgaagaattaactggcacctcagcaattctggattctgtggaggggctggaaggctatactacagacacacacccctgcaggataattctagctggaggccgcagcagggtggatgagaacatgcttctgcaaacctcttgggatgcatcactgactggattctggcgattagagcttccagcctgccagaaattcctcagtgcatgatctgctgagcagctctgacagggattcactggtgtcctggtagaatgtggagcccaggccctcagagctcccactctccagctggaagctgcccaccagctcctgaatccactgcaggtctgcggagagctcctgcctcagaatctcaaactgggcttgcagatggtccagtttcctggccatgcttccgaggctacatcccgtggcctggatgtcttctcgcagcagcttcttcaatgactccaccttgcggaactcatacctgagctgggacaggtcatgccgggcgctctcattctcctctcggtaccaagcttccttctcattgaagatggagaccagggcctccacatcgtcctggatggtatcgtgggcctccaccagggcacggcatcccaggtcgacccgagccacgtcttccaccacacaggcaaaacgctcgaagttgacataggagttgttgggaggcatgcttgagtggcatttgagagtgtactctctcaggtgcttggtcttcagctgggtgggctctgtcttccgctgttcaggggctctgccttctccttttgacgtgatccaggggtgtctgagagcctcttggattgtgagccgtttccgggtctctttaaccagaagcttccgaataaagtccttggccagctcgctcgtctggctgaagaattcctcatcaaagtcgtaactcactgctgtgatatttgccagtgtttcctgcttcgtgtctcccaggaaaggggatgctccacttaagcttggactcttctttctattcccttgccacatctgactggccaaaagcttccttgttggttccatttactaaatatctcttgaaagtcatccccatttccacagccactttcttagcatggtggcagcaaggtgcactgtacaaattttggtgttgcaatcctgggtttgaatcccagctcagccactcattagctgtgtgaagctagaaccccttgtgtagtttcctcatctgcaaaatgaagaaaataaaattcccacctcatgtgattgctgtgaagaatacatgcatacaaaagccttcatgcaatcctggcccacactaagggctctggaattaatggccattattattgtcattgtgagaacacaaaagccctctatgacttcccatcttctacaggatcacatctaaactcttgagcaaggcatcaagagttggtccttaccccacgcttggtacacttcagccacacttaaggtttaccgttccttttctcatgccatttcctcagccagcacagcccttccctcctccacccacagaattaacttcgttccctacatcccagttcaaattgatccatcaatcatgtgctgtctctatttctctctcaataaaccttcagcagtccagcaaaccagtggctccccatctgtgtctcaaagaggcatgttcattcctccagcctaaccttggttccactgggtgtgagttaggtgtatggtgtgtctcccacagacagggagccccagcaagcagggaagaccctccttcatgtcagtatcctagtgcctggtacagtgcctgccatggagcagacctcaacaaagctgttaaattcaaatgagccacaagaagactatgtgctcagtagacactgggattccatttttttttttttttgagacagggtcttgctctgttgcccaggacggagtgcagtggtgctactaca

SEQ ID NO: 12576 - RNA, 789 nt, Homo sapiens
  source 1..789: mol_type = other RNA
gagtgccttcttttggagcgtttattttcacttgatattctagattaacattcctttgctcttgatcaggatttggtttccattgtaaaagaacttgagccaaaccagtaactttaatggtgaaattgacaggtgggagaagtgaaatcttttcatcaggaagtaagtcagcttgcagtatctcagtggcccccaaaaggatgagtaatacatgcgccacgatgatcatatcctgtctacagacgatcctcttgttccgaccagtactcaacagaagatggcgaggaccgtgtctgtcgtgtctatgctcgtggctgcaaccccagcatctagcatagcgtcaggcacaggaccaatgctcaatgtgcctggcccttatctctgggtgcactttttaacttagaggcggttcttcactctttcatcatcacggctgtaatggttaaaaactctcaggcagcttccttcatgatgggatggcaacacgttttctctaagcaaatatggaggaggatttgtacagagcaactgtgcaggagctgaactggaactcccaacaaccaaactgctgtcaaacgaaagaatctctcgtccagatagccattatctgataactgtcttgtctgcattttcactctctttcagagttggtttgctctcttcaggagtgggaattaacttttactcatggtgacaaggtaaacaagttttccgtgggtactctaaagcgttgcatttctgttttgtttatgtgccttgtttggctacagtagttactgtgcctctgtc

SEQ ID NO: 12577 - RNA, 804 nt, Homo sapiens
  source 1..804: mol_type = other RNA
gagtgccttcttttggagcgtttattttcacttgatattctagattaacattcctttgctcttgatcaggatttggtttccattgtaaaagaacttgagccaaaccagtaactttaatggtgaaattgacaggtgggagaagtgaaatcttttcatcaggaagtaagtcagcttgcagtatctcagtggcccccaaaaggatgagtaatacatgcgccacgatgatcatatcctgtctacagacgatcctcttgttccgaccagtactcaacagaagatggcgaggaccgtgtctgtcgtgtctatgctcgtggctgcaaccccagcatctagcatagcgtcaggcacaggaccaatgctcaatgtgcctggcctgagaaatgcggtggccatgcgatgagaagcagcggcagggcattgagaacgaaccttatctctgggtgcactttttaacttagaggcggttcttcactctttcatcatcacggctgtaatggttaaaaactctcaggcagcttccttcatgatgggatggcaacacgttttctctaagcaaatatggaggaggatttgtacagagcaactgtgcaggagctgaactggaactcccaacaaccaaactgctgtcaaacgaaagaatctctcgtccagatagccattatctgataactgtcttgtctgcattttcactctctttcagagttggtttgctctcttcaggagtgggaattaacttttactcatggtgacaaggtaaacaagttttccgtgggtactctaaagcgttgcatttctgttttgttt

SEQ ID NO: 12578 - RNA, 873 nt, Homo sapiens
  source 1..873: mol_type = other RNA
gagtgccttcttttggagcgtttattttcacttgatattctagattaacattcctttgctcttgatcaggatttggtttccattgtaaaagaacttgagccaaaccagtaactttaatggtgaaattgacaggtgggagaagtgaaatcttttcatcaggaagtaagtcagcttgcagtatctcagtggcccccaaaaggatgagtaatacatgcgccacgatgatcatatcctttttcactatgaggatttaaagatgagtgaacatgacaggaaacttcaatctaaaacaatctgtagcctgtctacagacgatcctcttgttccgaccagtactcaacagaagatggcgaggaccgtgtctgtcgtgtctatgctcgtggctgcaaccccagcatctagcatagcgtcaggcacaggaccaatgctcaatgtgcctggcctgagaaatgcggtggccatgcgatgagaagcagcggcagggcattgagaacgaaccttatctctgggtgcactttttaacttagaggcggttcttcactctttcatcatcacggctgtaatggttaaaaactctcaggcagcttccttcatgatgggatggcaacacgttttctctaagcaaatatggaggaggatttgtacagagcaactgtgcaggagctgaactggaactcccaacaaccaaactgctgtcaaacgaaagaatctctcgtccagatagccattatctgataactgtcttgtctgcattttcactctctttcagagttggtttgctctcttcaggagtgggaattaacttttactcatggtgacaaggtaaacaagttttccgtgggtactctaaagcgttgcatttctgttttgttt

SEQ ID NO: 12579 - RNA, 1396 nt, Homo sapiens
  source 1..1396: mol_type = other RNA
gagtggataggggagtgtgtggagcaccctggctaatgctttttccccaccctatctggatgccattcactctaagaaacttctctgcactcagatcacaaaagctacctcctggtctgcccttggctgaagacttcccaaggtctctggacacacagattacaaagttcagaccccactaccaaatcagaggcatgtgtcaggagttccacgtgctgccagcatcagcagcatccaacaactagcatacatgaaacaggtaccatgtgccaggcattatacctgaactcttctagaatcttcagctgcagcccttctagcctgtgcaactctttgagataatgcatgccaatcctgagcacagtaccaggcagagccagcactcaatcactagtagctgttatagctattcatttttctgtacctttgcaatttatcttcacaactccttaaaatagaggtgtagctgttagctattgctgcgtaacaaaccaaccccaaacctagtagcttgaaacaatatccatttatccatgatcgcccatgagtccatgggtcagctggatgttctgtctttctgggaatgtctcagcagctattggctggctcacccttgcatctgtggtcatctggaaggtgggtgttctggaaggggatcagctgggacacttcacgtctgttgcatatggcctgtcatcttccaacaggccagcttgagctctccctgatggcttgaccaggggttgaggctctactttcaaggtggtgcactcacatgcccagcaagttcatgctggctgttggctgggggcctctccacagggctgctcagatgtcctcctcacatggcttccagacagagcagcaggagaaaaacaaaatcacagtgatcctttccatcctcttgcagcaaagaacctctccaaggagcgtcagcgtctgaatttgataccaactctggaaggttattaagtttgaactcccaactgcgttgtcagtagagttccagttcagtttccccattgtgaagtactcatgtgagacagagaccacttggtatttccgaagaattaaaacattcctccagccgggtctcactcgcaagtacaatatgatctcccatcgtatgcttttaaccataacctcctcaatatcccaacccaaacgtggtcagtgtaacttgcatggctccaattccaagacagggtcatcagacagtgatctctggaaaattcctcccaggtgggctacggtgggggaaaccggcctctctcggctccagagaggggagacggctctctagctgacttcctgtgtgggaaagagtcctctcactgacttccggtgtcagaaatgtccctctttccggccttcaaatatgagaaatgtttctctg

SEQ ID NO: 12580 - RNA, 34 nt, Homo sapiens
  source 1..34: mol_type = other RNA
gagtgtagttctgagcagagccacagagggaagt

SEQ ID NO: 12581 - RNA, 119 nt, Homo sapiens
  source 1..119: mol_type = other RNA
gagtgtagttctgagcagagccacagagggaagtgaggagacagagaacaggagaggccagcagagaagaaatgaaggcaggaggagggccaaggctcccagggaggggcaagggcaaa

SEQ ID NO: 12582 - RNA, 37 nt, Homo sapiens
  source 1..37: mol_type = other RNA
gagtgtagttctgagcagagcccacactgaatcctgg

SEQ ID NO: 12583 - RNA, 25 nt, Homo sapiens
  source 1..25: mol_type = other RNA
gatatcagctcagtaggcaccggag

SEQ ID NO: 12584 - RNA, 2798 nt, Homo sapiens
  source 1..2798: mol_type = other RNA
gatatcagctcagtaggcaccggagggcgggtccaatcgacagcccggagaagcagcgcctcagctgggagctccgtgggcaccgtctgctggcgcaggagacgcgaaggcctggactcgttaaaataacatttcggccaccacctgggctgaggacctatccatctgctccttggtccgctcgaagcacctacgggcgagctgctgctgtctggcgtcctcactcaccatcagctccccgtagaggtacacacccatggcctgatcctcctgaaggaacctctccacacttttgtaggctttcgtgaacttgtgcttaacaatgagttcacaccaccgatggcgaacctctgcatcctgatcctggaggtggtatgtcctctggaggctttgcagagttcgggggctcagagtcttctgctccaagagatgctccagaagcaagaccagctggtctggaagaagcttttcaaacacctcttccttctccctgcgcttccgttttcggggtctccggttcactccaatccatttcgtgacctcggcgcgcacttgccgcgcaagcccgcactccgccccggcgcgacgctccctctgcagcggctttggtattccggaactctcaagccagtcttggtagatgttttcaacagacagctcaagccttttttcttctggaatgttctccagtagcatttgaaggaaatcctgggaaagaatcagctgtccatgaaatgtgtgcacaaattttcttaaaaatgaaaaataggtttcatctccaagtcttttggcaagaaaccgaagaaggaagtagccctttaaataatgcacctgcatgaagatcttctccggattaagtccatgcttgataacagatgctcccgagtcacttgtgtggccagttttgtctttactgggtcttaacacctgcatctcctcgggggagcattgcatctcgtcctggaggcgacgccagcgcagacaagccctcagctcctgctgctcccgggcctcatagggggccagctgctgtgctgtggcccaaaacacatcctccaagtgagtggcgaagccttcactcagccactcctccgtccagtctcgggccccgatggctaggccaaaccaggcatgggcaatttcatggcagaggcgggtcccacagagatggttccctcctgtcaagatgctctgagagaggaacatgatgtgtgggctggccatccccagacttggaaagttggcagggacgatgagaacatccagccgagagaacgggtgtgctcccagaacagaatgtgctgctgagaggcaaggagggatcagccgcagaagggtctcttggcaggcacccgtgaggcacacaggggcaaagacccgatgaggaatgatctcctgggtggtggcagaagcattctggaagcggcaggggtattccatgtgactgcaaacaccaacatgcctgaagttggcctcagaaggtgagaagggtctctctgttgccaaatcatttgatgaccatgtctccatcttcatttctgtccagcatcccactgcaattgtgaaggtggaggctggcattggcatagttacatagtaataccagcttgagcactcttcccaaagctgcgttggtttggcagaattttccccactcattaaaacaacaaaagatgcagctgctcgaactgtagcctgccatgttgacatggcaacgggtggctcctggcatggaaaaagggccctgttgtttatgggagatcccacagtataaacacatggcctgccactctggtctgaggtccatgtaaccgatcgcccttcaggtttagttttgtaccatatcctgatagcatgaggaaagtcagtagctgtctgagcccctgtcttccttatctgcaagctccaagtgtcagtgtcaaagaggagttccccacagccaggagcctggctgcagcgagcgtaatagtctaactgctccctccaacgatttgcaggcaaagtcacaagttcacgtacaatctgattcctgaactcctcagaaacaaccgtgagctcaggagaccttgtaaatttttccagacctggcacagcagcaacatccacctcctcgacttttaacacagataaatcacagcagtccaacactagcaaaaaatcctcactcccatgattccctgtgtcacagcagtactttgagctagaaatcccagaagcatgttcctggttgtcatggttaccatctttatcagaagtatctttttcacctttactacagattgcaaaatcattatattccatttcagatgagaaggtccttgcatttgtcacgggaatatggcagggttcaggcatcccaaatttgcaggctttgtttgattctgattggcaggcttcctcaatagagctattctgtttcttgaatctgtttccatcctcgaggaaaagcactatggtcccctcaatgacttgactttcaaaatccacatccaaatccagtacatagtgcttcacaagtatgtggctggtgttggccatgagaggcaggtcatctctggcagggtccagctgtatgtccatgatgtggtttattgtttgagggatttattaaaatctcagatggggtttcctatctgccttaatcttccagaatcataaatagctgcttatcaaagaaaacaactgatgtcacaaattatggttcctttcagtctcctgtctcagccgcgtcccacgggtcaccacttccgcagactcggggttactacgggctaccccggcacgcgccgggtgacgtc

SEQ ID NO: 12585 - RNA, 5667 nt, Homo sapiens
  source 1..5667: mol_type = other RNA
gatatcagctcagtaggcaccggagggcgggtccaatcgacagcccggagaagcagcgcctcagctgggagctccgtgggcaccgtctgctggcgcaggagacgcgaaggcctggactgcaaatacaagagagagttcaccgcgcccagaacaacaggagctcctccgaaagccccgccccgccccgctcacagccatgagctaccacatgatttcacacgacttaggtgatgcatttggttttagttttttgtaagaagaatttttgcaactttcaatacatttgacctttcagacagatgtccgattagtgcatgtttctgtggacagacttaaggactcagtacatggctagcattcccagcaggagacagtgcatccttggggtcaagtggtctctcatcctccaggatcgcgctccgcacccaagctgactgtgcagcagcggccggcccgtcagcaacggcctctgccccagcggctccaacttaactgtccccatctcaccttctcttcaggtgcagaacttagccactgtgaacaaagcggaaaccaatcactgttcaccaatcagctaagctctgcaccttgttagagaggtcatcgctgggcataaataaagggacggtgaccggtgagcatcttcctcagctggtggcttcttttgtttccaaagaagagctacgagatgcacctgttctccaatctgcagtgagcgcgaccacggtttctggaggagcagccaaggtcgtggttgcgtggtaatccctggcaatgtgattttaatcttaagtcacaaatcagcatgccaggaacccaagcagccagagcacctgagagcagcgccaccccgtgctgtctgcacacactgggcttccgcggaaggacgccggcgacactgccgccttcacgcctgttatgctagcaaacaggtggagtttctgtttgttgttcgtttagttggcatcctagaggtataatttcttgaatcaaagggactccagagatgaccataaaaatgccagtgcagctttggaactgaagaaaaatgcagggaccggccatgcgacacacacaattgctaaaggcagctgtccttgctattagtttactgcctctaacccttggggacaagatcccttctctccaggcagattctagctgccctgggaaggctttggggactctcaagtcaggaggtccccctgctggaaggggccctgggacaatcccggccactgttcctcacggggactggttggggggcaggcttgcaacccctggatgcatctggaggggtggggacaggatcgaagatgctggggagggggaaaagggagacttgtgaccaagatgactcctttgcctgcctgggcaaaaattccccataaagagtggcgaggggtgtgccctgtggtgctgctccaaaacctgcaccaaagggaatgatgaaaggactagctggccttgtagtttcacacactttaacacgtacgccacgaaataacaaaacgaaagagaaacaccatttacactgattactattatgaggccggcagtgaggtaagtgcacagtctgtgtgccgccagcccgtcctggaggggagccgcgtcaagtctgcagcaggcgtttcgctacgagacgctcagtcccgtttccctttcctggcacacatggttcctgactcttctggaagaatatgatcatgcttctgaaaaactttttatttcttttcattattagagttctttcagataaataagctacttaaacacgttacacagaaatggttttcataagcacaaaacattagaagaaaactcaatgttcaaaactgagtgaagaatatcaacaccaaatattcaatatccatgaaaaattatagagaagctataacacgaaaaatgcttcagatttgataaagtttttttaaagatacaaaattagacatcccctattaatatcatataaaacactgaagaaaaacggagcagacacagaaataatgatgattgttagagaaaaaaaatctcacagctatcctaacaaaaccttgtgtactaccgctaggttgctttaatagtgtagaaacccatactgagcaactaactgctaggaagtaaatctaacaggttaattccaggcacaattaacagaggaagtgatttaaataatctaggactccaatagaagccaggggagaaattccgctccaacacaacaaagcaaaaagtaggacctgccctcaagacacagggtcatggaggccatatgccacgtgtgctgtgtgcgccgcgggtgctgtgtggtgcgtgcactgtgtgtgccacatgtgctctgtgtggtgcgtgcggtgtgtgctgtgtgtgccgcaggtgctctgtgtggtgcacgcgctgtgtgtggtgtgtgtgctgcatgcagtgtgcgcgctacgtgtggtgcatgtgctgtgtgtgctctgtgttgtgcatgcgctgtgtgtggtgtgtgtgccgcgtgtactctgcgtggtgtgtgtgctgtgggtgctccaggtgctctgtgtggtgtgtgtgctgcgtgtgccgcgtgtgctctgtgtggtgcgtgcgctgtttggtgtgtatgctgcatgtgccgtgtgtgctctgcgtggtgcgtgcgctgtgtgtgctgtgtgtgccgcgtgtgctctgtgtggtgcgtgcgctgtgtggtgtgtgctgtgcgtgctctgtgtggtgcgtcctctggtgtgtgtgtgctgcatgcagtgtgtgtgctacgtgtggtgcatgtgctgtgtgtgctgcgtgtgcctggagagcctcctgccagccgatgaccaggcgtggacagcccaaggaacctccaattcacacatggctagaagaaaacatctgcttgcagaagctaggctttggagtcacacggccgcttaaactcctgtatcagccgtgaccctgaagactggaccagcgcttctgccaggcttcccattccatctctaaacctactcaagatgttcccccacaatttttgtttcaacagattataaaacctgaagtggccaaaatagtgccaaggagtgccgctgtgcctccaggtggacagcctctgcttcccggtgactgccacagccaggcaaggtgctccagggacccggggctcccataccagcccagcacccacttggccagttactctccaggccctgggccagggagccgactattgatgctgcgggtagtcttggctaactattcggcttactgatttagttggctcctaaaaggagtatctggttagaactaaatgacagaaaggaaagggagagaatcacctcgttaaaataacatttcggccaccacctgggctgaggacctatccatctgctccttggtccgctcgaagcacctacgggcgagctgctgctgtctggcgtcctcactcaccatcagctccccgtagaggtacacacccatggcctgatcctcctgaaggaacctctccacacttttgtaggctttcgtgaacttgtgcttaacaatgagttcacaccaccgatggcgaacctctgcatcctgatcctggaggtggtatgtcctctggaggctttgcagagttcgggggctcagagtcttctgctccaagagatgctccagaagcaagaccagctggtctggaagaagcttttcaaacacctcttccttctccctgcgcttccgttttcggggtctccggttcactccaatccatttcgtgacctcggcgcgcacttgccgcgcaagcccgcactccgccccggcgcgacgctccctctgcagcggctttggtattccggaactctcaagccagtcttggtagatgttttcaacagacagctcaagcctgggaaagaatcagctgtccatgaaatgtgtgcacaaattttcttaaaaatgaaaaataggtttcatctccaagtcttttggcaagaaaccgaagaaggaagtagccctttaaataatgcacctgcatgaagatcttctccggattaagtccatgcttgataacagatgctcccgagtcacttgtgtggccagttttgtctttactgggtctggccatccccagacttggaaagttggcagggacgatgagaacatccagccgagagaacgggtgtgctcccagaacagaatgtgctgctgagaggcaaggagggatcagccgcagaagggtctcttggcaggcacccgtgaggcacacaggggcaaagacccgatgaggaatgatctcctgggtggtggcagaagcattctggaagcggcaggggtattccatgtgactgcaaacaccaacatgcctgaagttggcctcagaaggtgagaagggtctctctgttgccaaatcatttgatgaccatgtctccatcttcatttctgtccagcatcccactgcaattgtgaaggtggaggctggcattggcatagttacatagtaataccagcttgagcactcttcccaaagctgcgttggtttggcagaattttccccactcattaaaacaacaaaagatgcagctgctcgaactgtagcctgccatgttgacatggcaacgggtggctcctggcatggaaaaagggccctgttgtttatgggagatcccacagtataaacacatggcctgccactctggtctgaggtccatgtaaccgatcgcccttcaggtttagttttgtaccatatcctgatagcatgaggaaagtcagtagctgtctgagcccctgtcttccttatctgcaagctccaagtgtcagtgtcaaagaggagttccccacagccaggagcctggctgcagcgagcgtaatagtctaactgctccctccaacgatttgcaggcaaagtcacaagttcacgtacaatctgattcctgaactcctcagaaacaaccgtgagctcaggagaccttgtaaatttttccagacctggcacagcagcaacatccacctcctcgacttttaacacagataaatcacagcagtccaacactagcaaaaaatcctcactcccatgattccctgtgtcacagcagtactttgagctagaaatcccagaagcatgttcctggttgtcatggttaccatctttatcagaagtatctttttcacctttactacagattgcaaaatcattatattccatttcagatgagaaggtccttgcatttgtcacgggaatatggcagggttcaggcatcccaaatttgcaggctttgtttgattctgattggcaggcttcctcaatagagctattctgtttcttgaatctgtttccatcctcgaggaaaagcactatggtcccctcaatgacttgactttcaaaatccacatccaaatccagtacatagtgcttcacaagtatgtggctggtgttggccatgagaggcaggtcatctctggcagggtccagctgtatgtccatgatgtggtttattgtttgagggatttattaaaatctcagatggggtttcctatctgccttaatcttccagaatcataaatagctgcttatcaaagaaaacaactgatgtcacaaattatggttcctttcagtctcctgtctcagccgcgtcccacgggtcaccacttccgcagactcggggttactacgggctaccccggcacgcgccgggtgacgtc

SEQ ID NO: 12586 - RNA, 5544 nt, Homo sapiens
  source 1..5544: mol_type = other RNA
gatatcagctcagtaggcaccggagggcgggtccaatcgacagcccggagaagcagcgcctcagctgggagctccgtgggcaccgtctgctggcgcaggagacgcgaaggcctggactgcaaatacaagagagagttcaccgcgcccagaacaacaggagctcctccgaaagccccgccccgccccgctcacagccatgagctaccacatgatttcacacgacttaggtgatgcatttggttttagttttttgtaagaagaatttttgcaactttcaatacatttgacctttcagacagatgtccgattagtgcatgtttctgtggacagacttaaggactcagtacatggctagcattcccagcaggagacagtgcatccttggggtcaagtggtctctcatcctccaggatcgcgctccgcacccaagctgactgtgcagcagcggccggcccgtcagcaacggcctctgccccagcggctccaacttaactgtccccatctcaccttctcttcaggtgcagaacttagccactgtgaacaaagcggaaaccaatcactgttcaccaatcagctaagctctgcaccttgttagagaggtcatcgctgggcataaataaagggacggtgaccggtgagcatcttcctcagctggtggcttcttttgtttccaaagaagagctacgagatgcacctgttctccaatctgcagtgagcgcgaccacggtttctggaggagcagccaaggtcgtggttgcgtggtaatccctggcaatgtgattttaatcttaagtcacaaatcagcatgccaggaacccaagcagccagagcacctgagagcagcgccaccccgtgctgtctgcacacactgggcttccgcggaaggacgccggcgacactgccgccttcacgcctgttatgctagcaaacaggtggagtttctgtttgttgttcgtttagttggcatcctagaggtataatttcttgaatcaaagggactccagagatgaccataaaaatgccagtgcagctttggaactgaagaaaaatgcagggaccggccatgcgacacacacaattgctaaaggcagctgtccttgctattagtttactgcctctaacccttggggacaagatcccttctctccaggcagattctagctgccctgggaaggctttggggactctcaagtcaggaggtccccctgctggaaggggccctgggacaatcccggccactgttcctcacggggactggttggggggcaggcttgcaacccctggatgcatctggaggggtggggacaggatcgaagatgctggggagggggaaaagggagacttgtgaccaagatgactcctttgcctgcctgggcaaaaattccccataaagagtggcgaggggtgtgccctgtggtgctgctccaaaacctgcaccaaagggaatgatgaaaggactagctggccttgtagtttcacacactttaacacgtacgccacgaaataacaaaacgaaagagaaacaccatttacactgattactattatgaggccggcagtgaggtaagtgcacagtctgtgtgccgccagcccgtcctggaggggagccgcgtcaagtctgcagcaggcgtttcgctacgagacgctcagtcccgtttccctttcctggcacacatggttcctgactcttctggaagaatatgatcatgcttctgaaaaactttttatttcttttcattattagagttctttcagataaataagctacttaaacacgttacacagaaatggttttcataagcacaaaacattagaagaaaactcaatgttcaaaactgagtgaagaatatcaacaccaaatattcaatatccatgaaaaattatagagaagctataacacgaaaaatgcttcagatttgataaagtttttttaaagatacaaaattagacatcccctattaatatcatataaaacactgaagaaaaacggagcagacacagaaataatgatgattgttagagaaaaaaaatctcacagctatcctaacaaaaccttgtgtactaccgctaggttgctttaatagtgtagaaacccatactgagcaactaactgctaggaagtaaatctaacaggttaattccaggcacaattaacagaggaagtgatttaaataatctaggactccaatagaagccaggggagaaattccgctccaacacaacaaagcaaaaagtaggacctgccctcaagacacagggtcatggaggccatatgccacgtgtgctgtgtgcgccgcgggtgctgtgtggtgcgtgcactgtgtgtgccacatgtgctctgtgtggtgcgtgcggtgtgtgctgtgtgtgccgcaggtgctctgtgtggtgcacgcgctgtgtgtggtgtgtgtgctgcatgcagtgtgcgcgctacgtgtggtgcatgtgctgtgtgtgctctgtgttgtgcatgcgctgtgtgtggtgtgtgtgccgcgtgtactctgcgtggtgtgtgtgctgtgggtgctccaggtgctctgtgtggtgtgtgtgctgcgtgtgccgcgtgtgctctgtgtggtgcgtgcgctgtttggtgtgtatgctgcatgtgccgtgtgtgctctgcgtggtgcgtgcgctgtgtgtgctgtgtgtgccgcgtgtgctctgtgtggtgcgtgcgctgtgtggtgtgtgctgtgcgtgctctgtgtggtgcgtcctctggtgtgtgtgtgctgcatgcagtgtgtgtgctacgtgtggtgcatgtgctgtgtgtgctgcgtgtgcctggagagcctcctgccagccgatgaccaggcgtggacagcccaaggaacctccaattcacacatggctagaagaaaacatctgcttgcagaagctaggctttggagtcacacggccgcttaaactcctgtatcagccgtgaccctgaagactggaccagcgcttctgccaggcttcccattccatctctaaacctactcaagatgttcccccacaatttttgtttcaacagattataaaacctgaagtggccaaaatagtgccaaggagtgccgctgtgcctccaggtggacagcctctgcttcccggtgactgccacagccaggcaaggtgctccagggacccggggctcccataccagcccagcacccacttggccagttactctccaggccctgggccagggagccgactattgatgctgcgggtagtcttggctaactattcggcttactgatttagttggctcctaaaaggagtatctggttagaactaaatgacagaaaggaaagggagagaatcacctcgttaaaataacatttcggccaccacctgggctgaggacctatccatctgctccttggtccgctcgaagcacctacgggcgagctgctgctgtctggcgtcctcactcaccatcagctccccgtagaggtacacacccatggcctgatcctcctgaaggaacctctccacacttttgtaggctttcgtgaacttgtgcttaacaatgagttcacaccaccgatggcgaacctctgcatcctgatcctggaggtggtatgtcctctggaggctttgcagagttcgggggctcagagtcttctgctccaagagatgctccagaagcaagaccagctggtctggaagaagcttttcaaacacctcttccttctccctgcgcttccgttttcggggtctccggttcactccaatccatttcgtgacctcggcgcgcacttgccgcgcaagcccgcactccgccccggcgcgacgctccctctgcagcggctttggtattccggaactctcaagccagtcttggtagatgttttcaacagacagctcaagccttttttcttctggaatgttctccagtagcatttgaaggaaatcctgggaaagaatcagctgtccatgaaatgtgtgcacaaattttcttaaaaatgaaaaataggtttcatctccaagtcttttggcaagaaaccgaagaaggaagtagccctttaaataatgcacctgcatgaagatcttctccggattaagtccatgcttgataacagatgctcccgagtcacttgtgtggccagttttgtctttactgggtctggccatccccagacttggaaagttggcagggacgatgagaacatccagccgagagaacgggtgtgctcccagaacagaatgtgctgctgagaggcaaggagggatcagccgcagaagggtctcttggcaggcacccgtgaggcacacaggggcaaagacccgatgaggaatgatctcctgggtggtggcagaagcattctggaagcggcaggggtattccatgtgactgcaaacaccaacatgcctgaagttggcctcagaaggtgagaagggtctctctgttgccaaatcatttgatgaccatgtctccatcttcatttctgtccagcatcccactgcaattgtgaaggtggaggctggcattggcatagttacatagtaataccagcttgagcactctgccactctggtctgaggtccatgtaaccgatcgcccttcaggtttagttttgtaccatatcctgatagcatgaggaaagtcagtagctgtctgagcccctgtcttccttatctgcaagctccaagtgtcagtgtcaaagaggagttccccacagccaggagcctggctgcagcgagcgtaatagtctaactgctccctccaacgatttgcaggcaaagtcacaagttcacgtacaatctgattcctgaactcctcagaaacaaccgtgagctcaggagaccttgtaaatttttccagacctggcacagcagcaacatccacctcctcgacttttaacacagataaatcacagcagtccaacactagcaaaaaatcctcactcccatgattccctgtgtcacagcagtactttgagctagaaatcccagaagcatgttcctggttgtcatggttaccatctttatcagaagtatctttttcacctttactacagattgcaaaatcattatattccatttcagatgagaaggtccttgcatttgtcacgggaatatggcagggttcaggcatcccaaatttgcaggctttgtttgattctgattggcaggcttcctcaatagagctattctgtttcttgaatctgtttccatcctcgaggaaaagcactatggtcccctcaatgacttgactttcaaaatccacatccaaatccagtacatagtgcttcacaagtatgtggctggtgttggccatgagaggcaggtcatctctggcagggtccagctgtatgtccatgatgtggtttattgtttgagggatttattaaaatctcagatggggtttcctatctgccttaatcttccagaatcataaatagctgcttatcaaagaaaacaactgatgtcacaaattatggttcctttcagtctcctgtctcagccgcgtcccacgggtcaccacttccgcagactcggggttactacgggctaccccggcacgcgccgggtgacgtc

SEQ ID NO: 12587 - RNA, 5711 nt, Homo sapiens
  source 1..5711: mol_type = other RNA
gatatcagctcagtaggcaccggagggcgggtccaatcgacagcccggagaagcagcgcctcagctgggagctccgtgggcaccgtctgctggcgcaggagacgcgaaggcctggactgcaaatacaagagagagttcaccgcgcccagaacaacaggagctcctccgaaagccccgccccgccccgctcacagccatgagctaccacatgatttcacacgacttaggtgatgcatttggttttagttttttgtaagaagaatttttgcaactttcaatacatttgacctttcagacagatgtccgattagtgcatgtttctgtggacagacttaaggactcagtacatggctagcattcccagcaggagacagtgcatccttggggtcaagtggtctctcatcctccaggatcgcgctccgcacccaagctgactgtgcagcagcggccggcccgtcagcaacggcctctgccccagcggctccaacttaactgtccccatctcaccttctcttcaggtgcagaacttagccactgtgaacaaagcggaaaccaatcactgttcaccaatcagctaagctctgcaccttgttagagaggtcatcgctgggcataaataaagggacggtgaccggtgagcatcttcctcagctggtggcttcttttgtttccaaagaagagctacgagatgcacctgttctccaatctgcagtgagcgcgaccacggtttctggaggagcagccaaggtcgtggttgcgtggtaatccctggcaatgtgattttaatcttaagtcacaaatcagcatgccaggaacccaagcagccagagcacctgagagcagcgccaccccgtgctgtctgcacacactgggcttccgcggaaggacgccggcgacactgccgccttcacgcctgttatgctagcaaacaggtggagtttctgtttgttgttcgtttagttggcatcctagaggtataatttcttgaatcaaagggactccagagatgaccataaaaatgccagtgcagctttggaactgaagaaaaatgcagggaccggccatgcgacacacacaattgctaaaggcagctgtccttgctattagtttactgcctctaacccttggggacaagatcccttctctccaggcagattctagctgccctgggaaggctttggggactctcaagtcaggaggtccccctgctggaaggggccctgggacaatcccggccactgttcctcacggggactggttggggggcaggcttgcaacccctggatgcatctggaggggtggggacaggatcgaagatgctggggagggggaaaagggagacttgtgaccaagatgactcctttgcctgcctgggcaaaaattccccataaagagtggcgaggggtgtgccctgtggtgctgctccaaaacctgcaccaaagggaatgatgaaaggactagctggccttgtagtttcacacactttaacacgtacgccacgaaataacaaaacgaaagagaaacaccatttacactgattactattatgaggccggcagtgaggtaagtgcacagtctgtgtgccgccagcccgtcctggaggggagccgcgtcaagtctgcagcaggcgtttcgctacgagacgctcagtcccgtttccctttcctggcacacatggttcctgactcttctggaagaatatgatcatgcttctgaaaaactttttatttcttttcattattagagttctttcagataaataagctacttaaacacgttacacagaaatggttttcataagcacaaaacattagaagaaaactcaatgttcaaaactgagtgaagaatatcaacaccaaatattcaatatccatgaaaaattatagagaagctataacacgaaaaatgcttcagatttgataaagtttttttaaagatacaaaattagacatcccctattaatatcatataaaacactgaagaaaaacggagcagacacagaaataatgatgattgttagagaaaaaaaatctcacagctatcctaacaaaaccttgtgtactaccgctaggttgctttaatagtgtagaaacccatactgagcaactaactgctaggaagtaaatctaacaggttaattccaggcacaattaacagaggaagtgatttaaataatctaggactccaatagaagccaggggagaaattccgctccaacacaacaaagcaaaaagtaggacctgccctcaagacacagggtcatggaggccatatgccacgtgtgctgtgtgcgccgcgggtgctgtgtggtgcgtgcactgtgtgtgccacatgtgctctgtgtggtgcgtgcggtgtgtgctgtgtgtgccgcaggtgctctgtgtggtgcacgcgctgtgtgtggtgtgtgtgctgcatgcagtgtgcgcgctacgtgtggtgcatgtgctgtgtgtgctctgtgttgtgcatgcgctgtgtgtggtgtgtgtgccgcgtgtactctgcgtggtgtgtgtgctgtgggtgctccaggtgctctgtgtggtgtgtgtgctgcgtgtgccgcgtgtgctctgtgtggtgcgtgcgctgtttggtgtgtatgctgcatgtgccgtgtgtgctctgcgtggtgcgtgcgctgtgtgtgctgtgtgtgccgcgtgtgctctgtgtggtgcgtgcgctgtgtggtgtgtgctgtgcgtgctctgtgtggtgcgtcctctggtgtgtgtgtgctgcatgcagtgtgtgtgctacgtgtggtgcatgtgctgtgtgtgctgcgtgtgcctggagagcctcctgccagccgatgaccaggcgtggacagcccaaggaacctccaattcacacatggctagaagaaaacatctgcttgcagaagctaggctttggagtcacacggccgcttaaactcctgtatcagccgtgaccctgaagactggaccagcgcttctgccaggcttcccattccatctctaaacctactcaagatgttcccccacaatttttgtttcaacagattataaaacctgaagtggccaaaatagtgccaaggagtgccgctgtgcctccaggtggacagcctctgcttcccggtgactgccacagccaggcaaggtgctccagggacccggggctcccataccagcccagcacccacttggccagttactctccaggccctgggccagggagccgactattgatgctgcgggtagtcttggctaactattcggcttactgatttagttggctcctaaaaggagtatctggttagaactaaatgacagaaaggaaagggagagaatcacctcgttaaaataacatttcggccaccacctgggctgaggacctatccatctgctccttggtccgctcgaagcacctacgggcgagctgctgctgtctggcgtcctcactcaccatcagctccccgtagaggtacacacccatggcctgatcctcctgaaggaacctctccacacttttgtaggctttcgtgaacttgtgcttaacaatgagttcacaccaccgatggcgaacctctgcatcctgatcctggaggtggtatgtcctctggaggctttgcagagttcgggggctcagagtcttctgctccaagagatgctccagaagcaagaccagctggtctggaagaagcttttcaaacacctcttccttctccctgcgcttccgttttcggggtctccggttcactccaatccatttcgtgacctcggcgcgcacttgccgcgcaagcccgcactccgccccggcgcgacgctccctctgcagcggctttggtattccggaactctcaagccagtcttggtagatgttttcaacagacagctcaagccttttttcttctggaatgttctccagtagcatttgaaggaaatcctgggaaagaatcagctgtccatgaaatgtgtgcacaaattttcttaaaaatgaaaaataggtttcatctccaagtcttttggcaagaaaccgaagaaggaagtagccctttaaataatgcacctgcatgaagatcttctccggattaagtccatgcttgataacagatgctcccgagtcacttgtgtggccagttttgtctttactgggtctggccatccccagacttggaaagttggcagggacgatgagaacatccagccgagagaacgggtgtgctcccagaacagaatgtgctgctgagaggcaaggagggatcagccgcagaagggtctcttggcaggcacccgtgaggcacacaggggcaaagacccgatgaggaatgatctcctgggtggtggcagaagcattctggaagcggcaggggtattccatgtgactgcaaacaccaacatgcctgaagttggcctcagaaggtgagaagggtctctctgttgccaaatcatttgatgaccatgtctccatcttcatttctgtccagcatcccactgcaattgtgaaggtggaggctggcattggcatagttacatagtaataccagcttgagcactcttcccaaagctgcgttggtttggcagaattttccccactcattaaaacaacaaaagatgcagctgctcgaactgtagcctgccatgttgacatggcaacgggtggctcctggcatggaaaaagggccctgttgtttatgggagatcccacagtataaacacatggcctgccactctggtctgaggtccatgtaaccgatcgcccttcaggtttagttttgtaccatatcctgatagcatgaggaaagtcagtagctgtctgagcccctgtcttccttatctgcaagctccaagtgtcagtgtcaaagaggagttccccacagccaggagcctggctgcagcgagcgtaatagtctaactgctccctccaacgatttgcaggcaaagtcacaagttcacgtacaatctgattcctgaactcctcagaaacaaccgtgagctcaggagaccttgtaaatttttccagacctggcacagcagcaacatccacctcctcgacttttaacacagataaatcacagcagtccaacactagcaaaaaatcctcactcccatgattccctgtgtcacagcagtactttgagctagaaatcccagaagcatgttcctggttgtcatggttaccatctttatcagaagtatctttttcacctttactacagattgcaaaatcattatattccatttcagatgagaaggtccttgcatttgtcacgggaatatggcagggttcaggcatcccaaatttgcaggctttgtttgattctgattggcaggcttcctcaatagagctattctgtttcttgaatctgtttccatcctcgaggaaaagcactatggtcccctcaatgacttgactttcaaaatccacatccaaatccagtacatagtgcttcacaagtatgtggctggtgttggccatgagaggcaggtcatctctggcagggtccagctgtatgtccatgatgtggtttattgtttgagggatttattaaaatctcagatggggtttcctatctgccttaatcttccagaatcataaatagctgcttatcaaagaaaacaactgatgtcacaaattatggttcctttcagtctcctgtctcagccgcgtcccacgggtcaccacttccgcagactcggggttactacgggctaccccggcacgcgccgggtgacgtc

SEQ ID NO: 12588 - RNA, 6008 nt, Homo sapiens
  source 1..6008: mol_type = other RNA
gatatcagctcagtaggcaccggagggcgggtccaatcgacagcccggagaagcagcgcctcagctgggagctccgtgggcaccgtctgctggcgcaggagacgcgaaggcctggactgcaaatacaagagagagttcaccgcgcccagaacaacaggagctcctccgaaagccccgccccgccccgctcacagccatgagctaccacatgatttcacacgacttaggtgatgcatttggttttagttttttgtaagaagaatttttgcaactttcaatacatttgacctttcagacagatgtccgattagtgcatgtttctgtggacagacttaaggactcagtacatggctagcattcccagcaggagacagtgcatccttggggtcaagtggtctctcatcctccaggatcgcgctccgcacccaagctgactgtgcagcagcggccggcccgtcagcaacggcctctgccccagcggctccaacttaactgtccccatctcaccttctcttcaggtgcagaacttagccactgtgaacaaagcggaaaccaatcactgttcaccaatcagctaagctctgcaccttgttagagaggtcatcgctgggcataaataaagggacggtgaccggtgagcatcttcctcagctggtggcttcttttgtttccaaagaagagctacgagatgcacctgttctccaatctgcagtgagcgcgaccacggtttctggaggagcagccaaggtcgtggttgcgtggtaatccctggcaatgtgattttaatcttaagtcacaaatcagcatgccaggaacccaagcagccagagcacctgagagcagcgccaccccgtgctgtctgcacacactgggcttccgcggaaggacgccggcgacactgccgccttcacgcctgttatgctagcaaacaggtggagtttctgtttgttgttcgtttagttggcatcctagaggtataatttcttgaatcaaagggactccagagatgaccataaaaatgccagtgcagctttggaactgaagaaaaatgcagggaccggccatgcgacacacacaattgctaaaggcagctgtccttgctattagtttactgcctctaacccttggggacaagatcccttctctccaggcagattctagctgccctgggaaggctttggggactctcaagtcaggaggtccccctgctggaaggggccctgggacaatcccggccactgttcctcacggggactggttggggggcaggcttgcaacccctggatgcatctggaggggtggggacaggatcgaagatgctggggagggggaaaagggagacttgtgaccaagatgactcctttgcctgcctgggcaaaaattccccataaagagtggcgaggggtgtgccctgtggtgctgctccaaaacctgcaccaaagggaatgatgaaaggactagctggccttgtagtttcacacactttaacacgtacgccacgaaataacaaaacgaaagagaaacaccatttacactgattactattatgaggccggcagtgaggtaagtgcacagtctgtgtgccgccagcccgtcctggaggggagccgcgtcaagtctgcagcaggcgtttcgctacgagacgctcagtcccgtttccctttcctggcacacatggttcctgactcttctggaagaatatgatcatgcttctgaaaaactttttatttcttttcattattagagttctttcagataaataagctacttaaacacgttacacagaaatggttttcataagcacaaaacattagaagaaaactcaatgttcaaaactgagtgaagaatatcaacaccaaatattcaatatccatgaaaaattatagagaagctataacacgaaaaatgcttcagatttgataaagtttttttaaagatacaaaattagacatcccctattaatatcatataaaacactgaagaaaaacggagcagacacagaaataatgatgattgttagagaaaaaaaatctcacagctatcctaacaaaaccttgtgtactaccgctaggttgctttaatagtgtagaaacccatactgagcaactaactgctaggaagtaaatctaacaggttaattccaggcacaattaacagaggaagtgatttaaataatctaggactccaatagaagccaggggagaaattccgctccaacacaacaaagcaaaaagtaggacctgccctcaagacacagggtcatggaggccatatgccacgtgtgctgtgtgcgccgcgggtgctgtgtggtgcgtgcactgtgtgtgccacatgtgctctgtgtggtgcgtgcggtgtgtgctgtgtgtgccgcaggtgctctgtgtggtgcacgcgctgtgtgtggtgtgtgtgctgcatgcagtgtgcgcgctacgtgtggtgcatgtgctgtgtgtgctctgtgttgtgcatgcgctgtgtgtggtgtgtgtgccgcgtgtactctgcgtggtgtgtgtgctgtgggtgctccaggtgctctgtgtggtgtgtgtgctgcgtgtgccgcgtgtgctctgtgtggtgcgtgcgctgtttggtgtgtatgctgcatgtgccgtgtgtgctctgcgtggtgcgtgcgctgtgtgtgctgtgtgtgccgcgtgtgctctgtgtggtgcgtgcgctgtgtggtgtgtgctgtgcgtgctctgtgtggtgcgtcctctggtgtgtgtgtgctgcatgcagtgtgtgtgctacgtgtggtgcatgtgctgtgtgtgctgcgtgtgcctggagagcctcctgccagccgatgaccaggcgtggacagcccaaggaacctccaattcacacatggctagaagaaaacatctgcttgcagaagctaggctttggagtcacacggccgcttaaactcctgtatcagccgtgaccctgaagactggaccagcgcttctgccaggcttcccattccatctctaaacctactcaagatgttcccccacaatttttgtttcaacagattataaaacctgaagtggccaaaatagtgccaaggagtgccgctgtgcctccaggtggacagcctctgcttcccggtgactgccacagccaggcaaggtgctccagggacccggggctcccataccagcccagcacccacttggccagttactctccaggccctgggccagggagccgactattgatgctgcgggtagtcttggctaactattcggcttactgatttagttggctcctaaaaggagtatctggttagaactaaatgacagaaaggaaagggagagaatcacctcgttaaaataacatttcggccaccacctgggctgaggacctatccatctgctccttggtccgctcgaagcacctacgggcgagctgctgctgtctggcgtcctcactcaccatcagctccccgtagaggtacacacccatggcctgatcctcctgaaggaacctctccacacttttgtaggctttcgtgaacttgtgcttaacaatgagttcacaccaccgatggcgaacctctgcatcctgatcctggaggtggtatgtcctctggaggctttgcagagttcgggggctcagagtcttctgctccaagagatgctccagaagcaagaccagctggtctggaagaagcttttcaaacacctcttccttctccctgcgcttccgttttcggggtctccggttcactccaatccatttcgtgacctcggcgcgcacttgccgcgcaagcccgcactccgccccggcgcgacgctccctctgcagcggctttggtattccggaactctcaagccagtcttggtagatgttttcaacagacagctcaagccttttttcttctggaatgttctccagtagcatttgaaggaaatcctgggaaagaatcagctgtccatgaaatgtgtgcacaaattttcttaaaaatgaaaaataggtttcatctccaagtcttttggcaagaaaccgaagaaggaagtagccctttaaataatgcacctgcatgaagatcttctccggattaagtccatgcttgataacagatgctcccgagtcacttgtgtggccagttttgtctttactgggtcttaacacctgcatctcctcgggggagcattgcatctcgtcctggaggcgacgccagcgcagacaagccctcagctcctgctgctcccgggcctcatagggggccagctgctgtgctgtggcccaaaacacatcctccaagtgagtggcgaagccttcactcagccactcctccgtccagtctcgggccccgatggctaggccaaaccaggcatgggcaatttcatggcagaggcgggtcccacagagatggttccctcctgtcaagatgctctgagagaggaacatgatgtgtgggctggccatccccagacttggaaagttggcagggacgatgagaacatccagccgagagaacgggtgtgctcccagaacagaatgtgctgctgagaggcaaggagggatcagccgcagaagggtctcttggcaggcacccgtgaggcacacaggggcaaagacccgatgaggaatgatctcctgggtggtggcagaagcattctggaagcggcaggggtattccatgtgactgcaaacaccaacatgcctgaagttggcctcagaaggtgagaagggtctctctgttgccaaatcatttgatgaccatgtctccatcttcatttctgtccagcatcccactgcaattgtgaaggtggaggctggcattggcatagttacatagtaataccagcttgagcactcttcccaaagctgcgttggtttggcagaattttccccactcattaaaacaacaaaagatgcagctgctcgaactgtagcctgccatgttgacatggcaacgggtggctcctggcatggaaaaagggccctgttgtttatgggagatcccacagtataaacacatggcctgccactctggtctgaggtccatgtaaccgatcgcccttcaggtttagttttgtaccatatcctgatagcatgaggaaagtcagtagctgtctgagcccctgtcttccttatctgcaagctccaagtgtcagtgtcaaagaggagttccccacagccaggagcctggctgcagcgagcgtaatagtctaactgctccctccaacgatttgcaggcaaagtcacaagttcacgtacaatctgattcctgaactcctcagaaacaaccgtgagctcaggagaccttgtaaatttttccagacctggcacagcagcaacatccacctcctcgacttttaacacagataaatcacagcagtccaacactagcaaaaaatcctcactcccatgattccctgtgtcacagcagtactttgagctagaaatcccagaagcatgttcctggttgtcatggttaccatctttatcagaagtatctttttcacctttactacagattgcaaaatcattatattccatttcagatgagaaggtccttgcatttgtcacgggaatatggcagggttcaggcatcccaaatttgcaggctttgtttgattctgattggcaggcttcctcaatagagctattctgtttcttgaatctgtttccatcctcgaggaaaagcactatggtcccctcaatgacttgactttcaaaatccacatccaaatccagtacatagtgcttcacaagtatgtggctggtgttggccatgagaggcaggtcatctctggcagggtccagctgtatgtccatgatgtggtttattgtttgagggatttattaaaatctcagatggggtttcctatctgccttaatcttccagaatcataaatagctgcttatcaaagaaaacaactgatgtcacaaattatggttcctttcagtctcctgtctcagccgcgtcccacgggtcaccacttccgcagactcggggttactacgggctaccccggcacgcgccgggtgacgtc

SEQ ID NO: 12589 - RNA, 34 nt, Homo sapiens
  source 1..34: mol_type = other RNA
gatctcactttgttgcccaggatgaagtgcagtg

SEQ ID NO: 12590 - RNA, 6781 nt, Homo sapiens
  source 1..6781: mol_type = other RNA
gatctcactttgttgcccaggatggagtgcaggggcatgatcatagctcactgtagccttgaactactggactcaagctaacctcctgcctcagcctcctcagtaggtgggactaccggcacttgccactacacctggctgatcttttttttgagatggaggcttgttctgtcgcccagcctggagtgcagtggtgcaatcttggctcactgcaactgccacctcctaggttcaagcaattcttctgcctcagcctcccgagtagatgggattacaggcacgtgccaccacacctggctgacttttgtatttttagtagagacggggtttcaccatgttagccacactggtcttgaaatcctgacctcaagtgatctgcccacctcggcctcccaaagtgctgggattacaggcatgagccacggcgcctgaccacacctggctaatctttttaaaaagtttttgtacagacagggtctccctatattggtcaggcttgtctcgaactcctgggttccagcaatcctccagcctcagccttcccaagtgctggtattacatggatgagccactgcacctggctaattttactttaaaggaatctttctactattttatcattaagtatgacatttgtgttttcagaacatatattccctaccaagttacaggagttaattttaattcccaacttaatagtattttagtgtcatctatgggtgttaaattccatcaagtgatttatcagcatatactgagataatccttatgagttttatctggtagttaattaaaatattttctaatattaaatcttccaaacatactcttctgttttttgagacagggtctagttctgtcacccagggtggagtacagtggtacgatctcagctcactgcaacttccgcctcctagattcaagtgattctcccgtcccagcctcccaagtagctgggattataggtgtcagttaccatgccctgctatttttttgtatttttagtagagaggggtttcaccatgttggccaggctggtctcaaactcctgacctcaggtgatccaccatctcagcctcctgaagtgctgggattataggtgtgagccaccgtgcctggccccatatatctctttttaagtgggcatactgccattataaataatagtgattctgctggtaatgaacaaaggatgctggatccactaatagtctgttaaacctaatatcatgactttcttgttagctatacattggtttgctataattccatttagaatttttaaacctatgttcacaaatatggatttttaaacctatgttcacaaatatggatttttaaacctatgttcacaaatatggtttgcaagtcattttttctcctaaatttctatttgatggggaagttgtaaaatattggggttatttttccttggattttccttataataactattcctgaaaagtctctggaatgtctttcttttctggggctggggtagaaggactagatagatttacaaaccagtaactcaatttctgttttgtaaaattttcatttcattaaataataagtcctaatcaagtattattctttcccacagtatgtgagtgctgtcctcaatactgtcaacacttctggcttctaccaggcaaggctgcatgtagatttgcatctgaaaaaacaacaaactaaaatctaaccctaggtagtagtaaactgaatataaactttctcttatgaatttattctgtcttctttggtacatcaataataatatacacctttacagtatttcccagattgggggatacactttagcaagtatctgcgattatttgtttatgtaagatgtcccttcccttctgtgaatcatcattcttcaccccaagtatcttgagattggattctgtataagcagaatacaacagttaggcattcaggtatcattaaattcctccgcttcaaggatgaaaatttctttgggtatctaatagagtacaaagcagaaggtgtttcagaaatatttgcagtattgaatccgcatattcctccaagatagccctaatctaactggcagggtcccactcttcccagattaatgcccactcacataacaaacctgatgaggtagtgaagaaaactaactttgtgagtaagcaactggcagagtttttcaccactgtgactctatagctacatgtaactaagtagtatcactgacacataatcttaaattgaagttttaagatcattattctccatgttatacatgggtatcaaaagcattcccctcttgaccactccagaattctgtttaaaatttttcaatgacaacttatccatttccccaaagcctcagtgagcacatgatgccaacaattcatttcatgacttcatagcatgggccaagtttcttgcttaaaagacttccatcctgtcttgggaaacaaccatttccaaatatccacatatccttgcaagtttctgcctactcctctaccacccatttctgaagccatctgatttagtaagctgtatgcaaaagatacacaatggctaatgcaatcaaacaaggaatgtattaaaagcacacccaatagctcaaaataaaagacaagtgaacaaagttaagaaaatgacagtaacaaaagctgttctgggaacctctattgaaatagctacttattacatcaacatgctaccacagaacaaaagctcatgttgcttttctgaacttgaaaaacccattaacaatgtacagttctgagcctcagctgaccatagtgctcatgccaagtcctgagcagggcatcttgaatggtggttccctcatgactacatacaccgttagggaatgtttcgttaagaggaaatcaagatgttctaacctgtgaaggtagaatagattccaggctacacaaacacatgaagtgtgccttatattgattactaaagaggttgctgccaagactgcttccaaagggcagaagatagccctaaaaaatgtttgcagtgtggaaatgcatttttagtaagtcatattctagtaacaagttgcatttggtaagacacaaagaaacaatgttggtatgcagagtagaaatctctggaagatgatattgtcatatcagagatattgtcagtatcagagatactgaaatctctggaagatgatttttgtctcacatatggcattcgcaagtaaaatgccaaactgcaaaattcatattatgtagtacacataggaagatatctaaatatccctgtaggctctgggatgttatttcttattcttaacctccttactagattcacttgtacaatgaaataatctgtatcttattatttataattgagaattttctcaaaccttttcctgaaattttggaacacctggaataaaatttcttaaaatgattcctaaaagaaataattcttcaaaattaatattaagatataataacaggttggtttttttttttttttttttttttttttttagaatgaagcttctaaggtgaggttaacagtccagctgtggtttatttggtacattcataagatgttcactcctatatatattttttccctaggggtttctcatttctagatttacactttcccttatagcatggtccctccaaggtatatgcttccgatacataaaatgtttgtaattttgttaattctgccattcattagctcaataatttctctcattaaaattctgtaaactatgaatttcaaagaagtctattctatattcatctggttcatgaagtttcctctttgtgaatcttattttagtaaaatgactttacaacgtttaacatggttcctcacctgtatgaactttttaaaaaaaggtatgacttgctgctaaaaattttcagagtggttactaaattcagttttcctgtgtattgtctactatctttttgcatgtaaagaacagctttctgtggatgcctttccatatgctgtgcattcataaagtttctattcagtatgagttttctggaagatgacaagatgattccacttacagagtttctctttatatatgattgtttctatctcttgtgaatccacttttcagagtttcgtaaaattatcaatgtttgtcatctacatgagttctctgatgcataatgagctgtgacttccaacaaaaggctttcccacattcagtgcacttacaaggcttctctcctgtatgtgttctctgatgtgcactgagaattgatttttgagagaaggttttcccacattcattgcacccatagggtttctctcctgaatgagttctttgatgtacaatgagttgagaattcctaatgaaggcttttccacactcactgcattcatatggtttctctcttgtgtgcattctctggtgtacaagaaggcgtaatttcccactgaaggatttctcacattgactgcatttataagggttgacccctgcatgagttcgctcatgtacaatgagtagtgatttccaaatgaaggctttcccacattcattacattcatatggtttttcacctgaatgagttctcatgtgtataattaggtatgacttgctgctaaaagctttcccacattcactgcacccataaggcttttcccctgcatgagttcgctgatgtgaaatgagctggtctttcctattaaaggctttcccacattcactgcattcatagggattttctcctgtgtgaattctctgatgcacaatgagttgtgaattgaaactaaaggatttcccgcattccctgcactcatgtggtttctctcctgtatgagttctcatatgtataataaggtatgacttgctcctgaaggctttcccacactcactgcatccatatggttttactcctgtgtgacttctctgatgtacaatgagctgggacttcaaactaaaggtttttgcacattgactgcatccatagggttttactccagtgtgcactcctttatgtacaatgagctgtgatttgaacgtaaaggcttttccacattcattacaactatagggtttctctcctgtatgagttctctgatgtacaatcaggtttgactttgtattaaaggctttctgacactcactacattcaaatggtttctcccctgtatgagttctctggtgtataataagctgtgactttaaaccaaaagcctttccacagtcggtgcattcataaggcttctctcctgcatgagttctctggtgtgaaataagctggtatttccgactgaaggctttcccacattcatggcattcataggggttctctcctgtatgaatcctctgatgtataatgagctgtgatttaaaactgaaggctttcccacaattgttgcattcatggagtttttctcctgtatgagtccttgtatgtataataaggtatgacttgctcctgaaggctttgccacattcattgcatacataaggtttcattcctgtgtgacttctctgatgtacaatgagctgtgatttcaaactgaatcctttaccacactgaatacacccatagggctttactcctgtgtgaatcccctgatgtacaatgagctgtgacttgaatgtaaaggcttttccacaatcactacaaacataaggtttctcccctgtatgggttctctgatgtaccataaggtttgactttgtattaaaggctttctgacattcattgcattcatatggtttctctcctgtatgaattctttcatgtataatgagctgtgattttaaaccaaaagctttcccacattcattacacacatatggtttctgtcctgaatgagttttctggtgtgaaacaagctggtctttcctactgaagactttcccacattcacagcactcatagggattctcacctgtgtgaattctctgatgtataacaagctgtgaatggaaactgaatgttttcctgcattcactgcattcatgtagtttctctcctgtatgaattctctgatgtacaatgaggtatgatttactactgaagtctttcccacattcattacaaccatagggtttctcttcggcatgagtttgctgatgcactagaaggtatgacttgctgctgaaggctttctcacaacagctgcatccaaagggtttttcgcccatatacatttgttggcacataagttgcgatttcttattgacggtttttccagattcaatactttcacagtattttattccaataacagtttgctcatgtttagaatggaagaatgattttccatgtacctgaaacccattaggattatttctagcataatcactagtgaaatctatatatttcaaactctttccatgcgtgccacatttatgaggtttttgtcttgaaagatactttgtactaagaagacatagttttccaaatgtagtgcattcaaagctttttgccgtacttcccagcttgtctttattttcctgatgccaatccataagatcatcaattttccagactgtgtccaaatagaagctgtccggaccctggtggccatccctacggtcagttttgtgtgcctcgctggaagtgacaggacgcgagggatgctccggctcctccaaaccctgaaggggcagcagaatagagtccagggtactgcctccacctccagatctgcagccagaagggttcgcaaccactccagactcggctggcccgttgaccacgacgggcgatgaacgctatctgaggaacaaggatctcgccatcggcgcggaacaatggcggccgctacgtat

SEQ ID NO: 12591 - RNA, 6982 nt, Homo sapiens
  source 1..6982: mol_type = other RNA
gatctcactttgttgcccaggatggagtgcaggggcatgatcatagctcactgtagccttgaactactggactcaagctaacctcctgcctcagcctcctcagtaggtgggactaccggcacttgccactacacctggctgatcttttttttgagatggaggcttgttctgtcgcccagcctggagtgcagtggtgcaatcttggctcactgcaactgccacctcctaggttcaagcaattcttctgcctcagcctcccgagtagatgggattacaggcacgtgccaccacacctggctgacttttgtatttttagtagagacggggtttcaccatgttagccacactggtcttgaaatcctgacctcaagtgatctgcccacctcggcctcccaaagtgctgggattacaggcatgagccacggcgcctgaccacacctggctaatctttttaaaaagtttttgtacagacagggtctccctatattggtcaggcttgtctcgaactcctgggttccagcaatcctccagcctcagccttcccaagtgctggtattacatggatgagccactgcacctggctaattttactttaaaggaatctttctactattttatcattaagtatgacatttgtgttttcagaacatatattccctaccaagttacaggagttaattttaattcccaacttaatagtattttagtgtcatctatgggtgttaaattccatcaagtgatttatcagcatatactgagataatccttatgagttttatctggtagttaattaaaatattttctaatattaaatcttccaaacatactcttctgttttttgagacagggtctagttctgtcacccagggtggagtacagtggtacgatctcagctcactgcaacttccgcctcctagattcaagtgattctcccgtcccagcctcccaagtagctgggattataggtgtcagttaccatgccctgctatttttttgtatttttagtagagaggggtttcaccatgttggccaggctggtctcaaactcctgacctcaggtgatccaccatctcagcctcctgaagtgctgggattataggtgtgagccaccgtgcctggccccatatatctctttttaagtgggcatactgccattataaataatagtgattctgctggtaatgaacaaaggatgctggatccactaatagtctgttaaacctaatatcatgactttcttgttagctatacattggtttgctataattccatttagaatttttaaacctatgttcacaaatatggatttttaaacctatgttcacaaatatggatttttaaacctatgttcacaaatatggtttgcaagtcattttttctcctaaatttctatttgatggggaagttgtaaaatattggggttatttttccttggattttccttataataactattcctgaaaagtctctggaatgtctttcttttctggggctggggtagaaggactagatagatttacaaaccagtaactcaatttctgttttgtaaaattttcatttcattaaataataagtcctaatcaagtattattctttcccacagtatgtgagtgctgtcctcaatactgtcaacacttctggcttctaccaggcaaggctgcatgtagatttgcatctgaaaaaacaacaaactaaaatctaaccctaggtagtagtaaactgaatataaactttctcttatgaatttattctgtcttctttggtacatcaataataatatacacctttacagtatttcccagattgggggatacactttagcaagtatctgcgattatttgtttatgtaagatgtcccttcccttctgtgaatcatcattcttcaccccaagtatcttgagattggattctgtataagcagaatacaacagttaggcattcaggtatcattaaattcctccgcttcaaggatgaaaatttctttgggtatctaatagagtacaaagcagaaggtgtttcagaaatatttgcagtattgaatccgcatattcctccaagatagccctaatctaactggcagggtcccactcttcccagattaatgcccactcacataacaaacctgatgaggtagtgaagaaaactaactttgtgagtaagcaactggcagagtttttcaccactgtgactctatagctacatgtaactaagtagtatcactgacacataatcttaaattgaagttttaagatcattattctccatgttatacatgggtatcaaaagcattcccctcttgaccactccagaattctgtttaaaatttttcaatgacaacttatccatttccccaaagcctcagtgagcacatgatgccaacaattcatttcatgacttcatagcatgggccaagtttcttgcttaaaagacttccatcctgtcttgggaaacaaccatttccaaatatccacatatccttgcaagtttctgcctactcctctaccacccatttctgaagccatctgatttagtaagctgtatgcaaaagatacacaatggctaatgcaatcaaacaaggaatgtattaaaagcacacccaatagctcaaaataaaagacaagtgaacaaagttaagaaaatgacagtaacaaaagctgttctgggaacctctattgaaatagctacttattacatcaacatgctaccacagaacaaaagctcatgttgcttttctgaacttgaaaaacccattaacaatgtacagttctgagcctcagctgaccatagtgctcatgccaagtcctgagcagggcatcttgaatggtggttccctcatgactacatacaccgttagggaatgtttcgttaagaggaaatcaagatgttctaacctgtgaaggtagaatagattccaggctacacaaacacatgaagtgtgccttatattgattactaaagaggttgctgccaagactgcttccaaagggcagaagatagccctaaaaaatgtttgcagtgtggaaatgcatttttagtaagtcatattctagtaacaagttgcatttggtaagacacaaagaaacaatgttggtatgcagagtagaaatctctggaagatgatattgtcatatcagagatattgtcagtatcagagatactgaaatctctggaagatgatttttgtctcacatatggcattcgcaagtaaaatgccaaactgcaaaattcatattatgtagtacacataggaagatatctaaatatccctgtaggctctgggatgttatttcttattcttaacctccttactagattcacttgtacaatgaaataatctgtatcttattatttataattgagaattttctcaaaccttttcctgaaattttggaacacctggaataaaatttcttaaaatgattcctaaaagaaataattcttcaaaattaatattaagatataataacaggttggtttttttttttttttttttttttttttttagaatgaagcttctaaggtgaggttaacagtccagctgtggtttatttggtacattcataagatgttcactcctatatatattttttccctaggggtttctcatttctagatttacactttcccttatagcatggtccctccaaggtatatgcttccgatacataaaatgtttgtaattttgttaattctgccattcattagctcaataatttctctcattaaaattctgtaaactatgaatttcaaagaagtctattctatattcatctggttcatgaagtttcctctttgtgaatcttattttagtaaaatgactttacaacgtttaacatggttcctcacctgtatgaactttttaaaaaaaggtatgacttgctgctaaaaattttcagagtggttactaaattcagttttcctgtgtattgtctactatctttttgcatgtaaagaacagctttctgtggatgcctttccatatgctgtgcattcataaagtttctattcagtatgagttttctggaagatgacaagatgattccacttacagagtttctctttatatatgattgtttctatctcttgtgaatccacttttcagagtttcgtaaaattatcaatgtttgtcatctacatgagttctctgatgcataatgagctgtgacttccaacaaaaggctttcccacattcagtgcacttacaaggcttctctcctgtatgtgttctctgatgtgcactgagaattgatttttgagagaaggttttcccacattcattgcacccatagggtttctctcctgaatgagttctttgatgtacaatgagttgagaattcctaatgaaggcttttccacactcactgcattcatatggtttctctcttgtgtgcattctctggtgtacaagaaggcgtaatttcccactgaaggatttctcacattgactgcatttataagggttgacccctgcatgagttcgctcatgtacaatgagtagtgatttccaaatgaaggctttcccacattcattacattcatatggtttttcacctgaatgagttctcatgtgtataattaggtatgacttgctgctaaaagctttcccacattcactgcacccataaggcttttcccctgcatgagttcgctgatgtgaaatgagctggtctttcctattaaaggctttcccacattcactgcattcatagggattttctcctgtgtgaattctctgatgcacaatgagttgtgaattgaaactaaaggatttcccgcattccctgcactcatgtggtttctctcctgtatgagttctcatatgtataataaggtatgacttgctcctgaaggctttcccacactcactgcatccatatggttttactcctgtgtgacttctctgatgtacaatgagctgggacttcaaactaaaggtttttgcacattgactgcatccatagggttttactccagtgtgcactcctttatgtacaatgagctgtgatttgaacgtaaaggcttttccacattcattacaactatagggtttctctcctgtatgagttctctgatgtacaatcaggtttgactttgtattaaaggctttctgacactcactacattcaaatggtttctcccctgtatgagttctctggtgtataataagctgtgactttaaaccaaaagcctttccacagtcggtgcattcataaggcttctctcctgcatgagttctctggtgtgaaataagctggtatttccgactgaaggctttcccacattcatggcattcataggggttctctcctgtatgaatcctctgatgtataatgagctgtgatttaaaactgaaggctttcccacaattgttgcattcatggagtttttctcctgtatgagtccttgtatgtataataaggtatgacttgctcctgaaggctttgccacattcattgcatacataaggtttcattcctgtgtgacttctctgatgtacaatgagctgtgatttcaaactgaatcctttaccacactgaatacacccatagggctttactcctgtgtgaatcccctgatgtacaatgagctgtgacttgaatgtaaaggcttttccacaatcactacaaacataaggtttctcccctgtatgggttctctgatgtaccataaggtttgactttgtattaaaggctttctgacattcattgcattcatatggtttctctcctgtatgaattctttcatgtataatgagctgtgattttaaaccaaaagctttcccacattcattacacacatatggtttctgtcctgaatgagttttctggtgtgaaacaagctggtctttcctactgaagactttcccacattcacagcactcatagggattctcacctgtgtgaattctctgatgtataacaagctgtgaatggaaactgaatgttttcctgcattcactgcattcatgtagtttctctcctgtatgaattctctgatgtacaatgaggtatgatttactactgaagtctttcccacattcattacaaccatagggtttctcttcggcatgagtttgctgatgcactagaaggtatgacttgctgctgaaggctttctcacaacagctgcatccaaagggtttttcgcccatatacatttgttggcacataagttgcgatttcttattgacggtttttccagattcaatactttcacagtattttattccaataacagtttgctcatgtttagaatggaagaatgattttccatgtacctgaaacccattaggattatttctagcataatcactagtgaaatctatatatttcaaactctttccatgcgtgccacatttatgaggtttttgtcttgaaagatactttgtactaagaagacatagttttccaaatgtagtgcattcaaagctttttgccgtacttcccagcttgtctttattttcctgatgccaatccataagatcatcaattttccagactgtgtccaggacttggtgatttttggctgctcttgggaaataaacagccactctaggactttctctattctgcgactcttctgcttctgcctgggtgttccagggagaggttgcagaccaggagtcccttggcccaagatggattcctgaccttggagctttctgatcctatcccatgaactgtttcgttcttggagaggtgggacccaaatagaagctgtccggaccctggtggccatccctacggtcagttttgtgtgcctcgctggaagtgacaggacgcgagggatgctccggctcctccaaaccctgaaggggcagcagaatagagtccagggtactgcctccacctccagatctgcagccagaagggttcgcaaccactccagactcggctggcccgttgaccacgacgggcgatgaacgctatctgaggaacaaggatctcgccatcggcgcggaacaatggcggccgctacgtat

SEQ ID NO: 12592 - RNA, 7110 nt, Homo sapiens
  source 1..7110: mol_type = other RNA
gatctcactttgttgcccaggatggagtgcaggggcatgatcatagctcactgtagccttgaactactggactcaagctaacctcctgcctcagcctcctcagtaggtgggactaccggcacttgccactacacctggctgatcttttttttgagatggaggcttgttctgtcgcccagcctggagtgcagtggtgcaatcttggctcactgcaactgccacctcctaggttcaagcaattcttctgcctcagcctcccgagtagatgggattacaggcacgtgccaccacacctggctgacttttgtatttttagtagagacggggtttcaccatgttagccacactggtcttgaaatcctgacctcaagtgatctgcccacctcggcctcccaaagtgctgggattacaggcatgagccacggcgcctgaccacacctggctaatctttttaaaaagtttttgtacagacagggtctccctatattggtcaggcttgtctcgaactcctgggttccagcaatcctccagcctcagccttcccaagtgctggtattacatggatgagccactgcacctggctaattttactttaaaggaatctttctactattttatcattaagtatgacatttgtgttttcagaacatatattccctaccaagttacaggagttaattttaattcccaacttaatagtattttagtgtcatctatgggtgttaaattccatcaagtgatttatcagcatatactgagataatccttatgagttttatctggtagttaattaaaatattttctaatattaaatcttccaaacatactcttctgttttttgagacagggtctagttctgtcacccagggtggagtacagtggtacgatctcagctcactgcaacttccgcctcctagattcaagtgattctcccgtcccagcctcccaagtagctgggattataggtgtcagttaccatgccctgctatttttttgtatttttagtagagaggggtttcaccatgttggccaggctggtctcaaactcctgacctcaggtgatccaccatctcagcctcctgaagtgctgggattataggtgtgagccaccgtgcctggccccatatatctctttttaagtgggcatactgccattataaataatagtgattctgctggtaatgaacaaaggatgctggatccactaatagtctgttaaacctaatatcatgactttcttgttagctatacattggtttgctataattccatttagaatttttaaacctatgttcacaaatatggatttttaaacctatgttcacaaatatggatttttaaacctatgttcacaaatatggtttgcaagtcattttttctcctaaatttctatttgatggggaagttgtaaaatattggggttatttttccttggattttccttataataactattcctgaaaagtctctggaatgtctttcttttctggggctggggtagaaggactagatagatttacaaaccagtaactcaatttctgttttgtaaaattttcatttcattaaataataagtcctaatcaagtattattctttcccacagtatgtgagtgctgtcctcaatactgtcaacacttctggcttctaccaggcaaggctgcatgtagatttgcatctgaaaaaacaacaaactaaaatctaaccctaggtagtagtaaactgaatataaactttctcttatgaatttattctgtcttctttggtacatcaataataatatacacctttacagtatttcccagattgggggatacactttagcaagtatctgcgattatttgtttatgtaagatgtcccttcccttctgtgaatcatcattcttcaccccaagtatcttgagattggattctgtataagcagaatacaacagttaggcattcaggtatcattaaattcctccgcttcaaggatgaaaatttctttgggtatctaatagagtacaaagcagaaggtgtttcagaaatatttgcagtattgaatccgcatattcctccaagatagccctaatctaactggcagggtcccactcttcccagattaatgcccactcacataacaaacctgatgaggtagtgaagaaaactaactttgtgagtaagcaactggcagagtttttcaccactgtgactctatagctacatgtaactaagtagtatcactgacacataatcttaaattgaagttttaagatcattattctccatgttatacatgggtatcaaaagcattcccctcttgaccactccagaattctgtttaaaatttttcaatgacaacttatccatttccccaaagcctcagtgagcacatgatgccaacaattcatttcatgacttcatagcatgggccaagtttcttgcttaaaagacttccatcctgtcttgggaaacaaccatttccaaatatccacatatccttgcaagtttctgcctactcctctaccacccatttctgaagccatctgatttagtaagctgtatgcaaaagatacacaatggctaatgcaatcaaacaaggaatgtattaaaagcacacccaatagctcaaaataaaagacaagtgaacaaagttaagaaaatgacagtaacaaaagctgttctgggaacctctattgaaatagctacttattacatcaacatgctaccacagaacaaaagctcatgttgcttttctgaacttgaaaaacccattaacaatgtacagttctgagcctcagctgaccatagtgctcatgccaagtcctgagcagggcatcttgaatggtggttccctcatgactacatacaccgttagggaatgtttcgttaagaggaaatcaagatgttctaacctgtgaaggtagaatagattccaggctacacaaacacatgaagtgtgccttatattgattactaaagaggttgctgccaagactgcttccaaagggcagaagatagccctaaaaaatgtttgcagtgtggaaatgcatttttagtaagtcatattctagtaacaagttgcatttggtaagacacaaagaaacaatgttggtatgcagagtagaaatctctggaagatgatattgtcatatcagagatattgtcagtatcagagatactgaaatctctggaagatgatttttgtctcacatatggcattcgcaagtaaaatgccaaactgcaaaattcatattatgtagtacacataggaagatatctaaatatccctgtaggctctgggatgttatttcttattcttaacctccttactagattcacttgtacaatgaaataatctgtatcttattatttataattgagaattttctcaaaccttttcctgaaattttggaacacctggaataaaatttcttaaaatgattcctaaaagaaataattcttcaaaattaatattaagatataataacaggttggtttttttttttttttttttttttttttttagaatgaagcttctaaggtgaggttaacagtccagctgtggtttatttggtacattcataagatgttcactcctatatatattttttccctaggggtttctcatttctagatttacactttcccttatagcatggtccctccaaggtatatgcttccgatacataaaatgtttgtaattttgttaattctgccattcattagctcaataatttctctcattaaaattctgtaaactatgaatttcaaagaagtctattctatattcatctggttcatgaagtttcctctttgtgaatcttattttagtaaaatgactttacaacgtttaacatggttcctcacctgtatgaactttttaaaaaaaggtatgacttgctgctaaaaattttcagagtggttactaaattcagttttcctgtgtattgtctactatctttttgcatgtaaagaacagctttctgtggatgcctttccatatgctgtgcattcataaagtttctattcagtatgagttttctggaagatgacaagatgattccacttacagagtttctctttatatatgattgtttctatctcttgtgaatccacttttcagagtttcgtaaaattatcaatgtttgtcatctacatgagttctctgatgcataatgagctgtgacttccaacaaaaggctttcccacattcagtgcacttacaaggcttctctcctgtatgtgttctctgatgtgcactgagaattgatttttgagagaaggttttcccacattcattgcacccatagggtttctctcctgaatgagttctttgatgtacaatgagttgagaattcctaatgaaggcttttccacactcactgcattcatatggtttctctcttgtgtgcattctctggtgtacaagaaggcgtaatttcccactgaaggatttctcacattgactgcatttataagggttgacccctgcatgagttcgctcatgtacaatgagtagtgatttccaaatgaaggctttcccacattcattacattcatatggtttttcacctgaatgagttctcatgtgtataattaggtatgacttgctgctaaaagctttcccacattcactgcacccataaggcttttcccctgcatgagttcgctgatgtgaaatgagctggtctttcctattaaaggctttcccacattcactgcattcatagggattttctcctgtgtgaattctctgatgcacaatgagttgtgaattgaaactaaaggatttcccgcattccctgcactcatgtggtttctctcctgtatgagttctcatatgtataataaggtatgacttgctcctgaaggctttcccacactcactgcatccatatggttttactcctgtgtgacttctctgatgtacaatgagctgggacttcaaactaaaggtttttgcacattgactgcatccatagggttttactccagtgtgcactcctttatgtacaatgagctgtgatttgaacgtaaaggcttttccacattcattacaactatagggtttctctcctgtatgagttctctgatgtacaatcaggtttgactttgtattaaaggctttctgacactcactacattcaaatggtttctcccctgtatgagttctctggtgtataataagctgtgactttaaaccaaaagcctttccacagtcggtgcattcataaggcttctctcctgcatgagttctctggtgtgaaataagctggtatttccgactgaaggctttcccacattcatggcattcataggggttctctcctgtatgaatcctctgatgtataatgagctgtgatttaaaactgaaggctttcccacaattgttgcattcatggagtttttctcctgtatgagtccttgtatgtataataaggtatgacttgctcctgaaggctttgccacattcattgcatacataaggtttcattcctgtgtgacttctctgatgtacaatgagctgtgatttcaaactgaatcctttaccacactgaatacacccatagggctttactcctgtgtgaatcccctgatgtacaatgagctgtgacttgaatgtaaaggcttttccacaatcactacaaacataaggtttctcccctgtatgggttctctgatgtaccataaggtttgactttgtattaaaggctttctgacattcattgcattcatatggtttctctcctgtatgaattctttcatgtataatgagctgtgattttaaaccaaaagctttcccacattcattacacacatatggtttctgtcctgaatgagttttctggtgtgaaacaagctggtctttcctactgaagactttcccacattcacagcactcatagggattctcacctgtgtgaattctctgatgtataacaagctgtgaatggaaactgaatgttttcctgcattcactgcattcatgtagtttctctcctgtatgaattctctgatgtacaatgaggtatgatttactactgaagtctttcccacattcattacaaccatagggtttctcttcggcatgagtttgctgatgcactagaaggtatgacttgctgctgaaggctttctcacaacagctgcatccaaagggtttttcgcccatatacatttgttggcacataagttgcgatttcttattgacggtttttccagattcaatactttcacagtattttattccaataacagtttgctcatgtttagaatggaagaatgattttccatgtacctgaaacccattaggattatttctagcataatcactagtgaaatctatatatttcaaactctttccatgcgtgccacatttatgaggtttttgtcttgaaagatactttgtactaagaagacatagttttccaaatgtagtgcattcaaagctttttgccgtacttcccagcttgtctttattttcctgatgccaatccataagatcatcaattttccagactgtgtctccagaggatgcagcaacaaggcgtcatcttggaagcacagagcaggccctcaccagacaccaaacctgccagcaccttggctttggactttccagccttcaaaattggacaggtctgatttggaacttgggcctgcaccatacacagctcttctccttgttccaacttgaagatgatatcaggtttggtgtgttggtaccctagggacaccaggttgctatagttctccaacatcacactcctgtacaggcacttctgtgctgggtctagcagctgccactcctcccaggtaaaatccacaaacacatccatgaatgacaaaggtccccaaatagaagctgtccggaccctggtggccatccctacggtcagttttgtgtgcctcgctggaagtgacaggacgcgagggatgctccggctcctccaaaccctgaaggggcagcagaatagagtccagggtactgcctccacctccagatctgcagccagaagggttcgcaaccactccagactcggctggcccgttgaccacgacgggcgatgaacgctatctgaggaacaaggatctcgccatcggcgcggaacaatggcggccgctacgtat

SEQ ID NO: 12593 - RNA, 7311 nt, Homo sapiens
  source 1..7311: mol_type = other RNA
gatctcactttgttgcccaggatggagtgcaggggcatgatcatagctcactgtagccttgaactactggactcaagctaacctcctgcctcagcctcctcagtaggtgggactaccggcacttgccactacacctggctgatcttttttttgagatggaggcttgttctgtcgcccagcctggagtgcagtggtgcaatcttggctcactgcaactgccacctcctaggttcaagcaattcttctgcctcagcctcccgagtagatgggattacaggcacgtgccaccacacctggctgacttttgtatttttagtagagacggggtttcaccatgttagccacactggtcttgaaatcctgacctcaagtgatctgcccacctcggcctcccaaagtgctgggattacaggcatgagccacggcgcctgaccacacctggctaatctttttaaaaagtttttgtacagacagggtctccctatattggtcaggcttgtctcgaactcctgggttccagcaatcctccagcctcagccttcccaagtgctggtattacatggatgagccactgcacctggctaattttactttaaaggaatctttctactattttatcattaagtatgacatttgtgttttcagaacatatattccctaccaagttacaggagttaattttaattcccaacttaatagtattttagtgtcatctatgggtgttaaattccatcaagtgatttatcagcatatactgagataatccttatgagttttatctggtagttaattaaaatattttctaatattaaatcttccaaacatactcttctgttttttgagacagggtctagttctgtcacccagggtggagtacagtggtacgatctcagctcactgcaacttccgcctcctagattcaagtgattctcccgtcccagcctcccaagtagctgggattataggtgtcagttaccatgccctgctatttttttgtatttttagtagagaggggtttcaccatgttggccaggctggtctcaaactcctgacctcaggtgatccaccatctcagcctcctgaagtgctgggattataggtgtgagccaccgtgcctggccccatatatctctttttaagtgggcatactgccattataaataatagtgattctgctggtaatgaacaaaggatgctggatccactaatagtctgttaaacctaatatcatgactttcttgttagctatacattggtttgctataattccatttagaatttttaaacctatgttcacaaatatggatttttaaacctatgttcacaaatatggatttttaaacctatgttcacaaatatggtttgcaagtcattttttctcctaaatttctatttgatggggaagttgtaaaatattggggttatttttccttggattttccttataataactattcctgaaaagtctctggaatgtctttcttttctggggctggggtagaaggactagatagatttacaaaccagtaactcaatttctgttttgtaaaattttcatttcattaaataataagtcctaatcaagtattattctttcccacagtatgtgagtgctgtcctcaatactgtcaacacttctggcttctaccaggcaaggctgcatgtagatttgcatctgaaaaaacaacaaactaaaatctaaccctaggtagtagtaaactgaatataaactttctcttatgaatttattctgtcttctttggtacatcaataataatatacacctttacagtatttcccagattgggggatacactttagcaagtatctgcgattatttgtttatgtaagatgtcccttcccttctgtgaatcatcattcttcaccccaagtatcttgagattggattctgtataagcagaatacaacagttaggcattcaggtatcattaaattcctccgcttcaaggatgaaaatttctttgggtatctaatagagtacaaagcagaaggtgtttcagaaatatttgcagtattgaatccgcatattcctccaagatagccctaatctaactggcagggtcccactcttcccagattaatgcccactcacataacaaacctgatgaggtagtgaagaaaactaactttgtgagtaagcaactggcagagtttttcaccactgtgactctatagctacatgtaactaagtagtatcactgacacataatcttaaattgaagttttaagatcattattctccatgttatacatgggtatcaaaagcattcccctcttgaccactccagaattctgtttaaaatttttcaatgacaacttatccatttccccaaagcctcagtgagcacatgatgccaacaattcatttcatgacttcatagcatgggccaagtttcttgcttaaaagacttccatcctgtcttgggaaacaaccatttccaaatatccacatatccttgcaagtttctgcctactcctctaccacccatttctgaagccatctgatttagtaagctgtatgcaaaagatacacaatggctaatgcaatcaaacaaggaatgtattaaaagcacacccaatagctcaaaataaaagacaagtgaacaaagttaagaaaatgacagtaacaaaagctgttctgggaacctctattgaaatagctacttattacatcaacatgctaccacagaacaaaagctcatgttgcttttctgaacttgaaaaacccattaacaatgtacagttctgagcctcagctgaccatagtgctcatgccaagtcctgagcagggcatcttgaatggtggttccctcatgactacatacaccgttagggaatgtttcgttaagaggaaatcaagatgttctaacctgtgaaggtagaatagattccaggctacacaaacacatgaagtgtgccttatattgattactaaagaggttgctgccaagactgcttccaaagggcagaagatagccctaaaaaatgtttgcagtgtggaaatgcatttttagtaagtcatattctagtaacaagttgcatttggtaagacacaaagaaacaatgttggtatgcagagtagaaatctctggaagatgatattgtcatatcagagatattgtcagtatcagagatactgaaatctctggaagatgatttttgtctcacatatggcattcgcaagtaaaatgccaaactgcaaaattcatattatgtagtacacataggaagatatctaaatatccctgtaggctctgggatgttatttcttattcttaacctccttactagattcacttgtacaatgaaataatctgtatcttattatttataattgagaattttctcaaaccttttcctgaaattttggaacacctggaataaaatttcttaaaatgattcctaaaagaaataattcttcaaaattaatattaagatataataacaggttggtttttttttttttttttttttttttttttagaatgaagcttctaaggtgaggttaacagtccagctgtggtttatttggtacattcataagatgttcactcctatatatattttttccctaggggtttctcatttctagatttacactttcccttatagcatggtccctccaaggtatatgcttccgatacataaaatgtttgtaattttgttaattctgccattcattagctcaataatttctctcattaaaattctgtaaactatgaatttcaaagaagtctattctatattcatctggttcatgaagtttcctctttgtgaatcttattttagtaaaatgactttacaacgtttaacatggttcctcacctgtatgaactttttaaaaaaaggtatgacttgctgctaaaaattttcagagtggttactaaattcagttttcctgtgtattgtctactatctttttgcatgtaaagaacagctttctgtggatgcctttccatatgctgtgcattcataaagtttctattcagtatgagttttctggaagatgacaagatgattccacttacagagtttctctttatatatgattgtttctatctcttgtgaatccacttttcagagtttcgtaaaattatcaatgtttgtcatctacatgagttctctgatgcataatgagctgtgacttccaacaaaaggctttcccacattcagtgcacttacaaggcttctctcctgtatgtgttctctgatgtgcactgagaattgatttttgagagaaggttttcccacattcattgcacccatagggtttctctcctgaatgagttctttgatgtacaatgagttgagaattcctaatgaaggcttttccacactcactgcattcatatggtttctctcttgtgtgcattctctggtgtacaagaaggcgtaatttcccactgaaggatttctcacattgactgcatttataagggttgacccctgcatgagttcgctcatgtacaatgagtagtgatttccaaatgaaggctttcccacattcattacattcatatggtttttcacctgaatgagttctcatgtgtataattaggtatgacttgctgctaaaagctttcccacattcactgcacccataaggcttttcccctgcatgagttcgctgatgtgaaatgagctggtctttcctattaaaggctttcccacattcactgcattcatagggattttctcctgtgtgaattctctgatgcacaatgagttgtgaattgaaactaaaggatttcccgcattccctgcactcatgtggtttctctcctgtatgagttctcatatgtataataaggtatgacttgctcctgaaggctttcccacactcactgcatccatatggttttactcctgtgtgacttctctgatgtacaatgagctgggacttcaaactaaaggtttttgcacattgactgcatccatagggttttactccagtgtgcactcctttatgtacaatgagctgtgatttgaacgtaaaggcttttccacattcattacaactatagggtttctctcctgtatgagttctctgatgtacaatcaggtttgactttgtattaaaggctttctgacactcactacattcaaatggtttctcccctgtatgagttctctggtgtataataagctgtgactttaaaccaaaagcctttccacagtcggtgcattcataaggcttctctcctgcatgagttctctggtgtgaaataagctggtatttccgactgaaggctttcccacattcatggcattcataggggttctctcctgtatgaatcctctgatgtataatgagctgtgatttaaaactgaaggctttcccacaattgttgcattcatggagtttttctcctgtatgagtccttgtatgtataataaggtatgacttgctcctgaaggctttgccacattcattgcatacataaggtttcattcctgtgtgacttctctgatgtacaatgagctgtgatttcaaactgaatcctttaccacactgaatacacccatagggctttactcctgtgtgaatcccctgatgtacaatgagctgtgacttgaatgtaaaggcttttccacaatcactacaaacataaggtttctcccctgtatgggttctctgatgtaccataaggtttgactttgtattaaaggctttctgacattcattgcattcatatggtttctctcctgtatgaattctttcatgtataatgagctgtgattttaaaccaaaagctttcccacattcattacacacatatggtttctgtcctgaatgagttttctggtgtgaaacaagctggtctttcctactgaagactttcccacattcacagcactcatagggattctcacctgtgtgaattctctgatgtataacaagctgtgaatggaaactgaatgttttcctgcattcactgcattcatgtagtttctctcctgtatgaattctctgatgtacaatgaggtatgatttactactgaagtctttcccacattcattacaaccatagggtttctcttcggcatgagtttgctgatgcactagaaggtatgacttgctgctgaaggctttctcacaacagctgcatccaaagggtttttcgcccatatacatttgttggcacataagttgcgatttcttattgacggtttttccagattcaatactttcacagtattttattccaataacagtttgctcatgtttagaatggaagaatgattttccatgtacctgaaacccattaggattatttctagcataatcactagtgaaatctatatatttcaaactctttccatgcgtgccacatttatgaggtttttgtcttgaaagatactttgtactaagaagacatagttttccaaatgtagtgcattcaaagctttttgccgtacttcccagcttgtctttattttcctgatgccaatccataagatcatcaattttccagactgtgtctccagaggatgcagcaacaaggcgtcatcttggaagcacagagcaggccctcaccagacaccaaacctgccagcaccttggctttggactttccagccttcaaaattggacaggtctgatttggaacttgggcctgcaccatacacagctcttctccttgttccaacttgaagatgatatcaggtttggtgtgttggtaccctagggacaccaggttgctatagttctccaacatcacactcctgtacaggcacttctgtgctgggtctagcagctgccactcctcccaggtaaaatccacaaacacatccatgaatgacaaaggtccccaggacttggtgatttttggctgctcttgggaaataaacagccactctaggactttctctattctgcgactcttctgcttctgcctgggtgttccagggagaggttgcagaccaggagtcccttggcccaagatggattcctgaccttggagctttctgatcctatcccatgaactgtttcgttcttggagaggtgggacccaaatagaagctgtccggaccctggtggccatccctacggtcagttttgtgtgcctcgctggaagtgacaggacgcgagggatgctccggctcctccaaaccctgaaggggcagcagaatagagtccagggtactgcctccacctccagatctgcagccagaagggttcgcaaccactccagactcggctggcccgttgaccacgacgggcgatgaacgctatctgaggaacaaggatctcgccatcggcgcggaacaatggcggccgctacgtat

SEQ ID NO: 12594 - RNA, 6877 nt, Homo sapiens
  source 1..6877: mol_type = other RNA
gatctcactttgttgcccaggatggagtgcaggggcatgatcatagctcactgtagccttgaactactggactcaagctaacctcctgcctcagcctcctcagtaggtgggactaccggcacttgccactacacctggctgatcttttttttgagatggaggcttgttctgtcgcccagcctggagtgcagtggtgcaatcttggctcactgcaactgccacctcctaggttcaagcaattcttctgcctcagcctcccgagtagatgggattacaggcacgtgccaccacacctggctgacttttgtatttttagtagagacggggtttcaccatgttagccacactggtcttgaaatcctgacctcaagtgatctgcccacctcggcctcccaaagtgctgggattacaggcatgagccacggcgcctgaccacacctggctaatctttttaaaaagtttttgtacagacagggtctccctatattggtcaggcttgtctcgaactcctgggttccagcaatcctccagcctcagccttcccaagtgctggtattacatggatgagccactgcacctggctaattttactttaaaggaatctttctactattttatcattaagtatgacatttgtgttttcagaacatatattccctaccaagttacaggagttaattttaattcccaacttaatagtattttagtgtcatctatgggtgttaaattccatcaagtgatttatcagcatatactgagataatccttatgagttttatctggtagttaattaaaatattttctaatattaaatcttccaaacatactcttctgttttttgagacagggtctagttctgtcacccagggtggagtacagtggtacgatctcagctcactgcaacttccgcctcctagattcaagtgattctcccgtcccagcctcccaagtagctgggattataggtgtcagttaccatgccctgctatttttttgtatttttagtagagaggggtttcaccatgttggccaggctggtctcaaactcctgacctcaggtgatccaccatctcagcctcctgaagtgctgggattataggtgtgagccaccgtgcctggccccatatatctctttttaagtgggcatactgccattataaataatagtgattctgctggtaatgaacaaaggatgctggatccactaatagtctgttaaacctaatatcatgactttcttgttagctatacattggtttgctataattccatttagaatttttaaacctatgttcacaaatatggatttttaaacctatgttcacaaatatggatttttaaacctatgttcacaaatatggtttgcaagtcattttttctcctaaatttctatttgatggggaagttgtaaaatattggggttatttttccttggattttccttataataactattcctgaaaagtctctggaatgtctttcttttctggggctggggtagaaggactagatagatttacaaaccagtaactcaatttctgttttgtaaaattttcatttcattaaataataagtcctaatcaagtattattctttcccacagtatgtgagtgctgtcctcaatactgtcaacacttctggcttctaccaggcaaggctgcatgtagatttgcatctgaaaaaacaacaaactaaaatctaaccctaggtagtagtaaactgaatataaactttctcttatgaatttattctgtcttctttggtacatcaataataatatacacctttacagtatttcccagattgggggatacactttagcaagtatctgcgattatttgtttatgtaagatgtcccttcccttctgtgaatcatcattcttcaccccaagtatcttgagattggattctgtataagcagaatacaacagttaggcattcaggtatcattaaattcctccgcttcaaggatgaaaatttctttgggtatctaatagagtacaaagcagaaggtgtttcagaaatatttgcagtattgaatccgcatattcctccaagatagccctaatctaactggcagggtcccactcttcccagattaatgcccactcacataacaaacctgatgaggtagtgaagaaaactaactttgtgagtaagcaactggcagagtttttcaccactgtgactctatagctacatgtaactaagtagtatcactgacacataatcttaaattgaagttttaagatcattattctccatgttatacatgggtatcaaaagcattcccctcttgaccactccagaattctgtttaaaatttttcaatgacaacttatccatttccccaaagcctcagtgagcacatgatgccaacaattcatttcatgacttcatagcatgggccaagtttcttgcttaaaagacttccatcctgtcttgggaaacaaccatttccaaatatccacatatccttgcaagtttctgcctactcctctaccacccatttctgaagccatctgatttagtaagctgtatgcaaaagatacacaatggctaatgcaatcaaacaaggaatgtattaaaagcacacccaatagctcaaaataaaagacaagtgaacaaagttaagaaaatgacagtaacaaaagctgttctgggaacctctattgaaatagctacttattacatcaacatgctaccacagaacaaaagctcatgttgcttttctgaacttgaaaaacccattaacaatgtacagttctgagcctcagctgaccatagtgctcatgccaagtcctgagcagggcatcttgaatggtggttccctcatgactacatacaccgttagggaatgtttcgttaagaggaaatcaagatgttctaacctgtgaaggtagaatagattccaggctacacaaacacatgaagtgtgccttatattgattactaaagaggttgctgccaagactgcttccaaagggcagaagatagccctaaaaaatgtttgcagtgtggaaatgcatttttagtaagtcatattctagtaacaagttgcatttggtaagacacaaagaaacaatgttggtatgcagagtagaaatctctggaagatgatattgtcatatcagagatattgtcagtatcagagatactgaaatctctggaagatgatttttgtctcacatatggcattcgcaagtaaaatgccaaactgcaaaattcatattatgtagtacacataggaagatatctaaatatccctgtaggctctgggatgttatttcttattcttaacctccttactagattcacttgtacaatgaaataatctgtatcttattatttataattgagaattttctcaaaccttttcctgaaattttggaacacctggaataaaatttcttaaaatgattcctaaaagaaataattcttcaaaattaatattaagatataataacaggttggtttttttttttttttttttttttttttttagaatgaagcttctaaggtgaggttaacagtccagctgtggtttatttggtacattcataagatgttcactcctatatatattttttccctaggggtttctcatttctagatttacactttcccttatagcatggtccctccaaggtatatgcttccgatacataaaatgtttgtaattttgttaattctgccattcattagctcaataatttctctcattaaaattctgtaaactatgaatttcaaagaagtctattctatattcatctggttcatgaagtttcctctttgtgaatcttattttagtaaaatgactttacaacgtttaacatggttcctcacctgtatgaactttttaaaaaaaggtatgacttgctgctaaaaattttcagagtggttactaaattcagttttcctgtgtattgtctactatctttttgcatgtaaagaacagctttctgtggatgcctttccatatgctgtgcattcataaagtttctattcagtatgagttttctggaagatgacaagatgattccacttacagagtttctctttatatatgattgtttctatctcttgtgaatccacttttcagagtttcgtaaaattatcaatgtttgtcatctacatgagttctctgatgcataatgagctgtgacttccaacaaaaggctttcccacattcagtgcacttacaaggcttctctcctgtatgtgttctctgatgtgcactgagaattgatttttgagagaaggttttcccacattcattgcacccatagggtttctctcctgaatgagttctttgatgtacaatgagttgagaattcctaatgaaggcttttccacactcactgcattcatatggtttctctcttgtgtgcattctctggtgtacaagaaggcgtaatttcccactgaaggatttctcacattgactgcatttataagggttgacccctgcatgagttcgctcatgtacaatgagtagtgatttccaaatgaaggctttcccacattcattacattcatatggtttttcacctgaatgagttctcatgtgtataattaggtatgacttgctgctaaaagctttcccacattcactgcacccataaggcttttcccctgcatgagttcgctgatgtgaaatgagctggtctttcctattaaaggctttcccacattcactgcattcatagggattttctcctgtgtgaattctctgatgcacaatgagttgtgaattgaaactaaaggatttcccgcattccctgcactcatgtggtttctctcctgtatgagttctcatatgtataataaggtatgacttgctcctgaaggctttcccacactcactgcatccatatggttttactcctgtgtgacttctctgatgtacaatgagctgggacttcaaactaaaggtttttgcacattgactgcatccatagggttttactccagtgtgcactcctttatgtacaatgagctgtgatttgaacgtaaaggcttttccacattcattacaactatagggtttctctcctgtatgagttctctgatgtacaatcaggtttgactttgtattaaaggctttctgacactcactacattcaaatggtttctcccctgtatgagttctctggtgtataataagctgtgactttaaaccaaaagcctttccacagtcggtgcattcataaggcttctctcctgcatgagttctctggtgtgaaataagctggtatttccgactgaaggctttcccacattcatggcattcataggggttctctcctgtatgaatcctctgatgtataatgagctgtgatttaaaactgaaggctttcccacaattgttgcattcatggagtttttctcctgtatgagtccttgtatgtataataaggtatgacttgctcctgaaggctttgccacattcattgcatacataaggtttcattcctgtgtgacttctctgatgtacaatgagctgtgatttcaaactgaatcctttaccacactgaatacacccatagggctttactcctgtgtgaatcccctgatgtacaatgagctgtgacttgaatgtaaaggcttttccacaatcactacaaacataaggtttctcccctgtatgggttctctgatgtaccataaggtttgactttgtattaaaggctttctgacattcattgcattcatatggtttctctcctgtatgaattctttcatgtataatgagctgtgattttaaaccaaaagctttcccacattcattacacacatatggtttctgtcctgaatgagttttctggtgtgaaacaagctggtctttcctactgaagactttcccacattcacagcactcatagggattctcacctgtgtgaattctctgatgtataacaagctgtgaatggaaactgaatgttttcctgcattcactgcattcatgtagtttctctcctgtatgaattctctgatgtacaatgaggtatgatttactactgaagtctttcccacattcattacaaccatagggtttctcttcggcatgagtttgctgatgcactagaaggtatgacttgctgctgaaggctttctcacaacagctgcatccaaagggtttttcgcccatatacatttgttggcacataagttgcgatttcttattgacggtttttccagattcaatactttcacagtattttattccaataacagtttgctcatgtttagaatggaagaatgattttccatgtacctgaaacccattaggattatttctagcataatcactagtgaaatctatatatttcaaactctttccatgcgtgccacatttatgaggtttttgtcttgaaagatactttgtactaagaagacatagttttccaaatgtagtgcattcaaagctttttgccgtacttcccagcttgtctttattttcctgatgccaatccataagatcatcaattttccagactgtgtttggacaggtctgatttggaacttgggcctgcaccatacacagctcttctccttgttccaacttgaagatgatatcaggtttggtgtgttggtaccccaaatagaagctgtccggaccctggtggccatccctacggtcagttttgtgtgcctcgctggaagtgacaggacgcgagggatgctccggctcctccaaaccctgaaggggcagcagaatagagtccagggtactgcctccacctccagatctgcagccagaagggttcgcaaccactccagactcggctggcccgttgaccacgacgggcgatgaacgctatctgaggaacaaggatctcgccatcggcgcggaacaatggcggccgctacgtat

SEQ ID NO: 12595 - RNA, 7078 nt, Homo sapiens
  source 1..7078: mol_type = other RNA
gatctcactttgttgcccaggatggagtgcaggggcatgatcatagctcactgtagccttgaactactggactcaagctaacctcctgcctcagcctcctcagtaggtgggactaccggcacttgccactacacctggctgatcttttttttgagatggaggcttgttctgtcgcccagcctggagtgcagtggtgcaatcttggctcactgcaactgccacctcctaggttcaagcaattcttctgcctcagcctcccgagtagatgggattacaggcacgtgccaccacacctggctgacttttgtatttttagtagagacggggtttcaccatgttagccacactggtcttgaaatcctgacctcaagtgatctgcccacctcggcctcccaaagtgctgggattacaggcatgagccacggcgcctgaccacacctggctaatctttttaaaaagtttttgtacagacagggtctccctatattggtcaggcttgtctcgaactcctgggttccagcaatcctccagcctcagccttcccaagtgctggtattacatggatgagccactgcacctggctaattttactttaaaggaatctttctactattttatcattaagtatgacatttgtgttttcagaacatatattccctaccaagttacaggagttaattttaattcccaacttaatagtattttagtgtcatctatgggtgttaaattccatcaagtgatttatcagcatatactgagataatccttatgagttttatctggtagttaattaaaatattttctaatattaaatcttccaaacatactcttctgttttttgagacagggtctagttctgtcacccagggtggagtacagtggtacgatctcagctcactgcaacttccgcctcctagattcaagtgattctcccgtcccagcctcccaagtagctgggattataggtgtcagttaccatgccctgctatttttttgtatttttagtagagaggggtttcaccatgttggccaggctggtctcaaactcctgacctcaggtgatccaccatctcagcctcctgaagtgctgggattataggtgtgagccaccgtgcctggccccatatatctctttttaagtgggcatactgccattataaataatagtgattctgctggtaatgaacaaaggatgctggatccactaatagtctgttaaacctaatatcatgactttcttgttagctatacattggtttgctataattccatttagaatttttaaacctatgttcacaaatatggatttttaaacctatgttcacaaatatggatttttaaacctatgttcacaaatatggtttgcaagtcattttttctcctaaatttctatttgatggggaagttgtaaaatattggggttatttttccttggattttccttataataactattcctgaaaagtctctggaatgtctttcttttctggggctggggtagaaggactagatagatttacaaaccagtaactcaatttctgttttgtaaaattttcatttcattaaataataagtcctaatcaagtattattctttcccacagtatgtgagtgctgtcctcaatactgtcaacacttctggcttctaccaggcaaggctgcatgtagatttgcatctgaaaaaacaacaaactaaaatctaaccctaggtagtagtaaactgaatataaactttctcttatgaatttattctgtcttctttggtacatcaataataatatacacctttacagtatttcccagattgggggatacactttagcaagtatctgcgattatttgtttatgtaagatgtcccttcccttctgtgaatcatcattcttcaccccaagtatcttgagattggattctgtataagcagaatacaacagttaggcattcaggtatcattaaattcctccgcttcaaggatgaaaatttctttgggtatctaatagagtacaaagcagaaggtgtttcagaaatatttgcagtattgaatccgcatattcctccaagatagccctaatctaactggcagggtcccactcttcccagattaatgcccactcacataacaaacctgatgaggtagtgaagaaaactaactttgtgagtaagcaactggcagagtttttcaccactgtgactctatagctacatgtaactaagtagtatcactgacacataatcttaaattgaagttttaagatcattattctccatgttatacatgggtatcaaaagcattcccctcttgaccactccagaattctgtttaaaatttttcaatgacaacttatccatttccccaaagcctcagtgagcacatgatgccaacaattcatttcatgacttcatagcatgggccaagtttcttgcttaaaagacttccatcctgtcttgggaaacaaccatttccaaatatccacatatccttgcaagtttctgcctactcctctaccacccatttctgaagccatctgatttagtaagctgtatgcaaaagatacacaatggctaatgcaatcaaacaaggaatgtattaaaagcacacccaatagctcaaaataaaagacaagtgaacaaagttaagaaaatgacagtaacaaaagctgttctgggaacctctattgaaatagctacttattacatcaacatgctaccacagaacaaaagctcatgttgcttttctgaacttgaaaaacccattaacaatgtacagttctgagcctcagctgaccatagtgctcatgccaagtcctgagcagggcatcttgaatggtggttccctcatgactacatacaccgttagggaatgtttcgttaagaggaaatcaagatgttctaacctgtgaaggtagaatagattccaggctacacaaacacatgaagtgtgccttatattgattactaaagaggttgctgccaagactgcttccaaagggcagaagatagccctaaaaaatgtttgcagtgtggaaatgcatttttagtaagtcatattctagtaacaagttgcatttggtaagacacaaagaaacaatgttggtatgcagagtagaaatctctggaagatgatattgtcatatcagagatattgtcagtatcagagatactgaaatctctggaagatgatttttgtctcacatatggcattcgcaagtaaaatgccaaactgcaaaattcatattatgtagtacacataggaagatatctaaatatccctgtaggctctgggatgttatttcttattcttaacctccttactagattcacttgtacaatgaaataatctgtatcttattatttataattgagaattttctcaaaccttttcctgaaattttggaacacctggaataaaatttcttaaaatgattcctaaaagaaataattcttcaaaattaatattaagatataataacaggttggtttttttttttttttttttttttttttttagaatgaagcttctaaggtgaggttaacagtccagctgtggtttatttggtacattcataagatgttcactcctatatatattttttccctaggggtttctcatttctagatttacactttcccttatagcatggtccctccaaggtatatgcttccgatacataaaatgtttgtaattttgttaattctgccattcattagctcaataatttctctcattaaaattctgtaaactatgaatttcaaagaagtctattctatattcatctggttcatgaagtttcctctttgtgaatcttattttagtaaaatgactttacaacgtttaacatggttcctcacctgtatgaactttttaaaaaaaggtatgacttgctgctaaaaattttcagagtggttactaaattcagttttcctgtgtattgtctactatctttttgcatgtaaagaacagctttctgtggatgcctttccatatgctgtgcattcataaagtttctattcagtatgagttttctggaagatgacaagatgattccacttacagagtttctctttatatatgattgtttctatctcttgtgaatccacttttcagagtttcgtaaaattatcaatgtttgtcatctacatgagttctctgatgcataatgagctgtgacttccaacaaaaggctttcccacattcagtgcacttacaaggcttctctcctgtatgtgttctctgatgtgcactgagaattgatttttgagagaaggttttcccacattcattgcacccatagggtttctctcctgaatgagttctttgatgtacaatgagttgagaattcctaatgaaggcttttccacactcactgcattcatatggtttctctcttgtgtgcattctctggtgtacaagaaggcgtaatttcccactgaaggatttctcacattgactgcatttataagggttgacccctgcatgagttcgctcatgtacaatgagtagtgatttccaaatgaaggctttcccacattcattacattcatatggtttttcacctgaatgagttctcatgtgtataattaggtatgacttgctgctaaaagctttcccacattcactgcacccataaggcttttcccctgcatgagttcgctgatgtgaaatgagctggtctttcctattaaaggctttcccacattcactgcattcatagggattttctcctgtgtgaattctctgatgcacaatgagttgtgaattgaaactaaaggatttcccgcattccctgcactcatgtggtttctctcctgtatgagttctcatatgtataataaggtatgacttgctcctgaaggctttcccacactcactgcatccatatggttttactcctgtgtgacttctctgatgtacaatgagctgggacttcaaactaaaggtttttgcacattgactgcatccatagggttttactccagtgtgcactcctttatgtacaatgagctgtgatttgaacgtaaaggcttttccacattcattacaactatagggtttctctcctgtatgagttctctgatgtacaatcaggtttgactttgtattaaaggctttctgacactcactacattcaaatggtttctcccctgtatgagttctctggtgtataataagctgtgactttaaaccaaaagcctttccacagtcggtgcattcataaggcttctctcctgcatgagttctctggtgtgaaataagctggtatttccgactgaaggctttcccacattcatggcattcataggggttctctcctgtatgaatcctctgatgtataatgagctgtgatttaaaactgaaggctttcccacaattgttgcattcatggagtttttctcctgtatgagtccttgtatgtataataaggtatgacttgctcctgaaggctttgccacattcattgcatacataaggtttcattcctgtgtgacttctctgatgtacaatgagctgtgatttcaaactgaatcctttaccacactgaatacacccatagggctttactcctgtgtgaatcccctgatgtacaatgagctgtgacttgaatgtaaaggcttttccacaatcactacaaacataaggtttctcccctgtatgggttctctgatgtaccataaggtttgactttgtattaaaggctttctgacattcattgcattcatatggtttctctcctgtatgaattctttcatgtataatgagctgtgattttaaaccaaaagctttcccacattcattacacacatatggtttctgtcctgaatgagttttctggtgtgaaacaagctggtctttcctactgaagactttcccacattcacagcactcatagggattctcacctgtgtgaattctctgatgtataacaagctgtgaatggaaactgaatgttttcctgcattcactgcattcatgtagtttctctcctgtatgaattctctgatgtacaatgaggtatgatttactactgaagtctttcccacattcattacaaccatagggtttctcttcggcatgagtttgctgatgcactagaaggtatgacttgctgctgaaggctttctcacaacagctgcatccaaagggtttttcgcccatatacatttgttggcacataagttgcgatttcttattgacggtttttccagattcaatactttcacagtattttattccaataacagtttgctcatgtttagaatggaagaatgattttccatgtacctgaaacccattaggattatttctagcataatcactagtgaaatctatatatttcaaactctttccatgcgtgccacatttatgaggtttttgtcttgaaagatactttgtactaagaagacatagttttccaaatgtagtgcattcaaagctttttgccgtacttcccagcttgtctttattttcctgatgccaatccataagatcatcaattttccagactgtgtttggacaggtctgatttggaacttgggcctgcaccatacacagctcttctccttgttccaacttgaagatgatatcaggtttggtgtgttggtaccccaggacttggtgatttttggctgctcttgggaaataaacagccactctaggactttctctattctgcgactcttctgcttctgcctgggtgttccagggagaggttgcagaccaggagtcccttggcccaagatggattcctgaccttggagctttctgatcctatcccatgaactgtttcgttcttggagaggtgggacccaaatagaagctgtccggaccctggtggccatccctacggtcagttttgtgtgcctcgctggaagtgacaggacgcgagggatgctccggctcctccaaaccctgaaggggcagcagaatagagtccagggtactgcctccacctccagatctgcagccagaagggttcgcaaccactccagactcggctggcccgttgaccacgacgggcgatgaacgctatctgaggaacaaggatctcgccatcggcgcggaacaatggcggccgctacgtat

SEQ ID NO: 12596 - RNA, 7146 nt, Homo sapiens
  source 1..7146: mol_type = other RNA
gatctcactttgttgcccaggatggagtgcaggggcatgatcatagctcactgtagccttgaactactggactcaagctaacctcctgcctcagcctcctcagtaggtgggactaccggcacttgccactacacctggctgatcttttttttgagatggaggcttgttctgtcgcccagcctggagtgcagtggtgcaatcttggctcactgcaactgccacctcctaggttcaagcaattcttctgcctcagcctcccgagtagatgggattacaggcacgtgccaccacacctggctgacttttgtatttttagtagagacggggtttcaccatgttagccacactggtcttgaaatcctgacctcaagtgatctgcccacctcggcctcccaaagtgctgggattacaggcatgagccacggcgcctgaccacacctggctaatctttttaaaaagtttttgtacagacagggtctccctatattggtcaggcttgtctcgaactcctgggttccagcaatcctccagcctcagccttcccaagtgctggtattacatggatgagccactgcacctggctaattttactttaaaggaatctttctactattttatcattaagtatgacatttgtgttttcagaacatatattccctaccaagttacaggagttaattttaattcccaacttaatagtattttagtgtcatctatgggtgttaaattccatcaagtgatttatcagcatatactgagataatccttatgagttttatctggtagttaattaaaatattttctaatattaaatcttccaaacatactcttctgttttttgagacagggtctagttctgtcacccagggtggagtacagtggtacgatctcagctcactgcaacttccgcctcctagattcaagtgattctcccgtcccagcctcccaagtagctgggattataggtgtcagttaccatgccctgctatttttttgtatttttagtagagaggggtttcaccatgttggccaggctggtctcaaactcctgacctcaggtgatccaccatctcagcctcctgaagtgctgggattataggtgtgagccaccgtgcctggccccatatatctctttttaagtgggcatactgccattataaataatagtgattctgctggtaatgaacaaaggatgctggatccactaatagtctgttaaacctaatatcatgactttcttgttagctatacattggtttgctataattccatttagaatttttaaacctatgttcacaaatatggatttttaaacctatgttcacaaatatggatttttaaacctatgttcacaaatatggtttgcaagtcattttttctcctaaatttctatttgatggggaagttgtaaaatattggggttatttttccttggattttccttataataactattcctgaaaagtctctggaatgtctttcttttctggggctggggtagaaggactagatagatttacaaaccagtaactcaatttctgttttgtaaaattttcatttcattaaataataagtcctaatcaagtattattctttcccacagtatgtgagtgctgtcctcaatactgtcaacacttctggcttctaccaggcaaggctgcatgtagatttgcatctgaaaaaacaacaaactaaaatctaaccctaggtagtagtaaactgaatataaactttctcttatgaatttattctgtcttctttggtacatcaataataatatacacctttacagtatttcccagattgggggatacactttagcaagtatctgcgattatttgtttatgtaagatgtcccttcccttctgtgaatcatcattcttcaccccaagtatcttgagattggattctgtataagcagaatacaacagttaggcattcaggtatcattaaattcctccgcttcaaggatgaaaatttctttgggtatctaatagagtacaaagcagaaggtgtttcagaaatatttgcagtattgaatccgcatattcctccaagatagccctaatctaactggcagggtcccactcttcccagattaatgcccactcacataacaaacctgatgaggtagtgaagaaaactaactttgtgagtaagcaactggcagagtttttcaccactgtgactctatagctacatgtaactaagtagtatcactgacacataatcttaaattgaagttttaagatcattattctccatgttatacatgggtatcaaaagcattcccctcttgaccactccagaattctgtttaaaatttttcaatgacaacttatccatttccccaaagcctcagtgagcacatgatgccaacaattcatttcatgacttcatagcatgggccaagtttcttgcttaaaagacttccatcctgtcttgggaaacaaccatttccaaatatccacatatccttgcaagtttctgcctactcctctaccacccatttctgaagccatctgatttagtaagctgtatgcaaaagatacacaatggctaatgcaatcaaacaaggaatgtattaaaagcacacccaatagctcaaaataaaagacaagtgaacaaagttaagaaaatgacagtaacaaaagctgttctgggaacctctattgaaatagctacttattacatcaacatgctaccacagaacaaaagctcatgttgcttttctgaacttgaaaaacccattaacaatgtacagttctgagcctcagctgaccatagtgctcatgccaagtcctgagcagggcatcttgaatggtggttccctcatgactacatacaccgttagggaatgtttcgttaagaggaaatcaagatgttctaacctgtgaaggtagaatagattccaggctacacaaacacatgaagtgtgccttatattgattactaaagaggttgctgccaagactgcttccaaagggcagaagatagccctaaaaaatgtttgcagtgtggaaatgcatttttagtaagtcatattctagtaacaagttgcatttggtaagacacaaagaaacaatgttggtatgcagagtagaaatctctggaagatgatattgtcatatcagagatattgtcagtatcagagatactgaaatctctggaagatgatttttgtctcacatatggcattcgcaagtaaaatgccaaactgcaaaattcatattatgtagtacacataggaagatatctaaatatccctgtaggctctgggatgttatttcttattcttaacctccttactagattcacttgtacaatgaaataatctgtatcttattatttataattgagaattttctcaaaccttttcctgaaattttggaacacctggaataaaatttcttaaaatgattcctaaaagaaataattcttcaaaattaatattaagatataataacaggttggtttttttttttttttttttttttttttttagaatgaagcttctaaggtgaggttaacagtccagctgtggtttatttggtacattcataagatgttcactcctatatatattttttccctaggggtttctcatttctagatttacactttcccttatagcatggtccctccaaggtatatgcttccgatacataaaatgtttgtaattttgttaattctgccattcattagctcaataatttctctcattaaaattctgtaaactatgaatttcaaagaagtctattctatattcatctggttcatgaagtttcctctttgtgaatcttattttagtaaaatgactttacaacgtttaacatggttcctcacctgtatgaactttttaaaaaaaggtatgacttgctgctaaaaattttcagagtggttactaaattcagttttcctgtgtattgtctactatctttttgcatgtaaagaacagctttctgtggatgcctttccatatgctgtgcattcataaagtttctattcagtatgagttttctggaagatgacaagatgattccacttacagagtttctctttatatatgattgtttctatctcttgtgaatccacttttcagagtttcgtaaaattatcaatgtttgtcatctacatgagttctctgatgcataatgagctgtgacttccaacaaaaggctttcccacattcagtgcacttacaaggcttctctcctgtatgtgttctctgatgtgcactgagaattgatttttgagagaaggttttcccacattcattgcacccatagggtttctctcctgaatgagttctttgatgtacaatgagttgagaattcctaatgaaggcttttccacactcactgcattcatatggtttctctcttgtgtgcattctctggtgtacaagaaggcgtaatttcccactgaaggatttctcacattgactgcatttataagggttgacccctgcatgagttcgctcatgtacaatgagtagtgatttccaaatgaaggctttcccacattcattacattcatatggtttttcacctgaatgagttctcatgtgtataattaggtatgacttgctgctaaaagctttcccacattcactgcacccataaggcttttcccctgcatgagttcgctgatgtgaaatgagctggtctttcctattaaaggctttcccacattcactgcattcatagggattttctcctgtgtgaattctctgatgcacaatgagttgtgaattgaaactaaaggatttcccgcattccctgcactcatgtggtttctctcctgtatgagttctcatatgtataataaggtatgacttgctcctgaaggctttcccacactcactgcatccatatggttttactcctgtgtgacttctctgatgtacaatgagctgggacttcaaactaaaggtttttgcacattgactgcatccatagggttttactccagtgtgcactcctttatgtacaatgagctgtgatttgaacgtaaaggcttttccacattcattacaactatagggtttctctcctgtatgagttctctgatgtacaatcaggtttgactttgtattaaaggctttctgacactcactacattcaaatggtttctcccctgtatgagttctctggtgtataataagctgtgactttaaaccaaaagcctttccacagtcggtgcattcataaggcttctctcctgcatgagttctctggtgtgaaataagctggtatttccgactgaaggctttcccacattcatggcattcataggggttctctcctgtatgaatcctctgatgtataatgagctgtgatttaaaactgaaggctttcccacaattgttgcattcatggagtttttctcctgtatgagtccttgtatgtataataaggtatgacttgctcctgaaggctttgccacattcattgcatacataaggtttcattcctgtgtgacttctctgatgtacaatgagctgtgatttcaaactgaatcctttaccacactgaatacacccatagggctttactcctgtgtgaatcccctgatgtacaatgagctgtgacttgaatgtaaaggcttttccacaatcactacaaacataaggtttctcccctgtatgggttctctgatgtaccataaggtttgactttgtattaaaggctttctgacattcattgcattcatatggtttctctcctgtatgaattctttcatgtataatgagctgtgattttaaaccaaaagctttcccacattcattacacacatatggtttctgtcctgaatgagttttctggtgtgaaacaagctggtctttcctactgaagactttcccacattcacagcactcatagggattctcacctgtgtgaattctctgatgtataacaagctgtgaatggaaactgaatgttttcctgcattcactgcattcatgtagtttctctcctgtatgaattctctgatgtacaatgaggtatgatttactactgaagtctttcccacattcattacaaccatagggtttctcttcggcatgagtttgctgatgcactagaaggtatgacttgctgctgaaggctttctcacaacagctgcatccaaagggtttttcgcccatatacatttgttggcacataagttgcgatttcttattgacggtttttccagattcaatactttcacagtattttattccaataacagtttgctcatgtttagaatggaagaatgattttccatgtacctgaaacccattaggattatttctagcataatcactagtgaaatctatatatttcaaactctttccatgcgtgccacatttatgaggtttttgtcttgaaagatactttgtactaagaagacatagttttccaaatgtagtgcattcaaagctttttgccgtacttcccagcttgtctttattttcctgatgccaatccataagatcatcaattttccagactgtgtttggacaggtctgatttggaacttgggcctgcaccatacacagctcttctccttgttccaacttgaagatgatatcaggtttggtgtgttggtaccctagggacaccaggttgctatagttctccaacatcacactcctgtacaggcacttctgtgctgggtctagcagctgccactcctcccaggtaaaatccacaaacacatccatgaatgacaaaggtccccaggacttggtgatttttggctgctcttgggaaataaacagccactctaggactttctctattctgcgactcttctgcttctgcctgggtgttccagggagaggttgcagaccaggagtcccttggcccaagatggattcctgaccttggagctttctgatcctatcccatgaactgtttcgttcttggagaggtgggacccaaatagaagctgtccggaccctggtggccatccctacggtcagttttgtgtgcctcgctggaagtgacaggacgcgagggatgctccagatctgcagccagaagggttcgcaaccactccagactcggctggcccgttgaccacgacgggcgatgaacgctatctgaggaacaaggatctcgccatcggcgcggaacaatggcggccgctacgtat

SEQ ID NO: 12597 - RNA, 7205 nt, Homo sapiens
  source 1..7205: mol_type = other RNA
gatctcactttgttgcccaggatggagtgcaggggcatgatcatagctcactgtagccttgaactactggactcaagctaacctcctgcctcagcctcctcagtaggtgggactaccggcacttgccactacacctggctgatcttttttttgagatggaggcttgttctgtcgcccagcctggagtgcagtggtgcaatcttggctcactgcaactgccacctcctaggttcaagcaattcttctgcctcagcctcccgagtagatgggattacaggcacgtgccaccacacctggctgacttttgtatttttagtagagacggggtttcaccatgttagccacactggtcttgaaatcctgacctcaagtgatctgcccacctcggcctcccaaagtgctgggattacaggcatgagccacggcgcctgaccacacctggctaatctttttaaaaagtttttgtacagacagggtctccctatattggtcaggcttgtctcgaactcctgggttccagcaatcctccagcctcagccttcccaagtgctggtattacatggatgagccactgcacctggctaattttactttaaaggaatctttctactattttatcattaagtatgacatttgtgttttcagaacatatattccctaccaagttacaggagttaattttaattcccaacttaatagtattttagtgtcatctatgggtgttaaattccatcaagtgatttatcagcatatactgagataatccttatgagttttatctggtagttaattaaaatattttctaatattaaatcttccaaacatactcttctgttttttgagacagggtctagttctgtcacccagggtggagtacagtggtacgatctcagctcactgcaacttccgcctcctagattcaagtgattctcccgtcccagcctcccaagtagctgggattataggtgtcagttaccatgccctgctatttttttgtatttttagtagagaggggtttcaccatgttggccaggctggtctcaaactcctgacctcaggtgatccaccatctcagcctcctgaagtgctgggattataggtgtgagccaccgtgcctggccccatatatctctttttaagtgggcatactgccattataaataatagtgattctgctggtaatgaacaaaggatgctggatccactaatagtctgttaaacctaatatcatgactttcttgttagctatacattggtttgctataattccatttagaatttttaaacctatgttcacaaatatggatttttaaacctatgttcacaaatatggatttttaaacctatgttcacaaatatggtttgcaagtcattttttctcctaaatttctatttgatggggaagttgtaaaatattggggttatttttccttggattttccttataataactattcctgaaaagtctctggaatgtctttcttttctggggctggggtagaaggactagatagatttacaaaccagtaactcaatttctgttttgtaaaattttcatttcattaaataataagtcctaatcaagtattattctttcccacagtatgtgagtgctgtcctcaatactgtcaacacttctggcttctaccaggcaaggctgcatgtagatttgcatctgaaaaaacaacaaactaaaatctaaccctaggtagtagtaaactgaatataaactttctcttatgaatttattctgtcttctttggtacatcaataataatatacacctttacagtatttcccagattgggggatacactttagcaagtatctgcgattatttgtttatgtaagatgtcccttcccttctgtgaatcatcattcttcaccccaagtatcttgagattggattctgtataagcagaatacaacagttaggcattcaggtatcattaaattcctccgcttcaaggatgaaaatttctttgggtatctaatagagtacaaagcagaaggtgtttcagaaatatttgcagtattgaatccgcatattcctccaagatagccctaatctaactggcagggtcccactcttcccagattaatgcccactcacataacaaacctgatgaggtagtgaagaaaactaactttgtgagtaagcaactggcagagtttttcaccactgtgactctatagctacatgtaactaagtagtatcactgacacataatcttaaattgaagttttaagatcattattctccatgttatacatgggtatcaaaagcattcccctcttgaccactccagaattctgtttaaaatttttcaatgacaacttatccatttccccaaagcctcagtgagcacatgatgccaacaattcatttcatgacttcatagcatgggccaagtttcttgcttaaaagacttccatcctgtcttgggaaacaaccatttccaaatatccacatatccttgcaagtttctgcctactcctctaccacccatttctgaagccatctgatttagtaagctgtatgcaaaagatacacaatggctaatgcaatcaaacaaggaatgtattaaaagcacacccaatagctcaaaataaaagacaagtgaacaaagttaagaaaatgacagtaacaaaagctgttctgggaacctctattgaaatagctacttattacatcaacatgctaccacagaacaaaagctcatgttgcttttctgaacttgaaaaacccattaacaatgtacagttctgagcctcagctgaccatagtgctcatgccaagtcctgagcagggcatcttgaatggtggttccctcatgactacatacaccgttagggaatgtttcgttaagaggaaatcaagatgttctaacctgtgaaggtagaatagattccaggctacacaaacacatgaagtgtgccttatattgattactaaagaggttgctgccaagactgcttccaaagggcagaagatagccctaaaaaatgtttgcagtgtggaaatgcatttttagtaagtcatattctagtaacaagttgcatttggtaagacacaaagaaacaatgttggtatgcagagtagaaatctctggaagatgatattgtcatatcagagatattgtcagtatcagagatactgaaatctctggaagatgatttttgtctcacatatggcattcgcaagtaaaatgccaaactgcaaaattcatattatgtagtacacataggaagatatctaaatatccctgtaggctctgggatgttatttcttattcttaacctccttactagattcacttgtacaatgaaataatctgtatcttattatttataattgagaattttctcaaaccttttcctgaaattttggaacacctggaataaaatttcttaaaatgattcctaaaagaaataattcttcaaaattaatattaagatataataacaggttggtttttttttttttttttttttttttttttagaatgaagcttctaaggtgaggttaacagtccagctgtggtttatttggtacattcataagatgttcactcctatatatattttttccctaggggtttctcatttctagatttacactttcccttatagcatggtccctccaaggtatatgcttccgatacataaaatgtttgtaattttgttaattctgccattcattagctcaataatttctctcattaaaattctgtaaactatgaatttcaaagaagtctattctatattcatctggttcatgaagtttcctctttgtgaatcttattttagtaaaatgactttacaacgtttaacatggttcctcacctgtatgaactttttaaaaaaaggtatgacttgctgctaaaaattttcagagtggttactaaattcagttttcctgtgtattgtctactatctttttgcatgtaaagaacagctttctgtggatgcctttccatatgctgtgcattcataaagtttctattcagtatgagttttctggaagatgacaagatgattccacttacagagtttctctttatatatgattgtttctatctcttgtgaatccacttttcagagtttcgtaaaattatcaatgtttgtcatctacatgagttctctgatgcataatgagctgtgacttccaacaaaaggctttcccacattcagtgcacttacaaggcttctctcctgtatgtgttctctgatgtgcactgagaattgatttttgagagaaggttttcccacattcattgcacccatagggtttctctcctgaatgagttctttgatgtacaatgagttgagaattcctaatgaaggcttttccacactcactgcattcatatggtttctctcttgtgtgcattctctggtgtacaagaaggcgtaatttcccactgaaggatttctcacattgactgcatttataagggttgacccctgcatgagttcgctcatgtacaatgagtagtgatttccaaatgaaggctttcccacattcattacattcatatggtttttcacctgaatgagttctcatgtgtataattaggtatgacttgctgctaaaagctttcccacattcactgcacccataaggcttttcccctgcatgagttcgctgatgtgaaatgagctggtctttcctattaaaggctttcccacattcactgcattcatagggattttctcctgtgtgaattctctgatgcacaatgagttgtgaattgaaactaaaggatttcccgcattccctgcactcatgtggtttctctcctgtatgagttctcatatgtataataaggtatgacttgctcctgaaggctttcccacactcactgcatccatatggttttactcctgtgtgacttctctgatgtacaatgagctgggacttcaaactaaaggtttttgcacattgactgcatccatagggttttactccagtgtgcactcctttatgtacaatgagctgtgatttgaacgtaaaggcttttccacattcattacaactatagggtttctctcctgtatgagttctctgatgtacaatcaggtttgactttgtattaaaggctttctgacactcactacattcaaatggtttctcccctgtatgagttctctggtgtataataagctgtgactttaaaccaaaagcctttccacagtcggtgcattcataaggcttctctcctgcatgagttctctggtgtgaaataagctggtatttccgactgaaggctttcccacattcatggcattcataggggttctctcctgtatgaatcctctgatgtataatgagctgtgatttaaaactgaaggctttcccacaattgttgcattcatggagtttttctcctgtatgagtccttgtatgtataataaggtatgacttgctcctgaaggctttgccacattcattgcatacataaggtttcattcctgtgtgacttctctgatgtacaatgagctgtgatttcaaactgaatcctttaccacactgaatacacccatagggctttactcctgtgtgaatcccctgatgtacaatgagctgtgacttgaatgtaaaggcttttccacaatcactacaaacataaggtttctcccctgtatgggttctctgatgtaccataaggtttgactttgtattaaaggctttctgacattcattgcattcatatggtttctctcctgtatgaattctttcatgtataatgagctgtgattttaaaccaaaagctttcccacattcattacacacatatggtttctgtcctgaatgagttttctggtgtgaaacaagctggtctttcctactgaagactttcccacattcacagcactcatagggattctcacctgtgtgaattctctgatgtataacaagctgtgaatggaaactgaatgttttcctgcattcactgcattcatgtagtttctctcctgtatgaattctctgatgtacaatgaggtatgatttactactgaagtctttcccacattcattacaaccatagggtttctcttcggcatgagtttgctgatgcactagaaggtatgacttgctgctgaaggctttctcacaacagctgcatccaaagggtttttcgcccatatacatttgttggcacataagttgcgatttcttattgacggtttttccagattcaatactttcacagtattttattccaataacagtttgctcatgtttagaatggaagaatgattttccatgtacctgaaacccattaggattatttctagcataatcactagtgaaatctatatatttcaaactctttccatgcgtgccacatttatgaggtttttgtcttgaaagatactttgtactaagaagacatagttttccaaatgtagtgcattcaaagctttttgccgtacttcccagcttgtctttattttcctgatgccaatccataagatcatcaattttccagactgtgtttggacaggtctgatttggaacttgggcctgcaccatacacagctcttctccttgttccaacttgaagatgatatcaggtttggtgtgttggtaccctagggacaccaggttgctatagttctccaacatcacactcctgtacaggcacttctgtgctgggtctagcagctgccactcctcccaggtaaaatccacaaacacatccatgaatgacaaaggtccccaggacttggtgatttttggctgctcttgggaaataaacagccactctaggactttctctattctgcgactcttctgcttctgcctgggtgttccagggagaggttgcagaccaggagtcccttggcccaagatggattcctgaccttggagctttctgatcctatcccatgaactgtttcgttcttggagaggtgggacccaaatagaagctgtccggaccctggtggccatccctacggtcagttttgtgtgcctcgctggaagtgacaggacgcgagggatgctccggctcctccaaaccctgaaggggcagcagaatagagtccagggtactgcctccacctccagatctgcagccagaagggttcgcaaccactccagactcggctggcccgttgaccacgacgggcgatgaacgctatctgaggaacaaggatctcgccatcggcgcggaacaatggcggccgctacgtat

SEQ ID NO: 12598 - RNA, 7153 nt, Homo sapiens
  source 1..7153: mol_type = other RNA
gatctcactttgttgcccaggatggagtgcaggggcatgatcatagctcactgtagccttgaactactggactcaagctaacctcctgcctcagcctcctcagtaggtgggactaccggcacttgccactacacctggctgatcttttttttgagatggaggcttgttctgtcgcccagcctggagtgcagtggtgcaatcttggctcactgcaactgccacctcctaggttcaagcaattcttctgcctcagcctcccgagtagatgggattacaggcacgtgccaccacacctggctgacttttgtatttttagtagagacggggtttcaccatgttagccacactggtcttgaaatcctgacctcaagtgatctgcccacctcggcctcccaaagtgctgggattacaggcatgagccacggcgcctgaccacacctggctaatctttttaaaaagtttttgtacagacagggtctccctatattggtcaggcttgtctcgaactcctgggttccagcaatcctccagcctcagccttcccaagtgctggtattacatggatgagccactgcacctggctaattttactttaaaggaatctttctactattttatcattaagtatgacatttgtgttttcagaacatatattccctaccaagttacaggagttaattttaattcccaacttaatagtattttagtgtcatctatgggtgttaaattccatcaagtgatttatcagcatatactgagataatccttatgagttttatctggtagttaattaaaatattttctaatattaaatcttccaaacatactcttctgttttttgagacagggtctagttctgtcacccagggtggagtacagtggtacgatctcagctcactgcaacttccgcctcctagattcaagtgattctcccgtcccagcctcccaagtagctgggattataggtgtcagttaccatgccctgctatttttttgtatttttagtagagaggggtttcaccatgttggccaggctggtctcaaactcctgacctcaggtgatccaccatctcagcctcctgaagtgctgggattataggtgtgagccaccgtgcctggccccatatatctctttttaagtgggcatactgccattataaataatagtgattctgctggtaatgaacaaaggatgctggatccactaatagtctgttaaacctaatatcatgactttcttgttagctatacattggtttgctataattccatttagaatttttaaacctatgttcacaaatatggatttttaaacctatgttcacaaatatggatttttaaacctatgttcacaaatatggtttgcaagtcattttttctcctaaatttctatttgatggggaagttgtaaaatattggggttatttttccttggattttccttataataactattcctgaaaagtctctggaatgtctttcttttctggggctggggtagaaggactagatagatttacaaaccagtaactcaatttctgttttgtaaaattttcatttcattaaataataagtcctaatcaagtattattctttcccacagtatgtgagtgctgtcctcaatactgtcaacacttctggcttctaccaggcaaggctgcatgtagatttgcatctgaaaaaacaacaaactaaaatctaaccctaggtagtagtaaactgaatataaactttctcttatgaatttattctgtcttctttggtacatcaataataatatacacctttacagtatttcccagattgggggatacactttagcaagtatctgcgattatttgtttatgtaagatgtcccttcccttctgtgaatcatcattcttcaccccaagtatcttgagattggattctgtataagcagaatacaacagttaggcattcaggtatcattaaattcctccgcttcaaggatgaaaatttctttgggtatctaatagagtacaaagcagaaggtgtttcagaaatatttgcagtattgaatccgcatattcctccaagatagccctaatctaactggcagggtcccactcttcccagattaatgcccactcacataacaaacctgatgaggtagtgaagaaaactaactttgtgagtaagcaactggcagagtttttcaccactgtgactctatagctacatgtaactaagtagtatcactgacacataatcttaaattgaagttttaagatcattattctccatgttatacatgggtatcaaaagcattcccctcttgaccactccagaattctgtttaaaatttttcaatgacaacttatccatttccccaaagcctcagtgagcacatgatgccaacaattcatttcatgacttcatagcatgggccaagtttcttgcttaaaagacttccatcctgtcttgggaaacaaccatttccaaatatccacatatccttgcaagtttctgcctactcctctaccacccatttctgaagccatctgatttagtaagctgtatgcaaaagatacacaatggctaatgcaatcaaacaaggaatgtattaaaagcacacccaatagctcaaaataaaagacaagtgaacaaagttaagaaaatgacagtaacaaaagctgttctgggaacctctattgaaatagctacttattacatcaacatgctaccacagaacaaaagctcatgttgcttttctgaacttgaaaaacccattaacaatgtacagttctgagcctcagctgaccatagtgctcatgccaagtcctgagcagggcatcttgaatggtggttccctcatgactacatacaccgttagggaatgtttcgttaagaggaaatcaagatgttctaacctgtgaaggtagaatagattccaggctacacaaacacatgaagtgtgccttatattgattactaaagaggttgctgccaagactgcttccaaagggcagaagatagccctaaaaaatgtttgcagtgtggaaatgcatttttagtaagtcatattctagtaacaagttgcatttggtaagacacaaagaaacaatgttggtatgcagagtagaaatctctggaagatgatattgtcatatcagagatattgtcagtatcagagatactgaaatctctggaagatgatttttgtctcacatatggcattcgcaagtaaaatgccaaactgcaaaattcatattatgtagtacacataggaagatatctaaatatccctgtaggctctgggatgttatttcttattcttaacctccttactagattcacttgtacaatgaaataatctgtatcttattatttataattgagaattttctcaaaccttttcctgaaattttggaacacctggaataaaatttcttaaaatgattcctaaaagaaataattcttcaaaattaatattaagatataataacaggttggtttttttttttttttttttttttttttttagaatgaagcttctaaggtgaggttaacagtccagctgtggtttatttggtacattcataagatgttcactcctatatatattttttccctaggggtttctcatttctagatttacactttcccttatagcatggtccctccaaggtatatgcttccgatacataaaatgtttgtaattttgttaattctgccattcattagctcaataatttctctcattaaaattctgtaaactatgaatttcaaagaagtctattctatattcatctggttcatgaagtttcctctttgtgaatcttattttagtaaaatgactttacaacgtttaacatggttcctcacctgtatgaactttttaaaaaaaggtatgacttgctgctaaaaattttcagagtggttactaaattcagttttcctgtgtattgtctactatctttttgcatgtaaagaacagctttctgtggatgcctttccatatgctgtgcattcataaagtttctattcagtatgagttttctggaagatgacaagatgattccacttacagagtttctctttatatatgattgtttctatctcttgtgaatccacttttcagagtttcgtaaaattatcaatgtttgtcatctacatgagttctctgatgcataatgagctgtgacttccaacaaaaggctttcccacattcagtgcacttacaaggcttctctcctgtatgtgttctctgatgtgcactgagaattgatttttgagagaaggttttcccacattcattgcacccatagggtttctctcctgaatgagttctttgatgtacaatgagttgagaattcctaatgaaggcttttccacactcactgcattcatatggtttctctcttgtgtgcattctctggtgtacaagaaggcgtaatttcccactgaaggatttctcacattgactgcatttataagggttgacccctgcatgagttcgctcatgtacaatgagtagtgatttccaaatgaaggctttcccacattcattacattcatatggtttttcacctgaatgagttctcatgtgtataattaggtatgacttgctgctaaaagctttcccacattcactgcacccataaggcttttcccctgcatgagttcgctgatgtgaaatgagctggtctttcctattaaaggctttcccacattcactgcattcatagggattttctcctgtgtgaattctctgatgcacaatgagttgtgaattgaaactaaaggatttcccgcattccctgcactcatgtggtttctctcctgtatgagttctcatatgtataataaggtatgacttgctcctgaaggctttcccacactcactgcatccatatggttttactcctgtgtgacttctctgatgtacaatgagctgggacttcaaactaaaggtttttgcacattgactgcatccatagggttttactccagtgtgcactcctttatgtacaatgagctgtgatttgaacgtaaaggcttttccacattcattacaactatagggtttctctcctgtatgagttctctgatgtacaatcaggtttgactttgtattaaaggctttctgacactcactacattcaaatggtttctcccctgtatgagttctctggtgtataataagctgtgactttaaaccaaaagcctttccacagtcggtgcattcataaggcttctctcctgcatgagttctctggtgtgaaataagctggtatttccgactgaaggctttcccacattcatggcattcataggggttctctcctgtatgaatcctctgatgtataatgagctgtgatttaaaactgaaggctttcccacaattgttgcattcatggagtttttctcctgtatgagtccttgtatgtataataaggtatgacttgctcctgaaggctttgccacattcattgcatacataaggtttcattcctgtgtgacttctctgatgtacaatgagctgtgatttcaaactgaatcctttaccacactgaatacacccatagggctttactcctgtgtgaatcccctgatgtacaatgagctgtgacttgaatgtaaaggcttttccacaatcactacaaacataaggtttctcccctgtatgggttctctgatgtaccataaggtttgactttgtattaaaggctttctgacattcattgcattcatatggtttctctcctgtatgaattctttcatgtataatgagctgtgattttaaaccaaaagctttcccacattcattacacacatatggtttctgtcctgaatgagttttctggtgtgaaacaagctggtctttcctactgaagactttcccacattcacagcactcatagggattctcacctgtgtgaattctctgatgtataacaagctgtgaatggaaactgaatgttttcctgcattcactgcattcatgtagtttctctcctgtatgaattctctgatgtacaatgaggtatgatttactactgaagtctttcccacattcattacaaccatagggtttctcttcggcatgagtttgctgatgcactagaaggtatgacttgctgctgaaggctttctcacaacagctgcatccaaagggtttttcgcccatatacatttgttggcacataagttgcgatttcttattgacggtttttccagattcaatactttcacagtattttattccaataacagtttgctcatgtttagaatggaagaatgattttccatgtacctgaaacccattaggattatttctagcataatcactagtgaaatctatatatttcaaactctttccatgcgtgccacatttatgaggtttttgtcttgaaagatactttgtactaagaagacatagttttccaaatgtagtgcattcaaagctttttgccgtacttcccagcttgtctttattttcctgatgccaatccataagatcatcaattttccagactgtgtttggacaggtctgatttggaacttgggcctgcaccatacacagctcttctccttgttccaacttgaagatgatatcaggtttggtgtgttggtaccctagggacaccaggttgctatagttctccaacatcacactcctgtacaggcacttctgtgctgggtctagcagctgccactcctcccaggtaaaatccacaaacacatccatgaatgacaaaggtccccaggacttggtgatttttggctgctcttgggaaataaacagccactctaggactttctctattctgcgactcttctgcttctgcctgggtgttccagggagaggttgcagaccaggagtcccttggcccaagatggattcctgaccttggagctttctgatcctatcccatgaactgtttcgttcttggagaggtgggacctgtggaccaaatagaagctgtccggaccctggtggccatccctacggtcagttttgtgtgcctcgctggaagtgacaggacgcgagggatgctccagatctgcagccagaagggttcgcaaccactccagactcggctggcccgttgaccacgacgggcgatgaacgctatctgaggaacaaggatctcgccatcggcgcggaacaatggcggccgctacgtat

SEQ ID NO: 12599 - RNA, 50 nt, Homo sapiens
  source 1..50: mol_type = other RNA
gatctcactttgttgcccaggctagagggtagtggcacaatcttggctca

SEQ ID NO: 12600 - RNA, 191 nt, Homo sapiens
  source 1..191: mol_type = other RNA
gatctcactttgttgcccaggctagcctcaaacttctggcttcaagtcatcctcatgcctcagcctctagttggtggaggagaagatacattgtgtccatatgcactaaaacaacggctaagatcatttttatcatctgcatttcatcttttcatcattgtaagataattattaaatcaaagaaaagctca

SEQ ID NO: 12601 - RNA, 9648 nt, Homo sapiens
  source 1..9648: mol_type = other RNA
gatctcactttgttgcccaggctattttctggatgtctattaaaaaaaaattagtcctgcacagtgttctagaaagggtttttcttttcagaatatccatattctccaagtagcaagttagaatataaggaatatttgccattaaacctttctgttagaaatgtaaacatgaaattgcctaatatagacctatctcagatgctaaatagaattgtttataacacctttggaatataattatgtgagctacacttaaccatctggcattttgcttcctgcggacaatttgcaatagcatagaaaaatattttgtttgtgtatttcttatcaaacagatatgctaaagttctgtttagagagtaatagcattttattctaacttttaaaataaggtagtccatttgcagcagcttgatatataagtaaacaaaaatttttaatattaataaaacactagcacatacactgaaagcatctaagaaattcaaaatataaaacacttaccaagtaatgaccatatgagtggtaacatattgaataaaggccctttgaagaagttggagagttatgattactgagcaggctagataattaaataattacacattttgattgaaaaatatatgtagttcattaaaatagggactctaactccacttctctagctaagcttctattcagatgccacgtttgtactttaattagaacaaaagaccgacattaacttcaatgcaacataataattcataataatgattgtatattaatctcttgagcttgcaggaatatagcacatgacatatggcatgatacaggcacctgtgtgatcctttggggacttaggtggtgcatattaattagcccctggaaaataaaatctgtttccttctgagaaaagctacctcagtgcttattggcttaagccatcaaagaaattagatgaaatactgttaggctgggtctgcactcattaaagctttgtctagatgtaagcactgaatcaactgcctctgagttaagtcttgactgaatggtgcataagaaatcagagtaatcatgcatttctttggccttgatgattggattttggcatttaaaaaatccatcaaaattaccattttggttacagaaaattatgtaattgtataattcaaacaaaataatgtaaccagaaacactaaaatttgaagccacttcattttcctaaatgctgcttgaaactgcctcaatttaacccttttatttgtaaattcagattcaacccgaatatgagattataaatggcttaagaaatatgtcatcttgcaataatcagggtaacaagattcttgacggtcccaggtctgctaaaggcacttcagtgtgtatatctttgtcaggcaatggaacgatattatgaaactaaaactctggctgattaacagatcatttaaattgagactgatagatcttaaaattacttctcagggggaaaaagttacaatgctagagtgtacctagaaaacagaaacttgagtagacatggtaatgaccagaaaaggctatctttatacatttcttttgctacgcttcaaattcatgtcacctaaaagttgtgaagtgcacaaaacaaatctacttaactgaaaattattttcaatgaatgggatgtttagaactctgtgagggtttttaaggtcttttcgaatagcaaattctaatgaggcttttttaagttggcaatttaaactcatacaagaaataaaaactcaccagtgtggctgggcagaatatatatattttctcaaatattgtttgtttgttttttccctgcactgtatccatggtcccatgatgaaactgttatattgctgatatatttattggaatatgtgggccaacttcctttccactcaacatatggattggtagtttaaaataattcctttctattaagcaaatgtgtggctaaggcacatttaaatagcccattaaaccaatgagatgacaatgtgttaccctcagagaaagcttaatttttggagtaatcaattacacatatcacagaatgtctcatgagaacatttttggctaggtctaccaatttatcatacaaataattatagattttcatttgaggcaaagatgctgattcatcattagtaacatggtcacaaataatcatttattttatttttgttaacatctgtctttcctgtggggaaacttactatatgctctacgtttatttaatttaaaaagtcaattggttattctgaatttttaaaaataacataaaactgttgttctaaatcacagcacctgcttttctttttttagtgaaattatataagcatttagagaatgaaagtgtaagacttgtggtttctggtctctttttactgtttgtaagcctactcgtcatgatattccacaatggtgcacttgccttttaatgctcttatagatatcttcaaacttgcctacatatatacgcctttgttggagtgggctaccatcatcaggaatgatgtcatttgtttcttcaaactcctttattataccaaaaaagtgacagactccacagtctgatcagttttggagaaatatgttaacattttcaattatctcactttctagaatcaaaatagtctgattttttttttcggcactcagtgtaaagaacaaagaactgaatacagtgggcccagaagagaaatatgcctcatcatttttattagctttggaactgtggacaagtcactcaacctagttttctcattttgaaatgggttgttgtgggaattaaaaaaaaaaaaaaaaaaaaaaaaggatacatgggaaaaattctaaaacaccagtgcctgggatgtagcaggcacaaatataagctgcaactgaattgttttcttagagataaaatgggtccacttttcttttctcataatgattccattaataacaaatctttacgtctttcttgttattatgactcttcaatttatttagaaatgtcaattagtgttttcttggaaactacgattaacgtagattggaaattcttaaacttcagtgtgtgtaacagacatccagaaatcttgctgaagatgtagattcctagccctgtctttctaaatttcacattttgagaaacggtgatttagattgttgacttaacactggcctgacttgccctcttacagatatattttgctcaatgtccttcttcctgacttctggtgttctgtaaggattctccccactttctctcaagtacccagtctttgtgtcctttgcctgaattctcggggagagttttgtttgtcaggtacagtcagagaatgaactagccttgaattaaaagcagtgtttccagcccatgcaacatctgacagaatggctggttacatcgaatgcactggaaaagatcatttataaccctgtctcctcagggagaagcaagatatactgcatgagaaagcagagaagcttaaattccagtggtgcttttgttactaactaaatacatgactatgtccaagtttcttactcactttgggtttagttactatatctggtgggggtaattgataatgccttctctggctgaaggcaagatctcagggcttagaccagaatctttattaggctttcttttgattctgagacttatgcttttccataaagggcagtatctcatgtgtaccctgcctgaacataaatttcaccgttacacctttaccacattttcttcagagaatatttatgattcattatttcctaggcacaattctatgtatgaaagattgtgagaagtaccaggcatatagacgactcagcaacagcttaaacctactaccaattcacattaacacttgctattaatttgctcaggattttatttatttgaatctattgggggtggggaggggaggggagtgaaatgatatacatttggaggcaccctcaggtaatcacactatagaaataatgctgctagttaagaggtttgttgcaaagatgtaaagcagcatgtacagaatttgttggacgtctgctttaggtataatttaatatctccacgtatcttttaatagactaataaaaaaccatagttaactacagttttcaaatagcaaataacatataatttagaggtgaggaatacagaagaaggtttttatctatacagtgtgacttacctaggtacgcaatctttaaacaaaatgaagaagaaacatgttttctgttctcagtgctattgtaggttatgggaataaattaatttagaaatttgttctaaaataatgaactaccaaactgataatagcttgcctttatttgttttagtttcatctgtaagtgaataactggaatgaacacatcaacctttggttaaatataaggctttctagcttttgggcttacatgcacctgcttgtgtattcccacctcttttctgatgatctctgaagaggaagaaagagcatgaatgcctaggtatgcacaagcctatttatttctagacctttcctatacacactcttcaacatggcaaatgtttgcaaacaaatacattggttaaaaaaataatattgtaaggtagtttcatttttcatctaaaaatatgtgcacacaggcaatttcgatgaaaatggatttctgcttgaattatctagctaattgcctctattccctgctttgccttgagcatataaaaattatttagggtagacagtgttgaaccttataaatcaattaatcagtattgattaattatttcccctcaactttagtttgcctttaaactaagactaggtttatgctcatccataaaaagtgaaaatttaaacatacacagactgtctgcaatgtcactctggcggtgtatcatggggagatatgtttgaattagatagagaaaatttatatgaaatactctgaggctatgtttcctaaggggaattgctttatccagtataggaaaaccatttttcacataaatttctaaagataaattagaactttaacctgacacctaataggtagaattttagggtttgggggaataataatagttgctagagctattcaatggcaatgtcaatataaaaagcttagttttccacatgagagaagaactgaagtgtagacgagacactctcttacagtaacactgcagaaacttagaagcatgaatattttctagatttccatcttagtcacaattaaggataaagaagaaaaaatatgaaaagtttcttcataatattaaggggcttttattgataaaacaactatttctttcatagtaagttctttttgtcagaggcagaaatagaaatttgattctttagaagacattttgggtttcaaagagaaactctgctactttactgttgaaaatatatagtactctgagaaagctgccttacagcaaggagtttcagaaaagatacaagaaagaaaaccaatgtgagatgctttcattttagagtccctgcttcagtgtttccaacagaaacaagagaaaaagtaataagaaatatttttttctccctcttaagacatacatcactcctgaaattcttagaaaatcaactgaggcaaattaggggtttcaaagctagtcaccttgtaagttgttaggaaaaaaatttgcatttaaattgctctatgtagctcccttgagattttctcctggaatgcttatggctcttttttcattaatacttaaaaaaatacaatttcataaccagtgtattactacatctagttgtgttaagaagagaaacttcatttcataaaatagaaacattcaaagtggtttaggtcaaccaatcactcagtcagaatacttgaattcttcatattgaacacttaatagtgaagttaatctgaaccatatcaactctccatttcttttacagaaactaagtcattaatagctctatcagagagaataaactgtgttcctatatgccctccccataggaacaaagatagtccagaacttcttggaaatttttccttaaaatagtacatatttttatatatcagatttctttttaataggtaattcttaagtcctatttcaataacttgctttacatattcagaaatgtagatataagaaaaatattaaatgtgcaaaatgttctttctatatttacatttaaaaaatacaatgtaataatagctttatacttgtcaaaaagccattggggaaaataagccttcaatgtcagaaaatctggttaaattagagcttttgcttgtggaattgtaaacaaacttttaaaaatgctcagagttttctcaattcttcccatccaagacactcttgaacacatcaagtcctgctttgaagtaaacctgagctgaattaatgctgttcaacacctctgacagggcttcttgaagggtctcatttgatgcaaggggtttgcagtgttcccaagcctctataagtattgaaaaccggcttgtcttttcatcaaggtggtagaggatgtttctataaaaacctggtggtgcctgctttaccagaaagcttttctccatgtcttggagaatgtcattcagcatccggatgcggatgggtgctctctccttgggatcattagcaggtcgcatctcatcagactgaaaaagttcagcactctcccgcaggcgtaacgccatggctaacagttgatgagtgttgggttgatcacctttaaggttgttttgaacttctaaagctatatcaagtgcattaaagggcagaacaggttcgttggcaatttgcaaaatcacttctcctgagagcttagtaatggtttcatgaaggttgaaagagggatccatttcttcaatttttgttgctcgtgtagaaaaacgggcctcggagagaaaacttggaccctctaatgttttgatgtcctcgtaagcaaactgcacgatgggaactccaagatggttgatgaaataatcagcatcaccttgtatctgtatagaactgatattggtttctgggcactgggctcttctggtacagttgaaattatttttctctactaccagttgctgaagagatggtgatgctacaggatacagactagagttcccccttatgggactgtggaggctaatataagccacaacatttttctgaagaaccttcttgaaatcctctccccattcatatgagccaatattgccaaaagctgttcctccccaagaacagaaaacaatagttcggtctggtctccaccctctcttaacttttgacatcaaggcacggataaacgctgtgattattgcagtactactggcccattcttgtccattataactgtgtgcagtgtgatgatggctgccaactatgatataccggtctggagatgtcaagcccattacaaatccaacaacattagtaactgttttcaattttgtgactgtctgaacttgcatgctgacgactcttatttcattatttggaagctctagagagctacacgcttcatttttggttctagcttttggcgaagagatcagttttgcaacgaggggtgcagagatgggctgcactaatagagaggtgaggtttgatcggctttgtctaaaactttcatcgacacttgggtaaccaggcgtagaagggtctcctcctggattcagtgacaccatgaaggtatcatggctaggattcacagtctttggcaaatcacaaggatcgatatacagaagaacacctccaaatccagccttttccaatgaggaaagcttataaagcagtggcaattttcctaatttcaggagtgcgatctgatttgttacgttttttattttcctaatcctttttaaatcatctgccattccataactcacatcgatgacttcagccttgagagttcctttggcagaataggctgcatatgaatagagcaggtcttggctgctatcttttctggcttcttcactgcaaggctggccattaggatgaaagcattgaccactgctgctcagagtcacagtgctgggagaagggcctggcagatcaagcagcacagagtaatttacaaactgtacatcttctaggcccaaagaggtccactgagtcttaatcttctttgaaatttccatgtcatcttcatttttatatagttgtaccaaatttctctttactttcttgctgaattccataaagaagtttgaaaagcctcccttgcagctagggaaggctatatgacaaaaatatgcccaatgtaaaatgaaagcctgttgaaagattcgggaaaagcatttatcttcctgataaaagtgattaatgtggctacagttgcctttcctctcctattcctgcttagatgcctagatctgtggtggctttctaatgaccctgaggtaaaaagtgtaaggatgaaaaccaagatgttgaaactggcaatgtcacaatgtgcatgggtttgtgacatcatcaatgatcaactgaaccaacaacagtgaccacctaactccaaacatcttgttttatttgtctaagccaatgttaactgaattttccgttacttgaaacttaaaactgctattattacttcgcctaattatatgttagattgtagaatttgatcatgcccaaatagcttcagtattctcacgaaaagcggcagagacccctacaaacagaagaagtcaaatatttaaatgaagtggaaccaagttagataatccacttaaccacatagacacaaacacaagagatgggcaaaaacaacacagaggtctgcaatctgatttggaaagtatcttagatggctaccctgatgttcttttctctttccttaagaggaaaaaaactatccctttgcaagtacaaatattacatttttagacaaaaagaaaaaacacaaaaattgaataacatatagctttgttcttaagaaacatgatatggttgaagaaaacaaaactgataatcaagaatgcttaagtgcttaatgctaatatactgtcagagcacaaaatttaacatggtcaattgtgttttatagaagattggtaagggctttgataatgtttcacagtggaggaaatacgtaagttgactcttgaaagattaatatgtattcactagagatacagaagaggggatgtaaggcagaggcagcagtttaagctaagaacacatggaaagtaaacggtagggtgcatctagacaactgcaggtaacccagctggaggcacagtagaaagagaaagtccgaaatagaggagccaggtcatgacctgaagccataattaagaatttggatagttttctgtaattaatatgtgacaatgagtatatcaagaacaatgtcaaatttttattagggcatagcacccaagcactagtgtggataggcactatgccaagtactcggaagttaaaaaggtttcatgacagaaatcatgacttgggaccattgccctaccatctattagtaccaccatccgtacatgtcctgaactgcattagtcattgcttagttcaaaagtctgagcactttataatcaacaaaaatctccatattctaatgtcttctcttggtttaaggacttttccaagtgattttgtccttcctattttaaaaattttaaaggtaatttttaaaagatgtctgctatggcttgaatgtcccctcc

SEQ ID NO: 12602 - RNA, 12109 nt, Homo sapiens
  source 1..12109: mol_type = other RNA
gatctcactttgttgcccaggctattttctggatgtctattaaaaaaaaattagtcctgcacagtgttctagaaagggtttttcttttcagaatatccatattctccaagtagcaagttagaatataaggaatatttgccattaaacctttctgttagaaatgtaaacatgaaattgcctaatatagacctatctcagatgctaaatagaattgtttataacacctttggaatataattatgtgagctacacttaaccatctggcattttgcttcctgcggacaatttgcaatagcatagaaaaatattttgtttgtgtatttcttatcaaacagatatgctaaagttctgtttagagagtaatagcattttattctaacttttaaaataaggtagtccatttgcagcagcttgatatataagtaaacaaaaatttttaatattaataaaacactagcacatacactgaaagcatctaagaaattcaaaatataaaacacttaccaagtaatgaccatatgagtggtaacatattgaataaaggccctttgaagaagttggagagttatgattactgagcaggctagataattaaataattacacattttgattgaaaaatatatgtagttcattaaaatagggactctaactccacttctctagctaagcttctattcagatgccacgtttgtactttaattagaacaaaagaccgacattaacttcaatgcaacataataattcataataatgattgtatattaatctcttgagcttgcaggaatatagcacatgacatatggcatgatacaggcacctgtgtgatcctttggggacttaggtggtgcatattaattagcccctggaaaataaaatctgtttccttctgagaaaagctacctcagtgcttattggcttaagccatcaaagaaattagatgaaatactgttaggctgggtctgcactcattaaagctttgtctagatgtaagcactgaatcaactgcctctgagttaagtcttgactgaatggtgcataagaaatcagagtaatcatgcatttctttggccttgatgattggattttggcatttaaaaaatccatcaaaattaccattttggttacagaaaattatgtaattgtataattcaaacaaaataatgtaaccagaaacactaaaatttgaagccacttcattttcctaaatgctgcttgaaactgcctcaatttaacccttttatttgtaaattcagattcaacccgaatatgagattataaatggcttaagaaatatgtcatcttgcaataatcagggtaacaagattcttgacggtcccaggtctgctaaaggcacttcagtgtgtatatctttgtcaggcaatggaacgatattatgaaactaaaactctggctgattaacagatcatttaaattgagactgatagatcttaaaattacttctcagggggaaaaagttacaatgctagagtgtacctagaaaacagaaacttgagtagacatggtaatgaccagaaaaggctatctttatacatttcttttgctacgcttcaaattcatgtcacctaaaagttgtgaagtgcacaaaacaaatctacttaactgaaaattattttcaatgaatgggatgtttagaactctgtgagggtttttaaggtcttttcgaatagcaaattctaatgaggcttttttaagttggcaatttaaactcatacaagaaataaaaactcaccagtgtggctgggcagaatatatatattttctcaaatattgtttgtttgttttttccctgcactgtatccatggtcccatgatgaaactgttatattgctgatatatttattggaatatgtgggccaacttcctttccactcaacatatggattggtagtttaaaataattcctttctattaagcaaatgtgtggctaaggcacatttaaatagcccattaaaccaatgagatgacaatgtgttaccctcagagaaagcttaatttttggagtaatcaattacacatatcacagaatgtctcatgagaacatttttggctaggtctaccaatttatcatacaaataattatagattttcatttgaggcaaagatgctgattcatcattagtaacatggtcacaaataatcatttattttatttttgttaacatctgtctttcctgtggggaaacttactatatgctctacgtttatttaatttaaaaagtcaattggttattctgaatttttaaaaataacataaaactgttgttctaaatcacagcacctgcttttctttttttagtgaaattatataagcatttagagaatgaaagtgtaagacttgtggtttctggtctctttttactgtttgtaagcctactcgtcatgatattccacaatggtgcacttgccttttaatgctcttatagatatcttcaaacttgcctacatatatacgcctttgttggagtgggctaccatcatcaggaatgatgtcatttgtttcttcaaactcctttattataccaaaaaagtgacagactccacagtctgatcagttttggagaaatatgttaacattttcaattatctcactttctagaatcaaaatagtctgattttttttttcggcactcagtgtaaagaacaaagaactgaatacagtgggcccagaagagaaatatgcctcatcatttttattagctttggaactgtggacaagtcactcaacctagttttctcattttgaaatgggttgttgtgggaattaaaaaaaaaaaaaaaaaaaaaaaaggatacatgggaaaaattctaaaacaccagtgcctgggatgtagcaggcacaaatataagctgcaactgaattgttttcttagagataaaatgggtccacttttcttttctcataatgattccattaataacaaatctttacgtctttcttgttattatgactcttcaatttatttagaaatgtcaattagtgttttcttggaaactacgattaacgtagattggaaattcttaaacttcagtgtgtgtaacagacatccagaaatcttgctgaagatgtagattcctagccctgtctttctaaatttcacattttgagaaacggtgatttagattgttgacttaacactggcctgacttgccctcttacagatatattttgctcaatgtccttcttcctgacttctggtgttctgtaaggattctccccactttctctcaagtacccagtctttgtgtcctttgcctgaattctcggggagagttttgtttgtcaggtacagtcagagaatgaactagccttgaattaaaagcagtgtttccagcccatgcaacatctgacagaatggctggttacatcgaatgcactggaaaagatcatttataaccctgtctcctcagggagaagcaagatatactgcatgagaaagcagagaagcttaaattccagtggtgcttttgttactaactaaatacatgactatgtccaagtttcttactcactttgggtttagttactatatctggtgggggtaattgataatgccttctctggctgaaggcaagatctcagggcttagaccagaatctttattaggctttcttttgattctgagacttatgcttttccataaagggcagtatctcatgtgtaccctgcctgaacataaatttcaccgttacacctttaccacattttcttcagagaatatttatgattcattatttcctaggcacaattctatgtatgaaagattgtgagaagtaccaggcatatagacgactcagcaacagcttaaacctactaccaattcacattaacacttgctattaatttgctcaggattttatttatttgaatctattgggggtggggaggggaggggagtgaaatgatatacatttggaggcaccctcaggtaatcacactatagaaataatgctgctagttaagaggtttgttgcaaagatgtaaagcagcatgtacagaatttgttggacgtctgctttaggtataatttaatatctccacgtatcttttaatagactaataaaaaaccatagttaactacagttttcaaatagcaaataacatataatttagaggtgaggaatacagaagaaggtttttatctatacagtgtgacttacctaggtacgcaatctttaaacaaaatgaagaagaaacatgttttctgttctcagtgctattgtaggttatgggaataaattaatttagaaatttgttctaaaataatgaactaccaaactgataatagcttgcctttatttgttttagtttcatctgtaagtgaataactggaatgaacacatcaacctttggttaaatataaggctttctagcttttgggcttacatgcacctgcttgtgtattcccacctcttttctgatgatctctgaagaggaagaaagagcatgaatgcctaggtatgcacaagcctatttatttctagacctttcctatacacactcttcaacatggcaaatgtttgcaaacaaatacattggttaaaaaaataatattgtaaggtagtttcatttttcatctaaaaatatgtgcacacaggcaatttcgatgaaaatggatttctgcttgaattatctagctaattgcctctattccctgctttgccttgagcatataaaaattatttagggtagacagtgttgaaccttataaatcaattaatcagtattgattaattatttcccctcaactttagtttgcctttaaactaagactaggtttatgctcatccataaaaagtgaaaatttaaacatacacagactgtctgcaatgtcactctggcggtgtatcatggggagatatgtttgaattagatagagaaaatttatatgaaatactctgaggctatgtttcctaaggggaattgctttatccagtataggaaaaccatttttcacataaatttctaaagataaattagaactttaacctgacacctaataggtagaattttagggtttgggggaataataatagttgctagagctattcaatggcaatgtcaatataaaaagcttagttttccacatgagagaagaactgaagtgtagacgagacactctcttacagtaacactgcagaaacttagaagcatgaatattttctagatttccatcttagtcacaattaaggataaagaagaaaaaatatgaaaagtttcttcataatattaaggggcttttattgataaaacaactatttctttcatagtaagttctttttgtcagaggcagaaatagaaatttgattctttagaagacattttgggtttcaaagagaaactctgctactttactgttgaaaatatatagtactctgagaaagctgccttacagcaaggagtttcagaaaagatacaagaaagaaaaccaatgtgagatgctttcattttagagtccctgcttcagtgtttccaacagaaacaagagaaaaagtaataagaaatatttttttctccctcttaagacatacatcactcctgaaattcttagaaaatcaactgaggcaaattaggggtttcaaagctagtcaccttgtaagttgttaggaaaaaaatttgcatttaaattgctctatgtagctcccttgagattttctcctggaatgcttatggctcttttttcattaatacttaaaaaaatacaatttcataaccagtgtattactacatctagttgtgttaagaagagaaacttcatttcataaaatagaaacattcaaagtggtttaggtcaaccaatcactcagtcagaatacttgaattcttcatattgaacacttaatagtgaagttaatctgaaccatatcaactctccatttcttttacagaaactaagtcattaatagctctatcagagagaataaactgtgttcctatatgccctccccataggaacaaagatagtccagaacttcttggaaatttttccttaaaatagtacatatttttatatatcagatttctttttaataggtaattcttaagtcctatttcaataacttgctttacatattcagaaatgtagatataagaaaaatattaaatgtgcaaaatgttctttctatatttacatttaaaaaatacaatgtaataatagctttatacttgtcaaaaagccattggggaaaataagccttcaatgtcagaaaatctggttaaattagagcttttgcttgtggaattgtaaacaaacttttaaaaatgctcagagttttctcaattcttcccatccaagacactcttgaacacatcaagtcctgctttgaagtaaacctgagctgaattaatgctgttcaacacctctgacagggcttcttgaagggtctcatttgatgcaaggggtttgcagtgttcccaagcctctataagtattgaaaaccggcttgtcttttcatcaaggtggtagaggatgtttctataaaaacctggtggtgcctgctttaccagaaagcttttctccatgtcttggagaatgtcattcagcatccggatgcggatgggtgctctctccttgggatcattagcaggtcgcatctcatcagactgaaaaagttcagcactctcccgcaggcgtaacgccatggctaacagttgatgagtgttgggttgatcacctttaaggttgttttgaacttctaaagctatatcaagtgcattaaagggcagaacaggttcgttggcaatttgcaaaatcacttctcctgagagcttagtaatggtttcatgaaggttgaaagagggatccatttcttcaatttttgttgctcgtgtagaaaaacgggcctcggagagaaaacttggaccctctaatgttttgatgtcctcgtaagcaaactgcacgatgggaactccaagatggttgatgaaataatcagcatcaccttgtatctgtatagaactgatattggtttctgggcactgggctcttctggtacagttgaaattatttttctctactaccagttgctgaagagatggtgatgctacaggatacagactagagttcccccttatgggactgtggaggctaatataagccacaacatttttctgaagaaccttcttgaaatcctctccccattcatatgagccaatattgccaaaagctgttcctccccaagaacagaaaacaatagttcggtctggtctccaccctctcttaacttttgacatcaaggcacggataaacgctgtgattattgcagtactactggcccattcttgtccattataactgtgtgcagtgtgatgatggctgccaactatgatataccggtctggagatgtcaagcccattacaaatccaacaacattagtaactgttttcaattttgtgactgtctgaacttgcatgctgacgactcttatttcattatttggaagctctagagagctacacgcttcatttttggttctagcttttggcgaagagatcagttttgcaacgaggggtgcagagatgggctgcactaatagagaggtgaggtttgatcggctttgtctaaaactttcatcgacacttgggtaaccaggcgtagaagggtctcctcctggattcagtgacaccatgaaggtatcatggctaggattcacagtctttggcaaatcacaaggatcgatatacagaagaacacctccaaatccagccttttccaatgaggaaagcttataaagcagtggcaattttcctaatttcaggagtgcgatctgatttgttacgttttttattttcctaatcctttttaaatcatctgccattccataactcacatcgatgacttcagccttgagagttcctttggcagaataggctgcatatgaatagagcaggtcttggctgctatcttttctggcttcttcactgcaaggctggccattaggatgaaagcattgaccactgctgctcagagtcacagtgctgggagaagggcctggcagatcaagcagcacagagtaatttacaaactgtacatcttctaggcccaaagaggtccactgagtcttaatcttctttgaaatttccatgtcatcttcatttttatatagttgtaccaaatttctgaaagacttcttaatatcttctgcctggattgtcttgagaatctcttgatataactgaggatcaactgttcctgaagatggagcatctgaagggcaatttgtatgtacataataacctatcaaaatcccaaaaataaataaaatggtggctgtgcaaagtatttttaagacgtggcaaaagttgcagcgattgctctttggtgcagatcgtgtataatgggtaatgtagtcagattcttcttgaagtctctggaaccttcctttgggtgaagttgctggttgaatggaatcaagattgaggtctatagtctctgaatgccctaggttctgattctcagcaccgtctagctggaattggtcaaaaccagactcctctagttccttctccatgtcccactctaagtcaagggcagtggcttgaaggtcatcattgtctaagtactgtgagtgtcctggagctctttgatctgcatggaccttctgataggccatctttttaccagtcacctctttcattatccatcttctagcaatcacttccatccactgcctcatgccaatgtcgagtgccattgcttcaaatgctgtatacagtttttacttgtttctggaaagagggtaaatccagtccttgatattttaaccaaatgcacaaatattttttcttccacatttaattctacaaatatatttgattgactgtcctacccttatgaatcagtcactatgtcaaaatgaagcggactatacaattagcaagaacctagtctcatatccaaacctgtggacctatgtgttctattgccagtatcagggagaaagagtaaaagcatactccagaccaccaaaactaatagctatcagaatccacttcagaaaatacgttcttatcttaaaaaaggacttttgggggatggcaattccattgcactgatttgtggtttagtgcatcaagcattcctcaggcacattcggtgtgccaggtaaggtggtggcccctgagaaccgtgagataaacaagatgcaagtgcagcctggaagctcatattccagagtttccctttcgccctgcttgtcagttttgcgaaagcattcacagcccctacctcttctgttcacctctcccgttctaggcaatagtcatgggatagctttggcctaaaatggtacattattaatttggggcccatatttcagatgtcacattttaaagatgaagaaacaagggaagaggagggtcaagtcacatgtcacaggtgaagtggccatcaattaacaaacttgatattgttgaagtgttgaatatgactaatatggtgtgtactgaggcccctcactccccactgctcgtcccactattccacagagcgtcatcctgcctggactgcaggactggatattaactcctacctgcatatgtaaaattaactcctacctttcctgctattttaaaaccaaataaattacctcaccattcactaaataaaactcactattttcttatgtttactgcttattcctcagttcccacccccaaagtcaaggagtactattctcttttccttagctaactcatcagacccacatttaataaactggaaaattttttattaaataatgttgagtggaaaaaaggataacaaatttctatgtaaaaagtgatgcagttattttaaaatatatagttatacacacacacaaagactttaagttagcatgccaaaatattagtaatttttgaaaaatctggattgttaatttatgggtaatgtttactttactcttcacacttttttgtttctaaccttctgacgatctctatgtgatatatatatatgtatataaactattaaaataaagttattcttaaagccaatctctaaaaaatcaactacattctgattaaaatctctgatgaacacaatttagataaaattatattttatttgtgctacagtattgcagaaagcattgcaaatacaatacattgcatatgtgattctttataatctctatttgaattatatgacacttgaaggcagaaaatgtatattttaaaaaatatcttctaatacttaacttgtgtagttaaatatattaaccaaatgttacaaatgttacaattgtgcatttcttgcctgggaatcctaaaggaaatcgaaataataaaaacagctgacaattatgacattcatactatgtgctaggttctgttacagatagttttacagcttctatctcatttaatcctcagaatagtccttttagagttcgttttatacatgaagaaactcaaaagtaggaagagatcaaattatctaaagtgccatagctagaacgtgacagagccagtatttgaaaccaagtaggtaaccccacagtctgtgcactaacccaccacacaatccatattttgaatgtttcaacaatattagaaatcttggagtagggataatgatataaagcagggatttgttaatacagattgtttatcatgatttcctcattactagtatctacctcaaaggactattttaacagttaaatatatgatcatgagtttgcacaagtgtctggtgtgtatagagtgctctataattgttttttgagatggaattttgctcttgttgcccaggctggagtgcaatggcactgtcttggctcatggcgacctctgtctcccgggattcaagcaattctcctgtctcagccttccaagtagctgggattacaggcacccgtcaccatgccaggataatttttgtatttttagtagagacggtatatcaccatgttggccaggctggtcttgaactcctgacctcaggtgaggtgatccgcctgcctgggtctcccaaactcctgggattacaggtgtgagccaccgtgcctagcctataaatttagctaatactgttacatgcatattttagctactgtgaattcagttaagatgaaatagctacacaactaaggagatctttttttttttttctgagtatgataaactaaggacatgccttaagtctaagaaaatctgtttactgcaggcttttctgcacaaattttcctttatcatcaaggttgctatagccatccctctttcggattccttttcttctttaaaattagaggctttgctttacactgttatttttaaatggctggatacctgccatagatctaataattggttgtaaaaatccagacaaacatcaatttttaattcttaatttttaatcttgtttgaaacaaacatgtaaactaaaataaaaacttaataaagccaggttcaaatcttgcctgttttagtatataagtcaaatttttattaaattaacttcagatcctattaattatgaaagcaagaggttatatttctaatgaatactaagatcttattagaaattccttctccatcactttgtttttctcttcattagatatacccgcacaaatgacctaaaattcaacccactttgaaaataaattttcaaggcttagtgaaaaaagcctaatttctgtagccactggcctgtttctagagccatcgttgactgatggcttataaagcctttttatacagcactgacattttaaagatactggccagtctgaactttccatctggcgtgcttgatttcctttgtcccactttcccatagtgacttattctgtccttgagctctaaaactactttgatttaatttaggcctgggggtgtgaagacatggtgaaatttatttaaacaagagacgatagtaatgcctccaacagtgcatagtaataggaaagcaaataactgacttcctggcatttatttgtgtaataacttcaccaccaagtgcaaccagagaggtattccagaactttccatgcaattacataaaactagcaagagctagtcagcacttgtaaaatcaagtgggagataaaggaaattattttatctcaggccaaaaaaaaa

SEQ ID NO: 12603 - RNA, 8759 nt, Homo sapiens
  source 1..8759: mol_type = other RNA
gatctcactttgttgcccaggctattttctggatgtctattaaaaaaaaattagtcctgcacagtgttctagaaagggtttttcttttcagaatatccatattctccaagtagcaagttagaatataaggaatatttgccattaaacctttctgttagaaatgtaaacatgaaattgcctaatatagacctatctcagatgctaaatagaattgtttataacacctttggaatataattatgtgagctacacttaaccatctggcattttgcttcctgcggacaatttgcaatagcatagaaaaatattttgtttgtgtatttcttatcaaacagatatgctaaagttctgtttagagagtaatagcattttattctaacttttaaaataaggtagtccatttgcagcagcttgatatataagtaaacaaaaatttttaatattaataaaacactagcacatacactgaaagcatctaagaaattcaaaatataaaacacttaccaagtaatgaccatatgagtggtaacatattgaataaaggccctttgaagaagttggagagttatgattactgagcaggctagataattaaataattacacattttgattgaaaaatatatgtagttcattaaaatagggactctaactccacttctctagctaagcttctattcagatgccacgtttgtactttaattagaacaaaagaccgacattaacttcaatgcaacataataattcataataatgattgtatattaatctcttgagcttgcaggaatatagcacatgacatatggcatgatacaggcacctgtgtgatcctttggggacttaggtggtgcatattaattagcccctggaaaataaaatctgtttccttctgagaaaagctacctcagtgcttattggcttaagccatcaaagaaattagatgaaatactgttaggctgggtctgcactcattaaagctttgtctagatgtaagcactgaatcaactgcctctgagttaagtcttgactgaatggtgcataagaaatcagagtaatcatgcatttctttggccttgatgattggattttggcatttaaaaaatccatcaaaattaccattttggttacagaaaattatgtaattgtataattcaaacaaaataatgtaaccagaaacactaaaatttgaagccacttcattttcctaaatgctgcttgaaactgcctcaatttaacccttttatttgtaaattcagattcaacccgaatatgagattataaatggcttaagaaatatgtcatcttgcaataatcagggtaacaagattcttgacggtcccaggtctgctaaaggcacttcagtgtgtatatctttgtcaggcaatggaacgatattatgaaactaaaactctggctgattaacagatcatttaaattgagactgatagatcttaaaattacttctcagggggaaaaagttacaatgctagagtgtacctagaaaacagaaacttgagtagacatggtaatgaccagaaaaggctatctttatacatttcttttgctacgcttcaaattcatgtcacctaaaagttgtgaagtgcacaaaacaaatctacttaactgaaaattattttcaatgaatgggatgtttagaactctgtgagggtttttaaggtcttttcgaatagcaaattctaatgaggcttttttaagttggcaatttaaactcatacaagaaataaaaactcaccagtgtggctgggcagaatatatatattttctcaaatattgtttgtttgttttttccctgcactgtatccatggtcccatgatgaaactgttatattgctgatatatttattggaatatgtgggccaacttcctttccactcaacatatggattggtagtttaaaataattcctttctattaagcaaatgtgtggctaaggcacatttaaatagcccattaaaccaatgagatgacaatgtgttaccctcagagaaagcttaatttttggagtaatcaattacacatatcacagaatgtctcatgagaacatttttggctaggtctaccaatttatcatacaaataattatagattttcatttgaggcaaagatgctgattcatcattagtaacatggtcacaaataatcatttattttatttttgttaacatctgtctttcctgtggggaaacttactatatgctctacgtttatttaatttaaaaagtcaattggttattctgaatttttaaaaataacataaaactgttgttctaaatcacagcacctgcttttctttttttagtgaaattatataagcatttagagaatgaaagtgtaagacttgtggtttctggtctctttttactgtttgtaagcctactcgtcatgatattccacaatggtgcacttgccttttaatgctcttatagatatcttcaaacttgcctacatatatacgcctttgttggagtgggctaccatcatcaggaatgatgtcatttgtttcttcaaactcctttattataccaaaaaagtgacagactccacagtctgatcagttttggagaaatatgttaacattttcaattatctcactttctagaatcaaaatagtctgattttttttttcggcactcagtgtaaagaacaaagaactgaatacagtgggcccagaagagaaatatgcctcatcatttttattagctttggaactgtggacaagtcactcaacctagttttctcattttgaaatgggttgttgtgggaattaaaaaaaaaaaaaaaaaaaaaaaaggatacatgggaaaaattctaaaacaccagtgcctgggatgtagcaggcacaaatataagctgcaactgaattgttttcttagagataaaatgggtccacttttcttttctcataatgattccattaataacaaatctttacgtctttcttgttattatgactcttcaatttatttagaaatgtcaattagtgttttcttggaaactacgattaacgtagattggaaattcttaaacttcagtgtgtgtaacagacatccagaaatcttgctgaagatgtagattcctagccctgtctttctaaatttcacattttgagaaacggtgatttagattgttgacttaacactggcctgacttgccctcttacagatatattttgctcaatgtccttcttcctgacttctggtgttctgtaaggattctccccactttctctcaagtacccagtctttgtgtcctttgcctgaattctcggggagagttttgtttgtcaggtacagtcagagaatgaactagccttgaattaaaagcagtgtttccagcccatgcaacatctgacagaatggctggttacatcgaatgcactggaaaagatcatttataaccctgtctcctcagggagaagcaagatatactgcatgagaaagcagagaagcttaaattccagtggtgcttttgttactaactaaatacatgactatgtccaagtttcttactcactttgggtttagttactatatctggtgggggtaattgataatgccttctctggctgaaggcaagatctcagggcttagaccagaatctttattaggctttcttttgattctgagacttatgcttttccataaagggcagtatctcatgtgtaccctgcctgaacataaatttcaccgttacacctttaccacattttcttcagagaatatttatgattcattatttcctaggcacaattctatgtatgaaagattgtgagaagtaccaggcatatagacgactcagcaacagcttaaacctactaccaattcacattaacacttgctattaatttgctcaggattttatttatttgaatctattgggggtggggaggggaggggagtgaaatgatatacatttggaggcaccctcaggtaatcacactatagaaataatgctgctagttaagaggtttgttgcaaagatgtaaagcagcatgtacagaatttgttggacgtctgctttaggtataatttaatatctccacgtatcttttaatagactaataaaaaaccatagttaactacagttttcaaatagcaaataacatataatttagaggtgaggaatacagaagaaggtttttatctatacagtgtgacttacctaggtacgcaatctttaaacaaaatgaagaagaaacatgttttctgttctcagtgctattgtaggttatgggaataaattaatttagaaatttgttctaaaataatgaactaccaaactgataatagcttgcctttatttgttttagtttcatctgtaagtgaataactggaatgaacacatcaacctttggttaaatataaggctttctagcttttgggcttacatgcacctgcttgtgtattcccacctcttttctgatgatctctgaagaggaagaaagagcatgaatgcctaggtatgcacaagcctatttatttctagacctttcctatacacactcttcaacatggcaaatgtttgcaaacaaatacattggttaaaaaaataatattgtaaggtagtttcatttttcatctaaaaatatgtgcacacaggcaatttcgatgaaaatggatttctgcttgaattatctagctaattgcctctattccctgctttgccttgagcatataaaaattatttagggtagacagtgttgaaccttataaatcaattaatcagtattgattaattatttcccctcaactttagtttgcctttaaactaagactaggtttatgctcatccataaaaagtgaaaatttaaacatacacagactgtctgcaatgtcactctggcggtgtatcatggggagatatgtttgaattagatagagaaaatttatatgaaatactctgaggctatgtttcctaaggggaattgctttatccagtataggaaaaccatttttcacataaatttctaaagataaattagaactttaacctgacacctaataggtagaattttagggtttgggggaataataatagttgctagagctattcaatggcaatgtcaatataaaaagcttagttttccacatgagagaagaactgaagtgtagacgagacactctcttacagtaacactgcagaaacttagaagcatgaatattttctagatttccatcttagtcacaattaaggataaagaagaaaaaatatgaaaagtttcttcataatattaaggggcttttattgataaaacaactatttctttcatagtaagttctttttgtcagaggcagaaatagaaatttgattctttagaagacattttgggtttcaaagagaaactctgctactttactgttgaaaatatatagtactctgagaaagctgccttacagcaaggagtttcagaaaagatacaagaaagaaaaccaatgtgagatgctttcattttagagtccctgcttcagtgtttccaacagaaacaagagaaaaagtaataagaaatatttttttctccctcttaagacatacatcactcctgaaattcttagaaaatcaactgaggcaaattaggggtttcaaagctagtcaccttgtaagttgttaggaaaaaaatttgcatttaaattgctctatgtagctcccttgagattttctcctggaatgcttatggctcttttttcattaatacttaaaaaaatacaatttcataaccagtgtattactacatctagttgtgttaagaagagaaacttcatttcataaaatagaaacattcaaagtggtttaggtcaaccaatcactcagtcagaatacttgaattcttcatattgaacacttaatagtgaagttaatctgaaccatatcaactctccatttcttttacagaaactaagtcattaatagctctatcagagagaataaactgtgttcctatatgccctccccataggaacaaagatagtccagaacttcttggaaatttttccttaaaatagtacatatttttatatatcagatttctttttaataggtaattcttaagtcctatttcaataacttgctttacatattcagaaatgtagatataagaaaaatattaaatgtgcaaaatgttctttctatatttacatttaaaaaatacaatgtaataatagctttatacttgtcaaaaagccattggggaaaataagccttcaatgtcagaaaatctggttaaattagagcttttgcttgtggaattgtaaacaaacttttaaaaatgctcagagttttctcaattcttcccatccaagacactcttgaacacatcaagtcctgctttgaagtaaacctgagctgaattaatgctgttcaacacctctgacagggcttcttgaagggtctcatttgatgcaaggggtttgcagtgttcccaagcctctataagtattgaaaaccggcttgtcttttcatcaaggtggtagaggatgtttctataaaaacctggtggtgcctgctttaccagaaagcttttctccatgtcttggagaatgtcattcagcatccggatgcggatgggtgctctctccttgggatcattagcaggtcgcatctcatcagactgaaaaagttcagcactctcccgcaggcgtaacgccatggctaacagttgatgagtgttgggttgatcacctttaaggttgttttgaacttctaaagctatatcaagtgcattaaagggcagaacaggttcgttggcaatttgcaaaatcacttctcctgagagcttagtaatggtttcatgaaggttgaaagagggatccatttcttcaatttttgttgctcgtgtagaaaaacgggcctcggagagaaaacttggaccctctaatgttttgatgtcctcgtaagcaaactgcacgatgggaactccaagatggttgatgaaataatcagcatcaccttgtatctgtatagaactgatattggtttctgggcactgggctcttctggtacagttgaaattatttttctctactaccagttgctgaagagatggtgatgctacaggatacagactagagttcccccttatgggactgtggaggctaatataagccacaacatttttctgaagaaccttcttgaaatcctctccccattcatatgagccaatattgccaaaagctgttcctccccaagaacagaaaacaatagttcggtctggtctccaccctctcttaacttttgacatcaaggcacggataaacgctgtgattattgcagtactactggcccattcttgtccattataactgtgtgcagtgtgatgatggctgccaactatgatataccggtctggagatgtcaagcccattacaaatccaacaacattagtaactgttttcaattttgtgactgtctgaacttgcatgctgacgactcttatttcattatttggaagctctagagagctacacgcttcatttttggttctagcttttggcgaagagatcagttttgcaacgaggggtgcagagatgggctgcactaatagagaggtgaggtttgatcggctttgtctaaaactttcatcgacacttgggtaaccaggcgtagaagggtctcctcctggattcagtgacaccatgaaggtatcatggctaggattcacagtctttggcaaatcacaaggatcgatatacagaagaacacctccaaatccagccttttccaatgaggaaagcttataaagcagtggcaattttcctaatttcaggagtgcgatctgatttgttacgttttttattttcctaatcctttttaaatcatctgccattccataactcacatcgatgacttcagccttgagagttcctttggcagaataggctgcatatgaatagagcaggtcttggctgctatcttttctggcttcttcactgcaaggctggccattaggatgaaagcattgaccactgctgctcagagtcacagtgctgggagaagggcctggcagatcaagcagcacagagtaatttacaaactgtacatcttctaggcccaaagaggtccactgagtcttaatcttctttgaaatttccatgtcatcttcatttttatatagttgtaccaaatttctgaaagacttcttaatatcttctgcctggattgtcttgagaatctcttgatataactgaggatcaactgttcctgaagatggagcatctgaagggcaatttgtatgtacataataacctatcaaaatcccaaaaataaataaaatggtggctgtgcaaagtatttttaagacgtggcaaaagttgcagcgattgctctttggtgcagatcgtgtataatgggtaatgtagtcagattcttcttgaagtctctggaaccttcctttgggtgaagttgctggttgaatggaatcaagattgaggtctatagtctctgaatgccctaggttctgattctcagcaccgtctagctggaattggtcaaaaccagactcctctagttccttctccatgtcccactctaagtcaagggcagtggcttgaaggtcatcattgtctaagtactgtgagtgtcctggagctctttgatctgcatggaccttctgataggccatctttttaccttgcaaagacgtgttaggtaaacttgcttcattctctcccattttattatttctttttaaagagggccaagcagtttcaagttgtgtcacttaccctgcaagctttgtgaccttct

SEQ ID NO: 12604 - RNA, 8917 nt, Homo sapiens
  source 1..8917: mol_type = other RNA
gatctcactttgttgcccaggctattttctggatgtctattaaaaaaaaattagtcctgcacagtgttctagaaagggtttttcttttcagaatatccatattctccaagtagcaagttagaatataaggaatatttgccattaaacctttctgttagaaatgtaaacatgaaattgcctaatatagacctatctcagatgctaaatagaattgtttataacacctttggaatataattatgtgagctacacttaaccatctggcattttgcttcctgcggacaatttgcaatagcatagaaaaatattttgtttgtgtatttcttatcaaacagatatgctaaagttctgtttagagagtaatagcattttattctaacttttaaaataaggtagtccatttgcagcagcttgatatataagtaaacaaaaatttttaatattaataaaacactagcacatacactgaaagcatctaagaaattcaaaatataaaacacttaccaagtaatgaccatatgagtggtaacatattgaataaaggccctttgaagaagttggagagttatgattactgagcaggctagataattaaataattacacattttgattgaaaaatatatgtagttcattaaaatagggactctaactccacttctctagctaagcttctattcagatgccacgtttgtactttaattagaacaaaagaccgacattaacttcaatgcaacataataattcataataatgattgtatattaatctcttgagcttgcaggaatatagcacatgacatatggcatgatacaggcacctgtgtgatcctttggggacttaggtggtgcatattaattagcccctggaaaataaaatctgtttccttctgagaaaagctacctcagtgcttattggcttaagccatcaaagaaattagatgaaatactgttaggctgggtctgcactcattaaagctttgtctagatgtaagcactgaatcaactgcctctgagttaagtcttgactgaatggtgcataagaaatcagagtaatcatgcatttctttggccttgatgattggattttggcatttaaaaaatccatcaaaattaccattttggttacagaaaattatgtaattgtataattcaaacaaaataatgtaaccagaaacactaaaatttgaagccacttcattttcctaaatgctgcttgaaactgcctcaatttaacccttttatttgtaaattcagattcaacccgaatatgagattataaatggcttaagaaatatgtcatcttgcaataatcagggtaacaagattcttgacggtcccaggtctgctaaaggcacttcagtgtgtatatctttgtcaggcaatggaacgatattatgaaactaaaactctggctgattaacagatcatttaaattgagactgatagatcttaaaattacttctcagggggaaaaagttacaatgctagagtgtacctagaaaacagaaacttgagtagacatggtaatgaccagaaaaggctatctttatacatttcttttgctacgcttcaaattcatgtcacctaaaagttgtgaagtgcacaaaacaaatctacttaactgaaaattattttcaatgaatgggatgtttagaactctgtgagggtttttaaggtcttttcgaatagcaaattctaatgaggcttttttaagttggcaatttaaactcatacaagaaataaaaactcaccagtgtggctgggcagaatatatatattttctcaaatattgtttgtttgttttttccctgcactgtatccatggtcccatgatgaaactgttatattgctgatatatttattggaatatgtgggccaacttcctttccactcaacatatggattggtagtttaaaataattcctttctattaagcaaatgtgtggctaaggcacatttaaatagcccattaaaccaatgagatgacaatgtgttaccctcagagaaagcttaatttttggagtaatcaattacacatatcacagaatgtctcatgagaacatttttggctaggtctaccaatttatcatacaaataattatagattttcatttgaggcaaagatgctgattcatcattagtaacatggtcacaaataatcatttattttatttttgttaacatctgtctttcctgtggggaaacttactatatgctctacgtttatttaatttaaaaagtcaattggttattctgaatttttaaaaataacataaaactgttgttctaaatcacagcacctgcttttctttttttagtgaaattatataagcatttagagaatgaaagtgtaagacttgtggtttctggtctctttttactgtttgtaagcctactcgtcatgatattccacaatggtgcacttgccttttaatgctcttatagatatcttcaaacttgcctacatatatacgcctttgttggagtgggctaccatcatcaggaatgatgtcatttgtttcttcaaactcctttattataccaaaaaagtgacagactccacagtctgatcagttttggagaaatatgttaacattttcaattatctcactttctagaatcaaaatagtctgattttttttttcggcactcagtgtaaagaacaaagaactgaatacagtgggcccagaagagaaatatgcctcatcatttttattagctttggaactgtggacaagtcactcaacctagttttctcattttgaaatgggttgttgtgggaattaaaaaaaaaaaaaaaaaaaaaaaaggatacatgggaaaaattctaaaacaccagtgcctgggatgtagcaggcacaaatataagctgcaactgaattgttttcttagagataaaatgggtccacttttcttttctcataatgattccattaataacaaatctttacgtctttcttgttattatgactcttcaatttatttagaaatgtcaattagtgttttcttggaaactacgattaacgtagattggaaattcttaaacttcagtgtgtgtaacagacatccagaaatcttgctgaagatgtagattcctagccctgtctttctaaatttcacattttgagaaacggtgatttagattgttgacttaacactggcctgacttgccctcttacagatatattttgctcaatgtccttcttcctgacttctggtgttctgtaaggattctccccactttctctcaagtacccagtctttgtgtcctttgcctgaattctcggggagagttttgtttgtcaggtacagtcagagaatgaactagccttgaattaaaagcagtgtttccagcccatgcaacatctgacagaatggctggttacatcgaatgcactggaaaagatcatttataaccctgtctcctcagggagaagcaagatatactgcatgagaaagcagagaagcttaaattccagtggtgcttttgttactaactaaatacatgactatgtccaagtttcttactcactttgggtttagttactatatctggtgggggtaattgataatgccttctctggctgaaggcaagatctcagggcttagaccagaatctttattaggctttcttttgattctgagacttatgcttttccataaagggcagtatctcatgtgtaccctgcctgaacataaatttcaccgttacacctttaccacattttcttcagagaatatttatgattcattatttcctaggcacaattctatgtatgaaagattgtgagaagtaccaggcatatagacgactcagcaacagcttaaacctactaccaattcacattaacacttgctattaatttgctcaggattttatttatttgaatctattgggggtggggaggggaggggagtgaaatgatatacatttggaggcaccctcaggtaatcacactatagaaataatgctgctagttaagaggtttgttgcaaagatgtaaagcagcatgtacagaatttgttggacgtctgctttaggtataatttaatatctccacgtatcttttaatagactaataaaaaaccatagttaactacagttttcaaatagcaaataacatataatttagaggtgaggaatacagaagaaggtttttatctatacagtgtgacttacctaggtacgcaatctttaaacaaaatgaagaagaaacatgttttctgttctcagtgctattgtaggttatgggaataaattaatttagaaatttgttctaaaataatgaactaccaaactgataatagcttgcctttatttgttttagtttcatctgtaagtgaataactggaatgaacacatcaacctttggttaaatataaggctttctagcttttgggcttacatgcacctgcttgtgtattcccacctcttttctgatgatctctgaagaggaagaaagagcatgaatgcctaggtatgcacaagcctatttatttctagacctttcctatacacactcttcaacatggcaaatgtttgcaaacaaatacattggttaaaaaaataatattgtaaggtagtttcatttttcatctaaaaatatgtgcacacaggcaatttcgatgaaaatggatttctgcttgaattatctagctaattgcctctattccctgctttgccttgagcatataaaaattatttagggtagacagtgttgaaccttataaatcaattaatcagtattgattaattatttcccctcaactttagtttgcctttaaactaagactaggtttatgctcatccataaaaagtgaaaatttaaacatacacagactgtctgcaatgtcactctggcggtgtatcatggggagatatgtttgaattagatagagaaaatttatatgaaatactctgaggctatgtttcctaaggggaattgctttatccagtataggaaaaccatttttcacataaatttctaaagataaattagaactttaacctgacacctaataggtagaattttagggtttgggggaataataatagttgctagagctattcaatggcaatgtcaatataaaaagcttagttttccacatgagagaagaactgaagtgtagacgagacactctcttacagtaacactgcagaaacttagaagcatgaatattttctagatttccatcttagtcacaattaaggataaagaagaaaaaatatgaaaagtttcttcataatattaaggggcttttattgataaaacaactatttctttcatagtaagttctttttgtcagaggcagaaatagaaatttgattctttagaagacattttgggtttcaaagagaaactctgctactttactgttgaaaatatatagtactctgagaaagctgccttacagcaaggagtttcagaaaagatacaagaaagaaaaccaatgtgagatgctttcattttagagtccctgcttcagtgtttccaacagaaacaagagaaaaagtaataagaaatatttttttctccctcttaagacatacatcactcctgaaattcttagaaaatcaactgaggcaaattaggggtttcaaagctagtcaccttgtaagttgttaggaaaaaaatttgcatttaaattgctctatgtagctcccttgagattttctcctggaatgcttatggctcttttttcattaatacttaaaaaaatacaatttcataaccagtgtattactacatctagttgtgttaagaagagaaacttcatttcataaaatagaaacattcaaagtggtttaggtcaaccaatcactcagtcagaatacttgaattcttcatattgaacacttaatagtgaagttaatctgaaccatatcaactctccatttcttttacagaaactaagtcattaatagctctatcagagagaataaactgtgttcctatatgccctccccataggaacaaagatagtccagaacttcttggaaatttttccttaaaatagtacatatttttatatatcagatttctttttaataggtaattcttaagtcctatttcaataacttgctttacatattcagaaatgtagatataagaaaaatattaaatgtgcaaaatgttctttctatatttacatttaaaaaatacaatgtaataatagctttatacttgtcaaaaagccattggggaaaataagccttcaatgtcagaaaatctggttaaattagagcttttgcttgtggaattgtaaacaaacttttaaaaatgctcagagttttctcaattcttcccatccaagacactcttgaacacatcaagtcctgctttgaagtaaacctgagctgaattaatgctgttcaacacctctgacagggcttcttgaagggtctcatttgatgcaaggggtttgcagtgttcccaagcctctataagtattgaaaaccggcttgtcttttcatcaaggtggtagaggatgtttctataaaaacctggtggtgcctgctttaccagaaagcttttctccatgtcttggagaatgtcattcagcatccggatgcggatgggtgctctctccttgggatcattagcaggtcgcatctcatcagactgaaaaagttcagcactctcccgcaggcgtaacgccatggctaacagttgatgagtgttgggttgatcacctttaaggttgttttgaacttctaaagctatatcaagtgcattaaagggcagaacaggttcgttggcaatttgcaaaatcacttctcctgagagcttagtaatggtttcatgaaggttgaaagagggatccatttcttcaatttttgttgctcgtgtagaaaaacgggcctcggagagaaaacttggaccctctaatgttttgatgtcctcgtaagcaaactgcacgatgggaactccaagatggttgatgaaataatcagcatcaccttgtatctgtatagaactgatattggtttctgggcactgggctcttctggtacagttgaaattatttttctctactaccagttgctgaagagatggtgatgctacaggatacagactagagttcccccttatgggactgtggaggctaatataagccacaacatttttctgaagaaccttcttgaaatcctctccccattcatatgagccaatattgccaaaagctgttcctccccaagaacagaaaacaatagttcggtctggtctccaccctctcttaacttttgacatcaaggcacggataaacgctgtgattattgcagtactactggcccattcttgtccattataactgtgtgcagtgtgatgatggctgccaactatgatataccggtctggagatgtcaagcccattacaaatccaacaacattagtaactgttttcaattttgtgactgtctgaacttgcatgctgacgactcttatttcattatttggaagctctagagagctacacgcttcatttttggttctagcttttggcgaagagatcagttttgcaacgaggggtgcagagatgggctgcactaatagagaggtgaggtttgatcggctttgtctaaaactttcatcgacacttgggtaaccaggcgtagaagggtctcctcctggattcagtgacaccatgaaggtatcatggctaggattcacagtctttggcaaatcacaaggatcgatatacagaagaacacctccaaatccagccttttccaatgaggaaagcttataaagcagtggcaattttcctaatttcaggagtgcgatctgatttgttacgttttttattttcctaatcctttttaaatcatctgccattccataactcacatcgatgacttcagccttgagagttcctttggcagaataggctgcatatgaatagagcaggtcttggctgctatcttttctggcttcttcactgcaaggctggccattaggatgaaagcattgaccactgctgctcagagtcacagtgctgggagaagggcctggcagatcaagcagcacagagtaatttacaaactgtacatcttctaggcccaaagaggtccactgagtcttaatcttctttgaaatttccatgtcatcttcatttttatatagttgtaccaaatttctgaaagacttcttaatatcttctgcctggattgtcttgagaatctcttgatataactgaggatcaactgttcctgaagatggagcatctgaagggcaatttgtatgtacataataacctatcaaaatcccaaaaataaataaaatggtggctgtgcaaagtatttttaagacgtggcaaaagttgcagcgattgctctttggtgcagatcgtgtataatgggtaatgtagtcagattcttcttgaagtctctggaaccttcctttgggtgaagttgctggttgaatggaatcaagattgaggtctatagtctctgaatgccctaggttctgattctcagcaccgtctagctggaattggtcaaaaccagactcctctagttccttctccatgtcccactctaagtcaagggcagtggcttgaaggtcatcattgtctaagtactgtgagtgtcctggagctctttgatctgcatggaccttctgataggccatctttttaccttggatttcatgccttgacattttcagcaactttctttgctccaaatttgcttgattttgttttgagattatgagactttccagcaaagattctggaaatttcaactccaagatgtcctgttacctcaatatctaaatgtcaactctgaaattcctcaggtcttcaagtgtttgaacctatcatgaagggctagtgaaagccttcctcatggaacacaggtccaacaggagctccttgcacttctgttaattgaaaatgctattaaagttctgt

SEQ ID NO: 12605 - RNA, 11583 nt, Homo sapiens
  source 1..11583: mol_type = other RNA
gatctcactttgttgcccaggctattttctggatgtctattaaaaaaaaattagtcctgcacagtgttctagaaagggtttttcttttcagaatatccatattctccaagtagcaagttagaatataaggaatatttgccattaaacctttctgttagaaatgtaaacatgaaattgcctaatatagacctatctcagatgctaaatagaattgtttataacacctttggaatataattatgtgagctacacttaaccatctggcattttgcttcctgcggacaatttgcaatagcatagaaaaatattttgtttgtgtatttcttatcaaacagatatgctaaagttctgtttagagagtaatagcattttattctaacttttaaaataaggtagtccatttgcagcagcttgatatataagtaaacaaaaatttttaatattaataaaacactagcacatacactgaaagcatctaagaaattcaaaatataaaacacttaccaagtaatgaccatatgagtggtaacatattgaataaaggccctttgaagaagttggagagttatgattactgagcaggctagataattaaataattacacattttgattgaaaaatatatgtagttcattaaaatagggactctaactccacttctctagctaagcttctattcagatgccacgtttgtactttaattagaacaaaagaccgacattaacttcaatgcaacataataattcataataatgattgtatattaatctcttgagcttgcaggaatatagcacatgacatatggcatgatacaggcacctgtgtgatcctttggggacttaggtggtgcatattaattagcccctggaaaataaaatctgtttccttctgagaaaagctacctcagtgcttattggcttaagccatcaaagaaattagatgaaatactgttaggctgggtctgcactcattaaagctttgtctagatgtaagcactgaatcaactgcctctgagttaagtcttgactgaatggtgcataagaaatcagagtaatcatgcatttctttggccttgatgattggattttggcatttaaaaaatccatcaaaattaccattttggttacagaaaattatgtaattgtataattcaaacaaaataatgtaaccagaaacactaaaatttgaagccacttcattttcctaaatgctgcttgaaactgcctcaatttaacccttttatttgtaaattcagattcaacccgaatatgagattataaatggcttaagaaatatgtcatcttgcaataatcagggtaacaagattcttgacggtcccaggtctgctaaaggcacttcagtgtgtatatctttgtcaggcaatggaacgatattatgaaactaaaactctggctgattaacagatcatttaaattgagactgatagatcttaaaattacttctcagggggaaaaagttacaatgctagagtgtacctagaaaacagaaacttgagtagacatggtaatgaccagaaaaggctatctttatacatttcttttgctacgcttcaaattcatgtcacctaaaagttgtgaagtgcacaaaacaaatctacttaactgaaaattattttcaatgaatgggatgtttagaactctgtgagggtttttaaggtcttttcgaatagcaaattctaatgaggcttttttaagttggcaatttaaactcatacaagaaataaaaactcaccagtgtggctgggcagaatatatatattttctcaaatattgtttgtttgttttttccctgcactgtatccatggtcccatgatgaaactgttatattgctgatatatttattggaatatgtgggccaacttcctttccactcaacatatggattggtagtttaaaataattcctttctattaagcaaatgtgtggctaaggcacatttaaatagcccattaaaccaatgagatgacaatgtgttaccctcagagaaagcttaatttttggagtaatcaattacacatatcacagaatgtctcatgagaacatttttggctaggtctaccaatttatcatacaaataattatagattttcatttgaggcaaagatgctgattcatcattagtaacatggtcacaaataatcatttattttatttttgttaacatctgtctttcctgtggggaaacttactatatgctctacgtttatttaatttaaaaagtcaattggttattctgaatttttaaaaataacataaaactgttgttctaaatcacagcacctgcttttctttttttagtgaaattatataagcatttagagaatgaaagtgtaagacttgtggtttctggtctctttttactgtttgtaagcctactcgtcatgatattccacaatggtgcacttgccttttaatgctcttatagatatcttcaaacttgcctacatatatacgcctttgttggagtgggctaccatcatcaggaatgatgtcatttgtttcttcaaactcctttattataccaaaaaagtgacagactccacagtctgatcagttttggagaaatatgttaacattttcaattatctcactttctagaatcaaaatagtctgattttttttttcggcactcagtgtaaagaacaaagaactgaatacagtgggcccagaagagaaatatgcctcatcatttttattagctttggaactgtggacaagtcactcaacctagttttctcattttgaaatgggttgttgtgggaattaaaaaaaaaaaaaaaaaaaaaaaaggatacatgggaaaaattctaaaacaccagtgcctgggatgtagcaggcacaaatataagctgcaactgaattgttttcttagagataaaatgggtccacttttcttttctcataatgattccattaataacaaatctttacgtctttcttgttattatgactcttcaatttatttagaaatgtcaattagtgttttcttggaaactacgattaacgtagattggaaattcttaaacttcagtgtgtgtaacagacatccagaaatcttgctgaagatgtagattcctagccctgtctttctaaatttcacattttgagaaacggtgatttagattgttgacttaacactggcctgacttgccctcttacagatatattttgctcaatgtccttcttcctgacttctggtgttctgtaaggattctccccactttctctcaagtacccagtctttgtgtcctttgcctgaattctcggggagagttttgtttgtcaggtacagtcagagaatgaactagccttgaattaaaagcagtgtttccagcccatgcaacatctgacagaatggctggttacatcgaatgcactggaaaagatcatttataaccctgtctcctcagggagaagcaagatatactgcatgagaaagcagagaagcttaaattccagtggtgcttttgttactaactaaatacatgactatgtccaagtttcttactcactttgggtttagttactatatctggtgggggtaattgataatgccttctctggctgaaggcaagatctcagggcttagaccagaatctttattaggctttcttttgattctgagacttatgcttttccataaagggcagtatctcatgtgtaccctgcctgaacataaatttcaccgttacacctttaccacattttcttcagagaatatttatgattcattatttcctaggcacaattctatgtatgaaagattgtgagaagtaccaggcatatagacgactcagcaacagcttaaacctactaccaattcacattaacacttgctattaatttgctcaggattttatttatttgaatctattgggggtggggaggggaggggagtgaaatgatatacatttggaggcaccctcaggtaatcacactatagaaataatgctgctagttaagaggtttgttgcaaagatgtaaagcagcatgtacagaatttgttggacgtctgctttaggtataatttaatatctccacgtatcttttaatagactaataaaaaaccatagttaactacagttttcaaatagcaaataacatataatttagaggtgaggaatacagaagaaggtttttatctatacagtgtgacttacctaggtacgcaatctttaaacaaaatgaagaagaaacatgttttctgttctcagtgctattgtaggttatgggaataaattaatttagaaatttgttctaaaataatgaactaccaaactgataatagcttgcctttatttgttttagtttcatctgtaagtgaataactggaatgaacacatcaacctttggttaaatataaggctttctagcttttgggcttacatgcacctgcttgtgtattcccacctcttttctgatgatctctgaagaggaagaaagagcatgaatgcctaggtatgcacaagcctatttatttctagacctttcctatacacactcttcaacatggcaaatgtttgcaaacaaatacattggttaaaaaaataatattgtaaggtagtttcatttttcatctaaaaatatgtgcacacaggcaatttcgatgaaaatggatttctgcttgaattatctagctaattgcctctattccctgctttgccttgagcatataaaaattatttagggtagacagtgttgaaccttataaatcaattaatcagtattgattaattatttcccctcaactttagtttgcctttaaactaagactaggtttatgctcatccataaaaagtgaaaatttaaacatacacagactgtctgcaatgtcactctggcggtgtatcatggggagatatgtttgaattagatagagaaaatttatatgaaatactctgaggctatgtttcctaaggggaattgctttatccagtataggaaaaccatttttcacataaatttctaaagataaattagaactttaacctgacacctaataggtagaattttagggtttgggggaataataatagttgctagagctattcaatggcaatgtcaatataaaaagcttagttttccacatgagagaagaactgaagtgtagacgagacactctcttacagtaacactgcagaaacttagaagcatgaatattttctagatttccatcttagtcacaattaaggataaagaagaaaaaatatgaaaagtttcttcataatattaaggggcttttattgataaaacaactatttctttcatagtaagttctttttgtcagaggcagaaatagaaatttgattctttagaagacattttgggtttcaaagagaaactctgctactttactgttgaaaatatatagtactctgagaaagctgccttacagcaaggagtttcagaaaagatacaagaaagaaaaccaatgtgagatgctttcattttagagtccctgcttcagtgtttccaacagaaacaagagaaaaagtaataagaaatatttttttctccctcttaagacatacatcactcctgaaattcttagaaaatcaactgaggcaaattaggggtttcaaagctagtcaccttgtaagttgttaggaaaaaaatttgcatttaaattgctctatgtagctcccttgagattttctcctggaatgcttatggctcttttttcattaatacttaaaaaaatacaatttcataaccagtgtattactacatctagttgtgttaagaagagaaacttcatttcataaaatagaaacattcaaagtggtttaggtcaaccaatcactcagtcagaatacttgaattcttcatattgaacacttaatagtgaagttaatctgaaccatatcaactctccatttcttttacagaaactaagtcattaatagctctatcagagagaataaactgtgttcctatatgccctccccataggaacaaagatagtccagaacttcttggaaatttttccttaaaatagtacatatttttatatatcagatttctttttaataggtaattcttaagtcctatttcaataacttgctttacatattcagaaatgtagatataagaaaaatattaaatgtgcaaaatgttctttctatatttacatttaaaaaatacaatgtaataatagctttatacttgtcaaaaagccattggggaaaataagccttcaatgtcagaaaatctggttaaattagagcttttgcttgtggaattgtaaacaaacttttaaaaatgctcagagttttctcaattcttcccatccaagacactcttgaacacatcaagtcctgctttgaagtaaacctgagctgaattaatgctgttcaacacctctgacagggcttcttgaagggtctcatttgatgcaaggggtttgcagtgttcccaagcctctataagtattgaaaaccggcttgtcttttcatcaaggtggtagaggatgtttctataaaaacctggtggtgcctgctttaccagaaagcttttctccatgtcttggagaatgtcattcagcatccggatgcggatgggtgctctctccttgggatcattagcaggtcgcatctcatcagactgaaaaagttcagcactctcccgcaggcgtaacgccatggctaacagttgatgagtgttgggttgatcacctttaaggttgttttgaacttctaaagctatatcaagtgcattaaagggcagaacaggttcgttggcaatttgcaaaatcacttctcctgagagcttagtaatggtttcatgaaggttgaaagagggatccatttcttcaatttttgttgctcgtgtagaaaaacgggcctcggagagaaaacttggaccctctaatgttttgatgtcctcgtaagcaaactgcacgatgggaactccaagatggttgatgaaataatcagcatcaccttgtatctgtatagaactgatattggtttctgggcactgggctcttctggtacagttgaaattatttttctctactaccagttgctgaagagatggtgatgctacaggatacagactagagttcccccttatgggactgtggaggctaatataagccacaacatttttctgaagaaccttcttgaaatcctctccccattcatatgagccaatattgccaaaagctgttcctccccaagaacagaaaacaatagttcggtctggtctccaccctctcttaacttttgacatcaaggcacggataaacgctgtgattattgcagtactactggcccattcttgtccattataactgtgtgcagtgtgatgatggctgccaactatgatataccggtctggagatgtcaagcccattacaaatccaacaacattagtaactgttttcaattttgtgactgtctgaacttgcatgctgacgactcttatttcattatttggaagctctagagagctacacgcttcatttttggttctagcttttggcgaagagatcagttttgcaacgaggggtgcagagatgggctgcactaatagagaggtgaggtttgatcggctttgtctaaaactttcatcgacacttgggtaaccaggcgtagaagggtctcctcctggattcagtgacaccatgaaggtatcatggctaggattcacagtctttggcaaatcacaaggatcgatatacagaagaacacctccaaatccagccttttccaatgaggaaagcttataaagcagtggcaattttcctaatttcaggagtgcgatctgatttgttacgttttttattttcctaatcctttttaaatcatctgccattccataactcacatcgatgacttcagccttgagagttcctttggcagaataggctgcatatgaatagagcaggtcttggctgctatcttttctggcttcttcactgcaaggctggccattaggatgaaagcattgaccactgctgctcagagtcacagtgctgggagaagggcctggcagatcaagcagcacagagtaatttacaaactgtacatcttctaggcccaaagaggtccactgagtcttaatcttctttgaaatttccatgtcatcttcatttttatatagttgtaccaaatttctgaaagacttcttaatatcttctgcctggattgtcttgagaatctcttgatataactgaggatcaactgttcctgaagatggagcatctgaagggcaatttgtatgtacataataacctatcaaaatcccaaaaataaataaaatggtggctgtgcaaagtatttttaagacgtggcaaaagttgcagcgattgctctttggtgcagatcgtgtataatgggtaatgtagtcagattcttcttgaagtctctggaaccttcctttgggtgaagttgctggttgaatggaatcaagattgaggtctatagtctctgaatgccctaggttctgattctcagcaccgtctagctggaattggtcaaaaccagactcctctagttccttctccatgtcccactctaagtcaagggcagtggcttgaaggtcatcattgtctaagtactgtgagtgtcctggagctctttgatctgcatggaccttctgataggccatctttttacttcaattgaatgttcctagtgcaactggagggcttctgcaggttacaggagactgacaatctggacccagtcttcatccaggtgcctaatagtcaatgctcatttccaatattaacaggagttttgaagaagtggatttcaaccctcaaggatgacttggagtgtttcaagacttcagaggaagaagtaacttgtttttaatcgttttctttatagaaactaaatttcatttaaattattcttttcttccctcagcctcatgtaaagttcttagtctccaaggcaacaggttgtcaagagtcacattgtatcattgggaaaatgctttgtcctaatgcaaatcaactgcttttgtcccagtccctggaaatctgcatagctagggttgaataaaagacgccctaagacatcaaaagctattttgaacgtccagctgggagatctgagcggcgcgggcgcgggctcgtctgcggtacggctgccgggccaggccggattttcagcagccgtaaagcgggagaagcgggcgcgagccgcggcgcgaaccctcgcccccgagcggcggccccggcgcctccgccgcgagcgtcagccgcttggcaaggaacgggctgggctgagtcataataaaagacgcgtttgtcgagccaagtgggaagaagagccgcgggcagcagtgttcaatggcacaagcctcaaaaattgggaaggattttttttttaatgggcaaaactggaaacttgcccccatggtgcccatcaaaagatatgtttcgtttataatttgcatatattttatacatagtctttgaatctaataaaacttttaaaagaatttttaaagcccattgcttgcagagccaaattcctggttatagcttcgtgacttacgcaagttacttgaattctgtgcttttgtttttcatccatgaaacaggataataaaggtacctccctcaagagagactgcgagagagcttggcatcctgcctgcacttagcactcgctaaatgttaattgttattttaaaataggagggaggagataataaagaggaacttagataacagttttgaatggaagaagatacgaatataaatcaagatttttcttttttcaagtggagtaaattagacaaattaccaatggaagagaagaaagtggagcctggaaggaacaaacggggctaagagaagtagctgaagcgagggaaggaagaagggggaaggaggaaagaagagaggaagaggggtgaataaaagcctccaaggaacaaacgaggctgaaagatgtggctgaaggtagggaaggaagaaaaagggaggaagagaggaagaaataaaaccaaggaagcaagaataaagctaggctgcgtgggaagaggggaggaaggaaggagagagaaattcaactaggctcagtggccaaaatgctgaagtgtgtcctgccgggagggagtggaggaatatgtttactcactatttagaaatgcatgacaaactccatccgctgagggagatttttacaatgtataaacagagaaacaactgtctaaaaatgagccccaaatgaggagcctttgctccagtgaatgagatttggcagttctgcaaaatgaggaaattcttccttgtgcggcatcttgaagggttgagtcatgaaacccacagcaaatattagtgggctggattcctgaaaggcatgccagatggacgcattctggttagttttactgtgtgatgttcccttctgtacttctgtcaattttagaagaaaagagtgtgaataaagatttgagaagtgaacttaaaagccaaactagttacttaatgtacgagtatccacccaccaggagcttacagttacagattccaaaacaagcaaccgtttctcccactttcattttccctcccctttgtttctactttcaccgtattgctttttatccatttttataatatgattttttacagtggaaccgcctacgggaaaggtgcttttaattaatacgaaagaatggaaggaatttcagctaggcctctctaagagggtaaagctttgtgaaagaaaggttttttagctgaagttttaatgagaataagagtagttggcagatgtgaaatcagaagttttttcagacaagaaaataatacgactcgagtgaaagggaatggactagaaatcagaaacagttctattccttaattaccgtaagaaccaaagactggaggaaagtttttcctattctataaagaaaaatgggggcctccctccaccagccagaccttcaaaaaaggaaaaaataaaaattaaaaacctctattagattcttgtaatgatttgctttttcttaggagaacttcttcagggtaaaagacgtgaaagtgcttctttcggcaacttctgacgaaatacttttgtagaagcaaaatttctgaagggataatttttgctcaagcaaaaaactattagtaagataagaatcccttttcctttgtttcaattttgctaagccttcaggctgaggcaaacagattatcattaaacctttattaatgtgaaaccaaaaaaagataaaatcttaaatgctgcgaagcccttaacctaaaaggagcaagaaaacaaaccaaggcccagaaaatagagaaagggattaggaagcctttctaaggggaacctttgaactgtgggctgtaaaatgaatgtctgtgacttgccttaaacaaataggcaatataaactaaagctgggaactaagaagatctcctcagatcagataaaaagcttaccttgtgtgaaacactgtggtcaaagaagaaaattcctttcatcttaagtggagacaaaaacgtgtatcacttgttttgtgtgtgctcataaaacacctccatcacctgaatcccttgggtgcaattttttgatggacttggcattctttaaa

SEQ ID NO: 12606 - RNA, 9501 nt, Homo sapiens
  source 1..9501: mol_type = other RNA
gatctcactttgttgcccaggctattttctggatgtctattaaaaaaaaattagtcctgcacagtgttctagaaagggtttttcttttcagaatatccatattctccaagtagcaagttagaatataaggaatatttgccattaaacctttctgttagaaatgtaaacatgaaattgcctaatatagacctatctcagatgctaaatagaattgtttataacacctttggaatataattatgtgagctacacttaaccatctggcattttgcttcctgcggacaatttgcaatagcatagaaaaatattttgtttgtgtatttcttatcaaacagatatgctaaagttctgtttagagagtaatagcattttattctaacttttaaaataaggtagtccatttgcagcagcttgatatataagtaaacaaaaatttttaatattaataaaacactagcacatacactgaaagcatctaagaaattcaaaatataaaacacttaccaagtaatgaccatatgagtggtaacatattgaataaaggccctttgaagaagttggagagttatgattactgagcaggctagataattaaataattacacattttgattgaaaaatatatgtagttcattaaaatagggactctaactccacttctctagctaagcttctattcagatgccacgtttgtactttaattagaacaaaagaccgacattaacttcaatgcaacataataattcataataatgattgtatattaatctcttgagcttgcaggaatatagcacatgacatatggcatgatacaggcacctgtgtgatcctttggggacttaggtggtgcatattaattagcccctggaaaataaaatctgtttccttctgagaaaagctacctcagtgcttattggcttaagccatcaaagaaattagatgaaatactgttaggctgggtctgcactcattaaagctttgtctagatgtaagcactgaatcaactgcctctgagttaagtcttgactgaatggtgcataagaaatcagagtaatcatgcatttctttggccttgatgattggattttggcatttaaaaaatccatcaaaattaccattttggttacagaaaattatgtaattgtataattcaaacaaaataatgtaaccagaaacactaaaatttgaagccacttcattttcctaaatgctgcttgaaactgcctcaatttaacccttttatttgtaaattcagattcaacccgaatatgagattataaatggcttaagaaatatgtcatcttgcaataatcagggtaacaagattcttgacggtcccaggtctgctaaaggcacttcagtgtgtatatctttgtcaggcaatggaacgatattatgaaactaaaactctggctgattaacagatcatttaaattgagactgatagatcttaaaattacttctcagggggaaaaagttacaatgctagagtgtacctagaaaacagaaacttgagtagacatggtaatgaccagaaaaggctatctttatacatttcttttgctacgcttcaaattcatgtcacctaaaagttgtgaagtgcacaaaacaaatctacttaactgaaaattattttcaatgaatgggatgtttagaactctgtgagggtttttaaggtcttttcgaatagcaaattctaatgaggcttttttaagttggcaatttaaactcatacaagaaataaaaactcaccagtgtggctgggcagaatatatatattttctcaaatattgtttgtttgttttttccctgcactgtatccatggtcccatgatgaaactgttatattgctgatatatttattggaatatgtgggccaacttcctttccactcaacatatggattggtagtttaaaataattcctttctattaagcaaatgtgtggctaaggcacatttaaatagcccattaaaccaatgagatgacaatgtgttaccctcagagaaagcttaatttttggagtaatcaattacacatatcacagaatgtctcatgagaacatttttggctaggtctaccaatttatcatacaaataattatagattttcatttgaggcaaagatgctgattcatcattagtaacatggtcacaaataatcatttattttatttttgttaacatctgtctttcctgtggggaaacttactatatgctctacgtttatttaatttaaaaagtcaattggttattctgaatttttaaaaataacataaaactgttgttctaaatcacagcacctgcttttctttttttagtgaaattatataagcatttagagaatgaaagtgtaagacttgtggtttctggtctctttttactgtttgtaagcctactcgtcatgatattccacaatggtgcacttgccttttaatgctcttatagatatcttcaaacttgcctacatatatacgcctttgttggagtgggctaccatcatcaggaatgatgtcatttgtttcttcaaactcctttattataccaaaaaagtgacagactccacagtctgatcagttttggagaaatatgttaacattttcaattatctcactttctagaatcaaaatagtctgattttttttttcggcactcagtgtaaagaacaaagaactgaatacagtgggcccagaagagaaatatgcctcatcatttttattagctttggaactgtggacaagtcactcaacctagttttctcattttgaaatgggttgttgtgggaattaaaaaaaaaaaaaaaaaaaaaaaaggatacatgggaaaaattctaaaacaccagtgcctgggatgtagcaggcacaaatataagctgcaactgaattgttttcttagagataaaatgggtccacttttcttttctcataatgattccattaataacaaatctttacgtctttcttgttattatgactcttcaatttatttagaaatgtcaattagtgttttcttggaaactacgattaacgtagattggaaattcttaaacttcagtgtgtgtaacagacatccagaaatcttgctgaagatgtagattcctagccctgtctttctaaatttcacattttgagaaacggtgatttagattgttgacttaacactggcctgacttgccctcttacagatatattttgctcaatgtccttcttcctgacttctggtgttctgtaaggattctccccactttctctcaagtacccagtctttgtgtcctttgcctgaattctcggggagagttttgtttgtcaggtacagtcagagaatgaactagccttgaattaaaagcagtgtttccagcccatgcaacatctgacagaatggctggttacatcgaatgcactggaaaagatcatttataaccctgtctcctcagggagaagcaagatatactgcatgagaaagcagagaagcttaaattccagtggtgcttttgttactaactaaatacatgactatgtccaagtttcttactcactttgggtttagttactatatctggtgggggtaattgataatgccttctctggctgaaggcaagatctcagggcttagaccagaatctttattaggctttcttttgattctgagacttatgcttttccataaagggcagtatctcatgtgtaccctgcctgaacataaatttcaccgttacacctttaccacattttcttcagagaatatttatgattcattatttcctaggcacaattctatgtatgaaagattgtgagaagtaccaggcatatagacgactcagcaacagcttaaacctactaccaattcacattaacacttgctattaatttgctcaggattttatttatttgaatctattgggggtggggaggggaggggagtgaaatgatatacatttggaggcaccctcaggtaatcacactatagaaataatgctgctagttaagaggtttgttgcaaagatgtaaagcagcatgtacagaatttgttggacgtctgctttaggtataatttaatatctccacgtatcttttaatagactaataaaaaaccatagttaactacagttttcaaatagcaaataacatataatttagaggtgaggaatacagaagaaggtttttatctatacagtgtgacttacctaggtacgcaatctttaaacaaaatgaagaagaaacatgttttctgttctcagtgctattgtaggttatgggaataaattaatttagaaatttgttctaaaataatgaactaccaaactgataatagcttgcctttatttgttttagtttcatctgtaagtgaataactggaatgaacacatcaacctttggttaaatataaggctttctagcttttgggcttacatgcacctgcttgtgtattcccacctcttttctgatgatctctgaagaggaagaaagagcatgaatgcctaggtatgcacaagcctatttatttctagacctttcctatacacactcttcaacatggcaaatgtttgcaaacaaatacattggttaaaaaaataatattgtaaggtagtttcatttttcatctaaaaatatgtgcacacaggcaatttcgatgaaaatggatttctgcttgaattatctagctaattgcctctattccctgctttgccttgagcatataaaaattatttagggtagacagtgttgaaccttataaatcaattaatcagtattgattaattatttcccctcaactttagtttgcctttaaactaagactaggtttatgctcatccataaaaagtgaaaatttaaacatacacagactgtctgcaatgtcactctggcggtgtatcatggggagatatgtttgaattagatagagaaaatttatatgaaatactctgaggctatgtttcctaaggggaattgctttatccagtataggaaaaccatttttcacataaatttctaaagataaattagaactttaacctgacacctaataggtagaattttagggtttgggggaataataatagttgctagagctattcaatggcaatgtcaatataaaaagcttagttttccacatgagagaagaactgaagtgtagacgagacactctcttacagtaacactgcagaaacttagaagcatgaatattttctagatttccatcttagtcacaattaaggataaagaagaaaaaatatgaaaagtttcttcataatattaaggggcttttattgataaaacaactatttctttcatagtaagttctttttgtcagaggcagaaatagaaatttgattctttagaagacattttgggtttcaaagagaaactctgctactttactgttgaaaatatatagtactctgagaaagctgccttacagcaaggagtttcagaaaagatacaagaaagaaaaccaatgtgagatgctttcattttagagtccctgcttcagtgtttccaacagaaacaagagaaaaagtaataagaaatatttttttctccctcttaagacatacatcactcctgaaattcttagaaaatcaactgaggcaaattaggggtttcaaagctagtcaccttgtaagttgttaggaaaaaaatttgcatttaaattgctctatgtagctcccttgagattttctcctggaatgcttatggctcttttttcattaatacttaaaaaaatacaatttcataaccagtgtattactacatctagttgtgttaagaagagaaacttcatttcataaaatagaaacattcaaagtggtttaggtcaaccaatcactcagtcagaatacttgaattcttcatattgaacacttaatagtgaagttaatctgaaccatatcaactctccatttcttttacagaaactaagtcattaatagctctatcagagagaataaactgtgttcctatatgccctccccataggaacaaagatagtccagaacttcttggaaatttttccttaaaatagtacatatttttatatatcagatttctttttaataggtaattcttaagtcctatttcaataacttgctttacatattcagaaatgtagatataagaaaaatattaaatgtgcaaaatgttctttctatatttacatttaaaaaatacaatgtaataatagctttatacttgtcaaaaagccattggggaaaataagccttcaatgtcagaaaatctggttaaattagagcttttgcttgtggaattgtaaacaaacttttaaaaatgctcagagttttctcaattcttcccatccaagacactcttgaacacatcaagtcctgctttgaagtaaacctgagctgaattaatgctgttcaacacctctgacagggcttcttgaagggtctcatttgatgcaaggggtttgcagtgttcccaagcctctataagtattgaaaaccggcttgtcttttcatcaaggtggtagaggatgtttctataaaaacctggtggtgcctgctttaccagaaagcttttctccatgtcttggagaatgtcattcagcatccggatgcggatgggtgctctctccttgggatcattagcaggtcgcatctcatcagactgaaaaagttcagcactctcccgcaggcgtaacgccatggctaacagttgatgagtgttgggttgatcacctttaaggttgttttgaacttctaaagctatatcaagtgcattaaagggcagaacaggttcgttggcaatttgcaaaatcacttctcctgagagcttagtaatggtttcatgaaggttgaaagagggatccatttcttcaatttttgttgctcgtgtagaaaaacgggcctcggagagaaaacttggaccctctaatgttttgatgtcctcgtaagcaaactgcacgatgggaactccaagatggttgatgaaataatcagcatcaccttgtatctgtatagaactgatattggtttctgggcactgggctcttctggtacagttgaaattatttttctctactaccagttgctgaagagatggtgatgctacaggatacagactagagttcccccttatgggactgtggaggctaatataagccacaacatttttctgaagaaccttcttgaaatcctctccccattcatatgagccaatattgccaaaagctgttcctccccaagaacagaaaacaatagttcggtctggtctccaccctctcttaacttttgacatcaaggcacggataaacgctgtgattattgcagtactactggcccattcttgtccattataactgtgtgcagtgtgatgatggctgccaactatgatataccggtctggagatgtcaagcccattacaaatccaacaacattagtaactgttttcaattttgtgactgtctgaacttgcatgctgacgactcttatttcattatttggaagctctagagagctacacgcttcatttttggttctagcttttggcgaagagatcagttttgcaacgaggggtgcagagatgggctgcactaatagagaggtgaggtttgatcggctttgtctaaaactttcatcgacacttgggtaaccaggcgtagaagggtctcctcctggattcagtgacaccatgaaggtatcatggctaggattcacagtctttggcaaatcacaaggatcgatatacagaagaacacctccaaatccagccttttccaatgaggaaagcttataaagcagtggcaattttcctaatttcaggagtgcgatctgatttgttacgttttttattttcctaatcctttttaaatcatctgccattccataactcacatcgatgacttcagccttgagagttcctttggcagaataggctgcatatgaatagagcaggtcttggctgctatcttttctggcttcttcactgcaaggctggccattaggatgaaagcattgaccactgctgctcagagtcacagtgctgggagaagggcctggcagatcaagcagcacagagtaatttacaaactgtacatcttctaggcccaaagaggtccactgagtcttaatcttctttgaaatttccatgtcatcttcatttttatatagttgtaccaaatttctgaaagacttcttaatatcttctgcctggattgtcttgagaatctcttgatataactgaggatcaactgttcctgaagatggagcatctgaagggcaatttgtatgtacataataacctatcaaaatcccaaaaataaataaaatggtggctgtgcaaagtatttttaagacgtggcaaaagttgcagcgattgctctttggtgcagatcgtgtataatgggtaatgtagtcagattcttcttgaagtctctggaaccttcctttgggtgaagttgctggttgaatggaatcaagattgaggtctatagtctctgaatgccctaggttctgattctcagcaccgtctagctggaattggtcaaaaccagactcctctagttccttctccatgtcccactctaagtcaagggcagtggcttgaaggtcatcattgtctaagtactgtgagtgtcctggagctctttgatctgcatggaccttctgataggccatctttttacttcaattgaatgttcctagtgcaactggagggcttctgcaggttacaggagactgacaatctggacccagtcttcatccaggtgcctaatagtcaatgctcatttccaatattaacaggagttttgaagaagtggatttcaaccctcaaggatgacttggagtgtttcaagacttcagaggaagaagtaacttgtttttaatcgttttctttatagaaactaaatttcatttaaattattcttttcttccctcagcctcatgtaaagttcttagtctccaaggcaacaggttgtcaagagtcacattgtatcattgggaaaatgctttgtcctaatgcaaatcaactgcttttgtcccagtccctggaaatctgcatagctagggttgaataaaagacgccctaagacatcaaaagctattttgaacgtccagctgggagatctgtaaatgaatgatagaaagttcgaaaatcctcacaaaagattgactctcagtgaactttgctcctgataaattctacccacaatgtttattcaaatttagttttaaaaagagaaagcagactttggagagatggcctttacgtggattttatttgctgatgataatgatgatgcacagtgcctcttcacaagattacatgagttaaaaggtaatcccactatcactcttgcaccgatgagtgctctacttgagtgctgatctcaatttttgactccaagctttattacaggaaagcttaaacgaaatgcatttgtgtaagagatgtagatacaaacttcagaatattcatgttaaccatcattgatctctgctttgatggaggtgatttttgatgtaaaataagccgaaattaca

SEQ ID NO: 12607 - RNA, 11519 nt, Homo sapiens
  source 1..11519: mol_type = other RNA
gatctcactttgttgcccaggctattttctggatgtctattaaaaaaaaattagtcctgcacagtgttctagaaagggtttttcttttcagaatatccatattctccaagtagcaagttagaatataaggaatatttgccattaaacctttctgttagaaatgtaaacatgaaattgcctaatatagacctatctcagatgctaaatagaattgtttataacacctttggaatataattatgtgagctacacttaaccatctggcattttgcttcctgcggacaatttgcaatagcatagaaaaatattttgtttgtgtatttcttatcaaacagatatgctaaagttctgtttagagagtaatagcattttattctaacttttaaaataaggtagtccatttgcagcagcttgatatataagtaaacaaaaatttttaatattaataaaacactagcacatacactgaaagcatctaagaaattcaaaatataaaacacttaccaagtaatgaccatatgagtggtaacatattgaataaaggccctttgaagaagttggagagttatgattactgagcaggctagataattaaataattacacattttgattgaaaaatatatgtagttcattaaaatagggactctaactccacttctctagctaagcttctattcagatgccacgtttgtactttaattagaacaaaagaccgacattaacttcaatgcaacataataattcataataatgattgtatattaatctcttgagcttgcaggaatatagcacatgacatatggcatgatacaggcacctgtgtgatcctttggggacttaggtggtgcatattaattagcccctggaaaataaaatctgtttccttctgagaaaagctacctcagtgcttattggcttaagccatcaaagaaattagatgaaatactgttaggctgggtctgcactcattaaagctttgtctagatgtaagcactgaatcaactgcctctgagttaagtcttgactgaatggtgcataagaaatcagagtaatcatgcatttctttggccttgatgattggattttggcatttaaaaaatccatcaaaattaccattttggttacagaaaattatgtaattgtataattcaaacaaaataatgtaaccagaaacactaaaatttgaagccacttcattttcctaaatgctgcttgaaactgcctcaatttaacccttttatttgtaaattcagattcaacccgaatatgagattataaatggcttaagaaatatgtcatcttgcaataatcagggtaacaagattcttgacggtcccaggtctgctaaaggcacttcagtgtgtatatctttgtcaggcaatggaacgatattatgaaactaaaactctggctgattaacagatcatttaaattgagactgatagatcttaaaattacttctcagggggaaaaagttacaatgctagagtgtacctagaaaacagaaacttgagtagacatggtaatgaccagaaaaggctatctttatacatttcttttgctacgcttcaaattcatgtcacctaaaagttgtgaagtgcacaaaacaaatctacttaactgaaaattattttcaatgaatgggatgtttagaactctgtgagggtttttaaggtcttttcgaatagcaaattctaatgaggcttttttaagttggcaatttaaactcatacaagaaataaaaactcaccagtgtggctgggcagaatatatatattttctcaaatattgtttgtttgttttttccctgcactgtatccatggtcccatgatgaaactgttatattgctgatatatttattggaatatgtgggccaacttcctttccactcaacatatggattggtagtttaaaataattcctttctattaagcaaatgtgtggctaaggcacatttaaatagcccattaaaccaatgagatgacaatgtgttaccctcagagaaagcttaatttttggagtaatcaattacacatatcacagaatgtctcatgagaacatttttggctaggtctaccaatttatcatacaaataattatagattttcatttgaggcaaagatgctgattcatcattagtaacatggtcacaaataatcatttattttatttttgttaacatctgtctttcctgtggggaaacttactatatgctctacgtttatttaatttaaaaagtcaattggttattctgaatttttaaaaataacataaaactgttgttctaaatcacagcacctgcttttctttttttagtgaaattatataagcatttagagaatgaaagtgtaagacttgtggtttctggtctctttttactgtttgtaagcctactcgtcatgatattccacaatggtgcacttgccttttaatgctcttatagatatcttcaaacttgcctacatatatacgcctttgttggagtgggctaccatcatcaggaatgatgtcatttgtttcttcaaactcctttattataccaaaaaagtgacagactccacagtctgatcagttttggagaaatatgttaacattttcaattatctcactttctagaatcaaaatagtctgattttttttttcggcactcagtgtaaagaacaaagaactgaatacagtgggcccagaagagaaatatgcctcatcatttttattagctttggaactgtggacaagtcactcaacctagttttctcattttgaaatgggttgttgtgggaattaaaaaaaaaaaaaaaaaaaaaaaaggatacatgggaaaaattctaaaacaccagtgcctgggatgtagcaggcacaaatataagctgcaactgaattgttttcttagagataaaatgggtccacttttcttttctcataatgattccattaataacaaatctttacgtctttcttgttattatgactcttcaatttatttagaaatgtcaattagtgttttcttggaaactacgattaacgtagattggaaattcttaaacttcagtgtgtgtaacagacatccagaaatcttgctgaagatgtagattcctagccctgtctttctaaatttcacattttgagaaacggtgatttagattgttgacttaacactggcctgacttgccctcttacagatatattttgctcaatgtccttcttcctgacttctggtgttctgtaaggattctccccactttctctcaagtacccagtctttgtgtcctttgcctgaattctcggggagagttttgtttgtcaggtacagtcagagaatgaactagccttgaattaaaagcagtgtttccagcccatgcaacatctgacagaatggctggttacatcgaatgcactggaaaagatcatttataaccctgtctcctcagggagaagcaagatatactgcatgagaaagcagagaagcttaaattccagtggtgcttttgttactaactaaatacatgactatgtccaagtttcttactcactttgggtttagttactatatctggtgggggtaattgataatgccttctctggctgaaggcaagatctcagggcttagaccagaatctttattaggctttcttttgattctgagacttatgcttttccataaagggcagtatctcatgtgtaccctgcctgaacataaatttcaccgttacacctttaccacattttcttcagagaatatttatgattcattatttcctaggcacaattctatgtatgaaagattgtgagaagtaccaggcatatagacgactcagcaacagcttaaacctactaccaattcacattaacacttgctattaatttgctcaggattttatttatttgaatctattgggggtggggaggggaggggagtgaaatgatatacatttggaggcaccctcaggtaatcacactatagaaataatgctgctagttaagaggtttgttgcaaagatgtaaagcagcatgtacagaatttgttggacgtctgctttaggtataatttaatatctccacgtatcttttaatagactaataaaaaaccatagttaactacagttttcaaatagcaaataacatataatttagaggtgaggaatacagaagaaggtttttatctatacagtgtgacttacctaggtacgcaatctttaaacaaaatgaagaagaaacatgttttctgttctcagtgctattgtaggttatgggaataaattaatttagaaatttgttctaaaataatgaactaccaaactgataatagcttgcctttatttgttttagtttcatctgtaagtgaataactggaatgaacacatcaacctttggttaaatataaggctttctagcttttgggcttacatgcacctgcttgtgtattcccacctcttttctgatgatctctgaagaggaagaaagagcatgaatgcctaggtatgcacaagcctatttatttctagacctttcctatacacactcttcaacatggcaaatgtttgcaaacaaatacattggttaaaaaaataatattgtaaggtagtttcatttttcatctaaaaatatgtgcacacaggcaatttcgatgaaaatggatttctgcttgaattatctagctaattgcctctattccctgctttgccttgagcatataaaaattatttagggtagacagtgttgaaccttataaatcaattaatcagtattgattaattatttcccctcaactttagtttgcctttaaactaagactaggtttatgctcatccataaaaagtgaaaatttaaacatacacagactgtctgcaatgtcactctggcggtgtatcatggggagatatgtttgaattagatagagaaaatttatatgaaatactctgaggctatgtttcctaaggggaattgctttatccagtataggaaaaccatttttcacataaatttctaaagataaattagaactttaacctgacacctaataggtagaattttagggtttgggggaataataatagttgctagagctattcaatggcaatgtcaatataaaaagcttagttttccacatgagagaagaactgaagtgtagacgagacactctcttacagtaacactgcagaaacttagaagcatgaatattttctagatttccatcttagtcacaattaaggataaagaagaaaaaatatgaaaagtttcttcataatattaaggggcttttattgataaaacaactatttctttcatagtaagttctttttgtcagaggcagaaatagaaatttgattctttagaagacattttgggtttcaaagagaaactctgctactttactgttgaaaatatatagtactctgagaaagctgccttacagcaaggagtttcagaaaagatacaagaaagaaaaccaatgtgagatgctttcattttagagtccctgcttcagtgtttccaacagaaacaagagaaaaagtaataagaaatatttttttctccctcttaagacatacatcactcctgaaattcttagaaaatcaactgaggcaaattaggggtttcaaagctagtcaccttgtaagttgttaggaaaaaaatttgcatttaaattgctctatgtagctcccttgagattttctcctggaatgcttatggctcttttttcattaatacttaaaaaaatacaatttcataaccagtgtattactacatctagttgtgttaagaagagaaacttcatttcataaaatagaaacattcaaagtggtttaggtcaaccaatcactcagtcagaatacttgaattcttcatattgaacacttaatagtgaagttaatctgaaccatatcaactctccatttcttttacagaaactaagtcattaatagctctatcagagagaataaactgtgttcctatatgccctccccataggaacaaagatagtccagaacttcttggaaatttttccttaaaatagtacatatttttatatatcagatttctttttaataggtaattcttaagtcctatttcaataacttgctttacatattcagaaatgtagatataagaaaaatattaaatgtgcaaaatgttctttctatatttacatttaaaaaatacaatgtaataatagctttatacttgtcaaaaagccattggggaaaataagccttcaatgtcagaaaatctggttaaattagagcttttgcttgtggaattgtaaacaaacttttaaaaatgctcagagttttctcaattcttcccatccaagacactcttgaacacatcaagtcctgctttgaagtaaacctgagctgaattaatgctgttcaacacctctgacagggcttcttgaagggtctcatttgatgcaaggggtttgcagtgttcccaagcctctataagtattgaaaaccggcttgtcttttcatcaaggtggtagaggatgtttctataaaaacctggtggtgcctgctttaccagaaagcttttctccatgtcttggagaatgtcattcagcatccggatgcggatgggtgctctctccttgggatcattagcaggtcgcatctcatcagactgaaaaagttcagcactctcccgcaggcgtaacgccatggctaacagttgatgagtgttgggttgatcacctttaaggttgttttgaacttctaaagctatatcaagtgcattaaagggcagaacaggttcgttggcaatttgcaaaatcacttctcctgagagcttagtaatggtttcatgaaggttgaaagagggatccatttcttcaatttttgttgctcgtgtagaaaaacgggcctcggagagaaaacttggaccctctaatgttttgatgtcctcgtaagcaaactgcacgatgggaactccaagatggttgatgaaataatcagcatcaccttgtatctgtatagaactgatattggtttctgggcactgggctcttctggtacagttgaaattatttttctctactaccagttgctgaagagatggtgatgctacaggatacagactagagttcccccttatgggactgtggaggctaatataagccacaacatttttctgaagaaccttcttgaaatcctctccccattcatatgagccaatattgccaaaagctgttcctccccaagaacagaaaacaatagttcggtctggtctccaccctctcttaacttttgacatcaaggcacggataaacgctgtgattattgcagtactactggcccattcttgtccattataactgtgtgcagtgtgatgatggctgccaactatgatataccggtctggagatgtcaagcccattacaaatccaacaacattagtaactgttttcaattttgtgactgtctgaacttgcatgctgacgactcttatttcattatttggaagctctagagagctacacgcttcatttttggttctagcttttggcgaagagatcagttttgcaacgaggggtgcagagatgggctgcactaatagagaggtgaggtttgatcggctttgtctaaaactttcatcgacacttgggtaaccaggcgtagaagggtctcctcctggattcagtgacaccatgaaggtatcatggctaggattcacagtctttggcaaatcacaaggatcgatatacagaagaacacctccaaatccagccttttccaatgaggaaagcttataaagcagtggcaattttcctaatttcaggagtgcgatctgatttgttacgttttttattttcctaatcctttttaaatcatctgccattccataactcacatcgatgacttcagccttgagagttcctttggcagaataggctgcatatgaatagagcaggtcttggctgctatcttttctggcttcttcactgcaaggctggccattaggatgaaagcattgaccactgctgctcagagtcacagtgctgggagaagggcctggcagatcaagcagcacagagtaatttacaaactgtacatcttctaggcccaaagaggtccactgagtcttaatcttctttgaaatttccatgtcatcttcatttttatatagttgtaccaaatttctgaaagacttcttaatatcttctgcctggattgtcttgagaatctcttgatataactgaggatcaactgttcctgaagatggagcatctgaagggcaatttgtatgtacataataacctatcaaaatcccaaaaataaataaaatggtggctgtgcaaagtatttttaagacgtggcaaaagttgcagcgattgctctttggtgcagatcgtgtataatgggtaatgtagtcagattcttcttgaagtctctggaaccttcctttgggtgaagttgctggttgaatggaatcaagattgaggtctatagtctctgaatgccctaggttctgattctcagcaccgtctagctggaattggtcaaaaccagactcctctagttccttctccatgtcccactctaagtcaagggcagtggcttgaaggtcatcattgtctaagtactgtgagtgtcctggagctctttgatctgcatggaccttctgataggccatctttttacttcaattgaatgttcctagtgcaactggagggcttctgcaggttacaggagactgacaatctggacccagtcttcatccaggtgcctaatagtcaatgctcatttccaatattaacaggagttttgaagaagtggatttcaaccctcaaggatgacttggagtgtttcaagacttcagaggaagaagtaacttgtttttaatcgttttctttatagaaactaaatttcatttaaattattcttttcttccctcagcctcctagggttgaataaaagacgccctaagacatcaaaagctattttgaacgtccagctgggagatctgtaaatgaatgatagaaagttcgaaaatcctcacaaaagattgactctcagtgaactttgctcctgataaattctacccacaatgtttattcaaatttagttttaaaaagagaaagcagactttggagagatggcctttacgtggattttatttgctgatgataatgatgatgcacagtgcctcttcacaagattacatgagttaaaaggtaatcccactatcactcttgcaccgatgagtgctctacttgagtgctgatctcaatttttgactccaagctttattacaggaaagcttaaacgaaatgcatttgtgtaagagatgtagatacaaacttcagaatattcatgttaaccatcattgatctctgctttgatggaggtgatttttgatgtaaaataagccgaaattacacaaatattgatttgaaccattattattgcttctaataaaactctcattaatatcttttatatgttgaatgtgtttgtcttgcaggtggtaggtgatggagacagagaaagagagataaagaaatacagagagataccttgttaactcagagatattctaacaaatttttataatgtcatcagagatttttctactctgaataattcaaatcattgagcttttgccttaaaaaaatgcagaatacaaagagatttatcatgtgagtgcaactacttctgctttctcaaaaggttgaccaggcttatggtctttgaaagggcaactgagataaccatgtgctcaatacaattagaatatatctaaactttttaatggtttacctatcttctttttcacacatcaagtcaaatgggtagggaaagaggcttataaacaagagaaaacctaactaactattgaacgaattcaatctggctaaaacatggaatataaagaggaatggcaagagatgaagttaaataggccagataataagggtcttacaggtcatgttaaggtgattaaattttattctgaggttaatgaagaatctttgaaagatgtgaagcagggttgtgatttactttatagtaagatcatttctctatctcaaatgtgataatggacttggaaacactacaagcaaagagatcagttaggaagcagtggcattaatcagctaaaagatgagtttaaaaagttgggaatcaaaaacgtatttaaaattattttatgtaaaaaactatccctaagcctcccattactggacagaaagtattaaacagaaagtattaaagacaaatcgttaaatgatagatcctagagcagtttgcttgtatgtagctgatggccaatgttggtccagacagtattttaaaaaaatttgccaaactttaaaaatcaggaaattacatacacacaggcacatacatccagatttgtagcctctctaggtaacaggaagatgttgtaacctgggccatcattcccacatagtaaaaattgactacagctggttagtgattactcatcttaaatagggcatacattctccagttttttcgagtctgtgcaattttttacttatcagcatggataccatctgttaattaccattgatcacctctacacttcagtcgtctatttcacctacattgcctctacaggcatttgagattgggacttgtgtataaaagaatatgtaaatactttacttaatttttaaaaatgacattctgtcatttaaaatgacattttaaaatgacattctgtttttaggaggaaatcagtgagtgacagaaacacaatatactagagatttctgaaagaaacatgtacaaggacatgagaaagttaacagaataattccttgtatcatcaatgtaggagtaatcacaggtctttatttaacttggtaccacatatcacttggtgtcactttggtctcataacaactcaaatctcttctctccaaaaaagaaaaagtacattttaaaagttcaacttggatttaaaacttctcaaaatgaaccaaatacacaatcagctgttcattagctaactacctcatctagattttcttcagataaaattatttttaaagtgattaaaaaagagaaagaacagaataccaaaagtaaaagcagaaacacttgccattttagattaccttaccagaaaagtattctaatatttgtaccaacactattttcaattaaatctaataagcaaatataattccaaggatatgaaaaggaactgctaagataattgttctgaaagcactccaattaaagatgaaaatacataatgctttattttggcaaaagaatgatccagtggcacagacaagcagtgacttctgtaacatttaataatctgtagacaaaatgcaaatagcaacaacccccaaaacctctataatataaatcttaatcagaatataaaactgtgttaattttctcttatagaaaataaaacaaaaaataatcttcacatcacaacctacgttgtaaccatacgttttactatatgaacatctaattcattttaaaaattaatattaaaagtaattatagcaagggagcttttcgcaattt

SEQ ID NO: 12608 - RNA, 9100 nt, Homo sapiens
  source 1..9100: mol_type = other RNA
gatctcactttgttgcccaggctattttctggatgtctattaaaaaaaaattagtcctgcacagtgttctagaaagggtttttcttttcagaatatccatattctccaagtagcaagttagaatataaggaatatttgccattaaacctttctgttagaaatgtaaacatgaaattgcctaatatagacctatctcagatgctaaatagaattgtttataacacctttggaatataattatgtgagctacacttaaccatctggcattttgcttcctgcggacaatttgcaatagcatagaaaaatattttgtttgtgtatttcttatcaaacagatatgctaaagttctgtttagagagtaatagcattttattctaacttttaaaataaggtagtccatttgcagcagcttgatatataagtaaacaaaaatttttaatattaataaaacactagcacatacactgaaagcatctaagaaattcaaaatataaaacacttaccaagtaatgaccatatgagtggtaacatattgaataaaggccctttgaagaagttggagagttatgattactgagcaggctagataattaaataattacacattttgattgaaaaatatatgtagttcattaaaatagggactctaactccacttctctagctaagcttctattcagatgccacgtttgtactttaattagaacaaaagaccgacattaacttcaatgcaacataataattcataataatgattgtatattaatctcttgagcttgcaggaatatagcacatgacatatggcatgatacaggcacctgtgtgatcctttggggacttaggtggtgcatattaattagcccctggaaaataaaatctgtttccttctgagaaaagctacctcagtgcttattggcttaagccatcaaagaaattagatgaaatactgttaggctgggtctgcactcattaaagctttgtctagatgtaagcactgaatcaactgcctctgagttaagtcttgactgaatggtgcataagaaatcagagtaatcatgcatttctttggccttgatgattggattttggcatttaaaaaatccatcaaaattaccattttggttacagaaaattatgtaattgtataattcaaacaaaataatgtaaccagaaacactaaaatttgaagccacttcattttcctaaatgctgcttgaaactgcctcaatttaacccttttatttgtaaattcagattcaacccgaatatgagattataaatggcttaagaaatatgtcatcttgcaataatcagggtaacaagattcttgacggtcccaggtctgctaaaggcacttcagtgtgtatatctttgtcaggcaatggaacgatattatgaaactaaaactctggctgattaacagatcatttaaattgagactgatagatcttaaaattacttctcagggggaaaaagttacaatgctagagtgtacctagaaaacagaaacttgagtagacatggtaatgaccagaaaaggctatctttatacatttcttttgctacgcttcaaattcatgtcacctaaaagttgtgaagtgcacaaaacaaatctacttaactgaaaattattttcaatgaatgggatgtttagaactctgtgagggtttttaaggtcttttcgaatagcaaattctaatgaggcttttttaagttggcaatttaaactcatacaagaaataaaaactcaccagtgtggctgggcagaatatatatattttctcaaatattgtttgtttgttttttccctgcactgtatccatggtcccatgatgaaactgttatattgctgatatatttattggaatatgtgggccaacttcctttccactcaacatatggattggtagtttaaaataattcctttctattaagcaaatgtgtggctaaggcacatttaaatagcccattaaaccaatgagatgacaatgtgttaccctcagagaaagcttaatttttggagtaatcaattacacatatcacagaatgtctcatgagaacatttttggctaggtctaccaatttatcatacaaataattatagattttcatttgaggcaaagatgctgattcatcattagtaacatggtcacaaataatcatttattttatttttgttaacatctgtctttcctgtggggaaacttactatatgctctacgtttatttaatttaaaaagtcaattggttattctgaatttttaaaaataacataaaactgttgttctaaatcacagcacctgcttttctttttttagtgaaattatataagcatttagagaatgaaagtgtaagacttgtggtttctggtctctttttactgtttgtaagcctactcgtcatgatattccacaatggtgcacttgccttttaatgctcttatagatatcttcaaacttgcctacatatatacgcctttgttggagtgggctaccatcatcaggaatgatgtcatttgtttcttcaaactcctttattataccaaaaaagtgacagactccacagtctgatcagttttggagaaatatgttaacattttcaattatctcactttctagaatcaaaatagtctgattttttttttcggcactcagtgtaaagaacaaagaactgaatacagtgggcccagaagagaaatatgcctcatcatttttattagctttggaactgtggacaagtcactcaacctagttttctcattttgaaatgggttgttgtgggaattaaaaaaaaaaaaaaaaaaaaaaaaggatacatgggaaaaattctaaaacaccagtgcctgggatgtagcaggcacaaatataagctgcaactgaattgttttcttagagataaaatgggtccacttttcttttctcataatgattccattaataacaaatctttacgtctttcttgttattatgactcttcaatttatttagaaatgtcaattagtgttttcttggaaactacgattaacgtagattggaaattcttaaacttcagtgtgtgtaacagacatccagaaatcttgctgaagatgtagattcctagccctgtctttctaaatttcacattttgagaaacggtgatttagattgttgacttaacactggcctgacttgccctcttacagatatattttgctcaatgtccttcttcctgacttctggtgttctgtaaggattctccccactttctctcaagtacccagtctttgtgtcctttgcctgaattctcggggagagttttgtttgtcaggtacagtcagagaatgaactagccttgaattaaaagcagtgtttccagcccatgcaacatctgacagaatggctggttacatcgaatgcactggaaaagatcatttataaccctgtctcctcagggagaagcaagatatactgcatgagaaagcagagaagcttaaattccagtggtgcttttgttactaactaaatacatgactatgtccaagtttcttactcactttgggtttagttactatatctggtgggggtaattgataatgccttctctggctgaaggcaagatctcagggcttagaccagaatctttattaggctttcttttgattctgagacttatgcttttccataaagggcagtatctcatgtgtaccctgcctgaacataaatttcaccgttacacctttaccacattttcttcagagaatatttatgattcattatttcctaggcacaattctatgtatgaaagattgtgagaagtaccaggcatatagacgactcagcaacagcttaaacctactaccaattcacattaacacttgctattaatttgctcaggattttatttatttgaatctattgggggtggggaggggaggggagtgaaatgatatacatttggaggcaccctcaggtaatcacactatagaaataatgctgctagttaagaggtttgttgcaaagatgtaaagcagcatgtacagaatttgttggacgtctgctttaggtataatttaatatctccacgtatcttttaatagactaataaaaaaccatagttaactacagttttcaaatagcaaataacatataatttagaggtgaggaatacagaagaaggtttttatctatacagtgtgacttacctaggtacgcaatctttaaacaaaatgaagaagaaacatgttttctgttctcagtgctattgtaggttatgggaataaattaatttagaaatttgttctaaaataatgaactaccaaactgataatagcttgcctttatttgttttagtttcatctgtaagtgaataactggaatgaacacatcaacctttggttaaatataaggctttctagcttttgggcttacatgcacctgcttgtgtattcccacctcttttctgatgatctctgaagaggaagaaagagcatgaatgcctaggtatgcacaagcctatttatttctagacctttcctatacacactcttcaacatggcaaatgtttgcaaacaaatacattggttaaaaaaataatattgtaaggtagtttcatttttcatctaaaaatatgtgcacacaggcaatttcgatgaaaatggatttctgcttgaattatctagctaattgcctctattccctgctttgccttgagcatataaaaattatttagggtagacagtgttgaaccttataaatcaattaatcagtattgattaattatttcccctcaactttagtttgcctttaaactaagactaggtttatgctcatccataaaaagtgaaaatttaaacatacacagactgtctgcaatgtcactctggcggtgtatcatggggagatatgtttgaattagatagagaaaatttatatgaaatactctgaggctatgtttcctaaggggaattgctttatccagtataggaaaaccatttttcacataaatttctaaagataaattagaactttaacctgacacctaataggtagaattttagggtttgggggaataataatagttgctagagctattcaatggcaatgtcaatataaaaagcttagttttccacatgagagaagaactgaagtgtagacgagacactctcttacagtaacactgcagaaacttagaagcatgaatattttctagatttccatcttagtcacaattaaggataaagaagaaaaaatatgaaaagtttcttcataatattaaggggcttttattgataaaacaactatttctttcatagtaagttctttttgtcagaggcagaaatagaaatttgattctttagaagacattttgggtttcaaagagaaactctgctactttactgttgaaaatatatagtactctgagaaagctgccttacagcaaggagtttcagaaaagatacaagaaagaaaaccaatgtgagatgctttcattttagagtccctgcttcagtgtttccaacagaaacaagagaaaaagtaataagaaatatttttttctccctcttaagacatacatcactcctgaaattcttagaaaatcaactgaggcaaattaggggtttcaaagctagtcaccttgtaagttgttaggaaaaaaatttgcatttaaattgctctatgtagctcccttgagattttctcctggaatgcttatggctcttttttcattaatacttaaaaaaatacaatttcataaccagtgtattactacatctagttgtgttaagaagagaaacttcatttcataaaatagaaacattcaaagtggtttaggtcaaccaatcactcagtcagaatacttgaattcttcatattgaacacttaatagtgaagttaatctgaaccatatcaactctccatttcttttacagaaactaagtcattaatagctctatcagagagaataaactgtgttcctatatgccctccccataggaacaaagatagtccagaacttcttggaaatttttccttaaaatagtacatatttttatatatcagatttctttttaataggtaattcttaagtcctatttcaataacttgctttacatattcagaaatgtagatataagaaaaatattaaatgtgcaaaatgttctttctatatttacatttaaaaaatacaatgtaataatagctttatacttgtcaaaaagccattggggaaaataagccttcaatgtcagaaaatctggttaaattagagcttttgcttgtggaattgtaaacaaacttttaaaaatgctcagagttttctcaattcttcccatccaagacactcttgaacacatcaagtcctgctttgaagtaaacctgagctgaattaatgctgttcaacacctctgacagggcttcttgaagggtctcatttgatgcaaggggtttgcagtgttcccaagcctctataagtattgaaaaccggcttgtcttttcatcaaggtggtagaggatgtttctataaaaacctggtggtgcctgctttaccagaaagcttttctccatgtcttggagaatgtcattcagcatccggatgcggatgggtgctctctccttgggatcattagcaggtcgcatctcatcagactgaaaaagttcagcactctcccgcaggcgtaacgccatggctaacagttgatgagtgttgggttgatcacctttaaggttgttttgaacttctaaagctatatcaagtgcattaaagggcagaacaggttcgttggcaatttgcaaaatcacttctcctgagagcttagtaatggtttcatgaaggttgaaagagggatccatttcttcaatttttgttgctcgtgtagaaaaacgggcctcggagagaaaacttggaccctctaatgttttgatgtcctcgtaagcaaactgcacgatgggaactccaagatggttgatgaaataatcagcatcaccttgtatctgtatagaactgatattggtttctgggcactgggctcttctggtacagttgaaattatttttctctactaccagttgctgaagagatggtgatgctacaggatacagactagagttcccccttatgggactgtggaggctaatataagccacaacatttttctgaagaaccttcttgaaatcctctccccattcatatgagccaatattgccaaaagctgttcctccccaagaacagaaaacaatagttcggtctggtctccaccctctcttaacttttgacatcaaggcacggataaacgctgtgattattgcagtactactggcccattcttgtccattataactgtgtgcagtgtgatgatggctgccaactatgatataccggtctggagatgtcaagcccattacaaatccaacaacattagtaactgttttcaattttgtgactgtctgaacttgcatgctgacgactcttatttcattatttggaagctctagagagctacacgcttcatttttggttctagcttttggcgaagagatcagttttgcaacgaggggtgcagagatgggctgcactaatagagaggtgaggtttgatcggctttgtctaaaactttcatcgacacttgggtaaccaggcgtagaagggtctcctcctggattcagtgacaccatgaaggtatcatggctaggattcacagtctttggcaaatcacaaggatcgatatacagaagaacacctccaaatccagccttttccaatgaggaaagcttataaagcagtggcaattttcctaatttcaggagtgcgatctgatttgttacgttttttattttcctaatcctttttaaatcatctgccattccataactcacatcgatgacttcagccttgagagttcctttggcagaataggctgcatatgaatagagcaggtcttggctgctatcttttctggcttcttcactgcaaggctggccattaggatgaaagcattgaccactgctgctcagagtcacagtgctgggagaagggcctggcagatcaagcagcacagagtaatttacaaactgtacatcttctaggcccaaagaggtccactgagtcttaatcttctttgaaatttccatgtcatcttcatttttatatagttgtaccaaatttctgaaagacttcttaatatcttctgcctggattgtcttgagaatctcttgatataactgaggatcaactgttcctgaagatggagcatctgaagggcaatttgtatgtacataataacctatcaaaatcccaaaaataaataaaatggtggctgtgcaaagtatttttaagacgtggcaaaagttgcagcgattgctctttggtgcagatcgtgtataatgggtaatgtagtcagattcttcttgaagtctctggaaccttcctttgggtgaagttgctggttgaatggaatcaagattgaggtctatagtctctgaatgccctaggttctgattctcagcaccgtctagctggaattggtcaaaaccagactcctctagttccttctccatgtcccactctaagtcaagggcagtggcttgaaggtcatcattgtctaagtactgtgagtgtcctggagctctttgatctgcatggaccttctgataggccatctttttacttcaattgaatgttcctagtgcaactggagggcttctgcaggttacaggagactgacaatctggacccagtcttcatccaggtgcctaatagtcaatgctcatttccaatattaacaggagttttgaagaagtggatttcaaccctcaaggatgacttggagtgtttcaagacttcagaggaagaagtaacttgtttttaatcgttttctttatagaaactaaatttcatttaaattattcttttcttccctcagcctcctagggttgaataaaagacgccctaagacatcaaaagctattttgaacgtccagctgggagatctttattacaggaaagcttaaacgaaatgcatttgtgtaagagatgtagatacaaacttcagaatattcatgttaaccatcattgatctctgctttgatggaggtgatttttgatgtaaaataagccgaaattaca

SEQ ID NO: 12609 - RNA, 11400 nt, Homo sapiens
  source 1..11400: mol_type = other RNA
gatctcactttgttgcccaggctattttctggatgtctattaaaaaaaaattagtcctgcacagtgttctagaaagggtttttcttttcagaatatccatattctccaagtagcaagttagaatataaggaatatttgccattaaacctttctgttagaaatgtaaacatgaaattgcctaatatagacctatctcagatgctaaatagaattgtttataacacctttggaatataattatgtgagctacacttaaccatctggcattttgcttcctgcggacaatttgcaatagcatagaaaaatattttgtttgtgtatttcttatcaaacagatatgctaaagttctgtttagagagtaatagcattttattctaacttttaaaataaggtagtccatttgcagcagcttgatatataagtaaacaaaaatttttaatattaataaaacactagcacatacactgaaagcatctaagaaattcaaaatataaaacacttaccaagtaatgaccatatgagtggtaacatattgaataaaggccctttgaagaagttggagagttatgattactgagcaggctagataattaaataattacacattttgattgaaaaatatatgtagttcattaaaatagggactctaactccacttctctagctaagcttctattcagatgccacgtttgtactttaattagaacaaaagaccgacattaacttcaatgcaacataataattcataataatgattgtatattaatctcttgagcttgcaggaatatagcacatgacatatggcatgatacaggcacctgtgtgatcctttggggacttaggtggtgcatattaattagcccctggaaaataaaatctgtttccttctgagaaaagctacctcagtgcttattggcttaagccatcaaagaaattagatgaaatactgttaggctgggtctgcactcattaaagctttgtctagatgtaagcactgaatcaactgcctctgagttaagtcttgactgaatggtgcataagaaatcagagtaatcatgcatttctttggccttgatgattggattttggcatttaaaaaatccatcaaaattaccattttggttacagaaaattatgtaattgtataattcaaacaaaataatgtaaccagaaacactaaaatttgaagccacttcattttcctaaatgctgcttgaaactgcctcaatttaacccttttatttgtaaattcagattcaacccgaatatgagattataaatggcttaagaaatatgtcatcttgcaataatcagggtaacaagattcttgacggtcccaggtctgctaaaggcacttcagtgtgtatatctttgtcaggcaatggaacgatattatgaaactaaaactctggctgattaacagatcatttaaattgagactgatagatcttaaaattacttctcagggggaaaaagttacaatgctagagtgtacctagaaaacagaaacttgagtagacatggtaatgaccagaaaaggctatctttatacatttcttttgctacgcttcaaattcatgtcacctaaaagttgtgaagtgcacaaaacaaatctacttaactgaaaattattttcaatgaatgggatgtttagaactctgtgagggtttttaaggtcttttcgaatagcaaattctaatgaggcttttttaagttggcaatttaaactcatacaagaaataaaaactcaccagtgtggctgggcagaatatatatattttctcaaatattgtttgtttgttttttccctgcactgtatccatggtcccatgatgaaactgttatattgctgatatatttattggaatatgtgggccaacttcctttccactcaacatatggattggtagtttaaaataattcctttctattaagcaaatgtgtggctaaggcacatttaaatagcccattaaaccaatgagatgacaatgtgttaccctcagagaaagcttaatttttggagtaatcaattacacatatcacagaatgtctcatgagaacatttttggctaggtctaccaatttatcatacaaataattatagattttcatttgaggcaaagatgctgattcatcattagtaacatggtcacaaataatcatttattttatttttgttaacatctgtctttcctgtggggaaacttactatatgctctacgtttatttaatttaaaaagtcaattggttattctgaatttttaaaaataacataaaactgttgttctaaatcacagcacctgcttttctttttttagtgaaattatataagcatttagagaatgaaagtgtaagacttgtggtttctggtctctttttactgtttgtaagcctactcgtcatgatattccacaatggtgcacttgccttttaatgctcttatagatatcttcaaacttgcctacatatatacgcctttgttggagtgggctaccatcatcaggaatgatgtcatttgtttcttcaaactcctttattataccaaaaaagtgacagactccacagtctgatcagttttggagaaatatgttaacattttcaattatctcactttctagaatcaaaatagtctgattttttttttcggcactcagtgtaaagaacaaagaactgaatacagtgggcccagaagagaaatatgcctcatcatttttattagctttggaactgtggacaagtcactcaacctagttttctcattttgaaatgggttgttgtgggaattaaaaaaaaaaaaaaaaaaaaaaaaggatacatgggaaaaattctaaaacaccagtgcctgggatgtagcaggcacaaatataagctgcaactgaattgttttcttagagataaaatgggtccacttttcttttctcataatgattccattaataacaaatctttacgtctttcttgttattatgactcttcaatttatttagaaatgtcaattagtgttttcttggaaactacgattaacgtagattggaaattcttaaacttcagtgtgtgtaacagacatccagaaatcttgctgaagatgtagattcctagccctgtctttctaaatttcacattttgagaaacggtgatttagattgttgacttaacactggcctgacttgccctcttacagatatattttgctcaatgtccttcttcctgacttctggtgttctgtaaggattctccccactttctctcaagtacccagtctttgtgtcctttgcctgaattctcggggagagttttgtttgtcaggtacagtcagagaatgaactagccttgaattaaaagcagtgtttccagcccatgcaacatctgacagaatggctggttacatcgaatgcactggaaaagatcatttataaccctgtctcctcagggagaagcaagatatactgcatgagaaagcagagaagcttaaattccagtggtgcttttgttactaactaaatacatgactatgtccaagtttcttactcactttgggtttagttactatatctggtgggggtaattgataatgccttctctggctgaaggcaagatctcagggcttagaccagaatctttattaggctttcttttgattctgagacttatgcttttccataaagggcagtatctcatgtgtaccctgcctgaacataaatttcaccgttacacctttaccacattttcttcagagaatatttatgattcattatttcctaggcacaattctatgtatgaaagattgtgagaagtaccaggcatatagacgactcagcaacagcttaaacctactaccaattcacattaacacttgctattaatttgctcaggattttatttatttgaatctattgggggtggggaggggaggggagtgaaatgatatacatttggaggcaccctcaggtaatcacactatagaaataatgctgctagttaagaggtttgttgcaaagatgtaaagcagcatgtacagaatttgttggacgtctgctttaggtataatttaatatctccacgtatcttttaatagactaataaaaaaccatagttaactacagttttcaaatagcaaataacatataatttagaggtgaggaatacagaagaaggtttttatctatacagtgtgacttacctaggtacgcaatctttaaacaaaatgaagaagaaacatgttttctgttctcagtgctattgtaggttatgggaataaattaatttagaaatttgttctaaaataatgaactaccaaactgataatagcttgcctttatttgttttagtttcatctgtaagtgaataactggaatgaacacatcaacctttggttaaatataaggctttctagcttttgggcttacatgcacctgcttgtgtattcccacctcttttctgatgatctctgaagaggaagaaagagcatgaatgcctaggtatgcacaagcctatttatttctagacctttcctatacacactcttcaacatggcaaatgtttgcaaacaaatacattggttaaaaaaataatattgtaaggtagtttcatttttcatctaaaaatatgtgcacacaggcaatttcgatgaaaatggatttctgcttgaattatctagctaattgcctctattccctgctttgccttgagcatataaaaattatttagggtagacagtgttgaaccttataaatcaattaatcagtattgattaattatttcccctcaactttagtttgcctttaaactaagactaggtttatgctcatccataaaaagtgaaaatttaaacatacacagactgtctgcaatgtcactctggcggtgtatcatggggagatatgtttgaattagatagagaaaatttatatgaaatactctgaggctatgtttcctaaggggaattgctttatccagtataggaaaaccatttttcacataaatttctaaagataaattagaactttaacctgacacctaataggtagaattttagggtttgggggaataataatagttgctagagctattcaatggcaatgtcaatataaaaagcttagttttccacatgagagaagaactgaagtgtagacgagacactctcttacagtaacactgcagaaacttagaagcatgaatattttctagatttccatcttagtcacaattaaggataaagaagaaaaaatatgaaaagtttcttcataatattaaggggcttttattgataaaacaactatttctttcatagtaagttctttttgtcagaggcagaaatagaaatttgattctttagaagacattttgggtttcaaagagaaactctgctactttactgttgaaaatatatagtactctgagaaagctgccttacagcaaggagtttcagaaaagatacaagaaagaaaaccaatgtgagatgctttcattttagagtccctgcttcagtgtttccaacagaaacaagagaaaaagtaataagaaatatttttttctccctcttaagacatacatcactcctgaaattcttagaaaatcaactgaggcaaattaggggtttcaaagctagtcaccttgtaagttgttaggaaaaaaatttgcatttaaattgctctatgtagctcccttgagattttctcctggaatgcttatggctcttttttcattaatacttaaaaaaatacaatttcataaccagtgtattactacatctagttgtgttaagaagagaaacttcatttcataaaatagaaacattcaaagtggtttaggtcaaccaatcactcagtcagaatacttgaattcttcatattgaacacttaatagtgaagttaatctgaaccatatcaactctccatttcttttacagaaactaagtcattaatagctctatcagagagaataaactgtgttcctatatgccctccccataggaacaaagatagtccagaacttcttggaaatttttccttaaaatagtacatatttttatatatcagatttctttttaataggtaattcttaagtcctatttcaataacttgctttacatattcagaaatgtagatataagaaaaatattaaatgtgcaaaatgttctttctatatttacatttaaaaaatacaatgtaataatagctttatacttgtcaaaaagccattggggaaaataagccttcaatgtcagaaaatctggttaaattagagcttttgcttgtggaattgtaaacaaacttttaaaaatgctcagagttttctcaattcttcccatccaagacactcttgaacacatcaagtcctgctttgaagtaaacctgagctgaattaatgctgttcaacacctctgacagggcttcttgaagggtctcatttgatgcaaggggtttgcagtgttcccaagcctctataagtattgaaaaccggcttgtcttttcatcaaggtggtagaggatgtttctataaaaacctggtggtgcctgctttaccagaaagcttttctccatgtcttggagaatgtcattcagcatccggatgcggatgggtgctctctccttgggatcattagcaggtcgcatctcatcagactgaaaaagttcagcactctcccgcaggcgtaacgccatggctaacagttgatgagtgttgggttgatcacctttaaggttgttttgaacttctaaagctatatcaagtgcattaaagggcagaacaggttcgttggcaatttgcaaaatcacttctcctgagagcttagtaatggtttcatgaaggttgaaagagggatccatttcttcaatttttgttgctcgtgtagaaaaacgggcctcggagagaaaacttggaccctctaatgttttgatgtcctcgtaagcaaactgcacgatgggaactccaagatggttgatgaaataatcagcatcaccttgtatctgtatagaactgatattggtttctgggcactgggctcttctggtacagttgaaattatttttctctactaccagttgctgaagagatggtgatgctacaggatacagactagagttcccccttatgggactgtggaggctaatataagccacaacatttttctgaagaaccttcttgaaatcctctccccattcatatgagccaatattgccaaaagctgttcctccccaagaacagaaaacaatagttcggtctggtctccaccctctcttaacttttgacatcaaggcacggataaacgctgtgattattgcagtactactggcccattcttgtccattataactgtgtgcagtgtgatgatggctgccaactatgatataccggtctggagatgtcaagcccattacaaatccaacaacattagtaactgttttcaattttgtgactgtctgaacttgcatgctgacgactcttatttcattatttggaagctctagagagctacacgcttcatttttggttctagcttttggcgaagagatcagttttgcaacgaggggtgcagagatgggctgcactaatagagaggtgaggtttgatcggctttgtctaaaactttcatcgacacttgggtaaccaggcgtagaagggtctcctcctggattcagtgacaccatgaaggtatcatggctaggattcacagtctttggcaaatcacaaggatcgatatacagaagaacacctccaaatccagccttttccaatgaggaaagcttataaagcagtggcaattttcctaatttcaggagtgcgatctgatttgttacgttttttattttcctaatcctttttaaatcatctgccattccataactcacatcgatgacttcagccttgagagttcctttggcagaataggctgcatatgaatagagcaggtcttggctgctatcttttctggcttcttcactgcaaggctggccattaggatgaaagcattgaccactgctgctcagagtcacagtgctgggagaagggcctggcagatcaagcagcacagagtaatttacaaactgtacatcttctaggcccaaagaggtccactgagtcttaatcttctttgaaatttccatgtcatcttcatttttatatagttgtaccaaatttctgaaagacttcttaatatcttctgcctggattgtcttgagaatctcttgatataactgaggatcaactgttcctgaagatggagcatctgaagggcaatttgtatgtacataataacctatcaaaatcccaaaaataaataaaatggtggctgtgcaaagtatttttaagacgtggcaaaagttgcagcgattgctctttggtgcagatcgtgtataatgggtaatgtagtcagattcttcttgaagtctctggaaccttcctttgggtgaagttgctggttgaatggaatcaagattgaggtctatagtctctgaatgccctaggttctgattctcagcaccgtctagctggaattggtcaaaaccagactcctctagttccttctccatgtcccactctaagtcaagggcagtggcttgaaggtcatcattgtctaagtactgtgagtgtcctggagctctttgatctgcatggaccttctgataggccatctttttacttcaattgaatgttcctagtgcaactggagggcttctgcaggttacaggagactgacaatctggacccagtcttcatccaggtgcctaatagtcaatgctcatttccaatattaacaggagttttgaagaagtggatttcaaccctcaaggatgacttggagtgtttcaagacttcagaggaagaagtaacttgtttttaatcgttttctttatagaaactaaatttcatttaaattattcttttcttccctcagcctcctgagcggcgcgggcgcgggctcgtctgcggtacggctgccgggccaggccggattttcagcagccgtaaagcgggagaagcgggcgcgagccgcggcgcgaaccctcgcccccgagcggcggccccggcgcctccgccgcgagcgtcagccgcttggcaaggaacgggctgggctgagtcataataaaagacgcgtttgtcgagccaagtgggaagaagagccgcgggcagcagtgttcaatggcacaagcctcaaaaattgggaaggattttttttttaatgggcaaaactggaaacttgcccccatggtgcccatcaaaagatatgtttcgtttataatttgcatatattttatacatagtctttgaatctaataaaacttttaaaagaatttttaaagcccattgcttgcagagccaaattcctggttatagcttcgtgacttacgcaagttacttgaattctgtgcttttgtttttcatccatgaaacaggataataaaggtacctccctcaagagagactgcgagagagcttggcatcctgcctgcacttagcactcgctaaatgttaattgttattttaaaataggagggaggagataataaagaggaacttagataacagttttgaatggaagaagatacgaatataaatcaagatttttcttttttcaagtggagtaaattagacaaattaccaatggaagagaagaaagtggagcctggaaggaacaaacggggctaagagaagtagctgaagcgagggaaggaagaagggggaaggaggaaagaagagaggaagaggggtgaataaaagcctccaaggaacaaacgaggctgaaagatgtggctgaaggtagggaaggaagaaaaagggaggaagagaggaagaaataaaaccaaggaagcaagaataaagctaggctgcgtgggaagaggggaggaaggaaggagagagaaattcaactaggctcagtggccaaaatgctgaagtgtgtcctgccgggagggagtggaggaatatgtttactcactatttagaaatgcatgacaaactccatccgctgagggagatttttacaatgtataaacagagaaacaactgtctaaaaatgagccccaaatgaggagcctttgctccagtgaatgagatttggcagttctgcaaaatgaggaaattcttccttgtgcggcatcttgaagggttgagtcatgaaacccacagcaaatattagtgggctggattcctgaaaggcatgccagatggacgcattctggttagttttactgtgtgatgttcccttctgtacttctgtcaattttagaagaaaagagtgtgaataaagatttgagaagtgaacttaaaagccaaactagttacttaatgtacgagtatccacccaccaggagcttacagttacagattccaaaacaagcaaccgtttctcccactttcattttccctcccctttgtttctactttcaccgtattgctttttatccatttttataatatgattttttacagtggaaccgcctacgggaaaggtgcttttaattaatacgaaagaatggaaggaatttcagctaggcctctctaagagggtaaagctttgtgaaagaaaggttttttagctgaagttttaatgagaataagagtagttggcagatgtgaaatcagaagttttttcagacaagaaaataatacgactcgagtgaaagggaatggactagaaatcagaaacagttctattccttaattaccgtaagaaccaaagactggaggaaagtttttcctattctataaagaaaaatgggggcctccctccaccagccagaccttcaaaaaaggaaaaaataaaaattaaaaacctctattagattcttgtaatgatttgctttttcttaggagaacttcttcagggtaaaagacgtgaaagtgcttctttcggcaacttctgacgaaatacttttgtagaagcaaaatttctgaagggataatttttgctcaagcaaaaaactattagtaagataagaatcccttttcctttgtttcaattttgctaagccttcaggctgaggcaaacagattatcattaaacctttattaatgtgaaaccaaaaaaagataaaatcttaaatgctgcgaagcccttaacctaaaaggagcaagaaaacaaaccaaggcccagaaaatagagaaagggattaggaagcctttctaaggggaacctttgaactgtgggctgtaaaatgaatgtctgtgacttgccttaaacaaataggcaatataaactaaagctgggaactaagaagatctcctcagatcagataaaaagcttaccttgtgtgaaacactgtggtcaaagaagaaaattcctttcatcttaagtggagacaaaaacgtgtatcacttgttttgtgtgtgctcataaaacacctccatcacctgaatcccttgggtgcaattttttgatggacttggcattctttaaa

SEQ ID NO: 12610 - RNA, 9037 nt, Homo sapiens
  source 1..9037: mol_type = other RNA
gatctcactttgttgcccaggctattttctggatgtctattaaaaaaaaattagtcctgcacagtgttctagaaagggtttttcttttcagaatatccatattctccaagtagcaagttagaatataaggaatatttgccattaaacctttctgttagaaatgtaaacatgaaattgcctaatatagacctatctcagatgctaaatagaattgtttataacacctttggaatataattatgtgagctacacttaaccatctggcattttgcttcctgcggacaatttgcaatagcatagaaaaatattttgtttgtgtatttcttatcaaacagatatgctaaagttctgtttagagagtaatagcattttattctaacttttaaaataaggtagtccatttgcagcagcttgatatataagtaaacaaaaatttttaatattaataaaacactagcacatacactgaaagcatctaagaaattcaaaatataaaacacttaccaagtaatgaccatatgagtggtaacatattgaataaaggccctttgaagaagttggagagttatgattactgagcaggctagataattaaataattacacattttgattgaaaaatatatgtagttcattaaaatagggactctaactccacttctctagctaagcttctattcagatgccacgtttgtactttaattagaacaaaagaccgacattaacttcaatgcaacataataattcataataatgattgtatattaatctcttgagcttgcaggaatatagcacatgacatatggcatgatacaggcacctgtgtgatcctttggggacttaggtggtgcatattaattagcccctggaaaataaaatctgtttccttctgagaaaagctacctcagtgcttattggcttaagccatcaaagaaattagatgaaatactgttaggctgggtctgcactcattaaagctttgtctagatgtaagcactgaatcaactgcctctgagttaagtcttgactgaatggtgcataagaaatcagagtaatcatgcatttctttggccttgatgattggattttggcatttaaaaaatccatcaaaattaccattttggttacagaaaattatgtaattgtataattcaaacaaaataatgtaaccagaaacactaaaatttgaagccacttcattttcctaaatgctgcttgaaactgcctcaatttaacccttttatttgtaaattcagattcaacccgaatatgagattataaatggcttaagaaatatgtcatcttgcaataatcagggtaacaagattcttgacggtcccaggtctgctaaaggcacttcagtgtgtatatctttgtcaggcaatggaacgatattatgaaactaaaactctggctgattaacagatcatttaaattgagactgatagatcttaaaattacttctcagggggaaaaagttacaatgctagagtgtacctagaaaacagaaacttgagtagacatggtaatgaccagaaaaggctatctttatacatttcttttgctacgcttcaaattcatgtcacctaaaagttgtgaagtgcacaaaacaaatctacttaactgaaaattattttcaatgaatgggatgtttagaactctgtgagggtttttaaggtcttttcgaatagcaaattctaatgaggcttttttaagttggcaatttaaactcatacaagaaataaaaactcaccagtgtggctgggcagaatatatatattttctcaaatattgtttgtttgttttttccctgcactgtatccatggtcccatgatgaaactgttatattgctgatatatttattggaatatgtgggccaacttcctttccactcaacatatggattggtagtttaaaataattcctttctattaagcaaatgtgtggctaaggcacatttaaatagcccattaaaccaatgagatgacaatgtgttaccctcagagaaagcttaatttttggagtaatcaattacacatatcacagaatgtctcatgagaacatttttggctaggtctaccaatttatcatacaaataattatagattttcatttgaggcaaagatgctgattcatcattagtaacatggtcacaaataatcatttattttatttttgttaacatctgtctttcctgtggggaaacttactatatgctctacgtttatttaatttaaaaagtcaattggttattctgaatttttaaaaataacataaaactgttgttctaaatcacagcacctgcttttctttttttagtgaaattatataagcatttagagaatgaaagtgtaagacttgtggtttctggtctctttttactgtttgtaagcctactcgtcatgatattccacaatggtgcacttgccttttaatgctcttatagatatcttcaaacttgcctacatatatacgcctttgttggagtgggctaccatcatcaggaatgatgtcatttgtttcttcaaactcctttattataccaaaaaagtgacagactccacagtctgatcagttttggagaaatatgttaacattttcaattatctcactttctagaatcaaaatagtctgattttttttttcggcactcagtgtaaagaacaaagaactgaatacagtgggcccagaagagaaatatgcctcatcatttttattagctttggaactgtggacaagtcactcaacctagttttctcattttgaaatgggttgttgtgggaattaaaaaaaaaaaaaaaaaaaaaaaaggatacatgggaaaaattctaaaacaccagtgcctgggatgtagcaggcacaaatataagctgcaactgaattgttttcttagagataaaatgggtccacttttcttttctcataatgattccattaataacaaatctttacgtctttcttgttattatgactcttcaatttatttagaaatgtcaattagtgttttcttggaaactacgattaacgtagattggaaattcttaaacttcagtgtgtgtaacagacatccagaaatcttgctgaagatgtagattcctagccctgtctttctaaatttcacattttgagaaacggtgatttagattgttgacttaacactggcctgacttgccctcttacagatatattttgctcaatgtccttcttcctgacttctggtgttctgtaaggattctccccactttctctcaagtacccagtctttgtgtcctttgcctgaattctcggggagagttttgtttgtcaggtacagtcagagaatgaactagccttgaattaaaagcagtgtttccagcccatgcaacatctgacagaatggctggttacatcgaatgcactggaaaagatcatttataaccctgtctcctcagggagaagcaagatatactgcatgagaaagcagagaagcttaaattccagtggtgcttttgttactaactaaatacatgactatgtccaagtttcttactcactttgggtttagttactatatctggtgggggtaattgataatgccttctctggctgaaggcaagatctcagggcttagaccagaatctttattaggctttcttttgattctgagacttatgcttttccataaagggcagtatctcatgtgtaccctgcctgaacataaatttcaccgttacacctttaccacattttcttcagagaatatttatgattcattatttcctaggcacaattctatgtatgaaagattgtgagaagtaccaggcatatagacgactcagcaacagcttaaacctactaccaattcacattaacacttgctattaatttgctcaggattttatttatttgaatctattgggggtggggaggggaggggagtgaaatgatatacatttggaggcaccctcaggtaatcacactatagaaataatgctgctagttaagaggtttgttgcaaagatgtaaagcagcatgtacagaatttgttggacgtctgctttaggtataatttaatatctccacgtatcttttaatagactaataaaaaaccatagttaactacagttttcaaatagcaaataacatataatttagaggtgaggaatacagaagaaggtttttatctatacagtgtgacttacctaggtacgcaatctttaaacaaaatgaagaagaaacatgttttctgttctcagtgctattgtaggttatgggaataaattaatttagaaatttgttctaaaataatgaactaccaaactgataatagcttgcctttatttgttttagtttcatctgtaagtgaataactggaatgaacacatcaacctttggttaaatataaggctttctagcttttgggcttacatgcacctgcttgtgtattcccacctcttttctgatgatctctgaagaggaagaaagagcatgaatgcctaggtatgcacaagcctatttatttctagacctttcctatacacactcttcaacatggcaaatgtttgcaaacaaatacattggttaaaaaaataatattgtaaggtagtttcatttttcatctaaaaatatgtgcacacaggcaatttcgatgaaaatggatttctgcttgaattatctagctaattgcctctattccctgctttgccttgagcatataaaaattatttagggtagacagtgttgaaccttataaatcaattaatcagtattgattaattatttcccctcaactttagtttgcctttaaactaagactaggtttatgctcatccataaaaagtgaaaatttaaacatacacagactgtctgcaatgtcactctggcggtgtatcatggggagatatgtttgaattagatagagaaaatttatatgaaatactctgaggctatgtttcctaaggggaattgctttatccagtataggaaaaccatttttcacataaatttctaaagataaattagaactttaacctgacacctaataggtagaattttagggtttgggggaataataatagttgctagagctattcaatggcaatgtcaatataaaaagcttagttttccacatgagagaagaactgaagtgtagacgagacactctcttacagtaacactgcagaaacttagaagcatgaatattttctagatttccatcttagtcacaattaaggataaagaagaaaaaatatgaaaagtttcttcataatattaaggggcttttattgataaaacaactatttctttcatagtaagttctttttgtcagaggcagaaatagaaatttgattctttagaagacattttgggtttcaaagagaaactctgctactttactgttgaaaatatatagtactctgagaaagctgccttacagcaaggagtttcagaaaagatacaagaaagaaaaccaatgtgagatgctttcattttagagtccctgcttcagtgtttccaacagaaacaagagaaaaagtaataagaaatatttttttctccctcttaagacatacatcactcctgaaattcttagaaaatcaactgaggcaaattaggggtttcaaagctagtcaccttgtaagttgttaggaaaaaaatttgcatttaaattgctctatgtagctcccttgagattttctcctggaatgcttatggctcttttttcattaatacttaaaaaaatacaatttcataaccagtgtattactacatctagttgtgttaagaagagaaacttcatttcataaaatagaaacattcaaagtggtttaggtcaaccaatcactcagtcagaatacttgaattcttcatattgaacacttaatagtgaagttaatctgaaccatatcaactctccatttcttttacagaaactaagtcattaatagctctatcagagagaataaactgtgttcctatatgccctccccataggaacaaagatagtccagaacttcttggaaatttttccttaaaatagtacatatttttatatatcagatttctttttaataggtaattcttaagtcctatttcaataacttgctttacatattcagaaatgtagatataagaaaaatattaaatgtgcaaaatgttctttctatatttacatttaaaaaatacaatgtaataatagctttatacttgtcaaaaagccattggggaaaataagccttcaatgtcagaaaatctggttaaattagagcttttgcttgtggaattgtaaacaaacttttaaaaatgctcagagttttctcaattcttcccatccaagacactcttgaacacatcaagtcctgctttgaagtaaacctgagctgaattaatgctgttcaacacctctgacagggcttcttgaagggtctcatttgatgcaaggggtttgcagtgttcccaagcctctataagtattgaaaaccggcttgtcttttcatcaaggtggtagaggatgtttctataaaaacctggtggtgcctgctttaccagaaagcttttctccatgtcttggagaatgtcattcagcatccggatgcggatgggtgctctctccttgggatcattagcaggtcgcatctcatcagactgaaaaagttcagcactctcccgcaggcgtaacgccatggctaacagttgatgagtgttgggttgatcacctttaaggttgttttgaacttctaaagctatatcaagtgcattaaagggcagaacaggttcgttggcaatttgcaaaatcacttctcctgagagcttagtaatggtttcatgaaggttgaaagagggatccatttcttcaatttttgttgctcgtgtagaaaaacgggcctcggagagaaaacttggaccctctaatgttttgatgtcctcgtaagcaaactgcacgatgggaactccaagatggttgatgaaataatcagcatcaccttgtatctgtatagaactgatattggtttctgggcactgggctcttctggtacagttgaaattatttttctctactaccagttgctgaagagatggtgatgctacaggatacagactagagttcccccttatgggactgtggaggctaatataagccacaacatttttctgaagaaccttcttgaaatcctctccccattcatatgagccaatattgccaaaagctgttcctccccaagaacagaaaacaatagttcggtctggtctccaccctctcttaacttttgacatcaaggcacggataaacgctgtgattattgcagtactactggcccattcttgtccattataactgtgtgcagtgtgatgatggctgccaactatgatataccggtctggagatgtcaagcccattacaaatccaacaacattagtaactgttttcaattttgtgactgtctgaacttgcatgctgacgactcttatttcattatttggaagctctagagagctacacgcttcatttttggttctagcttttggcgaagagatcagttttgcaacgaggggtgcagagatgggctgcactaatagagaggtgaggtttgatcggctttgtctaaaactttcatcgacacttgggtaaccaggcgtagaagggtctcctcctggattcagtgacaccatgaaggtatcatggctaggattcacagtctttggcaaatcacaaggatcgatatacagaagaacacctccaaatccagccttttccaatgaggaaagcttataaagcagtggcaattttcctaatttcaggagtgcgatctgatttgttacgttttttattttcctaatcctttttaaatcatctgccattccataactcacatcgatgacttcagccttgagagttcctttggcagaataggctgcatatgaatagagcaggtcttggctgctatcttttctggcttcttcactgcaaggctggccattaggatgaaagcattgaccactgctgctcagagtcacagtgctgggagaagggcctggcagatcaagcagcacagagtaatttacaaactgtacatcttctaggcccaaagaggtccactgagtcttaatcttctttgaaatttccatgtcatcttcatttttatatagttgtaccaaatttctgaaagacttcttaatatcttctgcctggattgtcttgagaatctcttgatataactgaggatcaactgttcctgaagatggagcatctgaagggcaatttgtatgtacataataacctatcaaaatcccaaaaataaataaaatggtggctgtgcaaagtatttttaagacgtggcaaaagttgcagcgattgctctttggtgcagatcgtgtataatgggtaatgtagtcagattcttcttgaagtctctggaaccttcctttgggtgaagttgctggttgaatggaatcaagattgaggtctatagtctctgaatgccctaggttctgattctcagcaccgtctagctggaattggtcaaaaccagactcctctagttccttctccatgtcccactctaagtcaagggcagtggcttgaaggtcatcattgtctaagtactgtgagtgtcctggagctctttgatctgcatggaccttctgataggccatctttttacttcaattgaatgttcctagtgcaactggagggcttctgcaggttacaggagactgacaatctggacccagtcttcatccaggtgcctaatagtcaatgctcatttccaatattaacaggagttttgaagaagtggatttcaaccctcaaggatgacttggagtgtttcaagacttcagaggaagaagtaacttgtttttaatcgttttctttatagaaactaaatttcatttaaattattcttttcttccctcagcctcctttattacaggaaagcttaaacgaaatgcatttgtgtaagagatgtagatacaaacttcagaatattcatgttaaccatcattgatctctgctttgatggaggtgatttttgatgtaaaataagccgaaattaca

SEQ ID NO: 12611 - RNA, 9367 nt, Homo sapiens
  source 1..9367: mol_type = other RNA
gatctcactttgttgcccaggctattttctggatgtctattaaaaaaaaattagtcctgcacagtgttctagaaagggtttttcttttcagaatatccatattctccaagtagcaagttagaatataaggaatatttgccattaaacctttctgttagaaatgtaaacatgaaattgcctaatatagacctatctcagatgctaaatagaattgtttataacacctttggaatataattatgtgagctacacttaaccatctggcattttgcttcctgcggacaatttgcaatagcatagaaaaatattttgtttgtgtatttcttatcaaacagatatgctaaagttctgtttagagagtaatagcattttattctaacttttaaaataaggtagtccatttgcagcagcttgatatataagtaaacaaaaatttttaatattaataaaacactagcacatacactgaaagcatctaagaaattcaaaatataaaacacttaccaagtaatgaccatatgagtggtaacatattgaataaaggccctttgaagaagttggagagttatgattactgagcaggctagataattaaataattacacattttgattgaaaaatatatgtagttcattaaaatagggactctaactccacttctctagctaagcttctattcagatgccacgtttgtactttaattagaacaaaagaccgacattaacttcaatgcaacataataattcataataatgattgtatattaatctcttgagcttgcaggaatatagcacatgacatatggcatgatacaggcacctgtgtgatcctttggggacttaggtggtgcatattaattagcccctggaaaataaaatctgtttccttctgagaaaagctacctcagtgcttattggcttaagccatcaaagaaattagatgaaatactgttaggctgggtctgcactcattaaagctttgtctagatgtaagcactgaatcaactgcctctgagttaagtcttgactgaatggtgcataagaaatcagagtaatcatgcatttctttggccttgatgattggattttggcatttaaaaaatccatcaaaattaccattttggttacagaaaattatgtaattgtataattcaaacaaaataatgtaaccagaaacactaaaatttgaagccacttcattttcctaaatgctgcttgaaactgcctcaatttaacccttttatttgtaaattcagattcaacccgaatatgagattataaatggcttaagaaatatgtcatcttgcaataatcagggtaacaagattcttgacggtcccaggtctgctaaaggcacttcagtgtgtatatctttgtcaggcaatggaacgatattatgaaactaaaactctggctgattaacagatcatttaaattgagactgatagatcttaaaattacttctcagggggaaaaagttacaatgctagagtgtacctagaaaacagaaacttgagtagacatggtaatgaccagaaaaggctatctttatacatttcttttgctacgcttcaaattcatgtcacctaaaagttgtgaagtgcacaaaacaaatctacttaactgaaaattattttcaatgaatgggatgtttagaactctgtgagggtttttaaggtcttttcgaatagcaaattctaatgaggcttttttaagttggcaatttaaactcatacaagaaataaaaactcaccagtgtggctgggcagaatatatatattttctcaaatattgtttgtttgttttttccctgcactgtatccatggtcccatgatgaaactgttatattgctgatatatttattggaatatgtgggccaacttcctttccactcaacatatggattggtagtttaaaataattcctttctattaagcaaatgtgtggctaaggcacatttaaatagcccattaaaccaatgagatgacaatgtgttaccctcagagaaagcttaatttttggagtaatcaattacacatatcacagaatgtctcatgagaacatttttggctaggtctaccaatttatcatacaaataattatagattttcatttgaggcaaagatgctgattcatcattagtaacatggtcacaaataatcatttattttatttttgttaacatctgtctttcctgtggggaaacttactatatgctctacgtttatttaatttaaaaagtcaattggttattctgaatttttaaaaataacataaaactgttgttctaaatcacagcacctgcttttctttttttagtgaaattatataagcatttagagaatgaaagtgtaagacttgtggtttctggtctctttttactgtttgtaagcctactcgtcatgatattccacaatggtgcacttgccttttaatgctcttatagatatcttcaaacttgcctacatatatacgcctttgttggagtgggctaccatcatcaggaatgatgtcatttgtttcttcaaactcctttattataccaaaaaagtgacagactccacagtctgatcagttttggagaaatatgttaacattttcaattatctcactttctagaatcaaaatagtctgattttttttttcggcactcagtgtaaagaacaaagaactgaatacagtgggcccagaagagaaatatgcctcatcatttttattagctttggaactgtggacaagtcactcaacctagttttctcattttgaaatgggttgttgtgggaattaaaaaaaaaaaaaaaaaaaaaaaaggatacatgggaaaaattctaaaacaccagtgcctgggatgtagcaggcacaaatataagctgcaactgaattgttttcttagagataaaatgggtccacttttcttttctcataatgattccattaataacaaatctttacgtctttcttgttattatgactcttcaatttatttagaaatgtcaattagtgttttcttggaaactacgattaacgtagattggaaattcttaaacttcagtgtgtgtaacagacatccagaaatcttgctgaagatgtagattcctagccctgtctttctaaatttcacattttgagaaacggtgatttagattgttgacttaacactggcctgacttgccctcttacagatatattttgctcaatgtccttcttcctgacttctggtgttctgtaaggattctccccactttctctcaagtacccagtctttgtgtcctttgcctgaattctcggggagagttttgtttgtcaggtacagtcagagaatgaactagccttgaattaaaagcagtgtttccagcccatgcaacatctgacagaatggctggttacatcgaatgcactggaaaagatcatttataaccctgtctcctcagggagaagcaagatatactgcatgagaaagcagagaagcttaaattccagtggtgcttttgttactaactaaatacatgactatgtccaagtttcttactcactttgggtttagttactatatctggtgggggtaattgataatgccttctctggctgaaggcaagatctcagggcttagaccagaatctttattaggctttcttttgattctgagacttatgcttttccataaagggcagtatctcatgtgtaccctgcctgaacataaatttcaccgttacacctttaccacattttcttcagagaatatttatgattcattatttcctaggcacaattctatgtatgaaagattgtgagaagtaccaggcatatagacgactcagcaacagcttaaacctactaccaattcacattaacacttgctattaatttgctcaggattttatttatttgaatctattgggggtggggaggggaggggagtgaaatgatatacatttggaggcaccctcaggtaatcacactatagaaataatgctgctagttaagaggtttgttgcaaagatgtaaagcagcatgtacagaatttgttggacgtctgctttaggtataatttaatatctccacgtatcttttaatagactaataaaaaaccatagttaactacagttttcaaatagcaaataacatataatttagaggtgaggaatacagaagaaggtttttatctatacagtgtgacttacctaggtacgcaatctttaaacaaaatgaagaagaaacatgttttctgttctcagtgctattgtaggttatgggaataaattaatttagaaatttgttctaaaataatgaactaccaaactgataatagcttgcctttatttgttttagtttcatctgtaagtgaataactggaatgaacacatcaacctttggttaaatataaggctttctagcttttgggcttacatgcacctgcttgtgtattcccacctcttttctgatgatctctgaagaggaagaaagagcatgaatgcctaggtatgcacaagcctatttatttctagacctttcctatacacactcttcaacatggcaaatgtttgcaaacaaatacattggttaaaaaaataatattgtaaggtagtttcatttttcatctaaaaatatgtgcacacaggcaatttcgatgaaaatggatttctgcttgaattatctagctaattgcctctattccctgctttgccttgagcatataaaaattatttagggtagacagtgttgaaccttataaatcaattaatcagtattgattaattatttcccctcaactttagtttgcctttaaactaagactaggtttatgctcatccataaaaagtgaaaatttaaacatacacagactgtctgcaatgtcactctggcggtgtatcatggggagatatgtttgaattagatagagaaaatttatatgaaatactctgaggctatgtttcctaaggggaattgctttatccagtataggaaaaccatttttcacataaatttctaaagataaattagaactttaacctgacacctaataggtagaattttagggtttgggggaataataatagttgctagagctattcaatggcaatgtcaatataaaaagcttagttttccacatgagagaagaactgaagtgtagacgagacactctcttacagtaacactgcagaaacttagaagcatgaatattttctagatttccatcttagtcacaattaaggataaagaagaaaaaatatgaaaagtttcttcataatattaaggggcttttattgataaaacaactatttctttcatagtaagttctttttgtcagaggcagaaatagaaatttgattctttagaagacattttgggtttcaaagagaaactctgctactttactgttgaaaatatatagtactctgagaaagctgccttacagcaaggagtttcagaaaagatacaagaaagaaaaccaatgtgagatgctttcattttagagtccctgcttcagtgtttccaacagaaacaagagaaaaagtaataagaaatatttttttctccctcttaagacatacatcactcctgaaattcttagaaaatcaactgaggcaaattaggggtttcaaagctagtcaccttgtaagttgttaggaaaaaaatttgcatttaaattgctctatgtagctcccttgagattttctcctggaatgcttatggctcttttttcattaatacttaaaaaaatacaatttcataaccagtgtattactacatctagttgtgttaagaagagaaacttcatttcataaaatagaaacattcaaagtggtttaggtcaaccaatcactcagtcagaatacttgaattcttcatattgaacacttaatagtgaagttaatctgaaccatatcaactctccatttcttttacagaaactaagtcattaatagctctatcagagagaataaactgtgttcctatatgccctccccataggaacaaagatagtccagaacttcttggaaatttttccttaaaatagtacatatttttatatatcagatttctttttaataggtaattcttaagtcctatttcaataacttgctttacatattcagaaatgtagatataagaaaaatattaaatgtgcaaaatgttctttctatatttacatttaaaaaatacaatgtaataatagctttatacttgtcaaaaagccattggggaaaataagccttcaatgtcagaaaatctggttaaattagagcttttgcttgtggaattgtaaacaaacttttaaaaatgctcagagttttctcaattcttcccatccaagacactcttgaacacatcaagtcctgctttgaagtaaacctgagctgaattaatgctgttcaacacctctgacagggcttcttgaagggtctcatttgatgcaaggggtttgcagtgttcccaagcctctataagtattgaaaaccggcttgtcttttcatcaaggtggtagaggatgtttctataaaaacctggtggtgcctgctttaccagaaagcttttctccatgtcttggagaatgtcattcagcatccggatgcggatgggtgctctctccttgggatcattagcaggtcgcatctcatcagactgaaaaagttcagcactctcccgcaggcgtaacgccatggctaacagttgatgagtgttgggttgatcacctttaaggttgttttgaacttctaaagctatatcaagtgcattaaagggcagaacaggttcgttggcaatttgcaaaatcacttctcctgagagcttagtaatggtttcatgaaggttgaaagagggatccatttcttcaatttttgttgctcgtgtagaaaaacgggcctcggagagaaaacttggaccctctaatgttttgatgtcctcgtaagcaaactgcacgatgggaactccaagatggttgatgaaataatcagcatcaccttgtatctgtatagaactgatattggtttctgggcactgggctcttctggtacagttgaaattatttttctctactaccagttgctgaagagatggtgatgctacaggatacagactagagttcccccttatgggactgtggaggctaatataagccacaacatttttctgaagaaccttcttgaaatcctctccccattcatatgagccaatattgccaaaagctgttcctccccaagaacagaaaacaatagttcggtctggtctccaccctctcttaacttttgacatcaaggcacggataaacgctgtgattattgcagtactactggcccattcttgtccattataactgtgtgcagtgtgatgatggctgccaactatgatataccggtctggagatgtcaagcccattacaaatccaacaacattagtaactgttttcaattttgtgactgtctgaacttgcatgctgacgactcttatttcattatttggaagctctagagagctacacgcttcatttttggttctagcttttggcgaagagatcagttttgcaacgaggggtgcagagatgggctgcactaatagagaggtgaggtttgatcggctttgtctaaaactttcatcgacacttgggtaaccaggcgtagaagggtctcctcctggattcagtgacaccatgaaggtatcatggctaggattcacagtctttggcaaatcacaaggatcgatatacagaagaacacctccaaatccagccttttccaatgaggaaagcttataaagcagtggcaattttcctaatttcaggagtgcgatctgatttgttacgttttttattttcctaatcctttttaaatcatctgccattccataactcacatcgatgacttcagccttgagagttcctttggcagaataggctgcatatgaatagagcaggtcttggctgctatcttttctggcttcttcactgcaaggctggccattaggatgaaagcattgaccactgctgctcagagtcacagtgctgggagaagggcctggcagatcaagcagcacagagtaatttacaaactgtacatcttctaggcccaaagaggtccactgagtcttaatcttctttgaaatttccatgtcatcttcatttttatatagttgtaccaaatttctgaaagacttcttaatatcttctgcctggattgtcttgagaatctcttgatataactgaggatcaactgttcctgaagatggagcatctgaagggcaatttgtatgtacataataacctatcaaaatcccaaaaataaataaaatggtggctgtgcaaagtatttttaagacgtggcaaaagttgcagcgattgctctttggtgcagatcgtgtataatgggtaatgtagtcagattcttcttgaagtctctggaaccttcctttgggtgaagttgctggttgaatggaatcaagattgaggtctatagtctctgaatgccctaggttctgattctcagcaccgtctagctggaattggtcaaaaccagactcctctagttccttctccatgtcccactctaagtcaagggcagtggcttgaaggtcatcattgtctaagtactgtgagtgtcctggagctctttgatctgcatggaccttctgataggccatctttttacttcaattgaatgttcctagtgcaactggagggcttctgcaggttacaggagactgacaatctggacccagtcttcatccaggtgcctaatagtcaatgctcatttccctctgttaagttagtttccttcctcctcagtttttcacactcatttcaatatcttccatcttccttaagcttgtttttaatcgttttctttatagaaactaaatttcatttaaattattcttttcttccctcagcctcctagggttgaataaaagacgccctaagacatcaaaagctattttgaacgtccagctgggagatctgtaaatgaatgatagaaagttcgaaaatcctcacaaaagattgactctcagtgaactttgctcctgataaattctacccacaatgtttattcaaatttagttttaaaaagagaaagcagactttggagagatggcctttacgtggattttatttgctgatgataatgatgatgcacagtgcctcttcacaagattacatgagttaaaaggtaatcccactatcactcttgcaccgatgagtgctctacttgagtgctgatctcaatttttgactccaagctttattacaggaaagcttaaacgaaatgcatttgtgtaagagatgtagatacaaacttcagaatattcatgttaaccatcattgatctctgctttgatggaggtgatttttgatgtaaaataagccgaaattaca

SEQ ID NO: 12612 - RNA, 9742 nt, Homo sapiens
  source 1..9742: mol_type = other RNA
gatctcactttgttgcccaggctattttctggatgtctattaaaaaaaaattagtcctgcacagtgttctagaaagggtttttcttttcagaatatccatattctccaagtagcaagttagaatataaggaatatttgccattaaacctttctgttagaaatgtaaacatgaaattgcctaatatagacctatctcagatgctaaatagaattgtttataacacctttggaatataattatgtgagctacacttaaccatctggcattttgcttcctgcggacaatttgcaatagcatagaaaaatattttgtttgtgtatttcttatcaaacagatatgctaaagttctgtttagagagtaatagcattttattctaacttttaaaataaggtagtccatttgcagcagcttgatatataagtaaacaaaaatttttaatattaataaaacactagcacatacactgaaagcatctaagaaattcaaaatataaaacacttaccaagtaatgaccatatgagtggtaacatattgaataaaggccctttgaagaagttggagagttatgattactgagcaggctagataattaaataattacacattttgattgaaaaatatatgtagttcattaaaatagggactctaactccacttctctagctaagcttctattcagatgccacgtttgtactttaattagaacaaaagaccgacattaacttcaatgcaacataataattcataataatgattgtatattaatctcttgagcttgcaggaatatagcacatgacatatggcatgatacaggcacctgtgtgatcctttggggacttaggtggtgcatattaattagcccctggaaaataaaatctgtttccttctgagaaaagctacctcagtgcttattggcttaagccatcaaagaaattagatgaaatactgttaggctgggtctgcactcattaaagctttgtctagatgtaagcactgaatcaactgcctctgagttaagtcttgactgaatggtgcataagaaatcagagtaatcatgcatttctttggccttgatgattggattttggcatttaaaaaatccatcaaaattaccattttggttacagaaaattatgtaattgtataattcaaacaaaataatgtaaccagaaacactaaaatttgaagccacttcattttcctaaatgctgcttgaaactgcctcaatttaacccttttatttgtaaattcagattcaacccgaatatgagattataaatggcttaagaaatatgtcatcttgcaataatcagggtaacaagattcttgacggtcccaggtctgctaaaggcacttcagtgtgtatatctttgtcaggcaatggaacgatattatgaaactaaaactctggctgattaacagatcatttaaattgagactgatagatcttaaaattacttctcagggggaaaaagttacaatgctagagtgtacctagaaaacagaaacttgagtagacatggtaatgaccagaaaaggctatctttatacatttcttttgctacgcttcaaattcatgtcacctaaaagttgtgaagtgcacaaaacaaatctacttaactgaaaattattttcaatgaatgggatgtttagaactctgtgagggtttttaaggtcttttcgaatagcaaattctaatgaggcttttttaagttggcaatttaaactcatacaagaaataaaaactcaccagtgtggctgggcagaatatatatattttctcaaatattgtttgtttgttttttccctgcactgtatccatggtcccatgatgaaactgttatattgctgatatatttattggaatatgtgggccaacttcctttccactcaacatatggattggtagtttaaaataattcctttctattaagcaaatgtgtggctaaggcacatttaaatagcccattaaaccaatgagatgacaatgtgttaccctcagagaaagcttaatttttggagtaatcaattacacatatcacagaatgtctcatgagaacatttttggctaggtctaccaatttatcatacaaataattatagattttcatttgaggcaaagatgctgattcatcattagtaacatggtcacaaataatcatttattttatttttgttaacatctgtctttcctgtggggaaacttactatatgctctacgtttatttaatttaaaaagtcaattggttattctgaatttttaaaaataacataaaactgttgttctaaatcacagcacctgcttttctttttttagtgaaattatataagcatttagagaatgaaagtgtaagacttgtggtttctggtctctttttactgtttgtaagcctactcgtcatgatattccacaatggtgcacttgccttttaatgctcttatagatatcttcaaacttgcctacatatatacgcctttgttggagtgggctaccatcatcaggaatgatgtcatttgtttcttcaaactcctttattataccaaaaaagtgacagactccacagtctgatcagttttggagaaatatgttaacattttcaattatctcactttctagaatcaaaatagtctgattttttttttcggcactcagtgtaaagaacaaagaactgaatacagtgggcccagaagagaaatatgcctcatcatttttattagctttggaactgtggacaagtcactcaacctagttttctcattttgaaatgggttgttgtgggaattaaaaaaaaaaaaaaaaaaaaaaaaggatacatgggaaaaattctaaaacaccagtgcctgggatgtagcaggcacaaatataagctgcaactgaattgttttcttagagataaaatgggtccacttttcttttctcataatgattccattaataacaaatctttacgtctttcttgttattatgactcttcaatttatttagaaatgtcaattagtgttttcttggaaactacgattaacgtagattggaaattcttaaacttcagtgtgtgtaacagacatccagaaatcttgctgaagatgtagattcctagccctgtctttctaaatttcacattttgagaaacggtgatttagattgttgacttaacactggcctgacttgccctcttacagatatattttgctcaatgtccttcttcctgacttctggtgttctgtaaggattctccccactttctctcaagtacccagtctttgtgtcctttgcctgaattctcggggagagttttgtttgtcaggtacagtcagagaatgaactagccttgaattaaaagcagtgtttccagcccatgcaacatctgacagaatggctggttacatcgaatgcactggaaaagatcatttataaccctgtctcctcagggagaagcaagatatactgcatgagaaagcagagaagcttaaattccagtggtgcttttgttactaactaaatacatgactatgtccaagtttcttactcactttgggtttagttactatatctggtgggggtaattgataatgccttctctggctgaaggcaagatctcagggcttagaccagaatctttattaggctttcttttgattctgagacttatgcttttccataaagggcagtatctcatgtgtaccctgcctgaacataaatttcaccgttacacctttaccacattttcttcagagaatatttatgattcattatttcctaggcacaattctatgtatgaaagattgtgagaagtaccaggcatatagacgactcagcaacagcttaaacctactaccaattcacattaacacttgctattaatttgctcaggattttatttatttgaatctattgggggtggggaggggaggggagtgaaatgatatacatttggaggcaccctcaggtaatcacactatagaaataatgctgctagttaagaggtttgttgcaaagatgtaaagcagcatgtacagaatttgttggacgtctgctttaggtataatttaatatctccacgtatcttttaatagactaataaaaaaccatagttaactacagttttcaaatagcaaataacatataatttagaggtgaggaatacagaagaaggtttttatctatacagtgtgacttacctaggtacgcaatctttaaacaaaatgaagaagaaacatgttttctgttctcagtgctattgtaggttatgggaataaattaatttagaaatttgttctaaaataatgaactaccaaactgataatagcttgcctttatttgttttagtttcatctgtaagtgaataactggaatgaacacatcaacctttggttaaatataaggctttctagcttttgggcttacatgcacctgcttgtgtattcccacctcttttctgatgatctctgaagaggaagaaagagcatgaatgcctaggtatgcacaagcctatttatttctagacctttcctatacacactcttcaacatggcaaatgtttgcaaacaaatacattggttaaaaaaataatattgtaaggtagtttcatttttcatctaaaaatatgtgcacacaggcaatttcgatgaaaatggatttctgcttgaattatctagctaattgcctctattccctgctttgccttgagcatataaaaattatttagggtagacagtgttgaaccttataaatcaattaatcagtattgattaattatttcccctcaactttagtttgcctttaaactaagactaggtttatgctcatccataaaaagtgaaaatttaaacatacacagactgtctgcaatgtcactctggcggtgtatcatggggagatatgtttgaattagatagagaaaatttatatgaaatactctgaggctatgtttcctaaggggaattgctttatccagtataggaaaaccatttttcacataaatttctaaagataaattagaactttaacctgacacctaataggtagaattttagggtttgggggaataataatagttgctagagctattcaatggcaatgtcaatataaaaagcttagttttccacatgagagaagaactgaagtgtagacgagacactctcttacagtaacactgcagaaacttagaagcatgaatattttctagatttccatcttagtcacaattaaggataaagaagaaaaaatatgaaaagtttcttcataatattaaggggcttttattgataaaacaactatttctttcatagtaagttctttttgtcagaggcagaaatagaaatttgattctttagaagacattttgggtttcaaagagaaactctgctactttactgttgaaaatatatagtactctgagaaagctgccttacagcaaggagtttcagaaaagatacaagaaagaaaaccaatgtgagatgctttcattttagagtccctgcttcagtgtttccaacagaaacaagagaaaaagtaataagaaatatttttttctccctcttaagacatacatcactcctgaaattcttagaaaatcaactgaggcaaattaggggtttcaaagctagtcaccttgtaagttgttaggaaaaaaatttgcatttaaattgctctatgtagctcccttgagattttctcctggaatgcttatggctcttttttcattaatacttaaaaaaatacaatttcataaccagtgtattactacatctagttgtgttaagaagagaaacttcatttcataaaatagaaacattcaaagtggtttaggtcaaccaatcactcagtcagaatacttgaattcttcatattgaacacttaatagtgaagttaatctgaaccatatcaactctccatttcttttacagaaactaagtcattaatagctctatcagagagaataaactgtgttcctatatgccctccccataggaacaaagatagtccagaacttcttggaaatttttccttaaaatagtacatatttttatatatcagatttctttttaataggtaattcttaagtcctatttcaataacttgctttacatattcagaaatgtagatataagaaaaatattaaatgtgcaaaatgttctttctatatttacatttaaaaaatacaatgtaataatagctttatacttgtcaaaaagccattggggaaaataagccttcaatgtcagaaaatctggttaaattagagcttttgcttgtggaattgtaaacaaacttttaaaaatgctcagagttttctcaattcttcccatccaagacactcttgaacacatcaagtcctgctttgaagtaaacctgagctgaattaatgctgttcaacacctctgacagggcttcttgaagggtctcatttgatgcaaggggtttgcagtgttcccaagcctctataagtattgaaaaccggcttgtcttttcatcaaggtggtagaggatgtttctataaaaacctggtggtgcctgctttaccagaaagcttttctccatgtcttggagaatgtcattcagcatccggatgcggatgggtgctctctccttgggatcattagcaggtcgcatctcatcagactgaaaaagttcagcactctcccgcaggcgtaacgccatggctaacagttgatgagtgttgggttgatcacctttaaggttgttttgaacttctaaagctatatcaagtgcattaaagggcagaacaggttcgttggcaatttgcaaaatcacttctcctgagagcttagtaatggtttcatgaaggttgaaagagggatccatttcttcaatttttgttgctcgtgtagaaaaacgggcctcggagagaaaacttggaccctctaatgttttgatgtcctcgtaagcaaactgcacgatgggaactccaagatggttgatgaaataatcagcatcaccttgtatctgtatagaactgatattggtttctgggcactgggctcttctggtacagttgaaattatttttctctactaccagttgctgaagagatggtgatgctacaggatacagactagagttcccccttatgggactgtggaggctaatataagccacaacatttttctgaagaaccttcttgaaatcctctccccattcatatgagccaatattgccaaaagctgttcctccccaagaacagaaaacaatagttcggtctggtctccaccctctcttaacttttgacatcaaggcacggataaacgctgtgattattgcagtactactggcccattcttgtccattataactgtgtgcagtgtgatgatggctgccaactatgatataccggtctggagatgtcaagcccattacaaatccaacaacattagtaactgttttcaattttgtgactgtctgaacttgcatgctgacgactcttatttcattatttggaagctctagagagctacacgcttcatttttggttctagcttttggcgaagagatcagttttgcaacgaggggtgcagagatgggctgcactaatagagaggtgaggtttgatcggctttgtctaaaactttcatcgacacttgggtaaccaggcgtagaagggtctcctcctggattcagtgacaccatgaaggtatcatggctaggattcacagtctttggcaaatcacaaggatcgatatacagaagaacacctccaaatccagccttttccaatgaggaaagcttataaagcagtggcaattttcctaatttcaggagtgcgatctgatttgttacgttttttattttcctaatcctttttaaatcatctgccattccataactcacatcgatgacttcagccttgagagttcctttggcagaataggctgcatatgaatagagcaggtcttggctgctatcttttctggcttcttcactgcaaggctggccattaggatgaaagcattgaccactgctgctcagagtcacagtgctgggagaagggcctggcagatcaagcagcacagagtaatttacaaactgtacatcttctaggcccaaagaggtccactgagtcttaatcttctttgaaatttccatgtcatcttcatttttatatagttgtaccaaatttctgaaagacttcttaatatcttctgcctggattgtcttgagaatctcttgatataactgaggatcaactgttcctgaagatggagcatctgaagggcaatttgtatgtacataataacctatcaaaatcccaaaaataaataaaatggtggctgtgcaaagtatttttaagacgtggcaaaagttgcagcgattgctctttggtgcagatcgtgtataatgggtaatgtagtcagattcttcttgaagtctctggaaccttcctttgggtgaagttgctggttgaatggaatcaagattgaggtctatagtctctgaatgccctaggttctgattctcagcaccgtctagctggaattggtcaaaaccagactcctctagttccttctccatgtcccactctaagtcaagggcagtggcttgaaggtcatcattgtctaagtactgtgagtgtcctggagctctttgatctgcatggaccttctgataggccatctttttacttcaattgaatgttcctagtgcaactggagggcttctgcaggttacaggagactgacaatctggacccagtcttcatccaggtgcctaatagtcaatgctcatttccctctgttaagttagtttccttcctcctcagtttttcacactcatttcaatatcttccatcttccttaagctttacataagaaataataatgtgtcataaatttctcaactaccaaaatacagaataaaataataattctgaatttttgtcttaaattccttctgcttttagagaaaaaggtgcttaaggtagatcttgtaaattcaccaatttagaagtgctatctaaatcttctttcttttctcacaaagaaagaactgcttgatgaggataacctaactaggctaatacatgaattaaatgcaacctagacttacctatcctcaaatgttatggaccggatgttggtgttttcccaaaattcgtatgttgaagccctaatctccaatgttataatatttggaggtgggtcctgagagtttgcacactctctctctgccatgtaagaacctgacaagaaggagacgatctgcaagagagcccttgaaaactggttggaactttgatcttggacttcccagtatccagaactggtgaaaataaattcctgttgtttaatccacccagtctgtgggattttgctatagcagctcaatcttcaaataaactctttagttcaataatgctattaccacattagtatggatacacacatgtgcatacctgcctatacacacacataattcaggacatttaatattatctcatttgtggagaataaaagaaatatggaatgaggaggattggaaatcactacctaattctcaaattttatttaagtgcctcaagattctattcatgggtaagggtatgcaagaaattaatgataattttagtacaaatgtgggtttctgctccccctcaacaccgaaaatgaaaaagtgaaaccaacccagtagtcccatagacaggttttggggttttctggataaatatggaaattgacccttctggtcttaaagcttgaagcttacatttgttttacctgaattt

SEQ ID NO: 12613 - RNA, 11247 nt, Homo sapiens
  source 1..11247: mol_type = other RNA
gatctcactttgttgcccaggctattttctggatgtctattaaaaaaaaattagtcctgcacagtgttctagaaagggtttttcttttcagaatatccatattctccaagtagcaagttagaatataaggaatatttgccattaaacctttctgttagaaatgtaaacatgaaattgcctaatatagacctatctcagatgctaaatagaattgtttataacacctttggaatataattatgtgagctacacttaaccatctggcattttgcttcctgcggacaatttgcaatagcatagaaaaatattttgtttgtgtatttcttatcaaacagatatgctaaagttctgtttagagagtaatagcattttattctaacttttaaaataaggtagtccatttgcagcagcttgatatataagtaaacaaaaatttttaatattaataaaacactagcacatacactgaaagcatctaagaaattcaaaatataaaacacttaccaagtaatgaccatatgagtggtaacatattgaataaaggccctttgaagaagttggagagttatgattactgagcaggctagataattaaataattacacattttgattgaaaaatatatgtagttcattaaaatagggactctaactccacttctctagctaagcttctattcagatgccacgtttgtactttaattagaacaaaagaccgacattaacttcaatgcaacataataattcataataatgattgtatattaatctcttgagcttgcaggaatatagcacatgacatatggcatgatacaggcacctgtgtgatcctttggggacttaggtggtgcatattaattagcccctggaaaataaaatctgtttccttctgagaaaagctacctcagtgcttattggcttaagccatcaaagaaattagatgaaatactgttaggctgggtctgcactcattaaagctttgtctagatgtaagcactgaatcaactgcctctgagttaagtcttgactgaatggtgcataagaaatcagagtaatcatgcatttctttggccttgatgattggattttggcatttaaaaaatccatcaaaattaccattttggttacagaaaattatgtaattgtataattcaaacaaaataatgtaaccagaaacactaaaatttgaagccacttcattttcctaaatgctgcttgaaactgcctcaatttaacccttttatttgtaaattcagattcaacccgaatatgagattataaatggcttaagaaatatgtcatcttgcaataatcagggtaacaagattcttgacggtcccaggtctgctaaaggcacttcagtgtgtatatctttgtcaggcaatggaacgatattatgaaactaaaactctggctgattaacagatcatttaaattgagactgatagatcttaaaattacttctcagggggaaaaagttacaatgctagagtgtacctagaaaacagaaacttgagtagacatggtaatgaccagaaaaggctatctttatacatttcttttgctacgcttcaaattcatgtcacctaaaagttgtgaagtgcacaaaacaaatctacttaactgaaaattattttcaatgaatgggatgtttagaactctgtgagggtttttaaggtcttttcgaatagcaaattctaatgaggcttttttaagttggcaatttaaactcatacaagaaataaaaactcaccagtgtggctgggcagaatatatatattttctcaaatattgtttgtttgttttttccctgcactgtatccatggtcccatgatgaaactgttatattgctgatatatttattggaatatgtgggccaacttcctttccactcaacatatggattggtagtttaaaataattcctttctattaagcaaatgtgtggctaaggcacatttaaatagcccattaaaccaatgagatgacaatgtgttaccctcagagaaagcttaatttttggagtaatcaattacacatatcacagaatgtctcatgagaacatttttggctaggtctaccaatttatcatacaaataattatagattttcatttgaggcaaagatgctgattcatcattagtaacatggtcacaaataatcatttattttatttttgttaacatctgtctttcctgtggggaaacttactatatgctctacgtttatttaatttaaaaagtcaattggttattctgaatttttaaaaataacataaaactgttgttctaaatcacagcacctgcttttctttttttagtgaaattatataagcatttagagaatgaaagtgtaagacttgtggtttctggtctctttttactgtttgtaagcctactcgtcatgatattccacaatggtgcacttgccttttaatgctcttatagatatcttcaaacttgcctacatatatacgcctttgttggagtgggctaccatcatcaggaatgatgtcatttgtttcttcaaactcctttattataccaaaaaagtgacagactccacagtctgatcagttttggagaaatatgttaacattttcaattatctcactttctagaatcaaaatagtctgattttttttttcggcactcagtgtaaagaacaaagaactgaatacagtgggcccagaagagaaatatgcctcatcatttttattagctttggaactgtggacaagtcactcaacctagttttctcattttgaaatgggttgttgtgggaattaaaaaaaaaaaaaaaaaaaaaaaaggatacatgggaaaaattctaaaacaccagtgcctgggatgtagcaggcacaaatataagctgcaactgaattgttttcttagagataaaatgggtccacttttcttttctcataatgattccattaataacaaatctttacgtctttcttgttattatgactcttcaatttatttagaaatgtcaattagtgttttcttggaaactacgattaacgtagattggaaattcttaaacttcagtgtgtgtaacagacatccagaaatcttgctgaagatgtagattcctagccctgtctttctaaatttcacattttgagaaacggtgatttagattgttgacttaacactggcctgacttgccctcttacagatatattttgctcaatgtccttcttcctgacttctggtgttctgtaaggattctccccactttctctcaagtacccagtctttgtgtcctttgcctgaattctcggggagagttttgtttgtcaggtacagtcagagaatgaactagccttgaattaaaagcagtgtttccagcccatgcaacatctgacagaatggctggttacatcgaatgcactggaaaagatcatttataaccctgtctcctcagggagaagcaagatatactgcatgagaaagcagagaagcttaaattccagtggtgcttttgttactaactaaatacatgactatgtccaagtttcttactcactttgggtttagttactatatctggtgggggtaattgataatgccttctctggctgaaggcaagatctcagggcttagaccagaatctttattaggctttcttttgattctgagacttatgcttttccataaagggcagtatctcatgtgtaccctgcctgaacataaatttcaccgttacacctttaccacattttcttcagagaatatttatgattcattatttcctaggcacaattctatgtatgaaagattgtgagaagtaccaggcatatagacgactcagcaacagcttaaacctactaccaattcacattaacacttgctattaatttgctcaggattttatttatttgaatctattgggggtggggaggggaggggagtgaaatgatatacatttggaggcaccctcaggtaatcacactatagaaataatgctgctagttaagaggtttgttgcaaagatgtaaagcagcatgtacagaatttgttggacgtctgctttaggtataatttaatatctccacgtatcttttaatagactaataaaaaaccatagttaactacagttttcaaatagcaaataacatataatttagaggtgaggaatacagaagaaggtttttatctatacagtgtgacttacctaggtacgcaatctttaaacaaaatgaagaagaaacatgttttctgttctcagtgctattgtaggttatgggaataaattaatttagaaatttgttctaaaataatgaactaccaaactgataatagcttgcctttatttgttttagtttcatctgtaagtgaataactggaatgaacacatcaacctttggttaaatataaggctttctagcttttgggcttacatgcacctgcttgtgtattcccacctcttttctgatgatctctgaagaggaagaaagagcatgaatgcctaggtatgcacaagcctatttatttctagacctttcctatacacactcttcaacatggcaaatgtttgcaaacaaatacattggttaaaaaaataatattgtaaggtagtttcatttttcatctaaaaatatgtgcacacaggcaatttcgatgaaaatggatttctgcttgaattatctagctaattgcctctattccctgctttgccttgagcatataaaaattatttagggtagacagtgttgaaccttataaatcaattaatcagtattgattaattatttcccctcaactttagtttgcctttaaactaagactaggtttatgctcatccataaaaagtgaaaatttaaacatacacagactgtctgcaatgtcactctggcggtgtatcatggggagatatgtttgaattagatagagaaaatttatatgaaatactctgaggctatgtttcctaaggggaattgctttatccagtataggaaaaccatttttcacataaatttctaaagataaattagaactttaacctgacacctaataggtagaattttagggtttgggggaataataatagttgctagagctattcaatggcaatgtcaatataaaaagcttagttttccacatgagagaagaactgaagtgtagacgagacactctcttacagtaacactgcagaaacttagaagcatgaatattttctagatttccatcttagtcacaattaaggataaagaagaaaaaatatgaaaagtttcttcataatattaaggggcttttattgataaaacaactatttctttcatagtaagttctttttgtcagaggcagaaatagaaatttgattctttagaagacattttgggtttcaaagagaaactctgctactttactgttgaaaatatatagtactctgagaaagctgccttacagcaaggagtttcagaaaagatacaagaaagaaaaccaatgtgagatgctttcattttagagtccctgcttcagtgtttccaacagaaacaagagaaaaagtaataagaaatatttttttctccctcttaagacatacatcactcctgaaattcttagaaaatcaactgaggcaaattaggggtttcaaagctagtcaccttgtaagttgttaggaaaaaaatttgcatttaaattgctctatgtagctcccttgagattttctcctggaatgcttatggctcttttttcattaatacttaaaaaaatacaatttcataaccagtgtattactacatctagttgtgttaagaagagaaacttcatttcataaaatagaaacattcaaagtggtttaggtcaaccaatcactcagtcagaatacttgaattcttcatattgaacacttaatagtgaagttaatctgaaccatatcaactctccatttcttttacagaaactaagtcattaatagctctatcagagagaataaactgtgttcctatatgccctccccataggaacaaagatagtccagaacttcttggaaatttttccttaaaatagtacatatttttatatatcagatttctttttaataggtaattcttaagtcctatttcaataacttgctttacatattcagaaatgtagatataagaaaaatattaaatgtgcaaaatgttctttctatatttacatttaaaaaatacaatgtaataatagctttatacttgtcaaaaagccattggggaaaataagccttcaatgtcagaaaatctggttaaattagagcttttgcttgtggaattgtaaacaaacttttaaaaatgctcagagttttctcaattcttcccatccaagacactcttgaacacatcaagtcctgctttgaagtaaacctgagctgaattaatgctgttcaacacctctgacagggcttcttgaagggtctcatttgatgcaaggggtttgcagtgttcccaagcctctataagtattgaaaaccggcttgtcttttcatcaaggtggtagaggatgtttctataaaaacctggtggtgcctgctttaccagaaagcttttctccatgtcttggagaatgtcattcagcatccggatgcggatgggtgctctctccttgggatcattagcaggtcgcatctcatcagactgaaaaagttcagcactctcccgcaggcgtaacgccatggctaacagttgatgagtgttgggttgatcacctttaaggttgttttgaacttctaaagctatatcaagtgcattaaagggcagaacaggttcgttggcaatttgcaaaatcacttctcctgagagcttagtaatggtttcatgaaggttgaaagagggatccatttcttcaatttttgttgctcgtgtagaaaaacgggcctcggagagaaaacttggaccctctaatgttttgatgtcctcgtaagcaaactgcacgatgggaactccaagatggttgatgaaataatcagcatcaccttgtatctgtatagaactgatattggtttctgggcactgggctcttctggtacagttgaaattatttttctctactaccagttgctgaagagatggtgatgctacaggatacagactagagttcccccttatgggactgtggaggctaatataagccacaacatttttctgaagaaccttcttgaaatcctctccccattcatatgagccaatattgccaaaagctgttcctccccaagaacagaaaacaatagttcggtctggtctccaccctctcttaacttttgacatcaaggcacggataaacgctgtgattattgcagtactactggcccattcttgtccattataactgtgtgcagtgtgatgatggctgccaactatgatataccggtctggagatgtcaagcccattacaaatccaacaacattagtaactgttttcaattttgtgactgtctgaacttgcatgctgacgactcttatttcattatttggaagctctagagagctacacgcttcatttttggttctagcttttggcgaagagatcagttttgcaacgaggggtgcagagatgggctgcactaatagagaggtgaggtttgatcggctttgtctaaaactttcatcgacacttgggtaaccaggcgtagaagggtctcctcctggattcagtgacaccatgaaggtatcatggctaggattcacagtctttggcaaatcacaaggatcgatatacagaagaacacctccaaatccagccttttccaatgaggaaagcttataaagcagtggcaattttcctaatttcaggagtgcgatctgatttgttacgttttttattttcctaatcctttttaaatcatctgccattccataactcacatcgatgacttcagccttgagagttcctttggcagaataggctgcatatgaatagagcaggtcttggctgctatcttttctggcttcttcactgcaaggctggccattaggatgaaagcattgaccactgctgctcagagtcacagtgctgggagaagggcctggcagatcaagcagcacagagtaatttacaaactgtacatcttctaggcccaaagaggtccactgagtcttaatcttctttgaaatttccatgtcatcttcatttttatatagttgtaccaaatttctgaaagacttcttaatatcttctgcctggattgtcttgagaatctcttgatataactgaggatcaactgttcctgaagatggagcatctgaagggcaatttgtatgtacataataacctatcaaaatcccaaaaataaataaaatggtggctgtgcaaagtatttttaagacgtggcaaaagttgcagcgattgctctttggtgcagatcgtgtataatgggtaatgtagtcagattcttcttgaagtctctggaaccttcctttgggtgaagttgctggttgaatggaatcaagattgaggtctatagtctctgaatgccctaggttctgattctcagcaccgtctagctggaattggtcaaaaccagactcctctagttccttctccatgtcccactctaagtcaagggcagtggcttgaaggtcatcattgtctaagtactgtgagtgtcctggagctctttgatctgcatggaccttctgataggccatctttttacttcaattgaatgttcctagtgcaactggagggcttctgcaggttacaggagactgacaatctggacccagtcttcatccaggtgcctaatagtcaatgctcatttcctgagcggcgcgggcgcgggctcgtctgcggtacggctgccgggccaggccggattttcagcagccgtaaagcgggagaagcgggcgcgagccgcggcgcgaaccctcgcccccgagcggcggccccggcgcctccgccgcgagcgtcagccgcttggcaaggaacgggctgggctgagtcataataaaagacgcgtttgtcgagccaagtgggaagaagagccgcgggcagcagtgttcaatggcacaagcctcaaaaattgggaaggattttttttttaatgggcaaaactggaaacttgcccccatggtgcccatcaaaagatatgtttcgtttataatttgcatatattttatacatagtctttgaatctaataaaacttttaaaagaatttttaaagcccattgcttgcagagccaaattcctggttatagcttcgtgacttacgcaagttacttgaattctgtgcttttgtttttcatccatgaaacaggataataaaggtacctccctcaagagagactgcgagagagcttggcatcctgcctgcacttagcactcgctaaatgttaattgttattttaaaataggagggaggagataataaagaggaacttagataacagttttgaatggaagaagatacgaatataaatcaagatttttcttttttcaagtggagtaaattagacaaattaccaatggaagagaagaaagtggagcctggaaggaacaaacggggctaagagaagtagctgaagcgagggaaggaagaagggggaaggaggaaagaagagaggaagaggggtgaataaaagcctccaaggaacaaacgaggctgaaagatgtggctgaaggtagggaaggaagaaaaagggaggaagagaggaagaaataaaaccaaggaagcaagaataaagctaggctgcgtgggaagaggggaggaaggaaggagagagaaattcaactaggctcagtggccaaaatgctgaagtgtgtcctgccgggagggagtggaggaatatgtttactcactatttagaaatgcatgacaaactccatccgctgagggagatttttacaatgtataaacagagaaacaactgtctaaaaatgagccccaaatgaggagcctttgctccagtgaatgagatttggcagttctgcaaaatgaggaaattcttccttgtgcggcatcttgaagggttgagtcatgaaacccacagcaaatattagtgggctggattcctgaaaggcatgccagatggacgcattctggttagttttactgtgtgatgttcccttctgtacttctgtcaattttagaagaaaagagtgtgaataaagatttgagaagtgaacttaaaagccaaactagttacttaatgtacgagtatccacccaccaggagcttacagttacagattccaaaacaagcaaccgtttctcccactttcattttccctcccctttgtttctactttcaccgtattgctttttatccatttttataatatgattttttacagtggaaccgcctacgggaaaggtgcttttaattaatacgaaagaatggaaggaatttcagctaggcctctctaagagggtaaagctttgtgaaagaaaggttttttagctgaagttttaatgagaataagagtagttggcagatgtgaaatcagaagttttttcagacaagaaaataatacgactcgagtgaaagggaatggactagaaatcagaaacagttctattccttaattaccgtaagaaccaaagactggaggaaagtttttcctattctataaagaaaaatgggggcctccctccaccagccagaccttcaaaaaaggaaaaaataaaaattaaaaacctctattagattcttgtaatgatttgctttttcttaggagaacttcttcagggtaaaagacgtgaaagtgcttctttcggcaacttctgacgaaatacttttgtagaagcaaaatttctgaagggataatttttgctcaagcaaaaaactattagtaagataagaatcccttttcctttgtttcaattttgctaagccttcaggctgaggcaaacagattatcattaaacctttattaatgtgaaaccaaaaaaagataaaatcttaaatgctgcgaagcccttaacctaaaaggagcaagaaaacaaaccaaggcccagaaaatagagaaagggattaggaagcctttctaaggggaacctttgaactgtgggctgtaaaatgaatgtctgtgacttgccttaaacaaataggcaatataaactaaagctgggaactaagaagatctcctcagatcagataaaaagcttaccttgtgtgaaacactgtggtcaaagaagaaaattcctttcatcttaagtggagacaaaaacgtgtatcacttgttttgtgtgtgctcataaaacacctccatcacctgaatcccttgggtgcaattttttgatggacttggcattctttaaa

SEQ ID NO: 12614 - RNA, 11379 nt, Homo sapiens
  source 1..11379: mol_type = other RNA
gatctcactttgttgcccaggctattttctggatgtctattaaaaaaaaattagtcctgcacagtgttctagaaagggtttttcttttcagaatatccatattctccaagtagcaagttagaatataaggaatatttgccattaaacctttctgttagaaatgtaaacatgaaattgcctaatatagacctatctcagatgctaaatagaattgtttataacacctttggaatataattatgtgagctacacttaaccatctggcattttgcttcctgcggacaatttgcaatagcatagaaaaatattttgtttgtgtatttcttatcaaacagatatgctaaagttctgtttagagagtaatagcattttattctaacttttaaaataaggtagtccatttgcagcagcttgatatataagtaaacaaaaatttttaatattaataaaacactagcacatacactgaaagcatctaagaaattcaaaatataaaacacttaccaagtaatgaccatatgagtggtaacatattgaataaaggccctttgaagaagttggagagttatgattactgagcaggctagataattaaataattacacattttgattgaaaaatatatgtagttcattaaaatagggactctaactccacttctctagctaagcttctattcagatgccacgtttgtactttaattagaacaaaagaccgacattaacttcaatgcaacataataattcataataatgattgtatattaatctcttgagcttgcaggaatatagcacatgacatatggcatgatacaggcacctgtgtgatcctttggggacttaggtggtgcatattaattagcccctggaaaataaaatctgtttccttctgagaaaagctacctcagtgcttattggcttaagccatcaaagaaattagatgaaatactgttaggctgggtctgcactcattaaagctttgtctagatgtaagcactgaatcaactgcctctgagttaagtcttgactgaatggtgcataagaaatcagagtaatcatgcatttctttggccttgatgattggattttggcatttaaaaaatccatcaaaattaccattttggttacagaaaattatgtaattgtataattcaaacaaaataatgtaaccagaaacactaaaatttgaagccacttcattttcctaaatgctgcttgaaactgcctcaatttaacccttttatttgtaaattcagattcaacccgaatatgagattataaatggcttaagaaatatgtcatcttgcaataatcagggtaacaagattcttgacggtcccaggtctgctaaaggcacttcagtgtgtatatctttgtcaggcaatggaacgatattatgaaactaaaactctggctgattaacagatcatttaaattgagactgatagatcttaaaattacttctcagggggaaaaagttacaatgctagagtgtacctagaaaacagaaacttgagtagacatggtaatgaccagaaaaggctatctttatacatttcttttgctacgcttcaaattcatgtcacctaaaagttgtgaagtgcacaaaacaaatctacttaactgaaaattattttcaatgaatgggatgtttagaactctgtgagggtttttaaggtcttttcgaatagcaaattctaatgaggcttttttaagttggcaatttaaactcatacaagaaataaaaactcaccagtgtggctgggcagaatatatatattttctcaaatattgtttgtttgttttttccctgcactgtatccatggtcccatgatgaaactgttatattgctgatatatttattggaatatgtgggccaacttcctttccactcaacatatggattggtagtttaaaataattcctttctattaagcaaatgtgtggctaaggcacatttaaatagcccattaaaccaatgagatgacaatgtgttaccctcagagaaagcttaatttttggagtaatcaattacacatatcacagaatgtctcatgagaacatttttggctaggtctaccaatttatcatacaaataattatagattttcatttgaggcaaagatgctgattcatcattagtaacatggtcacaaataatcatttattttatttttgttaacatctgtctttcctgtggggaaacttactatatgctctacgtttatttaatttaaaaagtcaattggttattctgaatttttaaaaataacataaaactgttgttctaaatcacagcacctgcttttctttttttagtgaaattatataagcatttagagaatgaaagtgtaagacttgtggtttctggtctctttttactgtttgtaagcctactcgtcatgatattccacaatggtgcacttgccttttaatgctcttatagatatcttcaaacttgcctacatatatacgcctttgttggagtgggctaccatcatcaggaatgatgtcatttgtttcttcaaactcctttattataccaaaaaagtgacagactccacagtctgatcagttttggagaaatatgttaacattttcaattatctcactttctagaatcaaaatagtctgattttttttttcggcactcagtgtaaagaacaaagaactgaatacagtgggcccagaagagaaatatgcctcatcatttttattagctttggaactgtggacaagtcactcaacctagttttctcattttgaaatgggttgttgtgggaattaaaaaaaaaaaaaaaaaaaaaaaaggatacatgggaaaaattctaaaacaccagtgcctgggatgtagcaggcacaaatataagctgcaactgaattgttttcttagagataaaatgggtccacttttcttttctcataatgattccattaataacaaatctttacgtctttcttgttattatgactcttcaatttatttagaaatgtcaattagtgttttcttggaaactacgattaacgtagattggaaattcttaaacttcagtgtgtgtaacagacatccagaaatcttgctgaagatgtagattcctagccctgtctttctaaatttcacattttgagaaacggtgatttagattgttgacttaacactggcctgacttgccctcttacagatatattttgctcaatgtccttcttcctgacttctggtgttctgtaaggattctccccactttctctcaagtacccagtctttgtgtcctttgcctgaattctcggggagagttttgtttgtcaggtacagtcagagaatgaactagccttgaattaaaagcagtgtttccagcccatgcaacatctgacagaatggctggttacatcgaatgcactggaaaagatcatttataaccctgtctcctcagggagaagcaagatatactgcatgagaaagcagagaagcttaaattccagtggtgcttttgttactaactaaatacatgactatgtccaagtttcttactcactttgggtttagttactatatctggtgggggtaattgataatgccttctctggctgaaggcaagatctcagggcttagaccagaatctttattaggctttcttttgattctgagacttatgcttttccataaagggcagtatctcatgtgtaccctgcctgaacataaatttcaccgttacacctttaccacattttcttcagagaatatttatgattcattatttcctaggcacaattctatgtatgaaagattgtgagaagtaccaggcatatagacgactcagcaacagcttaaacctactaccaattcacattaacacttgctattaatttgctcaggattttatttatttgaatctattgggggtggggaggggaggggagtgaaatgatatacatttggaggcaccctcaggtaatcacactatagaaataatgctgctagttaagaggtttgttgcaaagatgtaaagcagcatgtacagaatttgttggacgtctgctttaggtataatttaatatctccacgtatcttttaatagactaataaaaaaccatagttaactacagttttcaaatagcaaataacatataatttagaggtgaggaatacagaagaaggtttttatctatacagtgtgacttacctaggtacgcaatctttaaacaaaatgaagaagaaacatgttttctgttctcagtgctattgtaggttatgggaataaattaatttagaaatttgttctaaaataatgaactaccaaactgataatagcttgcctttatttgttttagtttcatctgtaagtgaataactggaatgaacacatcaacctttggttaaatataaggctttctagcttttgggcttacatgcacctgcttgtgtattcccacctcttttctgatgatctctgaagaggaagaaagagcatgaatgcctaggtatgcacaagcctatttatttctagacctttcctatacacactcttcaacatggcaaatgtttgcaaacaaatacattggttaaaaaaataatattgtaaggtagtttcatttttcatctaaaaatatgtgcacacaggcaatttcgatgaaaatggatttctgcttgaattatctagctaattgcctctattccctgctttgccttgagcatataaaaattatttagggtagacagtgttgaaccttataaatcaattaatcagtattgattaattatttcccctcaactttagtttgcctttaaactaagactaggtttatgctcatccataaaaagtgaaaatttaaacatacacagactgtctgcaatgtcactctggcggtgtatcatggggagatatgtttgaattagatagagaaaatttatatgaaatactctgaggctatgtttcctaaggggaattgctttatccagtataggaaaaccatttttcacataaatttctaaagataaattagaactttaacctgacacctaataggtagaattttagggtttgggggaataataatagttgctagagctattcaatggcaatgtcaatataaaaagcttagttttccacatgagagaagaactgaagtgtagacgagacactctcttacagtaacactgcagaaacttagaagcatgaatattttctagatttccatcttagtcacaattaaggataaagaagaaaaaatatgaaaagtttcttcataatattaaggggcttttattgataaaacaactatttctttcatagtaagttctttttgtcagaggcagaaatagaaatttgattctttagaagacattttgggtttcaaagagaaactctgctactttactgttgaaaatatatagtactctgagaaagctgccttacagcaaggagtttcagaaaagatacaagaaagaaaaccaatgtgagatgctttcattttagagtccctgcttcagtgtttccaacagaaacaagagaaaaagtaataagaaatatttttttctccctcttaagacatacatcactcctgaaattcttagaaaatcaactgaggcaaattaggggtttcaaagctagtcaccttgtaagttgttaggaaaaaaatttgcatttaaattgctctatgtagctcccttgagattttctcctggaatgcttatggctcttttttcattaatacttaaaaaaatacaatttcataaccagtgtattactacatctagttgtgttaagaagagaaacttcatttcataaaatagaaacattcaaagtggtttaggtcaaccaatcactcagtcagaatacttgaattcttcatattgaacacttaatagtgaagttaatctgaaccatatcaactctccatttcttttacagaaactaagtcattaatagctctatcagagagaataaactgtgttcctatatgccctccccataggaacaaagatagtccagaacttcttggaaatttttccttaaaatagtacatatttttatatatcagatttctttttaataggtaattcttaagtcctatttcaataacttgctttacatattcagaaatgtagatataagaaaaatattaaatgtgcaaaatgttctttctatatttacatttaaaaaatacaatgtaataatagctttatacttgtcaaaaagccattggggaaaataagccttcaatgtcagaaaatctggttaaattagagcttttgcttgtggaattgtaaacaaacttttaaaaatgctcagagttttctcaattcttcccatccaagacactcttgaacacatcaagtcctgctttgaagtaaacctgagctgaattaatgctgttcaacacctctgacagggcttcttgaagggtctcatttgatgcaaggggtttgcagtgttcccaagcctctataagtattgaaaaccggcttgtcttttcatcaaggtggtagaggatgtttctataaaaacctggtggtgcctgctttaccagaaagcttttctccatgtcttggagaatgtcattcagcatccggatgcggatgggtgctctctccttgggatcattagcaggtcgcatctcatcagactgaaaaagttcagcactctcccgcaggcgtaacgccatggctaacagttgatgagtgttgggttgatcacctttaaggttgttttgaacttctaaagctatatcaagtgcattaaagggcagaacaggttcgttggcaatttgcaaaatcacttctcctgagagcttagtaatggtttcatgaaggttgaaagagggatccatttcttcaatttttgttgctcgtgtagaaaaacgggcctcggagagaaaacttggaccctctaatgttttgatgtcctcgtaagcaaactgcacgatgggaactccaagatggttgatgaaataatcagcatcaccttgtatctgtatagaactgatattggtttctgggcactgggctcttctggtacagttgaaattatttttctctactaccagttgctgaagagatggtgatgctacaggatacagactagagttcccccttatgggactgtggaggctaatataagccacaacatttttctgaagaaccttcttgaaatcctctccccattcatatgagccaatattgccaaaagctgttcctccccaagaacagaaaacaatagttcggtctggtctccaccctctcttaacttttgacatcaaggcacggataaacgctgtgattattgcagtactactggcccattcttgtccattataactgtgtgcagtgtgatgatggctgccaactatgatataccggtctggagatgtcaagcccattacaaatccaacaacattagtaactgttttcaattttgtgactgtctgaacttgcatgctgacgactcttatttcattatttggaagctctagagagctacacgcttcatttttggttctagcttttggcgaagagatcagttttgcaacgaggggtgcagagatgggctgcactaatagagaggtgaggtttgatcggctttgtctaaaactttcatcgacacttgggtaaccaggcgtagaagggtctcctcctggattcagtgacaccatgaaggtatcatggctaggattcacagtctttggcaaatcacaaggatcgatatacagaagaacacctccaaatccagccttttccaatgaggaaagcttataaagcagtggcaattttcctaatttcaggagtgcgatctgatttgttacgttttttattttcctaatcctttttaaatcatctgccattccataactcacatcgatgacttcagccttgagagttcctttggcagaataggctgcatatgaatagagcaggtcttggctgctatcttttctggcttcttcactgcaaggctggccattaggatgaaagcattgaccactgctgctcagagtcacagtgctgggagaagggcctggcagatcaagcagcacagagtaatttacaaactgtacatcttctaggcccaaagaggtccactgagtcttaatcttctttgaaatttccatgtcatcttcatttttatatagttgtaccaaatttctgaaagacttcttaatatcttctgcctggattgtcttgagaatctcttgatataactgaggatcaactgttcctgaagatggagcatctgaagggcaatttgtatgtacataataacctatcaaaatcccaaaaataaataaaatggtggctgtgcaaagtatttttaagacgtggcaaaagttgcagcgattgctctttggtgcagatcgtgtataatgggtaatgtagtcagattcttcttgaagtctctggaaccttcctttgggtgaagttgctggttgaatggaatcaagattgaggtctatagtctctgaatgccctaggttctgattctcagcaccgtctagctggaattggtcaaaaccagactcctctagttccttctccatgtcccactctaagtcaagggcagtggcttgaaggtcatcattgtctaagtactgtgagtgtcctggagctctttgatctgcatggaccttctgataggccatctttttacttcaattgaatgttcctagtgcaactggagggcttctgcaggttacaggagactgacaatctggacccagtcttcatccaggtgcctaatagtcaatgctcatttccttgtttttaatcgttttctttatagaaactaaatttcatttaaattattcttttcttccctcagcctcctagggttgaataaaagacgccctaagacatcaaaagctattttgaacgtccagctgggagatctgagcggcgcgggcgcgggctcgtctgcggtacggctgccgggccaggccggattttcagcagccgtaaagcgggagaagcgggcgcgagccgcggcgcgaaccctcgcccccgagcggcggccccggcgcctccgccgcgagcgtcagccgcttggcaaggaacgggctgggctgagtcataataaaagacgcgtttgtcgagccaagtgggaagaagagccgcgggcagcagtgttcaatggcacaagcctcaaaaattgggaaggattttttttttaatgggcaaaactggaaacttgcccccatggtgcccatcaaaagatatgtttcgtttataatttgcatatattttatacatagtctttgaatctaataaaacttttaaaagaatttttaaagcccattgcttgcagagccaaattcctggttatagcttcgtgacttacgcaagttacttgaattctgtgcttttgtttttcatccatgaaacaggataataaaggtacctccctcaagagagactgcgagagagcttggcatcctgcctgcacttagcactcgctaaatgttaattgttattttaaaataggagggaggagataataaagaggaacttagataacagttttgaatggaagaagatacgaatataaatcaagatttttcttttttcaagtggagtaaattagacaaattaccaatggaagagaagaaagtggagcctggaaggaacaaacggggctaagagaagtagctgaagcgagggaaggaagaagggggaaggaggaaagaagagaggaagaggggtgaataaaagcctccaaggaacaaacgaggctgaaagatgtggctgaaggtagggaaggaagaaaaagggaggaagagaggaagaaataaaaccaaggaagcaagaataaagctaggctgcgtgggaagaggggaggaaggaaggagagagaaattcaactaggctcagtggccaaaatgctgaagtgtgtcctgccgggagggagtggaggaatatgtttactcactatttagaaatgcatgacaaactccatccgctgagggagatttttacaatgtataaacagagaaacaactgtctaaaaatgagccccaaatgaggagcctttgctccagtgaatgagatttggcagttctgcaaaatgaggaaattcttccttgtgcggcatcttgaagggttgagtcatgaaacccacagcaaatattagtgggctggattcctgaaaggcatgccagatggacgcattctggttagttttactgtgtgatgttcccttctgtacttctgtcaattttagaagaaaagagtgtgaataaagatttgagaagtgaacttaaaagccaaactagttacttaatgtacgagtatccacccaccaggagcttacagttacagattccaaaacaagcaaccgtttctcccactttcattttccctcccctttgtttctactttcaccgtattgctttttatccatttttataatatgattttttacagtggaaccgcctacgggaaaggtgcttttaattaatacgaaagaatggaaggaatttcagctaggcctctctaagagggtaaagctttgtgaaagaaaggttttttagctgaagttttaatgagaataagagtagttggcagatgtgaaatcagaagttttttcagacaagaaaataatacgactcgagtgaaagggaatggactagaaatcagaaacagttctattccttaattaccgtaagaaccaaagactggaggaaagtttttcctattctataaagaaaaatgggggcctccctccaccagccagaccttcaaaaaaggaaaaaataaaaattaaaaacctctattagattcttgtaatgatttgctttttcttaggagaacttcttcagggtaaaagacgtgaaagtgcttctttcggcaacttctgacgaaatacttttgtagaagcaaaatttctgaagggataatttttgctcaagcaaaaaactattagtaagataagaatcccttttcctttgtttcaattttgctaagccttcaggctgaggcaaacagattatcattaaacctttattaatgtgaaaccaaaaaaagataaaatcttaaatgctgcgaagcccttaacctaaaaggagcaagaaaacaaaccaaggcccagaaaatagagaaagggattaggaagcctttctaaggggaacctttgaactgtgggctgtaaaatgaatgtctgtgacttgccttaaacaaataggcaatataaactaaagctgggaactaagaagatctcctcagatcagataaaaagcttaccttgtgtgaaacactgtggtcaaagaagaaaattcctttcatcttaagtggagacaaaaacgtgtatcacttgttttgtgtgtgctcataaaacacctccatcacctgaatcccttgggtgcaattttttgatggacttggcattctttaaa

SEQ ID NO: 12615 - RNA, 9297 nt, Homo sapiens
  source 1..9297: mol_type = other RNA
gatctcactttgttgcccaggctattttctggatgtctattaaaaaaaaattagtcctgcacagtgttctagaaagggtttttcttttcagaatatccatattctccaagtagcaagttagaatataaggaatatttgccattaaacctttctgttagaaatgtaaacatgaaattgcctaatatagacctatctcagatgctaaatagaattgtttataacacctttggaatataattatgtgagctacacttaaccatctggcattttgcttcctgcggacaatttgcaatagcatagaaaaatattttgtttgtgtatttcttatcaaacagatatgctaaagttctgtttagagagtaatagcattttattctaacttttaaaataaggtagtccatttgcagcagcttgatatataagtaaacaaaaatttttaatattaataaaacactagcacatacactgaaagcatctaagaaattcaaaatataaaacacttaccaagtaatgaccatatgagtggtaacatattgaataaaggccctttgaagaagttggagagttatgattactgagcaggctagataattaaataattacacattttgattgaaaaatatatgtagttcattaaaatagggactctaactccacttctctagctaagcttctattcagatgccacgtttgtactttaattagaacaaaagaccgacattaacttcaatgcaacataataattcataataatgattgtatattaatctcttgagcttgcaggaatatagcacatgacatatggcatgatacaggcacctgtgtgatcctttggggacttaggtggtgcatattaattagcccctggaaaataaaatctgtttccttctgagaaaagctacctcagtgcttattggcttaagccatcaaagaaattagatgaaatactgttaggctgggtctgcactcattaaagctttgtctagatgtaagcactgaatcaactgcctctgagttaagtcttgactgaatggtgcataagaaatcagagtaatcatgcatttctttggccttgatgattggattttggcatttaaaaaatccatcaaaattaccattttggttacagaaaattatgtaattgtataattcaaacaaaataatgtaaccagaaacactaaaatttgaagccacttcattttcctaaatgctgcttgaaactgcctcaatttaacccttttatttgtaaattcagattcaacccgaatatgagattataaatggcttaagaaatatgtcatcttgcaataatcagggtaacaagattcttgacggtcccaggtctgctaaaggcacttcagtgtgtatatctttgtcaggcaatggaacgatattatgaaactaaaactctggctgattaacagatcatttaaattgagactgatagatcttaaaattacttctcagggggaaaaagttacaatgctagagtgtacctagaaaacagaaacttgagtagacatggtaatgaccagaaaaggctatctttatacatttcttttgctacgcttcaaattcatgtcacctaaaagttgtgaagtgcacaaaacaaatctacttaactgaaaattattttcaatgaatgggatgtttagaactctgtgagggtttttaaggtcttttcgaatagcaaattctaatgaggcttttttaagttggcaatttaaactcatacaagaaataaaaactcaccagtgtggctgggcagaatatatatattttctcaaatattgtttgtttgttttttccctgcactgtatccatggtcccatgatgaaactgttatattgctgatatatttattggaatatgtgggccaacttcctttccactcaacatatggattggtagtttaaaataattcctttctattaagcaaatgtgtggctaaggcacatttaaatagcccattaaaccaatgagatgacaatgtgttaccctcagagaaagcttaatttttggagtaatcaattacacatatcacagaatgtctcatgagaacatttttggctaggtctaccaatttatcatacaaataattatagattttcatttgaggcaaagatgctgattcatcattagtaacatggtcacaaataatcatttattttatttttgttaacatctgtctttcctgtggggaaacttactatatgctctacgtttatttaatttaaaaagtcaattggttattctgaatttttaaaaataacataaaactgttgttctaaatcacagcacctgcttttctttttttagtgaaattatataagcatttagagaatgaaagtgtaagacttgtggtttctggtctctttttactgtttgtaagcctactcgtcatgatattccacaatggtgcacttgccttttaatgctcttatagatatcttcaaacttgcctacatatatacgcctttgttggagtgggctaccatcatcaggaatgatgtcatttgtttcttcaaactcctttattataccaaaaaagtgacagactccacagtctgatcagttttggagaaatatgttaacattttcaattatctcactttctagaatcaaaatagtctgattttttttttcggcactcagtgtaaagaacaaagaactgaatacagtgggcccagaagagaaatatgcctcatcatttttattagctttggaactgtggacaagtcactcaacctagttttctcattttgaaatgggttgttgtgggaattaaaaaaaaaaaaaaaaaaaaaaaaggatacatgggaaaaattctaaaacaccagtgcctgggatgtagcaggcacaaatataagctgcaactgaattgttttcttagagataaaatgggtccacttttcttttctcataatgattccattaataacaaatctttacgtctttcttgttattatgactcttcaatttatttagaaatgtcaattagtgttttcttggaaactacgattaacgtagattggaaattcttaaacttcagtgtgtgtaacagacatccagaaatcttgctgaagatgtagattcctagccctgtctttctaaatttcacattttgagaaacggtgatttagattgttgacttaacactggcctgacttgccctcttacagatatattttgctcaatgtccttcttcctgacttctggtgttctgtaaggattctccccactttctctcaagtacccagtctttgtgtcctttgcctgaattctcggggagagttttgtttgtcaggtacagtcagagaatgaactagccttgaattaaaagcagtgtttccagcccatgcaacatctgacagaatggctggttacatcgaatgcactggaaaagatcatttataaccctgtctcctcagggagaagcaagatatactgcatgagaaagcagagaagcttaaattccagtggtgcttttgttactaactaaatacatgactatgtccaagtttcttactcactttgggtttagttactatatctggtgggggtaattgataatgccttctctggctgaaggcaagatctcagggcttagaccagaatctttattaggctttcttttgattctgagacttatgcttttccataaagggcagtatctcatgtgtaccctgcctgaacataaatttcaccgttacacctttaccacattttcttcagagaatatttatgattcattatttcctaggcacaattctatgtatgaaagattgtgagaagtaccaggcatatagacgactcagcaacagcttaaacctactaccaattcacattaacacttgctattaatttgctcaggattttatttatttgaatctattgggggtggggaggggaggggagtgaaatgatatacatttggaggcaccctcaggtaatcacactatagaaataatgctgctagttaagaggtttgttgcaaagatgtaaagcagcatgtacagaatttgttggacgtctgctttaggtataatttaatatctccacgtatcttttaatagactaataaaaaaccatagttaactacagttttcaaatagcaaataacatataatttagaggtgaggaatacagaagaaggtttttatctatacagtgtgacttacctaggtacgcaatctttaaacaaaatgaagaagaaacatgttttctgttctcagtgctattgtaggttatgggaataaattaatttagaaatttgttctaaaataatgaactaccaaactgataatagcttgcctttatttgttttagtttcatctgtaagtgaataactggaatgaacacatcaacctttggttaaatataaggctttctagcttttgggcttacatgcacctgcttgtgtattcccacctcttttctgatgatctctgaagaggaagaaagagcatgaatgcctaggtatgcacaagcctatttatttctagacctttcctatacacactcttcaacatggcaaatgtttgcaaacaaatacattggttaaaaaaataatattgtaaggtagtttcatttttcatctaaaaatatgtgcacacaggcaatttcgatgaaaatggatttctgcttgaattatctagctaattgcctctattccctgctttgccttgagcatataaaaattatttagggtagacagtgttgaaccttataaatcaattaatcagtattgattaattatttcccctcaactttagtttgcctttaaactaagactaggtttatgctcatccataaaaagtgaaaatttaaacatacacagactgtctgcaatgtcactctggcggtgtatcatggggagatatgtttgaattagatagagaaaatttatatgaaatactctgaggctatgtttcctaaggggaattgctttatccagtataggaaaaccatttttcacataaatttctaaagataaattagaactttaacctgacacctaataggtagaattttagggtttgggggaataataatagttgctagagctattcaatggcaatgtcaatataaaaagcttagttttccacatgagagaagaactgaagtgtagacgagacactctcttacagtaacactgcagaaacttagaagcatgaatattttctagatttccatcttagtcacaattaaggataaagaagaaaaaatatgaaaagtttcttcataatattaaggggcttttattgataaaacaactatttctttcatagtaagttctttttgtcagaggcagaaatagaaatttgattctttagaagacattttgggtttcaaagagaaactctgctactttactgttgaaaatatatagtactctgagaaagctgccttacagcaaggagtttcagaaaagatacaagaaagaaaaccaatgtgagatgctttcattttagagtccctgcttcagtgtttccaacagaaacaagagaaaaagtaataagaaatatttttttctccctcttaagacatacatcactcctgaaattcttagaaaatcaactgaggcaaattaggggtttcaaagctagtcaccttgtaagttgttaggaaaaaaatttgcatttaaattgctctatgtagctcccttgagattttctcctggaatgcttatggctcttttttcattaatacttaaaaaaatacaatttcataaccagtgtattactacatctagttgtgttaagaagagaaacttcatttcataaaatagaaacattcaaagtggtttaggtcaaccaatcactcagtcagaatacttgaattcttcatattgaacacttaatagtgaagttaatctgaaccatatcaactctccatttcttttacagaaactaagtcattaatagctctatcagagagaataaactgtgttcctatatgccctccccataggaacaaagatagtccagaacttcttggaaatttttccttaaaatagtacatatttttatatatcagatttctttttaataggtaattcttaagtcctatttcaataacttgctttacatattcagaaatgtagatataagaaaaatattaaatgtgcaaaatgttctttctatatttacatttaaaaaatacaatgtaataatagctttatacttgtcaaaaagccattggggaaaataagccttcaatgtcagaaaatctggttaaattagagcttttgcttgtggaattgtaaacaaacttttaaaaatgctcagagttttctcaattcttcccatccaagacactcttgaacacatcaagtcctgctttgaagtaaacctgagctgaattaatgctgttcaacacctctgacagggcttcttgaagggtctcatttgatgcaaggggtttgcagtgttcccaagcctctataagtattgaaaaccggcttgtcttttcatcaaggtggtagaggatgtttctataaaaacctggtggtgcctgctttaccagaaagcttttctccatgtcttggagaatgtcattcagcatccggatgcggatgggtgctctctccttgggatcattagcaggtcgcatctcatcagactgaaaaagttcagcactctcccgcaggcgtaacgccatggctaacagttgatgagtgttgggttgatcacctttaaggttgttttgaacttctaaagctatatcaagtgcattaaagggcagaacaggttcgttggcaatttgcaaaatcacttctcctgagagcttagtaatggtttcatgaaggttgaaagagggatccatttcttcaatttttgttgctcgtgtagaaaaacgggcctcggagagaaaacttggaccctctaatgttttgatgtcctcgtaagcaaactgcacgatgggaactccaagatggttgatgaaataatcagcatcaccttgtatctgtatagaactgatattggtttctgggcactgggctcttctggtacagttgaaattatttttctctactaccagttgctgaagagatggtgatgctacaggatacagactagagttcccccttatgggactgtggaggctaatataagccacaacatttttctgaagaaccttcttgaaatcctctccccattcatatgagccaatattgccaaaagctgttcctccccaagaacagaaaacaatagttcggtctggtctccaccctctcttaacttttgacatcaaggcacggataaacgctgtgattattgcagtactactggcccattcttgtccattataactgtgtgcagtgtgatgatggctgccaactatgatataccggtctggagatgtcaagcccattacaaatccaacaacattagtaactgttttcaattttgtgactgtctgaacttgcatgctgacgactcttatttcattatttggaagctctagagagctacacgcttcatttttggttctagcttttggcgaagagatcagttttgcaacgaggggtgcagagatgggctgcactaatagagaggtgaggtttgatcggctttgtctaaaactttcatcgacacttgggtaaccaggcgtagaagggtctcctcctggattcagtgacaccatgaaggtatcatggctaggattcacagtctttggcaaatcacaaggatcgatatacagaagaacacctccaaatccagccttttccaatgaggaaagcttataaagcagtggcaattttcctaatttcaggagtgcgatctgatttgttacgttttttattttcctaatcctttttaaatcatctgccattccataactcacatcgatgacttcagccttgagagttcctttggcagaataggctgcatatgaatagagcaggtcttggctgctatcttttctggcttcttcactgcaaggctggccattaggatgaaagcattgaccactgctgctcagagtcacagtgctgggagaagggcctggcagatcaagcagcacagagtaatttacaaactgtacatcttctaggcccaaagaggtccactgagtcttaatcttctttgaaatttccatgtcatcttcatttttatatagttgtaccaaatttctgaaagacttcttaatatcttctgcctggattgtcttgagaatctcttgatataactgaggatcaactgttcctgaagatggagcatctgaagggcaatttgtatgtacataataacctatcaaaatcccaaaaataaataaaatggtggctgtgcaaagtatttttaagacgtggcaaaagttgcagcgattgctctttggtgcagatcgtgtataatgggtaatgtagtcagattcttcttgaagtctctggaaccttcctttgggtgaagttgctggttgaatggaatcaagattgaggtctatagtctctgaatgccctaggttctgattctcagcaccgtctagctggaattggtcaaaaccagactcctctagttccttctccatgtcccactctaagtcaagggcagtggcttgaaggtcatcattgtctaagtactgtgagtgtcctggagctctttgatctgcatggaccttctgataggccatctttttacttcaattgaatgttcctagtgcaactggagggcttctgcaggttacaggagactgacaatctggacccagtcttcatccaggtgcctaatagtcaatgctcatttccttgtttttaatcgttttctttatagaaactaaatttcatttaaattattcttttcttccctcagcctcctagggttgaataaaagacgccctaagacatcaaaagctattttgaacgtccagctgggagatctgtaaatgaatgatagaaagttcgaaaatcctcacaaaagattgactctcagtgaactttgctcctgataaattctacccacaatgtttattcaaatttagttttaaaaagagaaagcagactttggagagatggcctttacgtggattttatttgctgatgataatgatgatgcacagtgcctcttcacaagattacatgagttaaaaggtaatcccactatcactcttgcaccgatgagtgctctacttgagtgctgatctcaatttttgactccaagctttattacaggaaagcttaaacgaaatgcatttgtgtaagagatgtagatacaaacttcagaatattcatgttaaccatcattgatctctgctttgatggaggtgatttttgatgtaaaataagccgaaattaca

SEQ ID NO: 12616 - RNA, 8855 nt, Homo sapiens
  source 1..8855: mol_type = other RNA
gatctcactttgttgcccaggctattttctggatgtctattaaaaaaaaattagtcctgcacagtgttctagaaagggtttttcttttcagaatatccatattctccaagtagcaagttagaatataaggaatatttgccattaaacctttctgttagaaatgtaaacatgaaattgcctaatatagacctatctcagatgctaaatagaattgtttataacacctttggaatataattatgtgagctacacttaaccatctggcattttgcttcctgcggacaatttgcaatagcatagaaaaatattttgtttgtgtatttcttatcaaacagatatgctaaagttctgtttagagagtaatagcattttattctaacttttaaaataaggtagtccatttgcagcagcttgatatataagtaaacaaaaatttttaatattaataaaacactagcacatacactgaaagcatctaagaaattcaaaatataaaacacttaccaagtaatgaccatatgagtggtaacatattgaataaaggccctttgaagaagttggagagttatgattactgagcaggctagataattaaataattacacattttgattgaaaaatatatgtagttcattaaaatagggactctaactccacttctctagctaagcttctattcagatgccacgtttgtactttaattagaacaaaagaccgacattaacttcaatgcaacataataattcataataatgattgtatattaatctcttgagcttgcaggaatatagcacatgacatatggcatgatacaggcacctgtgtgatcctttggggacttaggtggtgcatattaattagcccctggaaaataaaatctgtttccttctgagaaaagctacctcagtgcttattggcttaagccatcaaagaaattagatgaaatactgttaggctgggtctgcactcattaaagctttgtctagatgtaagcactgaatcaactgcctctgagttaagtcttgactgaatggtgcataagaaatcagagtaatcatgcatttctttggccttgatgattggattttggcatttaaaaaatccatcaaaattaccattttggttacagaaaattatgtaattgtataattcaaacaaaataatgtaaccagaaacactaaaatttgaagccacttcattttcctaaatgctgcttgaaactgcctcaatttaacccttttatttgtaaattcagattcaacccgaatatgagattataaatggcttaagaaatatgtcatcttgcaataatcagggtaacaagattcttgacggtcccaggtctgctaaaggcacttcagtgtgtatatctttgtcaggcaatggaacgatattatgaaactaaaactctggctgattaacagatcatttaaattgagactgatagatcttaaaattacttctcagggggaaaaagttacaatgctagagtgtacctagaaaacagaaacttgagtagacatggtaatgaccagaaaaggctatctttatacatttcttttgctacgcttcaaattcatgtcacctaaaagttgtgaagtgcacaaaacaaatctacttaactgaaaattattttcaatgaatgggatgtttagaactctgtgagggtttttaaggtcttttcgaatagcaaattctaatgaggcttttttaagttggcaatttaaactcatacaagaaataaaaactcaccagtgtggctgggcagaatatatatattttctcaaatattgtttgtttgttttttccctgcactgtatccatggtcccatgatgaaactgttatattgctgatatatttattggaatatgtgggccaacttcctttccactcaacatatggattggtagtttaaaataattcctttctattaagcaaatgtgtggctaaggcacatttaaatagcccattaaaccaatgagatgacaatgtgttaccctcagagaaagcttaatttttggagtaatcaattacacatatcacagaatgtctcatgagaacatttttggctaggtctaccaatttatcatacaaataattatagattttcatttgaggcaaagatgctgattcatcattagtaacatggtcacaaataatcatttattttatttttgttaacatctgtctttcctgtggggaaacttactatatgctctacgtttatttaatttaaaaagtcaattggttattctgaatttttaaaaataacataaaactgttgttctaaatcacagcacctgcttttctttttttagtgaaattatataagcatttagagaatgaaagtgtaagacttgtggtttctggtctctttttactgtttgtaagcctactcgtcatgatattccacaatggtgcacttgccttttaatgctcttatagatatcttcaaacttgcctacatatatacgcctttgttggagtgggctaccatcatcaggaatgatgtcatttgtttcttcaaactcctttattataccaaaaaagtgacagactccacagtctgatcagttttggagaaatatgttaacattttcaattatctcactttctagaatcaaaatagtctgattttttttttcggcactcagtgtaaagaacaaagaactgaatacagtgggcccagaagagaaatatgcctcatcatttttattagctttggaactgtggacaagtcactcaacctagttttctcattttgaaatgggttgttgtgggaattaaaaaaaaaaaaaaaaaaaaaaaaggatacatgggaaaaattctaaaacaccagtgcctgggatgtagcaggcacaaatataagctgcaactgaattgttttcttagagataaaatgggtccacttttcttttctcataatgattccattaataacaaatctttacgtctttcttgttattatgactcttcaatttatttagaaatgtcaattagtgttttcttggaaactacgattaacgtagattggaaattcttaaacttcagtgtgtgtaacagacatccagaaatcttgctgaagatgtagattcctagccctgtctttctaaatttcacattttgagaaacggtgatttagattgttgacttaacactggcctgacttgccctcttacagatatattttgctcaatgtccttcttcctgacttctggtgttctgtaaggattctccccactttctctcaagtacccagtctttgtgtcctttgcctgaattctcggggagagttttgtttgtcaggtacagtcagagaatgaactagccttgaattaaaagcagtgtttccagcccatgcaacatctgacagaatggctggttacatcgaatgcactggaaaagatcatttataaccctgtctcctcagggagaagcaagatatactgcatgagaaagcagagaagcttaaattccagtggtgcttttgttactaactaaatacatgactatgtccaagtttcttactcactttgggtttagttactatatctggtgggggtaattgataatgccttctctggctgaaggcaagatctcagggcttagaccagaatctttattaggctttcttttgattctgagacttatgcttttccataaagggcagtatctcatgtgtaccctgcctgaacataaatttcaccgttacacctttaccacattttcttcagagaatatttatgattcattatttcctaggcacaattctatgtatgaaagattgtgagaagtaccaggcatatagacgactcagcaacagcttaaacctactaccaattcacattaacacttgctattaatttgctcaggattttatttatttgaatctattgggggtggggaggggaggggagtgaaatgatatacatttggaggcaccctcaggtaatcacactatagaaataatgctgctagttaagaggtttgttgcaaagatgtaaagcagcatgtacagaatttgttggacgtctgctttaggtataatttaatatctccacgtatcttttaatagactaataaaaaaccatagttaactacagttttcaaatagcaaataacatataatttagaggtgaggaatacagaagaaggtttttatctatacagtgtgacttacctaggtacgcaatctttaaacaaaatgaagaagaaacatgttttctgttctcagtgctattgtaggttatgggaataaattaatttagaaatttgttctaaaataatgaactaccaaactgataatagcttgcctttatttgttttagtttcatctgtaagtgaataactggaatgaacacatcaacctttggttaaatataaggctttctagcttttgggcttacatgcacctgcttgtgtattcccacctcttttctgatgatctctgaagaggaagaaagagcatgaatgcctaggtatgcacaagcctatttatttctagacctttcctatacacactcttcaacatggcaaatgtttgcaaacaaatacattggttaaaaaaataatattgtaaggtagtttcatttttcatctaaaaatatgtgcacacaggcaatttcgatgaaaatggatttctgcttgaattatctagctaattgcctctattccctgctttgccttgagcatataaaaattatttagggtagacagtgttgaaccttataaatcaattaatcagtattgattaattatttcccctcaactttagtttgcctttaaactaagactaggtttatgctcatccataaaaagtgaaaatttaaacatacacagactgtctgcaatgtcactctggcggtgtatcatggggagatatgtttgaattagatagagaaaatttatatgaaatactctgaggctatgtttcctaaggggaattgctttatccagtataggaaaaccatttttcacataaatttctaaagataaattagaactttaacctgacacctaataggtagaattttagggtttgggggaataataatagttgctagagctattcaatggcaatgtcaatataaaaagcttagttttccacatgagagaagaactgaagtgtagacgagacactctcttacagtaacactgcagaaacttagaagcatgaatattttctagatttccatcttagtcacaattaaggataaagaagaaaaaatatgaaaagtttcttcataatattaaggggcttttattgataaaacaactatttctttcatagtaagttctttttgtcagaggcagaaatagaaatttgattctttagaagacattttgggtttcaaagagaaactctgctactttactgttgaaaatatatagtactctgagaaagctgccttacagcaaggagtttcagaaaagatacaagaaagaaaaccaatgtgagatgctttcattttagagtccctgcttcagtgtttccaacagaaacaagagaaaaagtaataagaaatatttttttctccctcttaagacatacatcactcctgaaattcttagaaaatcaactgaggcaaattaggggtttcaaagctagtcaccttgtaagttgttaggaaaaaaatttgcatttaaattgctctatgtagctcccttgagattttctcctggaatgcttatggctcttttttcattaatacttaaaaaaatacaatttcataaccagtgtattactacatctagttgtgttaagaagagaaacttcatttcataaaatagaaacattcaaagtggtttaggtcaaccaatcactcagtcagaatacttgaattcttcatattgaacacttaatagtgaagttaatctgaaccatatcaactctccatttcttttacagaaactaagtcattaatagctctatcagagagaataaactgtgttcctatatgccctccccataggaacaaagatagtccagaacttcttggaaatttttccttaaaatagtacatatttttatatatcagatttctttttaataggtaattcttaagtcctatttcaataacttgctttacatattcagaaatgtagatataagaaaaatattaaatgtgcaaaatgttctttctatatttacatttaaaaaatacaatgtaataatagctttatacttgtcaaaaagccattggggaaaataagccttcaatgtcagaaaatctggttaaattagagcttttgcttgtggaattgtaaacaaacttttaaaaatgctcagagttttctcaattcttcccatccaagacactcttgaacacatcaagtcctgctttgaagtaaacctgagctgaattaatgctgttcaacacctctgacagggcttcttgaagggtctcatttgatgcaaggggtttgcagtgttcccaagcctctataagtattgaaaaccggcttgtcttttcatcaaggtggtagaggatgtttctataaaaacctggtggtgcctgctttaccagaaagcttttctccatgtcttggagaatgtcattcagcatccggatgcggatgggtgctctctccttgggatcattagcaggtcgcatctcatcagactgaaaaagttcagcactctcccgcaggcgtaacgccatggctaacagttgatgagtgttgggttgatcacctttaaggttgttttgaacttctaaagctatatcaagtgcattaaagggcagaacaggttcgttggcaatttgcaaaatcacttctcctgagagcttagtaatggtttcatgaaggttgaaagagggatccatttcttcaatttttgttgctcgtgtagaaaaacgggcctcggagagaaaacttggaccctctaatgttttgatgtcctcgtaagcaaactgcacgatgggaactccaagatggttgatgaaataatcagcatcaccttgtatctgtatagaactgatattggtttctgggcactgggctcttctggtacagttgaaattatttttctctactaccagttgctgaagagatggtgatgctacaggatacagactagagttcccccttatgggactgtggaggctaatataagccacaacatttttctgaagaaccttcttgaaatcctctccccattcatatgagccaatattgccaaaagctgttcctccccaagaacagaaaacaatagttcggtctggtctccaccctctcttaacttttgacatcaaggcacggataaacgctgtgattattgcagtactactggcccattcttgtccattataactgtgtgcagtgtgatgatggctgccaactatgatataccggtctggagatgtcaagcccattacaaatccaacaacattagtaactgttttcaattttgtgactgtctgaacttgcatgctgacgactcttatttcattatttggaagctctagagagctacacgcttcatttttggttctagcttttggcgaagagatcagttttgcaacgaggggtgcagagatgggctgcactaatagagaggtgaggtttgatcggctttgtctaaaactttcatcgacacttgggtaaccaggcgtagaagggtctcctcctggattcagtgacaccatgaaggtatcatggctaggattcacagtctttggcaaatcacaaggatcgatatacagaagaacacctccaaatccagccttttccaatgaggaaagcttataaagcagtggcaattttcctaatttcaggagtgcgatctgatttgttacgttttttattttcctaatcctttttaaatcatctgccattccataactcacatcgatgacttcagccttgagagttcctttggcagaataggctgcatatgaatagagcaggtcttggctgctatcttttctggcttcttcactgcaaggctggccattaggatgaaagcattgaccactgctgctcagagtcacagtgctgggagaagggcctggcagatcaagcagcacagagtaatttacaaactgtacatcttctaggcccaaagaggtccactgagtcttaatcttctttgaaatttccatgtcatcttcatttttatatagttgtaccaaatttctgaaagacttcttaatatcttctgcctggattgtcttgagaatctcttgatataactgaggatcaactgttcctgaagatggagcatctgaagggcaatttgtatgtacataataacctatcaaaatcccaaaaataaataaaatggtggctgtgcaaagtatttttaagacgtggcaaaagttgcagcgattgctctttggtgcagatcgtgtataatgggtaatgtagtcagattcttcttgaagtctctggaaccttcctttgggtgaagttgctggttgaatggaatcaagattgaggtctatagtctctgaatgccctaggttctgattctcagcaccgtctagctggaattggtcaaaaccagactcctctagttccttctccatgtcccactctaagtcaagggcagtggcttgaaggtcatcattgtctaagtactgtgagtgtcctggagctctttgatctgcatggaccttctgataggccatctttttacttcaattgaatgttcctagtgcaactggagggcttctgcaggttacaggagactgacaatctggacccagtcttcatccaggtgcctaatagtcaatgctcatttccttgtttttaatcgttttctttatagaaactaaatttcatttaaattattcttttcttccctcagcctcctgagcggcgcgggcgcgggctcgtctgcggtacggct

SEQ ID NO: 12617 - RNA, 8401 nt, Homo sapiens
  source 1..8401: mol_type = other RNA
gatctcactttgttgcccaggctattttctggatgtctattaaaaaaaaattagtcctgcacagtgttctagaaagggtttttcttttcagaatatccatattctccaagtagcaagttagaatataaggaatatttgccattaaacctttctgttagaaatgtaaacatgaaattgcctaatatagacctatctcagatgctaaatagaattgtttataacacctttggaatataattatgtgagctacacttaaccatctggcattttgcttcctgcggacaatttgcaatagcatagaaaaatattttgtttgtgtatttcttatcaaacagatatgctaaagttctgtttagagagtaatagcattttattctaacttttaaaataaggtagtccatttgcagcagcttgatatataagtaaacaaaaatttttaatattaataaaacactagcacatacactgaaagcatctaagaaattcaaaatataaaacacttaccaagtaatgaccatatgagtggtaacatattgaataaaggccctttgaagaagttggagagttatgattactgagcaggctagataattaaataattacacattttgattgaaaaatatatgtagttcattaaaatagggactctaactccacttctctagctaagcttctattcagatgccacgtttgtactttaattagaacaaaagaccgacattaacttcaatgcaacataataattcataataatgattgtatattaatctcttgagcttgcaggaatatagcacatgacatatggcatgatacaggcacctgtgtgatcctttggggacttaggtggtgcatattaattagcccctggaaaataaaatctgtttccttctgagaaaagctacctcagtgcttattggcttaagccatcaaagaaattagatgaaatactgttaggctgggtctgcactcattaaagctttgtctagatgtaagcactgaatcaactgcctctgagttaagtcttgactgaatggtgcataagaaatcagagtaatcatgcatttctttggccttgatgattggattttggcatttaaaaaatccatcaaaattaccattttggttacagaaaattatgtaattgtataattcaaacaaaataatgtaaccagaaacactaaaatttgaagccacttcattttcctaaatgctgcttgaaactgcctcaatttaacccttttatttgtaaattcagattcaacccgaatatgagattataaatggcttaagaaatatgtcatcttgcaataatcagggtaacaagattcttgacggtcccaggtctgctaaaggcacttcagtgtgtatatctttgtcaggcaatggaacgatattatgaaactaaaactctggctgattaacagatcatttaaattgagactgatagatcttaaaattacttctcagggggaaaaagttacaatgctagagtgtacctagaaaacagaaacttgagtagacatggtaatgaccagaaaaggctatctttatacatttcttttgctacgcttcaaattcatgtcacctaaaagttgtgaagtgcacaaaacaaatctacttaactgaaaattattttcaatgaatgggatgtttagaactctgtgagggtttttaaggtcttttcgaatagcaaattctaatgaggcttttttaagttggcaatttaaactcatacaagaaataaaaactcaccagtgtggctgggcagaatatatatattttctcaaatattgtttgtttgttttttccctgcactgtatccatggtcccatgatgaaactgttatattgctgatatatttattggaatatgtgggccaacttcctttccactcaacatatggattggtagtttaaaataattcctttctattaagcaaatgtgtggctaaggcacatttaaatagcccattaaaccaatgagatgacaatgtgttaccctcagagaaagcttaatttttggagtaatcaattacacatatcacagaatgtctcatgagaacatttttggctaggtctaccaatttatcatacaaataattatagattttcatttgaggcaaagatgctgattcatcattagtaacatggtcacaaataatcatttattttatttttgttaacatctgtctttcctgtggggaaacttactatatgctctacgtttatttaatttaaaaagtcaattggttattctgaatttttaaaaataacataaaactgttgttctaaatcacagcacctgcttttctttttttagtgaaattatataagcatttagagaatgaaagtgtaagacttgtggtttctggtctctttttactgtttgtaagcctactcgtcatgatattccacaatggtgcacttgccttttaatgctcttatagatatcttcaaacttgcctacatatatacgcctttgttggagtgggctaccatcatcaggaatgatgtcatttgtttcttcaaactcctttattataccaaaaaagtgacagactccacagtctgatcagttttggagaaatatgttaacattttcaattatctcactttctagaatcaaaatagtctgattttttttttcggcactcagtgtaaagaacaaagaactgaatacagtgggcccagaagagaaatatgcctcatcatttttattagctttggaactgtggacaagtcactcaacctagttttctcattttgaaatgggttgttgtgggaattaaaaaaaaaaaaaaaaaaaaaaaaggatacatgggaaaaattctaaaacaccagtgcctgggatgtagcaggcacaaatataagctgcaactgaattgttttcttagagataaaatgggtccacttttcttttctcataatgattccattaataacaaatctttacgtctttcttgttattatgactcttcaatttatttagaaatgtcaattagtgttttcttggaaactacgattaacgtagattggaaattcttaaacttcagtgtgtgtaacagacatccagaaatcttgctgaagatgtagattcctagccctgtctttctaaatttcacattttgagaaacggtgatttagattgttgacttaacactggcctgacttgccctcttacagatatattttgctcaatgtccttcttcctgacttctggtgttctgtaaggattctccccactttctctcaagtacccagtctttgtgtcctttgcctgaattctcggggagagttttgtttgtcaggtacagtcagagaatgaactagccttgaattaaaagcagtgtttccagcccatgcaacatctgacagaatggctggttacatcgaatgcactggaaaagatcatttataaccctgtctcctcagggagaagcaagatatactgcatgagaaagcagagaagcttaaattccagtggtgcttttgttactaactaaatacatgactatgtccaagtttcttactcactttgggtttagttactatatctggtgggggtaattgataatgccttctctggctgaaggcaagatctcagggcttagaccagaatctttattaggctttcttttgattctgagacttatgcttttccataaagggcagtatctcatgtgtaccctgcctgaacataaatttcaccgttacacctttaccacattttcttcagagaatatttatgattcattatttcctaggcacaattctatgtatgaaagattgtgagaagtaccaggcatatagacgactcagcaacagcttaaacctactaccaattcacattaacacttgctattaatttgctcaggattttatttatttgaatctattgggggtggggaggggaggggagtgaaatgatatacatttggaggcaccctcaggtaatcacactatagaaataatgctgctagttaagaggtttgttgcaaagatgtaaagcagcatgtacagaatttgttggacgtctgctttaggtataatttaatatctccacgtatcttttaatagactaataaaaaaccatagttaactacagttttcaaatagcaaataacatataatttagaggtgaggaatacagaagaaggtttttatctatacagtgtgacttacctaggtacgcaatctttaaacaaaatgaagaagaaacatgttttctgttctcagtgctattgtaggttatgggaataaattaatttagaaatttgttctaaaataatgaactaccaaactgataatagcttgcctttatttgttttagtttcatctgtaagtgaataactggaatgaacacatcaacctttggttaaatataaggctttctagcttttgggcttacatgcacctgcttgtgtattcccacctcttttctgatgatctctgaagaggaagaaagagcatgaatgcctaggtatgcacaagcctatttatttctagacctttcctatacacactcttcaacatggcaaatgtttgcaaacaaatacattggttaaaaaaataatattgtaaggtagtttcatttttcatctaaaaatatgtgcacacaggcaatttcgatgaaaatggatttctgcttgaattatctagctaattgcctctattccctgctttgccttgagcatataaaaattatttagggtagacagtgttgaaccttataaatcaattaatcagtattgattaattatttcccctcaactttagtttgcctttaaactaagactaggtttatgctcatccataaaaagtgaaaatttaaacatacacagactgtctgcaatgtcactctggcggtgtatcatggggagatatgtttgaattagatagagaaaatttatatgaaatactctgaggctatgtttcctaaggggaattgctttatccagtataggaaaaccatttttcacataaatttctaaagataaattagaactttaacctgacacctaataggtagaattttagggtttgggggaataataatagttgctagagctattcaatggcaatgtcaatataaaaagcttagttttccacatgagagaagaactgaagtgtagacgagacactctcttacagtaacactgcagaaacttagaagcatgaatattttctagatttccatcttagtcacaattaaggataaagaagaaaaaatatgaaaagtttcttcataatattaaggggcttttattgataaaacaactatttctttcatagtaagttctttttgtcagaggcagaaatagaaatttgattctttagaagacattttgggtttcaaagagaaactctgctactttactgttgaaaatatatagtactctgagaaagctgccttacagcaaggagtttcagaaaagatacaagaaagaaaaccaatgtgagatgctttcattttagagtccctgcttcagtgtttccaacagaaacaagagaaaaagtaataagaaatatttttttctccctcttaagacatacatcactcctgaaattcttagaaaatcaactgaggcaaattaggggtttcaaagctagtcaccttgtaagttgttaggaaaaaaatttgcatttaaattgctctatgtagctcccttgagattttctcctggaatgcttatggctcttttttcattaatacttaaaaaaatacaatttcataaccagtgtattactacatctagttgtgttaagaagagaaacttcatttcataaaatagaaacattcaaagtggtttaggtcaaccaatcactcagtcagaatacttgaattcttcatattgaacacttaatagtgaagttaatctgaaccatatcaactctccatttcttttacagaaactaagtcattaatagctctatcagagagaataaactgtgttcctatatgccctccccataggaacaaagatagtccagaacttcttggaaatttttccttaaaatagtacatatttttatatatcagatttctttttaataggtaattcttaagtcctatttcaataacttgctttacatattcagaaatgtagatataagaaaaatattaaatgtgcaaaatgttctttctatatttacatttaaaaaatacaatgtaataatagctttatacttgtcaaaaagccattggggaaaataagccttcaatgtcagaaaatctggttaaattagagcttttgcttgtggaattgtaaacaaacttttaaaaatgctcagagttttctcaattcttcccatccaagacactcttgaacacatcaagtcctgctttgaagtaaacctgagctgaattaatgctgttcaacacctctgacagggcttcttgaagggtctcatttgatgcaaggggtttgcagtgttcccaagcctctataagtattgaaaaccggcttgtcttttcatcaaggtggtagaggatgtttctataaaaacctggtggtgcctgctttaccagaaagcttttctccatgtcttggagaatgtcattcagcatccggatgcggatgggtgctctctccttgggatcattagcaggtcgcatctcatcagactgaaaaagttcagcactctcccgcaggcgtaacgccatggctaacagttgatgagtgttgggttgatcacctttaaggttgttttgaacttctaaagctatatcaagtgcattaaagggcagaacaggttcgttggcaatttgcaaaatcacttctcctgagagcttagtaatggtttcatgaaggttgaaagagggatccatttcttcaatttttgttgctcgtgtagaaaaacgggcctcggagagaaaacttggaccctctaatgttttgatgtcctcgtaagcaaactgcacgatgggaactccaagatggttgatgaaataatcagcatcaccttgtatctgtatagaactgatattggtttctgggcactgggctcttctggtacagttgaaattatttttctctactaccagttgctgaagagatggtgatgctacaggatacagactagagttcccccttatgggactgtggaggctaatataagccacaacatttttctgaagaaccttcttgaaatcctctccccattcatatgagccaatattgccaaaagctgttcctccccaagaacagaaaacaatagttcggtctggtctccaccctctcttaacttttgacatcaaggcacggataaacgctgtgattattgcagtactactggcccattcttgtccattataactgtgtgcagtgtgatgatggctgccaactatgatataccggtctggagatgtcaagcccattacaaatccaacaacattagtaactgttttcaattttgtgactgtctgaacttgcatgctgacgactcttatttcattatttggaagctctagagagctacacgcttcatttttggttctagcttttggcgaagagatcagttttgcaacgaggggtgcagagatgggctgcactaatagagaggtgaggtttgatcggctttgtctaaaactttcatcgacacttgggtaaccaggcgtagaagggtctcctcctggattcagtgacaccatgaaggtatcatggctaggattcacagtctttggcaaatcacaaggatcgatatacagaagaacacctccaaatccagccttttccaatgaggaaagcttataaagcagtggcaattttcctaatttcaggagtgcgatctgatttgttacgttttttattttcctaatcctttttaaatcatctgccattccataactcacatcgatgacttcagccttgagagttcctttggcagaataggctgcatatgaatagagcaggtcttggctgctatcttttctggcttcttcactgcaaggctggccattaggatgaaagcattgaccactgctgctcagagtcacagtgctgggagaagggcctggcagatcaagcagcacagagtaatttacaaactgtacatcttctaggcccaaagaggtccactgagtcttaatcttctttgaaatttccatgtcatcttcatttttatatagttgtaccaaatttctgtgacattcaagcttcttctaagttaaagagctttctcaaccgtcctaggtaaacatggtttatacaagataaccagcatctcaactggcttaagctgattagattagggacaagcacttgacagagagtcacgaacatctttggtccacaaaaggataataatgacatttcatcctgaaagacttcttaatatcttctgcctggattgtcttgagaatctcttgatataactgaggatcaactgttcctgaagatgga

SEQ ID NO: 12618 - RNA, 11966 nt, Homo sapiens
  source 1..11966: mol_type = other RNA
gatctcactttgttgcccaggctattttctggatgtctattaaaaaaaaattagtcctgcacagtgttctagaaagggtttttcttttcagaatatccatattctccaagtagcaagttagaatataaggaatatttgccattaaacctttctgttagaaatgtaaacatgaaattgcctaatatagacctatctcagatgctaaatagaattgtttataacacctttggaatataattatgtgagctacacttaaccatctggcattttgcttcctgcggacaatttgcaatagcatagaaaaatattttgtttgtgtatttcttatcaaacagatatgctaaagttctgtttagagagtaatagcattttattctaacttttaaaataaggtagtccatttgcagcagcttgatatataagtaaacaaaaatttttaatattaataaaacactagcacatacactgaaagcatctaagaaattcaaaatataaaacacttaccaagtaatgaccatatgagtggtaacatattgaataaaggccctttgaagaagttggagagttatgattactgagcaggctagataattaaataattacacattttgattgaaaaatatatgtagttcattaaaatagggactctaactccacttctctagctaagcttctattcagatgccacgtttgtactttaattagaacaaaagaccgacattaacttcaatgcaacataataattcataataatgattgtatattaatctcttgagcttgcaggaatatagcacatgacatatggcatgatacaggcacctgtgtgatcctttggggacttaggtggtgcatattaattagcccctggaaaataaaatctgtttccttctgagaaaagctacctcagtgcttattggcttaagccatcaaagaaattagatgaaatactgttaggctgggtctgcactcattaaagctttgtctagatgtaagcactgaatcaactgcctctgagttaagtcttgactgaatggtgcataagaaatcagagtaatcatgcatttctttggccttgatgattggattttggcatttaaaaaatccatcaaaattaccattttggttacagaaaattatgtaattgtataattcaaacaaaataatgtaaccagaaacactaaaatttgaagccacttcattttcctaaatgctgcttgaaactgcctcaatttaacccttttatttgtaaattcagattcaacccgaatatgagattataaatggcttaagaaatatgtcatcttgcaataatcagggtaacaagattcttgacggtcccaggtctgctaaaggcacttcagtgtgtatatctttgtcaggcaatggaacgatattatgaaactaaaactctggctgattaacagatcatttaaattgagactgatagatcttaaaattacttctcagggggaaaaagttacaatgctagagtgtacctagaaaacagaaacttgagtagacatggtaatgaccagaaaaggctatctttatacatttcttttgctacgcttcaaattcatgtcacctaaaagttgtgaagtgcacaaaacaaatctacttaactgaaaattattttcaatgaatgggatgtttagaactctgtgagggtttttaaggtcttttcgaatagcaaattctaatgaggcttttttaagttggcaatttaaactcatacaagaaataaaaactcaccagtgtggctgggcagaatatatatattttctcaaatattgtttgtttgttttttccctgcactgtatccatggtcccatgatgaaactgttatattgctgatatatttattggaatatgtgggccaacttcctttccactcaacatatggattggtagtttaaaataattcctttctattaagcaaatgtgtggctaaggcacatttaaatagcccattaaaccaatgagatgacaatgtgttaccctcagagaaagcttaatttttggagtaatcaattacacatatcacagaatgtctcatgagaacatttttggctaggtctaccaatttatcatacaaataattatagattttcatttgaggcaaagatgctgattcatcattagtaacatggtcacaaataatcatttattttatttttgttaacatctgtctttcctgtggggaaacttactatatgctctacgtttatttaatttaaaaagtcaattggttattctgaatttttaaaaataacataaaactgttgttctaaatcacagcacctgcttttctttttttagtgaaattatataagcatttagagaatgaaagtgtaagacttgtggtttctggtctctttttactgtttgtaagcctactcgtcatgatattccacaatggtgcacttgccttttaatgctcttatagatatcttcaaacttgcctacatatatacgcctttgttggagtgggctaccatcatcaggaatgatgtcatttgtttcttcaaactcctttattataccaaaaaagtgacagactccacagtctgatcagttttggagaaatatgttaacattttcaattatctcactttctagaatcaaaatagtctgattttttttttcggcactcagtgtaaagaacaaagaactgaatacagtgggcccagaagagaaatatgcctcatcatttttattagctttggaactgtggacaagtcactcaacctagttttctcattttgaaatgggttgttgtgggaattaaaaaaaaaaaaaaaaaaaaaaaaggatacatgggaaaaattctaaaacaccagtgcctgggatgtagcaggcacaaatataagctgcaactgaattgttttcttagagataaaatgggtccacttttcttttctcataatgattccattaataacaaatctttacgtctttcttgttattatgactcttcaatttatttagaaatgtcaattagtgttttcttggaaactacgattaacgtagattggaaattcttaaacttcagtgtgtgtaacagacatccagaaatcttgctgaagatgtagattcctagccctgtctttctaaatttcacattttgagaaacggtgatttagattgttgacttaacactggcctgacttgccctcttacagatatattttgctcaatgtccttcttcctgacttctggtgttctgtaaggattctccccactttctctcaagtacccagtctttgtgtcctttgcctgaattctcggggagagttttgtttgtcaggtacagtcagagaatgaactagccttgaattaaaagcagtgtttccagcccatgcaacatctgacagaatggctggttacatcgaatgcactggaaaagatcatttataaccctgtctcctcagggagaagcaagatatactgcatgagaaagcagagaagcttaaattccagtggtgcttttgttactaactaaatacatgactatgtccaagtttcttactcactttgggtttagttactatatctggtgggggtaattgataatgccttctctggctgaaggcaagatctcagggcttagaccagaatctttattaggctttcttttgattctgagacttatgcttttccataaagggcagtatctcatgtgtaccctgcctgaacataaatttcaccgttacacctttaccacattttcttcagagaatatttatgattcattatttcctaggcacaattctatgtatgaaagattgtgagaagtaccaggcatatagacgactcagcaacagcttaaacctactaccaattcacattaacacttgctattaatttgctcaggattttatttatttgaatctattgggggtggggaggggaggggagtgaaatgatatacatttggaggcaccctcaggtaatcacactatagaaataatgctgctagttaagaggtttgttgcaaagatgtaaagcagcatgtacagaatttgttggacgtctgctttaggtataatttaatatctccacgtatcttttaatagactaataaaaaaccatagttaactacagttttcaaatagcaaataacatataatttagaggtgaggaatacagaagaaggtttttatctatacagtgtgacttacctaggtacgcaatctttaaacaaaatgaagaagaaacatgttttctgttctcagtgctattgtaggttatgggaataaattaatttagaaatttgttctaaaataatgaactaccaaactgataatagcttgcctttatttgttttagtttcatctgtaagtgaataactggaatgaacacatcaacctttggttaaatataaggctttctagcttttgggcttacatgcacctgcttgtgtattcccacctcttttctgatgatctctgaagaggaagaaagagcatgaatgcctaggtatgcacaagcctatttatttctagacctttcctatacacactcttcaacatggcaaatgtttgcaaacaaatacattggttaaaaaaataatattgtaaggtagtttcatttttcatctaaaaatatgtgcacacaggcaatttcgatgaaaatggatttctgcttgaattatctagctaattgcctctattccctgctttgccttgagcatataaaaattatttagggtagacagtgttgaaccttataaatcaattaatcagtattgattaattatttcccctcaactttagtttgcctttaaactaagactaggtttatgctcatccataaaaagtgaaaatttaaacatacacagactgtctgcaatgtcactctggcggtgtatcatggggagatatgtttgaattagatagagaaaatttatatgaaatactctgaggctatgtttcctaaggggaattgctttatccagtataggaaaaccatttttcacataaatttctaaagataaattagaactttaacctgacacctaataggtagaattttagggtttgggggaataataatagttgctagagctattcaatggcaatgtcaatataaaaagcttagttttccacatgagagaagaactgaagtgtagacgagacactctcttacagtaacactgcagaaacttagaagcatgaatattttctagatttccatcttagtcacaattaaggataaagaagaaaaaatatgaaaagtttcttcataatattaaggggcttttattgataaaacaactatttctttcatagtaagttctttttgtcagaggcagaaatagaaatttgattctttagaagacattttgggtttcaaagagaaactctgctactttactgttgaaaatatatagtactctgagaaagctgccttacagcaaggagtttcagaaaagatacaagaaagaaaaccaatgtgagatgctttcattttagagtccctgcttcagtgtttccaacagaaacaagagaaaaagtaataagaaatatttttttctccctcttaagacatacatcactcctgaaattcttagaaaatcaactgaggcaaattaggggtttcaaagctagtcaccttgtaagttgttaggaaaaaaatttgcatttaaattgctctatgtagctcccttgagattttctcctggaatgcttatggctcttttttcattaatacttaaaaaaatacaatttcataaccagtgtattactacatctagttgtgttaagaagagaaacttcatttcataaaatagaaacattcaaagtggtttaggtcaaccaatcactcagtcagaatacttgaattcttcatattgaacacttaatagtgaagttaatctgaaccatatcaactctccatttcttttacagaaactaagtcattaatagctctatcagagagaataaactgtgttcctatatgccctccccataggaacaaagatagtccagaacttcttggaaatttttccttaaaatagtacatatttttatatatcagatttctttttaataggtaattcttaagtcctatttcaataacttgctttacatattcagaaatgtagatataagaaaaatattaaatgtgcaaaatgttctttctatatttacatttaaaaaatacaatgtaataatagctttatacttgtcaaaaagccattggggaaaataagccttcaatgtcagaaaatctggttaaattagagcttttgcttgtggaattgtaaacaaacttttaaaaatgctcagagttttctcaattcttcccatccaagacactcttgaacacatcaagtcctgctttgaagtaaacctgagctgaattaatgctgttcaacacctctgacagggcttcttgaagggtctcatttgatgcaaggggtttgcagtgttcccaagcctctataagtattgaaaaccggcttgtcttttcatcaaggtggtagaggatgtttctataaaaacctggtggtgcctgctttaccagaaagcttttctccatgtcttggagaatgtcattcagcatccggatgcggatgggtgctctctccttgggatcattagcaggtcgcatctcatcagactgaaaaagttcagcactctcccgcaggcgtaacgccatggctaacagttgatgagtgttgggttgatcacctttaaggttgttttgaacttctaaagctatatcaagtgcattaaagggcagaacaggttcgttggcaatttgcaaaatcacttctcctgagagcttagtaatggtttcatgaaggttgaaagagggatccatttcttcaatttttgttgctcgtgtagaaaaacgggcctcggagagaaaacttggaccctctaatgttttgatgtcctcgtaagcaaactgcacgatgggaactccaagatggttgatgaaataatcagcatcaccttgtatctgtatagaactgatattggtttctgggcactgggctcttctggtacagttgaaattatttttctctactaccagttgctgaagagatggtgatgctacaggatacagactagagttcccccttatgggactgtggaggctaatataagccacaacatttttctgaagaaccttcttgaaatcctctccccattcatatgagccaatattgccaaaagctgttcctccccaagaacagaaaacaatagttcggtctggtctccaccctctcttaacttttgacatcaaggcacggataaacgctgtgattattgcagtactactggcccattcttgtccattataactgtgtgcagtgtgatgatggctgccaactatgatataccggtctggagatgtcaagcccattacaaatccaacaacattagtaactgttttcaattttgtgactgtctgaacttgcatgctgacgactcttatttcgacacttgggtaaccaggcgtagaagggtctcctcctggattcagtgacaccatgaaggtatcatggctaggattcacagtctttggcaaatcacaaggatcgatatacagaagaacacctccaaatccagccttttccaatgaggaaagcttataaagcagtggcaattttcctaatttcaggagtgcgatctgatttgttacgttttttattttcctaatcctttttaaatcatctgccattccataactcacatcgatgacttcagccttgagagttcctttggcagaataggctgcatatgaatagagcaggtcttggctgctatcttttctggcttcttcactgcaaggctggccattaggatgaaagcattgaccactgctgctcagagtcacagtgctgggagaagggcctggcagatcaagcagcacagagtaatttacaaactgtacatcttctaggcccaaagaggtccactgagtcttaatcttctttgaaatttccatgtcatcttcatttttatatagttgtaccaaatttctgaaagacttcttaatatcttctgcctggattgtcttgagaatctcttgatataactgaggatcaactgttcctgaagatggagcatctgaagggcaatttgtatgtacataataacctatcaaaatcccaaaaataaataaaatggtggctgtgcaaagtatttttaagacgtggcaaaagttgcagcgattgctctttggtgcagatcgtgtataatgggtaatgtagtcagattcttcttgaagtctctggaaccttcctttgggtgaagttgctggttgaatggaatcaagattgaggtctatagtctctgaatgccctaggttctgattctcagcaccgtctagctggaattggtcaaaaccagactcctctagttccttctccatgtcccactctaagtcaagggcagtggcttgaaggtcatcattgtctaagtactgtgagtgtcctggagctctttgatctgcatggaccttctgataggccatctttttaccagtcacctctttcattatccatcttctagcaatcacttccatccactgcctcatgccaatgtcgagtgccattgcttcaaatgctgtatacagtttttacttgtttctggaaagagggtaaatccagtccttgatattttaaccaaatgcacaaatattttttcttccacatttaattctacaaatatatttgattgactgtcctacccttatgaatcagtcactatgtcaaaatgaagcggactatacaattagcaagaacctagtctcatatccaaacctgtggacctatgtgttctattgccagtatcagggagaaagagtaaaagcatactccagaccaccaaaactaatagctatcagaatccacttcagaaaatacgttcttatcttaaaaaaggacttttgggggatggcaattccattgcactgatttgtggtttagtgcatcaagcattcctcaggcacattcggtgtgccaggtaaggtggtggcccctgagaaccgtgagataaacaagatgcaagtgcagcctggaagctcatattccagagtttccctttcgccctgcttgtcagttttgcgaaagcattcacagcccctacctcttctgttcacctctcccgttctaggcaatagtcatgggatagctttggcctaaaatggtacattattaatttggggcccatatttcagatgtcacattttaaagatgaagaaacaagggaagaggagggtcaagtcacatgtcacaggtgaagtggccatcaattaacaaacttgatattgttgaagtgttgaatatgactaatatggtgtgtactgaggcccctcactccccactgctcgtcccactattccacagagcgtcatcctgcctggactgcaggactggatattaactcctacctgcatatgtaaaattaactcctacctttcctgctattttaaaaccaaataaattacctcaccattcactaaataaaactcactattttcttatgtttactgcttattcctcagttcccacccccaaagtcaaggagtactattctcttttccttagctaactcatcagacccacatttaataaactggaaaattttttattaaataatgttgagtggaaaaaaggataacaaatttctatgtaaaaagtgatgcagttattttaaaatatatagttatacacacacacaaagactttaagttagcatgccaaaatattagtaatttttgaaaaatctggattgttaatttatgggtaatgtttactttactcttcacacttttttgtttctaaccttctgacgatctctatgtgatatatatatatgtatataaactattaaaataaagttattcttaaagccaatctctaaaaaatcaactacattctgattaaaatctctgatgaacacaatttagataaaattatattttatttgtgctacagtattgcagaaagcattgcaaatacaatacattgcatatgtgattctttataatctctatttgaattatatgacacttgaaggcagaaaatgtatattttaaaaaatatcttctaatacttaacttgtgtagttaaatatattaaccaaatgttacaaatgttacaattgtgcatttcttgcctgggaatcctaaaggaaatcgaaataataaaaacagctgacaattatgacattcatactatgtgctaggttctgttacagatagttttacagcttctatctcatttaatcctcagaatagtccttttagagttcgttttatacatgaagaaactcaaaagtaggaagagatcaaattatctaaagtgccatagctagaacgtgacagagccagtatttgaaaccaagtaggtaaccccacagtctgtgcactaacccaccacacaatccatattttgaatgtttcaacaatattagaaatcttggagtagggataatgatataaagcagggatttgttaatacagattgtttatcatgatttcctcattactagtatctacctcaaaggactattttaacagttaaatatatgatcatgagtttgcacaagtgtctggtgtgtatagagtgctctataattgttttttgagatggaattttgctcttgttgcccaggctggagtgcaatggcactgtcttggctcatggcgacctctgtctcccgggattcaagcaattctcctgtctcagccttccaagtagctgggattacaggcacccgtcaccatgccaggataatttttgtatttttagtagagacggtatatcaccatgttggccaggctggtcttgaactcctgacctcaggtgaggtgatccgcctgcctgggtctcccaaactcctgggattacaggtgtgagccaccgtgcctagcctataaatttagctaatactgttacatgcatattttagctactgtgaattcagttaagatgaaatagctacacaactaaggagatctttttttttttttctgagtatgataaactaaggacatgccttaagtctaagaaaatctgtttactgcaggcttttctgcacaaattttcctttatcatcaaggttgctatagccatccctctttcggattccttttcttctttaaaattagaggctttgctttacactgttatttttaaatggctggatacctgccatagatctaataattggttgtaaaaatccagacaaacatcaatttttaattcttaatttttaatcttgtttgaaacaaacatgtaaactaaaataaaaacttaataaagccaggttcaaatcttgcctgttttagtatataagtcaaatttttattaaattaacttcagatcctattaattatgaaagcaagaggttatatttctaatgaatactaagatcttattagaaattccttctccatcactttgtttttctcttcattagatatacccgcacaaatgacctaaaattcaacccactttgaaaataaattttcaaggcttagtgaaaaaagcctaatttctgtagccactggcctgtttctagagccatcgttgactgatggcttataaagcctttttatacagcactgacattttaaagatactggccagtctgaactttccatctggcgtgcttgatttcctttgtcccactttcccatagtgacttattctgtccttgagctctaaaactactttgatttaatttaggcctgggggtgtgaagacatggtgaaatttatttaaacaagagacgatagtaatgcctccaacagtgcatagtaataggaaagcaaataactgacttcctggcatttatttgtgtaataacttcaccaccaagtgcaaccagagaggtattccagaactttccatgcaattacataaaactagcaagagctagtcagcacttgtaaaatcaagtgggagataaaggaaattattttatctcaggccaaaaaaaaaa

SEQ ID NO: 12619 - RNA, 11962 nt, Homo sapiens
  source 1..11962: mol_type = other RNA
gatctcactttgttgcccaggctattttctggatgtctattaaaaaaaaattagtcctgcacagtgttctagaaagggtttttcttttcagaatatccatattctccaagtagcaagttagaatataaggaatatttgccattaaacctttctgttagaaatgtaaacatgaaattgcctaatatagacctatctcagatgctaaatagaattgtttataacacctttggaatataattatgtgagctacacttaaccatctggcattttgcttcctgcggacaatttgcaatagcatagaaaaatattttgtttgtgtatttcttatcaaacagatatgctaaagttctgtttagagagtaatagcattttattctaacttttaaaataaggtagtccatttgcagcagcttgatatataagtaaacaaaaatttttaatattaataaaacactagcacatacactgaaagcatctaagaaattcaaaatataaaacacttaccaagtaatgaccatatgagtggtaacatattgaataaaggccctttgaagaagttggagagttatgattactgagcaggctagataattaaataattacacattttgattgaaaaatatatgtagttcattaaaatagggactctaactccacttctctagctaagcttctattcagatgccacgtttgtactttaattagaacaaaagaccgacattaacttcaatgcaacataataattcataataatgattgtatattaatctcttgagcttgcaggaatatagcacatgacatatggcatgatacaggcacctgtgtgatcctttggggacttaggtggtgcatattaattagcccctggaaaataaaatctgtttccttctgagaaaagctacctcagtgcttattggcttaagccatcaaagaaattagatgaaatactgttaggctgggtctgcactcattaaagctttgtctagatgtaagcactgaatcaactgcctctgagttaagtcttgactgaatggtgcataagaaatcagagtaatcatgcatttctttggccttgatgattggattttggcatttaaaaaatccatcaaaattaccattttggttacagaaaattatgtaattgtataattcaaacaaaataatgtaaccagaaacactaaaatttgaagccacttcattttcctaaatgctgcttgaaactgcctcaatttaacccttttatttgtaaattcagattcaacccgaatatgagattataaatggcttaagaaatatgtcatcttgcaataatcagggtaacaagattcttgacggtcccaggtctgctaaaggcacttcagtgtgtatatctttgtcaggcaatggaacgatattatgaaactaaaactctggctgattaacagatcatttaaattgagactgatagatcttaaaattacttctcagggggaaaaagttacaatgctagagtgtacctagaaaacagaaacttgagtagacatggtaatgaccagaaaaggctatctttatacatttcttttgctacgcttcaaattcatgtcacctaaaagttgtgaagtgcacaaaacaaatctacttaactgaaaattattttcaatgaatgggatgtttagaactctgtgagggtttttaaggtcttttcgaatagcaaattctaatgaggcttttttaagttggcaatttaaactcatacaagaaataaaaactcaccagtgtggctgggcagaatatatatattttctcaaatattgtttgtttgttttttccctgcactgtatccatggtcccatgatgaaactgttatattgctgatatatttattggaatatgtgggccaacttcctttccactcaacatatggattggtagtttaaaataattcctttctattaagcaaatgtgtggctaaggcacatttaaatagcccattaaaccaatgagatgacaatgtgttaccctcagagaaagcttaatttttggagtaatcaattacacatatcacagaatgtctcatgagaacatttttggctaggtctaccaatttatcatacaaataattatagattttcatttgaggcaaagatgctgattcatcattagtaacatggtcacaaataatcatttattttatttttgttaacatctgtctttcctgtggggaaacttactatatgctctacgtttatttaatttaaaaagtcaattggttattctgaatttttaaaaataacataaaactgttgttctaaatcacagcacctgcttttctttttttagtgaaattatataagcatttagagaatgaaagtgtaagacttgtggtttctggtctctttttactgtttgtaagcctactcgtcatgatattccacaatggtgcacttgccttttaatgctcttatagatatcttcaaacttgcctacatatatacgcctttgttggagtgggctaccatcatcaggaatgatgtcatttgtttcttcaaactcctttattataccaaaaaagtgacagactccacagtctgatcagttttggagaaatatgttaacattttcaattatctcactttctagaatcaaaatagtctgattttttttttcggcactcagtgtaaagaacaaagaactgaatacagtgggcccagaagagaaatatgcctcatcatttttattagctttggaactgtggacaagtcactcaacctagttttctcattttgaaatgggttgttgtgggaattaaaaaaaaaaaaaaaaaaaaaaaaggatacatgggaaaaattctaaaacaccagtgcctgggatgtagcaggcacaaatataagctgcaactgaattgttttcttagagataaaatgggtccacttttcttttctcataatgattccattaataacaaatctttacgtctttcttgttattatgactcttcaatttatttagaaatgtcaattagtgttttcttggaaactacgattaacgtagattggaaattcttaaacttcagtgtgtgtaacagacatccagaaatcttgctgaagatgtagattcctagccctgtctttctaaatttcacattttgagaaacggtgatttagattgttgacttaacactggcctgacttgccctcttacagatatattttgctcaatgtccttcttcctgacttctggtgttctgtaaggattctccccactttctctcaagtacccagtctttgtgtcctttgcctgaattctcggggagagttttgtttgtcaggtacagtcagagaatgaactagccttgaattaaaagcagtgtttccagcccatgcaacatctgacagaatggctggttacatcgaatgcactggaaaagatcatttataaccctgtctcctcagggagaagcaagatatactgcatgagaaagcagagaagcttaaattccagtggtgcttttgttactaactaaatacatgactatgtccaagtttcttactcactttgggtttagttactatatctggtgggggtaattgataatgccttctctggctgaaggcaagatctcagggcttagaccagaatctttattaggctttcttttgattctgagacttatgcttttccataaagggcagtatctcatgtgtaccctgcctgaacataaatttcaccgttacacctttaccacattttcttcagagaatatttatgattcattatttcctaggcacaattctatgtatgaaagattgtgagaagtaccaggcatatagacgactcagcaacagcttaaacctactaccaattcacattaacacttgctattaatttgctcaggattttatttatttgaatctattgggggtggggaggggaggggagtgaaatgatatacatttggaggcaccctcaggtaatcacactatagaaataatgctgctagttaagaggtttgttgcaaagatgtaaagcagcatgtacagaatttgttggacgtctgctttaggtataatttaatatctccacgtatcttttaatagactaataaaaaaccatagttaactacagttttcaaatagcaaataacatataatttagaggtgaggaatacagaagaaggtttttatctatacagtgtgacttacctaggtacgcaatctttaaacaaaatgaagaagaaacatgttttctgttctcagtgctattgtaggttatgggaataaattaatttagaaatttgttctaaaataatgaactaccaaactgataatagcttgcctttatttgttttagtttcatctgtaagtgaataactggaatgaacacatcaacctttggttaaatataaggctttctagcttttgggcttacatgcacctgcttgtgtattcccacctcttttctgatgatctctgaagaggaagaaagagcatgaatgcctaggtatgcacaagcctatttatttctagacctttcctatacacactcttcaacatggcaaatgtttgcaaacaaatacattggttaaaaaaataatattgtaaggtagtttcatttttcatctaaaaatatgtgcacacaggcaatttcgatgaaaatggatttctgcttgaattatctagctaattgcctctattccctgctttgccttgagcatataaaaattatttagggtagacagtgttgaaccttataaatcaattaatcagtattgattaattatttcccctcaactttagtttgcctttaaactaagactaggtttatgctcatccataaaaagtgaaaatttaaacatacacagactgtctgcaatgtcactctggcggtgtatcatggggagatatgtttgaattagatagagaaaatttatatgaaatactctgaggctatgtttcctaaggggaattgctttatccagtataggaaaaccatttttcacataaatttctaaagataaattagaactttaacctgacacctaataggtagaattttagggtttgggggaataataatagttgctagagctattcaatggcaatgtcaatataaaaagcttagttttccacatgagagaagaactgaagtgtagacgagacactctcttacagtaacactgcagaaacttagaagcatgaatattttctagatttccatcttagtcacaattaaggataaagaagaaaaaatatgaaaagtttcttcataatattaaggggcttttattgataaaacaactatttctttcatagtaagttctttttgtcagaggcagaaatagaaatttgattctttagaagacattttgggtttcaaagagaaactctgctactttactgttgaaaatatatagtactctgagaaagctgccttacagcaaggagtttcagaaaagatacaagaaagaaaaccaatgtgagatgctttcattttagagtccctgcttcagtgtttccaacagaaacaagagaaaaagtaataagaaatatttttttctccctcttaagacatacatcactcctgaaattcttagaaaatcaactgaggcaaattaggggtttcaaagctagtcaccttgtaagttgttaggaaaaaaatttgcatttaaattgctctatgtagctcccttgagattttctcctggaatgcttatggctcttttttcattaatacttaaaaaaatacaatttcataaccagtgtattactacatctagttgtgttaagaagagaaacttcatttcataaaatagaaacattcaaagtggtttaggtcaaccaatcactcagtcagaatacttgaattcttcatattgaacacttaatagtgaagttaatctgaaccatatcaactctccatttcttttacagaaactaagtcattaatagctctatcagagagaataaactgtgttcctatatgccctccccataggaacaaagatagtccagaacttcttggaaatttttccttaaaatagtacatatttttatatatcagatttctttttaataggtaattcttaagtcctatttcaataacttgctttacatattcagaaatgtagatataagaaaaatattaaatgtgcaaaatgttctttctatatttacatttaaaaaatacaatgtaataatagctttatacttgtcaaaaagccattggggaaaataagccttcaatgtcagaaaatctggttaaattagagcttttgcttgtggaattgtaaacaaacttttaaaaatgctcagagttttctcaattcttcccatccaagacactcttgaacacatcaagtcctgctttgaagtaaacctgagctgaattaatgctgttcaacacctctgacagggcttcttgaagggtctcatttgatgcaaggggtttgcagtgttcccaagcctctataagtattgaaaaccggcttgtcttttcatcaaggtggtagaggatgtttctataaaaacctggtggtgcctgctttaccagaaagcttttctccatgtcttggagaatgtcattcagcatccggatgcggatgggtgctctctccttgggatcattagcaggtcgcatctcatcagactgaaaaagttcagcactctcccgcaggcgtaacgccatggctaacagttgatgagtgttgggttgatcacctttaaggttgttttgaacttctaaagctatatcaagtgcattaaagggcagaacaggttcgttggcaatttgcaaaatcacttctcctgagagcttagtaatggtttcatgaaggttgaaagagggatccatttcttcaatttttgttgctcgtgtagaaaaacgggcctcggagagaaaacttggaccctctactaccagttgctgaagagatggtgatgctacaggatacagactagagttcccccttatgggactgtggaggctaatataagccacaacatttttctgaagaaccttcttgaaatcctctccccattcatatgagccaatattgccaaaagctgttcctccccaagaacagaaaacaatagttcggtctggtctccaccctctcttaacttttgacatcaaggcacggataaacgctgtgattattgcagtactactggcccattcttgtccattataactgtgtgcagtgtgatgatggctgccaactatgatataccggtctggagatgtcaagcccattacaaatccaacaacattagtaactgttttcaattttgtgactgtctgaacttgcatgctgacgactcttatttcattatttggaagctctagagagctacacgcttcatttttggttctagcttttggcgaagagatcagttttgcaacgaggggtgcagagatgggctgcactaatagagaggtgaggtttgatcggctttgtctaaaactttcatcgacacttgggtaaccaggcgtagaagggtctcctcctggattcagtgacaccatgaaggtatcatggctaggattcacagtctttggcaaatcacaaggatcgatatacagaagaacacctccaaatccagccttttccaatgaggaaagcttataaagcagtggcaattttcctaatttcaggagtgcgatctgatttgttacgttttttattttcctaatcctttttaaatcatctgccattccataactcacatcgatgacttcagccttgagagttcctttggcagaataggctgcatatgaatagagcaggtcttggctgctatcttttctggcttcttcactgcaaggctggccattaggatgaaagcattgaccactgctgctcagagtcacagtgctgggagaagggcctggcagatcaagcagcacagagtaatttacaaactgtacatcttctaggcccaaagaggtccactgagtcttaatcttctttgaaatttccatgtcatcttcatttttatatagttgtaccaaatttctgaaagacttcttaatatcttctgcctggattgtcttgagaatctcttgatataactgaggatcaactgttcctgaagatggagcatctgaagggcaatttgtatgtacataataacctatcaaaatcccaaaaataaataaaatggtggctgtgcaaagtatttttaagacgtggcaaaagttgcagcgattgctctttggtgcagatcgtgtataatgggtaatgtagtcagattcttcttgaagtctctggaaccttcctttgggtgaagttgctggttgaatggaatcaagattgaggtctatagtctctgaatgccctaggttctgattctcagcaccgtctagctggaattggtcaaaaccagactcctctagttccttctccatgtcccactctaagtcaagggcagtggcttgaaggtcatcattgtctaagtactgtgagtgtcctggagctctttgatctgcatggaccttctgataggccatctttttaccagtcacctctttcattatccatcttctagcaatcacttccatccactgcctcatgccaatgtcgagtgccattgcttcaaatgctgtatacagtttttacttgtttctggaaagagggtaaatccagtccttgatattttaaccaaatgcacaaatattttttcttccacatttaattctacaaatatatttgattgactgtcctacccttatgaatcagtcactatgtcaaaatgaagcggactatacaattagcaagaacctagtctcatatccaaacctgtggacctatgtgttctattgccagtatcagggagaaagagtaaaagcatactccagaccaccaaaactaatagctatcagaatccacttcagaaaatacgttcttatcttaaaaaaggacttttgggggatggcaattccattgcactgatttgtggtttagtgcatcaagcattcctcaggcacattcggtgtgccaggtaaggtggtggcccctgagaaccgtgagataaacaagatgcaagtgcagcctggaagctcatattccagagtttccctttcgccctgcttgtcagttttgcgaaagcattcacagcccctacctcttctgttcacctctcccgttctaggcaatagtcatgggatagctttggcctaaaatggtacattattaatttggggcccatatttcagatgtcacattttaaagatgaagaaacaagggaagaggagggtcaagtcacatgtcacaggtgaagtggccatcaattaacaaacttgatattgttgaagtgttgaatatgactaatatggtgtgtactgaggcccctcactccccactgctcgtcccactattccacagagcgtcatcctgcctggactgcaggactggatattaactcctacctgcatatgtaaaattaactcctacctttcctgctattttaaaaccaaataaattacctcaccattcactaaataaaactcactattttcttatgtttactgcttattcctcagttcccacccccaaagtcaaggagtactattctcttttccttagctaactcatcagacccacatttaataaactggaaaattttttattaaataatgttgagtggaaaaaaggataacaaatttctatgtaaaaagtgatgcagttattttaaaatatatagttatacacacacacaaagactttaagttagcatgccaaaatattagtaatttttgaaaaatctggattgttaatttatgggtaatgtttactttactcttcacacttttttgtttctaaccttctgacgatctctatgtgatatatatatatgtatataaactattaaaataaagttattcttaaagccaatctctaaaaaatcaactacattctgattaaaatctctgatgaacacaatttagataaaattatattttatttgtgctacagtattgcagaaagcattgcaaatacaatacattgcatatgtgattctttataatctctatttgaattatatgacacttgaaggcagaaaatgtatattttaaaaaatatcttctaatacttaacttgtgtagttaaatatattaaccaaatgttacaaatgttacaattgtgcatttcttgcctgggaatcctaaaggaaatcgaaataataaaaacagctgacaattatgacattcatactatgtgctaggttctgttacagatagttttacagcttctatctcatttaatcctcagaatagtccttttagagttcgttttatacatgaagaaactcaaaagtaggaagagatcaaattatctaaagtgccatagctagaacgtgacagagccagtatttgaaaccaagtaggtaaccccacagtctgtgcactaacccaccacacaatccatattttgaatgtttcaacaatattagaaatcttggagtagggataatgatataaagcagggatttgttaatacagattgtttatcatgatttcctcattactagtatctacctcaaaggactattttaacagttaaatatatgatcatgagtttgcacaagtgtctggtgtgtatagagtgctctataattgttttttgagatggaattttgctcttgttgcccaggctggagtgcaatggcactgtcttggctcatggcgacctctgtctcccgggattcaagcaattctcctgtctcagccttccaagtagctgggattacaggcacccgtcaccatgccaggataatttttgtatttttagtagagacggtatatcaccatgttggccaggctggtcttgaactcctgacctcaggtgaggtgatccgcctgcctgggtctcccaaactcctgggattacaggtgtgagccaccgtgcctagcctataaatttagctaatactgttacatgcatattttagctactgtgaattcagttaagatgaaatagctacacaactaaggagatctttttttttttttctgagtatgataaactaaggacatgccttaagtctaagaaaatctgtttactgcaggcttttctgcacaaattttcctttatcatcaaggttgctatagccatccctctttcggattccttttcttctttaaaattagaggctttgctttacactgttatttttaaatggctggatacctgccatagatctaataattggttgtaaaaatccagacaaacatcaatttttaattcttaatttttaatcttgtttgaaacaaacatgtaaactaaaataaaaacttaataaagccaggttcaaatcttgcctgttttagtatataagtcaaatttttattaaattaacttcagatcctattaattatgaaagcaagaggttatatttctaatgaatactaagatcttattagaaattccttctccatcactttgtttttctcttcattagatatacccgcacaaatgacctaaaattcaacccactttgaaaataaattttcaaggcttagtgaaaaaagcctaatttctgtagccactggcctgtttctagagccatcgttgactgatggcttataaagcctttttatacagcactgacattttaaagatactggccagtctgaactttccatctggcgtgcttgatttcctttgtcccactttcccatagtgacttattctgtccttgagctctaaaactactttgatttaatttaggcctgggggtgtgaagacatggtgaaatttatttaaacaagagacgatagtaatgcctccaacagtgcatagtaataggaaagcaaataactgacttcctggcatttatttgtgtaataacttcaccaccaagtgcaaccagagaggtattccagaactttccatgcaattacataaaactagcaagagctagtcagcacttgtaaaatcaagtgggagataaaggaaattattttatctcaggccaaaaaaaaa

SEQ ID NO: 12620 - RNA, 11095 nt, Homo sapiens
  source 1..11095: mol_type = other RNA
gatctcactttgttgcccaggctattttctggatgtctattaaaaaaaaattagtcctgcacagtgttctagaaagggtttttcttttcagaatatccatattctccaagtagcaagttagaatataaggaatatttgccattaaacctttctgttagaaatgtaaacatgaaattgcctaatatagacctatctcagatgctaaatagaattgtttataacacctttggaatataattatgtgagctacacttaaccatctggcattttgcttcctgcggacaatttgcaatagcatagaaaaatattttgtttgtgtatttcttatcaaacagatatgctaaagttctgtttagagagtaatagcattttattctaacttttaaaataaggtagtccatttgcagcagcttgatatataagtaaacaaaaatttttaatattaataaaacactagcacatacactgaaagcatctaagaaattcaaaatataaaacacttaccaagtaatgaccatatgagtggtaacatattgaataaaggccctttgaagaagttggagagttatgattactgagcaggctagataattaaataattacacattttgattgaaaaatatatgtagttcattaaaatagggactctaactccacttctctagctaagcttctattcagatgccacgtttgtactttaattagaacaaaagaccgacattaacttcaatgcaacataataattcataataatgattgtatattaatctcttgagcttgcaggaatatagcacatgacatatggcatgatacaggcacctgtgtgatcctttggggacttaggtggtgcatattaattagcccctggaaaataaaatctgtttccttctgagaaaagctacctcagtgcttattggcttaagccatcaaagaaattagatgaaatactgttaggctgggtctgcactcattaaagctttgtctagatgtaagcactgaatcaactgcctctgagttaagtcttgactgaatggtgcataagaaatcagagtaatcatgcatttctttggccttgatgattggattttggcatttaaaaaatccatcaaaattaccattttggttacagaaaattatgtaattgtataattcaaacaaaataatgtaaccagaaacactaaaatttgaagccacttcattttcctaaatgctgcttgaaactgcctcaatttaacccttttatttgtaaattcagattcaacccgaatatgagattataaatggcttaagaaatatgtcatcttgcaataatcagggtaacaagattcttgacggtcccaggtctgctaaaggcacttcagtgtgtatatctttgtcaggcaatggaacgatattatgaaactaaaactctggctgattaacagatcatttaaattgagactgatagatcttaaaattacttctcagggggaaaaagttacaatgctagagtgtacctagaaaacagaaacttgagtagacatggtaatgaccagaaaaggctatctttatacatttcttttgctacgcttcaaattcatgtcacctaaaagttgtgaagtgcacaaaacaaatctacttaactgaaaattattttcaatgaatgggatgtttagaactctgtgagggtttttaaggtcttttcgaatagcaaattctaatgaggcttttttaagttggcaatttaaactcatacaagaaataaaaactcaccagtgtggctgggcagaatatatatattttctcaaatattgtttgtttgttttttccctgcactgtatccatggtcccatgatgaaactgttatattgctgatatatttattggaatatgtgggccaacttcctttccactcaacatatggattggtagtttaaaataattcctttctattaagcaaatgtgtggctaaggcacatttaaatagcccattaaaccaatgagatgacaatgtgttaccctcagagaaagcttaatttttggagtaatcaattacacatatcacagaatgtctcatgagaacatttttggctaggtctaccaatttatcatacaaataattatagattttcatttgaggcaaagatgctgattcatcattagtaacatggtcacaaataatcatttattttatttttgttaacatctgtctttcctgtggggaaacttactatatgctctacgtttatttaatttaaaaagtcaattggttattctgaatttttaaaaataacataaaactgttgttctaaatcacagcacctgcttttctttttttagtgaaattatataagcatttagagaatgaaagtgtaagacttgtggtttctggtctctttttactgtttgtaagcctactcgtcatgatattccacaatggtgcacttgccttttaatgctcttatagatatcttcaaacttgcctacatatatacgcctttgttggagtgggctaccatcatcaggaatgatgtcatttgtttcttcaaactcctttattataccaaaaaagtgacagactccacagtctgatcagttttggagaaatatgttaacattttcaattatctcactttctagaatcaaaatagtctgattttttttttcggcactcagtgtaaagaacaaagaactgaatacagtgggcccagaagagaaatatgcctcatcatttttattagctttggaactgtggacaagtcactcaacctagttttctcattttgaaatgggttgttgtgggaattaaaaaaaaaaaaaaaaaaaaaaaaggatacatgggaaaaattctaaaacaccagtgcctgggatgtagcaggcacaaatataagctgcaactgaattgttttcttagagataaaatgggtccacttttcttttctcataatgattccattaataacaaatctttacgtctttcttgttattatgactcttcaatttatttagaaatgtcaattagtgttttcttggaaactacgattaacgtagattggaaattcttaaacttcagtgtgtgtaacagacatccagaaatcttgctgaagatgtagattcctagccctgtctttctaaatttcacattttgagaaacggtgatttagattgttgacttaacactggcctgacttgccctcttacagatatattttgctcaatgtccttcttcctgacttctggtgttctgtaaggattctccccactttctctcaagtacccagtctttgtgtcctttgcctgaattctcggggagagttttgtttgtcaggtacagtcagagaatgaactagccttgaattaaaagcagtgtttccagcccatgcaacatctgacagaatggctggttacatcgaatgcactggaaaagatcatttataaccctgtctcctcagggagaagcaagatatactgcatgagaaagcagagaagcttaaattccagtggtgcttttgttactaactaaatacatgactatgtccaagtttcttactcactttgggtttagttactatatctggtgggggtaattgataatgccttctctggctgaaggcaagatctcagggcttagaccagaatctttattaggctttcttttgattctgagacttatgcttttccataaagggcagtatctcatgtgtaccctgcctgaacataaatttcaccgttacacctttaccacattttcttcagagaatatttatgattcattatttcctaggcacaattctatgtatgaaagattgtgagaagtaccaggcatatagacgactcagcaacagcttaaacctactaccaattcacattaacacttgctattaatttgctcaggattttatttatttgaatctattgggggtggggaggggaggggagtgaaatgatatacatttggaggcaccctcaggtaatcacactatagaaataatgctgctagttaagaggtttgttgcaaagatgtaaagcagcatgtacagaatttgttggacgtctgctttaggtataatttaatatctccacgtatcttttaatagactaataaaaaaccatagttaactacagttttcaaatagcaaataacatataatttagaggtgaggaatacagaagaaggtttttatctatacagtgtgacttacctaggtacgcaatctttaaacaaaatgaagaagaaacatgttttctgttctcagtgctattgtaggttatgggaataaattaatttagaaatttgttctaaaataatgaactaccaaactgataatagcttgcctttatttgttttagtttcatctgtaagtgaataactggaatgaacacatcaacctttggttaaatataaggctttctagcttttgggcttacatgcacctgcttgtgtattcccacctcttttctgatgatctctgaagaggaagaaagagcatgaatgcctaggtatgcacaagcctatttatttctagacctttcctatacacactcttcaacatggcaaatgtttgcaaacaaatacattggttaaaaaaataatattgtaaggtagtttcatttttcatctaaaaatatgtgcacacaggcaatttcgatgaaaatggatttctgcttgaattatctagctaattgcctctattccctgctttgccttgagcatataaaaattatttagggtagacagtgttgaaccttataaatcaattaatcagtattgattaattatttcccctcaactttagtttgcctttaaactaagactaggtttatgctcatccataaaaagtgaaaatttaaacatacacagactgtctgcaatgtcactctggcggtgtatcatggggagatatgtttgaattagatagagaaaatttatatgaaatactctgaggctatgtttcctaaggggaattgctttatccagtataggaaaaccatttttcacataaatttctaaagataaattagaactttaacctgacacctaataggtagaattttagggtttgggggaataataatagttgctagagctattcaatggcaatgtcaatataaaaagcttagttttccacatgagagaagaactgaagtgtagacgagacactctcttacagtaacactgcagaaacttagaagcatgaatattttctagatttccatcttagtcacaattaaggataaagaagaaaaaatatgaaaagtttcttcataatattaaggggcttttattgataaaacaactatttctttcatagtaagttctttttgtcagaggcagaaatagaaatttgattctttagaagacattttgggtttcaaagagaaactctgctactttactgttgaaaatatatagtactctgagaaagctgccttacagcaaggagtttcagaaaagatacaagaaagaaaaccaatgtgagatgctttcattttagagtccctgcttcagtgtttccaacagaaacaagagaaaaagtaataagaaatatttttttctccctcttaagacatacatcactcctgaaattcttagaaaatcaactgaggcaaattaggggtttcaaagctagtcaccttgtaagttgttaggaaaaaaatttgcatttaaattgctctatgtagctcccttgagattttctcctggaatgcttatggctcttttttcattaatacttaaaaaaatacaatttcataaccagtgtattactacatctagttgtgttaagaagagaaacttcatttcataaaatagaaacattcaaagtggtttaggtcaaccaatcactcagtcagaatacttgaattcttcatattgaacacttaatagtgaagttaatctgaaccatatcaactctccatttcttttacagaaactaagtcattaatagctctatcagagagaataaactgtgttcctatatgccctccccataggaacaaagatagtccagaacttcttggaaatttttccttaaaatagtacatatttttatatatcagatttctttttaataggtaattcttaagtcctatttcaataacttgctttacatattcagaaatgtagatataagaaaaatattaaatgtgcaaaatgttctttctatatttacatttaaaaaatacaatgtaataatagctttatacttgtcaaaaagccattggggaaaataagccttcaatgtcagaaaatctggttaaattagagcttttgcttgtggaattgtaaacaaacttttaaaaatgctcagagttttctcaattcttcccatccaagacactcttgaacacatcaagtcctgctttgaagtaaacctgagctgaattaatgctgttcaacacctctgacagggcttcttgaagggtctcatttgatgcaaggggtttgcagtgttcccaagcctctataagtattgaaaaccggcttgtcttttcatcaaggtggtagaggatgtttctataaaaacctggtggtgcctgctttaccagaaagcttttctccatgtcttggagaatgtcattcagcatccggatgcggatgggtgctctctccttgggatcattagcaggtcgcatctcatcagactgaaaaagttcagcactctcccgcaggcgtaacgccatggctaacagttgatgagtgttgggttgatcacctttaaggttgttttgaacttctaaagctatatcaagtgcattaaagggcagaacaggttcgttggcaatttgcaaaatcacttctcctgagagcttagtaatggtttcatgaaggttgaaagagggatccatttcttcaatttttgttgctcgtgtagaaaaacgggcctcggagagaaaacttggaccctctactaccagttgctgaagagatggtgatgctacaggatacagactagagttcccccttatgggactgtggaggctaatataagccacaacatttttctgaagaaccttcttgaaatcctctccccattcatatgagccaatattgccaaaagctgttcctccccaagaacagaaaacaatagttcggtctggtctccaccctctcttaacttttgacatcaaggcacggataaacgctgtgattattgcagtactactggcccattcttgtccattataactgtgtgcagtgtgatgatggctgccaactatgatataccggtctggagatgtcaagcccattacaaatccaacaacattagtaactgttttcaattttgtgactgtctgaacttgcatgctgacgactcttatttcgacacttgggtaaccaggcgtagaagggtctcctcctggattcagtgacaccatgaaggtatcatggctaggattcacagtctttggcaaatcacaaggatcgatatacagaagaacacctccaaatccagccttttccaatgaggaaagcttataaagcagtggcaattttcctaatttcaggagtgcgatctgatttgttacgttttttattttcctaatcctttttaaatcatctgccattccataactcacatcgatgacttcagccttgagagttcctttggcagaataggctgcatatgaatagagcaggtcttggctgctatcttttctggcttcttcactgcaaggctggccattaggatgaaagcattgaccactgctgctcagagtcacagtgctgggagaagggcctggcagatcaagcagcacagagtaatttacaaactgtacatcttctaggcccaaagaggtccactgagtcttaatcttctttgaaatttccatgtcatcttcatttttatatagttgtaccaaatttctgaaagacttcttaatatcttctgcctggattgtcttgagaatctcttgatataactgaggatcaactgttcctgaagatggagcatctgaagggcaatttgtatgtacataataacctatcaaaatcccaaaaataaataaaatggtggctgtgcaaagtatttttaagacgtggcaaaagttgcagcgattgctctttggtgcagatcgtgtataatgggtaatgtagtcagattcttcttgaagtctctggaaccttcctttgggtgaagttgctggttgaatggaatcaagattgaggtctatagtctctgaatgccctaggttctgattctcagcaccgtctagctggaattggtcaaaaccagactcctctagttccttctccatgtcccactctaagtcaagggcagtggcttgaaggtcatcattgtctaagtactgtgagtgtcctggagctctttgatctgcatggaccttctgataggccatctttttacttcaattgaatgttcctagtgcaactggagggcttctgcaggttacaggagactgacaatctggacccagtcttcatccaggtgcctaatagtcaatgctcatttccctctgttaagttagtttccttcctcctcagtttttcacactcatttcaatatcttccatcttccttaagcttgtttttaatcgttttctttatagaaactaaatttcatttaaattattcttttcttccctcagcctcctgagcggcgcgggcgcgggctcgtctgcggtacggctgccgggccaggccggattttcagcagccgtaaagcgggagaagcgggcgcgagccgcggcgcgaaccctcgcccccgagcggcggccccggcgcctccgccgcgagcgtcagccgcttggcaaggaacgggctgggctgagtcataataaaagacgcgtttgtcgagccaagtgggaagaagagccgcgggcagcagtgttcaatggcacaagcctcaaaaattgggaaggattttttttttaatgggcaaaactggaaacttgcccccatggtgcccatcaaaagatatgtttcgtttataatttgcatatattttatacatagtctttgaatctaataaaacttttaaaagaatttttaaagcccattgcttgcagagccaaattcctggttatagcttcgtgacttacgcaagttacttgaattctgtgcttttgtttttcatccatgaaacaggataataaaggtacctccctcaagagagactgcgagagagcttggcatcctgcctgcacttagcactcgctaaatgttaattgttattttaaaataggagggaggagataataaagaggaacttagataacagttttgaatggaagaagatacgaatataaatcaagatttttcttttttcaagtggagtaaattagacaaattaccaatggaagagaagaaagtggagcctggaaggaacaaacggggctaagagaagtagctgaagcgagggaaggaagaagggggaaggaggaaagaagagaggaagaggggtgaataaaagcctccaaggaacaaacgaggctgaaagatgtggctgaaggtagggaaggaagaaaaagggaggaagagaggaagaaataaaaccaaggaagcaagaataaagctaggctgcgtgggaagaggggaggaaggaaggagagagaaattcaactaggctcagtggccaaaatgctgaagtgtgtcctgccgggagggagtggaggaatatgtttactcactatttagaaatgcatgacaaactccatccgctgagggagatttttacaatgtataaacagagaaacaactgtctaaaaatgagccccaaatgaggagcctttgctccagtgaatgagatttggcagttctgcaaaatgaggaaattcttccttgtgcggcatcttgaagggttgagtcatgaaacccacagcaaatattagtgggctggattcctgaaaggcatgccagatggacgcattctggttagttttactgtgtgatgttcccttctgtacttctgtcaattttagaagaaaagagtgtgaataaagatttgagaagtgaacttaaaagccaaactagttacttaatgtacgagtatccacccaccaggagcttacagttacagattccaaaacaagcaaccgtttctcccactttcattttccctcccctttgtttctactttcaccgtattgctttttatccatttttataatatgattttttacagtggaaccgcctacgggaaaggtgcttttaattaatacgaaagaatggaaggaatttcagctaggcctctctaagagggtaaagctttgtgaaagaaaggttttttagctgaagttttaatgagaataagagtagttggcagatgtgaaatcagaagttttttcagacaagaaaataatacgactcgagtgaaagggaatggactagaaatcagaaacagttctattccttaattaccgtaagaaccaaagactggaggaaagtttttcctattctataaagaaaaatgggggcctccctccaccagccagaccttcaaaaaaggaaaaaataaaaattaaaaacctctattagattcttgtaatgatttgctttttcttaggagaacttcttcagggtaaaagacgtgaaagtgcttctttcggcaacttctgacgaaatacttttgtagaagcaaaatttctgaagggataatttttgctcaagcaaaaaactattagtaagataagaatcccttttcctttgtttcaattttgctaagccttcaggctgaggcaaacagattatcattaaacctttattaatgtgaaaccaaaaaaagataaaatcttaaatgctgcgaagcccttaacctaaaaggagcaagaaaacaaaccaaggcccagaaaatagagaaagggattaggaagcctttctaaggggaacctttgaactgtgggctgtaaaatgaatgtctgtgacttgccttaaacaaataggcaatataaactaaagctgggaactaagaagatctcctcagatcagataaaaagcttaccttgtgtgaaacactgtggtcaaagaagaaaattcctttcatcttaagtggagacaaaaacgtgtatcacttgttttgtgtgtgctcataaaacacctccatcacctgaatcccttgggtgcaattttttgatggacttggcattctttaaa

SEQ ID NO: 12621 - RNA, 6765 nt, Homo sapiens
  source 1..6765: mol_type = other RNA
gatctcactttgttgcccaggctgcgattctactgcctcagcctcctgagtagctgggattaaggtgcacaccaccatgcccggctaatttttgtacttttagtagagacggggtttcaccatgttggccaggctggtctcgaactcctgacctcaagtgatctgtccacctcggcctcccaaagtgctggaattacaggcatgagccaccgcacctggccaatgtatcttggttgatttcttatgttacttgatctctgtaacatttaacattgttaactacttaacaatatagtcttggttttctcccaactctaagggtagttattcttctgtttaagggatcttctgattaaagtttctacatatcatcttaaatctctgaaaaatctgaaatcacttcagtatgaagttttccctaaggtccagccttttctcttttcacagcaagtcaagagatctagtgatagaaaatcttttaaattatgtgaagctgattagtgacacatagaggctttgcctaagcagaggtggggcagctgtgtcaatgatgcagctatgcgggggctgagatggactctaggagctgttccctgagattgagagctcatcacaatttctccacatctgtagaggctgcagaagaactgaaggagcagctgaggtcagtgcctctttacagctcttatgttcacaacacaatcagagttgtttattctggcattcaacatggtctgactctgctgaaacatctcctttctaaggctttccagaagggctgtctaggaaaaggaggaaatggagttggtgctgtgtgacttttaatgggataatccaacagcaagtgattagtcacctatagaatctaaagctaagcaattaggatttggctttattttcactaacttatgtggatcctcagtgctctacctttagacactgacaagaagaaaaagcatacatttgttaagctgggtccctgtagcttgtgtggaggaaatggtctcactgtgatgttgtaagctgggatcagagacccaggcactaattcagattcttctgcttgatgatgttgtggattcactgtagtgagtttggtccaagaaccagaagaagcttaatatctccaaacattctcttaaatggaagcattaagagcagacattaagtttttcttgagcactgatgtagccctaaggataaaaaagctgtagtgtggaattcatttccacactttttatccagtgccgtattttgggcattgtcatcaaggacgctggaccatgggaagctgtgctgatatatacggttcatttacacttgctttgtggccatcatatttccaatgtgattctatattcttgagtaaataaactgggaactcaagctaatcttatacaagtgtatatgtgtaatcttgatacacctccattgtccacctgaaacaatacagcttataggtgtgttctgaaaactaaagttgttacaatttgtttataattaagtaatctttttaaagagttagaagaatgtaagtgcagcattaatatttacttgacttttgtttttaaagtacttcaccaaaagttcattcctgaaagctgagctacatctgggctacttcatgttgtggactatggaagatctggtttaaaacttattttcatcaccccgggtgagtcatttactcttacacaaagatgtcatgagaatgagatccctcaaaacagaaaaataaccacccttagagtcggaggaaaaaaaaagtttaggtctcttaggtgtgggtgcaatggtgatggtagtactggggaaggaagtagtggtactggtagttagcataatcttatgaaatagtcataggatttcatatttcccttaagcatttttcatttattccagagaaactgtcaaaaacccataccctcgcatataaaacattcaataacctaagaaaaaaggaacttcctcaacatgtagagtacgtatgaaaaagccagagctaatgtcatactcaatggtgaaaagactaaaagtttttctcctaagaacaaaaacaagacaaggatgtcctcttctgctacttttatacaacacagtactacacatttttgccagagcaagtgagtaagaaaaagaaagggtatccaaatcggaaaggaagaagcaaaactatctttattcacagatgatatgatttatatgtagaaaaccctaaagaatgcaccaaaaaactggttagaactaaatctgcataagtcgcaggatacaaaatcaacacaggaaaatcagttgtatttctatccattagcgatgaacaatttcaaaaggaaatgaaggaaactattccatttacagtagtatccaaaagaataaaatgcccacaaataactttaagaaagtgaaaggcttgtacactgaaaactaaaacactgctcaaagaaattaaagaagacataagtggaaagacagcctgtgttcatggattggaagacttaaaattgctaagatgacaacactccctaaagcaatatgagggttcaatgcactctgtaacaaaatctcaatggtgttttgggcagaaatggaaaaactgatcctaaaattcctatgaaatttcaagtaacccacaatggtgtgtgtgtgtatatatacatatggcatgtatatatatgccatatatatatacgtgccatatatatatatatggaagaacaaaattggaagactcacacttccccatttcaaaacttactgcaaagctacagtagtcaaaacagtgtggtactggcataaagacagacatatagaccaacagaagagagttgagagcccagaaataatccctcacatgtgtggtcaactgatttttgacaagggtgctaagatcattcaatgcagaaagaacatctcctcaacaaatggtgctgggaaaactggctatccacatgcaaaagaatgaagttgggcacttacctcataccgtatacaaaaattaacttgaaatggatcaaagtcctaaatttaataaataaaactgtaaaattcatagaagaaaacacaggagcaaatcttcatgactttgcatttggcaacatgaaaagcctaagcaacaaaagaaaaaatggataagctggacttaataaaaattaaagtctgtctgcatcaaaagatacagtcaaaagagtaaaaggacaacccacagaatgggagaaaatacttgcaaaccatctatctgataagggcttaatatccagactctatgaagaaaagacaaacaacccagttttaaaaataggcaaaggacttgaatagacatttctttaaagaagatacaaaatagacaataagcatatgaaaagatgctcaacatcattagtcattagagaaatacaaatcaaaaccacaatgagacaccacttaacagctaccaagatggctataattttttaaaaaataacaagtgttgccagggatatggaaaaactagaactcttgtagattgctggtgggaatgtaaaatggtgccttcactatggaaaacagtttggtagtttcccaaaaagttaagcatagaattactgtatgactcagaaattccactcctatgtatacatccaagagaactgaaacaacagataaacaaatagattattatatgtaaatgttcatagcagtatcattcacaatagcccattggctattaatgaaaacaatctaagtgcccatcatcagaggaatggataaacaaaatgtggtatatatccatacaatggaatattattcagtcataaaaaaggaatgaagttctgatacacactacaacacagatgaaccttgaaaatgtgctaagtgaaataagccagatacaaaaggtcaaatgttgtatggttccatgaatatgaactgcttagaactggcaaattcacagaaaggttaccaggggtaggggataggggaatggagttattgcttaatgagaagagtttatgtttggagtgatggaaaaatgttggaaatggatagtggtgatggttgcctaacattgtgaatgtaattaatgtcactgaatttacacttaaaatcattacaatggcaaattttatattttatcacacacacaaaaataggcaaaggtaaagtttctacagtctcatgaagaaaagattaaataaaaagcttagtcacacctgacttgtgtgacagtaaaattatccctggacttgaggtcagaagatcagagttaactctcgatctcttgaccttgtgatctgcctgccttggtctcccaaagtgctgggattacaggcatgagccaccatgcccggcccagagttaagtctcttattgggctcctggtttgcactcttgggcccacaagagttattctctatacagccaccagaaaaaaaaagaaagaaagaaagaaactaagtactcatctaaaaattatctaaaaaagaacaatgaaagaaaccagaagaaactaggaaaaaattaagaagaatgaagtaaaaattaattaactagggaataaaaattgtagtaagtagaataagtaaaaaagcttatactttgaaaatacctatagataaaacatttgcaagactgatcacaaaaaaagcaaacattgacaagattactatccagaaataagacataaactctgatataatacatactgatagaattctaggacaataaatagagcatgcaggtgtgtgacagcagatttgaaaacacagaggtactaaatggtttccatttagtatatggtgaccaaaattgaccaaagtagaagtggaaaactgaaaagaccaatttcagagatgaaattagaagagttatttgacgtttaatggcaaaaaccaccagggaagtttggataaactattacaaatatcctctcaaaaccattataagagatcaagagaaagtaagggaaattcccagggaaccaaatagaggtgaaaacaggaggagtaagctacagctgggaccgaagctctgaagtccagcttgccaacctcagtaacaaaggagtttagaatacagtgactgtggcaggacaagacatagtcccatgggactacataaagtagggagaggaactgagaccctgacatgaagctggggcaccagaaatgaaaaggtaaatcagaaaaaaaaaaaaaaaaaaaaatcttccaagaaagctcaggtgtttcagcaagggctctaggtgggctctgtgtgtttcttccctatcacattctcaagtcattccctcaagataactattatcctggattttgtgtttgtgtttacacagagttctgcttgattttaagtaaaaaattgtatactaaggtagtcttctgtgacttgagtttttcacttagtattgtgtttatgaaaaaatttaaaccctatgtttactgataaccacaaggaataacagacacaatatttaataaaaaaaggaacaaaatatcgaaaccatctatatactgtaatgtacctttaaaccaatgctagggaaaaacaaagggaaaacacaaaactgcaataaacttcatcttctctcccaggtttttcttgaacaattcccacccccattccctactatgtatccttaacttctttagacagtgaatgagaaattaatactaaaagccctcaaatgaaccctagggacatttcctgggttttcccttcttctcccctctccaaccgtgccgtgaagggcaagcccctcagccctaaaatctgaggaggcccagagtggtggctggggcagaggagtgggctacccctgcagagtagagacgtgtatagtgggggatatccactgggagccccagtcccaggtgaaagcacactggtgctcctgggcaaggaggcccggctgtccccacaatctcccgtggggaagcatcattggttggtcgactgcccatcttgctgcggttatagaaccaaactcgaaccacatccttctgcagctggaggcacccagcaatgtggctgatttgctggggtgtgggcttagggcaccgctggaagaatttctccaggctgtttccgattcgtcgctctctgcttgcccgtctccacttcccagactgttgcaggatcatctccattttgcataagcccagaaggttctctgcttccacttccttcagccactttttcagcagtggtcgcagcttccacatgttggcgacgcttagctgctgggcctcgaagcggcagatggtcgtctggctaagcaccttcccaaacagagctcccacagcgatccccacatcggcctgcgagtaccctaggctcaacctcttctgcctcaactccttggccaattgctgcaactctttcagtatgcccgagatgtcctctggcggcggcaacttcggaatgctccgcagggcaatgtagggccccgggagggcgccttcggaggggcgtcgcaaccagtcccctgcctcactagctccaagacggggcctgcagggtgctatccagccccggaattcgtgtggcaggggacccaggggaatcctccacacgtcagggcctgggcagatccctggcctgactgccggccagaccatcaccctgccaggggccgcctgggtgctcaaccaggtcagagtgtcaacccgcaggggcatcggccctctggggccgcccccaccactgcctggaagggggcagaagtggtttgagggcctgtgtccggccatgggtggaatggcacccgcagcggctctggtaggaact

SEQ ID NO: 12622 - RNA, 2459 nt, Homo sapiens
  source 1..2459: mol_type = other RNA
gatctcactttgttgcccaggctggagcacagtggcgtgatctcagctcgctgcaacctctgcctcctgtgttcaagcaattctcctgcctcagcctcctgagtagctgggattacaggcgtgtgccaccacactcagctaatttttgtatttttagtagagactgtttcaccatgttggtcaggctggtcttgaactcctgacttcgtgatccgcccaccttagcctcccaaagtgctgggattacaggtgagccaccttgcccggccgaagttaaagatgcagtttgggataagaccatcataaggatattttcttcccctttactcataaaagttgtcagcttaggccgggcgcgatggctcacgcctgtaatcctagtactttgggaggctgaggcgggcagatcacctgaggtcaggagtttgtgaccagcctggccaacatgacaaaaccctgtctctactaaaaatacaaaattagccaggtgtggtggtggacacctgtagtcccagctattcgggaggctgaggcaggagaatcacttgaacctgggaggcagaggttgtagtgagctgagatcttgccatcacactccagcctggaggacaagagcaaactctgtctcaaaaaaaaaaaaaaaaagttgtcagcttaaaaaatccttcaacgagagctttcttatgctctaaaacctttctctttattttaaatctgtctgcagtgtttgaaggcaagacagataatcagcaaacttacctcgcaatataaggatctgagctggactcctgggattacagactgtggtttagttccatttctaccagcactgtgatgtgaggtactatggttcttttagttacaagaggtgttaggaatgaatgcccactcacatttaataatagcttatgtagcacacaactctgcagcataataccaacaacaggagtgttttaaagcaggatggagaagaaagtagacaatacaacttaaggtttcctttgtcctttcccctgttttcaccatgagaattcagctgaaaaacaactctccagaatgcccacccatattgtcctttgacccaccacattccaaacttctgacttctgatcccaagctcttggagccttagcctttagtgatgtatccttctctgatgaggaaatcatagattttccgggttttgttcacatctatcttgatgagtgctcttgcctgcgccagtcttaagcctccttgcttgttacattcgttcaatagagcagatttgtattctaaataggctccagggaccaacctcaccatctgacagagctccttttctttttcattcagcttctctgtgccagggaggccagtgaggttcaagggtggtgcactccgtctacctgaattcgaagccattggaatggaaggactcaggccggaatcaatgtcagcttgccggcggagccactgctggcaagcactactgtcctggatatactggagaacttctgagagcatagtgcgtttaaggcgctcttcctcccgtgtcttcttgaggtgatcgtaggttctggcactacaaaaattggtaatgcctgctgtcctgtattcttggagcctcttgatttcccttcggagttcaaattccaatgcatggctttcaatgaatttgtcatgttccactggccccacaattcttgcaaatcgcctcattgtttcatacaggtcctggacctccttgggataccgccgttccattaattgaaactttctaaggttgattaatccatggtctcttataattttttttcgtctttgtctctcctttaacctggaatgatagatatctaccacagccatcttcagagagtgaaatggaatggctgtgtcagcagtttttgcttcctctgcttgtttcaggttcagcagggtagatgcaaacagagggttattgatgaaatgcttcatatagtgcttctcacactcctccttggtcttggtgcacatttgattggctacatcctgccaatttccaaagccacagtccatcacagcttctaaaagggccatttcttcttgagcagtccagctgggatcaaggacaggaaaatctgaagtcattatttcataagtatgatcgctttgatgtttcttgtactcaaagcctcgagtgaaacactgcaagcagaggaaaaaaggaggtggcccacattcagcacacttgatataaggctccatgaggtaggaggagcagcctcggcaaggtggcttatcagagggatcattgctaaaggaacccaaacggtccattccctaattggcaacgagtgctgctttggtcttcctcagcagagcttcttcaagacttcagaaccggccaacacatacaccaaagcttgatgactccctcgccgagaccccctaatccgcgccaaagagccgccggtcgcgcgcgcctccgggctttgcgt

SEQ ID NO: 12623 - RNA, 2532 nt, Homo sapiens
  source 1..2532: mol_type = other RNA
gatctcactttgttgcccaggctggagcacagtggcgtgatctcagctcgctgcaacctctgcctcctgtgttcaagcaattctcctgcctcagcctcctgagtagctgggattacaggcgtgtgccaccacactcagctaatttttgtatttttagtagagactgtttcaccatgttggtcaggctggtcttgaactcctgacttcgtgatccgcccaccttagcctcccaaagtgctgggattacaggtgagccaccttgcccggccgaagttaaagatgcagtttgggataagaccatcataaggatattttcttcccctttactcataaaagttgtcagcttaggccgggcgcgatggctcacgcctgtaatcctagtactttgggaggctgaggcgggcagatcacctgaggtcaggagtttgtgaccagcctggccaacatgacaaaaccctgtctctactaaaaatacaaaattagccaggtgtggtggtggacacctgtagtcccagctattcgggaggctgaggcaggagaatcacttgaacctgggaggcagaggttgtagtgagctgagatcttgccatcacactccagcctggaggacaagagcaaactctgtctcaaaaaaaaaaaaaaaaagttgtcagcttaaaaaatccttcaacgagagctttcttatgctctaaaacctttctctttattttaaatctgtctgcagtgtttgaaggcaagacagataatcagcaaacttacctcgcaatataaggatctgagctggactcctgggattacagactgtggtttagttccatttctaccagcactgtgatgtgaggtactatggttcttttagttacaagaggtgttaggaatgaatgcccactcacatttaataatagcttatgtagcacacaactctgcagcataataccaacaacaggagtgttttaaagcaggatggagaagaaagtagacaatacaacttaaggtttcctttgtcctttcccctgttttcaccatgagaattcagctgaaaaacaactctccagaatgcccacccatattgtcctttgacccaccacattccaaacttctgacttctgatcccaagctcttggagccttagcctttagtgatgtatccttctctgatgaggaaatcatagattttccgggttttgttcacatctatcttgatgagtgctcttgcctgcgccagtcttaagcctccttgcttgttacattcgttcaatagagcagatttgtattctaaataggctccagggaccaacctcaccatctgacagagctccttttctttttcattcagcttctctgtgccagggaggccagtgaggttcaagggtggtgcactccgtctacctgaattcgaagccattggaatggaaggactcaggccggaatcaatgtcagcttgccggcggagccactgctggcaagcactactgtcctggatatactggagaacttctgagagcatagtgcgtttaaggcgctcttcctcccgtgtcttcttgaggtgatcgtaggttctggcactacaaaaattggtaatgcctgctgtcctgtattcttggagcctcttgatttcccttcggagttcaaattccaatgcatggctttcaatgaatttgtcatgttccactggccccacaattcttgcaaatcgcctcattgtttcatacaggtcctggacctccttgggataccgccgttccattaattgaaactttctaaggttgattaatccatggtctcttataattttttttcgtctttgtctctcctttaacctggaatgatagatatctaccacagccatcttcagagcatgtaaaatgtccgagtcatcttcaacaaaatcaatgtctctcaagtcccattctgcataattgtcaaattcagtgaaatggaatggctgtgtcagcagtttttgcttcctctgcttgtttcaggttcagcagggtagatgcaaacagagggttattgatgaaatgcttcatatagtgcttctcacactcctccttggtcttggtgcacatttgattggctacatcctgccaatttccaaagccacagtccatcacagcttctaaaagggccatttcttcttgagcagtccagctgggatcaaggacaggaaaatctgaagtcattatttcataagtatgatcgctttgatgtttcttgtactcaaagcctcgagtgaaacactgcaagcagaggaaaaaaggaggtggcccacattcagcacacttgatataaggctccatgaggtaggaggagcagcctcggcaaggtggcttatcagagggatcattgctaaaggaacccaaacggtccattccctaattggcaacgagtgctgctttggtcttcctcagcagagcttcttcaagacttcagaaccggccaacacatacaccaaagcttgatgactccctcgccgagaccccctaatccgcgccaaagagccgccggtcgcgcgcgcctccgggctttgcgt

SEQ ID NO: 12624 - RNA, 2830 nt, Homo sapiens
  source 1..2830: mol_type = other RNA
gatctcactttgttgcccaggctggagcacagtggcgtgatctcagctcgctgcaacctctgcctcctgtgttcaagcaattctcctgcctcagcctcctgagtagctgggattacaggcgtgtgccaccacactcagctaatttttgtatttttagtagagactgtttcaccatgttggtcaggctggtcttgaactcctgacttcgtgatccgcccaccttagcctcccaaagtgctgggattacaggtgagccaccttgcccggccgaagttaaagatgcagtttgggataagaccatcataaggatattttcttcccctttactcataaaagttgtcagcttaggccgggcgcgatggctcacgcctgtaatcctagtactttgggaggctgaggcgggcagatcacctgaggtcaggagtttgtgaccagcctggccaacatgacaaaaccctgtctctactaaaaatacaaaattagccaggtgtggtggtggacacctgtagtcccagctattcgggaggctgaggcaggagaatcacttgaacctgggaggcagaggttgtagtgagctgagatcttgccatcacactccagcctggaggacaagagcaaactctgtctcaaaaaaaaaaaaaaaaagttgtcagcttaaaaaatccttcaacgagagctttcttatgctctaaaacctttctctttattttaaatctgtctgcagtgtttgaaggcaagacagataatcagcaaacttacctcgcaatataaggatctgagctggactcctgggattacagactgtggtttagttccatttctaccagcactgtgatgtgaggtactatggttcttttagttacaagaggtgttaggaatgaatgcccactcacatttaataatagcttatgtagcacacaactctgcagcataataccaacaacaggagtgttttaaagcaggatggagaagaaagtagacaatacaacttaaggtttcctttgtcctttcccctgttttcaccatgagaattcagctgaaaaacaactctccagaatgcccacccatattgtcctttgacccaccacattccaaacttctgacttctgatcccaagctcttggagccttagcctttagtgatgtatccttctctgatgaggaaatcatagattttccgggttttgttcacatctatcttgatgagtgctcttgcctgcgccagtcttaagcctccttgcttgttacattcgttcaatagagcagatttgtattctaaataggctccagggaccaacctcaccatctgacagagctccttttctttttcattcagcttctctgtgccagggaggccagtgaggttcaagggtggtgcactccgtctacctgaattcgaagccattggaatggaaggactcaggccggaatcaatgtcagcttgccggcggagccactgctggcaagcactactgtcctggatatactggagaacttctgagagcatagtgcgtttaaggcgctcttcctcccgtgtcttcttgaggtgatcgtaggttctggcactacaaaaattggtaatgcctgctgtcctgtattcttggagcctcttgatttcccttcggagttcaaattccaatgcatggctttcaatgaatttgtcatgttccactggccccacaattcttgcaaatcgcctcattgtttcatacaggtcctggacctccttgggataccgccgttccattaattgaaactttctaaggttgattaatccatggtctcttataattttttttcgtctttgtctctcctttaacctggaatgatagatatctaccacagccatcttcagagcatgtaaaatgtccgagtcatcttcaacaaaatcaatgtctctcaagtcccattctgcataattgtcaaattcctcaatgaaatctgctcgagctggcatgtacccggccatgtcccgagaaagcaaggagtcaaaggtaggtcggggagggtcatctgtagagtgaaatggaatggctgtgtcagcagtttttgcttcctctgcttgtttcaggttcagcagggtagatgcaaacagagggttattgatgaaatgcttcatatagtgcttctcacactcctccttggtcttggtgcacatttgattggctacatcctgccaatttccaaagccacagtccatcacagcttctaaaagggccatttcttcttgagcagtccagctgggatcaaggacaggaaaatctgaagtcattatttcataagtatgatcgctttgatgtttcttgtactcaaagcctcgagtgaaacactgcaagcagaggaaaaaaggaggtggcccacattcagcacacttgatataaggctccatgaggtaggaggagcagcctcggcaaggtggcttatcagagggatcattgctaaaggaacccaaacggtccattccctaattggcaacgagtgctgctttggtcttcctcagcagagcttcttcaagacttcagaaccggccaacacatacaccaaagcttgatgactcccgggagaaggaagtgaggcacttcgccgggcaggagtccacgttgggaggaggaaaggcgcaggctcccgagttgtggagccaacgttcaaatccttacggggtgggaccggcctgggccagtcattttacctgcgcctcagctctaacagggtactgaaatacctactttggggggcctgctaggaaattcaaatgggcaacgctggtcaggggcatctggcacagtggccattcttggtagagctacgcgctccagggctgagcgggaaat

SEQ ID NO: 12625 - RNA, 2621 nt, Homo sapiens
  source 1..2621: mol_type = other RNA
gatctcactttgttgcccaggctggagcacagtggcgtgatctcagctcgctgcaacctctgcctcctgtgttcaagcaattctcctgcctcagcctcctgagtagctgggattacaggcgtgtgccaccacactcagctaatttttgtatttttagtagagactgtttcaccatgttggtcaggctggtcttgaactcctgacttcgtgatccgcccaccttagcctcccaaagtgctgggattacaggtgagccaccttgcccggccgaagttaaagatgcagtttgggataagaccatcataaggatattttcttcccctttactcataaaagttgtcagcttaggccgggcgcgatggctcacgcctgtaatcctagtactttgggaggctgaggcgggcagatcacctgaggtcaggagtttgtgaccagcctggccaacatgacaaaaccctgtctctactaaaaatacaaaattagccaggtgtggtggtggacacctgtagtcccagctattcgggaggctgaggcaggagaatcacttgaacctgggaggcagaggttgtagtgagctgagatcttgccatcacactccagcctggaggacaagagcaaactctgtctcaaaaaaaaaaaaaaaaagttgtcagcttaaaaaatccttcaacgagagctttcttatgctctaaaacctttctctttattttaaatctgtctgcagtgtttgaaggcaagacagataatcagcaaacttacctcgcaatataaggatctgagctggactcctgggattacagactgtggtttagttccatttctaccagcactgtgatgtgaggtactatggttcttttagttacaagaggtgttaggaatgaatgcccactcacatttaataatagcttatgtagcacacaactctgcagcataataccaacaacaggagtgttttaaagcaggatggagaagaaagtagacaatacaacttaaggtttcctttgtcctttcccctgttttcaccatgagaattcagctgaaaaacaactctccagaatgcccacccatattgtcctttgacccaccacattccaaacttctgacttctgatcccaagctcttggagccttagcctttagtgatgtatccttctctgatgaggaaatcatagattttccgggttttgttcacatctatcttgatgagtgctcttgcctgcgccagtcttaagcctccttgcttgttacattcgttcaatagagcagatttgtattctaaataggctccagggaccaacctcaccatctgacagagctccttttctttttcattcagcttctctgtgccagggaggccagtgaggttcaagggtggtgcactccgtctacctgaattcgaagccattggaatggaaggactcaggccggaatcaatgtcagcttgccggcggagccactgctggcaagcactactgtcctggatatactggagaacttctgagagcatagtgcgtttaaggcgctcttcctcccgtgtcttcttgaggtgatcgtaggttctggcactacaaaaattggtaatgcctgctgtcctgtattcttggagcctcttgatttcccttcggagttcaaattccaatgcatggctttcaatgaatttgtcatgttccactggccccacaattcttgcaaatcgcctcattgtttcatacaggtcctggacctccttgggataccgccgttccattaattgaaactttctaaggttgattaatccatggtctcttataattttttttcgtctttgtctctcctttaacctggaatgatagatatctaccacagccatcttcagagcatgtaaaatgtccgagtcatcttcaacaaaatcaatgtctctcaagtcccattctgcataattgtcaaattcctcaatgaaatctgctcgagctggcatgtacccggccatgtcccgagaaagcaaggagtcaaaggtaggtcggggagggtcatctgtagagtgaaatggaatggctgtgtcagcagtttttgcttcctctgcttgtttcaggttcagcagggtagatgcaaacagagggttattgatgaaatgcttcatatagtgcttctcacactcctccttggtcttggtgcacatttgattggctacatcctgccaatttccaaagccacagtccatcacagcttctaaaagggccatttcttcttgagcagtccagctgggatcaaggacaggaaaatctgaagtcattatttcataagtatgatcgctttgatgtttcttgtactcaaagcctcgagtgaaacactgcaagcagaggaaaaaaggaggtggcccacattcagcacacttgatataaggctccatgaggtaggaggagcagcctcggcaaggtggcttatcagagggatcattgctaaaggaacccaaacggtccattccctaattggcaacgagtgctgctttggtcttcctcagcagagcttcttcaagacttcagaaccggccaacacatacaccaaagcttgatgactccctcgccgagaccccctaatccgcgccaaagagccgccggtcgcgcgcgcctccgggctttgcgt

SEQ ID NO: 12626 - RNA, 2742 nt, Homo sapiens
  source 1..2742: mol_type = other RNA
gatctcactttgttgcccaggctggagcacagtggcgtgatctcagctcgctgcaacctctgcctcctgtgttcaagcaattctcctgcctcagcctcctgagtagctgggattacaggcgtgtgccaccacactcagctaatttttgtatttttagtagagactgtttcaccatgttggtcaggctggtcttgaactcctgacttcgtgatccgcccaccttagcctcccaaagtgctgggattacaggtgagccaccttgcccggccgaagttaaagatgcagtttgggataagaccatcataaggatattttcttcccctttactcataaaagttgtcagcttaggccgggcgcgatggctcacgcctgtaatcctagtactttgggaggctgaggcgggcagatcacctgaggtcaggagtttgtgaccagcctggccaacatgacaaaaccctgtctctactaaaaatacaaaattagccaggtgtggtggtggacacctgtagtcccagctattcgggaggctgaggcaggagaatcacttgaacctgggaggcagaggttgtagtgagctgagatcttgccatcacactccagcctggaggacaagagcaaactctgtctcaaaaaaaaaaaaaaaaagttgtcagcttaaaaaatccttcaacgagagctttcttatgctctaaaacctttctctttattttaaatctgtctgcagtgtttgaaggcaagacagataatcagcaaacttacctcgcaatataaggatctgagctggactcctgggattacagactgtggtttagttccatttctaccagcactgtgatgtgaggtactatggttcttttagttacaagaggtgttaggaatgaatgcccactcacatttaataatagcttatgtagcacacaactctgcagcataataccaacaacaggagtgttttaaagcaggatggagaagaaagtagacaatacaacttaaggtttcctttgtcctttcccctgttttcaccatgagaattcagctgaaaaacaactctccagaatgcccacccatattgtcctttgacccaccacattccaaacttctgacttctgatcccaagctcttggagccttagcctttagtgatgtatccttctctgatgaggaaatcatagattttccgggttttgttcacatctatcttgatgagtgctcttgcctgcgccagtcttaagcctccttgcttgttacattcgttcaatagagcagatttgtattctaaataggctccagggaccaacctcaccatctgacagagctccttttctttttcattcagcttctctgtgccagggaggccagtgaggttcaagggtggtgcactccgtctacctgaattcgaagccattggaatggaaggactcaggccggaatcaatgtcagcttgccggcggagccactgctggcaagcactactgtcctggatatactggagaacttctgagagcatagtgcgtttaaggcgctcttcctcccgtgtcttcttgaggtgatcgtaggttctggcactacaaaaattggtaatgcctgctgtcctgtattcttggagcctcttgatttcccttcggagttcaaattccaatgcatggctttcaatgaatttgtcatgttccactggccccacaattcttgcaaatcgcctcattgtttcatacaggtcctggacctccttgggataccgccgttccattaattgaaactttctaaggttgattaatccatggtctcttataattttttttcgtctttgtctctcctttaacctggaatgatagatatctaccacagccatcttcagagcatgtaaaatgtccgagtcatcttcaacaaaatcaatgtctctcaagtcccattctgcataattgtcaaattcctcaatgaaatctgctcgagctggcatgtacccggccatgtcccgagaaagcaaggagtcaaaggtaggtcggggagggtcatctgtagagtgaaatggaatggctgtgtcagcagtttttgcttcctctgcttgtttcaggttcagcagggtagatgcaaacagagggttattgatgaaatgcttcatatagtgcttctcacactcctccttggtcttggtgcacatttgattggctacatcctgccaatttccaaagccacagtccatcacagcttctaaaagggccatttcttcttgagcagtccagctgggatcaaggacaggaaaatctgaagtcattatttcataagtatgatcgctttgatgtttcttgtactcaaagcctcgagtgaaacatgctaaaggaacccaaacggtccattccctaattggcaacgagtgctgctttggtcttcctcagcagagcttcttcaagacttcagaaccggccaacacatacaccaaagcttgatgactcccgggagaaggaagtgaggcacttcgccgggcaggagtccacgttgggaggaggaaaggcgcaggctcccgagttgtggagccaacgttcaaatccttacggggtgggaccggcctgggccagtcattttacctgcgcctcagctctaacagggtactgaaatacctactttggggggcctgctaggaaattcaaatgggcaacgctggtcaggggcatctggcacagtggccattcttggtagagctacgcgctccagggctgagcgggaaatggcgaggccggggcactgg

SEQ ID NO: 12627 - RNA, 2523 nt, Homo sapiens
  source 1..2523: mol_type = other RNA
gatctcactttgttgcccaggctggagcacagtggcgtgatctcagctcgctgcaacctctgcctcctgtgttcaagcaattctcctgcctcagcctcctgagtagctgggattacaggcgtgtgccaccacactcagctaatttttgtatttttagtagagactgtttcaccatgttggtcaggctggtcttgaactcctgacttcgtgatccgcccaccttagcctcccaaagtgctgggattacaggtgagccaccttgcccggccgaagttaaagatgcagtttgggataagaccatcataaggatattttcttcccctttactcataaaagttgtcagcttaggccgggcgcgatggctcacgcctgtaatcctagtactttgggaggctgaggcgggcagatcacctgaggtcaggagtttgtgaccagcctggccaacatgacaaaaccctgtctctactaaaaatacaaaattagccaggtgtggtggtggacacctgtagtcccagctattcgggaggctgaggcaggagaatcacttgaacctgggaggcagaggttgtagtgagctgagatcttgccatcacactccagcctggaggacaagagcaaactctgtctcaaaaaaaaaaaaaaaaagttgtcagcttaaaaaatccttcaacgagagctttcttatgctctaaaacctttctctttattttaaatctgtctgcagtgtttgaaggcaagacagataatcagcaaacttacctcgcaatataaggatctgagctggactcctgggattacagactgtggtttagttccatttctaccagcactgtgatgtgaggtactatggttcttttagttacaagaggtgttaggaatgaatgcccactcacatttaataatagcttatgtagcacacaactctgcagcataataccaacaacaggagtgttttaaagcaggatggagaagaaagtagacaatacaacttaaggtttcctttgtcctttcccctgttttcaccatgagaattcagctgaaaaacaactctccagaatgcccacccatattgtcctttgacccaccacattccaaacttctgacttctgatcccaagctcttggagccttagcctttagtgatgtatccttctctgatgaggaaatcatagattttccgggttttgttcacatctatcttgatgagtgctcttgcctgcgccagtcttaagcctccttgcttgttacattcgttcaatagagcagatttgtattctaaataggctccagggaccaacctcaccatctgacagagctccttttctttttcattcagcttctctgtgccagggaggccagtgaggttcaagggtggtgcactccgtctacctgaattcgaagccattggaatggaaggactcaggccggaatcaatgtcagcttgccggcggagccactgctggcaagcactactgtcctggatatactggagaacttctgagagcatagtgcgtttaaggcgctcttcctcccgtgtcttcttgaggtgatcgtaggttctggcactacaaaaattggtaatgcctgctgtcctgtattcttggagcctcttgatttcccttcggagttcaaattccaatgcatggctttcaatgaatttgtcatgttccactggccccacaattcttgcaaatcgcctcattgtttcatacaggtcctggacctccttgggataccgccgttccattaattgaaactttctaaggttgattaatccatggtctcttataattttttttcgtctttgtctctcctttaacctggaatgatagatatctaccacagccatcttcagagcatgtaaaatgtccgagtcatcttcaacaaaatcaatgtctctcaagtcccattctgcataattgtcaaattcctcaatgaaatctgctcgagctggcatgtacccggccatgtcccgagaaagcaaggagtcaaaggtaggtcggggagggtcatctgtagagtgaaatggaatggctgtgtcagcagtttttgcttcctctgcttgtttcaggttcagcagggtagatgcaaacagagggttattgatgaaatgcttcatatagtgcttctcacactcctccttggtcttggtgcacatttgattggctacatcctgccaatttccaaagccacagtccatcacagcttctaaaagggccatttcttcttgagcagtccagctgggatcaaggacaggaaaatctgaagtcattatttcataagtatgatcgctttgatgtttcttgtactcaaagcctcgagtgaaacatgctaaaggaacccaaacggtccattccctaattggcaacgagtgctgctttggtcttcctcagcagagcttcttcaagacttcagaaccggccaacacatacaccaaagcttgatgactccctcgccgagaccccctaatccgcgccaaagagccgccggtcgcgcgcgcctccgggctttgcgtgcgcgcccc

SEQ ID NO: 12628 - RNA, 2557 nt, Homo sapiens
  source 1..2557: mol_type = other RNA
gatctcactttgttgcccaggctggagcacagtggcgtgatctcagctcgctgcaacctctgcctcctgtgttcaagcaattctcctgcctcagcctcctgagtagctgggattacaggcgtgtgccaccacactcagctaatttttgtatttttagtagagactgtttcaccatgttggtcaggctggtcttgaactcctgacttcgtgatccgcccaccttagcctcccaaagtgctgggattacaggtgagccaccttgcccggccgaagttaaagatgcagtttgggataagaccatcataaggatattttcttcccctttactcataaaagttgtcagcttaggccgggcgcgatggctcacgcctgtaatcctagtactttgggaggctgaggcgggcagatcacctgaggtcaggagtttgtgaccagcctggccaacatgacaaaaccctgtctctactaaaaatacaaaattagccaggtgtggtggtggacacctgtagtcccagctattcgggaggctgaggcaggagaatcacttgaacctgggaggcagaggttgtagtgagctgagatcttgccatcacactccagcctggaggacaagagcaaactctgtctcaaaaaaaaaaaaaaaaagttgtcagcttaaaaaatccttcaacgagagctttcttatgctctaaaacctttctctttattttaaatctgtctgcagtgtttgaaggcaagacagataatcagcaaacttacctcgcaatataaggatctgagctggactcctgggattacagactgtggtttagttccatttctaccagcactgtgatgtgaggtactatggttcttttagttacaagaggtgttaggaatgaatgcccactcacatttaataatagcttatgtagcacacaactctgcagcataataccaacaacaggagtgttttaaagcaggatggagaagaaagtagacaatacaacttaaggtttcctttgtcctttcccctgttttcaccatgagaattcagctgaaaaacaactctccagaatgcccacccatattgtcctttgacccaccacattccaaacttctgacttctgatcccaagctcttggagccttagcctttagtgatgtatccttctctgatgaggaaatcatagattttccgggttttgttcacatctatcttgatgagtgctcttgcctgcgccagtcttaagcctccttgcttgttacattcgttcaatagagcagatttgtattctaaataggctccagggaccaacctcaccatctgacagagctccttttctttttcattcagcttctctgtgccagggaggccagtgaggttcaagggtggtgcactccgtctacctgaattcgaagccattggaatggaaggactcaggccggaatcaatgtcagcttgccggcggagccactgctggcaagcactactgtcctggatatactggagaacttctgagagcatagtgcgtttaaggcgctcttcctcccgtgtcttcttgaggtgatcgtaggttctggcactacaaaaattggtaatgcctgctgtcctgtattcttggagcctcttgatttcccttcggagttcaaattccaatgcatggctttcaatgaatttgtcatgttccactggccccacaattcttgcaaatcgcctcattgtttcatacaggtcctggacctccttgggataccgccgttccattaattgaaactttctaaggttgattaatccatggtctcttataattttttttcgtctttgtctctcctttaacctggaatgatagatatctaccacagccatcttcagagcatgtaaaatgtccgagtcatcttcaacaaaatcaatgtctctcaagtcccattctgcataattgtcaaattcctcaatgaaatctgctcgagctggcatgtacccggccatgtcccgagaaagcaaggagtcaaaggtaggtcggggagggtcatctgtagagtgaaatggaatggctgtgtcagcagtttttgcttcctctgcttgtttcaggttcagcagggtagatgcaaacagagggttattgatgaaatgcttcatatagtgcttctcacactcctccttggtcttggtgcacatttgattggctacatcctgccaatttccaaagccacagtccatcacagcttctaaaagggccatttcttcttgagcagtccagctgggatcaaggacaggaaaatctgaagtctgcaagcagaggaaaaaaggaggtggcccacattcagcacacttgatataaggctccatgaggtaggaggagcagcctcggcaaggtggcttatcagagggatcattgctaaaggaacccaaacggtccattccctaattggcaacgagtgctgctttggtcttcctcagcagagcttcttcaagacttcagaaccggccaacacatacaccaaagcttgatgactccctcgccgagaccccctaatccgcgccaaagagccgccggtcgcgcgcgcctccgggcttt

SEQ ID NO: 12629 - RNA, 2538 nt, Homo sapiens
  source 1..2538: mol_type = other RNA
gatctcactttgttgcccaggctggagcacagtggcgtgatctcagctcgctgcaacctctgcctcctgtgttcaagcaattctcctgcctcagcctcctgagtagctgggattacaggcgtgtgccaccacactcagctaatttttgtatttttagtagagactgtttcaccatgttggtcaggctggtcttgaactcctgacttcgtgatccgcccaccttagcctcccaaagtgctgggattacaggtgagccaccttgcccggccgaagttaaagatgcagtttgggataagaccatcataaggatattttcttcccctttactcataaaagttgtcagcttaggccgggcgcgatggctcacgcctgtaatcctagtactttgggaggctgaggcgggcagatcacctgaggtcaggagtttgtgaccagcctggccaacatgacaaaaccctgtctctactaaaaatacaaaattagccaggtgtggtggtggacacctgtagtcccagctattcgggaggctgaggcaggagaatcacttgaacctgggaggcagaggttgtagtgagctgagatcttgccatcacactccagcctggaggacaagagcaaactctgtctcaaaaaaaaaaaaaaaaagttgtcagcttaaaaaatccttcaacgagagctttcttatgctctaaaacctttctctttattttaaatctgtctgcagtgtttgaaggcaagacagataatcagcaaacttacctcgcaatataaggatctgagctggactcctgggattacagactgtggtttagttccatttctaccagcactgtgatgtgaggtactatggttcttttagttacaagaggtgttaggaatgaatgcccactcacatttaataatagcttatgtagcacacaactctgcagcataataccaacaacaggagtgttttaaagcaggatggagaagaaagtagacaatacaacttaaggtttcctttgtcctttcccctgttttcaccatgagaattcagctgaaaaacaactctccagaatgcccacccatattgtcctttgacccaccacattccaaacttctgacttctgatcccaagctcttggagccttagcctttagtgatgtatccttctctgatgaggaaatcatagattttccgggttttgttcacatctatcttgatgagtgctcttgcctgcgccagtcttaagcctccttgcttgttacattcgttcaatagagcagatttgtattctaaataggctccagggaccaacctcaccatctgacagagctccttttctttttcattcagcttctctgtgccagggaggccagtgaggttcaagggtggtgcactccgtctacctgaattcgaagccattggaatggaaggactcaggccggaatcaatgtcagcttgccggcggagccactgctggcaagcactactgtcctggatatactggagaacttctgagagcatagtgcgtttaaggcgctcttcctcccgtgtcttcttgaggtgatcgtaggttctggcactacaaaaattggtaatgcctgctgtcctgtattcttggagcctcttgatttcccttcggagttcaaattccaatgcatggctttcaatgaatttgtcatgttccactggccccacaattcttgcaaatcgcctcattgtttcatacaggtcctggacctccttgggataccgccgttccattaattgaaactttctaaggttgattaatccatggtctcttataattttttttcgtctttgtctctcctttaacctggaatgatagatatctaccacagccatcttcagagcatgtaaaatgtccgagtcatcttcaacaaaatcaatgtctctcaagtcccattctgcataattgtcaaattcctcaatgaaatctgctcgagctggcatgtacccggccatgtcccgagaaagcaaggagtcaaaggtaggtcggggagggtcatctgtagagtgaaatggaatggctgtgtcagcagtttttgcttcctctgcttgtttcaggttcagcagggtagatgcaaacagagggttattgatgaaatgcttcatatagtgcttctcacactcctccttggtcttggtgcacatttgattggctacatcctgccattatttcataagtatgatcgctttgatgtttcttgtactcaaagcctcgagtgaaacactgcaagcagaggaaaaaaggaggtggcccacattcagcacacttgatataaggctccatgaggtaggaggagcagcctcggcaaggtggcttatcagagggatcattgctaaaggaacccaaacggtccattccctaattggcaacgagtgctgctttggtcttcctcagcagagcttcttcaagacttcagaaccggccaacacatacaccaaagcttgatgactccctcgccgagaccccctaatccgcgccaaagagccgccggtcgcgcgcgcctccgggctttgcgtgcgcgcccc

SEQ ID NO: 12630 - RNA, 2431 nt, Homo sapiens
  source 1..2431: mol_type = other RNA
gatctcactttgttgcccaggctggagcacagtggcgtgatctcagctcgctgcaacctctgcctcctgtgttcaagcaattctcctgcctcagcctcctgagtagctgggattacaggcgtgtgccaccacactcagctaatttttgtatttttagtagagactgtttcaccatgttggtcaggctggtcttgaactcctgacttcgtgatccgcccaccttagcctcccaaagtgctgggattacaggtgagccaccttgcccggccgaagttaaagatgcagtttgggataagaccatcataaggatattttcttcccctttactcataaaagttgtcagcttaggccgggcgcgatggctcacgcctgtaatcctagtactttgggaggctgaggcgggcagatcacctgaggtcaggagtttgtgaccagcctggccaacatgacaaaaccctgtctctactaaaaatacaaaattagccaggtgtggtggtggacacctgtagtcccagctattcgggaggctgaggcaggagaatcacttgaacctgggaggcagaggttgtagtgagctgagatcttgccatcacactccagcctggaggacaagagcaaactctgtctcaaaaaaaaaaaaaaaaagttgtcagcttaaaaaatccttcaacgagagctttcttatgctctaaaacctttctctttattttaaatctgtctgcagtgtttgaaggcaagacagataatcagcaaacttacctcgcaatataaggatctgagctggactcctgggattacagactgtggtttagttccatttctaccagcactgtgatgtgaggtactatggttcttttagttacaagaggtgttaggaatgaatgcccactcacatttaataatagcttatgtagcacacaactctgcagcataataccaacaacaggagtgttttaaagcaggatggagaagaaagtagacaatacaacttaaggtttcctttgtcctttcccctgttttcaccatgagaattcagctgaaaaacaactctccagaatgcccacccatattgtcctttgacccaccacattccaaacttctgacttctgatcccaagctcttggagccttagcctttagtgatgtatccttctctgatgaggaaatcatagattttccgggttttgttcacatctatcttgatgagtgctcttgcctgcgccagtcttaagcctccttgcttgttacattcgttcaatagagcagatttgtattctaaataggctccagggaccaacctcaccatctgacagagctccttttctttttcattcagcttctctgtgccagggaggccagtgaggttcaagggtggtgcactccgtctacctgaattcgaagccattggaatggaaggactcaggccggaatcaatgtcagcttgccggcggagccactgctggcaagcactactgtcctggatatactggagaacttctgagagcatagtgcgtttaaggcgctcttcctcccgtgtcttcttgaggtgatcgtaggttctggcactacaaaaattggtaatgcctgctgtcctgtattcttggagcctcttgatttcccttcggagttcaaattccaatgcatggctttcaatgaatttgtcatgttccactggccccacaattcttgcaaatcgcctcattgtttcatacaggtcctggacctccttgggataccgccgttccattaattgaaactttctaaggttgattaatccatggtctcttataattttttttcgtctttgtctctcctttaacctggaatgatagatatctaccacagccatcttcagagcatgtaaaatgtccgagtcatcttcaacaaaatcaatgtctctcaagtcccattctgcataattgtcaaattcctcaatgaaatctgctcgagctggcatgtacccggccatgtcccgagaaagcaaggagtcaaaggtaggtcggggagggtcatctgtagagtgaaatggaatggctgtgtcagcagtttttgcttcctctgcttgtttcaggttcagcagggtagatgcaaacagagggttattgatgaaatgcttcatatagtgcttctcacactcctccttggtcttggtgcacatttgattggctacatcctgccattatttcataagtatgatcgctttgatgtttcttgtactcaaagcctcgagtgaaacatgctaaaggaacccaaacggtccattccctaattggcaacgagtgctgctttggtcttcctcagcagagcttcttcaagacttcagaaccggccaacacatacaccaaagcttgatgactccctcgccgagaccccctaatccgcgccaaagagccgccggtcgcgcgcgcctccgggctttgcgtgcgcgcccc

SEQ ID NO: 12631 - RNA, 2750 nt, Homo sapiens
  source 1..2750: mol_type = other RNA
gatctcactttgttgcccaggctggagcacagtggcgtgatctcagctcgctgcaacctctgcctcctgtgttcaagcaattctcctgcctcagcctcctgagtagctgggattacaggcgtgtgccaccacactcagctaatttttgtatttttagtagagactgtttcaccatgttggtcaggctggtcttgaactcctgacttcgtgatccgcccaccttagcctcccaaagtgctgggattacaggtgagccaccttgcccggccgaagttaaagatgcagtttgggataagaccatcataaggatattttcttcccctttactcataaaagttgtcagcttaggccgggcgcgatggctcacgcctgtaatcctagtactttgggaggctgaggcgggcagatcacctgaggtcaggagtttgtgaccagcctggccaacatgacaaaaccctgtctctactaaaaatacaaaattagccaggtgtggtggtggacacctgtagtcccagctattcgggaggctgaggcaggagaatcacttgaacctgggaggcagaggttgtagtgagctgagatcttgccatcacactccagcctggaggacaagagcaaactctgtctcaaaaaaaaaaaaaaaaagttgtcagcttaaaaaatccttcaacgagagctttcttatgctctaaaacctttctctttattttaaatctgtctgcagtgtttgaaggcaagacagataatcagcaaacttacctcgcaatataaggatctgagctggactcctgggattacagactgtggtttagttccatttctaccagcactgtgatgtgaggtactatggttcttttagttacaagaggtgttaggaatgaatgcccactcacatttaataatagcttatgtagcacacaactctgcagcataataccaacaacaggagtgttttaaagcaggatggagaagaaagtagacaatacaacttaaggtttcctttgtcctttcccctgttttcaccatgagaattcagctgaaaaacaactctccagaatgcccacccatattgtcctttgacccaccacattccaaacttctgacttctgatcccaagctcttggagccttagcctttagtgatgtatccttctctgatgaggaaatcatagattttccgggttttgttcacatctatcttgatgagtgctcttgcctgcgccagtcttaagcctccttgcttgttacattcgttcaatagagcagatttgtattctaaataggctccagggaccaacctcaccatctgacagagctccttttctttttcattcagcttctctgtgccagggaggccagtgaggttcaagggtggtgcactccgtctacctgaattcgaagccattggaatggaaggactcaggccggaatcaatgtcagcttgccggcggagccactgctggcaagcactactgtcctggatatactggagaacttctgagagcatagtgcgtttaaggcgctcttcctcccgtgtcttcttgaggtgatcgtaggttctggcactacaaaaattggtaatgcctgctgtcctgtattcttggagcctcttgatttcccttcggagttcaaattccaatgcatggctttcaatgaatttgtcatgttccactggccccacaattcttgcaaatcgcctcattgtttcatacaggtcctggacctccttgggataccgccgttccattaattgaaactttctaaggttgattaatccatggtctcttataattttttttcgtctttgtctctcctttaacctggaatgatagatatctaccacagccatcttcagagcatgtaaaatgtccgagtcatcttcaacaaaatcaatgtctctcaagtcccattctgcataattgtcaaattcctcaatgaaatctgctcgagctggcatgtacccggccatgtcccgagaaagcaaggagtcaaaggtaggtcggggagggtcatctgtagagtgaaatggaatggctgtgtcagcagtttttgcttcctctgcttgtttcaggttcagcagggtagatgcaaacagagggttattgatgaaatgcttcatatagtgcttctcacactcctccttggtcttggtgcacatttgattggctacatcctgcctctaaatcatgggttgataggaaagcaacacatactttctcttcctgaggttccttcctttactcttcaacaacagcttcttctctgagtccactagggcaggacaactcttaacaccaagctcttaccaatttccaaagccacagtccatcacagcttctaaaagggccatttcttcttgagcagtccagctgggatcaaggacaggaaaatctgaagtcattatttcataagtatgatcgctttgatgtttcttgtactcaaagcctcgagtgaaacactgcaagcagaggaaaaaaggaggtggcccacattcagcacacttgatataaggctccatgaggtaggaggagcagcctcggcaaggtggcttatcagagggatcattgctaaaggaacccaaacggtccattccctaattggcaacgagtgctgctttggtcttcctcagcagagcttcttcaagacttcagaaccggccaacacatacaccaaagcttgatgactccctcgccgagaccccctaatccgcgccaaagagccgccggtcgcgcgcgcctccgggctttgcgt

SEQ ID NO: 12632 - RNA, 2699 nt, Homo sapiens
  source 1..2699: mol_type = other RNA
gatctcactttgttgcccaggctggagcacagtggcgtgatctcagctcgctgcaacctctgcctcctgtgttcaagcaattctcctgcctcagcctcctgagtagctgggattacaggcgtgtgccaccacactcagctaatttttgtatttttagtagagactgtttcaccatgttggtcaggctggtcttgaactcctgacttcgtgatccgcccaccttagcctcccaaagtgctgggattacaggtgagccaccttgcccggccgaagttaaagatgcagtttgggataagaccatcataaggatattttcttcccctttactcataaaagttgtcagcttaggccgggcgcgatggctcacgcctgtaatcctagtactttgggaggctgaggcgggcagatcacctgaggtcaggagtttgtgaccagcctggccaacatgacaaaaccctgtctctactaaaaatacaaaattagccaggtgtggtggtggacacctgtagtcccagctattcgggaggctgaggcaggagaatcacttgaacctgggaggcagaggttgtagtgagctgagatcttgccatcacactccagcctggaggacaagagcaaactctgtctcaaaaaaaaaaaaaaaaagttgtcagcttaaaaaatccttcaacgagagctttcttatgctctaaaacctttctctttattttaaatctgtctgcagtgtttgaaggcaagacagataatcagcaaacttacctcgcaatataaggatctgagctggactcctgggattacagactgtggtttagttccatttctaccagcactgtgatgtgaggtactatggttcttttagttacaagaggtgttaggaatgaatgcccactcacatttaataatagcttatgtagcacacaactctgcagcataataccaacaacaggagtgttttaaagcaggatggagaagaaagtagacaatacaacttaaggtttcctttgtcctttcccctgttttcaccatgagaattcagctgaaaaacaactctccagaatgcccacccatattgtcctttgacccaccacattccaaacttctgacttctgatcccaagctcttggagccttagcctttagtgatgtatccttctctgatgaggaaatcatagattttccgggttttgttcacatctatcttgatgagtgctcttgcctgcgccagtcttaagcctccttgcttgttacattcgttcaatagagcagatttgtattctaaataggctccagggaccaacctcaccatctgacagagctccttttctttttcattcagcttctctgtgccagggaggccagtgaggttcaagggtggtgcactccgtctacctgaattcgaagccattggaatggaaggactcaggccggaatcaatgtcagcttgccggcggagccactgctggcaagcactactgtcctggatatactggagaacttctgagagcatagtgcgtttaaggcgctcttcctcccgtgtcttcttgaggtgatcgtaggttctggcactacaaaaattggtaatgcctgctgtcctgtattcttggagcctcttgatttcccttcggagttcaaattccaatgcatggctttcaatgaatttgtcatgttccactggccccacaattcttgcaaatcgcctcattgtttcatacaggtcctggacctccttgggataccgccgttccattaattgaaactttctaaggttgattaatccatggtctcttataattttttttcgtctttgtctctcctttaacctggaatgatagatatctaccacagccatcttcagagcatgtaaaatgtccgagtcatcttcaacaaaatcaatgtctctcaagtcccattctgcataattgtcaaattcctcaatgaaatctgctcgagctggcatgtacccggccatgtcccgagaaagcaaggagtcaaaggtaggtcggggagggtcatctgtagagtgaaatggaatggctgtgtcagcagtttttgcttcctctgcttgtttcaggttcagcagggtagatgcaaacagagggttattgatgaaatgcttcatatagtgcttctcacactcctccttggtcttggtgcacatttgattggctacatcctgcctctaaatcatgggttgataggaaagcaacacatactttctcttcctgaggttccttcctttactcttcaacaacagcttcttctctgagtccactagggcaggacaactcttaacaccaagctcttaccaatttccaaagccacagtccatcacagcttctaaaagggccatttcttcttgagcagtccagctgggatcaaggacaggaaaatctgaagtctgcaagcagaggaaaaaaggaggtggcccacattcagcacacttgatataaggctccatgaggtaggaggagcagcctcggcaaggtggcttatcagagggatcattgctaaaggaacccaaacggtccattccctaattggcaacgagtgctgctttggtcttcctcagcagagcttcttcaagacttcagaaccggccaacacatacaccaaagcttgatgactccctcgccgagaccccctaatccgcgccaaagagccgccggtcgcgcgcgcctccgggctttgcgtgcgcgcccc

SEQ ID NO: 12633 - RNA, 2714 nt, Homo sapiens
  source 1..2714: mol_type = other RNA
gatctcactttgttgcccaggctggagcacagtggcgtgatctcagctcgctgcaacctctgcctcctgtgttcaagcaattctcctgcctcagcctcctgagtagctgggattacaggcgtgtgccaccacactcagctaatttttgtatttttagtagagactgtttcaccatgttggtcaggctggtcttgaactcctgacttcgtgatccgcccaccttagcctcccaaagtgctgggattacaggtgagccaccttgcccggccgaagttaaagatgcagtttgggataagaccatcataaggatattttcttcccctttactcataaaagttgtcagcttaggccgggcgcgatggctcacgcctgtaatcctagtactttgggaggctgaggcgggcagatcacctgaggtcaggagtttgtgaccagcctggccaacatgacaaaaccctgtctctactaaaaatacaaaattagccaggtgtggtggtggacacctgtagtcccagctattcgggaggctgaggcaggagaatcacttgaacctgggaggcagaggttgtagtgagctgagatcttgccatcacactccagcctggaggacaagagcaaactctgtctcaaaaaaaaaaaaaaaaagttgtcagcttaaaaaatccttcaacgagagctttcttatgctctaaaacctttctctttattttaaatctgtctgcagtgtttgaaggcaagacagataatcagcaaacttacctcgcaatataaggatctgagctggactcctgggattacagactgtggtttagttccatttctaccagcactgtgatgtgaggtactatggttcttttagttacaagaggtgttaggaatgaatgcccactcacatttaataatagcttatgtagcacacaactctgcagcataataccaacaacaggagtgttttaaagcaggatggagaagaaagtagacaatacaacttaaggtttcctttgtcctttcccctgttttcaccatgagaattcagctgaaaaacaactctccagaatgcccacccatattgtcctttgacccaccacattccaaacttctgacttctgatcccaagctcttggagccttagcctttagtgatgtatccttctctgatgaggaaatcatagattttccgggttttgttcacatctatcttgatgagtgctcttgcctgcgccagtcttaagcctccttgcttgttacattcgttcaatagagcagatttgtattctaaataggctccagggaccaacctcaccatctgacagagctccttttctttttcattcagcttctctgtgccagggaggccagtgaggttcaagggtggtgcactccgtctacctgaattcgaagccattggaatggaaggactcaggccggaatcaatgtcagcttgccggcggagccactgctggcaagcactactgtcctggatatactggagaacttctgagagcatagtgcgtttaaggcgctcttcctcccgtgtcttcttgaggtgatcgtaggttctggcactacaaaaattggtaatgcctgctgtcctgtattcttggagcctcttgatttcccttcggagttcaaattccaatgcatggctttcaatgaatttgtcatgttccactggccccacaattcttgcaaatcgcctcattgtttcatacaggtcctggacctccttgggataccgccgttccattaattgaaactttctaaggttgattaatccatggtctcttataattttttttcgtctttgtctctcctttaacctggaatgatagatatctaccacagccatcttcagagcatgtaaaatgtccgagtcatcttcaacaaaatcaatgtctctcaagtcccattctgcataattgtcaaattcctcaatgaaatctgctcgagctggcatgtacccggccatgtcccgagaaagcaaggagtcaaaggtaggtcggggagggtcatctgtagagtgaaatggaatggctgtgtcagcagtttttgcttcctctgcttgtttcaggttcagcagggtagatgcaaacagagggttattgatgaaatgcttcatatagtgcttctcacactcctccttggtcttggtgcacatttgattggctacatcctgctttctcttcctgaggttccttcctttactcttcaacaacagcttcttctctgagtccactagggcaggacaactcttaacaccaagctcttaccaatttccaaagccacagtccatcacagcttctaaaagggccatttcttcttgagcagtccagctgggatcaaggacaggaaaatctgaagtcattatttcataagtatgatcgctttgatgtttcttgtactcaaagcctcgagtgaaacactgcaagcagaggaaaaaaggaggtggcccacattcagcacacttgatataaggctccatgaggtaggaggagcagcctcggcaaggtggcttatcagagggatcattgctaaaggaacccaaacggtccattccctaattggcaacgagtgctgctttggtcttcctcagcagagcttcttcaagacttcagaaccggccaacacatacaccaaagcttgatgactccctcgccgagaccccctaatccgcgccaaagagccgccggtcgcgcgcgcctccgggctttgcgt

SEQ ID NO: 12634 - RNA, 2945 nt, Homo sapiens
  source 1..2945: mol_type = other RNA
gatctcactttgttgcccaggctggagtgcaatggcgtgatcttggctcactggaacctctgcctcccaggttgaagtggttctcctgcctcagcctcccgagtagctaggatcacaggtgcccatcaccgcctggctaattctgtttttttttgtagagacggggtttcaccatgttggcaaggctggtcttgaactcctgaccttaggtgatccgcccacctcagcctcctagagtgctgggattacaggcgtaagccaccgcgcctggccttctgcatttttaagtttctatggttccaccattctcaccttggcctgttctttcattatggctttctgtttctacttcaaaaatggcacattttctggtatttttttgaagaggcccaatagtttcttgaaaatttcttctaactcctgaaactgagattatacactgatcatatatgattttatgactctttaaaacaatgtttctcagtatcctgtcctaagtcccaagttttaccacctttacttcacccagacctgtggccactttactcatctttggctataccaagagatatctctggtaacaggacgattatttttgtttacctttcaatgtttaaaaaatgtcttgccttgtatatacatgctccagtaataattattttgaaaacaaaagtttttaaacctgtgaacagcataataaaaaactttttctatcccacaaagagcacaataaaaaaaaaatcaacatctgttaatctaggatacagtatatagaaaagttatggtatcaagatgatagtttaaagatatacatttttgctttcaaaagcaaggattctaatatattaggaaaatagaaagacagtattatttaaccctgttctcacataagcaccaattttattccaaataatcacataattttaagaaataattttcctaatatatttttacaaaaagtcacttcagtgtcatacattctagaaacgccatcttgtatattagtattaccttacctgaactgaaacattccaaaagttccaataccttctacagatttcatttttacagttcaaaaaaattatttatttttcatgataaatgatgctactgataactttacttggtagaattgtagttactttggtaatttctacatgtttataaataagcaccacatatactatattaaaaaattagccagtctaagggcttgcactggagaccagggagttacattttgttaaacccagattgaacagagttgaatttagattaatacagagaaatgcatgctctgggtttgttgtcctttgtatttcttgaagcatcagatgaatcgtaaaaagttcaaagagcttcttattactccttgagtgactgttttgagaacaattaaggttgataaaaatctcaatggcaaattggagctcttaaagaaagcagctgtctttggtttattctccacagaatgctgtggagaattatcctgaattcctttagttaccactcctttaaaaatgtcttcacccaatctcctcaatgttgatgtcatagtcgagtgctgtgctccagcatctagctgccttagggaccaatatataaattttacaaaaggctcgtgaagtttgatattcacaaatggcatccactgtagctgctctgtcattagaggcaaaagctttacacacttctcctgaatatcatttctctgggaagcaaatttgagttgtggttttttaccatccattccagattcttcatgtttcactttgctaagatgatgatccgaaatccagtccatgaagacagttaaaagttcataaacttgcccattaagtggtaccttgtaagtttttgaaactggtgctttttcttgttttaaacttttcatttcatgaacagcatgggaacttcctttcaatctctgtattgtcataaactcgtacttcctctgtaaattatctaaacgagcttgaactcttttagcctgaatgtctatcttcctgttttcttcacttgcttcatttaactgtttttttaaggtatcattcaattctttcaatgcatcaaaagaggacctcagtctcttggtttctttattcttttccttaagaacttcggttaagtgttcaacttctgcatcatgctgctcttttataatttgaaatcttgtaagaacctcttcttcaacacctttaattttactcaaggcattttcatgtctgaaaagcagttgttctctttcaagtaaaaaacgttctcgcttttgaagttcttcagcaaatttctgttgtgctgcagtttcacactgcaatttcagatgtatctgaaataattcgtcatatatctgactgatctgatgtggaagtaaactccgcttgtctgatgctttagattttggacagctgacaggtttcaaaggagagtcacctgcatcactacaacactcagtccgaggtctcgatgaggtcgtattagttggcaaggcaactttttctatttctttaaaagactgcttggttattttcgaggtactaactctataatcattttcaattaactcttcttctgtttcctgtttcttcaaatcatggaaagaatccagttcatcatctaggcaattcacatttacgtgcttgaataagctgcccaatggtgttctacaatgcttgctttcatcagaatattttaacgatgaaccaactttatctccagagtagatatccaaatcacctggggaggttagagttcttctcttatacttagactgataaaaatttgaaaaatcatactcaggcggcggcttcacctcgtcggggcagctgcccccgagtccgtagcggcttttgagactctccactactaaatcctgccccggtggcttgacgaccctcggctccatagcacacagcaaccgtaccagtctccccgggaaccgcgtt

SEQ ID NO: 12635 - RNA, 3084 nt, Homo sapiens
  source 1..3084: mol_type = other RNA
gatctcactttgttgcccaggctggagtgcaatggcgtgatcttggctcactggaacctctgcctcccaggttgaagtggttctcctgcctcagcctcccgagtagctaggatcacaggtgcccatcaccgcctggctaattctgtttttttttgtagagacggggtttcaccatgttggcaaggctggtcttgaactcctgaccttaggtgatccgcccacctcagcctcctagagtgctgggattacaggcgtaagccaccgcgcctggccttctgcatttttaagtttctatggttccaccattctcaccttggcctgttctttcattatggctttctgtttctacttcaaaaatggcacattttctggtatttttttgaagaggcccaatagtttcttgaaaatttcttctaactcctgaaactgagattatacactgatcatatatgattttatgactctttaaaacaatgtttctcagtatcctgtcctaagtcccaagttttaccacctttacttcacccagacctgtggccactttactcatctttggctataccaagagatatctctggtaacaggacgattatttttgtttacctttcaatgtttaaaaaatgtcttgccttgtatatacatgctccagtaataattattttgaaaacaaaagtttttaaacctgtgaacagcataataaaaaactttttctatcccacaaagagcacaataaaaaaaaaatcaacatctgttaatctaggatacagtatatagaaaagttatggtatcaagatgatagtttaaagatatacatttttgctttcaaaagcaaggattctaatatattaggaaaatagaaagacagtattatttaaccctgttctcacataagcaccaattttattccaaataatcacataattttaagaaataattttcctaatatatttttacaaaaagtcacttcagtgtcatacattctagaaacgccatcttgtatattagtattaccttacctgaactgaaacattccaaaagttccaataccttctacagatttcatttttacagttcaaaaaaattatttatttttcatgataaatgatgctactgataactttacttggtagaattgtagttactttggtaatttctacatgtttataaataagcaccacatatactatattaaaaaattagccagtctaagggcttgcactggagaccagggagttacattttgttaaacccagattgaacagagttgaatttagattaatacagagaaatgcatgctctgggtttgttgtcctttgtatttcttgaagcatcagatgaatcgtaaaaagttcaaagagcttcttattactcttgattttggaaagtttctgtaaaataatactgagtttttctagtatttgaagatcaagcttaggggctcgaagcagcacagagcaagtacgaaaaaataaagagttgctacaggcttccaggaaaggctgcaaggattcttgagtgactgttttgagaacaattaaggttgataaaaatctcaatggcaaattggagctcttaaagaaagcagctgtctttggtttattctccacagaatgctgtggagaattatcctgaattcctttagttaccactcctttaaaaatgtcttcacccaatctcctcaatgttgatgtcatagtcgagtgctgtgctccagcatctagctgccttagggaccaatatataaattttacaaaaggctcgtgaagtttgatattcacaaatggcatccactgtagctgctctgtcattagaggcaaaagctttacacacttctcctgaatatcatttctctgggaagcaaatttgagttgtggttttttaccatccattccagattcttcatgtttcactttgctaagatgatgatccgaaatccagtccatgaagacagttaaaagttcataaacttgcccattaagtggtaccttgtaagtttttgaaactggtgctttttcttgttttaaacttttcatttcatgaacagcatgggaacttcctttcaatctctgtattgtcataaactcgtacttcctctgtaaattatctaaacgagcttgaactcttttagcctgaatgtctatcttcctgttttcttcacttgcttcatttaactgtttttttaaggtatcattcaattctttcaatgcatcaaaagaggacctcagtctcttggtttctttattcttttccttaagaacttcggttaagtgttcaacttctgcatcatgctgctcttttataatttgaaatcttgtaagaacctcttcttcaacacctttaattttactcaaggcattttcatgtctgaaaagcagttgttctctttcaagtaaaaaacgttctcgcttttgaagttcttcagcaaatttctgttgtgctgcagtttcacactgcaatttcagatgtatctgaaataattcgtcatatatctgactgatctgatgtggaagtaaactccgcttgtctgatgctttagattttggacagctgacaggtttcaaaggagagtcacctgcatcactacaacactcagtccgaggtctcgatgaggtcgtattagttggcaaggcaactttttctatttctttaaaagactgcttggttattttcgaggtactaactctataatcattttcaattaactcttcttctgtttcctgtttcttcaaatcatggaaagaatccagttcatcatctaggcaattcacatttacgtgcttgaataagctgcccaatggtgttctacaatgcttgctttcatcagaatattttaacgatgaaccaactttatctccagagtagatatccaaatcacctggggaggttagagttcttctcttatacttagactgataaaaatttgaaaaatcatactcaggcggcggcttcacctcgtcggggcagctgcccccgagtccgtagcggcttttgagactctccactactaaatcctgccccggtggcttgacgaccctcggctccatagcacacagcaaccgtaccagtctccccgggaaccgcgtt

SEQ ID NO: 12636 - RNA, 2774 nt, Homo sapiens
  source 1..2774: mol_type = other RNA
gatctcactttgttgcccaggctggagtgcaatggcgtgatcttggctcactggaacctctgcctcccaggttgaagtggttctcctgcctcagcctcccgagtagctaggatcacaggtgcccatcaccgcctggctaattctgtttttttttgtagagacggggtttcaccatgttggcaaggctggtcttgaactcctgaccttaggtgatccgcccacctcagcctcctagagtgctgggattacaggcgtaagccaccgcgcctggccttctgcatttttaagtttctatggttccaccattctcaccttggcctgttctttcattatggctttctgtttctacttcaaaaatggcacattttctggtatttttttgaagaggcccaatagtttcttgaaaatttcttctaactcctgaaactgagattatacactgatcatatatgattttatgactctttaaaacaatgtttctcagtatcctgtcctaagtcccaagttttaccacctttacttcacccagacctgtggccactttactcatctttggctataccaagagatatctctggtaacaggacgattatttttgtttacctttcaatgtttaaaaaatgtcttgccttgtatatacatgctccagtaataattattttgaaaacaaaagtttttaaacctgtgaacagcataataaaaaactttttctatcccacaaagagcacaataaaaaaaaaatcaacatctgttaatctaggatacagtatatagaaaagttatggtatcaagatgatagtttaaagatatacatttttgctttcaaaagcaaggattctaatatattaggaaaatagaaagacagtattatttaaccctgttctcacataagcaccaattttattccaaataatcacataattttaagaaataattttcctaatatatttttacaaaaagtcacttcagtgtcatacattctagaaacgccatcttgtatattagtattaccttacctgaactgaaacattccaaaagttccaataccttctacagatttcatttttacagttcaaaaaaattatttatttttcatgataaatgatgctactgataactttacttggtagaattgtagttactttggtaatttctacatgtttataaataagcaccacatatactatattaaaaaattagccagtctaagggcttgcactggagaccagggagttacattttgttaaacccagattgaacagagttgaatttagattaatacagagaaatgcatgctctgggtttgttgtcctttgtatttcttgaagcatcagatgaatcgtaaaaagttcaaagagcttcttattactcttgattttggaaagtttctgtaaaataatactgagtttttctagtatttgaagatcaagcttaggggctcgaagcagcacagagcaagtacgaaaaaataaagagttgctacaggcttccaggaaaggctgcaaggattctttacacacttctcctgaatatcatttctctgggaagcaaatttgagttgtggttttttaccatccattccagattcttcatgtttcactttgctaagatgatgatccgaaatccagtccatgaagacagttaaaagttcataaacttgcccattaagtggtaccttgtaagtttttgaaactggtgctttttcttgttttaaacttttcatttcatgaacagcatgggaacttcctttcaatctctgtattgtcataaactcgtacttcctctgtaaattatctaaacgagcttgaactcttttagcctgaatgtctatcttcctgttttcttcacttgcttcatttaactgtttttttaaggtatcattcaattctttcaatgcatcaaaagaggacctcagtctcttggtttctttattcttttccttaagaacttcggttaagtgttcaacttctgcatcatgctgctcttttataatttgaaatcttgtaagaacctcttcttcaacacctttaattttactcaaggcattttcatgtctgaaaagcagttgttctctttcaagtaaaaaacgttctcgcttttgaagttcttcagcaaatttctgttgtgctgcagtttcacactgcaatttcagatgtatctgaaataattcgtcatatatctgactgatctgatgtggaagtaaactccgcttgtctgatgctttagattttggacagctgacaggtttcaaaggagagtcacctgcatcactacaacactcagtccgaggtctcgatgaggtcgtattagttggcaaggcaactttttctatttctttaaaagactgcttggttattttcgaggtactaactctataatcattttcaattaactcttcttctgtttcctgtttcttcaaatcatggaaagaatccagttcatcatctaggcaattcacatttacgtgcttgaataagctgcccaatggtgttctacaatgcttgctttcatcagaatattttaacgatgaaccaactttatctccagagtagatatccaaatcacctggggaggttagagttcttctcttatacttagactgataaaaatttgaaaaatcatactcaggcggcggcttcacctcgtcggggcagctgcccccgagtccgtagcggcttttgagactctccactactaaatcctgccccggtggcttgacgaccctcggctccatagcacacagcaaccgtaccagtctccccgggaaccgcgtt

SEQ ID NO: 12637 - RNA, 3258 nt, Homo sapiens
  source 1..3258: mol_type = other RNA
gatctcactttgttgcccaggctggagtgcaatggcgtgatcttggctcactggaacctctgcctcccaggttgaagtggttctcctgcctcagcctcccgagtagctaggatcacaggtgcccatcaccgcctggctaattctgtttttttttgtagagacggggtttcaccatgttggcaaggctggtcttgaactcctgaccttaggtgatccgcccacctcagcctcctagagtgctgggattacaggcgtaagccaccgcgcctggccttctgcatttttaagtttctatggttccaccattctcaccttggcctgttctttcattatggctttctgtttctacttcaaaaatggcacattttctggtatttttttgaagaggcccaatagtttcttgaaaatttcttctaactcctgaaactgagattatacactgatcatatatgattttatgactctttaaaacaatgtttctcagtatcctgtcctaagtcccaagttttaccacctttacttcacccagacctgtggccactttactcatctttggctataccaagagatatctctggtaacaggacgattatttttgtttacctttcaatgtttaaaaaatgtcttgccttgtatatacatgctccagtaataattattttgaaaacaaaagtttttaaacctgtgaacagcataataaaaaactttttctatcccacaaagagcacaataaaaaaaaaatcaacatctgttaatctaggatacagtatatagaaaagttatggtatcaagatgatagtttaaagatatacatttttgctttcaaaagcaaggattctaatatattaggaaaatagaaagacagtattatttaaccctgttctcacataagcaccaattttattccaaataatcacataattttaagaaataattttcctaatatatttttacaaaaagtcacttcagtgtcatacattctagaaacgccatcttgtatattagtattaccttacctgaactgaaacattccaaaagttccaataccttctacagatttcatttttacagttcaaaaaaattatttatttttcatgataaatgatgctactgataactttacttggtagaattgtagttactttggtaatttctacatgtttataaataagcaccacatatactatattaaaaaattagccagtctaagggcttgcactggagaccagggagttacattttgttaaacccagattgaacagagttgaatttagattaatacagagaaatgcatgctctgggtttgttgtcctttgtatttcttgaagcatcagatgaatcgtaaaaagttcaaagagcttcttattactcttgattttggaaagtttctgtaaaataatactgagtttttctagtatttgaagatcaagcttaggggctcgaagcagcacagagcaagtacgaaaaaataaagagttgctacaggcttccaggaaaggctgcaaggatttagattccaccgtcatctggagcaaactatcaataacattagacaggagtcctttactggatattcttagatgacttaatattactggaacagcctgatactccaaaaacaaggtttttccttcttctgtcttcaagtccaaacaaagagaatcaaatgcctgagccaggtaatcagcttgagtgactgttttgagaacaattaaggttgataaaaatctcaatggcaaattggagctcttaaagaaagcagctgtctttggtttattctccacagaatgctgtggagaattatcctgaattcctttagttaccactcctttaaaaatgtcttcacccaatctcctcaatgttgatgtcatagtcgagtgctgtgctccagcatctagctgccttagggaccaatatataaattttacaaaaggctcgtgaagtttgatattcacaaatggcatccactgtagctgctctgtcattagaggcaaaagctttacacacttctcctgaatatcatttctctgggaagcaaatttgagttgtggttttttaccatccattccagattcttcatgtttcactttgctaagatgatgatccgaaatccagtccatgaagacagttaaaagttcataaacttgcccattaagtggtaccttgtaagtttttgaaactggtgctttttcttgttttaaacttttcatttcatgaacagcatgggaacttcctttcaatctctgtattgtcataaactcgtacttcctctgtaaattatctaaacgagcttgaactcttttagcctgaatgtctatcttcctgttttcttcacttgcttcatttaactgtttttttaaggtatcattcaattctttcaatgcatcaaaagaggacctcagtctcttggtttctttattcttttccttaagaacttcggttaagtgttcaacttctgcatcatgctcttttataatttgaaatcttgtaagaacctcttcttcaacacctttaattttactcaaggcattttcatgtctgaaaagcagttgttctctttcaagtaaaaaacgttctcgcttttgaagttcttcagcaaatttctgttgtgctgcagtttcacactgcaatttcagatgtatctgaaataattcgtcatatatctgactgatctgatgtggaagtaaactccgcttgtctgatgctttagattttggacagctgacaggtttcaaaggagagtcacctgcatcactacaacactcagtccgaggtctcgatgaggtcgtattagttggcaaggcaactttttctatttctttaaaagactgcttggttattttcgaggtactaactctataatcattttcaattaactcttcttctgtttcctgtttcttcaaatcatggaaagaatccagttcatcatctaggcaattcacatttacgtgcttgaataagctgcccaatggtgttctacaatgcttgctttcatcagaatattttaacgatgaaccaactttatctccagagtagatatccaaatcacctggggaggttagagttcttctcttatacttagactgataaaaatttgaaaaatcatactcaggcggcggcttcacctcgtcggggcagctgcccccgagtccgtagcggcttttgagactctccactactaaatcctgccccggtggcttgacgaccctcggctccatagcacacagcaaccgtaccagtctccccgggaaccgcgtt

SEQ ID NO: 12638 - RNA, 3271 nt, Homo sapiens
  source 1..3271: mol_type = other RNA
gatctcactttgttgcccaggctggagtgcaatggcgtgatcttggctcactggaacctctgcctcccaggttgaagtggttctcctgcctcagcctcccgagtagctaggatcacaggtgcccatcaccgcctggctaattctgtttttttttgtagagacggggtttcaccatgttggcaaggctggtcttgaactcctgaccttaggtgatccgcccacctcagcctcctagagtgctgggattacaggcgtaagccaccgcgcctggccttctgcatttttaagtttctatggttccaccattctcaccttggcctgttctttcattatggctttctgtttctacttcaaaaatggcacattttctggtatttttttgaagaggcccaatagtttcttgaaaatttcttctaactcctgaaactgagattatacactgatcatatatgattttatgactctttaaaacaatgtttctcagtatcctgtcctaagtcccaagttttaccacctttacttcacccagacctgtggccactttactcatctttggctataccaagagatatctctggtaacaggacgattatttttgtttacctttcaatgtttaaaaaatgtcttgccttgtatatacatgctccagtaataattattttgaaaacaaaagtttttaaacctgtgaacagcataataaaaaactttttctatcccacaaagagcacaataaaaaaaaaatcaacatctgttaatctaggatacagtatatagaaaagttatggtatcaagatgatagtttaaagatatacatttttgctttcaaaagcaaggattctaatatattaggaaaatagaaagacagtattatttaaccctgttctcacataagcaccaattttattccaaataatcacataattttaagaaataattttcctaatatatttttacaaaaagtcacttcagtgtcatacattctagaaacgccatcttgtatattagtattaccttacctgaactgaaacattccaaaagttccaataccttctacagatttcatttttacagttcaaaaaaattatttatttttcatgataaatgatgctactgataactttacttggtagaattgtagttactttggtaatttctacatgtttataaataagcaccacatatactatattaaaaaattagccagtctaagggcttgcactggagaccagggagttacattttgttaaacccagattgaacagagttgaatttagattaatacagagaaatgcatgctctgggtttgttgtcctttgtatttcttgaagcatcagatgaatcgtaaaaagttcaaagagcttcttattactcttgattttggaaagtttctgtaaaataatactgagtttttctagtatttgaagatcaagcttaggggctcgaagcagcacagagcaagtacgaaaaaataaagagttgctacaggcttccaggaaaggctgcaaggatttagattccaccgtcatctggagcaaactatcaataacattagacaggagtcctttactggatattcttagatgacttaatattactggaacagcctgatactccaaaaacaaggtttttccttcttctgtcttcaagtccaaacaaagagaatcaaatgcctgagccaggtaatcagcttgagtgactgttttgagaacaattaaggttgataaaaatctcaatggcaaattggagctcttaaagaaagcagctgtctttggtttattctccacagaatgctgtggagaattatcctgaattcctttagttaccactcctttaaaaatgtcttcacccaatctcctcaatgttgatgtcatagtcgagtgctgtgctccagcatctagctgccttagggaccaatatataaattttacaaaaggctcgtgaagtttgatattcacaaatggcatccactgtagctgctctgtcattagaggcaaaagctttacacacttctcctgaatatcatttctctgggaagcaaatttgagttgtggttttttaccatccattccagattcttcatgtttcactttgctaagatgatgatccgaaatccagtccatgaagacagttaaaagttcataaacttgcccattaagtggtaccttgtaagtttttgaaactggtgctttttcttgttttaaacttttcatttcatgaacagcatgggaacttcctttcaatctctgtattgtcataaactcgtacttcctctgtaaattatctaaacgagcttgaactcttttagcctgaatgtctatcttcctgttttcttcacttgcttcatttaactgtttttttaaggtatcattcaattctttcaatgcatcaaaagaggacctcagtctcttggtttctttattcttttccttaagaacttcggttaagtgttcaacttctgcatcatgctcttttataatttgaaatcttgtaagaacctcttcttcaacacctttaattttactcaaggcattttcatgtctgaaaagcagttgttctctttcaagtaaaaaacgttctcgcttttgaagttcttcagcaaatttctgttgtgctgcagtttcacactgcaatttcagatgtatctgaaataattcgtcatatatctgactgatctgatgtggaagtaaactccgcttgtctgatgctttagattttggacagctgacaggtttcaaaggagagtcacctgcatcactacaacactcagtccgaggtctcgatgaggtcgtattagttggcaaggcaactttttctatttctttaaaagactgcttggttattttcgaggtactaactctataatcattttcaattaactcttcttctgtttcctgtttcttcaaatcatggaaagaatccagttcatcatctaggcaattcacatttacgtgcttgaataagctgcccaatggtgttctacaatgcttgctttcatcagaatattttaacgatgaaccaactttatctccagagtagatatccaaatcacctggggaggttagagttcttctcttatacttagactgataaaaatttgaaaaatcatactcgtcggggcagctgcccccgagtccgtagcggcttttgagactctccactactaaatcctgccccggtggcttgacgaccctcggctccatagcacacagcaaccgtaccagtctccccgggaaccgcgttcatcaaacccgcggcgctacgcggccgcagt

SEQ ID NO: 12639 - RNA, 3175 nt, Homo sapiens
  source 1..3175: mol_type = other RNA
gatctcactttgttgcccaggctggagtgcaatggcgtgatcttggctcactggaacctctgcctcccaggttgaagtggttctcctgcctcagcctcccgagtagctaggatcacaggtgcccatcaccgcctggctaattctgtttttttttgtagagacggggtttcaccatgttggcaaggctggtcttgaactcctgaccttaggtgatccgcccacctcagcctcctagagtgctgggattacaggcgtaagccaccgcgcctggccttctgcatttttaagtttctatggttccaccattctcaccttggcctgttctttcattatggctttctgtttctacttcaaaaatggcacattttctggtatttttttgaagaggcccaatagtttcttgaaaatttcttctaactcctgaaactgagattatacactgatcatatatgattttatgactctttaaaacaatgtttctcagtatcctgtcctaagtcccaagttttaccacctttacttcacccagacctgtggccactttactcatctttggctataccaagagatatctctggtaacaggacgattatttttgtttacctttcaatgtttaaaaaatgtcttgccttgtatatacatgctccagtaataattattttgaaaacaaaagtttttaaacctgtgaacagcataataaaaaactttttctatcccacaaagagcacaataaaaaaaaaatcaacatctgttaatctaggatacagtatatagaaaagttatggtatcaagatgatagtttaaagatatacatttttgctttcaaaagcaaggattctaatatattaggaaaatagaaagacagtattatttaaccctgttctcacataagcaccaattttattccaaataatcacataattttaagaaataattttcctaatatatttttacaaaaagtcacttcagtgtcatacattctagaaacgccatcttgtatattagtattaccttacctgaactgaaacattccaaaagttccaataccttctacagatttcatttttacagttcaaaaaaattatttatttttcatgataaatgatgctactgataactttacttggtagaattgtagttactttggtaatttctacatgtttataaataagcaccacatatactatattaaaaaattagccagtctaagggcttgcactggagaccagggagttacattttgttaaacccagattgaacagagttgaatttagattaatacagagaaatgcatgctctgggtttgttgtcctttgtatttcttgaagcatcagatgaatcgtaaaaagttcaaagagcttcttattactcttgattttggaaagtttctgtaaaataatactgagtttttctagtatttgaagatcaagcttaggggctcgaagcagcacagagcaagtacgaaaaaataaagagttgctacaggcttccaggaaaggctgcaaggatttagattccaccgtcatctggagcaaactatcaataacattagacaggagtcctttactggatattcttagatgacttaatattactggaacagcctgatactccaaaaacaaggtttttccttcttctgtcttcaagtccaaacaaagagaatcaaatgcctgagccaggtaatcagcttgagtgactgttttgagaacaattaaggttgataaaaatctcaatggcaaattggagctcttaaagaaagcagctgtctttggtttattctccacagaatgctgtggagaattatcctgaattcctttagttaccactcctttaaaaatgtcttcacccaatctcctcaatgttgatgtcatagtcgagtgctgtgctccagcatctagctgccttagggaccaatatataaattttacaaaaggctcgtgaagtttgatattcacaaatggcatccactgtagctgctctgtcattagaggcaaaagctttacacacttctcctgaatatcatttctctgggaagcaaatttgagttgtggttttttaccatccattccagattcttcatgtttcactttgctaagatgatgatccgaaatccagtccatgaagacagttaaaagttcataaacttgcccattaagtggtaccttgtaagtttttgaaactggtgctttttcttgttttaaacttttcatttcatgaacagcatgggaacttcctttcaatctctgtattgtcataaactcgtacttcctctgtaaattatctaaacgagcttgaactcttttagcctgaatgtctatcttcctgttttcttcacttgcttcatttaactgtttttttaaggtatcattcaattctttcaatgcatcaaaagaggacctcagtctcttggtttctttattcttttccttaagaacttcggttaagtgttcaacttctgcatcatgctgctcttttataatttgaaatcttgtaagaacctcttcttcaacacctttaattttactcaaggcattttcatgtctgaaaagcagttgttctctttcaagtaaaaaacgttctcgcttttgaagttcttcagcaaatttctgttgtgctgcagtttcacactgcaatttcagatgtatctgaaataattcgtcatatatctgactgatctgatgtggaagtaaactccgcttgtctgatgctttagattttggacagctgacaggtttcaaaggagagtcacctgcatcactacaacactcagtccgaggtctcgatgaggtcgtattagttggcaaggcaactttttctatttctttaaaagactgcttggttattttcgaggtactaactctataatcattttcaattaactcttcttctgtttcctgtttcttcaaatcatggaaagaatccagttcatcatcaattcacatttacgtgcttgaataagctgcccaatggtgttctacaatgcttgctttcatcagaatattttaacgatgaaccaactttatctccagagtagatatccaaatcacctcgtcggggcagctgcccccgagtccgtagcggcttttgagactctccactactaaatcctgccccggtggcttgacgaccctcggctccatagcacacagcaaccgtaccagtctccccgggaacc

SEQ ID NO: 12640 - RNA, 3160 nt, Homo sapiens
  source 1..3160: mol_type = other RNA
gatctcactttgttgcccaggctggagtgcaatggcgtgatcttggctcactggaacctctgcctcccaggttgaagtggttctcctgcctcagcctcccgagtagctaggatcacaggtgcccatcaccgcctggctaattctgtttttttttgtagagacggggtttcaccatgttggcaaggctggtcttgaactcctgaccttaggtgatccgcccacctcagcctcctagagtgctgggattacaggcgtaagccaccgcgcctggccttctgcatttttaagtttctatggttccaccattctcaccttggcctgttctttcattatggctttctgtttctacttcaaaaatggcacattttctggtatttttttgaagaggcccaatagtttcttgaaaatttcttctaactcctgaaactgagattatacactgatcatatatgattttatgactctttaaaacaatgtttctcagtatcctgtcctaagtcccaagttttaccacctttacttcacccagacctgtggccactttactcatctttggctataccaagagatatctctggtaacaggacgattatttttgtttacctttcaatgtttaaaaaatgtcttgccttgtatatacatgctccagtaataattattttgaaaacaaaagtttttaaacctgtgaacagcataataaaaaactttttctatcccacaaagagcacaataaaaaaaaaatcaacatctgttaatctaggatacagtatatagaaaagttatggtatcaagatgatagtttaaagatatacatttttgctttcaaaagcaaggattctaatatattaggaaaatagaaagacagtattatttaaccctgttctcacataagcaccaattttattccaaataatcacataattttaagaaataattttcctaatatatttttacaaaaagtcacttcagtgtcatacattctagaaacgccatcttgtatattagtattaccttacctgaactgaaacattccaaaagttccaataccttctacagatttcatttttacagttcaaaaaaattatttatttttcatgataaatgatgctactgataactttacttggtagaattgtagttactttggtaatttctacatgtttataaataagcaccacatatactatattaaaaaattagccagtctaagggcttgcactggagaccagggagttacattttgttaaacccagattgaacagagttgaatttagattaatacagagaaatgcatgctctgggtttgttgtcctttgtatttcttgaagcatcagatgaatcgtaaaaagttcaaagagcttcttattactcttgattttggaaagtttctgtaaaataatactgagtttttctagtatttgaagatcaagcttaggggctcgaagcagcacagagcaagtacgaaaaaataaagagttgctacaggcttccaggaaaggctgcaaggatttagattccaccgtcatctggagcaaactatcaataacattagacaggagtcctttactggatattcttagatgacttaatattactggaacagcctgatactccaaaaacaaggtttttccttcttctgtcttcaagtccaaacaaagagaatcaaatgcctgagccaggtaatcagcttgagtgactgttttgagaacaattaaggttgataaaaatctcaatggcaaattggagctcttaaagaaagcagctgtctttggtttattctccacagaatgctgtggagaattatcctgaattcctttagttaccactcctttaaaaatgtcttcacccaatctcctcaatgttgatgtcatagtcgagtgctgtgctccagcatctagctgccttagggaccaatatataaattttacaaaaggctcgtgaagtttgatattcacaaatggcatccactgtagctgctctgtcattagaggcaaaagctttacacacttctcctgaatatcatttctctgggaagcaaatttgagttgtggttttttaccatccattccagattcttcatgtttcactttgctaagatgatgatccgaaatccagtccatgaagacagttaaaagttcataaacttgcccattaagtggtaccttgtaagtttttgaaactggtgctttttcttgttttaaacttttcatttcatgaacagcatgggaacttcctttcaatctctgtattgtcataaactcgtacttcctctgtaaattatctaaacgagcttgaactcttttagcctgaatgtctatcttcctgttttcttcacttgcttcatttaactgtttttttaaggtatcattcaattctttcaatgcatcaaaagaggacctcagtctcttggtttctttattcttttccttaagaacttcggttaagtgttcaacttctgcatcatgctgctcttttataatttgaaatcttgtaagaacctcttcttcaacacctttaattttactcaaggcattttcatgtctgaaaagcagttgttctctttcaagtaaaaaacgttctcgcttttgaagttcttcagcaaatttctgttgtgctgcagtttcacactgcaatttcagatgtatctgaaataattcgtcatatatctgactgatctgatgtggaagtaaactccgcttgtctgatgctttagattttggacagctgacaggtttcaaaggagagtcacctgcatcactacaacactcagtccgaggtctcgatgaggtcgtattagttggcaaggcaactttttctatttctttaaaagactgcttggttattttcgaggtactaactctataatcattttcaattaactcttcttctgtttcctgtttcttcaaatcatggaaagaatccagttcatcatcaattcacatttacgtgcttgaataagctgcccaatggtgttctacaatgcttgctttcatcagaatattttaacgatgaaccaactttatctccagagtagatatccaaatcacctggggaggttagagttcttctcttatacttagactgataaaaatttgaaaaatcatacagtctccccgggaaccgcgttcatcaaacccgcggcgctacgcggccgcagtgc

SEQ ID NO: 12641 - RNA, 3221 nt, Homo sapiens
  source 1..3221: mol_type = other RNA
gatctcactttgttgcccaggctggagtgcaatggcgtgatcttggctcactggaacctctgcctcccaggttgaagtggttctcctgcctcagcctcccgagtagctaggatcacaggtgcccatcaccgcctggctaattctgtttttttttgtagagacggggtttcaccatgttggcaaggctggtcttgaactcctgaccttaggtgatccgcccacctcagcctcctagagtgctgggattacaggcgtaagccaccgcgcctggccttctgcatttttaagtttctatggttccaccattctcaccttggcctgttctttcattatggctttctgtttctacttcaaaaatggcacattttctggtatttttttgaagaggcccaatagtttcttgaaaatttcttctaactcctgaaactgagattatacactgatcatatatgattttatgactctttaaaacaatgtttctcagtatcctgtcctaagtcccaagttttaccacctttacttcacccagacctgtggccactttactcatctttggctataccaagagatatctctggtaacaggacgattatttttgtttacctttcaatgtttaaaaaatgtcttgccttgtatatacatgctccagtaataattattttgaaaacaaaagtttttaaacctgtgaacagcataataaaaaactttttctatcccacaaagagcacaataaaaaaaaaatcaacatctgttaatctaggatacagtatatagaaaagttatggtatcaagatgatagtttaaagatatacatttttgctttcaaaagcaaggattctaatatattaggaaaatagaaagacagtattatttaaccctgttctcacataagcaccaattttattccaaataatcacataattttaagaaataattttcctaatatatttttacaaaaagtcacttcagtgtcatacattctagaaacgccatcttgtatattagtattaccttacctgaactgaaacattccaaaagttccaataccttctacagatttcatttttacagttcaaaaaaattatttatttttcatgataaatgatgctactgataactttacttggtagaattgtagttactttggtaatttctacatgtttataaataagcaccacatatactatattaaaaaattagccagtctaagggcttgcactggagaccagggagttacattttgttaaacccagattgaacagagttgaatttagattaatacagagaaatgcatgctctgggtttgttgtcctttgtatttcttgaagcatcagatgaatcgtaaaaagttcaaagagcttcttattactcttgattttggaaagtttctgtaaaataatactgagtttttctagtatttgaagatcaagcttaggggctcgaagcagcacagagcaagtacgaaaaaataaagagttgctacaggcttccaggaaaggctgcaaggatttagattccaccgtcatctggagcaaactatcaataacattagacaggagtcctttactggatattcttagatgacttaatattactggaacagcctgatactccaaaaacaaggtttttccttcttctgtcttcaagtccaaacaaagagaatcaaatgcctgagccaggtaatcagcttgagtgactgttttgagaacaattaaggttgataaaaatctcaatggcaaattggagctcttaaagaaagcagctgtctttggtttattctccacagaatgctgtggagaattatcctgaattcctttagttaccactcctttaaaaatgtcttcacccaatctcctcaatgttgatgtcatagtcgagtgctgtgctccagcatctagctgccttagggaccaatatataaattttacaaaaggctcgtgaagtttgatattcacaaatggcatccactgtagctgctctgtcattagaggcaaaagctttacacacttctcctgaatatcatttctctgggaagcaaatttgagttgtggttttttaccatccattccagattcttcatgtttcactttgctaagatgatgatccgaaatccagtccatgaagacagttaaaagttcataaacttgcccattaagtggtaccttgtaagtttttgaaactggtgctttttcttgttttaaacttttcatttcatgaacagcatgggaacttcctttcaatctctgtattgtcataaactcgtacttcctctgtaaattatctaaacgagcttgaactcttttagcctgaatgtctatcttcctgttttcttcacttgcttcatttaactgtttttttaaggtatcattcaattctttcaatgcatcaaaagaggacctcagtctcttggtttctttattcttttccttaagaacttcggttaagtgttcaacttctgcatcatgctgctcttttataatttgaaatcttgtaagaacctcttcttcaacacctttaattttactcaaggcattttcatgtctgaaaagcagttgttctctttcaagtaaaaaacgttctcgcttttgaagttcttcagcaaatttctgttgtgctgcagtttcacactgcaatttcagatgtatctgaaataattcgtcatatatctgactgatctgatgtggaagtaaactccgcttgtctgatgctttagattttggacagctgacaggtttcaaaggagagtcacctgcatcactacaacactcagtccgaggtctcgatgaggtcgtattagttggcaaggcaactttttctatttctttaaaagactgcttggttattttcgaggtactaactctataatcattttcaattaactcttcttctgtttcctgtttcttcaaatcatggaaagaatccagttcatcatcaattcacatttacgtgcttgaataagctgcccaatggtgttctacaatgcttgctttcatcagaatattttaacgatgaaccaactttatctccagagtagatatccaaatcacctggggaggttagagttcttctcttatacttagactgataaaaatttgaaaaatcatactcaggcggcggcttcacctcgtcggggcagctgcccccgagtccgtagcggcttttgagactctccactactaaatcctgccccggtggcttgacgaccctcggctccatagcac

SEQ ID NO: 12642 - RNA, 3116 nt, Homo sapiens
  source 1..3116: mol_type = other RNA
gatctcactttgttgcccaggctggagtgcaatggcgtgatcttggctcactggaacctctgcctcccaggttgaagtggttctcctgcctcagcctcccgagtagctaggatcacaggtgcccatcaccgcctggctaattctgtttttttttgtagagacggggtttcaccatgttggcaaggctggtcttgaactcctgaccttaggtgatccgcccacctcagcctcctagagtgctgggattacaggcgtaagccaccgcgcctggccttctgcatttttaagtttctatggttccaccattctcaccttggcctgttctttcattatggctttctgtttctacttcaaaaatggcacattttctggtatttttttgaagaggcccaatagtttcttgaaaatttcttctaactcctgaaactgagattatacactgatcatatatgattttatgactctttaaaacaatgtttctcagtatcctgtcctaagtcccaagttttaccacctttacttcacccagacctgtggccactttactcatctttggctataccaagagatatctctggtaacaggacgattatttttgtttacctttcaatgtttaaaaaatgtcttgccttgtatatacatgctccagtaataattattttgaaaacaaaagtttttaaacctgtgaacagcataataaaaaactttttctatcccacaaagagcacaataaaaaaaaaatcaacatctgttaatctaggatacagtatatagaaaagttatggtatcaagatgatagtttaaagatatacatttttgctttcaaaagcaaggattctaatatattaggaaaatagaaagacagtattatttaaccctgttctcacataagcaccaattttattccaaataatcacataattttaagaaataattttcctaatatatttttacaaaaagtcacttcagtgtcatacattctagaaacgccatcttgtatattagtattaccttacctgaactgaaacattccaaaagttccaataccttctacagatttcatttttacagttcaaaaaaattatttatttttcatgataaatgatgctactgataactttacttggtagaattgtagttactttggtaatttctacatgtttataaataagcaccacatatactatattaaaaaattagccagtctaagggcttgcactggagaccagggagttacattttgttaaacccagattgaacagagttgaatttagattaatacagagaaatgcatgctctgggtttgttgtcctttgtatttcttgaagcatcagatgaatcgtaaaaagttcaaagagcttcttattactcttgattttggaaagtttctgtaaaataatactgagtttttctagtatttgaagatcaagcttaggggctcgaagcagcacagagcaagtacgaaaaaataaagagttgctacaggcttccaggaaaggctgcaaggatttagattccaccgtcatctggagcaaactatcaataacattagacaggagtcctttactggatattcttagatgacttaatattactggaacagcctgatactccaaaaacaaggtttttccttcttctgtcttcaagtccaaacaaagagaatcaaatgcctgagccaggtaatcagcttgagtgactgttttgagaacaattaaggttgataaaaatctcaatggcaaattggagctcttaaagaaagcagctgtctttggtttattctccacagaatgctgtggagaattatcctgaattcctttagttaccactcctttaaaaatgtcttcacccaatctcctcaatgttgatgtcatagtcgagtgctttacacacttctcctgaatatcatttctctgggaagcaaatttgagttgtggttttttaccatccattccagattcttcatgtttcactttgctaagatgatgatccgaaatccagtccatgaagacagttaaaagttcataaacttgcccattaagtggtaccttgtaagtttttgaaactggtgctttttcttgttttaaacttttcatttcatgaacagcatgggaacttcctttcaatctctgtattgtcataaactcgtacttcctctgtaaattatctaaacgagcttgaactcttttagcctgaatgtctatcttcctgttttcttcacttgcttcatttaactgtttttttaaggtatcattcaattctttcaatgcatcaaaagaggacctcagtctcttggtttctttattcttttccttaagaacttcggttaagtgttcaacttctgcatcatgctgctcttttataatttgaaatcttgtaagaacctcttcttcaacacctttaattttactcaaggcattttcatgtctgaaaagcagttgttctctttcaagtaaaaaacgttctcgcttttgaagttcttcagcaaatttctgttgtgctgcagtttcacactgcaatttcagatgtatctgaaataattcgtcatatatctgactgatctgatgtggaagtaaactccgcttgtctgatgctttagattttggacagctgacaggtttcaaaggagagtcacctgcatcactacaacactcagtccgaggtctcgatgaggtcgtattagttggcaaggcaactttttctatttctttaaaagactgcttggttattttcgaggtactaactctataatcattttcaattaactcttcttctgtttcctgtttcttcaaatcatggaaagaatccagttcatcatctaggcaattcacatttacgtgcttgaataagctgcccaatggtgttctacaatgcttgctttcatcagaatattttaacgatgaaccaactttatctccagagtagatatccaaatcacctcgtcggggcagctgcccccgagtccgtagcggcttttgagactctccactactaaatcctgccccggtggcttgacgaccctcggctccatagcacacagcaaccgtaccagtctccccgggaaccgcgttcatcaaacccgcggcgctacgcggccgcagtgcgtcacgacgtgccag

SEQ ID NO: 12643 - RNA, 3144 nt, Homo sapiens
  source 1..3144: mol_type = other RNA
gatctcactttgttgcccaggctggagtgcaatggcgtgatcttggctcactggaacctctgcctcccaggttgaagtggttctcctgcctcagcctcccgagtagctaggatcacaggtgcccatcaccgcctggctaattctgtttttttttgtagagacggggtttcaccatgttggcaaggctggtcttgaactcctgaccttaggtgatccgcccacctcagcctcctagagtgctgggattacaggcgtaagccaccgcgcctggccttctgcatttttaagtttctatggttccaccattctcaccttggcctgttctttcattatggctttctgtttctacttcaaaaatggcacattttctggtatttttttgaagaggcccaatagtttcttgaaaatttcttctaactcctgaaactgagattatacactgatcatatatgattttatgactctttaaaacaatgtttctcagtatcctgtcctaagtcccaagttttaccacctttacttcacccagacctgtggccactttactcatctttggctataccaagagatatctctggtaacaggacgattatttttgtttacctttcaatgtttaaaaaatgtcttgccttgtatatacatgctccagtaataattattttgaaaacaaaagtttttaaacctgtgaacagcataataaaaaactttttctatcccacaaagagcacaataaaaaaaaaatcaacatctgttaatctaggatacagtatatagaaaagttatggtatcaagatgatagtttaaagatatacatttttgctttcaaaagcaaggattctaatatattaggaaaatagaaagacagtattatttaaccctgttctcacataagcaccaattttattccaaataatcacataattttaagaaataattttcctaatatatttttacaaaaagtcacttcagtgtcatacattctagaaacgccatcttgtatattagtattaccttacctgaactgaaacattccaaaagttccaataccttctacagatttcatttttacagttcaaaaaaattatttatttttcatgataaatgatgctactgataactttacttggtagaattgtagttactttggtaatttctacatgtttataaataagcaccacatatactatattaaaaaattagccagtctaagggcttgcactggagaccagggagttacattttgttaaacccagattgaacagagttgaatttagattaatacagagaaatgcatgctctgggtttgttgtcctttgtatttcttgaagcatcagatgaatcgtaaaaagttcaaagagcttcttattactcttgattttggaaagtttctgtaaaataatactgagtttttctagtatttgaagatcaagcttaggggctcgaagcagcacagagcaagtacgaaaaaataaagagttgctacaggcttccaggaaaggctgcaaggatttagattccaccgtcatctggagcaaactatcaataacattagacaggagtcctttactggatattcttagatgacttaatattactggaacagcctgatactccaaaaacaaggtttttccttcttctgtcttcaagtccaaacaaagagaatcaaatgcctgagccaggtaatcagcttgagtgactgttttgagaacaattaaggttgataaaaatctcaatggcaaattggagctcttaaagaaagcagctgtctttggtttattctccacagaatgctgtggagaattatcctgaattcctttagttaccactcctttaaaaatgtcttcacccaatctcctcaatgttgatgtcatagtcgagtgctttacacacttctcctgaatatcatttctctgggaagcaaatttgagttgtggttttttaccatccattccagattcttcatgtttcactttgctaagatgatgatccgaaatccagtccatgaagacagttaaaagttcataaacttgcccattaagtggtaccttgtaagtttttgaaactggtgctttttcttgttttaaacttttcatttcatgaacagcatgggaacttcctttcaatctctgtattgtcataaactcgtacttcctctgtaaattatctaaacgagcttgaactcttttagcctgaatgtctatcttcctgttttcttcacttgcttcatttaactgtttttttaaggtatcattcaattctttcaatgcatcaaaagaggacctcagtctcttggtttctttattcttttccttaagaacttcggttaagtgttcaacttctgcatcatgctgctcttttataatttgaaatcttgtaagaacctcttcttcaacacctttaattttactcaaggcattttcatgtctgaaaagcagttgttctctttcaagtaaaaaacgttctcgcttttgaagttcttcagcaaatttctgttgtgctgcagtttcacactgcaatttcagatgtatctgaaataattcgtcatatatctgactgatctgatgtggaagtaaactccgcttgtctgatgctttagattttggacagctgacaggtttcaaaggagagtcacctgcatcactacaacactcagtccgaggtctcgatgaggtcgtattagttggcaaggcaactttttctatttctttaaaagactgcttggttattttcgaggtactaactctataatcattttcaattaactcttcttctgtttcctgtttcttcaaatcatggaaagaatccagttcatcatctaggcaattcacatttacgtgcttgaataagctgcccaatggtgttctacaatgcttgctttcatcagaatattttaacgatgaaccaactttatctccagagtagatatccaaatcacctggggaggttagagttcttctcttatacttagactgataaaaatttgaaaaatcatactcaggcggcggcttcacctcgtcggggcagctgcccccgagtccgtagcggcttttgagactctccactactaaatcctgccccggtggcttgacgaccctcggctccatagcacacagcaaccgtaccagtctccccgggaaccgcgtt

SEQ ID NO: 12644 - RNA, 3206 nt, Homo sapiens
  source 1..3206: mol_type = other RNA
gatctcactttgttgcccaggctggagtgcagtaggcatgatcttggctcactgcaacctccacctcctgggttcaagcgattctcatgcctcaaccaggcgccaccacacctggctaatttttgtatttttagtagagatggggtttcaccatgttggccaggctggtcttgaactcctgacctcaggtgatccacccacctcggcctcccaaagtgctgggattacaggcgtgagccaccgcgcctggcctcatctaaccaatttggattctggttggagttcaggaaaaactaagttcccattacttccagattattttaaaataaaaaatcatgatgacttgtgaggaaaaggaagaacatgtcagatcctgagcttcctctcaggcttgagtgcctcaagaggactgtattgctgtgttacgagaggtacagtgcaatgctttcatctgatatgccagtgtggtaagaaggctttccctggaggtagagactcttttatcagaaggttgggggtctccagaaggttttccccaccaggaattggatttgatggctggaatttagagcctacacatttgggtctcacaatcagggcagggcaggtaaggctaatggtgcaaactgtgtctctgcacaggcagtcatctaggggaaggggtgtggtgcagccagtaaaacctggaacctgcaagtggttcagaactttggtggccagtaagggaaaaactcctcaagcatgctacaatattgaaaggttcaaaagcactgacaaagtgttgttttgcccccggtgcagcacataagactctgttccagtgaaatgctacattcaaagtgctgtccacctcagaagatcccagaggatgcaattctggctgtgctgggaagtgctaaagttccctccatatgtcactttggagaaggaagcagcaaagcagccatgttgattcctctctcaacctttggcatcatggacgatggtagcgtgtaaaatgtttgctctcttcatgaacctccatctcggagcttttaaattcatttaattcttttcttatggcagccttgtcagcaggggtcagtttggtccaaggtttgtcggctcgccggtcataatcttgagcatctgttacctctacatattcattaaacctcagaatcttcctggcaaggagttcagcgacagttggcctttgactgagctttctagtgagccgacgtttaatttctcgtttttctgcctgacgatcagcttcatttttaggttgcaatatattgcgttgttctagttcttctggtgttggtctttgactcagtcgccggatcagtgtgtttccaatctggtgccgtatttcattccactcctccttgcttttacaaggccaagaattcaggttcaactctggttcactgggtctgtggttcaacttcattgccagtgtgtctttcctcttcactttgttggcgagagcactctgatagctttcatcttcatcttcttcatctcggtactgaatgggaccttctgaatcagagtcgctctccttctcttcttcctcccgtagacactgtggtaatttaggaatgactgaggtaggtgtcatttcttcactgaatgtggatggacaggtttgctcctcttcttcttcatcgtctggaacttttagcatttcaatagtgatgggaagagacctggtccgacccagcgtactgctgtcctcagaaaagctgtcactgttttcaaaaagcaacgaatgagctctgtgagaaccctccagaataggagtcatgggaagtgggctggtgagggcctgctggattcgaatatgcagtgggagtggaggcagcctagagggtatatggggctccccaaagttctggtccagtatcctcttggggacttcctttttctgatcttcctgctggggaatctcctggtgtagatctaaggatggtggaaactcaatttctggcacaacttgaaaagtcttagcagggaatggaggggtgcgtggaggctctggaggtatatgagtaggcagtgggggggacggagagcgaggtgagatcattggtagtagttccgagcccatagaacacgtgctcttctctctttcatcacttggtgtttttgtggtgatggcagcagcagactccaaggtgggtactgaggttgatggaatgcctctcttaggtggtaagggtggggacggttttgataacaatgtaccactgtttattgcttgggacagttcagcaatgacagggttgctatttctgtgagctggtttagggggagggatagggggctgcttggcagggaccatatgagtgaggcttggggtagcagtagtgttagtgctggcaggagcagcaggcagagtcctgggtgctggggaaggggtgacagagagattaacagtctttgcaaggcttgtggcagcagtggtggcagcgggtgctgtggtgatggaggtggagatgatgaaccttgccgtgccgccagaggaagtggcatcctttgcttgcccttcacttgcttcatgagaagaggacaagggtcttttgggaggaagtaaaggtggtttgggtacattctcaggaacagactctgcttcagaattaggctggcttccagttgagcctagtcgtttctttaggtcctcttctggaatagctttcctaagacttgctaatcttactggctcttcctctacttggactggactagatgatctggcattccctatgggggtggtatggccattctttaacatggcatcgcttggctttcctggatcctcaccaccttgctcagggtcttccaacagaacccctcttttaaccagctcttctcttggctttcgcatagatattttccgttctaaaacttctgaagtctctttaaatttatcactacttttttttttcctccatttccagggcttgaagatcttgccaaagcctgagaacttgctcttccttttggtaggaggtgttgtgtctcctgcttccacactgtccaggaccatgcctggctctgtagtgggctggtctgcttcctcaaatggatcttccatgccactattaaccagtttagggaggtgagatactgtttccagatctccgccgccgcctcctcagcctccacagcagcctctcccggaaatcctacctggcccgttggccgccaggcagcagccg

SEQ ID NO: 12645 - RNA, 3306 nt, Homo sapiens
  source 1..3306: mol_type = other RNA
gatctcactttgttgcccaggctggagtgcagtaggcatgatcttggctcactgcaacctccacctcctgggttcaagcgattctcatgcctcaaccaggcgccaccacacctggctaatttttgtatttttagtagagatggggtttcaccatgttggccaggctggtcttgaactcctgacctcaggtgatccacccacctcggcctcccaaagtgctgggattacaggcgtgagccaccgcgcctggcctcatctaaccaatttggattctggttggagttcaggaaaaactaagttcccattacttccagattattttaaaataaaaaatcatgatgacttgtgaggaaaaggaagaacatgtcagatcctgagcttcctctcaggcttgagtgcctcaagaggactgtattgctgtgttacgagaggtacagtgcaatgctttcatctgatatgccagtgtggtaagaaggctttccctggaggtagagactcttttatcagaaggttgggggtctccagaaggttttccccaccaggaattggatttgatggctggaatttagagcctacacatttgggtctcacaatcagggcagggcaggtaaggctaatggtgcaaactgtgtctctgcacaggcagtcatctaggggaaggggtgtggtgcagccagtaaaacctggaacctgcaagtggttcagaactttggtggccagtaagggaaaaactcctcaagcatgctacaatattgaaaggttcaaaagcactgacaaagtgttgttttgcccccggtgcagcacataagactctgttccagtgaaatgctacattcaaagtgctgtccacctcagaagatcccagaggatgcaattctggctgtgctgggaagtgctaaagttccctccatatgtcactttggagaaggaagcagcaaagcagccatgttgattcctctctcaacctttggcatcatggacgatggtagcgtgtaaaatgtttgctctcttcatgaacctccatctcggagcttttaaattcatttaattcttttcttatggcagccttgtcagcaggggtcagtttggtccaaggtttgtcggctcgccggtcataatcttgagcatctgttacctctacatattcattaaacctcagaatcttcctggcaaggagttcagcgacagttggcctttgactgagctttctagtgagccgacgtttaatttctcgtttttctgcctgacgatcagcttcatttttaggttgcaatatattgcgttgttctagttcttctggtgttggtctttgactcagtcgccggatcagtgtgtttccaatctggtgccgtatttcattccactcctccttgcttttacaaggccaagaattcaggttcaactctggttcactgggtctgtggttcaacttcattgccagtgtgtctttcctcttcactttgttggcgagagcactctgatagctttcatcttcatcttcttcatctcggtactgaatgggaccttctgaatcagagtcgctctccttctcttcttcctcccgtagacactgtggtaatttaggaatgactgaggtaggtgtcatttcttcactgaatgtggatggacaggtttgctcctcttcttcttcatcgtctggaacttttagcatttcaatagtgatgggaagagacctggtccgacccagcgtactgctgtcctcagaaaagctgtcactgttttcaaaaagcaacgaatgagctctgtgagaaccctccagaataggagtcatgggaagtgggctggtgagggcctgctggattcgaatatgcagtgggagtggaggcagcctagagggtatatggggctccccaaagttctggtccagtatcctcttggggacttcctttttctgatcttcctgctggggaatctcctggtgtagatctaaggatggtggaaactcaatttctggcacaacttgaaaagtcttagcagggaatggaggggtgcgtggaggctctggaggtatatgagtaggcagtgggggggacggagagcgaggtgagatcattggtagtagttccgagcccatagaacacgtgctcttctctctttcatcacttggtgtttttgtggtgatggcagcagcagactccaaggtgggtactgaggttgatggaatgcctctcttaggtggtaagggtggggacggttttgataacaatgtaccactgtttattgcttgggacagttcagcaatgacagggttgctatttctgtgagctggtttagggggagggatagggggctgcttggcagggaccatatgagtgaggcttggggtagcagtagtgttagtgctggcaggagcagcaggcagagtcctgggtgctggggaaggggtgacagagagattaacagtctttgcaaggcttgtggcagcagtggtggcagcgggtgctgtggtgatggaggtggagatgatgaaccttgccgtgccgccagaggaagtggcatcctttgcttgcccttcacttgcttcatgagaagaggacaagggtcttttgggaggaagtaaaggtggtttgggtacattctcaggaacagactctgcttcagaattaggctggcttccagttgagcctagtcgtttctttaggtcctcttctggaatagctttcctaagacttgctaatcttactggctcttcctctacttggactggactagatgatctggcattccctatgggggtggtatggccattctttaacatggcatcgcttggctttcctggatcctcaccaccttgctcagggtcttccaacagaacccctcttttaaccagctcttctcttggctttcgcatagatattttccgttctaaaacttctgaagtctctttaaatttatcactacttttttttttcctccatttccagggcttgaagatcttgccaaagcctgagaacttgctcttccttttggtaggaggtgttgtgtctcctgcttccacactgtccaggaccatgcctggctctgtagtgggctggtctgcttcctcaaatggatcttccatgccactattaaccagtttagggaggtgagatactgttttgtgcactgtgattgtaacttctgcaatgtggagtacaacagcaaaactagcacaattttcttttttcgtcttcacaatttcacagatagaaaattcattccagatctccgccgccgcctcctcagcctccacagcagcctctcccggaaatcctacctggcccgttggccgccaggcagcagccg

SEQ ID NO: 12646 - RNA, 3347 nt, Homo sapiens
  source 1..3347: mol_type = other RNA
gatctcactttgttgcccaggctggagtgcagtaggcatgatcttggctcactgcaacctccacctcctgggttcaagcgattctcatgcctcaaccaggcgccaccacacctggctaatttttgtatttttagtagagatggggtttcaccatgttggccaggctggtcttgaactcctgacctcaggtgatccacccacctcggcctcccaaagtgctgggattacaggcgtgagccaccgcgcctggcctcatctaaccaatttggattctggttggagttcaggaaaaactaagttcccattacttccagattattttaaaataaaaaatcatgatgacttgtgaggaaaaggaagaacatgtcagatcctgagcttcctctcaggcttgagtgcctcaagaggactgtattgctgtgttacgagaggtacagtgcaatgctttcatctgatatgccagtgtggtaagaaggctttccctggaggtagagactcttttatcagaaggttgggggtctccagaaggttttccccaccaggaattggatttgatggctggaatttagagcctacacatttgggtctcacaatcagggcagggcaggtaaggctaatggtgcaaactgtgtctctgcacaggcagtcatctaggggaaggggtgtggtgcagccagtaaaacctggaacctgcaagtggttcagaactttggtggccagtaagggaaaaactcctcaagcatgctacaatattgaaaggttcaaaagcactgacaaagtgttgttttgcccccggtgcagcacataagactctgttccagtgaaatgctacattcaaagtgctgtccacctcagaagatcccagaggatgcaattctggctgtgctgggaagtgctaaagttccctccatatgtcactttggagaaggaagcagcaaagcagccatgttgattcctctctcaacctttggcatcatggacgatggtagcgtgtaaaatgtttgctctcttcatgaacctccatctcggagcttttaaattcatttaattcttttcttatggcagccttgtcagcaggggtcagtttggtccaaggtttgtcggctcgccggtcataatcttgagcatctgttacctctacatattcattaaacctcagaatcttcctggcaaggagttcagcgacagttggcctttgactgagctttctagtgagccgacgtttaatttctcgtttttctgcctgacgatcagcttcatttttaggttgcaatatattgcgttgttctagttcttctggtgttggtctttgactcagtcgccggatcagtgtgtttccaatctggtgccgtatttcattccactcctccttgcttttacaaggccaagaattcaggttcaactctggttcactgggtctgtggttcaacttcattgccagtgtgtctttcctcttcactttgttggcgagagcactctgatagctttcatcttcatcttcttcatctcggtactgaatgggaccttctgaatcagagtcgctctccttctcttcttcctcccgtagacactgtggtaatttaggaatgactgaggtaggtgtcatttcttcactgaatgtggatggacaggtttgctcctcttcttcttcatcgtctggaacttttagcatttcaatagtgatgggaagagacctggtccgacccagcgtactgctgtcctcagaaaagctgtcactgttttcaaaaagcaacgaatgagctctgtgagaaccctccagaataggagtcatgggaagtgggctggtgagggcctgctggattcgaatatgcagtgggagtggaggcagcctagagggtatatggggctccccaaagttctggtccagtatcctcttggggacttcctttttctgatcttcctgctggggaatctcctggtgtagatctaaggatggtggaaactcaatttctggcacaacttgaaaagtcttagcagggaatggaggggtgcgtggaggctctggaggtatatgagtaggcagtgggggggacggagagcgaggtgagatcattggtagtagttccgagcccatagaacacgtgctcttctctctttcatcacttggtgtttttgtggtgatggcagcagcagactccaaggtgggtactgaggttgatggaatgcctctcttaggtggtaagggtggggacggttttgataacaatgtaccactgtttattgcttgggacagttcagcaatgacagggttgctatttctgtgagctggtttagggggagggatagggggctgcttggcagggaccatatgagtgaggcttggggtagcagtagtgttagtgctggcaggagcagcaggcagagtcctgggtgctggggaaggggtgacagagagattaacagtctttgcaaggcttgtggcagcagtggtggcagcgggtgctgtggtgatggaggtggagatgatgaaccttgccgtgccgccagaggaagtggcatcctttgcttgcccttcacttgcttcatgagaagaggacaagggtcttttgggaggaagtaaaggtggtttgggtacattctcaggaacagactctgcttcagaattaggctggcttccagttgagcctagtcgtttctttaggtcctcttctggaatagctttcctaagacttgctaatcttactggctcttcctctacttggactggactagatgatctggcattccctatgggggtggtatggccattctttaacatggcatcgcttggctttcctggatcctcaccaccttgctcagggtcttccaacagaacccctcttttaaccagctcttctcttggctttcgcatagatattttccgttctaaaacttctgaagtctctttaaatttatcactacttttttttttcctccatttccagggcttgaagatcttgccaaagcctgagaacttgctcttccttttggtaggaggtgttgtgtctcctgcttccacactgtccaggaccatgcctggctctgtagtgggctggtctgcttcctcaactgcatctggatttaccggtctggagacatcagcttgtcccatgattatattgtctgatgtatctcacgacaacaaactgtcccggacaaaagcaaacttttcataaaagataaatccacataaagaggggacatgcggtcctctttcagtgtcactgccaaacatcaggaaatggcataaggtcagttcatctgctgaagtttctgtttcccatacagcctgagcacttgcagttcttacaaaactgtcttcacactggcactcttcacacaggaat

SEQ ID NO: 12647 - RNA, 3234 nt, Homo sapiens
  source 1..3234: mol_type = other RNA
gatctcactttgttgcccaggctggagtgcagtaggcatgatcttggctcactgcaacctccacctcctgggttcaagcgattctcatgcctcaaccaggcgccaccacacctggctaatttttgtatttttagtagagatggggtttcaccatgttggccaggctggtcttgaactcctgacctcaggtgatccacccacctcggcctcccaaagtgctgggattacaggcgtgagccaccgcgcctggcctcatctaaccaatttggattctggttggagttcaggaaaaactaagttcccattacttccagattattttaaaataaaaaatcatgatgacttgtgaggaaaaggaagaacatgtcagatcctgagcttcctctcaggcttgagtgcctcaagaggactgtattgctgtgttacgagaggtacagtgcaatgctttcatctgatatgccagtgtggtaagaaggctttccctggaggtagagactcttttatcagaaggttgggggtctccagaaggttttccccaccaggaattggatttgatggctggaatttagagcctacacatttgggtctcacaatcagggcagggcaggtaaggctaatggtgcaaactgtgtctctgcacaggcagtcatctaggggaaggggtgtggtgcagccagtaaaacctggaacctgcaagtggttcagaactttggtggccagtaagggaaaaactcctcaagcatgctacaatattgaaaggttcaaaagcactgacaaagtgttgttttgcccccggtgcagcacataagactctgttccagtgaaatgctacattcaaagtgctgtccacctcagaagatcccagaggatgcaattctggctgtgctgggaagtgctaaagttccctccatatgtcactttggagaaggaagcagcaaagcagccatgttgattcctctctcaacctttggcatcatggacgatggtagcgtgtaaaatgtttgctctcttcatgaacctccatctcggagcttttaaattcatttaattcttttcttatggcagccttgtcagcaggggtcagtttggtccaaggtttgtcggctcgccggtcataatcttgagcatctgttacctctacatattcattaaacctcagaatcttcctggcaaggagttcagcgacagttggcctttgactgagctttctagtgagccgacgtttaatttctcgtttttctgcctgacgatcagcttcatttttaggttgcaatatattgcgttgttctagttcttctggtgttggtctttgactcagtcgccggatcagtgtgtttccaatctggtgccgtatttcattccactcctccttgcttttacaaggccaagaattcaggttcaactctggttcactgggtctgtggttcaacttcattgccagtgtgtctttcctcttcactttgttggcgagagcactctgatagctttcatcttcatcttcttcatctcggtactgaatgggaccttctgaatcagagtcgctctccttctcttcttcctcccgtagacactgtggtaatttaggaatgactgaggtaggtgtcatttcttcactgaatgtggatggacaggtttgctcctcttcttcttcatcgtctggaacttttagcatttcaatagtgatgggaagagacctggtccgacccagcgtactgctgtcctcagaaaagctgtcactgttttcaaaaagcaacgaatgagctctgtgagaaccctccagaataggagtcatgggaagtgggctggtgagggcctgctggattcgaatatgcagtgggagtggaggcagcctagagggtatatggggctccccaaagttctggtccagtatcctcttggggacttcctttttctgatcttcctgctggggaatctcctggtgtagatctaaggatggtggaaactcaatttctggcacaacttgaaaagtcttagcagggaatggaggggtgcgtggaggctctggaggtatatgagtaggcagtgggggggacggagagcgaggtgagatcattggtagtagttccgagcccatagaacacgtgctcttctctctttcatcacttggtgtttttgtggtgatggcagcagcagactccaaggtgggtactgaggttgatggaatgcctctcttaggtggtaagggtggggacggttttgataacaatgtaccactgtttattgcttgggacagttcagcaatgacagggttgctatttctgtgagctggtttagggggagggatagggggctgcttggcagggaccatatgagtgaggcttggggtagcagtagtgttagtgctggcaggagcagcaggcagagtcctgggtgctggggaaggggtgacagagagattaacagtctttgcaaggcttgtggcagcagtggtggcagcgggtgctgtggtgatggaggtggagatgatgaaccttgccgtgccgccagaggaagtggcatcctttgcttgcccttcacttgcttcatgagaagaggacaagggtcttttgggaggaagtaaaggtggtttgggtacattctcaggaacagactctgcttcagaattaggctggcttccagttgagcctagtcgtttctttaggtcctcttctggaatagctttcctaagacttgctaatcttactggctcttcctctacttggactggactagatgatctggcattccctatgggggtggtatggccattctttaacatggcatcgcttggctttcctggatcctcaccaccttgctcagggtcttccaacagaacccctcttttaaccagctcttctcttggctttcgcatagatattttccgttctaaaacttctgaagtctctttaaatttatcactacttttttttttcctccatttccagggcttgaagatcttgccaaagcctgagaacttgctcttccttttggtaggaggtgttgtgtctcctgcttccacactgtccaggaccatgcctggctctgtagtgggctggtctgcttcctctactgttccaaggttctctggagaagtcaaatggatcttccatgccactattaaccagtttagggaggtgagatactgtttccagatctccgccgccgcctcctcagcctccacagcagcctctcccggaaatcctacctggcccgttggccgccaggcagcagccg

SEQ ID NO: 12648 - RNA, 3230 nt, Homo sapiens
  source 1..3230: mol_type = other RNA
gatctcactttgttgcccaggctggagtgcagtaggcatgatcttggctcactgcaacctccacctcctgggttcaagcgattctcatgcctcaaccaggcgccaccacacctggctaatttttgtatttttagtagagatggggtttcaccatgttggccaggctggtcttgaactcctgacctcaggtgatccacccacctcggcctcccaaagtgctgggattacaggcgtgagccaccgcgcctggcctcatctaaccaatttggattctggttggagttcaggaaaaactaagttcccattacttccagattattttaaaataaaaaatcatgatgacttgtgaggaaaaggaagaacatgtcagatcctgagcttcctctcaggcttgagtgcctcaagaggactgtattgctgtgttacgagaggtacagtgcaatgctttcatctgatatgccagtgtggtaagaaggctttccctggaggtagagactcttttatcagaaggttgggggtctccagaaggttttccccaccaggaattggatttgatggctggaatttagagcctacacatttgggtctcacaatcagggcagggcaggtaaggctaatggtgcaaactgtgtctctgcacaggcagtcatctaggggaaggggtgtggtgcagccagtaaaacctggaacctgcaagtggttcagaactttggtggccagtaagggaaaaactcctcaagcatgctacaatattgaaaggttcaaaagcactgacaaagtgttgttttgcccccggtgcagcacataagactctgttccagtgaaatgctacattcaaagtgctgtccacctcagaagatcccagaggatgcaattctggctgtgctgggaagtgctaaagttccctccatatgtcactttggagaaggaagcagcaaagcagccatgttgattcctctctcaacctttggcatcatggacgatggtagcgtgtaaaatgtttgctctcttcatgaacctccatctcggagcttttaaattcatttaattcttttcttatggcagccttgtcagcaggggtcagtttggtccaaggtttgtcggctcgccggtcataatcttgagcatctgttacctctacatattcattaaacctcagaatcttcctggcaaggagttcagcgacagttggcctttgactgagctttctagtgagccgacgtttaatttctcgtttttctgcctgacgatcagcttcatttttaggttgcaatatattgcgttgttctagttcttctggtgttggtctttgactcagtcgccggatcagtgtgtttccaatctggtgccgtatttcattccactcctccttgcttttacaaggccaagaattcaggttcaactctggttcactgggtctgtggttcaacttcattgccagtgtgtctttcctcttcactttgttggcgagagcactctgatagctttcatcttcatcttcttcatctcggtactgaatgggaccttctgaatcagagtcgctctccttctcttcttcctcccgtagacactgtggtaatttaggaatgactgaggtaggtgtcatttcttcactgaatgtggatggacaggtttgctcctcttcttcttcatcgtctggaacttttagcatttcaatagtgatgggaagagacctggtccgacccagcgtactgctgtcctcagaaaagctgtcactgttttcaaaaagcaacgaatgagctctgtgagaaccctccagaataggagtcatgggaagtgggctggtgagggcctgctggattcgaatatgcagtgggagtggaggcagcctagagggtatatggggctccccaaagttctggtccagtatcctcttggggacttcctttttctgatcttcctgctggggaatctcctggtgtagatctaaggatggtggaaactcaatttctggcacaacttgaaaagtcttagcagggaatggaggggtgcgtggaggctctggaggtatatgagtaggcagtgggggggacggagagcgaggtgagatcattggtagtagttccgagcccatagaacacgtgctcttctctctttcatcacttggtgtttttgtggtgatggcagcagcagactccaaggtgggtactgaggttgatggaatgcctctcttaggtggtaagggtggggacggttttgataacaatgtaccactgtttattgcttgggacagttcagcaatgacagggttgctatttctgtgagctggtttagggggagggatagggggctgcttggcagggaccatatgagtgaggcttggggtagcagtagtgttagtgctggcaggagcagcaggcagagtcctgggtgctggggaaggggtgacagagagattaacagtctttgcaaggcttgtggcagcagtggtggcagcgggtgctgtggtgatggaggtggagatgatgaaccttgccgtgccgccagaggaagtggcatcctttgcttgcccttcacttgcttcatgagaagaggacaagggtcttttgggaggaagtaaaggtggtttgggtacattctcaggaacagactctgcttcagaattaggctggcttccagttgagcctagtcgtttctttaggtcctcttctggaatagctttcctaagacttgctaatcttactggctcttcctctacttggactggactagatgatctggcattccctatgggggtggtatggccattctttaacatggcatcgcttggctttcctggatcctcaccaccttgctcagggtcttccaacagaacccctcttttaaccagctcttctcttggctttcgcatagatattttccgttctaaaacttctgaagtctctttaaatttatcactacttttttttttcctccatttccagggcttgaagatcttgccaaagcctgagaacttgctcttccttttggtaggaggtgttgtgtctcctgcttccacactgtccaggaccatgcctggctctgtagtgggctggtctgcttccttgttccaaggttctctggagaagtcaaatggatcttccatgccactattaaccagtttagggaggtgagatactgtttccagatctccgccgccgcctcctcagcctccacagcagcctctcccggaaatcctacctggcccgttggccgccaggcagcagccg

SEQ ID NO: 12649 - RNA, 3330 nt, Homo sapiens
  source 1..3330: mol_type = other RNA
gatctcactttgttgcccaggctggagtgcagtaggcatgatcttggctcactgcaacctccacctcctgggttcaagcgattctcatgcctcaaccaggcgccaccacacctggctaatttttgtatttttagtagagatggggtttcaccatgttggccaggctggtcttgaactcctgacctcaggtgatccacccacctcggcctcccaaagtgctgggattacaggcgtgagccaccgcgcctggcctcatctaaccaatttggattctggttggagttcaggaaaaactaagttcccattacttccagattattttaaaataaaaaatcatgatgacttgtgaggaaaaggaagaacatgtcagatcctgagcttcctctcaggcttgagtgcctcaagaggactgtattgctgtgttacgagaggtacagtgcaatgctttcatctgatatgccagtgtggtaagaaggctttccctggaggtagagactcttttatcagaaggttgggggtctccagaaggttttccccaccaggaattggatttgatggctggaatttagagcctacacatttgggtctcacaatcagggcagggcaggtaaggctaatggtgcaaactgtgtctctgcacaggcagtcatctaggggaaggggtgtggtgcagccagtaaaacctggaacctgcaagtggttcagaactttggtggccagtaagggaaaaactcctcaagcatgctacaatattgaaaggttcaaaagcactgacaaagtgttgttttgcccccggtgcagcacataagactctgttccagtgaaatgctacattcaaagtgctgtccacctcagaagatcccagaggatgcaattctggctgtgctgggaagtgctaaagttccctccatatgtcactttggagaaggaagcagcaaagcagccatgttgattcctctctcaacctttggcatcatggacgatggtagcgtgtaaaatgtttgctctcttcatgaacctccatctcggagcttttaaattcatttaattcttttcttatggcagccttgtcagcaggggtcagtttggtccaaggtttgtcggctcgccggtcataatcttgagcatctgttacctctacatattcattaaacctcagaatcttcctggcaaggagttcagcgacagttggcctttgactgagctttctagtgagccgacgtttaatttctcgtttttctgcctgacgatcagcttcatttttaggttgcaatatattgcgttgttctagttcttctggtgttggtctttgactcagtcgccggatcagtgtgtttccaatctggtgccgtatttcattccactcctccttgcttttacaaggccaagaattcaggttcaactctggttcactgggtctgtggttcaacttcattgccagtgtgtctttcctcttcactttgttggcgagagcactctgatagctttcatcttcatcttcttcatctcggtactgaatgggaccttctgaatcagagtcgctctccttctcttcttcctcccgtagacactgtggtaatttaggaatgactgaggtaggtgtcatttcttcactgaatgtggatggacaggtttgctcctcttcttcttcatcgtctggaacttttagcatttcaatagtgatgggaagagacctggtccgacccagcgtactgctgtcctcagaaaagctgtcactgttttcaaaaagcaacgaatgagctctgtgagaaccctccagaataggagtcatgggaagtgggctggtgagggcctgctggattcgaatatgcagtgggagtggaggcagcctagagggtatatggggctccccaaagttctggtccagtatcctcttggggacttcctttttctgatcttcctgctggggaatctcctggtgtagatctaaggatggtggaaactcaatttctggcacaacttgaaaagtcttagcagggaatggaggggtgcgtggaggctctggaggtatatgagtaggcagtgggggggacggagagcgaggtgagatcattggtagtagttccgagcccatagaacacgtgctcttctctctttcatcacttggtgtttttgtggtgatggcagcagcagactccaaggtgggtactgaggttgatggaatgcctctcttaggtggtaagggtggggacggttttgataacaatgtaccactgtttattgcttgggacagttcagcaatgacagggttgctatttctgtgagctggtttagggggagggatagggggctgcttggcagggaccatatgagtgaggcttggggtagcagtagtgttagtgctggcaggagcagcaggcagagtcctgggtgctggggaaggggtgacagagagattaacagtctttgcaaggcttgtggcagcagtggtggcagcgggtgctgtggtgatggaggtggagatgatgaaccttgccgtgccgccagaggaagtggcatcctttgcttgcccttcacttgcttcatgagaagaggacaagggtcttttgggaggaagtaaaggtggtttgggtacattctcaggaacagactctgcttcagaattaggctggcttccagttgagcctagtcgtttctttaggtcctcttctggaatagctttcctaagacttgctaatcttactggctcttcctctacttggactggactagatgatctggcattccctatgggggtggtatggccattctttaacatggcatcgcttggctttcctggatcctcaccaccttgctcagggtcttccaacagaacccctcttttaaccagctcttctcttggctttcgcatagatattttccgttctaaaacttctgaagtctctttaaatttatcactacttttttttttcctccatttccagggcttgaagatcttgccaaagcctgagaacttgctcttccttttggtaggaggtgttgtgtctcctgcttccacactgtccaggaccatgcctggctctgtagtgggctggtctgcttccttgttccaaggttctctggagaagtcaaatggatcttccatgccactattaaccagtttagggaggtgagatactgttttgtgcactgtgattgtaacttctgcaatgtggagtacaacagcaaaactagcacaattttcttttttcgtcttcacaatttcacagatagaaaattcattccagatctccgccgccgcctcctcagcctccacagcagcctctcccggaaatcctacctggcccgttggccgccaggcagcagccg

SEQ ID NO: 12650 - RNA, 3257 nt, Homo sapiens
  source 1..3257: mol_type = other RNA
gatctcactttgttgcccaggctggagtgcagtggcacaaacatggctcactgcagctttgaactctctagctcaagtgatccgcctccctcagcctcctgagtagctgggactatcagtgtgcaccaccacgcctggctaatcttttttttttttttgtagagacagggtctcattatgttgctcaggctcagactcttttatgtatgtgatcatttaacacttaggaacaagaaatccatcccgttgcactgattcaacatctgagattcagaaattatctgctgttttggaagactacaagatgaaccaggcaatctcttcagtttctgttgtcagggaactttacttagattttctgaaagagccactgagcagttttgagtcatttgcctcttcaagagattgttcctatttcagaggtctttcatttttcctttttgtattttgactagagtttatctgatctaaatacatgttttctcacagaaggcacaaaatgcttcataaggagtcattttgtcctttctttcttctgatgaacctgccctctcctcctctgcaaggtttcacagtgatgtgcaacgtccactctccatgctaagtgacagtgactgtaatttgctgagagagcagtgaccaaaccattggctccttcagaggctggttatttcaaccatctggagaaaaatggaggctcctaatgcagagtgaggaccttaagttgtctagggcaaagactcatttgttcattcattcattaattcacccatgcactcattggacaaacttgaatagggtactatgccccaggggtgtgaggaaggataaactatggagtggcccattcacaacaactgcacatcagggcagagcagaagtgctctaacagcaccagctccaggtcacccaaggatgaccaggaaggctccaggcagatcaagcattcgagctgggcttggaggaatatccttgattctggaggtggagttgggaagcagccatcccagcaaagaacatggcagcagagaagctgaagacaccaggatgaggagtggaccagtcggaatccttactcctggatgtgctgggggacagatggactcctccaaagagctgaatgctgggctgaacagttttagtccttaggagctactgactgttgtcaacagaaggtgacagcgcctaccctggcagctgcccatggggagtgatgagccggggaggaagatcctcaagacagtgaggacagaatgcaatatccctggcgtgttctaggggaaggcagtgaaggctaaaacttgggcaccggcagggagaataggtgggacaggagagccgtggaagacaggatgaagccagaaggagagctggagaaggacctgaggtgggggtgaagatggtgggagtgtcaaggggattctcacatttttatttttaactttaaaaagtttttaaacagaaacaaggtcttgccatcttgcccaggctggtctcgaattcctgggctaaagtgatcctcctgtctcagtctctcaaagtgctgggattacaggcatgagccaccatgcccacctgatcctcacattcttttttttttttttttttctgatacagagtcttgctctgccgcccaggctggagtgcagtggcatgatcttggctcactgcaacctccgcctccgaggttcaagagattctcctgcctcggcctcccaagtagctgggattacaggtgtgcaccaccacacctggctaatttttgtatttttagtagagacagggtttcaccatgttggccaggctgatctggaactcctgaccttgagtgatctgcccacctctgcctcccaaagtgctgggattacaggcatgagccaccatacctgactgattctcagattctgaaatgacagttaagcccaggactcaagccagggacagaagcagataacctggttttggtgagaaggttatgcacttgcttctgaaaatgttgatgatgagactaagtcttatagtttcttgtgcacctcccttggtgcctagaagaaaggttaaaacaggatacattacagagggactatcttgagagaggagttacctgggcacagcccaggggcccttgggagtgacatgcaagggcagcactggcttgccttatttggttctcccgctctttcttctttcccttgtaaaagtaactgaagcttaaaggtgaaaatgacttaaataatagaaaccatgttagccttactccccttccccattagccacaaattggtggcgatcaccattttgtgcaccgagcctgggtctcacgcttgcaagtccttgggctcatctggagtcagcttcatcagtttgtccacacagagcaggatgagggtgaggaaccagaggctccagccaacagctgccgcgatccagccgtactcgtccactcctgtgcggcagcaccgggctgcttgtgggcagaagtccacgttgaggcactgctccagggtcccagggtctgggtggtgagcggtcaagcttgagctgttgctgctgcttgctgccgagcaagccgagtggagggaggcaaaggccaggctgaggatcagggtggcccgggtggcagcggggaggcgctgcatgctggaggctgtgctgagtgcccggtgcaggtgagccggtcctgcggagttgtgccgagtgcctgctgcaggtgagtcgactcccacctgcaggagctggaaagcaactctgccagaggtgaacttatgctgggtgtttgggggaaacaccatggggtggagcaaaggaaacttggcctgtcacaccttctctcacctctctagaagggaagccaaaccgttggctgaggaaggaagggaggggcaagctgtgcccttctcccctgagcgcaaatattgtccttattgagaaacaaggggaggacaagagagatctgtgtcatgctggttcctgggacatgagtttgctgcctctcccatctgcaggtgtagcatggatgctcaattccatttgggccaatattcactgagcacccactatgctgaagttgggagatacctgctgtcgaagtgcgttaattacaaacacgcatcattcaaccccagaaccgtgtttgaggaatggcttgggaggataaagcactgtgggtttcaacagtggaggccacatctgctgatgggatgcttcaagaagaaaatggcatttgaggttgggcatgggggctcaccctgtagtcc

SEQ ID NO: 12651 - RNA, 2753 nt, Homo sapiens
  source 1..2753: mol_type = other RNA
gatctcactttgttgcccaggctggagtgcagtggcacaaacatggctcactgcagctttgaactctctagctcaagtgatccgcctccctcagcctcctgagtagctgggactatcagtgtgcaccaccacgcctggctaatcttttttttttttttgtagagacagggtctcattatgttgctcaggctcagactcttttatgtatgtgatcatttaacacttaggaacaagaaatccatcccgttgcactgattcaacatctgagattcagaaattatctgctgttttggaagactacaagatgaaccaggcaatctcttcagtttctgttgtcagggaactttacttagattttctgaaagagccactgagcagttttgagtcatttgcctcttcaagagattgttcctatttcagaggtctttcatttttcctttttgtattttgactagagtttatctgatctaaatacatgttttctcacagaaggcacaaaatgcttcataaggagtcattttgtcctttctttcttctgatgaacctgccctctcctcctctgcaaggtttcacagtgatgtgcaacgtccactctccatgctaagtgacagtgactgtaatttgctgagagagcagtgaccaaaccattggctccttcagaggctggttatttcaaccatctggagaaaaatggaggctcctaatgcagagtgaggaccttaagttgtctagggcaaagactcatttgttcattcattcattaattcacccatgcactcattggacaaacttgaatagggtactatgccccaggggtgtgaggaaggataaactatggagtggcccattcacaacaactgcacatcagggcagagcagaagtgctctaacagcaccagctccaggtcacccaaggatgaccaggaaggctccaggcagatcaagcattcgagctgggcttggaggaatatccttgattctggaggtggagttgggaagcagccatcccagcaaagaacatggcagcagagaagctgaagacaccaggatgaggagtggaccagtcggaatccttactcctggatgtgctgggggacagatggactcctccaaagagctgaatgctgggctgaacagttttagtccttaggagctactgactgttgtcaacagaaggtgacagcgcctaccctggcagctgcccatggggagtgatgagccggggaggaagatcctcaagacagtgaggacagaatgcaatatccctggcgtgttctaggggaaggcagtgaaggctaaaacttgggcaccggcagggagaataggtgggacaggagagccgtggaagacaggatgaagccagaaggagagctggagaaggacctgaggtgggggtgaagatggtgggagtgtcaaggggattctcacatttttatttttaactttaaaaagtttttaaacagaaacaaggtcttgccatcttgcccaggctggtctcgaattcctgggctaaagtgatcctcctgtctcagtctctcaaagtgctgggattacaggcatgagccaccatgcccacctgatcctcacattcttttttttttttttttttctgatacagagtcttgctctgccgcccaggctggagtgcagtggcatgatcttggctcactgcaacctccgcctccgaggttcaagagattctcctgcctcggcctcccaagtagctgggattacaggtgtgcaccaccacacctggctaatttttgtatttttagtagagacagggtttcaccatgttggccaggctgatctggaactcctgaccttgagtgatctgcccacctctgcctcccaaagtgctgggattacaggcatgagccaccatacctgactgattctcagattctgaaatgacagttaagcccaggactcaagccagggacagaagcagataacctggttttggtgagaaggttatgcacttgcttctgaaaatgttgatgatgagactaagtcttatagtttcttgtgcacctcccttggtgcctagaagaaaggttaaaacaggatacattacagagggactatcttgagagaggagttacctgggcacagcccaggggcccttgggagtgacatgcaagggcagcactggcttgccttatttggttctcccgctctttcttctttcccttgtaaaagtaactgaagcttaaaggtgaaaatgacttaaataatagaaaccatgttagccttactccccttccccattagccacaaattggtggcgatcaccattttgtgcaccgagcctgggtctcacgcttgcaagtccttgggctcatctggagtcagcttcatcagtttgtccacacagagcaggatgagggtgaggaaccagaggctccagccaacagctgccgcgatccagccgtactcgtccactcctgtgcggcagcaccgggctgcttgtgggcagaagtccacgttgaggcactgctccagggtcccagggtctgggtggtgagcggtcaagcttgagctgttgctgctgcttgcttctgccgagcaagccgagtggagggaggcaaaggccaggctgaggatcagggtggcccgggtggcagcggggaggcgctgcatgctggaggctgtgctgagtgcccggtgcaggtgagccggtcctgcggagttgtgccgagtgcctgctgcaggtgagtcgactcccacctgcaggagctggaaagcaactct

SEQ ID NO: 12652 - RNA, 16239 nt, Homo sapiens
  source 1..16239: mol_type = other RNA
gatctcactttgttgcccaggctggagtgcagtggcacagtcatggctcactataacctcaaactcctgggctcaggcaatcctctgcctcatcttcccaagtagctgggactacaggtgtctaccaccatgcccggctaattttataaaattttttatagagacgggggtcttgctgtgttgctcaggtcttgaactcctggcctcaagtgcacctcctgccttggcctcccaaaacactgggattacagatgcaggccactgtacctggcccccatatttattaatcacattttattcattcattcatttaactttcctgtgaagttttgcaaatggcttcctcaattcccccttgttaagctttttttccttctcaaaccatgcttatatcctttctggttccagccacatattttgggtcagacagtcctagcactgtacttttaatatcacctggagtgacttcagagacttctttgaagccacaagaccatctggttcaataccaatattttgaaatctaatgactcactattctagaacattctcaacattaagtttcttaaagatggcttaaatactttttaaatttaaataaatgtacagaaaacaaaaatcttttcatttaaaacctaccaaatatagccacacatggtagggcatacctatagtcccagttactcaggaggctgaggcaggaggattacttgagccaaggagttcagggctgcagtgcactatgattgtgcctgcaaaaaggcactgcactccagcgtcggccacagagaaagacctagttttttgtttttgtttttgtttttgagacagagtcttgttctgtcgcccaggctggaatgcagtctggagtgcagtggctcattgcaacctccacctcctgggttcaagcaattctcctgcctcagcctcctgagtagctgggattacaggggcacaccaccacgcccaactaacttttgtatttttagtagagatggagtttcgccatgttggccaggttggtctcaaactcctgggctcaagtgattcacctaccttggcctcccaaagtgctgggattacaggcgtgagccactgcatccagccataagactcagtttcttttcttttttttttttggagatggagttttgctcttttgtccaggctggagtgaagtggtgcgaccatggttcactgcaacctctaccctcccggttcaagcaattctcctgcctcagcctcccaagtagctgggattataggcacccactactacgcccagctaatttttgtatttttagtagagacgaggtttcgccatgttggctaggctggtctcaaactcctgacctcaggtgatccacccgcttcggccttgcaaagtgctgagattacaggcatgagtcaccacgcctggccggcaagaccctgtttctaaaaaacaaaataaaaaataaatcttccaactatttataatatgatctctgttcatctttactgttataaacattcctcaggtacttgaaaggagtgtgtgttctaggcttgttgagtacagataacctattagacaaggttactaacttccctgctgcctgctctatcacctctattagaagtatttaaaatctcaattttccttttaattttcatgctgttttctgggttgttcatgattgctatgtttgtggtggattgttctttaaaaaaaaaaatcttgatcctattaacactttttgcctcaaattctattttgtctgctattgatattactacccaaaatccccgcaccccgcccttttttttgagacaggatctcactctgtcactcaagctggagtgcagttcaccatcacggtggctcattgcagcctcgacctccctgggcttgggtgatcctcccacctcagcctcccgagtagctgggatcacaggcacataccaccatacctggctaatttttgtactttttatagagacggggattcaccatgttggccaggctggtcttaaactcctgatctcaagtgatccgcccaccttggcctcccaaagtgctgggattataggcatgagccaccacacccagccggcagcaaactgtttatggactggtactggggcccagaccctaccttgagtggtactgggctagaggacttattaattgcatgatctaggagtagttcataaattctgtgatggtcattctttgggtgaactccatttctagcagattctagataagcagcatgacttcctctgattctctgacacctgagggtggggaaattcagactgtcccacttgggttgtgcgtcttcacgctggggaagagggtgaggccaaagttgtgttgggagataaataatgaaattcaagaactccatggtaacagcccttgtctttcctctctggggccacacagtgcagtgtggggagaggagtggacagaaggaatgtcagcatttccttggcaaaatctcttgcgtttcagaacagcagtgagattttggaggtatgagagagtcacaggtgtgacattcctgtgaggaatgctatttgagtacaagcagtggatgtcctcatgatgttatgatttcagaagaatagcactgtgcttggctgaaaagttctgcattcaataactccatgccaataagcagccatttcctcccagcacacagttgctcaccaatgtccatggtcctatggcactgggaggcctctgatgcagctgtctcccactatggtcttaggaaattcctggaacgttattagagtgagtttttcctagatctgcttactgaatacctgttgaactttcacactgatggccagttccaagacttaagcatgaccttgcgaccattggtgatagtgctttcttgatctgctgaatcaaattgaagcagaactgggggtactactaggaatgaggggtgactagggatggggctggggcgaggggtatattgggtaactgaggatgaccagtgtcagagagcacaaagatgatggtgaagggcaggtagaccacctcccacttggtgggaaagtctgttcctggctggaactggttcattcattccaagccagcaacagctccaggtttggacgccatttatgaatctacatgccaccagaccagtccctgtcttccacacaccccactctctggagtctggaaaaatggcgggggtggggctagctactagtttttgtttttttttttctttttgagacacagtttcattctgtcatccaggctggagtgcagtggcatgatctcagctcactgcaacctccgcctcccaggttcaagcgattctcgtgccttagctttcagagtagctgggactacaggtgcacaccatcacagctgactaatttttcttttctttttttttttttgagacggagtctcactctgtctcccaggctggagtgcagtgatgtgatctcagctcactgcaacctacgtctccagggttcatgtgagtttcctgcctcagcctcctgagtgagtagctgggattacaggcgcctgccaccacgtccagctaatttttgtatttttagtagagattgggtttcaccatgttggccaggctggtctccaactcctgacctcaagtgatccacctgcctcggcctcccaaatcgctgggattacaggcgtgagtcatcatgcctggccttttttttttttttgtgagacagagttttgctcttgtcacccaggctggagtgtaatggcatgatctcggctcactgaaacctctgccaggcacacgtcaccatgcccggctaatttttgtatttttggtagaaacggggtttcaccatgttggccaggctggtctccaactcctgacctcaagtgatcctcctgccttggcctcccaaagtgctgggattacaggtgttagctaccaagtctggcctttttttttttttttttttttttttttttttgagacagagtttcgctcttgtcacccaggctggagtgtaatagtgtgattccagcttactgcaacctctgcctctcgggttcaagccattctcctgcctcagcctcctgagcagctgggattacaggcacacgccagcatgcctggctaatttttatatttttagtagagacggggtttcaccatgttggccaggctggtctcgaactcctgacctcaggtgatccatctgcctcagcctcccaaactgctgggatgacaggcgtgagccaccacgccaggccctatttttatttttaaccagtgctgtagtttgaatatttgtctcctccaaaactcatctggaaacatccccaatgtggcaatattgagagatggcgcctttaaaaggtgactgggtcatgaaggctctgcccagtgagactggtgcctttataagaagaggaagagagacctgagctaccatgctcaagtccctcaccacgtgaggccctctgccaccttgggtctctgcagagagttcccaggaacaagaagtctctcaccagatgtggaccctgtaccttggacttctcagtctccactattgtaagaaataaattccttttctttataaatgacccagtttcaggtattctgttctatgcaacacaaaatggactaagacaacgagtacgcttagttgttgcttcctgagttccaaagtccgacagacagagcaggtcctccattcttgcccctttttaccccaaatgctcattggcattcttgcagctacgagtaataattaaaagtggctaagccaggctggcatggttgctcacgcctgtaatatcagcactttgggaggctgaggcaggaggatcacttgaacccaggagtgagaccagccagggcaacatagcaacaccctgtctctaattattattatttttttaagtgagtaagccaaataggggtttacttttcatctagaacaagaagacgtgttggccaggctggtctcaaactactgggctcaagtgatccacccacctcagcctcccaaagtgttgggattatgcgtgagccaccgcacctggccacaagacccaatttcttttattttatctttttttttttttttttaagagatagggcatctaacggcattgttttagctgctcaacacttttttttttttgcttatttttgtttgttttgtttgtttttgagacagggtctccctctgttgcccagcatatagtgcagtggcatgatcatggctcactgcagcctcaacctcccaggatcaggcaatcctcctgcttcagcttcctgagtagctgagaccacaggtgcacaccaatatacctaatttttttttttttgagatggagtttcactcttgttgcccaggctggagtgcaatggcgtggtctcagctcactgcaacctctgcctccctggttcaagcgattctcctgtctcagcctgccgagtagctggggttacaggcataagccactacgcccagctaattttgtatttttagtagagacagggtttctccatgttggtcaggctggtctcgaactcctgacctcaggtgatccacccacctcagccttccaaagtgctgagattgcaggtgtgaaccactacgcctggccacctgactaatttttaagttattcacagagaacaggttttgcaatgttgcccaggctggtctcaaactcctgggctcaaatgatcctcctccctcggcctcccaaagtgctggggttacaggtgtgccactgtgcctggtcggctcaccactttcagatctggctctcttcacctctcttttatagtcataagctgattagcacaattctagacatccgcagctacatttaaggcaggaaggaggtggtaatagacactaccagccacatctgtcccttttaatcaggataccctagaaatcctcagcagactttgaattatgtgccattggtgaaatgtcatatgatcatccctctacaaggcaacgaggtaaaaagagaatttagtatttctagcctctagagtggagatgaacaaagaataggaatgggcatttgcttaggaaaccaactgtgccttacaacatttttgcacttttttctgtaacattttgtgttaaatcatataaaaatgctgatcctaacaaatatggtcaatgagtcacaccataattctctaagaactccagtccaaaaaggttaatcttgcttttaaactccaggcgcggtgtttcacagctgtaattttagcacttcgggaggcagagcaagaggatcacttgaggccaggagttggagaccagcctggcaacatagcaagaccccgtctctacaaaaaataaaattatctgggcctgttggtgcacacctgtagtcccagctactcaggaggctgaggtgggaggatcacttgagcctaggaattcgaggctgcagtgagctgtgattgcaccactgcactccagcctgggtgacagagggagaacctatctccaaaacaaaacaaaataaaaacaaaacaaaactccaagcagagaaagacttgacgagtcggatgagtctgatgattcctaaaggaaatcctttttgagattccaggagattccatctcctcaacagagtaattgattttgagcctcccacctcctgaattaaggcccacccatccctatcctgcactgaactgtagactcttttttacttccttacaaaagtttattcttaaatgtacaacagactccaagacgacactttattgtagctataggtggcaaaagatgttatggcagagaatccagatgtttaaataggaatggggtcaagggtcaccgccccaagcacggataacaaaatttattttttgccagatttctttaattccacctgtgactggtgagggctggtggcggggtggctttcacttttagctcctctttttgtttctgcttgaacgtcccatcttccttacccacccccttgacctgcttcttgagctttctcagggcttcttgccacctttgcagctgtacatggcacctgccatagggctctaattttaaactgagaaattgagaaaacaggaaactgactctttttggggggagagtaagacaaacaggaaaaggaaaatgaagacgtggttgatacagatcgttggatttcaaaaggaaaagtctacggataaccgaaaaaaataaatatttagaaatgcatagtcttggctggttaaataagtatccatgcttgttcttgtggcatagtagttacgagacatttttagttaaatggaaaaatgtgaattactatagtttgagtgatatgctgctttccaaattaaaagcagcataacaaaaacattcccctaatactcataaataattcattgaattggcaataattcacctcctaatgacttcatatgaagtataaagtaacttcgatacatcagaagaaatcctatcttctaatataagaaagtaatatgattacattaaatgcgtctcatataagttataaaaatggtatctatgagtaaagaaatgcttgtgaacaaaaaaattgatcttataaaggtcaaacaggccaggcgtggtggctcacacctgtaatcccagcactttgggaggctgaggtgggcggagtacctgaggtcaggagttcaagaccagcctggccaacatggtgataccctgtctctacaaaaatacaaaaaattagctgggcatgatggtgggtgcctgtaatctcagctactcgggaggcagaggcgggagaatcgcttgaacccgggaggcggaggttgcagtgaactgagattgagccacaacaaccaagcctgggagacagaggaaactctgtctcaaaaaataaaaaataaaaattaaaattaaaaaaaaggtcaaacaaaccaaacccttctgattaatttattcaatctacttttattataagcaaatgagaaattataattttaatctgaaaaagcagaatcaggggattttggagctggacagtcccctggaaattatttggatcaaagccctcattttataggtgaagaaactgagaagtaagatttgagcaagctgcccaaaggctttgccaaaggctataccagtgaatggcagagtctggactggaagtcccagtgctgccgtccaggtgagacctgttccactgcatgctactagctcccgggctgagaccggacttttgcttggcaggtttctttctttcgaaactattaattattgtattttttgtagagacagggttttgccatgatgcccaggctggtcttgaactcctgagctcaagagatccacccagcttggcctctcaaaaatgttgggattacaggcataagccacagtgcccggcccattttcctcccacctctttgttccttctctgtttcttttgcagcattatgttctatcattgtataccagagttcctcaacttcagttatagtctgttcttgctttatgctatcttcttcagcaagctcatcttggtctgttttcctccttatcaggcataccccagaaactcctgttttatctccacctcaactaaacattttcctgagttctgggcctctataaactaattatttgattaacatcttttttttttttttctgagatagagtctctctctgtcacccaggctggagtgcagtggtgcaatctcagatcactgcagcttctgcctcccagattcaagcgattctcctgcctcagcctcctaagtagctgggattataggcatgcaccaccgcacacagctaatttttgtacttttagtagagacggggtttcaccatgttggtcaggctggtctcaaactcctgatctgaagtgatctgactgcctcagcttcccaaagtgctgggattacaagcctgagccaccatgcctggccaacatctttaattggatatctcagtatcaagaaggcccataatattcctctgcctcatccctctcctcagtcctcttcttgtgtttcctagttcagagaatggcaccattctctatcaagctgcgcaaatcagacatgtgtgattttttgttgttgttgagacagggactcactctgtcacccaggctagagtgcagtggcgtgatcatggcgcactgaagcctcaaactcctgggctcaggagatcctcccgcctcagcctcctgagtagctgggaccacaggcccacaccaccatgcccagctaattttgtattctttgtagagatggggtttcatcatgtttgcccaggctggtctcgaactcctggactcaagcaatccacccacctcagcctcccaaagtgctgggattacaggcatgagccactgtgcccagctgaagtgtgatccttaacttcaccccttctcatgccctccatttccaatccatctccagtccagttgactccagctactcaattatttccacttatctcattccactacctttgaagctaccaccatctctaactacagtcatctcccaactaactggtctcctggcatctctctggttctcctccactaatttcaaaaaaagaaatttactgtgacagtgctcacaacactcccccttgctcttactaaagatgcttaccatagcctccaggtattgtatggcctgaggtctatctacatttccaggtgcaggacacaccatgtctccccactcccaaatttagtctccagactccatcctttttacagttctttaaaagcatcacaattcctccaaccactaggcatttgtatgtgctattccctctttccagaatgcaataccctccctctgcctagctagctaacttctatgtatctatgactgcagctcaaactttcctcatggactccctccacaagtgccaagcctgggccagattcttttgttatgtgctcacagaacgatgttccctttagcattcattgagtttgctgtttaattattcttgtcttgtttttgtttaattagtcctatctctaatactagacaaatgttccttaagatcacaggaaatataggactgtctctacataaaaactgttttatatccataatgcctaggacagtacctggcacacagtatatgctcaataaatttttgttgaatgaatgcaattatcattatattcctgatattagcaggtataatccagtttaagtttgggaacagaaagacaaaacggaccacatctaataaatccggtctcctttcttttattatttatttatttgagacagttttgctcttgttgcccaggctgcagtgcaatggcatgatcttggctcactgaaacctccgcctcccaagttcaagggattctccagcctcagcctcccaagtagctgggattacaggcatccaccaccacgcccagctaatttttttgtatttttagtagagatggggtttcaccatgttggccaggctggtctcgaactcctgacctcaggtgatccacccacctcagcctcccaaagtgttgggattacaggcgtgagccaccgtgcccggccaaggtctcctttcttttaatcaaactctcacctttggccattctgcagtcattcacccgacagtatttactgacggagtgaatacagagtgcttgattaatgttgctgctttgttattattattattattattgagatggagtcttgctctgttgcccaggctggagtgcagtggcgtgatctcggctcactgcaacctccgcctcccgggttcaagccattctcctgcctcagcctcccaagtagctgggactacaggcatgcaacaccacacctggctaatttttgtatttttagtagagacaaggtttcaccatattggccaggctggtcttgaactcctgacctcaggtgatctgcccacctcagcttcccaaagtgctgggattacaggcgtgagccaccatacccaacctaatgtttctgctttgaaatacaatttcaaaaagtcattaataggttgaaaacagcaagattttaaaagtattttaaaaagtgaaacagaagaatgcttacttcatttcacagagatagatttctcctttatgttatttctaaaaggagatggaattttgtttcattcatttctgcttatttggacaggccaaatatgaacagctgaacacgtcagcgttaccatgcatatgttacacagatgccatccttcttccatcagctctcatatgcaatacagaagtaaaaagaggttctctttatttttaaaaggtaaaaattgaaattcagtcacttaacacagaataaacaataattacaattacactggtaacaaaggacagcaagcatgttttctttgaaagcactgtatctggtttgtctccgtgcttggtcctagtatctggcatattttccccagagttttcttttcagtgggatgattatcttcggggcaaaaaagtttatcagactcaagttttagcagtacttattttattcatttatatacatgtaaccccatcctgtcttactccaatcttcttactgccttcctactgacacatatattatataacaccctccccaagttctatttacggttaaaaatttctttttttttttctttttttgagacagagtttcactctcgtcacccaggctggtgtgcaatggcgcagtctcggctcactgcaacctccgactccctggttcaagtgattctcctgtctcagcctcccgagtagctggaattacaggcgcccgccaccatgcccagctaatttttgtatttttagtagagacagtgtttcgccatgttggccaggctggtctcaaactcctgacctcaggtgatccacccgccttggcctctcaaagtgctgggattataggcgtaagccactgcgcccagcctacagttacgaatttctaaatggcacaaataaactcagctgttctcagtgcagacgtcaaatcctcactgtgctgaaacattttcctcagcttttgggaaataattacaatttaaacatacacagagaatgtttcttagacaaacataatacccgaggcttatctggtaaaaactaattgctctgtccttagcacaaaaaatatatatctttgtaaaatgagaagaaccaaagaatatttaaaacaaagaaggaagccacacgtactaattacacaagagactgactgacaaactggaattctccaaaacagattttcagcgaggcttctcatttcagagtccaggaaaaaaaaatcctaaaaaccccaaaggtatattatatgtgtgtatatatatttttattgtgttaaaaaacacaaaacataaaatttactgtcttatcaaaaggtatattttgtcgctcttccctttttttttttttttttttcccgagacagagtccagtctgtcgcccaggctgaagtgcagtggcatgatctcggctcactgcaacctgcatcttctgggctcaagcaatcctcccacctcagcctcctgagtagatggagctacaggcacgtgccactaggcccggctaatttttgtattttttgcagacagggttttgccatgttgcccgggctggtctttgttctcctaagagttgttttctccatgaaagttgataaataacatttagaaaatgaattattacaagagtaatgatatgtctcaatttattatatgaaattatcaacaactgcttttaatattcagatgtcaagaagatgaaaagcagaaatacattttgcaaacatgtagcactccataaatggaaatcatgtatttcctctaatatcccaatttttctatattgggatcttatatggctgtttctatatggctattttgtcccaacttgctgtacaagaattttccccagccaccttagaaaggttggatgtagttcactccaagtttgcagttcactccaagtgtttcagtaccacagaaagctccatggaagcctcaaatgtacgggctaggcaatagaagcagggaggtaggattaagaaattactggccaggtgtggtggctcaggcctgtaatcccagcacttcgagaggctgaggcagacagatggcttgagctcaagagtttgagatcagcctgagcaacatggcaaaactctgtctctacaaaaaatataaaaatcagccaggtatgttggtgtgcacctgtagtcccagctactggggaggttgaggcaggaggattgcttgagcccaggaggctgaggctgcagtgagccatgattgtgccactgcattccagcctggtcgactgtaagacaaaaaataagaaaataaaaaatttaccaatataaaatgctcaaacagctaacaaacatgttcaattccatttatagtcttttctttgagccatttaaacatagggctattttttttttttttttttgagatggagtttcactcttgttgcccaggctggagagcaatggcatgatctcggctcaccacaacctctgcctcctgggttcaagcgattctcctgcctcagcctcccgagcagctgggattacaggcatgtgccaccatgcctggctaattttgtatttttagtagagacgggattcctccatgttggtcagactggtcttgaactcccaacctcaggtgatctgcctgcctcaaccttccaaagtgctgggattacaggtgtgagccactgagattggctgccgttttgttttttaactccatatagtttctatagttcactgaaaactcaaagagatgacctataaatgtatgaataatgtatgatttcttacatcaattttctactagaaaaaaatcatacttttagaattggattttgtcttacagtcatctttattatactttataaatgagatttcatttatataaatcaggaagctaaactaaaatagaaacactagatttaaattctgatttgaatactctgatcaaaataacaaatctcacactgggaaaccatctatcagcaagcagagagctactgtgtgtccttccttagaagagtttgaacaccgagaacccacagcatatttgcagtacagtaacagcaattcctttgtcattatcacagaactttaattttcatatactttgctgggaccaaccaaaccatcccatatatataaccatatccatatatatatatatatatatcccacatatatatgggatggtatatatatacacatgtatatgtatgtgtgtgtgtatatatgtgtatatatgtatacacacacacacacacacatatatatatatatacacacacacacatatatatatggagagagagagagagacagtgtcttgctctgtcgcccaggctggagtgcagtggtacgatcttggctcattgcaacctccgcctcccaggctcaagcgattctcatgtctcagtctcccaagtagctgggattacaggtgtgcaccaccacaccaggctaaccattccatacattttatacaatcatttttaaaaagaagcatgaaccatttcggttttagagaattaagtttttttaaaaaagagactcttaaaaaaaagtcattatatgaataaaatctgctttgtgttaattccgacaaatcattccatcattgagtctgtcaccaattttttttttttgaaatggagtttcgctcttgttgcccaggctggagtgcaatggtacgatctcggctcactgcaaccgccgcctcccgggttcaagtgattctcctgcctcagcctcccgagtagctgggattacaggcatgcgccaccacgcctggctaattttgtattattagttgagacagggtttctccatgttggtcaggctggtctcgaactcctgacctcaagtgatccgctggccttggcctcccaaagtgctgggattacaggcgtgagccaccgtgcctggcccaattttttttttttaataacttgcacacttaacaatattttttatcttcttgggacaacattcttttctccacaaaaacccaattaaggacgttgtgccagtttactcctacttccttcctgttcactgagcttaaagtgggtataggcgagaatgccaaataatgtacataaaatgccaagggcctgattaatggacagtggatccttaaataaaacatatcctccgaataaagtaatgcagaacttgaagtgtccgaacatgttataggtgacaggtgaagtgttcccaatgatccaataaattgataagttcaccatgaaagctattactccagatagcagcaccataagcaaagcagaaactgaccagggaccaaatattcctccttctccaaacactggctcaaagaagggcacagcaaccagcaacatggcagatgacatcggagcctggtagtacagcagctgcattgagttcacttgtaattcatgctgtttggctcctacccaaaacaggtaggtatttggtgagcatcacacacccaagtttctctgtctcctttcttctcttcaccttgagtcagacaacttatgcaattatgctttcttcccaacagtctattgtctctatactgtattttctaaaccttggaatacagcttcaaaatttatgaaatcagcgtgagctggattctggtggagaaggttttctggtagcagaaggtctggatggctatgatcaccggcgtggtcatggccttggccagctgataggtgcctatggtgttgttctgcagagaaaggttagtgaagaccacaaagccacagaagctgagggccaggaggaggagcctggagggcggcagacttttgggggcaaagatgtccagcttctggcagatatacaagcccagccaggtgaccacgaagtgcaccagggtcaggctcatgttggggaagccgtggtacacataaatccatttgttgaggaacacaatgcagatggacaccagcaggttgaacaggagcccggcggcgattcgccagtggccccgcactcggtccaccagcaatgccatgatccccgcgaagctggggccgtctagcctcggaaggggcgccgggcctgtctccggctgcccttctactccaccgccgcgtcctcgcagacgccgacctcaccgtctgacccaggagtggcatgcacagatcaaccccgggcgagtagcactcttaacagaggacacacaccccgccgccgccctgtaagccagctaggac

SEQ ID NO: 12653 - RNA, 16242 nt, Homo sapiens
  source 1..16242: mol_type = other RNA
gatctcactttgttgcccaggctggagtgcagtggcacagtcatggctcactataacctcaaactcctgggctcaggcaatcctctgcctcatcttcccaagtagctgggactacaggtgtctaccaccatgcccggctaattttataaaattttttatagagacgggggtcttgctgtgttgctcaggtcttgaactcctggcctcaagtgcacctcctgccttggcctcccaaaacactgggattacagatgcaggccactgtacctggcccccatatttattaatcacattttattcattcattcatttaactttcctgtgaagttttgcaaatggcttcctcaattcccccttgttaagctttttttccttctcaaaccatgcttatatcctttctggttccagccacatattttgggtcagacagtcctagcactgtacttttaatatcacctggagtgacttcagagacttctttgaagccacaagaccatctggttcaataccaatattttgaaatctaatgactcactattctagaacattctcaacattaagtttcttaaagatggcttaaatactttttaaatttaaataaatgtacagaaaacaaaaatcttttcatttaaaacctaccaaatatagccacacatggtagggcatacctatagtcccagttactcaggaggctgaggcaggaggattacttgagccaaggagttcagggctgcagtgcactatgattgtgcctgcaaaaaggcactgcactccagcgtcggccacagagaaagacctagttttttgtttttgtttttgtttttgagacagagtcttgttctgtcgcccaggctggaatgcagtctggagtgcagtggctcattgcaacctccacctcctgggttcaagcaattctcctgcctcagcctcctgagtagctgggattacaggggcacaccaccacgcccaactaacttttgtatttttagtagagatggagtttcgccatgttggccaggttggtctcaaactcctgggctcaagtgattcacctaccttggcctcccaaagtgctgggattacaggcgtgagccactgcatccagccataagactcagtttcttttcttttttttttttggagatggagttttgctcttttgtccaggctggagtgaagtggtgcgaccatggttcactgcaacctctaccctcccggttcaagcaattctcctgcctcagcctcccaagtagctgggattataggcacccactactacgcccagctaatttttgtatttttagtagagacgaggtttcgccatgttggctaggctggtctcaaactcctgacctcaggtgatccacccgcttcggccttgcaaagtgctgagattacaggcatgagtcaccacgcctggccggcaagaccctgtttctaaaaaacaaaataaaaaataaatcttccaactatttataatatgatctctgttcatctttactgttataaacattcctcaggtacttgaaaggagtgtgtgttctaggcttgttgagtacagataacctattagacaaggttactaacttccctgctgcctgctctatcacctctattagaagtatttaaaatctcaattttccttttaattttcatgctgttttctgggttgttcatgattgctatgtttgtggtggattgttctttaaaaaaaaaaatcttgatcctattaacactttttgcctcaaattctattttgtctgctattgatattactacccaaaatccccgcaccccgcccttttttttgagacaggatctcactctgtcactcaagctggagtgcagttcaccatcacggtggctcattgcagcctcgacctccctgggcttgggtgatcctcccacctcagcctcccgagtagctgggatcacaggcacataccaccatacctggctaatttttgtactttttatagagacggggattcaccatgttggccaggctggtcttaaactcctgatctcaagtgatccgcccaccttggcctcccaaagtgctgggattataggcatgagccaccacacccagccggcagcaaactgtttatggactggtactggggcccagaccctaccttgagtggtactgggctagaggacttattaattgcatgatctaggagtagttcataaattctgtgatggtcattctttgggtgaactccatttctagcagattctagataagcagcatgacttcctctgattctctgacacctgagggtggggaaattcagactgtcccacttgggttgtgcgtcttcacgctggggaagagggtgaggccaaagttgtgttgggagataaataatgaaattcaagaactccatggtaacagcccttgtctttcctctctggggccacacagtgcagtgtggggagaggagtggacagaaggaatgtcagcatttccttggcaaaatctcttgcgtttcagaacagcagtgagattttggaggtatgagagagtcacaggtgtgacattcctgtgaggaatgctatttgagtacaagcagtggatgtcctcatgatgttatgatttcagaagaatagcactgtgcttggctgaaaagttctgcattcaataactccatgccaataagcagccatttcctcccagcacacagttgctcaccaatgtccatggtcctatggcactgggaggcctctgatgcagctgtctcccactatggtcttaggaaattcctggaacgttattagagtgagtttttcctagatctgcttactgaatacctgttgaactttcacactgatggccagttccaagacttaagcatgaccttgcgaccattggtgatagtgctttcttgatctgctgaatcaaattgaagcagaactgggggtactactaggaatgaggggtgactagggatggggctggggcgaggggtatattgggtaactgaggatgaccagtgtcagagagcacaaagatgatggtgaagggcaggtagaccacctcccacttggtgggaaagtctgttcctggctggaactggttcattcattccaagccagcaacagctccaggtttggacgccatttatgaatctacatgccaccagaccagtccctgtcttccacacaccccactctctggagtctggaaaaatggcgggggtggggctagctactagtttttgtttttttttttctttttgagacacagtttcattctgtcatccaggctggagtgcagtggcatgatctcagctcactgcaacctccgcctcccaggttcaagcgattctcgtgccttagctttcagagtagctgggactacaggtgcacaccatcacagctgactaatttttcttttctttttttttttttgagacggagtctcactctgtctcccaggctggagtgcagtgatgtgatctcagctcactgcaacctacgtctccagggttcatgtgagtttcctgcctcagcctcctgagtgagtagctgggattacaggcgcctgccaccacgtccagctaatttttgtatttttagtagagattgggtttcaccatgttggccaggctggtctccaactcctgacctcaagtgatccacctgcctcggcctcccaaatcgctgggattacaggcgtgagtcatcatgcctggccttttttttttttttgtgagacagagttttgctcttgtcacccaggctggagtgtaatggcatgatctcggctcactgaaacctctgccaggcacacgtcaccatgcccggctaatttttgtatttttggtagaaacggggtttcaccatgttggccaggctggtctccaactcctgacctcaagtgatcctcctgccttggcctcccaaagtgctgggattacaggtgttagctaccaagtctggcctttttttttttttttttttttttttttttttgagacagagtttcgctcttgtcacccaggctggagtgtaatagtgtgattccagcttactgcaacctctgcctctcgggttcaagccattctcctgcctcagcctcctgagcagctgggattacaggcacacgccagcatgcctggctaatttttatatttttagtagagacggggtttcaccatgttggccaggctggtctcgaactcctgacctcaggtgatccatctgcctcagcctcccaaactgctgggatgacaggcgtgagccaccacgccaggccctatttttatttttaaccagtgctgtagtttgaatatttgtctcctccaaaactcatctggaaacatccccaatgtggcaatattgagagatggcgcctttaaaaggtgactgggtcatgaaggctctgcccagtgagactggtgcctttataagaagaggaagagagacctgagctaccatgctcaagtccctcaccacgtgaggccctctgccaccttgggtctctgcagagagttcccaggaacaagaagtctctcaccagatgtggaccctgtaccttggacttctcagtctccactattgtaagaaataaattccttttctttataaatgacccagtttcaggtattctgttctatgcaacacaaaatggactaagacaacgagtacgcttagttgttgcttcctgagttccaaagtccgacagacagagcaggtcctccattcttgcccctttttaccccaaatgctcattggcattcttgcagctacgagtaataattaaaagtggctaagccaggctggcatggttgctcacgcctgtaatatcagcactttgggaggctgaggcaggaggatcacttgaacccaggagtgagaccagccagggcaacatagcaacaccctgtctctaattattattatttttttaagtgagtaagccaaataggggtttacttttcatctagaacaagaagacgtgttggccaggctggtctcaaactactgggctcaagtgatccacccacctcagcctcccaaagtgttgggattatgcgtgagccaccgcacctggccacaagacccaatttcttttattttatctttttttttttttttttaagagatagggcatctaacggcattgttttagctgctcaacacttttttttttttgcttatttttgtttgttttgtttgtttttgagacagggtctccctctgttgcccagcatatagtgcagtggcatgatcatggctcactgcagcctcaacctcccaggatcaggcaatcctcctgcttcagcttcctgagtagctgagaccacaggtgcacaccaatatacctaatttttttttttttgagatggagtttcactcttgttgcccaggctggagtgcaatggcgtggtctcagctcactgcaacctctgcctccctggttcaagcgattctcctgtctcagcctgccgagtagctggggttacaggcataagccactacgcccagctaattttgtatttttagtagagacagggtttctccatgttggtcaggctggtctcgaactcctgacctcaggtgatccacccacctcagccttccaaagtgctgagattgcaggtgtgaaccactacgcctggccacctgactaatttttaagttattcacagagaacaggttttgcaatgttgcccaggctggtctcaaactcctgggctcaaatgatcctcctccctcggcctcccaaagtgctggggttacaggtgtgccactgtgcctggtcggctcaccactttcagatctggctctcttcacctctcttttatagtcataagctgattagcacaattctagacatccgcagctacatttaaggcaggaaggaggtggtaatagacactaccagccacatctgtcccttttaatcaggataccctagaaatcctcagcagactttgaattatgtgccattggtgaaatgtcatatgatcatccctctacaaggcaacgaggtaaaaagagaatttagtatttctagcctctagagtggagatgaacaaagaataggaatgggcatttgcttaggaaaccaactgtgccttacaacatttttgcacttttttctgtaacattttgtgttaaatcatataaaaatgctgatcctaacaaatatggtcaatgagtcacaccataattctctaagaactccagtccaaaaaggttaatcttgcttttaaactccaggcgcggtgtttcacagctgtaattttagcacttcgggaggcagagcaagaggatcacttgaggccaggagttggagaccagcctggcaacatagcaagaccccgtctctacaaaaaataaaattatctgggcctgttggtgcacacctgtagtcccagctactcaggaggctgaggtgggaggatcacttgagcctaggaattcgaggctgcagtgagctgtgattgcaccactgcactccagcctgggtgacagagggagaacctatctccaaaacaaaacaaaataaaaacaaaacaaaactccaagcagagaaagacttgacgagtcggatgagtctgatgattcctaaaggaaatcctttttgagattccaggagattccatctcctcaacagagtaattgattttgagcctcccacctcctgaattaaggcccacccatccctatcctgcactgaactgtagactcttttttacttccttacaaaagtttattcttaaatgtacaacagactccaagacgacactttattgtagctataggtggcaaaagatgttatggcagagaatccagatgtttaaataggaatggggtcaagggtcaccgccccaagcacggataacaaaatttattttttgccagatttctttaattccacctgtgactggtgagggctggtggcggggtggctttcacttttagctcctctttttgtttctgcttgaacgtcccatcttccttacccacccccttgacctgcttcttgagctttctcagggcttcttgccacctttgcagctgtacatggcacctgccatagggctctaattttaaactgagaaattgagaaaacaggaaactgactctttttggggggagagtaagacaaacaggaaaaggaaaatgaagacgtggttgatacagatcgttggatttcaaaaggaaaagtctacggataaccgaaaaaaataaatatttagaaatgcatagtcttggctggttaaataagtatccatgcttgttcttgtggcatagtagttacgagacatttttagttaaatggaaaaatgtgaattactatagtttgagtgatatgctgctttccaaattaaaagcagcataacaaaaacattcccctaatactcataaataattcattgaattggcaataattcacctcctaatgacttcatatgaagtataaagtaacttcgatacatcagaagaaatcctatcttctaatataagaaagtaatatgattacattaaatgcgtctcatataagttataaaaatggtatctatgagtaaagaaatgcttgtgaacaaaaaaattgatcttataaaggtcaaacaggccaggcgtggtggctcacacctgtaatcccagcactttgggaggctgaggtgggcggagtacctgaggtcaggagttcaagaccagcctggccaacatggtgataccctgtctctacaaaaatacaaaaaattagctgggcatgatggtgggtgcctgtaatctcagctactcgggaggcagaggcgggagaatcgcttgaacccgggaggcggaggttgcagtgaactgagattgagccacaacaaccaagcctgggagacagaggaaactctgtctcaaaaaataaaaaataaaaattaaaattaaaaaaaaggtcaaacaaaccaaacccttctgattaatttattcaatctacttttattataagcaaatgagaaattataattttaatctgaaaaagcagaatcaggggattttggagctggacagtcccctggaaattatttggatcaaagccctcattttataggtgaagaaactgagaagtaagatttgagcaagctgcccaaaggctttgccaaaggctataccagtgaatggcagagtctggactggaagtcccagtgctgccgtccaggtgagacctgttccactgcatgctactagctcccgggctgagaccggacttttgcttggcaggtttctttctttcgaaactattaattattgtattttttgtagagacagggttttgccatgatgcccaggctggtcttgaactcctgagctcaagagatccacccagcttggcctctcaaaaatgttgggattacaggcataagccacagtgcccggcccattttcctcccacctctttgttccttctctgtttcttttgcagcattatgttctatcattgtataccagagttcctcaacttcagttatagtctgttcttgctttatgctatcttcttcagcaagctcatcttggtctgttttcctccttatcaggcataccccagaaactcctgttttatctccacctcaactaaacattttcctgagttctgggcctctataaactaattatttgattaacatcttttttttttttttctgagatagagtctctctctgtcacccaggctggagtgcagtggtgcaatctcagatcactgcagcttctgcctcccagattcaagcgattctcctgcctcagcctcctaagtagctgggattataggcatgcaccaccgcacacagctaatttttgtacttttagtagagacggggtttcaccatgttggtcaggctggtctcaaactcctgatctgaagtgatctgactgcctcagcttcccaaagtgctgggattacaagcctgagccaccatgcctggccaacatctttaattggatatctcagtatcaagaaggcccataatattcctctgcctcatccctctcctcagtcctcttcttgtgtttcctagttcagagaatggcaccattctctatcaagctgcgcaaatcagacatgtgtgattttttgttgttgttgagacagggactcactctgtcacccaggctagagtgcagtggcgtgatcatggcgcactgaagcctcaaactcctgggctcaggagatcctcccgcctcagcctcctgagtagctgggaccacaggcccacaccaccatgcccagctaattttgtattctttgtagagatggggtttcatcatgtttgcccaggctggtctcgaactcctggactcaagcaatccacccacctcagcctcccaaagtgctgggattacaggcatgagccactgtgcccagctgaagtgtgatccttaacttcaccccttctcatgccctccatttccaatccatctccagtccagttgactccagctactcaattatttccacttatctcattccactacctttgaagctaccaccatctctaactacagtcatctcccaactaactggtctcctggcatctctctggttctcctccactaatttcaaaaaaagaaatttactgtgacagtgctcacaacactcccccttgctcttactaaagatgcttaccatagcctccaggtattgtatggcctgaggtctatctacatttccaggtgcaggacacaccatgtctccccactcccaaatttagtctccagactccatcctttttacagttctttaaaagcatcacaattcctccaaccactaggcatttgtatgtgctattccctctttccagaatgcaataccctccctctgcctagctagctaacttctatgtatctatgactgcagctcaaactttcctcatggactccctccacaagtgccaagcctgggccagattcttttgttatgtgctcacagaacgatgttccctttagcattcattgagtttgctgtttaattattcttgtcttgtttttgtttaattagtcctatctctaatactagacaaatgttccttaagatcacaggaaatataggactgtctctacataaaaactgttttatatccataatgcctaggacagtacctggcacacagtatatgctcaataaatttttgttgaatgaatgcaattatcattatattcctgatattagcaggtataatccagtttaagtttgggaacagaaagacaaaacggaccacatctaataaatccggtctcctttcttttattatttatttatttgagacagttttgctcttgttgcccaggctgcagtgcaatggcatgatcttggctcactgaaacctccgcctcccaagttcaagggattctccagcctcagcctcccaagtagctgggattacaggcatccaccaccacgcccagctaatttttttgtatttttagtagagatggggtttcaccatgttggccaggctggtctcgaactcctgacctcaggtgatccacccacctcagcctcccaaagtgttgggattacaggcgtgagccaccgtgcccggccaaggtctcctttcttttaatcaaactctcacctttggccattctgcagtcattcacccgacagtatttactgacggagtgaatacagagtgcttgattaatgttgctgctttgttattattattattattattgagatggagtcttgctctgttgcccaggctggagtgcagtggcgtgatctcggctcactgcaacctccgcctcccgggttcaagccattctcctgcctcagcctcccaagtagctgggactacaggcatgcaacaccacacctggctaatttttgtatttttagtagagacaaggtttcaccatattggccaggctggtcttgaactcctgacctcaggtgatctgcccacctcagcttcccaaagtgctgggattacaggcgtgagccaccatacccaacctaatgtttctgctttgaaatacaatttcaaaaagtcattaataggttgaaaacagcaagattttaaaagtattttaaaaagtgaaacagaagaatgcttacttcatttcacagagatagatttctcctttatgttatttctaaaaggagatggaattttgtttcattcatttctgcttatttggacaggccaaatatgaacagctgaacacgtcagcgttaccatgcatatgttacacagatgccatccttcttccatcagctctcatatgcaatacagaagtaaaaagaggttctctttatttttaaaaggtaaaaattgaaattcagtcacttaacacagaataaacaataattacaattacactggtaacaaaggacagcaagcatgttttctttgaaagcactgtatctggtttgtctccgtgcttggtcctagtatctggcatattttccccagagttttcttttcagtgggatgattatcttcggggcaaaaaagtttatcagactcaagttttagcagtacttattttattcatttatatacatgtaaccccatcctgtcttactccaatcttcttactgccttcctactgacacatatattatataacaccctccccaagttctatttacggttaaaaatttctttttttttttctttttttgagacagagtttcactctcgtcacccaggctggtgtgcaatggcgcagtctcggctcactgcaacctccgactccctggttcaagtgattctcctgtctcagcctcccgagtagctggaattacaggcgcccgccaccatgcccagctaatttttgtatttttagtagagacagtgtttcgccatgttggccaggctggtctcaaactcctgacctcaggtgatccacccgccttggcctctcaaagtgctgggattataggcgtaagccactgcgcccagcctacagttacgaatttctaaatggcacaaataaactcagctgttctcagtgcagacgtcaaatcctcactgtgctgaaacattttcctcagcttttgggaaataattacaatttaaacatacacagagaatgtttcttagacaaacataatacccgaggcttatctggtaaaaactaattgctctgtccttagcacaaaaaatatatatctttgtaaaatgagaagaaccaaagaatatttaaaacaaagaaggaagccacacgtactaattacacaagagactgactgacaaactggaattctccaaaacagattttcagcgaggcttctcatttcagagtccaggaaaaaaaaatcctaaaaaccccaaaggtatattatatgtgtgtatatatatttttattgtgttaaaaaacacaaaacataaaatttactgtcttatcaaaaggtatattttgtcgctcttccctttttttttttttttttttcccgagacagagtccagtctgtcgcccaggctgaagtgcagtggcatgatctcggctcactgcaacctgcatcttctgggctcaagcaatcctcccacctcagcctcctgagtagatggagctacaggcacgtgccactaggcccggctaatttttgtattttttgcagacagggttttgccatgttgcccgggctggtctttgttctcctaagagttgttttctccatgaaagttgataaataacatttagaaaatgaattattacaagagtaatgatatgtctcaatttattatatgaaattatcaacaactgcttttaatattcagatgtcaagaagatgaaaagcagaaatacattttgcaaacatgtagcactccataaatggaaatcatgtatttcctctaatatcccaatttttctatattgggatcttatatggctgtttctatatggctattttgtcccaacttgctgtacaagaattttccccagccaccttagaaaggttggatgtagttcactccaagtttgcagttcactccaagtgtttcagtaccacagaaagctccatggaagcctcaaatgtacgggctaggcaatagaagcagggaggtaggattaagaaattactggccaggtgtggtggctcaggcctgtaatcccagcacttcgagaggctgaggcagacagatggcttgagctcaagagtttgagatcagcctgagcaacatggcaaaactctgtctctacaaaaaatataaaaatcagccaggtatgttggtgtgcacctgtagtcccagctactggggaggttgaggcaggaggattgcttgagcccaggaggctgaggctgcagtgagccatgattgtgccactgcattccagcctggtcgactgtaagacaaaaaataagaaaataaaaaatttaccaatataaaatgctcaaacagctaacaaacatgttcaattccatttatagtcttttctttgagccatttaaacatagggctattttttttttttttttttgagatggagtttcactcttgttgcccaggctggagagcaatggcatgatctcggctcaccacaacctctgcctcctgggttcaagcgattctcctgcctcagcctcccgagcagctgggattacaggcatgtgccaccatgcctggctaattttgtatttttagtagagacgggattcctccatgttggtcagactggtcttgaactcccaacctcaggtgatctgcctgcctcaaccttccaaagtgctgggattacaggtgtgagccactgagattggctgccgttttgttttttaactccatatagtttctatagttcactgaaaactcaaagagatgacctataaatgtatgaataatgtatgatttcttacatcaattttctactagaaaaaaatcatacttttagaattggattttgtcttacagtcatctttattatactttataaatgagatttcatttatataaatcaggaagctaaactaaaatagaaacactagatttaaattctgatttgaatactctgatcaaaataacaaatctcacactgggaaaccatctatcagcaagcagagagctactgtgtgtccttccttagaagagtttgaacaccgagaacccacagcatatttgcagtacagtaacagcaattcctttgtcattatcacagaactttaattttcatatactttgctgggaccaaccaaaccatcccatatatataaccatatccatatatatatatatatatatcccacatatatatgggatggtatatatatacacatgtatatgtatgtgtgtgtgtatatatgtgtatatatgtatacacacacacacacacacatatatatatatatacacacacacacatatatatatggagagagagagagagacagtgtcttgctctgtcgcccaggctggagtgcagtggtacgatcttggctcattgcaacctccgcctcccaggctcaagcgattctcatgtctcagtctcccaagtagctgggattacaggtgtgcaccaccacaccaggctaaccattccatacattttatacaatcatttttaaaaagaagcatgaaccatttcggttttagagaattaagtttttttaaaaaagagactcttaaaaaaaagtcattatatgaataaaatctgctttgtgttaattccgacaaatcattccatcattgagtctgtcaccaattttttttttttgaaatggagtttcgctcttgttgcccaggctggagtgcaatggtacgatctcggctcactgcaaccgccgcctcccgggttcaagtgattctcctgcctcagcctcccgagtagctgggattacaggcatgcgccaccacgcctggctaattttgtattattagttgagacagggtttctccatgttggtcaggctggtctcgaactcctgacctcaagtgatccgctggccttggcctcccaaagtgctgggattacaggcgtgagccaccgtgcctggcccaattttttttttttaataacttgcacacttaacaatattttttatcttcttgggacaacattcttttctccacaaaaacccaattaaggacgttgtgccagtttactcctacttccttcctgttcactgagcttaaagtgggtataggcgagaatgccaaataatgtacataaaatgccaagggcctgattaatggacagtggatccttaaataaaacatatcctccgaataaagtaatgcagaacttgaagtgtccgaacatgttataggtgacaggtgaagtgttcccaatgatccaataaattgataagttcaccatgaaagctattactccagatagcagcaccataagcaaagcagaaactgaccagggaccaaatattcctccttctccaaacactggctcaaagaagggcacagcaaccagcaacatggcagatgacatcggagcctggtagtacagcagctgcattgagttcacttgtaattcatgctgtttggctcctacccaaaacaggtaggtatttggtgagcatcacacacccaagtttctctgtctcctttcttctcttcaccttgagtcagacaacttatgcaattatgctttcttcccaacagtctattgtctctatactgtattttctaaaccttggaatacagcttcaaaatttatgaaatctgcagcgtgagctggattctggtggagaaggttttctggtagcagaaggtctggatggctatgatcaccggcgtggtcatggccttggccagctgataggtgcctatggtgttgttctgcagagaaaggttagtgaagaccacaaagccacagaagctgagggccaggaggaggagcctggagggcggcagacttttgggggcaaagatgtccagcttctggcagatatacaagcccagccaggtgaccacgaagtgcaccagggtcaggctcatgttggggaagccgtggtacacataaatccatttgttgaggaacacaatgcagatggacaccagcaggttgaacaggagcccggcggcgattcgccagtggccccgcactcggtccaccagcaatgccatgatccccgcgaagctggggccgtctagcctcggaaggggcgccgggcctgtctccggctgcccttctactccaccgccgcgtcctcgcagacgccgacctcaccgtctgacccaggagtggcatgcacagatcaaccccgggcgagtagcactcttaacagaggacacacaccccgccgccgccctgtaagccagctaggac

SEQ ID NO: 12654 - RNA, 16183 nt, Homo sapiens
  source 1..16183: mol_type = other RNA
gatctcactttgttgcccaggctggagtgcagtggcacagtcatggctcactataacctcaaactcctgggctcaggcaatcctctgcctcatcttcccaagtagctgggactacaggtgtctaccaccatgcccggctaattttataaaattttttatagagacgggggtcttgctgtgttgctcaggtcttgaactcctggcctcaagtgcacctcctgccttggcctcccaaaacactgggattacagatgcaggccactgtacctggcccccatatttattaatcacattttattcattcattcatttaactttcctgtgaagttttgcaaatggcttcctcaattcccccttgttaagctttttttccttctcaaaccatgcttatatcctttctggttccagccacatattttgggtcagacagtcctagcactgtacttttaatatcacctggagtgacttcagagacttctttgaagccacaagaccatctggttcaataccaatattttgaaatctaatgactcactattctagaacattctcaacattaagtttcttaaagatggcttaaatactttttaaatttaaataaatgtacagaaaacaaaaatcttttcatttaaaacctaccaaatatagccacacatggtagggcatacctatagtcccagttactcaggaggctgaggcaggaggattacttgagccaaggagttcagggctgcagtgcactatgattgtgcctgcaaaaaggcactgcactccagcgtcggccacagagaaagacctagttttttgtttttgtttttgtttttgagacagagtcttgttctgtcgcccaggctggaatgcagtctggagtgcagtggctcattgcaacctccacctcctgggttcaagcaattctcctgcctcagcctcctgagtagctgggattacaggggcacaccaccacgcccaactaacttttgtatttttagtagagatggagtttcgccatgttggccaggttggtctcaaactcctgggctcaagtgattcacctaccttggcctcccaaagtgctgggattacaggcgtgagccactgcatccagccataagactcagtttcttttcttttttttttttggagatggagttttgctcttttgtccaggctggagtgaagtggtgcgaccatggttcactgcaacctctaccctcccggttcaagcaattctcctgcctcagcctcccaagtagctgggattataggcacccactactacgcccagctaatttttgtatttttagtagagacgaggtttcgccatgttggctaggctggtctcaaactcctgacctcaggtgatccacccgcttcggccttgcaaagtgctgagattacaggcatgagtcaccacgcctggccggcaagaccctgtttctaaaaaacaaaataaaaaataaatcttccaactatttataatatgatctctgttcatctttactgttataaacattcctcaggtacttgaaaggagtgtgtgttctaggcttgttgagtacagataacctattagacaaggttactaacttccctgctgcctgctctatcacctctattagaagtatttaaaatctcaattttccttttaattttcatgctgttttctgggttgttcatgattgctatgtttgtggtggattgttctttaaaaaaaaaaatcttgatcctattaacactttttgcctcaaattctattttgtctgctattgatattactacccaaaatccccgcaccccgcccttttttttgagacaggatctcactctgtcactcaagctggagtgcagttcaccatcacggtggctcattgcagcctcgacctccctgggcttgggtgatcctcccacctcagcctcccgagtagctgggatcacaggcacataccaccatacctggctaatttttgtactttttatagagacggggattcaccatgttggccaggctggtcttaaactcctgatctcaagtgatccgcccaccttggcctcccaaagtgctgggattataggcatgagccaccacacccagccggcagcaaactgtttatggactggtactggggcccagaccctaccttgagtggtactgggctagaggacttattaattgcatgatctaggagtagttcataaattctgtgatggtcattctttgggtgaactccatttctagcagattctagataagcagcatgacttcctctgattctctgacacctgagggtggggaaattcagactgtcccacttgggttgtgcgtcttcacgctggggaagagggtgaggccaaagttgtgttgggagataaataatgaaattcaagaactccatggtaacagcccttgtctttcctctctggggccacacagtgcagtgtggggagaggagtggacagaaggaatgtcagcatttccttggcaaaatctcttgcgtttcagaacagcagtgagattttggaggtatgagagagtcacaggtgtgacattcctgtgaggaatgctatttgagtacaagcagtggatgtcctcatgatgttatgatttcagaagaatagcactgtgcttggctgaaaagttctgcattcaataactccatgccaataagcagccatttcctcccagcacacagttgctcaccaatgtccatggtcctatggcactgggaggcctctgatgcagctgtctcccactatggtcttaggaaattcctggaacgttattagagtgagtttttcctagatctgcttactgaatacctgttgaactttcacactgatggccagttccaagacttaagcatgaccttgcgaccattggtgatagtgctttcttgatctgctgaatcaaattgaagcagaactgggggtactactaggaatgaggggtgactagggatggggctggggcgaggggtatattgggtaactgaggatgaccagtgtcagagagcacaaagatgatggtgaagggcaggtagaccacctcccacttggtgggaaagtctgttcctggctggaactggttcattcattccaagccagcaacagctccaggtttggacgccatttatgaatctacatgccaccagaccagtccctgtcttccacacaccccactctctggagtctggaaaaatggcgggggtggggctagctactagtttttgtttttttttttctttttgagacacagtttcattctgtcatccaggctggagtgcagtggcatgatctcagctcactgcaacctccgcctcccaggttcaagcgattctcgtgccttagctttcagagtagctgggactacaggtgcacaccatcacagctgactaatttttcttttctttttttttttttgagacggagtctcactctgtctcccaggctggagtgcagtgatgtgatctcagctcactgcaacctacgtctccagggttcatgtgagtttcctgcctcagcctcctgagtgagtagctgggattacaggcgcctgccaccacgtccagctaatttttgtatttttagtagagattgggtttcaccatgttggccaggctggtctccaactcctgacctcaagtgatccacctgcctcggcctcccaaatcgctgggattacaggcgtgagtcatcatgcctggccttttttttttttttgtgagacagagttttgctcttgtcacccaggctggagtgtaatggcatgatctcggctcactgaaacctctgccaggcacacgtcaccatgcccggctaatttttgtatttttggtagaaacggggtttcaccatgttggccaggctggtctccaactcctgacctcaagtgatcctcctgccttggcctcccaaagtgctgggattacaggtgttagctaccaagtctggcctttttttttttttttttttttttttttttttgagacagagtttcgctcttgtcacccaggctggagtgtaatagtgtgattccagcttactgcaacctctgcctctcgggttcaagccattctcctgcctcagcctcctgagcagctgggattacaggcacacgccagcatgcctggctaatttttatatttttagtagagacggggtttcaccatgttggccaggctggtctcgaactcctgacctcaggtgatccatctgcctcagcctcccaaactgctgggatgacaggcgtgagccaccacgccaggccctatttttatttttaaccagtgctgtagtttgaatatttgtctcctccaaaactcatctggaaacatccccaatgtggcaatattgagagatggcgcctttaaaaggtgactgggtcatgaaggctctgcccagtgagactggtgcctttataagaagaggaagagagacctgagctaccatgctcaagtccctcaccacgtgaggccctctgccaccttgggtctctgcagagagttcccaggaacaagaagtctctcaccagatgtggaccctgtaccttggacttctcagtctccactattgtaagaaataaattccttttctttataaatgacccagtttcaggtattctgttctatgcaacacaaaatggactaagacaacgagtacgcttagttgttgcttcctgagttccaaagtccgacagacagagcaggtcctccattcttgcccctttttaccccaaatgctcattggcattcttgcagctacgagtaataattaaaagtggctaagccaggctggcatggttgctcacgcctgtaatatcagcactttgggaggctgaggcaggaggatcacttgaacccaggagtgagaccagccagggcaacatagcaacaccctgtctctaattattattatttttttaagtgagtaagccaaataggggtttacttttcatctagaacaagaagacgtgttggccaggctggtctcaaactactgggctcaagtgatccacccacctcagcctcccaaagtgttgggattatgcgtgagccaccgcacctggccacaagacccaatttcttttattttatctttttttttttttttttaagagatagggcatctaacggcattgttttagctgctcaacacttttttttttttgcttatttttgtttgttttgtttgtttttgagacagggtctccctctgttgcccagcatatagtgcagtggcatgatcatggctcactgcagcctcaacctcccaggatcaggcaatcctcctgcttcagcttcctgagtagctgagaccacaggtgcacaccaatatacctaatttttttttttttgagatggagtttcactcttgttgcccaggctggagtgcaatggcgtggtctcagctcactgcaacctctgcctccctggttcaagcgattctcctgtctcagcctgccgagtagctggggttacaggcataagccactacgcccagctaattttgtatttttagtagagacagggtttctccatgttggtcaggctggtctcgaactcctgacctcaggtgatccacccacctcagccttccaaagtgctgagattgcaggtgtgaaccactacgcctggccacctgactaatttttaagttattcacagagaacaggttttgcaatgttgcccaggctggtctcaaactcctgggctcaaatgatcctcctccctcggcctcccaaagtgctggggttacaggtgtgccactgtgcctggtcggctcaccactttcagatctggctctcttcacctctcttttatagtcataagctgattagcacaattctagacatccgcagctacatttaaggcaggaaggaggtggtaatagacactaccagccacatctgtcccttttaatcaggataccctagaaatcctcagcagactttgaattatgtgccattggtgaaatgtcatatgatcatccctctacaaggcaacgaggtaaaaagagaatttagtatttctagcctctagagtggagatgaacaaagaataggaatgggcatttgcttaggaaaccaactgtgccttacaacatttttgcacttttttctgtaacattttgtgttaaatcatataaaaatgctgatcctaacaaatatggtcaatgagtcacaccataattctctaagaactccagtccaaaaaggttaatcttgcttttaaactccaggcgcggtgtttcacagctgtaattttagcacttcgggaggcagagcaagaggatcacttgaggccaggagttggagaccagcctggcaacatagcaagaccccgtctctacaaaaaataaaattatctgggcctgttggtgcacacctgtagtcccagctactcaggaggctgaggtgggaggatcacttgagcctaggaattcgaggctgcagtgagctgtgattgcaccactgcactccagcctgggtgacagagggagaacctatctccaaaacaaaacaaaataaaaacaaaacaaaactccaagcagagaaagacttgacgagtcggatgagtctgatgattcctaaaggaaatcctttttgagattccaggagattccatctcctcaacagagtaattgattttgagcctcccacctcctgaattaaggcccacccatccctatcctgcactgaactgtagactcttttttacttccttacaaaagtttattcttaaatgtacaacagactccaagacgacactttattgtagctataggtggcaaaagatgttatggcagagaatccagatgtttaaataggaatggggtcaagggtcaccgccccaagcacggataacaaaatttattttttgccagatttctttaattccacctgtgactggtgagggctggtggcggggtggctttcacttttagctcctctttttgtttctgcttgaacgtcccatcttccttacccacccccttgacctgcttcttgagctttctcagggcttcttgccacctttgcagctgtacatggcacctgccatagggctctaattttaaactgagaaattgagaaaacaggaaactgactctttttggggggagagtaagacaaacaggaaaaggaaaatgaagacgtggttgatacagatcgttggatttcaaaaggaaaagtctacggataaccgaaaaaaataaatatttagaaatgcatagtcttggctggttaaataagtatccatgcttgttcttgtggcatagtagttacgagacatttttagttaaatggaaaaatgtgaattactatagtttgagtgatatgctgctttccaaattaaaagcagcataacaaaaacattcccctaatactcataaataattcattgaattggcaataattcacctcctaatgacttcatatgaagtataaagtaacttcgatacatcagaagaaatcctatcttctaatataagaaagtaatatgattacattaaatgcgtctcatataagttataaaaatggtatctatgagtaaagaaatgcttgtgaacaaaaaaattgatcttataaaggtcaaacaggccaggcgtggtggctcacacctgtaatcccagcactttgggaggctgaggtgggcggagtacctgaggtcaggagttcaagaccagcctggccaacatggtgataccctgtctctacaaaaatacaaaaaattagctgggcatgatggtgggtgcctgtaatctcagctactcgggaggcagaggcgggagaatcgcttgaacccgggaggcggaggttgcagtgaactgagattgagccacaacaaccaagcctgggagacagaggaaactctgtctcaaaaaataaaaaataaaaattaaaattaaaaaaaaggtcaaacaaaccaaacccttctgattaatttattcaatctacttttattataagcaaatgagaaattataattttaatctgaaaaagcagaatcaggggattttggagctggacagtcccctggaaattatttggatcaaagccctcattttataggtgaagaaactgagaagtaagatttgagcaagctgcccaaaggctttgccaaaggctataccagtgaatggcagagtctggactggaagtcccagtgctgccgtccaggtgagacctgttccactgcatgctactagctcccgggctgagaccggacttttgcttggcaggtttctttctttcgaaactattaattattgtattttttgtagagacagggttttgccatgatgcccaggctggtcttgaactcctgagctcaagagatccacccagcttggcctctcaaaaatgttgggattacaggcataagccacagtgcccggcccattttcctcccacctctttgttccttctctgtttcttttgcagcattatgttctatcattgtataccagagttcctcaacttcagttatagtctgttcttgctttatgctatcttcttcagcaagctcatcttggtctgttttcctccttatcaggcataccccagaaactcctgttttatctccacctcaactaaacattttcctgagttctgggcctctataaactaattatttgattaacatcttttttttttttttctgagatagagtctctctctgtcacccaggctggagtgcagtggtgcaatctcagatcactgcagcttctgcctcccagattcaagcgattctcctgcctcagcctcctaagtagctgggattataggcatgcaccaccgcacacagctaatttttgtacttttagtagagacggggtttcaccatgttggtcaggctggtctcaaactcctgatctgaagtgatctgactgcctcagcttcccaaagtgctgggattacaagcctgagccaccatgcctggccaacatctttaattggatatctcagtatcaagaaggcccataatattcctctgcctcatccctctcctcagtcctcttcttgtgtttcctagttcagagaatggcaccattctctatcaagctgcgcaaatcagacatgtgtgattttttgttgttgttgagacagggactcactctgtcacccaggctagagtgcagtggcgtgatcatggcgcactgaagcctcaaactcctgggctcaggagatcctcccgcctcagcctcctgagtagctgggaccacaggcccacaccaccatgcccagctaattttgtattctttgtagagatggggtttcatcatgtttgcccaggctggtctcgaactcctggactcaagcaatccacccacctcagcctcccaaagtgctgggattacaggcatgagccactgtgcccagctgaagtgtgatccttaacttcaccccttctcatgccctccatttccaatccatctccagtccagttgactccagctactcaattatttccacttatctcattccactacctttgaagctaccaccatctctaactacagtcatctcccaactaactggtctcctggcatctctctggttctcctccactaatttcaaaaaaagaaatttactgtgacagtgctcacaacactcccccttgctcttactaaagatgcttaccatagcctccaggtattgtatggcctgaggtctatctacatttccaggtgcaggacacaccatgtctccccactcccaaatttagtctccagactccatcctttttacagttctttaaaagcatcacaattcctccaaccactaggcatttgtatgtgctattccctctttccagaatgcaataccctccctctgcctagctagctaacttctatgtatctatgactgcagctcaaactttcctcatggactccctccacaagtgccaagcctgggccagattcttttgttatgtgctcacagaacgatgttccctttagcattcattgagtttgctgtttaattattcttgtcttgtttttgtttaattagtcctatctctaatactagacaaatgttccttaagatcacaggaaatataggactgtctctacataaaaactgttttatatccataatgcctaggacagtacctggcacacagtatatgctcaataaatttttgttgaatgaatgcaattatcattatattcctgatattagcaggtataatccagtttaagtttgggaacagaaagacaaaacggaccacatctaataaatccggtctcctttcttttattatttatttatttgagacagttttgctcttgttgcccaggctgcagtgcaatggcatgatcttggctcactgaaacctccgcctcccaagttcaagggattctccagcctcagcctcccaagtagctgggattacaggcatccaccaccacgcccagctaatttttttgtatttttagtagagatggggtttcaccatgttggccaggctggtctcgaactcctgacctcaggtgatccacccacctcagcctcccaaagtgttgggattacaggcgtgagccaccgtgcccggccaaggtctcctttcttttaatcaaactctcacctttggccattctgcagtcattcacccgacagtatttactgacggagtgaatacagagtgcttgattaatgttgctgctttgttattattattattattattgagatggagtcttgctctgttgcccaggctggagtgcagtggcgtgatctcggctcactgcaacctccgcctcccgggttcaagccattctcctgcctcagcctcccaagtagctgggactacaggcatgcaacaccacacctggctaatttttgtatttttagtagagacaaggtttcaccatattggccaggctggtcttgaactcctgacctcaggtgatctgcccacctcagcttcccaaagtgctgggattacaggcgtgagccaccatacccaacctaatgtttctgctttgaaatacaatttcaaaaagtcattaataggttgaaaacagcaagattttaaaagtattttaaaaagtgaaacagaagaatgcttacttcatttcacagagatagatttctcctttatgttatttctaaaaggagatggaattttgtttcattcatttctgcttatttggacaggccaaatatgaacagctgaacacgtcagcgttaccatgcatatgttacacagatgccatccttcttccatcagctctcatatgcaatacagaagtaaaaagaggttctctttatttttaaaaggtaaaaattgaaattcagtcacttaacacagaataaacaataattacaattacactggtaacaaaggacagcaagcatgttttctttgaaagcactgtatctggtttgtctccgtgcttggtcctagtatctggcatattttccccagagttttcttttcagtgggatgattatcttcggggcaaaaaagtttatcagactcaagttttagcagtacttattttattcatttatatacatgtaaccccatcctgtcttactccaatcttcttactgccttcctactgacacatatattatataacaccctccccaagttctatttacggttaaaaatttctttttttttttctttttttgagacagagtttcactctcgtcacccaggctggtgtgcaatggcgcagtctcggctcactgcaacctccgactccctggttcaagtgattctcctgtctcagcctcccgagtagctggaattacaggcgcccgccaccatgcccagctaatttttgtatttttagtagagacagtgtttcgccatgttggccaggctggtctcaaactcctgacctcaggtgatccacccgccttggcctctcaaagtgctgggattataggcgtaagccactgcgcccagcctacagttacgaatttctaaatggcacaaataaactcagctgttctcagtgcagacgtcaaatcctcactgtgctgaaacattttcctcagcttttgggaaataattacaatttaaacatacacagagaatgtttcttagacaaacataatacccgaggcttatctggtaaaaactaattgctctgtccttagcacaaaaaatatatatctttgtaaaatgagaagaaccaaagaatatttaaaacaaagaaggaagccacacgtactaattacacaagagactgactgacaaactggaattctccaaaacagattttcagcgaggcttctcatttcagagtccaggaaaaaaaaatcctaaaaaccccaaaggtatattatatgtgtgtatatatatttttattgtgttaaaaaacacaaaacataaaatttactgtcttatcaaaaggtatattttgtcgctcttccctttttttttttttttttttcccgagacagagtccagtctgtcgcccaggctgaagtgcagtggcatgatctcggctcactgcaacctgcatcttctgggctcaagcaatcctcccacctcagcctcctgagtagatggagctacaggcacgtgccactaggcccggctaatttttgtattttttgcagacagggttttgccatgttgcccgggctggtctttgttctcctaagagttgttttctccatgaaagttgataaataacatttagaaaatgaattattacaagagtaatgatatgtctcaatttattatatgaaattatcaacaactgcttttaatattcagatgtcaagaagatgaaaagcagaaatacattttgcaaacatgtagcactccataaatggaaatcatgtatttcctctaatatcccaatttttctatattgggatcttatatggctgtttctatatggctattttgtcccaacttgctgtacaagaattttccccagccaccttagaaaggttggatgtagttcactccaagtttgcagttcactccaagtgtttcagtaccacagaaagctccatggaagcctcaaatgtacgggctaggcaatagaagcagggaggtaggattaagaaattactggccaggtgtggtggctcaggcctgtaatcccagcacttcgagaggctgaggcagacagatggcttgagctcaagagtttgagatcagcctgagcaacatggcaaaactctgtctctacaaaaaatataaaaatcagccaggtatgttggtgtgcacctgtagtcccagctactggggaggttgaggcaggaggattgcttgagcccaggaggctgaggctgcagtgagccatgattgtgccactgcattccagcctggtcgactgtaagacaaaaaataagaaaataaaaaatttaccaatataaaatgctcaaacagctaacaaacatgttcaattccatttatagtcttttctttgagccatttaaacatagggctattttttttttttttttttgagatggagtttcactcttgttgcccaggctggagagcaatggcatgatctcggctcaccacaacctctgcctcctgggttcaagcgattctcctgcctcagcctcccgagcagctgggattacaggcatgtgccaccatgcctggctaattttgtatttttagtagagacgggattcctccatgttggtcagactggtcttgaactcccaacctcaggtgatctgcctgcctcaaccttccaaagtgctgggattacaggtgtgagccactgagattggctgccgttttgttttttaactccatatagtttctatagttcactgaaaactcaaagagatgacctataaatgtatgaataatgtatgatttcttacatcaattttctactagaaaaaaatcatacttttagaattggattttgtcttacagtcatctttattatactttataaatgagatttcatttatataaatcaggaagctaaactaaaatagaaacactagatttaaattctgatttgaatactctgatcaaaataacaaatctcacactgggaaaccatctatcagcaagcagagagctactgtgtgtccttccttagaagagtttgaacaccgagaacccacagcatatttgcagtacagtaacagcaattcctttgtcattatcacagaactttaattttcatatactttgctgggaccaaccaaaccatcccatatatataaccatatccatatatatatatatatatatcccacatatatatgggatggtatatatatacacatgtatatgtatgtgtgtgtgtatatatgtgtatatatgtatacacacacacacacacacatatatatatatatacacacacacacatatatatatggagagagagagagagacagtgtcttgctctgtcgcccaggctggagtgcagtggtacgatcttggctcattgcaacctccgcctcccaggctcaagcgattctcatgtctcagtctcccaagtagctgggattacaggtgtgcaccaccacaccaggctaaccattccatacattttatacaatcatttttaaaaagaagcatgaaccatttcggttttagagaattaagtttttttaaaaaagagactcttaaaaaaaagtcattatatgaataaaatctgctttgtgttaattccgacaaatcattccatcattgagtctgtcaccaattttttttttttgaaatggagtttcgctcttgttgcccaggctggagtgcaatggtacgatctcggctcactgcaaccgccgcctcccgggttcaagtgattctcctgcctcagcctcccgagtagctgggattacaggcatgcgccaccacgcctggctaattttgtattattagttgagacagggtttctccatgttggtcaggctggtctcgaactcctgacctcaagtgatccgctggccttggcctcccaaagtgctgggattacaggcgtgagccaccgtgcctggcccaattttttttttttaataacttgcacacttaacaatattttttatcttcttgggacaacattcttttctccacaaaaacccaattaaggacgttgtgccagtttactcctacttccttcctgttcactgagcttaaagtgggtataggcgagaatgccaaataatgtacataaaatgccaagggcctgattaatggacagtggatccttaaataaaacatatcctccgaataaagtaatgcagaacttgaagtgtccgaacatgttataggtgacaggtgaagtgttcccaatgatccaataaattgataagttcaccatgaaagctattactccagatagcagcaccataagcaaagcagaaactgaccagggaccaaatattcctccttctccaaacactggctcaaagaagggcacagcaaccagcaacatggcagatgacatcggagcctggtagtacagcagctgcattgagttcacttgtaattcatgctgtttggctcctacccacacttgataaagggatgtaactaaaacaccaagagcagcaaacaccattccaaggaaattaaacttcacatcgtaataagaatttaggattacacctaaagttataggaatcagcgtgagctggattctggtggagaaggttttctggtagcagaaggtctggatggctatgatcaccggcgtggtcatggccttggccagctgataggtgcctatggtgttgttctgcagagaaaggttagtgaagaccacaaagccacagaagctgagggccaggaggaggagcctggagggcggcagacttttgggggcaaagatgtccagcttctggcagatatacaagcccagccaggtgaccacgaagtgcaccagggtcaggctcatgttggggaagccgtggtacacataaatccatttgttgaggaacacaatgcagatggacaccagcaggttgaacaggagcccggcggcgattcgccagtggccccgcactcggtccaccagcaatgccatgatccccgcgaagctggggccgtctagcctcggaaggggcgccgggcctgtctccggctgcccttctactccaccgccgcgtcctcgcagacgccgacctcaccgtctgacccaggagtggcatgcacagatcaaccccgggcgagtagcactcttaacagaggacacacaccccgccgccgccctgtaagccagctaggac

SEQ ID NO: 12655 - RNA, 16072 nt, Homo sapiens
  source 1..16072: mol_type = other RNA
gatctcactttgttgcccaggctggagtgcagtggcacagtcatggctcactataacctcaaactcctgggctcaggcaatcctctgcctcatcttcccaagtagctgggactacaggtgtctaccaccatgcccggctaattttataaaattttttatagagacgggggtcttgctgtgttgctcaggtcttgaactcctggcctcaagtgcacctcctgccttggcctcccaaaacactgggattacagatgcaggccactgtacctggcccccatatttattaatcacattttattcattcattcatttaactttcctgtgaagttttgcaaatggcttcctcaattcccccttgttaagctttttttccttctcaaaccatgcttatatcctttctggttccagccacatattttgggtcagacagtcctagcactgtacttttaatatcacctggagtgacttcagagacttctttgaagccacaagaccatctggttcaataccaatattttgaaatctaatgactcactattctagaacattctcaacattaagtttcttaaagatggcttaaatactttttaaatttaaataaatgtacagaaaacaaaaatcttttcatttaaaacctaccaaatatagccacacatggtagggcatacctatagtcccagttactcaggaggctgaggcaggaggattacttgagccaaggagttcagggctgcagtgcactatgattgtgcctgcaaaaaggcactgcactccagcgtcggccacagagaaagacctagttttttgtttttgtttttgtttttgagacagagtcttgttctgtcgcccaggctggaatgcagtctggagtgcagtggctcattgcaacctccacctcctgggttcaagcaattctcctgcctcagcctcctgagtagctgggattacaggggcacaccaccacgcccaactaacttttgtatttttagtagagatggagtttcgccatgttggccaggttggtctcaaactcctgggctcaagtgattcacctaccttggcctcccaaagtgctgggattacaggcgtgagccactgcatccagccataagactcagtttcttttcttttttttttttggagatggagttttgctcttttgtccaggctggagtgaagtggtgcgaccatggttcactgcaacctctaccctcccggttcaagcaattctcctgcctcagcctcccaagtagctgggattataggcacccactactacgcccagctaatttttgtatttttagtagagacgaggtttcgccatgttggctaggctggtctcaaactcctgacctcaggtgatccacccgcttcggccttgcaaagtgctgagattacaggcatgagtcaccacgcctggccggcaagaccctgtttctaaaaaacaaaataaaaaataaatcttccaactatttataatatgatctctgttcatctttactgttataaacattcctcaggtacttgaaaggagtgtgtgttctaggcttgttgagtacagataacctattagacaaggttactaacttccctgctgcctgctctatcacctctattagaagtatttaaaatctcaattttccttttaattttcatgctgttttctgggttgttcatgattgctatgtttgtggtggattgttctttaaaaaaaaaaatcttgatcctattaacactttttgcctcaaattctattttgtctgctattgatattactacccaaaatccccgcaccccgcccttttttttgagacaggatctcactctgtcactcaagctggagtgcagttcaccatcacggtggctcattgcagcctcgacctccctgggcttgggtgatcctcccacctcagcctcccgagtagctgggatcacaggcacataccaccatacctggctaatttttgtactttttatagagacggggattcaccatgttggccaggctggtcttaaactcctgatctcaagtgatccgcccaccttggcctcccaaagtgctgggattataggcatgagccaccacacccagccggcagcaaactgtttatggactggtactggggcccagaccctaccttgagtggtactgggctagaggacttattaattgcatgatctaggagtagttcataaattctgtgatggtcattctttgggtgaactccatttctagcagattctagataagcagcatgacttcctctgattctctgacacctgagggtggggaaattcagactgtcccacttgggttgtgcgtcttcacgctggggaagagggtgaggccaaagttgtgttgggagataaataatgaaattcaagaactccatggtaacagcccttgtctttcctctctggggccacacagtgcagtgtggggagaggagtggacagaaggaatgtcagcatttccttggcaaaatctcttgcgtttcagaacagcagtgagattttggaggtatgagagagtcacaggtgtgacattcctgtgaggaatgctatttgagtacaagcagtggatgtcctcatgatgttatgatttcagaagaatagcactgtgcttggctgaaaagttctgcattcaataactccatgccaataagcagccatttcctcccagcacacagttgctcaccaatgtccatggtcctatggcactgggaggcctctgatgcagctgtctcccactatggtcttaggaaattcctggaacgttattagagtgagtttttcctagatctgcttactgaatacctgttgaactttcacactgatggccagttccaagacttaagcatgaccttgcgaccattggtgatagtgctttcttgatctgctgaatcaaattgaagcagaactgggggtactactaggaatgaggggtgactagggatggggctggggcgaggggtatattgggtaactgaggatgaccagtgtcagagagcacaaagatgatggtgaagggcaggtagaccacctcccacttggtgggaaagtctgttcctggctggaactggttcattcattccaagccagcaacagctccaggtttggacgccatttatgaatctacatgccaccagaccagtccctgtcttccacacaccccactctctggagtctggaaaaatggcgggggtggggctagctactagtttttgtttttttttttctttttgagacacagtttcattctgtcatccaggctggagtgcagtggcatgatctcagctcactgcaacctccgcctcccaggttcaagcgattctcgtgccttagctttcagagtagctgggactacaggtgcacaccatcacagctgactaatttttcttttctttttttttttttgagacggagtctcactctgtctcccaggctggagtgcagtgatgtgatctcagctcactgcaacctacgtctccagggttcatgtgagtttcctgcctcagcctcctgagtgagtagctgggattacaggcgcctgccaccacgtccagctaatttttgtatttttagtagagattgggtttcaccatgttggccaggctggtctccaactcctgacctcaagtgatccacctgcctcggcctcccaaatcgctgggattacaggcgtgagtcatcatgcctggccttttttttttttttgtgagacagagttttgctcttgtcacccaggctggagtgtaatggcatgatctcggctcactgaaacctctgccaggcacacgtcaccatgcccggctaatttttgtatttttggtagaaacggggtttcaccatgttggccaggctggtctccaactcctgacctcaagtgatcctcctgccttggcctcccaaagtgctgggattacaggtgttagctaccaagtctggcctttttttttttttttttttttttttttttttgagacagagtttcgctcttgtcacccaggctggagtgtaatagtgtgattccagcttactgcaacctctgcctctcgggttcaagccattctcctgcctcagcctcctgagcagctgggattacaggcacacgccagcatgcctggctaatttttatatttttagtagagacggggtttcaccatgttggccaggctggtctcgaactcctgacctcaggtgatccatctgcctcagcctcccaaactgctgggatgacaggcgtgagccaccacgccaggccctatttttatttttaaccagtgctgtagtttgaatatttgtctcctccaaaactcatctggaaacatccccaatgtggcaatattgagagatggcgcctttaaaaggtgactgggtcatgaaggctctgcccagtgagactggtgcctttataagaagaggaagagagacctgagctaccatgctcaagtccctcaccacgtgaggccctctgccaccttgggtctctgcagagagttcccaggaacaagaagtctctcaccagatgtggaccctgtaccttggacttctcagtctccactattgtaagaaataaattccttttctttataaatgacccagtttcaggtattctgttctatgcaacacaaaatggactaagacaacgagtacgcttagttgttgcttcctgagttccaaagtccgacagacagagcaggtcctccattcttgcccctttttaccccaaatgctcattggcattcttgcagctacgagtaataattaaaagtggctaagccaggctggcatggttgctcacgcctgtaatatcagcactttgggaggctgaggcaggaggatcacttgaacccaggagtgagaccagccagggcaacatagcaacaccctgtctctaattattattatttttttaagtgagtaagccaaataggggtttacttttcatctagaacaagaagacgtgttggccaggctggtctcaaactactgggctcaagtgatccacccacctcagcctcccaaagtgttgggattatgcgtgagccaccgcacctggccacaagacccaatttcttttattttatctttttttttttttttttaagagatagggcatctaacggcattgttttagctgctcaacacttttttttttttgcttatttttgtttgttttgtttgtttttgagacagggtctccctctgttgcccagcatatagtgcagtggcatgatcatggctcactgcagcctcaacctcccaggatcaggcaatcctcctgcttcagcttcctgagtagctgagaccacaggtgcacaccaatatacctaatttttttttttttgagatggagtttcactcttgttgcccaggctggagtgcaatggcgtggtctcagctcactgcaacctctgcctccctggttcaagcgattctcctgtctcagcctgccgagtagctggggttacaggcataagccactacgcccagctaattttgtatttttagtagagacagggtttctccatgttggtcaggctggtctcgaactcctgacctcaggtgatccacccacctcagccttccaaagtgctgagattgcaggtgtgaaccactacgcctggccacctgactaatttttaagttattcacagagaacaggttttgcaatgttgcccaggctggtctcaaactcctgggctcaaatgatcctcctccctcggcctcccaaagtgctggggttacaggtgtgccactgtgcctggtcggctcaccactttcagatctggctctcttcacctctcttttatagtcataagctgattagcacaattctagacatccgcagctacatttaaggcaggaaggaggtggtaatagacactaccagccacatctgtcccttttaatcaggataccctagaaatcctcagcagactttgaattatgtgccattggtgaaatgtcatatgatcatccctctacaaggcaacgaggtaaaaagagaatttagtatttctagcctctagagtggagatgaacaaagaataggaatgggcatttgcttaggaaaccaactgtgccttacaacatttttgcacttttttctgtaacattttgtgttaaatcatataaaaatgctgatcctaacaaatatggtcaatgagtcacaccataattctctaagaactccagtccaaaaaggttaatcttgcttttaaactccaggcgcggtgtttcacagctgtaattttagcacttcgggaggcagagcaagaggatcacttgaggccaggagttggagaccagcctggcaacatagcaagaccccgtctctacaaaaaataaaattatctgggcctgttggtgcacacctgtagtcccagctactcaggaggctgaggtgggaggatcacttgagcctaggaattcgaggctgcagtgagctgtgattgcaccactgcactccagcctgggtgacagagggagaacctatctccaaaacaaaacaaaataaaaacaaaacaaaactccaagcagagaaagacttgacgagtcggatgagtctgatgattcctaaaggaaatcctttttgagattccaggagattccatctcctcaacagagtaattgattttgagcctcccacctcctgaattaaggcccacccatccctatcctgcactgaactgtagactcttttttacttccttacaaaagtttattcttaaatgtacaacagactccaagacgacactttattgtagctataggtggcaaaagatgttatggcagagaatccagatgtttaaataggaatggggtcaagggtcaccgccccaagcacggataacaaaatttattttttgccagatttctttaattccacctgtgactggtgagggctggtggcggggtggctttcacttttagctcctctttttgtttctgcttgaacgtcccatcttccttacccacccccttgacctgcttcttgagctttctcagggcttcttgccacctttgcagctgtacatggcacctgccatagggctctaattttaaactgagaaattgagaaaacaggaaactgactctttttggggggagagtaagacaaacaggaaaaggaaaatgaagacgtggttgatacagatcgttggatttcaaaaggaaaagtctacggataaccgaaaaaaataaatatttagaaatgcatagtcttggctggttaaataagtatccatgcttgttcttgtggcatagtagttacgagacatttttagttaaatggaaaaatgtgaattactatagtttgagtgatatgctgctttccaaattaaaagcagcataacaaaaacattcccctaatactcataaataattcattgaattggcaataattcacctcctaatgacttcatatgaagtataaagtaacttcgatacatcagaagaaatcctatcttctaatataagaaagtaatatgattacattaaatgcgtctcatataagttataaaaatggtatctatgagtaaagaaatgcttgtgaacaaaaaaattgatcttataaaggtcaaacaggccaggcgtggtggctcacacctgtaatcccagcactttgggaggctgaggtgggcggagtacctgaggtcaggagttcaagaccagcctggccaacatggtgataccctgtctctacaaaaatacaaaaaattagctgggcatgatggtgggtgcctgtaatctcagctactcgggaggcagaggcgggagaatcgcttgaacccgggaggcggaggttgcagtgaactgagattgagccacaacaaccaagcctgggagacagaggaaactctgtctcaaaaaataaaaaataaaaattaaaattaaaaaaaaggtcaaacaaaccaaacccttctgattaatttattcaatctacttttattataagcaaatgagaaattataattttaatctgaaaaagcagaatcaggggattttggagctggacagtcccctggaaattatttggatcaaagccctcattttataggtgaagaaactgagaagtaagatttgagcaagctgcccaaaggctttgccaaaggctataccagtgaatggcagagtctggactggaagtcccagtgctgccgtccaggtgagacctgttccactgcatgctactagctcccgggctgagaccggacttttgcttggcaggtttctttctttcgaaactattaattattgtattttttgtagagacagggttttgccatgatgcccaggctggtcttgaactcctgagctcaagagatccacccagcttggcctctcaaaaatgttgggattacaggcataagccacagtgcccggcccattttcctcccacctctttgttccttctctgtttcttttgcagcattatgttctatcattgtataccagagttcctcaacttcagttatagtctgttcttgctttatgctatcttcttcagcaagctcatcttggtctgttttcctccttatcaggcataccccagaaactcctgttttatctccacctcaactaaacattttcctgagttctgggcctctataaactaattatttgattaacatcttttttttttttttctgagatagagtctctctctgtcacccaggctggagtgcagtggtgcaatctcagatcactgcagcttctgcctcccagattcaagcgattctcctgcctcagcctcctaagtagctgggattataggcatgcaccaccgcacacagctaatttttgtacttttagtagagacggggtttcaccatgttggtcaggctggtctcaaactcctgatctgaagtgatctgactgcctcagcttcccaaagtgctgggattacaagcctgagccaccatgcctggccaacatctttaattggatatctcagtatcaagaaggcccataatattcctctgcctcatccctctcctcagtcctcttcttgtgtttcctagttcagagaatggcaccattctctatcaagctgcgcaaatcagacatgtgtgattttttgttgttgttgagacagggactcactctgtcacccaggctagagtgcagtggcgtgatcatggcgcactgaagcctcaaactcctgggctcaggagatcctcccgcctcagcctcctgagtagctgggaccacaggcccacaccaccatgcccagctaattttgtattctttgtagagatggggtttcatcatgtttgcccaggctggtctcgaactcctggactcaagcaatccacccacctcagcctcccaaagtgctgggattacaggcatgagccactgtgcccagctgaagtgtgatccttaacttcaccccttctcatgccctccatttccaatccatctccagtccagttgactccagctactcaattatttccacttatctcattccactacctttgaagctaccaccatctctaactacagtcatctcccaactaactggtctcctggcatctctctggttctcctccactaatttcaaaaaaagaaatttactgtgacagtgctcacaacactcccccttgctcttactaaagatgcttaccatagcctccaggtattgtatggcctgaggtctatctacatttccaggtgcaggacacaccatgtctccccactcccaaatttagtctccagactccatcctttttacagttctttaaaagcatcacaattcctccaaccactaggcatttgtatgtgctattccctctttccagaatgcaataccctccctctgcctagctagctaacttctatgtatctatgactgcagctcaaactttcctcatggactccctccacaagtgccaagcctgggccagattcttttgttatgtgctcacagaacgatgttccctttagcattcattgagtttgctgtttaattattcttgtcttgtttttgtttaattagtcctatctctaatactagacaaatgttccttaagatcacaggaaatataggactgtctctacataaaaactgttttatatccataatgcctaggacagtacctggcacacagtatatgctcaataaatttttgttgaatgaatgcaattatcattatattcctgatattagcaggtataatccagtttaagtttgggaacagaaagacaaaacggaccacatctaataaatccggtctcctttcttttattatttatttatttgagacagttttgctcttgttgcccaggctgcagtgcaatggcatgatcttggctcactgaaacctccgcctcccaagttcaagggattctccagcctcagcctcccaagtagctgggattacaggcatccaccaccacgcccagctaatttttttgtatttttagtagagatggggtttcaccatgttggccaggctggtctcgaactcctgacctcaggtgatccacccacctcagcctcccaaagtgttgggattacaggcgtgagccaccgtgcccggccaaggtctcctttcttttaatcaaactctcacctttggccattctgcagtcattcacccgacagtatttactgacggagtgaatacagagtgcttgattaatgttgctgctttgttattattattattattattgagatggagtcttgctctgttgcccaggctggagtgcagtggcgtgatctcggctcactgcaacctccgcctcccgggttcaagccattctcctgcctcagcctcccaagtagctgggactacaggcatgcaacaccacacctggctaatttttgtatttttagtagagacaaggtttcaccatattggccaggctggtcttgaactcctgacctcaggtgatctgcccacctcagcttcccaaagtgctgggattacaggcgtgagccaccatacccaacctaatgtttctgctttgaaatacaatttcaaaaagtcattaataggttgaaaacagcaagattttaaaagtattttaaaaagtgaaacagaagaatgcttacttcatttcacagagatagatttctcctttatgttatttctaaaaggagatggaattttgtttcattcatttctgcttatttggacaggccaaatatgaacagctgaacacgtcagcgttaccatgcatatgttacacagatgccatccttcttccatcagctctcatatgcaatacagaagtaaaaagaggttctctttatttttaaaaggtaaaaattgaaattcagtcacttaacacagaataaacaataattacaattacactggtaacaaaggacagcaagcatgttttctttgaaagcactgtatctggtttgtctccgtgcttggtcctagtatctggcatattttccccagagttttcttttcagtgggatgattatcttcggggcaaaaaagtttatcagactcaagttttagcagtacttattttattcatttatatacatgtaaccccatcctgtcttactccaatcttcttactgccttcctactgacacatatattatataacaccctccccaagttctatttacggttaaaaatttctttttttttttctttttttgagacagagtttcactctcgtcacccaggctggtgtgcaatggcgcagtctcggctcactgcaacctccgactccctggttcaagtgattctcctgtctcagcctcccgagtagctggaattacaggcgcccgccaccatgcccagctaatttttgtatttttagtagagacagtgtttcgccatgttggccaggctggtctcaaactcctgacctcaggtgatccacccgccttggcctctcaaagtgctgggattataggcgtaagccactgcgcccagcctacagttacgaatttctaaatggcacaaataaactcagctgttctcagtgcagacgtcaaatcctcactgtgctgaaacattttcctcagcttttgggaaataattacaatttaaacatacacagagaatgtttcttagacaaacataatacccgaggcttatctggtaaaaactaattgctctgtccttagcacaaaaaatatatatctttgtaaaatgagaagaaccaaagaatatttaaaacaaagaaggaagccacacgtactaattacacaagagactgactgacaaactggaattctccaaaacagattttcagcgaggcttctcatttcagagtccaggaaaaaaaaatcctaaaaaccccaaaggtatattatatgtgtgtatatatatttttattgtgttaaaaaacacaaaacataaaatttactgtcttatcaaaaggtatattttgtcgctcttccctttttttttttttttttttcccgagacagagtccagtctgtcgcccaggctgaagtgcagtggcatgatctcggctcactgcaacctgcatcttctgggctcaagcaatcctcccacctcagcctcctgagtagatggagctacaggcacgtgccactaggcccggctaatttttgtattttttgcagacagggttttgccatgttgcccgggctggtctttgttctcctaagagttgttttctccatgaaagttgataaataacatttagaaaatgaattattacaagagtaatgatatgtctcaatttattatatgaaattatcaacaactgcttttaatattcagatgtcaagaagatgaaaagcagaaatacattttgcaaacatgtagcactccataaatggaaatcatgtatttcctctaatatcccaatttttctatattgggatcttatatggctgtttctatatggctattttgtcccaacttgctgtacaagaattttccccagccaccttagaaaggttggatgtagttcactccaagtttgcagttcactccaagtgtttcagtaccacagaaagctccatggaagcctcaaatgtacgggctaggcaatagaagcagggaggtaggattaagaaattactggccaggtgtggtggctcaggcctgtaatcccagcacttcgagaggctgaggcagacagatggcttgagctcaagagtttgagatcagcctgagcaacatggcaaaactctgtctctacaaaaaatataaaaatcagccaggtatgttggtgtgcacctgtagtcccagctactggggaggttgaggcaggaggattgcttgagcccaggaggctgaggctgcagtgagccatgattgtgccactgcattccagcctggtcgactgtaagacaaaaaataagaaaataaaaaatttaccaatataaaatgctcaaacagctaacaaacatgttcaattccatttatagtcttttctttgagccatttaaacatagggctattttttttttttttttttgagatggagtttcactcttgttgcccaggctggagagcaatggcatgatctcggctcaccacaacctctgcctcctgggttcaagcgattctcctgcctcagcctcccgagcagctgggattacaggcatgtgccaccatgcctggctaattttgtatttttagtagagacgggattcctccatgttggtcagactggtcttgaactcccaacctcaggtgatctgcctgcctcaaccttccaaagtgctgggattacaggtgtgagccactgagattggctgccgttttgttttttaactccatatagtttctatagttcactgaaaactcaaagagatgacctataaatgtatgaataatgtatgatttcttacatcaattttctactagaaaaaaatcatacttttagaattggattttgtcttacagtcatctttattatactttataaatgagatttcatttatataaatcaggaagctaaactaaaatagaaacactagatttaaattctgatttgaatactctgatcaaaataacaaatctcacactgggaaaccatctatcagcaagcagagagctactgtgtgtccttccttagaagagtttgaacaccgagaacccacagcatatttgcagtacagtaacagcaattcctttgtcattatcacagaactttaattttcatatactttgctgggaccaaccaaaccatcccatatatataaccatatccatatatatatatatatatatcccacatatatatgggatggtatatatatacacatgtatatgtatgtgtgtgtgtatatatgtgtatatatgtatacacacacacacacacacatatatatatatatacacacacacacatatatatatggagagagagagagagacagtgtcttgctctgtcgcccaggctggagtgcagtggtacgatcttggctcattgcaacctccgcctcccaggctcaagcgattctcatgtctcagtctcccaagtagctgggattacaggtgtgcaccaccacaccaggctaaccattccatacattttatacaatcatttttaaaaagaagcatgaaccatttcggttttagagaattaagtttttttaaaaaagagactcttaaaaaaaagtcattatatgaataaaatctgctttgtgttaattccgacaaatcattccatcattgagtctgtcaccaattttttttttttgaaatggagtttcgctcttgttgcccaggctggagtgcaatggtacgatctcggctcactgcaaccgccgcctcccgggttcaagtgattctcctgcctcagcctcccgagtagctgggattacaggcatgcgccaccacgcctggctaattttgtattattagttgagacagggtttctccatgttggtcaggctggtctcgaactcctgacctcaagtgatccgctggccttggcctcccaaagtgctgggattacaggcgtgagccaccgtgcctggcccaattttttttttttaataacttgcacacttaacaatattttttatcttcttgggacaacattcttttctccacaaaaacccaattaaggacgttgtgccagtttactcctacttccttcctgttcactgagcttaaagtgggtataggcgagaatgccaaataatgtacataaaatgccaagggcctgattaatggacagtggatccttaaataaaacatatcctccgaataaagtaatgcagaacttgaagtgtccgaacatgttataggtgacaggtgaagtgttcccaatgatccaataaattgataagttcaccatgaaagctattactccagatagcagcaccataagcaaagcagaaactgaccagggaccaaatattcctccttctccaaacactggctcaaagaagggcacagcaaccagcaacatggcagatgacatcggagcctggtagtacagcagctgcattgagttcacttgtaattcatgctgtttggctcctacccacagcgtgagctggattctggtggagaaggttttctggtagcagaaggtctggatggctatgatcaccggcgtggtcatggccttggccagctgataggtgcctatggtgttgttctgcagagaaaggttagtgaagaccacaaagccacagaagctgagggccaggaggaggagcctggagggcggcagacttttgggggcaaagatgtccagcttctggcagatatacaagcccagccaggtgaccacgaagtgcaccagggtcaggctcatgttggggaagccgtggtacacataaatccatttgttgaggaacacaatgcagatggacaccagcaggttgaacaggagcccggcggcgattcgccagtggccccgcactcggtccaccagcaatgccatgatccccgcgaagctggggccgtctagcctcggaaggggcgccgggcctgtctccggctgcccttctactccaccgccgcgtcctcgcagacgccgacctcaccgtctgacccaggagtggcatgcacagatcaaccccgggcgagtagcactcttaacagaggacacacaccccgccgccgccctgtaagccagctaggac

SEQ ID NO: 12656 - RNA, 2505 nt, Homo sapiens
  source 1..2505: mol_type = other RNA
gatctcactttgttgcccaggctggagtgcagtggcaccatctaggcttactgcaacctccgcctcccaggttcaagcaattctcctgcctcagccacccgagtagctgggattacaggcgtgcaccaccacatcctgctaatttttgtatttttagtagagatggggtttctccatgttggccaggctggtcttgaactcctggcctcaagtgatccacccaccttggcagcccagagtgctgggattacaggcgtgagccactgggcgcagcccctctctggaatctctaaccccacaaaggcggaaattgcagagagaatgagcacaggctgcttccccaccaatggctaagcaggtcctgccagctcatgtctcctgccagctcatgtctcctgccagctcatgtctcctgccatgggggtcctgaggacatgcgtggcaagccccttgacagttgggaggatgggggtgagtgtcccgccccatccattgttctgtgccgagtaaaattgtgggactaagaggatgactccctgacatcctgagaacacccaacttttacagaaccatgagacgcaagtaggcaagatttctgaacaaagcaggggtgtgaagcagattgatgcaggtgctaggtgccctcctgcgtccctgagcctgtttctggccaaagctcacagagtacactgaaaacaaatggcacagctcacccatcacgtctgcttcccactaacaagcaagagtgccatgggatgaggtctcctaggccatgggcagaggcccctcaggggttcccaccatgcatggtcccctggagaagagcctgcaaggtggccgcgcccctgccctggctctcccagcccctgggctttgctgttctgcccactccaggacactgaggcctgctggagaggggggtaaaccctacctggggcaggcctcggggaagcctggcctcaggcttctcatgttgattgattcagagcaagtcaaatgcagcaggctcatccttgcttcagcttcaggtaggcctctttcttttccttttttgcaagaaatagattagatcccagtttgggtgcggatagcttgcgcctgtagtcccagcactttgggaggctgaggcgggcggatcacttgagctcaggagttcgagaccaacctggccaacatggtgaaaccccgtctctgtttcaactttaagcccacggcctttttgtacttgattaccaaaggaatttcatcaatttcttcaatattccacagtctcatggtcctatccttggaagcagacaggatccatttcttgttgttgctaatggcaacatccatcacccagtcattatggcccttcaaagagagcttccggtagccttctgctacatcccaaatagccacagtcctatcaaaccctccagaaatgagaaaagagctgtctctggcaaagtgacaggaactgacagaaccttcatggccctgcatcagagtcacacaggctccacagtttcgaaactcccctgtgtggacgttccatatttttaagtttttatcccaggagcttgtacacaggaaatggccactgaaggtaaaacagcagtttgagattgcattggaatgtgccttagtgatggtgagcagcgtggcctgggatgtaacatcccagatcttgatgcacctgtccaatgagacagaagccaccctctggctgtcggggtcaaagcagcatgacgtgatggaccttgtgtgatgatctttgatgacggaaacggtggtgatgttctcggcgtccattatgcagattccatgatccacgtcgaagcctgagaccacgtatttaccatcaggagaaaacttacaggagacgatgaaggtatcatacctgaccttccacagcagcttgcctgtctccaggtcccaggccctcactgtcttatcataggatgcggcaatgactctgctgctgtcgccggtgatgctgcactctacaacaggagctttgggcctgtgctcaaaatcgcgaaccacagaaccgtccaccggatcccacagcttcacagtgcagtcataggagccactgaggagctttgtgtcatccacacagaagtggcaggtgctcacagcgtgctcgtgcccactcagaattttaaatgggatcttggagagagggtcctggtcgccccagatcaatttctccggcacctggtgcttctcaggcaacagatgcggtggtggttccctgtccaaggccagggggtcgagggtggccagcaggtgcgtgtgcgggatcgacagcttgaagcggcctaaggccctcgccatggtcccccaggacagcttgccgggacaatactcgctggcgggggcggagggtggcggcaacttgcattccctgtcatgggctgtcggggagcaccgcggcggggaggccatctcgaagcccggtccgccggtggccgccgacaagcctggatgggaacggtggcgccgcgcgcccgcgcccgc

SEQ ID NO: 12657 - RNA, 3345 nt, Homo sapiens
  source 1..3345: mol_type = other RNA
gatctcactttgttgcccaggctggagtgcagtggcgcaatttccactcactgcaagctccgcctcctcggttcacgccattctcctgcctcaacctcatgagtagctgggactacaggcgccggccaccacgcccagctaattttgtatttttagtagagatggggtttcaccgtgttagccaggatggtctcgatctcctgaccttgtgatcctccctccttggcctcccaaagtgctggggttacaggcttgagccaccgcgcccggcctcagggtttcttttataactgtgatcaggaagatgtgcttttctttctacttggttaagcaactaatcaaactcagcacaacaaaacaaagattctccttttctcccaagaagttcaacagttctagcgttgtagaacatttcacaaataaaaccatcctagtttccttttcccataaacagttgaacacatcagtgtgataagatcacctcacactatttcttggcttaatgctagcattgcctcctgcatacagatttctcttacccttctagcagatttaattgcttcttcccctgtattcccacagcactgtatatactctattatagctagtttacgaataataatattaattctggaccataaaattgcaactggtcaatgcctggcatataatgaacactcaaatgaacaaggaattgaatcttgctttaatgaagtaagtcaagactaattatgtcagttccaatcttaagaacgtccttggcttttaatgaggggtcttcatctttgaacacagatttagtttcagacagtggtttttgctgcctgtaataactaaagtttgcaaaaaaattaattatttgaggacactatatttttaagaaatgaatttccttaaactattcctacaagggtaatatacagtaagtgaaaaaccactaacacggtagttctcatagtggttgcttttatgtatgcatacttaagataattttaagtggttagaataggtccagagaacacctatattctatggtgttgccatttaatgttttaattatttaaaatacttaaataatttaatatttaatttgaaaaattaaatactgagtttgttgtgggcaaattagtggtgataaaacattattaatctaaaatctgctcttaaaatttgttcagattatcattgactgattggccccgccctccccatattcactcataatatgatttgttattttgtgattcttgacagttaagaaagcaattttaatacctgaaatgcaagtctagctgtggcttcattttaagaatttggtaattttgtaaaagtgcttgaatgcttgttttaccattgttatatctcaattcttataagaccctcagcagaatcaatttacatgactggcagtactaagccactttaaaattattttaaataattttatttgcttgggttctacttgtttgggttttacatactactgtggcatccttcttttaaggatataaactataattagaaatgatatggaaaaaagtgactagaaaacaaatctgaaggcttttaaaaatttcagagtacattagtaaatgctttaaaagacaacccatccaataacatatatgcaagttaacactacaaattcaatgacataagaaaatagattggacttacttttacattcacctctacagatactctataatgaacacactagtatgatgataataaagcaatcaagaacaatttatctctcagtctgtgtatatgtgactatctacatatttatttcacacacacatgccaaatacccacataacttcaatcctatatccatttacctctcagagtgatttaaagtagccacagtggcacataaaaggaaaaaaataatgaattccaggcttcctagtaagtaaagccaaatcaaattgttcaagtgatactatagtgctatttttacaggaaaacacagatttctataatttctggtcatttacttcatcattaaagtactatttgccaatattggtttcacataatgacaataaaacattcttgacttatatactacatgaaaaaaatagattatgagcttattttttgaccagtcatcaaacatgttttcatttgaataaagaaaattcttccagtttaatatgtttatcaatttgttttttcaatgaaacaaagtaaatttacagtaaagttactggtctcaatataagtcttccaatcttcaaattcagccgaacagtacaaggattacaggagaaaaaaaaacacaattaatctcttgtggctatcattttaggggctggttttctcatattgctgaattctaccacaccctgtcgtatttccaaggtttggatggtgctttaaatctgaactgcctgagaagattcagaaagcctttgttcttgggcttacacagtaagcactttgcgtgattcctaatcacatttttatccagaacacagtgttacgggtcacatttttctcaataatgcttatattgattgatgctctataaatataaacatatttacatacagaatacacacactgacatgggggtatgaagttagccagccatccataggaagaatggaataaaaattgcaggaagggtagtgtatgataccaagcccgtacagactatagacgccaatcccaagactgctgaagcaagaacacttctctgatcacgaataattatcttcacagtctcacaaaacttgtcggactggggactgatcggggtgccatatctgcagtaggtcacgaagtgctcgcagttgttccacagcaggctgtagggggtaaagcccagcagcttttcagccctccgcgccacctcctcgttgagcagtgcctttttctggagggactcgtccaggtgattgaccaggatgttagctccgtaggcgaagtcctccactgtgtccacgcggatgctggccactttgacaataacgcccaggatgagacgcttgttggagaccaccttctgcgtgcgccccatgtcgtctgtcagggccaacaggatgtcgggcatcatgtgggcaacacggttgtctcctaggtagatgccatagtgggtcaggtgggtccggggcacctccagcacgtcgcctcggtggaaagagctggtttcataaaaactgttcctccctttgtcttcgcccgcggcgcccgaactaaagagcgtgaagttggagatgaggagcagcttctccagtagtaaagacaccacctccagcatggggttcttcatccctgagtagctggagagacctctggtttcccggaccgttaagaaaggtggctacattctgt

SEQ ID NO: 12658 - RNA, 3507 nt, Homo sapiens
  source 1..3507: mol_type = other RNA
gatctcactttgttgcccaggctggagtgcagtggcgcaatttccactcactgcaagctccgcctcctcggttcacgccattctcctgcctcaacctcatgagtagctgggactacaggcgccggccaccacgcccagctaattttgtatttttagtagagatggggtttcaccgtgttagccaggatggtctcgatctcctgaccttgtgatcctccctccttggcctcccaaagtgctggggttacaggcttgagccaccgcgcccggcctcagggtttcttttataactgtgatcaggaagatgtgcttttctttctacttggttaagcaactaatcaaactcagcacaacaaaacaaagattctccttttctcccaagaagttcaacagttctagcgttgtagaacatttcacaaataaaaccatcctagtttccttttcccataaacagttgaacacatcagtgtgataagatcacctcacactatttcttggcttaatgctagcattgcctcctgcatacagatttctcttacccttctagcagatttaattgcttcttcccctgtattcccacagcactgtatatactctattatagctagtttacgaataataatattaattctggaccataaaattgcaactggtcaatgcctggcatataatgaacactcaaatgaacaaggaattgaatcttgctttaatgaagtaagtcaagactaattatgtcagttccaatcttaagaacgtccttggcttttaatgaggggtcttcatctttgaacacagatttagtttcagacagtggtttttgctgcctgtaataactaaagtttgcaaaaaaattaattatttgaggacactatatttttaagaaatgaatttccttaaactattcctacaagggtaatatacagtaagtgaaaaaccactaacacggtagttctcatagtggttgcttttatgtatgcatacttaagataattttaagtggttagaataggtccagagaacacctatattctatggtgttgccatttaatgttttaattatttaaaatacttaaataatttaatatttaatttgaaaaattaaatactgagtttgttgtgggcaaattagtggtgataaaacattattaatctaaaatctgctcttaaaatttgttcagattatcattgactgattggccccgccctccccatattcactcataatatgatttgttattttgtgattcttgacagttaagaaagcaattttaatacctgaaatgcaagtctagctgtggcttcattttaagaatttggtaattttgtaaaagtgcttgaatgcttgttttaccattgttatatctcaattcttataagaccctcagcagaatcaatttacatgactggcagtactaagccactttaaaattattttaaataattttatttgcttgggttctacttgtttgggttttacatactactgtggcatccttcttttaaggatataaactataattagaaatgatatggaaaaaagtgactagaaaacaaatctgaaggcttttaaaaatttcagagtacattagtaaatgctttaaaagacaacccatccaataacatatatgcaagttaacactacaaattcaatgacataagaaaatagattggacttacttttacattcacctctacagatactctataatgaacacactagtatgatgataataaagcaatcaagaacaatttatctctcagtctgtgtatatgtgactatctacatatttatttcacacacacatgccaaatacccacataacttcaatcctatatccatttacctctcagagtgatttaaagtagccacagtggcacataaaaggaaaaaaataatgaattccaggcttcctagtaagtaaagccaaatcaaattgttcaagtgatactatagtgctatttttacaggaaaacacagatttctataatttctggtcatttacttcatcattaaagtactatttgccaatattggtttcacataatgacaataaaacattcttgacttatatactacatgaaaaaaatagattatgagcttattttttgaccagtcatcaaacatgttttcatttgaataaagaaaattcttccagtttaatatgtttatcaatttgttttttcaatgaaacaaagtaaatttacagtaaagttactggtctcaatataagtcttccaatcttcaaattcagccgaacagtacaaggattacaggagaaaaaaaaacacaattaatctcttgtggctatcattttaggggctggttttctcatattgctgaattctaccacaccctgtcgtatttccaaggtttggatggtgctttaaatctgaactgcctgagaagattcagaaagcctttgttcttgggcttacacagtaagcactttgcgtgattcctaatcacatttttatccagaacacagtgttacgggtcacatttttctcaataatgcttatattgattgatgctctataaatataaacatatttacatacagaatacacacactgacatgggggtatgaagttagccagccatccataggaagaatggaataaaaattgcaggaagggtagtgtatgataccaagcccgtacagactatagacgccaatcccaagactgctgaagcaagaacacttctctgatcacgaataattatcttcacagtctcacaaaacttgtcggactggggactgatcggggtgccatatctgcagtaggtcacgaagtgctcgcagttgttccacagcaggctgtagggggtaaagcccagcagcttttcagccctccgcgccacctcctcgttgagcagtgcctttttctggagggactcgtccaggtgattgaccaggatgttagctccgtaggcgaagtcctccactgtgtccacgcggatgctggccactttgacaataacgcccaggatgagacgcttgttggagaccaccttctgcgtgcgccccatgtcgtctgtcagggccaacaggatgtcgggcatcatgtgggcaacacggttgtctcctaggtagatgccatagtgggtcaggtgggtccggggcacctccagcacgtcgcctcggtggaaagagctggtttcataaaaactgttcctccctttgtcttcgcccgcggcgcccgaactaaagagcgtgaagttggagatgaggagcagcttctccagtagtaaagacaccacctccagcatggggttcttcatcctgcaggccaggtgaggtacggcgcaaagtacggccgctgaggagagaggaaggcaaaggaggacagcgaggcctggcgaccggctcagccaagccacaatggggaatgagacggataaggaaccggtggctgacggcggggacagtgagaccagtgctacaagcagccggagaaggagcgcacctgggggccgtgccgggggcagggccgcgcgcggtgctc

SEQ ID NO: 12659 - RNA, 1826 nt, Homo sapiens
  source 1..1826: mol_type = other RNA
gatctcactttgttgcccaggctggagtgcagtggtgcagtcttggctcactgcagcctgtcttctgggttaaaacgattctcctgcctcagcctccccagtagctgggatcataggcatgtgccaccacgcccagctaattattgtattttcagtagagaaggggtttcaccatgttggccaggctggtcttgaattcctggcctcaaatgatccacccacctcagcctcccaaagtgctggaattacaggtgtgagccaccaagcccagcctatatatatatatttaaagatgacaagaaattaacaactcagcattttgagaatggcatgtcaggttatcatgattagtacatgggcacctggctgtggctcatctactaccatattctttgttcttctagatccttcttggcttccatcttggcaactccaaaggcatggtggggaaaacagatgcagagatagatgcctatttctcctgcagtctctttcagcatagcaattaggcaagttatcaataagagtatataatctataacttatagtccacataaggcttcactcaatttgaaaaattgccagttctgtcaaatatgctaacactccaataaggtatttatgacacagaatctggacaagaaatgcttccgggtccctttgtgttcctttcattcctaggagagtagaaaaaatcactttgatgttgaagtcttctcccacttccacagcaagtcctttttgcttttcagcaacaataaaagcattgagaagtctagaatactctttgagattactataggagaatttatataagggagttaaactatataaagtccactgtttatgcagaaggaatgcaaccttttgagggtcaacatcttcctgcaactgcgaacactggggaattttccttcgaggtggagtcaggataaatgaactctgcttcctgaccgattctaatcgtttctgcagaggagtggcacctataaagtaatcttcaggtcttgaggatgcactaggagttgactctggtgcactgtaagaatccatggtctgtcaataaaatgccgtgatgacgctgtcacccattccggattcacgaatcattcttcaaaagtccggctccaaaactatgtggagactgaaatcccccagctctgcgaccctcgctcctgcggagtcagcttctgctcgcggagggggaagggcaaaaggacagtgcgtcccaacccgtccctctccagctgagcctgtcagagaccagcccagctctgaaatcaagccgttgagaaaagggaattcggccctccgccgcctcttcagtttaaaatcgtttcccgactcgctctgcggccccacgcaggaagcctccttggcgcctcgccgattccgtatcagtgaagcaactaaaattgccattttaactgagggcaaggccgagccacttaaccactatcgtcaacctttccaatcgtgctcggttgctcctcagttttcctaccggtgcgaagctttctctcaaatttccgcccgtagtaggcatggcggcggcacctcaccactgattcgttgaattccttcccggtaatcttgggcactagcgggcggagttgaagggcgcttggaccccagcggcgatctgtgtttgggttcgcgctctgggagaattttggctttgctcgccttcctctttcagaagactcgaaatcggccagcaggtctgcgagatttgaaacgcgactgttactccttgttttccggttctggccgcgggagcctctcgagaagcgtggaaagaggagaagggcgtataccttgtgacc

SEQ ID NO: 12660 - RNA, 1900 nt, Homo sapiens
  source 1..1900: mol_type = other RNA
gatctcactttgttgcccaggctggagtgcagtggtgcagtcttggctcactgcagcctgtcttctgggttaaaacgattctcctgcctcagcctccccagtagctgggatcataggcatgtgccaccacgcccagctaattattgtattttcagtagagaaggggtttcaccatgttggccaggctggtcttgaattcctggcctcaaatgatccacccacctcagcctcccaaagtgctggaattacaggtgtgagccaccaagcccagcctatatatatatatttaaagatgacaagaaattaacaactcagcattttgagaatggcatgtcaggttatcatgattagtacatgggcacctggctgtggctcatctactaccatattctttgttcttctagatccttcttggcttccatcttggcaactccaaaggcatggtggggaaaacagatgcagagatagatgcctatttctcctgcagtctctttcagcatagcaattaggcaagttatcaataagagtatataatctataacttatagtccacataaggcttcactcaatttgaaaaattgccagttctgtcaaatatgctaacactccaataaggtatttatgacacagaatctggacaagaaatgcttccgggtccctttgtgttcctttcattcctaggagagtagaaaaaatcactttgatgttgaagtcttctcccacttccacagcaagtcctttttgcttttcagcaacaataaaagcattgagaagtctagaatactctttgagattactataggagaatttatataagggagttaaactatataaagtccactgtttatgcagaaggaatgcaaccttttgagggtcaacatcttcctgcaactgcgaacactggggaattttccttcgaggtggagtcaggataaatgaactctgcttcctgaccgattctaatcgtttctgcagaggagtggcacctataaagtaatcttcaggtcttgaggatgcactaggagttgactctggtgcactgtaagaatccatggtctgtcaataaaatgccgtgatgacgctgtcacccattccggattcacgaatcattcttcaaaagtccggctccaaaactatgtggagactgaaatcccccaggaagacctccgctccctcagacgcggggcgggccctgcgacttcactctgggagggacatttccgctcacccagctctgcgaccctcgctcctgcggagtcagcttctgctcgcggagggggaagggcaaaaggacagtgcgtcccaacccgtccctctccagctgagcctgtcagagaccagcccagctctgaaatcaagccgttgagaaaagggaattcggccctccgccgcctcttcagtttaaaatcgtttcccgactcgctctgcggccccacgcaggaagcctccttggcgcctcgccgattccgtatcagtgaagcaactaaaattgccattttaactgagggcaaggccgagccacttaaccactatcgtcaacctttccaatcgtgctcggttgctcctcagttttcctaccggtgcgaagctttctctcaaatttccgcccgtagtaggcatggcggcggcacctcaccactgattcgttgaattccttcccggtaatcttgggcactagcgggcggagttgaagggcgcttggaccccagcggcgatctgtgtttgggttcgcgctctgggagaattttggctttgctcgccttcctctttcagaagactcgaaatcggccagcaggtctgcgagatttgaaacgcgactgttactccttgttttccggttctggccgcgggagcctctcgagaagcgtggaaagaggagaagggcgtataccttgtgacc

SEQ ID NO: 12661 - RNA, 2487 nt, Homo sapiens
  source 1..2487: mol_type = other RNA
gatctcactttgttgcccaggctggagtgcagtggtgcagtcttggctcactgcagcctgtcttctgggttaaaacgattctcctgcctcagcctccccagtagctgggatcataggcatgtgccaccacgcccagctaattattgtattttcagtagagaaggggtttcaccatgttggccaggctggtcttgaattcctggcctcaaatgatccacccacctcagcctcccaaagtgctggaattacaggtgtgagccaccaagcccagcctatatatatatatttaaagatgacaagaaattaacaactcagcattttgagaatggcatgtcaggttatcatgattagtacatgggcacctggctgtggctcatctactaccatattctttgttcttctagatccttcttggcttccatcttggcaactccaaaggcatggtggggaaaacagatgcagagatagatgcctatttctcctgcagtctctttcagcatagcaattaggcaagttatcaataagagtatataatctataacttatagtccacataaggcttcactcaatttgaaaaattgccagttctgtcaaatatgctaacactccaataaggtatttatgacacagaatctttatttttccatcagtatgtgctgaagctacagatgttgaaacacgaactaatcttgtggctgataaatgaattttgaaatgtctatggaaatgtgaataaaggcaatccatgaataggtcaacttcttcctgggtaacctccccaggtgttttgtggacactgtcccatagagcttttgcatcctctggatgtattgcgaaagaaatgtccagactttgagggctacagggtacagaccaaagaaattcagtagtagccacataatggtccattttgcatgcagtccacatggcagccatccaggaaagattaaatgcattgattgctaaaggactgaaataacagtcaaaggttttctgaaaccaagttccaattattgctgtgttagactctgctccatttgcaaggaataagggcagacaggtgaaatcttctgaaacagtctccagaagactgtctccaaatacacagcagaaccagccagtccacagcactttaccttctctattctcagatggcaattgagattttgacacaatccgagtgtggtggcatgcacctgcagtcccagctacttggaaggctaaggtggaaggatcacttgagcccaggagacagaggttgcagtcaaccaagatcgtgccactgtactccagcctggacaagaaatgcttccgggtccctttgtgttcctttcattcctaggagagtagaaaaaatcactttgatgttgaagtcttctcccacttccacagcaagtcctttttgcttttcagcaacaataaaagcattgagaagtctagaatactctttgagattactataggagaatttatataagggagttaaactatataaagtccactgtttatgcagaaggaatgcaaccttttgagggtcaacatcttcctgcaactgcgaacactggggaattttccttcgaggtggagtcaggataaatgaactctgcttcctgaccgattctaatcgtttctgcagaggagtggcacctataaagtaatcttcaggtcttgaggatgcactaggagttgactctggtgcactgtaagaatccatggtctgtcaataaaatgccgtgatgacgctgtcacccattccggattcacgaatcattcttcaaaagtccggctccaaaactatgtggagactgaaatcccccagctctgcgaccctcgctcctgcggagtcagcttctgctcgcggagggggaagggcaaaaggacagtgcgtcccaacccgtccctctccagctgagcctgtcagagaccagcccagctctgaaatcaagccgttgagaaaagggaattcggccctccgccgcctcttcagtttaaaatcgtttcccgactcgctctgcggccccacgcaggaagcctccttggcgcctcgccgattccgtatcagtgaagcaactaaaattgccattttaactgagggcaaggccgagccacttaaccactatcgtcaacctttccaatcgtgctcggttgctcctcagttttcctaccggtgcgaagctttctctcaaatttccgcccgtagtaggcatggcggcggcacctcaccactgattcgttgaattccttcccggtaatcttgggcactagcgggcggagttgaagggcgcttggaccccagcggcgatctgtgtttgggttcgcgctctgggagaattttggctttgctcgccttcctctttcagaagactcgaaatcggccagcaggtctgcgagatttgaaacgcgactgttactccttgttttccggttctggccgcgggagcctctcgagaagcgtggaaagaggagaagggcgtataccttgtgacc

SEQ ID NO: 12662 - RNA, 2471 nt, Homo sapiens
  source 1..2471: mol_type = other RNA
gatctcactttgttgcccaggctggagtgcagtggtgcagtcttggctcactgcagcctgtcttctgggttaaaacgattctcctgcctcagcctccccagtagctgggatcataggcatgtgccaccacgcccagctaattattgtattttcagtagagaaggggtttcaccatgttggccaggctggtcttgaattcctggcctcaaatgatccacccacctcagcctcccaaagtgctggaattacaggtgtgagccaccaagcccagcctatatatatatatttaaagatgacaagaaattaacaactcagcattttgagaatggcatgtcaggttatcatgattagtacatgggcacctggctgtggctcatctactaccatattctttgttcttctagatccttcttggcttccatcttggcaactccaaaggcatggtggggaaaacagatgcagagatagatgcctatttctcctgcagtctctttcagcatagcaattaggcaagttatcaataagagtatataatctataacttatagtccacataaggcttcactcaatttgaaaaattgccagttctgtcaaatatgctaacactccaataaggtatttatgacacagaatctttatttttccatcagtatgtgctgaagctacagatgttgaaacacgaactaatcttgtggctgataaatgaattttgaaatgtctatggaaatgtgaataaaggcaatccatgaataggtcaacttcttcctgggtaacctccccaggtgttttgtggacactgtcccatagagcttttgcatcctctggatgtattgcgaaagaaatgtccagactttgagggctacagggtacagaccaaagaaattcagtagtagccacataatggtccattttgcatgcagtccacatggcagccatccaggaaagattaaatgcattgattgctaaaggactgaaataacagtcaaaggttttctgaaaccaagttccaattattgctgtgttagactctgctccatttgcaaggaataagggcagacaggtgaaatcttctgaaacagtctccagaagactgtctccaaatacacagcagaaccagccagtccacagcactttaccttctctattctcagatggcaattgagattttgacacaatccgagtgtggtggcatgcacctgcagtcccagctacttggaaggctaaggtggaaggatcacttgagcccaggagacagaggttgcagtcaaccaagatcgtgccactgtactccagcctggacaagaaatgcttccgggtccctttgtgttcctttcattcctgcaactgcgaacactggggaattttccttcgaggtggagtcaggataaatgaactctgcttcctgaccgattctaatcgtttctgcagaggagtggcacctataaagtaatcttcaggtcttgaggatgcactaggagttgactctggtgcactgtaagaatccatggtctgtcaataaaatgccgtgatgacgctgtcacccattccggattcacgaatcattcttcaaaagtccggctccaaaactatgtggagactgaaatcccctgaagaaaaaaaaaaaaaaccgccaaaatgacagctaagacagaggccagactaacccctggccctcccaaattccctctcgctccacaagtgggttcacaagagacacaaacgcacccaggaagacctccgctccctcagacgcggggcgggccctgcgacttcactctgggagggacatttccgctcacccagctctgcgaccctcgctcctgcggagtcagcttctgctcgcggagggggaagggcaaaaggacagtgcgtcccaacccgtccctctccagctgagcctgtcagagaccagcccagctctgaaatcaagccgttgagaaaagggaattcggccctccgccgcctcttcagtttaaaatcgtttcccgactcgctctgcggccccacgcaggaagcctccttggcgcctcgccgattccgtatcagtgaagcaactaaaattgccattttaactgagggcaaggccgagccacttaaccactatcgtcaacctttccaatcgtgctcggttgctcctcagttttcctaccggtgcgaagctttctctcaaatttccgcccgtagtaggcatggcggcggcacctcaccactgattcgttgaattccttcccggtaatcttgggcactagcgggcggagttgaagggcgcttggaccccagcggcgatctgtgtttgggttcgcgctctgggagaattttggctttgctcgccttcctctttcagaagactcgaaatcggccagcaggtctgcgagatttgaaacgcgactgttactccttgttttccggttctggccgcgggagcctctcgagaagcgtggaaagaggagaagggcgtataccttgtgacc

SEQ ID NO: 12663 - RNA, 2581 nt, Homo sapiens
  source 1..2581: mol_type = other RNA
gatctcactttgttgcccaggctggagtgcagtggtgcagtcttggctcactgcagcctgtcttctgggttaaaacgattctcctgcctcagcctccccagtagctgggatcataggcatgtgccaccacgcccagctaattattgtattttcagtagagaaggggtttcaccatgttggccaggctggtcttgaattcctggcctcaaatgatccacccacctcagcctcccaaagtgctggaattacaggtgtgagccaccaagcccagcctatatatatatatttaaagatgacaagaaattaacaactcagcattttgagaatggcatgtcaggttatcatgattagtacatgggcacctggctgtggctcatctactaccatattctttgttcttctagatccttcttggcttccatcttggcaactccaaaggcatggtggggaaaacagatgcagagatagatgcctatttctcctgcagtctctttcagcatagcaattaggcaagttatcaataagagtatataatctataacttatagtccacataaggcttcactcaatttgaaaaattgccagttctgtcaaatatgctaacactccaataaggtatttatgacacagaatctttatttttccatcagtatgtgctgaagctacagatgttgaaacacgaactaatcttgtggctgataaatgaattttgaaatgtctatggaaatgtgaataaaggcaatccatgaataggtcaacttcttcctgggtaacctccccaggtgttttgtggacactgtcccatagagcttttgcatcctctggatgtattgcgaaagaaatgtccagactttgagggctacagggtacagaccaaagaaattcagtagtagccacataatggtccattttgcatgcagtccacatggcagccatccaggaaagattaaatgcattgattgctaaaggactgaaataacagtcaaaggttttctgaaaccaagttccaattattgctgtgttagactctgctccatttgcaaggaataagggcagacaggtgaaatcttctgaaacagtctccagaagactgtctccaaatacacagcagaaccagccagtccacagcactttaccttctctattctcagatggcaattgagattttgacacaatccgagtgtggtggcatgcacctgcagtcccagctacttggaaggctaaggtggaaggatcacttgagcccaggagacagaggttgcagtcaaccaagatcgtgccactgtactccagcctgggtgacaaaatgagaccctggacaagaaatgcttccgggtccctttgtgttcctttcattcctaggagagtagaaaaaatcactttgatgttgaagtcttctcccacttccacagcaagtcctttttgcttttcagcaacaataaaagcattgagaagtctagaatactctttgagattactataggagaatttatataagggagttaaactatataaagtccactgtttatgcagaaggaatgcaaccttttgagggtcaacatcttcctgcaactgcgaacactggggaattttccttcgaggtggagtcaggataaatgaactctgcttcctgaccgattctaatcgtttctgcagaggagtggcacctataaagtaatcttcaggtcttgaggatgcactaggagttgactctggtgcactgtaagaatccatggtctgtcaataaaatgccgtgatgacgctgtcacccattccggattcacgaatcattcttcaaaagtccggctccaaaactatgtggagactgaaatcccccaggaagacctccgctccctcagacgcggggcgggccctgcgacttcactctgggagggacatttccgctcacccagctctgcgaccctcgctcctgcggagtcagcttctgctcgcggagggggaagggcaaaaggacagtgcgtcccaacccgtccctctccagctgagcctgtcagagaccagcccagctctgaaatcaagccgttgagaaaagggaattcggccctccgccgcctcttcagtttaaaatcgtttcccgactcgctctgcggccccacgcaggaagcctccttggcgcctcgccgattccgtatcagtgaagcaactaaaattgccattttaactgagggcaaggccgagccacttaaccactatcgtcaacctttccaatcgtgctcggttgctcctcagttttcctaccggtgcgaagctttctctcaaatttccgcccgtagtaggcatggcggcggcacctcaccactgattcgttgaattccttcccggtaatcttgggcactagcgggcggagttgaagggcgcttggaccccagcggcgatctgtgtttgggttcgcgctctgggagaattttggctttgctcgccttcctctttcagaagactcgaaatcggccagcaggtctgcgagatttgaaacgcgactgttactccttgttttccggttctggccgcgggagcctctcgagaagcgtggaaagaggagaagggcgtataccttgtgacc

SEQ ID NO: 12664 - RNA, 2157 nt, Homo sapiens
  source 1..2157: mol_type = other RNA
gatctcactttgttgcccaggctggagtgcagtggtgcagtcttggctcactgcagcctgtcttctgggttaaaacgattctcctgcctcagcctccccagtagctgggatcataggcatgtgccaccacgcccagctaattattgtattttcagtagagaaggggtttcaccatgttggccaggctggtcttgaattcctggcctcaaatgatccacccacctcagcctcccaaagtgctggaattacaggtgtgagccaccaagcccagcctatatatatatatttaaagatgacaagaaattaacaactcagcattttgagaatggcatgtcaggttatcatgattagtacatgggcacctggctgtggctcatctactaccatattctttgttcttctagatccttcttggcttccatcttggcaactccaaaggcatggtggggaaaacagatgcagagatagatgcctatttctcctgcagtctctttcagcatagcaattaggcaagttatcaataagagtatataatctataacttatagtccacataaggcttcactcaatttgaaaaattgccagttctgtcaaatatgctaacactccaataaggtatttatgacacagaatctttatttttccatcagtatgtgctgaagctacagatgttgaaacacgaactaatcttgtggctgataaatgaattttgaaatgtctatggaaatgtgaataaaggcaatccatgaataggtcaacttcttcctgggtaacctccccaggtgttttgtggacactgtcccatagagcttttgcatcctctggatgtattgcgaaagaaatgtccagactttgagggctacagggtacagaccaaagaaattcagtagtagccacataatggtccattttgcatgcagtccacatggcagccatccaggaaagattaaatgcattgattgctaaaggactgaaataacagtcaaaggttttctgaaaccaagttccaattattgctgtgttagactctgctccatttgcaaggaataagggcagacaggtgaaatcttctgaaacagtctccagaagactgtctccaaatacacagcagaaccagccagtccacagcactttaccttctctattctcagatggcaattgagattttgacacaatccgagtgtggtggcatgcacctgcagtcccagctacttggaaggctaaggtggaaggatcacttgagcccaggagacagaggttgcagtcaaccaagatcgtgccactgtactccagcctgggtgacaaaatgagaccctggacaagaaatgcttccgggtccctttgtgttcctttcattcctaggagagtagaaaaaatcactttgatgttgaagtcttctcccacttccacagcaagtcctttttgcttttcagcaacaataaaagcattgagaagtctagaatactctttgagattactataggagaatttatataagggagttaaactatataaagtccactgtttatgcagaaggaatgcaaccttttgagggtcaacatcttcctgcaactgcgaacactggggaattttccttcgaggtggagtcaggataaatgaactctgcttcctgaccgattctaatcgtttctgcagaggagtggcacctataaagtaatcttcaggtcttgaggatgcactaggagttgactctggtgcactgtaagaatccatggtctgtcaataaaatgccgtgatgacgctgtcacccattccggattcacgaatcattcttcaaaagtccggctccaaaactatgtggagactgaaatccccggtgcgaagctttctctcaaatttccgcccgtagtaggcatggcggcggcacctcaccactgattcgttgaattccttcccggtaatcttgggcactagcgggcggagttgaagggcgcttggaccccagcggcgatctgtgtttgggttcgcgctctgggagaattttggctttgctcgccttcctctttcagaagactcgaaatcggccagcaggtctgcgagatttgaaacgcgactgttactccttgttttccggttctggccgcgggagcctctcgagaagcgtggaaagaggagaagggcgtataccttgtgacc

SEQ ID NO: 12665 - RNA, 2699 nt, Homo sapiens
  source 1..2699: mol_type = other RNA
gatctcactttgttgcccaggctggagtgcagtggtgcagtcttggctcactgcagcctgtcttctgggttaaaacgattctcctgcctcagcctccccagtagctgggatcataggcatgtgccaccacgcccagctaattattgtattttcagtagagaaggggtttcaccatgttggccaggctggtcttgaattcctggcctcaaatgatccacccacctcagcctcccaaagtgctggaattacaggtgtgagccaccaagcccagcctatatatatatatttaaagatgacaagaaattaacaactcagcattttgagaatggcatgtcaggttatcatgattagtacatgggcacctggctgtggctcatctactaccatattctttgttcttctagatccttcttggcttccatcttggcaactccaaaggcatggtggggaaaacagatgcagagatagatgcctatttctcctgcagtctctttcagcatagcaattaggcaagttatcaataagagtatataatctataacttatagtccacataaggcttcactcaatttgaaaaattgccagttctgtcaaatatgctaacactccaataaggtatttatgacacagaatctttatttttccatcagtatgtgctgaagctacagatgttgaaacacgaactaatcttgtggctgataaatgaattttgaaatgtctatggaaatgtgaataaaggcaatccatgaataggtcaacttcttcctgggtaacctccccaggtgttttgtggacactgtcccatagagcttttgcatcctctggatgtattgcgaaagaaatgtccagactttgagggctacagggtacagaccaaagaaattcagtagtagccacataatggtccattttgcatgcagtccacatggcagccatccaggaaagattaaatgcattgattgctaaaggactgaaataacagtcaaaggttttctgaaaccaagttccaattattgctgtgttagactctgctccatttgcaaggaataagggcagacaggtgaaatcttctgaaacagtctccagaagactgtctccaaatacacagcagaaccagccagtccacagcactttaccttctctattctcagatggcaattgagattttgacacaatccgagtgtggtggcatgcacctgcagtcccagctacttggaaggctaaggtggaaggatcacttgagcccaggagacagaggttgcagtcaaccaagatcgtgccactgtactccagcctgggtgacaaaatgagaccctggacaagaaatgcttccgggtccctttgtgttcctttcattcctaggagagtagaaaaaatcactttgatgttgaagtcttctcccacttccacagcaagtcctttttgcttttcagcaacaataaaagcattgagaagtctagaatactctttgagattactataggagaatttatataagggagttaaactatataaagtccactgtttatgcagaaggaatgcaaccttttgagggtcaacatcttcctgcaactgcgaacactggggaattttccttcgaggtggagtcaggataaatgaactctgcttcctgaccgattctaatcgtttctgcagaggagtggcacctataaagtaatcttcaggtcttgaggatgcactaggagttgactctggtgcactgtaagaatccatggtctgtcaataaaatgccgtgatgacgctgtcacccattccggattcacgaatcattcttcaaaagtccggctccaaaactatgtggagactgaaatcccctgaagaaaaaaaaaaaaaaccgccaaaatgacagctaagacagaggccagactaacccctggccctcccaaattccctctcgctccacaagtgggttcacaagagacacaaacgcacccaggaagacctccgctccctcagacgcggggcgggccctgcgacttcactctgggagggacatttccgctcacccagctctgcgaccctcgctcctgcggagtcagcttctgctcgcggagggggaagggcaaaaggacagtgcgtcccaacccgtccctctccagctgagcctgtcagagaccagcccagctctgaaatcaagccgttgagaaaagggaattcggccctccgccgcctcttcagtttaaaatcgtttcccgactcgctctgcggccccacgcaggaagcctccttggcgcctcgccgattccgtatcagtgaagcaactaaaattgccattttaactgagggcaaggccgagccacttaaccactatcgtcaacctttccaatcgtgctcggttgctcctcagttttcctaccggtgcgaagctttctctcaaatttccgcccgtagtaggcatggcggcggcacctcaccactgattcgttgaattccttcccggtaatcttgggcactagcgggcggagttgaagggcgcttggaccccagcggcgatctgtgtttgggttcgcgctctgggagaattttggctttgctcgccttcctctttcagaagactcgaaatcggccagcaggtctgcgagatttgaaacgcgactgttactccttgttttccggttctggccgcgggagcctctcgagaagcgtggaaagaggagaagggcgtataccttgtgacc

SEQ ID NO: 12666 - RNA, 2698 nt, Homo sapiens
  source 1..2698: mol_type = other RNA
gatctcactttgttgcccaggctggagtgcagtggtgcagtcttggctcactgcagcctgtcttctgggttaaaacgattctcctgcctcagcctccccagtagctgggatcataggcatgtgccaccacgcccagctaattattgtattttcagtagagaaggggtttcaccatgttggccaggctggtcttgaattcctggcctcaaatgatccacccacctcagcctcccaaagtgctggaattacaggtgtgagccaccaagcccagcctatatatatatatttaaagatgacaagaaattaacaactcagcattttgagaatggcatgtcaggttatcatgattagtacatgggcacctggctgtggctcatctactaccatattctttgttcttctagatccttcttggcttccatcttggcaactccaaaggcatggtggggaaaacagatgcagagatagatgcctatttctcctgcagtctctttcagcatagcaattaggcaagttatcaataagagtatataatctataacttatagtccacataaggcttcactcaatttgaaaaattgccagttctgtcaaatatgctaacactccaataaggtatttatgacacagaatctttatttttccatcagtatgtgctgaagctacagatgttgaaacacgaactaatcttgtggctgataaatgaattttgaaatgtctatggaaatgtgaataaaggcaatccatgaataggtcaacttcttcctgggtaacctccccaggtgttttgtggacactgtcccatagagcttttgcatcctctggatgtattgcgaaagaaatgtccagactttgagggctacagggtacagaccaaagaaattcagtagtagccacataatggtccattttgcatgcagtccacatggcagccatccaggaaagattaaatgcattgattgctaaaggactgaaataacagtcaaaggttttctgaaaccaagttccaattattgctgtgttagactctgctccatttgcaaggaataagggcagacaggtgaaatcttctgaaacagtctccagaagactgtctccaaatacacagcagaaccagccagtccacagcactttaccttctctattctcagatggcaattgagattttgacacaatccgagtgtggtggcatgcacctgcagtcccagctacttggaaggctaaggtggaaggatcacttgagcccaggagacagaggttgcagtcaaccaagatcgtgccactgtactccagcctgggtgacaaaatgagaccctggacaagaaatgcttccgggtccctttgtgttcctttcattcctaggagagtagaaaaaatcactttgatgttgaagtcttctcccacttccacagcaagtcctttttgcttttcagcaacaataaaagcattgagaagtctagaatactctttgagattactataggagaatttatataagggagttaaactatataaagtccactgtttatgcagaaggaatgcaaccttttgagggtcaacatcttcctgcaactgcgaacactggggaattttccttcgaggtggagtcaggataaatgaactctgcttcctgaccgattctaatcgtttctgcagaggagtggcacctataaagtaatcttcaggtcttgaggatgcactaggagttgactctggtgcactgtaagaatccatggtctgtctgtggtcccagctactcaggaggctgaagtaggactgcatgagcccaggaggtcaaggctgcagtgagatgtgatcatgccaccgaattccagcctgggtgacacagcaagaccctcaataaaatgccgtgatgacgctgtcacccattccggattcacgaatcattcttcaaaagtccggctccaaaactatgtggagactgaaatcccccaggaagacctccgctccctcagacgcggggcgggccctgcgacttcactctgggagggacatttccgctcacccagctctgcgaccctcgctcctgcggagtcagcttctgctcgcggagggggaagggcaaaaggacagtgcgtcccaacccgtccctctccagctgagcctgtcagagaccagcccagctctgaaatcaagccgttgagaaaagggaattcggccctccgccgcctcttcagtttaaaatcgtttcccgactcgctctgcggccccacgcaggaagcctccttggcgcctcgccgattccgtatcagtgaagcaactaaaattgccattttaactgagggcaaggccgagccacttaaccactatcgtcaacctttccaatcgtgctcggttgctcctcagttttcctaccggtgcgaagctttctctcaaatttccgcccgtagtaggcatggcggcggcacctcaccactgattcgttgaattccttcccggtaatcttgggcactagcgggcggagttgaagggcgcttggaccccagcggcgatctgtgtttgggttcgcgctctgggagaattttggctttgctcgccttcctctttcagaagactcgaaatcggccagcaggtctgcgagatttgaaacgcgactgttactccttgttttccggttctggccgcgggagcctctcgagaagcgtggaaagaggagaagggcgtataccttgtgacc

SEQ ID NO: 12667 - RNA, 2487 nt, Homo sapiens
  source 1..2487: mol_type = other RNA
gatctcactttgttgcccaggctggagtgcagtggtgcagtcttggctcactgcagcctgtcttctgggttaaaacgattctcctgcctcagcctccccagtagctgggatcataggcatgtgccaccacgcccagctaattattgtattttcagtagagaaggggtttcaccatgttggccaggctggtcttgaattcctggcctcaaatgatccacccacctcagcctcccaaagtgctggaattacaggtgtgagccaccaagcccagcctatatatatatatttaaagatgacaagaaattaacaactcagcattttgagaatggcatgtcaggttatcatgattagtacatgggcacctggctgtggctcatctactaccatattctttgttcttctagatccttcttggcttccatcttggcaactccaaaggcatggtggggaaaacagatgcagagatagatgcctatttctcctgcagtctctttcagcatagcaattaggcaagttatcaataagagtatataatctataacttatagtccacataaggcttcactcaatttgaaaaattgccagttctgtcaaatatgctaacactccaataaggtatttatgacacagaatctttatttttccatcagtatgtgctgaagctacagatgttgaaacacgaactaatcttgtggctgataaatgaattttgaaatgtctatggaaatgtgaataaaggcaatccatgaataggtcaacttcttcctgggtaacctccccaggtgttttgtggacactgtcccatagagcttttgcatcctctggatgtattgcgaaagaaatgtccagactttgagggctacagggtacagaccaaagaaattcagtagtagccacataatggtccattttgcatgcagtccacatggcagccatccaggaaagattaaatgcattgattgctaaaggactgaaataacagtcaaaggttttctgaaaccaagttccaattattgctgtgttagactctgctccatttgcaaggaataagggcagacaggtgaaatcttctgaaacagtctccagaagactgtctccaaatacacagcagaaccagccagtccacagcactttaccttctctattctcagatggcaattgagattttgacacaatctgcagtcccagctacttggaaggctaaggtggaaggatcacttgagcccaggagacagaggttgcagtcaaccaagatcgtgccactgtactccagcctgggtgacaaaatgagaccctggacaagaaatgcttccgggtccctttgtgttcctttcattcctaggagagtagaaaaaatcactttgatgttgaagtcttctcccacttccacagcaagtcctttttgcttttcagcaacaataaaagcattgagaagtctagaatactctttgagattactataggagaatttatataagggagttaaactatataaagtccactgtttatgcagaaggaatgcaaccttttgagggtcaacatcttcctgcaactgcgaacactggggaattttccttcgaggtggagtcaggataaatgaactctgcttcctgaccgattctaatcgtttctgcagaggagtggcacctataaagtaatcttcaggtcttgaggatgcactaggagttgactctggtgcactgtaagaatccatggtctgtcaataaaatgccgtgatgacgctgtcacccattccggattcacgaatcattcttcaaaagtccggctccaaaactatgtggagactgaaatcccccagctctgcgaccctcgctcctgcggagtcagcttctgctcgcggagggggaagggcaaaaggacagtgcgtcccaacccgtccctctccagctgagcctgtcagagaccagcccagctctgaaatcaagccgttgagaaaagggaattcggccctccgccgcctcttcagtttaaaatcgtttcccgactcgctctgcggccccacgcaggaagcctccttggcgcctcgccgattccgtatcagtgaagcaactaaaattgccattttaactgagggcaaggccgagccacttaaccactatcgtcaacctttccaatcgtgctcggttgctcctcagttttcctaccggtgcgaagctttctctcaaatttccgcccgtagtaggcatggcggcggcacctcaccactgattcgttgaattccttcccggtaatcttgggcactagcgggcggagttgaagggcgcttggaccccagcggcgatctgtgtttgggttcgcgctctgggagaattttggctttgctcgccttcctctttcagaagactcgaaatcggccagcaggtctgcgagatttgaaacgcgactgttactccttgttttccggttctggccgcgggagcctctcgagaagcgtggaaagaggagaagggcgtataccttgtgacc

SEQ ID NO: 12668 - RNA, 2369 nt, Homo sapiens
  source 1..2369: mol_type = other RNA
gatctcactttgttgcccaggctggagtgcagtggtgcagtcttggctcactgcagcctgtcttctgggttaaaacgattctcctgcctcagcctccccagtagctgggatcataggcatgtgccaccacgcccagctaattattgtattttcagtagagaaggggtttcaccatgttggccaggctggtcttgaattcctggcctcaaatgatccacccacctcagcctcccaaagtgctggaattacaggtgtgagccaccaagcccagcctatatatatatatttaaagatgacaagaaattaacaactcagcattttgagaatggcatgtcaggttatcatgattagtacatgggcacctggctgtggctcatctactaccatattctttgttcttctagatccttcttggcttccatcttggcaactccaaaggcatggtggggaaaacagatgcagagatagatgcctatttctcctgcagtctctttcagcatagcaattaggcaagttatcaataagagtatataatctataacttatagtccacataaggcttcactcaatttgaaaaattgccagttctgtcaaatatgctaacactccaataaggtatttatgacacagaatctttatttttccatcagtatgtgctgaagctacagatgttgaaacacgaactaatcttgtggctgataaatgaattttgaaatgtctatggaaatgtgaataaaggcaatccatgaataggtcaacttcttcctgggtaacctccccaggtgttttgtggacactgtcccatagagcttttgcatcctctggatgtattgcgaaagaaatgtccagactttgagggctacagggtacagaccaaagaaattcagtagtagccacataatggtccattttgcatgcagtccacatggcagccatccaggaaagattaaatgcattgattgctaaaggactgaaataacagtcaaaggttttctgaaaccaagttccaattattgctgtgttagactctgctccatttgcaaggaataagggcagacaggtgaaatcttctgaaacagtctccagaagactgtctccaaatacacagcagaaccagccagtccacagcactttaccttctctattctcagatggcaattgagattttgacacaatctggacaagaaatgcttccgggtccctttgtgttcctttcattcctaggagagtagaaaaaatcactttgatgttgaagtcttctcccacttccacagcaagtcctttttgcttttcagcaacaataaaagcattgagaagtctagaatactctttgagattactataggagaatttatataagggagttaaactatataaagtccactgtttatgcagaaggaatgcaaccttttgagggtcaacatcttcctgcaactgcgaacactggggaattttccttcgaggtggagtcaggataaatgaactctgcttcctgaccgattctaatcgtttctgcagaggagtggcacctataaagtaatcttcaggtcttgaggatgcactaggagttgactctggtgcactgtaagaatccatggtctgtcaataaaatgccgtgatgacgctgtcacccattccggattcacgaatcattcttcaaaagtccggctccaaaactatgtggagactgaaatcccccagctctgcgaccctcgctcctgcggagtcagcttctgctcgcggagggggaagggcaaaaggacagtgcgtcccaacccgtccctctccagctgagcctgtcagagaccagcccagctctgaaatcaagccgttgagaaaagggaattcggccctccgccgcctcttcagtttaaaatcgtttcccgactcgctctgcggccccacgcaggaagcctccttggcgcctcgccgattccgtatcagtgaagcaactaaaattgccattttaactgagggcaaggccgagccacttaaccactatcgtcaacctttccaatcgtgctcggttgctcctcagttttcctaccggtgcgaagctttctctcaaatttccgcccgtagtaggcatggcggcggcacctcaccactgattcgttgaattccttcccggtaatcttgggcactagcgggcggagttgaagggcgcttggaccccagcggcgatctgtgtttgggttcgcgctctgggagaattttggctttgctcgccttcctctttcagaagactcgaaatcggccagcaggtctgcgagatttgaaacgcgactgttactccttgttttccggttctggccgcgggagcctctcgagaagcgtggaaagaggagaagggcgtataccttgtgacc

SEQ ID NO: 12669 - RNA, 2443 nt, Homo sapiens
  source 1..2443: mol_type = other RNA
gatctcactttgttgcccaggctggagtgcagtggtgcagtcttggctcactgcagcctgtcttctgggttaaaacgattctcctgcctcagcctccccagtagctgggatcataggcatgtgccaccacgcccagctaattattgtattttcagtagagaaggggtttcaccatgttggccaggctggtcttgaattcctggcctcaaatgatccacccacctcagcctcccaaagtgctggaattacaggtgtgagccaccaagcccagcctatatatatatatttaaagatgacaagaaattaacaactcagcattttgagaatggcatgtcaggttatcatgattagtacatgggcacctggctgtggctcatctactaccatattctttgttcttctagatccttcttggcttccatcttggcaactccaaaggcatggtggggaaaacagatgcagagatagatgcctatttctcctgcagtctctttcagcatagcaattaggcaagttatcaataagagtatataatctataacttatagtccacataaggcttcactcaatttgaaaaattgccagttctgtcaaatatgctaacactccaataaggtatttatgacacagaatctttatttttccatcagtatgtgctgaagctacagatgttgaaacacgaactaatcttgtggctgataaatgaattttgaaatgtctatggaaatgtgaataaaggcaatccatgaataggtcaacttcttcctgggtaacctccccaggtgttttgtggacactgtcccatagagcttttgcatcctctggatgtattgcgaaagaaatgtccagactttgagggctacagggtacagaccaaagaaattcagtagtagccacataatggtccattttgcatgcagtccacatggcagccatccaggaaagattaaatgcattgattgctaaaggactgaaataacagtcaaaggttttctgaaaccaagttccaattattgctgtgttagactctgctccatttgcaaggaataagggcagacaggtgaaatcttctgaaacagtctccagaagactgtctccaaatacacagcagaaccagccagtccacagcactttaccttctctattctcagatggcaattgagattttgacacaatctggacaagaaatgcttccgggtccctttgtgttcctttcattcctaggagagtagaaaaaatcactttgatgttgaagtcttctcccacttccacagcaagtcctttttgcttttcagcaacaataaaagcattgagaagtctagaatactctttgagattactataggagaatttatataagggagttaaactatataaagtccactgtttatgcagaaggaatgcaaccttttgagggtcaacatcttcctgcaactgcgaacactggggaattttccttcgaggtggagtcaggataaatgaactctgcttcctgaccgattctaatcgtttctgcagaggagtggcacctataaagtaatcttcaggtcttgaggatgcactaggagttgactctggtgcactgtaagaatccatggtctgtcaataaaatgccgtgatgacgctgtcacccattccggattcacgaatcattcttcaaaagtccggctccaaaactatgtggagactgaaatcccccaggaagacctccgctccctcagacgcggggcgggccctgcgacttcactctgggagggacatttccgctcacccagctctgcgaccctcgctcctgcggagtcagcttctgctcgcggagggggaagggcaaaaggacagtgcgtcccaacccgtccctctccagctgagcctgtcagagaccagcccagctctgaaatcaagccgttgagaaaagggaattcggccctccgccgcctcttcagtttaaaatcgtttcccgactcgctctgcggccccacgcaggaagcctccttggcgcctcgccgattccgtatcagtgaagcaactaaaattgccattttaactgagggcaaggccgagccacttaaccactatcgtcaacctttccaatcgtgctcggttgctcctcagttttcctaccggtgcgaagctttctctcaaatttccgcccgtagtaggcatggcggcggcacctcaccactgattcgttgaattccttcccggtaatcttgggcactagcgggcggagttgaagggcgcttggaccccagcggcgatctgtgtttgggttcgcgctctgggagaattttggctttgctcgccttcctctttcagaagactcgaaatcggccagcaggtctgcgagatttgaaacgcgactgttactccttgttttccggttctggccgcgggagcctctcgagaagcgtggaaagaggagaagggcgtataccttgtgacc

SEQ ID NO: 12670 - RNA, 2019 nt, Homo sapiens
  source 1..2019: mol_type = other RNA
gatctcactttgttgcccaggctggagtgcagtggtgcagtcttggctcactgcagcctgtcttctgggttaaaacgattctcctgcctcagcctccccagtagctgggatcataggcatgtgccaccacgcccagctaattattgtattttcagtagagaaggggtttcaccatgttggccaggctggtcttgaattcctggcctcaaatgatccacccacctcagcctcccaaagtgctggaattacaggtgtgagccaccaagcccagcctatatatatatatttaaagatgacaagaaattaacaactcagcattttgagaatggcatgtcaggttatcatgattagtacatgggcacctggctgtggctcatctactaccatattctttgttcttctagatccttcttggcttccatcttggcaactccaaaggcatggtggggaaaacagatgcagagatagatgcctatttctcctgcagtctctttcagcatagcaattaggcaagttatcaataagagtatataatctataacttatagtccacataaggcttcactcaatttgaaaaattgccagttctgtcaaatatgctaacactccaataaggtatttatgacacagaatctttatttttccatcagtatgtgctgaagctacagatgttgaaacacgaactaatcttgtggctgataaatgaattttgaaatgtctatggaaatgtgaataaaggcaatccatgaataggtcaacttcttcctgggtaacctccccaggtgttttgtggacactgtcccatagagcttttgcatcctctggatgtattgcgaaagaaatgtccagactttgagggctacagggtacagaccaaagaaattcagtagtagccacataatggtccattttgcatgcagtccacatggcagccatccaggaaagattaaatgcattgattgctaaaggactgaaataacagtcaaaggttttctgaaaccaagttccaattattgctgtgttagactctgctccatttgcaaggaataagggcagacaggtgaaatcttctgaaacagtctccagaagactgtctccaaatacacagcagaaccagccagtccacagcactttaccttctctattctcagatggcaattgagattttgacacaatctggacaagaaatgcttccgggtccctttgtgttcctttcattcctaggagagtagaaaaaatcactttgatgttgaagtcttctcccacttccacagcaagtcctttttgcttttcagcaacaataaaagcattgagaagtctagaatactctttgagattactataggagaatttatataagggagttaaactatataaagtccactgtttatgcagaaggaatgcaaccttttgagggtcaacatcttcctgcaactgcgaacactggggaattttccttcgaggtggagtcaggataaatgaactctgcttcctgaccgattctaatcgtttctgcagaggagtggcacctataaagtaatcttcaggtcttgaggatgcactaggagttgactctggtgcactgtaagaatccatggtctgtcaataaaatgccgtgatgacgctgtcacccattccggattcacgaatcattcttcaaaagtccggctccaaaactatgtggagactgaaatccccggtgcgaagctttctctcaaatttccgcccgtagtaggcatggcggcggcacctcaccactgattcgttgaattccttcccggtaatcttgggcactagcgggcggagttgaagggcgcttggaccccagcggcgatctgtgtttgggttcgcgctctgggagaattttggctttgctcgccttcctctttcagaagactcgaaatcggccagcaggtctgcgagatttgaaacgcgactgttactccttgttttccggttctggccgcgggagcctctcgagaagcgtggaaagaggagaagggcgtataccttgtgacc

SEQ ID NO: 12671 - RNA, 2561 nt, Homo sapiens
  source 1..2561: mol_type = other RNA
gatctcactttgttgcccaggctggagtgcagtggtgcagtcttggctcactgcagcctgtcttctgggttaaaacgattctcctgcctcagcctccccagtagctgggatcataggcatgtgccaccacgcccagctaattattgtattttcagtagagaaggggtttcaccatgttggccaggctggtcttgaattcctggcctcaaatgatccacccacctcagcctcccaaagtgctggaattacaggtgtgagccaccaagcccagcctatatatatatatttaaagatgacaagaaattaacaactcagcattttgagaatggcatgtcaggttatcatgattagtacatgggcacctggctgtggctcatctactaccatattctttgttcttctagatccttcttggcttccatcttggcaactccaaaggcatggtggggaaaacagatgcagagatagatgcctatttctcctgcagtctctttcagcatagcaattaggcaagttatcaataagagtatataatctataacttatagtccacataaggcttcactcaatttgaaaaattgccagttctgtcaaatatgctaacactccaataaggtatttatgacacagaatctttatttttccatcagtatgtgctgaagctacagatgttgaaacacgaactaatcttgtggctgataaatgaattttgaaatgtctatggaaatgtgaataaaggcaatccatgaataggtcaacttcttcctgggtaacctccccaggtgttttgtggacactgtcccatagagcttttgcatcctctggatgtattgcgaaagaaatgtccagactttgagggctacagggtacagaccaaagaaattcagtagtagccacataatggtccattttgcatgcagtccacatggcagccatccaggaaagattaaatgcattgattgctaaaggactgaaataacagtcaaaggttttctgaaaccaagttccaattattgctgtgttagactctgctccatttgcaaggaataagggcagacaggtgaaatcttctgaaacagtctccagaagactgtctccaaatacacagcagaaccagccagtccacagcactttaccttctctattctcagatggcaattgagattttgacacaatctggacaagaaatgcttccgggtccctttgtgttcctttcattcctaggagagtagaaaaaatcactttgatgttgaagtcttctcccacttccacagcaagtcctttttgcttttcagcaacaataaaagcattgagaagtctagaatactctttgagattactataggagaatttatataagggagttaaactatataaagtccactgtttatgcagaaggaatgcaaccttttgagggtcaacatcttcctgcaactgcgaacactggggaattttccttcgaggtggagtcaggataaatgaactctgcttcctgaccgattctaatcgtttctgcagaggagtggcacctataaagtaatcttcaggtcttgaggatgcactaggagttgactctggtgcactgtaagaatccatggtctgtcaataaaatgccgtgatgacgctgtcacccattccggattcacgaatcattcttcaaaagtccggctccaaaactatgtggagactgaaatcccctgaagaaaaaaaaaaaaaaccgccaaaatgacagctaagacagaggccagactaacccctggccctcccaaattccctctcgctccacaagtgggttcacaagagacacaaacgcacccaggaagacctccgctccctcagacgcggggcgggccctgcgacttcactctgggagggacatttccgctcacccagctctgcgaccctcgctcctgcggagtcagcttctgctcgcggagggggaagggcaaaaggacagtgcgtcccaacccgtccctctccagctgagcctgtcagagaccagcccagctctgaaatcaagccgttgagaaaagggaattcggccctccgccgcctcttcagtttaaaatcgtttcccgactcgctctgcggccccacgcaggaagcctccttggcgcctcgccgattccgtatcagtgaagcaactaaaattgccattttaactgagggcaaggccgagccacttaaccactatcgtcaacctttccaatcgtgctcggttgctcctcagttttcctaccggtgcgaagctttctctcaaatttccgcccgtagtaggcatggcggcggcacctcaccactgattcgttgaattccttcccggtaatcttgggcactagcgggcggagttgaagggcgcttggaccccagcggcgatctgtgtttgggttcgcgctctgggagaattttggctttgctcgccttcctctttcagaagactcgaaatcggccagcaggtctgcgagatttgaaacgcgactgttactccttgttttccggttctggccgcgggagcctctcgagaagcgtggaaagaggagaagggcgtataccttgtgacc

SEQ ID NO: 12672 - RNA, 2558 nt, Homo sapiens
  source 1..2558: mol_type = other RNA
gatctcactttgttgcccaggctggagtgcagtggtgcagtcttggctcactgcagcctgtcttctgggttaaaacgattctcctgcctcagcctccccagtagctgggatcataggcatgtgccaccacgcccagctaattattgtattttcagtagagaaggggtttcaccatgttggccaggctggtcttgaattcctggcctcaaatgatccacccacctcagcctcccaaagtgctggaattacaggtgtgagccaccaagcccagcctatatatatatatttaaagatgacaagaaattaacaactcagcattttgagaatggcatgtcaggttatcatgattagtacatgggcacctggctgtggctcatctactaccatattctttgttcttctagatccttcttggcttccatcttggcaactccaaaggcatggtggggaaaacagatgcagagatagatgcctatttctcctgcagtctctttcagcatagcaattaggcaagttatcaataagagtatataatctataacttatagtccacataaggcttcactcaatttgaaaaattgccagttctgtcaaatatgctaacactccaataaggtatttatgacacagaatctttatttttccatcagtatgtgctgaagctacagatgttgaaacacgaactaatcttgtggctgataaatgaattttgaaatgtctatggaaatgtgaataaaggcaatccatgaataggtcaacttcttcctgggtaacctccccaggtgttttgtggacactgtcccatagagcttttgcatcctctggatgtattgcgaaagaaatgtccagactttgagggctacagggtacagaccaaagaaattcagtagtagccacataatggtccattttgcatgcagtccacatggcagccatccaggaaagattaaatgcattgattgctaaaggactgaaataacagtcaaaggttttctgaaaccaagttccaattattgctgtgttagactctgctccatttgcaaggaataagggcagacaggtgaaatcttctgaaacagtctccagaagactgtctccaaatacacagcagaaccagccagtccacagcactttaccttctctattctcagatggcaattgagattttgacacaatctggacaagaaatgcttccgggtccctttgtgttcctttcattcctaggagagtagaaaaaatcactttgatgttgaagtcttctcccacttccacagcaagtcctttttgcttttcagcaacaataaaagcattgagaagtctagaatactctttgagattactataggagaatttatataagggagttaaactatataaagtccactgtttatgcagaaggaatgcaaccttttgagggtcaacatcttcctgcaactgcgaacactggggaattttccttcgaggtggagtcaggataaatgaactctgcttcctgaccgattctaatcgtttctgcagaggagtggcacctataaagtaatcttcaggtcttgaggatgcactaggagttgactctggtgcactgtaagaatccatggtctgtctgtggtcccagctactcaggaggctgaagtaggactgcatgagcccaggaggtcaaggctgcagtgagatgtgatcatgccaccgaattccagcctgggtgacacagcaagacccaataaaatgccgtgatgacgctgtcacccattccggattcacgaatcattcttcaaaagtccggctccaaaactatgtggagactgaaatcccccaggaagacctccgctccctcagacgcggggcgggccctgcgacttcactctgggagggacatttccgctcacccagctctgcgaccctcgctcctgcggagtcagcttctgctcgcggagggggaagggcaaaaggacagtgcgtcccaacccgtccctctccagctgagcctgtcagagaccagcccagctctgaaatcaagccgttgagaaaagggaattcggccctccgccgcctcttcagtttaaaatcgtttcccgactcgctctgcggccccacgcaggaagcctccttggcgcctcgccgattccgtatcagtgaagcaactaaaattgccattttaactgagggcaaggccgagccacttaaccactatcgtcaacctttccaatcgtgctcggttgctcctcagttttcctaccggtgcgaagctttctctcaaatttccgcccgtagtaggcatggcggcggcacctcaccactgattcgttgaattccttcccggtaatcttgggcactagcgggcggagttgaagggcgcttggaccccagcggcgatctgtgtttgggttcgcgctctgggagaattttggctttgctcgccttcctctttcagaagactcgaaatcggccagcaggtctgcgagatttgaaacgcgactgttactccttgttttccggttctggccgcgggagcctctcgagaagcgtggaaagaggagaagggcgtataccttgtgacc

SEQ ID NO: 12673 - RNA, 2486 nt, Homo sapiens
  source 1..2486: mol_type = other RNA
gatctcactttgttgcccaggctggagtgcagtggtgcagtcttggctcactgcagcctgtcttctgggttaaaacgattctcctgcctcagcctccccagtagctgggatcataggcatgtgccaccacgcccagctaattattgtattttcagtagagaaggggtttcaccatgttggccaggctggtcttgaattcctggcctcaaatgatccacccacctcagcctcccaaagtgctggaattacaggtgtgagccaccaagcccagcctatatatatatatttaaagatgacaagaaattaacaactcagcattttgagaatggcatgtcaggttatcatgattagtacatgggcacctggctgtggctcatctactaccatattctttgttcttctagatccttcttggcttccatcttggcaactccaaaggcatggtggggaaaacagatgcagagatagatgcctatttctcctgcagtctctttcagcatagcaattaggcaagttatcaataagagtatataatctataacttatagtccacataaggcttcactcaatttgaaaaattgccagttctgtcaaatatgctaacactccaataaggtatttatgacacagaatctttatttttccatcagtatgtgctgaagctacagatgttgaaacacgaactaatcttgtggctgataaatgaattttgaaatgtctatggaaatgtgaataaaggcaatccatgaataggtcaacttcttcctgggtaacctccccaggtgttttgtggacactgtcccatagagcttttgcatcctctggatgtattgcgaaagaaatgtccagactttgagggctacagggtacagaccaaagaaattcagtagtagccacataatggtccattttgcatgcagtccacatggcagccatccaggaaagattaaatgcattgattgctaaaggactgaaataacagtcaaaggttttctgaaaccaagttccaattattgctgtgttagactctgctccatttgcaaggaataagggcagacaggtgaaatcttctgaaacagtctccagaagactgtctccaaatacacagcagaaccagccagtccacagcactttaccttctctattctcagatggcaattgagattttgacacaatctggacaagaaatgcttccgggtccctttgtgttcctttcattcctaggagagtagaaaaaatcactttgatgttgaagtcttctcccacttccacagcaagtcctttttgcttttcagcaacaataaaagcattgagaagtctagaatactctttgagattactataggagaatttatataagggagttaaactatataaagtccactgtttatgcagaaggaatgcaaccttttgagggtcaacatcttcctgcaactgcgaacactggggaattttccttcgaggtggagtcaggataaatgaactctgcttcctgaccgattctaatcgtttctgcagaggagtggcacctataaagtaatcttcaggtcttgaggatgcactaggagttgactctggtgcactgtaagaatccatggtctgtctgtggtcccagctactcaggaggctgaagtaggactgcatgagcccaggaggtcaaggctgcagtgagatgtgatcatgccaccgaattccagcctgggtgacacagcaagaccctcaataaaatgccgtgatgacgctgtcacccattccggattcacgaatcattcttcaaaagtccggctccaaaactatgtggagactgaaatcccccagctctgcgaccctcgctcctgcggagtcagcttctgctcgcggagggggaagggcaaaaggacagtgcgtcccaacccgtccctctccagctgagcctgtcagagaccagcccagctctgaaatcaagccgttgagaaaagggaattcggccctccgccgcctcttcagtttaaaatcgtttcccgactcgctctgcggccccacgcaggaagcctccttggcgcctcgccgattccgtatcagtgaagcaactaaaattgccattttaactgagggcaaggccgagccacttaaccactatcgtcaacctttccaatcgtgctcggttgctcctcagttttcctaccggtgcgaagctttctctcaaatttccgcccgtagtaggcatggcggcggcacctcaccactgattcgttgaattccttcccggtaatcttgggcactagcgggcggagttgaagggcgcttggaccccagcggcgatctgtgtttgggttcgcgctctgggagaattttggctttgctcgccttcctctttcagaagactcgaaatcggccagcaggtctgcgagatttgaaacgcgactgttactccttgttttccggttctggccgcgggagcctctcgagaagcgtggaaagaggagaagggcgtataccttgtgacc

SEQ ID NO: 12674 - RNA, 2303 nt, Homo sapiens
  source 1..2303: mol_type = other RNA
gatctcactttgttgcccaggctggagtgcagtggtgcagtcttggctcactgcagcctgtcttctgggttaaaacgattctcctgcctcagcctccccagtagctgggatcataggcatgtgccaccacgcccagctaattattgtattttcagtagagaaggggtttcaccatgttggccaggctggtcttgaattcctggcctcaaatgatccacccacctcagcctcccaaagtgctggaattacaggtgtgagccaccaagcccagcctatatatatatatttaaagatgacaagaaattaacaactcagcattttgagaatggcatgtcaggttatcatgattagtacatgggcacctggctgtggctcatctactaccatattctttgttcttctagatccttcttggcttccatcttggcaactccaaaggcatggtggggaaaacagatgcagagatagatgcctatttctcctgcagtctctttcagcatagcaattaggcaagttatcaataagagtatataatctataacttatagtccacataaggcttcactcaatttgaaaaattgccagttctgtcaaatatgctaacactccaataaggtatttatgacacagaatctttatttttccatcagtatgtgctgaagctacagatgttgaaacacgaactaatcttgtggctgataaatgaattttgaaatgtctatggaaatgtgaataaaggcaatccatgaataggtcaacttcttcctgggtaacctccccaggtgttttgtggacactgtcccatagagcttttgcatcctctggatgtattgcgaaagaaatgtccagactttgagggctacagggtacagaccaaagaaattcagtagtagccacataatggtccattttgcatgcagtccacatggcagccatccaggaaagattaaatgcattgattgctaaaggactgaaataacagtcaaaggttttctgaaaccaagttccaattattgctgtgttagactctgctccatttgcaaggaataagggcagacaggtgaaatcttctgaaacagtctccagaagactgtctccaaatacacagcagaaccagccagtccacagcactttaccttctctattctcagatggcaattgagattttgacacaattttgatgttgaagtcttctcccacttccacagcaagtcctttttgcttttcagcaacaataaaagcattgagaagtctagaatactctttgagattactataggagaatttatataagggagttaaactatataaagtccactgtttatgcagaaggaatgcaaccttttgagggtcaacatcttcctgcaactgcgaacactggggaattttccttcgaggtggagtcaggataaatgaactctgcttcctgaccgattctaatcgtttctgcagaggagtggcacctataaagtaatcttcaggtcttgaggatgcactaggagttgactctggtgcactgtaagaatccatggtctgtcaataaaatgccgtgatgacgctgtcacccattccggattcacgaatcattcttcaaaagtccggctccaaaactatgtggagactgaaatcccccagctctgcgaccctcgctcctgcggagtcagcttctgctcgcggagggggaagggcaaaaggacagtgcgtcccaacccgtccctctccagctgagcctgtcagagaccagcccagctctgaaatcaagccgttgagaaaagggaattcggccctccgccgcctcttcagtttaaaatcgtttcccgactcgctctgcggccccacgcaggaagcctccttggcgcctcgccgattccgtatcagtgaagcaactaaaattgccattttaactgagggcaaggccgagccacttaaccactatcgtcaacctttccaatcgtgctcggttgctcctcagttttcctaccggtgcgaagctttctctcaaatttccgcccgtagtaggcatggcggcggcacctcaccactgattcgttgaattccttcccggtaatcttgggcactagcgggcggagttgaagggcgcttggaccccagcggcgatctgtgtttgggttcgcgctctgggagaattttggctttgctcgccttcctctttcagaagactcgaaatcggccagcaggtctgcgagatttgaaacgcgactgttactccttgttttccggttctggccgcgggagcctctcgagaagcgtggaaagaggagaagggcgtataccttgtgacc

SEQ ID NO: 12675 - RNA, 2052 nt, Homo sapiens
  source 1..2052: mol_type = other RNA
gatctcactttgttgcccaggctggagtgcagtggtgcagtcttggctcactgcagcctgtcttctgggttaaaacgattctcctgcctcagcctccccagtagctgggatcataggcatgtgccaccacgcccagctaattattgtattttcagtagagaaggggtttcaccatgttggccaggctggtcttgaattcctggcctcaaatgatccacccacctcagcctcccaaagtgctggaattacaggtgtgagccaccaagcccagcctatatatatatatttaaagatgacaagaaattaacaactcagcattttgagaatggcatgtcaggttatcatgattagtacatgggcacctggctgtggctcatctactaccatattctttgttcttctagatccttcttggcttccatcttggcaactccaaaggcatggtggggaaaacagatgcagagatagatgcctatttctcctgcagtctctttcagcatagcaattaggcaagttatcaataagagtatataatctataacttatagtccacataaggcttcactcaatttgaaaaattgccagttctgtcaaatatgctaacactccaataaggtatttatgacacagaatctttatttttccatcagtatgtgctgaagctacagatgttgaaacacgaactaatcttgtggctgataaatgaattttgaaatgtctatggaaatgtgaataaaggcaatccatgaataggtcaacttcttcctgggtaacctccccaggtgttttgtggacactgtcccatagagcttttgcatcctctggatgtattgcgaaagaaatgtccagactttgagggctggacaagaaatgcttccgggtccctttgtgttcctttcattcctaggagagtagaaaaaatcactttgatgttgaagtcttctcccacttccacagcaagtcctttttgcttttcagcaacaataaaagcattgagaagtctagaatactctttgagattactataggagaatttatataagggagttaaactatataaagtccactgtttatgcagaaggaatgcaaccttttgagggtcaacatcttcctgcaactgcgaacactggggaattttccttcgaggtggagtcaggataaatgaactctgcttcctgaccgattctaatcgtttctgcagaggagtggcacctataaagtaatcttcaggtcttgaggatgcactaggagttgactctggtgcactgtaagaatccatggtctgtcaataaaatgccgtgatgacgctgtcacccattccggattcacgaatcattcttcaaaagtccggctccaaaactatgtggagactgaaatcccccagctctgcgaccctcgctcctgcggagtcagcttctgctcgcggagggggaagggcaaaaggacagtgcgtcccaacccgtccctctccagctgagcctgtcagagaccagcccagctctgaaatcaagccgttgagaaaagggaattcggccctccgccgcctcttcagtttaaaatcgtttcccgactcgctctgcggccccacgcaggaagcctccttggcgcctcgccgattccgtatcagtgaagcaactaaaattgccattttaactgagggcaaggccgagccacttaaccactatcgtcaacctttccaatcgtgctcggttgctcctcagttttcctaccggtgcgaagctttctctcaaatttccgcccgtagtaggcatggcggcggcacctcaccactgattcgttgaattccttcccggtaatcttgggcactagcgggcggagttgaagggcgcttggaccccagcggcgatctgtgtttgggttcgcgctctgggagaattttggctttgctcgccttcctctttcagaagactcgaaatcggccagcaggtctgcgagatttgaaacgcgactgttactccttgttttccggttctggccgcgggagcctctcgagaagcgtggaaagaggagaagggcgtataccttgtgacc

SEQ ID NO: 12676 - RNA, 1771 nt, Homo sapiens
  source 1..1771: mol_type = other RNA
gatctcactttgttgcccaggctggagtgcagtggtgccatctcggctcactgcaacctccgcctccagggttcaagcgattctcctgcctcagcctcccgagtagctgggattacaggcgcctgccaccacgcctagtttatttttgtattttcagtagagacggggttttgccatgttggccagggtggcctcgaactcctaacctcaggtgatccacccgcctcggcctcccaaagtgctggggttacaggcgtgagccaccgcgcccggccggtaatcatttctgtcactcaacaaatatttattgagcgcttgctatgtaccaggacctgttcttgcacaaaacaggcaatccatgcattgcttacattcacattctagtgggggtagtgacggaccataaaatcagcaagaaaaatgtatgttatgatagatggttatgagtgctttagagtaaaattaagtaggggaggcaggcaggaagtgtgtagtatgtttcaattttatattaggctggtcatggtttgtcatctatttcacctggctcacagttcttgcaggacaggaacaaatctcacttccatttgccttcatacttccagcacttaacacagcaccaggaactcagggaggcaataactttatactgaatccgttttatgccttcctagaggcaagcagttgagaaaggcgtgtaactagatattgcctataaggtccacaattggaataacgtaatcatttatgattaattttattcatttccattaacttaagctaagttcttttagcacgtttagattacagaacgaaagctgtgttaactagtattacaggacttttcacgtttttccaaacatcttctagccacctctttggccctacaactacgcataagcttttgcttttcaaaaaacctccacagcctttgccaattatttgttgatctcgagtagttgttataacagcacttggggtttaacactaaggttgcagatcgcgcccagttatcagttcctcgaacctcaaggaatcacaaagcaaggttccaccccccgaaaaactacgaaaagtgagaaagcctctaacactcctcgcgccgtgcccagccggaaccttgacctcaagatggcgtcccgtagtcgtaagattcagtcggctccaatcaaacatggtgggtcataatttacagttcgggcctttctagtaaccgctagacgctgcttctctatggttattcgtctcggcttggtgagtcagagccaacagcggagacgatctatatacgttcttctctatggttccgcgctccccgcccccggccgcagtgcacgccgggcaagaggaagacctccatcagctcgccgcgcagcgcggctgtatttgcggcctgtgcgagtaggcgcttgggcactcagtctccctggcgagcgacgggcagaaatctcgaaccagtggagcgcactcgtaacctggatcccagaaggtcgcgaaggcagtaccgtttcctcagcggcgggtgagtttgtgtctctgaacgcgtgtggaaaccgggagaccgggtgcctcagctttttagcagtctcctggcttgcttaagatagtcatgaattttgccatcctgcctcttttgcgcattggagggtgcagtaaactgtatatcgccattcattctaggcgattactaagctccacattaaaatgttactttctcatttttctttggtcgtcaatcctgcttttaaatacggttttccggaatagacgt

SEQ ID NO: 12677 - RNA, 2995 nt, Homo sapiens
  source 1..2995: mol_type = other RNA
gatctcactttgttgcccaggctggagtgcagtggtgcgatctcggctcactgcagcctccacttcctgggttcaagcaatactcctgtgtcagcctcccgagtagctgggactacaggcgcccgccaccacacctggctaatttttgtatttttagtagagacggggtttcaccatattggggaggctggtctcgaacacctgacctcaggtgatccgcccaccttggcctcccaaagtgctaggattacaggcatgaaccaccacacccagcctatttttattttttaaaaaaattttaatatttccatggaactctgcttgataccagctaatttatttttatgtttttgtagagacaggcatctccttatgttgtccaggctagtctcaacctcctggcctcaaactgtcctcctgcctcagcctcccaatgtattacaggcatgagccactgcaagtggcccatttaaatgttctataacaatattcagtgattacaatttctttgattcaaatacataagcaaatgcacaagcaataatgtatgcagtacatattaaacatcattactgcctaaacttgattaaacaaatgaataactttataattaaaaatatgtttctaggcaaagttaaatatattgacattagaagtaatatattcttgcatgtgtgggccacaaagaccttggctaaagtgtacattttaaaggtgcaaagcataaaaacagagcttttgagaatgacagcttcaagaagacaaaccaattaactcccaaatattggcttcaattcaagcgatatttctgtaaaatatacatttcatgacttcaattattacctaatgaatgcaaaaagccactatgactacactacacaggaattcaatgacagaacttctgtataaatacagtacagttgctcattttttagtagatttttttttcctccctgaatccacatgcatcaattctgttaactttgtaatatatgttacaaaatcaatagttaccttaaaatatttcatagcacactcaaattgtatgattcttatggtacttattgtactttggcttccagtagcccagtggacataacatgaccatgactgcttagacaactacttgtatgcctcagggcatctgcttcaagataggccattaaaagctcagtgcggcgaatgagtaactgcatgaggtcttcagctaaagtctctgtacttgaatagcgcaccttctcaaagtcaaaaatgtctttgagaaataaaagaacttgattcttaaaaaagcaacataaatcatacagagaatttctaggacccaaaaagccccaggctaggacaggactgatgtgttcacaaatggcataaaaatgggcaaaaaatccatctgggatctgcttcatctgttgtcttttctgtttcagcaccgaccaacaacttgaagccacagctgtttctttgaaggatgagtttagccatcgattatttactacattctgtatggatgtgggtgggttttccaaatcttcaaaggagtccattaatataaaatccagaacaacatcataaaaatttagatttttcacccctctagcagcaagttccatttcagtactaccccagtgatcggtctgctctaaaaaatagatcatttcatcaaaaacatcttcaaacttctttggattctttcgtgctttcacaattaaagctgataaaattttccttccgctctcagcgaggaatatcctgttagctgattctgaaagaattacctgaaaagcctgtcgaatacagtgaagtttggcaagaaaatcactgtctcctaggcactccaacatttcagttctcagtactctggagtaaatttttccttcttcaactaaatgcatggcttcctcgtaaaatgggcagtgacaaagggactccaggctgtaggtatgccgtacttctctgtgttctgcaagctctgctgcggaagcaaaggaatccgtggatgcgatgctcaaggtgtctcgcaggccaaagtcttccacattacccttcatggtgatatctgtatctttatcaatatcatcagcaagggaattaggatcagatgccccaagggtagcttcaaactcctcttggagacgataggctctttgcagcagagcttcgagtttatggataaattcagtactaataatatcatctacattttcttcagcaatggcatctcctgcacccagtttaatggaaccacaggcttcatcttcagcctgtctattgcgaaaggtcagagcttgttcccatcgacgcaatgcctcttcaaacaattccatacccattaagtataagttctctggagtagtcacaggaatattaacaagtttaatatcatcttcatctgctttgtcccaggaattagaattgccacaagcgcagctatgacaagaattgacactctggacagaggccaaactctgtgcagaacctgaatatttactgaaaagtcctccattagcatagttacaaacttgagatcctttgtctttggtagaacttaaagataatgtcaaattctgtctgctactggaacaacttgaacctttgtctgatgctgctcttttagtgtattcaagtatgaggtgctctggttcccatggtaatatttttcctttcttctttccacgttttcttttaaagtgatgagccagaaaaattacagatatagcactcactgcagttaccacaaacaactttttagccaccggagaaaatttgatctgggagagagaatagtaccaagtcagaggaagatcaaacactcttagcgctgctgtcttcaaggaaaactgtgattcacttactgtttcttctgacatggctcctcttctaatctggagctccaggccaggtacagctggcctgcccacgccagcttcccagctgatgcctggcgctgagcagcagtctgacatggagaaggcggagtccttccggggtcaggagt

SEQ ID NO: 12678 - RNA, 3037 nt, Homo sapiens
  source 1..3037: mol_type = other RNA
gatctcactttgttgcccaggctggagtgcagtggtgcgatctcggctcactgcagcctccacttcctgggttcaagcaatactcctgtgtcagcctcccgagtagctgggactacaggcgcccgccaccacacctggctaatttttgtatttttagtagagacggggtttcaccatattggggaggctggtctcgaacacctgacctcaggtgatccgcccaccttggcctcccaaagtgctaggattacaggcatgaaccaccacacccagcctatttttattttttaaaaaaattttaatatttccatggaactctgcttgataccagctaatttatttttatgtttttgtagagacaggcatctccttatgttgtccaggctagtctcaacctcctggcctcaaactgtcctcctgcctcagcctcccaatgtattacaggcatgagccactgcaagtggcccatttaaatgttctataacaatattcagtgattacaatttctttgattcaaatacataagcaaatgcacaagcaataatgtatgcagtacatattaaacatcattactgcctaaacttgattaaacaaatgaataactttataattaaaaatatgtttctaggcaaagttaaatatattgacattagaagtaatatattcttgcatgtgtgggccacaaagaccttggctaaagtgtacattttaaaggtgcaaagcataaaaacagagcttttgagaatgacagcttcaagaagacaaaccaattaactcccaaatattggcttcaattcaagcgatatttctgtaaaatatacatttcatgacttcaattattacctaatgaatgcaaaaagccactatgactacactacacaggaattcaatgacagaacttctgtataaatacagtacagttgctcattttttagtagatttttttttcctccctgaatccacatgcatcaattctgttaactttgtaatatatgttacaaaatcaatagttaccttaaaatatttcatagcacactcaaattgtatgattcttatggtacttattgtactttggcttccagtagcccagtggacataacatgaccatgactgcttagacaactacttgtatgcctcagggcatctgcttcaagataggccattaaaagctcagtgcggcgaatgagtaactgcatgaggtcttcagctaaagtctctgtacttgaatagcgcaccttctcaaagtcaaaaatgtctttgagaaataaaagaacttgattcttaaaaaagcaacataaatcatacagagaatttctaggacccaaaaagccccaggctaggacaggactgatgtgttcacaaatggcataaaaatgggcaaaaaatccatctgggatcttcatctgttgtcttttctgtttcagcaccgaccaacaacttgaagccacagctgtttctttgaaggatgagtttagccatcgattatttactacattctgtatggatgtgggtgggttttccaaatcttcaaaggagtccattaatataaaatccagaacaacatcataaaaatttagatttttcacccctctagcagcaagttccatttcagtactaccccagtgatcggtctgctctaaaaaatagatcatttcatcaaaaacatcttcaaacttctttggattctttcgtgctttcacaattaaagctgataaaattttccttccgctctcagcgaggaatatcctgttagctgattctgaaagaattacctgaaaagcctgtcgaatacagtgaagtttggcaagaaaatcactgtctcctaggcactccaacatttcagttctcagtactctggagtaaatttttccttcttcaactaaatgcatggcttcctcgtaaaatgggcagtgacaaagggactccaggctgtaggtatgccgtacttctctgtgttctgcaagctctgctgcggaagcaaaggaatccgtggatgcgatgctcaaggtgtctcgcaggccaaagtcttccacattacccttcatggtgatatctgtatctttatcaatatcatcagcaagggaattaggatcagatgccccaagggtagcttcaaactcctcttggagacgataggctctttgcagcagagcttcgagtttatggataaattcagtactaataatatcatctacattttcttcagcaatggcatctcctgcacccagtttaatggaaccacaggcttcatcttcagcctgtctattgcgaaaggtcagagcttgttcccatcgacgcaatgcctcttcaaacaattccatacccattaagtataagttctctggagtagtcacaggaatattaacaagtttaatatcatcttcatctgctttgtcccaggaattagaattgccacaagcgcagctatgacaagaattgacactctggacagaggccaaactctgtgcagaacctgaatatttactgaaaagtcctccattagcatagttacaaacttgagatcctttgtctttggtagaacttaaagataatgtcaaattctgtctgctactggaacaacttgaacctttgtctgatgctgctcttttagtgtattcaagtatgaggtgctctggttcccatggtaatatttttcctttcttctttccacgttttcttttaaagtgatgagccagaaaaattacagatatagcactcactgcagttaccacaaacaactttttagccaccggagaaaatttgatctgggagagagaatagtaccaagtcagaggaagatcaaacactcttagcgctgctgtcttcaaggaaaactgtgattcacttactgtttcttctgacatggctcctcttcaggcccgaccctgcttagcttctgagatgagacgaggtcgggggtgttcagggtggcacggccgtagaccctctggctttccgccgctccacctggcactccgagagctaacgccagcgatggagtccgcgccacccctgccccgaggcctctgccccaact

SEQ ID NO: 12679 - RNA, 3042 nt, Homo sapiens
  source 1..3042: mol_type = other RNA
gatctcactttgttgcccaggctggagtgcagtggtgcgatctcggctcactgcagcctccacttcctgggttcaagcaatactcctgtgtcagcctcccgagtagctgggactacaggcgcccgccaccacacctggctaatttttgtatttttagtagagacggggtttcaccatattggggaggctggtctcgaacacctgacctcaggtgatccgcccaccttggcctcccaaagtgctaggattacaggcatgaaccaccacacccagcctatttttattttttaaaaaaattttaatatttccatggaactctgcttgataccagctaatttatttttatgtttttgtagagacaggcatctccttatgttgtccaggctagtctcaacctcctggcctcaaactgtcctcctgcctcagcctcccaatgtattacaggcatgagccactgcaagtggcccatttaaatgttctataacaatattcagtgattacaatttctttgattcaaatacataagcaaatgcacaagcaataatgtatgcagtacatattaaacatcattactgcctaaacttgattaaacaaatgaataactttataattaaaaatatgtttctaggcaaagttaaatatattgacattagaagtaatatattcttgcatgtgtgggccacaaagaccttggctaaagtgtacattttaaaggtgcaaagcataaaaacagagcttttgagaatgacagcttcaagaagacaaaccaattaactcccaaatattggcttcaattcaagcgatatttctgtaaaatatacatttcatgacttcaattattacctaatgaatgcaaaaagccactatgactacactacacaggaattcaatgacagaacttctgtataaatacagtacagttgctcattttttagtagatttttttttcctccctgaatccacatgcatcaattctgttaactttgtaatatatgttacaaaatcaatagttaccttaaaatatttcatagcacactcaaattgtatgattcttatggtacttattgtactttggcttccagtagcccagtggacataacatgaccatgactgcttagacaactacttgtatgcctcagggcatctgcttcaagataggccattaaaagctcagtgcggcgaatgagtaactgcatgaggtcttcagctaaagtctctgtacttgaatagcgcaccttctcaaagtcaaaaatgtctttgagaaataaaagaacttgattcttaaaaaagcaacataaatcatacagagaatttctaggacccaaaaagccccaggctaggacaggactgatgtgttcacaaatggcataaaaatgggcaaaaaatccatctgggatcttcatctgttgtcttttctgtttcagcaccgaccaacaacttgaagccacagctgtttctttgaaggatgagtttagccatcgattatttactacattctgtatggatgtgggtgggttttccaaatcttcaaaggagtccattaatataaaatccagaacaacatcataaaaatttagatttttcacccctctagcagcaagttccatttcagtactaccccagtgatcggtctgctctaaaaaatagatcatttcatcaaaaacatcttcaaacttctttggattctttcgtgctttcacaattaaagctgataaaattttccttccgctctcagcgaggaatatcctgttagctgattctgaaagaattacctgaaaagcctgtcgaatacagtgaagtttggcaagaaaatcactgtctcctaggcactccaacatttcagttctcagtactctggagtaaatttttccttcttcaactaaatgcatggcttcctcgtaaaatgggcagtgacaaagggactccaggctgtaggtatgccgtacttctctgtgttctgcaagctctgctgcggaagcaaaggaatccgtggatgcgatgctcaaggtgtctcgcaggccaaagtcttccacattacccttcatggtgatatctgtatctttatcaatatcatcagcaagggaattaggatcagatgccccaagggtagcttcaaactcctcttggagacgataggctctttgcagcagagcttcgagtttatggataaattcagtactaataatatcatctacattttcttcagcaatggcatctcctgcacccagtttaatggaaccacaggcttcatcttcagcctgtctattgcgaaaggtcagagcttgttcccatcgacgcaatgcctcttcaaacaattccatacccattaagtataagttctctggagtagtcacaggaatattaacaagtttaatatcatcttcatctgctttgtcccaggaattagaattgccacaagcgcagctatgacaagaattgacactctggacagaggccaaactctgtgcagaacctgaatatttactgaaaagtcctccattagcatagttacaaacttgagatcctttgtctttggtagaacttaaagataatgtcaaattctgtctgctactggaacaacttgaacctttgtctgatgctgctcttttagtgtattcaagtatgaggtgctctggttcccatggtaatatttttcctttcttctttccacgttttcttttaaagtgatgagccagaaaaattacagatatagcactcactgcagttaccacaaacaactttttagccaccggagaaaatttgatctgggagagagaatagtaccaagtcagaggaagatcaaacactcttagcgctgctgtcttcaaggaaaactgtgattcacttactgtttcttctgacatggctcctcttctaatcaggcccgaccctgcttagcttctgagatgagacgaggtcgggggtgttcagggtggcacggccgtagaccctctggctttccgccgctccacctggcactccgagagctaacgccagcgatggagtccgcgccacccctgccccgaggcctctgccccaact

SEQ ID NO: 12680 - RNA, 3267 nt, Homo sapiens
  source 1..3267: mol_type = other RNA
gatctcactttgttgcccaggctggagtgcagtggtgcgatctcggctcactgcagcctccacttcctgggttcaagcaatactcctgtgtcagcctcccgagtagctgggactacaggcgcccgccaccacacctggctaatttttgtatttttagtagagacggggtttcaccatattggggaggctggtctcgaacacctgacctcaggtgatccgcccaccttggcctcccaaagtgctaggattacaggcatgaaccaccacacccagcctatttttattttttaaaaaaattttaatatttccatggaactctgcttgataccagctaatttatttttatgtttttgtagagacaggcatctccttatgttgtccaggctagtctcaacctcctggcctcaaactgtcctcctgcctcagcctcccaatgtattacaggcatgagccactgcaagtggcccatttaaatgttctataacaatattcagtgattacaatttctttgattcaaatacataagcaaatgcacaagcaataatgtatgcagtacatattaaacatcattactgcctaaacttgattaaacaaatgaataactttataattaaaaatatgtttctaggcaaagttaaatatattgacattagaagtaatatattcttgcatgtgtgggccacaaagaccttggctaaagtgtacattttaaaggtgcaaagcataaaaacagagcttttgagaatgacagcttcaagaagacaaaccaattaactcccaaatattggcttcaattcaagcgatatttctgtaaaatatacatttcatgacttcaattattacctaatgaatgcaaaaagccactatgactacactacacaggaattcaatgacagaacttctgtataaatacagtacagttgctcattttttagtagatttttttttcctccctgaatccacatgcatcaattctgttaactttgtaatatatgttacaaaatcaatagttaccttaaaatatttcatagcacactcaaattgtatgattcttatggtacttattgtactttggcttccagtagcccagtggacataacatgaccatgactgcttagacaactacttgtatgcctcagggcatctgcttcaagataggccattaaaagctcagtgcggcgaatgagtaactgcatgaggtcttcagctaaagtctctgtacttgaatagcgcaccttctcaaagtcaaaaatgtctttgagaaataaaagaacttgattcttaaaaaagcaacataaatcatacagagaatttctaggacccaaaaagccccaggctaggacaggactgatgtgttcacaaatggcataaaaatgggcaaaaaatccatctgggatcttcatctgttgtcttttctgtttcagcaccgaccaacaacttgaagccacagctgtttctttgaaggatgagtttagccatcgattatttactacattctgtatggatgtgggtgggttttccaaatcttcaaaggagtccattaatataaaatccagaacaacatcataaaaatttagatttttcacccctctagcagcaagttccatttcagtactaccccagtgatcggtctgctctaaaaaatagatcatttcatcaaaaacatcttcaaacttctttggattctttcgtgctttcacaattaaagctgataaaattttccttccgctctcagcgaggaatatcctgttagctgattctgaaagaattacctgaaaagcctgtcgaatacagtgaagtttggcaagaaaatcactgtctcctaggcactccaacatttcagttctcagtactctggagtaaatttttccttcttcaactaaatgcatggcttcctcgtaaaatgggcagtgacaaagggactccaggctgtaggtatgccgtacttctctgtgttctgcaagctctgctgcggaagcaaaggaatccgtggatgcgatgctcaaggtgtctcgcaggccaaagtcttccacattacccttcatggtgatatctgtatctttatcaatatcatcagcaagggaattaggatcagatgccccaagggtagcttcaaactcctcttggagacgataggctctttgcagcagagcttcgagtttatggataaattcagtactaataatatcatctacattttcttcagcaatggcatctcctgcacccagtttaatggaaccacaggcttcatcttcagcctgtctattgcgaaaggtcagagcttgttcccatcgacgcaatgcctcttcaaacaattccatacccattaagtataagttctctggagtagtcacaggaatattaacaagtttaatatcatcttcatctgctttgtcccaggaattagaattgccacaagcgcagctatgacaagaattgacactctggacagaggccaaactctgtgcagaacctgaatatttactgaaaagtcctccattagcatagttacaaacttgagatcctttgtctttggtagaacttaaagataatgtcaaattctgtctgctactggaacaacttgaacctttgtctgatgctgctcttttagtgtattcaagtatgaggtgctctggttcccatggtaatatttttcctttcttctttccacgttttcttttaaagtgatgagccagaaaaattacagatatagcactcactgcagttaccacaaacaactttttagccaccggagaaaatttgatctgggagagagaatagtaccaagtcagaggaagatcaaacactcttagcgctgctgtcttcaaggaaaactgtgattcacttactgtttcttctgacatggctcctcttctaatctccagcgcgctctcccccgaccccacagcagcccctcgcggagctctcctctgctgtcttcctttttctttgccaagaacaccagaaaagggggtccctccagctcggccgtccagacccttcctctggctcagagcagtggcgagcccatcccaattccgcgcttcctttgcaggcctccctctggcgtggggaccctcctgctttcctatgcaagtactaaccaggcccgaccctgcttagcttctgagatgagacgaggtcgggggtgttcagggtggcacggccgtagaccctctggctttccgccgctccacctggcactccgagagctaacgccagcgatggagtccgcgccacccctgccccgaggcctctgccccaact

SEQ ID NO: 12681 - RNA, 2992 nt, Homo sapiens
  source 1..2992: mol_type = other RNA
gatctcactttgttgcccaggctggagtgcagtggtgcgatctcggctcactgcagcctccacttcctgggttcaagcaatactcctgtgtcagcctcccgagtagctgggactacaggcgcccgccaccacacctggctaatttttgtatttttagtagagacggggtttcaccatattggggaggctggtctcgaacacctgacctcaggtgatccgcccaccttggcctcccaaagtgctaggattacaggcatgaaccaccacacccagcctatttttattttttaaaaaaattttaatatttccatggaactctgcttgataccagctaatttatttttatgtttttgtagagacaggcatctccttatgttgtccaggctagtctcaacctcctggcctcaaactgtcctcctgcctcagcctcccaatgtattacaggcatgagccactgcaagtggcccatttaaatgttctataacaatattcagtgattacaatttctttgattcaaatacataagcaaatgcacaagcaataatgtatgcagtacatattaaacatcattactgcctaaacttgattaaacaaatgaataactttataattaaaaatatgtttctaggcaaagttaaatatattgacattagaagtaatatattcttgcatgtgtgggccacaaagaccttggctaaagtgtacattttaaaggtgcaaagcataaaaacagagcttttgagaatgacagcttcaagaagacaaaccaattaactcccaaatattggcttcaattcaagcgatatttctgtaaaatatacatttcatgacttcaattattacctaatgaatgcaaaaagccactatgactacactacacaggaattcaatgacagaacttctgtataaatacagtacagttgctcattttttagtagatttttttttcctccctgaatccacatgcatcaattctgttaactttgtaatatatgttacaaaatcaatagttaccttaaaatatttcatagcacactcaaattgtatgattcttatggtacttattgtactttggcttccagtagcccagtggacataacatgaccatgactgcttagacaactacttgtatgcctcagggcatctgcttcaagataggccattaaaagctcagtgcggcgaatgagtaactgcatgaggtcttcagctaaagtctctgtacttgaatagcgcaccttctcaaagtcaaaaatgtctttgagaaataaaagaacttgattcttaaaaaagcaacataaatcatacagagaatttctaggacccaaaaagccccaggctaggacaggactgatgtgttcacaaatggcataaaaatgggcaaaaaatccatctgggatcttcatctgttgtcttttctgtttcagcaccgaccaacaacttgaagccacagctgtttctttgaaggatgagtttagccatcgattatttactacattctgtatggatgtgggtgggttttccaaatcttcaaaggagtccattaatataaaatccagaacaacatcataaaaatttagatttttcacccctctagcagcaagttccatttcagtactaccccagtgatcggtctgctctaaaaaatagatcatttcatcaaaaacatcttcaaacttctttggattctttcgtgctttcacaattaaagctgataaaattttccttccgctctcagcgaggaatatcctgttagctgattctgaaagaattacctgaaaagcctgtcgaatacagtgaagtttggcaagaaaatcactgtctcctaggcactccaacatttcagttctcagtactctggagtaaatttttccttcttcaactaaatgcatggcttcctcgtaaaatgggcagtgacaaagggactccaggctgtaggtatgccgtacttctctgtgttctgcaagctctgctgcggaagcaaaggaatccgtggatgcgatgctcaaggtgtctcgcaggccaaagtcttccacattacccttcatggtgatatctgtatctttatcaatatcatcagcaagggaattaggatcagatgccccaagggtagcttcaaactcctcttggagacgataggctctttgcagcagagcttcgagtttatggataaattcagtactaataatatcatctacattttcttcagcaatggcatctcctgcacccagtttaatggaaccacaggcttcatcttcagcctgtctattgcgaaaggtcagagcttgttcccatcgacgcaatgcctcttcaaacaattccatacccattaagtataagttctctggagtagtcacaggaatattaacaagtttaatatcatcttcatctgctttgtcccaggaattagaattgccacaagcgcagctatgacaagaattgacactctggacagaggccaaactctgtgcagaacctgaatatttactgaaaagtcctccattagcatagttacaaacttgagatcctttgtctttggtagaacttaaagataatgtcaaattctgtctgctactggaacaacttgaacctttgtctgatgctgctcttttagtgtattcaagtatgaggtgctctggttcccatggtaatatttttcctttcttctttccacgttttcttttaaagtgatgagccagaaaaattacagatatagcactcactgcagttaccacaaacaactttttagccaccggagaaaatttgatctgggagagagaatagtaccaagtcagaggaagatcaaacactcttagcgctgctgtcttcaaggaaaactgtgattcacttactgtttcttctgacatggctcctcttctaatctggagctccaggccaggtacagctggcctgcccacgccagcttcccagctgatgcctggcgctgagcagcagtctgacatggagaaggcggagtccttccggggtcaggagt

SEQ ID NO: 12682 - RNA, 5769 nt, Homo sapiens
  source 1..5769: mol_type = other RNA
gatctcactttgttgcccaggctggagtgcagtggtgggatctcagctcaccacaacctctgcctcccaggttcaagagattctcctgtctcagcctcccaagtagctgggatcacaggcatccaccaccatgcccagctaattttgtatttttagtagagacggaggtttcaccatgttggccagcctggactcaaactcccaacctcaggtgatcagcccgcttcggcctcccaaagtgctgggattacaggcgtgagccactgcacccggcctgtcactgttatcttgaacacgctgtcagtcagtactcctaggcatttatatttatttactatgttaagtaaaaaatggtttataaattgttgcaattgctggattcttttattaccagatcatattccttttcatattttaagatgaaaaaattatcatttctcttctgcaaactagctaagaagaagctgtacacactaaaactgttttgcagatttcctaagccaagcataagtaaacttgagtgctatccttttgtctatctacaatttagcttcaatagagagcctttacattacatcaaatcatctgtaacacaagaagcttaacaccagctgttttgaaagttgtgccatatggccaggtatcgaacactcaggaacataaacaggtatcttggggaaagttactgaatagttaatgcaaagcagattgtgttacagtaataaagagccaaaagtaagtaagactgaggtcagttagaaaagttttttgttggtttgtttgtttttgcttagcatagtggtcacatctgttcatcatgtatactcctatcagagcaaactacctgcagttccccaatgtaccacactcttccataactcaatgcctttgaccatagggtcatgccttccaaaaattatctctatgtatttctttacctggtgagcttctattttttctttttgactcaactgaaacaatccccaggtggaaacttctctcactttcctctgtttcaatggcacattgtctgtacctatattacaatatatattccttcgcttattgaaactgcttacttgctggttttgtcccctggaagtcagaaactatggcttcttcatcccagcatttccagtattacgtacagagcctggcactctgatataagaaatgatagccagcagagagatgttctgcaccttctgtcttgatatgcacaaacatgtgagttgatgccacctacacttccagtggtatagccacattctcaggtaggacacccatttatcttgaaatacttaacattctgaattctggaacagaattttaagatccatgtcgatgtccttgtaaggtaactccctctgtttaacaataaaaaaaaaagtctcacatttaacacgtgtttccacactcataaatacatacaaaagttgggagacctgtcttagaaacatgtttaaaatgaatatatataatattatgaaataaaatctgaataaaaattttattccaacaacacttctctattttaaatcatgtttattatttaagtttttatcacagtggagattaacttatgtttaatcatccaatcagtgcctactgtcaacttaatcaaattccaaaaaagtaaaatcaactcattcatacactctaagtcctcttactatcccaccattcattgcctgtgtcttttttcccttttaacggcaacatcgtaataagattgtgaaaaggtataactaataagtttctatgtatgtataataccatttcttcaagtattcagagagcagtacatttgtctgcattgtacattagaaaactacttgtgacattatttctaagtgcaggagagcagctcctggtgggagagtaatgaagttgtttgtcatagtgtatgccaaggatttacagcactctagaattttcacaactcttccatgttagtgaatgacattaggtaaatgttgtatttgcctactctcagctatcagatgtgggatttcaaactagaaacaaataaagcatacactcaaccaacaagggtagtgcaagtgctaagtaaacagaatgacatggaataaattcatagttgccaactagtgaatgcttcagcagggagaccctgattttatgatgtctgtgacttgcatccctgttctcaaatgaatactgtcactgctccatgtcagctacaatgaccggaaaaggctgctggggtgagggctgagtgaatgaggaagatgacaggaactcattttcacaaacaagtggttcaatttatctgtcacatctgtatatagtgtaaagtctgatttgttaacaagatctcaaacctctccagaaaaagcaggtaccaatatggaaaactgcaaatgttccatttaaaagaattaaatgttggcacctatgtaatatagattgtatggcccagacaataaaagggatcagaagatggttttttaaaagttaaactttggaaatgtaacacctgaacattcaaaaattacattatagaaaagccatcagttacataaacattcaacaatacaatggtgctgtttaaaaatgccctagaagcaataatcttcagtactttgaataaagtcagaatttcattgctttgtcttaattatgcatttaacatattgttactcattaaaatgaaatagaaaaaactataaaattcttccagaggaaaattattggtagtgggaaaacaaaagtaaaacgtgaaaaccaatgtatacatttacttaattacatgtttttcccccagaagtggccatactctatcagaaaagaaaaacaatacaaacaacaacaacaaaaaataactaaaaaaaaaaatacaaaaaactgtgccatttcttttttttttttcttcctctgcatccagttttggggggaagtgttctttcatggtagtgttctgagttcacacacattaaatgctagaaaagaaacatctggatcctgactatccttttactttattcttgagtgtgttgtaccctcaacaaatgtaacaagcagccagtaaaaattctcttaattaggacacacacacacacacacaaacacacacacacacacacacacatacacacacacacattattaagaaaaatgaaaccattcctgatccgggacacgcacatatcaagatttaaaactaaggtctgacacagtcactgaattgatttaaataattaaggcttctaaaaggttcagtgccaaaactctctacatcagtatttgaataaaatacatttctgcattttaggtttgtgctttttacagccatcttaattccacagaatttcattagtagatctcataagggcatgttagaattgtttactgatgttttacttttagtagctgttagactaaataatagcaataaaaattcaatgagtgaaccaatttatttctatcacctgggctgttggctcatttcactttcttttcatgtttaatatggccatttcttttgtacttgccattgaggattccattgtggtaatgtccattaactgtgctatgcttatttctagaccacagacttttgatttttctgtagataaattttgtcacccaagacaagagaaagtataacaaggcagcaccaagcaaaagcacaaaggcaatatccagtaaaaaatactgacaaaaggagatctgatggacagcggcacgtaggtgatgggctccattgtgacgaataatataatctatccaatagatagttcgattgacagggtgaccaggttgatccttgtgaatttccgaaagcttctgagccctctgacggtagctgggattattgataaccttcactagtgcttcatagagctctttttcagtaactgtcttccattctagcaatatccccatgccttttgcctgtactctggtcatagtatcataatggtctccaaagagtggaattcccactacaggcacaccatgatatatagtttcaaaaatactgttcaaaccaccatggctcaggaaggctttaatctttgaatgcccaagcaggtcattttgtggtaaccattctatgagtttagtgttgtttcctagattctttggtttgggtccagaaaacctccaaatcactttttgaggcaatctccccagagctcctgccagtttgttagcaatgtcttctgacagatacttgacaccagctccaaaagacaccaagacaaagccatgttcattagcaccatttacccatctttggagatcttctggtagtgggctggctggtttggttaggattcctcctacataaacaacattaggcagagtgggtcttgggaattccagtgctacgtcagtacacagcatccacaggctggacccatgaaccaaatcatacatggacttctctggcagcaggttgtacttctgcattatcctttcatatttgggaagaaccagaaagctgacccctaatctggaaatgaggtaaacaccggtatttttcatcctttgcagcaagttcatgcggtctgtgaggagtgagttaaactctgggacgtatgctaatggagcaggagcacccacttcagcaggataccaaaggccagttgaaaatacagcatatttaacccctaaaagatgagctatcacaaatccacacatatcattagggtccaccagcagcaggtcaaatttttctttcttcagaccctggatcagggcatggttgccaaccatcaggtcacagttcttagtatagtgatccagtatgtcaaacagttcgattgctgtcaatctcccagagaaaatattccgcatcttggactgtaggaaagcatctgaggtggtactgttaaagatccctgggtagcgctggaggctgtaatgattagatggggcgatgtctctgccttcagagaggaggaacactgtatggtggcctctctcgtgcaaggctgaggctagcgtcttgaaaatgtacatatggctttcaaacataattggcggcacgatgatgattttggcagccttcgctatcccaacagcactccacaggagaatgaaatatggagtgtaagacttcatagcaaaatagtattgtttttctctggatagtgtgaattataagagttttaacttttccttttatgtattcacaaaggaatccacagtgcgcatgtgttactctcactcgtctcttggctgccccgcgcgagtttgagtgtgtgtctgccgcgtaattgtatccgggacagaagggacctgtgtttgtgcgctgaatcaggtgtcgccgccttcggtggttcgggggcgtaagggaggcttcggagttagcgtgttggctaaggagggctctctgggttcacagttgatagcaatgctttaaccgtgtcctccctcgggtcctcagcgcgcctgctcgtccgcagctcccagcgggcggccaggccccccgccccccagccgcgccccgccctgcgtgcggcgagcagagtcggagcgcgccgctgcccttccgcacttggctcagcggggcacgacacgggccgccacgcgctcagcctagcatcactcgcctctgactgcgagcgcctccagctccccgggctggggcatggatgcagacgcgccttcgtaccacgcgctcgcaggctgggcaaggggcagcgcgttgggatccggccagtcgtccgctgagcgaggttggcttgcaggctgggacttttcgcgagccctctgggcgctcgagttgcgaactctgac

SEQ ID NO: 12683 - RNA, 5666 nt, Homo sapiens
  source 1..5666: mol_type = other RNA
gatctcactttgttgcccaggctggagtgcagtggtgggatctcagctcaccacaacctctgcctcccaggttcaagagattctcctgtctcagcctcccaagtagctgggatcacaggcatccaccaccatgcccagctaattttgtatttttagtagagacggaggtttcaccatgttggccagcctggactcaaactcccaacctcaggtgatcagcccgcttcggcctcccaaagtgctgggattacaggcgtgagccactgcacccggcctgtcactgttatcttgaacacgctgtcagtcagtactcctaggcatttatatttatttactatgttaagtaaaaaatggtttataaattgttgcaattgctggattcttttattaccagatcatattccttttcatattttaagatgaaaaaattatcatttctcttctgcaaactagctaagaagaagctgtacacactaaaactgttttgcagatttcctaagccaagcataagtaaacttgagtgctatccttttgtctatctacaatttagcttcaatagagagcctttacattacatcaaatcatctgtaacacaagaagcttaacaccagctgttttgaaagttgtgccatatggccaggtatcgaacactcaggaacataaacaggtatcttggggaaagttactgaatagttaatgcaaagcagattgtgttacagtaataaagagccaaaagtaagtaagactgaggtcagttagaaaagttttttgttggtttgtttgtttttgcttagcatagtggtcacatctgttcatcatgtatactcctatcagagcaaactacctgcagttccccaatgtaccacactcttccataactcaatgcctttgaccatagggtcatgccttccaaaaattatctctatgtatttctttacctggtgagcttctattttttctttttgactcaactgaaacaatccccaggtggaaacttctctcactttcctctgtttcaatggcacattgtctgtacctatattacaatatatattccttcgcttattgaaactgcttacttgctggttttgtcccctggaagtcagaaactatggcttcttcatcccagcatttccagtattacgtacagagcctggcactctgatataagaaatgatagccagcagagagatgttctgcaccttctgtcttgatatgcacaaacatgtgagttgatgccacctacacttccagtggtatagccacattctcaggtaggacacccatttatcttgaaatacttaacattctgaattctggaacagaattttaagatccatgtcgatgtccttgtaaggtaactccctctgtttaacaataaaaaaaaaagtctcacatttaacacgtgtttccacactcataaatacatacaaaagttgggagacctgtcttagaaacatgtttaaaatgaatatatataatattatgaaataaaatctgaataaaaattttattccaacaacacttctctattttaaatcatgtttattatttaagtttttatcacagtggagattaacttatgtttaatcatccaatcagtgcctactgtcaacttaatcaaattccaaaaaagtaaaatcaactcattcatacactctaagtcctcttactatcccaccattcattgcctgtgtcttttttcccttttaacggcaacatcgtaataagattgtgaaaaggtataactaataagtttctatgtatgtataataccatttcttcaagtattcagagagcagtacatttgtctgcattgtacattagaaaactacttgtgacattatttctaagtgcaggagagcagctcctggtgggagagtaatgaagttgtttgtcatagtgtatgccaaggatttacagcactctagaattttcacaactcttccatgttagtgaatgacattaggtaaatgttgtatttgcctactctcagctatcagatgtgggatttcaaactagaaacaaataaagcatacactcaaccaacaagggtagtgcaagtgctaagtaaacagaatgacatggaataaattcatagttgccaactagtgaatgcttcagcagggagaccctgattttatgatgtctgtgacttgcatccctgttctcaaatgaatactgtcactgctccatgtcagctacaatgaccggaaaaggctgctggggtgagggctgagtgaatgaggaagatgacaggaactcattttcacaaacaagtggttcaatttatctgtcacatctgtatatagtgtaaagtctgatttgttaacaagatctcaaacctctccagaaaaagcaggtaccaatatggaaaactgcaaatgttccatttaaaagaattaaatgttggcacctatgtaatatagattgtatggcccagacaataaaagggatcagaagatggttttttaaaagttaaactttggaaatgtaacacctgaacattcaaaaattacattatagaaaagccatcagttacataaacattcaacaatacaatggtgctgtttaaaaatgccctagaagcaataatcttcagtactttgaataaagtcagaatttcattgctttgtcttaattatgcatttaacatattgttactcattaaaatgaaatagaaaaaactataaaattcttccagaggaaaattattggtagtgggaaaacaaaagtaaaacgtgaaaaccaatgtatacatttacttaattacatgtttttcccccagaagtggccatactctatcagaaaagaaaaacaatacaaacaacaacaacaaaaaataactaaaaaaaaaaatacaaaaaactgtgccatttcttttttttttttcttcctctgcatccagttttggggggaagtgttctttcatggtagtgttctgagttcacacacattaaatgctagaaaagaaacatctggatcctgactatccttttactttattcttgagtgtgttgtaccctcaacaaatgtaacaagcagccagtaaaaattctcttaattaggacacacacacacacacacaaacacacacacacacacacacacatacacacacacacattattaagaaaaatgaaaccattcctgatccgggacacgcacatatcaagatttaaaactaaggtctgacacagtcactgaattgatttaaataattaaggcttctaaaaggttcagtgccaaaactctctacatcagtatttgaataaaatacatttctgcattttaggtttgtgctttttacagccatcttaattccacagaatttcattagtagatctcataagggcatgttagaattgtttactgatgttttacttttagtagctgttagactaaataatagcaataaaaattcaatgagtgaaccaatttatttctatcacctgggctgttggctcatttcactttcttttcatgtttaatatggccatttcttttgtacttgccattgaggattccattgtggtaatgtccattaactgtgctatgcttatttctagaccacagacttttgatttttctgtagataaattttgtcacccaagacaagagaaagtataacaaggcagcaccaagcaaaagcacaaaggcaatatccagtaaaaaatactgacaaaaggagatctgatggacagcggcacgtaggtgatgggctccattgtgacgaataatataatctatccaatagatagttcgattgacagggtgaccaggttgatccttgtgaatttccgaaagcttctgagccctctgacggtagctgggattattgataaccttcactagtgcttcatagagctctttttcagtaactgtcttccattctagcaatatccccatgccttttgcctgtactctggtcatagtatcataatggtctccaaagagtggaattcccactacaggcacaccatgatatatagtttcaaaaatactgttcaaaccaccatggctcaggaaggctttaatctttgaatgcccaagcaggtcattttgtggtaaccattctatgagtttagtgttgtttcctagattctttggtttgggtccagaaaacctccaaatcactttttgaggcaatctccccagagctcctgccagtttgttagcaatgtcttctgacagatacttgacaccagctccaaaagacaccaagacaaagccatgttcattagcaccatttacccatctttggagatcttctggtagtgggctggctggtttggttaggattcctcctacataaacaacattaggcagagtgggtcttgggaattccagtgctacgtcagtacacagcatccacaggctggacccatgaaccaaatcatacatggacttctctggcagcaggttgtacttctgcattatcctttcatatttgggaagaaccagaaagctgacccctaatctggaaatgaggtaaacaccggtatttttcatcctttgcagcaagttcatgcggtctgtgaggagtgagttaaactctgggacgtatgctaatggagcaggagcacccacttcagcaggataccaaaggccagttgaaaatacagcatatttaacccctaaaagatgagctatcacaaatccacacatatcattagggtccaccagcagcaggtcaaatttttctttcttcagaccctggatcagggcatggttgccaaccatcaggtcacagttcttagtatagtgatccagtatgtcaaacagttcgattgctgtcaatctcccagagaaaatattccgcatcttggactgtaggaaagcatctgaggtggtactgttaaagatccctgggtagcgctggaggctgtaatgattagatggggcgatgtctctgccttcagagaggaggaacactgtatggtggcctctctcgtgcaaggctgaggctagcgtcttgaaaatgtacatatggctttcaaacataattggcggcacgatgatgattttggcagccttcgctatcccaacagcactccacaggagaatgaaatatggagtgtaagacttcatagcaggctccctcgccgctcctccagtccatggaaggcgcccttctttttgccagcagcgcgtccttctctccccgcccgcaggcgctcacctcttctctaatcccgggggcccgcacaggcttctctaatgcaagggcaccccgtaccattcccaaatcggcgcggggacccgtgaaaccctgccaccactgtacactgtccattgtcgagagtcgcgcgggcacgcggaaacggcgggccccgaaaagtctcagcgagcttgtacagccccaagacattccccacccccaacacatcccgctcttgttcctccttagggggaagacggagtaaaggggagttgaagaggtcccgaagctcctcctggtcccccacctccatccctgccctggcagctggctctggcctctgggctccgcggtgcccatcccttcaggggtcaagtacaaggtcctcggccgaatcgcctccccgttataccctccctctgccttgagcgcacaaacgcgagagaaccctcgaacggatgccatatggcagaaacaggatcgcgggcgctatgaggggccagcc

SEQ ID NO: 12684 - RNA, 5696 nt, Homo sapiens
  source 1..5696: mol_type = other RNA
gatctcactttgttgcccaggctggagtgcagtggtgggatctcagctcaccacaacctctgcctcccaggttcaagagattctcctgtctcagcctcccaagtagctgggatcacaggcatccaccaccatgcccagctaattttgtatttttagtagagacggaggtttcaccatgttggccagcctggactcaaactcccaacctcaggtgatcagcccgcttcggcctcccaaagtgctgggattacaggcgtgagccactgcacccggcctgtcactgttatcttgaacacgctgtcagtcagtactcctaggcatttatatttatttactatgttaagtaaaaaatggtttataaattgttgcaattgctggattcttttattaccagatcatattccttttcatattttaagatgaaaaaattatcatttctcttctgcaaactagctaagaagaagctgtacacactaaaactgttttgcagatttcctaagccaagcataagtaaacttgagtgctatccttttgtctatctacaatttagcttcaatagagagcctttacattacatcaaatcatctgtaacacaagaagcttaacaccagctgttttgaaagttgtgccatatggccaggtatcgaacactcaggaacataaacaggtatcttggggaaagttactgaatagttaatgcaaagcagattgtgttacagtaataaagagccaaaagtaagtaagactgaggtcagttagaaaagttttttgttggtttgtttgtttttgcttagcatagtggtcacatctgttcatcatgtatactcctatcagagcaaactacctgcagttccccaatgtaccacactcttccataactcaatgcctttgaccatagggtcatgccttccaaaaattatctctatgtatttctttacctggtgagcttctattttttctttttgactcaactgaaacaatccccaggtggaaacttctctcactttcctctgtttcaatggcacattgtctgtacctatattacaatatatattccttcgcttattgaaactgcttacttgctggttttgtcccctggaagtcagaaactatggcttcttcatcccagcatttccagtattacgtacagagcctggcactctgatataagaaatgatagccagcagagagatgttctgcaccttctgtcttgatatgcacaaacatgtgagttgatgccacctacacttccagtggtatagccacattctcaggtaggacacccatttatcttgaaatacttaacattctgaattctggaacagaattttaagatccatgtcgatgtccttgtaaggtaactccctctgtttaacaataaaaaaaaaagtctcacatttaacacgtgtttccacactcataaatacatacaaaagttgggagacctgtcttagaaacatgtttaaaatgaatatatataatattatgaaataaaatctgaataaaaattttattccaacaacacttctctattttaaatcatgtttattatttaagtttttatcacagtggagattaacttatgtttaatcatccaatcagtgcctactgtcaacttaatcaaattccaaaaaagtaaaatcaactcattcatacactctaagtcctcttactatcccaccattcattgcctgtgtcttttttcccttttaacggcaacatcgtaataagattgtgaaaaggtataactaataagtttctatgtatgtataataccatttcttcaagtattcagagagcagtacatttgtctgcattgtacattagaaaactacttgtgacattatttctaagtgcaggagagcagctcctggtgggagagtaatgaagttgtttgtcatagtgtatgccaaggatttacagcactctagaattttcacaactcttccatgttagtgaatgacattaggtaaatgttgtatttgcctactctcagctatcagatgtgggatttcaaactagaaacaaataaagcatacactcaaccaacaagggtagtgcaagtgctaagtaaacagaatgacatggaataaattcatagttgccaactagtgaatgcttcagcagggagaccctgattttatgatgtctgtgacttgcatccctgttctcaaatgaatactgtcactgctccatgtcagctacaatgaccggaaaaggctgctggggtgagggctgagtgaatgaggaagatgacaggaactcattttcacaaacaagtggttcaatttatctgtcacatctgtatatagtgtaaagtctgatttgttaacaagatctcaaacctctccagaaaaagcaggtaccaatatggaaaactgcaaatgttccatttaaaagaattaaatgttggcacctatgtaatatagattgtatggcccagacaataaaagggatcagaagatggttttttaaaagttaaactttggaaatgtaacacctgaacattcaaaaattacattatagaaaagccatcagttacataaacattcaacaatacaatggtgctgtttaaaaatgccctagaagcaataatcttcagtactttgaataaagtcagaatttcattgctttgtcttaattatgcatttaacatattgttactcattaaaatgaaatagaaaaaactataaaattcttccagaggaaaattattggtagtgggaaaacaaaagtaaaacgtgaaaaccaatgtatacatttacttaattacatgtttttcccccagaagtggccatactctatcagaaaagaaaaacaatacaaacaacaacaacaaaaaataactaaaaaaaaaaatacaaaaaactgtgccatttcttttttttttttcttcctctgcatccagttttggggggaagtgttctttcatggtagtgttctgagttcacacacattaaatgctagaaaagaaacatctggatcctgactatccttttactttattcttgagtgtgttgtaccctcaacaaatgtaacaagcagccagtaaaaattctcttaattaggacacacacacacacacacaaacacacacacacacacacacacatacacacacacacattattaagaaaaatgaaaccattcctgatccgggacacgcacatatcaagatttaaaactaaggtctgacacagtcactgaattgatttaaataattaaggcttctaaaaggttcagtgccaaaactctctacatcagtatttgaataaaatacatttctgcattttaggtttgtgctttttacagccatcttaattccacagaatttcattagtagatctcataagggcatgttagaattgtttactgatgttttacttttagtagctgttagactaaataatagcaataaaaattcaatgagtgaaccaatttatttctatcacctgggctgttggctcatttcactttcttttcatgtttaatatggccatttcttttgtacttgccattgaggattccattgtggtaatgtccattaactgtgctatgcttatttctagaccacagacttttgatttttctgtagataaattttgtcacccaagacaagagaaagtataacaaggcagcaccaagcaaaagcacaaaggcaatatccagtaaaaaatactgacaaaaggagatctgatggacagcggcacgtaggtgatgggctccattgtgacgaataatataatctatccaatagatagttcgattgacagggtgaccaggttgatccttgtgaatttccgaaagcttctgagccctctgacggtagctgggattattgataaccttcactagtgcttcatagagctctttttcagtaactgtcttccattctagcaatatccccatgccttttgcctgtactctggtcatagtatcataatggtctccaaagagtggaattcccactacaggcacaccatgatatatagtttcaaaaatactgttcaaaccaccatggctcaggaaggctttaatctttgaatgcccaagcaggtcattttgtggtaaccattctatgagtttagtgttgtttcctagattctttggtttgggtccagaaaacctccaaatcactttttgaggcaatctccccagagctcctgccagtttgttagcaatgtcttctgacagatacttgacaccagctccaaaagacaccaagacaaagccatgttcattagcaccatttacccatctttggagatcttctggtagtgggctggctggtttggttaggattcctcctacataaacaacattaggcagagtgggtcttgggaattccagtgctacgtcagtacacagcatccacaggctggacccatgaaccaaatcatacatggacttctctggcagcaggttgtacttctgcattatcctttcatatttgggaagaaccagaaagctgacccctaatctggaaatgaggtaaacaccggtatttttcatcctttgcagcaagttcatgcggtctgtgaggagtgagttaaactctgggacgtatgctaatggagcaggagcacccacttcagcaggataccaaaggccagttgaaaatacagcatatttaacccctaaaagatgagctatcacaaatccacacatatcattagggtccaccagcagcaggtcaaatttttctttcttcagaccctggatcagggcatggttgccaaccatcaggtcacagttcttagtatagtgatccagtatgtcaaacagttcgattgctgtcaatctcccagagaaaatattccgcatcttggactgtaggaaagcatctgaggtggtactgttaaagatccctgggtagcgctggaggctgtaatgattagatggggcgatgtctctgccttcagagaggaggaacactgtatggtggcctctctcgtgcaaggctgaggctagcgtcttgaaaatgtacatatggctttcaaacataattggcggcacgatgatgattttggcagccttcgctatcccaacagcactccacaggagaatgaaatatggagtgtaagacttcatagctcagggagcaaacaacgcccctctcctccacccagaccgcccccccttccgccctctggaacggcgtggtccctccgctcacctcgtctcttggctgccccgcgcgagtttgagtgtgtgtctgccgcgtaattgtatccgggacagaagggacctgtgtttgtgcgctgaatcaggtgtcgccgccttcggtggttcgggggcgtaagggaggcttcggagttagcgtgttggctaaggagggctctctgggttcacagttgatagcaatgctttaaccgtgtcctccctcgggtcctcagcgcgcctgctcgtccgcagctcccagcgggcggccaggccccccgccccccagccgcgccccgccctgcgtgcggcgagcagagtcggagcgcgccgctgcccttccgcacttggctcagcggggcacgacacgggccgccacgcgctcagcctagcatcactcgcctctgactgcgagcgcctccagctccccgggctggggcatggatgcagacgcgccttcgtaccacgcgctcgcaggctgggcaaggggcagcgcgttgggatccggccagtcgtccgctgagcgaggttggctt

SEQ ID NO: 12685 - RNA, 5611 nt, Homo sapiens
  source 1..5611: mol_type = other RNA
gatctcactttgttgcccaggctggagtgcagtggtgggatctcagctcaccacaacctctgcctcccaggttcaagagattctcctgtctcagcctcccaagtagctgggatcacaggcatccaccaccatgcccagctaattttgtatttttagtagagacggaggtttcaccatgttggccagcctggactcaaactcccaacctcaggtgatcagcccgcttcggcctcccaaagtgctgggattacaggcgtgagccactgcacccggcctgtcactgttatcttgaacacgctgtcagtcagtactcctaggcatttatatttatttactatgttaagtaaaaaatggtttataaattgttgcaattgctggattcttttattaccagatcatattccttttcatattttaagatgaaaaaattatcatttctcttctgcaaactagctaagaagaagctgtacacactaaaactgttttgcagatttcctaagccaagcataagtaaacttgagtgctatccttttgtctatctacaatttagcttcaatagagagcctttacattacatcaaatcatctgtaacacaagaagcttaacaccagctgttttgaaagttgtgccatatggccaggtatcgaacactcaggaacataaacaggtatcttggggaaagttactgaatagttaatgcaaagcagattgtgttacagtaataaagagccaaaagtaagtaagactgaggtcagttagaaaagttttttgttggtttgtttgtttttgcttagcatagtggtcacatctgttcatcatgtatactcctatcagagcaaactacctgcagttccccaatgtaccacactcttccataactcaatgcctttgaccatagggtcatgccttccaaaaattatctctatgtatttctttacctggtgagcttctattttttctttttgactcaactgaaacaatccccaggtggaaacttctctcactttcctctgtttcaatggcacattgtctgtacctatattacaatatatattccttcgcttattgaaactgcttacttgctggttttgtcccctggaagtcagaaactatggcttcttcatcccagcatttccagtattacgtacagagcctggcactctgatataagaaatgatagccagcagagagatgttctgcaccttctgtcttgatatgcacaaacatgtgagttgatgccacctacacttccagtggtatagccacattctcaggtaggacacccatttatcttgaaatacttaacattctgaattctggaacagaattttaagatccatgtcgatgtccttgtaaggtaactccctctgtttaacaataaaaaaaaaagtctcacatttaacacgtgtttccacactcataaatacatacaaaagttgggagacctgtcttagaaacatgtttaaaatgaatatatataatattatgaaataaaatctgaataaaaattttattccaacaacacttctctattttaaatcatgtttattatttaagtttttatcacagtggagattaacttatgtttaatcatccaatcagtgcctactgtcaacttaatcaaattccaaaaaagtaaaatcaactcattcatacactctaagtcctcttactatcccaccattcattgcctgtgtcttttttcccttttaacggcaacatcgtaataagattgtgaaaaggtataactaataagtttctatgtatgtataataccatttcttcaagtattcagagagcagtacatttgtctgcattgtacattagaaaactacttgtgacattatttctaagtgcaggagagcagctcctggtgggagagtaatgaagttgtttgtcatagtgtatgccaaggatttacagcactctagaattttcacaactcttccatgttagtgaatgacattaggtaaatgttgtatttgcctactctcagctatcagatgtgggatttcaaactagaaacaaataaagcatacactcaaccaacaagggtagtgcaagtgctaagtaaacagaatgacatggaataaattcatagttgccaactagtgaatgcttcagcagggagaccctgattttatgatgtctgtgacttgcatccctgttctcaaatgaatactgtcactgctccatgtcagctacaatgaccggaaaaggctgctggggtgagggctgagtgaatgaggaagatgacaggaactcattttcacaaacaagtggttcaatttatctgtcacatctgtatatagtgtaaagtctgatttgttaacaagatctcaaacctctccagaaaaagcaggtaccaatatggaaaactgcaaatgttccatttaaaagaattaaatgttggcacctatgtaatatagattgtatggcccagacaataaaagggatcagaagatggttttttaaaagttaaactttggaaatgtaacacctgaacattcaaaaattacattatagaaaagccatcagttacataaacattcaacaatacaatggtgctgtttaaaaatgccctagaagcaataatcttcagtactttgaataaagtcagaatttcattgctttgtcttaattatgcatttaacatattgttactcattaaaatgaaatagaaaaaactataaaattcttccagaggaaaattattggtagtgggaaaacaaaagtaaaacgtgaaaaccaatgtatacatttacttaattacatgtttttcccccagaagtggccatactctatcagaaaagaaaaacaatacaaacaacaacaacaaaaaataactaaaaaaaaaaatacaaaaaactgtgccatttcttttttttttttcttcctctgcatccagttttggggggaagtgttctttcatggtagtgttctgagttcacacacattaaatgctagaaaagaaacatctggatcctgactatccttttactttattcttgagtgtgttgtaccctcaacaaatgtaacaagcagccagtaaaaattctcttaattaggacacacacacacacacacaaacacacacacacacacacacacatacacacacacacattattaagaaaaatgaaaccattcctgatccgggacacgcacatatcaagatttaaaactaaggtctgacacagtcactgaattgatttaaataattaaggcttctaaaaggttcagtgccaaaactctctacatcagtatttgaataaaatacatttctgcattttaggtttgtgctttttacagccatcttaattccacagaatttcattagtagatctcataagggcatgttagaattgtttactgatgttttacttttagtagctgttagactaaataatagcaataaaaattcaatgagtgaaccaatttatttctatcacctgggctgttggctcatttcactttcttttcatgtttaatatggccatttcttttgtacttgccattgaggattccattgtggtaatgtccattaactgtgctatgcttatttctagaccacagacttttgatttttctgtagataaattttgtcacccaagacaagagaaagtataacaaggcagcaccaagcaaaagcacaaaggcaatatccagtaaaaaatactgacaaaaggagatctgatggacagcggcacgtaggtgatgggctccattgtgacgaataatataatctatccaatagatagttcgattgacagggtgaccaggttgatccttgtgaatttccgaaagcttctgagccctctgacggtagctgggattattgataaccttcactagtgcttcatagagctctttttcagtaactgtcttccattctagcaatatccccatgccttttgcctgtactctggtcatagtatcataatggtctccaaagagtggaattcccactacaggcacaccatgatatatagtttcaaaaatactgttcaaaccaccatggctcaggaaggctttaatctttgaatgcccaagcaggtcattttgtggtaaccattctatgagtttagtgttgtttcctagattctttggtttgggtccagaaaacctccaaatcactttttgaggcaatctccccagagctcctgccagtttgttagcaatgtcttctgacagatacttgacaccagctccaaaagacaccaagacaaagccatgttcattagcaccatttacccatctttggagatcttctggtagtgggctggctggtttggttaggattcctcctacataaacaacattaggcagagtgggtcttgggaattccagtgctacgtcagtacacagcatccacaggctggacccatgaaccaaatcatacatggacttctctggcagcaggttgtacttctgcattatcctttcatatttgggaagaaccagaaagctgacccctaatctggaaatgaggtaaacaccggtatttttcatcctttgcagcaagttcatgcggtctgtgaggagtgagttaaactctgggacgtatgctaatggagcaggagcacccacttcagcaggataccaaaggccagttgaaaatacagcatatttaacccctaaaagatgagctatcacaaatccacacatatcattagggtccaccagcagcaggtcaaatttttctttcttcagaccctggatcagggcatggttgccaaccatcaggtcacagttcttagtatagtgatccagtatgtcaaacagttcgattgctgtcaatctcccagagaaaatattccgcatcttggactgtaggaaagcatctgaggtggtactgttaaagatccctgggtagcgctggaggctgtaatgattagatggggcgatgtctctgccttcagagaggaggaacactgtatggtggcctctctcgtgcaaggctgaggctagcgtcttgaaaatgtacatatggctttcaaacataattggcggcacgatgatgattttggcagccttcgctatcccaacagcactccacaggagaatgaaatatggagtgtaagacttcatagctcctcagattgtccttttgccccgacgcactgcatctacttgcactctccgatgcggtttgcctccttcaaatccaaaacacacataccaggctccctcgccgctcctccagtccatggaaggcgcccttctttttgccagcagcgcgtccttctctccccgcccgcaggcgctcacctcttctctaatcccgggggcccgcacaggcttctctaatgcaagggcaccccgtaccattcccaaatcggcgcggggacccgtgaaaccctgccaccactgtacactgtccattgtcgagagtcgcgcgggcacgcggaaacggcgggccccgaaaagtctcagcgagcttgtacagccccaagacattccccacccccaacacatcccgctcttgttcctccttagggggaagacggagtaaaggggagttgaagaggtcccgaagctcctcctggtcccccacctccatccctgccctggcagctggctctggcctctgggctccgcggtgcccatc

SEQ ID NO: 12686 - RNA, 5261 nt, Homo sapiens
  source 1..5261: mol_type = other RNA
gatctcactttgttgcccaggctggagtgcagtggtgggatctcagctcaccacaacctctgcctcccaggttcaagagattctcctgtctcagcctcccaagtagctgggatcacaggcatccaccaccatgcccagctaattttgtatttttagtagagacggaggtttcaccatgttggccagcctggactcaaactcccaacctcaggtgatcagcccgcttcggcctcccaaagtgctgggattacaggcgtgagccactgcacccggcctgtcactgttatcttgaacacgctgtcagtcagtactcctaggcatttatatttatttactatgttaagtaaaaaatggtttataaattgttgcaattgctggattcttttattaccagatcatattccttttcatattttaagatgaaaaaattatcatttctcttctgcaaactagctaagaagaagctgtacacactaaaactgttttgcagatttcctaagccaagcataagtaaacttgagtgctatccttttgtctatctacaatttagcttcaatagagagcctttacattacatcaaatcatctgtaacacaagaagcttaacaccagctgttttgaaagttgtgccatatggccaggtatcgaacactcaggaacataaacaggtatcttggggaaagttactgaatagttaatgcaaagcagattgtgttacagtaataaagagccaaaagtaagtaagactgaggtcagttagaaaagttttttgttggtttgtttgtttttgcttagcatagtggtcacatctgttcatcatgtatactcctatcagagcaaactacctgcagttccccaatgtaccacactcttccataactcaatgcctttgaccatagggtcatgccttccaaaaattatctctatgtatttctttacctggtgagcttctattttttctttttgactcaactgaaacaatccccaggtggaaacttctctcactttcctctgtttcaatggcacattgtctgtacctatattacaatatatattccttcgcttattgaaactgcttacttgctggttttgtcccctggaagtcagaaactatggcttcttcatcccagcatttccagtattacgtacagagcctggcactctgatataagaaatgatagccagcagagagatgttctgcaccttctgtcttgatatgcacaaacatgtgagttgatgccacctacacttccagtggtatagccacattctcaggtaggacacccatttatcttgaaatacttaacattctgaattctggaacagaattttaagatccatgtcgatgtccttgtaaggtaactccctctgtttaacaataaaaaaaaaagtctcacatttaacacgtgtttccacactcataaatacatacaaaagttgggagacctgtcttagaaacatgtttaaaatgaatatatataatattatgaaataaaatctgaataaaaattttattccaacaacacttctctattttaaatcatgtttattatttaagtttttatcacagtggagattaacttatgtttaatcatccaatcagtgcctactgtcaacttaatcaaattccaaaaaagtaaaatcaactcattcatacactctaagtcctcttactatcccaccattcattgcctgtgtcttttttcccttttaacggcaacatcgtaataagattgtgaaaaggtataactaataagtttctatgtatgtataataccatttcttcaagtattcagagagcagtacatttgtctgcattgtacattagaaaactacttgtgacattatttctaagtgcaggagagcagctcctggtgggagagtaatgaagttgtttgtcatagtgtatgccaaggatttacagcactctagaattttcacaactcttccatgttagtgaatgacattaggtaaatgttgtatttgcctactctcagctatcagatgtgggatttcaaactagaaacaaataaagcatacactcaaccaacaagggtagtgcaagtgctaagtaaacagaatgacatggaataaattcatagttgccaactagtgaatgcttcagcagggagaccctgattttatgatgtctgtgacttgcatccctgttctcaaatgaatactgtcactgctccatgtcagctacaatgaccggaaaaggctgctggggtgagggctgagtgaatgaggaagatgacaggaactcattttcacaaacaagtggttcaatttatctgtcacatctgtatatagtgtaaagtctgatttgttaacaagatctcaaacctctccagaaaaagcaggtaccaatatggaaaactgcaaatgttccatttaaaagaattaaatgttggcacctatgtaatatagattgtatggcccagacaataaaagggatcagaagatggttttttaaaagttaaactttggaaatgtaacacctgaacattcaaaaattacattatagaaaagccatcagttacataaacattcaacaatacaatggtgctgtttaaaaatgccctagaagcaataatcttcagtactttgaataaagtcagaatttcattgctttgtcttaattatgcatttaacatattgttactcattaaaatgaaatagaaaaaactataaaattcttccagaggaaaattattggtagtgggaaaacaaaagtaaaacgtgaaaaccaatgtatacatttacttaattacatgtttttcccccagaagtggccatactctatcagaaaagaaaaacaatacaaacaacaacaacaaaaaataactaaaaaaaaaaatacaaaaaactgtgccatttcttttttttttttcttcctctgcatccagttttggggggaagtgttctttcatggtagtgttctgagttcacacacattaaatgctagaaaagaaacatctggatcctgactatccttttactttattcttgagtgtgttgtaccctcaacaaatgtaacaagcagccagtaaaaattctcttaattaggacacacacacacacacacaaacacacacacacacacacacacatacacacacacacattattaagaaaaatgaaaccattcctgatccgggacacgcacatatcaagatttaaaactaaggtctgacacagtcactgaattgatttaaataattaaggcttctaaaaggttcagtgccaaaactctctacatcagtatttgaataaaatacatttctgcattttaggtttgtgctttttacagccatcttaattccacagaatttcattagtagatctcataagggcatgttagaattgtttactgatgttttacttttagtagctgttagactaaataatagcaataaaaattcaatgagtgaaccaatttatttctatcacctgggctgttggctcatttcactttcttttcatgtttaatatggccatttcttttgtacttgccattgaggattccattgtggtaatgtccattaactgtgctatgcttatttctagaccacagacttttgatttttctgtagataaattttgtcacccaagacaagagaaagtataacaaggcagcaccaagcaaaagcacaaaggcaatatccagtaaaaaatactgacaaaaggagatctgatggacagcggcacgtaggtgatgggctccattgtgacgaataatataatctatccaatagatagttcgattgacagggtgaccaggttgatccttgtgaatttccgaaagcttctgagccctctgacggtagctgggattattgataaccttcactagtgcttcatagagctctttttcagtaactgtcttccattctagcaatatccccatgccttttgcctgtactctggtcatagtatcataatggtctccaaagagtggaattcccactacaggcacaccatgatatatagtttcaaaaatactgttcaaaccaccatggctcaggaaggctttaatctttgaatgcccaagcaggtcattttgtggtaaccattctatgagtttagtgttgtttcctagattctttggtttgggtccagaaaacctccaaatcactttttgaggcaatctccccagagctcctgccagtttgttagcaatgtcttctgacagatacttgacaccagctccaaaagacaccaagacaaagccatgttcattagcaccatttacccatctttggagatcttctggtagtgggctggctggtttggttaggattcctcctacataaacaacattaggcagagtgggtcttgggaattccagtgctacgtcagtacacagcatccacaggctggacccatgaaccaaatcatacatggacttctctggcagcaggttgtacttctgcattatcctttcatatttgggaagaaccagaaagctgacccctaatctggaaatgaggtaaacaccggtatttttcatcctttgcagcaagttcatgcggtctgtgaggagtgagttaaactctgggacgtatgctaatggagcaggagcacccacttcagcaggataccaaaggccagttgaaaatacagcatatttaacccctaaaagatgagctatcacaaatccacacatatcattagggtccaccagcagcaggtcaaatttttctttcttcagaccctggatcagggcatggttgccaaccatcaggtcacagttcttagtatagtgatccagtatgtcaaacagttcgattgctgtcaatctcccagagaaaatattccgcatcttggactgtaggaaagcatctgaggtggtactgttaaagatccctgggtagcgctggaggctgtaatgattagatggggcgatgtctctgccttcagagaggaggaacactgtatggtggcctctctcgtgcaaggctgaggctagcgtcttgaaaatgtacatatggctttcaaacataattggcggcacgatgatgattttggcagccttcgctatcccaacagcactccacaggagaatgaaatatggagtgtaagacttcatagctcgtctcttggctgccccgcgcgagtttgagtgtgtgtctgccgcgtaattgtatccgggacagaagggacctgtgtttgtgcgctgaatcaggtgtcgccgccttcggtggttcgggggcgtaagggaggcttcggagttagcgtgttggctaaggagggctctct

SEQ ID NO: 12687 - RNA, 268 nt, Homo sapiens
  source 1..268: mol_type = other RNA
gatctcactttgttgcccaggctggagtgcagtgtcacgatcacagcttgctgcagtctcaagcttccagactcaagcgatcctcccacttcagcctccagtgagttgtcttctcatttttctgttccttcaacctctccctctccactagctggtttccctcacaggaccaacacgcatgtgcagtatttgcttccaccgaggtccgtgaggtgtgtgctaaccaaggggcggctcacaaccgtgacagactgccattcctgagtct

SEQ ID NO: 12688 - RNA, 416 nt, Homo sapiens
  source 1..416: mol_type = other RNA
gatctcactttgttgcccaggctggagtgcagtgtcacgatcacagcttgctgcagtctcaagcttccagactcaagcgatcctcccacttcagcctccagtgagttgtcttctcatttttctgttccttcaacctctccctctccactagctggtttccctcacaggaccaacacgcatgtgcagtatttgcttccaccgaggtccgtgaggtgtgtgctaaccaaggggcggctcacaaccgtgacagactgccattcctgagtctcttctggccatgggcccccggagccgtgagcgtcgggcaggcgcggtacagaacaccaacgacagcagcgccctcagcaagcgttccctggccgcgcgcgggtacgtgcaggacccctttgccgcgttgctggttccgggcgcggcgc

SEQ ID NO: 12689 - RNA, 387 nt, Homo sapiens
  source 1..387: mol_type = other RNA
gatctcactttgttgcccaggctggagtgcagtgtcacgatcacagcttgctgcagtctcaagcttccagactcaagcgatcctcccacttcagcctccagtgagttgtcttctcatttttctgttccttcaacctctccctctccactagctggtttccctcacaggaccaacacgcatgtgcagtatttgcttccacctcttagagatttctcaactacaaggacttaggcaaggtttcccttttgactggaaggcttgtagaaacgtgacaacccgccttccctaacactcatgtcacagcggtagcggaccgtattctgggacaaatggaactcacgacattccaaagaaaggtcagccgcaagcgaacttagcactggctac

SEQ ID NO: 12690 - RNA, 412 nt, Homo sapiens
  source 1..412: mol_type = other RNA
gatctcactttgttgcccaggctggagtgcagtgtcacgatcacagcttgctgcagtctcaagcttccagactcaagcgatcctcccacttcagcctccagtgagttgtcttctcatttttctgttccttcaacctctccctctccactagctggtttccctcacaggaccaacacgcatgtgcagtatttgcttccacctcttagagatttctcaactacaaggacttaggcaaggtttcccttttgactggaaggcttgtagaaacgtgacaacccgccttccctaacactcatgtcacagcggtagcggaccgtattctgggacaaatggaactcacgacattccaaagaaaggtcagccgcaagcgaacttagcactggctacaccctcctcaattctggttggcgag

SEQ ID NO: 12691 - RNA, 246 nt, Homo sapiens
  source 1..246: mol_type = other RNA
gatctcactttgttgcccaggctggagtgcagtgtcacgatcacagcttgctgcagtctcaagcttccagactcaagcgatcctcccacttcagcctccagtgagttgtcttctcatttttctgttccttcaacctctccctctccactagctggtttccctcacaggaccaacacgcatgtgcagtatttgcttccacgacattccaaagaaaggtcagccgcaagcgaacttagcactggctac

SEQ ID NO: 12692 - RNA, 285 nt, Homo sapiens
  source 1..285: mol_type = other RNA
gatctcactttgttgcccaggctggagtgcagtgtcacgatcacagcttgctgcagtctcaagcttccagactcaagcgatcctcccacttcagcctccagtgagttgtcttctcatttttctgttccttcaacctctccctctccactagctggtttccctcacaggaccaacacgcatgtgcagtatttgcttccacgacattccaaagaaaggtcagccgcaagcgaacttagcactggctacaccctcctcaattctggttggcgagatgcgctcttcccg

SEQ ID NO: 12693 - RNA, 282 nt, Homo sapiens
  source 1..282: mol_type = other RNA
gatctcactttgttgcccaggctggagtgcagtgtcacgatcacagcttgctgcagtctcaagcttccagactcaagcgatcctcccacttcagcctcctcttagagatttctcaactacaaggacttaggcaaggtttcccttttgactggaaggcttgtagaaacgtgacaacccgccttccctaacactcatgtcacagcggtagcggaccgtattctgggacaaatggaactcacgacattccaaagaaaggtcagccgcaagcgaacttagcactgg

SEQ ID NO: 12694 - RNA, 286 nt, Homo sapiens
  source 1..286: mol_type = other RNA
gatctcactttgttgcccaggctggagtgcagtgtcacgatcacagcttgctgcagtctcaagcttccagactcaagcgatcctcccacttcagcctcctcttagagatttctcaactacaaggacttaggcaaggtttcccttttgactggaaggcttgtagaaacgtgacaacccgccttccctaacactcatgtcacagcggtagcggaccgtattctgggacaaatggaactcacgacattccaaagaaaggtcagccgcaagcgaacttagcactggctac

SEQ ID NO: 12695 - RNA, 3106 nt, Homo sapiens
  source 1..3106: mol_type = other RNA
gatctcactttgttgcccaggctggcctccaaatcctggcttcaagagatctttctgcctcagcatccccaaaagtgttgggatcacaggtgtggagccaccgtgcccccacgccgtcatggacctttttaatgagtataacaggctgacaacatctgaatctttatcaatcttaacatcaaaaaagagagaaaaccagaatgtctcaagcttcctgacatgacacaacaggaagcacaaagcaccacccgtatttaaacagaacctgaatctaatccagcaagtaaacctaactataacttacaagtatgaatgacagtgaaatacagcaaatgataccatgagaaaggcaatcaaccaaatctagaatatgggatatgtaagacaaatgacctttcaacaaatgactgtttttttgaaagggaggggagagttattgttctagattaaaataatgagacataaccatcaacttatggagatataacaaccaattatttggtgtgaaccttaactggatctatactcaaataaaccaaacacaaagacttcttttggataatgggggaaatgtgaatgcggactgggtatcagatattatgttatgaggttttgtgtgacatggcactgcgatgacttcttctgtttacgtgttttaaatagagatgcacactaagatatttacagatgaaacagtaagtctggaatgtgccttaaaaaaactcatagagggtgtggcagctcacacctgtaatcccagcactttcggaggctgagacaggcagattgctagagctcaggagttcaagatcagcctggacaacatggcaaaatcccacctctagaaacctcccccaaacccccgcgtgtgcgcgcgtatgcacacacacacacacgcacacaaaatcagctaggcatggtggcacacgcctgtagtccttgccactcagcaggctgaggtgggaggatcacttgagcccagaagttcagcttgcgcaacacagtgagatcccctctcttaaaaaacatcagaaaaatactcagagtaatgacatgtaagagacacataaggaacccggaagttactttgtgcatgactgaaaacattctagtgttttctaaagtaacttgccttgatttatatatgctcctacaaatatagaaacaaaggaccaaactaaagaggattaaaagtaataagagggtagaaaaagcagagaatttagggattcaggaaaaacaggttccaatataaactaactacatggtcttaggcaagccattcaacctctcaagtatgtttcctcatgttaaaacaaggttaagcccaggtgtggtggctcacgcctgtaatcccagcactttgggaggctgaggcgggtggatcacgaggtcaggtattcgagaccagcctggccaacatggtgaaaccccatctctactaaaaatacaacacttaggcaggagtggtggcaggcgcctgtaatcccagctactcagaaggctaaggcaggagcatcagttgaacccaggaggcggaggttgcagtgagccaagactgtgccattgtactccagcctgggtgacaggatgagactccgtctcaaaaaacaaacaaacaaacaaaaaaaccgcacaaggttaactcccatctcataggattatggaaaatttaaattaagtaagattgaaagtgctctcatttcattcaccaatttgaaagccatttattaagtagccattaggtagcacacacataatatacataaaagagcattactgtgattaaaaatgaaatgagtaatcaaattccaattcaatctaatttaaacttaccatatgggctaaaaaagtcacacgttttaagagaggcttcataattagtaacaagttcctggattatagaaacctgggacaagagtcaaaggtaatcttctgggtgtaattgctttggggtgctgcttactaatttcttcataaatttgaagcctctcttctaaagtgctaatttgtagagctttttccaagccttcataataacaccaattttctgcatttcgatcaatcaagtttttgaacacttcactggcttcttttaatcttcccaatttcaacagtatttcccctttaatttcttccaccaaaagtttatcacatatttgtttctcatacatttctatatgttccaaagattcctgcaacagatctgcctctctcatcacttgattctggtataatatcaattcactatattcataatctattttgtttggaggaacttgctgagtttgtctaaattcttccaacagttttagggccatatcataatctttcagcaaatggtatgcaatagcatatccaatccaggaggcacgctgtgtggggcgcaactgaagaagctggtatcttgtctctcggtaaccttcaaggtctctcatttggatctgcaacagtgagagatccctcaaaatttgcaggttatctttatctaatttgagggcatttcggtaacattttatagcttcatcatattttttatcagaacgctgcaagagtccatatacatgccaacagacatgactcttgacatcattacgaagtcctttacgaacaaactcataagcttcttctttttttcctaaacagttcagtgttaatcctttcatagccaaagtctctccatgttcagcaaattttgggttcgacagaatcatcttgcaaaacttgaggccatttttgtactgcttctgttcataacatttcaagatgcgtttgaagaggttgctctccttgggcggcagcagcacgttcggcatcgtggccggcagggaggctaggtggccggcagggaggctaggtgcccgggcgctccgcttcgcgggggtgggcaccgggacgaaccgctgctgagagtcgggctgcgggcgatggattagttcattggtctacagttgcaattgggcagcctggctgttcggcacgggtggcaatggagaaggaaggcggtctgagcaggacacgcttcccctgggctccgctttttggccagcggcggcggcggcggttcccgcgcactgcaagatggcagccagggtccgcctcccga

SEQ ID NO: 12696 - RNA, 1077 nt, Homo sapiens
  source 1..1077: mol_type = other RNA
gatctcactttgttgcccaggctggcttcgaactcctggattcaggggatcctgctgcctcggcttcccaaagctctgggattgcaggcgtgagccccacgctggcccctcctccacttttaaggaccttgtgattacactgggccccccgggatgctccagggtcaccaccctagtttaaagtcagctgatccaaccttatttcatctgcaacctggatcccccgagccaggtagtcacaggctcccactaggatgtggacatcgatagggaacactatgctgccaaccaacccctgtctacaagccaaagagcatcccaccaggtagagcccacgaacactcaggggtcttgggcaggaggtgggtggacacagggcgggaaggagatgctcagtggggttgggggaagcaccggccgcgatgggcctcccagatctcagggccaaggcatgggaagctggcaccatgtccgggtccttggggctgtcggtaaacaagtggatcccccatgacacagcagctgctcccaagccccagccggggccggaacacagggcacgttgccatggaatcctggaatcctgcgctgaattgcagtttgtttcaggcaaggacgcccggcactcacgcagctgtgccaggcgggctcctcacagccagaggtgggaacagcaactctggggagaactgagggtgctgtggccaccgggtccctgaggctcacggaggagagtgaggcgaggagaaccatggagctgggccctgccttgggaaccaagcactcgccctttgcagctgcagagccgtcctgatgggcaggcgggggcggggtcgctgtgtagctgtgcagagagcgctccgaatgggggtctgtcaccagctcccaagctcgtgggttctctcaagattcttgtggcacatgattcattgcctttcttaacagcatcgctgaaaggagaaaaggccctttggaaattgattgcagtccctggatgtgtctcttggagcacatgtccctcggttcccacttggcaaaccaggcttcatgtccccaagacagggccaggcagcccat

SEQ ID NO: 12697 - RNA, 2285 nt, Homo sapiens
  source 1..2285: mol_type = other RNA
gatctcactttgttgcccaggctggggtatagtggcatgaacacagctcactgtagccttgatctcccgggctcaagcgatcctcctgcctcagcccccaagtagctgggactacaggcacacaccatcatgcccagctaatttttgtattttttgtagagatggggtttcattcactatgttgcccaggctggattttttttttttttttttttttttttgagacaagatcttgctctatcatccagcctggaatgcagtgtcatgaacataagctcactgcagcctagacctcctgggctcaagtgatcctctcacctcagcctactgaggagctggaactacagaggcaccagacccagctaactttgtgtagaaacagggttttgccatgttgcccaggctgttctcaaactcctgggctacaatctacctgccttggcttcccaaagtgctggccacggcccccagcctaacattttgaaaattattattattattattttcttgctctgtcacccaggctggagtgcagtggtgcaatctcagctctcagctcacctccgtctgctcggttcaattgattctcctgcctcagcctcctgagtagctgagattacaggcatgcgccaccatgcctggctaatttttgtagaaaattattatttctatgttacatcattttaacaatgcagtggttatctttgacctaaaaactaaagtttaaaaaccattttttaaattaaagaatgcaattagtacattcttgttgctgacatgaagattacagtgcatacctagctcctttcattatttataattcaaatctttgttgtacttcatctgcaatcattccagaaattgcaatggaagaagtagcagcaggagaaggtgcatttctcacatgaagaatgcgatttccaatatccccaactcctgcatcaaatacaaaatcttctaccagatttccatctctatccagggcctgggctcttactccagctgggcccctaagtatatcactgatagtaatttcagggatgaatttttgaagatacttcactgttgcaccaagaaaacatgctttatacatttcagtaactccataggaaaaattctgggatgccagtttaatcaagccactattgataattatatccataacatctgtggcactgaagtcaaagggtctgtaaccctctcgtttaaaggcaagaactgcattaggccctagccaaatactgccatccatccttggtgtgaagtgaactcctaggaaaggaaaccggctatctgggaccggataaatatttccttttacaagataacatttttctggcttcaaaagcaggtaatctccccggaatggtacaattcgaggatcaggagtgcagccactcaactctgaaatacggtctgagtaaagtcctgcacatgtcacaacatactgacatcgaatttcctctccctttgtattctttataacaattggatattgcattccatctatacttcttgaaggactttctttagccatttcaataccttttacttcaaaattggtcaagacagagccacctgcttcttggaaatcctgggcaaatgacaaagccacctgccgatagtccacaatgccagtatgtggacaatcaatagccattagacccctacaatatggctccttcttttttatatcctcctgctggatcagcctcaggcccgggacaccattctggaggcctttctcatatagggcctgaagtctgggaatttcttcttgttcaacagctactataagcttgccacactgcttgtaggaaattcccttttgctgacagtactcatagaggagggctgcaccttgtacacataatttggctttcagagactcaggtttataataaattccactatgtatgacaccactgttatgtccagtctggtgaacagctaaatctttctccttttccagaacaccaatagaaagtgatggatgtcgcaggatgagtgctctggcagaggcaagccccacaattccgccaccaacgatgactatatcaaatgagctggtgctggcgctgcggctacctccacacagcggtcttggcctcccagacgcgaacccgcacgccccaggggagccaccggcgaaaagcccgcgggcccgtccgcaggcaccaaccaaataacgcagcgctggcaccatcccctacgcacgctcccctccctcagcgctcagaagaagccacttgaccctccacggccgaggacccgcgctctttagc

SEQ ID NO: 12698 - RNA, 11649 nt, Homo sapiens
  source 1..11649: mol_type = other RNA
gatctcactttgttgcccaggctggtctcaaactcctaggttcaagcaatcctcccatcatggcctcccagcgtgctgggattatgggtatgagccactgcccctggctattattattaacttttaaaaatgtatgtcacatatgccataatcatttccaactctttcaaagtttttttaaatttcagctcaaaatattagaatgaaatgcacactcaagactaaagaagctatattctatgttcgagaaaatgtacaaatattgattctggttttttttgtttcttttttttttgagatggagtcttgccgtctcgcccaggctggagtgtagtggtgtgatcttagctcactgcaacctctgcctcctgggttcaagcaattctcctgcctcagcctctcgagtggctggaattacaggcacccaccaccacgcctggctaattattatattgttagagagatgaggtttcaccatgctggccaggctagtctcaaactcctgacctcaggtgatcaacctgcctcggcctcccaaagtgctgagaatacaggggggtgagccaccacgcctggcctacaaatattgattctatccatggtttggtgaaaaaccatacaagttcagcttattctctgtggcatcagcaggggtcatgtatcaggatggcagagtgctgtccagcgtgctgcagagggaaagtgctgagtgaacacgagttgttacccacttagctgtcccaagttaatcggaatgcggatggacgccgtgcataatcagcatgaaattttatgaagacctgatttgaggaagccacgaagggagctatgctggtgtcgcctccgcagtatggtccagaggatggagagctggcgttgggcccatcatagagtgtgagatagttctggacacagtctcctggatcgtcaatgctgatgaagtagaagttgatggtgacaagccttccagcaggagcaacaaggacccactcgcagtacgtgttgtttgggtatgtgcctggatagccggggctggtgaatgagcctctgtctccataaagagttccaccacatccagagggtgatgaagtccagatgatttcatatccacgatcagaagttacactatcactcttaaatcgtaggtatagttcattattttgagagaagacagggtttggcagcagagttccacagtacttgcccagtaatggtgaattgctgttacttccatttctcacctccaagaaatcgtttctgcattcaactgagttctcgatgccaagtgaatgaaaaaagagggaaatggtgtggttctggggggctgtgagagtaacggtgcaatccttgtcattgtcgtagttatctggccatccagggcttctcaggttgccaaatgccttgtgatagtctctgttgcaatctgcaatctgataggtgaaactcattctagagtttctgtttacaactccagatttgaaaatgaccattgcagtactcatagaagaataaaacactggcacagccgaagcatttctgccacagaactgaaatcttgaatttccgtgaccctgcggtgagtcctgaagctgtaagtaattctgcgtgcagtcttgcgaggtcagctgtaatgcccacacagttatcttgacctgctgatgcggaggggaatcaatgacccaagtacagatggaaaatgggacatctgggtctgatgaattgggtgatgaaatattttgtggggtccaagttgcattgtatgttccaccacaaggcatgtccatgatggtgtatgtagcattaaatccttccctctctaatgttaagtcactgatgaattgaaccgtaaggaagttaccagaagagataaaaggagcaggtactgtggaaccacaaaacgttccagccaagttcgcattttcactatccccatcatataactttacataatcataaaggcatctttgcctagtacttgctgcctccagagcaaatgtattgaaggtgaggtgaattactttgtttacaggtgcaattatgatccatacacagtttaaattcttgtcatacattccattcgaatcagaatcaggagaggcaaaggtattattcgagcctgtcagataaccaccacatccttgctgaggccccaatgtctgccggaaagacatcttccagccttttgctgtctgaaatgaatctgtcttgaacaccaggagcatactattattgctgctcttcacatttggtgggcgcttggaaccgcagaatttgccaagaaggggatcgctggtattggcaccatcgtaaattgccaggtagtcatgggagcaggaggtggagggaaccacatcaaaatcactgaacttgagctcgatcaccttgtcgtcactaacggtgatggtatacagacagtgcatatcatttgggtagtctgcgtatgaataggcaggacttgtgatgattccagaagagaaattgaacacaccaccacaggagattatcctataggaaaacttgaatccgaagtctgtgatttgctcgttggagtagaagttaagcagaaccggcccagcgatggtgaggggagctggcatctcatccccacacacagtagcaaatggggtggacatgacgctgtaacctctgataatgtgcacgccatcgttgacacagcttcccgtcacagcggaacgagcttctaagtggaaggacacaaaagtcaagaggaccactgacagaggattagcctctatgacataggtgcaattcatgttgttgtcatattgttttgggtaatttggagaaatgatgtaacctgaagggccagtgaaattacttccacatcggctaacaaaggacgcggagaagccctgagctggtgcctcctgagactggaagacggcagtgaatgtgttacttggtgtgataacgggacccggagccacgttcccacagccagtggctagcagggctttgtccacctcctcagttcctgcccacaccttcacgaagctattctgacattgtccatcaccgctggggattaggaagttgttgtcaaagctgatctccaagtgtttacttttgtgagtaatggccgtccaggaacatctgctgttttcgggaaaattctgaggccagtgaggggatctgattgtaccattatcagaatgaaatattccaccacaacctaaagtttgtgtgttccacgtagcataaaatccaccaccttgcaatgaatggtctgagttaaaagtcacgaccagctgattggaacctgactgtattgtcctggggtttgaatttccacagtattgtcctatgatgggtgattcaggggacccaccattcctgacagtgacagagtcccaagcacaagttgtatggggttcaatatcaaagtcactaaatgtgagagtgatggtgtgcccttgtggggcctccaacagcgaagagcagtgggtcaggctgtcataagcatttggatagttggggcttgtgatcactccactgtcacctatctgtattccgccacaatctgtaaaggaatactttgcatggaatccaatgtgttctacacgttcgttggtgacaaagtgaatccatacctgagaataaggtataaccaatggcaatgtaggctttgaaggaccacaaagtctccacatcaggggcccatcagcatcacccactcgaaactcgaggacatcaaattgacagtcttggtgactttctaggtaaaaatcttcaaagtgaatggaaatggatgaatttccctgatttggattgctgagagtccattcgcagttcaggtttcttgagtaattcctgactccgtcatagccaggagaagtaaagtttccttcaggagtatttggaagagacccaccacacactgcatcttcactggaggtataggaagcagtgaagccgccatatggcctggatccatccgtgaaaaaaatgactttcattgtgtttcctgaagatttaatctcattgcttacattcacactactacacagtttctctagctggggtgagttacttctaatgccattgaatactatcacatgctcattgttgcaggacggatgcgtggccagcctcaggttgttaaacattagggtgatccgccttccctccggggcagtgattctccactcgcagatccggccatgaggatttgggttcgggtagttgggagaagtaaatgttccaatagagccctgaagatccccaccacactcttccatactggattcaaatcgcagtctgaatcctgaggcagtcacagagccgtctgtgacaaacctgaccacagcagtattgctagaagtgtctatgctgtcaggaatggtgtttccacagtatctgcccaagatgtttccagaggtatgattgtcccagatctccacgaagtctttttcacagccagaagaattctgaaggttaaagtcttcaaaagagatggtgagatagtgtccagagagcccctggagatgccactcacagaataagttgtctctgtatggaagtgttggatgtccaatgctttcaacaacaccactttgccctggtactcttcccccacactgagctatagaatacttggccttgaatcccacatgtgtggggctgttgtcagatcgaaatctcaaatacataacctctcctgaggaccactgactgctgggcaaagatgtcccacaaaatttggaaagtattggtgcatccgaatccactccatcccgcaactcaaggtagttggaagtacagttgggtgttacttcaatatcgaatcgatcttcaaattgcagctgtatgcgtgtttccggtggagccgctaagatccaaatgcaatcagcgtgcgggggataattatgagggtggttgggggaggtcacatacccagcagaatcagcatcatggatgtagacgttgcccccacaggctaaactctttgcctcatatttgattttaaatccttgcccttcattactgtgatcagaaataaactgaacaaacatttgattatccgaggtgaacagagttgatgaagcatgactgccacaaaaatgaccatttcctccagggggtcccaagggtggagaacagatatcaggaccatttcttagcaccaagtaatccccctggttgcaagaagaatctccatttggaatctggaaaggctgttcaaaatggacagcaatggtcaggccactttggaccaggacgtgccaagaacagttgaggttggatgggtaagtctctggatacttgggggacgtgatgatccctctgtctgcatgcaaatatccaccgcagctcttgtgaaaggatgcattgaagcctgccctggttacactggagtccgaggtgaagcggatgaacatgtactctccagtagaccggatgggcccagggatctctctgccacagagaactgctagctgctgggccaagttattatctccatctcgtatcacaaggctatcataggcacacgttcggtgagattcaatgtccagggaaagaatgttgagttccacggtagagtcgggagcctggatgagccacgtacagtccactctattactgtaactgtcaggccagcccggggagaagagaaacacgggtgcatctcccgtcctcaggaagccaccacaagcacctggagcaatggtaggtaaaacaccatcaggtgcatccactgcaaaccactccagaaggaatcccttccctgagattgaagagtcggagtaaaaatgaaatgtcaaagaatttccagtggagctgaaagattcagtctgggtaccacagtaagctccaattaggcgggcgtgaatgctaggcccatcatagatccttaatttgtcataatagcagttttgtatttcttctatgtccatctccaagattctaccatggacaacgtgagatgcattcacatttactgtccattggtaattggagttatgtgggtagttttcaggccagaaaggagaggcgactttcccatgagttcccacaatattatcattgccaaatatcttcataaatgtggcctggaagcccgtgccgctgccagaaccatctgagataaatctgacccacagggtatgtccaacgatggaagaataattgagagggaaggagtttccacagtatcgtcccaccaagtgacccgtggcatttccttcacggatctccacaaaatctctgctgcagtcctgagagtcttccaactggaaagatataaaagacagctggagccggttgccaggggaactgacgatgttccagacacattccacattagggggataaatgtctgggtagccagggctgttgaagatgccttcagccatgtagaacgttccaccacaagccgacactgatgcggtgaccgtggtgtggaaacccccagcactgatgctagaatcagagacgaatctcagcgtcagggcgctgctgaaggatgtgataggatggggcatgtcggtgccacagtaacggcctcggaggggcgcgtcttcgtggccgccatccaaaatttctacaaagtcacgtgcacacgttgtgcttctttcaagttcaaagtgggtaaaagagagggtgatatgatttaatggaggttgcgcttgaatgatccagctgcagttctgattgtttggataattggcagggaaccgtggagaggaaacagtatcaaatgagctggtgaggatgtggcctccgcaggcttgcctgaattgagctcggaagcctctgttctgtctggaagggccagactgaaatctcaagaagaggctgtttcctgaggagacgatggggttagccagctgctcccttccacacgtcctggcaaggcgggacattgtggagcttaagccatcgtatgccataatacaagagtcttgtggttcaagatcaaagtcagtgaagttcaagagaacacgatgatttctgtcaacccgaatgacccaagaacagtctgtgttgctcctataaggactggggtaatttggagaatgaatctctccactgggagcctggaaaatcccaccacaacctccagtgactgcttgccatgacgcattgaagcctctcccatttatggacaagtcggtcttgaatcgaattgctagctcatttccagtgctggagacctgcatggggttctcaggtgatctctgggtacacagttgggctattctgggagagtggaaatcggggcctccatagatctccaagacatcaaagttgcaccttgaatgatactccacatcgaagtcatggatggtgagctgaatgctactcccggggtccgtcctaatgtaccagatacactccttgtttggtggatacctgttggggaacccggggctgctgaaggagcctgtggccccagacagctctccaccacaaccgtaaacaaaccactgcatctgaaatcctttctcacggcggccaaccccatctgtaaggagcagcacttgaagcttggagcttgtagtactccctggagggggcaggtctactccacagtagcgtcccatctgccgtggtccatcatagagctctaaataatctgtggagcagtttatgtgatgttccaagtcaaatgctaaaaatgtgtagttcacagtgttgcctgttgttgcccggatggtccagttgcaatgctgattttcagaataaggattcggataccctatactctctaagatgccataggtttgattgactattaccacattctcacatgtctgccggtattcagccttgaagccacgtccttgctgaccttcatctgtcctcagttttataaacatgctgtctccactagaacgaataagagggggtttctcatccccacaaagctgagttagcagatgagagttgctacttgggccatcatatacagccaggtaatctaaagtgcagtttggatgatgctccaagtgaaagtctttgaattccagttcaaatgcgctgccgtggctagatttcaaccaccagtagcattcagagctgtggtaatagggcatcgggtagttgggagatatgaacgtgccgcttgaagtggtgagattacccccgcaacctgttgatgacccatcccagtaagctgagaatccagaccttgtgtctatttggtcactcttaaattttaaccatagtttgttactatgagagatgattgttgggggtagatttgagccatagaatattcccagcaatggtgatttttcatagcctccatctctgatttccagaaaatctgtataatagtttccaatggcttcctccaaggagaagtttgtgaagtgcactgcaatcagttggccagttctcactgtgatccgataaatgcattcccagttgttgggataattattggggaagtttggagaagtgaatgtccccaaatcatctgtgtagtcttgcaaacatgctgttgctgcactgattgcttcatagtttattaagaagccttcataagcgaggtcggagtcagtcacaaacaccagcatcaatgagttaccactgcttgtgagagatggcgggatcgactttccacagtatcttccaagggatgtctcagagtcggtgtcataaacttccaagtagtcgtttgtgcaattgtaatgaaactccagatgaaatgtttcgaacattaaatgaatcaggtgattaggttggactaatatatgccaagtacagttgataccgtgggggtagacatttggatggccaggactttgaatggtccctgttgattctgtaagaatttctccacatgccaaatcctcagcactgaacttagccatgaaaccatggttttcagtagaagaacttttcacgaatgtgacataaagaaaattgtacacagatgttataaatgaaggtatgtctgtaccgcaatactttttattttcaggagaacccaaaatggaactgctaccaatctcaacataatctgtttcacagtgggcagaacttccaatttcaaagacagtgaagttgaggagaatgacttggctttggggctggtggatggtccacctacaggttctttctccaggatacacgttaggaaaaaaaggcgagcgaatgaccccttctccagttaattcatccccgcaagcgacttgataaacagctctgaaactagctttttcaacagaagcatctattttaaacctgatccagacactattagtaatggatttaatgtgagagatggttccgttgccacagacttttccaagtaaggtttcaccatctcgaacctcaatgtaattctgagaactgtcactctggcattgcagctccacgtgggtgaagttgatttgtatttgttctccctggggctgcttcatcatatagacgcattgcctggtgtgagtgaaaggcccagacaactcaggcaagaagagttcaccctctgggtccgtgtagttcccaccacaacgcagatccgaaggtgatgttaagtaggtgatatggaagccttggtcactaatctgggagtctgaatggaagtgaattctggcaaaggggccagtagtctggagcggtgggacagagaaagtggtgcagaacttcccaagaagggggtcctgatacaaaggaccatctcgaatctcaaggtaatctttgttgcagtcatcatggtgctcgaggctcaaggtcccaaaagtaaatgttaccaggaggtcaggactagttacaacaatccagacacaatctcttcctgggggatagtttccaggataccccggagacttaatagaaccgtaaggaccagtcaggatacctccacactctggttgctgtgtttcccatcttactgtaaagcctctcccatttcttaaatgttcagaatagagatgaaaatagagagcattgtcactgctgaggagttcatgagggaggctggagccacaaaatcttccaagttgaaaagcagaagaggaatctccatcataaacctgaagaaactcgtgtggacagttgtccatggattctaaccggaaaaaagtgaaagtgatacgcaggacctttcccatttcagttttgataacccagaagcagttaacatcatgaacataaccaacatccgggctcctgtagctgaagcttccatttattcctgagagggactctccacaaacttgctgaggaacctgacagagagctccagtccagagacgtgtgcattcacaactgaaagaatcaacgccatcaacacaagttcctccattcaaacaggggttgctcaaacactcattgatgttttctgtacagttgacacctgtccaacctgagtcacacttacaaaaataaccagagacagtgtcgatgcattgtccatttagacaggggtgacttaggcaaatattactgagctgcacacatccatttggcccataaccatttccagtataacccgggagacacgtgcagagaggtaaggaacctagagttgaggagcatgaggcatctgggtggcagcctccattactgactgagcagatgtctgtgagtgtgcacactcttccgtcaccctggtaccctggtggacaggcctggcagtgggaagacccaggtgtattcacacactcaacgggtggagccacagaacagccgccgttatttatctcacattcattgatatcttcgcaaatatatccattgccttgccagcctgttggacaggccccacagtagaaagagccttgagtgttgaaacactgcacaagtgtggagcaaggcccgggctggaagctgcactcgtctctgtccagcgtgcaggcagggctgttgggtgaaaacatccacccagcatcacagacgcagctgtacttgggctctccagcttgctctcgcattaaatcctcacagatgccatggacacagcgtgccacagaacccccttcacagtcgtcatatttggatgcacactggggtccgtacgtctcaggtgggcagtgacaactgtaacttcccattgtattaacacatgtgcctccattctggcagctcaagggtgttcctgagtaaatctcacattcgttaacatcagctgagcagagaggacccttccactgtgggggacagatacaaaaaaaggaatcatgcagattgaggcaggttccaccattctggcaaggattgctgctgcaaacctttttgtcaacagtctgctgcaagccttggaattttctctcaagatccaccagcttggaattaagctgatagatttgactagatatattttgaggcagaccaattgcactcccttttaactctataatatcttctttgtttttctggatctgatgtaaacactcactgagatcttcatcatttaatttaatttttcccagggatccggttctaaactcaatgttttgagcagaccccgtaagaaacaccaaatttcctctctctgtagccattcgaggctgttggagattgatgcttcttttttgtctctgcagctcaagttctccagcttcgccatttacttcagcaaatattaataaggtaagcaaactccaaagaaaaggtaaagacatgttcatcatcaacctcccaggttggcaggtaagagtgaggccactccaaccaact

SEQ ID NO: 12699 - RNA, 5997 nt, Homo sapiens
  source 1..5997: mol_type = other RNA
gatctcactttgttgcccaggctggtctcaaactcctgacctcaagtgatctgcctgcctcggctccccaaagtgcttgggattacaggcgtgagccactgcacccggcccctagcatgattattaaatctcctgattgtatatgaagcccttgtacacatctgggtctgcctctgggttctctgttctgtcactaaatcagaaagtccagggtgaagcccagcaaatctaatgaaagagcaagagtggagaatcctgactgcatggtaatagaatttgtgttagacacacacaaacactacattttccaacctcccttgcctctgggtgaggctgcgtgactaagctctggccagtgaagcaatggcaaaacctctgggtcggtccttaaagaggagtgccttcctctccccgtgcccacttgggagcataaggaattctctaatacgacatgggagaggcaggtgtcccaggaggaaggaaaaagacggaaggaccctagggtgctgatgacttggagtcccacagaggtgggccttttacacgggagggcagtcgtggatcgcaggggttctcaaacgtgagtgggcaccggcatcccccggagggtgtgttaaatacagatcactgggccccaccagcatctgatgcagctggggtggcacacagggatttatttgcgtgtccagtaagctcccagtgatgctgctggtctgggaaccacactgtgagaaccgctggtctgacctggttgcattgtttattttggggctctgtaaacacacctccagcccccaggcggacgaatccatccctgtgcccctcctgggcctccgggcccctcctcacctccggcacctgtcgagagtcattcattcccgtggagtgcctcagctggtcaactaaatgtgggcagagtggatcctctggcaccacccttgtcctaagcactcccctgttccgctccaggcggacgcctgaaacatggatctgtagaccccccgggccggtggggtcaggaagggtctgccaggaggaggctcctgggtgggagtccagggtgggaagctggaagaagccattctgctctggccagacagaggcgagagtggggtttggggaatgccattggcccctctgttcctctagccacacaggtggcagcagcctccttcctctaatgattgctgggcacttggcactctgtggctcctccagccttctcagagctttgtcatgatccaaccaccggtaccaaatccctgccatttgaaacaactctagttggggtctgttttcctgactggctctggcaggaggcagccacgtggggaggaacggggcctcgggcagctttcaccccacgccacccaaagccatgccttcaaactgcagtgagcgggctgggcacggtggctcacgcctgtaatcccagcactttgcggggccaaggagggaggatcccttgaggccaggagttcgaaaccagcctaggcaacatagcaacatcttgtctctaaaaacaaaaaacaaaaaacaaaaaaactcaaaacaaaacaaaacaaaacaaacctgcagtgagtgactgaaggcaccaaaaccagcagagttaccgtggggtcacagatgtggctgggcgagggagctccccgtctctgagcccgtggtttcttcagcaggagagtggagctcctagagctagctgttctcagtgcccgtggggtcgccgggcaccctggctgtgagccttgcgtttctgagatgctctgttctttgccgtccttatctgggtctggaaccatggtcacagaggcctcctgagctgctatctttctggaacaacttgttcacaaggtagaaggaattacctgctccttcaaagtctggtaaacctcatttgaggccaggcatggtggctcatgcctgtaatcccagcactttgggaggctgaggtgggtggatcacgaggtcaggagttcaagaccagtctggccaagatggcgaaatccagtctctactcaaaatacaaaaaattagcctggcgtggtggcaagcgcctgtaatcccagctacttgggaggctgaggcaggagaatcgcttgaacccaggaggcagaagttgcagtgagccaagatcgtgccactgcactccagcctgggcgacagagcgatactccgtctcaaaaaaaaaaaaaaaatctcatttgaaagtgcattcaagcctgaaaccttttatttattctggagtgtgtgtgcagtgaggagacagttattttggtcttgttttctatttcttcttttgccaatgttagcattttttttttttccagaaaggcatccacctcacctaagcctccaatacatcgcagagagcacagctgcttgcaccgctgggtttcactctgtgatgatccatctaggctgtgtttgcacttggcataggccctgccacacacacagtgctctgattcttggggtcaggacctgtgaagggtgggaggcgtggactaacctggaatctctgccctggccactcacttcccgagaggaccaggctgaggtctctggtgctgatgacgcctggctggctttggggacggaggctcactcctggctctctccccactccactgcctccctgggggctggggaggatgcagaaagtggagcccaacagggcctgaggcgcaaagtgccaggatgcagctgcagcagcgatggtggcatggccacctccatgccagtcagattccccccagcgtgggctcggctctgggctcctgcgtggaaggacacacttcacagggtgtctctccgaagccagcagctccaggccagtcagcctcagtcaatccccaaaagcccatctgcccactgaccaatttgccaaatggccttcaatttactaacttgggttagctcctactcaccaaacgcgctcaagacagcctttaaaaggttccaggaaattgcagatttggcaaactgggatcagtctgcacatggactgtggcaaactggctgcttccaggggtggggacaatcctgccccattctggggagtggcaggctgggggagcttactggctgctatgacctgaactccccactccccaccccacccttgccctgccttggctggaatcgtggtttgctcccagatccagaccctctccctgcaaattcccacccaagacagccgggcagggccccctgccccccacacatcgcacacagacacaaaacaagacaatgttttaattgtaaaactaactcgaggcaggggtgggcgggctggggctgcgctgaccgggcaggaacctggttcttcaggcagtggttctgccagggccaccccgcaggacagggaccatctgtcccccaataagggcaggggctagagtgttataaaatgacaatataaatagacttctagaaaagaggaggctgtccaggtgcagtagtcatttgctgcaggggctggagagggtggggggccctgacctgtctccccatccagccacagaaagggggcgcagggctacgggaaaaggccactcttcggacattcatgatcgacccccacaatggctcagggggagagggggctgggtgtcaggcaaggcgccagacaccccttgcaggctggaggacggggtggctggacctttgcacacacacacatgcacactcacacgcgtgcacacactcatacatgttcacctcttagtgttctctccacccccagcgacccccactgcagacttccagtgatgggagggccgctgcccttcctggagacagaagaacatgggggagggcctgtcccagagggtgggggtcctgggagcctcgcttgctcccacgagtccctgtgtttttctaaaagtcacgagatcaaaactggagttcagtagtagggtctcatctacccccagcaaggagggtggtgccacgcggagcatctcccgggctgggaggagtgggaggcctggccccctactggcctcagtggggcgggggtgacccggggggctctttggttgaggggaagggcgctgggcctcatctggtgcggttctggcgcatgaggggcacgatgctggcaggcggccctgccttggccaggaatgggtgcttcagcagctcggctgccgtggcccgctgggcagggtctcgcaccagcaggcggtccaggaagcccttcagggatggcgacaccttgtgcaggttcttcagtcggggtggcaggttgtcccgaatcatcttcatggctttgaggggtggctcgttgaagtaggggggctctccgtccaccatctcaatcaccattatccccagcgaccagatgtctacctctggcccgtagggaaggcgggagatgagctctggggccatccagtagggcgtgccgaccagcgacttccttcggggcacttccttgctcacctgggcgcagaacccaaagtctgacagcttcaccctgccatcatgggtcagcaggatcgagtcgctcttgatgtcccggtggatgacgccctgggcgtggagcaccgacagggcctgcagcactgcaaggcacacggccgcgatctgctcctcgttcatcctggtgtgggtgacgatgtcggtgagggcgcctccttccaggaactccatgaccacccagagctcgtcccccaccaggtagctgttgtacatctccaccacattctcgtgctggtagtccctcatgattaccacctcgttgaagagcagctcgcgcctctgctgcttgcgcaggtccatcttcttgacggccaccagcttgcccgagctgcgcacggtggcgatgcacacgatgcccgtggagccctcgccaatcttgatgaagttgtccaggtaggagcgggggtcgcctgggtccaccaccagctgcagggcagcccggaactgctcatgggatactcgctgtggctcccgctgtggtgagcgggggccagggggcccaggaacagcaggggcggcgggggtgcaggctggaggggccagctggggctctgaggcgtggggtcccagcactccagggctgggggcacctcgggctcgggtgggaggccgggaggaggaggaggaggactgggggatggccaggccccccgctgatggcccgttaggggccacgtcatgaggctccccctgggcaccccgggatgggtggtccgtgtcagccctcgggtaggtgttaaagggccggccagctgccagtttcgccccactggccagaccagcaggctggggggtgccgacatcaggcccggagagggggcgtttgtcccgggaggactcctggggaccccctgagccctccctggaagacttgggcctcttctctggccccgcccgtcgcctgtcaccactgccgccacccgcctcgctgtgaccggcgaaccggcctcggctgcctgccttccctgggccccctctggccgtggtggccggctcctctggcatcccattttcctggcgggcacgggcgggcggcggcgggctgtctctccgcagggagttggagcgtgtcaccgacatgttctcaaactcgtccagcagcagcgtgagggccccatctttggcacctttgctgccccgcacgatggtcttgggggccccgggctggatggaggtgatgcaggcggggtcgacgaggggcttgggccggcgagccgactcctcgatcaggctctgccactggcggggcagccccgtgaacttctgctcgtgctggtcgaagcccgtgtgcacgcggtgctcgaagttggacggcgcggagatctccacccgcttcttcctcttcccaaacatggtgccggggactcggtgcggccggctcggcgccgcagtcgctcgcggcctaactgctcgacctggaactccgcgccctcgcgcctccctcagctctcttgcaccgccaccaccgcggacactcccgccgccatgttgaatccccaacgaacatcc

SEQ ID NO: 12700 - RNA, 6070 nt, Homo sapiens
  source 1..6070: mol_type = other RNA
gatctcactttgttgcccaggctggtctcaaactcctgacctcaagtgatctgcctgcctcggctccccaaagtgcttgggattacaggcgtgagccactgcacccggcccctagcatgattattaaatctcctgattgtatatgaagcccttgtacacatctgggtctgcctctgggttctctgttctgtcactaaatcagaaagtccagggtgaagcccagcaaatctaatgaaagagcaagagtggagaatcctgactgcatggtaatagaatttgtgttagacacacacaaacactacattttccaacctcccttgcctctgggtgaggctgcgtgactaagctctggccagtgaagcaatggcaaaacctctgggtcggtccttaaagaggagtgccttcctctccccgtgcccacttgggagcataaggaattctctaatacgacatgggagaggcaggtgtcccaggaggaaggaaaaagacggaaggaccctagggtgctgatgacttggagtcccacagaggtgggccttttacacgggagggcagtcgtggatcgcaggggttctcaaacgtgagtgggcaccggcatcccccggagggtgtgttaaatacagatcactgggccccaccagcatctgatgcagctggggtggcacacagggatttatttgcgtgtccagtaagctcccagtgatgctgctggtctgggaaccacactgtgagaaccgctggtctgacctggttgcattgtttattttggggctctgtaaacacacctccagcccccaggcggacgaatccatccctgtgcccctcctgggcctccgggcccctcctcacctccggcacctgtcgagagtcattcattcccgtggagtgcctcagctggtcaactaaatgtgggcagagtggatcctctggcaccacccttgtcctaagcactcccctgttccgctccaggcggacgcctgaaacatggatctgtagaccccccgggccggtggggtcaggaagggtctgccaggaggaggctcctgggtgggagtccagggtgggaagctggaagaagccattctgctctggccagacagaggcgagagtggggtttggggaatgccattggcccctctgttcctctagccacacaggtggcagcagcctccttcctctaatgattgctgggcacttggcactctgtggctcctccagccttctcagagctttgtcatgatccaaccaccggtaccaaatccctgccatttgaaacaactctagttggggtctgttttcctgactggctctggcaggaggcagccacgtggggaggaacggggcctcgggcagctttcaccccacgccacccaaagccatgccttcaaactgcagtgagcgggctgggcacggtggctcacgcctgtaatcccagcactttgcggggccaaggagggaggatcccttgaggccaggagttcgaaaccagcctaggcaacatagcaacatcttgtctctaaaaacaaaaaacaaaaaacaaaaaaactcaaaacaaaacaaaacaaaacaaacctgcagtgagtgactgaaggcaccaaaaccagcagagttaccgtggggtcacagatgtggctgggcgagggagctccccgtctctgagcccgtggtttcttcagcaggagagtggagctcctagagctagctgttctcagtgcccgtggggtcgccgggcaccctggctgtgagccttgcgtttctgagatgctctgttctttgccgtccttatctgggtctggaaccatggtcacagaggcctcctgagctgctatctttctggaacaacttgttcacaaggtagaaggaattacctgctccttcaaagtctggtaaacctcatttgaggccaggcatggtggctcatgcctgtaatcccagcactttgggaggctgaggtgggtggatcacgaggtcaggagttcaagaccagtctggccaagatggcgaaatccagtctctactcaaaatacaaaaaattagcctggcgtggtggcaagcgcctgtaatcccagctacttgggaggctgaggcaggagaatcgcttgaacccaggaggcagaagttgcagtgagccaagatcgtgccactgcactccagcctgggcgacagagcgatactccgtctcaaaaaaaaaaaaaaaatctcatttgaaagtgcattcaagcctgaaaccttttatttattctggagtgtgtgtgcagtgaggagacagttattttggtcttgttttctatttcttcttttgccaatgttagcattttttttttttccagaaaggcatccacctcacctaagcctccaatacatcgcagagagcacagctgcttgcaccgctgggtttcactctgtgatgatccatctaggctgtgtttgcacttggcataggccctgccacacacacagtgctctgattcttggggtcaggacctgtgaagggtgggaggcgtggactaacctggaatctctgccctggccactcacttcccgagaggaccaggctgaggtctctggtgctgatgacgcctggctggctttggggacggaggctcactcctggctctctccccactccactgcctccctgggggctggggaggatgcagaaagtggagcccaacagggcctgaggcgcaaagtgccaggatgcagctgcagcagcgatggtggcatggccacctccatgccagtcagattccccccagcgtgggctcggctctgggctcctgcgtggaaggacacacttcacagggtgtctctccgaagccagcagctccaggccagtcagcctcagtcaatccccaaaagcccatctgcccactgaccaatttgccaaatggccttcaatttactaacttgggttagctcctactcaccaaacgcgctcaagacagcctttaaaaggttccaggaaattgcagatttggcaaactgggatcagtctgcacatggactgtggcaaactggctgcttccaggggtggggacaatcctgccccattctggggagtggcaggctgggggagcttactggctgctatgacctgaactccccactccccaccccacccttgccctgccttggctggaatcgtggtttgctcccagatccagaccctctccctgcaaattcccacccaagacagccgggcagggccccctgccccccacacatcgcacacagacacaaaacaagacaatgttttaattgtaaaactaactcgaggcaggggtgggcgggctggggctgcgctgaccgggcaggaacctggttcttcaggcagtggttctgccagggccaccccgcaggacagggaccatctgtcccccaataagggcaggggctagagtgttataaaatgacaatataaatagacttctagaaaagaggaggctgtccaggtgcagtagtcatttgctgcaggggctggagagggtggggggccctgacctgtctccccatccagccacagaaagggggcgcagggctacgggaaaaggccactcttcggacattcatgatcgacccccacaatggctcagggggagagggggctgggtgtcaggcaaggcgccagacaccccttgcaggctggaggacggggtggctggacctttgcacacacacacatgcacactcacacgcgtgcacacactcatacatgttcacctcttagtgttctctccacccccagcgacccccactgcagacttccagtgatgggagggccgctgcccttcctggagacagaagaacatgggggagggcctgtcccagagggtgggggtcctgggagcctcgcttgctcccacgagtccctgtgtttttctaaaagtcacgagatcaaaactggagttcagtagtagggtctcatctacccccagcaaggagggtggtgccacgcggagcatctcccgggctgggaggagtgggaggcctggccccctactggcctcagtggggcgggggtgacccggggggctctttggttgaggggaagggcgctgggcctcatctggtgcggttctggcgcatgaggggcacgatgctggcaggcggccctgccttggccaggaatgggtgcttcagcagctcggctgccgtggcccgctgggcagggtctcgcaccagcaggcggtccaggaagcccttcagggatggcgacaccttgtgcaggttcttcagtcggggtggcaggttgtcccgaatcatcttcatggctttgaggggtggctcgttgaagtaggggggctctccgtccaccatctcaatcaccattatccccagcgaccagatgtctacctctggcccgtagggaaggcgggagatgagctctggggccatccagtagggcgtgccgaccagcgacttccttcggggcacttccttgctcacctgggcgcagaacccaaagtctgacagcttcaccctgccatcatgggtcagcaggatcgagtcgctcttgatgtcccggtggatgacgccctgggcgtggagcaccgacagggcctgcagcactgcaaggcacacggccgcgatctgctcctcgttcatcctggtgtgggtgacgatgtcggtgagggcgcctccttccaggaactccatgaccacccagagctcgtcccccaccaggtagctgttgtacatctccaccacattctcgtgctggtagtccctcatgattaccacctcgttgaagagcagctcgcgcctctgctgcttgcgcaggtccatcttcttgacggccaccagcttgcccgagctgcgcacggtggcgatgcacacgatgcccgtggagccctcgccaatcttgatgaagttgtccaggtaggagcgggggtcgcctgggtccaccaccagctgcagggcagcccggaactgctcatgggatactcgctgtggctcccgctgtggtgagcgggggccagggggcccaggaacagcaggggcggcgggggtgcaggctggaggggccagctggggctctgaggcgtggggtcccagcactccagggctgggggcacctcgggctcgggtgggaggccgggaggaggaggaggaggactgggggatggccaggccccccgctgatggcccgttaggggccacgtcatgaggctccccctgggcaccccgggatgggtggtccgtgtcagccctcgggtaggtgttaaagggccggccagctgccagtttcgccccactggccagaccagcaggctggggggtgccgacatcaggcccggagagggggcgtttgtcccgggaggactcctggggaccccctgagccctccctggaagacttgggcctcttctctggccccgcccgtcgcctgtcaccactgccgccacccgcctcgctgtgaccggcgaaccggcctcggctgcctgccttccctgggccccctctggccgtggtggccggctcctctggcatcccattttcctggcgggcacgggcgggcggcggcgggctgtctctccgcagggagttggagcgtgtcaccgacatgttctcaaactcgtccagcagcagcgtgagggccccatctttggcacctttgctgccccgcacgatggtcttgggggccccgggctggatggaggtgatgcaggcggggtcgacgaggggcttgggccggcgagccgactcctcgatcaggctctgccactggcggggcagccccgtgaacttctgctcgtgctggtcgaagcccgtgtgcacgcggtgctcgaagttggacggcgcggagatctccacccgcttcttcctcttcccaaacatggtgccggggactcggtgcggcctggtctgatgctggtgggacagaagtgccctcaggcaggtgaccactcctctaggggcttcgggttactcatcggctcggcgccgcagtcgctcgcggcctaactgctcgacctggaactccgcgccctcgcgcctccctcagctctcttgcaccgccaccaccgcggacactcccgccgccatgttgaatccccaacgaacatcc

SEQ ID NO: 12701 - RNA, 6296 nt, Homo sapiens
  source 1..6296: mol_type = other RNA
gatctcactttgttgcccaggctggtctcaaactcctgacctcaagtgatctgcctgcctcggctccccaaagtgcttgggattacaggcgtgagccactgcacccggcccctagcatgattattaaatctcctgattgtatatgaagcccttgtacacatctgggtctgcctctgggttctctgttctgtcactaaatcagaaagtccagggtgaagcccagcaaatctaatgaaagagcaagagtggagaatcctgactgcatggtaatagaatttgtgttagacacacacaaacactacattttccaacctcccttgcctctgggtgaggctgcgtgactaagctctggccagtgaagcaatggcaaaacctctgggtcggtccttaaagaggagtgccttcctctccccgtgcccacttgggagcataaggaattctctaatacgacatgggagaggcaggtgtcccaggaggaaggaaaaagacggaaggaccctagggtgctgatgacttggagtcccacagaggtgggccttttacacgggagggcagtcgtggatcgcaggggttctcaaacgtgagtgggcaccggcatcccccggagggtgtgttaaatacagatcactgggccccaccagcatctgatgcagctggggtggcacacagggatttatttgcgtgtccagtaagctcccagtgatgctgctggtctgggaaccacactgtgagaaccgctggtctgacctggttgcattgtttattttggggctctgtaaacacacctccagcccccaggcggacgaatccatccctgtgcccctcctgggcctccgggcccctcctcacctccggcacctgtcgagagtcattcattcccgtggagtgcctcagctggtcaactaaatgtgggcagagtggatcctctggcaccacccttgtcctaagcactcccctgttccgctccaggcggacgcctgaaacatggatctgtagaccccccgggccggtggggtcaggaagggtctgccaggaggaggctcctgggtgggagtccagggtgggaagctggaagaagccattctgctctggccagacagaggcgagagtggggtttggggaatgccattggcccctctgttcctctagccacacaggtggcagcagcctccttcctctaatgattgctgggcacttggcactctgtggctcctccagccttctcagagctttgtcatgatccaaccaccggtaccaaatccctgccatttgaaacaactctagttggggtctgttttcctgactggctctggcaggaggcagccacgtggggaggaacggggcctcgggcagctttcaccccacgccacccaaagccatgccttcaaactgcagtgagcgggctgggcacggtggctcacgcctgtaatcccagcactttgcggggccaaggagggaggatcccttgaggccaggagttcgaaaccagcctaggcaacatagcaacatcttgtctctaaaaacaaaaaacaaaaaacaaaaaaactcaaaacaaaacaaaacaaaacaaacctgcagtgagtgactgaaggcaccaaaaccagcagagttaccgtggggtcacagatgtggctgggcgagggagctccccgtctctgagcccgtggtttcttcagcaggagagtggagctcctagagctagctgttctcagtgcccgtggggtcgccgggcaccctggctgtgagccttgcgtttctgagatgctctgttctttgccgtccttatctgggtctggaaccatggtcacagaggcctcctgagctgctatctttctggaacaacttgttcacaaggtagaaggaattacctgctccttcaaagtctggtaaacctcatttgaggccaggcatggtggctcatgcctgtaatcccagcactttgggaggctgaggtgggtggatcacgaggtcaggagttcaagaccagtctggccaagatggcgaaatccagtctctactcaaaatacaaaaaattagcctggcgtggtggcaagcgcctgtaatcccagctacttgggaggctgaggcaggagaatcgcttgaacccaggaggcagaagttgcagtgagccaagatcgtgccactgcactccagcctgggcgacagagcgatactccgtctcaaaaaaaaaaaaaaaatctcatttgaaagtgcattcaagcctgaaaccttttatttattctggagtgtgtgtgcagtgaggagacagttattttggtcttgttttctatttcttcttttgccaatgttagcattttttttttttccagaaaggcatccacctcacctaagcctccaatacatcgcagagagcacagctgcttgcaccgctgggtttcactctgtgatgatccatctaggctgtgtttgcacttggcataggccctgccacacacacagtgctctgattcttggggtcaggacctgtgaagggtgggaggcgtggactaacctggaatctctgccctggccactcacttcccgagaggaccaggctgaggtctctggtgctgatgacgcctggctggctttggggacggaggctcactcctggctctctccccactccactgcctccctgggggctggggaggatgcagaaagtggagcccaacagggcctgaggcgcaaagtgccaggatgcagctgcagcagcgatggtggcatggccacctccatgccagtcagattccccccagcgtgggctcggctctgggctcctgcgtggaaggacacacttcacagggtgtctctccgaagccagcagctccaggccagtcagcctcagtcaatccccaaaagcccatctgcccactgaccaatttgccaaatggccttcaatttactaacttgggttagctcctactcaccaaacgcgctcaagacagcctttaaaaggttccaggaaattgcagatttggcaaactgggatcagtctgcacatggactgtggcaaactggctgcttccaggggtggggacaatcctgccccattctggggagtggcaggctgggggagcttactggctgctatgacctgaactccccactccccaccccacccttgccctgccttggctggaatcgtggtttgctcccagatccagaccctctccctgcaaattcccacccaagacagccgggcagggccccctgccccccacacatcgcacacagacacaaaacaagacaatgttttaattgtaaaactaactcgaggcaggggtgggcgggctggggctgcgctgaccgggcaggaacctggttcttcaggcagtggttctgccagggccaccccgcaggacagggaccatctgtcccccaataagggcaggggctagagtgttataaaatgacaatataaatagacttctagaaaagaggaggctgtccaggtgcagtagtcatttgctgcaggggctggagagggtggggggccctgacctgtctccccatccagccacagaaagggggcgcagggctacgggaaaaggccactcttcggacattcatgatcgacccccacaatggctcagggggagagggggctgggtgtcaggcaaggcgccagacaccccttgcaggctggaggacggggtggctggacctttgcacacacacacatgcacactcacacgcgtgcacacactcatacatgttcacctcttagtgttctctccacccccagcgacccccactgcagacttccagtgatgggagggccgctgcccttcctggagacagaagaacatgggggagggcctgtcccagagggtgggggtcctgggagcctcgcttgctcccacgagtccctgtgtttttctaaaagtcacgagatcaaaactggagttcagtagtagggtctcatctacccccagcaaggagggtggtgccacgcggagcatctcccgggctgggaggagtgggaggcctggccccctactggcctcagtggggcgggggtgacccggggggctctttggttgaggggaagggcgctgggcctcatctggtgcggttctggcgcatgaggggcacgatgctggcaggcggccctgccttggccaggaatgggtgcttcagcagctcggctgccgtggcccgctgggcagggtctcgcaccagcaggcggtccaggaagcccttcagggatggcgacaccttgtgcaggttcttcagtcggggtggcaggttgtcccgaatcatcttcatggctttgaggggtggctcgttgaagtaggggggctctccgtccaccatctcaatcaccattatccccagcgaccagatgtctacctctggcccgtagggaaggcgggagatgagctctggggccatccagtagggcgtgccgaccagcgacttccttcggggcacttccttgctcacctgggcgcagaacccaaagtctgacagcttcaccctgccatcatgggtcagcaggatcgagtcgctcttgatgtcccggtggatgacgccctgggcgtggagcaccgacagggcctgcagcactgcaaggcacacggccgcgatctgctcctcgttcatcctggtgtgggtgacgatgtcggtgagggcgcctccttccaggaactccatgaccacccagagctcgtcccccaccaggtagctgttgtacatctccaccacattctcgtgctggtagtccctcatgattaccacctcgttgaagagcagctcgcgcctctgctgcttgcgcaggtccatcttcttgacggccaccagcttgcccgagctgcgcacggtggcgatgcacacgatgcccgtggagccctcgccaatcttgatgaagttgtccaggtaggagcgggggtcgcctgggtccaccaccagctgcagggcagcccggaactgctcatgggatactcgctgtggctcccgctgtggtgagcgggggccagggggcccaggaacagcaggggcggcgggggtgcaggctggaggggccagctggggctctgaggcgtggggtcccagcactccagggctgggggcacctcgggctcgggtgggaggccgggaggaggaggaggaggactgggggatggccaggccccccgctgatggcccgttaggggccacgtcatgaggctccccctgggcaccccgggatgggtggtccgtgtcagccctcgggtaggtgttaaagggccggccagctgccagtttcgccccactggccagaccagcaggctggggggtgccgacatcaggcccggagagggggcgtttgtcccgggaggactcctggggaccccctgagccctccctggaagacttgggcctcttctctggccccgcccgtcgcctgtcaccactgccgccacccgcctcgctgtgaccggcgaaccggcctcggctgcctgccttccctgggccccctctggccgtggtggccggctcctctggcatcccattttcctggcgggcacgggcgggcggcggcgggctgtctctccgcagggagttggagcgtgtcaccgacatgttctcaaactcgtccagcagcagcgtgagggccccatctttggcacctttgctgccccgcacgatggtcttgggggccccgggctggatggaggtgatgcaggcggggtcgacgaggggcttgggccggcgagccgactcctcgatcaggctctgccactggcggggcagccccgtgaacttctgctcgtgctggtcgaagcccgtgtgcacgcggtgctcgaagttggacggcgcggagatctccacccgcttcttcctcttcccaaacatggtgccggggactcggtgcggcctttggatattgactcagcacagggttactgatcccctgggttaagagggcaccccaggcagccttgtcgcgacactcccctatctttaggatctgtggtcttcaatcgggcccttgacacagtaccaagcacagagcaaatggtcgaccaaagccactttaaaaaacaaaggggctgaggaagagacattctgatggcggcatcccatagagagcctgcacacacctggtctgatgctggtgggacagaagtgccctcaggcaggtgaccactcctctaggggcttcgggttactcatcggctcggcgccgcagtcgctcgcggcctaactgctcgacctggaactccgcgccctcgcgcctccctcagctctcttgcaccgccaccaccgcggacactcccgccgccatgttgaatccccaacgaacatcc

SEQ ID NO: 12702 - RNA, 5538 nt, Homo sapiens
  source 1..5538: mol_type = other RNA
gatctcactttgttgcccaggctggtctcaaactcctgacctcaagtgatctgcctgcctcggctccccaaagtgcttgggattacaggcgtgagccactgcacccggcccctagcatgattattaaatctcctgattgtatatgaagcccttgtacacatctgggtctgcctctgggttctctgttctgtcactaaatcagaaagtccagggtgaagcccagcaaatctaatgaaagagcaagagtggagaatcctgactgcatggtaatagaatttgtgttagacacacacaaacactacattttccaacctcccttgcctctgggtgaggctgcgtgactaagctctggccagtgaagcaatggcaaaacctctgggtcggtccttaaagaggagtgccttcctctccccgtgcccacttgggagcataaggaattctctaatacgacatgggagaggcaggtgtcccaggaggaaggaaaaagacggaaggaccctagggtgctgatgacttggagtcccacagaggtgggccttttacacgggagggcagtcgtggatcgcaggggttctcaaacgtgagtgggcaccggcatcccccggagggtgtgttaaatacagatcactgggccccaccagcatctgatgcagctggggtggcacacagggatttatttgcgtgtccagtaagctcccagtgatgctgctggtctgggaaccacactgtgagaaccgctggtctgacctggttgcattgtttattttggggctctgtaaacacacctccagcccccaggcggacgaatccatccctgtgcccctcctgggcctccgggcccctcctcacctccggcacctgtcgagagtcattcattcccgtggagtgcctcagctggtcaactaaatgtgggcagagtggatcctctggcaccacccttgtcctaagcactcccctgttccgctccaggcggacgcctgaaacatggatctgtagaccccccgggccggtggggtcaggaagggtctgccaggaggaggctcctgggtgggagtccagggtgggaagctggaagaagccattctgctctggccagacagaggcgagagtggggtttggggaatgccattggcccctctgttcctctagccacacaggtggcagcagcctccttcctctaatgattgctgggcacttggcactctgtggctcctccagccttctcagagctttgtcatgatccaaccaccggtaccaaatccctgccatttgaaacaactctagttggggtctgttttcctgactggctctggcaggaggcagccacgtggggaggaacggggcctcgggcagctttcaccccacgccacccaaagccatgccttcaaactgcagtgagcgggctgggcacggtggctcacgcctgtaatcccagcactttgcggggccaaggagggaggatcccttgaggccaggagttcgaaaccagcctaggcaacatagcaacatcttgtctctaaaaacaaaaaacaaaaaacaaaaaaactcaaaacaaaacaaaacaaaacaaacctgcagtgagtgactgaaggcaccaaaaccagcagagttaccgtggggtcacagatgtggctgggcgagggagctccccgtctctgagcccgtggtttcttcagcaggagagtggagctcctagagctagctgttctcagtgcccgtggggtcgccgggcaccctggctgtgagccttgcgtttctgagatgctctgttctttgccgtccttatctgggtctggaaccatggtcacagaggcctcctgagctgctatctttctggaacaacttgttcacaaggtagaaggaattacctgctccttcaaagtctggtaaacctcatttgaggccaggcatggtggctcatgcctgtaatcccagcactttgggaggctgaggtgggtggatcacgaggtcaggagttcaagaccagtctggccaagatggcgaaatccagtctctactcaaaatacaaaaaattagcctggcgtggtggcaagcgcctgtaatcccagctacttgggaggctgaggcaggagaatcgcttgaacccaggaggcagaagttgcagtgagccaagatcgtgccactgcactccagcctgggcgacagagcgatactccgtctcaaaaaaaaaaaaaaaatctcatttgaaagtgcattcaagcctgaaaccttttatttattctggagtgtgtgtgcagtgaggagacagttattttggtcttgttttctatttcttcttttgccaatgttagcattttttttttttccagaaaggcatccacctcacctaagcctccaatacatcgcagagagcacagctgcttgcaccgctgggtttcactctgtgatgatccatctaggctgtgtttgcacttggcataggccctgccacacacacagtgctctgattcttggggtcaggacctgtgaagggtgggaggcgtggactaacctggaatctctgccctggccactcacttcccgagaggaccaggctgaggtctctggtgctgatgacgcctggctggctttggggacggaggctcactcctggctctctccccactccactgcctccctgggggctggggaggatgcagaaagtggagcccaacagggcctgaggcgcaaagtgccaggatgcagctgcagcagcgatggtggcatggccacctccatgccagtcagattccccccagcgtgggctcggctctgggctcctgcgtggaaggacacacttcacagggtgtctctccgaagccagcagctccaggccagtcagcctcagtcaatccccaaaagcccatctgcccactgaccaatttgccaaatggccttcaatttactaacttgggttagctcctactcaccaaacgcgctcaagacagcctttaaaaggttccaggaaattgcagatttggcaaactgggatcagtctgcacatggactgtggcaaactggctgcttccaggggtggggacaatcctgccccattctggggagtggcaggctgggggagcttactggctgctatgacctgaactccccactccccaccccacccttgccctgccttggctggaatcgtggtttgctcccagatccagaccctctccctgcaaattcccacccaagacagccgggcagggccccctgccccccacacatcgcacacagacacaaaacaagacaatgttttaattgtaaaactaactcgaggcaggggtgggcgggctggggctgcgctgaccgggcaggaacctggttcttcaggcagtggttctgccagggccaccccgcaggacagggaccatctgtcccccaataagggcaggggctagagtgttataaaatgacaatataaatagacttctagaaaagaggaggctgtccaggtgcagtagtcatttgctgcaggggctggagagggtggggggccctgacctgtctccccatccagccacagaaagggggcgcagggctacgggaaaaggccactcttcggacattcatgatcgacccccacaatggctcagggggagagggggctgggtgtcaggcaaggcgccagacaccccttgcaggctggaggacggggtggctggacctttgcacacacacacatgcacactcacacgcgtgcacacactcatacatgttcacctcttagtgttctctccacccccagcgacccccactgcagacttccagtgatgggagggccgctgcccttcctggagacagaagaacatgggggagggcctgtcccagagggtgggggtcctgggagcctcgcttgctcccacgagtccctgtgtttttctaaaagtcacgagatcaaaactggagttcagtagtagggtctcatctacccccagcaaggagggtggtgccacgcggagcatctcccgggctgggaggagtgggaggcctggccccctactggcctcagtggggcgggggtgacccggggggctctttggttgaggggaagggcgctgggcctcatctggtgcggttctggcgcatgaggggcacgatgctggcaggcggccctgccttggccaggaatgggtgcttcagcagctcggctgccgtggcccgctgggcagggtctcgcaccagcaggcggtccaggaagcccttcagggatggcgacaccttgtgcaggttcttcagtcggggtggcaggttgtcccgaatcatcttcatggctttgaggggtggctcgttgaagtaggggggctctccgtccaccatctcaatcaccattatccccagcgaccagatgtctacctctggcccgtagggaaggcgggagatgagctctggggccatccagtagggcgtgccgaccagcgacttccttcggggcacttccttgctcacctgggcgcagaacccaaagtctgacagcttcaccctgccatcatgggtcagcaggatcgagtcgctcttgatgtcccggtggatgacgccctgggcgtggagcaccgacagggcctgcagcactgcaaggcacacggccgcgatctgctcctcgttcatcctggtgtgggtgacgatgtcggtgagggcgcctccttccaggaactccatgaccacccagagctcgtcccccaccaggtagctgttgtacatctccaccacattctcgtgctggtagtccctcatgattaccacctcgttgaagagcagctcgcgcctctgctgcttgcgcaggtccatcttcttgacggccaccagcttgcccgagctgcgcacggtggcgatgcacacgatgcccgtggagccctcgccaatcttgatgaagttgtccaggtaggagcgggggtcgcctgggtccaccaccagctgcagggcagcccggaactgctcatgggatactcgctgtggctcccgctgtggtgagcgggggccagggggcccaggaacagcaggggcggcgggggtgcaggctggaggggccagctggggctctgaggcgtggggtcccagcactccagggctgggggcacctcgggctcgggtgggaggccgggaggaggaggaggaggactgggggatggccaggccccccgctgatggcccgttaggggccacgtcatgaggctcccccttgggggccccgggctggatggaggtgatgcaggcggggtcgacgaggggcttgggccggcgagccgactcctcgatcaggctctgccactggcggggcagccccgtgaacttctgctcgtgctggtcgaagcccgtgtgcacgcggtgctcgaagttggacggcgcggagatctccacccgcttcttcctcttcccaaacatggtgccggggactcggtgcggccggctcggcgccgcagtcgctcgcggcctaactgctcgacctggaactccgcgccctcgcgcctccctcagctctcttgcaccgccaccaccgcggacactcccgccgccatgttgaatccccaacgaacatcc

SEQ ID NO: 12703 - RNA, 5611 nt, Homo sapiens
  source 1..5611: mol_type = other RNA
gatctcactttgttgcccaggctggtctcaaactcctgacctcaagtgatctgcctgcctcggctccccaaagtgcttgggattacaggcgtgagccactgcacccggcccctagcatgattattaaatctcctgattgtatatgaagcccttgtacacatctgggtctgcctctgggttctctgttctgtcactaaatcagaaagtccagggtgaagcccagcaaatctaatgaaagagcaagagtggagaatcctgactgcatggtaatagaatttgtgttagacacacacaaacactacattttccaacctcccttgcctctgggtgaggctgcgtgactaagctctggccagtgaagcaatggcaaaacctctgggtcggtccttaaagaggagtgccttcctctccccgtgcccacttgggagcataaggaattctctaatacgacatgggagaggcaggtgtcccaggaggaaggaaaaagacggaaggaccctagggtgctgatgacttggagtcccacagaggtgggccttttacacgggagggcagtcgtggatcgcaggggttctcaaacgtgagtgggcaccggcatcccccggagggtgtgttaaatacagatcactgggccccaccagcatctgatgcagctggggtggcacacagggatttatttgcgtgtccagtaagctcccagtgatgctgctggtctgggaaccacactgtgagaaccgctggtctgacctggttgcattgtttattttggggctctgtaaacacacctccagcccccaggcggacgaatccatccctgtgcccctcctgggcctccgggcccctcctcacctccggcacctgtcgagagtcattcattcccgtggagtgcctcagctggtcaactaaatgtgggcagagtggatcctctggcaccacccttgtcctaagcactcccctgttccgctccaggcggacgcctgaaacatggatctgtagaccccccgggccggtggggtcaggaagggtctgccaggaggaggctcctgggtgggagtccagggtgggaagctggaagaagccattctgctctggccagacagaggcgagagtggggtttggggaatgccattggcccctctgttcctctagccacacaggtggcagcagcctccttcctctaatgattgctgggcacttggcactctgtggctcctccagccttctcagagctttgtcatgatccaaccaccggtaccaaatccctgccatttgaaacaactctagttggggtctgttttcctgactggctctggcaggaggcagccacgtggggaggaacggggcctcgggcagctttcaccccacgccacccaaagccatgccttcaaactgcagtgagcgggctgggcacggtggctcacgcctgtaatcccagcactttgcggggccaaggagggaggatcccttgaggccaggagttcgaaaccagcctaggcaacatagcaacatcttgtctctaaaaacaaaaaacaaaaaacaaaaaaactcaaaacaaaacaaaacaaaacaaacctgcagtgagtgactgaaggcaccaaaaccagcagagttaccgtggggtcacagatgtggctgggcgagggagctccccgtctctgagcccgtggtttcttcagcaggagagtggagctcctagagctagctgttctcagtgcccgtggggtcgccgggcaccctggctgtgagccttgcgtttctgagatgctctgttctttgccgtccttatctgggtctggaaccatggtcacagaggcctcctgagctgctatctttctggaacaacttgttcacaaggtagaaggaattacctgctccttcaaagtctggtaaacctcatttgaggccaggcatggtggctcatgcctgtaatcccagcactttgggaggctgaggtgggtggatcacgaggtcaggagttcaagaccagtctggccaagatggcgaaatccagtctctactcaaaatacaaaaaattagcctggcgtggtggcaagcgcctgtaatcccagctacttgggaggctgaggcaggagaatcgcttgaacccaggaggcagaagttgcagtgagccaagatcgtgccactgcactccagcctgggcgacagagcgatactccgtctcaaaaaaaaaaaaaaaatctcatttgaaagtgcattcaagcctgaaaccttttatttattctggagtgtgtgtgcagtgaggagacagttattttggtcttgttttctatttcttcttttgccaatgttagcattttttttttttccagaaaggcatccacctcacctaagcctccaatacatcgcagagagcacagctgcttgcaccgctgggtttcactctgtgatgatccatctaggctgtgtttgcacttggcataggccctgccacacacacagtgctctgattcttggggtcaggacctgtgaagggtgggaggcgtggactaacctggaatctctgccctggccactcacttcccgagaggaccaggctgaggtctctggtgctgatgacgcctggctggctttggggacggaggctcactcctggctctctccccactccactgcctccctgggggctggggaggatgcagaaagtggagcccaacagggcctgaggcgcaaagtgccaggatgcagctgcagcagcgatggtggcatggccacctccatgccagtcagattccccccagcgtgggctcggctctgggctcctgcgtggaaggacacacttcacagggtgtctctccgaagccagcagctccaggccagtcagcctcagtcaatccccaaaagcccatctgcccactgaccaatttgccaaatggccttcaatttactaacttgggttagctcctactcaccaaacgcgctcaagacagcctttaaaaggttccaggaaattgcagatttggcaaactgggatcagtctgcacatggactgtggcaaactggctgcttccaggggtggggacaatcctgccccattctggggagtggcaggctgggggagcttactggctgctatgacctgaactccccactccccaccccacccttgccctgccttggctggaatcgtggtttgctcccagatccagaccctctccctgcaaattcccacccaagacagccgggcagggccccctgccccccacacatcgcacacagacacaaaacaagacaatgttttaattgtaaaactaactcgaggcaggggtgggcgggctggggctgcgctgaccgggcaggaacctggttcttcaggcagtggttctgccagggccaccccgcaggacagggaccatctgtcccccaataagggcaggggctagagtgttataaaatgacaatataaatagacttctagaaaagaggaggctgtccaggtgcagtagtcatttgctgcaggggctggagagggtggggggccctgacctgtctccccatccagccacagaaagggggcgcagggctacgggaaaaggccactcttcggacattcatgatcgacccccacaatggctcagggggagagggggctgggtgtcaggcaaggcgccagacaccccttgcaggctggaggacggggtggctggacctttgcacacacacacatgcacactcacacgcgtgcacacactcatacatgttcacctcttagtgttctctccacccccagcgacccccactgcagacttccagtgatgggagggccgctgcccttcctggagacagaagaacatgggggagggcctgtcccagagggtgggggtcctgggagcctcgcttgctcccacgagtccctgtgtttttctaaaagtcacgagatcaaaactggagttcagtagtagggtctcatctacccccagcaaggagggtggtgccacgcggagcatctcccgggctgggaggagtgggaggcctggccccctactggcctcagtggggcgggggtgacccggggggctctttggttgaggggaagggcgctgggcctcatctggtgcggttctggcgcatgaggggcacgatgctggcaggcggccctgccttggccaggaatgggtgcttcagcagctcggctgccgtggcccgctgggcagggtctcgcaccagcaggcggtccaggaagcccttcagggatggcgacaccttgtgcaggttcttcagtcggggtggcaggttgtcccgaatcatcttcatggctttgaggggtggctcgttgaagtaggggggctctccgtccaccatctcaatcaccattatccccagcgaccagatgtctacctctggcccgtagggaaggcgggagatgagctctggggccatccagtagggcgtgccgaccagcgacttccttcggggcacttccttgctcacctgggcgcagaacccaaagtctgacagcttcaccctgccatcatgggtcagcaggatcgagtcgctcttgatgtcccggtggatgacgccctgggcgtggagcaccgacagggcctgcagcactgcaaggcacacggccgcgatctgctcctcgttcatcctggtgtgggtgacgatgtcggtgagggcgcctccttccaggaactccatgaccacccagagctcgtcccccaccaggtagctgttgtacatctccaccacattctcgtgctggtagtccctcatgattaccacctcgttgaagagcagctcgcgcctctgctgcttgcgcaggtccatcttcttgacggccaccagcttgcccgagctgcgcacggtggcgatgcacacgatgcccgtggagccctcgccaatcttgatgaagttgtccaggtaggagcgggggtcgcctgggtccaccaccagctgcagggcagcccggaactgctcatgggatactcgctgtggctcccgctgtggtgagcgggggccagggggcccaggaacagcaggggcggcgggggtgcaggctggaggggccagctggggctctgaggcgtggggtcccagcactccagggctgggggcacctcgggctcgggtgggaggccgggaggaggaggaggaggactgggggatggccaggccccccgctgatggcccgttaggggccacgtcatgaggctcccccttgggggccccgggctggatggaggtgatgcaggcggggtcgacgaggggcttgggccggcgagccgactcctcgatcaggctctgccactggcggggcagccccgtgaacttctgctcgtgctggtcgaagcccgtgtgcacgcggtgctcgaagttggacggcgcggagatctccacccgcttcttcctcttcccaaacatggtgccggggactcggtgcggcctggtctgatgctggtgggacagaagtgccctcaggcaggtgaccactcctctaggggcttcgggttactcatcggctcggcgccgcagtcgctcgcggcctaactgctcgacctggaactccgcgccctcgcgcctccctcagctctcttgcaccgccaccaccgcggacactcccgccgccatgttgaatccccaacgaacatcc

SEQ ID NO: 12704 - RNA, 481 nt, Homo sapiens
  source 1..481: mol_type = other RNA
gatctcactttgttgcccaggctggtctcaaactcctggctccaagtgatcctcctgccttggcctcctaaaatgaacatatcctcttttgatagagtacaattgctttcgataagtccagacaggttctctgaattgaatgaaacagctctagcttggcatccaggtccgcgtcagaggcaacaacatgttcatcttccttcttccctgtggctttaataaaggcctgcttcgtctcccaatatttctgttgcatcttatttacaactgacttatcttgagcatatcgatcctgtaagtcccagggataacatttgtgtcctgacatgttttcttcttcttctattgttgatgatttggggagaaggggcaggaaaaaagcatgagaggataagttatattataacctcggagccccggcccccaggagcctcccggccgcggtcggagcgtccctccggatcactcatccgacgtcagc

SEQ ID NO: 12705 - RNA, 484 nt, Homo sapiens
  source 1..484: mol_type = other RNA
gatctcactttgttgcccaggctggtctcaaactcctggctccaagtgatcctcctgccttggcctcctaaaatgaacatatcctcttttgatagagtacaattgctttcgataagtccagacaggttctctgaattgaatgaaacagctctagcttggcatccaggtccgcgtcagaggcaacaacatgttcatcttccttcttccctgtggctttaataaaggcctgcttcgtctcccaatatttctgttgcatcttatttacaactgacttatcttgagcatatcgatcctgtaagtcccagggataactgcatttgtgtcctgacatgttttcttcttcttctattgttgatgatttggggagaaggggcaggaaaaaagcatgagaggataagttatattataacctcggagccccggcccccaggagcctcccggccgcggtcggagcgtccctccggatcactcatccgacgtcagc

SEQ ID NO: 12706 - RNA, 526 nt, Homo sapiens
  source 1..526: mol_type = other RNA
gatctcactttgttgcccaggctggtctcaaactcctggctccaagtgatcctcctgccttggcctcctaaaatgaacatatcctcttttgatagagtacaattgctttcgataagtccagacaggttctctgaattgaatgaaacagctctagcttggcatccaggtccgcgtcagaggcaacaacatgttcatcttccttcttccctgtggctttaataaaggcctgcttcgtctcccaatatttctgttgcatcttatttacaactgacttatcttgagcatatcgatcctgtaagtcccagggataactgcatttgtgtcctgacatgttttcttcttcttctattgttgatgatttggggagaaggggcaggaaaaaagcatgagaggataagttatattataaccttgcttggggagggtcggggactcggggagtgagtttctctctctctactccccggggtctctcctcgacccccatctcctggggtatcccccgctcggatccgccgcccagagt

SEQ ID NO: 12707 - RNA, 419 nt, Homo sapiens
  source 1..419: mol_type = other RNA
gatctcactttgttgcccaggctggtctcaaactcctggctccaagtgatcctcctgccttggcctcctaaaatgaacatatcctcttttgatagagtacaattgctttcgataagtccagacaggttctctgaattgaatgaaacagctctagcttggcatccaggtccgcgtcagaggcaacaacatgttcatcttccttcttccctgtggctttaataaaggcctgcttcgtctcccaatatttctgttgcatcttatttacaactgacttatcttgagcatatcgatcctgtaagtcccagggataactgcatttgtgtcctgacatgttttcttcttcttctcggagccccggcccccaggagcctcccggccgcggtcggagcgtccctccggatcactcatccgacgtcagc

SEQ ID NO: 12708 - RNA, 1815 nt, Homo sapiens
  source 1..1815: mol_type = other RNA
gatctcactttgttgcccaggctggtctcaaactcctggctttaagcaaccttcccaccttagcctcccaaagagctgggattacaggtgtgagctattgtgcctggccacattctcttatctttccacaggaaaaaaatttccataatgaaatccaaatatgatgtcctatatccttctcatcccctatattctaggcctatataaaataaatcaaatcctacttccaaaaaatattctttaaatatctgaaaataactataatcgcaagtctcttttaacccagctaaatactaatcttccctttactgttcttcatgatttccagaccattctcccttctagtaaactcccctcaaaaatgaagctccaccactctgaacatctattaagtattctattaagtggggaagaacatgacacctcaagagttcacaccaatcatctaaaacacaggattgtttttatgaactctaattaaccaatctaacaaaccctggaattgaggttggtaagcaaagtacagaacttcctatttatctttatttaacttttacagtttaagtttctgttaagtttaacatcaaaatatcttctcaaatcctgaaatctagtgaacttctacttgtcgttttgaatcagctataaattacaaagcaagaccatctacattaatataaactgttaaataggacggggccaagtaaagaatcttacagcactctctgcatacttgtctcacaggtaacaaacatccagggaaaacttactttgggaatgacctttcactcatgcagctaaaaagccatgttcctctaccatgatccacaaattagctcaaaaggttgcctgtattgttctggctacaatgtccttgaccactccagcaatcctcggagaattctttcctcatggcaacgaagaaagtcccagattctaacagtgccgtcatcagagcatgtagcaaatttattatccgtgggtgagaaactggcctctctaatcgcctccttatgtgcctggaacatcttgacgttgttcatgttcgactgccaatatttcacatatcctccgtggtctgctgtcaacatccacatgtcattatgtgaccacgtcatggccctcactgggctgtcgtgagcctgtaatattgtttcaaaattgaaagtgagtccattccacagggtaaactccccactagaagctccagtgaccaagcgtcttccttctggagtccacctaacaacaaatacaggacactttactttatttgttgatgtccgaacaaattttgttgttactgcattcataggattattcaacattcctataggtgggaccagatcattgtaataacctgcatcaggctgaattgcccgcatatctctctggtctctttgccatattctgttctccaaatacttaattacagatggattgtagtctatggtttttcggttcacagcttttctcattcgttttccatcaaaagtaagctgttgcattgcttgctgttgtgcaaaatcaggtcgcttataaaacagctgtcgaggtgcctggtgctggaaccttggcatatggaaaaaacgaggaggagaaccaatttctgtagccatggtgatgttttccttctaggatacgtctggctttgagcagagctcctaaatggccagcgaagcgttcgccttcagagccagaaatgtctctcttgtttggtctccccaccccgatcctctcaatcccgctcctccaaaggagcagccgccatcttcccctatgggccaccgaacgcacgctctggggtcatcacgcact

SEQ ID NO: 12709 - RNA, 2806 nt, Homo sapiens
  source 1..2806: mol_type = other RNA
gatctcactttgttgcccaggctggtctcaaactcctgggctcaagcaaacctcccgcctcggacttccaaagtgctgggattacaggagtgagccaccatgcctggcccaactcacaatactctcataccattcatgatataccccttagtccaccaaacttctcaacaagttcaaaaagcctccttcgccagctgggatttggtctggcttctctaaagatgtaccaaaatagctacttccaagtaagagttgtccctaaagcacatcaacatatctatgatcacaacgttaccattgttcaaaatattcttgaaacttcttttggaattgtttctagaggcaacatctcattattttgaatagcctcaatagtgccaaatctttgtcctttgaaagtcaattatttttcgggaatagcatttgcatcatctccattgaaaagagtgagtgaataagctgggtaaaacttacggagaacaattattttaaaaaatgatcccttgtgtgggtcctacatgccttgatagctagtctaaaaggggtttctagaaatcttggaacaagaaaagcatatttgaactacctacaaaggatactaggtagatgcaaaaaaatttgggatgtttatagaaaaaccagttctgttatgtttcagttctgtgtctgggtgttatatctattctataacattattaggctatgtgtttatatttatgataatatgtcattcacaaataatgtgctatgaataaataaaatatgaaagagaaagaaaagactggaatactgctgttcttaccactactgaatactctgtgaaactctaaaattccaatactactacttgggttggggatggttggagaggcattgtgtctatactgtgactaaaaaaaaactggccaatttacaactccccttccttctccattgcccagtttttcccaggttgagttctagatttgttcctgatgcctctcctaactgccctagtgaagcagaaccagattcctcttgggtgactggagcagtggggtcaggcattaacaacaaccactattcctgctgtccccaagaatttttattcctatttgttggacccttgagtttctcattcactctttcattcactcgctcacataacaagtacttactaagtctcaccatgagccaggcactggctagtagaagctatagagattgataaaataagatcccatctgccctccaagaaacacagagcatagatagagcctttaattctaatttgaggaatcagagaagattttacagagaatgaagaatgaaagatgaataagagtttaaaaggtaaacaagggaagaagggcatgcgagagggcacacctgtgcaaggccccagaggcctggggagcatgaggtctttgaggatctgcattttcatgactctgatgtggaatccactaaggattagctgggagtggctaaaagaatcctggagtctcttttagggaacttcagtttcaatgggtaaccactgaaagcatttaagcaagagagtaacatgagcagctgcacattttaatgggatcatttgagtgacaccacagaaaataaaccagagagaaggacagagacagtagttaagaagggtgagttactagaagtagaaggagtagaaagctactgcaatattccagaagcgaaataatgaggccttgaattcacacaatggcagcagggatgaagaaaaggggtgccattggaaatagattcgaggtagaaaagacagaacctattgaccaaataaaaagacaggggattggggaaagggctgctgttgactccaaggtctccctcaagtctggataatgagtggatggtggtagtggggtcgaccaagacctagaacacaaggggaagatagaagaaaagatcaaggggaaggtggaaatgatgagctgtgctttgaacatgctgaatttgagggagttgtaggatgtgtccactgtaggcctgacattcagagatgaggtctggggcatggagaaagacattgacggaacatgaaaaaatggactggagtctttgaagaaacttcttgctacaggttgcaccaggttggatccatttcccatgtccttaaaaccacttcagtctgaagctttgagaagcactaaaatgatcaacttagaaagcattgtgcttagcagtggaaaatgtgatactctcctctgtttacctataaggaaattatttaaatcatcacagcaagaagaaaaactgaggaaactagctgcaagtaggaactgtctgagattacaggtgcagtttattctaaacgtgtccaaaatcactggaacattaactagataacctccattaggttttatattaacttgggggaaaaaaagtatcttccctaaggtcaatgattaattacattttcttcacaaggggtatacttggggatgtgtataaataagactaggacatataacggctggaaggagaccttttattctactctaattagatccttatccaaacacctgctatccacaaaaagacgggtcacagtgatgatcaaaaataacacttatatatgacacttttcatttatatatcacatttcacatataattattcatttaatcctcagacaactgatgaggccagtaaaattattatcctacgctacagtcatagaatgtgctagtgaattgtggagttgacttttagtacagtagaatcttttttatttatttatttatttatttatttttgagacggagtctcactctgttgcccaggctggagtgca

SEQ ID NO: 12710 - RNA, 3024 nt, Homo sapiens
  source 1..3024: mol_type = other RNA
gatctcactttgttgcccaggctggtctcaaactgggctcaagttatcttcccaccttggcctcccaaagtgctgggattataggcatgagccaccacattcagcccaaacatttctgagaccactacttgaactatcaagtctcctcttgtaactgattctcattagaaataatacacatttattgaatgtcattgatatataaagataccattctttgagtgggggaaatataatttaaaagtcgcaactactgacaatcaacaaataaactctaatgagaatcataaagcttgttcccagagaaccatgatacagggtgggacagtacgcaaataatgggctcctgttgtcagacttcatggtgattacattagtgctttctccagtatctttcttcctattgtactcctgaagcactcagaatgataaagataaatttctgatcattcctacaaagagtgcaggcaaagttaagatttaactgtgattgctggttgtttcatctcgaattcaaaatcctggatttccgaaacaatggagcttgatgtcacatttggctatcttgcttttgtctcctcttctggaaagaacaaatcatcttcctgaaaattacaggagacacttagtatgacaaaataaggcctctgaaactgtccaatctcacatgtaaaaagtgtaaaatcacagaactaaaatcaggttccggattttcctggaaatagaatgtcaccgggatctgttcaaaggtgagctttggctacattttataacagtgtttaaaactcgaatgcaaaaaactgctttcaatataatcagatatgtgcaaaaacaatttgttaaataacatgggaagattatattaacaaaagacatttccagaatactaacattcatgtgatttataaaggtgcattttctgtaaagagctatacagcccaaaaacatgaaattcttcaagggagtcccctttatcccatgagttggaagaatttattttcatattctatgcatggatcactgaagtgatgaatgtcactcgtcttcaagaaggaagcactctcagccttgtgaagaagaacctcaagggttcctggggctatgatcatgaagagcaccacaatgaagactgctgcgaagtctttttcacttcttcacatttgggatgtgaaatattttacagaaaaataagagtgtgcaaatccctctcacacatagaaaaacgattgtgtgaatattcttaaatttttaaaacttttaaaaactgtgatctttgcactgttttcaagagtcagcaactctgaagaaagatattcaccataagtgaccccatatggtgaagatattcacaataaatgacagttttgcaagatgactctttgggttggcattctgtttccggtcaccaggtttccgcaatctctgtgacagcccgcagcagctcggcaaatgtagggcggccttcaggtttctcatgccagcagctgtacatgacttcatatatggacattggtgccaggtgagggcgatatagcctgaagccttcagaaatagcttccacgacttgcaaatttgacttattttcaaaaggcatttttccttctgtaaaaacttcccacattaaaactccaaatgaccagacatcagatttactgctgtacttattgaaaagaaaaacttcaggaggggaccacttgattgggaacttggctccaaaagaactgacatactcatcatccaaaacgtaccttgtcattccaaagtctgaaatttttactatgcatgttgaactgaccaaacaattccttgccgccaaatccctatgaatatagccattcctctccagatattccattccttcacatatatcctggcatacactcagtagcatttccttcctaagctttcctttattctccctgagatagttaagcaggcagccattttccatgaactctgtcacaatgtaaaggggcttccgctgtatacagactccataaagttgcactagctttgaatgagataatttcatcatcactttggcctcttcaatgaaatcctcttcagacatggagccttcattgatggccttgatagctacctggatatgtgaccgccattcacctaaatggaccactccaaactgaccgcttccaatctcctttataaaagccaactcagatggatctatctcccacttttcgtagctaaacccagctgtggctggtaaacaactgcccatcagcccaactggatatcggagacgagtcatgagaccggctgcattgtgctggtgataccagattaactcagggattgattgaaaggcgtgtctttcagccacataccactgtcctgagtcattcttttttatctgataatgttttatggcagcctccgtacttcttctagctcccataaatacggaaattgtgtaggatcctaaatgtcttgaatctctgacaataaatgcaccttctttagactcttgtctcaatagatgttctgcctgatttctggtaatgtttctatggtaccaccccaaacggtctcttgccttccaccagtgaggattgtatttctccagtatcaggtattcttctgctctccttaaggctaaattacagggttctctgggcagaaaatcataaagtgccttgacttggatcttctcttcagcaacctcagagggtgggaggggaggcagtggctttcgttttgacggctgcacacggcccgtgttggattgcttcttatttgacaattggctgagccacggcctgcgacgctgggtgtatttttctggaagctcttcatctgtgctcaggcttatctgtgttctcatttgtctcatttgatggtgtctttttgttataaatagacatggtatagtgattaggaacaagagtttgaatcccagctccaccatttcatagtgtggccttgggtaagcaatgtaacctctctaatcttcaatttcctcatcgcttctgcactgaacagcaacagcagcaacagaaaacc

SEQ ID NO: 12711 - RNA, 4083 nt, Homo sapiens
  source 1..4083: mol_type = other RNA
gatctcactttgttgcccaggctggtctcaaactgggctcaagttatcttcccaccttggcctcccaaagtgctgggattataggcatgagccaccacattcagcccaaacatttctgagaccactacttgaactatcaagtctcctcttgtaactgattctcattagaaataatacacatttattgaatgtcattgatatataaagataccattctttgagtgggggaaatataatttaaaagtcgcaactactgacaatcaacaaataaactctaatgagaatcataaagcttgttcccagagaaccatgatacagggtgggacagtacgcaaataatgggctcctgttgtcagacttcatggtgattacattagtgctttctccagtatctttcttcctattgtactcctgaagcactcagaatgataaagataaatttctgatcattcctacaaagagtgcaggcaaagttaagatttaactgtgattgctggttgtttcatctcgaattcaaaatcctggatttccgaaacaatggagcttgatgtcacatttggctatcttgcttttgtctcctcttctggaaagaacaaatcatcttcctgaaaattacaggagacacttagtatgacaaaataaggcctctgaaactgtccaatctcacatgtaaaaagtgtaaaatcacagaactaaaatcaggttccggattttcctggaaatagaatgtcaccgggatctgttcaaaggtgagctttggctacattttataacagtgtttaaaactcgaatgcaaaaaactgctttcaatataatcagatatgtgcaaaaacaatttgttaaataacatgggaagattatattaacaaaagacatttccagaatactaacattcatgtgatttataaaggtgcattttctgtaaagagctatacagcccaaaaacatgaaattcttcaagggagtcccctttatcccatgagttggaagaatttattttcatattctatgcatggatcactgaagtgatgaatgtcactcgtcttcaagaaggaagcactctcagccttgtgaagaagaacctcaagggttcctggggctatgatcatgaagagcaccacaatgaagactgctgcgaagtctttttcacttcttcacatttgggatgtgaaatattttacagaaaaataagagtgtgcaaatccctctcacacatagaaaaacgattgtgtgaatattcttaaatttttaaaacttttaaaaactgtgatctttgcactgttttcaagagtcagcaactctgaagaaagatattcaccataagtgaccccatatggtgaagatattcacaataaatgacagttttgcaagatgactctttgggttggcattctgtttccggtcaccaggtttccgcaatctctgtgacagcccgcagcagctcggcaaatgtagggcggccttcaggtttctcatgccagcagctgtacatgacttcatatatggacattggtgccaggtgagggcgatatagcctgaagccttcagaaatagcttccacgacttgcaaatttgacttattttcaaaaggcatttttccttctgtaaaaacttcccacattaaaactccaaatgaccagacatcagatttactgctgtacttattgaaaagaaaaacttcaggaggggaccacttgattgggaacttggctccaaaagaactgacatactcatcatccaaaacgtaccttgtcattccaaagtctgaaatttttactatgcatgttgaactgaccaaacaattccttgccgccaaatccctatgaatatagccattcctctccagatattccattccttcacatatatcctggcatacactcagtagcatttccttcctaagctttcctttattctccctgagatagttaagcaggcagccattttccatgaactctgtcacaatgtaaaggggcttccgctgtatacagactccataaagttgcactagctttgaatgagataatttcatcatcactttggcctcttcaatgaaatcctcttcagacatggagccttcattgatggccttgatagctacctggatatgtgaccgccattcacctaaatggaccactccaaactgaccgcttccaatctcctttataaaagccaactcagatggatctatctcccacttttcgtagctaaacccagctgtggctggtaaacaactgcccatcagcccaactggatatcggagacgagtcatgagaccggctgcattgtgctggtgataccagattaactcagggattgattgaaaggcgtgtctttcagccacataccactgtcctgagtcattcttttttatctgataatgttttatggcagcctccgtacttcttctagctcccataaatacggaaattgtgtaggatcctaaatgtcttgaatctctgacaataaatgcaccttctttagactcttgtctcaatagatgttctgcctgatttctggtaatgtttctatggtaccactcatatatttctaaattagttattttgttttcagtcacatagttgcttgggattaagccttcattccccaaacggtctcttgccttccaccagtgaggattgtatttctccagtatcaggtattcttctgctctccttaaggctaaattacagggttctctgggcagaaaatcataaagtgccttgacttggatcttctcttcagcaacctcagagggtgggaggggaggcagtggctttcgttttgacggctgcacacggcccgtgttggattgcttcttatttgacaattggctgagccacggcctgcgacgctgggtgtatttttctggaagctcttcatctgtgctcaggcttatctgtgttctcatttgtaggaggaaaggatcatggtagccccttctgcggggagcacacaacagtcttcagttcttctgcggtgctctactcacaaaaacacatctttcaactgaaatcatagttcgctcaagatgtttctcacgggcagagttaaccccacctattttcctgttctgaaaacctcagaagagtataaatgacaaccaatggcatatataagaaagctcagtaatctccatcccaatctctgagggtatctgctattagtctctcatccccaaaggtgtgggtgactcgcaaacatcattttcaagaaatcacaaaattttggtaaaaggcacctttaaaattatcaaatcaaactgccctctctggactgggaaggaaatgaaggcacagacagaataagggacttgcccaaggccacaccgtgagtggcagaaacaattagattctaggctctggaatattgagtttagaatgttccatcctcccactcagcagacactttatttgggggaagtcaatctagtaataaccctaaaatgtgattgggggatggctgagaaatataaaaacaccaacaatacaaaacacacttgggagtttcacttcatcccactggaaagcataaccatgtgtcaactaattaacagagcaactttaatgaagacacagcatattctaatcgcccttccaatttcctggtttagattaaggtctccttagcattctgggtgatgactgttatttttacttcaccttttgcctttgttatgctttcgtataaaactttttttctaagtcttagtgaaaaatatttaaagatttttgaaggaaatgttgacaaatgttgccaggtgctatctatcttgttttcccataaaaagcatacactgaccattaggacagggactctatcttctcctcactctctttcataccacctagtacttcccgtagctcctcaaggtgaaaagggaagtatgggatgggaggagggaaggtcaggaaggaaggagaaaaggctgacagtgatagtaaggtagagtgtgccaggaccgactccttcaatgagctacaagtcagttaaaagttgtgcatggttagcaaccaaaatgcccatcaatgataggctggataaagaaaatgtggtacatatacaccgtggaatattatgcag

SEQ ID NO: 12712 - RNA, 3089 nt, Homo sapiens
  source 1..3089: mol_type = other RNA
gatctcactttgttgcccaggctggtctcaaactgggctcaagttatcttcccaccttggcctcccaaagtgctgggattataggcatgagccaccacattcagcccaaacatttctgagaccactacttgaactatcaagtctcctcttgtaactgattctcattagaaataatacacatttattgaatgtcattgatatataaagataccattctttgagtgggggaaatataatttaaaagtcgcaactactgacaatcaacaaataaactctaatgagaatcataaagcttgttcccagagaaccatgatacagggtgggacagtacgcaaataatgggctcctgttgtcagacttcatggtgattacattagtgctttctccagtatctttcttcctattgtactcctgaagcactcagaatgataaagataaatttctgatcattcctacaaagagtgcaggcaaagttaagatttaactgtgattgctggttgtttcatctcgaattcaaaatcctggatttccgaaacaatggagcttgatgtcacatttggctatcttgcttttgtctcctcttctggaaagaacaaatcatcttcctgaaaattacaggagacacttagtatgacaaaataaggcctctgaaactgtccaatctcacatgtaaaaagtgtaaaatcacagaactaaaatcaggttccggattttcctggaaatagaatgtcaccgggatctgttcaaaggtgagctttggctacattttataacagtgtttaaaactcgaatgcaaaaaactgctttcaatataatcagatatgtgcaaaaacaatttgttaaataacatgggaagattatattaacaaaagacatttccagaatactaacattcatgtgatttataaaggtgcattttctgtaaagagctatacagcccaaaaacatgaaattcttcaagggagtcccctttatcccatgagttggaagaatttattttcatattctatgcatggatcactgaagtgatgaatgtcactcgtcttcaagaaggaagcactctcagccttgtgaagaagaacctcaagggttcctggggctatgatcatgaagagcaccacaatgaagactgctgcgaagtctttttcacttcttcacatttgggatgtgaaatattttacagaaaaataagagtgtgcaaatccctctcacacatagaaaaacgattgtgtgaatattcttaaatttttaaaacttttaaaaactgtgatctttgcactgttttcaagagtcagcaactctgaagaaagatattcaccataagtgaccccatatggtgaagatattcacaataaatgacagttttgcaagatgactctttgggttggcattctgtttccggtcaccaggtttccgcaatctctgtgacagcccgcagcagctcggcaaatgtagggcggccttcaggtttctcatgccagcagctgtacatgacttcatatatggacattggtgccaggtgagggcgatatagcctgaagccttcagaaatagcttccacgacttgcaaatttgacttattttcaaaaggcatttttccttctgtaaaaacttcccacattaaaactccaaatgaccagacatcagatttactgctgtacttattgaaaagaaaaacttcaggaggggaccacttgattgggaacttggctccaaaagaactgacatactcatcatccaaaacgtaccttgtcattccaaagtctgaaatttttactatgcatgttgaactgaccaaacaattccttgccgccaaatccctatgaatatagccattcctctccagatattccattccttcacatatatcctggcatacactcagtagcatttccttcctaagctttcctttattctccctgagatagttaagcaggcagccattttccatgaactctgtcacaatgtaaaggggcttccgctgtatacagactccataaagttgcactagctttgaatgagataatttcatcatcactttggcctcttcaatgaaatcctcttcagacatggagccttcattgatggccttgatagctacctggatatgtgaccgccattcacctaaatggaccactccaaactgaccgcttccaatctcctttataaaagccaactcagatggatctatctcccacttttcgtagctaaacccagctgtggctggtaaacaactgcccatcagcccaactggatatcggagacgagtcatgagaccggctgcattgtgctggtgataccagattaactcagggattgattgaaaggcgtgtctttcagccacataccactgtcctgagtcattcttttttatctgataatgttttatggcagcctccgtacttcttctagctcccataaatacggaaattgtgtaggatcctaaatgtcttgaatctctgacaataaatgcaccttctttagactcttgtctcaatagatgttctgcctgatttctggtaatgtttctatggtaccactcatatatttctaaattagttattttgttttcagtcacatagttgcttgggattaagccttcattccccaaacggtctcttgccttccaccagtgaggattgtatttctccagtatcaggtattcttctgctctccttaaggctaaattacagggttctctgggcagaaaatcataaagtgccttgacttggatcttctcttcagcaacctcagagggtgggaggggaggcagtggctttcgttttgacggctgcacacggcccgtgttggattgcttcttatttgacaattggctgagccacggcctgcgacgctgggtgtatttttctggaagctcttcatctgtgctcaggcttatctgtgttctcatttgtctcatttgatggtgtctttttgttataaatagacatggtatagtgattaggaacaagagtttgaatcccagctccaccatttcatagtgtggccttgggtaagcaatgtaacctctctaatcttcaatttcctcatcgcttctgcactgaacagcaacagcagcaacagaaaac

SEQ ID NO: 12713 - RNA, 2507 nt, Homo sapiens
  source 1..2507: mol_type = other RNA
gatctcactttgttgcccaggctggtctcaaactgggctcaagttatcttcccaccttggcctcccaaagtgctgggattataggcatgagccaccacattcagcccaaacatttctgagaccactacttgaactatcaagtctcctcttgtaactgattctcattagaaataatacacatttattgaatgtcattgatatataaagataccattctttgagtgggggaaatataatttaaaagtcgcaactactgacaatcaacaaataaactctaatgagaatcataaagcttgttcccagagaaccatgatacagggtgggacagtacgcaaataatgggctcctgttgtcagacttcatggtgattacattagtgctttctccagtatctttcttcctattgtactcctgaagcactcagaatgataaagataaatttctgatcattcctacaaagagtgcaggcaaagttaagatttaactgtgattgctggttgtttcatctcgaattcaaaatcctggatttccgaaacaatggagcttgatgtcacatttggctatcttgcttttgtctcctcttctggaaagaacaaatcatcttcctgaaaattacaggagacacttagtatgacaaaataaggcctctgaaactgtccaatctcacatgtaaaaagtgtaaaatcacagaactaaaatcaggttccggattttcctggaaatagaatgtcaccgggatctgttcaaaggtgagctttggctacattttataacagtgtttaaaactcgaatgcaaaaaactgctttcaatataatcagatatgtgcaaaaacaatttgttaaataacatgggaagattatattaacaaaagacatttccagaatactaacattcatgtgatttataaaggtgcattttctgtaaagagctatacagcccaaaaacatgaaattcttcaagggagtcccctttatcccatgagttggaagaatttattttcatattctatgcatggatcactgaagtgatgaatgtcactcgtcttcaagaaggaagcactctcagccttgtgaagaagaacctcaagggttcctggggctatgatcatgaagagcaccacaatgaagactgctgcgaagtctttttcacttcttcacatttgggatgtgaaatattttacagaaaaataagagtgtgcaaatccctctcacacatagaaaaacgattgtgtgaatattcttaaatttttaaaacttttaaaaactgtgatctttgcactgttttcaagagtcagcaactctgaagaaagatattcaccataagtgaccccatatggtgaagatattcacaataaatgacagttttgcaagatgactctttgggttggcattctgtttccggtcaccaggtttccgcaatctctgtgacagcccgcagcagctcggcaaatgtagggcggccttcaggtttctcatgccagcagctgtacatgacttcatatatggacattggtgccaggtgagggcgatatagcctgaagccttcagaaatagcttccacgacttgcaaatttgacttattttcaaaaggcatttttccttctgtaaaaacttcccacattaaaactccaaatgaccagacatcagatttactgctgtacttattgaaaagaaaaacttcaggaggggaccacttgattgggaacttggctccaaaagaactgacatactcatcatccaaaacgtaccttgtcattccaaagtctgaaatttttactatgcatgttgaactgaccaaacaattccttgccgccaaatccctatgaatatagccattcctctccagatattccattccttcacatatatcctggcatacactcagtagcatttccttcctaagctttcctttattctccctgagatagttaagcaggcagccattttccatgaactctgtcacaatgtaaaggggcttccgctgtatacagactccataaagttgcactagctttgaatgagataatttcatcatcactttggcctcttcaatgaaatcctcttcagacatggagccttcattgatggccttgatagctacctggatatgtgaccgccattcacctaaatggaccactccaaactgaccgcttccaatctcctttataaaagccaactcagatggatctatctcccacttttcgtagctaaacccagctgtggctggtaaacaactgcccatcagcccaactggatatcggagacgagtcatgagaccggctgcattgtgctggtgataccagattaactcagggattgattgaaaggcgtgtctttcagccacataccactgtcctgagtcattcttttttatctgataatgttttatggcagcctccgtacttcttctagctcccataaatacggaaattgtgtaggatcctaaatgtcttgaatctctgacaataaatgcaccttctttagactgtagtcccagctactcagag

SEQ ID NO: 12714 - RNA, 2360 nt, Homo sapiens
  source 1..2360: mol_type = other RNA
gatctcactttgttgcccaggctggtctcaaactgggctcaagttatcttcccaccttggcctcccaaagtgctgggattataggcatgagccaccacattcagcccaaacatttctgagaccactacttgaactatcaagtctcctcttgtaactgattctcattagaaataatacacatttattgaatgtcattgatatataaagataccattctttgagtgggggaaatataatttaaaagtcgcaactactgacaatcaacaaataaactctaatgagaatcataaagcttgttcccagagaaccatgatacagggtgggacagtacgcaaataatgggctcctgttgtcagacttcatggtgattacattagtgctttctccagtatctttcttcctattgtactcctgaagcactcagaatgataaagataaatttctgatcattcctacaaagagtgcaggcaaagttaagatttaactgtgattgctggttgtttcatctcgaattcaaaatcctggatttccgaaacaatggagcttgatgtcacatttggctatcttgcttttgtctcctcttctggaaagaacaaatcatcttcctgaaaattacaggagacacttagtatgacaaaataaggcctctgaaactgtccaatctcacatgtaaaaagtgtaaaatcacagaactaaaatcaggttccggattttcctggaaatagaatgtcaccgggatctgttcaaaggtgagctttggctacattttataacagtgtttaaaactcgaatgcaaaaaactgctttcaatataatcagatatgtgcaaaaacaatttgttaaataacatgggaagattatattaacaaaagacatttccagaatactaacattcatgtgatttataaaggtgcattttctgtaaagagctatacagcccaaaaacatgaaattcttcaagggagtcccctttatcccatgagttggaagaatttattttcatattctatgcatggatcactgaagtgatgaatgtcactcgtcttcaagaaggaagcactctcagccttgtgaagaagaacctcaagggttcctggggctatgatcatgaagagcaccacaatgaagactgctgcgaagtctttttcacttcttcacatttgggatgtgaaatattttacagaaaaataagagtgtgcaaatccctctcacacatagaaaaacgattgtgtgaatattcttaaatttttaaaacttttaaaaactgtgatctttgcactgttttcaagagtcagcaactctgaagaaagatattcaccataagtgaccccatatggtgaagatattcacaataaatgacagttttgcaagatgactctttgggttggcattctgtttccggtcaccaggtttccgcaatctctgtgacagcccgcagcagctcggcaaatgtagggcggccttcaggtttctcatgccagcagctgtacatgacttcatatatggacattggtgccaggtgagggcgatatagcctgaagccttcagaaatagcttccacgacttgcaaatttgacttattttcaaaaggcatttttccttctgtaaaaacttcccacattaaaactccaaatgaccagacatcagatttactgctgtacttattgaaaagaaaaacttcaggaggggaccacttgattgggaacttggctccaaaagaactgacatactcatcatccaaaacgtaccttgtcattccaaagtctgaaatttttactatgcatgttgaactgaccaaacaattccttgccgccaaatccctatgaatatagccattcctctccagatattccattccttcacatatatcctggcatacactcagtagcatttccttcctaagctttcctttattctccctgagatagttaagcaggcagccattttccatgaactctgtcacaatgtaaaggggcttccgctgtatacagactccataaagttgcactagctttgaatgagataatttcatcatcactttggcctcttcaatgaaatcctcttcagacatggagccttcattgatggccttgatagctacctggatatgtgaccgccattcacctaaatggaccactccaaactgaccgcttccaatctcctttataaaagccaactcagatggatctatctcccacttttcgtagctaaacccagctgtggctggtaaacaactgcccatcagcccaactggatatcggagacgagtcatgagaccttctagctcccataaatacggaaattgtgtaggatcctaaatgtcttgaatctctgacaataaatgcaccttctttagactg

SEQ ID NO: 12715 - RNA, 2977 nt, Homo sapiens
  source 1..2977: mol_type = other RNA
gatctcactttgttgcccaggctggtctcaaactgggctcaagttatcttcccaccttggcctcccaaagtgctgggattataggcatgagccaccacattcagcccaaacatttctgagaccactacttgaactatcaagtctcctcttgtaactgattctcattagaaataatacacatttattgaatgtcattgatatataaagataccattctttgagtgggggaaatataatttaaaagtcgcaactactgacaatcaacaaataaactctaatgagaatcataaagcttgttcccagagaaccatgatacagggtgggacagtacgcaaataatgggctcctgttgtcagacttcatggtgattacattagtgctttctccagtatctttcttcctattgtactcctgaagcactcagaatgataaagataaatttctgatcattcctacaaagagtgcaggcaaagttaagatttaactgtgattgctggttgtttcatctcgaattcaaaatcctggatttccgaaacaatggagcttgatgtcacatttggctatcttgcttttgtctcctcttctggaaagaacaaatcatcttcctgaaaattacaggagacacttagtatgacaaaataaggcctctgaaactgtccaatctcacatgtaaaaagtgtaaaatcacagaactaaaatcaggttccggattttcctggaaatagaatgtcaccgggatctgttcaaaggtgagctttggctacattttataacagtgtttaaaactcgaatgcaaaaaactgctttcaatataatcagatatgtgcaaaaacaatttgttaaataacatgggaagattatattaacaaaagacatttccagaatactaacattcatgtgatttataaaggtgcattttctgtaaagagctatacagcccaaaaacatgaaattcttcaagggagtcccctttatcccatgagttggaagaatttattttcatattctatgcatggatcactgaagtgatgaatgtcactcgtcttcaagaaggaagcactctcagccttgtgaagaagaacctcaagggttcctggggctatgatcatgaagagcaccacaatgaagactgctgcgaagtctttttcacttcttcacatttgggatgtgaaatattttacagaaaaataagagtgtgcaaatccctctcacacatagaaaaacgattgtgtgaatattcttaaatttttaaaacttttaaaaactgtgatctttgcactgttttcaagagtcagcaactctgaagaaagatattcaccataagtgaccccatatggtgaagatattcacaataaatgacagttttgcaagatgactctttgggttggcattctgtttccggtcaccaggtttccgcaatctctgtgacagcccgcagcagctcggcaaatgtagggcggccttcaggtttctcatgccagcagctgtacatgacttcatatatggacattggtgccaggtgagggcgatatagcctgaagccttcagaaatagcttccacgacttgcaaatttgacttattttcaaaaggcatttttccttctgtaaaaacttcccacattaaaactccttgtcattccaaagtctgaaatttttactatgcatgttgaactgaccaaacaattccttgccgccaaatccctatgaatatagccattcctctccagatattccattccttcacatatatcctggcatacactcagtagcatttccttcctaagctttcctttattctccctgagatagttaagcaggcagccattttccatgaactctgtcacaatgtaaaggggcttccgctgtatacagactccataaagttgcactagctttgaatgagataatttcatcatcactttggcctcttcaatgaaatcctcttcagacatggagccttcattgatggccttgatagctacctggatatgtgaccgccattcacctaaatggaccactccaaactgaccgcttccaatctcctttataaaagccaactcagatggatctatctcccacttttcgtagctaaacccagctgtggctggtaaacaactgcccatcagcccaactggatatcggagacgagtcatgagaccggctgcattgtgctggtgataccagattaactcagggattgattgaaaggcgtgtctttcagccacataccactgtcctgagtcattcttttttatctgataatgttttatggcagcctccgtacttcttctagctcccataaatacggaaattgtgtaggatcctaaatgtcttgaatctctgacaataaatgcaccttctttagactcttgtctcaatagatgttctgcctgatttctggtaatgtttctatggtaccactcatatatttctaaattagttattttgttttcagtcacatagttgcttgggattaagccttcattccccaaacggtctcttgccttccaccagtgaggattgtatttctccagtatcaggtattcttctgctctccttaaggctaaattacagggttctctgggcagaaaatcataaagtgccttgacttggatcttctcttcagcaacctcagagggtgggaggggaggcagtggctttcgttttgacggctgcacacggcccgtgttggattgcttcttatttgacaattggctgagccacggcctgcgacgctgggtgtatttttctggaagctcttcatctgtgctcaggcttatctgtgttctcatttgtctcatttgatggtgtctttttgttataaatagacatggtatagtgattaggaacaagagtttgaatcccagctccaccatttcatagtgtggccttgggtaagcaatgtaacctctctaatcttcaatttcctcatcgcttctgcactgaacagcaacagcagcaacagaaaaccgactgg

SEQ ID NO: 12716 - RNA, 5795 nt, Homo sapiens
  source 1..5795: mol_type = other RNA
gatctcactttgttgcccaggctggtctccaactcctgggctcaagtgatacccagcctgggcctcccaaagtgctgggattacgggtatgagccactgtgcccagcctgatatacaatttcttcctcagacagtctggctctgtcgcccaggctggagtgcagtggcacaatcttggctcactgcaacctctgcctcccgggttcaagcaattctcctgcctcagcctcccgagtagctggaattacaggcatgcaccaccatgcctgaccaatttttgtatttttagtagagacctggggtttcatcatgttggccaggctgttcttgaactcctgacctcaagcaatccgcccacctcagcctcccaaagtgcttggatttcaggagtgagcttttgcacctggcctgatatacaatttctgatgctatagaagcaatgtataactcctaatttactagtgactgctatgcgcttcattaacattatggacatgtcgatcccaaaaatcatatagaaatgttactttttttttgagacagggtttcactctgtcgcccaggctggactgcaatggcgtaaacatggctcactgtagcctcaacctctcgggctcaagcaatcctcctgcctcagcctcccaaatagttgagactacaggcatgtgtcaccacaccccttaatttttgtattttcttttctcattatgttgtccaggatggtctcaaactcctgggctcaaggcatcctcctgccttggtctcctaaagtgttagaattacaggcatgagccactgtgcccagccagaaatgttaaactcactttatggtttcagaacaaggatcaaataaaataaaaatataaaaaataaaatatggttggccaagtgtggtggctcagccctctaatcccagccctttggaaggccaaggcagaaggctcgcttgagctcaggagttcaagactagccttggcaacatagcaagacctcatttctgctaaaaataaaaaacattagccagacatggtggtccacacttgcagtcccagttattcaagaggctgaggtgggaggatcacttgagcttgggagatcgaggctgcagtgagctatcatcgtgccactgcactccagtctggcgacagagcaagaccttctcaaaaataaaatatggtcgaaacgggacagacaaggcggctacctgtaaccctggccgctttaggagctggggcaggaaagttgcttgaggccaggaatccgagaccagcctgagcaacagcaggacccgtctatgaaaaaacaggagcaagtagtggcacatcccaattgtgtcagctaactgggaggctgaggcaggaggatcgcttgagcccaggagttcaaggctgtactccagcctgggcgacaaagcaagaaccctgttctctagggaaaaaaaaaaaaaagtcaaaacatttcataaaactttcacacaatggaggtttagttaagctgttactcttctgttcaattttgttgcacctatcagaaggcataatttcataaaatcaggattccttggcgttttaaccactctcaaaatatttgatcctactggaagttactatgcaatgctatcttgtccctgaatcaacataattcaactatcagcttcatatatatatatatatatatatattttttttttttgagacagagtttcgctgttgttgcccaggctggagtgcaatggcgcaatcttggctcaccacaacctccgcctcccgggttcaagcgattctcctgcctcagcctcctgagtagctgggattacaggcacgcaccaccaccgcagctaattttgtatttttagtagagacagggtttctccatgttggtcaggctggtcttgaactcccgacctcaggtgatccacccgcctcggcctcccagaatgctgggtttacaggcatgacccactgtgcctggcagtttcgtgtattcttactccactgggttctgctttatcgtattgacagtagacatttcattaaatgaaatgtaaaaagaacaccaatacatacatattaaaattttcttactagaatcttttagtataatttaaaaacctgaaatgagaattcgcatcactttaagtgggcctcttgggttttgaggatgaagtggctttctctcagaaatagctttgaaccgtaactctagtaactacagtggcaggctccatagcttgaacacagcgtattttgtatcaatgcccacaaataaaacctattataactcttaggaaataaaacttgaatcctgattggcagaactgcctcagtaagggctggctgaactgcatacccaaaatgttttagatctacggtccactttcacgttggctggactaatgcgtttctactgctcctcttacacgttgactgactttcctctcaggaagaggtagagactatgttccttttttcctcaatctgggacttggtttctgagacatcactgttgtaaccaagagcatggtaaaagtgatgttatgtgacattgaaggataagtcctaaaaagccaactctgccaagctctcctggagccccaaaataccacctaagtccagctgccctgaagccaccatgctagagattttcgggaaagactataccactaatagtgaaaagcacaaagagcatcctttcagctcagaagtgaaaagcttcatgagactcagaaccagaagagtctgatactcccgagttcttcacccacagaaaagcttatcatacaccattgatctttggatgctttgctaacatagcaagaaataatatacagttgatactgctaagcaccacagccaccacttggttgggttcagaagacatcctactttacctttttaaagtttggtccaaatttgtacctacaacttttccttttttcctgcagcacaggtaaaatgttggaacctttaacaagttcaggcaatgatgatataaagaagttaacatgcaactagctgcactggcttctaaattgagttcactgaccttaccatgagtttgtagtaacatttctctccaatctctgaaaaagtttttctctccaggccatctgtacgctttacgtagggactgttaaccaacccacgtattacacataaggactctaggtaaaatctagtgtttgaaaaacagcatgttatatattacactaggtttttcgttttttttccagtggtgggctgtcattacaaaagattgaacttttatacacttcctaatcaaacttaaggggaatctaaacacaaaaactaattcactttctaggagctctttaaaaatgggcttaaacctacaatccaatctcgtatctaagtatgatggaatgctttttccccagtggcattcatatagttcagctgtcaagcagtacctttcttaaaataccagactgaaaatagttcaattttctgtaaaaagtcagagccgggcacggtggctcatgcctataatcccagcagtttgggaggctgaggcgggcggatcacctgaggttggaagttcgagaccagcctgaccaacacagggaaaccccgtctctactaaaaatacaaaattagctgggcgtggtggcacatgcctgaaatcccagctacttgggaggctgaggcagaacaatcgcttgaacctgggaggcagaggttgccgtgaggcgagatcgcgacactacactcgtctgggcaacaagagtgaaactccgtctcaaaaaaaaaaaaagtcagatctgtgtaaagagaattagtgtacctgaaaattgttttcagctgtcaatcactttggtcctttactgtcattctaagaatcagcctaatttggtttaccttgtcttacaaataaggattagcaaactcaccaacataaaaaaggtgtagtacatgctgcaaaaatgtaagtatacactgacatttacttgccaaaataaccacaaatgactacacatatttaactataattaaatcaagtttttagaaatttaaagtctgcttccctagaaatacaggaactttgtgtgataaaacttgagacatatgacaatttctgaatagcaactggaatattcaaccaacaatggtcatggtcagttttgtattttttccttaacttatatacttcattctttccaactattttaaagctaaatcttttttaaaaaagttttaaaaataagtcacaggcaaatcatgaagagttgggtttatttcaacagtaaatctgaaactcttgccttaagcaagagtactacagtaattatatcaggaatagacaatttcctacactgtcaaatatataaaagttccttttgcactttcttcaacactgatcaacaagcagattcagtccacatttgctttgatctaactactgagttaacccaagcttcttcttcagagactctggcatctcgggtggaggagggcgaggaagtctgaagtagaccttcacggagtcatagataaaccactgtagtgcagtcagggtaccaatcatgatgatacgggcaaacagtcccttccatacacctttaaatccaagtctcttgaggaccagagaagcactgctacctttttctttattcaacacagataccacagaatcagcagggtgagaaacaattgcacaaaagactccagctatgtaacctgctacaaatgttacaaccagctgctctggctttgaacattcactgcggggcttaggaaccacaaacttgtacagtgcttcaacagtacgttcaaagcaggcgaacttcatcatggtgtatggtatctgtctcatccagagaggagcaacccccttgtagaatgcttttaggccttcttccttatacattttgggagctgcatccctcaaagtgttggcataacctggctgggtttgaattcgaaccttagcagcttccataggagccagggcaatgtcagcaaagaattcagcactggcagaggcagccaaatatagtgatgtgcgccagagataagtattctcctctccaagcatattgctatacaagactttaaagacttcataaaagccaaacttgcagagtccctgcatggagtagccaaggaaagtcggagcccatcctttagccaaaccacgaacaccatcctctttaagtgtaactgagaatccgttaaatatgcccttgtacttttgggggtccacctgcatacggcatttcactaaatccaggggaaccacagcagtgtgtgtcagaccacaacttaagaccccaccaaagccacacagtgcataatacttcgcggagccaaattcacaactgtactcttccacggcggcggctgccaggttgcgagggcggcggggctggcccgtgggccctggggagctgctgcggaggtccccgagaccatcgtgcaccagctgcagatgtggcgtgttgaaggggttcgcccgcgccaggtgcgccacggacgagaacatctttctaggggaggagggagcgacggttagaggacaggcaaggcgccggttaacgttaccggcgccctggaaccccaaccggggccttttccttcccgtctccacgcccttgaagaggtcacggcggccttcgaaagaggctgctcccggctgggcccaccgccaaagcagcggccccacaggagctctgggctccgctccccacacccgccacaggagaaggcccggccacactcactccctaagatggcgatcacacaaccactcccttggaaaggttgcggctcacagag

SEQ ID NO: 12717 - RNA, 5561 nt, Homo sapiens
  source 1..5561: mol_type = other RNA
gatctcactttgttgcccaggctggtctccaactcctgggctcaagtgatacccagcctgggcctcccaaagtgctgggattacgggtatgagccactgtgcccagcctgatatacaatttcttcctcagacagtctggctctgtcgcccaggctggagtgcagtggcacaatcttggctcactgcaacctctgcctcccgggttcaagcaattctcctgcctcagcctcccgagtagctggaattacaggcatgcaccaccatgcctgaccaatttttgtatttttagtagagacctggggtttcatcatgttggccaggctgttcttgaactcctgacctcaagcaatccgcccacctcagcctcccaaagtgcttggatttcaggagtgagcttttgcacctggcctgatatacaatttctgatgctatagaagcaatgtataactcctaatttactagtgactgctatgcgcttcattaacattatggacatgtcgatcccaaaaatcatatagaaatgttactttttttttgagacagggtttcactctgtcgcccaggctggactgcaatggcgtaaacatggctcactgtagcctcaacctctcgggctcaagcaatcctcctgcctcagcctcccaaatagttgagactacaggcatgtgtcaccacaccccttaatttttgtattttcttttctcattatgttgtccaggatggtctcaaactcctgggctcaaggcatcctcctgccttggtctcctaaagtgttagaattacaggcatgagccactgtgcccagccagaaatgttaaactcactttatggtttcagaacaaggatcaaataaaataaaaatataaaaaataaaatatggttggccaagtgtggtggctcagccctctaatcccagccctttggaaggccaaggcagaaggctcgcttgagctcaggagttcaagactagccttggcaacatagcaagacctcatttctgctaaaaataaaaaacattagccagacatggtggtccacacttgcagtcccagttattcaagaggctgaggtgggaggatcacttgagcttgggagatcgaggctgcagtgagctatcatcgtgccactgcactccagtctggcgacagagcaagaccttctcaaaaataaaatatggtcgaaacgggacagacaaggcggctacctgtaaccctggccgctttaggagctggggcaggaaagttgcttgaggccaggaatccgagaccagcctgagcaacagcaggacccgtctatgaaaaaacaggagcaagtagtggcacatcccaattgtgtcagctaactgggaggctgaggcaggaggatcgcttgagcccaggagttcaaggctgtactccagcctgggcgacaaagcaagaaccctgttctctagggaaaaaaaaaaaaaagtcaaaacatttcataaaactttcacacaatggaggtttagttaagctgttactcttctgttcaattttgttgcacctatcagaaggcataatttcataaaatcaggattccttggcgttttaaccactctcaaaatatttgatcctactggaagttactatgcaatgctatcttgtccctgaatcaacataattcaactatcagcttcatatatatatatatatatatatattttttttttttgagacagagtttcgctgttgttgcccaggctggagtgcaatggcgcaatcttggctcaccacaacctccgcctcccgggttcaagcgattctcctgcctcagcctcctgagtagctgggattacaggcacgcaccaccaccgcagctaattttgtatttttagtagagacagggtttctccatgttggtcaggctggtcttgaactcccgacctcaggtgatccacccgcctcggcctcccagaatgctgggtttacaggcatgacccactgtgcctggcagtttcgtgtattcttactccactgggttctgctttatcgtattgacagtagacatttcattaaatgaaatgtaaaaagaacaccaatacatacatattaaaattttcttactagaatcttttagtataatttaaaaacctgaaatgagaattcgcatcactttaagtgggcctcttgggttttgaggatgaagtggctttctctcagaaatagctttgaaccgtaactctagtaactacagtggcaggctccatagcttgaacacagcgtattttgtatcaatgcccacaaataaaacctattataactcttaggaaataaaacttgaatcctgattggcagaactgcctcagtaagggctggctgaactgcatacccaaaatgttttagatctacggtccactttcacgttggctggactaatgcgtttctactgctcctcttacacgttgactgactttcctctcaggaagaggtagagactatgttccttttttcctcaatctgggacttggtttctgagacatcactgttgtaaccaagagcatggtaaaagtgatgttatgtgacattgaaggataagtcctaaaaagccaactctgccaagctctcctggagccccaaaataccacctaagtccagctgccctgaagccaccatgctagagattttcgggaaagactataccactaatagtgaaaagcacaaagagcatcctttcagctcagaagtgaaaagcttcatgagactcagaaccagaagagtctgatactcccgagttcttcacccacagaaaagcttatcatacaccattgatctttggatgctttgctaacatagcaagaaataatatacagttgatactgctaagcaccacagccaccacttggttgggttcagaagacatcctactttacctttttaaagtttggtccaaatttgtacctacaacttttccttttttcctgcagcacaggtaaaatgttggaacctttaacaagttcaggcaatgatgatataaagaagttaacatgcaactagctgcactggcttctaaattgagttcactgaccttaccatgagtttgtagtaacatttctctccaatctctgaaaaagtttttctctccaggccatctgtacgctttacgtagggactgttaaccaacccacgtattacacataaggactctaggtaaaatctagtgtttgaaaaacagcatgttatatattacactaggtttttcgttttttttccagtggtgggctgtcattacaaaagattgaacttttatacacttcctaatcaaacttaaggggaatctaaacacaaaaactaattcactttctaggagctctttaaaaatgggcttaaacctacaatccaatctcgtatctaagtatgatggaatgctttttccccagtggcattcatatagttcagctgtcaagcagtacctttcttaaaataccagactgaaaatagttcaattttctgtaaaaagtcagagccgggcacggtggctcatgcctataatcccagcagtttgggaggctgaggcgggcggatcacctgaggttggaagttcgagaccagcctgaccaacacagggaaaccccgtctctactaaaaatacaaaattagctgggcgtggtggcacatgcctgaaatcccagctacttgggaggctgaggcagaacaatcgcttgaacctgggaggcagaggttgccgtgaggcgagatcgcgacactacactcgtctgggcaacaagagtgaaactccgtctcaaaaaaaaaaaaagtcagatctgtgtaaagagaattagtgtacctgaaaattgttttcagctgtcaatcactttggtcctttactgtcattctaagaatcagcctaatttggtttaccttgtcttacaaataaggattagcaaactcaccaacataaaaaaggtgtagtacatgctgcaaaaatgtaagtatacactgacatttacttgccaaaataaccacaaatgactacacatatttaactataattaaatcaagtttttagaaatttaaagtctgcttccctagaaatacaggaactttgtgtgataaaacttgagacatatgacaatttctgaatagcaactggaatattcaaccaacaatggtcatggtcagttttgtattttttccttaacttatatacttcattctttccaactattttaaagctaaatcttttttaaaaaagttttaaaaataagtcacaggcaaatcatgaagagttgggtttatttcaacagtaaatctgaaactcttgccttaagcaagagtactacagtaattatatcaggaatagacaatttcctacactgtcaaatatataaaagttccttttgcactttcttcaacactgatcaacaagcagattcagtccacatttgctttgatctaactactgagttaacccaagcttcttcttcagagactctggcatctcgggtggaggagggcgaggaagtctgaagtagaccttcacggagtcatagataaaccactgtagtgcagtcagggtaccaatcatgatgatacgggcaaacagtcccttccatacacctttaaatccaagtctcttgaggaccagagaagcactgctacctttttctttattcaacacagataccacagaatcagcagggtgagaaacaattgcacaaaagactccagctatgtaacctgctacaaatgttacaaccagctgctctggctttgaacattcactgcggggcttaggaaccacaaacttgtacagtgcttcaacagtacgttcaaagcaggcgaacttcatcatggtgtatggtatctgtctcatccagagaggagcaacccccttgtagaatgcttttaggccttcttccttatacattttgggagctgcatccctcaaagtgttggcataacctggctgggtttgaattcgaaccttagcagcttccataggagccagggcaatgtcagcaaagaattcagcactggcagaggcagccaaatatagtgatgtgcgccagagataagtattctcctctccaagcatattgctatacaagactttaaagacttcataaaagccaaacttgcagagtccctgcatggagtagccaaggaaagtcggagcccatcctttagccaaaccacgaacaccatcctctttaagtgtaactgagaatccgttaaatatgcccttgtacttttgggggtccacctgcatacggcatttcactaaatccaggggaaccacagcagtgtgtgtcagaccacaacttaagaccccaccaaagccacacagtgcataatacttcgcggagccaaattcacaactgtactcttccacggcggcggctgccaggttgcgagggcggcggggctggcccgtgggccctggggagctgctgcggaggtccccgagaccatcgtgcaccagctgcagatgtggcgtgttgaaggggttcgcccgcgccaggtgcgccacggacgagaacatcttttccctaagatggcgatcacacaaccactcccttggaaaggttgcggctcacagag

SEQ ID NO: 12718 - RNA, 5564 nt, Homo sapiens
  source 1..5564: mol_type = other RNA
gatctcactttgttgcccaggctggtctccaactcctgggctcaagtgatacccagcctgggcctcccaaagtgctgggattacgggtatgagccactgtgcccagcctgatatacaatttcttcctcagacagtctggctctgtcgcccaggctggagtgcagtggcacaatcttggctcactgcaacctctgcctcccgggttcaagcaattctcctgcctcagcctcccgagtagctggaattacaggcatgcaccaccatgcctgaccaatttttgtatttttagtagagacctggggtttcatcatgttggccaggctgttcttgaactcctgacctcaagcaatccgcccacctcagcctcccaaagtgcttggatttcaggagtgagcttttgcacctggcctgatatacaatttctgatgctatagaagcaatgtataactcctaatttactagtgactgctatgcgcttcattaacattatggacatgtcgatcccaaaaatcatatagaaatgttactttttttttgagacagggtttcactctgtcgcccaggctggactgcaatggcgtaaacatggctcactgtagcctcaacctctcgggctcaagcaatcctcctgcctcagcctcccaaatagttgagactacaggcatgtgtcaccacaccccttaatttttgtattttcttttctcattatgttgtccaggatggtctcaaactcctgggctcaaggcatcctcctgccttggtctcctaaagtgttagaattacaggcatgagccactgtgcccagccagaaatgttaaactcactttatggtttcagaacaaggatcaaataaaataaaaatataaaaaataaaatatggttggccaagtgtggtggctcagccctctaatcccagccctttggaaggccaaggcagaaggctcgcttgagctcaggagttcaagactagccttggcaacatagcaagacctcatttctgctaaaaataaaaaacattagccagacatggtggtccacacttgcagtcccagttattcaagaggctgaggtgggaggatcacttgagcttgggagatcgaggctgcagtgagctatcatcgtgccactgcactccagtctggcgacagagcaagaccttctcaaaaataaaatatggtcgaaacgggacagacaaggcggctacctgtaaccctggccgctttaggagctggggcaggaaagttgcttgaggccaggaatccgagaccagcctgagcaacagcaggacccgtctatgaaaaaacaggagcaagtagtggcacatcccaattgtgtcagctaactgggaggctgaggcaggaggatcgcttgagcccaggagttcaaggctgtactccagcctgggcgacaaagcaagaaccctgttctctagggaaaaaaaaaaaaaagtcaaaacatttcataaaactttcacacaatggaggtttagttaagctgttactcttctgttcaattttgttgcacctatcagaaggcataatttcataaaatcaggattccttggcgttttaaccactctcaaaatatttgatcctactggaagttactatgcaatgctatcttgtccctgaatcaacataattcaactatcagcttcatatatatatatatatatatatattttttttttttgagacagagtttcgctgttgttgcccaggctggagtgcaatggcgcaatcttggctcaccacaacctccgcctcccgggttcaagcgattctcctgcctcagcctcctgagtagctgggattacaggcacgcaccaccaccgcagctaattttgtatttttagtagagacagggtttctccatgttggtcaggctggtcttgaactcccgacctcaggtgatccacccgcctcggcctcccagaatgctgggtttacaggcatgacccactgtgcctggcagtttcgtgtattcttactccactgggttctgctttatcgtattgacagtagacatttcattaaatgaaatgtaaaaagaacaccaatacatacatattaaaattttcttactagaatcttttagtataatttaaaaacctgaaatgagaattcgcatcactttaagtgggcctcttgggttttgaggatgaagtggctttctctcagaaatagctttgaaccgtaactctagtaactacagtggcaggctccatagcttgaacacagcgtattttgtatcaatgcccacaaataaaacctattataactcttaggaaataaaacttgaatcctgattggcagaactgcctcagtaagggctggctgaactgcatacccaaaatgttttagatctacggtccactttcacgttggctggactaatgcgtttctactgctcctcttacacgttgactgactttcctctcaggaagaggtagagactatgttccttttttcctcaatctgggacttggtttctgagacatcactgttgtaaccaagagcatggtaaaagtgatgttatgtgacattgaaggataagtcctaaaaagccaactctgccaagctctcctggagccccaaaataccacctaagtccagctgccctgaagccaccatgctagagattttcgggaaagactataccactaatagtgaaaagcacaaagagcatcctttcagctcagaagtgaaaagcttcatgagactcagaaccagaagagtctgatactcccgagttcttcacccacagaaaagcttatcatacaccattgatctttggatgctttgctaacatagcaagaaataatatacagttgatactgctaagcaccacagccaccacttggttgggttcagaagacatcctactttacctttttaaagtttggtccaaatttgtacctacaacttttccttttttcctgcagcacaggtaaaatgttggaacctttaacaagttcaggcaatgatgatataaagaagttaacatgcaactagctgcactggcttctaaattgagttcactgaccttaccatgagtttgtagtaacatttctctccaatctctgaaaaagtttttctctccaggccatctgtacgctttacgtagggactgttaaccaacccacgtattacacataaggactctaggtaaaatctagtgtttgaaaaacagcatgttatatattacactaggtttttcgttttttttccagtggtgggctgtcattacaaaagattgaacttttatacacttcctaatcaaacttaaggggaatctaaacacaaaaactaattcactttctaggagctctttaaaaatgggcttaaacctacaatccaatctcgtatctaagtatgatggaatgctttttccccagtggcattcatatagttcagctgtcaagcagtacctttcttaaaataccagactgaaaatagttcaattttctgtaaaaagtcagagccgggcacggtggctcatgcctataatcccagcagtttgggaggctgaggcgggcggatcacctgaggttggaagttcgagaccagcctgaccaacacagggaaaccccgtctctactaaaaatacaaaattagctgggcgtggtggcacatgcctgaaatcccagctacttgggaggctgaggcagaacaatcgcttgaacctgggaggcagaggttgccgtgaggcgagatcgcgacactacactcgtctgggcaacaagagtgaaactccgtctcaaaaaaaaaaaaagtcagatctgtgtaaagagaattagtgtacctgaaaattgttttcagctgtcaatcactttggtcctttactgtcattctaagaatcagcctaatttggtttaccttgtcttacaaataaggattagcaaactcaccaacataaaaaaggtgtagtacatgctgcaaaaatgtaagtatacactgacatttacttgccaaaataaccacaaatgactacacatatttaactataattaaatcaagtttttagaaatttaaagtctgcttccctagaaatacaggaactttgtgtgataaaacttgagacatatgacaatttctgaatagcaactggaatattcaaccaacaatggtcatggtcagttttgtattttttccttaacttatatacttcattctttccaactattttaaagctaaatcttttttaaaaaagttttaaaaataagtcacaggcaaatcatgaagagttgggtttatttcaacagtaaatctgaaactcttgccttaagcaagagtactacagtaattatatcaggaatagacaatttcctacactgtcaaatatataaaagttccttttgcactttcttcaacactgatcaacaagcagattcagtccacatttgctttgatctaactactgagttaacccaagcttcttcttcagagactctggcatctcgggtggaggagggcgaggaagtctgaagtagaccttcacggagtcatagataaaccactgtagtgcagtcagggtaccaatcatgatgatacgggcaaacagtcccttccatacacctttaaatccaagtctcttgaggaccagagaagcactgctacctttttctttattcaacacagataccacagaatcagcagggtgagaaacaattgcacaaaagactccagctatgtaacctgctacaaatgttacaaccagctgctctggctttgaacattcactgcggggcttaggaaccacaaacttgtacagtgcttcaacagtacgttcaaagcaggcgaacttcatcatggtgtatggtatctgtctcatccagagaggagcaacccccttgtagaatgcttttaggccttcttccttatacattttgggagctgcatccctcaaagtgttggcataacctggctgggtttgaattcgaaccttagcagcttccataggagccagggcaatgtcagcaaagaattcagcactggcagaggcagccaaatatagtgatgtgcgccagagataagtattctcctctccaagcatattgctatacaagactttaaagacttcataaaagccaaacttgcagagtccctgcatggagtagccaaggaaagtcggagcccatcctttagccaaaccacgaacaccatcctctttaagtgtaactgagaatccgttaaatatgcccttgtacttttgggggtccacctgcattctgcatttaaccagatctagaggaaccaatgctgtatgtgttgtgccacagctaataattcctccaagtccacaaaggataaagaatctgccagatccatagtcacagctatactgctcttccacggcggcggctgccaggttgcgagggcggcggggctggcccgtgggccctggggagctgctgcggaggtccccgagaccatcgtgcaccagctgcagatgtggcgtgttgaaggggttcgcccgcgccaggtgcgccacggacgagaacatcttttccctaagatggcgatcacacaaccactcccttggaaaggttgcggctcacagag

SEQ ID NO: 12719 - RNA, 650 nt, Homo sapiens
  source 1..650: mol_type = other RNA
gatctcactttgttgcccaggctggtctccaattcgtggcctcaagtgactctctcacctctgccttatatttccgtttgagctgttattatcaactggagtaacatttctagttggggaaaaaagaactgatccttatctgtagatgaacacttatacattcagcacttacaaataactgaatgtgggcatgaaaaaaagaatgacagatgataaacatttactgttctcaaaataaattacctaatctcagttgagataaacacgactcagaattcaattaacagtataatataaagaagccccaaaccaatgagtgcaaaaagaaagactctcaaggaaggcttccctgagtaatatttaggttgagccctataagatagaaggaagatggataactcaagaaactaaaagcagcctgtgtggtaagatggtactgaccaaaggggaatgcacaggaaggtaaggctcagaaagtagacagaaccctatcaaagcaaaattttaaatagaaagcactcttctatttcaaaataactgttatttgttcacaataatacaaaggaattataaactactaaaactaacaaaccaaagtgggcaacataggaagaccccatctctacaaaaaaaaaaaaaaaaaaaaaaaa

SEQ ID NO: 12720 - RNA, 1572 nt, Homo sapiens
  source 1..1572: mol_type = other RNA
gatctcactttgttgcccaggctggtctcgaactcctgagctcaagcagtccccctgcctcggcctcccagtgtgctgggattacaggtgtgagccaccacgcccggcctgacttatttataattcactattttatctttcttccagacaaagcaaagcatttttctctaacaacataatagtcaggattttgcttattaacttacgtgggtggctttatactcccagaacaaatgatctagctgactactaggaaaaaggtttcatagtttaggaatatatcacatcacgtgttagttccaaatgtacatgaagacaatttttaattgctgcaatagcagaatattaaggcaacatcagaaagcagaggtgttttaaaacactaagccctactccctgcctggtggaaaacaaaatgatgttactaaatcccttaatacaaaaactttccaaaataatctgttgagcttgacttcgcagtttaatcttttacagtttgatggcagtgagagagaacctgcagctataattcccttggcaaaagaattcaacatctgatttactcacaatgcttaaaataaggaagggaaaatataaaataagttttccttgcttggcaaccatctttttaattatctatttttatactgtatccaggctatgcctgggtgtggatggctaactcgcatatagaaaatatcaagcatcacatctggaagaatcacaaacgagacaatgaacttctcaatcagtacatcaacagtcaaggtaagcaagaaaaggactttaccaagaaactaacatttacactttctgacggaactgaaatacactgaattacaggcatattcactgaaacaacaaaaaaaattctgtccatgtaaaggctatattttttacccccaaaaaagtgtttcaattctgatactcacaccacaactggttaagaaaataaagcgcagtgtttagcaactgagcatcctaactaccgtaagaggcactctgtgctcaccccttcctggcaaccgctgaggtcagcaaggccaggagcaaggagagcctcctatttttcaacacaagctgctgccgtctccttattaaagccccggatggagagatcatagaccacttcctctactttcttcacgtcatatttcaatccgtcgtagcgcttcctcagggagtcatttttcaggttgagaaggcgaaaaccggaatccagctcattgatgaaggtggagatgtggaggggtcgggagtagtctccagcagtcacgctgttgacagacagcctcgacagttcactggcaagaattagaactcctgagagataatcttctacatccagatgaaatcctttctcccgatctggctcaactctcggatgtcctgctcggcagccaaaaagccctgcagctccacgaagatctcgctcacagacatggcgccggctgcacaacaatcagccagtgtagcaagggcggccaaggaagtggacgccgcaggcaaccagcgcaatcaatcgcaacggccgccgctaccgccgcgtccccccggtcttacgccacgacc

SEQ ID NO: 12721 - RNA, 1796 nt, Homo sapiens
  source 1..1796: mol_type = other RNA
gatctcactttgttgcccaggctggtctcgaactcctgagctcaagcagtccccctgcctcggcctcccagtgtgctgggattacaggtgtgagccaccacgcccggcctgacttatttataattcactattttatctttcttccagacaaagcaaagcatttttctctaacaacataatagtcaggattttgcttattaacttacgtgggtggctttatactcccagaacaaatgatctagctgactactaggaaaaaggtttcatagtttaggaatatatcacatcacgtgttagttccaaatgtacatgaagacaatttttaattgctgcaatagcagaatattaaggcaacatcagaaagcagaggtgttttaaaacactaagccctactccctgcctggtggaaaacaaaatgatgttactaaatcccttaatacaaaaactttccaaaataatctgttgagcttgacttcgcagtttaatcttttacagtttgatggcagtgagagagaacctgcagctataattcccttggcaaaagaattcaacatctgatttactcacaatgcttaaaataaggaagggaaaatataaaataagttttccttgcttggcaaccatctttttaattatctatttttatactgtatccaggctatgcctgggtgtggatggctaactcgcatatagaaaatatcaagcatcacatctggaagaatcacaaacgagacaatgaacttctcaatcagtacatcaacagtcaaggtaagcaagaaaaggactttaccaagaaactaacatttacactttctgacggaactgaaatacactgaattacaggcatattcactgaaacaacaaaaaaaattctgtccatgtaaaggctatattttttacccccaaaaaagtgtttcaattctgatactcacaccacaactggttaagaaaataaagcgcagtgtttagcaactgagcatcctaactaccgtaagaggcactctgtgctcaccccttcctggcaaccgctgaggtcagcaaggccaggagcaaggagagcctcctatttttcaacacaagctgctgccgtctccttattaaagccccggatggagagatcatagaccacttcctctactttcttcacgtcatatttcaatccgtcgtagcgcttcctcagggagtcatttttcaggttgagaaggcgaaaaccggaatccagctcattgatgaaggtggagatgtggaggggtcgggagtagtctccagcagtcacgctgttgacagacagcctcgacagttcactggcaagaattagaactcctgagagataatcttctacatccagatgaaatcctttctcccgatctggctcaatgccaagaatttctgtaactgcttctcgagtcactagtgtttctgtttccaaatacacaacaaatgctgccaagaagaccaagcgctgcaacacaaacctccagtgctcatgaaatcctcggaggcgtccccaccgcccgagactgagcgacagaggagggccgggcgaagtggcccaactaggcatggaaaggcaaagggaatggggaagggagggggctcgcctctcggatgtcctgctcggcagccaaaaagccctgcagctccacgaagatctcgctcacagacatggcgccggctgcacaacaatcagccagtgtagcaagggcggccaaggaagtggacgccgcaggcaaccagcgcaatcaatcgcaacggccgccgctaccgccgcgtccccccggtcttacgccacgacc

SEQ ID NO: 12722 - RNA, 1688 nt, Homo sapiens
  source 1..1688: mol_type = other RNA
gatctcactttgttgcccaggctggtctcgaactcctgagctcaagcagtccccctgcctcggcctcccagtgtgctgggattacaggtgtgagccaccacgcccggcctgacttatttataattcactattttatctttcttccagacaaagcaaagcatttttctctaacaacataatagtcaggattttgcttattaacttacgtgggtggctttatactcccagaacaaatgatctagctgactactaggaaaaaggtttcatagtttaggaatatatcacatcacgtgttagttccaaatgtacatgaagacaatttttaattgctgcaatagcagaatattaaggcaacatcagaaagcagaggtgttttaaaacactaagccctactccctgcctggtggaaaacaaaatgatgttactaaatcccttaatacaaaaactttccaaaataatctgttgagcttgacttcgcagtttaatcttttacagtttgatggcagtgagagagaacctgcagctataattcccttggcaaaagaattcaacatctgatttactcacaatgcttaaaataaggaagggaaaatataaaataagttttccttgcttggcaaccatctttttaattatctatttttatactgtatccaggctatgcctgggtgtggatggctaactcgcatatagaaaatatcaagcatcacatctggaagaatcacaaacgagacaatgaacttctcaatcagtacatcaacagtcaaggtaagcaagaaaaggactttaccaagaaactaacatttacactttctgacggaactgaaatacactgaattacaggcatattcactgaaacaacaaaaaaaattctgtccatgtaaaggctatattttttacccccaaaaaagtgtttcaattctgatactcacaccacaactggttaagaaaataaagcgcagtgtttagcaactgagcatcctaactaccgtaagaggcactctgtgctcaccccttcctggcaaccgctgaggtcagcaaggccaggagcaaggagagcctcctatttttcaacacaagctgctgccgtctccttattaaagccccggatggagagatcatagaccacttcctctactttcttcacgtcatatttcaatccgtcgtagcgcttcctcagggagtcatttttcaggttgagaaggcgaaaaccggaatccagctcattgatgaaggtggagatgtggaggggtcgggagtagtctccagcagtcacgctgttgacagacagcctcgacagttcactggcaagaattagaactcctgagagataatcttctacatccagatgaaatcctttctcccgatctggctcaatgccaagaatttctgtaactgcttctcgagtcactagtgtttctgtttccaaatacacaacaaatgctgccaagaagaccaagcgctgcaacacaaacctccagtgctcatgaaatctctcggatgtcctgctcggcagccaaaaagccctgcagctccacgaagatctcgctcacagacatggcgccggctgcacaacaatcagccagtgtagcaagggcggccaaggaagtggacgccgcaggcaaccagcgcaatcaatcgcaacggccgccgctaccgccgcgtccccccggtcttacgccacgacc

SEQ ID NO: 12723 - RNA, 1785 nt, Homo sapiens
  source 1..1785: mol_type = other RNA
gatctcactttgttgcccaggctggtctcgaactcctgagctcaagcagtccccctgcctcggcctcccagtgtgctgggattacaggtgtgagccaccacgcccggcctgacttatttataattcactattttatctttcttccagacaaagcaaagcatttttctctaacaacataatagtcaggattttgcttattaacttacgtgggtggctttatactcccagaacaaatgatctagctgactactaggaaaaaggtttcatagtttaggaatatatcacatcacgtgttagttccaaatgtacatgaagacaatttttaattgctgcaatagcagaatattaaggcaacatcagaaagcagaggtgttttaaaacactaagccctactccctgcctggtggaaaacaaaatgatgttactaaatcccttaatacaaaaactttccaaaataatctgttgagcttgacttcgcagtttaatcttttacagtttgatggcagtgagagagaacctgcagctataattcccttggcaaaagaattcaacatctgatttactcacaatgcttaaaataaggaagggaaaatataaaataagttttccttgcttggcaaccatctttttaattatctatttttatactgtatccaggctatgcctgggtgtggatggctaactcgcatatagaaaatatcaagcatcacatctggaagaatcacaaacgagacaatgaacttctcaatcagtacatcaacagtcaaggtaagcaagaaaaggactttaccaagaaactaacatttacactttctgacggaactgaaatacactgaattacaggcatattcactgaaacaacaaaaaaaattctgtccatgtaaaggctatattttttacccccaaaaaagtgtttcaattctgatactcacaccacaactggttaagaaaataaagcgcagtgtttagcaactgagcatcctaactaccgtaagaggcactctgtgctcaccccttcctggcaaccgctgaggtcagcaaggccaggagcaaggagagcctcctatttttcaacacaagctgctgccgtctccttattaaagccccggatggagagatcatagaccacttcctctactttcttcacgtcatatttcaatccgtcgtagcgcttcctcagggagtcatttttcaggttgagaaggcgaaaaccggaatccagctcattgatgaaggtggagatgtggaggggtcgggagtagtctccagcagtcacgctgttgacagacagcctcgacagttcactggcaagaattagaactcctgagagataatcttctacatccagatgaaatcctttctcccgatctggctcaatgccaagaatttctgtaactgcttctcgagtcactagtgtttctgtttccaaatacacaacaaatgctgccaagaagaccaagcgctgcaacacaaacctccagtgctcatgaaatctgtaatactgttcagcaggaaatttggtcttcaaagatgttagatgtgtttttactgtaccaaaatgttctcgagctttcaaacacctctttggaactctcggatgtcctgctcggcagccaaaaagccctgcagctccacgaagatctcgctcacagacatggcgccggctgcacaacaatcagccagtgtagcaagggcggccaaggaagtggacgccgcaggcaaccagcgcaatcaatcgcaacggccgccgctaccgccgcgtccccccggtcttacgccacgacc

SEQ ID NO: 12724 - RNA, 1879 nt, Homo sapiens
  source 1..1879: mol_type = other RNA
gatctcactttgttgcccaggctggtctcgaactcctgagctcaagcagtccccctgcctcggcctcccagtgtgctgggattacaggtgtgagccaccacgcccggcctgacttatttataattcactattttatctttcttccagacaaagcaaagcatttttctctaacaacataatagtcaggattttgcttattaacttacgtgggtggctttatactcccagaacaaatgatctagctgactactaggaaaaaggtttcatagtttaggaatatatcacatcacgtgttagttccaaatgtacatgaagacaatttttaattgctgcaatagcagaatattaaggcaacatcagaaagcagaggtgttttaaaacactaagccctactccctgcctggtggaaaacaaaatgatgttactaaatcccttaatacaaaaactttccaaaataatctgttgagcttgacttcgcagtttaatcttttacagtttgatggcagtgagagagaacctgcagctataattcccttggcaaaagaattcaacatctgatttactcacaatgcttaaaataaggaagggaaaatataaaataagttttccttgcttggcaaccatctttttaattatctatttttatactgtatccaggctatgcctgggtgtggatggctaactcgcatatagaaaatatcaagcatcacatctggaagaatcacaaacgagacaatgaacttctcaatcagtacatcaacagtcaaggtaagcaagaaaaggactttaccaagaaactaacatttacactttctgacggaactgaaatacactgaattacaggcatattcactgaaacaacaaaaaaaattctgtccatgtaaaggctatattttttacccccaaaaaagtgtttcaattctgatactcacaccacaactggttaagaaaataaagcgcagtgtttagcaactgagcatcctaactaccgtaagaggcactctgtgctcaccccttcctggcaaccgctgaggtcagcaaggccaggagcaaggagagcctcctatttttcaacacaagctgctgccgtctccttattaaagccccggatggagagatcatagaccacttcctctactttcttcacgtcatatttcaatccgtcgtagcgcttcctcagggagtcatttttcaggttgagaaggcgaaaaccggaatccagctcattgatgaaggtggagatgtggaggggtcgggagtagtctccagcagtcacgctgttgacagacagcctcgacagttcactggcaagaattagaactcctgagagataatcttctacatccagatgaaatcctttctcccgatctggctcaatgccaagaatttctgtaactgcttctcgagtcactagtgtttctgtttccaaatacacaacaaatgctgccaagaagaccaagcgctgcaacacaaacctccagtgctcatgaaatctgtaatactgttcagcaggaaatttggtcttcaaagatgttagatgtgtttttactgtaccaaaatgttctcgagctttcaaacacctctttggaatgtcctgaaacccagcaccctgatggaccccttgcagtagagttaaaatctctcgagctgtttgttctaaactctgtacaacttttctgatttcctctcggatgtcctgctcggcagccaaaaagccctgcagctccacgaagatctcgctcacagacatggcgccggctgcacaacaatcagccagtgtagcaagggcggccaaggaagtggacgccgcaggcaaccagcgcaatcaatcgcaacggccgccgctaccgccgcgtccccccggtcttacgccacgacc

SEQ ID NO: 12725 - RNA, 1799 nt, Homo sapiens
  source 1..1799: mol_type = other RNA
gatctcactttgttgcccaggctggtctcgaactcctgagctcaagcagtccccctgcctcggcctcccagtgtgctgggattacaggtgtgagccaccacgcccggcctgacttatttataattcactattttatctttcttccagacaaagcaaagcatttttctctaacaacataatagtcaggattttgcttattaacttacgtgggtggctttatactcccagaacaaatgatctagctgactactaggaaaaaggtttcatagtttaggaatatatcacatcacgtgttagttccaaatgtacatgaagacaatttttaattgctgcaatagcagaatattaaggcaacatcagaaagcagaggtgttttaaaacactaagccctactccctgcctggtggaaaacaaaatgatgttactaaatcccttaatacaaaaactttccaaaataatctgttgagcttgacttcgcagtttaatcttttacagtttgatggcagtgagagagaacctgcagctataattcccttggcaaaagaattcaacatctgatttactcacaatgcttaaaataaggaagggaaaatataaaataagttttccttgcttggcaaccatctttttaattatctatttttatactgtatccaggctatgcctgggtgtggatggctaactcgcatatagaaaatatcaagcatcacatctggaagaatcacaaacgagacaatgaacttctcaatcagtacatcaacagtcaaggtaagcaagaaaaggactttaccaagaaactaacatttacactttctgacggaactgaaatacactgaattacaggcatattcactgaaacaacaaaaaaaattctgtccatgtaaaggctatattttttacccccaaaaaagtgtttcaattctgatactcacaccacaactggttaagaaaataaagcgcagtgtttagcaactgagcatcctaactaccgtaagaggcactctgtgctcaccccttcctggcaaccgctgaggtcagcaaggccaggagcaaggagagcctcctatttttcaacacaagctgctgccgtctccttattaaagccccggatggagagatcatagaccacttcctctactttcttcacgtcatatttcaatccgtcgtagcgcttcctcagggagtcatttttcaggttgagaaggcgaaaaccggaatccagctcattgatgaaggtggagatgtggaggggtcgggagtagtctccagcagtcacgctgttgacagacagcctcgatgccaagaatttctgtaactgcttctcgagtcactagtgtttctgtttccaaatacacaacaaatgctgccaagaagaccaagcgctgcaacacaaacctccagtgctcatgaaatctgtaatactgttcagcaggaaatttggtcttcaaagatgttagatgtgtttttactgtaccaaaatgttctcgagctttcaaacacctctttggaatgtcctgaaacccagcaccctgatggaccccttgcagtagagttaaaatctctcgagctgtttgttctaaactctgtacaacttttctgatttcctctcggatgtcctgctcggcagccaaaaagccctgcagctccacgaagatctcgctcacagacatggcgccggctgcacaacaatcagccagtgtagcaagggcggccaaggaagtggacgccgcaggcaaccagcgcaatcaatcgcaacggccgccgctaccgccgcgtccccccggtcttacgccacgacc

SEQ ID NO: 12726 - RNA, 3883 nt, Homo sapiens
  source 1..3883: mol_type = other RNA
gatctcactttgttgcccaggctggtctcttttacctgagctcaagtgatcctcctgccttagcctcccaaagtgctgcgattacaggcattagacactgcacccactctaatttgttttgttttgttttgtttcgttttgagatggagtctcactctgtcacctaggctggagtgcagtggagtgatctcagctcaatgcaaactccacctcctgggttcaagtgtttcttgttcctcagtctcccaagtagctgggattacaagtgcgtgccaccatgcccagctaatttttgtagttttagtagagatgaggtttcaccatattggccaggctaatctcgaactcctgacctcaagccatccgcctgccttggcctcccaaagtgctgggattacaggcgtgagccattgcacccagccatgtttttaagagaatgggtcttgctaccttgcccgggctggaatgcagtggttattcataggcgttataacacactctagtttctaactcctggcctcaagcaatcctcctgcctcagcctcctcagaacctgggactatagccttgcaccactgcactcggcttaacattttagcattaatgttgccatacagttttttgaaccctttcccaaaagccaacatcactgcctccctagctaaattcagtctgttctgtcacgtagaaaaataacagtaacatatctttttacctgaagggtcaaaccactctaactggcataggaaacatcctttatttttcatgattatgcaacttctttacatgagatgttggcattttgttcctagcatgtaacagaatcagtgatttaagatatcagattctgagttgtgagatttaaaagcataaaagttgaattgccttgcagcatttctcaagtgagaaatacaaaaatgatgttcacagcagacccaaattggggtcattcagcactagctgagacttgtttgcataatttcctttcctacccaattcattcaggctcctatgtagcttatacaggggtgggaatatgactcaaagtgcaaaaataaaatatttcacccagataaggaaggagcaagcttctgctatgtggcctaattgcaggcctcagaatgccagcaccttttctaagtttttgttttaaaatggaatgtaaaaactacataattaatattccaagcagcttaagctcattagttgggagtttaaattccaattccataaccatcctactgtcataactactgtaaaaaaatcattaaaaataaagtaacaaatgttatcatagatgtgaaattacttaaagtactaaatttctagtgttgtaaatagcagctaagttatatcacttcctgactgccaaattaagactaaatagaaagaatgtatatacaccattatatttaaaagtaaaaaacaacgaaactttttcatatccaagtatgtctgagactgtttacttccaacagccaagaatgataaatttcaaaaaccaaaaagttatattttgcgtgctgtaagtttcttttcaggagaaaacaattctttgcatgcatacctccctacttaacggcattaagaactttatctaacatctggtaaaacactcctatttggctcatttaataacaccattaaaaaagcataaaattgaactgtcatctaacaactatagcacaaagaagttattctgggtacctataccactaacattaagcccatttatttttatggatgcagccatttttccctcatgaatactcactgagggtcacactggcactgcatcttttgttgcatctttggtgaaatatgccagccctacatttgcattaatgaggagaccaatggcatcctagccagtactctgtcacgtcatctatggcctctttcattctcttcttatttcaggcatcctggtatgctcagtatatttaaagatggttcagaaggcaaaaactctttgtcagtaaaacagatcatgtcccagggttgcattttttaaaatgaaacaaagattagtccaaagaacaagtactgtcacttgttagggtttcttcttctaaaggtaataaggagcttcaaaacatattatttcttgactagagccctactggaaatcaatgaaaattcctcaaccagcaaactgctcaagttgacttgtttaaagttcaataagcaaatactcaacaggtaagggtacagcctgacttcaatcacaacattaagtcttcctaaagagaaggggcagaaaacatctacttaagctttctgttcaaatagctacataaggactcttgattgttctttcttgctttttataatcataactttgctcagaacagaaaactttactttgtcaacacataagccaggcatctaagaacaacctagggggagaacgcaaagttactcattttcaacaactattatatatttaatcacaaattcattagaaagatagtattcatccaattagtcttttcattattgctggttttgaaaatggccaacaatattcattaggtactgtgccattaacattgcattcaaaaaaagagaacatgggaaaccaaatccttgctctcctactctgctgatatgctctggtattggccagagtatggtagtacaaaaagagtcttgttgttatataaaaagcaataaacacatcaatagaataatgttcatgggcagccaagatgaagaagattccaaagaggttgagaacccaggataaagtgtgcaagaaattccagcttcttggtgtatattcggtgacaaagaaattcagcatagttaggacgactgtgtggccactaaacatgtaatctccacatgtgtgaacgccagtcagggtcataccaaagccactccaaatggcaaaggctcgatgtaatttctcccatacactgccatatatctttccagtacactgcaggtgttgtcctggcacggagagggaggtcacaaacatggtaaagcagcgaagcaagaatacagttcccatcagactacagagccttcgcagaagtattgacctgtgcttgtgaagaagaagaaccaggagccaaatatagcacagaatcatgccacatacttccgtcatggcaaaggcccatgggattctaggaacgctgtctaagaatatatctgggagtggtggataggtctgcatgtcaggcactcgctcatggactataaccataatgaaagatgtaaatccaaatactataaaaacatatatacaactcagtatagtcttccagtattctgggtccaatcttcgaacagaatgtttgtttttaccattcatgtactggtactgatcagaattcaagtcagttatgggtccgtcacagtcatgggaaagctccccattacagagccagtctgtactctgaagagcactgatgaaaggggtcatggaacccatgggactgtcactgttgtagcccatctcttctaaaacatcaatatgtattttctgcaattttcggactgagagcattaaccttttaatgtcccctaagactttgatttccagaggaggagaccggagatcatattcagtcaatgttagcaatgtgattccatcaagtcggtgcttattgcataaaatgtccacatattcaaaaaagccttcatccttcagccacacagctacatgcttggtagtccagcggcgaatgcagagttgattaggacctgccatttcctcctccgctgccaccaatgggttccatgtcactcccattcttgtagcattattcgttaggacagtttcctctcatactctgttcaaaatgattcttctcttcttttatatgtttttttccactgtcttagctcaccagttctttacaacctcaat

SEQ ID NO: 12727 - RNA, 3817 nt, Homo sapiens
  source 1..3817: mol_type = other RNA
gatctcactttgttgcccaggctggtctcttttacctgagctcaagtgatcctcctgccttagcctcccaaagtgctgcgattacaggcattagacactgcacccactctaatttgttttgttttgttttgtttcgttttgagatggagtctcactctgtcacctaggctggagtgcagtggagtgatctcagctcaatgcaaactccacctcctgggttcaagtgtttcttgttcctcagtctcccaagtagctgggattacaagtgcgtgccaccatgcccagctaatttttgtagttttagtagagatgaggtttcaccatattggccaggctaatctcgaactcctgacctcaagccatccgcctgccttggcctcccaaagtgctgggattacaggcgtgagccattgcacccagccatgtttttaagagaatgggtcttgctaccttgcccgggctggaatgcagtggttattcataggcgttataacacactctagtttctaactcctggcctcaagcaatcctcctgcctcagcctcctcagaacctgggactatagccttgcaccactgcactcggcttaacattttagcattaatgttgccatacagttttttgaaccctttcccaaaagccaacatcactgcctccctagctaaattcagtctgttctgtcacgtagaaaaataacagtaacatatctttttacctgaagggtcaaaccactctaactggcataggaaacatcctttatttttcatgattatgcaacttctttacatgagatgttggcattttgttcctagcatgtaacagaatcagtgatttaagatatcagattctgagttgtgagatttaaaagcataaaagttgaattgccttgcagcatttctcaagtgagaaatacaaaaatgatgttcacagcagacccaaattggggtcattcagcactagctgagacttgtttgcataatttcctttcctacccaattcattcaggctcctatgtagcttatacaggggtgggaatatgactcaaagtgcaaaaataaaatatttcacccagataaggaaggagcaagcttctgctatgtggcctaattgcaggcctcagaatgccagcaccttttctaagtttttgttttaaaatggaatgtaaaaactacataattaatattccaagcagcttaagctcattagttgggagtttaaattccaattccataaccatcctactgtcataactactgtaaaaaaatcattaaaaataaagtaacaaatgttatcatagatgtgaaattacttaaagtactaaatttctagtgttgtaaatagcagctaagttatatcacttcctgactgccaaattaagactaaatagaaagaatgtatatacaccattatatttaaaagtaaaaaacaacgaaactttttcatatccaagtatgtctgagactgtttacttccaacagccaagaatgataaatttcaaaaaccaaaaagttatattttgcgtgctgtaagtttcttttcaggagaaaacaattctttgcatgcatacctccctacttaacggcattaagaactttatctaacatctggtaaaacactcctatttggctcatttaataacaccattaaaaaagcataaaattgaactgtcatctaacaactatagcacaaagaagttattctgggtacctataccactaacattaagcccatttatttttatggatgcagccatttttccctcatgaatactcactgagggtcacactggcactgcatcttttgttgcatctttggtgaaatatgccagccctacatttgcattaatgaggagaccaatggcatcctagccagtactctgtcacgtcatctatggcctctttcattctcttcttatttcaggcatcctggtatgctcagtatatttaaagatggttcagaaggcaaaaactctttgtcagtaaaacagatcatgtcccagggttgcattttttaaaatgaaacaaagattagtccaaagaacaagtactgtcacttgttagggtttcttcttctaaaggtaataaggagcttcaaaacatattatttcttgactagagccctactggaaatcaatgaaaattcctcaaccagcaaactgctcaagttgacttgtttaaagttcaataagcaaatactcaacaggtaagggtacagcctgacttcaatcacaacattaagtcttcctaaagagaaggggcagaaaacatctacttaagctttctgttcaaatagctacataaggactcttgattgttctttcttgctttttataatcataactttgctcagaacagaaaactttactttgtcaacacataagccaggcatctaagaacaacctagggggagaacgcaaagttactcattttcaacaactattatatatttaatcacaaattcattagaaagatagtattcatccaattagtcttttcattattgctggttttgaaaatggccaacaatattcattaggtactgtgccattaacattgcattcaaaaaaagagaacatgggaaaccaaatccttgctctcctactctgctgatatgctctggtattggccagagtatggtagtacaaaaagagtcttgttgttatataaaaagcaataaacacatcaatagaataatgttcatgggcagccaagatgaagaagattccaaagaggttgagaacccaggataaagtgtgcaagaaattccagcttcttggtgtatattcggtgacaaagaaattcagcatagttaggacgactgtgtggccactaaacatgtaatctccacatgtgtgaacgccagtcagggtcataccaaagccactccaaatggcaaaggctcgatgtaatttctcccatacactgccatatatctttccagtacactgcaggtgttgtcctggcacggagagggaggtcacaaacatggtaaagcagcgaagcaagaatacagttcccatcagactacagagccttcgcagaagtattgacctgtgcttgtgaagaagaagaaccaggagccaaatatagcacagaatcatgccacatacttccgtcatggcaaaggcccatgggattctaggaacgctgtctaagaatatatctgggagtggtggataggtctgcatgtcaggcactcgctcatggactataaccataatgaaagatgtaaatccaaatactataaaaacatatatacaactcagtatagtcttccagtattctgggtccaatcttcgaacagaatgtttgtttttaccattcatgtactggtactgatcagaattcaagtcagttatgggtccgtcacagtcatgggaaagctccccattacagagccagtctgtactctgaagagcactgatgaaaggggtcatggaacccatgggactgtcactgttgtagcccatctcttctaaaacatcaatatgtattttctgcaattttcggactgagagcattaaccttttaatgtcccctaagactttgatttccagaggaggagaccggagatcatattcagtcaatgttagcaatgtgattccatcaagtcggtgcttattgcataaaatgtccacatattcaaaaaagccttcatccttcagccacacagctacatgcttggtagtccagcggcgaatgcagagttgattaggacctgccatttcctcctccgctgcccttggcagcaggcgccccccaagctcccctctcctcagcctcagctcccgctcacctccgcggtccgagtcgggctc

SEQ ID NO: 12728 - RNA, 3806 nt, Homo sapiens
  source 1..3806: mol_type = other RNA
gatctcactttgttgcccaggctggtctcttttacctgagctcaagtgatcctcctgccttagcctcccaaagtgctgcgattacaggcattagacactgcacccactctaatttgttttgttttgttttgtttcgttttgagatggagtctcactctgtcacctaggctggagtgcagtggagtgatctcagctcaatgcaaactccacctcctgggttcaagtgtttcttgttcctcagtctcccaagtagctgggattacaagtgcgtgccaccatgcccagctaatttttgtagttttagtagagatgaggtttcaccatattggccaggctaatctcgaactcctgacctcaagccatccgcctgccttggcctcccaaagtgctgggattacaggcgtgagccattgcacccagccatgtttttaagagaatgggtcttgctaccttgcccgggctggaatgcagtggttattcataggcgttataacacactctagtttctaactcctggcctcaagcaatcctcctgcctcagcctcctcagaacctgggactatagccttgcaccactgcactcggcttaacattttagcattaatgttgccatacagttttttgaaccctttcccaaaagccaacatcactgcctccctagctaaattcagtctgttctgtcacgtagaaaaataacagtaacatatctttttacctgaagggtcaaaccactctaactggcataggaaacatcctttatttttcatgattatgcaacttctttacatgagatgttggcattttgttcctagcatgtaacagaatcagtgatttaagatatcagattctgagttgtgagatttaaaagcataaaagttgaattgccttgcagcatttctcaagtgagaaatacaaaaatgatgttcacagcagacccaaattggggtcattcagcactagctgagacttgtttgcataatttcctttcctacccaattcattcaggctcctatgtagcttatacaggggtgggaatatgactcaaagtgcaaaaataaaatatttcacccagataaggaaggagcaagcttctgctatgtggcctaattgcaggcctcagaatgccagcaccttttctaagtttttgttttaaaatggaatgtaaaaactacataattaatattccaagcagcttaagctcattagttgggagtttaaattccaattccataaccatcctactgtcataactactgtaaaaaaatcattaaaaataaagtaacaaatgttatcatagatgtgaaattacttaaagtactaaatttctagtgttgtaaatagcagctaagttatatcacttcctgactgccaaattaagactaaatagaaagaatgtatatacaccattatatttaaaagtaaaaaacaacgaaactttttcatatccaagtatgtctgagactgtttacttccaacagccaagaatgataaatttcaaaaaccaaaaagttatattttgcgtgctgtaagtttcttttcaggagaaaacaattctttgcatgcatacctccctacttaacggcattaagaactttatctaacatctggtaaaacactcctatttggctcatttaataacaccattaaaaaagcataaaattgaactgtcatctaacaactatagcacaaagaagttattctgggtacctataccactaacattaagcccatttatttttatggatgcagccatttttccctcatgaatactcactgagggtcacactggcactgcatcttttgttgcatctttggtgaaatatgccagccctacatttgcattaatgaggagaccaatggcatcctagccagtactctgtcacgtcatctatggcctctttcattctcttcttatttcaggcatcctggtatgctcagtatatttaaagatggttcagaaggcaaaaactctttgtcagtaaaacagatcatgtcccagggttgcattttttaaaatgaaacaaagattagtccaaagaacaagtactgtcacttgttagggtttcttcttctaaaggtaataaggagcttcaaaacatattatttcttgactagagccctactggaaatcaatgaaaattcctcaaccagcaaactgctcaagttgacttgtttaaagttcaataagcaaatactcaacaggtaagggtacagcctgacttcaatcacaacattaagtcttcctaaagagaaggggcagaaaacatctacttaagctttctgttcaaatagctacataaggactcttgattgttctttcttgctttttataatcataactttgctcagaacagaaaactttactttgtcaacacataagccaggcatctaagaacaacctagggggagaacgcaaagttactcattttcaacaactattatatatttaatcacaaattcattagaaagatagtattcatccaattagtcttttcattattgctggttttgaaaatggccaacaatattcattaggtactgtgccattaacattgcattcaaaaaaagagaacatgggaaaccaaatccttgctctcctactctgctgatatgctctggtattggccagagtatggtagtacaaaaagagtcttgttgttatataaaaagcaataaacacatcaatagaataatgttcatgggcagccaagatgaagaagattccaaagaggttgagaacccaggataaagtgtgcaagaaattccagcttcttggtgtatattcggtgacaaagaaattcagcatagttaggacgactgtgtggccactaaacatgtaatctccacatgtgtgaacgccagtcagggtcataccaaagccactccaaatggcaaaggctcgatgtaatttctcccatacactgccatatatctttccagtacactgcaggtgttgtcctggcacggagagggaggtcacaaacatggtaaagcagcgaagcaagaatacagttcccatcagactacagagccttcgcagaagtattgacctgtgcttgtgaagaagaagaaccaggagccaaatatagcacagaatcatgccacatacttccgtcatggcaaaggcccatgggattctaggaacgctgtctaagaatatatctgggagtggtggataggtctgcatgtcaggcactcgctcatggactataaccataatgaaagatgtaaatccaaatactataaaaacatatatacaactcagtatagtcttccagtattctgggtccaatcttcgaacagaatgtttgtttttaccattcatgtactggtactgatcagaattcaagtcagttatgggtccgtcacagtcatgggaaagctccccattacagagccagtctgtactctgaagagcactgatgaaaggggtcatggaacccatgggactgtcactgttgtagcccatctcttctaaaacatcaatatgtattttctgcaattttcggactgagagcattaaccttttaatgtcccctaagactttgatttccagaggaggagaccggagatcatattcagtcaatgttagcaatgtgattccatcaagtcggtgcttattgcataaaatgtccacatattcaaaaaagccttcatccttcagccacacagctacatgcttggtagtccagcggcgaatgcagagttgattaggacctgccatttcctcctccgctgcctccgcggtccgagtcgggctccccggacccacctccgagtcggcgtccgagccgccgtcggagtcc

SEQ ID NO: 12729 - RNA, 3893 nt, Homo sapiens
  source 1..3893: mol_type = other RNA
gatctcactttgttgcccaggctggtctcttttacctgagctcaagtgatcctcctgccttagcctcccaaagtgctgcgattacaggcattagacactgcacccactctaatttgttttgttttgttttgtttcgttttgagatggagtctcactctgtcacctaggctggagtgcagtggagtgatctcagctcaatgcaaactccacctcctgggttcaagtgtttcttgttcctcagtctcccaagtagctgggattacaagtgcgtgccaccatgcccagctaatttttgtagttttagtagagatgaggtttcaccatattggccaggctaatctcgaactcctgacctcaagccatccgcctgccttggcctcccaaagtgctgggattacaggcgtgagccattgcacccagccatgtttttaagagaatgggtcttgctaccttgcccgggctggaatgcagtggttattcataggcgttataacacactctagtttctaactcctggcctcaagcaatcctcctgcctcagcctcctcagaacctgggactatagccttgcaccactgcactcggcttaacattttagcattaatgttgccatacagttttttgaaccctttcccaaaagccaacatcactgcctccctagctaaattcagtctgttctgtcacgtagaaaaataacagtaacatatctttttacctgaagggtcaaaccactctaactggcataggaaacatcctttatttttcatgattatgcaacttctttacatgagatgttggcattttgttcctagcatgtaacagaatcagtgatttaagatatcagattctgagttgtgagatttaaaagcataaaagttgaattgccttgcagcatttctcaagtgagaaatacaaaaatgatgttcacagcagacccaaattggggtcattcagcactagctgagacttgtttgcataatttcctttcctacccaattcattcaggctcctatgtagcttatacaggggtgggaatatgactcaaagtgcaaaaataaaatatttcacccagataaggaaggagcaagcttctgctatgtggcctaattgcaggcctcagaatgccagcaccttttctaagtttttgttttaaaatggaatgtaaaaactacataattaatattccaagcagcttaagctcattagttgggagtttaaattccaattccataaccatcctactgtcataactactgtaaaaaaatcattaaaaataaagtaacaaatgttatcatagatgtgaaattacttaaagtactaaatttctagtgttgtaaatagcagctaagttatatcacttcctgactgccaaattaagactaaatagaaagaatgtatatacaccattatatttaaaagtaaaaaacaacgaaactttttcatatccaagtatgtctgagactgtttacttccaacagccaagaatgataaatttcaaaaaccaaaaagttatattttgcgtgctgtaagtttcttttcaggagaaaacaattctttgcatgcatacctccctacttaacggcattaagaactttatctaacatctggtaaaacactcctatttggctcatttaataacaccattaaaaaagcataaaattgaactgtcatctaacaactatagcacaaagaagttattctgggtacctataccactaacattaagcccatttatttttatggatgcagccatttttccctcatgaatactcactgagggtcacactggcactgcatcttttgttgcatctttggtgaaatatgccagccctacatttgcattaatgaggagaccaatggcatcctagccagtactctgtcacgtcatctatggcctctttcattctcttcttatttcaggcatcctggtatgctcagtatatttaaagatggttcagaaggcaaaaactctttgtcagtaaaacagatcatgtcccagggttgcattttttaaaatgaaacaaagattagtccaaagaacaagtactgtcacttgttagggtttcttcttctaaaggtaataaggagcttcaaaacatattatttcttgactagagccctactggaaatcaatgaaaattcctcaaccagcaaactgctcaagttgacttgtttaaagttcaataagcaaatactcaacaggtaagggtacagcctgacttcaatcacaacattaagtcttcctaaagagaaggggcagaaaacatctacttaagctttctgttcaaatagctacataaggactcttgattgttctttcttgctttttataatcataactttgctcagaacagaaaactttactttgtcaacacataagccaggcatctaagaacaacctagggggagaacgcaaagttactcattttcaacaactattatatatttaatcacaaattcattagaaagatagtattcatccaattagtcttttcattattgctggttttgaaaatggccaacaatattcattaggtactgtgccattaacattgcattcaaaaaaagagaacatgggaaaccaaatccttgctctcctactctgctgatatgctctggtattggccagagtatggtagtacaaaaagagtcttgttgttatataaaaagcaataaacacatcaatagaataatgttcatgggcagccaagatgaagaagattccaaagaggttgagaacccaggataaagtgtgcaagaaattccagcttcttggtgtatattcggtgacaaagaaattcagcatagttaggacgactgtgtggccactaaacatgtaatctccacatgtgtgaacgccagtcagggtcataccaaagccactccaaatggcaaaggctcgatgtaatttctcccatacactgccatatatctttccagtacactgcaggtgttgtcctggcacggagagggaggtcacaaacatggtaaagcagcgaagcaagaatacagttcccatcagactacagagccttcgcagaagtattgacctgtgcttgtgaagaagaagaaccaggagccaaatatagcacagaatcatgccacatacttccgtcatggcaaaggcccatgggattctaggaacgctgtctaagaatatatctgggagtggtggataggtctgcatgtcaggcactcgctcatggactataaccataatgaaagatgtaaatccaaatactataaaaacatatatacaactcagtatagtcttccagtattctgggtccaatcttcgaacagaatgtttgtttttaccattcatgtactggtactgatcagaattcaagtcagttatgggtccgtcacagtcatgggaaagctccccattacagagccagtctgtactctgaagagcactgatgaaaggggtcatggaacccatgggactgtcactgttgtagcccatctcttctaaaacatcaatatgtattttctgcaattttcggactgagagcattaaccttttaatgtcccctaagactttgatttccagaggaggagaccggagatcatattcagtcaatgttagcaatgtgattccatcaagtcggtgcttattgcataaaatgtccacatattcaaaaaagccttcatccttcagccacacagctacatgcttggtagtccagcggcgaatgcagagttgattaggacctgccatttcctcctccgctgcctcttcaggtagactcccatcttcatggaggtttatggaaccaacggtcttcaatcccaaacagataccaagcagagaggaggcctgggggtttagagggaccggagggcccactgcagtccacaaggcctcagtcggctctcaggccccaccc

SEQ ID NO: 12730 - RNA, 3911 nt, Homo sapiens
  source 1..3911: mol_type = other RNA
gatctcactttgttgcccaggctggtctcttttacctgagctcaagtgatcctcctgccttagcctcccaaagtgctgcgattacaggcattagacactgcacccactctaatttgttttgttttgttttgtttcgttttgagatggagtctcactctgtcacctaggctggagtgcagtggagtgatctcagctcaatgcaaactccacctcctgggttcaagtgtttcttgttcctcagtctcccaagtagctgggattacaagtgcgtgccaccatgcccagctaatttttgtagttttagtagagatgaggtttcaccatattggccaggctaatctcgaactcctgacctcaagccatccgcctgccttggcctcccaaagtgctgggattacaggcgtgagccattgcacccagccatgtttttaagagaatgggtcttgctaccttgcccgggctggaatgcagtggttattcataggcgttataacacactctagtttctaactcctggcctcaagcaatcctcctgcctcagcctcctcagaacctgggactatagccttgcaccactgcactcggcttaacattttagcattaatgttgccatacagttttttgaaccctttcccaaaagccaacatcactgcctccctagctaaattcagtctgttctgtcacgtagaaaaataacagtaacatatctttttacctgaagggtcaaaccactctaactggcataggaaacatcctttatttttcatgattatgcaacttctttacatgagatgttggcattttgttcctagcatgtaacagaatcagtgatttaagatatcagattctgagttgtgagatttaaaagcataaaagttgaattgccttgcagcatttctcaagtgagaaatacaaaaatgatgttcacagcagacccaaattggggtcattcagcactagctgagacttgtttgcataatttcctttcctacccaattcattcaggctcctatgtagcttatacaggggtgggaatatgactcaaagtgcaaaaataaaatatttcacccagataaggaaggagcaagcttctgctatgtggcctaattgcaggcctcagaatgccagcaccttttctaagtttttgttttaaaatggaatgtaaaaactacataattaatattccaagcagcttaagctcattagttgggagtttaaattccaattccataaccatcctactgtcataactactgtaaaaaaatcattaaaaataaagtaacaaatgttatcatagatgtgaaattacttaaagtactaaatttctagtgttgtaaatagcagctaagttatatcacttcctgactgccaaattaagactaaatagaaagaatgtatatacaccattatatttaaaagtaaaaaacaacgaaactttttcatatccaagtatgtctgagactgtttacttccaacagccaagaatgataaatttcaaaaaccaaaaagttatattttgcgtgctgtaagtttcttttcaggagaaaacaattctttgcatgcatacctccctacttaacggcattaagaactttatctaacatctggtaaaacactcctatttggctcatttaataacaccattaaaaaagcataaaattgaactgtcatctaacaactatagcacaaagaagttattctgggtacctataccactaacattaagcccatttatttttatggatgcagccatttttccctcatgaatactcactgagggtcacactggcactgcatcttttgttgcatctttggtgaaatatgccagccctacatttgcattaatgaggagaccaatggcatcctagccagtactctgtcacgtcatctatggcctctttcattctcttcttatttcaggcatcctggtatgctcagtatatttaaagatggttcagaaggcaaaaactctttgtcagtaaaacagatcatgtcccagggttgcattttttaaaatgaaacaaagattagtccaaagaacaagtactgtcacttgttagggtttcttcttctaaaggtaataaggagcttcaaaacatattatttcttgactagagccctactggaaatcaatgaaaattcctcaaccagcaaactgctcaagttgacttgtttaaagttcaataagcaaatactcaacaggtaagggtacagcctgacttcaatcacaacattaagtcttcctaaagagaaggggcagaaaacatctacttaagctttctgttcaaatagctacataaggactcttgattgttctttcttgctttttataatcataactttgctcagaacagaaaactttactttgtcaacacataagccaggcatctaagaacaacctagggggagaacgcaaagttactcattttcaacaactattatatatttaatcacaaattcattagaaagatagtattcatccaattagtcttttcattattgctggttttgaaaatggccaacaatattcattaggtactgtgccattaacattgcattcaaaaaaagagaacatgggaaaccaaatccttgctctcctactctgctgatatgctctggtattggccagagtatggtagtacaaaaagagtcttgttgttatataaaaagcaataaacacatcaatagaataatgttcatgggcagccaagatgaagaagattccaaagaggttgagaacccaggataaagtgtgcaagaaattccagcttcttggtgtatattcggtgacaaagaaattcagcatagttaggacgactgtgtggccactaaacatgtaatctccacatgtgtgaacgccagtcagggtcataccaaagccactccaaatggcaaaggctcgatgtaatttctcccatacactgccatatatctttccagtacactgcaggtgttgtcctggcacggagagggaggtcacaaacatggtaaagcagcgaagcaagaatacagttcccatcagactacagagccttcgcagaagtattgacctgtgcttgtgaagaagaagaaccaggagccaaatatagcacagaatcatgccacatacttccgtcatggcaaaggcccatgggattctaggaacgctgtctaagaatatatctgggagtggtggataggtctgcatgtcaggcactcgctcatggactataaccataatgaaagatgtaaatccaaatactataaaaacatatatacaactcagtatagtcttccagtattctgggtccaatcttcgaacagaatgtttgtttttaccattcatgtactggtactgatcagaattcaagtcagttatgggtccgtcacagtcatgggaaagctccccattacagagccagtctgtactctgaagagcactgatgaaaggggtcatggaacccatgggactgtcactgttgtagcccatctcttctaaaacatcaatatgtattttctgcaattttcggactgagagcattaaccttttaatgtcccctaagactttgatttccagaggaggagaccggagatcatattcagtcaatgttagcaatgtgattccatcaagtcggtgcttattgcataaaatgtccacatattcaaaaaagccttcatccttcagccacacagctacatgcttggtagtccagcggcgaatgcagagttgattaggacctgccatttcctcctccgctgcctgggcgcggtggagtgtgcctgtagtcccagctactctgaggctgagtagctactctgaggctgagtagctactctcaggctgaggctggagagtcgcttgagccctggaggcagaggttgcagtgagccgagatcatgccactgtactccaacctgggagacagtgagac

SEQ ID NO: 12731 - RNA, 4033 nt, Homo sapiens
  source 1..4033: mol_type = other RNA
gatctcactttgttgcccaggctggtctcttttacctgagctcaagtgatcctcctgccttagcctcccaaagtgctgcgattacaggcattagacactgcacccactctaatttgttttgttttgttttgtttcgttttgagatggagtctcactctgtcacctaggctggagtgcagtggagtgatctcagctcaatgcaaactccacctcctgggttcaagtgtttcttgttcctcagtctcccaagtagctgggattacaagtgcgtgccaccatgcccagctaatttttgtagttttagtagagatgaggtttcaccatattggccaggctaatctcgaactcctgacctcaagccatccgcctgccttggcctcccaaagtgctgggattacaggcgtgagccattgcacccagccatgtttttaagagaatgggtcttgctaccttgcccgggctggaatgcagtggttattcataggcgttataacacactctagtttctaactcctggcctcaagcaatcctcctgcctcagcctcctcagaacctgggactatagccttgcaccactgcactcggcttaacattttagcattaatgttgccatacagttttttgaaccctttcccaaaagccaacatcactgcctccctagctaaattcagtctgttctgtcacgtagaaaaataacagtaacatatctttttacctgaagggtcaaaccactctaactggcataggaaacatcctttatttttcatgattatgcaacttctttacatgagatgttggcattttgttcctagcatgtaacagaatcagtgatttaagatatcagattctgagttgtgagatttaaaagcataaaagttgaattgccttgcagcatttctcaagtgagaaatacaaaaatgatgttcacagcagacccaaattggggtcattcagcactagctgagacttgtttgcataatttcctttcctacccaattcattcaggctcctatgtagcttatacaggggtgggaatatgactcaaagtgcaaaaataaaatatttcacccagataaggaaggagcaagcttctgctatgtggcctaattgcaggcctcagaatgccagcaccttttctaagtttttgttttaaaatggaatgtaaaaactacataattaatattccaagcagcttaagctcattagttgggagtttaaattccaattccataaccatcctactgtcataactactgtaaaaaaatcattaaaaataaagtaacaaatgttatcatagatgtgaaattacttaaagtactaaatttctagtgttgtaaatagcagctaagttatatcacttcctgactgccaaattaagactaaatagaaagaatgtatatacaccattatatttaaaagtaaaaaacaacgaaactttttcatatccaagtatgtctgagactgtttacttccaacagccaagaatgataaatttcaaaaaccaaaaagttatattttgcgtgctgtaagtttcttttcaggagaaaacaattctttgcatgcatacctccctacttaacggcattaagaactttatctaacatctggtaaaacactcctatttggctcatttaataacaccattaaaaaagcataaaattgaactgtcatctaacaactatagcacaaagaagttattctgggtacctataccactaacattaagcccatttatttttatggatgcagccatttttccctcatgaatactcactgagggtcacactggcactgcatcttttgttgcatctttggtgaaatatgccagccctacatttgcattaatgaggagaccaatggcatcctagccagtactctgtcacgtcatctatggcctctttcattctcttcttatttcaggcatcctggtatgctcagtatatttaaagatggttcagaaggcaaaaactctttgtcagtaaaacagatcatgtcccagggttgcattttttaaaatgaaacaaagattagtccaaagaacaagtactgtcacttgttagggtttcttcttctaaaggtaataaggagcttcaaaacatattatttcttgactagagccctactggaaatcaatgaaaattcctcaaccagcaaactgctcaagttgacttgtttaaagttcaataagcaaatactcaacaggtaagggtacagcctgacttcaatcacaacattaagtcttcctaaagagaaggggcagaaaacatctacttaagctttctgttcaaatagctacataaggactcttgattgttctttcttgctttttataatcataactttgctcagaacagaaaactttactttgtcaacacataagccaggcatctaagaacaacctagggggagaacgcaaagttactcattttcaacaactattatatatttaatcacaaattcattagaaagatagtattcatccaattagtcttttcattattgctggttttgaaaatggccaacaatattcattaggtactgtgccattaacattgcattcaaaaaaagagaacatgggaaaccaaatccttgctctcctactctgctgatatgctctggtattggccagagtatggtagtacaaaaagagtcttgttgttatataaaaagcaataaacacatcaatagaataatgttcatgggcagccaagatgaagaagattccaaagaggttgagaacccaggataaagtgtgcaagaaattccagcttcttggtgtatctaggaaaaggacagaaagatcattttaaagctacattccttccaatgcttctcagtcacgtttctcaggtcaggctgttttgccattcttcacaggatctgacacccttcccacagccttcactgcagctagttacctaatacgcatagaagcactaaaaagatacttacattcggtgacaaagaaattcagcatagttaggacgactgtgtggccactaaacatgtaatctccacatgtgtgaacgccagtcagggtcataccaaagccactccaaatggcaaaggctcgatgtaatttctcccatacactgccatatatctttccagtacactgcaggtgttgtcctggcacggagagggaggtcacaaacatggtaaagcagcgaagcaagaatacagttcccatcagactacagagccttcgcagaagtattgacctgtgcttgtgaagaagaagaaccaggagccaaatatagcacagaatcatgccacatacttccgtcatggcaaaggcccatgggattctaggaacgctgtctaagaatatatctgggagtggtggataggtctgcatgtcaggcactcgctcatggactataaccataatgaaagatgtaaatccaaatactataaaaacatatatacaactcagtatagtcttccagtattctgggtccaatcttcgaacagaatgtttgtttttaccattcatgtactggtactgatcagaattcaagtcagttatgggtccgtcacagtcatgggaaagctccccattacagagccagtctgtactctgaagagcactgatgaaaggggtcatggaacccatgggactgtcactgttgtagcccatctcttctaaaacatcaatatgtattttctgcaattttcggactgagagcattaaccttttaatgtcccctaagactttgatttccagaggaggagaccggagatcatattcagtcaatgttagcaatgtgattccatcaagtcggtgcttattgcataaaatgtccacatattcaaaaaagccttcatccttcagccacacagctacatgcttggtagtccagcggcgaatgcagagttgattaggacctgccatttcctcctccgctgcccttggcagcaggcgccccccaagctcccctctcctcagcctcagctcccgctcacctccgcggtccgagtcgggctccccggacccacctccgagtcggcgtccgagccgccgtcggagtcc

SEQ ID NO: 12732 - RNA, 6838 nt, Homo sapiens
  source 1..6838: mol_type = other RNA
gatctcactttgttgcccaggctggtctggaacccctgcctcaaatgatctgcctgcctaggcttccaaaattatgggactacaggcatgagcagtgaccaagttttaatttttaaaagttaattatctagaatgtaaacttagtgaaggctggaaatgtacaattattttcttaatccaaaatactttattatgggtaatactcatttaatatttattggtaatcactgagagccaaggtaaagtgatgatccaaatgaattgaatgtcatgatttaaataggcaattctcaaattagggggtttgggtagaaaaataatatcaaaaagttcttgtagttaaaaaaaaatcaatatgcttaacatgcctatttattttcttaaactacagaaagcaaatctcacatgctttgcttgtaagaatatgcaaaaaaagtaaatgctgtattaactgaaaaactctaagtactatattttaatttcgtgaatgatatgggtgatgtcatatagactgctattttcagtacattataaaattaccaaaatgttcaattttctacctttaaaaagtaggaaaatatccacttggcaaccaaccatcaaattaataactgattcaagtaagaattatcaacaatactaaaagtagcagatgcaagttggaagagaaacagcctatatgcagtatctgcccacaaattacttattatttccaaaaggaaaaacaggagtgttacactgaagaaactactttgtattggtgcatgcaaagaggtgaacatactgatgttgacagccagagtctttccatgtaattgcttaaagcaaaaattatcacatggttttgaaggttagctacataagcagaggtaatgcacatgtcaactatagcatgaaggatgagaagaggacagatggacctatatagttgcaaggtttctacattttaagttaagtggtacaatattaactctaagtggattgttaaaggacttattttgtcaaaattgataaaaaagcaagacccaattctatttgtttacaagtcatgaattttacatataaacataacaggttaaaagtaaactgatagaaaaagatatatcaggccaacagaaaacataataaggactaagtggctatgttattatcaaataaaatagacctcaagataaagattaccaaacataaaaagacatttcttaataagtaaatgtaacatctaatagcaaagttttgactagttttgttactaaagtttgaatggaacacagccatgactaatcatttatgtattgtctatggctgcttctgtgctgcaatagcagggttgagttgttgtgacagaaactatgttccagaaagcctaaaatatttactatctgcccctttacagaaaatgtttgctaaatcttgcaaaggattaagtcacaaacaggacacatggctggtacgatggtatatatgccaaaagcaaagttgtaaatatagttcataactatttgaaggcaggaaaagaatcaaattacagtaagactttgagttttaggaaatataacttgataagtacctgtaacatatgaatgaatgaccaaaggtagaagtagaaattcaaacatattttcatttaactgacagtgctaactcatgacagaatctctttttattcttaagtaactagtccttataatatataagtaaatagacccaaatggacactgacctgataatttcctaagacacagcatacagtttcattctttttttcctgacattaaattaatgaacaatttaatataaactttaaccaaccaaattttatgagatgtgtctatttgttcaagtggcaagtgtaaatagtaacggaactgtgttaatgtatactttggagacaaactctccccagcaaaattttaagaggatgcgagtaatcctaatataatgatgcacttcctaagttttgttttttccattaggaaatggacatgcatacacacatacaaaaccctgactatggtggtggttcaaatttgattaaatttttttttttagaaaaaaaatatttacacacacttttgcttttttaatatgaggtacacagtccaacaagaaaaaaaaagtaactgatatagtaaaggcactcagaaaaacaacagaaacaatatgaaaggtgttacaagagacagaaagagatgaaggatgatgattagtactcaccttcttcaaagctgcagtacggactttcttctttagggagagaagattagaaataaacaggttaaaattacattaagaaagggctactacatatatataatggggtaattatttatatagatctttaagaaaaggcaaattgagttctttaaacacatacttgtgagaatgggacagatctgcattatctaacaggatggttatcaaaattaaatttaataaaatcaaaaatttagttttttcagttgcaaaggccaaatttcaagtgctcaatggccacttttagccactggctatgggactggacatcatagaacactgtcattatcacagaaaattgtatagggtagcactaggctaggctgtctcaagatgtctaaattggaaagataaattgattttccctagaatttttggttcattcattcatttctttctttaacgttttgtctcttttattttatagacccttttattcttcagtcttatctatccacttaaactttttcatatttggttgaaaatgcatgcaatttcaaaagagaaacagaatgtatctcctctatagaacaaatagtaatttaaaatgttttactctgcataatattttttaaaaaatttccagaactgtacaaatctaaattcacttaaatcaaacagacatatggtgaagaaaacaccaagtaaaattaatgactgtattggtatagcaataaaatcaatcaaaatattgatgtaaaaacgtttcttacagagtagttagaggatatgattcaaatgaaaagtacagaaggacccttgtattttaaaaaaaataaagatatttaacctatgctttaaaattaaatgaaccaattaaaaactattaggacaacaaattaaatacaattcatatcagaattaacagtaaataatatttttctgaatatgcagcaagagtagaatccaaattatccttatgtaaatcataagaaacttataattaattatagatgatctggaccactatgcaacatttgaaaaaagagaaaaaaacactaaatataccttacaaataattctacaagttcttagattttttatgagacagctattgtgttaaatgtaatcatttaaatgtaatagtttaacacaatgacagttttctaatttttatacattttattaccattgcatttttttcaaatttagaaattatgctacagcagtataaaaattattttaaattcactaatattttcttttgtgcttcttcagagacaaacttctctagcagtaaaatcataccttctctctttttactttactttttacttttactctctctatatttttattttgtaatctttaggactgttataccaagaaagtttggtcttaagatctaaataatcacaaatgagaataaataagacaggcaaaacagaatagaaagcaactaagaaaaaggaaagaaccttagaaaaatgataatggaggttaaaaatgattttctaatgtaagaaccaaagaaaaccttaagccataaaagccagaaacaaaaagtaaaacttagaaaattaaatttctattcaaactatcaaataaaaaacatgcaacagatcagggtctttactaaattagataataacttcttattgttacgaagtcacaaattaactcccctacccaccccccctccaatagataaatacatcaaaaatatcatgagattacaaattccaaaatgccataatgtctatatactgagattcacagtttctggatttatttttccaccacttaaactgtggatcattgctatcatgtgggagtgtttgttcaattcctcttgctgaagtttcaccaaggactctttctcttccaaacgaccttctaattgtgccttttgaacctctagggaggaagccttaatgctcaactcttttcttatctgttctgttctgcttaattcttttctaaggatatcaatggtttcttccttatcttccctttccttttgtaaggttttaatcttttcttcttgtacttttgttttttgatgcaaatttgctagcttatgttctctgtctactagctgattctgtacttcttttctctgttcttctttctctattaattgggcaatacttttttcattttgttccttgagtgactcattcaactttttcactgtctcaatttgtttattcagagaatcacatgtgatctgtaaatctttattcttcttttcagtactttcatttctctgaagaagttccatgtaggattttgtcagtatttcatgttcttcagccacagactctaacttcctattatgttgaaagagatgctcaatatcactctgcgctctttctgattcaacttgctgcgccttcagcaacacactaagctcttcattttttctctcaacttctctcaacatactagcaagtgtccgtgcctctgtttcagcttgagttctttgacagcgatgctgagcaatcagtctatcagcctgtgcaagggctagagcttttgtttccaaaagatcttgtagcctgctttctttggaagctaatgtggatagtttcatttcatatacatccattatgtcagatattctcacatcacaaatctgatcctttaccaccattccagactgaagtttctctattaattcttcaatattcaatccaggaacaccatctttcaaatgaggagttaaacactttattgatgttggaaaactgtgatttgatgattgccagggcatttttctgggtatatgttctgtttcctgttgtctataggcattgtttgctgctatactttctccaagtactaaagcaggaaaatctggcagtggagcagcctccaataatattctcagtccagactgtacttgttctctattatctgacgttaaagcaaaagccaaaggagtaatcaaacgtgggtcctgaagtattttgtagaagcttacttccataccaggaaccaatggtttaagtttgttaatcaaatcaagagttttcaaaattacatcagcagcaagtttgcataattcagaatctgcaacctttgttccaaatcccaggtcaatcttgccatatgtaaattgttgttctataagagtggtacacttgacagttgtcaagatttttgcaatatgcatttttagtgtatcatctccacagagagttaacaaaacttcaatggccttggcaatcctttcacatttttttcttgttaaagcctcatctagattttgttctgtgaactgaagttgatcaaggattgtaggcagcagaagggtcacaaaacgatcagccgaggaacagttagcagcatctatgacatcctcaaatatttccttgaacaactccaatgctaaaacagaacagttttctgatccgtccaaaggttggcttaaccagcgcagtagagccacagtaggttctaaacatttagtatggcttcccagagtggcgctgccaggtggagactgttcaaacatcatctgagtgagcatatggcgcagctgagtcactgaacagaaggcaagaagtaattctaaaacctttgaagaggaatcaggatcctttccattaagaagacctaatacttggtgaagacatgaagaaaagtgctcatatctggtgagataatcagcaattttaggattcttaaggagatccatcagtaggtcaactgaatactttctagttagagtgccatcaccgtttatgagaatattaaatattagttgaaaagtctgatgaatgtttcgagcatggaatagcttttcccccacctcttcatttaatgtcaaactggataatattgaaagtgcaaacacaaccacagttaaactactatgggccaacaaggtgataagagttcgataaaaagatttcacattactcaatgtctttatgtgcgtttgaacagaaagattgtgccgacaaagatttgccaataatcctagacaaggcatttttaactcatcttcagaagattgaatgtgatctatcaggaacgtaattaattcatctatattggcaccagaatagaaaattttgacattatatgttaacttctgtagaagttgaatgcactgcaaaaacaccgaatcagtgtggctgctccgacaaaccactcccgccagcacactattcagattatatgtattctgaagacaatctctggtttcaatgtctactgctagttgagacagcaaaccgataatacttaagatcagtgaagcacttatgttggggtcttcaagtagctctacaaggcaactcaagcattcacttgttaatatctgatttgatgtaaatagtcgtgtgagtttctgtccagaaattactttgagggaggagaatgaaaaatgaagcccagagggtagttatgggattattccttctgcttcttcccaaagacaataggtgagctccaagtgccgcaaaagctgagtggcgttcgcctctgacttcacggctttgtactgactgacagtcaggagcaaggacttcaagcaggcagtggagtccattgcaccggccgcggcccggcttagggaccaccaccgcccagcgtgcgccggcctttagctttcgccgcgctttttttgatt

SEQ ID NO: 12733 - RNA, 6686 nt, Homo sapiens
  source 1..6686: mol_type = other RNA
gatctcactttgttgcccaggctggtctggaacccctgcctcaaatgatctgcctgcctaggcttccaaaattatgggactacaggcatgagcagtgaccaagttttaatttttaaaagttaattatctagaatgtaaacttagtgaaggctggaaatgtacaattattttcttaatccaaaatactttattatgggtaatactcatttaatatttattggtaatcactgagagccaaggtaaagtgatgatccaaatgaattgaatgtcatgatttaaataggcaattctcaaattagggggtttgggtagaaaaataatatcaaaaagttcttgtagttaaaaaaaaatcaatatgcttaacatgcctatttattttcttaaactacagaaagcaaatctcacatgctttgcttgtaagaatatgcaaaaaaagtaaatgctgtattaactgaaaaactctaagtactatattttaatttcgtgaatgatatgggtgatgtcatatagactgctattttcagtacattataaaattaccaaaatgttcaattttctacctttaaaaagtaggaaaatatccacttggcaaccaaccatcaaattaataactgattcaagtaagaattatcaacaatactaaaagtagcagatgcaagttggaagagaaacagcctatatgcagtatctgcccacaaattacttattatttccaaaaggaaaaacaggagtgttacactgaagaaactactttgtattggtgcatgcaaagaggtgaacatactgatgttgacagccagagtctttccatgtaattgcttaaagcaaaaattatcacatggttttgaaggttagctacataagcagaggtaatgcacatgtcaactatagcatgaaggatgagaagaggacagatggacctatatagttgcaaggtttctacattttaagttaagtggtacaatattaactctaagtggattgttaaaggacttattttgtcaaaattgataaaaaagcaagacccaattctatttgtttacaagtcatgaattttacatataaacataacaggttaaaagtaaactgatagaaaaagatatatcaggccaacagaaaacataataaggactaagtggctatgttattatcaaataaaatagacctcaagataaagattaccaaacataaaaagacatttcttaataagtaaatgtaacatctaatagcaaagttttgactagttttgttactaaagtttgaatggaacacagccatgactaatcatttatgtattgtctatggctgcttctgtgctgcaatagcagggttgagttgttgtgacagaaactatgttccagaaagcctaaaatatttactatctgcccctttacagaaaatgtttgctaaatcttgcaaaggattaagtcacaaacaggacacatggctggtacgatggtatatatgccaaaagcaaagttgtaaatatagttcataactatttgaaggcaggaaaagaatcaaattacagtaagactttgagttttaggaaatataacttgataagtacctgtaacatatgaatgaatgaccaaaggtagaagtagaaattcaaacatattttcatttaactgacagtgctaactcatgacagaatctctttttattcttaagtaactagtccttataatatataagtaaatagacccaaatggacactgacctgataatttcctaagacacagcatacagtttcattctttttttcctgacattaaattaatgaacaatttaatataaactttaaccaaccaaattttatgagatgtgtctatttgttcaagtggcaagtgtaaatagtaacggaactgtgttaatgtatactttggagacaaactctccccagcaaaattttaagaggatgcgagtaatcctaatataatgatgcacttcctaagttttgttttttccattaggaaatggacatgcatacacacatacaaaaccctgactatggtggtggttcaaatttgattaaatttttttttttagaaaaaaaatatttacacacacttttgcttttttaatatgaggtacacagtccaacaagaaaaaaaaagtaactgatatagtaaaggcactcagaaaaacaacagaaacaatatgaaaggtgttacaagagacagaaagagatgaaggatgatgattagtactcaccttcttcaaagctgcagtacggactttcttctttagggagagaagattagaaataaacaggttaaaattacattaagaaagggctactacatatatataatggggtaattatttatatagatctttaagaaaaggcaaattgagttctttaaacacatacttgtgagaatgggacagatctgcattatctaacaggatggttatcaaaattaaatttaataaaatcaaaaatttagttttttcagttgcaaaggccaaatttcaagtgctcaatggccacttttagccactggctatgggactggacatcatagaacactgtcattatcacagaaaattgtatagggtagcactaggctaggctgtctcaagatgtctaaattggaaagataaattgattttccctagaatttttggttcattcattcatttctttctttaacgttttgtctcttttattttatagacccttttattcttcagtcttatctatccacttaaactttttcatatttggttgaaaatgcatgcaatttcaaaagagaaacagaatgtatctcctctatagaacaaatagtaatttaaaatgttttactctgcataatattttttaaaaaatttccagaactgtacaaatctaaattcacttaaatcaaacagacatatggtgaagaaaacaccaagtaaaattaatgactgtattggtatagcaataaaatcaatcaaaatattgatgtaaaaacgtttcttacagagtagttagaggatatgattcaaatgaaaagtacagaaggacccttgtattttaaaaaaaataaagatatttaacctatgctttaaaattaaatgaaccaattaaaaactattaggacaacaaattaaatacaattcatatcagaattaacagtaaataatatttttctgaatatgcagcaagagtagaatccaaattatccttatgtaaatcataagaaacttataattaattatagatgatctggaccactatgcaacatttgaaaaaagagaaaaaaacactaaatataccttacaaataattctacaagttcttagattttttatgagacagctattgtgttaaatgtaatcatttaaatgtaatagtttaacacaatgacagttttctaatttttatacattttattaccattgcatttttttcaaatttagaaattatgctacagcagtataaaaattattttaaattcactaatattttcttttgtgcttcttcagagacaaacttctctagcagtaaaatcataccttctctctttttactttactttttacttttactctctctatatttttattttgtaatctttaggactgttataccaagaaagtttggtcttaagatctaaataatcacaaatgagaataaataagacaggcaaaacagaatagaaagcaactaagaaaaaggaaagaaccttagaaaaatgataatggaggttaaaaatgattttctaatgtaagaaccaaagaaaaccttaagccataaaagccagaaacaaaaagtaaaacttagaaaattaaatttctattcaaactatcaaataaaaaacatgcaacagatcagggtctttactaaattagataataacttcttattgttacgaagtcacaaattaactcccctacccaccccccctccaatagataaatacatcaaaaatatcatgagattacaaattccaaaatgccataatgtctatatactgagattcacagtttctggatttatttttccaccacttaaactgtggatcattgctatcatgtgggagtgtttgttcaattcctcttgctgaagtttcaccaaggactctttctcttccaaacgaccttctaattgtgccttttgaacctctagggaggaagccttaatgctcaactcttttcttatctgttctgttctgcttaattcttttctaaggatatcaatggtttcttccttatcttccctttccttttgtaaggttttaatcttttcttcttgtacttttgttttttgatgcaaatttgctagcttatgttctctgtctactagctgattctgtacttcttttctctgttcttctttctctattaattgggcaatacttttttcattttgttccttgagtgactcattcaactttttcactgtctcaatttgtttattcagagaatcacatgtgatctgtaaatctttattcttcttttcagtactttcatttctctgaagaagttccatgtaggattttgtcagtatttcatgttcttcagccacagactctaacttcctattatgttgaaagagatgctcaatatcactctgcgctctttctgattcaacttgctgcgccttcagcaacacactaagctcttcattttttctctcaacttctctcaacatactagcaagtgtccgtgcctctgtttcagcttgagttctttgacagcgatgctgagcaatcagtctatcagcctgtgcaagggctagagcttttgtttccaaaagatcttgtagcctgctttctttggaagctaatgtggatagtttcatttcatatacatccattatgtcagatattctcacatcacaaatctgatcctttaccaccattccagactgaagtttctctattaattcttcaatattcaatccaggaacaccatctttcaaatgaggagttaaacactttattgatgttggaaaactgtgatttgatgattgccagggcatttttctgggtatatgttctgtttcctgttgtctataggcattgtttgctgctatactttctccaagtactaaagcaggaaaatctggcagtggagcagcctccaataatattctcagtccagactgtacttgttctctattatctgacgttaaagcaaaagccaaaggagtaatcaaacgtgggtcctgaagtattttgtagaagcttacttccataccaggaaccaatggtttaagtttgttaatcaaatcaagagttttcaaaattacatcagcagcaagtttgcataattcagaatctgcaacctttgttccaaatcccaggtcaatcttgccatatgtaaattgttgttctataagagtggtacacttgacagttgtcaagatttttgcaatatgcatttttagtgtatcatctccacagagagttaacaaaacttcaatggccttggcaatcctttcacatttttttcttgttaaagcctcatctagattttgttctgtgaactgaagttgatcaaggattgtaggcagcagaagggtcacaaaacgatcagccgaggaacagttagcagcatctatgacatcctcaaatatttccttgaacaactccaatgctaaaacagaacagttttctgatccgtccaaaggttggcttaaccagcgcagtagagccacagtaggttctaaacatttagtatggcttcccagagtggcgctgccaggtggagactgttcaaacatcatctgagtgagcatatggcgcagctgagtcactgaacagaaggcaagaagtaattctaaaacctttgaagaggaatcaggatcctttccattaagaagacctaatacttggtgaagacatgaagaaaagtgctcatatctggtgagataatcagcaattttaggattcttaaggagatccatcagtaggtcaactgaatactttctagttagagtgccatcaccgtttatgagaatattaaatattagttgaaaagtctgatgaatgtttcgagcatggaatagcttttcccccacctcttcatttaatgtcaaactggataatattgaaagtgcaaacacaaccacagttaaactactatgggccaacaaggtgataagagttcgataaaaagatttcacattactcaatgtctttatgtgcgtttgaacagaaagattgtgccgacaaagatttgccaataatcctagacaaggcatttttaactcatcttcagaagattgaatgtgatctatcaggaacgtaattaattcatctgcaaaaacaccgaatcagtgtggctgctccgacaaaccactcccgccagcacactattcagattatatgtattctgaagacaatctctggtttcaatgtctactgctagttgagacagcaaaccgataatacttaagatcagtgaagcacttatgttggggtcttcaagtagctctacaaggcaactcaagcattcacttgttaatatctgatttgatgtaaatagtcgtgtgagtttctgtccagaaattacctccaagtgccgcaaaagctgagtggcgttcgcctctgacttcacggctttgtactgactgacagtcaggagcaaggacttcaagcaggcagtggagtccattgcaccggccgcggcccggcttagggaccaccaccgcccagcgtgcgccggcctttagctttcgccgcgcttttttt

SEQ ID NO: 12734 - RNA, 6807 nt, Homo sapiens
  source 1..6807: mol_type = other RNA
gatctcactttgttgcccaggctggtctggaacccctgcctcaaatgatctgcctgcctaggcttccaaaattatgggactacaggcatgagcagtgaccaagttttaatttttaaaagttaattatctagaatgtaaacttagtgaaggctggaaatgtacaattattttcttaatccaaaatactttattatgggtaatactcatttaatatttattggtaatcactgagagccaaggtaaagtgatgatccaaatgaattgaatgtcatgatttaaataggcaattctcaaattagggggtttgggtagaaaaataatatcaaaaagttcttgtagttaaaaaaaaatcaatatgcttaacatgcctatttattttcttaaactacagaaagcaaatctcacatgctttgcttgtaagaatatgcaaaaaaagtaaatgctgtattaactgaaaaactctaagtactatattttaatttcgtgaatgatatgggtgatgtcatatagactgctattttcagtacattataaaattaccaaaatgttcaattttctacctttaaaaagtaggaaaatatccacttggcaaccaaccatcaaattaataactgattcaagtaagaattatcaacaatactaaaagtagcagatgcaagttggaagagaaacagcctatatgcagtatctgcccacaaattacttattatttccaaaaggaaaaacaggagtgttacactgaagaaactactttgtattggtgcatgcaaagaggtgaacatactgatgttgacagccagagtctttccatgtaattgcttaaagcaaaaattatcacatggttttgaaggttagctacataagcagaggtaatgcacatgtcaactatagcatgaaggatgagaagaggacagatggacctatatagttgcaaggtttctacattttaagttaagtggtacaatattaactctaagtggattgttaaaggacttattttgtcaaaattgataaaaaagcaagacccaattctatttgtttacaagtcatgaattttacatataaacataacaggttaaaagtaaactgatagaaaaagatatatcaggccaacagaaaacataataaggactaagtggctatgttattatcaaataaaatagacctcaagataaagattaccaaacataaaaagacatttcttaataagtaaatgtaacatctaatagcaaagttttgactagttttgttactaaagtttgaatggaacacagccatgactaatcatttatgtattgtctatggctgcttctgtgctgcaatagcagggttgagttgttgtgacagaaactatgttccagaaagcctaaaatatttactatctgcccctttacagaaaatgtttgctaaatcttgcaaaggattaagtcacaaacaggacacatggctggtacgatggtatatatgccaaaagcaaagttgtaaatatagttcataactatttgaaggcaggaaaagaatcaaattacagtaagactttgagttttaggaaatataacttgataagtacctgtaacatatgaatgaatgaccaaaggtagaagtagaaattcaaacatattttcatttaactgacagtgctaactcatgacagaatctctttttattcttaagtaactagtccttataatatataagtaaatagacccaaatggacactgacctgataatttcctaagacacagcatacagtttcattctttttttcctgacattaaattaatgaacaatttaatataaactttaaccaaccaaattttatgagatgtgtctatttgttcaagtggcaagtgtaaatagtaacggaactgtgttaatgtatactttggagacaaactctccccagcaaaattttaagaggatgcgagtaatcctaatataatgatgcacttcctaagttttgttttttccattaggaaatggacatgcatacacacatacaaaaccctgactatggtggtggttcaaatttgattaaatttttttttttagaaaaaaaatatttacacacacttttgcttttttaatatgaggtacacagtccaacaagaaaaaaaaagtaactgatatagtaaaggcactcagaaaaacaacagaaacaatatgaaaggtgttacaagagacagaaagagatgaaggatgatgattagtactcaccttcttcaaagctgcagtacggactttcttctttagggagagaagattagaaataaacaggttaaaattacattaagaaagggctactacatatatataatggggtaattatttatatagatctttaagaaaaggcaaattgagttctttaaacacatacttgtgagaatgggacagatctgcattatctaacaggatggttatcaaaattaaatttaataaaatcaaaaatttagttttttcagttgcaaaggccaaatttcaagtgctcaatggccacttttagccactggctatgggactggacatcatagaacactgtcattatcacagaaaattgtatagggtagcactaggctaggctgtctcaagatgtctaaattggaaagataaattgattttccctagaatttttggttcattcattcatttctttctttaacgttttgtctcttttattttatagacccttttattcttcagtcttatctatccacttaaactttttcatatttggttgaaaatgcatgcaatttcaaaagagaaacagaatgtatctcctctatagaacaaatagtaatttaaaatgttttactctgcataatattttttaaaaaatttccagaactgtacaaatctaaattcacttaaatcaaacagacatatggtgaagaaaacaccaagtaaaattaatgactgtattggtatagcaataaaatcaatcaaaatattgatgtaaaaacgtttcttacagagtagttagaggatatgattcaaatgaaaagtacagaaggacccttgtattttaaaaaaaataaagatatttaacctatgctttaaaattaaatgaaccaattaaaaactattaggacaacaaattaaatacaattcatatcagaattaacagtaaataatatttttctgaatatgcagcaagagtagaatccaaattatccttatgtaaatcataagaaacttataattaattatagatgatctggaccactatgcaacatttgaaaaaagagaaaaaaacactaaatataccttacaaataattctacaagttcttagattttttatgagacagctattgtgttaaatgtaatcatttaaatgtaatagtttaacacaatgacagttttctaatttttatacattttattaccattgcatttttttcaaatttagaaattatgctacagcagtataaaaattattttaaattcactaatattttcttttgtgcttcttcagagacaaacttctctagcagtaaaatcataccttctctctttttactttactttttacttttactctctctatatttttattttgtaatctttaggactgttataccaagaaagtttggtcttaagatctaaataatcacaaatgagaataaataagacaggcaaaacagaatagaaagcaactaagaaaaaggaaagaaccttagaaaaatgataatggaggttaaaaatgattttctaatgtaagaaccaaagaaaaccttaagccataaaagccagaaacaaaaagtaaaacttagaaaattaaatttctattcaaactatcaaataaaaaacatgcaacagatcagggtctttactaaattagataataacttcttattgttacgaagtcacaaattaactcccctacccaccccccctccaatagataaatacatcaaaaatatcatgagattacaaattccaaaatgccataatgtctatatactgagattcacagtttctggatttatttttccaccacttaaactgtggatcattgctatcatgtgggagtgtttgttcaattcctcttgctgaagtttcaccaaggactctttctcttccaaacgaccttctaattgtgccttttgaacctctagggaggaagccttaatgctcaactcttttcttatctgttctgttctgcttaattcttttctaaggatatcaatggtttcttccttatcttccctttccttttgtaaggttttaatcttttcttcttgtacttttgttttttgatgcaaatttgctagcttatgttctctgtctactagctgattctgtacttcttttctctgttcttctttctctattaattgggcaatacttttttcattttgttccttgagtgactcattcaactttttcactgtctcaatttgtttattcagagaatcacatgtgatctgtaaatctttattcttcttttcagtactttcatttctctgaagaagttccatgtaggattttgtcagtatttcatgttcttcagccacagactctaacttcctattatgttgaaagagatgctcaatatcactctgcgctctttctgattcaacttgctgcgccttcagcaacacactaagctcttcattttttctctcaacttctctcaacatactagcaagtgtccgtgcctctgtttcagcttgagttctttgacagcgatgctgagcaatcagtctatcagcctgtgcaagggctagagcttttgtttccaaaagatcttgtagcctgctttctttggaagctaatgtggatagtttcatttcatatacatccattatgtcagatattctcacatcacaaatctgatcctttaccaccattccagactgaagtttctctattaattcttcaatattcaatccaggaacaccatctttcaaatgaggagttaaacactttattgatgttggaaaactgtgatttgatgattgccagggcatttttctgggtatatgttctgtttcctgttgtctataggcattgtttgctgctatactttctccaagtactaaagcaggaaaatctggcagtggagcagcctccaataatattctcagtccagactgtacttgttctctattatctgacgttaaagcaaaagccaaaggagtaatcaaacgtgggtcctgaagtattttgtagaagcttacttccataccaggaaccaatggtttaagtttgttaatcaaatcaagagttttcaaaattacatcagcagcaagtttgcataattcagaatctgcaacctttgttccaaatcccaggtcaatcttgccatatgtaaattgttgttctataagagtggtacacttgacagttgtcaagatttttgcaatatgcatttttagtgtatcatctccacagagagttaacaaaacttcaatggccttggcaatcctttcacatttttttcttgttaaagcctcatctagattttgttctgtgaactgaagttgatcaaggattgtaggcagcagaagggtcacaaaacgatcagccgaggaacagttagcagcatctatgacatcctcaaatatttccttgaacaactccaatgctaaaacagaacagttttctgatccgtccaaaggttggcttaaccagcgcagtagagccacagtaggttctaaacatttagtatggcttcccagagtggcgctgccaggtggagactgttcaaacatcatctgagtgagcatatggcgcagctgagtcactttgaagaggaatcaggatcctttccattaagaagacctaatacttggtgaagacatgaagaaaagtgctcatatctggtgagataatcagcaattttaggattcttaaggagatccatcagtaggtcaactgaatactttctagttagagtgccatcaccgtttatgagaatattaaatattagttgaaaagtctgatgaatgtttcgagcatggaatagcttttcccccacctcttcatttaatgtcaaactggataatattgaaagtgcaaacacaaccacagttaaactactatgggccaacaaggtgataagagttcgataaaaagatttcacattactcaatgtctttatgtgcgtttgaacagaaagattgtgccgacaaagatttgccaataatcctagacaaggcatttttaactcatcttcagaagattgaatgtgatctatcaggaacgtaattaattcatctatattggcaccagaatagaaaattttgacattatatgttaacttctgtagaagttgaatgcactgcaaaaacaccgaatcagtgtggctgctccgacaaaccactcccgccagcacactattcagattatatgtattctgaagacaatctctggtttcaatgtctactgctagttgagacagcaaaccgataatacttaagatcagtgaagcacttatgttggggtcttcaagtagctctacaaggcaactcaagcattcacttgttaatatctgatttgatgtaaatagtcgtgtgagtttctgtccagaaattactttgagggaggagaatgaaaaatgaagcccagagggtagttatgggattattccttctgcttcttcccaaagacaataggtgagctccaagtgccgcaaaagctgagtggcgttcgcctctgacttcacggctttgtactgactgacagtcaggagcaaggacttcaagcaggcagtggagtccattgcaccggccgcggcccggcttagggaccaccaccgcccagcgtgcgccggcctttagctttcgccgcgctttttttgatt

SEQ ID NO: 12735 - RNA, 12095 nt, Homo sapiens
  source 1..12095: mol_type = other RNA
gatctcactttgttgcccaggctggtcttaaactcctggcctcaagtgatccccttgtttcagccccgcaaagtgctgggattacaggtgtgagccaccatgcccgtgcccagccacctcatgagtcttgatggggggcagagaccaacaactccacagaagccagatgcttgctttcccagcctctcttgcagctagggcttgggcatgtgatccaggctcagccaatcagatggcactgactcttggcatgacatgggctaaggaggggctgcagggaatccatttgggctggggtggcagctgcactgggagcgacatcagtttccagagggagcagcagaatctggcatcaggcttggggcgtggtaggtgcaaccagactctgcacccagcagcagtggcagaatgggttctctgtggagagtctgtgtattgctccttccgctgaggccaccagcatctgcctccatgaacccctcagagcctgtgagcaactcaacagccttgaattttttcccttcctgtttgaatgagccagggttgtttcactgcttgaactaagagccgttcctgacatgaaaactaagccacatctttttgacccaaagattctggcatcctaaaatacccatctcattttaagttaaaaataaatccatgtttgagcatctactgtttcagttactgtgctaggtgttacaaagctaactaagagtgacaagtaaataactatcatcaccatgataaacagagaatggaaccctggtttttggaatacagacacaaaatgattaattctgcctggaagcgttttggaacatttcagagaggtagtgagctgggccaagagaagagcatacgcaaggaatggtggcatgaagttgcctggtgtgtcctgagaagaaagatgggctaagaaggactggggtagggcagagaagggggtcactggaggtgaggctgggaaagtgagccaaggctcaaatgcaaactgtctgaacttcattttctgtgcaagcaggagaagccgctgacatgggtttggaagatggactgaagccggagaaaaatggaagcaagaaaccctctcacaagaggccataaccacaaccaagtccatgagattgaaaaggaaggcagatatttgaaaaatatttaaagagatgtgaggggtaggacaggcacagtggctcatgcctgtagtcccagcactttgggaggccgaggtgggcagatccacgaggtcaggagatcaagaccatcctaacatggtaaaaccccatctctactaacaatacaaaaaattagtcaggtgtggtggcacgtgcctgtagtcccagctactcaggaggctgaggcaggagaatcgcttgaacctgggaggcggaggttgcagtgagccgagattgtgccactgcaccctagcctaggcaacagagcaagactctgtctcaaaaaaaataaaaaaaaaaaaaagagagaaagagagagagagatgaggagttgctgcactgctgggtgtggagagccgaggaggattcaaagatggtcctgaagtcccagctggaagaagtaggcggcagcaatgtttttaatactgtaaattcatcacgtagcacaggtttggggtggagaaagaaaaattgcattggcttcagggcatgcccagatctttcctcatcttaggcgtttgctaatacatgcattttctaagctgatgtcttgcgtttaatcactgctccattcaaaagagagaaggaggttgtttcaaacctagttgatatcatttgacttccatgctattcacagggctattttatttgaaacaggtataccacagccttaaattgcaagttaatccaggatgttcctaggttggcagttaggaacatgtaattctttggaagggctaaaagtcagctctttaaattatctccatatgaaccttctctccaccttagggtggatccacttatttagtccactgccagtaccacactagaacccgggtggtcactggactccagaaacaacagtagccctctctctgttctgtctctttttgactatctctattctgttcctgaccctgatttctcctgccaagctcaattttgacagctgacaacggcaagccatggcttcccaaaacattattttcaggtcaacttataaatttcaagaacacatttggctccgcttcctgtggtactaagcctacttcttgacagcatttgcctttgttgtaaatagcaaagttcttctagttggatttttgctaagaagtgtgtggatgtggcatgtgacgacatctttagcttggattctagaaaggcactaccattgtgcatttggctaaaggaaacacattttacccgtgaatgccttctatttacaaatgctcagctagcacacaaagctaagtacaagcaataagtactatcctacaatgttactcatttctgaaagcacaaaatgatgactggtatagctttggagatgttttctggaaacccaataaaggaacagatctttgttattccacacctacaaagtcagaagatgcacagtcttttattcatgtttgaacaagcttccttcttgaacaatcaactataaagtgatgtgattctctactagaccaggaactccttgaggacagaatgagggtctaatccatattctaaatccacaccacctggcacaatacatgttgcatggttagggtcaactaagagttggttgaattaatcaataacacacagcaagagaattcacaaagagaggggagtaatcccccagcctcaatcactcggcaagtggaatcgctgggcactgattccagctctgtctcagtgcttgagacagagctgaatgtaatgtgaacatttcaaatgaacaggaaaactagactcacggataagcagtgtagtcatcaagacaacactgtcttggaggtttttctgaagttaaaaccatgctacataagcaataaattatgaaggctgagcatgtgaataaaatttaatgttgtcataaattttataacaaagttaatctgacacatttaatgacatgcataatcattagtatgcagcactgtaatcagacattgataataagcagttcacaccagtgactgtaagagtctttacttgtgttcagccaagccaactgcttggtatatttttctcccttcttagtcgttagttttccatacctacaataactatcagtggtgatgggcttctctgaccatgtgaataatttaatcctcaatgcacagatacagaaacccttgctgaagacagtgtggagcagagaaggctgtctccactccttccacctgaaacacctctgcagatggatatgggagctctgcctacagcccttggacctaaccacttcagtgtgttccagtgagtgtctggacctcggcctgaaagatttttccgaaactaaagaaaatttctctgacctaaagaccttaacctccaccccagaagctctcaccaaggactacagggaactggtggggaaaatccttatcccttactcctcaaggcacagggcagtaatgctgaggcttgtgcgccacacttgctcccagaggtccccagcgggctacctgcggtggtgaatgacctcctaacacgccccttgacggccttcctttccttgcctcacttctccactctcctaccagcattgcagggttcacatcccaaatataccactggcacttgaatcctggtctccaggtctgtttctggaaaaacccaagtaagacattgccccagtaatggggctagatgtctgaggcttcctcaagtatctacctcgaaagctcttactgctgtacacacatgcacatacacacacgtgcgtacaaccagtcacatctaagcaccccgaataccagcctgttgaaggtagcagagagctgcactataagccaaggctgctcccaagagccgctccatcactgaattggcgccccagcaagatgaaggaatgtaatcattggaaggatggagaatgttctctgaatcactgacaaattggaaggggtggagggcaagagtccacctggtggagagatggaaagagcgagagagcctggaatgataatgccattgcttagaaaaggctgctccagatgccatatctacagaaattgtacagcccaaacatctctgagcaataggtctctggtagtcttgatgtctagaccaacaattcccagttcattcttctcagggaaggagccaggatagtccagagactctcattctgctgttagattgaaagggttaggcacaacagccttggcaaagtcacaagggcaaattcacactaaagtgtaaatgacccacaactcctcttctatttttaggttggggaggtgctttagaacataaggaggaactaaagaatattcctgttacatacaaggcagagaaaagggaaactagtggtgacaagacaaatcatccctttgacatttggctggctctacctattacagctctgggggtgaggtgggaacaaaaagatgctgtgtaaagaagtatcttatgccatccctactgtagtgaggtgcagtttagaggggacactgatcaagcagagacccagagtgtttcgttccaagccagaaacagaaatgtataaaacacagcctttccagcatcagaaatgagtagtggtagtggagaactacccaaaacaggaaagaggaccacgtgaggtagagtgtcaaggccctacattccagtgcctctgctcatgactgtaattttgggtaggtcacttaaagtctctggacctcagttttgccatctgtgaaatagggataatactatccagcataaaattggttatgaggctcatgtagggcctgcctgggatgatgtgttgctaatggttaagaacacaacttctggggtctgactggacaggctgaaatccctgcttaacacgttccagcagagccctgggcgatctatttaacttttgttttctcacctgtaagctgagacgaaagtacccactttataagattattccaataattagttgaaataatgcatgcagagaattaagcatggtacttgttatttgttaaactagctattaaaatgtgtaaaatataaagtattgtatggattttaggacaatgcaaagactctttgcttgctgcaatagttcggggccctttcagatggctaaaggcagaatttgtatgtgtaaatatggtgtgcttgtctctgctctggatactgagggcttaccctgttattaaacttatttagtaaatattgaactgtcatgaggcctaacatttagttccagttattagataaaacatttgctttgaatggtatttgaattgccaggttctagattattctggttgacaaactcttcgtattttataaagaggctaaaattggtaagctatcacagaacagatgtgccattttcaaggtatattaaaccatgattcactgtaacattgttcctactggcaacaaattcagagcaggctggactttatttggtgaagaaacattgagtggaagagaaatgacattattttatgtatttacattttcaaattactgtggcttaaacctgttcagccaacattacccaccttcagtctgctaaataaatgattcagtacatttctaatttacagaattttttaacaaaagaaaatgtaatttgatagccaaatcaacgttaaacattatacatttaaaaaaccacaggcaaagacacaaacatgatgacactaacttttgttaaagtatgcttacctatggtttcctctgaggcacgttctttcatgctaagcttccaacataatatgaaaatgaaggagatgcattttgcaaagcaaaacagaccttaagcaaaatattatacttctcaaattaacactgttacaaagttttagaatttaataagttcattaatttaaaagtttggatgtctgagtccttctatcccaaaacaagatcttggagggtcttccacagccatgtaataccatggtcacatgaccctttccaaaattattaatctgaatttactatatgaggataaatctatctttttgaaaatatttaggaaaatgagcttggtatttataaaatgaagctctctttgggtggtatcctaagacacgtcaagccaatcagcctgtaactgtgaaaaaaacattggtaggtacaaaagtggggtgggagaggagtgacttaactttgttaagtgatgggaaagaaacactaatagcattatctcaataaaatgtgatttaaaaaaatttaaaatactaaatcattgaactgacaaagaaatataaatcattcagaaataaactcattaggtcatcaaatcctgttaaatctgcaattaggaagagcaaggtgtacaatccatacatttaaactcacaggctcactttgcacaacgtcaatttactccttaatatgttattaatacgcattttccaaaaggatgtattagtaaatggtacacatctacttcttggcaacatcatataacctggtacaacataagcattcttcttatagttaagaaatgtggatggtatcaaaattagaaaaataaatgccctattatgttgtggtcaggtttaaggcatgtgaattttatcttcatacaaaagattaaaatctagatattaaaaagtagtgcagtatcagtgatgctgcctcagttcccaaaatgtcacatcacaaaaatatcccataattgcctgtagtttattccttggctttcctcttttctctctgcatctttgtaacaattttttaaaagtggaaatataattgttggcaatgctaacagctgtagaaatgattacaagatgtggaaaagcataacaggaatgtcaagaatctgtttctggcagtaatatatatggaacattgttcaggacaaaagaggagaaggaagaaaaaaaggagaggggtttatcatctctaagaattttcaaactaaacctcattgcttaataggaaaaaaagattccatatttaaagttaagtcacctctaactactagctaaagcatgacatcaccagcactggagtcagcggaagtgtgtttttgaaggacagtgttgcaggagaatctggacaggttttagagccaggagagagaaaataattctacctctgacagttgaaggaccttaggcaaatcagtttacctctgctagactacactccaaaatttggacattcaaaaatttgatattaataaccacatgaaagtctcgtgttgaggtgaatatgtatttgttggtgaaagatatgttggtttttaaacagacagcactctgcaattgtaggctattgttttgttttgccagttgtcaaattctatccagctatacacacttgtgtggcctcctaatggtgtttttccagtggctaaaggtttatgaataagacacttttcctaatggaattaacccgatgcttttcttaaacatgtaaccttgagttcaccgcaaaaaacaatgcttcgattagagcaatgcatataataaaggttaccctcgtttcttagacactagacatcattcacaaaaagagaactgcttttgaaagggatgtatttgcactggaaagaatagttttctacttctaattataaatgatttattggtgaaagcaaaacaacagcctgtctgagaggcacttctatgagcatcctcacgtgtgatttgcaaggttgaagaagagggaaaaatgcctcaattgtaccaatggtgagaaaacacccaaagtacaaagcaggtttcaaaaaaaccatactcataaccaaggacaataataaagcaatgtgttgacatatactctataagtcttcctccataaatagtttatagaaattttgtaatttctgtaaatgcatcctataataattttgcatcttgctttttttttacatttaatatcaagtagatttctaaagggcaattatttgaaaattatcccaaatacatggggaaatatacatcaagtgaaaaaatgcagtgggtgatagagatatcaggaagcgcctcaaatatttctcatctcgttggagaaaaacaaacatgttctcatttagaatgagtgggagttacctaattgatttaggcctctatatttaacttctagtcaaaaaaggtagttctatctagcaacaatattatggggaacaaaagaaaaaattaactctctaaatttgcagtagggtcttttcttcagaagtaccaaatcccatctattaccagctccatgcttcaggcctaaaatggatctccctgaagcaatgacagaatttttgccaagtgactaggatataaacaccactttggttgcacagtgagacatatgctccaaagaaaactggttcaaaaacaggcaagtgggtttctacagaataaatgagagccctgtcaatggcttcatcttcagggctttgtgtctgtgcttgcgtggtggctcttgtttcatctatggataatggtggcacacagttttcataattccttacattaatgaactgctataaatttgtttttggtattctagagagtcctaacttcagcttctgggcaatgctgaggaggcaccctatattctagacttaccttttgcaaggtgtactctcagcattgtgggcgatttccatgggagaatattctatttaaagaactactgtcccagcataaaacaaaaaatcatttatgaagatgcaggagactcggaaagctctcaattattgtttgcacaagcacaatgtcacagcctcctttccccattccacaagggggtcaggaagagagtactcagctgtgagaaaagacatacagaagaattcatgtggtcatgagagcgaggacatggccgatcccccaaggaggatgtgtcatacacttcatgagcccaagagtgtgctgtagggtctgaagggcaagatgctggttcactgatgtaaaggagagggaaaaaagcttcaaccaactagaaaaacagtctctatgcatgctatttttgattttaaacacaggtatcaattccttctctcagagagtccattttaaaataggatacatttttaaaggaatatttaaaggacacattcattaaaatttattttaaaaacttttcaaaagaaacaaaaggtatgaattttatttaatccttgaggaaatggttcttttctcacacacataaatcactcattttgtttttctttatctcctttattaatctacattagaaaaataaacttttcatacactaagaacaaggaaaccactctcaattgacaaaatgttccaatccaacacaatgattactttcacctttaatttacaggcagccagattcaaaatccttaaagttgcttaaacttaaaaatgacaatgacaacctaaaaggtataatgttgattggaacagacatttaattggaaaattgatgattttccatttccaattaaatctctagatagaaatgaaaaaaattaaaaatcgtatttaagaaaagccaaatcttgggttgtgaggtatctttttaaggatgtttcagcagaaaaaaacaaaggctctcacaattgtgtagctgcctagattaagtgggtatcctgatcaaggagatgggggatgatttggctttagtattccaatgataaagtttataatgagaataacatgttgctacaaaatccagtctcttcctcagatgccttccacagagggcaggaagctttgtcagttttgtttgctgatgatgcctggttccgtcaacaaataacacctgataggcctggatcaagcatgcagctgtggagaacacccctgggactctaactctggcactctgcaagctgggtacttgggcaggacagcagcagcactcatgaactgggcagcacctgttggtgagggctgatcacatggattctctcatcccagccttacaatcagtccttcaggtacatactttttctgactttgctgatgaggaaactatgcacagaggttacacagcttaacaaagggttctcacctaatgaacaatgaaatgggattttagcctttctttgcatctggtcttagagccaatacccaagaagcactgtactgtatgcattgtctcagagaaacttactcttcctgggcctcagtctttaaaaggtgggcagttgacttaataagaattaaagatcaatgattaaggttcaaggcactccaaaattctggtctttattgaaaaggctacagaagtctcaccttaataataccctatagacttgatattcttggttaattaaatattggaaaccaatttcatagtaattgaggtcagaaaaaagtactcatgacattttagaatatgatgacaaagccatagataaatttcaatgcacctgtaattacttaaaactgttatagcatgcaatgtgttaccacaacagccagagaaatactaatttactcagcctattcttctagaccagtaaacactaggattaaatagatattttcattgaatttgttctacccttcattgccatttatagatagcttacttgtcatagattactttctaattgttttatgtttcctaactagcctgcaatactttggcaaggacctcaaacaatagtagacagtaggtgtaaaatagatggctacattgaacagatgactaaaaggatgcctcctaagtacctatatcttgaaatatatattattgtgccttgctttcaatttgtgattttaaaatctagaaatcacctgttttatgtaataacaataaaatccttctttgttgaaaacatgcacaaataaagtttacaagctcaaaaaattaaacagcagtaacggtcaagctttccaacaataaaatacattttggtaaggttttcattttacaaaaactcaaaatagctttatgagttcacaaaataatatgatatttttcaagatattaacatattcttataccggaagagcatagaataaaatttacttggagattgagcatttgcttctttaagaaatacttcttttagtatttttactttaatattatgaaagctacataattacattcagattcattaactactccagtagttaatttttaaaacttatgatgaatagttttgtttaaaatatataacattggtaatatgcaaatctgaatctgtaataaagaaggatttgcattcctgatttttttttctgatacaaccaatgacaaaataactaatggttccacagaggataaaatgtctcaaatctgttggttctgaaggtgaagcgagatttttgtactgataccgtgtatcactgagataccaggaggaaatggaattaaactcagatagttcaaatggagagattttaatgaagggacgacctacagaggtgtcggcagggttggggggaatcagcgagatatgcttagaacccaccgactggcaaacctccccctgaagatggagaaggaggaaggagtgttactggaatgagagcttgagtccaggggaggaggatgggctgctgaggaggcgacaccatcctgaaagaagaatcctctgccagaggcttttcagggtcatttcttcacactctctgcagggaagcacggagacagcaggaagaaatatcctaacctcactctcttccctctacaggtgcttccattggccaaatccacccagaggccagttggtggcgatcagctctcttcaagtggtatttaaatttcttctttcattttccttctggtaacaaagaagtctgtggctcaaaagatgtttctctaagaccccatcctattaggtctctgagctgagggccgacgagtgggggcgggcaggagggccgagggaggcggaacaggatcgaggcgcgaggcgggagtcgagaaagcgagcggccgaggcgactctcagtgcgcggacgcgggcgcgcgcccgcgctcccttcgtcgactcacggcgagagcccaaccctgctgccgcgcgccacccgcctcgccgcgcct

SEQ ID NO: 12736 - RNA, 16776 nt, Homo sapiens
  source 1..16776: mol_type = other RNA
gatctcactttgttgcccaggctggtcttaaactcctggcctcaagtgatccccttgtttcagccccgcaaagtgctgggattacaggtgtgagccaccatgcccgtgcccagccacctcatgagtcttgatggggggcagagaccaacaactccacagaagccagatgcttgctttcccagcctctcttgcagctagggcttgggcatgtgatccaggctcagccaatcagatggcactgactcttggcatgacatgggctaaggaggggctgcagggaatccatttgggctggggtggcagctgcactgggagcgacatcagtttccagagggagcagcagaatctggcatcaggcttggggcgtggtaggtgcaaccagactctgcacccagcagcagtggcagaatgggttctctgtggagagtctgtgtattgctccttccgctgaggccaccagcatctgcctccatgaacccctcagagcctgtgagcaactcaacagccttgaattttttcccttcctgtttgaatgagccagggttgtttcactgcttgaactaagagccgttcctgacatgaaaactaagccacatctttttgacccaaagattctggcatcctaaaatacccatctcattttaagttaaaaataaatccatgtttgagcatctactgtttcagttactgtgctaggtgttacaaagctaactaagagtgacaagtaaataactatcatcaccatgataaacagagaatggaaccctggtttttggaatacagacacaaaatgattaattctgcctggaagcgttttggaacatttcagagaggtagtgagctgggccaagagaagagcatacgcaaggaatggtggcatgaagttgcctggtgtgtcctgagaagaaagatgggctaagaaggactggggtagggcagagaagggggtcactggaggtgaggctgggaaagtgagccaaggctcaaatgcaaactgtctgaacttcattttctgtgcaagcaggagaagccgctgacatgggtttggaagatggactgaagccggagaaaaatggaagcaagaaaccctctcacaagaggccataaccacaaccaagtccatgagattgaaaaggaaggcagatatttgaaaaatatttaaagagatgtgaggggtaggacaggcacagtggctcatgcctgtagtcccagcactttgggaggccgaggtgggcagatccacgaggtcaggagatcaagaccatcctaacatggtaaaaccccatctctactaacaatacaaaaaattagtcaggtgtggtggcacgtgcctgtagtcccagctactcaggaggctgaggcaggagaatcgcttgaacctgggaggcggaggttgcagtgagccgagattgtgccactgcaccctagcctaggcaacagagcaagactctgtctcaaaaaaaataaaaaaaaaaaaaagagagaaagagagagagagatgaggagttgctgcactgctgggtgtggagagccgaggaggattcaaagatggtcctgaagtcccagctggaagaagtaggcggcagcaatgtttttaatactgtaaattcatcacgtagcacaggtttggggtggagaaagaaaaattgcattggcttcagggcatgcccagatctttcctcatcttaggcgtttgctaatacatgcattttctaagctgatgtcttgcgtttaatcactgctccattcaaaagagagaaggaggttgtttcaaacctagttgatatcatttgacttccatgctattcacagggctattttatttgaaacaggtataccacagccttaaattgcaagttaatccaggatgttcctaggttggcagttaggaacatgtaattctttggaagggctaaaagtcagctctttaaattatctccatatgaaccttctctccaccttagggtggatccacttatttagtccactgccagtaccacactagaacccgggtggtcactggactccagaaacaacagtagccctctctctgttctgtctctttttgactatctctattctgttcctgaccctgatttctcctgccaagctcaattttgacagctgacaacggcaagccatggcttcccaaaacattattttcaggtcaacttataaatttcaagaacacatttggctccgcttcctgtggtactaagcctacttcttgacagcatttgcctttgttgtaaatagcaaagttcttctagttggatttttgctaagaagtgtgtggatgtggcatgtgacgacatctttagcttggattctagaaaggcactaccattgtgcatttggctaaaggaaacacattttacccgtgaatgccttctatttacaaatgctcagctagcacacaaagctaagtacaagcaataagtactatcctacaatgttactcatttctgaaagcacaaaatgatgactggtatagctttggagatgttttctggaaacccaataaaggaacagatctttgttattccacacctacaaagtcagaagatgcacagtcttttattcatgtttgaacaagcttccttcttgaacaatcaactataaagtgatgtgattctctactagaccaggaactccttgaggacagaatgagggtctaatccatattctaaatccacaccacctggcacaatacatgttgcatggttagggtcaactaagagttggttgaattaatcaataacacacagcaagagaattcacaaagagaggggagtaatcccccagcctcaatcactcggcaagtggaatcgctgggcactgattccagctctgtctcagtgcttgagacagagctgaatgtaatgtgaacatttcaaatgaacaggaaaactagactcacggataagcagtgtagtcatcaagacaacactgtcttggaggtttttctgaagttaaaaccatgctacataagcaataaattatgaaggctgagcatgtgaataaaatttaatgttgtcataaattttataacaaagttaatctgacacatttaatgacatgcataatcattagtatgcagcactgtaatcagacattgataataagcagttcacaccagtgactgtaagagtctttacttgtgttcagccaagccaactgcttggtatatttttctcccttcttagtcgttagttttccatacctacaataactatcagtggtgatgggcttctctgaccatgtgaataatttaatcctcaatgcacagatacagaaacccttgctgaagacagtgtggagcagagaaggctgtctccactccttccacctgaaacacctctgcagatggatatgggagctctgcctacagcccttggacctaaccacttcagtgtgttccagtgagtgtctggacctcggcctgaaagatttttccgaaactaaagaaaatttctctgacctaaagaccttaacctccaccccagaagctctcaccaaggactacagggaactggtggggaaaatccttatcccttactcctcaaggcacagggcagtaatgctgaggcttgtgcgccacacttgctcccagaggtccccagcgggctacctgcggtggtgaatgacctcctaacacgccccttgacggccttcctttccttgcctcacttctccactctcctaccagcattgcagggttcacatcccaaatataccactggcacttgaatcctggtctccaggtctgtttctggaaaaacccaagtaagacattgccccagtaatggggctagatgtctgaggcttcctcaagtatctacctcgaaagctcttactgctgtacacacatgcacatacacacacgtgcgtacaaccagtcacatctaagcaccccgaataccagcctgttgaaggtagcagagagctgcactataagccaaggctgctcccaagagccgctccatcactgaattggcgccccagcaagatgaaggaatgtaatcattggaaggatggagaatgttctctgaatcactgacaaattggaaggggtggagggcaagagtccacctggtggagagatggaaagagcgagagagcctggaatgataatgccattgcttagaaaaggctgctccagatgccatatctacagaaattgtacagcccaaacatctctgagcaataggtctctggtagtcttgatgtctagaccaacaattcccagttcattcttctcagggaaggagccaggatagtccagagactctcattctgctgttagattgaaagggttaggcacaacagccttggcaaagtcacaagggcaaattcacactaaagtgtaaatgacccacaactcctcttctatttttaggttggggaggtgctttagaacataaggaggaactaaagaatattcctgttacatacaaggcagagaaaagggaaactagtggtgacaagacaaatcatccctttgacatttggctggctctacctattacagctctgggggtgaggtgggaacaaaaagatgctgtgtaaagaagtatcttatgccatccctactgtagtgaggtgcagtttagaggggacactgatcaagcagagacccagagtgtttcgttccaagccagaaacagaaatgtataaaacacagcctttccagcatcagaaatgagtagtggtagtggagaactacccaaaacaggaaagaggaccacgtgaggtagagtgtcaaggccctacattccagtgcctctgctcatgactgtaattttgggtaggtcacttaaagtctctggacctcagttttgccatctgtgaaatagggataatactatccagcataaaattggttatgaggctcatgtagggcctgcctgggatgatgtgttgctaatggttaagaacacaacttctggggtctgactggacaggctgaaatccctgcttaacacgttccagcagagccctgggcgatctatttaacttttgttttctcacctgtaagctgagacgaaagtacccactttataagattattccaataattagttgaaataatgcatgcagagaattaagcatggtacttgttatttgttaaactagctattaaaatgtgtaaaatataaagtattgtatggattttaggacaatgcaaagactctttgcttgctgcaatagttcggggccctttcagatggctaaaggcagaatttgtatgtgtaaatatggtgtgcttgtctctgctctggatactgagggcttaccctgttattaaacttatttagtaaatattgaactgtcatgaggcctaacatttagttccagttattagataaaacatttgctttgaatggtatttgaattgccaggttctagattattctggttgacaaactcttcgtattttataaagaggctaaaattggtaagctatcacagaacagatgtgccattttcaaggtatattaaaccatgattcactgtaacattgttcctactggcaacaaattcagagcaggctggactttatttggtgaagaaacattgagtggaagagaaatgacattattttatgtatttacattttcaaattactgtggcttaaacctgttcagccaacattacccaccttcagtctgctaaataaatgattcagtacatttctaatttacagaattttttaacaaaagaaaatgtaatttgatagccaaatcaacgttaaacattatacatttaaaaaaccacaggcaaagacacaaacatgatgacactaacttttgttaaagtatgcttacctatggtttcctctgaggcacgttctttcatgctaagcttccaacataatatgaaaatgaaggagatgcattttgcaaagcaaaacagaccttaagcaaaatattatacttctcaaattaacactgttacaaagttttagaatttaataagttcattaatttaaaagtttggatgtctgagtccttctatcccaaaacaagatcttggagggtcttccacagccatgtaataccatggtcacatgaccctttccaaaattattaatctgaatttactatatgaggataaatctatctttttgaaaatatttaggaaaatgagcttggtatttataaaatgaagctctctttgggtggtatcctaagacacgtcaagccaatcagcctgtaactgtgaaaaaaacattggtaggtacaaaagtggggtgggagaggagtgacttaactttgttaagtgatgggaaagaaacactaatagcattatctcaataaaatgtgatttaaaaaaatttaaaatactaaatcattgaactgacaaagaaatataaatcattcagaaataaactcattaggtcatcaaatcctgttaaatctgcaattaggaagagcaaggtgtacaatccatacatttaaactcacaggctcactttgcacaacgtcaatttactccttaatatgttattaatacgcattttccaaaaggatgtattagtaaatggtacacatctacttcttggcaacatcatataacctggtacaacataagcattcttcttatagttaagaaatgtggatggtatcaaaattagaaaaataaatgccctattatgttgtggtcaggtttaaggcatgtgaattttatcttcatacaaaagattaaaatctagatattaaaaagtagtgcagtatcagtgatgctgcctcagttcccaaaatgtcacatcacaaaaatatcccataattgcctgtagtttattccttggctttcctcttttctctctgcatctttgtaacaattttttaaaagtggaaatataattgttggcaatgctaacagctgtagaaatgattacaagatgtggaaaagcataacaggaatgtcaagaatctgtttctggcagtaatatatatggaacattgttcaggacaaaagaggagaaggaagaaaaaaaggagaggggtttatcatctctaagaattttcaaactaaacctcattgcttaataggaaaaaaagattccatatttaaagttaagtcacctctaactactagctaaagcatgacatcaccagcactggagtcagcggaagtgtgtttttgaaggacagtgttgcaggagaatctggacaggttttagagccaggagagagaaaataattctacctctgacagttgaaggaccttaggcaaatcagtttacctctgctagactacactccaaaatttggacattcaaaaatttgatattaataaccacatgaaagtctcgtgttgaggtgaatatgtatttgttggtgaaagatatgttggtttttaaacagacagcactctgcaattgtaggctattgttttgttttgccagttgtcaaattctatccagctatacacacttgtgtggcctcctaatggtgtttttccagtggctaaaggtttatgaataagacacttttcctaatggaattaacccgatgcttttcttaaacatgtaaccttgagttcaccgcaaaaaacaatgcttcgattagagcaatgcatataataaaggttaccctcgtttcttagacactagacatcattcacaaaaagagaactgcttttgaaagggatgtatttgcactggaaagaatagttttctacttctaattataaatgatttattggtgaaagcaaaacaacagcctgtctgagaggcacttctatgagcatcctcacgtgtgatttgcaaggttgaagaagagggaaaaatgcctcaattgtaccaatggtgagaaaacacccaaagtacaaagcaggtttcaaaaaaaccatactcataaccaaggacaataataaagcaatgtgttgacatatactctataagtcttcctccataaatagtttatagaaattttgtaatttctgtaaatgcatcctataataattttgcatcttgctttttttttacatttaatatcaagtagatttctaaagggcaattatttgaaaattatcccaaatacatggggaaatatacatcaagtgaaaaaatgcagtgggtgatagagatatcaggaagcgcctcaaatatttctcatctcgttggagaaaaacaaacatgttctcatttagaatgagtgggagttacctaattgatttaggcctctatatttaacttctagtcaaaaaaggtagttctatctagcaacaatattatggggaacaaaagaaaaaattaactctctaaatttgcagtagggtcttttcttcagaagtaccaaatcccatctattaccagctccatgcttcaggcctaaaatggatctccctgaagcaatgacagaatttttgccaagtgactaggatataaacaccactttggttgcacagtgagacatatgctccaaagaaaactggttcaaaaacaggcaagtgggtttctacagaataaatgagagccctgtcaatggcttcatcttcagggctttgtgtctgtgcttgcgtggtggctcttgtttcatctatggataatggtggcacacagttttcataattccttacattaatgaactgctataaatttgtttttggtattctagagagtcctaacttcagcttctgggcaatgctgaggaggcaccctatattctagacttaccttttgcaaggtgtactctcagcattgtgggcgatttccatgggagaatattctatttaaagaactactgtcccagcataaaacaaaaaatcatttatgaagatgcaggagactcggaaagctctcaattattgtttgcacaagcacaatgtcacagcctcctttccccattccacaagggggtcaggaagagagtactcagctgtgagaaaagacatacagaagaattcatgtggtcatgagagcgaggacatggccgatcccccaaggaggatgtgtcatacacttcatgagcccaagagtgtgctgtagggtctgaagggcaagatgctggttcactgatgtaaaggagagggaaaaaagcttcaaccaactagaaaaacagtctctatgcatgctatttttgattttaaacacaggtatcaattccttctctcagagagtccattttaaaataggatacatttttaaaggaatatttaaaggacacattcattaaaatttattttaaaaacttttcaaaagaaacaaaaggtatgaattttatttaatccttgaggaaatggttcttttctcacacacataaatcactcattttgtttttctttatctcctttattaatctacattagaaaaataaacttttcatacactaagaacaaggaaaccactctcaattgacaaaatgttccaatccaacacaatgattactttcacctttaatttacaggcagccagattcaaaatccttaaagttgcttaaacttaaaaatgacaatgacaacctaaaaggtataatgttgattggaacagacatttaattggaaaattgatgattttccatttccaattaaatctctagatagaaatgaaaaaaattaaaaatcgtatttaagaaaagccaaatcttgggttgtgaggtatctttttaaggatgtttcagcagaaaaaaacaaaggctctcacaattgtgtagctgcctagattaagtgggtatcctgatcaaggagatgggggatgatttggctttagtattccaatgataaagtttataatgagaataacatgttgctacaaaatccagtctcttcctcagatgccttccacagagggcaggaagctttgtcagttttgtttgctgatgatgcctggttccgtcaacaaataacacctgataggcctggatcaagcatgcagctgtggagaacacccctgggactctaactctggcactctgcaagctgggtacttgggcaggacagcagcagcactcatgaactgggcagcacctgttggtgagggctgatcacatggattctctcatcccagccttacaatcagtccttcaggtacatactttttctgactttgctgatgaggaaactatgcacagaggttacacagcttaacaaagggttctcacctaatgaacaatgaaatgggattttagcctttctttgcatctggtcttagagccaatacccaagaagcactgtactgtatgcattgtctcagagaaacttactcttcctgggcctcagtctttaaaaggtgggcagttgacttaataagaattaaagatcaatgattaaggttcaaggcactccaaaattctggtctttattgaaaaggctacagaagtctcaccttaataataccctatagacttgatattcttggttaattaaatattggaaaccaatttcatagtaattgaggtcagaaaaaagtactcatgacattttagaatatgatgacaaagccatagataaatttcaatgcacctgtaattacttaaaactgttatagcatgcaatgtgttaccacaacagccagagaaatactaatttactcagcctattcttctagaccagtaaacactaggattaaatagatattttcattgaatttgttctacccttcattgccatttatagatagcttacttgtcatagattactttctaattgttttatgtttcctaactagcctgcaatactttggcaaggacctcaaacaatagtagacagtaggtgtaaaatagatggctacattgaacagatgactaaaaggatgcctcctaagtacctatatcttgaaatatatattattgtgccttgctttcaatttgtgattttaaaatctagaaatcacctgttttatgtaataacaataaaatccttctttgttgaaaacatgcacaaataaagtttacaagctcaaaaaattaaacagcagtaacggtcaagctttccaacaataaaatacattttggtaaggttttcattttacaaaaactcaaaatagctttatgagttcacaaaataatatgatatttttcaagatattaacatattcttataccggaagagcatagaataaaatttacttggagattgagcatttgcttctttaagaaatacttcttttagtatttttactttaatattatgaaagctacataattacattcagattcattaactactccagtagttaatttttaaaacttatgatgaatagttttgtttaaaatatataacattggtaatatgcaaatctgaatctgtaataaagaaggatttgcattcctgatttttttttctgatacaaccaatgacaaaataactaatggttccacagaggataaaatgtctcaaatctgttggttctgaaggtgaagcgagatttttgtactgataccgtgtatcactgagataccaggaggaaatggaattaaactcagatagttcaaatggagagattttaatgaagggacgacctacagaggtgtcggcagggttggggggaatcagcgagatatgcttagaacccaccgactggcaaacctccccctgaagatggagaaggaggaaggagtgttactggaatgagagcttgagtccaggggaggaggatgggctgctgaggaggcgacaccatcctgaaagaagaatcctctgccagaggcttttcagggtcatttcttcacactctctgcagggaagcacggagacagcaggaagaaatatcctaacctcactctcttccctctacaggtgcttccattggccaaatccacccagaggccagttggtggcgatcagctctcttcaagtggtatttaaatttcttctttcattttccttctggtaacaaagaagtctgtggctcaaaagatgtttctctaagaccccatcctattaggtctctgagctgtgggaagtatttatacaattgcttgtgaatataagatccaggaatttccctaagatccctaacaaaattggtgataagtagtcccacatgttaatccagccacccacggatgacagcacttaccatttctttgataaatgtcaaatgcatttgaagtacctacctgaaatatttgtttaaatgctatctaatctattaattttatatatgtgtgagtctgttttgtataccttctgattataggataaatgtaaataaatccaaagagtaatcaaagctaccactttcaagaagccttctttgtagaaccggaagagtcttaaataggcttttcaggtatgcatctcttattatcgctgaactccaagtcctgcaaggcaggcatcatgtgtgggtcacctttacagtaggcacaggccttaaaacagtgacatgcacattgcaggcactccataaatgtttgctgaattggctaaaccttggtttgttcccataatcaaccaccacaaacagcacacagataattacttcttggaaagattccaactagtgtttgatgttacctacgtggtttttctctcaagatcttaagagcagctctgtaggattacattattttctgttttttttttcctttgaccttaatgtcatctacttcaataacagcttcatacaaaattcctaccagcacataccacagcagattcaaggccttgttttaaaaatggtgccagcttctcttaatttggaagatatattgtctctcctgaacatgggctaagaaaatgtataatttggtattaacataagagctgaagacactttaaatgcattgtttcatttttataagataaaaaaaattttaagaatcaaaatgttatcaacagacttgtccttcattaaaaagtaaaactgcatttgcctacattttatgaaagtgtccaattatgaacaattttgaaatgtaacttttaaaaatgtaaacagcaaaaatgttgtatttaaaataaatctggaaaggcagaaaaacaaaaaatacccagaagacagagtttttggtgaaagttaagatatttcatctttgaacaacttagaatctttcctgcattttatagtctagttccaggcattaatttgaaataaccttggaatcctaaatctaacacccttcggaacaaagtagcttttctcttctgctttatgagcaaatggactaaatactagggaatggtactgtctgggcctttgaaccaagattgaaagagatgaaatcctatatgatatgtataaacattagagaatccattttgatttaataaaaggttgaatttgttctatatcctgtgagaaaatggttcccttttcctgaaaatgttacctcattccaacaatagaaagttggtttttttccagggtgtggtgttggcgggggacagagttgccatgaatatggcatctatgaagactgctgttatattcatttctcaaaatgcactgtggtaggaaattcagaacgcagtgagagaaaataaatgtttgacttcaaaatataaggccgcatttaaagcagaaggtaaagtatagaacagttgacagtataaattctttatctgcaatcttgcagttccctaaatctctgtaacacatcacttttaaaagcctcagataagtggttctataataatttaccaataattcaacccctcaaaagtcttagcaagttaaaccttataatcttacattttagaaatgacccaacttgatccttttattcttcagaatatctctctcaaattttcatttgtttttcattaattgatgaataatgagacattttaggtacctgtccacaaagaaatgaaattttcactttccaggaacctaacaaatgaaaagatagaaatcaattccaacagaatattaccaaagaaatcttttagaatggactgttaaaattatttatttgtatttatctggctctactatttgtggtacatttccacttcaaagctaaacctcaaataacatcatagtgagtggttgacttcatgtttaactgagatcttgaagactgaaaaagaccacgacaaacacacatctattttcttggctactgcatccgtgttcatcaccattctgatagtctgcaatgtattgcagctcaccctttgggaaggactaaagtagacatctgtttgttctgcttactcagcattcctaccctaattttcctttggagaacccctttattctagaccacgtgaagctaatgccaaaccccattccaggggatgcacctgaatccaacctccatcatctaaacagtgccttctccacgttcagagaagagcaagtgactcaaactgccctcataagaacagacctgggacttctgctgcaaatattgaagagtaagtactcttttttcttgctaggactaagctggtagtaccttctatgaggctatcatatggaaacaacttgtctgaaaatgaagccacaactagaaaacagatcctggtaacccggattgatggatccagccctaccttaaatggcaagacctaacccgaggctttttgcatcaaccaataaagtccttaagccagtttgagttggttttgtcacttgcagctaaaagaattctgactctaacaatgtgacaatagcaaaaataaacataactgcttttgaggtttctaatggattttcctccctatatacatgatttcatttaatcctcacaattcaggaaagcacatatctattaacattaaattaatattcattattttgaacacatgctatgtggataagggatgaggaaagccaaggaagtaatcaacgtgaaatctcacttatatgggagggaagtggaggttacatatctcagggcacttaacagatatcatcaaatgaaagaataaacagtgtgtgggagaggcagtaggtgattcttcatcaattcctggatgaaaaattaggagataatgaactccgaacaggcagcctaatgagaatggctcaagcaacaggacatagagagggagttaggttagacatggggttcttgggaattttcacctcgtgggggggcgggggggtcgtgcagctgttgtcagtgggaaagggaaaaaggaaaaggctgagtttggaaggcagggagggaggagacaatgtgagtcagtgaaaaagggcccttagaatgacaagtctggaccagagagaggctaagactgaaaatacaagttgggtaaccactggcatacagatggcagttcaggcttgggcactgcccaccagagcctcagcatgaagagaagagggggaggctggccaccacctccctctaggtaatcgtcatcctgatgctgagctcctgaaaacaggctctttcactcgccccatctcttgctcttgattgcaacccggcattcaggaggcaccctgtaatatctgtggagtgaccgacaacacagcgccagggcactgagaagatcccagggcgccagggactggttctacaagggtgcccctcccggtcccctccagcgcgccgccagagctgccagtcttggctgctacacgggaggcagcctcattatgcagctctcacctcttaaattagttcatgctctcacattaggtgtaatcacagcttgcaacgctttctggggatgtctcagaaagatctgagttgaaaaaatatttttgtgtcattttaatttaaagtaaaattgctgcttcttccccgcccctttctttcctcctggcccacccagcgaccctggccggccgtgctcaacgggggcgggggtcggaggtgagatttcctccacataattccttaaacagctatcaactaagtctcaaagaaaaaaaaaagagatctagaagcagagacgtggctgctggcgatcccaaagctggtgttcgctcttgggggagagcgtaccctgggggaggccgggaggccgggccagaggctagcccagaggcagagggcaggagcgctcagccggcgccccgcgtctctccagctcccgacgctgcgctggctccgctgagcacgccaggatcaaggtcgcctggtggggaccggagcgccaggagcctgtgggaagcgttccagccggcctctgactgggatccggcgccgcgtttctgctttggacttgactgacaggtccccccgccctcccgccgccctactaccagcctgggttcatccttcagggctacgtctaccgcacccgggctggaaagcctggagcgcgcccttcctctcctcatcttctcagctctcctttctccctgccacttggcaaagctgcattttgactttcacgttttggactacgtgtgtgtagttccaagtccatgcgtggcacgaaaatccacttagggtaaaaattattctcgaaaaatcgcccatctcaggatctggtgtctacactcaaggctaggaggtgcaggtacgggtgcgtaaagcatgccgtaagggtgcacagtaaataaaaagtacggatgcaaaatgtaaattttaagtgcaaaacagaaaagcagtactcgttgccgccccgcacgctgggttttaaggggcacgaaggtgggcctcggctgcttttgctcagccccgcgtcctcagcgcccggcccagtacccggtactccgtaggggttcaatgatctcccctgaataagtgaacgaattaacaaatgaatgaatgaccgctcgatccgacctccgcggccggcagagcagtcgctggagaggcgggagagagcgagaggccaagctccaccatcgcggccgccggctggggcagagggacacggagacactcggcgccccggctccgcaccgagtccccg

SEQ ID NO: 12737 - RNA, 13347 nt, Homo sapiens
  source 1..13347: mol_type = other RNA
gatctcactttgttgcccaggctggtcttaaactcctggcctcaagtgatccccttgtttcagccccgcaaagtgctgggattacaggtgtgagccaccatgcccgtgcccagccacctcatgagtcttgatggggggcagagaccaacaactccacagaagccagatgcttgctttcccagcctctcttgcagctagggcttgggcatgtgatccaggctcagccaatcagatggcactgactcttggcatgacatgggctaaggaggggctgcagggaatccatttgggctggggtggcagctgcactgggagcgacatcagtttccagagggagcagcagaatctggcatcaggcttggggcgtggtaggtgcaaccagactctgcacccagcagcagtggcagaatgggttctctgtggagagtctgtgtattgctccttccgctgaggccaccagcatctgcctccatgaacccctcagagcctgtgagcaactcaacagccttgaattttttcccttcctgtttgaatgagccagggttgtttcactgcttgaactaagagccgttcctgacatgaaaactaagccacatctttttgacccaaagattctggcatcctaaaatacccatctcattttaagttaaaaataaatccatgtttgagcatctactgtttcagttactgtgctaggtgttacaaagctaactaagagtgacaagtaaataactatcatcaccatgataaacagagaatggaaccctggtttttggaatacagacacaaaatgattaattctgcctggaagcgttttggaacatttcagagaggtagtgagctgggccaagagaagagcatacgcaaggaatggtggcatgaagttgcctggtgtgtcctgagaagaaagatgggctaagaaggactggggtagggcagagaagggggtcactggaggtgaggctgggaaagtgagccaaggctcaaatgcaaactgtctgaacttcattttctgtgcaagcaggagaagccgctgacatgggtttggaagatggactgaagccggagaaaaatggaagcaagaaaccctctcacaagaggccataaccacaaccaagtccatgagattgaaaaggaaggcagatatttgaaaaatatttaaagagatgtgaggggtaggacaggcacagtggctcatgcctgtagtcccagcactttgggaggccgaggtgggcagatccacgaggtcaggagatcaagaccatcctaacatggtaaaaccccatctctactaacaatacaaaaaattagtcaggtgtggtggcacgtgcctgtagtcccagctactcaggaggctgaggcaggagaatcgcttgaacctgggaggcggaggttgcagtgagccgagattgtgccactgcaccctagcctaggcaacagagcaagactctgtctcaaaaaaaataaaaaaaaaaaaaagagagaaagagagagagagatgaggagttgctgcactgctgggtgtggagagccgaggaggattcaaagatggtcctgaagtcccagctggaagaagtaggcggcagcaatgtttttaatactgtaaattcatcacgtagcacaggtttggggtggagaaagaaaaattgcattggcttcagggcatgcccagatctttcctcatcttaggcgtttgctaatacatgcattttctaagctgatgtcttgcgtttaatcactgctccattcaaaagagagaaggaggttgtttcaaacctagttgatatcatttgacttccatgctattcacagggctattttatttgaaacaggtataccacagccttaaattgcaagttaatccaggatgttcctaggttggcagttaggaacatgtaattctttggaagggctaaaagtcagctctttaaattatctccatatgaaccttctctccaccttagggtggatccacttatttagtccactgccagtaccacactagaacccgggtggtcactggactccagaaacaacagtagccctctctctgttctgtctctttttgactatctctattctgttcctgaccctgatttctcctgccaagctcaattttgacagctgacaacggcaagccatggcttcccaaaacattattttcaggtcaacttataaatttcaagaacacatttggctccgcttcctgtggtactaagcctacttcttgacagcatttgcctttgttgtaaatagcaaagttcttctagttggatttttgctaagaagtgtgtggatgtggcatgtgacgacatctttagcttggattctagaaaggcactaccattgtgcatttggctaaaggaaacacattttacccgtgaatgccttctatttacaaatgctcagctagcacacaaagctaagtacaagcaataagtactatcctacaatgttactcatttctgaaagcacaaaatgatgactggtatagctttggagatgttttctggaaacccaataaaggaacagatctttgttattccacacctacaaagtcagaagatgcacagtcttttattcatgtttgaacaagcttccttcttgaacaatcaactataaagtgatgtgattctctactagaccaggaactccttgaggacagaatgagggtctaatccatattctaaatccacaccacctggcacaatacatgttgcatggttagggtcaactaagagttggttgaattaatcaataacacacagcaagagaattcacaaagagaggggagtaatcccccagcctcaatcactcggcaagtggaatcgctgggcactgattccagctctgtctcagtgcttgagacagagctgaatgtaatgtgaacatttcaaatgaacaggaaaactagactcacggataagcagtgtagtcatcaagacaacactgtcttggaggtttttctgaagttaaaaccatgctacataagcaataaattatgaaggctgagcatgtgaataaaatttaatgttgtcataaattttataacaaagttaatctgacacatttaatgacatgcataatcattagtatgcagcactgtaatcagacattgataataagcagttcacaccagtgactgtaagagtctttacttgtgttcagccaagccaactgcttggtatatttttctcccttcttagtcgttagttttccatacctacaataactatcagtggtgatgggcttctctgaccatgtgaataatttaatcctcaatgcacagatacagaaacccttgctgaagacagtgtggagcagagaaggctgtctccactccttccacctgaaacacctctgcagatggatatgggagctctgcctacagcccttggacctaaccacttcagtgtgttccagtgagtgtctggacctcggcctgaaagatttttccgaaactaaagaaaatttctctgacctaaagaccttaacctccaccccagaagctctcaccaaggactacagggaactggtggggaaaatccttatcccttactcctcaaggcacagggcagtaatgctgaggcttgtgcgccacacttgctcccagaggtccccagcgggctacctgcggtggtgaatgacctcctaacacgccccttgacggccttcctttccttgcctcacttctccactctcctaccagcattgcagggttcacatcccaaatataccactggcacttgaatcctggtctccaggtctgtttctggaaaaacccaagtaagacattgccccagtaatggggctagatgtctgaggcttcctcaagtatctacctcgaaagctcttactgctgtacacacatgcacatacacacacgtgcgtacaaccagtcacatctaagcaccccgaataccagcctgttgaaggtagcagagagctgcactataagccaaggctgctcccaagagccgctccatcactgaattggcgccccagcaagatgaaggaatgtaatcattggaaggatggagaatgttctctgaatcactgacaaattggaaggggtggagggcaagagtccacctggtggagagatggaaagagcgagagagcctggaatgataatgccattgcttagaaaaggctgctccagatgccatatctacagaaattgtacagcccaaacatctctgagcaataggtctctggtagtcttgatgtctagaccaacaattcccagttcattcttctcagggaaggagccaggatagtccagagactctcattctgctgttagattgaaagggttaggcacaacagccttggcaaagtcacaagggcaaattcacactaaagtgtaaatgacccacaactcctcttctatttttaggttggggaggtgctttagaacataaggaggaactaaagaatattcctgttacatacaaggcagagaaaagggaaactagtggtgacaagacaaatcatccctttgacatttggctggctctacctattacagctctgggggtgaggtgggaacaaaaagatgctgtgtaaagaagtatcttatgccatccctactgtagtgaggtgcagtttagaggggacactgatcaagcagagacccagagtgtttcgttccaagccagaaacagaaatgtataaaacacagcctttccagcatcagaaatgagtagtggtagtggagaactacccaaaacaggaaagaggaccacgtgaggtagagtgtcaaggccctacattccagtgcctctgctcatgactgtaattttgggtaggtcacttaaagtctctggacctcagttttgccatctgtgaaatagggataatactatccagcataaaattggttatgaggctcatgtagggcctgcctgggatgatgtgttgctaatggttaagaacacaacttctggggtctgactggacaggctgaaatccctgcttaacacgttccagcagagccctgggcgatctatttaacttttgttttctcacctgtaagctgagacgaaagtacccactttataagattattccaataattagttgaaataatgcatgcagagaattaagcatggtacttgttatttgttaaactagctattaaaatgtgtaaaatataaagtattgtatggattttaggacaatgcaaagactctttgcttgctgcaatagttcggggccctttcagatggctaaaggcagaatttgtatgtgtaaatatggtgtgcttgtctctgctctggatactgagggcttaccctgttattaaacttatttagtaaatattgaactgtcatgaggcctaacatttagttccagttattagataaaacatttgctttgaatggtatttgaattgccaggttctagattattctggttgacaaactcttcgtattttataaagaggctaaaattggtaagctatcacagaacagatgtgccattttcaaggtatattaaaccatgattcactgtaacattgttcctactggcaacaaattcagagcaggctggactttatttggtgaagaaacattgagtggaagagaaatgacattattttatgtatttacattttcaaattactgtggcttaaacctgttcagccaacattacccaccttcagtctgctaaataaatgattcagtacatttctaatttacagaattttttaacaaaagaaaatgtaatttgatagccaaatcaacgttaaacattatacatttaaaaaaccacaggcaaagacacaaacatgatgacactaacttttgttaaagtatgcttacctatggtttcctctgaggcacgttctttcatgctaagcttccaacataatatgaaaatgaaggagatgcattttgcaaagcaaaacagaccttaagcaaaatattatacttctcaaattaacactgttacaaagttttagaatttaataagttcattaatttaaaagtttggatgtctgagtccttctatcccaaaacaagatcttggagggtcttccacagccatgtaataccatggtcacatgaccctttccaaaattattaatctgaatttactatatgaggataaatctatctttttgaaaatatttaggaaaatgagcttggtatttataaaatgaagctctctttgggtggtatcctaagacacgtcaagccaatcagcctgtaactgtgaaaaaaacattggtaggtacaaaagtggggtgggagaggagtgacttaactttgttaagtgatgggaaagaaacactaatagcattatctcaataaaatgtgatttaaaaaaatttaaaatactaaatcattgaactgacaaagaaatataaatcattcagaaataaactcattaggtcatcaaatcctgttaaatctgcaattaggaagagcaaggtgtacaatccatacatttaaactcacaggctcactttgcacaacgtcaatttactccttaatatgttattaatacgcattttccaaaaggatgtattagtaaatggtacacatctacttcttggcaacatcatataacctggtacaacataagcattcttcttatagttaagaaatgtggatggtatcaaaattagaaaaataaatgccctattatgttgtggtcaggtttaaggcatgtgaattttatcttcatacaaaagattaaaatctagatattaaaaagtagtgcagtatcagtgatgctgcctcagttcccaaaatgtcacatcacaaaaatatcccataattgcctgtagtttattccttggctttcctcttttctctctgcatctttgtaacaattttttaaaagtggaaatataattgttggcaatgctaacagctgtagaaatgattacaagatgtggaaaagcataacaggaatgtcaagaatctgtttctggcagtaatatatatggaacattgttcaggacaaaagaggagaaggaagaaaaaaaggagaggggtttatcatctctaagaattttcaaactaaacctcattgcttaataggaaaaaaagattccatatttaaagttaagtcacctctaactactagctaaagcatgacatcaccagcactggagtcagcggaagtgtgtttttgaaggacagtgttgcaggagaatctggacaggttttagagccaggagagagaaaataattctacctctgacagttgaaggaccttaggcaaatcagtttacctctgctagactacactccaaaatttggacattcaaaaatttgatattaataaccacatgaaagtctcgtgttgaggtgaatatgtatttgttggtgaaagatatgttggtttttaaacagacagcactctgcaattgtaggctattgttttgttttgccagttgtcaaattctatccagctatacacacttgtgtggcctcctaatggtgtttttccagtggctaaaggtttatgaataagacacttttcctaatggaattaacccgatgcttttcttaaacatgtaaccttgagttcaccgcaaaaaacaatgcttcgattagagcaatgcatataataaaggttaccctcgtttcttagacactagacatcattcacaaaaagagaactgcttttgaaagggatgtatttgcactggaaagaatagttttctacttctaattataaatgatttattggtgaaagcaaaacaacagcctgtctgagaggcacttctatgagcatcctcacgtgtgatttgcaaggttgaagaagagggaaaaatgcctcaattgtaccaatggtgagaaaacacccaaagtacaaagcaggtttcaaaaaaaccatactcataaccaaggacaataataaagcaatgtgttgacatatactctataagtcttcctccataaatagtttatagaaattttgtaatttctgtaaatgcatcctataataattttgcatcttgctttttttttacatttaatatcaagtagatttctaaagggcaattatttgaaaattatcccaaatacatggggaaatatacatcaagtgaaaaaatgcagtgggtgatagagatatcaggaagcgcctcaaatatttctcatctcgttggagaaaaacaaacatgttctcatttagaatgagtgggagttacctaattgatttaggcctctatatttaacttctagtcaaaaaaggtagttctatctagcaacaatattatggggaacaaaagaaaaaattaactctctaaatttgcagtagggtcttttcttcagaagtaccaaatcccatctattaccagctccatgcttcaggcctaaaatggatctccctgaagcaatgacagaatttttgccaagtgactaggatataaacaccactttggttgcacagtgagacatatgctccaaagaaaactggttcaaaaacaggcaagtgggtttctacagaataaatgagagccctgtcaatggcttcatcttcagggctttgtgtctgtgcttgcgtggtggctcttgtttcatctatggataatggtggcacacagttttcataattccttacattaatgaactgctataaatttgtttttggtattctagagagtcctaacttcagcttctgggcaatgctgaggaggcaccctatattctagacttaccttttgcaaggtgtactctcagcattgtgggcgatttccatgggagaatattctatttaaagaactactgtcccagcataaaacaaaaaatcatttatgaagatgcaggagactcggaaagctctcaattattgtttgcacaagcacaatgtcacagcctcctttccccattccacaagggggtcaggaagagagtactcagctgtgagaaaagacatacagaagaattcatgtggtcatgagagcgaggacatggccgatcccccaaggaggatgtgtcatacacttcatgagcccaagagtgtgctgtagggtctgaagggcaagatgctggttcactgatgtaaaggagagggaaaaaagcttcaaccaactagaaaaacagtctctatgcatgctatttttgattttaaacacaggtatcaattccttctctcagagagtccattttaaaataggatacatttttaaaggaatatttaaaggacacattcattaaaatttattttaaaaacttttcaaaagaaacaaaaggtatgaattttatttaatccttgaggaaatggttcttttctcacacacataaatcactcattttgtttttctttatctcctttattaatctacattagaaaaataaacttttcatacactaagaacaaggaaaccactctcaattgacaaaatgttccaatccaacacaatgattactttcacctttaatttacaggcagccagattcaaaatccttaaagttgcttaaacttaaaaatgacaatgacaacctaaaaggtataatgttgattggaacagacatttaattggaaaattgatgattttccatttccaattaaatctctagatagaaatgaaaaaaattaaaaatcgtatttaagaaaagccaaatcttgggttgtgaggtatctttttaaggatgtttcagcagaaaaaaacaaaggctctcacaattgtgtagctgcctagattaagtgggtatcctgatcaaggagatgggggatgatttggctttagtattccaatgataaagtttataatgagaataacatgttgctacaaaatccagtctcttcctcagatgccttccacagagggcaggaagctttgtcagttttgtttgctgatgatgcctggttccgtcaacaaataacacctgataggcctggatcaagcatgcagctgtggagaacacccctgggactctaactctggcactctgcaagctgggtacttgggcaggacagcagcagcactcatgaactgggcagcacctgttggtgagggctgatcacatggattctctcatcccagccttacaatcagtccttcaggtacatactttttctgactttgctgatgaggaaactatgcacagaggttacacagcttaacaaagggttctcacctctcttcaagtggtatttaaatttcttctttcattttccttctggtaacaaagaagtctgtggctcaaaagatgtttctctaagaccccatcctattaggtctctgagattttagaaatgacccaacttgatccttttattcttcagaatatctctctcaaattttcatttgtttttcattaattgatgaataatgagacattttaggtacctgtccacaaagaaatgaaattttcactttccaggaacctaacaaatgaaaagatagaaatcaattccaacagaatattaccaaagaaatcttttagaatggactgttaaaattatttatttgtatttatctggctctactatttgtggtacatttccacttcaaagctaaacctcaaataacatcatagtgagtggttgacttcatgtttaactgagatcttgaagactgaaaaagaccacgacaaacacacatctattttcttggctactgcatccgtgttcatcaccattctgatagtctgcaatgtattgcagctcaccctttgggaaggactaaagtagacatctgtttgttctgcttactcagcattcctaccctaattttcctttggagaacccctttattctagaccacgtgaagctaatgccaaaccccattccaggggatgcacctgaatccaacctccatcatctaaacagtgccttctccacgttcagagaagagcaagtgactcaaactgccctcataagaacagacctgggacttctgctgcaaatattgaagagtaagtactcttttttcttgctaggactaagctggtagtaccttctatgaggctatcatatggaaacaacttgtctgaaaatgaagccacaactagaaaacagatcctggtaacccggattgatggatccagccctaccttaaatggcaagacctaacccgaggctttttgcatcaaccaataaagtccttaagccagtttgagttggttttgtcacttgcagctaaaagaattctgactctaacaatgtgacaatagcaaaaataaacataactgcttttgaggtttctaatggattttcctccctatatacatgatttcatttaatcctcacaattcaggaaagcacatatctattaacattaaattaatattcattattttgaacacatgctatgtggataagggatgaggaaagccaaggaagtaatcaacgtgaaatctcacttatatgggagggaagtggaggttacatatctcagggcacttaacagatatcatcaaatgaaagaataaacagtgtgtgggagaggcagtaggtgattcttcatcaattcctggatgaaaaattaggagataatgaactccgaacaggcagcctaatgagaatggctcaagcaacaggacatagagagggagttaggttagacatggggttcttgggaattttcacctcgtgggggggcgggggggtcgtgcagctgttgtcagtgggaaagggaaaaaggaaaaggctgagtttggaaggcagggagggaggagacaatgtgagtcagtgaaaaagggcccttagaatgacaagtctggaccagagagaggctaagactgaaaatacaagttgggtaaccactggcatacagatggcagttcaggcttgggcactgcccaccagagcctcagcatgaagagaagagggggaggctggccaccacctccctctaggtaatcgtcatcctgatgctgagctcctgaaaacaggctctttcactcgccccatctcttgctcttgattgcaacccggcattcaggaggcaccctgtaatatctgtggagtgaccgacaacacagcgccagggcactgagaagatcccagggcgccagggactggttctacaagggtgcccctcccggtcccctccagcgcgccgccagagctgccagtcttggctgctacacgggaggcagcctcattatgcagctctcacctcttaaattagttcatgctctcacattaggtgtaatcacagcttgcaacgctttctggggatgtctcagaaagatctgagttgaaaaaatatttttgtgtcattttaatttaaagtaaaattgctgcttcttccccgcccctttctttcctcctggcccacccagcgaccctggccggccgtgctcaacgggggcgggggtcggaggtgagatttcctccacataattccttaaacagctatcaactaagtctcaaagaaaaaaaaaagagatctagaagcagagacgtggctgctggcgatcccaaagctggtgttcgctcttgggggagagcgtaccctgggggaggccgggaggccgggccagaggctagcccagaggcagagggcaggagcgctcagccggcgccccgcgtctctccagctcccgacgctgcgctggctccgctgagcacgccaggatcaaggtcgcctggtggggaccggagcgccaggagcctgtgggaagcgttccagccggcctctgactgggatccggcgccgcgtttctgctttggacttgactgacaggtccccccgccctcccgccgccctactaccagcctgggttcatccttcagggctacgtctaccgcacccgggctggaaagcctggagcgcgcccttcctctcctcatcttctcagctctcctttctccctgccacttggcaaagctgcattttgactttcacgttttggactacgtgtgtgtagttccaagtccatgcgtggcacgaaaatccacttagggtaaaaattattctcgaaaaatcgcccatctcaggatctggtgtctacactcaaggctaggaggtgcaggtacgggtgcgtaaagcatgccgtaagggtgcacagtaaataaaaagtacggatgcaaaatgtaaattttaagtgcaaaacagaaaagcagtactcgttgccgccccgcacgctgggttttaaggggcacgaaggtgggcctcggctgcttttgctcagccccgcgtcctcagcgcccggcccagtacccggtactccgtaggggttcaatgatctcccctgaataagtgaacgaattaacaaatgaatgaatgaccgctcgatccgacctccgcggccggcagagcagtcgctggagaggcgggagagagcgagaggccaagctccaccatcgcggccgccggctggggcagagggacacggagacactcggcgccccggctccgcaccgagtccc

SEQ ID NO: 12738 - RNA, 15088 nt, Homo sapiens
  source 1..15088: mol_type = other RNA
gatctcactttgttgcccaggctggtcttaaactcctggcctcaagtgatccccttgtttcagccccgcaaagtgctgggattacaggtgtgagccaccatgcccgtgcccagccacctcatgagtcttgatggggggcagagaccaacaactccacagaagccagatgcttgctttcccagcctctcttgcagctagggcttgggcatgtgatccaggctcagccaatcagatggcactgactcttggcatgacatgggctaaggaggggctgcagggaatccatttgggctggggtggcagctgcactgggagcgacatcagtttccagagggagcagcagaatctggcatcaggcttggggcgtggtaggtgcaaccagactctgcacccagcagcagtggcagaatgggttctctgtggagagtctgtgtattgctccttccgctgaggccaccagcatctgcctccatgaacccctcagagcctgtgagcaactcaacagccttgaattttttcccttcctgtttgaatgagccagggttgtttcactgcttgaactaagagccgttcctgacatgaaaactaagccacatctttttgacccaaagattctggcatcctaaaatacccatctcattttaagttaaaaataaatccatgtttgagcatctactgtttcagttactgtgctaggtgttacaaagctaactaagagtgacaagtaaataactatcatcaccatgataaacagagaatggaaccctggtttttggaatacagacacaaaatgattaattctgcctggaagcgttttggaacatttcagagaggtagtgagctgggccaagagaagagcatacgcaaggaatggtggcatgaagttgcctggtgtgtcctgagaagaaagatgggctaagaaggactggggtagggcagagaagggggtcactggaggtgaggctgggaaagtgagccaaggctcaaatgcaaactgtctgaacttcattttctgtgcaagcaggagaagccgctgacatgggtttggaagatggactgaagccggagaaaaatggaagcaagaaaccctctcacaagaggccataaccacaaccaagtccatgagattgaaaaggaaggcagatatttgaaaaatatttaaagagatgtgaggggtaggacaggcacagtggctcatgcctgtagtcccagcactttgggaggccgaggtgggcagatccacgaggtcaggagatcaagaccatcctaacatggtaaaaccccatctctactaacaatacaaaaaattagtcaggtgtggtggcacgtgcctgtagtcccagctactcaggaggctgaggcaggagaatcgcttgaacctgggaggcggaggttgcagtgagccgagattgtgccactgcaccctagcctaggcaacagagcaagactctgtctcaaaaaaaataaaaaaaaaaaaaagagagaaagagagagagagatgaggagttgctgcactgctgggtgtggagagccgaggaggattcaaagatggtcctgaagtcccagctggaagaagtaggcggcagcaatgtttttaatactgtaaattcatcacgtagcacaggtttggggtggagaaagaaaaattgcattggcttcagggcatgcccagatctttcctcatcttaggcgtttgctaatacatgcattttctaagctgatgtcttgcgtttaatcactgctccattcaaaagagagaaggaggttgtttcaaacctagttgatatcatttgacttccatgctattcacagggctattttatttgaaacaggtataccacagccttaaattgcaagttaatccaggatgttcctaggttggcagttaggaacatgtaattctttggaagggctaaaagtcagctctttaaattatctccatatgaaccttctctccaccttagggtggatccacttatttagtccactgccagtaccacactagaacccgggtggtcactggactccagaaacaacagtagccctctctctgttctgtctctttttgactatctctattctgttcctgaccctgatttctcctgccaagctcaattttgacagctgacaacggcaagccatggcttcccaaaacattattttcaggtcaacttataaatttcaagaacacatttggctccgcttcctgtggtactaagcctacttcttgacagcatttgcctttgttgtaaatagcaaagttcttctagttggatttttgctaagaagtgtgtggatgtggcatgtgacgacatctttagcttggattctagaaaggcactaccattgtgcatttggctaaaggaaacacattttacccgtgaatgccttctatttacaaatgctcagctagcacacaaagctaagtacaagcaataagtactatcctacaatgttactcatttctgaaagcacaaaatgatgactggtatagctttggagatgttttctggaaacccaataaaggaacagatctttgttattccacacctacaaagtcagaagatgcacagtcttttattcatgtttgaacaagcttccttcttgaacaatcaactataaagtgatgtgattctctactagaccaggaactccttgaggacagaatgagggtctaatccatattctaaatccacaccacctggcacaatacatgttgcatggttagggtcaactaagagttggttgaattaatcaataacacacagcaagagaattcacaaagagaggggagtaatcccccagcctcaatcactcggcaagtggaatcgctgggcactgattccagctctgtctcagtgcttgagacagagctgaatgtaatgtgaacatttcaaatgaacaggaaaactagactcacggataagcagtgtagtcatcaagacaacactgtcttggaggtttttctgaagttaaaaccatgctacataagcaataaattatgaaggctgagcatgtgaataaaatttaatgttgtcataaattttataacaaagttaatctgacacatttaatgacatgcataatcattagtatgcagcactgtaatcagacattgataataagcagttcacaccagtgactgtaagagtctttacttgtgttcagccaagccaactgcttggtatatttttctcccttcttagtcgttagttttccatacctacaataactatcagtggtgatgggcttctctgaccatgtgaataatttaatcctcaatgcacagatacagaaacccttgctgaagacagtgtggagcagagaaggctgtctccactccttccacctgaaacacctctgcagatggatatgggagctctgcctacagcccttggacctaaccacttcagtgtgttccagtgagtgtctggacctcggcctgaaagatttttccgaaactaaagaaaatttctctgacctaaagaccttaacctccaccccagaagctctcaccaaggactacagggaactggtggggaaaatccttatcccttactcctcaaggcacagggcagtaatgctgaggcttgtgcgccacacttgctcccagaggtccccagcgggctacctgcggtggtgaatgacctcctaacacgccccttgacggccttcctttccttgcctcacttctccactctcctaccagcattgcagggttcacatcccaaatataccactggcacttgaatcctggtctccaggtctgtttctggaaaaacccaagtaagacattgccccagtaatggggctagatgtctgaggcttcctcaagtatctacctcgaaagctcttactgctgtacacacatgcacatacacacacgtgcgtacaaccagtcacatctaagcaccccgaataccagcctgttgaaggtagcagagagctgcactataagccaaggctgctcccaagagccgctccatcactgaattggcgccccagcaagatgaaggaatgtaatcattggaaggatggagaatgttctctgaatcactgacaaattggaaggggtggagggcaagagtccacctggtggagagatggaaagagcgagagagcctggaatgataatgccattgcttagaaaaggctgctccagatgccatatctacagaaattgtacagcccaaacatctctgagcaataggtctctggtagtcttgatgtctagaccaacaattcccagttcattcttctcagggaaggagccaggatagtccagagactctcattctgctgttagattgaaagggttaggcacaacagccttggcaaagtcacaagggcaaattcacactaaagtgtaaatgacccacaactcctcttctatttttaggttggggaggtgctttagaacataaggaggaactaaagaatattcctgttacatacaaggcagagaaaagggaaactagtggtgacaagacaaatcatccctttgacatttggctggctctacctattacagctctgggggtgaggtgggaacaaaaagatgctgtgtaaagaagtatcttatgccatccctactgtagtgaggtgcagtttagaggggacactgatcaagcagagacccagagtgtttcgttccaagccagaaacagaaatgtataaaacacagcctttccagcatcagaaatgagtagtggtagtggagaactacccaaaacaggaaagaggaccacgtgaggtagagtgtcaaggccctacattccagtgcctctgctcatgactgtaattttgggtaggtcacttaaagtctctggacctcagttttgccatctgtgaaatagggataatactatccagcataaaattggttatgaggctcatgtagggcctgcctgggatgatgtgttgctaatggttaagaacacaacttctggggtctgactggacaggctgaaatccctgcttaacacgttccagcagagccctgggcgatctatttaacttttgttttctcacctgtaagctgagacgaaagtacccactttataagattattccaataattagttgaaataatgcatgcagagaattaagcatggtacttgttatttgttaaactagctattaaaatgtgtaaaatataaagtattgtatggattttaggacaatgcaaagactctttgcttgctgcaatagttcggggccctttcagatggctaaaggcagaatttgtatgtgtaaatatggtgtgcttgtctctgctctggatactgagggcttaccctgttattaaacttatttagtaaatattgaactgtcatgaggcctaacatttagttccagttattagataaaacatttgctttgaatggtatttgaattgccaggttctagattattctggttgacaaactcttcgtattttataaagaggctaaaattggtaagctatcacagaacagatgtgccattttcaaggtatattaaaccatgattcactgtaacattgttcctactggcaacaaattcagagcaggctggactttatttggtgaagaaacattgagtggaagagaaatgacattattttatgtatttacattttcaaattactgtggcttaaacctgttcagccaacattacccaccttcagtctgctaaataaatgattcagtacatttctaatttacagaattttttaacaaaagaaaatgtaatttgatagccaaatcaacgttaaacattatacatttaaaaaaccacaggcaaagacacaaacatgatgacactaacttttgttaaagtatgcttacctatggtttcctctgaggcacgttctttcatgctaagcttccaacataatatgaaaatgaaggagatgcattttgcaaagcaaaacagaccttaagcaaaatattatacttctcaaattaacactgttacaaagttttagaatttaataagttcattaatttaaaagtttggatgtctgagtccttctatcccaaaacaagatcttggagggtcttccacagccatgtaataccatggtcacatgaccctttccaaaattattaatctgaatttactatatgaggataaatctatctttttgaaaatatttaggaaaatgagcttggtatttataaaatgaagctctctttgggtggtatcctaagacacgtcaagccaatcagcctgtaactgtgaaaaaaacattggtaggtacaaaagtggggtgggagaggagtgacttaactttgttaagtgatgggaaagaaacactaatagcattatctcaataaaatgtgatttaaaaaaatttaaaatactaaatcattgaactgacaaagaaatataaatcattcagaaataaactcattaggtcatcaaatcctgttaaatctgcaattaggaagagcaaggtgtacaatccatacatttaaactcacaggctcactttgcacaacgtcaatttactccttaatatgttattaatacgcattttccaaaaggatgtattagtaaatggtacacatctacttcttggcaacatcatataacctggtacaacataagcattcttcttatagttaagaaatgtggatggtatcaaaattagaaaaataaatgccctattatgttgtggtcaggtttaaggcatgtgaattttatcttcatacaaaagattaaaatctagatattaaaaagtagtgcagtatcagtgatgctgcctcagttcccaaaatgtcacatcacaaaaatatcccataattgcctgtagtttattccttggctttcctcttttctctctgcatctttgtaacaattttttaaaagtggaaatataattgttggcaatgctaacagctgtagaaatgattacaagatgtggaaaagcataacaggaatgtcaagaatctgtttctggcagtaatatatatggaacattgttcaggacaaaagaggagaaggaagaaaaaaaggagaggggtttatcatctctaagaattttcaaactaaacctcattgcttaataggaaaaaaagattccatatttaaagttaagtcacctctaactactagctaaagcatgacatcaccagcactggagtcagcggaagtgtgtttttgaaggacagtgttgcaggagaatctggacaggttttagagccaggagagagaaaataattctacctctgacagttgaaggaccttaggcaaatcagtttacctctgctagactacactccaaaatttggacattcaaaaatttgatattaataaccacatgaaagtctcgtgttgaggtgaatatgtatttgttggtgaaagatatgttggtttttaaacagacagcactctgcaattgtaggctattgttttgttttgccagttgtcaaattctatccagctatacacacttgtgtggcctcctaatggtgtttttccagtggctaaaggtttatgaataagacacttttcctaatggaattaacccgatgcttttcttaaacatgtaaccttgagttcaccgcaaaaaacaatgcttcgattagagcaatgcatataataaaggttaccctcgtttcttagacactagacatcattcacaaaaagagaactgcttttgaaagggatgtatttgcactggaaagaatagttttctacttctaattataaatgatttattggtgaaagcaaaacaacagcctgtctgagaggcacttctatgagcatcctcacgtgtgatttgcaaggttgaagaagagggaaaaatgcctcaattgtaccaatggtgagaaaacacccaaagtacaaagcaggtttcaaaaaaaccatactcataaccaaggacaataataaagcaatgtgttgacatatactctataagtcttcctccataaatagtttatagaaattttgtaatttctgtaaatgcatcctataataattttgcatcttgctttttttttacatttaatatcaagtagatttctaaagggcaattatttgaaaattatcccaaatacatggggaaatatacatcaagtgaaaaaatgcagtgggtgatagagatatcaggaagcgcctcaaatatttctcatctcgttggagaaaaacaaacatgttctcatttagaatgagtgggagttacctaattgatttaggcctctatatttaacttctagtcaaaaaaggtagttctatctagcaacaatattatggggaacaaaagaaaaaattaactctctaaatttgcagtagggtcttttcttcagaagtaccaaatcccatctattaccagctccatgcttcaggcctaaaatggatctccctgaagcaatgacagaatttttgccaagtgactaggatataaacaccactttggttgcacagtgagacatatgctccaaagaaaactggttcaaaaacaggcaagtgggtttctacagaataaatgagagccctgtcaatggcttcatcttcagggctttgtgtctgtgcttgcgtggtggctcttgtttcatctatggataatggtggcacacagttttcataattccttacattaatgaactgctataaatttgtttttggtattctagagagtcctaacttcagcttctgggcaatgctgaggaggcaccctatattctagacttaccttttgcaaggtgtactctcagcattgtgggcgatttccatgggagaatattctatttaaagaactactgtcccagcataaaacaaaaaatcatttatgaagatgcaggagactcggaaagctctcaattattgtttgcacaagcacaatgtcacagcctcctttccccattccacaagggggtcaggaagagagtactcagctgtgagaaaagacatacagaagaattcatgtggtcatgagagcgaggacatggccgatcccccaaggaggatgtgtcatacacttcatgagcccaagagtgtgctgtagggtctgaagggcaagatgctggttcactgatgtaaaggagagggaaaaaagcttcaaccaactagaaaaacagtctctatgcatgctatttttgattttaaacacaggtatcaattccttctctcagagagtccattttaaaataggatacatttttaaaggaatatttaaaggacacattcattaaaatttattttaaaaacttttcaaaagaaacaaaaggtatgaattttatttaatccttgaggaaatggttcttttctcacacacataaatcactcattttgtttttctttatctcctttattaatctacattagaaaaataaacttttcatacactaagaacaaggaaaccactctcaattgacaaaatgttccaatccaacacaatgattactttcacctttaatttacaggcagccagattcaaaatccttaaagttgcttaaacttaaaaatgacaatgacaacctaaaaggtataatgttgattggaacagacatttaattggaaaattgatgattttccatttccaattaaatctctagatagaaatgaaaaaaattaaaaatcgtatttaagaaaagccaaatcttgggttgtgaggtatctttttaaggatgtttcagcagaaaaaaacaaaggctctcacaattgtgtagctgcctagattaagtgggtatcctgatcaaggagatgggggatgatttggctttagtattccaatgataaagtttataatgagaataacatgttgctacaaaatccagtctcttcctcagatgccttccacagagggcaggaagctttgtcagttttgtttgctgatgatgcctggttccgtcaacaaataacacctgataggcctggatcaagcatgcagctgtggagaacacccctgggactctaactctggcactctgcaagctgggtacttgggcaggacagcagcagcactcatgaactgggcagcacctgttggtgagggctgatcacatggattctctcatcccagccttacaatcagtccttcaggtacatactttttctgactttgctgatgaggaaactatgcacagaggttacacagcttaacaaagggttctcacctctcttcaagtggtatttaaatttcttctttcattttccttctggtaacaaagaagtctgtggctcaaaagatgtttctctaagaccccatcctattaggtctctgagctgtgggaagtatttatacaattgcttgtgaatataagatccaggaatttccctaagatccctaacaaaattggtgataagtagtcccacatgttaatccagccacccacggatgacagcacttaccatttctttgataaatgtcaaatgcatttgaagtacctacctgaaatatttgtttaaatgctatctaatctattaattttatatatgtgtgagtctgttttgtataccttctgattataggataaatgtaaataaatccaaagagtaatcaaagctaccactttcaagaagccttctttgtagaaccggaagagtcttaaataggcttttcaggtatgcatctcttattatcgctgaactccaagtcctgcaaggcaggcatcatgtgtgggtcacctttacagtaggcacaggccttaaaacagtgacatgcacattgcaggcactccataaatgtttgctgaattggctaaaccttggtttgttcccataatcaaccaccacaaacagcacacagataattacttcttggaaagattccaactagtgtttgatgttacctacgtggtttttctctcaagatcttaagagcagctctgtaggattacattattttctgttttttttttcctttgaccttaatgtcatctacttcaataacagcttcatacaaaattcctaccagcacataccacagcagattcaaggccttgttttaaaaatggtgccagcttctcttaatttggaagatatattgtctctcctgaacatgggctaagaaaatgtataatttggtattaacataagagctgaagacactttaaatgcattgtttcatttttataagataaaaaaaattttaagaatcaaaatgttatcaacagacttgtccttcattaaaaagtaaaactgcatttgcctacattttatgaaagtgtccaattatgaacaattttgaaatgtaacttttaaaaatgtaaacagcaaaaatgttgtatttaaaataaatctggaaaggcagaaaaacaaaaaatacccagaagacagagtttttggtgaaagttaagatatttcatctttgaacaacttagaatctttcctgcattttatagtctagttccaggcattaatttgaaataaccttggaatcctaaatctaacacccttcggaacaaagtagcttttctcttctgctttatgagcaaatggactaaatactagggaatggtactgtctgggcctttgaaccaagattgaaagagatgaaatcctatatgatatgtataaacattagagaatccattttgatttaataaaaggttgaatttgttctatatcctgtgagaaaatggttcccttttcctgaaaatgttacctcattccaacaatagaaagttggtttttttccagggtgtggtgttggcgggggacagagttgccatgaatatggcatctatgaagactgctgttatattcatttctcaaaatgcactgtggtaggaaattcagaacgcagtgagagaaaataaatgtttgacttcaaaatataaggccgcatttaaagcagaaggtaaagtatagaacagttgacagtataaattctttatctgcaatcttgcagttccctaaatctctgtaacacatcacttttaaaagcctcagataagtggttctataataatttaccaataattcaacccctcaaaagtcttagcaagttaaaccttataatcttacattttagaaatgacccaacttgatccttttattcttcagaatatctctctcaaattttcatttgtttttcattaattgatgaataatgagacattttaggtacctgtccacaaagaaatgaaattttcactttccaggaacctaacaaatgaaaagatagaaatcaattccaacagaatattaccaaagaaatcttttagaatggactgttaaaattatttatttgtatttatctggctctactatttgtggtacatttccacttcaaagctaaacctcaaataacatcatagtgagtggttgacttcatgtttaactgagatcttgaagactgaaaaagaccacgacaaacacacatctattttcttggctactgcatccgtgttcatcaccattctgatagtctgcaatgtattgcagctcaccctttgggaaggactaaagtagacatctgtttgttctgcttactcagcattcctaccctaattttcctttggagaacccctttattctagaccacgtgaagctaatgccaaaccccattccaggggatgcacctgaatccaacctccatcatctaaacagtgccttctccacgttcagagaagagcaagtgactcaaactgccctcataagaacagacctgggacttctgctgcaaatattgaagagtaagtactcttttttcttgctaggactaagctggtagtaccttctatgaggctatcatatggaaacaacttgtctgaaaatgaagccacaactagaaaacagatcctggtaacccggattgatggatccagccctaccttaaatggcaagacctaacccgaggctttttgcatcaaccaataaagtccttaagccagtttgagttggttttgtcacttgcagctaaaagaattctgactctaacaatgtgacaatagcaaaaataaacataactgcttttgaggtttctaatggattttcctccctatatacatgatttcatttaatcctcacaattcaggaaagcacatatctattaacattaaattaatattcattattttgaacacatgctatgtggataagggatgaggaaagccaaggaagtaatcaacgtgaaatctcacttatatgggagggaagtggaggttacatatctcagggcacttaacagatatcatcaaatgaaagaataaacagtgtgtgggagaggcagtaggtgattcttcatcaattcctggatgaaaaattaggagataatgaactccgaacaggcagcctaatgagaatggctcaagcaacaggacatagagagggagttaggttagacatggggttcttgggaattttcacctcgtgggggggcgggggggtcgtgcagctgttgtcagtgggaaagggaaaaaggaaaaggctgagtttggaaggcagggagggaggagacaatgtgagtcagtgaaaaagggcccttagaatgacaagtctggaccagagagaggctaagactgaaaatacaagttgggtaaccactggcatacagatggcagttcaggcttgggcactgcccaccagagcctcagcatgaagagaagagggggaggctggccaccacctccctctaggtaatcgtcatcctgatgctgagctcctgaaaacaggctctttcactcgccccatctcttgctcttgattgcaacccggcattcaggaggcaccctgtaatatctgtggagtgaccgacaacacagcgccagggcactgagaagatcccagggcgccagggactggttctacaagggtgcccctcccggtcccctccagcgcgccgccagagctgccagtcttggctgctacacgggaggcagcctcattatgcagctctcacctcttaaattagttcatgctctcacattaggtgtaatcacagcttgcaacgctttctggggatgtctcagaaagatctgagttgaaaaaatatttttgtgtcattttaatttaaagtaaaattgctgcttcttccccgcccctttctttcctcctggcccacccagcgaccctggccggccgtgctcaacgggggcgggggtcggaggtgagatttcctccacataattccttaaacagctatcaactaagtctcaaagaaaaaaaaaagagatctagaagcagagacgtggctgctggcgatcccaaagctggtgttcgctcttgggggagagcgtaccctgggggaggccgggaggccgggccagaggctagcccagaggcagagggcaggagcgctcagccggcgccccgcgtctctccagctcccgacgctgcgctggctccgctgagcacgccaggatcaaggtcgcctggtggggaccggagcgccaggagcctgtgggaagcgttccagccggcctctgactgggatccggcgccgcgtttctgctttggacttgactgacaggtccccccgccctcccgccgccctactaccagcctgggttcatccttcagggctacgtctaccgcacccgggctggaaagcctggagcgcgcccttcctctcctcatcttctcagctctcctttctccctgccacttggcaaagctgcattttgactttcacgttttggactacgtgtgtgtagttccaagtccatgcgtggcacgaaaatccacttagggtaaaaattattctcgaaaaatcgcccatctcaggatctggtgtctacactcaaggctaggaggtgcaggtacgggtgcgtaaagcatgccgtaagggtgcacagtaaataaaaagtacggatgcaaaatgtaaattttaagtgcaaaacagaaaagcagtactcgttgccgccccgcacgctgggttttaaggggcacgaaggtgggcctcggctgcttttgctcagccccgcgtcctcagcgcccggcccagtacccggtactccgtaggggttcaatgatctcccctgaataagtgaacgaattaacaaatgaatgaatgaccgctcgatccgacctccgcggccggcagagcagtcgctggagaggcgggagagagcgagaggccaagctccaccatcgcggccgccggctggggcagagggacacggagacactcggcgccccggctccgcaccgagtc

SEQ ID NO: 12739 - RNA, 15468 nt, Homo sapiens
  source 1..15468: mol_type = other RNA
gatctcactttgttgcccaggctggtcttaaactcctggcctcaagtgatccccttgtttcagccccgcaaagtgctgggattacaggtgtgagccaccatgcccgtgcccagccacctcatgagtcttgatggggggcagagaccaacaactccacagaagccagatgcttgctttcccagcctctcttgcagctagggcttgggcatgtgatccaggctcagccaatcagatggcactgactcttggcatgacatgggctaaggaggggctgcagggaatccatttgggctggggtggcagctgcactgggagcgacatcagtttccagagggagcagcagaatctggcatcaggcttggggcgtggtaggtgcaaccagactctgcacccagcagcagtggcagaatgggttctctgtggagagtctgtgtattgctccttccgctgaggccaccagcatctgcctccatgaacccctcagagcctgtgagcaactcaacagccttgaattttttcccttcctgtttgaatgagccagggttgtttcactgcttgaactaagagccgttcctgacatgaaaactaagccacatctttttgacccaaagattctggcatcctaaaatacccatctcattttaagttaaaaataaatccatgtttgagcatctactgtttcagttactgtgctaggtgttacaaagctaactaagagtgacaagtaaataactatcatcaccatgataaacagagaatggaaccctggtttttggaatacagacacaaaatgattaattctgcctggaagcgttttggaacatttcagagaggtagtgagctgggccaagagaagagcatacgcaaggaatggtggcatgaagttgcctggtgtgtcctgagaagaaagatgggctaagaaggactggggtagggcagagaagggggtcactggaggtgaggctgggaaagtgagccaaggctcaaatgcaaactgtctgaacttcattttctgtgcaagcaggagaagccgctgacatgggtttggaagatggactgaagccggagaaaaatggaagcaagaaaccctctcacaagaggccataaccacaaccaagtccatgagattgaaaaggaaggcagatatttgaaaaatatttaaagagatgtgaggggtaggacaggcacagtggctcatgcctgtagtcccagcactttgggaggccgaggtgggcagatccacgaggtcaggagatcaagaccatcctaacatggtaaaaccccatctctactaacaatacaaaaaattagtcaggtgtggtggcacgtgcctgtagtcccagctactcaggaggctgaggcaggagaatcgcttgaacctgggaggcggaggttgcagtgagccgagattgtgccactgcaccctagcctaggcaacagagcaagactctgtctcaaaaaaaataaaaaaaaaaaaaagagagaaagagagagagagatgaggagttgctgcactgctgggtgtggagagccgaggaggattcaaagatggtcctgaagtcccagctggaagaagtaggcggcagcaatgtttttaatactgtaaattcatcacgtagcacaggtttggggtggagaaagaaaaattgcattggcttcagggcatgcccagatctttcctcatcttaggcgtttgctaatacatgcattttctaagctgatgtcttgcgtttaatcactgctccattcaaaagagagaaggaggttgtttcaaacctagttgatatcatttgacttccatgctattcacagggctattttatttgaaacaggtataccacagccttaaattgcaagttaatccaggatgttcctaggttggcagttaggaacatgtaattctttggaagggctaaaagtcagctctttaaattatctccatatgaaccttctctccaccttagggtggatccacttatttagtccactgccagtaccacactagaacccgggtggtcactggactccagaaacaacagtagccctctctctgttctgtctctttttgactatctctattctgttcctgaccctgatttctcctgccaagctcaattttgacagctgacaacggcaagccatggcttcccaaaacattattttcaggtcaacttataaatttcaagaacacatttggctccgcttcctgtggtactaagcctacttcttgacagcatttgcctttgttgtaaatagcaaagttcttctagttggatttttgctaagaagtgtgtggatgtggcatgtgacgacatctttagcttggattctagaaaggcactaccattgtgcatttggctaaaggaaacacattttacccgtgaatgccttctatttacaaatgctcagctagcacacaaagctaagtacaagcaataagtactatcctacaatgttactcatttctgaaagcacaaaatgatgactggtatagctttggagatgttttctggaaacccaataaaggaacagatctttgttattccacacctacaaagtcagaagatgcacagtcttttattcatgtttgaacaagcttccttcttgaacaatcaactataaagtgatgtgattctctactagaccaggaactccttgaggacagaatgagggtctaatccatattctaaatccacaccacctggcacaatacatgttgcatggttagggtcaactaagagttggttgaattaatcaataacacacagcaagagaattcacaaagagaggggagtaatcccccagcctcaatcactcggcaagtggaatcgctgggcactgattccagctctgtctcagtgcttgagacagagctgaatgtaatgtgaacatttcaaatgaacaggaaaactagactcacggataagcagtgtagtcatcaagacaacactgtcttggaggtttttctgaagttaaaaccatgctacataagcaataaattatgaaggctgagcatgtgaataaaatttaatgttgtcataaattttataacaaagttaatctgacacatttaatgacatgcataatcattagtatgcagcactgtaatcagacattgataataagcagttcacaccagtgactgtaagagtctttacttgtgttcagccaagccaactgcttggtatatttttctcccttcttagtcgttagttttccatacctacaataactatcagtggtgatgggcttctctgaccatgtgaataatttaatcctcaatgcacagatacagaaacccttgctgaagacagtgtggagcagagaaggctgtctccactccttccacctgaaacacctctgcagatggatatgggagctctgcctacagcccttggacctaaccacttcagtgtgttccagtgagtgtctggacctcggcctgaaagatttttccgaaactaaagaaaatttctctgacctaaagaccttaacctccaccccagaagctctcaccaaggactacagggaactggtggggaaaatccttatcccttactcctcaaggcacagggcagtaatgctgaggcttgtgcgccacacttgctcccagaggtccccagcgggctacctgcggtggtgaatgacctcctaacacgccccttgacggccttcctttccttgcctcacttctccactctcctaccagcattgcagggttcacatcccaaatataccactggcacttgaatcctggtctccaggtctgtttctggaaaaacccaagtaagacattgccccagtaatggggctagatgtctgaggcttcctcaagtatctacctcgaaagctcttactgctgtacacacatgcacatacacacacgtgcgtacaaccagtcacatctaagcaccccgaataccagcctgttgaaggtagcagagagctgcactataagccaaggctgctcccaagagccgctccatcactgaattggcgccccagcaagatgaaggaatgtaatcattggaaggatggagaatgttctctgaatcactgacaaattggaaggggtggagggcaagagtccacctggtggagagatggaaagagcgagagagcctggaatgataatgccattgcttagaaaaggctgctccagatgccatatctacagaaattgtacagcccaaacatctctgagcaataggtctctggtagtcttgatgtctagaccaacaattcccagttcattcttctcagggaaggagccaggatagtccagagactctcattctgctgttagattgaaagggttaggcacaacagccttggcaaagtcacaagggcaaattcacactaaagtgtaaatgacccacaactcctcttctatttttaggttggggaggtgctttagaacataaggaggaactaaagaatattcctgttacatacaaggcagagaaaagggaaactagtggtgacaagacaaatcatccctttgacatttggctggctctacctattacagctctgggggtgaggtgggaacaaaaagatgctgtgtaaagaagtatcttatgccatccctactgtagtgaggtgcagtttagaggggacactgatcaagcagagacccagagtgtttcgttccaagccagaaacagaaatgtataaaacacagcctttccagcatcagaaatgagtagtggtagtggagaactacccaaaacaggaaagaggaccacgtgaggtagagtgtcaaggccctacattccagtgcctctgctcatgactgtaattttgggtaggtcacttaaagtctctggacctcagttttgccatctgtgaaatagggataatactatccagcataaaattggttatgaggctcatgtagggcctgcctgggatgatgtgttgctaatggttaagaacacaacttctggggtctgactggacaggctgaaatccctgcttaacacgttccagcagagccctgggcgatctatttaacttttgttttctcacctgtaagctgagacgaaagtacccactttataagattattccaataattagttgaaataatgcatgcagagaattaagcatggtacttgttatttgttaaactagctattaaaatgtgtaaaatataaagtattgtatggattttaggacaatgcaaagactctttgcttgctgcaatagttcggggccctttcagatggctaaaggcagaatttgtatgtgtaaatatggtgtgcttgtctctgctctggatactgagggcttaccctgttattaaacttatttagtaaatattgaactgtcatgaggcctaacatttagttccagttattagataaaacatttgctttgaatggtatttgaattgccaggttctagattattctggttgacaaactcttcgtattttataaagaggctaaaattggtaagctatcacagaacagatgtgccattttcaaggtatattaaaccatgattcactgtaacattgttcctactggcaacaaattcagagcaggctggactttatttggtgaagaaacattgagtggaagagaaatgacattattttatgtatttacattttcaaattactgtggcttaaacctgttcagccaacattacccaccttcagtctgctaaataaatgattcagtacatttctaatttacagaattttttaacaaaagaaaatgtaatttgatagccaaatcaacgttaaacattatacatttaaaaaaccacaggcaaagacacaaacatgatgacactaacttttgttaaagtatgcttacctatggtttcctctgaggcacgttctttcatgctaagcttccaacataatatgaaaatgaaggagatgcattttgcaaagcaaaacagaccttaagcaaaatattatacttctcaaattaacactgttacaaagttttagaatttaataagttcattaatttaaaagtttggatgtctgagtccttctatcccaaaacaagatcttggagggtcttccacagccatgtaataccatggtcacatgaccctttccaaaattattaatctgaatttactatatgaggataaatctatctttttgaaaatatttaggaaaatgagcttggtatttataaaatgaagctctctttgggtggtatcctaagacacgtcaagccaatcagcctgtaactgtgaaaaaaacattggtaggtacaaaagtggggtgggagaggagtgacttaactttgttaagtgatgggaaagaaacactaatagcattatctcaataaaatgtgatttaaaaaaatttaaaatactaaatcattgaactgacaaagaaatataaatcattcagaaataaactcattaggtcatcaaatcctgttaaatctgcaattaggaagagcaaggtgtacaatccatacatttaaactcacaggctcactttgcacaacgtcaatttactccttaatatgttattaatacgcattttccaaaaggatgtattagtaaatggtacacatctacttcttggcaacatcatataacctggtacaacataagcattcttcttatagttaagaaatgtggatggtatcaaaattagaaaaataaatgccctattatgttgtggtcaggtttaaggcatgtgaattttatcttcatacaaaagattaaaatctagatattaaaaagtagtgcagtatcagtgatgctgcctcagttcccaaaatgtcacatcacaaaaatatcccataattgcctgtagtttattccttggctttcctcttttctctctgcatctttgtaacaattttttaaaagtggaaatataattgttggcaatgctaacagctgtagaaatgattacaagatgtggaaaagcataacaggaatgtcaagaatctgtttctggcagtaatatatatggaacattgttcaggacaaaagaggagaaggaagaaaaaaaggagaggggtttatcatctctaagaattttcaaactaaacctcattgcttaataggaaaaaaagattccatatttaaagttaagtcacctctaactactagctaaagcatgacatcaccagcactggagtcagcggaagtgtgtttttgaaggacagtgttgcaggagaatctggacaggttttagagccaggagagagaaaataattctacctctgacagttgaaggaccttaggcaaatcagtttacctctgctagactacactccaaaatttggacattcaaaaatttgatattaataaccacatgaaagtctcgtgttgaggtgaatatgtatttgttggtgaaagatatgttggtttttaaacagacagcactctgcaattgtaggctattgttttgttttgccagttgtcaaattctatccagctatacacacttgtgtggcctcctaatggtgtttttccagtggctaaaggtttatgaataagacacttttcctaatggaattaacccgatgcttttcttaaacatgtaaccttgagttcaccgcaaaaaacaatgcttcgattagagcaatgcatataataaaggttaccctcgtttcttagacactagacatcattcacaaaaagagaactgcttttgaaagggatgtatttgcactggaaagaatagttttctacttctaattataaatgatttattggtgaaagcaaaacaacagcctgtctgagaggcacttctatgagcatcctcacgtgtgatttgcaaggttgaagaagagggaaaaatgcctcaattgtaccaatggtgagaaaacacccaaagtacaaagcaggtttcaaaaaaaccatactcataaccaaggacaataataaagcaatgtgttgacatatactctataagtcttcctccataaatagtttatagaaattttgtaatttctgtaaatgcatcctataataattttgcatcttgctttttttttacatttaatatcaagtagatttctaaagggcaattatttgaaaattatcccaaatacatggggaaatatacatcaagtgaaaaaatgcagtgggtgatagagatatcaggaagcgcctcaaatatttctcatctcgttggagaaaaacaaacatgttctcatttagaatgagtgggagttacctaattgatttaggcctctatatttaacttctagtcaaaaaaggtagttctatctagcaacaatattatggggaacaaaagaaaaaattaactctctaaatttgcagtagggtcttttcttcagaagtaccaaatcccatctattaccagctccatgcttcaggcctaaaatggatctccctgaagcaatgacagaatttttgccaagtgactaggatataaacaccactttggttgcacagtgagacatatgctccaaagaaaactggttcaaaaacaggcaagtgggtttctacagaataaatgagagccctgtcaatggcttcatcttcagggctttgtgtctgtgcttgcgtggtggctcttgtttcatctatggataatggtggcacacagttttcataattccttacattaatgaactgctataaatttgtttttggtattctagagagtcctaacttcagcttctgggcaatgctgaggaggcaccctatattctagacttaccttttgcaaggtgtactctcagcattgtgggcgatttccatgggagaatattctatttaaagaactactgtcccagcataaaacaaaaaatcatttatgaagatgcaggagactcggaaagctctcaattattgtttgcacaagcacaatgtcacagcctcctttccccattccacaagggggtcaggaagagagtactcagctgtgagaaaagacatacagaagaattcatgtggtcatgagagcgaggacatggccgatcccccaaggaggatgtgtcatacacttcatgagcccaagagtgtgctgtagggtctgaagggcaagatgctggttcactgatgtaaaggagagggaaaaaagcttcaaccaactagaaaaacagtctctatgcatgctatttttgattttaaacacaggtatcaattccttctctcagagagtccattttaaaataggatacatttttaaaggaatatttaaaggacacattcattaaaatttattttaaaaacttttcaaaagaaacaaaaggtatgaattttatttaatccttgaggaaatggttcttttctcacacacataaatcactcattttgtttttctttatctcctttattaatctacattagaaaaataaacttttcatacactaagaacaaggaaaccactctcaattgacaaaatgttccaatccaacacaatgattactttcacctttaatttacaggcagccagattcaaaatccttaaagttgcttaaacttaaaaatgacaatgacaacctaaaaggtataatgttgattggaacagacatttaattggaaaattgatgattttccatttccaattaaatctctagatagaaatgaaaaaaattaaaaatcgtatttaagaaaagccaaatcttgggttgtgaggtatctttttaaggatgtttcagcagaaaaaaacaaaggctctcacaattgtgtagctgcctagattaagtgggtatcctgatcaaggagatgggggatgatttggctttagtattccaatgataaagtttataatgagaataacatgttgctacaaaatccagtctcttcctcagatgccttccacagagggcaggaagctttgtcagttttgtttgctgatgatgcctggttccgtcaacaaataacacctgtcacacggtgggtagtcaatatacatttgttgaataaatatgaaaaaaagaaatgtacaatatgtttgtgaagccaactgtgtgtgcattgctattgaggtacacaaaaagtctttgttttaaatttgagaatgaggactttcaatggaatatatctataaaaatgaaaaaaagacattactgtctggacttttgtacagcaagagaagaaaaaccactagccaagagccaactcacctgataggcctggatcaagcatgcagctgtggagaacacccctgggactctaactctggcactctgcaagctgggtacttgggcaggacagcagcagcactcatgaactgggcagcaccgactggcaaacctccccctgaagatggagaaggaggaaggagtgttactggaatgagagcttgagtccaggggaggaggatgggctgctgaggaggcgacaccatcctgaaagaagaatcctctgccagaggcttttcagggtcatttcttcacactctctgcagggaagcacggagacagcaggaagaaatatcctaacctcactctcttccctctacaggtgcttccattggccaaatccacccagaggccagttggtggcgatcagctctcttcaagtggtatttaaatttcttctttcattttccttctggtaacaaagaagtctgtggctcaaaagatgtttctctaagaccccatcctattaggtctctgagctgtgggaagtatttatacaattgcttgtgaatataagatccaggaatttccctaagatccctaacaaaattggtgataagtagtcccacatgttaatccagccacccacggatgacagcacttaccatttctttgataaatgtcaaatgcatttgaagtacctacctgaaatatttgtttaaatgctatctaatctattaattttatatatgtgtgagtctgttttgtataccttctgattataggataaatgtaaataaatccaaagagtaatcaaagctaccactttcaagaagccttctttgtagaaccggaagagtcttaaataggcttttcaggtatgcatctcttattatcgctgaactccaagtcctgcaaggcaggcatcatgtgtgggtcacctttacagtaggcacaggccttaaaacagtgacatgcacattgcaggcactccataaatgtttgctgaattggctaaaccttggtttgttcccataatcaaccaccacaaacagcacacagataattacttcttggaaagattccaactagtgtttgatgttacctacgtggtttttctctcaagatcttaagagcagctctgtaggattacattattttctgttttttttttcctttgaccttaatgtcatctacttcaataacagcttcatacaaaattcctaccagcacataccacagcagattcaaggccttgttttaaaaatggtgccagcttctcttaatttggaagatatattgtctctcctgaacatgggctaagaaaatgtataatttggtattaacataagagctgaagacactttaaatgcattgtttcatttttataagataaaaaaaattttaagaatcaaaatgttatcaacagacttgtccttcattaaaaagtaaaactgcatttgcctacattttatgaaagtgtccaattatgaacaattttgaaatgtaacttttaaaaatgtaaacagcaaaaatgttgtatttaaaataaatctggaaaggcagaaaaacaaaaaatacccagaagacagagtttttggtgaaagttaagatatttcatctttgaacaacttagaatctttcctgcattttatagtctagttccaggcattaatttgaaataaccttggaatcctaaatctaacacccttcggaacaaagtagcttttctcttctgctttatgagcaaatggactaaatactagggaatggtactgtctgggcctttgaaccaagattgaaagagatgaaatcctatatgatatgtataaacattagagaatccattttgatttaataaaaggttgaatttgttctatatcctgtgagaaaatggttcccttttcctgaaaatgttacctcattccaacaatagaaagttggtttttttccagggtgtggtgttggcgggggacagagttgccatgaatatggcatctatgaagactgctgttatattcatttctcaaaatgcactgtggtaggaaattcagaacgcagtgagagaaaataaatgtttgacttcaaaatataaggccgcatttaaagcagaaggtaaagtatagaacagttgacagtataaattctttatctgcaatcttgcagttccctaaatctctgtaacacatcacttttaaaagcctcagataagtggttctataataatttaccaataattcaacccctcaaaagtcttagcaagttaaaccttataatcttacattttagaaatgacccaacttgatccttttattcttcagaatatctctctcaaattttcatttgtttttcattaattgatgaataatgagacattttaggtacctgtccacaaagaaatgaaattttcactttccaggaacctaacaaatgaaaagatagaaatcaattccaacagaatattaccaaagaaatcttttagaatggactgttaaaattatttatttgtatttatctggctctactatttgtggtacatttccacttcaaagctaaacctcaaataacatcatagtgagtggttgacttcatgtttaactgagatcttgaagactgaaaaagaccacgacaaacacacatctattttcttggctactgcatccgtgttcatcaccattctgatagtctgcaatgtattgcagctcaccctttgggaaggactaaagtagacatctgtttgttctgcttactcagcattcctaccctaattttcctttggagaacccctttattctagaccacgtgaagctaatgccaaaccccattccaggggatgcacctgaatccaacctccatcatctaaacagtgccttctccacgttcagagaagagcaagtgactcaaactgccctcataagaacagacctgggacttctgctgcaaatattgaagagtaagtactcttttttcttgctaggactaagctggtagtaccttctatgaggctatcatatggaaacaacttgtctgaaaatgaagccacaactagaaaacagatcctggtaacccggattgatggatccagccctaccttaaatggcaagacctaacccgaggctttttgcatcaaccaataaagtccttaagccagtttgagttggttttgtcacttgcagctaaaagaattctgactctaacaatgtgacaatagcaaaaataaacataactgcttttgaggtttctaatggattttcctccctatatacatgatttcatttaatcctcacaattcaggaaagcacatatctattaacattaaattaatattcattattttgaacacatgctatgtggataagggatgaggaaagccaaggaagtaatcaacgtgaaatctcacttatatgggagggaagtggaggttacatatctcagggcacttaacagatatcatcaaatgaaagaataaacagtgtgtgggagaggcagtaggtgattcttcatcaattcctggatgaaaaattaggagataatgaactccgaacaggcagcctaatgagaatggctcaagcaacaggacatagagagggagttaggttagacatggggttcttgggaattttcacctcgtgggggggcgggggggtcgtgcagctgttgtcagtgggaaagggaaaaaggaaaaggctgagtttggaaggcagggagggaggagacaatgtgagtcagtgaaaaagggcccttagaatgacaagtctggaccagagagaggctaagactgaaaatacaagttgggtaaccactggcatacagatggcagttcaggcttgggcactgcccaccagagcctcagcatgaagagaagagggggaggctggccaccacctccctctaggtaatcgtcatcctgatgctgagctcctgaaaacaggctctttcactcgccccatctcttgctcttgattgcaacccggcattcaggaggcaccctgtaatatctgtggagtgaccgacaacacagcgccagggcactgagaagatcccagggcgccagggactggttctacaagggtgcccctcccggtcccctccagcgcgccgccagagctgccagtcttggctgctacacgggaggcagcctcattatgcagctctcacctcttaaattagttcatgctctcacattaggtgtaatcacagcttgcaacgctttctggggatgtctcagaaagatctgagttgaaaaaatatttttgtgtcattttaatttaaagtaaaattgctgcttcttccccgcccctttctttcctcctggcccacccagcgaccctggccggccgtgctcaacgggggcgggggtcggaggtgagatttcctccacataattccttaaacagctatcaactaagtctcaaagaaaaaaaaaagagatctagaagcagagacgtggctgctggcgatcccaaagctggtgttcgctcttgggggagagcgtaccctgggggaggccgggaggccgggccagaggctagcccagaggcagagggcaggagcgctcagccggcgccccgcgtctctccagctcccgacgctgcgctggctccgctgagcacgccaggatcaaggtcgcctggtggggaccggagcgccaggagcctgtgggaagcgttccagccggcctctgactgggatccggcgccgcgtttctgctttggacttgactgacaggtccccccgccctcccgccgccctactaccagcctgggttcatccttcagggctacgtctaccgcacccgggctggaaagcctggagcgcgcccttcctctcctcatcttctcagctctcctttctccctgccacttggcaaagctgcattttgactttcacgttttggactacgtgtgtgtagttccaagtccatgcgtggcacgaaaatccacttagggtaaaaattattctcgaaaaatcgcccatctcaggatctggtgtctacactcaaggctaggaggtgcaggtacgggtgcgtaaagcatgccgtaagggtgcacagtaaataaaaagtacggatgcaaaatgtaaattttaagtgcaaaacagaaaagcagtactcgttgccgccccgcacgctgggttttaaggggcacgaaggtgggcctcggctgcttttgctcagccccgcgtcctcagcgcccggcccagtacccggtactccgtaggggttcaatgatctcccctgaataagtgaacgaattaacaaatgaatgaatgaccgctcgatccgacctccgcggccggcagagcagtcgctggagaggcgggagagagcgagaggccaagctccaccatcgcggccgccggctggggcagagggacacggagacactcggcgccccggctccgcaccgagtccccg

SEQ ID NO: 12740 - RNA, 13455 nt, Homo sapiens
  source 1..13455: mol_type = other RNA
gatctcactttgttgcccaggctggtcttaaactcctggcctcaagtgatccccttgtttcagccccgcaaagtgctgggattacaggtgtgagccaccatgcccgtgcccagccacctcatgagtcttgatggggggcagagaccaacaactccacagaagccagatgcttgctttcccagcctctcttgcagctagggcttgggcatgtgatccaggctcagccaatcagatggcactgactcttggcatgacatgggctaaggaggggctgcagggaatccatttgggctggggtggcagctgcactgggagcgacatcagtttccagagggagcagcagaatctggcatcaggcttggggcgtggtaggtgcaaccagactctgcacccagcagcagtggcagaatgggttctctgtggagagtctgtgtattgctccttccgctgaggccaccagcatctgcctccatgaacccctcagagcctgtgagcaactcaacagccttgaattttttcccttcctgtttgaatgagccagggttgtttcactgcttgaactaagagccgttcctgacatgaaaactaagccacatctttttgacccaaagattctggcatcctaaaatacccatctcattttaagttaaaaataaatccatgtttgagcatctactgtttcagttactgtgctaggtgttacaaagctaactaagagtgacaagtaaataactatcatcaccatgataaacagagaatggaaccctggtttttggaatacagacacaaaatgattaattctgcctggaagcgttttggaacatttcagagaggtagtgagctgggccaagagaagagcatacgcaaggaatggtggcatgaagttgcctggtgtgtcctgagaagaaagatgggctaagaaggactggggtagggcagagaagggggtcactggaggtgaggctgggaaagtgagccaaggctcaaatgcaaactgtctgaacttcattttctgtgcaagcaggagaagccgctgacatgggtttggaagatggactgaagccggagaaaaatggaagcaagaaaccctctcacaagaggccataaccacaaccaagtccatgagattgaaaaggaaggcagatatttgaaaaatatttaaagagatgtgaggggtaggacaggcacagtggctcatgcctgtagtcccagcactttgggaggccgaggtgggcagatccacgaggtcaggagatcaagaccatcctaacatggtaaaaccccatctctactaacaatacaaaaaattagtcaggtgtggtggcacgtgcctgtagtcccagctactcaggaggctgaggcaggagaatcgcttgaacctgggaggcggaggttgcagtgagccgagattgtgccactgcaccctagcctaggcaacagagcaagactctgtctcaaaaaaaataaaaaaaaaaaaaagagagaaagagagagagagatgaggagttgctgcactgctgggtgtggagagccgaggaggattcaaagatggtcctgaagtcccagctggaagaagtaggcggcagcaatgtttttaatactgtaaattcatcacgtagcacaggtttggggtggagaaagaaaaattgcattggcttcagggcatgcccagatctttcctcatcttaggcgtttgctaatacatgcattttctaagctgatgtcttgcgtttaatcactgctccattcaaaagagagaaggaggttgtttcaaacctagttgatatcatttgacttccatgctattcacagggctattttatttgaaacaggtataccacagccttaaattgcaagttaatccaggatgttcctaggttggcagttaggaacatgtaattctttggaagggctaaaagtcagctctttaaattatctccatatgaaccttctctccaccttagggtggatccacttatttagtccactgccagtaccacactagaacccgggtggtcactggactccagaaacaacagtagccctctctctgttctgtctctttttgactatctctattctgttcctgaccctgatttctcctgccaagctcaattttgacagctgacaacggcaagccatggcttcccaaaacattattttcaggtcaacttataaatttcaagaacacatttggctccgcttcctgtggtactaagcctacttcttgacagcatttgcctttgttgtaaatagcaaagttcttctagttggatttttgctaagaagtgtgtggatgtggcatgtgacgacatctttagcttggattctagaaaggcactaccattgtgcatttggctaaaggaaacacattttacccgtgaatgccttctatttacaaatgctcagctagcacacaaagctaagtacaagcaataagtactatcctacaatgttactcatttctgaaagcacaaaatgatgactggtatagctttggagatgttttctggaaacccaataaaggaacagatctttgttattccacacctacaaagtcagaagatgcacagtcttttattcatgtttgaacaagcttccttcttgaacaatcaactataaagtgatgtgattctctactagaccaggaactccttgaggacagaatgagggtctaatccatattctaaatccacaccacctggcacaatacatgttgcatggttagggtcaactaagagttggttgaattaatcaataacacacagcaagagaattcacaaagagaggggagtaatcccccagcctcaatcactcggcaagtggaatcgctgggcactgattccagctctgtctcagtgcttgagacagagctgaatgtaatgtgaacatttcaaatgaacaggaaaactagactcacggataagcagtgtagtcatcaagacaacactgtcttggaggtttttctgaagttaaaaccatgctacataagcaataaattatgaaggctgagcatgtgaataaaatttaatgttgtcataaattttataacaaagttaatctgacacatttaatgacatgcataatcattagtatgcagcactgtaatcagacattgataataagcagttcacaccagtgactgtaagagtctttacttgtgttcagccaagccaactgcttggtatatttttctcccttcttagtcgttagttttccatacctacaataactatcagtggtgatgggcttctctgaccatgtgaataatttaatcctcaatgcacagatacagaaacccttgctgaagacagtgtggagcagagaaggctgtctccactccttccacctgaaacacctctgcagatggatatgggagctctgcctacagcccttggacctaaccacttcagtgtgttccagtgagtgtctggacctcggcctgaaagatttttccgaaactaaagaaaatttctctgacctaaagaccttaacctccaccccagaagctctcaccaaggactacagggaactggtggggaaaatccttatcccttactcctcaaggcacagggcagtaatgctgaggcttgtgcgccacacttgctcccagaggtccccagcgggctacctgcggtggtgaatgacctcctaacacgccccttgacggccttcctttccttgcctcacttctccactctcctaccagcattgcagggttcacatcccaaatataccactggcacttgaatcctggtctccaggtctgtttctggaaaaacccaagtaagacattgccccagtaatggggctagatgtctgaggcttcctcaagtatctacctcgaaagctcttactgctgtacacacatgcacatacacacacgtgcgtacaaccagtcacatctaagcaccccgaataccagcctgttgaaggtagcagagagctgcactataagccaaggctgctcccaagagccgctccatcactgaattggcgccccagcaagatgaaggaatgtaatcattggaaggatggagaatgttctctgaatcactgacaaattggaaggggtggagggcaagagtccacctggtggagagatggaaagagcgagagagcctggaatgataatgccattgcttagaaaaggctgctccagatgccatatctacagaaattgtacagcccaaacatctctgagcaataggtctctggtagtcttgatgtctagaccaacaattcccagttcattcttctcagggaaggagccaggatagtccagagactctcattctgctgttagattgaaagggttaggcacaacagccttggcaaagtcacaagggcaaattcacactaaagtgtaaatgacccacaactcctcttctatttttaggttggggaggtgctttagaacataaggaggaactaaagaatattcctgttacatacaaggcagagaaaagggaaactagtggtgacaagacaaatcatccctttgacatttggctggctctacctattacagctctgggggtgaggtgggaacaaaaagatgctgtgtaaagaagtatcttatgccatccctactgtagtgaggtgcagtttagaggggacactgatcaagcagagacccagagtgtttcgttccaagccagaaacagaaatgtataaaacacagcctttccagcatcagaaatgagtagtggtagtggagaactacccaaaacaggaaagaggaccacgtgaggtagagtgtcaaggccctacattccagtgcctctgctcatgactgtaattttgggtaggtcacttaaagtctctggacctcagttttgccatctgtgaaatagggataatactatccagcataaaattggttatgaggctcatgtagggcctgcctgggatgatgtgttgctaatggttaagaacacaacttctggggtctgactggacaggctgaaatccctgcttaacacgttccagcagagccctgggcgatctatttaacttttgttttctcacctgtaagctgagacgaaagtacccactttataagattattccaataattagttgaaataatgcatgcagagaattaagcatggtacttgttatttgttaaactagctattaaaatgtgtaaaatataaagtattgtatggattttaggacaatgcaaagactctttgcttgctgcaatagttcggggccctttcagatggctaaaggcagaatttgtatgtgtaaatatggtgtgcttgtctctgctctggatactgagggcttaccctgttattaaacttatttagtaaatattgaactgtcatgaggcctaacatttagttccagttattagataaaacatttgctttgaatggtatttgaattgccaggttctagattattctggttgacaaactcttcgtattttataaagaggctaaaattggtaagctatcacagaacagatgtgccattttcaaggtatattaaaccatgattcactgtaacattgttcctactggcaacaaattcagagcaggctggactttatttggtgaagaaacattgagtggaagagaaatgacattattttatgtatttacattttcaaattactgtggcttaaacctgttcagccaacattacccaccttcagtctgctaaataaatgattcagtacatttctaatttacagaattttttaacaaaagaaaatgtaatttgatagccaaatcaacgttaaacattatacatttaaaaaaccacaggcaaagacacaaacatgatgacactaacttttgttaaagtatgcttacctatggtttcctctgaggcacgttctttcatgctaagcttccaacataatatgaaaatgaaggagatgcattttgcaaagcaaaacagaccttaagcaaaatattatacttctcaaattaacactgttacaaagttttagaatttaataagttcattaatttaaaagtttggatgtctgagtccttctatcccaaaacaagatcttggagggtcttccacagccatgtaataccatggtcacatgaccctttccaaaattattaatctgaatttactatatgaggataaatctatctttttgaaaatatttaggaaaatgagcttggtatttataaaatgaagctctctttgggtggtatcctaagacacgtcaagccaatcagcctgtaactgtgaaaaaaacattggtaggtacaaaagtggggtgggagaggagtgacttaactttgttaagtgatgggaaagaaacactaatagcattatctcaataaaatgtgatttaaaaaaatttaaaatactaaatcattgaactgacaaagaaatataaatcattcagaaataaactcattaggtcatcaaatcctgttaaatctgcaattaggaagagcaaggtgtacaatccatacatttaaactcacaggctcactttgcacaacgtcaatttactccttaatatgttattaatacgcattttccaaaaggatgtattagtaaatggtacacatctacttcttggcaacatcatataacctggtacaacataagcattcttcttatagttaagaaatgtggatggtatcaaaattagaaaaataaatgccctattatgttgtggtcaggtttaaggcatgtgaattttatcttcatacaaaagattaaaatctagatattaaaaagtagtgcagtatcagtgatgctgcctcagttcccaaaatgtcacatcacaaaaatatcccataattgcctgtagtttattccttggctttcctcttttctctctgcatctttgtaacaattttttaaaagtggaaatataattgttggcaatgctaacagctgtagaaatgattacaagatgtggaaaagcataacaggaatgtcaagaatctgtttctggcagtaatatatatggaacattgttcaggacaaaagaggagaaggaagaaaaaaaggagaggggtttatcatctctaagaattttcaaactaaacctcattgcttaataggaaaaaaagattccatatttaaagttaagtcacctctaactactagctaaagcatgacatcaccagcactggagtcagcggaagtgtgtttttgaaggacagtgttgcaggagaatctggacaggttttagagccaggagagagaaaataattctacctctgacagttgaaggaccttaggcaaatcagtttacctctgctagactacactccaaaatttggacattcaaaaatttgatattaataaccacatgaaagtctcgtgttgaggtgaatatgtatttgttggtgaaagatatgttggtttttaaacagacagcactctgcaattgtaggctattgttttgttttgccagttgtcaaattctatccagctatacacacttgtgtggcctcctaatggtgtttttccagtggctaaaggtttatgaataagacacttttcctaatggaattaacccgatgcttttcttaaacatgtaaccttgagttcaccgcaaaaaacaatgcttcgattagagcaatgcatataataaaggttaccctcgtttcttagacactagacatcattcacaaaaagagaactgcttttgaaagggatgtatttgcactggaaagaatagttttctacttctaattataaatgatttattggtgaaagcaaaacaacagcctgtctgagaggcacttctatgagcatcctcacgtgtgatttgcaaggttgaagaagagggaaaaatgcctcaattgtaccaatggtgagaaaacacccaaagtacaaagcaggtttcaaaaaaaccatactcataaccaaggacaataataaagcaatgtgttgacatatactctataagtcttcctccataaatagtttatagaaattttgtaatttctgtaaatgcatcctataataattttgcatcttgctttttttttacatttaatatcaagtagatttctaaagggcaattatttgaaaattatcccaaatacatggggaaatatacatcaagtgaaaaaatgcagtgggtgatagagatatcaggaagcgcctcaaatatttctcatctcgttggagaaaaacaaacatgttctcatttagaatgagtgggagttacctaattgatttaggcctctatatttaacttctagtcaaaaaaggtagttctatctagcaacaatattatggggaacaaaagaaaaaattaactctctaaatttgcagtagggtcttttcttcagaagtaccaaatcccatctattaccagctccatgcttcaggcctaaaatggatctccctgaagcaatgacagaatttttgccaagtgactaggatataaacaccactttggttgcacagtgagacatatgctccaaagaaaactggttcaaaaacaggcaagtgggtttctacagaataaatgagagccctgtcaatggcttcatcttcagggctttgtgtctgtgcttgcgtggtggctcttgtttcatctatggataatggtggcacacagttttcataattccttacattaatgaactgctataaatttgtttttggtattctagagagtcctaacttcagcttctgggcaatgctgaggaggcaccctatattctagacttaccttttgcaaggtgtactctcagcattgtgggcgatttccatgggagaatattctatttaaagaactactgtcccagcataaaacaaaaaatcatttatgaagatgcaggagactcggaaagctctcaattattgtttgcacaagcacaatgtcacagcctcctttccccattccacaagggggtcaggaagagagtactcagctgtgagaaaagacatacagaagaattcatgtggtcatgagagcgaggacatggccgatcccccaaggaggatgtgtcatacacttcatgagcccaagagtgtgctgtagggtctgaagggcaagatgctggttcactgatgtaaaggagagggaaaaaagcttcaaccaactagaaaaacagtctctatgcatgctatttttgattttaaacacaggtatcaattccttctctcagagagtccattttaaaataggatacatttttaaaggaatatttaaaggacacattcattaaaatttattttaaaaacttttcaaaagaaacaaaaggtatgaattttatttaatccttgaggaaatggttcttttctcacacacataaatcactcattttgtttttctttatctcctttattaatctacattagaaaaataaacttttcatacactaagaacaaggaaaccactctcaattgacaaaatgttccaatccaacacaatgattactttcacctttaatttacaggcagccagattcaaaatccttaaagttgcttaaacttaaaaatgacaatgacaacctaaaaggtataatgttgattggaacagacatttaattggaaaattgatgattttccatttccaattaaatctctagatagaaatgaaaaaaattaaaaatcgtatttaagaaaagccaaatcttgggttgtgaggtatctttttaaggatgtttcagcagaaaaaaacaaaggctctcacaattgtgtagctgcctagattaagtgggtatcctgatcaaggagatgggggatgatttggctttagtattccaatgataaagtttataatgagaataacatgttgctacaaaatccagtctcttcctcagatgccttccacagagggcaggaagctttgtcagttttgtttgctgatgatgcctggttccgtcaacaaataacacctgtcacacggtgggtagtcaatatacatttgttgaataaatatgaaaaaaagaaatgtacaatatgtttgtgaagccaactgtgtgtgcattgctattgaggtacacaaaaagtctttgttttaaatttgagaatgaggactttcaatggaatatatctataaaaatgaaaaaaagacattactgtctggacttttgtacagcaagagaagaaaaaccactagccaagagccaactcacctgataggcctggatcaagcatgcagctgtggagaacacccctgggactctaactctggcactctgcaagctgggtacttgggcaggacagcagcagcactcatgaactgggcagcacctctcttcaagtggtatttaaatttcttctttcattttccttctggtaacaaagaagtctgtggctcaaaagatgtttctctaagaccccatcctattaggtctctgagattttagaaatgacccaacttgatccttttattcttcagaatatctctctcaaattttcatttgtttttcattaattgatgaataatgagacattttaggtacctgtccacaaagaaatgaaattttcactttccaggaacctaacaaatgaaaagatagaaatcaattccaacagaatattaccaaagaaatcttttagaatggactgttaaaattatttatttgtatttatctggctctactatttgtggtacatttccacttcaaagctaaacctcaaataacatcatagtgagtggttgacttcatgtttaactgagatcttgaagactgaaaaagaccacgacaaacacacatctattttcttggctactgcatccgtgttcatcaccattctgatagtctgcaatgtattgcagctcaccctttgggaaggactaaagtagacatctgtttgttctgcttactcagcattcctaccctaattttcctttggagaacccctttattctagaccacgtgaagctaatgccaaaccccattccaggggatgcacctgaatccaacctccatcatctaaacagtgccttctccacgttcagagaagagcaagtgactcaaactgccctcataagaacagacctgggacttctgctgcaaatattgaagagtaagtactcttttttcttgctaggactaagctggtagtaccttctatgaggctatcatatggaaacaacttgtctgaaaatgaagccacaactagaaaacagatcctggtaacccggattgatggatccagccctaccttaaatggcaagacctaacccgaggctttttgcatcaaccaataaagtccttaagccagtttgagttggttttgtcacttgcagctaaaagaattctgactctaacaatgtgacaatagcaaaaataaacataactgcttttgaggtttctaatggattttcctccctatatacatgatttcatttaatcctcacaattcaggaaagcacatatctattaacattaaattaatattcattattttgaacacatgctatgtggataagggatgaggaaagccaaggaagtaatcaacgtgaaatctcacttatatgggagggaagtggaggttacatatctcagggcacttaacagatatcatcaaatgaaagaataaacagtgtgtgggagaggcagtaggtgattcttcatcaattcctggatgaaaaattaggagataatgaactccgaacaggcagcctaatgagaatggctcaagcaacaggacatagagagggagttaggttagacatggggttcttgggaattttcacctcgtgggggggcgggggggtcgtgcagctgttgtcagtgggaaagggaaaaaggaaaaggctgagtttggaaggcagggagggaggagacaatgtgagtcagtgaaaaagggcccttagaatgacaagtctggaccagagagaggctaagactgaaaatacaagttgggtaaccactggcatacagatggcagttcaggcttgggcactgcccaccagagcctcagcatgaagagaagagggggaggctggccaccacctccctctaggtaatcgtcatcctgatgctgagctcctgaaaacaggctctttcactcgccccatctcttgctcttgattgcaacccggcattcaggaggcaccctgtaatatctgtggagtgaccgacaacacagcgccagggcactgagaagatcccagggcgccagggactggttctacaagggtgcccctcccggtcccctccagcgcgccgccagagctgccagtcttggctgctacacgggaggcagcctcattatgcagctctcacctcttaaattagttcatgctctcacattaggtgtaatcacagcttgcaacgctttctggggatgtctcagaaagatctgagttgaaaaaatatttttgtgtcattttaatttaaagtaaaattgctgcttcttccccgcccctttctttcctcctggcccacccagcgaccctggccggccgtgctcaacgggggcgggggtcggaggtgagatttcctccacataattccttaaacagctatcaactaagtctcaaagaaaaaaaaaagagatctagaagcagagacgtggctgctggcgatcccaaagctggtgttcgctcttgggggagagcgtaccctgggggaggccgggaggccgggccagaggctagcccagaggcagagggcaggagcgctcagccggcgccccgcgtctctccagctcccgacgctgcgctggctccgctgagcacgccaggatcaaggtcgcctggtggggaccggagcgccaggagcctgtgggaagcgttccagccggcctctgactgggatccggcgccgcgtttctgctttggacttgactgacaggtccccccgccctcccgccgccctactaccagcctgggttcatccttcagggctacgtctaccgcacccgggctggaaagcctggagcgcgcccttcctctcctcatcttctcagctctcctttctccctgccacttggcaaagctgcattttgactttcacgttttggactacgtgtgtgtagttccaagtccatgcgtggcacgaaaatccacttagggtaaaaattattctcgaaaaatcgcccatctcaggatctggtgtctacactcaaggctaggaggtgcaggtacgggtgcgtaaagcatgccgtaagggtgcacagtaaataaaaagtacggatgcaaaatgtaaattttaagtgcaaaacagaaaagcagtactcgttgccgccccgcacgctgggttttaaggggcacgaaggtgggcctcggctgcttttgctcagccccgcgtcctcagcgcccggcccagtacccggtactccgtaggggttcaatgatctcccctgaataagtgaacgaattaacaaatgaatgaatgaccgctcgatccgacctccgcggccggcagagcagtcgctggagaggcgggagagagcgagaggccaagctccaccatcgcggccgccggctggggcagagggacacggagacactcggcgccccggctccgcaccgagtccccg

SEQ ID NO: 12741 - RNA, 15198 nt, Homo sapiens
  source 1..15198: mol_type = other RNA
gatctcactttgttgcccaggctggtcttaaactcctggcctcaagtgatccccttgtttcagccccgcaaagtgctgggattacaggtgtgagccaccatgcccgtgcccagccacctcatgagtcttgatggggggcagagaccaacaactccacagaagccagatgcttgctttcccagcctctcttgcagctagggcttgggcatgtgatccaggctcagccaatcagatggcactgactcttggcatgacatgggctaaggaggggctgcagggaatccatttgggctggggtggcagctgcactgggagcgacatcagtttccagagggagcagcagaatctggcatcaggcttggggcgtggtaggtgcaaccagactctgcacccagcagcagtggcagaatgggttctctgtggagagtctgtgtattgctccttccgctgaggccaccagcatctgcctccatgaacccctcagagcctgtgagcaactcaacagccttgaattttttcccttcctgtttgaatgagccagggttgtttcactgcttgaactaagagccgttcctgacatgaaaactaagccacatctttttgacccaaagattctggcatcctaaaatacccatctcattttaagttaaaaataaatccatgtttgagcatctactgtttcagttactgtgctaggtgttacaaagctaactaagagtgacaagtaaataactatcatcaccatgataaacagagaatggaaccctggtttttggaatacagacacaaaatgattaattctgcctggaagcgttttggaacatttcagagaggtagtgagctgggccaagagaagagcatacgcaaggaatggtggcatgaagttgcctggtgtgtcctgagaagaaagatgggctaagaaggactggggtagggcagagaagggggtcactggaggtgaggctgggaaagtgagccaaggctcaaatgcaaactgtctgaacttcattttctgtgcaagcaggagaagccgctgacatgggtttggaagatggactgaagccggagaaaaatggaagcaagaaaccctctcacaagaggccataaccacaaccaagtccatgagattgaaaaggaaggcagatatttgaaaaatatttaaagagatgtgaggggtaggacaggcacagtggctcatgcctgtagtcccagcactttgggaggccgaggtgggcagatccacgaggtcaggagatcaagaccatcctaacatggtaaaaccccatctctactaacaatacaaaaaattagtcaggtgtggtggcacgtgcctgtagtcccagctactcaggaggctgaggcaggagaatcgcttgaacctgggaggcggaggttgcagtgagccgagattgtgccactgcaccctagcctaggcaacagagcaagactctgtctcaaaaaaaataaaaaaaaaaaaaagagagaaagagagagagagatgaggagttgctgcactgctgggtgtggagagccgaggaggattcaaagatggtcctgaagtcccagctggaagaagtaggcggcagcaatgtttttaatactgtaaattcatcacgtagcacaggtttggggtggagaaagaaaaattgcattggcttcagggcatgcccagatctttcctcatcttaggcgtttgctaatacatgcattttctaagctgatgtcttgcgtttaatcactgctccattcaaaagagagaaggaggttgtttcaaacctagttgatatcatttgacttccatgctattcacagggctattttatttgaaacaggtataccacagccttaaattgcaagttaatccaggatgttcctaggttggcagttaggaacatgtaattctttggaagggctaaaagtcagctctttaaattatctccatatgaaccttctctccaccttagggtggatccacttatttagtccactgccagtaccacactagaacccgggtggtcactggactccagaaacaacagtagccctctctctgttctgtctctttttgactatctctattctgttcctgaccctgatttctcctgccaagctcaattttgacagctgacaacggcaagccatggcttcccaaaacattattttcaggtcaacttataaatttcaagaacacatttggctccgcttcctgtggtactaagcctacttcttgacagcatttgcctttgttgtaaatagcaaagttcttctagttggatttttgctaagaagtgtgtggatgtggcatgtgacgacatctttagcttggattctagaaaggcactaccattgtgcatttggctaaaggaaacacattttacccgtgaatgccttctatttacaaatgctcagctagcacacaaagctaagtacaagcaataagtactatcctacaatgttactcatttctgaaagcacaaaatgatgactggtatagctttggagatgttttctggaaacccaataaaggaacagatctttgttattccacacctacaaagtcagaagatgcacagtcttttattcatgtttgaacaagcttccttcttgaacaatcaactataaagtgatgtgattctctactagaccaggaactccttgaggacagaatgagggtctaatccatattctaaatccacaccacctggcacaatacatgttgcatggttagggtcaactaagagttggttgaattaatcaataacacacagcaagagaattcacaaagagaggggagtaatcccccagcctcaatcactcggcaagtggaatcgctgggcactgattccagctctgtctcagtgcttgagacagagctgaatgtaatgtgaacatttcaaatgaacaggaaaactagactcacggataagcagtgtagtcatcaagacaacactgtcttggaggtttttctgaagttaaaaccatgctacataagcaataaattatgaaggctgagcatgtgaataaaatttaatgttgtcataaattttataacaaagttaatctgacacatttaatgacatgcataatcattagtatgcagcactgtaatcagacattgataataagcagttcacaccagtgactgtaagagtctttacttgtgttcagccaagccaactgcttggtatatttttctcccttcttagtcgttagttttccatacctacaataactatcagtggtgatgggcttctctgaccatgtgaataatttaatcctcaatgcacagatacagaaacccttgctgaagacagtgtggagcagagaaggctgtctccactccttccacctgaaacacctctgcagatggatatgggagctctgcctacagcccttggacctaaccacttcagtgtgttccagtgagtgtctggacctcggcctgaaagatttttccgaaactaaagaaaatttctctgacctaaagaccttaacctccaccccagaagctctcaccaaggactacagggaactggtggggaaaatccttatcccttactcctcaaggcacagggcagtaatgctgaggcttgtgcgccacacttgctcccagaggtccccagcgggctacctgcggtggtgaatgacctcctaacacgccccttgacggccttcctttccttgcctcacttctccactctcctaccagcattgcagggttcacatcccaaatataccactggcacttgaatcctggtctccaggtctgtttctggaaaaacccaagtaagacattgccccagtaatggggctagatgtctgaggcttcctcaagtatctacctcgaaagctcttactgctgtacacacatgcacatacacacacgtgcgtacaaccagtcacatctaagcaccccgaataccagcctgttgaaggtagcagagagctgcactataagccaaggctgctcccaagagccgctccatcactgaattggcgccccagcaagatgaaggaatgtaatcattggaaggatggagaatgttctctgaatcactgacaaattggaaggggtggagggcaagagtccacctggtggagagatggaaagagcgagagagcctggaatgataatgccattgcttagaaaaggctgctccagatgccatatctacagaaattgtacagcccaaacatctctgagcaataggtctctggtagtcttgatgtctagaccaacaattcccagttcattcttctcagggaaggagccaggatagtccagagactctcattctgctgttagattgaaagggttaggcacaacagccttggcaaagtcacaagggcaaattcacactaaagtgtaaatgacccacaactcctcttctatttttaggttggggaggtgctttagaacataaggaggaactaaagaatattcctgttacatacaaggcagagaaaagggaaactagtggtgacaagacaaatcatccctttgacatttggctggctctacctattacagctctgggggtgaggtgggaacaaaaagatgctgtgtaaagaagtatcttatgccatccctactgtagtgaggtgcagtttagaggggacactgatcaagcagagacccagagtgtttcgttccaagccagaaacagaaatgtataaaacacagcctttccagcatcagaaatgagtagtggtagtggagaactacccaaaacaggaaagaggaccacgtgaggtagagtgtcaaggccctacattccagtgcctctgctcatgactgtaattttgggtaggtcacttaaagtctctggacctcagttttgccatctgtgaaatagggataatactatccagcataaaattggttatgaggctcatgtagggcctgcctgggatgatgtgttgctaatggttaagaacacaacttctggggtctgactggacaggctgaaatccctgcttaacacgttccagcagagccctgggcgatctatttaacttttgttttctcacctgtaagctgagacgaaagtacccactttataagattattccaataattagttgaaataatgcatgcagagaattaagcatggtacttgttatttgttaaactagctattaaaatgtgtaaaatataaagtattgtatggattttaggacaatgcaaagactctttgcttgctgcaatagttcggggccctttcagatggctaaaggcagaatttgtatgtgtaaatatggtgtgcttgtctctgctctggatactgagggcttaccctgttattaaacttatttagtaaatattgaactgtcatgaggcctaacatttagttccagttattagataaaacatttgctttgaatggtatttgaattgccaggttctagattattctggttgacaaactcttcgtattttataaagaggctaaaattggtaagctatcacagaacagatgtgccattttcaaggtatattaaaccatgattcactgtaacattgttcctactggcaacaaattcagagcaggctggactttatttggtgaagaaacattgagtggaagagaaatgacattattttatgtatttacattttcaaattactgtggcttaaacctgttcagccaacattacccaccttcagtctgctaaataaatgattcagtacatttctaatttacagaattttttaacaaaagaaaatgtaatttgatagccaaatcaacgttaaacattatacatttaaaaaaccacaggcaaagacacaaacatgatgacactaacttttgttaaagtatgcttacctatggtttcctctgaggcacgttctttcatgctaagcttccaacataatatgaaaatgaaggagatgcattttgcaaagcaaaacagaccttaagcaaaatattatacttctcaaattaacactgttacaaagttttagaatttaataagttcattaatttaaaagtttggatgtctgagtccttctatcccaaaacaagatcttggagggtcttccacagccatgtaataccatggtcacatgaccctttccaaaattattaatctgaatttactatatgaggataaatctatctttttgaaaatatttaggaaaatgagcttggtatttataaaatgaagctctctttgggtggtatcctaagacacgtcaagccaatcagcctgtaactgtgaaaaaaacattggtaggtacaaaagtggggtgggagaggagtgacttaactttgttaagtgatgggaaagaaacactaatagcattatctcaataaaatgtgatttaaaaaaatttaaaatactaaatcattgaactgacaaagaaatataaatcattcagaaataaactcattaggtcatcaaatcctgttaaatctgcaattaggaagagcaaggtgtacaatccatacatttaaactcacaggctcactttgcacaacgtcaatttactccttaatatgttattaatacgcattttccaaaaggatgtattagtaaatggtacacatctacttcttggcaacatcatataacctggtacaacataagcattcttcttatagttaagaaatgtggatggtatcaaaattagaaaaataaatgccctattatgttgtggtcaggtttaaggcatgtgaattttatcttcatacaaaagattaaaatctagatattaaaaagtagtgcagtatcagtgatgctgcctcagttcccaaaatgtcacatcacaaaaatatcccataattgcctgtagtttattccttggctttcctcttttctctctgcatctttgtaacaattttttaaaagtggaaatataattgttggcaatgctaacagctgtagaaatgattacaagatgtggaaaagcataacaggaatgtcaagaatctgtttctggcagtaatatatatggaacattgttcaggacaaaagaggagaaggaagaaaaaaaggagaggggtttatcatctctaagaattttcaaactaaacctcattgcttaataggaaaaaaagattccatatttaaagttaagtcacctctaactactagctaaagcatgacatcaccagcactggagtcagcggaagtgtgtttttgaaggacagtgttgcaggagaatctggacaggttttagagccaggagagagaaaataattctacctctgacagttgaaggaccttaggcaaatcagtttacctctgctagactacactccaaaatttggacattcaaaaatttgatattaataaccacatgaaagtctcgtgttgaggtgaatatgtatttgttggtgaaagatatgttggtttttaaacagacagcactctgcaattgtaggctattgttttgttttgccagttgtcaaattctatccagctatacacacttgtgtggcctcctaatggtgtttttccagtggctaaaggtttatgaataagacacttttcctaatggaattaacccgatgcttttcttaaacatgtaaccttgagttcaccgcaaaaaacaatgcttcgattagagcaatgcatataataaaggttaccctcgtttcttagacactagacatcattcacaaaaagagaactgcttttgaaagggatgtatttgcactggaaagaatagttttctacttctaattataaatgatttattggtgaaagcaaaacaacagcctgtctgagaggcacttctatgagcatcctcacgtgtgatttgcaaggttgaagaagagggaaaaatgcctcaattgtaccaatggtgagaaaacacccaaagtacaaagcaggtttcaaaaaaaccatactcataaccaaggacaataataaagcaatgtgttgacatatactctataagtcttcctccataaatagtttatagaaattttgtaatttctgtaaatgcatcctataataattttgcatcttgctttttttttacatttaatatcaagtagatttctaaagggcaattatttgaaaattatcccaaatacatggggaaatatacatcaagtgaaaaaatgcagtgggtgatagagatatcaggaagcgcctcaaatatttctcatctcgttggagaaaaacaaacatgttctcatttagaatgagtgggagttacctaattgatttaggcctctatatttaacttctagtcaaaaaaggtagttctatctagcaacaatattatggggaacaaaagaaaaaattaactctctaaatttgcagtagggtcttttcttcagaagtaccaaatcccatctattaccagctccatgcttcaggcctaaaatggatctccctgaagcaatgacagaatttttgccaagtgactaggatataaacaccactttggttgcacagtgagacatatgctccaaagaaaactggttcaaaaacaggcaagtgggtttctacagaataaatgagagccctgtcaatggcttcatcttcagggctttgtgtctgtgcttgcgtggtggctcttgtttcatctatggataatggtggcacacagttttcataattccttacattaatgaactgctataaatttgtttttggtattctagagagtcctaacttcagcttctgggcaatgctgaggaggcaccctatattctagacttaccttttgcaaggtgtactctcagcattgtgggcgatttccatgggagaatattctatttaaagaactactgtcccagcataaaacaaaaaatcatttatgaagatgcaggagactcggaaagctctcaattattgtttgcacaagcacaatgtcacagcctcctttccccattccacaagggggtcaggaagagagtactcagctgtgagaaaagacatacagaagaattcatgtggtcatgagagcgaggacatggccgatcccccaaggaggatgtgtcatacacttcatgagcccaagagtgtgctgtagggtctgaagggcaagatgctggttcactgatgtaaaggagagggaaaaaagcttcaaccaactagaaaaacagtctctatgcatgctatttttgattttaaacacaggtatcaattccttctctcagagagtccattttaaaataggatacatttttaaaggaatatttaaaggacacattcattaaaatttattttaaaaacttttcaaaagaaacaaaaggtatgaattttatttaatccttgaggaaatggttcttttctcacacacataaatcactcattttgtttttctttatctcctttattaatctacattagaaaaataaacttttcatacactaagaacaaggaaaccactctcaattgacaaaatgttccaatccaacacaatgattactttcacctttaatttacaggcagccagattcaaaatccttaaagttgcttaaacttaaaaatgacaatgacaacctaaaaggtataatgttgattggaacagacatttaattggaaaattgatgattttccatttccaattaaatctctagatagaaatgaaaaaaattaaaaatcgtatttaagaaaagccaaatcttgggttgtgaggtatctttttaaggatgtttcagcagaaaaaaacaaaggctctcacaattgtgtagctgcctagattaagtgggtatcctgatcaaggagatgggggatgatttggctttagtattccaatgataaagtttataatgagaataacatgttgctacaaaatccagtctcttcctcagatgccttccacagagggcaggaagctttgtcagttttgtttgctgatgatgcctggttccgtcaacaaataacacctgtcacacggtgggtagtcaatatacatttgttgaataaatatgaaaaaaagaaatgtacaatatgtttgtgaagccaactgtgtgtgcattgctattgaggtacacaaaaagtctttgttttaaatttgagaatgaggactttcaatggaatatatctataaaaatgaaaaaaagacattactgtctggacttttgtacagcaagagaagaaaaaccactagccaagagccaactcacctgataggcctggatcaagcatgcagctgtggagaacacccctgggactctaactctggcactctgcaagctgggtacttgggcaggacagcagcagcactcatgaactgggcagcacctctcttcaagtggtatttaaatttcttctttcattttccttctggtaacaaagaagtctgtggctcaaaagatgtttctctaagaccccatcctattaggtctctgagctgtgggaagtatttatacaattgcttgtgaatataagatccaggaatttccctaagatccctaacaaaattggtgataagtagtcccacatgttaatccagccacccacggatgacagcacttaccatttctttgataaatgtcaaatgcatttgaagtacctacctgaaatatttgtttaaatgctatctaatctattaattttatatatgtgtgagtctgttttgtataccttctgattataggataaatgtaaataaatccaaagagtaatcaaagctaccactttcaagaagccttctttgtagaaccggaagagtcttaaataggcttttcaggtatgcatctcttattatcgctgaactccaagtcctgcaaggcaggcatcatgtgtgggtcacctttacagtaggcacaggccttaaaacagtgacatgcacattgcaggcactccataaatgtttgctgaattggctaaaccttggtttgttcccataatcaaccaccacaaacagcacacagataattacttcttggaaagattccaactagtgtttgatgttacctacgtggtttttctctcaagatcttaagagcagctctgtaggattacattattttctgttttttttttcctttgaccttaatgtcatctacttcaataacagcttcatacaaaattcctaccagcacataccacagcagattcaaggccttgttttaaaaatggtgccagcttctcttaatttggaagatatattgtctctcctgaacatgggctaagaaaatgtataatttggtattaacataagagctgaagacactttaaatgcattgtttcatttttataagataaaaaaaattttaagaatcaaaatgttatcaacagacttgtccttcattaaaaagtaaaactgcatttgcctacattttatgaaagtgtccaattatgaacaattttgaaatgtaacttttaaaaatgtaaacagcaaaaatgttgtatttaaaataaatctggaaaggcagaaaaacaaaaaatacccagaagacagagtttttggtgaaagttaagatatttcatctttgaacaacttagaatctttcctgcattttatagtctagttccaggcattaatttgaaataaccttggaatcctaaatctaacacccttcggaacaaagtagcttttctcttctgctttatgagcaaatggactaaatactagggaatggtactgtctgggcctttgaaccaagattgaaagagatgaaatcctatatgatatgtataaacattagagaatccattttgatttaataaaaggttgaatttgttctatatcctgtgagaaaatggttcccttttcctgaaaatgttacctcattccaacaatagaaagttggtttttttccagggtgtggtgttggcgggggacagagttgccatgaatatggcatctatgaagactgctgttatattcatttctcaaaatgcactgtggtaggaaattcagaacgcagtgagagaaaataaatgtttgacttcaaaatataaggccgcatttaaagcagaaggtaaagtatagaacagttgacagtataaattctttatctgcaatcttgcagttccctaaatctctgtaacacatcacttttaaaagcctcagataagtggttctataataatttaccaataattcaacccctcaaaagtcttagcaagttaaaccttataatcttacattttagaaatgacccaacttgatccttttattcttcagaatatctctctcaaattttcatttgtttttcattaattgatgaataatgagacattttaggtacctgtccacaaagaaatgaaattttcactttccaggaacctaacaaatgaaaagatagaaatcaattccaacagaatattaccaaagaaatcttttagaatggactgttaaaattatttatttgtatttatctggctctactatttgtggtacatttccacttcaaagctaaacctcaaataacatcatagtgagtggttgacttcatgtttaactgagatcttgaagactgaaaaagaccacgacaaacacacatctattttcttggctactgcatccgtgttcatcaccattctgatagtctgcaatgtattgcagctcaccctttgggaaggactaaagtagacatctgtttgttctgcttactcagcattcctaccctaattttcctttggagaacccctttattctagaccacgtgaagctaatgccaaaccccattccaggggatgcacctgaatccaacctccatcatctaaacagtgccttctccacgttcagagaagagcaagtgactcaaactgccctcataagaacagacctgggacttctgctgcaaatattgaagagtaagtactcttttttcttgctaggactaagctggtagtaccttctatgaggctatcatatggaaacaacttgtctgaaaatgaagccacaactagaaaacagatcctggtaacccggattgatggatccagccctaccttaaatggcaagacctaacccgaggctttttgcatcaaccaataaagtccttaagccagtttgagttggttttgtcacttgcagctaaaagaattctgactctaacaatgtgacaatagcaaaaataaacataactgcttttgaggtttctaatggattttcctccctatatacatgatttcatttaatcctcacaattcaggaaagcacatatctattaacattaaattaatattcattattttgaacacatgctatgtggataagggatgaggaaagccaaggaagtaatcaacgtgaaatctcacttatatgggagggaagtggaggttacatatctcagggcacttaacagatatcatcaaatgaaagaataaacagtgtgtgggagaggcagtaggtgattcttcatcaattcctggatgaaaaattaggagataatgaactccgaacaggcagcctaatgagaatggctcaagcaacaggacatagagagggagttaggttagacatggggttcttgggaattttcacctcgtgggggggcgggggggtcgtgcagctgttgtcagtgggaaagggaaaaaggaaaaggctgagtttggaaggcagggagggaggagacaatgtgagtcagtgaaaaagggcccttagaatgacaagtctggaccagagagaggctaagactgaaaatacaagttgggtaaccactggcatacagatggcagttcaggcttgggcactgcccaccagagcctcagcatgaagagaagagggggaggctggccaccacctccctctaggtaatcgtcatcctgatgctgagctcctgaaaacaggctctttcactcgccccatctcttgctcttgattgcaacccggcattcaggaggcaccctgtaatatctgtggagtgaccgacaacacagcgccagggcactgagaagatcccagggcgccagggactggttctacaagggtgcccctcccggtcccctccagcgcgccgccagagctgccagtcttggctgctacacgggaggcagcctcattatgcagctctcacctcttaaattagttcatgctctcacattaggtgtaatcacagcttgcaacgctttctggggatgtctcagaaagatctgagttgaaaaaatatttttgtgtcattttaatttaaagtaaaattgctgcttcttccccgcccctttctttcctcctggcccacccagcgaccctggccggccgtgctcaacgggggcgggggtcggaggtgagatttcctccacataattccttaaacagctatcaactaagtctcaaagaaaaaaaaaagagatctagaagcagagacgtggctgctggcgatcccaaagctggtgttcgctcttgggggagagcgtaccctgggggaggccgggaggccgggccagaggctagcccagaggcagagggcaggagcgctcagccggcgccccgcgtctctccagctcccgacgctgcgctggctccgctgagcacgccaggatcaaggtcgcctggtggggaccggagcgccaggagcctgtgggaagcgttccagccggcctctgactgggatccggcgccgcgtttctgctttggacttgactgacaggtccccccgccctcccgccgccctactaccagcctgggttcatccttcagggctacgtctaccgcacccgggctggaaagcctggagcgcgcccttcctctcctcatcttctcagctctcctttctccctgccacttggcaaagctgcattttgactttcacgttttggactacgtgtgtgtagttccaagtccatgcgtggcacgaaaatccacttagggtaaaaattattctcgaaaaatcgcccatctcaggatctggtgtctacactcaaggctaggaggtgcaggtacgggtgcgtaaagcatgccgtaagggtgcacagtaaataaaaagtacggatgcaaaatgtaaattttaagtgcaaaacagaaaagcagtactcgttgccgccccgcacgctgggttttaaggggcacgaaggtgggcctcggctgcttttgctcagccccgcgtcctcagcgcccggcccagtacccggtactccgtaggggttcaatgatctcccctgaataagtgaacgaattaacaaatgaatgaatgaccgctcgatccgacctccgcggccggcagagcagtcgctggagaggcgggagagagcgagaggccaagctccaccatcgcggccgccggctggggcagagggacacggagacactcggcgccccggctccgcaccgagtccccg

SEQ ID NO: 12742 - RNA, 12314 nt, Homo sapiens
  source 1..12314: mol_type = other RNA
gatctcactttgttgcccaggctggtcttaaactcctggcctcaagtgatccccttgtttcagccccgcaaagtgctgggattacaggtgtgagccaccatgcccgtgcccagccacctcatgagtcttgatggggggcagagaccaacaactccacagaagccagatgcttgctttcccagcctctcttgcagctagggcttgggcatgtgatccaggctcagccaatcagatggcactgactcttggcatgacatgggctaaggaggggctgcagggaatccatttgggctggggtggcagctgcactgggagcgacatcagtttccagagggagcagcagaatctggcatcaggcttggggcgtggtaggtgcaaccagactctgcacccagcagcagtggcagaatgggttctctgtggagagtctgtgtattgctccttccgctgaggccaccagcatctgcctccatgaacccctcagagcctgtgagcaactcaacagccttgaattttttcccttcctgtttgaatgagccagggttgtttcactgcttgaactaagagccgttcctgacatgaaaactaagccacatctttttgacccaaagattctggcatcctaaaatacccatctcattttaagttaaaaataaatccatgtttgagcatctactgtttcagttactgtgctaggtgttacaaagctaactaagagtgacaagtaaataactatcatcaccatgataaacagagaatggaaccctggtttttggaatacagacacaaaatgattaattctgcctggaagcgttttggaacatttcagagaggtagtgagctgggccaagagaagagcatacgcaaggaatggtggcatgaagttgcctggtgtgtcctgagaagaaagatgggctaagaaggactggggtagggcagagaagggggtcactggaggtgaggctgggaaagtgagccaaggctcaaatgcaaactgtctgaacttcattttctgtgcaagcaggagaagccgctgacatgggtttggaagatggactgaagccggagaaaaatggaagcaagaaaccctctcacaagaggccataaccacaaccaagtccatgagattgaaaaggaaggcagatatttgaaaaatatttaaagagatgtgaggggtaggacaggcacagtggctcatgcctgtagtcccagcactttgggaggccgaggtgggcagatccacgaggtcaggagatcaagaccatcctaacatggtaaaaccccatctctactaacaatacaaaaaattagtcaggtgtggtggcacgtgcctgtagtcccagctactcaggaggctgaggcaggagaatcgcttgaacctgggaggcggaggttgcagtgagccgagattgtgccactgcaccctagcctaggcaacagagcaagactctgtctcaaaaaaaataaaaaaaaaaaaaagagagaaagagagagagagatgaggagttgctgcactgctgggtgtggagagccgaggaggattcaaagatggtcctgaagtcccagctggaagaagtaggcggcagcaatgtttttaatactgtaaattcatcacgtagcacaggtttggggtggagaaagaaaaattgcattggcttcagggcatgcccagatctttcctcatcttaggcgtttgctaatacatgcattttctaagctgatgtcttgcgtttaatcactgctccattcaaaagagagaaggaggttgtttcaaacctagttgatatcatttgacttccatgctattcacagggctattttatttgaaacaggtataccacagccttaaattgcaagttaatccaggatgttcctaggttggcagttaggaacatgtaattctttggaagggctaaaagtcagctctttaaattatctccatatgaaccttctctccaccttagggtggatccacttatttagtccactgccagtaccacactagaacccgggtggtcactggactccagaaacaacagtagccctctctctgttctgtctctttttgactatctctattctgttcctgaccctgatttctcctgccaagctcaattttgacagctgacaacggcaagccatggcttcccaaaacattattttcaggtcaacttataaatttcaagaacacatttggctccgcttcctgtggtactaagcctacttcttgacagcatttgcctttgttgtaaatagcaaagttcttctagttggatttttgctaagaagtgtgtggatgtggcatgtgacgacatctttagcttggattctagaaaggcactaccattgtgcatttggctaaaggaaacacattttacccgtgaatgccttctatttacaaatgctcagctagcacacaaagctaagtacaagcaataagtactatcctacaatgttactcatttctgaaagcacaaaatgatgactggtatagctttggagatgttttctggaaacccaataaaggaacagatctttgttattccacacctacaaagtcagaagatgcacagtcttttattcatgtttgaacaagcttccttcttgaacaatcaactataaagtgatgtgattctctactagaccaggaactccttgaggacagaatgagggtctaatccatattctaaatccacaccacctggcacaatacatgttgcatggttagggtcaactaagagttggttgaattaatcaataacacacagcaagagaattcacaaagagaggggagtaatcccccagcctcaatcactcggcaagtggaatcgctgggcactgattccagctctgtctcagtgcttgagacagagctgaatgtaatgtgaacatttcaaatgaacaggaaaactagactcacggataagcagtgtagtcatcaagacaacactgtcttggaggtttttctgaagttaaaaccatgctacataagcaataaattatgaaggctgagcatgtgaataaaatttaatgttgtcataaattttataacaaagttaatctgacacatttaatgacatgcataatcattagtatgcagcactgtaatcagacattgataataagcagttcacaccagtgactgtaagagtctttacttgtgttcagccaagccaactgcttggtatatttttctcccttcttagtcgttagttttccatacctacaataactatcagtggtgatgggcttctctgaccatgtgaataatttaatcctcaatgcacagatacagaaacccttgctgaagacagtgtggagcagagaaggctgtctccactccttccacctgaaacacctctgcagatggatatgggagctctgcctacagcccttggacctaaccacttcagtgtgttccagtgagtgtctggacctcggcctgaaagatttttccgaaactaaagaaaatttctctgacctaaagaccttaacctccaccccagaagctctcaccaaggactacagggaactggtggggaaaatccttatcccttactcctcaaggcacagggcagtaatgctgaggcttgtgcgccacacttgctcccagaggtccccagcgggctacctgcggtggtgaatgacctcctaacacgccccttgacggccttcctttccttgcctcacttctccactctcctaccagcattgcagggttcacatcccaaatataccactggcacttgaatcctggtctccaggtctgtttctggaaaaacccaagtaagacattgccccagtaatggggctagatgtctgaggcttcctcaagtatctacctcgaaagctcttactgctgtacacacatgcacatacacacacgtgcgtacaaccagtcacatctaagcaccccgaataccagcctgttgaaggtagcagagagctgcactataagccaaggctgctcccaagagccgctccatcactgaattggcgccccagcaagatgaaggaatgtaatcattggaaggatggagaatgttctctgaatcactgacaaattggaaggggtggagggcaagagtccacctggtggagagatggaaagagcgagagagcctggaatgataatgccattgcttagaaaaggctgctccagatgccatatctacagaaattgtacagcccaaacatctctgagcaataggtctctggtagtcttgatgtctagaccaacaattcccagttcattcttctcagggaaggagccaggatagtccagagactctcattctgctgttagattgaaagggttaggcacaacagccttggcaaagtcacaagggcaaattcacactaaagtgtaaatgacccacaactcctcttctatttttaggttggggaggtgctttagaacataaggaggaactaaagaatattcctgttacatacaaggcagagaaaagggaaactagtggtgacaagacaaatcatccctttgacatttggctggctctacctattacagctctgggggtgaggtgggaacaaaaagatgctgtgtaaagaagtatcttatgccatccctactgtagtgaggtgcagtttagaggggacactgatcaagcagagacccagagtgtttcgttccaagccagaaacagaaatgtataaaacacagcctttccagcatcagaaatgagtagtggtagtggagaactacccaaaacaggaaagaggaccacgtgaggtagagtgtcaaggccctacattccagtgcctctgctcatgactgtaattttgggtaggtcacttaaagtctctggacctcagttttgccatctgtgaaatagggataatactatccagcataaaattggttatgaggctcatgtagggcctgcctgggatgatgtgttgctaatggttaagaacacaacttctggggtctgactggacaggctgaaatccctgcttaacacgttccagcagagccctgggcgatctatttaacttttgttttctcacctgtaagctgagacgaaagtacccactttataagattattccaataattagttgaaataatgcatgcagagaattaagcatggtacttgttatttgttaaactagctattaaaatgtgtaaaatataaagtattgtatggattttaggacaatgcaaagactctttgcttgctgcaatagttcggggccctttcagatggctaaaggcagaatttgtatgtgtaaatatggtgtgcttgtctctgctctggatactgagggcttaccctgttattaaacttatttagtaaatattgaactgtcatgaggcctaacatttagttccagttattagataaaacatttgctttgaatggtatttgaattgccaggttctagattattctggttgacaaactcttcgtattttataaagaggctaaaattggtaagctatcacagaacagatgtgccattttcaaggtatattaaaccatgattcactgtaacattgttcctactggcaacaaattcagagcaggctggactttatttggtgaagaaacattgagtggaagagaaatgacattattttatgtatttacattttcaaattactgtggcttaaacctgttcagccaacattacccaccttcagtctgctaaataaatgattcagtacatttctaatttacagaattttttaacaaaagaaaatgtaatttgatagccaaatcaacgttaaacattatacatttaaaaaaccacaggcaaagacacaaacatgatgacactaacttttgttaaagtatgcttacctatggtttcctctgaggcacgttctttcatgctaagcttccaacataatatgaaaatgaaggagatgcattttgcaaagcaaaacagaccttaagcaaaatattatacttctcaaattaacactgttacaaagttttagaatttaataagttcattaatttaaaagtttggatgtctgagtccttctatcccaaaacaagatcttggagggtcttccacagccatgtaataccatggtcacatgaccctttccaaaattattaatctgaatttactatatgaggataaatctatctttttgaaaatatttaggaaaatgagcttggtatttataaaatgaagctctctttgggtggtatcctaagacacgtcaagccaatcagcctgtaactgtgaaaaaaacattggtaggtacaaaagtggggtgggagaggagtgacttaactttgttaagtgatgggaaagaaacactaatagcattatctcaataaaatgtgatttaaaaaaatttaaaatactaaatcattgaactgacaaagaaatataaatcattcagaaataaactcattaggtcatcaaatcctgttaaatctgcaattaggaagagcaaggtgtacaatccatacatttaaactcacaggctcactttgcacaacgtcaatttactccttaatatgttattaatacgcattttccaaaaggatgtattagtaaatggtacacatctacttcttggcaacatcatataacctggtacaacataagcattcttcttatagttaagaaatgtggatggtatcaaaattagaaaaataaatgccctattatgttgtggtcaggtttaaggcatgtgaattttatcttcatacaaaagattaaaatctagatattaaaaagtagtgcagtatcagtgatgctgcctcagttcccaaaatgtcacatcacaaaaatatcccataattgcctgtagtttattccttggctttcctcttttctctctgcatctttgtaacaattttttaaaagtggaaatataattgttggcaatgctaacagctgtagaaatgattacaagatgtggaaaagcataacaggaatgtcaagaatctgtttctggcagtaatatatatggaacattgttcaggacaaaagaggagaaggaagaaaaaaaggagaggggtttatcatctctaagaattttcaaactaaacctcattgcttaataggaaaaaaagattccatatttaaagttaagtcacctctaactactagctaaagcatgacatcaccagcactggagtcagcggaagtgtgtttttgaaggacagtgttgcaggagaatctggacaggttttagagccaggagagagaaaataattctacctctgacagttgaaggaccttaggcaaatcagtttacctctgctagactacactccaaaatttggacattcaaaaatttgatattaataaccacatgaaagtctcgtgttgaggtgaatatgtatttgttggtgaaagatatgttggtttttaaacagacagcactctgcaattgtaggctattgttttgttttgccagttgtcaaattctatccagctatacacacttgtgtggcctcctaatggtgtttttccagtggctaaaggtttatgaataagacacttttcctaatggaattaacccgatgcttttcttaaacatgtaaccttgagttcaccgcaaaaaacaatgcttcgattagagcaatgcatataataaaggttaccctcgtttcttagacactagacatcattcacaaaaagagaactgcttttgaaagggatgtatttgcactggaaagaatagttttctacttctaattataaatgatttattggtgaaagcaaaacaacagcctgtctgagaggcacttctatgagcatcctcacgtgtgatttgcaaggttgaagaagagggaaaaatgcctcaattgtaccaatggtgagaaaacacccaaagtacaaagcaggtttcaaaaaaaccatactcataaccaaggacaataataaagcaatgtgttgacatatactctataagtcttcctccataaatagtttatagaaattttgtaatttctgtaaatgcatcctataataattttgcatcttgctttttttttacatttaatatcaagtagatttctaaagggcaattatttgaaaattatcccaaatacatggggaaatatacatcaagtgaaaaaatgcagtgggtgatagagatatcaggaagcgcctcaaatatttctcatctcgttggagaaaaacaaacatgttctcatttagaatgagtgggagttacctaattgatttaggcctctatatttaacttctagtcaaaaaaggtagttctatctagcaacaatattatggggaacaaaagaaaaaattaactctctaaatttgcagtagggtcttttcttcagaagtaccaaatcccatctattaccagctccatgcttcaggcctaaaatggatctccctgaagcaatgacagaatttttgccaagtgactaggatataaacaccactttggttgcacagtgagacatatgctccaaagaaaactggttcaaaaacaggcaagtgggtttctacagaataaatgagagccctgtcaatggcttcatcttcagggctttgtgtctgtgcttgcgtggtggctcttgtttcatctatggataatggtggcacacagttttcataattccttacattaatgaactgctataaatttgtttttggtattctagagagtcctaacttcagcttctgggcaatgctgaggaggcaccctatattctagacttaccttttgcaaggtgtactctcagcattgtgggcgatttccatgggagaatattctatttaaagaactactgtcccagcataaaacaaaaaatcatttatgaagatgcaggagactcggaaagctctcaattattgtttgcacaagcacaatgtcacagcctcctttccccattccacaagggggtcaggaagagagtactcagctgtgagaaaagacatacagaagaattcatgtggtcatgagagcgaggacatggccgatcccccaaggaggatgtgtcatacacttcatgagcccaagagtgtgctgtagggtctgaagggcaagatgctggttcactgatgtaaaggagagggaaaaaagcttcaaccaactagaaaaacagtctctatgcatgctatttttgattttaaacacaggtatcaattccttctctcagagagtccattttaaaataggatacatttttaaaggaatatttaaaggacacattcattaaaatttattttaaaaacttttcaaaagaaacaaaaggtatgaattttatttaatccttgaggaaatggttcttttctcacacacataaatcactcattttgtttttctttatctcctttattaatctacattagaaaaataaacttttcatacactaagaacaaggaaaccactctcaattgacaaaatgttccaatccaacacaatgattactttcacctttaatttacaggcagccagattcaaaatccttaaagttgcttaaacttaaaaatgacaatgacaacctaaaaggtataatgttgattggaacagacatttaattggaaaattgatgattttccatttccaattaaatctctagatagaaatgaaaaaaattaaaaatcgtatttaagaaaagccaaatcttgggttgtgaggtatctttttaaggatgtttcagcagaaaaaaacaaaggctctcacaattgtgtagctgcctagattaagtgggtatcctgatcaaggagatgggggatgatttggctttagtattccaatgataaagtttataatgagaataacatgttgctacaaaatccagtctcttcctcagatgccttccacagagggcaggaagctttgtcagttttgtttgctgatgatgcctggttccgtcaacaaataacacctgtcacacggtgggtagtcaatatacatttgttgaataaatatgaaaaaaagaaatgtacaatatgtttgtgaagccaactgtgtgtgcattgctattgaggtacacaaaaagtctttgttttaaatttgagaatgaggactttcaatggaatatatctataaaaatgaaaaaaagacattactgtctggacttttgtacagcaagagaagaaaaaccactagccaagagccaactcacctgataggcctggatcaagcatgcagctgtggagaacacccctgggactctaactctggcactctgcaagctgggtacttgggcaggacagcagcagcactcatgaactgggcagcacctgttggtgagggctgatcacatggattctctcatcccagccttacaatcagtccttcaggtacatactttttctgactttgctgatgaggaaactatgcacagaggttacacagcttaacaaagggttctcacctaatgaacaatgaaatgggattttagcctttctttgcatctggtcttagagccaatacccaagaagcactgtactgtatgcattgtctcagagaaacttactcttcctgggcctcagtctttaaaaggtgggcagttgacttaataagaattaaagatcaatgattaaggttcaaggcactccaaaattctggtctttattgaaaaggctacagaagtctcaccttaataataccctatagacttgatattcttggttaattaaatattggaaaccaatttcatagtaattgaggtcagaaaaaagtactcatgacattttagaatatgatgacaaagccatagataaatttcaatgcacctgtaattacttaaaactgttatagcatgcaatgtgttaccacaacagccagagaaatactaatttactcagcctattcttctagaccagtaaacactaggattaaatagatattttcattgaatttgttctacccttcattgccatttatagatagcttacttgtcatagattactttctaattgttttatgtttcctaactagcctgcaatactttggcaaggacctcaaacaatagtagacagtaggtgtaaaatagatggctacattgaacagatgactaaaaggatgcctcctaagtacctatatcttgaaatatatattattgtgccttgctttcaatttgtgattttaaaatctagaaatcacctgttttatgtaataacaataaaatccttctttgttgaaaacatgcacaaataaagtttacaagctcaaaaaattaaacagcagtaacggtcaagctttccaacaataaaatacattttggtaaggttttcattttacaaaaactcaaaatagctttatgagttcacaaaataatatgatatttttcaagatattaacatattcttataccggaagagcatagaataaaatttacttggagattgagcatttgcttctttaagaaatacttcttttagtatttttactttaatattatgaaagctacataattacattcagattcattaactactccagtagttaatttttaaaacttatgatgaatagttttgtttaaaatatataacattggtaatatgcaaatctgaatctgtaataaagaaggatttgcattcctgatttttttttctgatacaaccaatgacaaaataactaatggttccacagaggataaaatgtctcaaatctgttggttctgaaggtgaagcgagatttttgtactgataccgtgtatcactgagataccaggaggaaatggaattaaactcagatagttcaaatggagagattttaatgaagggacgacctacagaggtgtcggcagggttggggggaatcagcgagatatgcttagaacccaccgactggcaaacctccccctgaagatggagaaggaggaaggagtgttactggaatgagagcttgagtccaggggaggaggatgggctgctgaggaggcgacaccatcctgaaagaagaatcctctgccagaggcttttcagggtcatttcttcacactctctctcttcaagtggtatttaaatttcttctttcattttccttctggtaacaaagaagtctgtggctcaaaagatgtttctctaagaccccatcctattaggtctctgagattttagaaatgacccaacttgatccttttattcttcagaatatctctctcaaattttcatttgtttttcattaattgatgaataatgagacattttaggtacctgagggccgacgagtgggggcgggcaggagggccgagggaggcggaacaggatcgaggcgcgaggcgggagtcgagaaagcgagcggccgaggcgactctcagtgcgcggacgcgggcgcgcgcccgcgctcccttcgtcgactcacggcgagagcccaaccctgctgccgcgcgccaccc

SEQ ID NO: 12743 - RNA, 15163 nt, Homo sapiens
  source 1..15163: mol_type = other RNA
gatctcactttgttgcccaggctggtcttaaactcctggcctcaagtgatccccttgtttcagccccgcaaagtgctgggattacaggtgtgagccaccatgcccgtgcccagccacctcatgagtcttgatggggggcagagaccaacaactccacagaagccagatgcttgctttcccagcctctcttgcagctagggcttgggcatgtgatccaggctcagccaatcagatggcactgactcttggcatgacatgggctaaggaggggctgcagggaatccatttgggctggggtggcagctgcactgggagcgacatcagtttccagagggagcagcagaatctggcatcaggcttggggcgtggtaggtgcaaccagactctgcacccagcagcagtggcagaatgggttctctgtggagagtctgtgtattgctccttccgctgaggccaccagcatctgcctccatgaacccctcagagcctgtgagcaactcaacagccttgaattttttcccttcctgtttgaatgagccagggttgtttcactgcttgaactaagagccgttcctgacatgaaaactaagccacatctttttgacccaaagattctggcatcctaaaatacccatctcattttaagttaaaaataaatccatgtttgagcatctactgtttcagttactgtgctaggtgttacaaagctaactaagagtgacaagtaaataactatcatcaccatgataaacagagaatggaaccctggtttttggaatacagacacaaaatgattaattctgcctggaagcgttttggaacatttcagagaggtagtgagctgggccaagagaagagcatacgcaaggaatggtggcatgaagttgcctggtgtgtcctgagaagaaagatgggctaagaaggactggggtagggcagagaagggggtcactggaggtgaggctgggaaagtgagccaaggctcaaatgcaaactgtctgaacttcattttctgtgcaagcaggagaagccgctgacatgggtttggaagatggactgaagccggagaaaaatggaagcaagaaaccctctcacaagaggccataaccacaaccaagtccatgagattgaaaaggaaggcagatatttgaaaaatatttaaagagatgtgaggggtaggacaggcacagtggctcatgcctgtagtcccagcactttgggaggccgaggtgggcagatccacgaggtcaggagatcaagaccatcctaacatggtaaaaccccatctctactaacaatacaaaaaattagtcaggtgtggtggcacgtgcctgtagtcccagctactcaggaggctgaggcaggagaatcgcttgaacctgggaggcggaggttgcagtgagccgagattgtgccactgcaccctagcctaggcaacagagcaagactctgtctcaaaaaaaataaaaaaaaaaaaaagagagaaagagagagagagatgaggagttgctgcactgctgggtgtggagagccgaggaggattcaaagatggtcctgaagtcccagctggaagaagtaggcggcagcaatgtttttaatactgtaaattcatcacgtagcacaggtttggggtggagaaagaaaaattgcattggcttcagggcatgcccagatctttcctcatcttaggcgtttgctaatacatgcattttctaagctgatgtcttgcgtttaatcactgctccattcaaaagagagaaggaggttgtttcaaacctagttgatatcatttgacttccatgctattcacagggctattttatttgaaacaggtataccacagccttaaattgcaagttaatccaggatgttcctaggttggcagttaggaacatgtaattctttggaagggctaaaagtcagctctttaaattatctccatatgaaccttctctccaccttagggtggatccacttatttagtccactgccagtaccacactagaacccgggtggtcactggactccagaaacaacagtagccctctctctgttctgtctctttttgactatctctattctgttcctgaccctgatttctcctgccaagctcaattttgacagctgacaacggcaagccatggcttcccaaaacattattttcaggtcaacttataaatttcaagaacacatttggctccgcttcctgtggtactaagcctacttcttgacagcatttgcctttgttgtaaatagcaaagttcttctagttggatttttgctaagaagtgtgtggatgtggcatgtgacgacatctttagcttggattctagaaaggcactaccattgtgcatttggctaaaggaaacacattttacccgtgaatgccttctatttacaaatgctcagctagcacacaaagctaagtacaagcaataagtactatcctacaatgttactcatttctgaaagcacaaaatgatgactggtatagctttggagatgttttctggaaacccaataaaggaacagatctttgttattccacacctacaaagtcagaagatgcacagtcttttattcatgtttgaacaagcttccttcttgaacaatcaactataaagtgatgtgattctctactagaccaggaactccttgaggacagaatgagggtctaatccatattctaaatccacaccacctggcacaatacatgttgcatggttagggtcaactaagagttggttgaattaatcaataacacacagcaagagaattcacaaagagaggggagtaatcccccagcctcaatcactcggcaagtggaatcgctgggcactgattccagctctgtctcagtgcttgagacagagctgaatgtaatgtgaacatttcaaatgaacaggaaaactagactcacggataagcagtgtagtcatcaagacaacactgtcttggaggtttttctgaagttaaaaccatgctacataagcaataaattatgaaggctgagcatgtgaataaaatttaatgttgtcataaattttataacaaagttaatctgacacatttaatgacatgcataatcattagtatgcagcactgtaatcagacattgataataagcagttcacaccagtgactgtaagagtctttacttgtgttcagccaagccaactgcttggtatatttttctcccttcttagtcgttagttttccatacctacaataactatcagtggtgatgggcttctctgaccatgtgaataatttaatcctcaatgcacagatacagaaacccttgctgaagacagtgtggagcagagaaggctgtctccactccttccacctgaaacacctctgcagatggatatgggagctctgcctacagcccttggacctaaccacttcagtgtgttccagtgagtgtctggacctcggcctgaaagatttttccgaaactaaagaaaatttctctgacctaaagaccttaacctccaccccagaagctctcaccaaggactacagggaactggtggggaaaatccttatcccttactcctcaaggcacagggcagtaatgctgaggcttgtgcgccacacttgctcccagaggtccccagcgggctacctgcggtggtgaatgacctcctaacacgccccttgacggccttcctttccttgcctcacttctccactctcctaccagcattgcagggttcacatcccaaatataccactggcacttgaatcctggtctccaggtctgtttctggaaaaacccaagtaagacattgccccagtaatggggctagatgtctgaggcttcctcaagtatctacctcgaaagctcttactgctgtacacacatgcacatacacacacgtgcgtacaaccagtcacatctaagcaccccgaataccagcctgttgaaggtagcagagagctgcactataagccaaggctgctcccaagagccgctccatcactgaattggcgccccagcaagatgaaggaatgtaatcattggaaggatggagaatgttctctgaatcactgacaaattggaaggggtggagggcaagagtccacctggtggagagatggaaagagcgagagagcctggaatgataatgccattgcttagaaaaggctgctccagatgccatatctacagaaattgtacagcccaaacatctctgagcaataggtctctggtagtcttgatgtctagaccaacaattcccagttcattcttctcagggaaggagccaggatagtccagagactctcattctgctgttagattgaaagggttaggcacaacagccttggcaaagtcacaagggcaaattcacactaaagtgtaaatgacccacaactcctcttctatttttaggttggggaggtgctttagaacataaggaggaactaaagaatattcctgttacatacaaggcagagaaaagggaaactagtggtgacaagacaaatcatccctttgacatttggctggctctacctattacagctctgggggtgaggtgggaacaaaaagatgctgtgtaaagaagtatcttatgccatccctactgtagtgaggtgcagtttagaggggacactgatcaagcagagacccagagtgtttcgttccaagccagaaacagaaatgtataaaacacagcctttccagcatcagaaatgagtagtggtagtggagaactacccaaaacaggaaagaggaccacgtgaggtagagtgtcaaggccctacattccagtgcctctgctcatgactgtaattttgggtaggtcacttaaagtctctggacctcagttttgccatctgtgaaatagggataatactatccagcataaaattggttatgaggctcatgtagggcctgcctgggatgatgtgttgctaatggttaagaacacaacttctggggtctgactggacaggctgaaatccctgcttaacacgttccagcagagccctgggcgatctatttaacttttgttttctcacctgtaagctgagacgaaagtacccactttataagattattccaataattagttgaaataatgcatgcagagaattaagcatggtacttgttatttgttaaactagctattaaaatgtgtaaaatataaagtattgtatggattttaggacaatgcaaagactctttgcttgctgcaatagttcggggccctttcagatggctaaaggcagaatttgtatgtgtaaatatggtgtgcttgtctctgctctggatactgagggcttaccctgttattaaacttatttagtaaatattgaactgtcatgaggcctaacatttagttccagttattagataaaacatttgctttgaatggtatttgaattgccaggttctagattattctggttgacaaactcttcgtattttataaagaggctaaaattggtaagctatcacagaacagatgtgccattttcaaggtatattaaaccatgattcactgtaacattgttcctactggcaacaaattcagagcaggctggactttatttggtgaagaaacattgagtggaagagaaatgacattattttatgtatttacattttcaaattactgtggcttaaacctgttcagccaacattacccaccttcagtctgctaaataaatgattcagtacatttctaatttacagaattttttaacaaaagaaaatgtaatttgatagccaaatcaacgttaaacattatacatttaaaaaaccacaggcaaagacacaaacatgatgacactaacttttgttaaagtatgcttacctatggtttcctctgaggcacgttctttcatgctaagcttccaacataatatgaaaatgaaggagatgcattttgcaaagcaaaacagaccttaagcaaaatattatacttctcaaattaacactgttacaaagttttagaatttaataagttcattaatttaaaagtttggatgtctgagtccttctatcccaaaacaagatcttggagggtcttccacagccatgtaataccatggtcacatgaccctttccaaaattattaatctgaatttactatatgaggataaatctatctttttgaaaatatttaggaaaatgagcttggtatttataaaatgaagctctctttgggtggtatcctaagacacgtcaagccaatcagcctgtaactgtgaaaaaaacattggtaggtacaaaagtggggtgggagaggagtgacttaactttgttaagtgatgggaaagaaacactaatagcattatctcaataaaatgtgatttaaaaaaatttaaaatactaaatcattgaactgacaaagaaatataaatcattcagaaataaactcattaggtcatcaaatcctgttaaatctgcaattaggaagagcaaggtgtacaatccatacatttaaactcacaggctcactttgcacaacgtcaatttactccttaatatgttattaatacgcattttccaaaaggatgtattagtaaatggtacacatctacttcttggcaacatcatataacctggtacaacataagcattcttcttatagttaagaaatgtggatggtatcaaaattagaaaaataaatgccctattatgttgtggtcaggtttaaggcatgtgaattttatcttcatacaaaagattaaaatctagatattaaaaagtagtgcagtatcagtgatgctgcctcagttcccaaaatgtcacatcacaaaaatatcccataattgcctgtagtttattccttggctttcctcttttctctctgcatctttgtaacaattttttaaaagtggaaatataattgttggcaatgctaacagctgtagaaatgattacaagatgtggaaaagcataacaggaatgtcaagaatctgtttctggcagtaatatatatggaacattgttcaggacaaaagaggagaaggaagaaaaaaaggagaggggtttatcatctctaagaattttcaaactaaacctcattgcttaataggaaaaaaagattccatatttaaagttaagtcacctctaactactagctaaagcatgacatcaccagcactggagtcagcggaagtgtgtttttgaaggacagtgttgcaggagaatctggacaggttttagagccaggagagagaaaataattctacctctgacagttgaaggaccttaggcaaatcagtttacctctgctagactacactccaaaatttggacattcaaaaatttgatattaataaccacatgaaagtctcgtgttgaggtgaatatgtatttgttggtgaaagatatgttggtttttaaacagacagcactctgcaattgtaggctattgttttgttttgccagttgtcaaattctatccagctatacacacttgtgtggcctcctaatggtgtttttccagtggctaaaggtttatgaataagacacttttcctaatggaattaacccgatgcttttcttaaacatgtaaccttgagttcaccgcaaaaaacaatgcttcgattagagcaatgcatataataaaggttaccctcgtttcttagacactagacatcattcacaaaaagagaactgcttttgaaagggatgtatttgcactggaaagaatagttttctacttctaattataaatgatttattggtgaaagcaaaacaacagcctgtctgagaggcacttctatgagcatcctcacgtgtgatttgcaaggttgaagaagagggaaaaatgcctcaattgtaccaatggtgagaaaacacccaaagtacaaagcaggtttcaaaaaaaccatactcataaccaaggacaataataaagcaatgtgttgacatatactctataagtcttcctccataaatagtttatagaaattttgtaatttctgtaaatgcatcctataataattttgcatcttgctttttttttacatttaatatcaagtagatttctaaagggcaattatttgaaaattatcccaaatacatggggaaatatacatcaagtgaaaaaatgcagtgggtgatagagatatcaggaagcgcctcaaatatttctcatctcgttggagaaaaacaaacatgttctcatttagaatgagtgggagttacctaattgatttaggcctctatatttaacttctagtcaaaaaaggtagttctatctagcaacaatattatggggaacaaaagaaaaaattaactctctaaatttgcagtagggtcttttcttcagaagtaccaaatcccatctattaccagctccatgcttcaggcctaaaatggatctccctgaagcaatgacagaatttttgccaagtgactaggatataaacaccactttggttgcacagtgagacatatgctccaaagaaaactggttcaaaaacaggcaagtgggtttctacagaataaatgagagccctgtcaatggcttcatcttcagggctttgtgtctgtgcttgcgtggtggctcttgtttcatctatggataatggtggcacacagttttcataattccttacattaatgaactgctataaatttgtttttggtattctagagagtcctaacttcagcttctgggcaatgctgaggaggcaccctatattctagacttaccttttgcaaggtgtactctcagcattgtgggcgatttccatgggagaatattctatttaaagaactactgtcccagcataaaacaaaaaatcatttatgaagatgcaggagactcggaaagctctcaattattgtttgcacaagcacaatgtcacagcctcctttccccattccacaagggggtcaggaagagagtactcagctgtgagaaaagacatacagaagaattcatgtggtcatgagagcgaggacatggccgatcccccaaggaggatgtgtcatacacttcatgagcccaagagtgtgctgtagggtctgaagggcaagatgctggttcactgatgtaaaggagagggaaaaaagcttcaaccaactagaaaaacagtctctatgcatgctatttttgattttaaacacaggtatcaattccttctctcagagagtccattttaaaataggatacatttttaaaggaatatttaaaggacacattcattaaaatttattttaaaaacttttcaaaagaaacaaaaggtatgaattttatttaatccttgaggaaatggttcttttctcacacacataaatcactcattttgtttttctttatctcctttattaatctacattagaaaaataaacttttcatacactaagaacaaggaaaccactctcaattgacaaaatgttccaatccaacacaatgattactttcacctttaatttacaggcagccagattcaaaatccttaaagttgcttaaacttaaaaatgacaatgacaacctaaaaggtataatgttgattggaacagacatttaattggaaaattgatgattttccatttccaattaaatctctagatagaaatgaaaaaaattaaaaatcgtatttaagaaaagccaaatcttgggttgtgaggtatctttttaaggatgtttcagcagaaaaaaacaaaggctctcacaattgtgtagctgcctagattaagtgggtatcctgatcaaggagatgggggatgatttggctttagtattccaatgataaagtttataatgagaataacatgttgctacaaaatccagtctcttcctcagatgccttccacagagggcaggaagctttgtcagttttgtttgctgatgatgcctggttccgtcaacaaataacacctgtcacacggtgggtagtcaatatacatttgttgaataaatatgaaaaaaagaaatgtacaatatgtttgtgaagccaactgtgtgtgcattgctattgaggtacacaaaaagtctttgttttaaatttgagaatgaggactttcaatggaatatatctataaaaatgaaaaaaagacattactgtctggacttttgtacagcaagagaagaaaaaccactagccaagagccaactcacctgataggcctggatcaagcatgcagctgtggagaacacccctgggactctaactctggcactctgcaagctgggtacttgggcaggacagcagcagcactcatgaactgggcagcacctgttggtgagggctgatcacatggattctctcatcccagccttacaatcagtccttcaggtacatactttttctgactttgctgatgaggaaactatgcacagaggttacacagcttaacaaagggttctcacctaatgaacaatgaaatgggattttagcctttctttgcatctggtcttagagccaatacccaagaagcactgtactgtatgcattgtctcagagaaacttactcttcctgggcctcagtctttaaaaggtgggcagttgacttaataagaattaaagatcaatgattaaggttcaaggcactccaaaattctggtctttattgaaaaggctacagaagtctcaccttaataataccctatagacttgatattcttggttaattaaatattggaaaccaatttcatagtaattgaggtcagaaaaaagtactcatgacattttagaatatgatgacaaagccatagataaatttcaatgcacctgtaattacttaaaactgttatagcatgcaatgtgttaccacaacagccagagaaatactaatttactcagcctattcttctagaccagtaaacactaggattaaatagatattttcattgaatttgttctacccttcattgccatttatagatagcttacttgtcatagattactttctaattgttttatgtttcctaactagcctgcaatactttggcaaggacctcaaacaatagtagacagtaggtgtaaaatagatggctacattgaacagatgactaaaaggatgcctcctaagtacctatatcttgaaatatatattattgtgccttgctttcaatttgtgattttaaaatctagaaatcacctgttttatgtaataacaataaaatccttctttgttgaaaacatgcacaaataaagtttacaagctcaaaaaattaaacagcagtaacggtcaagctttccaacaataaaatacattttggtaaggttttcattttacaaaaactcaaaatagctttatgagttcacaaaataatatgatatttttcaagatattaacatattcttataccggaagagcatagaataaaatttacttggagattgagcatttgcttctttaagaaatacttcttttagtatttttactttaatattatgaaagctacataattacattcagattcattaactactccagtagttaatttttaaaacttatgatgaatagttttgtttaaaatatataacattggtaatatgcaaatctgaatctgtaataaagaaggatttgcattcctgatttttttttctgatacaaccaatgacaaaataactaatggttccacagaggataaaatgtctcaaatctgttggttctgaaggtgaagcgagatttttgtactgataccgtgtatcactgagataccaggaggaaatggaattaaactcagatagttcaaatggagagattttaatgaagggacgacctacagaggtgtcggcagggttggggggaatcagcgagatatgcttagaacccaccgactggcaaacctccccctgaagatggagaaggaggaaggagtgttactggaatgagagcttgagtccaggggaggaggatgggctgctgaggaggcgacaccatcctgaaagaagaatcctctgccagaggcttttcagggtcatttcttcacactctctctcttcaagtggtatttaaatttcttctttcattttccttctggtaacaaagaagtctgtggctcaaaagatgtttctctaagaccccatcctattaggtctctgagattttagaaatgacccaacttgatccttttattcttcagaatatctctctcaaattttcatttgtttttcattaattgatgaataatgagacattttaggtacctgtccacaaagaaatgaaattttcactttccaggaacctaacaaatgaaaagatagaaatcaattccaacagaatattaccaaagaaatcttttagaatggactgttaaaattatttatttgtatttatctggctctactatttgtggtacatttccacttcaaagctaaacctcaaataacatcatagtgagtggttgacttcatgtttaactgagatcttgaagactgaaaaagaccacgacaaacacacatctattttcttggctactgcatccgtgttcatcaccattctgatagtctgcaatgtattgcagctcaccctttgggaaggactaaagtagacatctgtttgttctgcttactcagcattcctaccctaattttcctttggagaacccctttattctagaccacgtgaagctaatgccaaaccccattccaggggatgcacctgaatccaacctccatcatctaaacagtgccttctccacgttcagagaagagcaagtgactcaaactgccctcataagaacagacctgggacttctgctgcaaatattgaagagtaagtactcttttttcttgctaggactaagctggtagtaccttctatgaggctatcatatggaaacaacttgtctgaaaatgaagccacaactagaaaacagatcctggtaacccggattgatggatccagccctaccttaaatggcaagacctaacccgaggctttttgcatcaaccaataaagtccttaagccagtttgagttggttttgtcacttgcagctaaaagaattctgactctaacaatgtgacaatagcaaaaataaacataactgcttttgaggtttctaatggattttcctccctatatacatgatttcatttaatcctcacaattcaggaaagcacatatctattaacattaaattaatattcattattttgaacacatgctatgtggataagggatgaggaaagccaaggaagtaatcaacgtgaaatctcacttatatgggagggaagtggaggttacatatctcagggcacttaacagatatcatcaaatgaaagaataaacagtgtgtgggagaggcagtaggtgattcttcatcaattcctggatgaaaaattaggagataatgaactccgaacaggcagcctaatgagaatggctcaagcaacaggacatagagagggagttaggttagacatggggttcttgggaattttcacctcgtgggggggcgggggggtcgtgcagctgttgtcagtgggaaagggaaaaaggaaaaggctgagtttggaaggcagggagggaggagacaatgtgagtcagtgaaaaagggcccttagaatgacaagtctggaccagagagaggctaagactgaaaatacaagttgggtaaccactggcatacagatggcagttcaggcttgggcactgcccaccagagcctcagcatgaagagaagagggggaggctggccaccacctccctctaggtaatcgtcatcctgatgctgagctcctgaaaacaggctctttcactcgccccatctcttgctcttgattgcaacccggcattcaggaggcaccctgtaatatctgtggagtgaccgacaacacagcgccagggcactgagaagatcccagggcgccagggactggttctacaagggtgcccctcccggtcccctccagcgcgccgccagagctgccagtcttggctgctacacgggaggcagcctcattatgcagctctcacctcttaaattagttcatgctctcacattaggtgtaatcacagcttgcaacgctttctggggatgtctcagaaagatctgagttgaaaaaatatttttgtgtcattttaatttaaagtaaaattgctgcttcttccccgcccctttctttcctcctggcccacccagcgaccctggccggccgtgctcaacgggggcgggggtcggaggtgagatttcctccacataattccttaaacagctatcaactaagtctcaaagaaaaaaaaaagagatctagaagcagagacgtggctgctggcgatcccaaagctggtgttcgctcttgggggagagcgtaccctgggggaggccgggaggccgggccagaggctagcccagaggcagagggcaggagcgctcagccggcgccccgcgtctctccagctcccgacgctgcgctggctccgctgagcacgccaggatcaaggtcgcctggtggggaccggagcgccaggagcctgtgggaagcgttccagccggcctctgactgggatccggcgccgcgtttctgctttggacttgactgacaggtccccccgccctcccgccgccctactaccagcctgggttcatccttcagggctacgtctaccgcacccgggctggaaagcctggagcgcgcccttcctctcctcatcttctcagctctcctttctccctgccacttggcaaagctgcattttgactttcacgttttggactacgtgtgtgtagttccaagtccatgcgtggcacgaaaatccacttagggtaaaaattattctcgaaaaatcgcccatctcaggatctggtgtctacactcaaggctaggaggtgcaggtacgggtgcgtaaagcatgccgtaagggtgcacagtaaataaaaagtacggatgcaaaatgtaaattttaagtgcaaaacagaaaagcagtactcgttgccgccccgcacgctgggttttaaggggcacgaaggtgggcctcggctgcttttgctcagccccgcgtcctcagcgcccggcccagtacccggtactccgtaggggttcaatgatctcccctgaataagtgaacgaattaacaaatgaatgaatgaccgctcgatccgacctccgcggccggcagagcagtcgctggagaggcgggagagagcgagaggccaagctccaccatcgcggccgccggctggggcagagggacacggagacactcggcgccccggctccgcaccgagtccccg

SEQ ID NO: 12744 - RNA, 12364 nt, Homo sapiens
  source 1..12364: mol_type = other RNA
gatctcactttgttgcccaggctggtcttaaactcctggcctcaagtgatccccttgtttcagccccgcaaagtgctgggattacaggtgtgagccaccatgcccgtgcccagccacctcatgagtcttgatggggggcagagaccaacaactccacagaagccagatgcttgctttcccagcctctcttgcagctagggcttgggcatgtgatccaggctcagccaatcagatggcactgactcttggcatgacatgggctaaggaggggctgcagggaatccatttgggctggggtggcagctgcactgggagcgacatcagtttccagagggagcagcagaatctggcatcaggcttggggcgtggtaggtgcaaccagactctgcacccagcagcagtggcagaatgggttctctgtggagagtctgtgtattgctccttccgctgaggccaccagcatctgcctccatgaacccctcagagcctgtgagcaactcaacagccttgaattttttcccttcctgtttgaatgagccagggttgtttcactgcttgaactaagagccgttcctgacatgaaaactaagccacatctttttgacccaaagattctggcatcctaaaatacccatctcattttaagttaaaaataaatccatgtttgagcatctactgtttcagttactgtgctaggtgttacaaagctaactaagagtgacaagtaaataactatcatcaccatgataaacagagaatggaaccctggtttttggaatacagacacaaaatgattaattctgcctggaagcgttttggaacatttcagagaggtagtgagctgggccaagagaagagcatacgcaaggaatggtggcatgaagttgcctggtgtgtcctgagaagaaagatgggctaagaaggactggggtagggcagagaagggggtcactggaggtgaggctgggaaagtgagccaaggctcaaatgcaaactgtctgaacttcattttctgtgcaagcaggagaagccgctgacatgggtttggaagatggactgaagccggagaaaaatggaagcaagaaaccctctcacaagaggccataaccacaaccaagtccatgagattgaaaaggaaggcagatatttgaaaaatatttaaagagatgtgaggggtaggacaggcacagtggctcatgcctgtagtcccagcactttgggaggccgaggtgggcagatccacgaggtcaggagatcaagaccatcctaacatggtaaaaccccatctctactaacaatacaaaaaattagtcaggtgtggtggcacgtgcctgtagtcccagctactcaggaggctgaggcaggagaatcgcttgaacctgggaggcggaggttgcagtgagccgagattgtgccactgcaccctagcctaggcaacagagcaagactctgtctcaaaaaaaataaaaaaaaaaaaaagagagaaagagagagagagatgaggagttgctgcactgctgggtgtggagagccgaggaggattcaaagatggtcctgaagtcccagctggaagaagtaggcggcagcaatgtttttaatactgtaaattcatcacgtagcacaggtttggggtggagaaagaaaaattgcattggcttcagggcatgcccagatctttcctcatcttaggcgtttgctaatacatgcattttctaagctgatgtcttgcgtttaatcactgctccattcaaaagagagaaggaggttgtttcaaacctagttgatatcatttgacttccatgctattcacagggctattttatttgaaacaggtataccacagccttaaattgcaagttaatccaggatgttcctaggttggcagttaggaacatgtaattctttggaagggctaaaagtcagctctttaaattatctccatatgaaccttctctccaccttagggtggatccacttatttagtccactgccagtaccacactagaacccgggtggtcactggactccagaaacaacagtagccctctctctgttctgtctctttttgactatctctattctgttcctgaccctgatttctcctgccaagctcaattttgacagctgacaacggcaagccatggcttcccaaaacattattttcaggtcaacttataaatttcaagaacacatttggctccgcttcctgtggtactaagcctacttcttgacagcatttgcctttgttgtaaatagcaaagttcttctagttggatttttgctaagaagtgtgtggatgtggcatgtgacgacatctttagcttggattctagaaaggcactaccattgtgcatttggctaaaggaaacacattttacccgtgaatgccttctatttacaaatgctcagctagcacacaaagctaagtacaagcaataagtactatcctacaatgttactcatttctgaaagcacaaaatgatgactggtatagctttggagatgttttctggaaacccaataaaggaacagatctttgttattccacacctacaaagtcagaagatgcacagtcttttattcatgtttgaacaagcttccttcttgaacaatcaactataaagtgatgtgattctctactagaccaggaactccttgaggacagaatgagggtctaatccatattctaaatccacaccacctggcacaatacatgttgcatggttagggtcaactaagagttggttgaattaatcaataacacacagcaagagaattcacaaagagaggggagtaatcccccagcctcaatcactcggcaagtggaatcgctgggcactgattccagctctgtctcagtgcttgagacagagctgaatgtaatgtgaacatttcaaatgaacaggaaaactagactcacggataagcagtgtagtcatcaagacaacactgtcttggaggtttttctgaagttaaaaccatgctacataagcaataaattatgaaggctgagcatgtgaataaaatttaatgttgtcataaattttataacaaagttaatctgacacatttaatgacatgcataatcattagtatgcagcactgtaatcagacattgataataagcagttcacaccagtgactgtaagagtctttacttgtgttcagccaagccaactgcttggtatatttttctcccttcttagtcgttagttttccatacctacaataactatcagtggtgatgggcttctctgaccatgtgaataatttaatcctcaatgcacagatacagaaacccttgctgaagacagtgtggagcagagaaggctgtctccactccttccacctgaaacacctctgcagatggatatgggagctctgcctacagcccttggacctaaccacttcagtgtgttccagtgagtgtctggacctcggcctgaaagatttttccgaaactaaagaaaatttctctgacctaaagaccttaacctccaccccagaagctctcaccaaggactacagggaactggtggggaaaatccttatcccttactcctcaaggcacagggcagtaatgctgaggcttgtgcgccacacttgctcccagaggtccccagcgggctacctgcggtggtgaatgacctcctaacacgccccttgacggccttcctttccttgcctcacttctccactctcctaccagcattgcagggttcacatcccaaatataccactggcacttgaatcctggtctccaggtctgtttctggaaaaacccaagtaagacattgccccagtaatggggctagatgtctgaggcttcctcaagtatctacctcgaaagctcttactgctgtacacacatgcacatacacacacgtgcgtacaaccagtcacatctaagcaccccgaataccagcctgttgaaggtagcagagagctgcactataagccaaggctgctcccaagagccgctccatcactgaattggcgccccagcaagatgaaggaatgtaatcattggaaggatggagaatgttctctgaatcactgacaaattggaaggggtggagggcaagagtccacctggtggagagatggaaagagcgagagagcctggaatgataatgccattgcttagaaaaggctgctccagatgccatatctacagaaattgtacagcccaaacatctctgagcaataggtctctggtagtcttgatgtctagaccaacaattcccagttcattcttctcagggaaggagccaggatagtccagagactctcattctgctgttagattgaaagggttaggcacaacagccttggcaaagtcacaagggcaaattcacactaaagtgtaaatgacccacaactcctcttctatttttaggttggggaggtgctttagaacataaggaggaactaaagaatattcctgttacatacaaggcagagaaaagggaaactagtggtgacaagacaaatcatccctttgacatttggctggctctacctattacagctctgggggtgaggtgggaacaaaaagatgctgtgtaaagaagtatcttatgccatccctactgtagtgaggtgcagtttagaggggacactgatcaagcagagacccagagtgtttcgttccaagccagaaacagaaatgtataaaacacagcctttccagcatcagaaatgagtagtggtagtggagaactacccaaaacaggaaagaggaccacgtgaggtagagtgtcaaggccctacattccagtgcctctgctcatgactgtaattttgggtaggtcacttaaagtctctggacctcagttttgccatctgtgaaatagggataatactatccagcataaaattggttatgaggctcatgtagggcctgcctgggatgatgtgttgctaatggttaagaacacaacttctggggtctgactggacaggctgaaatccctgcttaacacgttccagcagagccctgggcgatctatttaacttttgttttctcacctgtaagctgagacgaaagtacccactttataagattattccaataattagttgaaataatgcatgcagagaattaagcatggtacttgttatttgttaaactagctattaaaatgtgtaaaatataaagtattgtatggattttaggacaatgcaaagactctttgcttgctgcaatagttcggggccctttcagatggctaaaggcagaatttgtatgtgtaaatatggtgtgcttgtctctgctctggatactgagggcttaccctgttattaaacttatttagtaaatattgaactgtcatgaggcctaacatttagttccagttattagataaaacatttgctttgaatggtatttgaattgccaggttctagattattctggttgacaaactcttcgtattttataaagaggctaaaattggtaagctatcacagaacagatgtgccattttcaaggtatattaaaccatgattcactgtaacattgttcctactggcaacaaattcagagcaggctggactttatttggtgaagaaacattgagtggaagagaaatgacattattttatgtatttacattttcaaattactgtggcttaaacctgttcagccaacattacccaccttcagtctgctaaataaatgattcagtacatttctaatttacagaattttttaacaaaagaaaatgtaatttgatagccaaatcaacgttaaacattatacatttaaaaaaccacaggcaaagacacaaacatgatgacactaacttttgttaaagtatgcttacctatggtttcctctgaggcacgttctttcatgctaagcttccaacataatatgaaaatgaaggagatgcattttgcaaagcaaaacagaccttaagcaaaatattatacttctcaaattaacactgttacaaagttttagaatttaataagttcattaatttaaaagtttggatgtctgagtccttctatcccaaaacaagatcttggagggtcttccacagccatgtaataccatggtcacatgaccctttccaaaattattaatctgaatttactatatgaggataaatctatctttttgaaaatatttaggaaaatgagcttggtatttataaaatgaagctctctttgggtggtatcctaagacacgtcaagccaatcagcctgtaactgtgaaaaaaacattggtaggtacaaaagtggggtgggagaggagtgacttaactttgttaagtgatgggaaagaaacactaatagcattatctcaataaaatgtgatttaaaaaaatttaaaatactaaatcattgaactgacaaagaaatataaatcattcagaaataaactcattaggtcatcaaatcctgttaaatctgcaattaggaagagcaaggtgtacaatccatacatttaaactcacaggctcactttgcacaacgtcaatttactccttaatatgttattaatacgcattttccaaaaggatgtattagtaaatggtacacatctacttcttggcaacatcatataacctggtacaacataagcattcttcttatagttaagaaatgtggatggtatcaaaattagaaaaataaatgccctattatgttgtggtcaggtttaaggcatgtgaattttatcttcatacaaaagattaaaatctagatattaaaaagtagtgcagtatcagtgatgctgcctcagttcccaaaatgtcacatcacaaaaatatcccataattgcctgtagtttattccttggctttcctcttttctctctgcatctttgtaacaattttttaaaagtggaaatataattgttggcaatgctaacagctgtagaaatgattacaagatgtggaaaagcataacaggaatgtcaagaatctgtttctggcagtaatatatatggaacattgttcaggacaaaagaggagaaggaagaaaaaaaggagaggggtttatcatctctaagaattttcaaactaaacctcattgcttaataggaaaaaaagattccatatttaaagttaagtcacctctaactactagctaaagcatgacatcaccagcactggagtcagcggaagtgtgtttttgaaggacagtgttgcaggagaatctggacaggttttagagccaggagagagaaaataattctacctctgacagttgaaggaccttaggcaaatcagtttacctctgctagactacactccaaaatttggacattcaaaaatttgatattaataaccacatgaaagtctcgtgttgaggtgaatatgtatttgttggtgaaagatatgttggtttttaaacagacagcactctgcaattgtaggctattgttttgttttgccagttgtcaaattctatccagctatacacacttgtgtggcctcctaatggtgtttttccagtggctaaaggtttatgaataagacacttttcctaatggaattaacccgatgcttttcttaaacatgtaaccttgagttcaccgcaaaaaacaatgcttcgattagagcaatgcatataataaaggttaccctcgtttcttagacactagacatcattcacaaaaagagaactgcttttgaaagggatgtatttgcactggaaagaatagttttctacttctaattataaatgatttattggtgaaagcaaaacaacagcctgtctgagaggcacttctatgagcatcctcacgtgtgatttgcaaggttgaagaagagggaaaaatgcctcaattgtaccaatggtgagaaaacacccaaagtacaaagcaggtttcaaaaaaaccatactcataaccaaggacaataataaagcaatgtgttgacatatactctataagtcttcctccataaatagtttatagaaattttgtaatttctgtaaatgcatcctataataattttgcatcttgctttttttttacatttaatatcaagtagatttctaaagggcaattatttgaaaattatcccaaatacatggggaaatatacatcaagtgaaaaaatgcagtgggtgatagagatatcaggaagcgcctcaaatatttctcatctcgttggagaaaaacaaacatgttctcatttagaatgagtgggagttacctaattgatttaggcctctatatttaacttctagtcaaaaaaggtagttctatctagcaacaatattatggggaacaaaagaaaaaattaactctctaaatttgcagtagggtcttttcttcagaagtaccaaatcccatctattaccagctccatgcttcaggcctaaaatggatctccctgaagcaatgacagaatttttgccaagtgactaggatataaacaccactttggttgcacagtgagacatatgctccaaagaaaactggttcaaaaacaggcaagtgggtttctacagaataaatgagagccctgtcaatggcttcatcttcagggctttgtgtctgtgcttgcgtggtggctcttgtttcatctatggataatggtggcacacagttttcataattccttacattaatgaactgctataaatttgtttttggtattctagagagtcctaacttcagcttctgggcaatgctgaggaggcaccctatattctagacttaccttttgcaaggtgtactctcagcattgtgggcgatttccatgggagaatattctatttaaagaactactgtcccagcataaaacaaaaaatcatttatgaagatgcaggagactcggaaagctctcaattattgtttgcacaagcacaatgtcacagcctcctttccccattccacaagggggtcaggaagagagtactcagctgtgagaaaagacatacagaagaattcatgtggtcatgagagcgaggacatggccgatcccccaaggaggatgtgtcatacacttcatgagcccaagagtgtgctgtagggtctgaagggcaagatgctggttcactgatgtaaaggagagggaaaaaagcttcaaccaactagaaaaacagtctctatgcatgctatttttgattttaaacacaggtatcaattccttctctcagagagtccattttaaaataggatacatttttaaaggaatatttaaaggacacattcattaaaatttattttaaaaacttttcaaaagaaacaaaaggtatgaattttatttaatccttgaggaaatggttcttttctcacacacataaatcactcattttgtttttctttatctcctttattaatctacattagaaaaataaacttttcatacactaagaacaaggaaaccactctcaattgacaaaatgttccaatccaacacaatgattactttcacctttaatttacaggcagccagattcaaaatccttaaagttgcttaaacttaaaaatgacaatgacaacctaaaaggtataatgttgattggaacagacatttaattggaaaattgatgattttccatttccaattaaatctctagatagaaatgaaaaaaattaaaaatcgtatttaagaaaagccaaatcttgggttgtgaggtatctttttaaggatgtttcagcagaaaaaaacaaaggctctcacaattgtgtagctgcctagattaagtgggtatcctgatcaaggagatgggggatgatttggctttagtattccaatgataaagtttataatgagaataacatgttgctacaaaatccagtctcttcctcagatgccttccacagagggcaggaagctttgtcagttttgtttgctgatgatgcctggttccgtcaacaaataacacctgtcacacggtgggtagtcaatatacatttgttgaataaatatgaaaaaaagaaatgtacaatatgtttgtgaagccaactgtgtgtgcattgctattgaggtacacaaaaagtctttgttttaaatttgagaatgaggactttcaatggaatatatctataaaaatgaaaaaaagacattactgtctggacttttgtacagcaagagaagaaaaaccactagccaagagccaactcacctgataggcctggatcaagcatgcagctgtggagaacacccctgggactctaactctggcactctgcaagctgggtacttgggcaggacagcagcagcactcatgaactgggcagcacctgttggtgagggctgatcacatggattctctcatcccagccttacaatcagtccttcaggtacatactttttctgactttgctgatgaggaaactatgcacagaggttacacagcttaacaaagggttctcacctaatgaacaatgaaatgggattttagcctttctttgcatctggtcttagagccaatacccaagaagcactgtactgtatgcattgtctcagagaaacttactcttcctgggcctcagtctttaaaaggtgggcagttgacttaataagaattaaagatcaatgattaaggttcaaggcactccaaaattctggtctttattgaaaaggctacagaagtctcaccttaataataccctatagacttgatattcttggttaattaaatattggaaaccaatttcatagtaattgaggtcagaaaaaagtactcatgacattttagaatatgatgacaaagccatagataaatttcaatgcacctgtaattacttaaaactgttatagcatgcaatgtgttaccacaacagccagagaaatactaatttactcagcctattcttctagaccagtaaacactaggattaaatagatattttcattgaatttgttctacccttcattgccatttatagatagcttacttgtcatagattactttctaattgttttatgtttcctaactagcctgcaatactttggcaaggacctcaaacaatagtagacagtaggtgtaaaatagatggctacattgaacagatgactaaaaggatgcctcctaagtacctatatcttgaaatatatattattgtgccttgctttcaatttgtgattttaaaatctagaaatcacctgttttatgtaataacaataaaatccttctttgttgaaaacatgcacaaataaagtttacaagctcaaaaaattaaacagcagtaacggtcaagctttccaacaataaaatacattttggtaaggttttcattttacaaaaactcaaaatagctttatgagttcacaaaataatatgatatttttcaagatattaacatattcttataccggaagagcatagaataaaatttacttggagattgagcatttgcttctttaagaaatacttcttttagtatttttactttaatattatgaaagctacataattacattcagattcattaactactccagtagttaatttttaaaacttatgatgaatagttttgtttaaaatatataacattggtaatatgcaaatctgaatctgtaataaagaaggatttgcattcctgatttttttttctgatacaaccaatgacaaaataactaatggttccacagaggataaaatgtctcaaatctgttggttctgaaggtgaagcgagatttttgtactgataccgtgtatcactgagataccaggaggaaatggaattaaactcagatagttcaaatggagagattttaatgaagggacgacctacagaggtgtcggcagggttggggggaatcagcgagatatgcttagaacccaccgactggcaaacctccccctgaagatggagaaggaggaaggagtgttactggaatgagagcttgagtccaggggaggaggatgggctgctgaggaggcgacaccatcctgaaagaagaatcctctgccagaggcttttcagggtcatttcttcacactctctctcttcaagtggtatttaaatttcttctttcattttccttctggtaacaaagaagtctgtggctcaaaagatgtttctctaagaccccatcctattaggtctctgagattttagaaatgacccaacttgatccttttattcttcagaatatctctctcaaattttcatttgtttttcattaattgatgaataatgagacattttaggtacctgtccacaaagaaatgaaattttcactttccaggaacctgagggccgacgagtgggggcgggcaggagggccgagggaggcggaacaggatcgaggcgcgaggcgggagtcgagaaagcgagcggccgaggcgactctcagtgcgcggacgcgggcgcgcgcccgcgctcccttcgtcgactcacggcgagagcccaaccctgctgccgcgcgccacccgcctcgccgcgc

SEQ ID NO: 12745 - RNA, 12225 nt, Homo sapiens
  source 1..12225: mol_type = other RNA
gatctcactttgttgcccaggctggtcttaaactcctggcctcaagtgatccccttgtttcagccccgcaaagtgctgggattacaggtgtgagccaccatgcccgtgcccagccacctcatgagtcttgatggggggcagagaccaacaactccacagaagccagatgcttgctttcccagcctctcttgcagctagggcttgggcatgtgatccaggctcagccaatcagatggcactgactcttggcatgacatgggctaaggaggggctgcagggaatccatttgggctggggtggcagctgcactgggagcgacatcagtttccagagggagcagcagaatctggcatcaggcttggggcgtggtaggtgcaaccagactctgcacccagcagcagtggcagaatgggttctctgtggagagtctgtgtattgctccttccgctgaggccaccagcatctgcctccatgaacccctcagagcctgtgagcaactcaacagccttgaattttttcccttcctgtttgaatgagccagggttgtttcactgcttgaactaagagccgttcctgacatgaaaactaagccacatctttttgacccaaagattctggcatcctaaaatacccatctcattttaagttaaaaataaatccatgtttgagcatctactgtttcagttactgtgctaggtgttacaaagctaactaagagtgacaagtaaataactatcatcaccatgataaacagagaatggaaccctggtttttggaatacagacacaaaatgattaattctgcctggaagcgttttggaacatttcagagaggtagtgagctgggccaagagaagagcatacgcaaggaatggtggcatgaagttgcctggtgtgtcctgagaagaaagatgggctaagaaggactggggtagggcagagaagggggtcactggaggtgaggctgggaaagtgagccaaggctcaaatgcaaactgtctgaacttcattttctgtgcaagcaggagaagccgctgacatgggtttggaagatggactgaagccggagaaaaatggaagcaagaaaccctctcacaagaggccataaccacaaccaagtccatgagattgaaaaggaaggcagatatttgaaaaatatttaaagagatgtgaggggtaggacaggcacagtggctcatgcctgtagtcccagcactttgggaggccgaggtgggcagatccacgaggtcaggagatcaagaccatcctaacatggtaaaaccccatctctactaacaatacaaaaaattagtcaggtgtggtggcacgtgcctgtagtcccagctactcaggaggctgaggcaggagaatcgcttgaacctgggaggcggaggttgcagtgagccgagattgtgccactgcaccctagcctaggcaacagagcaagactctgtctcaaaaaaaataaaaaaaaaaaaaagagagaaagagagagagagatgaggagttgctgcactgctgggtgtggagagccgaggaggattcaaagatggtcctgaagtcccagctggaagaagtaggcggcagcaatgtttttaatactgtaaattcatcacgtagcacaggtttggggtggagaaagaaaaattgcattggcttcagggcatgcccagatctttcctcatcttaggcgtttgctaatacatgcattttctaagctgatgtcttgcgtttaatcactgctccattcaaaagagagaaggaggttgtttcaaacctagttgatatcatttgacttccatgctattcacagggctattttatttgaaacaggtataccacagccttaaattgcaagttaatccaggatgttcctaggttggcagttaggaacatgtaattctttggaagggctaaaagtcagctctttaaattatctccatatgaaccttctctccaccttagggtggatccacttatttagtccactgccagtaccacactagaacccgggtggtcactggactccagaaacaacagtagccctctctctgttctgtctctttttgactatctctattctgttcctgaccctgatttctcctgccaagctcaattttgacagctgacaacggcaagccatggcttcccaaaacattattttcaggtcaacttataaatttcaagaacacatttggctccgcttcctgtggtactaagcctacttcttgacagcatttgcctttgttgtaaatagcaaagttcttctagttggatttttgctaagaagtgtgtggatgtggcatgtgacgacatctttagcttggattctagaaaggcactaccattgtgcatttggctaaaggaaacacattttacccgtgaatgccttctatttacaaatgctcagctagcacacaaagctaagtacaagcaataagtactatcctacaatgttactcatttctgaaagcacaaaatgatgactggtatagctttggagatgttttctggaaacccaataaaggaacagatctttgttattccacacctacaaagtcagaagatgcacagtcttttattcatgtttgaacaagcttccttcttgaacaatcaactataaagtgatgtgattctctactagaccaggaactccttgaggacagaatgagggtctaatccatattctaaatccacaccacctggcacaatacatgttgcatggttagggtcaactaagagttggttgaattaatcaataacacacagcaagagaattcacaaagagaggggagtaatcccccagcctcaatcactcggcaagtggaatcgctgggcactgattccagctctgtctcagtgcttgagacagagctgaatgtaatgtgaacatttcaaatgaacaggaaaactagactcacggataagcagtgtagtcatcaagacaacactgtcttggaggtttttctgaagttaaaaccatgctacataagcaataaattatgaaggctgagcatgtgaataaaatttaatgttgtcataaattttataacaaagttaatctgacacatttaatgacatgcataatcattagtatgcagcactgtaatcagacattgataataagcagttcacaccagtgactgtaagagtctttacttgtgttcagccaagccaactgcttggtatatttttctcccttcttagtcgttagttttccatacctacaataactatcagtggtgatgggcttctctgaccatgtgaataatttaatcctcaatgcacagatacagaaacccttgctgaagacagtgtggagcagagaaggctgtctccactccttccacctgaaacacctctgcagatggatatgggagctctgcctacagcccttggacctaaccacttcagtgtgttccagtgagtgtctggacctcggcctgaaagatttttccgaaactaaagaaaatttctctgacctaaagaccttaacctccaccccagaagctctcaccaaggactacagggaactggtggggaaaatccttatcccttactcctcaaggcacagggcagtaatgctgaggcttgtgcgccacacttgctcccagaggtccccagcgggctacctgcggtggtgaatgacctcctaacacgccccttgacggccttcctttccttgcctcacttctccactctcctaccagcattgcagggttcacatcccaaatataccactggcacttgaatcctggtctccaggtctgtttctggaaaaacccaagtaagacattgccccagtaatggggctagatgtctgaggcttcctcaagtatctacctcgaaagctcttactgctgtacacacatgcacatacacacacgtgcgtacaaccagtcacatctaagcaccccgaataccagcctgttgaaggtagcagagagctgcactataagccaaggctgctcccaagagccgctccatcactgaattggcgccccagcaagatgaaggaatgtaatcattggaaggatggagaatgttctctgaatcactgacaaattggaaggggtggagggcaagagtccacctggtggagagatggaaagagcgagagagcctggaatgataatgccattgcttagaaaaggctgctccagatgccatatctacagaaattgtacagcccaaacatctctgagcaataggtctctggtagtcttgatgtctagaccaacaattcccagttcattcttctcagggaaggagccaggatagtccagagactctcattctgctgttagattgaaagggttaggcacaacagccttggcaaagtcacaagggcaaattcacactaaagtgtaaatgacccacaactcctcttctatttttaggttggggaggtgctttagaacataaggaggaactaaagaatattcctgttacatacaaggcagagaaaagggaaactagtggtgacaagacaaatcatccctttgacatttggctggctctacctattacagctctgggggtgaggtgggaacaaaaagatgctgtgtaaagaagtatcttatgccatccctactgtagtgaggtgcagtttagaggggacactgatcaagcagagacccagagtgtttcgttccaagccagaaacagaaatgtataaaacacagcctttccagcatcagaaatgagtagtggtagtggagaactacccaaaacaggaaagaggaccacgtgaggtagagtgtcaaggccctacattccagtgcctctgctcatgactgtaattttgggtaggtcacttaaagtctctggacctcagttttgccatctgtgaaatagggataatactatccagcataaaattggttatgaggctcatgtagggcctgcctgggatgatgtgttgctaatggttaagaacacaacttctggggtctgactggacaggctgaaatccctgcttaacacgttccagcagagccctgggcgatctatttaacttttgttttctcacctgtaagctgagacgaaagtacccactttataagattattccaataattagttgaaataatgcatgcagagaattaagcatggtacttgttatttgttaaactagctattaaaatgtgtaaaatataaagtattgtatggattttaggacaatgcaaagactctttgcttgctgcaatagttcggggccctttcagatggctaaaggcagaatttgtatgtgtaaatatggtgtgcttgtctctgctctggatactgagggcttaccctgttattaaacttatttagtaaatattgaactgtcatgaggcctaacatttagttccagttattagataaaacatttgctttgaatggtatttgaattgccaggttctagattattctggttgacaaactcttcgtattttataaagaggctaaaattggtaagctatcacagaacagatgtgccattttcaaggtatattaaaccatgattcactgtaacattgttcctactggcaacaaattcagagcaggctggactttatttggtgaagaaacattgagtggaagagaaatgacattattttatgtatttacattttcaaattactgtggcttaaacctgttcagccaacattacccaccttcagtctgctaaataaatgattcagtacatttctaatttacagaattttttaacaaaagaaaatgtaatttgatagccaaatcaacgttaaacattatacatttaaaaaaccacaggcaaagacacaaacatgatgacactaacttttgttaaagtatgcttacctatggtttcctctgaggcacgttctttcatgctaagcttccaacataatatgaaaatgaaggagatgcattttgcaaagcaaaacagaccttaagcaaaatattatacttctcaaattaacactgttacaaagttttagaatttaataagttcattaatttaaaagtttggatgtctgagtccttctatcccaaaacaagatcttggagggtcttccacagccatgtaataccatggtcacatgaccctttccaaaattattaatctgaatttactatatgaggataaatctatctttttgaaaatatttaggaaaatgagcttggtatttataaaatgaagctctctttgggtggtatcctaagacacgtcaagccaatcagcctgtaactgtgaaaaaaacattggtaggtacaaaagtggggtgggagaggagtgacttaactttgttaagtgatgggaaagaaacactaatagcattatctcaataaaatgtgatttaaaaaaatttaaaatactaaatcattgaactgacaaagaaatataaatcattcagaaataaactcattaggtcatcaaatcctgttaaatctgcaattaggaagagcaaggtgtacaatccatacatttaaactcacaggctcactttgcacaacgtcaatttactccttaatatgttattaatacgcattttccaaaaggatgtattagtaaatggtacacatctacttcttggcaacatcatataacctggtacaacataagcattcttcttatagttaagaaatgtggatggtatcaaaattagaaaaataaatgccctattatgttgtggtcaggtttaaggcatgtgaattttatcttcatacaaaagattaaaatctagatattaaaaagtagtgcagtatcagtgatgctgcctcagttcccaaaatgtcacatcacaaaaatatcccataattgcctgtagtttattccttggctttcctcttttctctctgcatctttgtaacaattttttaaaagtggaaatataattgttggcaatgctaacagctgtagaaatgattacaagatgtggaaaagcataacaggaatgtcaagaatctgtttctggcagtaatatatatggaacattgttcaggacaaaagaggagaaggaagaaaaaaaggagaggggtttatcatctctaagaattttcaaactaaacctcattgcttaataggaaaaaaagattccatatttaaagttaagtcacctctaactactagctaaagcatgacatcaccagcactggagtcagcggaagtgtgtttttgaaggacagtgttgcaggagaatctggacaggttttagagccaggagagagaaaataattctacctctgacagttgaaggaccttaggcaaatcagtttacctctgctagactacactccaaaatttggacattcaaaaatttgatattaataaccacatgaaagtctcgtgttgaggtgaatatgtatttgttggtgaaagatatgttggtttttaaacagacagcactctgcaattgtaggctattgttttgttttgccagttgtcaaattctatccagctatacacacttgtgtggcctcctaatggtgtttttccagtggctaaaggtttatgaataagacacttttcctaatggaattaacccgatgcttttcttaaacatgtaaccttgagttcaccgcaaaaaacaatgcttcgattagagcaatgcatataataaaggttaccctcgtttcttagacactagacatcattcacaaaaagagaactgcttttgaaagggatgtatttgcactggaaagaatagttttctacttctaattataaatgatttattggtgaaagcaaaacaacagcctgtctgagaggcacttctatgagcatcctcacgtgtgatttgcaaggttgaagaagagggaaaaatgcctcaattgtaccaatggtgagaaaacacccaaagtacaaagcaggtttcaaaaaaaccatactcataaccaaggacaataataaagcaatgtgttgacatatactctataagtcttcctccataaatagtttatagaaattttgtaatttctgtaaatgcatcctataataattttgcatcttgctttttttttacatttaatatcaagtagatttctaaagggcaattatttgaaaattatcccaaatacatggggaaatatacatcaagtgaaaaaatgcagtgggtgatagagatatcaggaagcgcctcaaatatttctcatctcgttggagaaaaacaaacatgttctcatttagaatgagtgggagttacctaattgatttaggcctctatatttaacttctagtcaaaaaaggtagttctatctagcaacaatattatggggaacaaaagaaaaaattaactctctaaatttgcagtagggtcttttcttcagaagtaccaaatcccatctattaccagctccatgcttcaggcctaaaatggatctccctgaagcaatgacagaatttttgccaagtgactaggatataaacaccactttggttgcacagtgagacatatgctccaaagaaaactggttcaaaaacaggcaagtgggtttctacagaataaatgagagccctgtcaatggcttcatcttcagggctttgtgtctgtgcttgcgtggtggctcttgtttcatctatggataatggtggcacacagttttcataattccttacattaatgaactgctataaatttgtttttggtattctagagagtcctaacttcagcttctgggcaatgctgaggaggcaccctatattctagacttaccttttgcaaggtgtactctcagcattgtgggcgatttccatgggagaatattctatttaaagaactactgtcccagcataaaacaaaaaatcatttatgaagatgcaggagactcggaaagctctcaattattgtttgcacaagcacaatgtcacagcctcctttccccattccacaagggggtcaggaagagagtactcagctgtgagaaaagacatacagaagaattcatgtggtcatgagagcgaggacatggccgatcccccaaggaggatgtgtcatacacttcatgagcccaagagtgtgctgtagggtctgaagggcaagatgctggttcactgatgtaaaggagagggaaaaaagcttcaaccaactagaaaaacagtctctatgcatgctatttttgattttaaacacaggtatcaattccttctctcagagagtccattttaaaataggatacatttttaaaggaatatttaaaggacacattcattaaaatttattttaaaaacttttcaaaagaaacaaaaggtatgaattttatttaatccttgaggaaatggttcttttctcacacacataaatcactcattttgtttttctttatctcctttattaatctacattagaaaaataaacttttcatacactaagaacaaggaaaccactctcaattgacaaaatgttccaatccaacacaatgattactttcacctttaatttacaggcagccagattcaaaatccttaaagttgcttaaacttaaaaatgacaatgacaacctaaaaggtataatgttgattggaacagacatttaattggaaaattgatgattttccatttccaattaaatctctagatagaaatgaaaaaaattaaaaatcgtatttaagaaaagccaaatcttgggttgtgaggtatctttttaaggatgtttcagcagaaaaaaacaaaggctctcacaattgtgtagctgcctagattaagtgggtatcctgatcaaggagatgggggatgatttggctttagtattccaatgataaagtttataatgagaataacatgttgctacaaaatccagtctcttcctcagatgccttccacagagggcaggaagctttgtcagttttgtttgctgatgatgcctggttccgtcaacaaataacacctgtcacacggtgggtagtcaatatacatttgttgaataaatatgaaaaaaagaaatgtacaatatgtttgtgaagccaactgtgtgtgcattgctattgaggtacacaaaaagtctttgttttaaatttgagaatgaggactttcaatggaatatatctataaaaatgaaaaaaagacattactgtctggacttttgtacagcaagagaagaaaaaccactagccaagagccaactcacctgataggcctggatcaagcatgcagctgtggagaacacccctgggactctaactctggcactctgcaagctgggtacttgggcaggacagcagcagcactcatgaactgggcagcacctgttggtgagggctgatcacatggattctctcatcccagccttacaatcagtccttcaggtacatactttttctgactttgctgatgaggaaactatgcacagaggttacacagcttaacaaagggttctcacctaatgaacaatgaaatgggattttagcctttctttgcatctggtcttagagccaatacccaagaagcactgtactgtatgcattgtctcagagaaacttactcttcctgggcctcagtctttaaaaggtgggcagttgacttaataagaattaaagatcaatgattaaggttcaaggcactccaaaattctggtctttattgaaaaggctacagaagtctcaccttaataataccctatagacttgatattcttggttaattaaatattggaaaccaatttcatagtaattgaggtcagaaaaaagtactcatgacattttagaatatgatgacaaagccatagataaatttcaatgcacctgtaattacttaaaactgttatagcatgcaatgtgttaccacaacagccagagaaatactaatttactcagcctattcttctagaccagtaaacactaggattaaatagatattttcattgaatttgttctacccttcattgccatttatagatagcttacttgtcatagattactttctaattgttttatgtttcctaactagcctgcaatactttggcaaggacctcaaacaatagtagacagtaggtgtaaaatagatggctacattgaacagatgactaaaaggatgcctcctaagtacctatatcttgaaatatatattattgtgccttgctttcaatttgtgattttaaaatctagaaatcacctgttttatgtaataacaataaaatccttctttgttgaaaacatgcacaaataaagtttacaagctcaaaaaattaaacagcagtaacggtcaagctttccaacaataaaatacattttggtaaggttttcattttacaaaaactcaaaatagctttatgagttcacaaaataatatgatatttttcaagatattaacatattcttataccggaagagcatagaataaaatttacttggagattgagcatttgcttctttaagaaatacttcttttagtatttttactttaatattatgaaagctacataattacattcagattcattaactactccagtagttaatttttaaaacttatgatgaatagttttgtttaaaatatataacattggtaatatgcaaatctgaatctgtaataaagaaggatttgcattcctgatttttttttctgatacaaccaatgacaaaataactaatggttccacagaggataaaatgtctcaaatctgttggttctgaaggtgaagcgagatttttgtactgataccgtgtatcactgagataccaggaggaaatggaattaaactcagatagttcaaatggagagattttaatgaagggacgacctacagaggtgtcggcagggttggggggaatcagcgagatatgcttagaacccaccgactggcaaacctccccctgaagatggagaaggaggaaggagtgttactggaatgagagcttgagtccaggggaggaggatgggctgctgaggaggcgacaccatcctgaaagaagaatcctctgccagaggcttttcagggtcatttcttcacactctctctcttcaagtggtatttaaatttcttctttcattttccttctggtaacaaagaagtctgtggctcaaaagatgtttctctaagaccccatcctattaggtctctgagctgagggccgacgagtgggggcgggcaggagggccgagggaggcggaacaggatcgaggcgcgaggcgggagtcgagaaagcgagcggccgaggcgactctcagtgcgcggacgcgggcgcgcgcccgcgctcccttcgtcgactcacggcgagagcccaaccctgctgccgcgcgccacccgcctcgccgcgcct

SEQ ID NO: 12746 - RNA, 12249 nt, Homo sapiens
  source 1..12249: mol_type = other RNA
gatctcactttgttgcccaggctggtcttaaactcctggcctcaagtgatccccttgtttcagccccgcaaagtgctgggattacaggtgtgagccaccatgcccgtgcccagccacctcatgagtcttgatggggggcagagaccaacaactccacagaagccagatgcttgctttcccagcctctcttgcagctagggcttgggcatgtgatccaggctcagccaatcagatggcactgactcttggcatgacatgggctaaggaggggctgcagggaatccatttgggctggggtggcagctgcactgggagcgacatcagtttccagagggagcagcagaatctggcatcaggcttggggcgtggtaggtgcaaccagactctgcacccagcagcagtggcagaatgggttctctgtggagagtctgtgtattgctccttccgctgaggccaccagcatctgcctccatgaacccctcagagcctgtgagcaactcaacagccttgaattttttcccttcctgtttgaatgagccagggttgtttcactgcttgaactaagagccgttcctgacatgaaaactaagccacatctttttgacccaaagattctggcatcctaaaatacccatctcattttaagttaaaaataaatccatgtttgagcatctactgtttcagttactgtgctaggtgttacaaagctaactaagagtgacaagtaaataactatcatcaccatgataaacagagaatggaaccctggtttttggaatacagacacaaaatgattaattctgcctggaagcgttttggaacatttcagagaggtagtgagctgggccaagagaagagcatacgcaaggaatggtggcatgaagttgcctggtgtgtcctgagaagaaagatgggctaagaaggactggggtagggcagagaagggggtcactggaggtgaggctgggaaagtgagccaaggctcaaatgcaaactgtctgaacttcattttctgtgcaagcaggagaagccgctgacatgggtttggaagatggactgaagccggagaaaaatggaagcaagaaaccctctcacaagaggccataaccacaaccaagtccatgagattgaaaaggaaggcagatatttgaaaaatatttaaagagatgtgaggggtaggacaggcacagtggctcatgcctgtagtcccagcactttgggaggccgaggtgggcagatccacgaggtcaggagatcaagaccatcctaacatggtaaaaccccatctctactaacaatacaaaaaattagtcaggtgtggtggcacgtgcctgtagtcccagctactcaggaggctgaggcaggagaatcgcttgaacctgggaggcggaggttgcagtgagccgagattgtgccactgcaccctagcctaggcaacagagcaagactctgtctcaaaaaaaataaaaaaaaaaaaaagagagaaagagagagagagatgaggagttgctgcactgctgggtgtggagagccgaggaggattcaaagatggtcctgaagtcccagctggaagaagtaggcggcagcaatgtttttaatactgtaaattcatcacgtagcacaggtttggggtggagaaagaaaaattgcattggcttcagggcatgcccagatctttcctcatcttaggcgtttgctaatacatgcattttctaagctgatgtcttgcgtttaatcactgctccattcaaaagagagaaggaggttgtttcaaacctagttgatatcatttgacttccatgctattcacagggctattttatttgaaacaggtataccacagccttaaattgcaagttaatccaggatgttcctaggttggcagttaggaacatgtaattctttggaagggctaaaagtcagctctttaaattatctccatatgaaccttctctccaccttagggtggatccacttatttagtccactgccagtaccacactagaacccgggtggtcactggactccagaaacaacagtagccctctctctgttctgtctctttttgactatctctattctgttcctgaccctgatttctcctgccaagctcaattttgacagctgacaacggcaagccatggcttcccaaaacattattttcaggtcaacttataaatttcaagaacacatttggctccgcttcctgtggtactaagcctacttcttgacagcatttgcctttgttgtaaatagcaaagttcttctagttggatttttgctaagaagtgtgtggatgtggcatgtgacgacatctttagcttggattctagaaaggcactaccattgtgcatttggctaaaggaaacacattttacccgtgaatgccttctatttacaaatgctcagctagcacacaaagctaagtacaagcaataagtactatcctacaatgttactcatttctgaaagcacaaaatgatgactggtatagctttggagatgttttctggaaacccaataaaggaacagatctttgttattccacacctacaaagtcagaagatgcacagtcttttattcatgtttgaacaagcttccttcttgaacaatcaactataaagtgatgtgattctctactagaccaggaactccttgaggacagaatgagggtctaatccatattctaaatccacaccacctggcacaatacatgttgcatggttagggtcaactaagagttggttgaattaatcaataacacacagcaagagaattcacaaagagaggggagtaatcccccagcctcaatcactcggcaagtggaatcgctgggcactgattccagctctgtctcagtgcttgagacagagctgaatgtaatgtgaacatttcaaatgaacaggaaaactagactcacggataagcagtgtagtcatcaagacaacactgtcttggaggtttttctgaagttaaaaccatgctacataagcaataaattatgaaggctgagcatgtgaataaaatttaatgttgtcataaattttataacaaagttaatctgacacatttaatgacatgcataatcattagtatgcagcactgtaatcagacattgataataagcagttcacaccagtgactgtaagagtctttacttgtgttcagccaagccaactgcttggtatatttttctcccttcttagtcgttagttttccatacctacaataactatcagtggtgatgggcttctctgaccatgtgaataatttaatcctcaatgcacagatacagaaacccttgctgaagacagtgtggagcagagaaggctgtctccactccttccacctgaaacacctctgcagatggatatgggagctctgcctacagcccttggacctaaccacttcagtgtgttccagtgagtgtctggacctcggcctgaaagatttttccgaaactaaagaaaatttctctgacctaaagaccttaacctccaccccagaagctctcaccaaggactacagggaactggtggggaaaatccttatcccttactcctcaaggcacagggcagtaatgctgaggcttgtgcgccacacttgctcccagaggtccccagcgggctacctgcggtggtgaatgacctcctaacacgccccttgacggccttcctttccttgcctcacttctccactctcctaccagcattgcagggttcacatcccaaatataccactggcacttgaatcctggtctccaggtctgtttctggaaaaacccaagtaagacattgccccagtaatggggctagatgtctgaggcttcctcaagtatctacctcgaaagctcttactgctgtacacacatgcacatacacacacgtgcgtacaaccagtcacatctaagcaccccgaataccagcctgttgaaggtagcagagagctgcactataagccaaggctgctcccaagagccgctccatcactgaattggcgccccagcaagatgaaggaatgtaatcattggaaggatggagaatgttctctgaatcactgacaaattggaaggggtggagggcaagagtccacctggtggagagatggaaagagcgagagagcctggaatgataatgccattgcttagaaaaggctgctccagatgccatatctacagaaattgtacagcccaaacatctctgagcaataggtctctggtagtcttgatgtctagaccaacaattcccagttcattcttctcagggaaggagccaggatagtccagagactctcattctgctgttagattgaaagggttaggcacaacagccttggcaaagtcacaagggcaaattcacactaaagtgtaaatgacccacaactcctcttctatttttaggttggggaggtgctttagaacataaggaggaactaaagaatattcctgttacatacaaggcagagaaaagggaaactagtggtgacaagacaaatcatccctttgacatttggctggctctacctattacagctctgggggtgaggtgggaacaaaaagatgctgtgtaaagaagtatcttatgccatccctactgtagtgaggtgcagtttagaggggacactgatcaagcagagacccagagtgtttcgttccaagccagaaacagaaatgtataaaacacagcctttccagcatcagaaatgagtagtggtagtggagaactacccaaaacaggaaagaggaccacgtgaggtagagtgtcaaggccctacattccagtgcctctgctcatgactgtaattttgggtaggtcacttaaagtctctggacctcagttttgccatctgtgaaatagggataatactatccagcataaaattggttatgaggctcatgtagggcctgcctgggatgatgtgttgctaatggttaagaacacaacttctggggtctgactggacaggctgaaatccctgcttaacacgttccagcagagccctgggcgatctatttaacttttgttttctcacctgtaagctgagacgaaagtacccactttataagattattccaataattagttgaaataatgcatgcagagaattaagcatggtacttgttatttgttaaactagctattaaaatgtgtaaaatataaagtattgtatggattttaggacaatgcaaagactctttgcttgctgcaatagttcggggccctttcagatggctaaaggcagaatttgtatgtgtaaatatggtgtgcttgtctctgctctggatactgagggcttaccctgttattaaacttatttagtaaatattgaactgtcatgaggcctaacatttagttccagttattagataaaacatttgctttgaatggtatttgaattgccaggttctagattattctggttgacaaactcttcgtattttataaagaggctaaaattggtaagctatcacagaacagatgtgccattttcaaggtatattaaaccatgattcactgtaacattgttcctactggcaacaaattcagagcaggctggactttatttggtgaagaaacattgagtggaagagaaatgacattattttatgtatttacattttcaaattactgtggcttaaacctgttcagccaacattacccaccttcagtctgctaaataaatgattcagtacatttctaatttacagaattttttaacaaaagaaaatgtaatttgatagccaaatcaacgttaaacattatacatttaaaaaaccacaggcaaagacacaaacatgatgacactaacttttgttaaagtatgcttacctatggtttcctctgaggcacgttctttcatgctaagcttccaacataatatgaaaatgaaggagatgcattttgcaaagcaaaacagaccttaagcaaaatattatacttctcaaattaacactgttacaaagttttagaatttaataagttcattaatttaaaagtttggatgtctgagtccttctatcccaaaacaagatcttggagggtcttccacagccatgtaataccatggtcacatgaccctttccaaaattattaatctgaatttactatatgaggataaatctatctttttgaaaatatttaggaaaatgagcttggtatttataaaatgaagctctctttgggtggtatcctaagacacgtcaagccaatcagcctgtaactgtgaaaaaaacattggtaggtacaaaagtggggtgggagaggagtgacttaactttgttaagtgatgggaaagaaacactaatagcattatctcaataaaatgtgatttaaaaaaatttaaaatactaaatcattgaactgacaaagaaatataaatcattcagaaataaactcattaggtcatcaaatcctgttaaatctgcaattaggaagagcaaggtgtacaatccatacatttaaactcacaggctcactttgcacaacgtcaatttactccttaatatgttattaatacgcattttccaaaaggatgtattagtaaatggtacacatctacttcttggcaacatcatataacctggtacaacataagcattcttcttatagttaagaaatgtggatggtatcaaaattagaaaaataaatgccctattatgttgtggtcaggtttaaggcatgtgaattttatcttcatacaaaagattaaaatctagatattaaaaagtagtgcagtatcagtgatgctgcctcagttcccaaaatgtcacatcacaaaaatatcccataattgcctgtagtttattccttggctttcctcttttctctctgcatctttgtaacaattttttaaaagtggaaatataattgttggcaatgctaacagctgtagaaatgattacaagatgtggaaaagcataacaggaatgtcaagaatctgtttctggcagtaatatatatggaacattgttcaggacaaaagaggagaaggaagaaaaaaaggagaggggtttatcatctctaagaattttcaaactaaacctcattgcttaataggaaaaaaagattccatatttaaagttaagtcacctctaactactagctaaagcatgacatcaccagcactggagtcagcggaagtgtgtttttgaaggacagtgttgcaggagaatctggacaggttttagagccaggagagagaaaataattctacctctgacagttgaaggaccttaggcaaatcagtttacctctgctagactacactccaaaatttggacattcaaaaatttgatattaataaccacatgaaagtctcgtgttgaggtgaatatgtatttgttggtgaaagatatgttggtttttaaacagacagcactctgcaattgtaggctattgttttgttttgccagttgtcaaattctatccagctatacacacttgtgtggcctcctaatggtgtttttccagtggctaaaggtttatgaataagacacttttcctaatggaattaacccgatgcttttcttaaacatgtaaccttgagttcaccgcaaaaaacaatgcttcgattagagcaatgcatataataaaggttaccctcgtttcttagacactagacatcattcacaaaaagagaactgcttttgaaagggatgtatttgcactggaaagaatagttttctacttctaattataaatgatttattggtgaaagcaaaacaacagcctgtctgagaggcacttctatgagcatcctcacgtgtgatttgcaaggttgaagaagagggaaaaatgcctcaattgtaccaatggtgagaaaacacccaaagtacaaagcaggtttcaaaaaaaccatactcataaccaaggacaataataaagcaatgtgttgacatatactctataagtcttcctccataaatagtttatagaaattttgtaatttctgtaaatgcatcctataataattttgcatcttgctttttttttacatttaatatcaagtagatttctaaagggcaattatttgaaaattatcccaaatacatggggaaatatacatcaagtgaaaaaatgcagtgggtgatagagatatcaggaagcgcctcaaatatttctcatctcgttggagaaaaacaaacatgttctcatttagaatgagtgggagttacctaattgatttaggcctctatatttaacttctagtcaaaaaaggtagttctatctagcaacaatattatggggaacaaaagaaaaaattaactctctaaatttgcagtagggtcttttcttcagaagtaccaaatcccatctattaccagctccatgcttcaggcctaaaatggatctccctgaagcaatgacagaatttttgccaagtgactaggatataaacaccactttggttgcacagtgagacatatgctccaaagaaaactggttcaaaaacaggcaagtgggtttctacagaataaatgagagccctgtcaatggcttcatcttcagggctttgtgtctgtgcttgcgtggtggctcttgtttcatctatggataatggtggcacacagttttcataattccttacattaatgaactgctataaatttgtttttggtattctagagagtcctaacttcagcttctgggcaatgctgaggaggcaccctatattctagacttaccttttgcaaggtgtactctcagcattgtgggcgatttccatgggagaatattctatttaaagaactactgtcccagcataaaacaaaaaatcatttatgaagatgcaggagactcggaaagctctcaattattgtttgcacaagcacaatgtcacagcctcctttccccattccacaagggggtcaggaagagagtactcagctgtgagaaaagacatacagaagaattcatgtggtcatgagagcgaggacatggccgatcccccaaggaggatgtgtcatacacttcatgagcccaagagtgtgctgtagggtctgaagggcaagatgctggttcactgatgtaaaggagagggaaaaaagcttcaaccaactagaaaaacagtctctatgcatgctatttttgattttaaacacaggtatcaattccttctctcagagagtccattttaaaataggatacatttttaaaggaatatttaaaggacacattcattaaaatttattttaaaaacttttcaaaagaaacaaaaggtatgaattttatttaatccttgaggaaatggttcttttctcacacacataaatcactcattttgtttttctttatctcctttattaatctacattagaaaaataaacttttcatacactaagaacaaggaaaccactctcaattgacaaaatgttccaatccaacacaatgattactttcacctttaatttacaggcagccagattcaaaatccttaaagttgcttaaacttaaaaatgacaatgacaacctaaaaggtataatgttgattggaacagacatttaattggaaaattgatgattttccatttccaattaaatctctagatagaaatgaaaaaaattaaaaatcgtatttaagaaaagccaaatcttgggttgtgaggtatctttttaaggatgtttcagcagaaaaaaacaaaggctctcacaattgtgtagctgcctagattaagtgggtatcctgatcaaggagatgggggatgatttggctttagtattccaatgataaagtttataatgagaataacatgttgctacaaaatccagtctcttcctcagatgccttccacagagggcaggaagctttgtcagttttgtttgctgatgatgcctggttccgtcaacaaataacacctgtcacacggtgggtagtcaatatacatttgttgaataaatatgaaaaaaagaaatgtacaatatgtttgtgaagccaactgtgtgtgcattgctattgaggtacacaaaaagtctttgttttaaatttgagaatgaggactttcaatggaatatatctataaaaatgaaaaaaagacattactgtctggacttttgtacagcaagagaagaaaaaccactagccaagagccaactcacctgataggcctggatcaagcatgcagctgtggagaacacccctgggactctaactctggcactctgcaagctgggtacttgggcaggacagcagcagcactcatgaactgggcagcacctgttggtgagggctgatcacatggattctctcatcccagccttacaatcagtccttcaggtacatactttttctgactttgctgatgaggaaactatgcacagaggttacacagcttaacaaagggttctcacctaatgaacaatgaaatgggattttagcctttctttgcatctggtcttagagccaatacccaagaagcactgtactgtatgcattgtctcagagaaacttactcttcctgggcctcagtctttaaaaggtgggcagttgacttaataagaattaaagatcaatgattaaggttcaaggcactccaaaattctggtctttattgaaaaggctacagaagtctcaccttaataataccctatagacttgatattcttggttaattaaatattggaaaccaatttcatagtaattgaggtcagaaaaaagtactcatgacattttagaatatgatgacaaagccatagataaatttcaatgcacctgtaattacttaaaactgttatagcatgcaatgtgttaccacaacagccagagaaatactaatttactcagcctattcttctagaccagtaaacactaggattaaatagatattttcattgaatttgttctacccttcattgccatttatagatagcttacttgtcatagattactttctaattgttttatgtttcctaactagcctgcaatactttggcaaggacctcaaacaatagtagacagtaggtgtaaaatagatggctacattgaacagatgactaaaaggatgcctcctaagtacctatatcttgaaatatatattattgtgccttgctttcaatttgtgattttaaaatctagaaatcacctgttttatgtaataacaataaaatccttctttgttgaaaacatgcacaaataaagtttacaagctcaaaaaattaaacagcagtaacggtcaagctttccaacaataaaatacattttggtaaggttttcattttacaaaaactcaaaatagctttatgagttcacaaaataatatgatatttttcaagatattaacatattcttataccggaagagcatagaataaaatttacttggagattgagcatttgcttctttaagaaatacttcttttagtatttttactttaatattatgaaagctacataattacattcagattcattaactactccagtagttaatttttaaaacttatgatgaatagttttgtttaaaatatataacattggtaatatgcaaatctgaatctgtaataaagaaggatttgcattcctgatttttttttctgatacaaccaatgacaaaataactaatggttccacagaggataaaatgtctcaaatctgttggttctgaaggtgaagcgagatttttgtactgataccgtgtatcactgagataccaggaggaaatggaattaaactcagatagttcaaatggagagattttaatgaagggacgacctacagaggtgtcggcagggttggggggaatcagcgagatatgcttagaacccaccgactggcaaacctccccctgaagatggagaaggaggaaggagtgttactggaatgagagcttgagtccaggggaggaggatgggctgctgaggaggcgacaccatcctgaaagaagaatcctctgccagaggcttttcagggtcatttcttcacactctctctcttcaagtggtatttaaatttcttctttcattttccttctggtaacaaagaagtctgtggctcaaaagatgtttctctaagaccccatcctattaggtctctgagctgtccacaaagaaatgaaattttcactttccaggaacctgagggccgacgagtgggggcgggcaggagggccgagggaggcggaacaggatcgaggcgcgaggcgggagtcgagaaagcgagcggccgaggcgactctcagtgcgcggacgcgggcgcgcgcccgcgctcccttcgtcgactcacggcgagagcccaaccctgctgccgcgcgccaccc

SEQ ID NO: 12747 - RNA, 16906 nt, Homo sapiens
  source 1..16906: mol_type = other RNA
gatctcactttgttgcccaggctggtcttaaactcctggcctcaagtgatccccttgtttcagccccgcaaagtgctgggattacaggtgtgagccaccatgcccgtgcccagccacctcatgagtcttgatggggggcagagaccaacaactccacagaagccagatgcttgctttcccagcctctcttgcagctagggcttgggcatgtgatccaggctcagccaatcagatggcactgactcttggcatgacatgggctaaggaggggctgcagggaatccatttgggctggggtggcagctgcactgggagcgacatcagtttccagagggagcagcagaatctggcatcaggcttggggcgtggtaggtgcaaccagactctgcacccagcagcagtggcagaatgggttctctgtggagagtctgtgtattgctccttccgctgaggccaccagcatctgcctccatgaacccctcagagcctgtgagcaactcaacagccttgaattttttcccttcctgtttgaatgagccagggttgtttcactgcttgaactaagagccgttcctgacatgaaaactaagccacatctttttgacccaaagattctggcatcctaaaatacccatctcattttaagttaaaaataaatccatgtttgagcatctactgtttcagttactgtgctaggtgttacaaagctaactaagagtgacaagtaaataactatcatcaccatgataaacagagaatggaaccctggtttttggaatacagacacaaaatgattaattctgcctggaagcgttttggaacatttcagagaggtagtgagctgggccaagagaagagcatacgcaaggaatggtggcatgaagttgcctggtgtgtcctgagaagaaagatgggctaagaaggactggggtagggcagagaagggggtcactggaggtgaggctgggaaagtgagccaaggctcaaatgcaaactgtctgaacttcattttctgtgcaagcaggagaagccgctgacatgggtttggaagatggactgaagccggagaaaaatggaagcaagaaaccctctcacaagaggccataaccacaaccaagtccatgagattgaaaaggaaggcagatatttgaaaaatatttaaagagatgtgaggggtaggacaggcacagtggctcatgcctgtagtcccagcactttgggaggccgaggtgggcagatccacgaggtcaggagatcaagaccatcctaacatggtaaaaccccatctctactaacaatacaaaaaattagtcaggtgtggtggcacgtgcctgtagtcccagctactcaggaggctgaggcaggagaatcgcttgaacctgggaggcggaggttgcagtgagccgagattgtgccactgcaccctagcctaggcaacagagcaagactctgtctcaaaaaaaataaaaaaaaaaaaaagagagaaagagagagagagatgaggagttgctgcactgctgggtgtggagagccgaggaggattcaaagatggtcctgaagtcccagctggaagaagtaggcggcagcaatgtttttaatactgtaaattcatcacgtagcacaggtttggggtggagaaagaaaaattgcattggcttcagggcatgcccagatctttcctcatcttaggcgtttgctaatacatgcattttctaagctgatgtcttgcgtttaatcactgctccattcaaaagagagaaggaggttgtttcaaacctagttgatatcatttgacttccatgctattcacagggctattttatttgaaacaggtataccacagccttaaattgcaagttaatccaggatgttcctaggttggcagttaggaacatgtaattctttggaagggctaaaagtcagctctttaaattatctccatatgaaccttctctccaccttagggtggatccacttatttagtccactgccagtaccacactagaacccgggtggtcactggactccagaaacaacagtagccctctctctgttctgtctctttttgactatctctattctgttcctgaccctgatttctcctgccaagctcaattttgacagctgacaacggcaagccatggcttcccaaaacattattttcaggtcaacttataaatttcaagaacacatttggctccgcttcctgtggtactaagcctacttcttgacagcatttgcctttgttgtaaatagcaaagttcttctagttggatttttgctaagaagtgtgtggatgtggcatgtgacgacatctttagcttggattctagaaaggcactaccattgtgcatttggctaaaggaaacacattttacccgtgaatgccttctatttacaaatgctcagctagcacacaaagctaagtacaagcaataagtactatcctacaatgttactcatttctgaaagcacaaaatgatgactggtatagctttggagatgttttctggaaacccaataaaggaacagatctttgttattccacacctacaaagtcagaagatgcacagtcttttattcatgtttgaacaagcttccttcttgaacaatcaactataaagtgatgtgattctctactagaccaggaactccttgaggacagaatgagggtctaatccatattctaaatccacaccacctggcacaatacatgttgcatggttagggtcaactaagagttggttgaattaatcaataacacacagcaagagaattcacaaagagaggggagtaatcccccagcctcaatcactcggcaagtggaatcgctgggcactgattccagctctgtctcagtgcttgagacagagctgaatgtaatgtgaacatttcaaatgaacaggaaaactagactcacggataagcagtgtagtcatcaagacaacactgtcttggaggtttttctgaagttaaaaccatgctacataagcaataaattatgaaggctgagcatgtgaataaaatttaatgttgtcataaattttataacaaagttaatctgacacatttaatgacatgcataatcattagtatgcagcactgtaatcagacattgataataagcagttcacaccagtgactgtaagagtctttacttgtgttcagccaagccaactgcttggtatatttttctcccttcttagtcgttagttttccatacctacaataactatcagtggtgatgggcttctctgaccatgtgaataatttaatcctcaatgcacagatacagaaacccttgctgaagacagtgtggagcagagaaggctgtctccactccttccacctgaaacacctctgcagatggatatgggagctctgcctacagcccttggacctaaccacttcagtgtgttccagtgagtgtctggacctcggcctgaaagatttttccgaaactaaagaaaatttctctgacctaaagaccttaacctccaccccagaagctctcaccaaggactacagggaactggtggggaaaatccttatcccttactcctcaaggcacagggcagtaatgctgaggcttgtgcgccacacttgctcccagaggtccccagcgggctacctgcggtggtgaatgacctcctaacacgccccttgacggccttcctttccttgcctcacttctccactctcctaccagcattgcagggttcacatcccaaatataccactggcacttgaatcctggtctccaggtctgtttctggaaaaacccaagtaagacattgccccagtaatggggctagatgtctgaggcttcctcaagtatctacctcgaaagctcttactgctgtacacacatgcacatacacacacgtgcgtacaaccagtcacatctaagcaccccgaataccagcctgttgaaggtagcagagagctgcactataagccaaggctgctcccaagagccgctccatcactgaattggcgccccagcaagatgaaggaatgtaatcattggaaggatggagaatgttctctgaatcactgacaaattggaaggggtggagggcaagagtccacctggtggagagatggaaagagcgagagagcctggaatgataatgccattgcttagaaaaggctgctccagatgccatatctacagaaattgtacagcccaaacatctctgagcaataggtctctggtagtcttgatgtctagaccaacaattcccagttcattcttctcagggaaggagccaggatagtccagagactctcattctgctgttagattgaaagggttaggcacaacagccttggcaaagtcacaagggcaaattcacactaaagtgtaaatgacccacaactcctcttctatttttaggttggggaggtgctttagaacataaggaggaactaaagaatattcctgttacatacaaggcagagaaaagggaaactagtggtgacaagacaaatcatccctttgacatttggctggctctacctattacagctctgggggtgaggtgggaacaaaaagatgctgtgtaaagaagtatcttatgccatccctactgtagtgaggtgcagtttagaggggacactgatcaagcagagacccagagtgtttcgttccaagccagaaacagaaatgtataaaacacagcctttccagcatcagaaatgagtagtggtagtggagaactacccaaaacaggaaagaggaccacgtgaggtagagtgtcaaggccctacattccagtgcctctgctcatgactgtaattttgggtaggtcacttaaagtctctggacctcagttttgccatctgtgaaatagggataatactatccagcataaaattggttatgaggctcatgtagggcctgcctgggatgatgtgttgctaatggttaagaacacaacttctggggtctgactggacaggctgaaatccctgcttaacacgttccagcagagccctgggcgatctatttaacttttgttttctcacctgtaagctgagacgaaagtacccactttataagattattccaataattagttgaaataatgcatgcagagaattaagcatggtacttgttatttgttaaactagctattaaaatgtgtaaaatataaagtattgtatggattttaggacaatgcaaagactctttgcttgctgcaatagttcggggccctttcagatggctaaaggcagaatttgtatgtgtaaatatggtgtgcttgtctctgctctggatactgagggcttaccctgttattaaacttatttagtaaatattgaactgtcatgaggcctaacatttagttccagttattagataaaacatttgctttgaatggtatttgaattgccaggttctagattattctggttgacaaactcttcgtattttataaagaggctaaaattggtaagctatcacagaacagatgtgccattttcaaggtatattaaaccatgattcactgtaacattgttcctactggcaacaaattcagagcaggctggactttatttggtgaagaaacattgagtggaagagaaatgacattattttatgtatttacattttcaaattactgtggcttaaacctgttcagccaacattacccaccttcagtctgctaaataaatgattcagtacatttctaatttacagaattttttaacaaaagaaaatgtaatttgatagccaaatcaacgttaaacattatacatttaaaaaaccacaggcaaagacacaaacatgatgacactaacttttgttaaagtatgcttacctatggtttcctctgaggcacgttctttcatgctaagcttccaacataatatgaaaatgaaggagatgcattttgcaaagcaaaacagaccttaagcaaaatattatacttctcaaattaacactgttacaaagttttagaatttaataagttcattaatttaaaagtttggatgtctgagtccttctatcccaaaacaagatcttggagggtcttccacagccatgtaataccatggtcacatgaccctttccaaaattattaatctgaatttactatatgaggataaatctatctttttgaaaatatttaggaaaatgagcttggtatttataaaatgaagctctctttgggtggtatcctaagacacgtcaagccaatcagcctgtaactgtgaaaaaaacattggtaggtacaaaagtggggtgggagaggagtgacttaactttgttaagtgatgggaaagaaacactaatagcattatctcaataaaatgtgatttaaaaaaatttaaaatactaaatcattgaactgacaaagaaatataaatcattcagaaataaactcattaggtcatcaaatcctgttaaatctgcaattaggaagagcaaggtgtacaatccatacatttaaactcacaggctcactttgcacaacgtcaatttactccttaatatgttattaatacgcattttccaaaaggatgtattagtaaatggtacacatctacttcttggcaacatcatataacctggtacaacataagcattcttcttatagttaagaaatgtggatggtatcaaaattagaaaaataaatgccctattatgttgtggtcaggtttaaggcatgtgaattttatcttcatacaaaagattaaaatctagatattaaaaagtagtgcagtatcagtgatgctgcctcagttcccaaaatgtcacatcacaaaaatatcccataattgcctgtagtttattccttggctttcctcttttctctctgcatctttgtaacaattttttaaaagtggaaatataattgttggcaatgctaacagctgtagaaatgattacaagatgtggaaaagcataacaggaatgtcaagaatctgtttctggcagtaatatatatggaacattgttcaggacaaaagaggagaaggaagaaaaaaaggagaggggtttatcatctctaagaattttcaaactaaacctcattgcttaataggaaaaaaagattccatatttaaagttaagtcacctctaactactagctaaagcatgacatcaccagcactggagtcagcggaagtgtgtttttgaaggacagtgttgcaggagaatctggacaggttttagagccaggagagagaaaataattctacctctgacagttgaaggaccttaggcaaatcagtttacctctgctagactacactccaaaatttggacattcaaaaatttgatattaataaccacatgaaagtctcgtgttgaggtgaatatgtatttgttggtgaaagatatgttggtttttaaacagacagcactctgcaattgtaggctattgttttgttttgccagttgtcaaattctatccagctatacacacttgtgtggcctcctaatggtgtttttccagtggctaaaggtttatgaataagacacttttcctaatggaattaacccgatgcttttcttaaacatgtaaccttgagttcaccgcaaaaaacaatgcttcgattagagcaatgcatataataaaggttaccctcgtttcttagacactagacatcattcacaaaaagagaactgcttttgaaagggatgtatttgcactggaaagaatagttttctacttctaattataaatgatttattggtgaaagcaaaacaacagcctgtctgagaggcacttctatgagcatcctcacgtgtgatttgcaaggttgaagaagagggaaaaatgcctcaattgtaccaatggtgagaaaacacccaaagtacaaagcaggtttcaaaaaaaccatactcataaccaaggacaataataaagcaatgtgttgacatatactctataagtcttcctccataaatagtttatagaaattttgtaatttctgtaaatgcatcctataataattttgcatcttgctttttttttacatttaatatcaagtagatttctaaagggcaattatttgaaaattatcccaaatacatggggaaatatacatcaagtgaaaaaatgcagtgggtgatagagatatcaggaagcgcctcaaatatttctcatctcgttggagaaaaacaaacatgttctcatttagaatgagtgggagttacctaattgatttaggcctctatatttaacttctagtcaaaaaaggtagttctatctagcaacaatattatggggaacaaaagaaaaaattaactctctaaatttgcagtagggtcttttcttcagaagtaccaaatcccatctattaccagctccatgcttcaggcctaaaatggatctccctgaagcaatgacagaatttttgccaagtgactaggatataaacaccactttggttgcacagtgagacatatgctccaaagaaaactggttcaaaaacaggcaagtgggtttctacagaataaatgagagccctgtcaatggcttcatcttcagggctttgtgtctgtgcttgcgtggtggctcttgtttcatctatggataatggtggcacacagttttcataattccttacattaatgaactgctataaatttgtttttggtattctagagagtcctaacttcagcttctgggcaatgctgaggaggcaccctatattctagacttaccttttgcaaggtgtactctcagcattgtgggcgatttccatgggagaatattctatttaaagaactactgtcccagcataaaacaaaaaatcatttatgaagatgcaggagactcggaaagctctcaattattgtttgcacaagcacaatgtcacagcctcctttccccattccacaagggggtcaggaagagagtactcagctgtgagaaaagacatacagaagaattcatgtggtcatgagagcgaggacatggccgatcccccaaggaggatgtgtcatacacttcatgagcccaagagtgtgctgtagggtctgaagggcaagatgctggttcactgatgtaaaggagagggaaaaaagcttcaaccaactagaaaaacagtctctatgcatgctatttttgattttaaacacaggtatcaattccttctctcagagagtccattttaaaataggatacatttttaaaggaatatttaaaggacacattcattaaaatttattttaaaaacttttcaaaagaaacaaaaggtatgaattttatttaatccttgaggaaatggttcttttctcacacacataaatcactcattttgtttttctttatctcctttattaatctacattagaaaaataaacttttcatacactaagaacaaggaaaccactctcaattgacaaaatgttccaatccaacacaatgattactttcacctttaatttacaggcagccagattcaaaatccttaaagttgcttaaacttaaaaatgacaatgacaacctaaaaggtataatgttgattggaacagacatttaattggaaaattgatgattttccatttccaattaaatctctagatagaaatgaaaaaaattaaaaatcgtatttaagaaaagccaaatcttgggttgtgaggtatctttttaaggatgtttcagcagaaaaaaacaaaggctctcacaattgtgtagctgcctagattaagtgggtatcctgatcaaggagatgggggatgatttggctttagtattccaatgataaagtttataatgagaataacatgttgctacaaaatccagtctcttcctcagatgccttccacagagggcaggaagctttgtcagttttgtttgctgatgatgcctggttccgtcaacaaataacacctgtcacacggtgggtagtcaatatacatttgttgaataaatatgaaaaaaagaaatgtacaatatgtttgtgaagccaactgtgtgtgcattgctattgaggtacacaaaaagtctttgttttaaatttgagaatgaggactttcaatggaatatatctataaaaatgaaaaaaagacattactgtctggacttttgtacagcaagagaagaaaaaccactagccaagagccaactcacctgataggcctggatcaagcatgcagctgtggagaacacccctgggactctaactctggcactctgcaagctgggtacttgggcaggacagcagcagcactcatgaactgggcagcacctgttggtgagggctgatcacatggattctctcatcccagccttacaatcagtccttcaggtacatactttttctgactttgctgatgaggaaactatgcacagaggttacacagcttaacaaagggttctcacctaatgaacaatgaaatgggattttagcctttctttgcatctggtcttagagccaatacccaagaagcactgtactgtatgcattgtctcagagaaacttactcttcctgggcctcagtctttaaaaggtgggcagttgacttaataagaattaaagatcaatgattaaggttcaaggcactccaaaattctggtctttattgaaaaggctacagaagtctcaccttaataataccctatagacttgatattcttggttaattaaatattggaaaccaatttcatagtaattgaggtcagaaaaaagtactcatgacattttagaatatgatgacaaagccatagataaatttcaatgcacctgtaattacttaaaactgttatagcatgcaatgtgttaccacaacagccagagaaatactaatttactcagcctattcttctagaccagtaaacactaggattaaatagatattttcattgaatttgttctacccttcattgccatttatagatagcttacttgtcatagattactttctaattgttttatgtttcctaactagcctgcaatactttggcaaggacctcaaacaatagtagacagtaggtgtaaaatagatggctacattgaacagatgactaaaaggatgcctcctaagtacctatatcttgaaatatatattattgtgccttgctttcaatttgtgattttaaaatctagaaatcacctgttttatgtaataacaataaaatccttctttgttgaaaacatgcacaaataaagtttacaagctcaaaaaattaaacagcagtaacggtcaagctttccaacaataaaatacattttggtaaggttttcattttacaaaaactcaaaatagctttatgagttcacaaaataatatgatatttttcaagatattaacatattcttataccggaagagcatagaataaaatttacttggagattgagcatttgcttctttaagaaatacttcttttagtatttttactttaatattatgaaagctacataattacattcagattcattaactactccagtagttaatttttaaaacttatgatgaatagttttgtttaaaatatataacattggtaatatgcaaatctgaatctgtaataaagaaggatttgcattcctgatttttttttctgatacaaccaatgacaaaataactaatggttccacagaggataaaatgtctcaaatctgttggttctgaaggtgaagcgagatttttgtactgataccgtgtatcactgagataccaggaggaaatggaattaaactcagatagttcaaatggagagattttaatgaagggacgacctacagaggtgtcggcagggttggggggaatcagcgagatatgcttagaacccaccgactggcaaacctccccctgaagatggagaaggaggaaggagtgttactggaatgagagcttgagtccaggggaggaggatgggctgctgaggaggcgacaccatcctgaaagaagaatcctctgccagaggcttttcagggtcatttcttcacactctctctcttcaagtggtatttaaatttcttctttcattttccttctggtaacaaagaagtctgtggctcaaaagatgtttctctaagaccccatcctattaggtctctgagctgtgggaagtatttatacaattgcttgtgaatataagatccaggaatttccctaagatccctaacaaaattggtgataagtagtcccacatgttaatccagccacccacggatgacagcacttaccatttctttgataaatgtcaaatgcatttgaagtacctacctgaaatatttgtttaaatgctatctaatctattaattttatatatgtgtgagtctgttttgtataccttctgattataggataaatgtaaataaatccaaagagtaatcaaagctaccactttcaagaagccttctttgtagaaccggaagagtcttaaataggcttttcaggtatgcatctcttattatcgctgaactccaagtcctgcaaggcaggcatcatgtgtgggtcacctttacagtaggcacaggccttaaaacagtgacatgcacattgcaggcactccataaatgtttgctgaattggctaaaccttggtttgttcccataatcaaccaccacaaacagcacacagataattacttcttggaaagattccaactagtgtttgatgttacctacgtggtttttctctcaagatcttaagagcagctctgtaggattacattattttctgttttttttttcctttgaccttaatgtcatctacttcaataacagcttcatacaaaattcctaccagcacataccacagcagattcaaggccttgttttaaaaatggtgccagcttctcttaatttggaagatatattgtctctcctgaacatgggctaagaaaatgtataatttggtattaacataagagctgaagacactttaaatgcattgtttcatttttataagataaaaaaaattttaagaatcaaaatgttatcaacagacttgtccttcattaaaaagtaaaactgcatttgcctacattttatgaaagtgtccaattatgaacaattttgaaatgtaacttttaaaaatgtaaacagcaaaaatgttgtatttaaaataaatctggaaaggcagaaaaacaaaaaatacccagaagacagagtttttggtgaaagttaagatatttcatctttgaacaacttagaatctttcctgcattttatagtctagttccaggcattaatttgaaataaccttggaatcctaaatctaacacccttcggaacaaagtagcttttctcttctgctttatgagcaaatggactaaatactagggaatggtactgtctgggcctttgaaccaagattgaaagagatgaaatcctatatgatatgtataaacattagagaatccattttgatttaataaaaggttgaatttgttctatatcctgtgagaaaatggttcccttttcctgaaaatgttacctcattccaacaatagaaagttggtttttttccagggtgtggtgttggcgggggacagagttgccatgaatatggcatctatgaagactgctgttatattcatttctcaaaatgcactgtggtaggaaattcagaacgcagtgagagaaaataaatgtttgacttcaaaatataaggccgcatttaaagcagaaggtaaagtatagaacagttgacagtataaattctttatctgcaatcttgcagttccctaaatctctgtaacacatcacttttaaaagcctcagataagtggttctataataatttaccaataattcaacccctcaaaagtcttagcaagttaaaccttataatcttacattttagaaatgacccaacttgatccttttattcttcagaatatctctctcaaattttcatttgtttttcattaattgatgaataatgagacattttaggtacctgtccacaaagaaatgaaattttcactttccaggaacctaacaaatgaaaagatagaaatcaattccaacagaatattaccaaagaaatcttttagaatggactgttaaaattatttatttgtatttatctggctctactatttgtggtacatttccacttcaaagctaaacctcaaataacatcatagtgagtggttgacttcatgtttaactgagatcttgaagactgaaaaagaccacgacaaacacacatctattttcttggctactgcatccgtgttcatcaccattctgatagtctgcaatgtattgcagctcaccctttgggaaggactaaagtagacatctgtttgttctgcttactcagcattcctaccctaattttcctttggagaacccctttattctagaccacgtgaagctaatgccaaaccccattccaggggatgcacctgaatccaacctccatcatctaaacagtgccttctccacgttcagagaagagcaagtgactcaaactgccctcataagaacagacctgggacttctgctgcaaatattgaagagtaagtactcttttttcttgctaggactaagctggtagtaccttctatgaggctatcatatggaaacaacttgtctgaaaatgaagccacaactagaaaacagatcctggtaacccggattgatggatccagccctaccttaaatggcaagacctaacccgaggctttttgcatcaaccaataaagtccttaagccagtttgagttggttttgtcacttgcagctaaaagaattctgactctaacaatgtgacaatagcaaaaataaacataactgcttttgaggtttctaatggattttcctccctatatacatgatttcatttaatcctcacaattcaggaaagcacatatctattaacattaaattaatattcattattttgaacacatgctatgtggataagggatgaggaaagccaaggaagtaatcaacgtgaaatctcacttatatgggagggaagtggaggttacatatctcagggcacttaacagatatcatcaaatgaaagaataaacagtgtgtgggagaggcagtaggtgattcttcatcaattcctggatgaaaaattaggagataatgaactccgaacaggcagcctaatgagaatggctcaagcaacaggacatagagagggagttaggttagacatggggttcttgggaattttcacctcgtgggggggcgggggggtcgtgcagctgttgtcagtgggaaagggaaaaaggaaaaggctgagtttggaaggcagggagggaggagacaatgtgagtcagtgaaaaagggcccttagaatgacaagtctggaccagagagaggctaagactgaaaatacaagttgggtaaccactggcatacagatggcagttcaggcttgggcactgcccaccagagcctcagcatgaagagaagagggggaggctggccaccacctccctctaggtaatcgtcatcctgatgctgagctcctgaaaacaggctctttcactcgccccatctcttgctcttgattgcaacccggcattcaggaggcaccctgtaatatctgtggagtgaccgacaacacagcgccagggcactgagaagatcccagggcgccagggactggttctacaagggtgcccctcccggtcccctccagcgcgccgccagagctgccagtcttggctgctacacgggaggcagcctcattatgcagctctcacctcttaaattagttcatgctctcacattaggtgtaatcacagcttgcaacgctttctggggatgtctcagaaagatctgagttgaaaaaatatttttgtgtcattttaatttaaagtaaaattgctgcttcttccccgcccctttctttcctcctggcccacccagcgaccctggccggccgtgctcaacgggggcgggggtcggaggtgagatttcctccacataattccttaaacagctatcaactaagtctcaaagaaaaaaaaaagagatctagaagcagagacgtggctgctggcgatcccaaagctggtgttcgctcttgggggagagcgtaccctgggggaggccgggaggccgggccagaggctagcccagaggcagagggcaggagcgctcagccggcgccccgcgtctctccagctcccgacgctgcgctggctccgctgagcacgccaggatcaaggtcgcctggtggggaccggagcgccaggagcctgtgggaagcgttccagccggcctctgactgggatccggcgccgcgtttctgctttggacttgactgacaggtccccccgccctcccgccgccctactaccagcctgggttcatccttcagggctacgtctaccgcacccgggctggaaagcctggagcgcgcccttcctctcctcatcttctcagctctcctttctccctgccacttggcaaagctgcattttgactttcacgttttggactacgtgtgtgtagttccaagtccatgcgtggcacgaaaatccacttagggtaaaaattattctcgaaaaatcgcccatctcaggatctggtgtctacactcaaggctaggaggtgcaggtacgggtgcgtaaagcatgccgtaagggtgcacagtaaataaaaagtacggatgcaaaatgtaaattttaagtgcaaaacagaaaagcagtactcgttgccgccccgcacgctgggttttaaggggcacgaaggtgggcctcggctgcttttgctcagccccgcgtcctcagcgcccggcccagtacccggtactccgtaggggttcaatgatctcccctgaataagtgaacgaattaacaaatgaatgaatgaccgctcgatccgacctccgcggccggcagagcagtcgctggagaggcgggagagagcgagaggccaagctccaccatcgcggccgccggctggggcagagggacacggagacactcggcgccccggctccgcaccgagtccccg

SEQ ID NO: 12748 - RNA, 12424 nt, Homo sapiens
  source 1..12424: mol_type = other RNA
gatctcactttgttgcccaggctggtcttaaactcctggcctcaagtgatccccttgtttcagccccgcaaagtgctgggattacaggtgtgagccaccatgcccgtgcccagccacctcatgagtcttgatggggggcagagaccaacaactccacagaagccagatgcttgctttcccagcctctcttgcagctagggcttgggcatgtgatccaggctcagccaatcagatggcactgactcttggcatgacatgggctaaggaggggctgcagggaatccatttgggctggggtggcagctgcactgggagcgacatcagtttccagagggagcagcagaatctggcatcaggcttggggcgtggtaggtgcaaccagactctgcacccagcagcagtggcagaatgggttctctgtggagagtctgtgtattgctccttccgctgaggccaccagcatctgcctccatgaacccctcagagcctgtgagcaactcaacagccttgaattttttcccttcctgtttgaatgagccagggttgtttcactgcttgaactaagagccgttcctgacatgaaaactaagccacatctttttgacccaaagattctggcatcctaaaatacccatctcattttaagttaaaaataaatccatgtttgagcatctactgtttcagttactgtgctaggtgttacaaagctaactaagagtgacaagtaaataactatcatcaccatgataaacagagaatggaaccctggtttttggaatacagacacaaaatgattaattctgcctggaagcgttttggaacatttcagagaggtagtgagctgggccaagagaagagcatacgcaaggaatggtggcatgaagttgcctggtgtgtcctgagaagaaagatgggctaagaaggactggggtagggcagagaagggggtcactggaggtgaggctgggaaagtgagccaaggctcaaatgcaaactgtctgaacttcattttctgtgcaagcaggagaagccgctgacatgggtttggaagatggactgaagccggagaaaaatggaagcaagaaaccctctcacaagaggccataaccacaaccaagtccatgagattgaaaaggaaggcagatatttgaaaaatatttaaagagatgtgaggggtaggacaggcacagtggctcatgcctgtagtcccagcactttgggaggccgaggtgggcagatccacgaggtcaggagatcaagaccatcctaacatggtaaaaccccatctctactaacaatacaaaaaattagtcaggtgtggtggcacgtgcctgtagtcccagctactcaggaggctgaggcaggagaatcgcttgaacctgggaggcggaggttgcagtgagccgagattgtgccactgcaccctagcctaggcaacagagcaagactctgtctcaaaaaaaataaaaaaaaaaaaaagagagaaagagagagagagatgaggagttgctgcactgctgggtgtggagagccgaggaggattcaaagatggtcctgaagtcccagctggaagaagtaggcggcagcaatgtttttaatactgtaaattcatcacgtagcacaggtttggggtggagaaagaaaaattgcattggcttcagggcatgcccagatctttcctcatcttaggcgtttgctaatacatgcattttctaagctgatgtcttgcgtttaatcactgctccattcaaaagagagaaggaggttgtttcaaacctagttgatatcatttgacttccatgctattcacagggctattttatttgaaacaggtataccacagccttaaattgcaagttaatccaggatgttcctaggttggcagttaggaacatgtaattctttggaagggctaaaagtcagctctttaaattatctccatatgaaccttctctccaccttagggtggatccacttatttagtccactgccagtaccacactagaacccgggtggtcactggactccagaaacaacagtagccctctctctgttctgtctctttttgactatctctattctgttcctgaccctgatttctcctgccaagctcaattttgacagctgacaacggcaagccatggcttcccaaaacattattttcaggtcaacttataaatttcaagaacacatttggctccgcttcctgtggtactaagcctacttcttgacagcatttgcctttgttgtaaatagcaaagttcttctagttggatttttgctaagaagtgtgtggatgtggcatgtgacgacatctttagcttggattctagaaaggcactaccattgtgcatttggctaaaggaaacacattttacccgtgaatgccttctatttacaaatgctcagctagcacacaaagctaagtacaagcaataagtactatcctacaatgttactcatttctgaaagcacaaaatgatgactggtatagctttggagatgttttctggaaacccaataaaggaacagatctttgttattccacacctacaaagtcagaagatgcacagtcttttattcatgtttgaacaagcttccttcttgaacaatcaactataaagtgatgtgattctctactagaccaggaactccttgaggacagaatgagggtctaatccatattctaaatccacaccacctggcacaatacatgttgcatggttagggtcaactaagagttggttgaattaatcaataacacacagcaagagaattcacaaagagaggggagtaatcccccagcctcaatcactcggcaagtggaatcgctgggcactgattccagctctgtctcagtgcttgagacagagctgaatgtaatgtgaacatttcaaatgaacaggaaaactagactcacggataagcagtgtagtcatcaagacaacactgtcttggaggtttttctgaagttaaaaccatgctacataagcaataaattatgaaggctgagcatgtgaataaaatttaatgttgtcataaattttataacaaagttaatctgacacatttaatgacatgcataatcattagtatgcagcactgtaatcagacattgataataagcagttcacaccagtgactgtaagagtctttacttgtgttcagccaagccaactgcttggtatatttttctcccttcttagtcgttagttttccatacctacaataactatcagtggtgatgggcttctctgaccatgtgaataatttaatcctcaatgcacagatacagaaacccttgctgaagacagtgtggagcagagaaggctgtctccactccttccacctgaaacacctctgcagatggatatgggagctctgcctacagcccttggacctaaccacttcagtgtgttccagtgagtgtctggacctcggcctgaaagatttttccgaaactaaagaaaatttctctgacctaaagaccttaacctccaccccagaagctctcaccaaggactacagggaactggtggggaaaatccttatcccttactcctcaaggcacagggcagtaatgctgaggcttgtgcgccacacttgctcccagaggtccccagcgggctacctgcggtggtgaatgacctcctaacacgccccttgacggccttcctttccttgcctcacttctccactctcctaccagcattgcagggttcacatcccaaatataccactggcacttgaatcctggtctccaggtctgtttctggaaaaacccaagtaagacattgccccagtaatggggctagatgtctgaggcttcctcaagtatctacctcgaaagctcttactgctgtacacacatgcacatacacacacgtgcgtacaaccagtcacatctaagcaccccgaataccagcctgttgaaggtagcagagagctgcactataagccaaggctgctcccaagagccgctccatcactgaattggcgccccagcaagatgaaggaatgtaatcattggaaggatggagaatgttctctgaatcactgacaaattggaaggggtggagggcaagagtccacctggtggagagatggaaagagcgagagagcctggaatgataatgccattgcttagaaaaggctgctccagatgccatatctacagaaattgtacagcccaaacatctctgagcaataggtctctggtagtcttgatgtctagaccaacaattcccagttcattcttctcagggaaggagccaggatagtccagagactctcattctgctgttagattgaaagggttaggcacaacagccttggcaaagtcacaagggcaaattcacactaaagtgtaaatgacccacaactcctcttctatttttaggttggggaggtgctttagaacataaggaggaactaaagaatattcctgttacatacaaggcagagaaaagggaaactagtggtgacaagacaaatcatccctttgacatttggctggctctacctattacagctctgggggtgaggtgggaacaaaaagatgctgtgtaaagaagtatcttatgccatccctactgtagtgaggtgcagtttagaggggacactgatcaagcagagacccagagtgtttcgttccaagccagaaacagaaatgtataaaacacagcctttccagcatcagaaatgagtagtggtagtggagaactacccaaaacaggaaagaggaccacgtgaggtagagtgtcaaggccctacattccagtgcctctgctcatgactgtaattttgggtaggtcacttaaagtctctggacctcagttttgccatctgtgaaatagggataatactatccagcataaaattggttatgaggctcatgtagggcctgcctgggatgatgtgttgctaatggttaagaacacaacttctggggtctgactggacaggctgaaatccctgcttaacacgttccagcagagccctgggcgatctatttaacttttgttttctcacctgtaagctgagacgaaagtacccactttataagattattccaataattagttgaaataatgcatgcagagaattaagcatggtacttgttatttgttaaactagctattaaaatgtgtaaaatataaagtattgtatggattttaggacaatgcaaagactctttgcttgctgcaatagttcggggccctttcagatggctaaaggcagaatttgtatgtgtaaatatggtgtgcttgtctctgctctggatactgagggcttaccctgttattaaacttatttagtaaatattgaactgtcatgaggcctaacatttagttccagttattagataaaacatttgctttgaatggtatttgaattgccaggttctagattattctggttgacaaactcttcgtattttataaagaggctaaaattggtaagctatcacagaacagatgtgccattttcaaggtatattaaaccatgattcactgtaacattgttcctactggcaacaaattcagagcaggctggactttatttggtgaagaaacattgagtggaagagaaatgacattattttatgtatttacattttcaaattactgtggcttaaacctgttcagccaacattacccaccttcagtctgctaaataaatgattcagtacatttctaatttacagaattttttaacaaaagaaaatgtaatttgatagccaaatcaacgttaaacattatacatttaaaaaaccacaggcaaagacacaaacatgatgacactaacttttgttaaagtatgcttacctatggtttcctctgaggcacgttctttcatgctaagcttccaacataatatgaaaatgaaggagatgcattttgcaaagcaaaacagaccttaagcaaaatattatacttctcaaattaacactgttacaaagttttagaatttaataagttcattaatttaaaagtttggatgtctgagtccttctatcccaaaacaagatcttggagggtcttccacagccatgtaataccatggtcacatgaccctttccaaaattattaatctgaatttactatatgaggataaatctatctttttgaaaatatttaggaaaatgagcttggtatttataaaatgaagctctctttgggtggtatcctaagacacgtcaagccaatcagcctgtaactgtgaaaaaaacattggtaggtacaaaagtggggtgggagaggagtgacttaactttgttaagtgatgggaaagaaacactaatagcattatctcaataaaatgtgatttaaaaaaatttaaaatactaaatcattgaactgacaaagaaatataaatcattcagaaataaactcattaggtcatcaaatcctgttaaatctgcaattaggaagagcaaggtgtacaatccatacatttaaactcacaggctcactttgcacaacgtcaatttactccttaatatgttattaatacgcattttccaaaaggatgtattagtaaatggtacacatctacttcttggcaacatcatataacctggtacaacataagcattcttcttatagttaagaaatgtggatggtatcaaaattagaaaaataaatgccctattatgttgtggtcaggtttaaggcatgtgaattttatcttcatacaaaagattaaaatctagatattaaaaagtagtgcagtatcagtgatgctgcctcagttcccaaaatgtcacatcacaaaaatatcccataattgcctgtagtttattccttggctttcctcttttctctctgcatctttgtaacaattttttaaaagtggaaatataattgttggcaatgctaacagctgtagaaatgattacaagatgtggaaaagcataacaggaatgtcaagaatctgtttctggcagtaatatatatggaacattgttcaggacaaaagaggagaaggaagaaaaaaaggagaggggtttatcatctctaagaattttcaaactaaacctcattgcttaataggaaaaaaagattccatatttaaagttaagtcacctctaactactagctaaagcatgacatcaccagcactggagtcagcggaagtgtgtttttgaaggacagtgttgcaggagaatctggacaggttttagagccaggagagagaaaataattctacctctgacagttgaaggaccttaggcaaatcagtttacctctgctagactacactccaaaatttggacattcaaaaatttgatattaataaccacatgaaagtctcgtgttgaggtgaatatgtatttgttggtgaaagatatgttggtttttaaacagacagcactctgcaattgtaggctattgttttgttttgccagttgtcaaattctatccagctatacacacttgtgtggcctcctaatggtgtttttccagtggctaaaggtttatgaataagacacttttcctaatggaattaacccgatgcttttcttaaacatgtaaccttgagttcaccgcaaaaaacaatgcttcgattagagcaatgcatataataaaggttaccctcgtttcttagacactagacatcattcacaaaaagagaactgcttttgaaagggatgtatttgcactggaaagaatagttttctacttctaattataaatgatttattggtgaaagcaaaacaacagcctgtctgagaggcacttctatgagcatcctcacgtgtgatttgcaaggttgaagaagagggaaaaatgcctcaattgtaccaatggtgagaaaacacccaaagtacaaagcaggtttcaaaaaaaccatactcataaccaaggacaataataaagcaatgtgttgacatatactctataagtcttcctccataaatagtttatagaaattttgtaatttctgtaaatgcatcctataataattttgcatcttgctttttttttacatttaatatcaagtagatttctaaagggcaattatttgaaaattatcccaaatacatggggaaatatacatcaagtgaaaaaatgcagtgggtgatagagatatcaggaagcgcctcaaatatttctcatctcgttggagaaaaacaaacatgttctcatttagaatgagtgggagttacctaattgatttaggcctctatatttaacttctagtcaaaaaaggtagttctatctagcaacaatattatggggaacaaaagaaaaaattaactctctaaatttgcagtagggtcttttcttcagaagtaccaaatcccatctattaccagctccatgcttcaggcctaaaatggatctccctgaagcaatgacagaatttttgccaagtgactaggatataaacaccactttggttgcacagtgagacatatgctccaaagaaaactggttcaaaaacaggcaagtgggtttctacagaataaatgagagccctgtcaatggcttcatcttcagggctttgtgtctgtgcttgcgtggtggctcttgtttcatctatggataatggtggcacacagttttcataattccttacattaatgaactgctataaatttgtttttggtattctagagagtcctaacttcagcttctgggcaatgctgaggaggcaccctatattctagacttaccttttgcaaggtgtactctcagcattgtgggcgatttccatgggagaatattctatttaaagaactactgtcccagcataaaacaaaaaatcatttatgaagatgcaggagactcggaaagctctcaattattgtttgcacaagcacaatgtcacagcctcctttccccattccacaagggggtcaggaagagagtactcagctgtgagaaaagacatacagaagaattcatgtggtcatgagagcgaggacatggccgatcccccaaggaggatgtgtcatacacttcatgagcccaagagtgtgctgtagggtctgaagggcaagatgctggttcactgatgtaaaggagagggaaaaaagcttcaaccaactagaaaaacagtctctatgcatgctatttttgattttaaacacaggtatcaattccttctctcagagagtccattttaaaataggatacatttttaaaggaatatttaaaggacacattcattaaaatttattttaaaaacttttcaaaagaaacaaaaggtatgaattttatttaatccttgaggaaatggttcttttctcacacacataaatcactcattttgtttttctttatctcctttattaatctacattagaaaaataaacttttcatacactaagaacaaggaaaccactctcaattgacaaaatgttccaatccaacacaatgattactttcacctttaatttacaggcagccagattcaaaatccttaaagttgcttaaacttaaaaatgacaatgacaacctaaaaggtataatgttgattggaacagacatttaattggaaaattgatgattttccatttccaattaaatctctagatagaaatgaaaaaaattaaaaatcgtatttaagaaaagccaaatcttgggttgtgaggtatctttttaaggatgtttcagcagaaaaaaacaaaggctctcacaattgtgtagctgcctagattaagtgggtatcctgatcaaggagatgggggatgatttggctttagtattccaatgataaagtttataatgagaataacatgttgctacaaaatccagtctcttcctcagatgccttccacagagggcaggaagctttgtcagttttgtttgctgatgatgcctggttccgtcaacaaataacacctgtcacacggtgggtagtcaatatacatttgttgaataaatatgaaaaaaagaaatgtacaatatgtttgtgaagccaactgtgtgtgcattgctattgaggtacacaaaaagtctttgttttaaatttgagaatgaggactttcaatggaatatatctataaaaatgaaaaaaagacattactgtctggacttttgtacagcaagagaagaaaaaccactagccaagagccaactcacctgataggcctggatcaagcatgcagctgtggagaacacccctgggactctaactctggcactctgcaagctgggtacttgggcaggacagcagcagcactcatgaactgggcagcacctgttggtgagggctgatcacatggattctctcatcccagccttacaatcagtccttcaggtacatactttttctgactttgctgatgaggaaactatgcacagaggttacacagcttaacaaagggttctcacctaatgaacaatgaaatgggattttagcctttctttgcatctggtcttagagccaatacccaagaagcactgtactgtatgcattgtctcagagaaacttactcttcctgggcctcagtctttaaaaggtgggcagttgacttaataagaattaaagatcaatgattaaggttcaaggcactccaaaattctggtctttattgaaaaggctacagaagtctcaccttaataataccctatagacttgatattcttggttaattaaatattggaaaccaatttcatagtaattgaggtcagaaaaaagtactcatgacattttagaatatgatgacaaagccatagataaatttcaatgcacctgtaattacttaaaactgttatagcatgcaatgtgttaccacaacagccagagaaatactaatttactcagcctattcttctagaccagtaaacactaggattaaatagatattttcattgaatttgttctacccttcattgccatttatagatagcttacttgtcatagattactttctaattgttttatgtttcctaactagcctgcaatactttggcaaggacctcaaacaatagtagacagtaggtgtaaaatagatggctacattgaacagatgactaaaaggatgcctcctaagtacctatatcttgaaatatatattattgtgccttgctttcaatttgtgattttaaaatctagaaatcacctgttttatgtaataacaataaaatccttctttgttgaaaacatgcacaaataaagtttacaagctcaaaaaattaaacagcagtaacggtcaagctttccaacaataaaatacattttggtaaggttttcattttacaaaaactcaaaatagctttatgagttcacaaaataatatgatatttttcaagatattaacatattcttataccggaagagcatagaataaaatttacttggagattgagcatttgcttctttaagaaatacttcttttagtatttttactttaatattatgaaagctacataattacattcagattcattaactactccagtagttaatttttaaaacttatgatgaatagttttgtttaaaatatataacattggtaatatgcaaatctgaatctgtaataaagaaggatttgcattcctgatttttttttctgatacaaccaatgacaaaataactaatggttccacagaggataaaatgtctcaaatctgttggttctgaaggtgaagcgagatttttgtactgataccgtgtatcactgagataccaggaggaaatggaattaaactcagatagttcaaatggagagattttaatgaagggacgacctacagaggtgtcggcagggttggggggaatcagcgagatatgcttagaacccaccgactggcaaacctccccctgaagatggagaaggaggaaggagtgttactggaatgagagcttgagtccaggggaggaggatgggctgctgaggaggcgacaccatcctgaaagaagaatcctctgccagaggcttttcagggtcatttcttcacactctctgcagggaagcacggagacagcaggaagaaatatcctaacctcactctcttccctctacaggtgcttccattggccaaatccacccagaggccagttggtggcgatcagctctcttcaagtggtatttaaatttcttctttcattttccttctggtaacaaagaagtctgtggctcaaaagatgtttctctaagaccccatcctattaggtctctgagattttagaaatgacccaacttgatccttttattcttcagaatatctctctcaaattttcatttgtttttcattaattgatgaataatgagacattttaggtacctgagggccgacgagtgggggcgggcaggagggccgagggaggcggaacaggatcgaggcgcgaggcgggagtcgagaaagcgagcggccgaggcgactctcagtgcgcggacgcgggcgcgcgcccgcgctcccttcgtcgactcacggcgagagcccaaccctgctgccgcgcgccaccc

SEQ ID NO: 12749 - RNA, 15273 nt, Homo sapiens
  source 1..15273: mol_type = other RNA
gatctcactttgttgcccaggctggtcttaaactcctggcctcaagtgatccccttgtttcagccccgcaaagtgctgggattacaggtgtgagccaccatgcccgtgcccagccacctcatgagtcttgatggggggcagagaccaacaactccacagaagccagatgcttgctttcccagcctctcttgcagctagggcttgggcatgtgatccaggctcagccaatcagatggcactgactcttggcatgacatgggctaaggaggggctgcagggaatccatttgggctggggtggcagctgcactgggagcgacatcagtttccagagggagcagcagaatctggcatcaggcttggggcgtggtaggtgcaaccagactctgcacccagcagcagtggcagaatgggttctctgtggagagtctgtgtattgctccttccgctgaggccaccagcatctgcctccatgaacccctcagagcctgtgagcaactcaacagccttgaattttttcccttcctgtttgaatgagccagggttgtttcactgcttgaactaagagccgttcctgacatgaaaactaagccacatctttttgacccaaagattctggcatcctaaaatacccatctcattttaagttaaaaataaatccatgtttgagcatctactgtttcagttactgtgctaggtgttacaaagctaactaagagtgacaagtaaataactatcatcaccatgataaacagagaatggaaccctggtttttggaatacagacacaaaatgattaattctgcctggaagcgttttggaacatttcagagaggtagtgagctgggccaagagaagagcatacgcaaggaatggtggcatgaagttgcctggtgtgtcctgagaagaaagatgggctaagaaggactggggtagggcagagaagggggtcactggaggtgaggctgggaaagtgagccaaggctcaaatgcaaactgtctgaacttcattttctgtgcaagcaggagaagccgctgacatgggtttggaagatggactgaagccggagaaaaatggaagcaagaaaccctctcacaagaggccataaccacaaccaagtccatgagattgaaaaggaaggcagatatttgaaaaatatttaaagagatgtgaggggtaggacaggcacagtggctcatgcctgtagtcccagcactttgggaggccgaggtgggcagatccacgaggtcaggagatcaagaccatcctaacatggtaaaaccccatctctactaacaatacaaaaaattagtcaggtgtggtggcacgtgcctgtagtcccagctactcaggaggctgaggcaggagaatcgcttgaacctgggaggcggaggttgcagtgagccgagattgtgccactgcaccctagcctaggcaacagagcaagactctgtctcaaaaaaaataaaaaaaaaaaaaagagagaaagagagagagagatgaggagttgctgcactgctgggtgtggagagccgaggaggattcaaagatggtcctgaagtcccagctggaagaagtaggcggcagcaatgtttttaatactgtaaattcatcacgtagcacaggtttggggtggagaaagaaaaattgcattggcttcagggcatgcccagatctttcctcatcttaggcgtttgctaatacatgcattttctaagctgatgtcttgcgtttaatcactgctccattcaaaagagagaaggaggttgtttcaaacctagttgatatcatttgacttccatgctattcacagggctattttatttgaaacaggtataccacagccttaaattgcaagttaatccaggatgttcctaggttggcagttaggaacatgtaattctttggaagggctaaaagtcagctctttaaattatctccatatgaaccttctctccaccttagggtggatccacttatttagtccactgccagtaccacactagaacccgggtggtcactggactccagaaacaacagtagccctctctctgttctgtctctttttgactatctctattctgttcctgaccctgatttctcctgccaagctcaattttgacagctgacaacggcaagccatggcttcccaaaacattattttcaggtcaacttataaatttcaagaacacatttggctccgcttcctgtggtactaagcctacttcttgacagcatttgcctttgttgtaaatagcaaagttcttctagttggatttttgctaagaagtgtgtggatgtggcatgtgacgacatctttagcttggattctagaaaggcactaccattgtgcatttggctaaaggaaacacattttacccgtgaatgccttctatttacaaatgctcagctagcacacaaagctaagtacaagcaataagtactatcctacaatgttactcatttctgaaagcacaaaatgatgactggtatagctttggagatgttttctggaaacccaataaaggaacagatctttgttattccacacctacaaagtcagaagatgcacagtcttttattcatgtttgaacaagcttccttcttgaacaatcaactataaagtgatgtgattctctactagaccaggaactccttgaggacagaatgagggtctaatccatattctaaatccacaccacctggcacaatacatgttgcatggttagggtcaactaagagttggttgaattaatcaataacacacagcaagagaattcacaaagagaggggagtaatcccccagcctcaatcactcggcaagtggaatcgctgggcactgattccagctctgtctcagtgcttgagacagagctgaatgtaatgtgaacatttcaaatgaacaggaaaactagactcacggataagcagtgtagtcatcaagacaacactgtcttggaggtttttctgaagttaaaaccatgctacataagcaataaattatgaaggctgagcatgtgaataaaatttaatgttgtcataaattttataacaaagttaatctgacacatttaatgacatgcataatcattagtatgcagcactgtaatcagacattgataataagcagttcacaccagtgactgtaagagtctttacttgtgttcagccaagccaactgcttggtatatttttctcccttcttagtcgttagttttccatacctacaataactatcagtggtgatgggcttctctgaccatgtgaataatttaatcctcaatgcacagatacagaaacccttgctgaagacagtgtggagcagagaaggctgtctccactccttccacctgaaacacctctgcagatggatatgggagctctgcctacagcccttggacctaaccacttcagtgtgttccagtgagtgtctggacctcggcctgaaagatttttccgaaactaaagaaaatttctctgacctaaagaccttaacctccaccccagaagctctcaccaaggactacagggaactggtggggaaaatccttatcccttactcctcaaggcacagggcagtaatgctgaggcttgtgcgccacacttgctcccagaggtccccagcgggctacctgcggtggtgaatgacctcctaacacgccccttgacggccttcctttccttgcctcacttctccactctcctaccagcattgcagggttcacatcccaaatataccactggcacttgaatcctggtctccaggtctgtttctggaaaaacccaagtaagacattgccccagtaatggggctagatgtctgaggcttcctcaagtatctacctcgaaagctcttactgctgtacacacatgcacatacacacacgtgcgtacaaccagtcacatctaagcaccccgaataccagcctgttgaaggtagcagagagctgcactataagccaaggctgctcccaagagccgctccatcactgaattggcgccccagcaagatgaaggaatgtaatcattggaaggatggagaatgttctctgaatcactgacaaattggaaggggtggagggcaagagtccacctggtggagagatggaaagagcgagagagcctggaatgataatgccattgcttagaaaaggctgctccagatgccatatctacagaaattgtacagcccaaacatctctgagcaataggtctctggtagtcttgatgtctagaccaacaattcccagttcattcttctcagggaaggagccaggatagtccagagactctcattctgctgttagattgaaagggttaggcacaacagccttggcaaagtcacaagggcaaattcacactaaagtgtaaatgacccacaactcctcttctatttttaggttggggaggtgctttagaacataaggaggaactaaagaatattcctgttacatacaaggcagagaaaagggaaactagtggtgacaagacaaatcatccctttgacatttggctggctctacctattacagctctgggggtgaggtgggaacaaaaagatgctgtgtaaagaagtatcttatgccatccctactgtagtgaggtgcagtttagaggggacactgatcaagcagagacccagagtgtttcgttccaagccagaaacagaaatgtataaaacacagcctttccagcatcagaaatgagtagtggtagtggagaactacccaaaacaggaaagaggaccacgtgaggtagagtgtcaaggccctacattccagtgcctctgctcatgactgtaattttgggtaggtcacttaaagtctctggacctcagttttgccatctgtgaaatagggataatactatccagcataaaattggttatgaggctcatgtagggcctgcctgggatgatgtgttgctaatggttaagaacacaacttctggggtctgactggacaggctgaaatccctgcttaacacgttccagcagagccctgggcgatctatttaacttttgttttctcacctgtaagctgagacgaaagtacccactttataagattattccaataattagttgaaataatgcatgcagagaattaagcatggtacttgttatttgttaaactagctattaaaatgtgtaaaatataaagtattgtatggattttaggacaatgcaaagactctttgcttgctgcaatagttcggggccctttcagatggctaaaggcagaatttgtatgtgtaaatatggtgtgcttgtctctgctctggatactgagggcttaccctgttattaaacttatttagtaaatattgaactgtcatgaggcctaacatttagttccagttattagataaaacatttgctttgaatggtatttgaattgccaggttctagattattctggttgacaaactcttcgtattttataaagaggctaaaattggtaagctatcacagaacagatgtgccattttcaaggtatattaaaccatgattcactgtaacattgttcctactggcaacaaattcagagcaggctggactttatttggtgaagaaacattgagtggaagagaaatgacattattttatgtatttacattttcaaattactgtggcttaaacctgttcagccaacattacccaccttcagtctgctaaataaatgattcagtacatttctaatttacagaattttttaacaaaagaaaatgtaatttgatagccaaatcaacgttaaacattatacatttaaaaaaccacaggcaaagacacaaacatgatgacactaacttttgttaaagtatgcttacctatggtttcctctgaggcacgttctttcatgctaagcttccaacataatatgaaaatgaaggagatgcattttgcaaagcaaaacagaccttaagcaaaatattatacttctcaaattaacactgttacaaagttttagaatttaataagttcattaatttaaaagtttggatgtctgagtccttctatcccaaaacaagatcttggagggtcttccacagccatgtaataccatggtcacatgaccctttccaaaattattaatctgaatttactatatgaggataaatctatctttttgaaaatatttaggaaaatgagcttggtatttataaaatgaagctctctttgggtggtatcctaagacacgtcaagccaatcagcctgtaactgtgaaaaaaacattggtaggtacaaaagtggggtgggagaggagtgacttaactttgttaagtgatgggaaagaaacactaatagcattatctcaataaaatgtgatttaaaaaaatttaaaatactaaatcattgaactgacaaagaaatataaatcattcagaaataaactcattaggtcatcaaatcctgttaaatctgcaattaggaagagcaaggtgtacaatccatacatttaaactcacaggctcactttgcacaacgtcaatttactccttaatatgttattaatacgcattttccaaaaggatgtattagtaaatggtacacatctacttcttggcaacatcatataacctggtacaacataagcattcttcttatagttaagaaatgtggatggtatcaaaattagaaaaataaatgccctattatgttgtggtcaggtttaaggcatgtgaattttatcttcatacaaaagattaaaatctagatattaaaaagtagtgcagtatcagtgatgctgcctcagttcccaaaatgtcacatcacaaaaatatcccataattgcctgtagtttattccttggctttcctcttttctctctgcatctttgtaacaattttttaaaagtggaaatataattgttggcaatgctaacagctgtagaaatgattacaagatgtggaaaagcataacaggaatgtcaagaatctgtttctggcagtaatatatatggaacattgttcaggacaaaagaggagaaggaagaaaaaaaggagaggggtttatcatctctaagaattttcaaactaaacctcattgcttaataggaaaaaaagattccatatttaaagttaagtcacctctaactactagctaaagcatgacatcaccagcactggagtcagcggaagtgtgtttttgaaggacagtgttgcaggagaatctggacaggttttagagccaggagagagaaaataattctacctctgacagttgaaggaccttaggcaaatcagtttacctctgctagactacactccaaaatttggacattcaaaaatttgatattaataaccacatgaaagtctcgtgttgaggtgaatatgtatttgttggtgaaagatatgttggtttttaaacagacagcactctgcaattgtaggctattgttttgttttgccagttgtcaaattctatccagctatacacacttgtgtggcctcctaatggtgtttttccagtggctaaaggtttatgaataagacacttttcctaatggaattaacccgatgcttttcttaaacatgtaaccttgagttcaccgcaaaaaacaatgcttcgattagagcaatgcatataataaaggttaccctcgtttcttagacactagacatcattcacaaaaagagaactgcttttgaaagggatgtatttgcactggaaagaatagttttctacttctaattataaatgatttattggtgaaagcaaaacaacagcctgtctgagaggcacttctatgagcatcctcacgtgtgatttgcaaggttgaagaagagggaaaaatgcctcaattgtaccaatggtgagaaaacacccaaagtacaaagcaggtttcaaaaaaaccatactcataaccaaggacaataataaagcaatgtgttgacatatactctataagtcttcctccataaatagtttatagaaattttgtaatttctgtaaatgcatcctataataattttgcatcttgctttttttttacatttaatatcaagtagatttctaaagggcaattatttgaaaattatcccaaatacatggggaaatatacatcaagtgaaaaaatgcagtgggtgatagagatatcaggaagcgcctcaaatatttctcatctcgttggagaaaaacaaacatgttctcatttagaatgagtgggagttacctaattgatttaggcctctatatttaacttctagtcaaaaaaggtagttctatctagcaacaatattatggggaacaaaagaaaaaattaactctctaaatttgcagtagggtcttttcttcagaagtaccaaatcccatctattaccagctccatgcttcaggcctaaaatggatctccctgaagcaatgacagaatttttgccaagtgactaggatataaacaccactttggttgcacagtgagacatatgctccaaagaaaactggttcaaaaacaggcaagtgggtttctacagaataaatgagagccctgtcaatggcttcatcttcagggctttgtgtctgtgcttgcgtggtggctcttgtttcatctatggataatggtggcacacagttttcataattccttacattaatgaactgctataaatttgtttttggtattctagagagtcctaacttcagcttctgggcaatgctgaggaggcaccctatattctagacttaccttttgcaaggtgtactctcagcattgtgggcgatttccatgggagaatattctatttaaagaactactgtcccagcataaaacaaaaaatcatttatgaagatgcaggagactcggaaagctctcaattattgtttgcacaagcacaatgtcacagcctcctttccccattccacaagggggtcaggaagagagtactcagctgtgagaaaagacatacagaagaattcatgtggtcatgagagcgaggacatggccgatcccccaaggaggatgtgtcatacacttcatgagcccaagagtgtgctgtagggtctgaagggcaagatgctggttcactgatgtaaaggagagggaaaaaagcttcaaccaactagaaaaacagtctctatgcatgctatttttgattttaaacacaggtatcaattccttctctcagagagtccattttaaaataggatacatttttaaaggaatatttaaaggacacattcattaaaatttattttaaaaacttttcaaaagaaacaaaaggtatgaattttatttaatccttgaggaaatggttcttttctcacacacataaatcactcattttgtttttctttatctcctttattaatctacattagaaaaataaacttttcatacactaagaacaaggaaaccactctcaattgacaaaatgttccaatccaacacaatgattactttcacctttaatttacaggcagccagattcaaaatccttaaagttgcttaaacttaaaaatgacaatgacaacctaaaaggtataatgttgattggaacagacatttaattggaaaattgatgattttccatttccaattaaatctctagatagaaatgaaaaaaattaaaaatcgtatttaagaaaagccaaatcttgggttgtgaggtatctttttaaggatgtttcagcagaaaaaaacaaaggctctcacaattgtgtagctgcctagattaagtgggtatcctgatcaaggagatgggggatgatttggctttagtattccaatgataaagtttataatgagaataacatgttgctacaaaatccagtctcttcctcagatgccttccacagagggcaggaagctttgtcagttttgtttgctgatgatgcctggttccgtcaacaaataacacctgtcacacggtgggtagtcaatatacatttgttgaataaatatgaaaaaaagaaatgtacaatatgtttgtgaagccaactgtgtgtgcattgctattgaggtacacaaaaagtctttgttttaaatttgagaatgaggactttcaatggaatatatctataaaaatgaaaaaaagacattactgtctggacttttgtacagcaagagaagaaaaaccactagccaagagccaactcacctgataggcctggatcaagcatgcagctgtggagaacacccctgggactctaactctggcactctgcaagctgggtacttgggcaggacagcagcagcactcatgaactgggcagcacctgttggtgagggctgatcacatggattctctcatcccagccttacaatcagtccttcaggtacatactttttctgactttgctgatgaggaaactatgcacagaggttacacagcttaacaaagggttctcacctaatgaacaatgaaatgggattttagcctttctttgcatctggtcttagagccaatacccaagaagcactgtactgtatgcattgtctcagagaaacttactcttcctgggcctcagtctttaaaaggtgggcagttgacttaataagaattaaagatcaatgattaaggttcaaggcactccaaaattctggtctttattgaaaaggctacagaagtctcaccttaataataccctatagacttgatattcttggttaattaaatattggaaaccaatttcatagtaattgaggtcagaaaaaagtactcatgacattttagaatatgatgacaaagccatagataaatttcaatgcacctgtaattacttaaaactgttatagcatgcaatgtgttaccacaacagccagagaaatactaatttactcagcctattcttctagaccagtaaacactaggattaaatagatattttcattgaatttgttctacccttcattgccatttatagatagcttacttgtcatagattactttctaattgttttatgtttcctaactagcctgcaatactttggcaaggacctcaaacaatagtagacagtaggtgtaaaatagatggctacattgaacagatgactaaaaggatgcctcctaagtacctatatcttgaaatatatattattgtgccttgctttcaatttgtgattttaaaatctagaaatcacctgttttatgtaataacaataaaatccttctttgttgaaaacatgcacaaataaagtttacaagctcaaaaaattaaacagcagtaacggtcaagctttccaacaataaaatacattttggtaaggttttcattttacaaaaactcaaaatagctttatgagttcacaaaataatatgatatttttcaagatattaacatattcttataccggaagagcatagaataaaatttacttggagattgagcatttgcttctttaagaaatacttcttttagtatttttactttaatattatgaaagctacataattacattcagattcattaactactccagtagttaatttttaaaacttatgatgaatagttttgtttaaaatatataacattggtaatatgcaaatctgaatctgtaataaagaaggatttgcattcctgatttttttttctgatacaaccaatgacaaaataactaatggttccacagaggataaaatgtctcaaatctgttggttctgaaggtgaagcgagatttttgtactgataccgtgtatcactgagataccaggaggaaatggaattaaactcagatagttcaaatggagagattttaatgaagggacgacctacagaggtgtcggcagggttggggggaatcagcgagatatgcttagaacccaccgactggcaaacctccccctgaagatggagaaggaggaaggagtgttactggaatgagagcttgagtccaggggaggaggatgggctgctgaggaggcgacaccatcctgaaagaagaatcctctgccagaggcttttcagggtcatttcttcacactctctgcagggaagcacggagacagcaggaagaaatatcctaacctcactctcttccctctacaggtgcttccattggccaaatccacccagaggccagttggtggcgatcagctctcttcaagtggtatttaaatttcttctttcattttccttctggtaacaaagaagtctgtggctcaaaagatgtttctctaagaccccatcctattaggtctctgagattttagaaatgacccaacttgatccttttattcttcagaatatctctctcaaattttcatttgtttttcattaattgatgaataatgagacattttaggtacctgtccacaaagaaatgaaattttcactttccaggaacctaacaaatgaaaagatagaaatcaattccaacagaatattaccaaagaaatcttttagaatggactgttaaaattatttatttgtatttatctggctctactatttgtggtacatttccacttcaaagctaaacctcaaataacatcatagtgagtggttgacttcatgtttaactgagatcttgaagactgaaaaagaccacgacaaacacacatctattttcttggctactgcatccgtgttcatcaccattctgatagtctgcaatgtattgcagctcaccctttgggaaggactaaagtagacatctgtttgttctgcttactcagcattcctaccctaattttcctttggagaacccctttattctagaccacgtgaagctaatgccaaaccccattccaggggatgcacctgaatccaacctccatcatctaaacagtgccttctccacgttcagagaagagcaagtgactcaaactgccctcataagaacagacctgggacttctgctgcaaatattgaagagtaagtactcttttttcttgctaggactaagctggtagtaccttctatgaggctatcatatggaaacaacttgtctgaaaatgaagccacaactagaaaacagatcctggtaacccggattgatggatccagccctaccttaaatggcaagacctaacccgaggctttttgcatcaaccaataaagtccttaagccagtttgagttggttttgtcacttgcagctaaaagaattctgactctaacaatgtgacaatagcaaaaataaacataactgcttttgaggtttctaatggattttcctccctatatacatgatttcatttaatcctcacaattcaggaaagcacatatctattaacattaaattaatattcattattttgaacacatgctatgtggataagggatgaggaaagccaaggaagtaatcaacgtgaaatctcacttatatgggagggaagtggaggttacatatctcagggcacttaacagatatcatcaaatgaaagaataaacagtgtgtgggagaggcagtaggtgattcttcatcaattcctggatgaaaaattaggagataatgaactccgaacaggcagcctaatgagaatggctcaagcaacaggacatagagagggagttaggttagacatggggttcttgggaattttcacctcgtgggggggcgggggggtcgtgcagctgttgtcagtgggaaagggaaaaaggaaaaggctgagtttggaaggcagggagggaggagacaatgtgagtcagtgaaaaagggcccttagaatgacaagtctggaccagagagaggctaagactgaaaatacaagttgggtaaccactggcatacagatggcagttcaggcttgggcactgcccaccagagcctcagcatgaagagaagagggggaggctggccaccacctccctctaggtaatcgtcatcctgatgctgagctcctgaaaacaggctctttcactcgccccatctcttgctcttgattgcaacccggcattcaggaggcaccctgtaatatctgtggagtgaccgacaacacagcgccagggcactgagaagatcccagggcgccagggactggttctacaagggtgcccctcccggtcccctccagcgcgccgccagagctgccagtcttggctgctacacgggaggcagcctcattatgcagctctcacctcttaaattagttcatgctctcacattaggtgtaatcacagcttgcaacgctttctggggatgtctcagaaagatctgagttgaaaaaatatttttgtgtcattttaatttaaagtaaaattgctgcttcttccccgcccctttctttcctcctggcccacccagcgaccctggccggccgtgctcaacgggggcgggggtcggaggtgagatttcctccacataattccttaaacagctatcaactaagtctcaaagaaaaaaaaaagagatctagaagcagagacgtggctgctggcgatcccaaagctggtgttcgctcttgggggagagcgtaccctgggggaggccgggaggccgggccagaggctagcccagaggcagagggcaggagcgctcagccggcgccccgcgtctctccagctcccgacgctgcgctggctccgctgagcacgccaggatcaaggtcgcctggtggggaccggagcgccaggagcctgtgggaagcgttccagccggcctctgactgggatccggcgccgcgtttctgctttggacttgactgacaggtccccccgccctcccgccgccctactaccagcctgggttcatccttcagggctacgtctaccgcacccgggctggaaagcctggagcgcgcccttcctctcctcatcttctcagctctcctttctccctgccacttggcaaagctgcattttgactttcacgttttggactacgtgtgtgtagttccaagtccatgcgtggcacgaaaatccacttagggtaaaaattattctcgaaaaatcgcccatctcaggatctggtgtctacactcaaggctaggaggtgcaggtacgggtgcgtaaagcatgccgtaagggtgcacagtaaataaaaagtacggatgcaaaatgtaaattttaagtgcaaaacagaaaagcagtactcgttgccgccccgcacgctgggttttaaggggcacgaaggtgggcctcggctgcttttgctcagccccgcgtcctcagcgcccggcccagtacccggtactccgtaggggttcaatgatctcccctgaataagtgaacgaattaacaaatgaatgaatgaccgctcgatccgacctccgcggccggcagagcagtcgctggagaggcgggagagagcgagaggccaagctccaccatcgcggccgccggctggggcagagggacacggagacactcggcgccccggctccgcaccgagtccccg

SEQ ID NO: 12750 - RNA, 12476 nt, Homo sapiens
  source 1..12476: mol_type = other RNA
gatctcactttgttgcccaggctggtcttaaactcctggcctcaagtgatccccttgtttcagccccgcaaagtgctgggattacaggtgtgagccaccatgcccgtgcccagccacctcatgagtcttgatggggggcagagaccaacaactccacagaagccagatgcttgctttcccagcctctcttgcagctagggcttgggcatgtgatccaggctcagccaatcagatggcactgactcttggcatgacatgggctaaggaggggctgcagggaatccatttgggctggggtggcagctgcactgggagcgacatcagtttccagagggagcagcagaatctggcatcaggcttggggcgtggtaggtgcaaccagactctgcacccagcagcagtggcagaatgggttctctgtggagagtctgtgtattgctccttccgctgaggccaccagcatctgcctccatgaacccctcagagcctgtgagcaactcaacagccttgaattttttcccttcctgtttgaatgagccagggttgtttcactgcttgaactaagagccgttcctgacatgaaaactaagccacatctttttgacccaaagattctggcatcctaaaatacccatctcattttaagttaaaaataaatccatgtttgagcatctactgtttcagttactgtgctaggtgttacaaagctaactaagagtgacaagtaaataactatcatcaccatgataaacagagaatggaaccctggtttttggaatacagacacaaaatgattaattctgcctggaagcgttttggaacatttcagagaggtagtgagctgggccaagagaagagcatacgcaaggaatggtggcatgaagttgcctggtgtgtcctgagaagaaagatgggctaagaaggactggggtagggcagagaagggggtcactggaggtgaggctgggaaagtgagccaaggctcaaatgcaaactgtctgaacttcattttctgtgcaagcaggagaagccgctgacatgggtttggaagatggactgaagccggagaaaaatggaagcaagaaaccctctcacaagaggccataaccacaaccaagtccatgagattgaaaaggaaggcagatatttgaaaaatatttaaagagatgtgaggggtaggacaggcacagtggctcatgcctgtagtcccagcactttgggaggccgaggtgggcagatccacgaggtcaggagatcaagaccatcctaacatggtaaaaccccatctctactaacaatacaaaaaattagtcaggtgtggtggcacgtgcctgtagtcccagctactcaggaggctgaggcaggagaatcgcttgaacctgggaggcggaggttgcagtgagccgagattgtgccactgcaccctagcctaggcaacagagcaagactctgtctcaaaaaaaataaaaaaaaaaaaaagagagaaagagagagagagatgaggagttgctgcactgctgggtgtggagagccgaggaggattcaaagatggtcctgaagtcccagctggaagaagtaggcggcagcaatgtttttaatactgtaaattcatcacgtagcacaggtttggggtggagaaagaaaaattgcattggcttcagggcatgcccagatctttcctcatcttaggcgtttgctaatacatgcattttctaagctgatgtcttgcgtttaatcactgctccattcaaaagagagaaggaggttgtttcaaacctagttgatatcatttgacttccatgctattcacagggctattttatttgaaacaggtataccacagccttaaattgcaagttaatccaggatgttcctaggttggcagttaggaacatgtaattctttggaagggctaaaagtcagctctttaaattatctccatatgaaccttctctccaccttagggtggatccacttatttagtccactgccagtaccacactagaacccgggtggtcactggactccagaaacaacagtagccctctctctgttctgtctctttttgactatctctattctgttcctgaccctgatttctcctgccaagctcaattttgacagctgacaacggcaagccatggcttcccaaaacattattttcaggtcaacttataaatttcaagaacacatttggctccgcttcctgtggtactaagcctacttcttgacagcatttgcctttgttgtaaatagcaaagttcttctagttggatttttgctaagaagtgtgtggatgtggcatgtgacgacatctttagcttggattctagaaaggcactaccattgtgcatttggctaaaggaaacacattttacccgtgaatgccttctatttacaaatgctcagctagcacacaaagctaagtacaagcaataagtactatcctacaatgttactcatttctgaaagcacaaaatgatgactggtatagctttggagatgttttctggaaacccaataaaggaacagatctttgttattccacacctacaaagtcagaagatgcacagtcttttattcatgtttgaacaagcttccttcttgaacaatcaactataaagtgatgtgattctctactagaccaggaactccttgaggacagaatgagggtctaatccatattctaaatccacaccacctggcacaatacatgttgcatggttagggtcaactaagagttggttgaattaatcaataacacacagcaagagaattcacaaagagaggggagtaatcccccagcctcaatcactcggcaagtggaatcgctgggcactgattccagctctgtctcagtgcttgagacagagctgaatgtaatgtgaacatttcaaatgaacaggaaaactagactcacggataagcagtgtagtcatcaagacaacactgtcttggaggtttttctgaagttaaaaccatgctacataagcaataaattatgaaggctgagcatgtgaataaaatttaatgttgtcataaattttataacaaagttaatctgacacatttaatgacatgcataatcattagtatgcagcactgtaatcagacattgataataagcagttcacaccagtgactgtaagagtctttacttgtgttcagccaagccaactgcttggtatatttttctcccttcttagtcgttagttttccatacctacaataactatcagtggtgatgggcttctctgaccatgtgaataatttaatcctcaatgcacagatacagaaacccttgctgaagacagtgtggagcagagaaggctgtctccactccttccacctgaaacacctctgcagatggatatgggagctctgcctacagcccttggacctaaccacttcagtgtgttccagtgagtgtctggacctcggcctgaaagatttttccgaaactaaagaaaatttctctgacctaaagaccttaacctccaccccagaagctctcaccaaggactacagggaactggtggggaaaatccttatcccttactcctcaaggcacagggcagtaatgctgaggcttgtgcgccacacttgctcccagaggtccccagcgggctacctgcggtggtgaatgacctcctaacacgccccttgacggccttcctttccttgcctcacttctccactctcctaccagcattgcagggttcacatcccaaatataccactggcacttgaatcctggtctccaggtctgtttctggaaaaacccaagtaagacattgccccagtaatggggctagatgtctgaggcttcctcaagtatctacctcgaaagctcttactgctgtacacacatgcacatacacacacgtgcgtacaaccagtcacatctaagcaccccgaataccagcctgttgaaggtagcagagagctgcactataagccaaggctgctcccaagagccgctccatcactgaattggcgccccagcaagatgaaggaatgtaatcattggaaggatggagaatgttctctgaatcactgacaaattggaaggggtggagggcaagagtccacctggtggagagatggaaagagcgagagagcctggaatgataatgccattgcttagaaaaggctgctccagatgccatatctacagaaattgtacagcccaaacatctctgagcaataggtctctggtagtcttgatgtctagaccaacaattcccagttcattcttctcagggaaggagccaggatagtccagagactctcattctgctgttagattgaaagggttaggcacaacagccttggcaaagtcacaagggcaaattcacactaaagtgtaaatgacccacaactcctcttctatttttaggttggggaggtgctttagaacataaggaggaactaaagaatattcctgttacatacaaggcagagaaaagggaaactagtggtgacaagacaaatcatccctttgacatttggctggctctacctattacagctctgggggtgaggtgggaacaaaaagatgctgtgtaaagaagtatcttatgccatccctactgtagtgaggtgcagtttagaggggacactgatcaagcagagacccagagtgtttcgttccaagccagaaacagaaatgtataaaacacagcctttccagcatcagaaatgagtagtggtagtggagaactacccaaaacaggaaagaggaccacgtgaggtagagtgtcaaggccctacattccagtgcctctgctcatgactgtaattttgggtaggtcacttaaagtctctggacctcagttttgccatctgtgaaatagggataatactatccagcataaaattggttatgaggctcatgtagggcctgcctgggatgatgtgttgctaatggttaagaacacaacttctggggtctgactggacaggctgaaatccctgcttaacacgttccagcagagccctgggcgatctatttaacttttgttttctcacctgtaagctgagacgaaagtacccactttataagattattccaataattagttgaaataatgcatgcagagaattaagcatggtacttgttatttgttaaactagctattaaaatgtgtaaaatataaagtattgtatggattttaggacaatgcaaagactctttgcttgctgcaatagttcggggccctttcagatggctaaaggcagaatttgtatgtgtaaatatggtgtgcttgtctctgctctggatactgagggcttaccctgttattaaacttatttagtaaatattgaactgtcatgaggcctaacatttagttccagttattagataaaacatttgctttgaatggtatttgaattgccaggttctagattattctggttgacaaactcttcgtattttataaagaggctaaaattggtaagctatcacagaacagatgtgccattttcaaggtatattaaaccatgattcactgtaacattgttcctactggcaacaaattcagagcaggctggactttatttggtgaagaaacattgagtggaagagaaatgacattattttatgtatttacattttcaaattactgtggcttaaacctgttcagccaacattacccaccttcagtctgctaaataaatgattcagtacatttctaatttacagaattttttaacaaaagaaaatgtaatttgatagccaaatcaacgttaaacattatacatttaaaaaaccacaggcaaagacacaaacatgatgacactaacttttgttaaagtatgcttacctatggtttcctctgaggcacgttctttcatgctaagcttccaacataatatgaaaatgaaggagatgcattttgcaaagcaaaacagaccttaagcaaaatattatacttctcaaattaacactgttacaaagttttagaatttaataagttcattaatttaaaagtttggatgtctgagtccttctatcccaaaacaagatcttggagggtcttccacagccatgtaataccatggtcacatgaccctttccaaaattattaatctgaatttactatatgaggataaatctatctttttgaaaatatttaggaaaatgagcttggtatttataaaatgaagctctctttgggtggtatcctaagacacgtcaagccaatcagcctgtaactgtgaaaaaaacattggtaggtacaaaagtggggtgggagaggagtgacttaactttgttaagtgatgggaaagaaacactaatagcattatctcaataaaatgtgatttaaaaaaatttaaaatactaaatcattgaactgacaaagaaatataaatcattcagaaataaactcattaggtcatcaaatcctgttaaatctgcaattaggaagagcaaggtgtacaatccatacatttaaactcacaggctcactttgcacaacgtcaatttactccttaatatgttattaatacgcattttccaaaaggatgtattagtaaatggtacacatctacttcttggcaacatcatataacctggtacaacataagcattcttcttatagttaagaaatgtggatggtatcaaaattagaaaaataaatgccctattatgttgtggtcaggtttaaggcatgtgaattttatcttcatacaaaagattaaaatctagatattaaaaagtagtgcagtatcagtgatgctgcctcagttcccaaaatgtcacatcacaaaaatatcccataattgcctgtagtttattccttggctttcctcttttctctctgcatctttgtaacaattttttaaaagtggaaatataattgttggcaatgctaacagctgtagaaatgattacaagatgtggaaaagcataacaggaatgtcaagaatctgtttctggcagtaatatatatggaacattgttcaggacaaaagaggagaaggaagaaaaaaaggagaggggtttatcatctctaagaattttcaaactaaacctcattgcttaataggaaaaaaagattccatatttaaagttaagtcacctctaactactagctaaagcatgacatcaccagcactggagtcagcggaagtgtgtttttgaaggacagtgttgcaggagaatctggacaggttttagagccaggagagagaaaataattctacctctgacagttgaaggaccttaggcaaatcagtttacctctgctagactacactccaaaatttggacattcaaaaatttgatattaataaccacatgaaagtctcgtgttgaggtgaatatgtatttgttggtgaaagatatgttggtttttaaacagacagcactctgcaattgtaggctattgttttgttttgccagttgtcaaattctatccagctatacacacttgtgtggcctcctaatggtgtttttccagtggctaaaggtttatgaataagacacttttcctaatggaattaacccgatgcttttcttaaacatgtaaccttgagttcaccgcaaaaaacaatgcttcgattagagcaatgcatataataaaggttaccctcgtttcttagacactagacatcattcacaaaaagagaactgcttttgaaagggatgtatttgcactggaaagaatagttttctacttctaattataaatgatttattggtgaaagcaaaacaacagcctgtctgagaggcacttctatgagcatcctcacgtgtgatttgcaaggttgaagaagagggaaaaatgcctcaattgtaccaatggtgagaaaacacccaaagtacaaagcaggtttcaaaaaaaccatactcataaccaaggacaataataaagcaatgtgttgacatatactctataagtcttcctccataaatagtttatagaaattttgtaatttctgtaaatgcatcctataataattttgcatcttgctttttttttacatttaatatcaagtagatttctaaagggcaattatttgaaaattatcccaaatacatggggaaatatacatcaagtgaaaaaatgcagtgggtgatagagatatcaggaagcgcctcaaatatttctcatctcgttggagaaaaacaaacatgttctcatttagaatgagtgggagttacctaattgatttaggcctctatatttaacttctagtcaaaaaaggtagttctatctagcaacaatattatggggaacaaaagaaaaaattaactctctaaatttgcagtagggtcttttcttcagaagtaccaaatcccatctattaccagctccatgcttcaggcctaaaatggatctccctgaagcaatgacagaatttttgccaagtgactaggatataaacaccactttggttgcacagtgagacatatgctccaaagaaaactggttcaaaaacaggcaagtgggtttctacagaataaatgagagccctgtcaatggcttcatcttcagggctttgtgtctgtgcttgcgtggtggctcttgtttcatctatggataatggtggcacacagttttcataattccttacattaatgaactgctataaatttgtttttggtattctagagagtcctaacttcagcttctgggcaatgctgaggaggcaccctatattctagacttaccttttgcaaggtgtactctcagcattgtgggcgatttccatgggagaatattctatttaaagaactactgtcccagcataaaacaaaaaatcatttatgaagatgcaggagactcggaaagctctcaattattgtttgcacaagcacaatgtcacagcctcctttccccattccacaagggggtcaggaagagagtactcagctgtgagaaaagacatacagaagaattcatgtggtcatgagagcgaggacatggccgatcccccaaggaggatgtgtcatacacttcatgagcccaagagtgtgctgtagggtctgaagggcaagatgctggttcactgatgtaaaggagagggaaaaaagcttcaaccaactagaaaaacagtctctatgcatgctatttttgattttaaacacaggtatcaattccttctctcagagagtccattttaaaataggatacatttttaaaggaatatttaaaggacacattcattaaaatttattttaaaaacttttcaaaagaaacaaaaggtatgaattttatttaatccttgaggaaatggttcttttctcacacacataaatcactcattttgtttttctttatctcctttattaatctacattagaaaaataaacttttcatacactaagaacaaggaaaccactctcaattgacaaaatgttccaatccaacacaatgattactttcacctttaatttacaggcagccagattcaaaatccttaaagttgcttaaacttaaaaatgacaatgacaacctaaaaggtataatgttgattggaacagacatttaattggaaaattgatgattttccatttccaattaaatctctagatagaaatgaaaaaaattaaaaatcgtatttaagaaaagccaaatcttgggttgtgaggtatctttttaaggatgtttcagcagaaaaaaacaaaggctctcacaattgtgtagctgcctagattaagtgggtatcctgatcaaggagatgggggatgatttggctttagtattccaatgataaagtttataatgagaataacatgttgctacaaaatccagtctcttcctcagatgccttccacagagggcaggaagctttgtcagttttgtttgctgatgatgcctggttccgtcaacaaataacacctgtcacacggtgggtagtcaatatacatttgttgaataaatatgaaaaaaagaaatgtacaatatgtttgtgaagccaactgtgtgtgcattgctattgaggtacacaaaaagtctttgttttaaatttgagaatgaggactttcaatggaatatatctataaaaatgaaaaaaagacattactgtctggacttttgtacagcaagagaagaaaaaccactagccaagagccaactcacctgataggcctggatcaagcatgcagctgtggagaacacccctgggactctaactctggcactctgcaagctgggtacttgggcaggacagcagcagcactcatgaactgggcagcacctgttggtgagggctgatcacatggattctctcatcccagccttacaatcagtccttcaggtacatactttttctgactttgctgatgaggaaactatgcacagaggttacacagcttaacaaagggttctcacctaatgaacaatgaaatgggattttagcctttctttgcatctggtcttagagccaatacccaagaagcactgtactgtatgcattgtctcagagaaacttactcttcctgggcctcagtctttaaaaggtgggcagttgacttaataagaattaaagatcaatgattaaggttcaaggcactccaaaattctggtctttattgaaaaggctacagaagtctcaccttaataataccctatagacttgatattcttggttaattaaatattggaaaccaatttcatagtaattgaggtcagaaaaaagtactcatgacattttagaatatgatgacaaagccatagataaatttcaatgcacctgtaattacttaaaactgttatagcatgcaatgtgttaccacaacagccagagaaatactaatttactcagcctattcttctagaccagtaaacactaggattaaatagatattttcattgaatttgttctacccttcattgccatttatagatagcttacttgtcatagattactttctaattgttttatgtttcctaactagcctgcaatactttggcaaggacctcaaacaatagtagacagtaggtgtaaaatagatggctacattgaacagatgactaaaaggatgcctcctaagtacctatatcttgaaatatatattattgtgccttgctttcaatttgtgattttaaaatctagaaatcacctgttttatgtaataacaataaaatccttctttgttgaaaacatgcacaaataaagtttacaagctcaaaaaattaaacagcagtaacggtcaagctttccaacaataaaatacattttggtaaggttttcattttacaaaaactcaaaatagctttatgagttcacaaaataatatgatatttttcaagatattaacatattcttataccggaagagcatagaataaaatttacttggagattgagcatttgcttctttaagaaatacttcttttagtatttttactttaatattatgaaagctacataattacattcagattcattaactactccagtagttaatttttaaaacttatgatgaatagttttgtttaaaatatataacattggtaatatgcaaatctgaatctgtaataaagaaggatttgcattcctgatttttttttctgatacaaccaatgacaaaataactaatggttccacagaggataaaatgtctcaaatctgttggttctgaaggtgaagcgagatttttgtactgataccgtgtatcactgagataccaggaggaaatggaattaaactcagatagttcaaatggagagattttaatgaagggacgacctacagaggtgtcggcagggttggggggaatcagcgagatatgcttagaacccaccgactggcaaacctccccctgaagatggagaaggaggaaggagtgttactggaatgagagcttgagtccaggggaggaggatgggctgctgaggaggcgacaccatcctgaaagaagaatcctctgccagaggcttttcagggtcatttcttcacactctctgcagggaagcacggagacagcaggaagaaatatcctaacctcactctcttccctctacaggtgcttccattggccaaatccacccagaggccagttggtggcgatcagctctcttcaagtggtatttaaatttcttctttcattttccttctggtaacaaagaagtctgtggctcaaaagatgtttctctaagaccccatcctattaggtctctgagattttagaaatgacccaacttgatccttttattcttcagaatatctctctcaaattttcatttgtttttcattaattgatgaataatgagacattttaggtacctgtccacaaagaaatgaaattttcactttccaggaacctgagggccgacgagtgggggcgggcaggagggccgagggaggcggaacaggatcgaggcgcgaggcgggagtcgagaaagcgagcggccgaggcgactctcagtgcgcggacgcgggcgcgcgcccgcgctcccttcgtcgactcacggcgagagcccaaccctgctgccgcgcgccacccgcctcgccgcgcct

SEQ ID NO: 12751 - RNA, 12335 nt, Homo sapiens
  source 1..12335: mol_type = other RNA
gatctcactttgttgcccaggctggtcttaaactcctggcctcaagtgatccccttgtttcagccccgcaaagtgctgggattacaggtgtgagccaccatgcccgtgcccagccacctcatgagtcttgatggggggcagagaccaacaactccacagaagccagatgcttgctttcccagcctctcttgcagctagggcttgggcatgtgatccaggctcagccaatcagatggcactgactcttggcatgacatgggctaaggaggggctgcagggaatccatttgggctggggtggcagctgcactgggagcgacatcagtttccagagggagcagcagaatctggcatcaggcttggggcgtggtaggtgcaaccagactctgcacccagcagcagtggcagaatgggttctctgtggagagtctgtgtattgctccttccgctgaggccaccagcatctgcctccatgaacccctcagagcctgtgagcaactcaacagccttgaattttttcccttcctgtttgaatgagccagggttgtttcactgcttgaactaagagccgttcctgacatgaaaactaagccacatctttttgacccaaagattctggcatcctaaaatacccatctcattttaagttaaaaataaatccatgtttgagcatctactgtttcagttactgtgctaggtgttacaaagctaactaagagtgacaagtaaataactatcatcaccatgataaacagagaatggaaccctggtttttggaatacagacacaaaatgattaattctgcctggaagcgttttggaacatttcagagaggtagtgagctgggccaagagaagagcatacgcaaggaatggtggcatgaagttgcctggtgtgtcctgagaagaaagatgggctaagaaggactggggtagggcagagaagggggtcactggaggtgaggctgggaaagtgagccaaggctcaaatgcaaactgtctgaacttcattttctgtgcaagcaggagaagccgctgacatgggtttggaagatggactgaagccggagaaaaatggaagcaagaaaccctctcacaagaggccataaccacaaccaagtccatgagattgaaaaggaaggcagatatttgaaaaatatttaaagagatgtgaggggtaggacaggcacagtggctcatgcctgtagtcccagcactttgggaggccgaggtgggcagatccacgaggtcaggagatcaagaccatcctaacatggtaaaaccccatctctactaacaatacaaaaaattagtcaggtgtggtggcacgtgcctgtagtcccagctactcaggaggctgaggcaggagaatcgcttgaacctgggaggcggaggttgcagtgagccgagattgtgccactgcaccctagcctaggcaacagagcaagactctgtctcaaaaaaaataaaaaaaaaaaaaagagagaaagagagagagagatgaggagttgctgcactgctgggtgtggagagccgaggaggattcaaagatggtcctgaagtcccagctggaagaagtaggcggcagcaatgtttttaatactgtaaattcatcacgtagcacaggtttggggtggagaaagaaaaattgcattggcttcagggcatgcccagatctttcctcatcttaggcgtttgctaatacatgcattttctaagctgatgtcttgcgtttaatcactgctccattcaaaagagagaaggaggttgtttcaaacctagttgatatcatttgacttccatgctattcacagggctattttatttgaaacaggtataccacagccttaaattgcaagttaatccaggatgttcctaggttggcagttaggaacatgtaattctttggaagggctaaaagtcagctctttaaattatctccatatgaaccttctctccaccttagggtggatccacttatttagtccactgccagtaccacactagaacccgggtggtcactggactccagaaacaacagtagccctctctctgttctgtctctttttgactatctctattctgttcctgaccctgatttctcctgccaagctcaattttgacagctgacaacggcaagccatggcttcccaaaacattattttcaggtcaacttataaatttcaagaacacatttggctccgcttcctgtggtactaagcctacttcttgacagcatttgcctttgttgtaaatagcaaagttcttctagttggatttttgctaagaagtgtgtggatgtggcatgtgacgacatctttagcttggattctagaaaggcactaccattgtgcatttggctaaaggaaacacattttacccgtgaatgccttctatttacaaatgctcagctagcacacaaagctaagtacaagcaataagtactatcctacaatgttactcatttctgaaagcacaaaatgatgactggtatagctttggagatgttttctggaaacccaataaaggaacagatctttgttattccacacctacaaagtcagaagatgcacagtcttttattcatgtttgaacaagcttccttcttgaacaatcaactataaagtgatgtgattctctactagaccaggaactccttgaggacagaatgagggtctaatccatattctaaatccacaccacctggcacaatacatgttgcatggttagggtcaactaagagttggttgaattaatcaataacacacagcaagagaattcacaaagagaggggagtaatcccccagcctcaatcactcggcaagtggaatcgctgggcactgattccagctctgtctcagtgcttgagacagagctgaatgtaatgtgaacatttcaaatgaacaggaaaactagactcacggataagcagtgtagtcatcaagacaacactgtcttggaggtttttctgaagttaaaaccatgctacataagcaataaattatgaaggctgagcatgtgaataaaatttaatgttgtcataaattttataacaaagttaatctgacacatttaatgacatgcataatcattagtatgcagcactgtaatcagacattgataataagcagttcacaccagtgactgtaagagtctttacttgtgttcagccaagccaactgcttggtatatttttctcccttcttagtcgttagttttccatacctacaataactatcagtggtgatgggcttctctgaccatgtgaataatttaatcctcaatgcacagatacagaaacccttgctgaagacagtgtggagcagagaaggctgtctccactccttccacctgaaacacctctgcagatggatatgggagctctgcctacagcccttggacctaaccacttcagtgtgttccagtgagtgtctggacctcggcctgaaagatttttccgaaactaaagaaaatttctctgacctaaagaccttaacctccaccccagaagctctcaccaaggactacagggaactggtggggaaaatccttatcccttactcctcaaggcacagggcagtaatgctgaggcttgtgcgccacacttgctcccagaggtccccagcgggctacctgcggtggtgaatgacctcctaacacgccccttgacggccttcctttccttgcctcacttctccactctcctaccagcattgcagggttcacatcccaaatataccactggcacttgaatcctggtctccaggtctgtttctggaaaaacccaagtaagacattgccccagtaatggggctagatgtctgaggcttcctcaagtatctacctcgaaagctcttactgctgtacacacatgcacatacacacacgtgcgtacaaccagtcacatctaagcaccccgaataccagcctgttgaaggtagcagagagctgcactataagccaaggctgctcccaagagccgctccatcactgaattggcgccccagcaagatgaaggaatgtaatcattggaaggatggagaatgttctctgaatcactgacaaattggaaggggtggagggcaagagtccacctggtggagagatggaaagagcgagagagcctggaatgataatgccattgcttagaaaaggctgctccagatgccatatctacagaaattgtacagcccaaacatctctgagcaataggtctctggtagtcttgatgtctagaccaacaattcccagttcattcttctcagggaaggagccaggatagtccagagactctcattctgctgttagattgaaagggttaggcacaacagccttggcaaagtcacaagggcaaattcacactaaagtgtaaatgacccacaactcctcttctatttttaggttggggaggtgctttagaacataaggaggaactaaagaatattcctgttacatacaaggcagagaaaagggaaactagtggtgacaagacaaatcatccctttgacatttggctggctctacctattacagctctgggggtgaggtgggaacaaaaagatgctgtgtaaagaagtatcttatgccatccctactgtagtgaggtgcagtttagaggggacactgatcaagcagagacccagagtgtttcgttccaagccagaaacagaaatgtataaaacacagcctttccagcatcagaaatgagtagtggtagtggagaactacccaaaacaggaaagaggaccacgtgaggtagagtgtcaaggccctacattccagtgcctctgctcatgactgtaattttgggtaggtcacttaaagtctctggacctcagttttgccatctgtgaaatagggataatactatccagcataaaattggttatgaggctcatgtagggcctgcctgggatgatgtgttgctaatggttaagaacacaacttctggggtctgactggacaggctgaaatccctgcttaacacgttccagcagagccctgggcgatctatttaacttttgttttctcacctgtaagctgagacgaaagtacccactttataagattattccaataattagttgaaataatgcatgcagagaattaagcatggtacttgttatttgttaaactagctattaaaatgtgtaaaatataaagtattgtatggattttaggacaatgcaaagactctttgcttgctgcaatagttcggggccctttcagatggctaaaggcagaatttgtatgtgtaaatatggtgtgcttgtctctgctctggatactgagggcttaccctgttattaaacttatttagtaaatattgaactgtcatgaggcctaacatttagttccagttattagataaaacatttgctttgaatggtatttgaattgccaggttctagattattctggttgacaaactcttcgtattttataaagaggctaaaattggtaagctatcacagaacagatgtgccattttcaaggtatattaaaccatgattcactgtaacattgttcctactggcaacaaattcagagcaggctggactttatttggtgaagaaacattgagtggaagagaaatgacattattttatgtatttacattttcaaattactgtggcttaaacctgttcagccaacattacccaccttcagtctgctaaataaatgattcagtacatttctaatttacagaattttttaacaaaagaaaatgtaatttgatagccaaatcaacgttaaacattatacatttaaaaaaccacaggcaaagacacaaacatgatgacactaacttttgttaaagtatgcttacctatggtttcctctgaggcacgttctttcatgctaagcttccaacataatatgaaaatgaaggagatgcattttgcaaagcaaaacagaccttaagcaaaatattatacttctcaaattaacactgttacaaagttttagaatttaataagttcattaatttaaaagtttggatgtctgagtccttctatcccaaaacaagatcttggagggtcttccacagccatgtaataccatggtcacatgaccctttccaaaattattaatctgaatttactatatgaggataaatctatctttttgaaaatatttaggaaaatgagcttggtatttataaaatgaagctctctttgggtggtatcctaagacacgtcaagccaatcagcctgtaactgtgaaaaaaacattggtaggtacaaaagtggggtgggagaggagtgacttaactttgttaagtgatgggaaagaaacactaatagcattatctcaataaaatgtgatttaaaaaaatttaaaatactaaatcattgaactgacaaagaaatataaatcattcagaaataaactcattaggtcatcaaatcctgttaaatctgcaattaggaagagcaaggtgtacaatccatacatttaaactcacaggctcactttgcacaacgtcaatttactccttaatatgttattaatacgcattttccaaaaggatgtattagtaaatggtacacatctacttcttggcaacatcatataacctggtacaacataagcattcttcttatagttaagaaatgtggatggtatcaaaattagaaaaataaatgccctattatgttgtggtcaggtttaaggcatgtgaattttatcttcatacaaaagattaaaatctagatattaaaaagtagtgcagtatcagtgatgctgcctcagttcccaaaatgtcacatcacaaaaatatcccataattgcctgtagtttattccttggctttcctcttttctctctgcatctttgtaacaattttttaaaagtggaaatataattgttggcaatgctaacagctgtagaaatgattacaagatgtggaaaagcataacaggaatgtcaagaatctgtttctggcagtaatatatatggaacattgttcaggacaaaagaggagaaggaagaaaaaaaggagaggggtttatcatctctaagaattttcaaactaaacctcattgcttaataggaaaaaaagattccatatttaaagttaagtcacctctaactactagctaaagcatgacatcaccagcactggagtcagcggaagtgtgtttttgaaggacagtgttgcaggagaatctggacaggttttagagccaggagagagaaaataattctacctctgacagttgaaggaccttaggcaaatcagtttacctctgctagactacactccaaaatttggacattcaaaaatttgatattaataaccacatgaaagtctcgtgttgaggtgaatatgtatttgttggtgaaagatatgttggtttttaaacagacagcactctgcaattgtaggctattgttttgttttgccagttgtcaaattctatccagctatacacacttgtgtggcctcctaatggtgtttttccagtggctaaaggtttatgaataagacacttttcctaatggaattaacccgatgcttttcttaaacatgtaaccttgagttcaccgcaaaaaacaatgcttcgattagagcaatgcatataataaaggttaccctcgtttcttagacactagacatcattcacaaaaagagaactgcttttgaaagggatgtatttgcactggaaagaatagttttctacttctaattataaatgatttattggtgaaagcaaaacaacagcctgtctgagaggcacttctatgagcatcctcacgtgtgatttgcaaggttgaagaagagggaaaaatgcctcaattgtaccaatggtgagaaaacacccaaagtacaaagcaggtttcaaaaaaaccatactcataaccaaggacaataataaagcaatgtgttgacatatactctataagtcttcctccataaatagtttatagaaattttgtaatttctgtaaatgcatcctataataattttgcatcttgctttttttttacatttaatatcaagtagatttctaaagggcaattatttgaaaattatcccaaatacatggggaaatatacatcaagtgaaaaaatgcagtgggtgatagagatatcaggaagcgcctcaaatatttctcatctcgttggagaaaaacaaacatgttctcatttagaatgagtgggagttacctaattgatttaggcctctatatttaacttctagtcaaaaaaggtagttctatctagcaacaatattatggggaacaaaagaaaaaattaactctctaaatttgcagtagggtcttttcttcagaagtaccaaatcccatctattaccagctccatgcttcaggcctaaaatggatctccctgaagcaatgacagaatttttgccaagtgactaggatataaacaccactttggttgcacagtgagacatatgctccaaagaaaactggttcaaaaacaggcaagtgggtttctacagaataaatgagagccctgtcaatggcttcatcttcagggctttgtgtctgtgcttgcgtggtggctcttgtttcatctatggataatggtggcacacagttttcataattccttacattaatgaactgctataaatttgtttttggtattctagagagtcctaacttcagcttctgggcaatgctgaggaggcaccctatattctagacttaccttttgcaaggtgtactctcagcattgtgggcgatttccatgggagaatattctatttaaagaactactgtcccagcataaaacaaaaaatcatttatgaagatgcaggagactcggaaagctctcaattattgtttgcacaagcacaatgtcacagcctcctttccccattccacaagggggtcaggaagagagtactcagctgtgagaaaagacatacagaagaattcatgtggtcatgagagcgaggacatggccgatcccccaaggaggatgtgtcatacacttcatgagcccaagagtgtgctgtagggtctgaagggcaagatgctggttcactgatgtaaaggagagggaaaaaagcttcaaccaactagaaaaacagtctctatgcatgctatttttgattttaaacacaggtatcaattccttctctcagagagtccattttaaaataggatacatttttaaaggaatatttaaaggacacattcattaaaatttattttaaaaacttttcaaaagaaacaaaaggtatgaattttatttaatccttgaggaaatggttcttttctcacacacataaatcactcattttgtttttctttatctcctttattaatctacattagaaaaataaacttttcatacactaagaacaaggaaaccactctcaattgacaaaatgttccaatccaacacaatgattactttcacctttaatttacaggcagccagattcaaaatccttaaagttgcttaaacttaaaaatgacaatgacaacctaaaaggtataatgttgattggaacagacatttaattggaaaattgatgattttccatttccaattaaatctctagatagaaatgaaaaaaattaaaaatcgtatttaagaaaagccaaatcttgggttgtgaggtatctttttaaggatgtttcagcagaaaaaaacaaaggctctcacaattgtgtagctgcctagattaagtgggtatcctgatcaaggagatgggggatgatttggctttagtattccaatgataaagtttataatgagaataacatgttgctacaaaatccagtctcttcctcagatgccttccacagagggcaggaagctttgtcagttttgtttgctgatgatgcctggttccgtcaacaaataacacctgtcacacggtgggtagtcaatatacatttgttgaataaatatgaaaaaaagaaatgtacaatatgtttgtgaagccaactgtgtgtgcattgctattgaggtacacaaaaagtctttgttttaaatttgagaatgaggactttcaatggaatatatctataaaaatgaaaaaaagacattactgtctggacttttgtacagcaagagaagaaaaaccactagccaagagccaactcacctgataggcctggatcaagcatgcagctgtggagaacacccctgggactctaactctggcactctgcaagctgggtacttgggcaggacagcagcagcactcatgaactgggcagcacctgttggtgagggctgatcacatggattctctcatcccagccttacaatcagtccttcaggtacatactttttctgactttgctgatgaggaaactatgcacagaggttacacagcttaacaaagggttctcacctaatgaacaatgaaatgggattttagcctttctttgcatctggtcttagagccaatacccaagaagcactgtactgtatgcattgtctcagagaaacttactcttcctgggcctcagtctttaaaaggtgggcagttgacttaataagaattaaagatcaatgattaaggttcaaggcactccaaaattctggtctttattgaaaaggctacagaagtctcaccttaataataccctatagacttgatattcttggttaattaaatattggaaaccaatttcatagtaattgaggtcagaaaaaagtactcatgacattttagaatatgatgacaaagccatagataaatttcaatgcacctgtaattacttaaaactgttatagcatgcaatgtgttaccacaacagccagagaaatactaatttactcagcctattcttctagaccagtaaacactaggattaaatagatattttcattgaatttgttctacccttcattgccatttatagatagcttacttgtcatagattactttctaattgttttatgtttcctaactagcctgcaatactttggcaaggacctcaaacaatagtagacagtaggtgtaaaatagatggctacattgaacagatgactaaaaggatgcctcctaagtacctatatcttgaaatatatattattgtgccttgctttcaatttgtgattttaaaatctagaaatcacctgttttatgtaataacaataaaatccttctttgttgaaaacatgcacaaataaagtttacaagctcaaaaaattaaacagcagtaacggtcaagctttccaacaataaaatacattttggtaaggttttcattttacaaaaactcaaaatagctttatgagttcacaaaataatatgatatttttcaagatattaacatattcttataccggaagagcatagaataaaatttacttggagattgagcatttgcttctttaagaaatacttcttttagtatttttactttaatattatgaaagctacataattacattcagattcattaactactccagtagttaatttttaaaacttatgatgaatagttttgtttaaaatatataacattggtaatatgcaaatctgaatctgtaataaagaaggatttgcattcctgatttttttttctgatacaaccaatgacaaaataactaatggttccacagaggataaaatgtctcaaatctgttggttctgaaggtgaagcgagatttttgtactgataccgtgtatcactgagataccaggaggaaatggaattaaactcagatagttcaaatggagagattttaatgaagggacgacctacagaggtgtcggcagggttggggggaatcagcgagatatgcttagaacccaccgactggcaaacctccccctgaagatggagaaggaggaaggagtgttactggaatgagagcttgagtccaggggaggaggatgggctgctgaggaggcgacaccatcctgaaagaagaatcctctgccagaggcttttcagggtcatttcttcacactctctgcagggaagcacggagacagcaggaagaaatatcctaacctcactctcttccctctacaggtgcttccattggccaaatccacccagaggccagttggtggcgatcagctctcttcaagtggtatttaaatttcttctttcattttccttctggtaacaaagaagtctgtggctcaaaagatgtttctctaagaccccatcctattaggtctctgagctgagggccgacgagtgggggcgggcaggagggccgagggaggcggaacaggatcgaggcgcgaggcgggagtcgagaaagcgagcggccgaggcgactctcagtgcgcggacgcgggcgcgcgcccgcgctcccttcgtcgactcacggcgagagcccaaccctgctgccgcgcgccacccgcctcgccgcgcct

SEQ ID NO: 12752 - RNA, 15170 nt, Homo sapiens
  source 1..15170: mol_type = other RNA
gatctcactttgttgcccaggctggtcttaaactcctggcctcaagtgatccccttgtttcagccccgcaaagtgctgggattacaggtgtgagccaccatgcccgtgcccagccacctcatgagtcttgatggggggcagagaccaacaactccacagaagccagatgcttgctttcccagcctctcttgcagctagggcttgggcatgtgatccaggctcagccaatcagatggcactgactcttggcatgacatgggctaaggaggggctgcagggaatccatttgggctggggtggcagctgcactgggagcgacatcagtttccagagggagcagcagaatctggcatcaggcttggggcgtggtaggtgcaaccagactctgcacccagcagcagtggcagaatgggttctctgtggagagtctgtgtattgctccttccgctgaggccaccagcatctgcctccatgaacccctcagagcctgtgagcaactcaacagccttgaattttttcccttcctgtttgaatgagccagggttgtttcactgcttgaactaagagccgttcctgacatgaaaactaagccacatctttttgacccaaagattctggcatcctaaaatacccatctcattttaagttaaaaataaatccatgtttgagcatctactgtttcagttactgtgctaggtgttacaaagctaactaagagtgacaagtaaataactatcatcaccatgataaacagagaatggaaccctggtttttggaatacagacacaaaatgattaattctgcctggaagcgttttggaacatttcagagaggtagtgagctgggccaagagaagagcatacgcaaggaatggtggcatgaagttgcctggtgtgtcctgagaagaaagatgggctaagaaggactggggtagggcagagaagggggtcactggaggtgaggctgggaaagtgagccaaggctcaaatgcaaactgtctgaacttcattttctgtgcaagcaggagaagccgctgacatgggtttggaagatggactgaagccggagaaaaatggaagcaagaaaccctctcacaagaggccataaccacaaccaagtccatgagattgaaaaggaaggcagatatttgaaaaatatttaaagagatgtgaggggtaggacaggcacagtggctcatgcctgtagtcccagcactttgggaggccgaggtgggcagatccacgaggtcaggagatcaagaccatcctaacatggtaaaaccccatctctactaacaatacaaaaaattagtcaggtgtggtggcacgtgcctgtagtcccagctactcaggaggctgaggcaggagaatcgcttgaacctgggaggcggaggttgcagtgagccgagattgtgccactgcaccctagcctaggcaacagagcaagactctgtctcaaaaaaaataaaaaaaaaaaaaagagagaaagagagagagagatgaggagttgctgcactgctgggtgtggagagccgaggaggattcaaagatggtcctgaagtcccagctggaagaagtaggcggcagcaatgtttttaatactgtaaattcatcacgtagcacaggtttggggtggagaaagaaaaattgcattggcttcagggcatgcccagatctttcctcatcttaggcgtttgctaatacatgcattttctaagctgatgtcttgcgtttaatcactgctccattcaaaagagagaaggaggttgtttcaaacctagttgatatcatttgacttccatgctattcacagggctattttatttgaaacaggtataccacagccttaaattgcaagttaatccaggatgttcctaggttggcagttaggaacatgtaattctttggaagggctaaaagtcagctctttaaattatctccatatgaaccttctctccaccttagggtggatccacttatttagtccactgccagtaccacactagaacccgggtggtcactggactccagaaacaacagtagccctctctctgttctgtctctttttgactatctctattctgttcctgaccctgatttctcctgccaagctcaattttgacagctgacaacggcaagccatggcttcccaaaacattattttcaggtcaacttataaatttcaagaacacatttggctccgcttcctgtggtactaagcctacttcttgacagcatttgcctttgttgtaaatagcaaagttcttctagttggatttttgctaagaagtgtgtggatgtggcatgtgacgacatctttagcttggattctagaaaggcactaccattgtgcatttggctaaaggaaacacattttacccgtgaatgccttctatttacaaatgctcagctagcacacaaagctaagtacaagcaataagtactatcctacaatgttactcatttctgaaagcacaaaatgatgactggtatagctttggagatgttttctggaaacccaataaaggaacagatctttgttattccacacctacaaagtcagaagatgcacagtcttttattcatgtttgaacaagcttccttcttgaacaatcaactataaagtgatgtgattctctactagaccaggaactccttgaggacagaatgagggtctaatccatattctaaatccacaccacctggcacaatacatgttgcatggttagggtcaactaagagttggttgaattaatcaataacacacagcaagagaattcacaaagagaggggagtaatcccccagcctcaatcactcggcaagtggaatcgctgggcactgattccagctctgtctcagtgcttgagacagagctgaatgtaatgtgaacatttcaaatgaacaggaaaactagactcacggataagcagtgtagtcatcaagacaacactgtcttggaggtttttctgaagttaaaaccatgctacataagcaataaattatgaaggctgagcatgtgaataaaatttaatgttgtcataaattttataacaaagttaatctgacacatttaatgacatgcataatcattagtatgcagcactgtaatcagacattgataataagcagttcacaccagtgactgtaagagtctttacttgtgttcagccaagccaactgcttggtatatttttctcccttcttagtcgttagttttccatacctacaataactatcagtggtgatgggcttctctgaccatgtgaataatttaatcctcaatgcacagatacagaaacccttgctgaagacagtgtggagcagagaaggctgtctccactccttccacctgaaacacctctgcagatggatatgggagctctgcctacagcccttggacctaaccacttcagtgtgttccagtgagtgtctggacctcggcctgaaagatttttccgaaactaaagaaaatttctctgacctaaagaccttaacctccaccccagaagctctcaccaaggactacagggaactggtggggaaaatccttatcccttactcctcaaggcacagggcagtaatgctgaggcttgtgcgccacacttgctcccagaggtccccagcgggctacctgcggtggtgaatgacctcctaacacgccccttgacggccttcctttccttgcctcacttctccactctcctaccagcattgcagggttcacatcccaaatataccactggcacttgaatcctggtctccaggtctgtttctggaaaaacccaagtaagacattgccccagtaatggggctagatgtctgaggcttcctcaagtatctacctcgaaagctcttactgctgtacacacatgcacatacacacacgtgcgtacaaccagtcacatctaagcaccccgaataccagcctgttgaaggtagcagagagctgcactataagccaaggctgctcccaagagccgctccatcactgaattggcgccccagcaagatgaaggaatgtaatcattggaaggatggagaatgttctctgaatcactgacaaattggaaggggtggagggcaagagtccacctggtggagagatggaaagagcgagagagcctggaatgataatgccattgcttagaaaaggctgctccagatgccatatctacagaaattgtacagcccaaacatctctgagcaataggtctctggtagtcttgatgtctagaccaacaattcccagttcattcttctcagggaaggagccaggatagtccagagactctcattctgctgttagattgaaagggttaggcacaacagccttggcaaagtcacaagggcaaattcacactaaagtgtaaatgacccacaactcctcttctatttttaggttggggaggtgctttagaacataaggaggaactaaagaatattcctgttacatacaaggcagagaaaagggaaactagtggtgacaagacaaatcatccctttgacatttggctggctctacctattacagctctgggggtgaggtgggaacaaaaagatgctgtgtaaagaagtatcttatgccatccctactgtagtgaggtgcagtttagaggggacactgatcaagcagagacccagagtgtttcgttccaagccagaaacagaaatgtataaaacacagcctttccagcatcagaaatgagtagtggtagtggagaactacccaaaacaggaaagaggaccacgtgaggtagagtgtcaaggccctacattccagtgcctctgctcatgactgtaattttgggtaggtcacttaaagtctctggacctcagttttgccatctgtgaaatagggataatactatccagcataaaattggttatgaggctcatgtagggcctgcctgggatgatgtgttgctaatggttaagaacacaacttctggggtctgactggacaggctgaaatccctgcttaacacgttccagcagagccctgggcgatctatttaacttttgttttctcacctgtaagctgagacgaaagtacccactttataagattattccaataattagttgaaataatgcatgcagagaattaagcatggtacttgttatttgttaaactagctattaaaatgtgtaaaatataaagtattgtatggattttaggacaatgcaaagactctttgcttgctgcaatagttcggggccctttcagatggctaaaggcagaatttgtatgtgtaaatatggtgtgcttgtctctgctctggatactgagggcttaccctgttattaaacttatttagtaaatattgaactgtcatgaggcctaacatttagttccagttattagataaaacatttgctttgaatggtatttgaattgccaggttctagattattctggttgacaaactcttcgtattttataaagaggctaaaattggtaagctatcacagaacagatgtgccattttcaaggtatattaaaccatgattcactgtaacattgttcctactggcaacaaattcagagcaggctggactttatttggtgaagaaacattgagtggaagagaaatgacattattttatgtatttacattttcaaattactgtggcttaaacctgttcagccaacattacccaccttcagtctgctaaataaatgattcagtacatttctaatttacagaattttttaacaaaagaaaatgtaatttgatagccaaatcaacgttaaacattatacatttaaaaaaccacaggcaaagacacaaacatgatgacactaacttttgttaaagtatgcttacctatggtttcctctgaggcacgttctttcatgctaagcttccaacataatatgaaaatgaaggagatgcattttgcaaagcaaaacagaccttaagcaaaatattatacttctcaaattaacactgttacaaagttttagaatttaataagttcattaatttaaaagtttggatgtctgagtccttctatcccaaaacaagatcttggagggtcttccacagccatgtaataccatggtcacatgaccctttccaaaattattaatctgaatttactatatgaggataaatctatctttttgaaaatatttaggaaaatgagcttggtatttataaaatgaagctctctttgggtggtatcctaagacacgtcaagccaatcagcctgtaactgtgaaaaaaacattggtaggtacaaaagtggggtgggagaggagtgacttaactttgttaagtgatgggaaagaaacactaatagcattatctcaataaaatgtgatttaaaaaaatttaaaatactaaatcattgaactgacaaagaaatataaatcattcagaaataaactcattaggtcatcaaatcctgttaaatctgcaattaggaagagcaaggtgtacaatccatacatttaaactcacaggctcactttgcacaacgtcaatttactccttaatatgttattaatacgcattttccaaaaggatgtattagtaaatggtacacatctacttcttggcaacatcatataacctggtacaacataagcattcttcttatagttaagaaatgtggatggtatcaaaattagaaaaataaatgccctattatgttgtggtcaggtttaaggcatgtgaattttatcttcatacaaaagattaaaatctagatattaaaaagtagtgcagtatcagtgatgctgcctcagttcccaaaatgtcacatcacaaaaatatcccataattgcctgtagtttattccttggctttcctcttttctctctgcatctttgtaacaattttttaaaagtggaaatataattgttggcaatgctaacagctgtagaaatgattacaagatgtggaaaagcataacaggaatgtcaagaatctgtttctggcagtaatatatatggaacattgttcaggacaaaagaggagaaggaagaaaaaaaggagaggggtttatcatctctaagaattttcaaactaaacctcattgcttaataggaaaaaaagattccatatttaaagttaagtcacctctaactactagctaaagcatgacatcaccagcactggagtcagcggaagtgtgtttttgaaggacagtgttgcaggagaatctggacaggttttagagccaggagagagaaaataattctacctctgacagttgaaggaccttaggcaaatcagtttacctctgctagactacactccaaaatttggacattcaaaaatttgatattaataaccacatgaaagtctcgtgttgaggtgaatatgtatttgttggtgaaagatatgttggtttttaaacagacagcactctgcaattgtaggctattgttttgttttgccagttgtcaaattctatccagctatacacacttgtgtggcctcctaatggtgtttttccagtggctaaaggtttatgaataagacacttttcctaatggaattaacccgatgcttttcttaaacatgtaaccttgagttcaccgcaaaaaacaatgcttcgattagagcaatgcatataataaaggttaccctcgtttcttagacactagacatcattcacaaaaagagaactgcttttgaaagggatgtatttgcactggaaagaatagttttctacttctaattataaatgatttattggtgaaagcaaaacaacagcctgtctgagaggcacttctatgagcatcctcacgtgtgatttgcaaggttgaagaagagggaaaaatgcctcaattgtaccaatggtgagaaaacacccaaagtacaaagcaggtttcaaaaaaaccatactcataaccaaggacaataataaagcaatgtgttgacatatactctataagtcttcctccataaatagtttatagaaattttgtaatttctgtaaatgcatcctataataattttgcatcttgctttttttttacatttaatatcaagtagatttctaaagggcaattatttgaaaattatcccaaatacatggggaaatatacatcaagtgaaaaaatgcagtgggtgatagagatatcaggaagcgcctcaaatatttctcatctcgttggagaaaaacaaacatgttctcatttagaatgagtgggagttacctaattgatttaggcctctatatttaacttctagtcaaaaaaggtagttctatctagcaacaatattatggggaacaaaagaaaaaattaactctctaaatttgcagtagggtcttttcttcagaagtaccaaatcccatctattaccagctccatgcttcaggcctaaaatggatctccctgaagcaatgacagaatttttgccaagtgactaggatataaacaccactttggttgcacagtgagacatatgctccaaagaaaactggttcaaaaacaggcaagtgggtttctacagaataaatgagagccctgtcaatggcttcatcttcagggctttgtgtctgtgcttgcgtggtggctcttgtttcatctatggataatggtggcacacagttttcataattccttacattaatgaactgctataaatttgtttttggtattctagagagtcctaacttcagcttctgggcaatgctgaggaggcaccctatattctagacttaccttttgcaaggtgtactctcagcattgtgggcgatttccatgggagaatattctatttaaagaactactgtcccagcataaaacaaaaaatcatttatgaagatgcaggagactcggaaagctctcaattattgtttgcacaagcacaatgtcacagcctcctttccccattccacaagggggtcaggaagagagtactcagctgtgagaaaagacatacagaagaattcatgtggtcatgagagcgaggacatggccgatcccccaaggaggatgtgtcatacacttcatgagcccaagagtgtgctgtagggtctgaagggcaagatgctggttcactgatgtaaaggagagggaaaaaagcttcaaccaactagaaaaacagtctctatgcatgctatttttgattttaaacacaggtatcaattccttctctcagagagtccattttaaaataggatacatttttaaaggaatatttaaaggacacattcattaaaatttattttaaaaacttttcaaaagaaacaaaaggtatgaattttatttaatccttgaggaaatggttcttttctcacacacataaatcactcattttgtttttctttatctcctttattaatctacattagaaaaataaacttttcatacactaagaacaaggaaaccactctcaattgacaaaatgttccaatccaacacaatgattactttcacctttaatttacaggcagccagattcaaaatccttaaagttgcttaaacttaaaaatgacaatgacaacctaaaaggtataatgttgattggaacagacatttaattggaaaattgatgattttccatttccaattaaatctctagatagaaatgaaaaaaattaaaaatcgtatttaagaaaagccaaatcttgggttgtgaggtatctttttaaggatgtttcagcagaaaaaaacaaaggctctcacaattgtgtagctgcctagattaagtgggtatcctgatcaaggagatgggggatgatttggctttagtattccaatgataaagtttataatgagaataacatgttgctacaaaatccagtctcttcctcagatgccttccacagagggcaggaagctttgtcagttttgtttgctgatgatgcctggttccgtcaacaaataacacctgtcacacggtgggtagtcaatatacatttgttgaataaatatgaaaaaaagaaatgtacaatatgtttgtgaagccaactgtgtgtgcattgctattgaggtacacaaaaagtctttgttttaaatttgagaatgaggactttcaatggaatatatctataaaaatgaaaaaaagacattactgtctggacttttgtacagcaagagaagaaaaaccactagccaagagccaactcacctgataggcctggatcaagcatgcagctgtggagaacacccctgggactctaactctggcactctgcaagctgggtacttgggcaggacagcagcagcactcatgaactgggcagcacctgttggtgagggctgatcacatggattctctcatcccagccttacaatcagtccttcaggtacatactttttctgactttgctgatgaggaaactatgcacagaggttacacagcttaacaaagggttctcacctaatgaacaatgaaatgggattttagcctttctttgcatctggtcttagagccaatacccaagaagcactgtactgtatgcattgtctcagagaaacttactcttcctgggcctcagtctttaaaaggtgggcagttgacttaataagaattaaagatcaatgattaaggttcaaggcactccaaaattctggtctttattgaaaaggctacagaagtctcaccttaataataccctatagacttgatattcttggttaattaaatattggaaaccaatttcatagtaattgaggtcagaaaaaagtactcatgacattttagaatatgatgacaaagccatagataaatttcaatgcacctgtaattacttaaaactgttatagcatgcaatgtgttaccacaacagccagagaaatactaatttactcagcctattcttctagaccagtaaacactaggattaaatagatattttcattgaatttgttctacccttcattgccatttatagatagcttacttgtcatagattactttctaattgttttatgtttcctaactagcctgcaatactttggcaaggacctcaaacaatagtagacagtaggtgtaaaatagatggctacattgaacagatgactaaaaggatgcctcctaagtacctatatcttgaaatatatattattgtgccttgctttcaatttgtgattttaaaatctagaaatcacctgttttatgtaataacaataaaatccttctttgttgaaaacatgcacaaataaagtttacaagctcaaaaaattaaacagcagtaacggtcaagctttccaacaataaaatacattttggtaaggttttcattttacaaaaactcaaaatagctttatgagttcacaaaataatatgatatttttcaagatattaacatattcttataccggaagagcatagaataaaatttacttggagattgagcatttgcttctttaagaaatacttcttttagtatttttactttaatattatgaaagctacataattacattcagattcattaactactccagtagttaatttttaaaacttatgatgaatagttttgtttaaaatatataacattggtaatatgcaaatctgaatctgtaataaagaaggatttgcattcctgatttttttttctgatacaaccaatgacaaaataactaatggttccacagaggataaaatgtctcaaatctgttggttctgaaggtgaagcgagatttttgtactgataccgtgtatcactgagataccaggaggaaatggaattaaactcagatagttcaaatggagagattttaatgaagggacgacctacagaggtgtcggcagggttggggggaatcagcgagatatgcttagaacccaccgactggcaaacctccccctgaagatggagaaggaggaaggagtgttactggaatgagagcttgagtccaggggaggaggatgggctgctgaggaggcgacaccatcctgaaagaagaatcctctgccagaggcttttcagggtcatttcttcacactctctgcagggaagcacggagacagcaggaagaaatatcctaacctcactctcttccctctacaggtgcttccattggccaaatccacccagaggccagttggtggcgatcagctctcttcaagtggtatttaaatttcttctttcattttccttctggtaacaaagaagtctgtggctcaaaagatgtttctctaagaccccatcctattaggtctctgagctgtccacaaagaaatgaaattttcactttccaggaacctaacaaatgaaaagatagaaatcaattccaacagaatattaccaaagaaatcttttagaatggactgttaaaattatttatttgtatttatctggctctactatttgtggtacatttccacttcaaagctaaacctcaaataacatcatagtgagtggttgacttcatgtttaactgagatcttgaagactgaaaaagaccacgacaaacacacatctattttcttggctactgcatccgtgttcatcaccattctgatagtctgcaatgtattgcagctcaccctttgggaaggactaaagtagacatctgtttgttctgcttactcagcattcctaccctaattttcctttggagaacccctttattctagaccacgtgaagctaatgccaaaccccattccaggggatgcacctgaatccaacctccatcatctaaacagtgccttctccacgttcagagaagagcaagtgactcaaactgccctcataagaacagacctgggacttctgctgcaaatattgaagagtaagtactcttttttcttgctaggactaagctggtagtaccttctatgaggctatcatatggaaacaacttgtctgaaaatgaagccacaactagaaaacagatcctggtaacccggattgatggatccagccctaccttaaatggcaagacctaacccgaggctttttgcatcaaccaataaagtccttaagccagtttgagttggttttgtcacttgcagctaaaagaattctgactctaacaatgtgacaatagcaaaaataaacataactgcttttgaggtttctaatggattttcctccctatatacatgatttcatttaatcctcacaattcaggaaagcacatatctattaacattaaattaatattcattattttgaacacatgctatgtggataagggatgaggaaagccaaggaagtaatcaacgtgaaatctcacttatatgggagggaagtggaggttacatatctcagggcacttaacagatatcatcaaatgaaagaataaacagtgtgtgggagaggcagtaggtgattcttcatcaattcctggatgaaaaattaggagataatgaactccgaacaggcagcctaatgagaatggctcaagcaacaggacatagagagggagttaggttagacatggggttcttgggaattttcacctcgtgggggggcgggggggtcgtgcagctgttgtcagtgggaaagggaaaaaggaaaaggctgagtttggaaggcagggagggaggagacaatgtgagtcagtgaaaaagggcccttagaatgacaagtctggaccagagagaggctaagactgaaaatacaagttgggtaaccactggcatacagatggcagttcaggcttgggcactgcccaccagagcctcagcatgaagagaagagggggaggctggccaccacctccctctaggtaatcgtcatcctgatgctgagctcctgaaaacaggctctttcactcgccccatctcttgctcttgattgcaacccggcattcaggaggcaccctgtaatatctgtggagtgaccgacaacacagcgccagggcactgagaagatcccagggcgccagggactggttctacaagggtgcccctcccggtcccctccagcgcgccgccagagctgccagtcttggctgctacacgggaggcagcctcattatgcagctctcacctcttaaattagttcatgctctcacattaggtgtaatcacagcttgcaacgctttctggggatgtctcagaaagatctgagttgaaaaaatatttttgtgtcattttaatttaaagtaaaattgctgcttcttccccgcccctttctttcctcctggcccacccagcgaccctggccggccgtgctcaacgggggcgggggtcggaggtgagatttcctccacataattccttaaacagctatcaactaagtctcaaagaaaaaaaaaagagatctagaagcagagacgtggctgctggcgatcccaaagctggtgttcgctcttgggggagagcgtaccctgggggaggccgggaggccgggccagaggctagcccagaggcagagggcaggagcgctcagccggcgccccgcgtctctccagctcccgacgctgcgctggctccgctgagcacgccaggatcaaggtcgcctggtggggaccggagcgccaggagcctgtgggaagcgttccagccggcctctgactgggatccggcgccgcgtttctgctttggacttgactgacaggtccccccgccctcccgccgccctactaccagcctgggttcatccttcagggctacgtctaccgcacccgggctggaaagcctggagcgcgcccttcctctcctcatcttctcagctctcctttctccctgccacttggcaaagctgcattttgactttcacgttttggactacgtgtgtgtagttccaagtccatgcgtggcacgaaaatccacttagggtaaaaattattctcgaaaaatcgcccatctcaggatctggtgtctacactcaaggctaggaggtgcaggtacgggtgcgtaaagcatgccgtaagggtgcacagtaaataaaaagtacggatgcaaaatgtaaattttaagtgcaaaacagaaaagcagtactcgttgccgccccgcacgctgggttttaaggggcacgaaggtgggcctcggctgcttttgctcagccccgcgtcctcagcgcccggcccagtacccggtactccgtaggggttcaatgatctcccctgaataagtgaacgaattaacaaatgaatgaatgaccgctcgatccgacctccgcggccggcagagcagtcgctggagaggcgggagagagcgagaggccaagctccaccatcgcggccgccggctggggcagagggacacggagacactcggcgccccggctccgcaccgagtccccg

SEQ ID NO: 12753 - RNA, 12359 nt, Homo sapiens
  source 1..12359: mol_type = other RNA
gatctcactttgttgcccaggctggtcttaaactcctggcctcaagtgatccccttgtttcagccccgcaaagtgctgggattacaggtgtgagccaccatgcccgtgcccagccacctcatgagtcttgatggggggcagagaccaacaactccacagaagccagatgcttgctttcccagcctctcttgcagctagggcttgggcatgtgatccaggctcagccaatcagatggcactgactcttggcatgacatgggctaaggaggggctgcagggaatccatttgggctggggtggcagctgcactgggagcgacatcagtttccagagggagcagcagaatctggcatcaggcttggggcgtggtaggtgcaaccagactctgcacccagcagcagtggcagaatgggttctctgtggagagtctgtgtattgctccttccgctgaggccaccagcatctgcctccatgaacccctcagagcctgtgagcaactcaacagccttgaattttttcccttcctgtttgaatgagccagggttgtttcactgcttgaactaagagccgttcctgacatgaaaactaagccacatctttttgacccaaagattctggcatcctaaaatacccatctcattttaagttaaaaataaatccatgtttgagcatctactgtttcagttactgtgctaggtgttacaaagctaactaagagtgacaagtaaataactatcatcaccatgataaacagagaatggaaccctggtttttggaatacagacacaaaatgattaattctgcctggaagcgttttggaacatttcagagaggtagtgagctgggccaagagaagagcatacgcaaggaatggtggcatgaagttgcctggtgtgtcctgagaagaaagatgggctaagaaggactggggtagggcagagaagggggtcactggaggtgaggctgggaaagtgagccaaggctcaaatgcaaactgtctgaacttcattttctgtgcaagcaggagaagccgctgacatgggtttggaagatggactgaagccggagaaaaatggaagcaagaaaccctctcacaagaggccataaccacaaccaagtccatgagattgaaaaggaaggcagatatttgaaaaatatttaaagagatgtgaggggtaggacaggcacagtggctcatgcctgtagtcccagcactttgggaggccgaggtgggcagatccacgaggtcaggagatcaagaccatcctaacatggtaaaaccccatctctactaacaatacaaaaaattagtcaggtgtggtggcacgtgcctgtagtcccagctactcaggaggctgaggcaggagaatcgcttgaacctgggaggcggaggttgcagtgagccgagattgtgccactgcaccctagcctaggcaacagagcaagactctgtctcaaaaaaaataaaaaaaaaaaaaagagagaaagagagagagagatgaggagttgctgcactgctgggtgtggagagccgaggaggattcaaagatggtcctgaagtcccagctggaagaagtaggcggcagcaatgtttttaatactgtaaattcatcacgtagcacaggtttggggtggagaaagaaaaattgcattggcttcagggcatgcccagatctttcctcatcttaggcgtttgctaatacatgcattttctaagctgatgtcttgcgtttaatcactgctccattcaaaagagagaaggaggttgtttcaaacctagttgatatcatttgacttccatgctattcacagggctattttatttgaaacaggtataccacagccttaaattgcaagttaatccaggatgttcctaggttggcagttaggaacatgtaattctttggaagggctaaaagtcagctctttaaattatctccatatgaaccttctctccaccttagggtggatccacttatttagtccactgccagtaccacactagaacccgggtggtcactggactccagaaacaacagtagccctctctctgttctgtctctttttgactatctctattctgttcctgaccctgatttctcctgccaagctcaattttgacagctgacaacggcaagccatggcttcccaaaacattattttcaggtcaacttataaatttcaagaacacatttggctccgcttcctgtggtactaagcctacttcttgacagcatttgcctttgttgtaaatagcaaagttcttctagttggatttttgctaagaagtgtgtggatgtggcatgtgacgacatctttagcttggattctagaaaggcactaccattgtgcatttggctaaaggaaacacattttacccgtgaatgccttctatttacaaatgctcagctagcacacaaagctaagtacaagcaataagtactatcctacaatgttactcatttctgaaagcacaaaatgatgactggtatagctttggagatgttttctggaaacccaataaaggaacagatctttgttattccacacctacaaagtcagaagatgcacagtcttttattcatgtttgaacaagcttccttcttgaacaatcaactataaagtgatgtgattctctactagaccaggaactccttgaggacagaatgagggtctaatccatattctaaatccacaccacctggcacaatacatgttgcatggttagggtcaactaagagttggttgaattaatcaataacacacagcaagagaattcacaaagagaggggagtaatcccccagcctcaatcactcggcaagtggaatcgctgggcactgattccagctctgtctcagtgcttgagacagagctgaatgtaatgtgaacatttcaaatgaacaggaaaactagactcacggataagcagtgtagtcatcaagacaacactgtcttggaggtttttctgaagttaaaaccatgctacataagcaataaattatgaaggctgagcatgtgaataaaatttaatgttgtcataaattttataacaaagttaatctgacacatttaatgacatgcataatcattagtatgcagcactgtaatcagacattgataataagcagttcacaccagtgactgtaagagtctttacttgtgttcagccaagccaactgcttggtatatttttctcccttcttagtcgttagttttccatacctacaataactatcagtggtgatgggcttctctgaccatgtgaataatttaatcctcaatgcacagatacagaaacccttgctgaagacagtgtggagcagagaaggctgtctccactccttccacctgaaacacctctgcagatggatatgggagctctgcctacagcccttggacctaaccacttcagtgtgttccagtgagtgtctggacctcggcctgaaagatttttccgaaactaaagaaaatttctctgacctaaagaccttaacctccaccccagaagctctcaccaaggactacagggaactggtggggaaaatccttatcccttactcctcaaggcacagggcagtaatgctgaggcttgtgcgccacacttgctcccagaggtccccagcgggctacctgcggtggtgaatgacctcctaacacgccccttgacggccttcctttccttgcctcacttctccactctcctaccagcattgcagggttcacatcccaaatataccactggcacttgaatcctggtctccaggtctgtttctggaaaaacccaagtaagacattgccccagtaatggggctagatgtctgaggcttcctcaagtatctacctcgaaagctcttactgctgtacacacatgcacatacacacacgtgcgtacaaccagtcacatctaagcaccccgaataccagcctgttgaaggtagcagagagctgcactataagccaaggctgctcccaagagccgctccatcactgaattggcgccccagcaagatgaaggaatgtaatcattggaaggatggagaatgttctctgaatcactgacaaattggaaggggtggagggcaagagtccacctggtggagagatggaaagagcgagagagcctggaatgataatgccattgcttagaaaaggctgctccagatgccatatctacagaaattgtacagcccaaacatctctgagcaataggtctctggtagtcttgatgtctagaccaacaattcccagttcattcttctcagggaaggagccaggatagtccagagactctcattctgctgttagattgaaagggttaggcacaacagccttggcaaagtcacaagggcaaattcacactaaagtgtaaatgacccacaactcctcttctatttttaggttggggaggtgctttagaacataaggaggaactaaagaatattcctgttacatacaaggcagagaaaagggaaactagtggtgacaagacaaatcatccctttgacatttggctggctctacctattacagctctgggggtgaggtgggaacaaaaagatgctgtgtaaagaagtatcttatgccatccctactgtagtgaggtgcagtttagaggggacactgatcaagcagagacccagagtgtttcgttccaagccagaaacagaaatgtataaaacacagcctttccagcatcagaaatgagtagtggtagtggagaactacccaaaacaggaaagaggaccacgtgaggtagagtgtcaaggccctacattccagtgcctctgctcatgactgtaattttgggtaggtcacttaaagtctctggacctcagttttgccatctgtgaaatagggataatactatccagcataaaattggttatgaggctcatgtagggcctgcctgggatgatgtgttgctaatggttaagaacacaacttctggggtctgactggacaggctgaaatccctgcttaacacgttccagcagagccctgggcgatctatttaacttttgttttctcacctgtaagctgagacgaaagtacccactttataagattattccaataattagttgaaataatgcatgcagagaattaagcatggtacttgttatttgttaaactagctattaaaatgtgtaaaatataaagtattgtatggattttaggacaatgcaaagactctttgcttgctgcaatagttcggggccctttcagatggctaaaggcagaatttgtatgtgtaaatatggtgtgcttgtctctgctctggatactgagggcttaccctgttattaaacttatttagtaaatattgaactgtcatgaggcctaacatttagttccagttattagataaaacatttgctttgaatggtatttgaattgccaggttctagattattctggttgacaaactcttcgtattttataaagaggctaaaattggtaagctatcacagaacagatgtgccattttcaaggtatattaaaccatgattcactgtaacattgttcctactggcaacaaattcagagcaggctggactttatttggtgaagaaacattgagtggaagagaaatgacattattttatgtatttacattttcaaattactgtggcttaaacctgttcagccaacattacccaccttcagtctgctaaataaatgattcagtacatttctaatttacagaattttttaacaaaagaaaatgtaatttgatagccaaatcaacgttaaacattatacatttaaaaaaccacaggcaaagacacaaacatgatgacactaacttttgttaaagtatgcttacctatggtttcctctgaggcacgttctttcatgctaagcttccaacataatatgaaaatgaaggagatgcattttgcaaagcaaaacagaccttaagcaaaatattatacttctcaaattaacactgttacaaagttttagaatttaataagttcattaatttaaaagtttggatgtctgagtccttctatcccaaaacaagatcttggagggtcttccacagccatgtaataccatggtcacatgaccctttccaaaattattaatctgaatttactatatgaggataaatctatctttttgaaaatatttaggaaaatgagcttggtatttataaaatgaagctctctttgggtggtatcctaagacacgtcaagccaatcagcctgtaactgtgaaaaaaacattggtaggtacaaaagtggggtgggagaggagtgacttaactttgttaagtgatgggaaagaaacactaatagcattatctcaataaaatgtgatttaaaaaaatttaaaatactaaatcattgaactgacaaagaaatataaatcattcagaaataaactcattaggtcatcaaatcctgttaaatctgcaattaggaagagcaaggtgtacaatccatacatttaaactcacaggctcactttgcacaacgtcaatttactccttaatatgttattaatacgcattttccaaaaggatgtattagtaaatggtacacatctacttcttggcaacatcatataacctggtacaacataagcattcttcttatagttaagaaatgtggatggtatcaaaattagaaaaataaatgccctattatgttgtggtcaggtttaaggcatgtgaattttatcttcatacaaaagattaaaatctagatattaaaaagtagtgcagtatcagtgatgctgcctcagttcccaaaatgtcacatcacaaaaatatcccataattgcctgtagtttattccttggctttcctcttttctctctgcatctttgtaacaattttttaaaagtggaaatataattgttggcaatgctaacagctgtagaaatgattacaagatgtggaaaagcataacaggaatgtcaagaatctgtttctggcagtaatatatatggaacattgttcaggacaaaagaggagaaggaagaaaaaaaggagaggggtttatcatctctaagaattttcaaactaaacctcattgcttaataggaaaaaaagattccatatttaaagttaagtcacctctaactactagctaaagcatgacatcaccagcactggagtcagcggaagtgtgtttttgaaggacagtgttgcaggagaatctggacaggttttagagccaggagagagaaaataattctacctctgacagttgaaggaccttaggcaaatcagtttacctctgctagactacactccaaaatttggacattcaaaaatttgatattaataaccacatgaaagtctcgtgttgaggtgaatatgtatttgttggtgaaagatatgttggtttttaaacagacagcactctgcaattgtaggctattgttttgttttgccagttgtcaaattctatccagctatacacacttgtgtggcctcctaatggtgtttttccagtggctaaaggtttatgaataagacacttttcctaatggaattaacccgatgcttttcttaaacatgtaaccttgagttcaccgcaaaaaacaatgcttcgattagagcaatgcatataataaaggttaccctcgtttcttagacactagacatcattcacaaaaagagaactgcttttgaaagggatgtatttgcactggaaagaatagttttctacttctaattataaatgatttattggtgaaagcaaaacaacagcctgtctgagaggcacttctatgagcatcctcacgtgtgatttgcaaggttgaagaagagggaaaaatgcctcaattgtaccaatggtgagaaaacacccaaagtacaaagcaggtttcaaaaaaaccatactcataaccaaggacaataataaagcaatgtgttgacatatactctataagtcttcctccataaatagtttatagaaattttgtaatttctgtaaatgcatcctataataattttgcatcttgctttttttttacatttaatatcaagtagatttctaaagggcaattatttgaaaattatcccaaatacatggggaaatatacatcaagtgaaaaaatgcagtgggtgatagagatatcaggaagcgcctcaaatatttctcatctcgttggagaaaaacaaacatgttctcatttagaatgagtgggagttacctaattgatttaggcctctatatttaacttctagtcaaaaaaggtagttctatctagcaacaatattatggggaacaaaagaaaaaattaactctctaaatttgcagtagggtcttttcttcagaagtaccaaatcccatctattaccagctccatgcttcaggcctaaaatggatctccctgaagcaatgacagaatttttgccaagtgactaggatataaacaccactttggttgcacagtgagacatatgctccaaagaaaactggttcaaaaacaggcaagtgggtttctacagaataaatgagagccctgtcaatggcttcatcttcagggctttgtgtctgtgcttgcgtggtggctcttgtttcatctatggataatggtggcacacagttttcataattccttacattaatgaactgctataaatttgtttttggtattctagagagtcctaacttcagcttctgggcaatgctgaggaggcaccctatattctagacttaccttttgcaaggtgtactctcagcattgtgggcgatttccatgggagaatattctatttaaagaactactgtcccagcataaaacaaaaaatcatttatgaagatgcaggagactcggaaagctctcaattattgtttgcacaagcacaatgtcacagcctcctttccccattccacaagggggtcaggaagagagtactcagctgtgagaaaagacatacagaagaattcatgtggtcatgagagcgaggacatggccgatcccccaaggaggatgtgtcatacacttcatgagcccaagagtgtgctgtagggtctgaagggcaagatgctggttcactgatgtaaaggagagggaaaaaagcttcaaccaactagaaaaacagtctctatgcatgctatttttgattttaaacacaggtatcaattccttctctcagagagtccattttaaaataggatacatttttaaaggaatatttaaaggacacattcattaaaatttattttaaaaacttttcaaaagaaacaaaaggtatgaattttatttaatccttgaggaaatggttcttttctcacacacataaatcactcattttgtttttctttatctcctttattaatctacattagaaaaataaacttttcatacactaagaacaaggaaaccactctcaattgacaaaatgttccaatccaacacaatgattactttcacctttaatttacaggcagccagattcaaaatccttaaagttgcttaaacttaaaaatgacaatgacaacctaaaaggtataatgttgattggaacagacatttaattggaaaattgatgattttccatttccaattaaatctctagatagaaatgaaaaaaattaaaaatcgtatttaagaaaagccaaatcttgggttgtgaggtatctttttaaggatgtttcagcagaaaaaaacaaaggctctcacaattgtgtagctgcctagattaagtgggtatcctgatcaaggagatgggggatgatttggctttagtattccaatgataaagtttataatgagaataacatgttgctacaaaatccagtctcttcctcagatgccttccacagagggcaggaagctttgtcagttttgtttgctgatgatgcctggttccgtcaacaaataacacctgtcacacggtgggtagtcaatatacatttgttgaataaatatgaaaaaaagaaatgtacaatatgtttgtgaagccaactgtgtgtgcattgctattgaggtacacaaaaagtctttgttttaaatttgagaatgaggactttcaatggaatatatctataaaaatgaaaaaaagacattactgtctggacttttgtacagcaagagaagaaaaaccactagccaagagccaactcacctgataggcctggatcaagcatgcagctgtggagaacacccctgggactctaactctggcactctgcaagctgggtacttgggcaggacagcagcagcactcatgaactgggcagcacctgttggtgagggctgatcacatggattctctcatcccagccttacaatcagtccttcaggtacatactttttctgactttgctgatgaggaaactatgcacagaggttacacagcttaacaaagggttctcacctaatgaacaatgaaatgggattttagcctttctttgcatctggtcttagagccaatacccaagaagcactgtactgtatgcattgtctcagagaaacttactcttcctgggcctcagtctttaaaaggtgggcagttgacttaataagaattaaagatcaatgattaaggttcaaggcactccaaaattctggtctttattgaaaaggctacagaagtctcaccttaataataccctatagacttgatattcttggttaattaaatattggaaaccaatttcatagtaattgaggtcagaaaaaagtactcatgacattttagaatatgatgacaaagccatagataaatttcaatgcacctgtaattacttaaaactgttatagcatgcaatgtgttaccacaacagccagagaaatactaatttactcagcctattcttctagaccagtaaacactaggattaaatagatattttcattgaatttgttctacccttcattgccatttatagatagcttacttgtcatagattactttctaattgttttatgtttcctaactagcctgcaatactttggcaaggacctcaaacaatagtagacagtaggtgtaaaatagatggctacattgaacagatgactaaaaggatgcctcctaagtacctatatcttgaaatatatattattgtgccttgctttcaatttgtgattttaaaatctagaaatcacctgttttatgtaataacaataaaatccttctttgttgaaaacatgcacaaataaagtttacaagctcaaaaaattaaacagcagtaacggtcaagctttccaacaataaaatacattttggtaaggttttcattttacaaaaactcaaaatagctttatgagttcacaaaataatatgatatttttcaagatattaacatattcttataccggaagagcatagaataaaatttacttggagattgagcatttgcttctttaagaaatacttcttttagtatttttactttaatattatgaaagctacataattacattcagattcattaactactccagtagttaatttttaaaacttatgatgaatagttttgtttaaaatatataacattggtaatatgcaaatctgaatctgtaataaagaaggatttgcattcctgatttttttttctgatacaaccaatgacaaaataactaatggttccacagaggataaaatgtctcaaatctgttggttctgaaggtgaagcgagatttttgtactgataccgtgtatcactgagataccaggaggaaatggaattaaactcagatagttcaaatggagagattttaatgaagggacgacctacagaggtgtcggcagggttggggggaatcagcgagatatgcttagaacccaccgactggcaaacctccccctgaagatggagaaggaggaaggagtgttactggaatgagagcttgagtccaggggaggaggatgggctgctgaggaggcgacaccatcctgaaagaagaatcctctgccagaggcttttcagggtcatttcttcacactctctgcagggaagcacggagacagcaggaagaaatatcctaacctcactctcttccctctacaggtgcttccattggccaaatccacccagaggccagttggtggcgatcagctctcttcaagtggtatttaaatttcttctttcattttccttctggtaacaaagaagtctgtggctcaaaagatgtttctctaagaccccatcctattaggtctctgagctgtccacaaagaaatgaaattttcactttccaggaacctgagggccgacgagtgggggcgggcaggagggccgagggaggcggaacaggatcgaggcgcgaggcgggagtcgagaaagcgagcggccgaggcgactctcagtgcgcggacgcgggcgcgcgcccgcgctcccttcgtcgactcacggcgagagcccaaccctgctgccgcgcgccaccc

SEQ ID NO: 12754 - RNA, 14167 nt, Homo sapiens
  source 1..14167: mol_type = other RNA
gatctcactttgttgcccaggctggtcttaaactcctggcctcaagtgatccccttgtttcagccccgcaaagtgctgggattacaggtgtgagccaccatgcccgtgcccagccacctcatgagtcttgatggggggcagagaccaacaactccacagaagccagatgcttgctttcccagcctctcttgcagctagggcttgggcatgtgatccaggctcagccaatcagatggcactgactcttggcatgacatgggctaaggaggggctgcagggaatccatttgggctggggtggcagctgcactgggagcgacatcagtttccagagggagcagcagaatctggcatcaggcttggggcgtggtaggtgcaaccagactctgcacccagcagcagtggcagaatgggttctctgtggagagtctgtgtattgctccttccgctgaggccaccagcatctgcctccatgaacccctcagagcctgtgagcaactcaacagccttgaattttttcccttcctgtttgaatgagccagggttgtttcactgcttgaactaagagccgttcctgacatgaaaactaagccacatctttttgacccaaagattctggcatcctaaaatacccatctcattttaagttaaaaataaatccatgtttgagcatctactgtttcagttactgtgctaggtgttacaaagctaactaagagtgacaagtaaataactatcatcaccatgataaacagagaatggaaccctggtttttggaatacagacacaaaatgattaattctgcctggaagcgttttggaacatttcagagaggtagtgagctgggccaagagaagagcatacgcaaggaatggtggcatgaagttgcctggtgtgtcctgagaagaaagatgggctaagaaggactggggtagggcagagaagggggtcactggaggtgaggctgggaaagtgagccaaggctcaaatgcaaactgtctgaacttcattttctgtgcaagcaggagaagccgctgacatgggtttggaagatggactgaagccggagaaaaatggaagcaagaaaccctctcacaagaggccataaccacaaccaagtccatgagattgaaaaggaaggcagatatttgaaaaatatttaaagagatgtgaggggtaggacaggcacagtggctcatgcctgtagtcccagcactttgggaggccgaggtgggcagatccacgaggtcaggagatcaagaccatcctaacatggtaaaaccccatctctactaacaatacaaaaaattagtcaggtgtggtggcacgtgcctgtagtcccagctactcaggaggctgaggcaggagaatcgcttgaacctgggaggcggaggttgcagtgagccgagattgtgccactgcaccctagcctaggcaacagagcaagactctgtctcaaaaaaaataaaaaaaaaaaaaagagagaaagagagagagagatgaggagttgctgcactgctgggtgtggagagccgaggaggattcaaagatggtcctgaagtcccagctggaagaagtaggcggcagcaatgtttttaatactgtaaattcatcacgtagcacaggtttggggtggagaaagaaaaattgcattggcttcagggcatgcccagatctttcctcatcttaggcgtttgctaatacatgcattttctaagctgatgtcttgcgtttaatcactgctccattcaaaagagagaaggaggttgtttcaaacctagttgatatcatttgacttccatgctattcacagggctattttatttgaaacaggtataccacagccttaaattgcaagttaatccaggatgttcctaggttggcagttaggaacatgtaattctttggaagggctaaaagtcagctctttaaattatctccatatgaaccttctctccaccttagggtggatccacttatttagtccactgccagtaccacactagaacccgggtggtcactggactccagaaacaacagtagccctctctctgttctgtctctttttgactatctctattctgttcctgaccctgatttctcctgccaagctcaattttgacagctgacaacggcaagccatggcttcccaaaacattattttcaggtcaacttataaatttcaagaacacatttggctccgcttcctgtggtactaagcctacttcttgacagcatttgcctttgttgtaaatagcaaagttcttctagttggatttttgctaagaagtgtgtggatgtggcatgtgacgacatctttagcttggattctagaaaggcactaccattgtgcatttggctaaaggaaacacattttacccgtgaatgccttctatttacaaatgctcagctagcacacaaagctaagtacaagcaataagtactatcctacaatgttactcatttctgaaagcacaaaatgatgactggtatagctttggagatgttttctggaaacccaataaaggaacagatctttgttattccacacctacaaagtcagaagatgcacagtcttttattcatgtttgaacaagcttccttcttgaacaatcaactataaagtgatgtgattctctactagaccaggaactccttgaggacagaatgagggtctaatccatattctaaatccacaccacctggcacaatacatgttgcatggttagggtcaactaagagttggttgaattaatcaataacacacagcaagagaattcacaaagagaggggagtaatcccccagcctcaatcactcggcaagtggaatcgctgggcactgattccagctctgtctcagtgcttgagacagagctgaatgtaatgtgaacatttcaaatgaacaggaaaactagactcacggataagcagtgtagtcatcaagacaacactgtcttggaggtttttctgaagttaaaaccatgctacataagcaataaattatgaaggctgagcatgtgaataaaatttaatgttgtcataaattttataacaaagttaatctgacacatttaatgacatgcataatcattagtatgcagcactgtaatcagacattgataataagcagttcacaccagtgactgtaagagtctttacttgtgttcagccaagccaactgcttggtatatttttctcccttcttagtcgttagttttccatacctacaataactatcagtggtgatgggcttctctgaccatgtgaataatttaatcctcaatgcacagatacagaaacccttgctgaagacagtgtggagcagagaaggctgtctccactccttccacctgaaacacctctgcagatggatatgggagctctgcctacagcccttggacctaaccacttcagtgtgttccagtgagtgtctggacctcggcctgaaagatttttccgaaactaaagaaaatttctctgacctaaagaccttaacctccaccccagaagctctcaccaaggactacagggaactggtggggaaaatccttatcccttactcctcaaggcacagggcagtaatgctgaggcttgtgcgccacacttgctcccagaggtccccagcgggctacctgcggtggtgaatgacctcctaacacgccccttgacggccttcctttccttgcctcacttctccactctcctaccagcattgcagggttcacatcccaaatataccactggcacttgaatcctggtctccaggtctgtttctggaaaaacccaagtaagacattgccccagtaatggggctagatgtctgaggcttcctcaagtatctacctcgaaagctcttactgctgtacacacatgcacatacacacacgtgcgtacaaccagtcacatctaagcaccccgaataccagcctgttgaaggtagcagagagctgcactataagccaaggctgctcccaagagccgctccatcactgaattggcgccccagcaagatgaaggaatgtaatcattggaaggatggagaatgttctctgaatcactgacaaattggaaggggtggagggcaagagtccacctggtggagagatggaaagagcgagagagcctggaatgataatgccattgcttagaaaaggctgctccagatgccatatctacagaaattgtacagcccaaacatctctgagcaataggtctctggtagtcttgatgtctagaccaacaattcccagttcattcttctcagggaaggagccaggatagtccagagactctcattctgctgttagattgaaagggttaggcacaacagccttggcaaagtcacaagggcaaattcacactaaagtgtaaatgacccacaactcctcttctatttttaggttggggaggtgctttagaacataaggaggaactaaagaatattcctgttacatacaaggcagagaaaagggaaactagtggtgacaagacaaatcatccctttgacatttggctggctctacctattacagctctgggggtgaggtgggaacaaaaagatgctgtgtaaagaagtatcttatgccatccctactgtagtgaggtgcagtttagaggggacactgatcaagcagagacccagagtgtttcgttccaagccagaaacagaaatgtataaaacacagcctttccagcatcagaaatgagtagtggtagtggagaactacccaaaacaggaaagaggaccacgtgaggtagagtgtcaaggccctacattccagtgcctctgctcatgactgtaattttgggtaggtcacttaaagtctctggacctcagttttgccatctgtgaaatagggataatactatccagcataaaattggttatgaggctcatgtagggcctgcctgggatgatgtgttgctaatggttaagaacacaacttctggggtctgactggacaggctgaaatccctgcttaacacgttccagcagagccctgggcgatctatttaacttttgttttctcacctgtaagctgagacgaaagtacccactttataagattattccaataattagttgaaataatgcatgcagagaattaagcatggtacttgttatttgttaaactagctattaaaatgtgtaaaatataaagtattgtatggattttaggacaatgcaaagactctttgcttgctgcaatagttcggggccctttcagatggctaaaggcagaatttgtatgtgtaaatatggtgtgcttgtctctgctctggatactgagggcttaccctgttattaaacttatttagtaaatattgaactgtcatgaggcctaacatttagttccagttattagataaaacatttgctttgaatggtatttgaattgccaggttctagattattctggttgacaaactcttcgtattttataaagaggctaaaattggtaagctatcacagaacagatgtgccattttcaaggtatattaaaccatgattcactgtaacattgttcctactggcaacaaattcagagcaggctggactttatttggtgaagaaacattgagtggaagagaaatgacattattttatgtatttacattttcaaattactgtggcttaaacctgttcagccaacattacccaccttcagtctgctaaataaatgattcagtacatttctaatttacagaattttttaacaaaagaaaatgtaatttgatagccaaatcaacgttaaacattatacatttaaaaaaccacaggcaaagacacaaacatgatgacactaacttttgttaaagtatgcttacctatggtttcctctgaggcacgttctttcatgctaagcttccaacataatatgaaaatgaaggagatgcattttgcaaagcaaaacagaccttaagcaaaatattatacttctcaaattaacactgttacaaagttttagaatttaataagttcattaatttaaaagtttggatgtctgagtccttctatcccaaaacaagatcttggagggtcttccacagccatgtaataccatggtcacatgaccctttccaaaattattaatctgaatttactatatgaggataaatctatctttttgaaaatatttaggaaaatgagcttggtatttataaaatgaagctctctttgggtggtatcctaagacacgtcaagccaatcagcctgtaactgtgaaaaaaacattggtaggtacaaaagtggggtgggagaggagtgacttaactttgttaagtgatgggaaagaaacactaatagcattatctcaataaaatgtgatttaaaaaaatttaaaatactaaatcattgaactgacaaagaaatataaatcattcagaaataaactcattaggtcatcaaatcctgttaaatctgcaattaggaagagcaaggtgtacaatccatacatttaaactcacaggctcactttgcacaacgtcaatttactccttaatatgttattaatacgcattttccaaaaggatgtattagtaaatggtacacatctacttcttggcaacatcatataacctggtacaacataagcattcttcttatagttaagaaatgtggatggtatcaaaattagaaaaataaatgccctattatgttgtggtcaggtttaaggcatgtgaattttatcttcatacaaaagattaaaatctagatattaaaaagtagtgcagtatcagtgatgctgcctcagttcccaaaatgtcacatcacaaaaatatcccataattgcctgtagtttattccttggctttcctcttttctctctgcatctttgtaacaattttttaaaagtggaaatataattgttggcaatgctaacagctgtagaaatgattacaagatgtggaaaagcataacaggaatgtcaagaatctgtttctggcagtaatatatatggaacattgttcaggacaaaagaggagaaggaagaaaaaaaggagaggggtttatcatctctaagaattttcaaactaaacctcattgcttaataggaaaaaaagattccatatttaaagttaagtcacctctaactactagctaaagcatgacatcaccagcactggagtcagcggaagtgtgtttttgaaggacagtgttgcaggagaatctggacaggttttagagccaggagagagaaaataattctacctctgacagttgaaggaccttaggcaaatcagtttacctctgctagactacactccaaaatttggacattcaaaaatttgatattaataaccacatgaaagtctcgtgttgaggtgaatatgtatttgttggtgaaagatatgttggtttttaaacagacagcactctgcaattgtaggctattgttttgttttgccagttgtcaaattctatccagctatacacacttgtgtggcctcctaatggtgtttttccagtggctaaaggtttatgaataagacacttttcctaatggaattaacccgatgcttttcttaaacatgtaaccttgagttcaccgcaaaaaacaatgcttcgattagagcaatgcatataataaaggttaccctcgtttcttagacactagacatcattcacaaaaagagaactgcttttgaaagggatgtatttgcactggaaagaatagttttctacttctaattataaatgatttattggtgaaagcaaaacaacagcctgtctgagaggcacttctatgagcatcctcacgtgtgatttgcaaggttgaagaagagggaaaaatgcctcaattgtaccaatggtgagaaaacacccaaagtacaaagcaggtttcaaaaaaaccatactcataaccaaggacaataataaagcaatgtgttgacatatactctataagtcttcctccataaatagtttatagaaattttgtaatttctgtaaatgcatcctataataattttgcatcttgctttttttttacatttaatatcaagtagatttctaaagggcaattatttgaaaattatcccaaatacatggggaaatatacatcaagtgaaaaaatgcagtgggtgatagagatatcaggaagcgcctcaaatatttctcatctcgttggagaaaaacaaacatgttctcatttagaatgagtgggagttacctaattgatttaggcctctatatttaacttctagtcaaaaaaggtagttctatctagcaacaatattatggggaacaaaagaaaaaattaactctctaaatttgcagtagggtcttttcttcagaagtaccaaatcccatctattaccagctccatgcttcaggcctaaaatggatctccctgaagcaatgacagaatttttgccaagtgactaggatataaacaccactttggttgcacagtgagacatatgctccaaagaaaactggttcaaaaacaggcaagtgggtttctacagaataaatgagagccctgtcaatggcttcatcttcagggctttgtgtctgtgcttgcgtggtggctcttgtttcatctatggataatggtggcacacagttttcataattccttacattaatgaactgctataaatttgtttttggtattctagagagtcctaacttcagcttctgggcaatgctgaggaggcaccctatattctagacttaccttttgcaaggtgtactctcagcattgtgggcgatttccatgggagaatattctatttaaagaactactgtcccagcataaaacaaaaaatcatttatgaagatgcaggagactcggaaagctctcaattattgtttgcacaagcacaatgtcacagcctcctttccccattccacaagggggtcaggaagagagtactcagctgtgagaaaagacatacagaagaattcatgtggtcatgagagcgaggacatggccgatcccccaaggaggatgtgtcatacacttcatgagcccaagagtgtgctgtagggtctgaagggcaagatgctggttcactgatgtaaaggagagggaaaaaagcttcaaccaactagaaaaacagtctctatgcatgctatttttgattttaaacacaggtatcaattccttctctcagagagtccattttaaaataggatacatttttaaaggaatatttaaaggacacattcattaaaatttattttaaaaacttttcaaaagaaacaaaaggtatgaattttatttaatccttgaggaaatggttcttttctcacacacataaatcactcattttgtttttctttatctcctttattaatctacattagaaaaataaacttttcatacactaagaacaaggaaaccactctcaattgacaaaatgttccaatccaacacaatgattactttcacctttaatttacaggcagccagattcaaaatccttaaagttgcttaaacttaaaaatgacaatgacaacctaaaaggtataatgttgattggaacagacatttaattggaaaattgatgattttccatttccaattaaatctctagatagaaatgaaaaaaattaaaaatcgtatttaagaaaagccaaatcttgggttgtgaggtatctttttaaggatgtttcagcagaaaaaaacaaaggctctcacaattgtgtagctgcctagattaagtgggtatcctgatcaaggagatgggggatgatttggctttagtattccaatgataaagtttataatgagaataacatgttgctacaaaatccagtctcttcctcagatgccttccacagagggcaggaagctttgtcagttttgtttgctgatgatgcctggttccgtcaacaaataacacctgtcacacggtgggtagtcaatatacatttgttgaataaatatgaaaaaaagaaatgtacaatatgtttgtgaagccaactgtgtgtgcattgctattgaggtacacaaaaagtctttgttttaaatttgagaatgaggactttcaatggaatatatctataaaaatgaaaaaaagacattactgtctggacttttgtacagcaagagaagaaaaaccactagccaagagccaactcacctgataggcctggatcaagcatgcagctgtggagaacacccctgggactctaactctggcactctgcaagctgggtacttgggcaggacagcagcagcactcatgaactgggcagcacctgttggtgagggctgatcacatggattctctcatcccagccttacaatcagtccttcaggtacatactttttctgactttgctgatgaggaaactatgcacagaggttacacagcttaacaaagggttctcacctaatgaacaatgaaatgggattttagcctttctttgcatctggtcttagagccaatacccaagaagcactgtactgtatgcattgtctcagagaaacttactcttcctgggcctcagtctttaaaaggtgggcagttgacttaataagaattaaagatcaatgattaaggttcaaggcactccaaaattctggtctttattgaaaaggctacagaagtctcaccttaataataccctatagacttgatattcttggttaattaaatattggaaaccaatttcatagtaattgaggtcagaaaaaagtactcatgacattttagaatatgatgacaaagccatagataaatttcaatgcacctgtaattacttaaaactgttatagcatgcaatgtgttaccacaacagccagagaaatactaatttactcagcctattcttctagaccagtaaacactaggattaaatagatattttcattgaatttgttctacccttcattgccatttatagatagcttacttgtcatagattactttctaattgttttatgtttcctaactagcctgcaatactttggcaaggacctcaaacaatagtagacagtaggtgtaaaatagatggctacattgaacagatgactaaaaggatgcctcctaagtacctatatcttgaaatatatattattgtgccttgctttcaatttgtgattttaaaatctagaaatcacctgttttatgtaataacaataaaatccttctttgttgaaaacatgcacaaataaagtttacaagctcaaaaaattaaacagcagtaacggtcaagctttccaacaataaaatacattttggtaaggttttcattttacaaaaactcaaaatagctttatgagttcacaaaataatatgatatttttcaagatattaacatattcttataccggaagagcatagaataaaatttacttggagattgagcatttgcttctttaagaaatacttcttttagtatttttactttaatattatgaaagctacataattacattcagattcattaactactccagtagttaatttttaaaacttatgatgaatagttttgtttaaaatatataacattggtaatatgcaaatctgaatctgtaataaagaaggatttgcattcctgatttttttttctgatacaaccaatgacaaaataactaatggttccacagaggataaaatgtctcaaatctgttggttctgaaggtgaagcgagatttttgtactgataccgtgtatcactgagataccaggaggaaatggaattaaactcagatagttcaaatggagagattttaatgaagggacgacctacagaggtgtcggcagggttggggggaatcagcgagatatgcttagaacccaccgactggcaaacctccccctgaagatggagaaggaggaaggagtgttactggaatgagagcttgagtccaggggaggaggatgggctgctgaggaggcgacaccatcctgaaagaagaatcctctgccagaggcttttcagggtcatttcttcacactctctgcagggaagcacggagacagcaggaagaaatatcctaacctcactctcttccctctacaggtgcttccattggccaaatccacccagaggccagttggtggcgatcagctctcttcaagtggtatttaaatttcttctttcattttccttctggtaacaaagaagtctgtggctcaaaagatgtttctctaagaccccatcctattaggtctctgagctgtgggaagtatttatacaattgcttgtgaatataagatccaggaatttccctaagatccctaacaaaattggtgataagtagtcccacatgttaatccagccacccacggatgacagcacttaccatttctttgataaatgtcaaatgcatttgaagtacctacctgaaatatttgtttaaatgctatctaatctattaattttatatatgtgtgagtctgttttgtataccttctgattataggataaatgtaaataaatccaaagagtaatcaaagctaccactttcaagaagccttctttgtagaaccggaagagtcttaaataggcttttcaggtatgcatctcttattatcgctgaactccaagtcctgcaaggcaggcatcatgtgtgggtcacctttacagtaggcacaggccttaaaacagtgacatgcacattgcaggcactccataaatgtttgctgaattggctaaaccttggtttgttcccataatcaaccaccacaaacagcacacagataattacttcttggaaagattccaactagtgtttgatgttacctacgtggtttttctctcaagatcttaagagcagctctgtaggattacattattttctgttttttttttcctttgaccttaatgtcatctacttcaataacagcttcatacaaaattcctaccagcacataccacagcagattcaaggccttgttttaaaaatggtgccagcttctcttaatttggaagatatattgtctctcctgaacatgggctaagaaaatgtataatttggtattaacataagagctgaagacactttaaatgcattgtttcatttttataagataaaaaaaattttaagaatcaaaatgttatcaacagacttgtccttcattaaaaagtaaaactgcatttgcctacattttatgaaagtgtccaattatgaacaattttgaaatgtaacttttaaaaatgtaaacagcaaaaatgttgtatttaaaataaatctggaaaggcagaaaaacaaaaaatacccagaagacagagtttttggtgaaagttaagatatttcatctttgaacaacttagaatctttcctgcattttatagtctagttccaggcattaatttgaaataaccttggaatcctaaatctaacacccttcggaacaaagtagcttttctcttctgctttatgagcaaatggactaaatactagggaatggtactgtctgggcctttgaaccaagattgaaagagatgaaatcctatatgatatgtataaacattagagaatccattttgatttaataaaaggttgaatttgttctatatcctgtgagaaaatggttcccttttcctgaaaatgttacctcattccaacaatagaaagttggtttttttccagggtgtggtgttggcgggggacagagttgccatgaatatggcatctatgaagactgctgttatattcatttctcaaaatgcactgtggtaggaaattcagaacgcagtgagagaaaataaatgtttgacttcaaaatataaggccgcatttaaagcagaaggtaaagtatagaacagttgacagtataaattctttatctgcaatcttgcagttccctaaatctctgtaacacatcacttttaaaagcctcagataagtggttctataataatttaccaataattcaacccctcaaaagtcttagcaagttaaaccttataatcttacattttagaaatgacccaacttgatccttttattcttcagaatatctctctcaaattttcatttgtttttcattaattgatgaataatgagacattttaggtacctgagggccgacgagtgggggcgggcaggagggccgagggaggcggaacaggatcgaggcgcgaggcgggagtcgagaaagcgagcggccgaggcgactctcagtgcgcggacgcgggcgcgcgcccgcgctcccttcgtcgactcacggcgagagcccaaccctgctgccgcgcgccaccc

SEQ ID NO: 12755 - RNA, 16016 nt, Homo sapiens
  source 1..16016: mol_type = other RNA
gatctcactttgttgcccaggctggtcttaaactcctggcctcaagtgatccccttgtttcagccccgcaaagtgctgggattacaggtgtgagccaccatgcccgtgcccagccacctcatgagtcttgatggggggcagagaccaacaactccacagaagccagatgcttgctttcccagcctctcttgcagctagggcttgggcatgtgatccaggctcagccaatcagatggcactgactcttggcatgacatgggctaaggaggggctgcagggaatccatttgggctggggtggcagctgcactgggagcgacatcagtttccagagggagcagcagaatctggcatcaggcttggggcgtggtaggtgcaaccagactctgcacccagcagcagtggcagaatgggttctctgtggagagtctgtgtattgctccttccgctgaggccaccagcatctgcctccatgaacccctcagagcctgtgagcaactcaacagccttgaattttttcccttcctgtttgaatgagccagggttgtttcactgcttgaactaagagccgttcctgacatgaaaactaagccacatctttttgacccaaagattctggcatcctaaaatacccatctcattttaagttaaaaataaatccatgtttgagcatctactgtttcagttactgtgctaggtgttacaaagctaactaagagtgacaagtaaataactatcatcaccatgataaacagagaatggaaccctggtttttggaatacagacacaaaatgattaattctgcctggaagcgttttggaacatttcagagaggtagtgagctgggccaagagaagagcatacgcaaggaatggtggcatgaagttgcctggtgtgtcctgagaagaaagatgggctaagaaggactggggtagggcagagaagggggtcactggaggtgaggctgggaaagtgagccaaggctcaaatgcaaactgtctgaacttcattttctgtgcaagcaggagaagccgctgacatgggtttggaagatggactgaagccggagaaaaatggaagcaagaaaccctctcacaagaggccataaccacaaccaagtccatgagattgaaaaggaaggcagatatttgaaaaatatttaaagagatgtgaggggtaggacaggcacagtggctcatgcctgtagtcccagcactttgggaggccgaggtgggcagatccacgaggtcaggagatcaagaccatcctaacatggtaaaaccccatctctactaacaatacaaaaaattagtcaggtgtggtggcacgtgcctgtagtcccagctactcaggaggctgaggcaggagaatcgcttgaacctgggaggcggaggttgcagtgagccgagattgtgccactgcaccctagcctaggcaacagagcaagactctgtctcaaaaaaaataaaaaaaaaaaaaagagagaaagagagagagagatgaggagttgctgcactgctgggtgtggagagccgaggaggattcaaagatggtcctgaagtcccagctggaagaagtaggcggcagcaatgtttttaatactgtaaattcatcacgtagcacaggtttggggtggagaaagaaaaattgcattggcttcagggcatgcccagatctttcctcatcttaggcgtttgctaatacatgcattttctaagctgatgtcttgcgtttaatcactgctccattcaaaagagagaaggaggttgtttcaaacctagttgatatcatttgacttccatgctattcacagggctattttatttgaaacaggtataccacagccttaaattgcaagttaatccaggatgttcctaggttggcagttaggaacatgtaattctttggaagggctaaaagtcagctctttaaattatctccatatgaaccttctctccaccttagggtggatccacttatttagtccactgccagtaccacactagaacccgggtggtcactggactccagaaacaacagtagccctctctctgttctgtctctttttgactatctctattctgttcctgaccctgatttctcctgccaagctcaattttgacagctgacaacggcaagccatggcttcccaaaacattattttcaggtcaacttataaatttcaagaacacatttggctccgcttcctgtggtactaagcctacttcttgacagcatttgcctttgttgtaaatagcaaagttcttctagttggatttttgctaagaagtgtgtggatgtggcatgtgacgacatctttagcttggattctagaaaggcactaccattgtgcatttggctaaaggaaacacattttacccgtgaatgccttctatttacaaatgctcagctagcacacaaagctaagtacaagcaataagtactatcctacaatgttactcatttctgaaagcacaaaatgatgactggtatagctttggagatgttttctggaaacccaataaaggaacagatctttgttattccacacctacaaagtcagaagatgcacagtcttttattcatgtttgaacaagcttccttcttgaacaatcaactataaagtgatgtgattctctactagaccaggaactccttgaggacagaatgagggtctaatccatattctaaatccacaccacctggcacaatacatgttgcatggttagggtcaactaagagttggttgaattaatcaataacacacagcaagagaattcacaaagagaggggagtaatcccccagcctcaatcactcggcaagtggaatcgctgggcactgattccagctctgtctcagtgcttgagacagagctgaatgtaatgtgaacatttcaaatgaacaggaaaactagactcacggataagcagtgtagtcatcaagacaacactgtcttggaggtttttctgaagttaaaaccatgctacataagcaataaattatgaaggctgagcatgtgaataaaatttaatgttgtcataaattttataacaaagttaatctgacacatttaatgacatgcataatcattagtatgcagcactgtaatcagacattgataataagcagttcacaccagtgactgtaagagtctttacttgtgttcagccaagccaactgcttggtatatttttctcccttcttagtcgttagttttccatacctacaataactatcagtggtgatgggcttctctgaccatgtgaataatttaatcctcaatgcacagatacagaaacccttgctgaagacagtgtggagcagagaaggctgtctccactccttccacctgaaacacctctgcagatggatatgggagctctgcctacagcccttggacctaaccacttcagtgtgttccagtgagtgtctggacctcggcctgaaagatttttccgaaactaaagaaaatttctctgacctaaagaccttaacctccaccccagaagctctcaccaaggactacagggaactggtggggaaaatccttatcccttactcctcaaggcacagggcagtaatgctgaggcttgtgcgccacacttgctcccagaggtccccagcgggctacctgcggtggtgaatgacctcctaacacgccccttgacggccttcctttccttgcctcacttctccactctcctaccagcattgcagggttcacatcccaaatataccactggcacttgaatcctggtctccaggtctgtttctggaaaaacccaagtaagacattgccccagtaatggggctagatgtctgaggcttcctcaagtatctacctcgaaagctcttactgctgtacacacatgcacatacacacacgtgcgtacaaccagtcacatctaagcaccccgaataccagcctgttgaaggtagcagagagctgcactataagccaaggctgctcccaagagccgctccatcactgaattggcgccccagcaagatgaaggaatgtaatcattggaaggatggagaatgttctctgaatcactgacaaattggaaggggtggagggcaagagtccacctggtggagagatggaaagagcgagagagcctggaatgataatgccattgcttagaaaaggctgctccagatgccatatctacagaaattgtacagcccaaacatctctgagcaataggtctctggtagtcttgatgtctagaccaacaattcccagttcattcttctcagggaaggagccaggatagtccagagactctcattctgctgttagattgaaagggttaggcacaacagccttggcaaagtcacaagggcaaattcacactaaagtgtaaatgacccacaactcctcttctatttttaggttggggaggtgctttagaacataaggaggaactaaagaatattcctgttacatacaaggcagagaaaagggaaactagtggtgacaagacaaatcatccctttgacatttggctggctctacctattacagctctgggggtgaggtgggaacaaaaagatgctgtgtaaagaagtatcttatgccatccctactgtagtgaggtgcagtttagaggggacactgatcaagcagagacccagagtgtttcgttccaagccagaaacagaaatgtataaaacacagcctttccagcatcagaaatgagtagtggtagtggagaactacccaaaacaggaaagaggaccacgtgaggtagagtgtcaaggccctacattccagtgcctctgctcatgactgtaattttgggtaggtcacttaaagtctctggacctcagttttgccatctgtgaaatagggataatactatccagcataaaattggttatgaggctcatgtagggcctgcctgggatgatgtgttgctaatggttaagaacacaacttctggggtctgactggacaggctgaaatccctgcttaacacgttccagcagagccctgggcgatctatttaacttttgttttctcacctgtaagctgagacgaaagtacccactttataagattattccaataattagttgaaataatgcatgcagagaattaagcatggtacttgttatttgttaaactagctattaaaatgtgtaaaatataaagtattgtatggattttaggacaatgcaaagactctttgcttgctgcaatagttcggggccctttcagatggctaaaggcagaatttgtatgtgtaaatatggtgtgcttgtctctgctctggatactgagggcttaccctgttattaaacttatttagtaaatattgaactgtcatgaggcctaacatttagttccagttattagataaaacatttgctttgaatggtatttgaattgccaggttctagattattctggttgacaaactcttcgtattttataaagaggctaaaattggtaagctatcacagaacagatgtgccattttcaaggtatattaaaccatgattcactgtaacattgttcctactggcaacaaattcagagcaggctggactttatttggtgaagaaacattgagtggaagagaaatgacattattttatgtatttacattttcaaattactgtggcttaaacctgttcagccaacattacccaccttcagtctgctaaataaatgattcagtacatttctaatttacagaattttttaacaaaagaaaatgtaatttgatagccaaatcaacgttaaacattatacatttaaaaaaccacaggcaaagacacaaacatgatgacactaacttttgttaaagtatgcttacctatggtttcctctgaggcacgttctttcatgctaagcttccaacataatatgaaaatgaaggagatgcattttgcaaagcaaaacagaccttaagcaaaatattatacttctcaaattaacactgttacaaagttttagaatttaataagttcattaatttaaaagtttggatgtctgagtccttctatcccaaaacaagatcttggagggtcttccacagccatgtaataccatggtcacatgaccctttccaaaattattaatctgaatttactatatgaggataaatctatctttttgaaaatatttaggaaaatgagcttggtatttataaaatgaagctctctttgggtggtatcctaagacacgtcaagccaatcagcctgtaactgtgaaaaaaacattggtaggtacaaaagtggggtgggagaggagtgacttaactttgttaagtgatgggaaagaaacactaatagcattatctcaataaaatgtgatttaaaaaaatttaaaatactaaatcattgaactgacaaagaaatataaatcattcagaaataaactcattaggtcatcaaatcctgttaaatctgcaattaggaagagcaaggtgtacaatccatacatttaaactcacaggctcactttgcacaacgtcaatttactccttaatatgttattaatacgcattttccaaaaggatgtattagtaaatggtacacatctacttcttggcaacatcatataacctggtacaacataagcattcttcttatagttaagaaatgtggatggtatcaaaattagaaaaataaatgccctattatgttgtggtcaggtttaaggcatgtgaattttatcttcatacaaaagattaaaatctagatattaaaaagtagtgcagtatcagtgatgctgcctcagttcccaaaatgtcacatcacaaaaatatcccataattgcctgtagtttattccttggctttcctcttttctctctgcatctttgtaacaattttttaaaagtggaaatataattgttggcaatgctaacagctgtagaaatgattacaagatgtggaaaagcataacaggaatgtcaagaatctgtttctggcagtaatatatatggaacattgttcaggacaaaagaggagaaggaagaaaaaaaggagaggggtttatcatctctaagaattttcaaactaaacctcattgcttaataggaaaaaaagattccatatttaaagttaagtcacctctaactactagctaaagcatgacatcaccagcactggagtcagcggaagtgtgtttttgaaggacagtgttgcaggagaatctggacaggttttagagccaggagagagaaaataattctacctctgacagttgaaggaccttaggcaaatcagtttacctctgctagactacactccaaaatttggacattcaaaaatttgatattaataaccacatgaaagtctcgtgttgaggtgaatatgtatttgttggtgaaagatatgttggtttttaaacagacagcactctgcaattgtaggctattgttttgttttgccagttgtcaaattctatccagctatacacacttgtgtggcctcctaatggtgtttttccagtggctaaaggtttatgaataagacacttttcctaatggaattaacccgatgcttttcttaaacatgtaaccttgagttcaccgcaaaaaacaatgcttcgattagagcaatgcatataataaaggttaccctcgtttcttagacactagacatcattcacaaaaagagaactgcttttgaaagggatgtatttgcactggaaagaatagttttctacttctaattataaatgatttattggtgaaagcaaaacaacagcctgtctgagaggcacttctatgagcatcctcacgtgtgatttgcaaggttgaagaagagggaaaaatgcctcaattgtaccaatggtgagaaaacacccaaagtacaaagcaggtttcaaaaaaaccatactcataaccaaggacaataataaagcaatgtgttgacatatactctataagtcttcctccataaatagtttatagaaattttgtaatttctgtaaatgcatcctataataattttgcatcttgctttttttttacatttaatatcaagtagatttctaaagggcaattatttgaaaattatcccaaatacatggggaaatatacatcaagtgaaaaaatgcagtgggtgatagagatatcaggaagcgcctcaaatatttctcatctcgttggagaaaaacaaacatgttctcatttagaatgagtgggagttacctaattgatttaggcctctatatttaacttctagtcaaaaaaggtagttctatctagcaacaatattatggggaacaaaagaaaaaattaactctctaaatttgcagtagggtcttttcttcagaagtaccaaatcccatctattaccagctccatgcttcaggcctaaaatggatctccctgaagcaatgacagaatttttgccaagtgactaggatataaacaccactttggttgcacagtgagacatatgctccaaagaaaactggttcaaaaacaggcaagtgggtttctacagaataaatgagagccctgtcaatggcttcatcttcagggctttgtgtctgtgcttgcgtggtggctcttgtttcatctatggataatggtggcacacagttttcataattccttacattaatgaactgctataaatttgtttttggtattctagagagtcctaacttcagcttctgggcaatgctgaggaggcaccctatattctagacttaccttttgcaaggtgtactctcagcattgtgggcgatttccatgggagaatattctatttaaagaactactgtcccagcataaaacaaaaaatcatttatgaagatgcaggagactcggaaagctctcaattattgtttgcacaagcacaatgtcacagcctcctttccccattccacaagggggtcaggaagagagtactcagctgtgagaaaagacatacagaagaattcatgtggtcatgagagcgaggacatggccgatcccccaaggaggatgtgtcatacacttcatgagcccaagagtgtgctgtagggtctgaagggcaagatgctggttcactgatgtaaaggagagggaaaaaagcttcaaccaactagaaaaacagtctctatgcatgctatttttgattttaaacacaggtatcaattccttctctcagagagtccattttaaaataggatacatttttaaaggaatatttaaaggacacattcattaaaatttattttaaaaacttttcaaaagaaacaaaaggtatgaattttatttaatccttgaggaaatggttcttttctcacacacataaatcactcattttgtttttctttatctcctttattaatctacattagaaaaataaacttttcatacactaagaacaaggaaaccactctcaattgacaaaatgttccaatccaacacaatgattactttcacctttaatttacaggcagccagattcaaaatccttaaagttgcttaaacttaaaaatgacaatgacaacctaaaaggtataatgttgattggaacagacatttaattggaaaattgatgattttccatttccaattaaatctctagatagaaatgaaaaaaattaaaaatcgtatttaagaaaagccaaatcttgggttgtgaggtatctttttaaggatgtttcagcagaaaaaaacaaaggctctcacaattgtgtagctgcctagattaagtgggtatcctgatcaaggagatgggggatgatttggctttagtattccaatgataaagtttataatgagaataacatgttgctacaaaatccagtctcttcctcagatgccttccacagagggcaggaagctttgtcagttttgtttgctgatgatgcctggttccgtcaacaaataacacctgtcacacggtgggtagtcaatatacatttgttgaataaatatgaaaaaaagaaatgtacaatatgtttgtgaagccaactgtgtgtgcattgctattgaggtacacaaaaagtctttgttttaaatttgagaatgaggactttcaatggaatatatctataaaaatgaaaaaaagacattactgtctggacttttgtacagcaagagaagaaaaaccactagccaagagccaactcacctgataggcctggatcaagcatgcagctgtggagaacacccctgggactctaactctggcactctgcaagctgggtacttgggcaggacagcagcagcactcatgaactgggcagcacctgttggtgagggctgatcacatggattctctcatcccagccttacaatcagtccttcaggtacatactttttctgactttgctgatgaggaaactatgcacagaggttacacagcttaacaaagggttctcacctaatgaacaatgaaatgggattttagcctttctttgcatctggtcttagagccaatacccaagaagcactgtactgtatgcattgtctcagagaaacttactcttcctgggcctcagtctttaaaaggtgggcagttgacttaataagaattaaagatcaatgattaaggttcaaggcactccaaaattctggtctttattgaaaaggctacagaagtctcaccttaataataccctatagacttgatattcttggttaattaaatattggaaaccaatttcatagtaattgaggtcagaaaaaagtactcatgacattttagaatatgatgacaaagccatagataaatttcaatgcacctgtaattacttaaaactgttatagcatgcaatgtgttaccacaacagccagagaaatactaatttactcagcctattcttctagaccagtaaacactaggattaaatagatattttcattgaatttgttctacccttcattgccatttatagatagcttacttgtcatagattactttctaattgttttatgtttcctaactagcctgcaatactttggcaaggacctcaaacaatagtagacagtaggtgtaaaatagatggctacattgaacagatgactaaaaggatgcctcctaagtacctatatcttgaaatatatattattgtgccttgctttcaatttgtgattttaaaatctagaaatcacctgttttatgtaataacaataaaatccttctttgttgaaaacatgcacaaataaagtttacaagctcaaaaaattaaacagcagtaacggtcaagctttccaacaataaaatacattttggtaaggttttcattttacaaaaactcaaaatagctttatgagttcacaaaataatatgatatttttcaagatattaacatattcttataccggaagagcatagaataaaatttacttggagattgagcatttgcttctttaagaaatacttcttttagtatttttactttaatattatgaaagctacataattacattcagattcattaactactccagtagttaatttttaaaacttatgatgaatagttttgtttaaaatatataacattggtaatatgcaaatctgaatctgtaataaagaaggatttgcattcctgatttttttttctgatacaaccaatgacaaaataactaatggttccacagaggataaaatgtctcaaatctgttggttctgaaggtgaagcgagatttttgtactgataccgtgtatcactgagataccaggaggaaatggaattaaactcagatagttcaaatggagagattttaatgaagggacgacctacagaggtgtcggcagggttggggggaatcagcgagatatgcttagaacccaccgactggcaaacctccccctgaagatggagaaggaggaaggagtgttactggaatgagagcttgagtccaggggaggaggatgggctgctgaggaggcgacaccatcctgaaagaagaatcctctgccagaggcttttcagggtcatttcttcacactctctgcagggaagcacggagacagcaggaagaaatatcctaacctcactctcttccctctacaggtgcttccattggccaaatccacccagaggccagttggtggcgatcagctctcttcaagtggtatttaaatttcttctttcattttccttctggtaacaaagaagtctgtggctcaaaagatgtttctctaagaccccatcctattaggtctctgagctgtgggaagtatttatacaattgcttgtgaatataagatccaggaatttccctaagatccctaacaaaattggtgataagtagtcccacatgttaatccagccacccacggatgacagcacttaccatttctttgataaatgtcaaatgcatttgaagtacctacctgaaatatttgtttaaatgctatctaatctattaattttatatatgtgtgagtctgttttgtataccttctgattataggataaatgtaaataaatccaaagagtaatcaaagctaccactttcaagaagccttctttgtagaaccggaagagtcttaaataggcttttcaggtatgcatctcttattatcgctgaactccaagtcctgcaaggcaggcatcatgtgtgggtcacctttacagtaggcacaggccttaaaacagtgacatgcacattgcaggcactccataaatgtttgctgaattggctaaaccttggtttgttcccataatcaaccaccacaaacagcacacagataattacttcttggaaagattccaactagtgtttgatgttacctacgtggtttttctctcaagatcttaagagcagctctgtaggattacattattttctgttttttttttcctttgaccttaatgtcatctacttcaataacagcttcatacaaaattcctaccagcacataccacagcagattcaaggccttgttttaaaaatggtgccagcttctcttaatttggaagatatattgtctctcctgaacatgggctaagaaaatgtataatttggtattaacataagagctgaagacactttaaatgcattgtttcatttttataagataaaaaaaattttaagaatcaaaatgttatcaacagacttgtccttcattaaaaagtaaaactgcatttgcctacattttatgaaagtgtccaattatgaacaattttgaaatgtaacttttaaaaatgtaaacagcaaaaatgttgtatttaaaataaatctggaaaggcagaaaaacaaaaaatacccagaagacagagtttttggtgaaagttaagatatttcatctttgaacaacttagaatctttcctgcattttatagtctagttccaggcattaatttgaaataaccttggaatcctaaatctaacacccttcggaacaaagtagcttttctcttctgctttatgagcaaatggactaaatactagggaatggtactgtctgggcctttgaaccaagattgaaagagatgaaatcctatatgatatgtataaacattagagaatccattttgatttaataaaaggttgaatttgttctatatcctgtgagaaaatggttcccttttcctgaaaatgttacctcattccaacaatagaaagttggtttttttccagggtgtggtgttggcgggggacagagttgccatgaatatggcatctatgaagactgctgttatattcatttctcaaaatgcactgtggtaggaaattcagaacgcagtgagagaaaataaatgtttgacttcaaaatataaggccgcatttaaagcagaaggtaaagtatagaacagttgacagtataaattctttatctgcaatcttgcagttccctaaatctctgtaacacatcacttttaaaagcctcagataagtggttctataataatttaccaataattcaacccctcaaaagtcttagcaagttaaaccttataatcttacattttagaaatgacccaacttgatccttttattcttcagaatatctctctcaaattttcatttgtttttcattaattgatgaataatgagacattttaggtacctgtccacaaagaaatgaaattttcactttccaggaacctaacaaatgaaaagatagaaatcaattccaacagaatattaccaaagaaatcttttagaatggactgttaaaattatttatttgtatttatctggctctactatttgtggtacatttccacttcaaagctaaacctcaaataacatcatagtgagtggttgacttcatgtttaactgagatcttgaagactgaaaaagaccacgacaaacacacatctattttcttggctactgcatccgtgttcatcaccattctgatagtctgcaatgtattgcagctcaccctttgggaaggactaaagtagacatctgtttgttctgcttactcagcattcctaccctaattttcctttggagaacccctttattctagaccacgtgaagctaatgccaaaccccattccaggggatgcacctgaatccaacctccatcatctaaacagtgccttctccacgttcagagaagagcaagtgactcaaactgccctcataagaacagacctgggacttctgctgcaaatattgaagagtaagtactcttttttcttgctaggactaagctggtagtaccttctatgaggctatcatatggaaacaacttgtctgaaaatgaagccacaactagaaaacagatcctggtaacccggattgatggatccagccctaccttaaatggcaagacctaacccgaggctttttgcatcaaccaataaagtccttaagccagtttgagttggttttgtcacttgcagctaaaagaattctgactctaacaatgtgacaatagcaaaaataaacataactgcttttgaggtttctaatggattttcctccctatatacatgatttcatttaatcctcacaattcaggaaagcacatatctattaacattaaattaatattcattattttgaacacatgctatgtggataagggatgaggaaagccaaggaagtaatcaacgtgaaatctcacttatatgggagggaagtggaggttacatatctcagggcacttaacagatatcatcaaatgaaagaataaacagtgtgtgggagaggcagtaggtgattcttcatcaattcctggatgaaaaattaggagataatgaactccgaacaggcagcctaatgagaatggctcaagcaacaggacatagagagggagttaggttagacatggggttcttgggaattttcacctcgtgggggggcgggggggtcgtgcagctgttgtcagtgggaaagggaaaaaggaaaaggctgagtttggaaggcagggagggaggagacaatgtgagtcagtgaaaaagggcccttagaatgacaagtctggaccagagagaggctaagactgaaaatacaagttgggtaaccactggcatacagatggcagttcaggcttgggcactgcccaccagagcctcagcatgaagagaagagggggaggctggccaccacctccctctaggtaatcgtcatcctgatgctgagctcctgaaaacaggctctttcactcgccccatctcttgctcttgattgcaacccggcattcaggaggcaccctgtaatatctgtggagtgaccgacaacacagcgccagggcactgagaagatcccagggcgccagggactggttctacaagggtgcccctcccggtcccctccagcgcgccgccagagctgccagtcttggctgctacacgggaggcagcctcattatgcagctctcacctcttaaattagttcatgctctcacattaggtgtaatcacagcttgcaacgctttctggggatgtctcagaaagatctgagggccgacgagtgggggcgggcaggagggccgagggaggcggaacaggatcgaggcgcgaggcgggagtcgagaaagcgagcggccgaggcgactctcagtgcgcggacgcgggcgcgcgcccgcgctcccttcgtcgactcacggcgagagcccaaccctgctgccgcgcgccaccc

SEQ ID NO: 12756 - RNA, 17016 nt, Homo sapiens
  source 1..17016: mol_type = other RNA
gatctcactttgttgcccaggctggtcttaaactcctggcctcaagtgatccccttgtttcagccccgcaaagtgctgggattacaggtgtgagccaccatgcccgtgcccagccacctcatgagtcttgatggggggcagagaccaacaactccacagaagccagatgcttgctttcccagcctctcttgcagctagggcttgggcatgtgatccaggctcagccaatcagatggcactgactcttggcatgacatgggctaaggaggggctgcagggaatccatttgggctggggtggcagctgcactgggagcgacatcagtttccagagggagcagcagaatctggcatcaggcttggggcgtggtaggtgcaaccagactctgcacccagcagcagtggcagaatgggttctctgtggagagtctgtgtattgctccttccgctgaggccaccagcatctgcctccatgaacccctcagagcctgtgagcaactcaacagccttgaattttttcccttcctgtttgaatgagccagggttgtttcactgcttgaactaagagccgttcctgacatgaaaactaagccacatctttttgacccaaagattctggcatcctaaaatacccatctcattttaagttaaaaataaatccatgtttgagcatctactgtttcagttactgtgctaggtgttacaaagctaactaagagtgacaagtaaataactatcatcaccatgataaacagagaatggaaccctggtttttggaatacagacacaaaatgattaattctgcctggaagcgttttggaacatttcagagaggtagtgagctgggccaagagaagagcatacgcaaggaatggtggcatgaagttgcctggtgtgtcctgagaagaaagatgggctaagaaggactggggtagggcagagaagggggtcactggaggtgaggctgggaaagtgagccaaggctcaaatgcaaactgtctgaacttcattttctgtgcaagcaggagaagccgctgacatgggtttggaagatggactgaagccggagaaaaatggaagcaagaaaccctctcacaagaggccataaccacaaccaagtccatgagattgaaaaggaaggcagatatttgaaaaatatttaaagagatgtgaggggtaggacaggcacagtggctcatgcctgtagtcccagcactttgggaggccgaggtgggcagatccacgaggtcaggagatcaagaccatcctaacatggtaaaaccccatctctactaacaatacaaaaaattagtcaggtgtggtggcacgtgcctgtagtcccagctactcaggaggctgaggcaggagaatcgcttgaacctgggaggcggaggttgcagtgagccgagattgtgccactgcaccctagcctaggcaacagagcaagactctgtctcaaaaaaaataaaaaaaaaaaaaagagagaaagagagagagagatgaggagttgctgcactgctgggtgtggagagccgaggaggattcaaagatggtcctgaagtcccagctggaagaagtaggcggcagcaatgtttttaatactgtaaattcatcacgtagcacaggtttggggtggagaaagaaaaattgcattggcttcagggcatgcccagatctttcctcatcttaggcgtttgctaatacatgcattttctaagctgatgtcttgcgtttaatcactgctccattcaaaagagagaaggaggttgtttcaaacctagttgatatcatttgacttccatgctattcacagggctattttatttgaaacaggtataccacagccttaaattgcaagttaatccaggatgttcctaggttggcagttaggaacatgtaattctttggaagggctaaaagtcagctctttaaattatctccatatgaaccttctctccaccttagggtggatccacttatttagtccactgccagtaccacactagaacccgggtggtcactggactccagaaacaacagtagccctctctctgttctgtctctttttgactatctctattctgttcctgaccctgatttctcctgccaagctcaattttgacagctgacaacggcaagccatggcttcccaaaacattattttcaggtcaacttataaatttcaagaacacatttggctccgcttcctgtggtactaagcctacttcttgacagcatttgcctttgttgtaaatagcaaagttcttctagttggatttttgctaagaagtgtgtggatgtggcatgtgacgacatctttagcttggattctagaaaggcactaccattgtgcatttggctaaaggaaacacattttacccgtgaatgccttctatttacaaatgctcagctagcacacaaagctaagtacaagcaataagtactatcctacaatgttactcatttctgaaagcacaaaatgatgactggtatagctttggagatgttttctggaaacccaataaaggaacagatctttgttattccacacctacaaagtcagaagatgcacagtcttttattcatgtttgaacaagcttccttcttgaacaatcaactataaagtgatgtgattctctactagaccaggaactccttgaggacagaatgagggtctaatccatattctaaatccacaccacctggcacaatacatgttgcatggttagggtcaactaagagttggttgaattaatcaataacacacagcaagagaattcacaaagagaggggagtaatcccccagcctcaatcactcggcaagtggaatcgctgggcactgattccagctctgtctcagtgcttgagacagagctgaatgtaatgtgaacatttcaaatgaacaggaaaactagactcacggataagcagtgtagtcatcaagacaacactgtcttggaggtttttctgaagttaaaaccatgctacataagcaataaattatgaaggctgagcatgtgaataaaatttaatgttgtcataaattttataacaaagttaatctgacacatttaatgacatgcataatcattagtatgcagcactgtaatcagacattgataataagcagttcacaccagtgactgtaagagtctttacttgtgttcagccaagccaactgcttggtatatttttctcccttcttagtcgttagttttccatacctacaataactatcagtggtgatgggcttctctgaccatgtgaataatttaatcctcaatgcacagatacagaaacccttgctgaagacagtgtggagcagagaaggctgtctccactccttccacctgaaacacctctgcagatggatatgggagctctgcctacagcccttggacctaaccacttcagtgtgttccagtgagtgtctggacctcggcctgaaagatttttccgaaactaaagaaaatttctctgacctaaagaccttaacctccaccccagaagctctcaccaaggactacagggaactggtggggaaaatccttatcccttactcctcaaggcacagggcagtaatgctgaggcttgtgcgccacacttgctcccagaggtccccagcgggctacctgcggtggtgaatgacctcctaacacgccccttgacggccttcctttccttgcctcacttctccactctcctaccagcattgcagggttcacatcccaaatataccactggcacttgaatcctggtctccaggtctgtttctggaaaaacccaagtaagacattgccccagtaatggggctagatgtctgaggcttcctcaagtatctacctcgaaagctcttactgctgtacacacatgcacatacacacacgtgcgtacaaccagtcacatctaagcaccccgaataccagcctgttgaaggtagcagagagctgcactataagccaaggctgctcccaagagccgctccatcactgaattggcgccccagcaagatgaaggaatgtaatcattggaaggatggagaatgttctctgaatcactgacaaattggaaggggtggagggcaagagtccacctggtggagagatggaaagagcgagagagcctggaatgataatgccattgcttagaaaaggctgctccagatgccatatctacagaaattgtacagcccaaacatctctgagcaataggtctctggtagtcttgatgtctagaccaacaattcccagttcattcttctcagggaaggagccaggatagtccagagactctcattctgctgttagattgaaagggttaggcacaacagccttggcaaagtcacaagggcaaattcacactaaagtgtaaatgacccacaactcctcttctatttttaggttggggaggtgctttagaacataaggaggaactaaagaatattcctgttacatacaaggcagagaaaagggaaactagtggtgacaagacaaatcatccctttgacatttggctggctctacctattacagctctgggggtgaggtgggaacaaaaagatgctgtgtaaagaagtatcttatgccatccctactgtagtgaggtgcagtttagaggggacactgatcaagcagagacccagagtgtttcgttccaagccagaaacagaaatgtataaaacacagcctttccagcatcagaaatgagtagtggtagtggagaactacccaaaacaggaaagaggaccacgtgaggtagagtgtcaaggccctacattccagtgcctctgctcatgactgtaattttgggtaggtcacttaaagtctctggacctcagttttgccatctgtgaaatagggataatactatccagcataaaattggttatgaggctcatgtagggcctgcctgggatgatgtgttgctaatggttaagaacacaacttctggggtctgactggacaggctgaaatccctgcttaacacgttccagcagagccctgggcgatctatttaacttttgttttctcacctgtaagctgagacgaaagtacccactttataagattattccaataattagttgaaataatgcatgcagagaattaagcatggtacttgttatttgttaaactagctattaaaatgtgtaaaatataaagtattgtatggattttaggacaatgcaaagactctttgcttgctgcaatagttcggggccctttcagatggctaaaggcagaatttgtatgtgtaaatatggtgtgcttgtctctgctctggatactgagggcttaccctgttattaaacttatttagtaaatattgaactgtcatgaggcctaacatttagttccagttattagataaaacatttgctttgaatggtatttgaattgccaggttctagattattctggttgacaaactcttcgtattttataaagaggctaaaattggtaagctatcacagaacagatgtgccattttcaaggtatattaaaccatgattcactgtaacattgttcctactggcaacaaattcagagcaggctggactttatttggtgaagaaacattgagtggaagagaaatgacattattttatgtatttacattttcaaattactgtggcttaaacctgttcagccaacattacccaccttcagtctgctaaataaatgattcagtacatttctaatttacagaattttttaacaaaagaaaatgtaatttgatagccaaatcaacgttaaacattatacatttaaaaaaccacaggcaaagacacaaacatgatgacactaacttttgttaaagtatgcttacctatggtttcctctgaggcacgttctttcatgctaagcttccaacataatatgaaaatgaaggagatgcattttgcaaagcaaaacagaccttaagcaaaatattatacttctcaaattaacactgttacaaagttttagaatttaataagttcattaatttaaaagtttggatgtctgagtccttctatcccaaaacaagatcttggagggtcttccacagccatgtaataccatggtcacatgaccctttccaaaattattaatctgaatttactatatgaggataaatctatctttttgaaaatatttaggaaaatgagcttggtatttataaaatgaagctctctttgggtggtatcctaagacacgtcaagccaatcagcctgtaactgtgaaaaaaacattggtaggtacaaaagtggggtgggagaggagtgacttaactttgttaagtgatgggaaagaaacactaatagcattatctcaataaaatgtgatttaaaaaaatttaaaatactaaatcattgaactgacaaagaaatataaatcattcagaaataaactcattaggtcatcaaatcctgttaaatctgcaattaggaagagcaaggtgtacaatccatacatttaaactcacaggctcactttgcacaacgtcaatttactccttaatatgttattaatacgcattttccaaaaggatgtattagtaaatggtacacatctacttcttggcaacatcatataacctggtacaacataagcattcttcttatagttaagaaatgtggatggtatcaaaattagaaaaataaatgccctattatgttgtggtcaggtttaaggcatgtgaattttatcttcatacaaaagattaaaatctagatattaaaaagtagtgcagtatcagtgatgctgcctcagttcccaaaatgtcacatcacaaaaatatcccataattgcctgtagtttattccttggctttcctcttttctctctgcatctttgtaacaattttttaaaagtggaaatataattgttggcaatgctaacagctgtagaaatgattacaagatgtggaaaagcataacaggaatgtcaagaatctgtttctggcagtaatatatatggaacattgttcaggacaaaagaggagaaggaagaaaaaaaggagaggggtttatcatctctaagaattttcaaactaaacctcattgcttaataggaaaaaaagattccatatttaaagttaagtcacctctaactactagctaaagcatgacatcaccagcactggagtcagcggaagtgtgtttttgaaggacagtgttgcaggagaatctggacaggttttagagccaggagagagaaaataattctacctctgacagttgaaggaccttaggcaaatcagtttacctctgctagactacactccaaaatttggacattcaaaaatttgatattaataaccacatgaaagtctcgtgttgaggtgaatatgtatttgttggtgaaagatatgttggtttttaaacagacagcactctgcaattgtaggctattgttttgttttgccagttgtcaaattctatccagctatacacacttgtgtggcctcctaatggtgtttttccagtggctaaaggtttatgaataagacacttttcctaatggaattaacccgatgcttttcttaaacatgtaaccttgagttcaccgcaaaaaacaatgcttcgattagagcaatgcatataataaaggttaccctcgtttcttagacactagacatcattcacaaaaagagaactgcttttgaaagggatgtatttgcactggaaagaatagttttctacttctaattataaatgatttattggtgaaagcaaaacaacagcctgtctgagaggcacttctatgagcatcctcacgtgtgatttgcaaggttgaagaagagggaaaaatgcctcaattgtaccaatggtgagaaaacacccaaagtacaaagcaggtttcaaaaaaaccatactcataaccaaggacaataataaagcaatgtgttgacatatactctataagtcttcctccataaatagtttatagaaattttgtaatttctgtaaatgcatcctataataattttgcatcttgctttttttttacatttaatatcaagtagatttctaaagggcaattatttgaaaattatcccaaatacatggggaaatatacatcaagtgaaaaaatgcagtgggtgatagagatatcaggaagcgcctcaaatatttctcatctcgttggagaaaaacaaacatgttctcatttagaatgagtgggagttacctaattgatttaggcctctatatttaacttctagtcaaaaaaggtagttctatctagcaacaatattatggggaacaaaagaaaaaattaactctctaaatttgcagtagggtcttttcttcagaagtaccaaatcccatctattaccagctccatgcttcaggcctaaaatggatctccctgaagcaatgacagaatttttgccaagtgactaggatataaacaccactttggttgcacagtgagacatatgctccaaagaaaactggttcaaaaacaggcaagtgggtttctacagaataaatgagagccctgtcaatggcttcatcttcagggctttgtgtctgtgcttgcgtggtggctcttgtttcatctatggataatggtggcacacagttttcataattccttacattaatgaactgctataaatttgtttttggtattctagagagtcctaacttcagcttctgggcaatgctgaggaggcaccctatattctagacttaccttttgcaaggtgtactctcagcattgtgggcgatttccatgggagaatattctatttaaagaactactgtcccagcataaaacaaaaaatcatttatgaagatgcaggagactcggaaagctctcaattattgtttgcacaagcacaatgtcacagcctcctttccccattccacaagggggtcaggaagagagtactcagctgtgagaaaagacatacagaagaattcatgtggtcatgagagcgaggacatggccgatcccccaaggaggatgtgtcatacacttcatgagcccaagagtgtgctgtagggtctgaagggcaagatgctggttcactgatgtaaaggagagggaaaaaagcttcaaccaactagaaaaacagtctctatgcatgctatttttgattttaaacacaggtatcaattccttctctcagagagtccattttaaaataggatacatttttaaaggaatatttaaaggacacattcattaaaatttattttaaaaacttttcaaaagaaacaaaaggtatgaattttatttaatccttgaggaaatggttcttttctcacacacataaatcactcattttgtttttctttatctcctttattaatctacattagaaaaataaacttttcatacactaagaacaaggaaaccactctcaattgacaaaatgttccaatccaacacaatgattactttcacctttaatttacaggcagccagattcaaaatccttaaagttgcttaaacttaaaaatgacaatgacaacctaaaaggtataatgttgattggaacagacatttaattggaaaattgatgattttccatttccaattaaatctctagatagaaatgaaaaaaattaaaaatcgtatttaagaaaagccaaatcttgggttgtgaggtatctttttaaggatgtttcagcagaaaaaaacaaaggctctcacaattgtgtagctgcctagattaagtgggtatcctgatcaaggagatgggggatgatttggctttagtattccaatgataaagtttataatgagaataacatgttgctacaaaatccagtctcttcctcagatgccttccacagagggcaggaagctttgtcagttttgtttgctgatgatgcctggttccgtcaacaaataacacctgtcacacggtgggtagtcaatatacatttgttgaataaatatgaaaaaaagaaatgtacaatatgtttgtgaagccaactgtgtgtgcattgctattgaggtacacaaaaagtctttgttttaaatttgagaatgaggactttcaatggaatatatctataaaaatgaaaaaaagacattactgtctggacttttgtacagcaagagaagaaaaaccactagccaagagccaactcacctgataggcctggatcaagcatgcagctgtggagaacacccctgggactctaactctggcactctgcaagctgggtacttgggcaggacagcagcagcactcatgaactgggcagcacctgttggtgagggctgatcacatggattctctcatcccagccttacaatcagtccttcaggtacatactttttctgactttgctgatgaggaaactatgcacagaggttacacagcttaacaaagggttctcacctaatgaacaatgaaatgggattttagcctttctttgcatctggtcttagagccaatacccaagaagcactgtactgtatgcattgtctcagagaaacttactcttcctgggcctcagtctttaaaaggtgggcagttgacttaataagaattaaagatcaatgattaaggttcaaggcactccaaaattctggtctttattgaaaaggctacagaagtctcaccttaataataccctatagacttgatattcttggttaattaaatattggaaaccaatttcatagtaattgaggtcagaaaaaagtactcatgacattttagaatatgatgacaaagccatagataaatttcaatgcacctgtaattacttaaaactgttatagcatgcaatgtgttaccacaacagccagagaaatactaatttactcagcctattcttctagaccagtaaacactaggattaaatagatattttcattgaatttgttctacccttcattgccatttatagatagcttacttgtcatagattactttctaattgttttatgtttcctaactagcctgcaatactttggcaaggacctcaaacaatagtagacagtaggtgtaaaatagatggctacattgaacagatgactaaaaggatgcctcctaagtacctatatcttgaaatatatattattgtgccttgctttcaatttgtgattttaaaatctagaaatcacctgttttatgtaataacaataaaatccttctttgttgaaaacatgcacaaataaagtttacaagctcaaaaaattaaacagcagtaacggtcaagctttccaacaataaaatacattttggtaaggttttcattttacaaaaactcaaaatagctttatgagttcacaaaataatatgatatttttcaagatattaacatattcttataccggaagagcatagaataaaatttacttggagattgagcatttgcttctttaagaaatacttcttttagtatttttactttaatattatgaaagctacataattacattcagattcattaactactccagtagttaatttttaaaacttatgatgaatagttttgtttaaaatatataacattggtaatatgcaaatctgaatctgtaataaagaaggatttgcattcctgatttttttttctgatacaaccaatgacaaaataactaatggttccacagaggataaaatgtctcaaatctgttggttctgaaggtgaagcgagatttttgtactgataccgtgtatcactgagataccaggaggaaatggaattaaactcagatagttcaaatggagagattttaatgaagggacgacctacagaggtgtcggcagggttggggggaatcagcgagatatgcttagaacccaccgactggcaaacctccccctgaagatggagaaggaggaaggagtgttactggaatgagagcttgagtccaggggaggaggatgggctgctgaggaggcgacaccatcctgaaagaagaatcctctgccagaggcttttcagggtcatttcttcacactctctgcagggaagcacggagacagcaggaagaaatatcctaacctcactctcttccctctacaggtgcttccattggccaaatccacccagaggccagttggtggcgatcagctctcttcaagtggtatttaaatttcttctttcattttccttctggtaacaaagaagtctgtggctcaaaagatgtttctctaagaccccatcctattaggtctctgagctgtgggaagtatttatacaattgcttgtgaatataagatccaggaatttccctaagatccctaacaaaattggtgataagtagtcccacatgttaatccagccacccacggatgacagcacttaccatttctttgataaatgtcaaatgcatttgaagtacctacctgaaatatttgtttaaatgctatctaatctattaattttatatatgtgtgagtctgttttgtataccttctgattataggataaatgtaaataaatccaaagagtaatcaaagctaccactttcaagaagccttctttgtagaaccggaagagtcttaaataggcttttcaggtatgcatctcttattatcgctgaactccaagtcctgcaaggcaggcatcatgtgtgggtcacctttacagtaggcacaggccttaaaacagtgacatgcacattgcaggcactccataaatgtttgctgaattggctaaaccttggtttgttcccataatcaaccaccacaaacagcacacagataattacttcttggaaagattccaactagtgtttgatgttacctacgtggtttttctctcaagatcttaagagcagctctgtaggattacattattttctgttttttttttcctttgaccttaatgtcatctacttcaataacagcttcatacaaaattcctaccagcacataccacagcagattcaaggccttgttttaaaaatggtgccagcttctcttaatttggaagatatattgtctctcctgaacatgggctaagaaaatgtataatttggtattaacataagagctgaagacactttaaatgcattgtttcatttttataagataaaaaaaattttaagaatcaaaatgttatcaacagacttgtccttcattaaaaagtaaaactgcatttgcctacattttatgaaagtgtccaattatgaacaattttgaaatgtaacttttaaaaatgtaaacagcaaaaatgttgtatttaaaataaatctggaaaggcagaaaaacaaaaaatacccagaagacagagtttttggtgaaagttaagatatttcatctttgaacaacttagaatctttcctgcattttatagtctagttccaggcattaatttgaaataaccttggaatcctaaatctaacacccttcggaacaaagtagcttttctcttctgctttatgagcaaatggactaaatactagggaatggtactgtctgggcctttgaaccaagattgaaagagatgaaatcctatatgatatgtataaacattagagaatccattttgatttaataaaaggttgaatttgttctatatcctgtgagaaaatggttcccttttcctgaaaatgttacctcattccaacaatagaaagttggtttttttccagggtgtggtgttggcgggggacagagttgccatgaatatggcatctatgaagactgctgttatattcatttctcaaaatgcactgtggtaggaaattcagaacgcagtgagagaaaataaatgtttgacttcaaaatataaggccgcatttaaagcagaaggtaaagtatagaacagttgacagtataaattctttatctgcaatcttgcagttccctaaatctctgtaacacatcacttttaaaagcctcagataagtggttctataataatttaccaataattcaacccctcaaaagtcttagcaagttaaaccttataatcttacattttagaaatgacccaacttgatccttttattcttcagaatatctctctcaaattttcatttgtttttcattaattgatgaataatgagacattttaggtacctgtccacaaagaaatgaaattttcactttccaggaacctaacaaatgaaaagatagaaatcaattccaacagaatattaccaaagaaatcttttagaatggactgttaaaattatttatttgtatttatctggctctactatttgtggtacatttccacttcaaagctaaacctcaaataacatcatagtgagtggttgacttcatgtttaactgagatcttgaagactgaaaaagaccacgacaaacacacatctattttcttggctactgcatccgtgttcatcaccattctgatagtctgcaatgtattgcagctcaccctttgggaaggactaaagtagacatctgtttgttctgcttactcagcattcctaccctaattttcctttggagaacccctttattctagaccacgtgaagctaatgccaaaccccattccaggggatgcacctgaatccaacctccatcatctaaacagtgccttctccacgttcagagaagagcaagtgactcaaactgccctcataagaacagacctgggacttctgctgcaaatattgaagagtaagtactcttttttcttgctaggactaagctggtagtaccttctatgaggctatcatatggaaacaacttgtctgaaaatgaagccacaactagaaaacagatcctggtaacccggattgatggatccagccctaccttaaatggcaagacctaacccgaggctttttgcatcaaccaataaagtccttaagccagtttgagttggttttgtcacttgcagctaaaagaattctgactctaacaatgtgacaatagcaaaaataaacataactgcttttgaggtttctaatggattttcctccctatatacatgatttcatttaatcctcacaattcaggaaagcacatatctattaacattaaattaatattcattattttgaacacatgctatgtggataagggatgaggaaagccaaggaagtaatcaacgtgaaatctcacttatatgggagggaagtggaggttacatatctcagggcacttaacagatatcatcaaatgaaagaataaacagtgtgtgggagaggcagtaggtgattcttcatcaattcctggatgaaaaattaggagataatgaactccgaacaggcagcctaatgagaatggctcaagcaacaggacatagagagggagttaggttagacatggggttcttgggaattttcacctcgtgggggggcgggggggtcgtgcagctgttgtcagtgggaaagggaaaaaggaaaaggctgagtttggaaggcagggagggaggagacaatgtgagtcagtgaaaaagggcccttagaatgacaagtctggaccagagagaggctaagactgaaaatacaagttgggtaaccactggcatacagatggcagttcaggcttgggcactgcccaccagagcctcagcatgaagagaagagggggaggctggccaccacctccctctaggtaatcgtcatcctgatgctgagctcctgaaaacaggctctttcactcgccccatctcttgctcttgattgcaacccggcattcaggaggcaccctgtaatatctgtggagtgaccgacaacacagcgccagggcactgagaagatcccagggcgccagggactggttctacaagggtgcccctcccggtcccctccagcgcgccgccagagctgccagtcttggctgctacacgggaggcagcctcattatgcagctctcacctcttaaattagttcatgctctcacattaggtgtaatcacagcttgcaacgctttctggggatgtctcagaaagatctgagttgaaaaaatatttttgtgtcattttaatttaaagtaaaattgctgcttcttccccgcccctttctttcctcctggcccacccagcgaccctggccggccgtgctcaacgggggcgggggtcggaggtgagatttcctccacataattccttaaacagctatcaactaagtctcaaagaaaaaaaaaagagatctagaagcagagacgtggctgctggcgatcccaaagctggtgttcgctcttgggggagagcgtaccctgggggaggccgggaggccgggccagaggctagcccagaggcagagggcaggagcgctcagccggcgccccgcgtctctccagctcccgacgctgcgctggctccgctgagcacgccaggatcaaggtcgcctggtggggaccggagcgccaggagcctgtgggaagcgttccagccggcctctgactgggatccggcgccgcgtttctgctttggacttgactgacaggtccccccgccctcccgccgccctactaccagcctgggttcatccttcagggctacgtctaccgcacccgggctggaaagcctggagcgcgcccttcctctcctcatcttctcagctctcctttctccctgccacttggcaaagctgcattttgactttcacgttttggactacgtgtgtgtagttccaagtccatgcgtggcacgaaaatccacttagggtaaaaattattctcgaaaaatcgcccatctcaggatctggtgtctacactcaaggctaggaggtgcaggtacgggtgcgtaaagcatgccgtaagggtgcacagtaaataaaaagtacggatgcaaaatgtaaattttaagtgcaaaacagaaaagcagtactcgttgccgccccgcacgctgggttttaaggggcacgaaggtgggcctcggctgcttttgctcagccccgcgtcctcagcgcccggcccagtacccggtactccgtaggggttcaatgatctcccctgaataagtgaacgaattaacaaatgaatgaatgaccgctcgatccgacctccgcggccggcagagcagtcgctggagaggcgggagagagcgagaggccaagctccaccatcgcggccgccggctggggcagagggacacggagacactcggcgccccggctccgcaccgagtccccg

SEQ ID NO: 12757 - RNA, 14205 nt, Homo sapiens
  source 1..14205: mol_type = other RNA
gatctcactttgttgcccaggctggtcttaaactcctggcctcaagtgatccccttgtttcagccccgcaaagtgctgggattacaggtgtgagccaccatgcccgtgcccagccacctcatgagtcttgatggggggcagagaccaacaactccacagaagccagatgcttgctttcccagcctctcttgcagctagggcttgggcatgtgatccaggctcagccaatcagatggcactgactcttggcatgacatgggctaaggaggggctgcagggaatccatttgggctggggtggcagctgcactgggagcgacatcagtttccagagggagcagcagaatctggcatcaggcttggggcgtggtaggtgcaaccagactctgcacccagcagcagtggcagaatgggttctctgtggagagtctgtgtattgctccttccgctgaggccaccagcatctgcctccatgaacccctcagagcctgtgagcaactcaacagccttgaattttttcccttcctgtttgaatgagccagggttgtttcactgcttgaactaagagccgttcctgacatgaaaactaagccacatctttttgacccaaagattctggcatcctaaaatacccatctcattttaagttaaaaataaatccatgtttgagcatctactgtttcagttactgtgctaggtgttacaaagctaactaagagtgacaagtaaataactatcatcaccatgataaacagagaatggaaccctggtttttggaatacagacacaaaatgattaattctgcctggaagcgttttggaacatttcagagaggtagtgagctgggccaagagaagagcatacgcaaggaatggtggcatgaagttgcctggtgtgtcctgagaagaaagatgggctaagaaggactggggtagggcagagaagggggtcactggaggtgaggctgggaaagtgagccaaggctcaaatgcaaactgtctgaacttcattttctgtgcaagcaggagaagccgctgacatgggtttggaagatggactgaagccggagaaaaatggaagcaagaaaccctctcacaagaggccataaccacaaccaagtccatgagattgaaaaggaaggcagatatttgaaaaatatttaaagagatgtgaggggtaggacaggcacagtggctcatgcctgtagtcccagcactttgggaggccgaggtgggcagatccacgaggtcaggagatcaagaccatcctaacatggtaaaaccccatctctactaacaatacaaaaaattagtcaggtgtggtggcacgtgcctgtagtcccagctactcaggaggctgaggcaggagaatcgcttgaacctgggaggcggaggttgcagtgagccgagattgtgccactgcaccctagcctaggcaacagagcaagactctgtctcaaaaaaaataaaaaaaaaaaaaagagagaaagagagagagagatgaggagttgctgcactgctgggtgtggagagccgaggaggattcaaagatggtcctgaagtcccagctggaagaagtaggcggcagcaatgtttttaatactgtaaattcatcacgtagcacaggtttggggtggagaaagaaaaattgcattggcttcagggcatgcccagatctttcctcatcttaggcgtttgctaatacatgcattttctaagctgatgtcttgcgtttaatcactgctccattcaaaagagagaaggaggttgtttcaaacctagttgatatcatttgacttccatgctattcacagggctattttatttgaaacaggtataccacagccttaaattgcaagttaatccaggatgttcctaggttggcagttaggaacatgtaattctttggaagggctaaaagtcagctctttaaattatctccatatgaaccttctctccaccttagggtggatccacttatttagtccactgccagtaccacactagaacccgggtggtcactggactccagaaacaacagtagccctctctctgttctgtctctttttgactatctctattctgttcctgaccctgatttctcctgccaagctcaattttgacagctgacaacggcaagccatggcttcccaaaacattattttcaggtcaacttataaatttcaagaacacatttggctccgcttcctgtggtactaagcctacttcttgacagcatttgcctttgttgtaaatagcaaagttcttctagttggatttttgctaagaagtgtgtggatgtggcatgtgacgacatctttagcttggattctagaaaggcactaccattgtgcatttggctaaaggaaacacattttacccgtgaatgccttctatttacaaatgctcagctagcacacaaagctaagtacaagcaataagtactatcctacaatgttactcatttctgaaagcacaaaatgatgactggtatagctttggagatgttttctggaaacccaataaaggaacagatctttgttattccacacctacaaagtcagaagatgcacagtcttttattcatgtttgaacaagcttccttcttgaacaatcaactataaagtgatgtgattctctactagaccaggaactccttgaggacagaatgagggtctaatccatattctaaatccacaccacctggcacaatacatgttgcatggttagggtcaactaagagttggttgaattaatcaataacacacagcaagagaattcacaaagagaggggagtaatcccccagcctcaatcactcggcaagtggaatcgctgggcactgattccagctctgtctcagtgcttgagacagagctgaatgtaatgtgaacatttcaaatgaacaggaaaactagactcacggataagcagtgtagtcatcaagacaacactgtcttggaggtttttctgaagttaaaaccatgctacataagcaataaattatgaaggctgagcatgtgaataaaatttaatgttgtcataaattttataacaaagttaatctgacacatttaatgacatgcataatcattagtatgcagcactgtaatcagacattgataataagcagttcacaccagtgactgtaagagtctttacttgtgttcagccaagccaactgcttggtatatttttctcccttcttagtcgttagttttccatacctacaataactatcagtggtgatgggcttctctgaccatgtgaataatttaatcctcaatgcacagatacagaaacccttgctgaagacagtgtggagcagagaaggctgtctccactccttccacctgaaacacctctgcagatggatatgggagctctgcctacagcccttggacctaaccacttcagtgtgttccagtgagtgtctggacctcggcctgaaagatttttccgaaactaaagaaaatttctctgacctaaagaccttaacctccaccccagaagctctcaccaaggactacagggaactggtggggaaaatccttatcccttactcctcaaggcacagggcagtaatgctgaggcttgtgcgccacacttgctcccagaggtccccagcgggctacctgcggtggtgaatgacctcctaacacgccccttgacggccttcctttccttgcctcacttctccactctcctaccagcattgcagggttcacatcccaaatataccactggcacttgaatcctggtctccaggtctgtttctggaaaaacccaagtaagacattgccccagtaatggggctagatgtctgaggcttcctcaagtatctacctcgaaagctcttactgctgtacacacatgcacatacacacacgtgcgtacaaccagtcacatctaagcaccccgaataccagcctgttgaaggtagcagagagctgcactataagccaaggctgctcccaagagccgctccatcactgaattggcgccccagcaagatgaaggaatgtaatcattggaaggatggagaatgttctctgaatcactgacaaattggaaggggtggagggcaagagtccacctggtggagagatggaaagagcgagagagcctggaatgataatgccattgcttagaaaaggctgctccagatgccatatctacagaaattgtacagcccaaacatctctgagcaataggtctctggtagtcttgatgtctagaccaacaattcccagttcattcttctcagggaaggagccaggatagtccagagactctcattctgctgttagattgaaagggttaggcacaacagccttggcaaagtcacaagggcaaattcacactaaagtgtaaatgacccacaactcctcttctatttttaggttggggaggtgctttagaacataaggaggaactaaagaatattcctgttacatacaaggcagagaaaagggaaactagtggtgacaagacaaatcatccctttgacatttggctggctctacctattacagctctgggggtgaggtgggaacaaaaagatgctgtgtaaagaagtatcttatgccatccctactgtagtgaggtgcagtttagaggggacactgatcaagcagagacccagagtgtttcgttccaagccagaaacagaaatgtataaaacacagcctttccagcatcagaaatgagtagtggtagtggagaactacccaaaacaggaaagaggaccacgtgaggtagagtgtcaaggccctacattccagtgcctctgctcatgactgtaattttgggtaggtcacttaaagtctctggacctcagttttgccatctgtgaaatagggataatactatccagcataaaattggttatgaggctcatgtagggcctgcctgggatgatgtgttgctaatggttaagaacacaacttctggggtctgactggacaggctgaaatccctgcttaacacgttccagcagagccctgggcgatctatttaacttttgttttctcacctgtaagctgagacgaaagtacccactttataagattattccaataattagttgaaataatgcatgcagagaattaagcatggtacttgttatttgttaaactagctattaaaatgtgtaaaatataaagtattgtatggattttaggacaatgcaaagactctttgcttgctgcaatagttcggggccctttcagatggctaaaggcagaatttgtatgtgtaaatatggtgtgcttgtctctgctctggatactgagggcttaccctgttattaaacttatttagtaaatattgaactgtcatgaggcctaacatttagttccagttattagataaaacatttgctttgaatggtatttgaattgccaggttctagattattctggttgacaaactcttcgtattttataaagaggctaaaattggtaagctatcacagaacagatgtgccattttcaaggtatattaaaccatgattcactgtaacattgttcctactggcaacaaattcagagcaggctggactttatttggtgaagaaacattgagtggaagagaaatgacattattttatgtatttacattttcaaattactgtggcttaaacctgttcagccaacattacccaccttcagtctgctaaataaatgattcagtacatttctaatttacagaattttttaacaaaagaaaatgtaatttgatagccaaatcaacgttaaacattatacatttaaaaaaccacaggcaaagacacaaacatgatgacactaacttttgttaaagtatgcttacctatggtttcctctgaggcacgttctttcatgctaagcttccaacataatatgaaaatgaaggagatgcattttgcaaagcaaaacagaccttaagcaaaatattatacttctcaaattaacactgttacaaagttttagaatttaataagttcattaatttaaaagtttggatgtctgagtccttctatcccaaaacaagatcttggagggtcttccacagccatgtaataccatggtcacatgaccctttccaaaattattaatctgaatttactatatgaggataaatctatctttttgaaaatatttaggaaaatgagcttggtatttataaaatgaagctctctttgggtggtatcctaagacacgtcaagccaatcagcctgtaactgtgaaaaaaacattggtaggtacaaaagtggggtgggagaggagtgacttaactttgttaagtgatgggaaagaaacactaatagcattatctcaataaaatgtgatttaaaaaaatttaaaatactaaatcattgaactgacaaagaaatataaatcattcagaaataaactcattaggtcatcaaatcctgttaaatctgcaattaggaagagcaaggtgtacaatccatacatttaaactcacaggctcactttgcacaacgtcaatttactccttaatatgttattaatacgcattttccaaaaggatgtattagtaaatggtacacatctacttcttggcaacatcatataacctggtacaacataagcattcttcttatagttaagaaatgtggatggtatcaaaattagaaaaataaatgccctattatgttgtggtcaggtttaaggcatgtgaattttatcttcatacaaaagattaaaatctagatattaaaaagtagtgcagtatcagtgatgctgcctcagttcccaaaatgtcacatcacaaaaatatcccataattgcctgtagtttattccttggctttcctcttttctctctgcatctttgtaacaattttttaaaagtggaaatataattgttggcaatgctaacagctgtagaaatgattacaagatgtggaaaagcataacaggaatgtcaagaatctgtttctggcagtaatatatatggaacattgttcaggacaaaagaggagaaggaagaaaaaaaggagaggggtttatcatctctaagaattttcaaactaaacctcattgcttaataggaaaaaaagattccatatttaaagttaagtcacctctaactactagctaaagcatgacatcaccagcactggagtcagcggaagtgtgtttttgaaggacagtgttgcaggagaatctggacaggttttagagccaggagagagaaaataattctacctctgacagttgaaggaccttaggcaaatcagtttacctctgctagactacactccaaaatttggacattcaaaaatttgatattaataaccacatgaaagtctcgtgttgaggtgaatatgtatttgttggtgaaagatatgttggtttttaaacagacagcactctgcaattgtaggctattgttttgttttgccagttgtcaaattctatccagctatacacacttgtgtggcctcctaatggtgtttttccagtggctaaaggtttatgaataagacacttttcctaatggaattaacccgatgcttttcttaaacatgtaaccttgagttcaccgcaaaaaacaatgcttcgattagagcaatgcatataataaaggttaccctcgtttcttagacactagacatcattcacaaaaagagaactgcttttgaaagggatgtatttgcactggaaagaatagttttctacttctaattataaatgatttattggtgaaagcaaaacaacagcctgtctgagaggcacttctatgagcatcctcacgtgtgatttgcaaggttgaagaagagggaaaaatgcctcaattgtaccaatggtgagaaaacacccaaagtacaaagcaggtttcaaaaaaaccatactcataaccaaggacaataataaagcaatgtgttgacatatactctataagtcttcctccataaatagtttatagaaattttgtaatttctgtaaatgcatcctataataattttgcatcttgctttttttttacatttaatatcaagtagatttctaaagggcaattatttgaaaattatcccaaatacatggggaaatatacatcaagtgaaaaaatgcagtgggtgatagagatatcaggaagcgcctcaaatatttctcatctcgttggagaaaaacaaacatgttctcatttagaatgagtgggagttacctaattgatttaggcctctatatttaacttctagtcaaaaaaggtagttctatctagcaacaatattatggggaacaaaagaaaaaattaactctctaaatttgcagtagggtcttttcttcagaagtaccaaatcccatctattaccagctccatgcttcaggcctaaaatggatctccctgaagcaatgacagaatttttgccaagtgactaggatataaacaccactttggttgcacagtgagacatatgctccaaagaaaactggttcaaaaacaggcaagtgggtttctacagaataaatgagagccctgtcaatggcttcatcttcagggctttgtgtctgtgcttgcgtggtggctcttgtttcatctatggataatggtggcacacagttttcataattccttacattaatgaactgctataaatttgtttttggtattctagagagtcctaacttcagcttctgggcaatgctgaggaggcaccctatattctagacttaccttttgcaaggtgtactctcagcattgtgggcgatttccatgggagaatattctatttaaagaactactgtcccagcataaaacaaaaaatcatttatgaagatgcaggagactcggaaagctctcaattattgtttgcacaagcacaatgtcacagcctcctttccccattccacaagggggtcaggaagagagtactcagctgtgagaaaagacatacagaagaattcatgtggtcatgagagcgaggacatggccgatcccccaaggaggatgtgtcatacacttcatgagcccaagagtgtgctgtagggtctgaagggcaagatgctggttcactgatgtaaaggagagggaaaaaagcttcaaccaactagaaaaacagtctctatgcatgctatttttgattttaaacacaggtatcaattccttctctcagagagtccattttaaaataggatacatttttaaaggaatatttaaaggacacattcattaaaatttattttaaaaacttttcaaaagaaacaaaaggtatgaattttatttaatccttgaggaaatggttcttttctcacacacataaatcactcattttgtttttctttatctcctttattaatctacattagaaaaataaacttttcatacactaagaacaaggaaaccactctcaattgacaaaatgttccaatccaacacaatgattactttcacctttaatttacaggcagccagattcaaaatccttaaagttgcttaaacttaaaaatgacaatgacaacctaaaaggtataatgttgattggaacagacatttaattggaaaattgatgattttccatttccaattaaatctctagatagaaatgaaaaaaattaaaaatcgtatttaagaaaagccaaatcttgggttgtgaggtatctttttaaggatgtttcagcagaaaaaaacaaaggctctcacaattgtgtagctgcctagattaagtgggtatcctgatcaaggagatgggggatgatttggctttagtattccaatgataaagtttataatgagaataacatgttgctacaaaatccagtctcttcctcagatgccttccacagagggcaggaagctttgtcagttttgtttgctgatgatgcctggttccgtcaacaaataacacctgtcacacggtgggtagtcaatatacatttgttgaataaatatgaaaaaaagaaatgtacaatatgtttgtgaagccaactgtgtgtgcattgctattgaggtacacaaaaagtctttgttttaaatttgagaatgaggactttcaatggaatatatctataaaaatgaaaaaaagacattactgtctggacttttgtacagcaagagaagaaaaaccactagccaagagccaactcacctgataggcctggatcaagcatgcagctgtggagaacacccctgggactctaactctggcactctgcaagctgggtacttgggcaggacagcagcagcactcatgaactgggcagcacctgttggtgagggctgatcacatggattctctcatcccagccttacaatcagtccttcaggtacatactttttctgactttgctgatgaggaaactatgcacagaggttacacagcttaacaaagggttctcacctaatgaacaatgaaatgggattttagcctttctttgcatctggtcttagagccaatacccaagaagcactgtactgtatgcattgtctcagagaaacttactcttcctgggcctcagtctttaaaaggtgggcagttgacttaataagaattaaagatcaatgattaaggttcaaggcactccaaaattctggtctttattgaaaaggctacagaagtctcaccttaataataccctatagacttgatattcttggttaattaaatattggaaaccaatttcatagtaattgaggtcagaaaaaagtactcatgacattttagaatatgatgacaaagccatagataaatttcaatgcacctgtaattacttaaaactgttatagcatgcaatgtgttaccacaacagccagagaaatactaatttactcagcctattcttctagaccagtaaacactaggattaaatagatattttcattgaatttgttctacccttcattgccatttatagatagcttacttgtcatagattactttctaattgttttatgtttcctaactagcctgcaatactttggcaaggacctcaaacaatagtagacagtaggtgtaaaatagatggctacattgaacagatgactaaaaggatgcctcctaagtacctatatcttgaaatatatattattgtgccttgctttcaatttgtgattttaaaatctagaaatcacctgttttatgtaataacaataaaatccttctttgttgaaaacatgcacaaataaagtttacaagctcaaaaaattaaacagcagtaacggtcaagctttccaacaataaaatacattttggtaaggttttcattttacaaaaactcaaaatagctttatgagttcacaaaataatatgatatttttcaagatattaacatattcttataccggaagagcatagaataaaatttacttggagattgagcatttgcttctttaagaaatacttcttttagtatttttactttaatattatgaaagctacataattacattcagattcattaactactccagtagttaatttttaaaacttatgatgaatagttttgtttaaaatatataacattggtaatatgcaaatctgaatctgtaataaagaaggatttgcattcctgatttttttttctgatacaaccaatgacaaaataactaatggttccacagaggataaaatgtctcaaatctgttggttctgaaggtgaagcgagatttttgtactgataccgtgtatcactgagataccaggaggaaatggaattaaactcagatagttcaaatggagagattttaatgaagggacgacctacagaggtgtcggcagggttggggggaatcagcgagatatgcttagaacccaccgactggcaaacctccccctgaagatggagaaggaggaaggagtgttactggaatgagagcttgagtccaggggaggaggatgggctgctgaggaggcgacaccatcctgaaagaagaatcctctgccagaggcttttcagggtcatttcttcacactctctgcagggaagcacggagacagcaggaagaaatatcctaacctcactctcttccctctacaggtgcttccattggccaaatccacccagaggccagttggtggcgatcagctctcttcaagtggtatttaaatttcttctttcattttccttctggtaacaaagaagtctgtggctcaaaagatgtttctctaagaccccatcctattaggtctctgagctgtgggaagtatttatacaattgcttgtgaatataagatccaggaatttccctaagatccctaacaaaattggtgataagtagtcccacatgttaatccagccacccacggatgacagcacttaccatttctttgataaatgtcaaatgcatttgaagtacctacctgaaatatttgtttaaatgctatctaatctattaattttatatatgtgtgagtctgttttgtataccttctgattataggataaatgtaaataaatccaaagagtaatcaaagctaccactttcaagaagccttctttgtagaaccggaagagtcttaaataggcttttcaggtatgcatctcttattatcgctgaactccaagtcctgcaaggcaggcatcatgtgtgggtcacctttacagtaggcacaggccttaaaacagtgacatgcacattgcaggcactccataaatgtttgctgaattggctaaaccttggtttgttcccataatcaaccaccacaaacagcacacagataattacttcttggaaagattccaactagtgtttgatgttacctacgtggtttttctctcaagatcttaagagcagctctgtaggattacattattttctgttttttttttcctttgaccttaatgtcatctacttcaataacagcttcatacaaaattcctaccagcacataccacagcagattcaaggccttgttttaaaaatggtgccagcttctcttaatttggaagatatattgtctctcctgaacatgggctaagaaaatgtataatttggtattaacataagagctgaagacactttaaatgcattgtttcatttttataagataaaaaaaattttaagaatcaaaatgttatcaacagacttgtccttcattaaaaagtaaaactgcatttgcctacattttatgaaagtgtccaattatgaacaattttgaaatgtaacttttaaaaatgtaaacagcaaaaatgttgtatttaaaataaatctggaaaggcagaaaaacaaaaaatacccagaagacagagtttttggtgaaagttaagatatttcatctttgaacaacttagaatctttcctgcattttatagtctagttccaggcattaatttgaaataaccttggaatcctaaatctaacacccttcggaacaaagtagcttttctcttctgctttatgagcaaatggactaaatactagggaatggtactgtctgggcctttgaaccaagattgaaagagatgaaatcctatatgatatgtataaacattagagaatccattttgatttaataaaaggttgaatttgttctatatcctgtgagaaaatggttcccttttcctgaaaatgttacctcattccaacaatagaaagttggtttttttccagggtgtggtgttggcgggggacagagttgccatgaatatggcatctatgaagactgctgttatattcatttctcaaaatgcactgtggtaggaaattcagaacgcagtgagagaaaataaatgtttgacttcaaaatataaggccgcatttaaagcagaaggtaaagtatagaacagttgacagtataaattctttatctgcaatcttgcagttccctaaatctctgtaacacatcacttttaaaagcctcagataagtggttctataataatttaccaataattcaacccctcaaaagtcttagcaagttaaaccttataatcttacattttagaaatgacccaacttgatccttttattcttcagaatatctctctcaaattttcatttgtttttcattaattgatgaataatgagacattttaggtacctgtccacaaagaaatgaaattttcactttccaggaacctgagggccgacgagtgggggcgggcaggagggccgagggaggcggaacaggatcgaggcgcgaggcgggagtcgagaaagcgagcggccgaggcgactctcagtgcgcggacgcgggcgcgcgcccgcgctcccttcgtcgactcacggcgagagcccaaccctgctgccgcgcgccaccc

SEQ ID NO: 12758 - RNA, 10790 nt, Homo sapiens
  source 1..10790: mol_type = other RNA
gatctcactttgttgcccaggctggtcttaaactcctggcctcaagtgatccccttgtttcagccccgcaaagtgctgggattacaggtgtgagccaccatgcccgtgcccagccacctcatgagtcttgatggggggcagagaccaacaactccacagaagccagatgcttgctttcccagcctctcttgcagctagggcttgggcatgtgatccaggctcagccaatcagatggcactgactcttggcatgacatgggctaaggaggggctgcagggaatccatttgggctggggtggcagctgcactgggagcgacatcagtttccagagggagcagcagaatctggcatcaggcttggggcgtggtaggtgcaaccagactctgcacccagcagcagtggcagaatgggttctctgtggagagtctgtgtattgctccttccgctgaggccaccagcatctgcctccatgaacccctcagagcctgtgagcaactcaacagccttgaattttttcccttcctgtttgaatgagccagggttgtttcactgcttgaactaagagccgttcctgacatgaaaactaagccacatctttttgacccaaagattctggcatcctaaaatacccatctcattttaagttaaaaataaatccatgtttgagcatctactgtttcagttactgtgctaggtgttacaaagctaactaagagtgacaagtaaataactatcatcaccatgataaacagagaatggaaccctggtttttggaatacagacacaaaatgattaattctgcctggaagcgttttggaacatttcagagaggtagtgagctgggccaagagaagagcatacgcaaggaatggtggcatgaagttgcctggtgtgtcctgagaagaaagatgggctaagaaggactggggtagggcagagaagggggtcactggaggtgaggctgggaaagtgagccaaggctcaaatgcaaactgtctgaacttcattttctgtgcaagcaggagaagccgctgacatgggtttggaagatggactgaagccggagaaaaatggaagcaagaaaccctctcacaagaggccataaccacaaccaagtccatgagattgaaaaggaaggcagatatttgaaaaatatttaaagagatgtgaggggtaggacaggcacagtggctcatgcctgtagtcccagcactttgggaggccgaggtgggcagatccacgaggtcaggagatcaagaccatcctaacatggtaaaaccccatctctactaacaatacaaaaaattagtcaggtgtggtggcacgtgcctgtagtcccagctactcaggaggctgaggcaggagaatcgcttgaacctgggaggcggaggttgcagtgagccgagattgtgccactgcaccctagcctaggcaacagagcaagactctgtctcaaaaaaaataaaaaaaaaaaaaagagagaaagagagagagagatgaggagttgctgcactgctgggtgtggagagccgaggaggattcaaagatggtcctgaagtcccagctggaagaagtaggcggcagcaatgtttttaatactgtaaattcatcacgtagcacaggtttggggtggagaaagaaaaattgcattggcttcagggcatgcccagatctttcctcatcttaggcgtttgctaatacatgcattttctaagctgatgtcttgcgtttaatcactgctccattcaaaagagagaaggaggttgtttcaaacctagttgatatcatttgacttccatgctattcacagggctattttatttgaaacaggtataccacagccttaaattgcaagttaatccaggatgttcctaggttggcagttaggaacatgtaattctttggaagggctaaaagtcagctctttaaattatctccatatgaaccttctctccaccttagggtggatccacttatttagtccactgccagtaccacactagaacccgggtggtcactggactccagaaacaacagtagccctctctctgttctgtctctttttgactatctctattctgttcctgaccctgatttctcctgccaagctcaattttgacagctgacaacggcaagccatggcttcccaaaacattattttcaggtcaacttataaatttcaagaacacatttggctccgcttcctgtggtactaagcctacttcttgacagcatttgcctttgttgtaaatagcaaagttcttctagttggatttttgctaagaagtgtgtggatgtggcatgtgacgacatctttagcttggattctagaaaggcactaccattgtgcatttggctaaaggaaacacattttacccgtgaatgccttctatttacaaatgctcagctagcacacaaagctaagtacaagcaataagtactatcctacaatgttactcatttctgaaagcacaaaatgatgactggtatagctttggagatgttttctggaaacccaataaaggaacagatctttgttattccacacctacaaagtcagaagatgcacagtcttttattcatgtttgaacaagcttccttcttgaacaatcaactataaagtgatgtgattctctactagaccaggaactccttgaggacagaatgagggtctaatccatattctaaatccacaccacctggcacaatacatgttgcatggttagggtcaactaagagttggttgaattaatcaataacacacagcaagagaattcacaaagagaggggagtaatcccccagcctcaatcactcggcaagtggaatcgctgggcactgattccagctctgtctcagtgcttgagacagagctgaatgtaatgtgaacatttcaaatgaacaggaaaactagactcacggataagcagtgtagtcatcaagacaacactgtcttggaggtttttctgaagttaaaaccatgctacataagcaataaattatgaaggctgagcatgtgaataaaatttaatgttgtcataaattttataacaaagttaatctgacacatttaatgacatgcataatcattagtatgcagcactgtaatcagacattgataataagcagttcacaccagtgactgtaagagtctttacttgtgttcagccaagccaactgcttggtatatttttctcccttcttagtcgttagttttccatacctacaataactatcagtggtgatgggcttctctgaccatgtgaataatttaatcctcaatgcacagatacagaaacccttgctgaagacagtgtggagcagagaaggctgtctccactccttccacctgaaacacctctgcagatggatatgggagctctgcctacagcccttggacctaaccacttcagtgtgttccagtgagtgtctggacctcggcctgaaagatttttccgaaactaaagaaaatttctctgacctaaagaccttaacctccaccccagaagctctcaccaaggactacagggaactggtggggaaaatccttatcccttactcctcaaggcacagggcagtaatgctgaggcttgtgcgccacacttgctcccagaggtccccagcgggctacctgcggtggtgaatgacctcctaacacgccccttgacggccttcctttccttgcctcacttctccactctcctaccagcattgcagggttcacatcccaaatataccactggcacttgaatcctggtctccaggtctgtttctggaaaaacccaagtaagacattgccccagtaatggggctagatgtctgaggcttcctcaagtatctacctcgaaagctcttactgctgtacacacatgcacatacacacacgtgcgtacaaccagtcacatctaagcaccccgaataccagcctgttgaaggtagcagagagctgcactataagccaaggctgctcccaagagccgctccatcactgaattggcgccccagcaagatgaaggaatgtaatcattggaaggatggagaatgttctctgaatcactgacaaattggaaggggtggagggcaagagtccacctggtggagagatggaaagagcgagagagcctggaatgataatgccattgcttagaaaaggctgctccagatgccatatctacagaaattgtacagcccaaacatctctgagcaataggtctctggtagtcttgatgtctagaccaacaattcccagttcattcttctcagggaaggagccaggatagtccagagactctcattctgctgttagattgaaagggttaggcacaacagccttggcaaagtcacaagggcaaattcacactaaagtgtaaatgacccacaactcctcttctatttttaggttggggaggtgctttagaacataaggaggaactaaagaatattcctgttacatacaaggcagagaaaagggaaactagtggtgacaagacaaatcatccctttgacatttggctggctctacctattacagctctgggggtgaggtgggaacaaaaagatgctgtgtaaagaagtatcttatgccatccctactgtagtgaggtgcagtttagaggggacactgatcaagcagagacccagagtgtttcgttccaagccagaaacagaaatgtataaaacacagcctttccagcatcagaaatgagtagtggtagtggagaactacccaaaacaggaaagaggaccacgtgaggtagagtgtcaaggccctacattccagtgcctctgctcatgactgtaattttgggtaggtcacttaaagtctctggacctcagttttgccatctgtgaaatagggataatactatccagcataaaattggttatgaggctcatgtagggcctgcctgggatgatgtgttgctaatggttaagaacacaacttctggggtctgactggacaggctgaaatccctgcttaacacgttccagcagagccctgggcgatctatttaacttttgttttctcacctgtaagctgagacgaaagtacccactttataagattattccaataattagttgaaataatgcatgcagagaattaagcatggtacttgttatttgttaaactagctattaaaatgtgtaaaatataaagtattgtatggattttaggacaatgcaaagactctttgcttgctgcaatagttcggggccctttcagatggctaaaggcagaatttgtatgtgtaaatatggtgtgcttgtctctgctctggatactgagggcttaccctgttattaaacttatttagtaaatattgaactgtcatgaggcctaacatttagttccagttattagataaaacatttgctttgaatggtatttgaattgccaggttctagattattctggttgacaaactcttcgtattttataaagaggctaaaattggtaagctatcacagaacagatgtgccattttcaaggtatattaaaccatgattcactgtaacattgttcctactggcaacaaattcagagcaggctggactttatttggtgaagaaacattgagtggaagagaaatgacattattttatgtatttacattttcaaattactgtggcttaaacctgttcagccaacattacccaccttcagtctgctaaataaatgattcagtacatttctaatttacagaattttttaacaaaagaaaatgtaatttgatagccaaatcaacgttaaacattatacatttaaaaaaccacaggcaaagacacaaacatgatgacactaacttttgttaaagtatgcttacctatggtttcctctgaggcacgttctttcatgctaagcttccaacataatatgaaaatgaaggagatgcattttgcaaagcaaaacagaccttaagcaaaatattatacttctcaaattaacactgttacaaagttttagaatttaataagttcattaatttaaaagtttggatgtctgagtccttctatcccaaaacaagatcttggagggtcttccacagccatgtaataccatggtcacatgaccctttccaaaattattaatctgaatttactatatgaggataaatctatctttttgaaaatatttaggaaaatgagcttggtatttataaaatgaagctctctttgggtggtatcctaagacacgtcaagccaatcagcctgtaactgtgaaaaaaacattggtaggtacaaaagtggggtgggagaggagtgacttaactttgttaagtgatgggaaagaaacactaatagcattatctcaataaaatgtgatttaaaaaaatttaaaatactaaatcattgaactgacaaagaaatataaatcattcagaaataaactcattaggtcatcaaatcctgttaaatctgcaattaggaagagcaaggtgtacaatccatacatttaaactcacaggctcactttgcacaacgtcaatttactccttaatatgttattaatacgcattttccaaaaggatgtattagtaaatggtacacatctacttcttggcaacatcatataacctggtacaacataagcattcttcttatagttaagaaatgtggatggtatcaaaattagaaaaataaatgccctattatgttgtggtcaggtttaaggcatgtgaattttatcttcatacaaaagattaaaatctagatattaaaaagtagtgcagtatcagtgatgctgcctcagttcccaaaatgtcacatcacaaaaatatcccataattgcctgtagtttattccttggctttcctcttttctctctgcatctttgtaacaattttttaaaagtggaaatataattgttggcaatgctaacagctgtagaaatgattacaagatgtggaaaagcataacaggaatgtcaagaatctgtttctggcagtaatatatatggaacattgttcaggacaaaagaggagaaggaagaaaaaaaggagaggggtttatcatctctaagaattttcaaactaaacctcattgcttaataggaaaaaaagattccatatttaaagttaagtcacctctaactactagctaaagcatgacatcaccagcactggagtcagcggaagtgtgtttttgaaggacagtgttgcaggagaatctggacaggttttagagccaggagagagaaaataattctacctctgacagttgaaggaccttaggcaaatcagtttacctctgctagactacactccaaaatttggacattcaaaaatttgatattaataaccacatgaaagtctcgtgttgaggtgaatatgtatttgttggtgaaagatatgttggtttttaaacagacagcactctgcaattgtaggctattgttttgttttgccagttgtcaaattctatccagctatacacacttgtgtggcctcctaatggtgtttttccagtggctaaaggtttatgaataagacacttttcctaatggaattaacccgatgcttttcttaaacatgtaaccttgagttcaccgcaaaaaacaatgcttcgattagagcaatgcatataataaaggttaccctcgtttcttagacactagacatcattcacaaaaagagaactgcttttgaaagggatgtatttgcactggaaagaatagttttctacttctaattataaatgatttattggtgaaagcaaaacaacagcctgtctgagaggcacttctatgagcatcctcacgtgtgatttgcaaggttgaagaagagggaaaaatgcctcaattgtaccaatggtgagaaaacacccaaagtacaaagcaggtttcaaaaaaaccatactcataaccaaggacaataataaagcaatgtgttgacatatactctataagtcttcctccataaatagtttatagaaattttgtaatttctgtaaatgcatcctataataattttgcatcttgctttttttttacatttaatatcaagtagatttctaaagggcaattatttgaaaattatcccaaatacatggggaaatatacatcaagtgaaaaaatgcagtgggtgatagagatatcaggaagcgcctcaaatatttctcatctcgttggagaaaaacaaacatgttctcatttagaatgagtgggagttacctaattgatttaggcctctatatttaacttctagtcaaaaaaggtagttctatctagcaacaatattatggggaacaaaagaaaaaattaactctctaaatttgcagtagggtcttttcttcagaagtaccaaatcccatctattaccagctccatgcttcaggcctaaaatggatctccctgaagcaatgacagaatttttgccaagtgactaggatataaacaccactttggttgcacagtgagacatatgctccaaagaaaactggttcaaaaacaggcaagtgggtttctacagaataaatgagagccctgtcaatggcttcatcttcagggctttgtgtctgtgcttgcgtggtggctcttgtttcatctatggataatggtggcacacagttttcataattccttacattaatgaactgctataaatttgtttttggtattctagagagtcctaacttcagcttctgggcaatgctgaggaggcaccctatattctagacttaccttttgcaaggtgtactctcagcattgtgggcgatttccatgggagaatattctatttaaagaactactgtcccagcataaaacaaaaaatcatttatgaagatgcaggagactcggaaagctctcaattattgtttgcacaagcacaatgtcacagcctcctttccccattccacaagggggtcaggaagagagtactcagctgtgagaaaagacatacagaagaattcatgtggtcatgagagcgaggacatggccgatcccccaaggaggatgtgtcatacacttcatgagcccaagagtgtgctgtagggtctgaagggcaagatgctggttcactgatgtaaaggagagggaaaaaagcttcaaccaactagaaaaacagtctctatgcatgctatttttgattttaaacacaggtatcaattccttctctcagagagtccattttaaaataggatacatttttaaaggaatatttaaaggacacattcattaaaatttattttaaaaacttttcaaaagaaacaaaaggtatgaattttatttaatccttgaggaaatggttcttttctcacacacataaatcactcattttgtttttctttatctcctttattaatctacattagaaaaataaacttttcatacactaagaacaaggaaaccactctcaattgacaaaatgttccaatccaacacaatgattactttcacctttaatttacaggcagccagattcaaaatccttaaagttgcttaaacttaaaaatgacaatgacaacctaaaaggtataatgttgattggaacagacatttaattggaaaattgatgattttccatttccaattaaatctctagatagaaatgaaaaaaattaaaaatcgtatttaagaaaagccaaatcttgggttgtgaggtatctttttaaggatgtttcagcagaaaaaaacaaaggctctcacaattgtgtagctgcctagattaagtgggtatcctgatcaaggagatgggggatgatttggctttagtattccaatgataaagtttataatgagaataacatgttgctacaaaatccagtctcttcctcagatgccttccacagagggcaggaagctttgtcagttttgtttgctgatgatgcctggttccgtcaacaaataacacctgtcacacggtgggtagtcaatatacatttgttgaataaatatgaaaaaaagaaatgtacaatatgtttgtgaagccaactgtgtgtgcattgctattgaggtacacaaaaagtctttgttttaaatttgagaatgaggactttcaatggaatatatctataaaaatgaaaaaaagacattactgtctggacttttgtacagcaagagaagaaaaaccactagccaagagccaactcacctgataggcctggatcaagcatgcagctgtggagaacacccctgggactctaactctggcactctgcaagctgggtacttgggcaggacagcagcagcactcatgaactgggcagcacctgttggtgagggctgatcacatggattctctcatcccagccttacaatcagtccttcaggtacatactttttctgactttgctgatgaggaaactatgcacagaggttacacagcttaacaaagggttctcacctctcttcaagtggtatttaaatttcttctttcattttccttctggtaacaaagaagtctgtggctcaaaagatgtttctctaagaccccatcctattaggtctctgagattttagaaatgacccaacttgatccttttattcttcagaatatctctctcaaattttcatttgtttttcattaattgatgaataatgagacattttaggtacctgtccacaaagaaatgaaattttcactttccaggaacctgagggccgacgagtgggggcgggcaggagggccgagggaggcggaacaggatcgaggcgcgaggcgggagtcgagaaagcgagcggccgaggcgactctcagtgcgcggacgcgggcgcgcgcccgcgctcccttcgtcgactcacggcgagagcccaaccctgctgccgcgcgccacccgcctcgccgcgc

SEQ ID NO: 12759 - RNA, 15332 nt, Homo sapiens
  source 1..15332: mol_type = other RNA
gatctcactttgttgcccaggctggtcttaaactcctggcctcaagtgatccccttgtttcagccccgcaaagtgctgggattacaggtgtgagccaccatgcccgtgcccagccacctcatgagtcttgatggggggcagagaccaacaactccacagaagccagatgcttgctttcccagcctctcttgcagctagggcttgggcatgtgatccaggctcagccaatcagatggcactgactcttggcatgacatgggctaaggaggggctgcagggaatccatttgggctggggtggcagctgcactgggagcgacatcagtttccagagggagcagcagaatctggcatcaggcttggggcgtggtaggtgcaaccagactctgcacccagcagcagtggcagaatgggttctctgtggagagtctgtgtattgctccttccgctgaggccaccagcatctgcctccatgaacccctcagagcctgtgagcaactcaacagccttgaattttttcccttcctgtttgaatgagccagggttgtttcactgcttgaactaagagccgttcctgacatgaaaactaagccacatctttttgacccaaagattctggcatcctaaaatacccatctcattttaagttaaaaataaatccatgtttgagcatctactgtttcagttactgtgctaggtgttacaaagctaactaagagtgacaagtaaataactatcatcaccatgataaacagagaatggaaccctggtttttggaatacagacacaaaatgattaattctgcctggaagcgttttggaacatttcagagaggtagtgagctgggccaagagaagagcatacgcaaggaatggtggcatgaagttgcctggtgtgtcctgagaagaaagatgggctaagaaggactggggtagggcagagaagggggtcactggaggtgaggctgggaaagtgagccaaggctcaaatgcaaactgtctgaacttcattttctgtgcaagcaggagaagccgctgacatgggtttggaagatggactgaagccggagaaaaatggaagcaagaaaccctctcacaagaggccataaccacaaccaagtccatgagattgaaaaggaaggcagatatttgaaaaatatttaaagagatgtgaggggtaggacaggcacagtggctcatgcctgtagtcccagcactttgggaggccgaggtgggcagatccacgaggtcaggagatcaagaccatcctaacatggtaaaaccccatctctactaacaatacaaaaaattagtcaggtgtggtggcacgtgcctgtagtcccagctactcaggaggctgaggcaggagaatcgcttgaacctgggaggcggaggttgcagtgagccgagattgtgccactgcaccctagcctaggcaacagagcaagactctgtctcaaaaaaaataaaaaaaaaaaaaagagagaaagagagagagagatgaggagttgctgcactgctgggtgtggagagccgaggaggattcaaagatggtcctgaagtcccagctggaagaagtaggcggcagcaatgtttttaatactgtaaattcatcacgtagcacaggtttggggtggagaaagaaaaattgcattggcttcagggcatgcccagatctttcctcatcttaggcgtttgctaatacatgcattttctaagctgatgtcttgcgtttaatcactgctccattcaaaagagagaaggaggttgtttcaaacctagttgatatcatttgacttccatgctattcacagggctattttatttgaaacaggtataccacagccttaaattgcaagttaatccaggatgttcctaggttggcagttaggaacatgtaattctttggaagggctaaaagtcagctctttaaattatctccatatgaaccttctctccaccttagggtggatccacttatttagtccactgccagtaccacactagaacccgggtggtcactggactccagaaacaacagtagccctctctctgttctgtctctttttgactatctctattctgttcctgaccctgatttctcctgccaagctcaattttgacagctgacaacggcaagccatggcttcccaaaacattattttcaggtcaacttataaatttcaagaacacatttggctccgcttcctgtggtactaagcctacttcttgacagcatttgcctttgttgtaaatagcaaagttcttctagttggatttttgctaagaagtgtgtggatgtggcatgtgacgacatctttagcttggattctagaaaggcactaccattgtgcatttggctaaaggaaacacattttacccgtgaatgccttctatttacaaatgctcagctagcacacaaagctaagtacaagcaataagtactatcctacaatgttactcatttctgaaagcacaaaatgatgactggtatagctttggagatgttttctggaaacccaataaaggaacagatctttgttattccacacctacaaagtcagaagatgcacagtcttttattcatgtttgaacaagcttccttcttgaacaatcaactataaagtgatgtgattctctactagaccaggaactccttgaggacagaatgagggtctaatccatattctaaatccacaccacctggcacaatacatgttgcatggttagggtcaactaagagttggttgaattaatcaataacacacagcaagagaattcacaaagagaggggagtaatcccccagcctcaatcactcggcaagtggaatcgctgggcactgattccagctctgtctcagtgcttgagacagagctgaatgtaatgtgaacatttcaaatgaacaggaaaactagactcacggataagcagtgtagtcatcaagacaacactgtcttggaggtttttctgaagttaaaaccatgctacataagcaataaattatgaaggctgagcatgtgaataaaatttaatgttgtcataaattttataacaaagttaatctgacacatttaatgacatgcataatcattagtatgcagcactgtaatcagacattgataataagcagttcacaccagtgactgtaagagtctttacttgtgttcagccaagccaactgcttggtatatttttctcccttcttagtcgttagttttccatacctacaataactatcagtggtgatgggcttctctgaccatgtgaataatttaatcctcaatgcacagatacagaaacccttgctgaagacagtgtggagcagagaaggctgtctccactccttccacctgaaacacctctgcagatggatatgggagctctgcctacagcccttggacctaaccacttcagtgtgttccagtgagtgtctggacctcggcctgaaagatttttccgaaactaaagaaaatttctctgacctaaagaccttaacctccaccccagaagctctcaccaaggactacagggaactggtggggaaaatccttatcccttactcctcaaggcacagggcagtaatgctgaggcttgtgcgccacacttgctcccagaggtccccagcgggctacctgcggtggtgaatgacctcctaacacgccccttgacggccttcctttccttgcctcacttctccactctcctaccagcattgcagggttcacatcccaaatataccactggcacttgaatcctggtctccaggtctgtttctggaaaaacccaagtaagacattgccccagtaatggggctagatgtctgaggcttcctcaagtatctacctcgaaagctcttactgctgtacacacatgcacatacacacacgtgcgtacaaccagtcacatctaagcaccccgaataccagcctgttgaaggtagcagagagctgcactataagccaaggctgctcccaagagccgctccatcactgaattggcgccccagcaagatgaaggaatgtaatcattggaaggatggagaatgttctctgaatcactgacaaattggaaggggtggagggcaagagtccacctggtggagagatggaaagagcgagagagcctggaatgataatgccattgcttagaaaaggctgctccagatgccatatctacagaaattgtacagcccaaacatctctgagcaataggtctctggtagtcttgatgtctagaccaacaattcccagttcattcttctcagggaaggagccaggatagtccagagactctcattctgctgttagattgaaagggttaggcacaacagccttggcaaagtcacaagggcaaattcacactaaagtgtaaatgacccacaactcctcttctatttttaggttggggaggtgctttagaacataaggaggaactaaagaatattcctgttacatacaaggcagagaaaagggaaactagtggtgacaagacaaatcatccctttgacatttggctggctctacctattacagctctgggggtgaggtgggaacaaaaagatgctgtgtaaagaagtatcttatgccatccctactgtagtgaggtgcagtttagaggggacactgatcaagcagagacccagagtgtttcgttccaagccagaaacagaaatgtataaaacacagcctttccagcatcagaaatgagtagtggtagtggagaactacccaaaacaggaaagaggaccacgtgaggtagagtgtcaaggccctacattccagtgcctctgctcatgactgtaattttgggtaggtcacttaaagtctctggacctcagttttgccatctgtgaaatagggataatactatccagcataaaattggttatgaggctcatgtagggcctgcctgggatgatgtgttgctaatggttaagaacacaacttctggggtctgactggacaggctgaaatccctgcttaacacgttccagcagagccctgggcgatctatttaacttttgttttctcacctgtaagctgagacgaaagtacccactttataagattattccaataattagttgaaataatgcatgcagagaattaagcatggtacttgttatttgttaaactagctattaaaatgtgtaaaatataaagtattgtatggattttaggacaatgcaaagactctttgcttgctgcaatagttcggggccctttcagatggctaaaggcagaatttgtatgtgtaaatatggtgtgcttgtctctgctctggatactgagggcttaccctgttattaaacttatttagtaaatattgaactgtcatgaggcctaacatttagttccagttattagataaaacatttgctttgaatggtatttgaattgccaggttctagattattctggttgacaaactcttcgtattttataaagaggctaaaattggtaagctatcacagaacagatgtgccattttcaaggtatattaaaccatgattcactgtaacattgttcctactggcaacaaattcagagcaggctggactttatttggtgaagaaacattgagtggaagagaaatgacattattttatgtatttacattttcaaattactgtggcttaaacctgttcagccaacattacccaccttcagtctgctaaataaatgattcagtacatttctaatttacagaattttttaacaaaagaaaatgtaatttgatagccaaatcaacgttaaacattatacatttaaaaaaccacaggcaaagacacaaacatgatgacactaacttttgttaaagtatgcttacctatggtttcctctgaggcacgttctttcatgctaagcttccaacataatatgaaaatgaaggagatgcattttgcaaagcaaaacagaccttaagcaaaatattatacttctcaaattaacactgttacaaagttttagaatttaataagttcattaatttaaaagtttggatgtctgagtccttctatcccaaaacaagatcttggagggtcttccacagccatgtaataccatggtcacatgaccctttccaaaattattaatctgaatttactatatgaggataaatctatctttttgaaaatatttaggaaaatgagcttggtatttataaaatgaagctctctttgggtggtatcctaagacacgtcaagccaatcagcctgtaactgtgaaaaaaacattggtaggtacaaaagtggggtgggagaggagtgacttaactttgttaagtgatgggaaagaaacactaatagcattatctcaataaaatgtgatttaaaaaaatttaaaatactaaatcattgaactgacaaagaaatataaatcattcagaaataaactcattaggtcatcaaatcctgttaaatctgcaattaggaagagcaaggtgtacaatccatacatttaaactcacaggctcactttgcacaacgtcaatttactccttaatatgttattaatacgcattttccaaaaggatgtattagtaaatggtacacatctacttcttggcaacatcatataacctggtacaacataagcattcttcttatagttaagaaatgtggatggtatcaaaattagaaaaataaatgccctattatgttgtggtcaggtttaaggcatgtgaattttatcttcatacaaaagattaaaatctagatattaaaaagtagtgcagtatcagtgatgctgcctcagttcccaaaatgtcacatcacaaaaatatcccataattgcctgtagtttattccttggctttcctcttttctctctgcatctttgtaacaattttttaaaagtggaaatataattgttggcaatgctaacagctgtagaaatgattacaagatgtggaaaagcataacaggaatgtcaagaatctgtttctggcagtaatatatatggaacattgttcaggacaaaagaggagaaggaagaaaaaaaggagaggggtttatcatctctaagaattttcaaactaaacctcattgcttaataggaaaaaaagattccatatttaaagttaagtcacctctaactactagctaaagcatgacatcaccagcactggagtcagcggaagtgtgtttttgaaggacagtgttgcaggagaatctggacaggttttagagccaggagagagaaaataattctacctctgacagttgaaggaccttaggcaaatcagtttacctctgctagactacactccaaaatttggacattcaaaaatttgatattaataaccacatgaaagtctcgtgttgaggtgaatatgtatttgttggtgaaagatatgttggtttttaaacagacagcactctgcaattgtaggctattgttttgttttgccagttgtcaaattctatccagctatacacacttgtgtggcctcctaatggtgtttttccagtggctaaaggtttatgaataagacacttttcctaatggaattaacccgatgcttttcttaaacatgtaaccttgagttcaccgcaaaaaacaatgcttcgattagagcaatgcatataataaaggttaccctcgtttcttagacactagacatcattcacaaaaagagaactgcttttgaaagggatgtatttgcactggaaagaatagttttctacttctaattataaatgatttattggtgaaagcaaaacaacagcctgtctgagaggcacttctatgagcatcctcacgtgtgatttgcaaggttgaagaagagggaaaaatgcctcaattgtaccaatggtgagaaaacacccaaagtacaaagcaggtttcaaaaaaaccatactcataaccaaggacaataataaagcaatgtgttgacatatactctataagtcttcctccataaatagtttatagaaattttgtaatttctgtaaatgcatcctataataattttgcatcttgctttttttttacatttaatatcaagtagatttctaaagggcaattatttgaaaattatcccaaatacatggggaaatatacatcaagtgaaaaaatgcagtgggtgatagagatatcaggaagcgcctcaaatatttctcatctcgttggagaaaaacaaacatgttctcatttagaatgagtgggagttacctaattgatttaggcctctatatttaacttctagtcaaaaaaggtagttctatctagcaacaatattatggggaacaaaagaaaaaattaactctctaaatttgcagtagggtcttttcttcagaagtaccaaatcccatctattaccagctccatgcttcaggcctaaaatggatctccctgaagcaatgacagaatttttgccaagtgactaggatataaacaccactttggttgcacagtgagacatatgctccaaagaaaactggttcaaaaacaggcaagtgggtttctacagaataaatgagagccctgtcaatggcttcatcttcagggctttgtgtctgtgcttgcgtggtggctcttgtttcatctatggataatggtggcacacagttttcataattccttacattaatgaactgctataaatttgtttttggtattctagagagtcctaacttcagcttctgggcaatgctgaggaggcaccctatattctagacttaccttttgcaaggtgtactctcagcattgtgggcgatttccatgggagaatattctatttaaagaactactgtcccagcataaaacaaaaaatcatttatgaagatgcaggagactcggaaagctctcaattattgtttgcacaagcacaatgtcacagcctcctttccccattccacaagggggtcaggaagagagtactcagctgtgagaaaagacatacagaagaattcatgtggtcatgagagcgaggacatggccgatcccccaaggaggatgtgtcatacacttcatgagcccaagagtgtgctgtagggtctgaagggcaagatgctggttcactgatgtaaaggagagggaaaaaagcttcaaccaactagaaaaacagtctctatgcatgctatttttgattttaaacacaggtatcaattccttctctcagagagtccattttaaaataggatacatttttaaaggaatatttaaaggacacattcattaaaatttattttaaaaacttttcaaaagaaacaaaaggtatgaattttatttaatccttgaggaaatggttcttttctcacacacataaatcactcattttgtttttctttatctcctttattaatctacattagaaaaataaacttttcatacactaagaacaaggaaaccactctcaattgacaaaatgttccaatccaacacaatgattactttcacctttaatttacaggcagccagattcaaaatccttaaagttgcttaaacttaaaaatgacaatgacaacctaaaaggtataatgttgattggaacagacatttaattggaaaattgatgattttccatttccaattaaatctctagatagaaatgaaaaaaattaaaaatcgtatttaagaaaagccaaatcttgggttgtgaggtatctttttaaggatgtttcagcagaaaaaaacaaaggctctcacaattgtgtagctgcctagattaagtgggtatcctgatcaaggagatgggggatgatttggctttagtattccaatgataaagtttataatgagaataacatgttgctacaaaatccagtctcttcctcagatgccttccacagagggcaggaagctttgtcagttttgtttgctgatgatgcctggttccgtcaacaaataacacctgtcacacggtgggtagtcaatatacatttgttgaataaatatgaaaaaaagaaatgtacaatatgtttgtgaagccaactgtgtgtgcattgctattgaggtacacaaaaagtctttgttttaaatttgagaatgaggactttcaatggaatatatctataaaaatgaaaaaaagacattactgtctggacttttgtacagcaagagaagaaaaaccactagccaagagccaactcacctgataggcctggatcaagcatgcagctgtggagaacacccctgggactctaactctggcactctgcaagctgggtacttgggcaggacagcagcagcactcatgaactgggcagcacctgttggtgagggctgatcacatggattctctcatcccagccttacaatcagtccttcaggtacatactttttctgactttgctgatgaggaaactatgcacagaggttacacagcttaacaaagggttctcacctctcttcaagtggtatttaaatttcttctttcattttccttctggtaacaaagaagtctgtggctcaaaagatgtttctctaagaccccatcctattaggtctctgagctgtgggaagtatttatacaattgcttgtgaatataagatccaggaatttccctaagatccctaacaaaattggtgataagtagtcccacatgttaatccagccacccacggatgacagcacttaccatttctttgataaatgtcaaatgcatttgaagtacctacctgaaatatttgtttaaatgctatctaatctattaattttatatatgtgtgagtctgttttgtataccttctgattataggataaatgtaaataaatccaaagagtaatcaaagctaccactttcaagaagccttctttgtagaaccggaagagtcttaaataggcttttcaggtatgcatctcttattatcgctgaactccaagtcctgcaaggcaggcatcatgtgtgggtcacctttacagtaggcacaggccttaaaacagtgacatgcacattgcaggcactccataaatgtttgctgaattggctaaaccttggtttgttcccataatcaaccaccacaaacagcacacagataattacttcttggaaagattccaactagtgtttgatgttacctacgtggtttttctctcaagatcttaagagcagctctgtaggattacattattttctgttttttttttcctttgaccttaatgtcatctacttcaataacagcttcatacaaaattcctaccagcacataccacagcagattcaaggccttgttttaaaaatggtgccagcttctcttaatttggaagatatattgtctctcctgaacatgggctaagaaaatgtataatttggtattaacataagagctgaagacactttaaatgcattgtttcatttttataagataaaaaaaattttaagaatcaaaatgttatcaacagacttgtccttcattaaaaagtaaaactgcatttgcctacattttatgaaagtgtccaattatgaacaattttgaaatgtaacttttaaaaatgtaaacagcaaaaatgttgtatttaaaataaatctggaaaggcagaaaaacaaaaaatacccagaagacagagtttttggtgaaagttaagatatttcatctttgaacaacttagaatctttcctgcattttatagtctagttccaggcattaatttgaaataaccttggaatcctaaatctaacacccttcggaacaaagtagcttttctcttctgctttatgagcaaatggactaaatactagggaatggtactgtctgggcctttgaaccaagattgaaagagatgaaatcctatatgatatgtataaacattagagaatccattttgatttaataaaaggttgaatttgttctatatcctgtgagaaaatggttcccttttcctgaaaatgttacctcattccaacaatagaaagttggtttttttccagggtgtggtgttggcgggggacagagttgccatgaatatggcatctatgaagactgctgttatattcatttctcaaaatgcactgtggtaggaaattcagaacgcagtgagagaaaataaatgtttgacttcaaaatataaggccgcatttaaagcagaaggtaaagtatagaacagttgacagtataaattctttatctgcaatcttgcagttccctaaatctctgtaacacatcacttttaaaagcctcagataagtggttctataataatttaccaataattcaacccctcaaaagtcttagcaagttaaaccttataatcttacattttagaaatgacccaacttgatccttttattcttcagaatatctctctcaaattttcatttgtttttcattaattgatgaataatgagacattttaggtacctgtccacaaagaaatgaaattttcactttccaggaacctaacaaatgaaaagatagaaatcaattccaacagaatattaccaaagaaatcttttagaatggactgttaaaattatttatttgtatttatctggctctactatttgtggtacatttccacttcaaagctaaacctcaaataacatcatagtgagtggttgacttcatgtttaactgagatcttgaagactgaaaaagaccacgacaaacacacatctattttcttggctactgcatccgtgttcatcaccattctgatagtctgcaatgtattgcagctcaccctttgggaaggactaaagtagacatctgtttgttctgcttactcagcattcctaccctaattttcctttggagaacccctttattctagaccacgtgaagctaatgccaaaccccattccaggggatgcacctgaatccaacctccatcatctaaacagtgccttctccacgttcagagaagagcaagtgactcaaactgccctcataagaacagacctgggacttctgctgcaaatattgaagagtaagtactcttttttcttgctaggactaagctggtagtaccttctatgaggctatcatatggaaacaacttgtctgaaaatgaagccacaactagaaaacagatcctggtaacccggattgatggatccagccctaccttaaatggcaagacctaacccgaggctttttgcatcaaccaataaagtccttaagccagtttgagttggttttgtcacttgcagctaaaagaattctgactctaacaatgtgacaatagcaaaaataaacataactgcttttgaggtttctaatggattttcctccctatatacatgatttcatttaatcctcacaattcaggaaagcacatatctattaacattaaattaatattcattattttgaacacatgctatgtggataagggatgaggaaagccaaggaagtaatcaacgtgaaatctcacttatatgggagggaagtggaggttacatatctcagggcacttaacagatatcatcaaatgaaagaataaacagtgtgtgggagaggcagtaggtgattcttcatcaattcctggatgaaaaattaggagataatgaactccgaacaggcagcctaatgagaatggctcaagcaacaggacatagagagggagttaggttagacatggggttcttgggaattttcacctcgtgggggggcgggggggtcgtgcagctgttgtcagtgggaaagggaaaaaggaaaaggctgagtttggaaggcagggagggaggagacaatgtgagtcagtgaaaaagggcccttagaatgacaagtctggaccagagagaggctaagactgaaaatacaagttgggtaaccactggcatacagatggcagttcaggcttgggcactgcccaccagagcctcagcatgaagagaagagggggaggctggccaccacctccctctaggtaatcgtcatcctgatgctgagctcctgaaaacaggctctttcactcgccccatctcttgctcttgattgcaacccggcattcaggaggcaccctgtaatatctgtggagtgaccgacaacacagcgccagggcactgagaagatcccagggcgccagggactggttctacaagggtgcccctcccggtcccctccagcgcgccgccagagctgccagtcttggctgctacacgggaggcagcctcattatgcagctctcacctcttaaattagttcatgctctcacattaggtgtaatcacagcttgcaacgctttctggggatgtctcagaaagatctgagttgaaaaaatatttttgtgtcattttaatttaaagtaaaattgctgcttcttccccgcccctttctttcctcctggcccacccagcgaccctggccggccgtgctcaacgggggcgggggtcggaggtgagatttcctccacataattccttaaacagctatcaactaagtctcaaagaaaaaaaaaagagatctagaagcagagacgtggctgctggcgatcccaaagctggtgttcgctcttgggggagagcgtaccctgggggaggccgggaggccgggccagaggctagcccagaggcagagggcaggagcgctcagccggcgccccgcgtctctccagctcccgacgctgcgctggctccgctgagcacgccaggatcaaggtcgcctggtggggaccggagcgccaggagcctgtgggaagcgttccagccggcctctgactgggatccggcgccgcgtttctgctttggacttgactgacaggtccccccgccctcccgccgccctactaccagcctgggttcatccttcagggctacgtctaccgcacccgggctggaaagcctggagcgcgcccttcctctcctcatcttctcagctctcctttctccctgccacttggcaaagctgcattttgactttcacgttttggactacgtgtgtgtagttccaagtccatgcgtggcacgaaaatccacttagggtaaaaattattctcgaaaaatcgcccatctcaggatctggtgtctacactcaaggctaggaggtgcaggtacgggtgcgtaaagcatgccgtaagggtgcacagtaaataaaaagtacggatgcaaaatgtaaattttaagtgcaaaacagaaaagcagtactcgttgccgccccgcacgctgggttttaaggggcacgaaggtgggcctcggctgcttttgctcagccccgcgtcctcagcgcccggcccagtacccggtactccgtaggggttcaatgatctcccctgaataagtgaacgaattaacaaatgaatgaatgaccgctcgatccgacctccgcggccggcagagcagtcgctggagaggcgggagagagcgagaggccaagctccaccatcgcggccgccggctggggcagagggacacggagacactcggcgccccggctccgcaccgagtccccg

SEQ ID NO: 12760 - RNA, 15292 nt, Homo sapiens
  source 1..15292: mol_type = other RNA
gatctcactttgttgcccaggctggtcttaaactcctggcctcaagtgatccccttgtttcagccccgcaaagtgctgggattacaggtgtgagccaccatgcccgtgcccagccacctcatgagtcttgatggggggcagagaccaacaactccacagaagccagatgcttgctttcccagcctctcttgcagctagggcttgggcatgtgatccaggctcagccaatcagatggcactgactcttggcatgacatgggctaaggaggggctgcagggaatccatttgggctggggtggcagctgcactgggagcgacatcagtttccagagggagcagcagaatctggcatcaggcttggggcgtggtaggtgcaaccagactctgcacccagcagcagtggcagaatgggttctctgtggagagtctgtgtattgctccttccgctgaggccaccagcatctgcctccatgaacccctcagagcctgtgagcaactcaacagccttgaattttttcccttcctgtttgaatgagccagggttgtttcactgcttgaactaagagccgttcctgacatgaaaactaagccacatctttttgacccaaagattctggcatcctaaaatacccatctcattttaagttaaaaataaatccatgtttgagcatctactgtttcagttactgtgctaggtgttacaaagctaactaagagtgacaagtaaataactatcatcaccatgataaacagagaatggaaccctggtttttggaatacagacacaaaatgattaattctgcctggaagcgttttggaacatttcagagaggtagtgagctgggccaagagaagagcatacgcaaggaatggtggcatgaagttgcctggtgtgtcctgagaagaaagatgggctaagaaggactggggtagggcagagaagggggtcactggaggtgaggctgggaaagtgagccaaggctcaaatgcaaactgtctgaacttcattttctgtgcaagcaggagaagccgctgacatgggtttggaagatggactgaagccggagaaaaatggaagcaagaaaccctctcacaagaggccataaccacaaccaagtccatgagattgaaaaggaaggcagatatttgaaaaatatttaaagagatgtgaggggtaggacaggcacagtggctcatgcctgtagtcccagcactttgggaggccgaggtgggcagatccacgaggtcaggagatcaagaccatcctaacatggtaaaaccccatctctactaacaatacaaaaaattagtcaggtgtggtggcacgtgcctgtagtcccagctactcaggaggctgaggcaggagaatcgcttgaacctgggaggcggaggttgcagtgagccgagattgtgccactgcaccctagcctaggcaacagagcaagactctgtctcaaaaaaaataaaaaaaaaaaaaagagagaaagagagagagagatgaggagttgctgcactgctgggtgtggagagccgaggaggattcaaagatggtcctgaagtcccagctggaagaagtaggcggcagcaatgtttttaatactgtaaattcatcacgtagcacaggtttggggtggagaaagaaaaattgcattggcttcagggcatgcccagatctttcctcatcttaggcgtttgctaatacatgcattttctaagctgatgtcttgcgtttaatcactgctccattcaaaagagagaaggaggttgtttcaaacctagttgatatcatttgacttccatgctattcacagggctattttatttgaaacaggtataccacagccttaaattgcaagttaatccaggatgttcctaggttggcagttaggaacatgtaattctttggaagggctaaaagtcagctctttaaattatctccatatgaaccttctctccaccttagggtggatccacttatttagtccactgccagtaccacactagaacccgggtggtcactggactccagaaacaacagtagccctctctctgttctgtctctttttgactatctctattctgttcctgaccctgatttctcctgccaagctcaattttgacagctgacaacggcaagccatggcttcccaaaacattattttcaggtcaacttataaatttcaagaacacatttggctccgcttcctgtggtactaagcctacttcttgacagcatttgcctttgttgtaaatagcaaagttcttctagttggatttttgctaagaagtgtgtggatgtggcatgtgacgacatctttagcttggattctagaaaggcactaccattgtgcatttggctaaaggaaacacattttacccgtgaatgccttctatttacaaatgctcagctagcacacaaagctaagtacaagcaataagtactatcctacaatgttactcatttctgaaagcacaaaatgatgactggtatagctttggagatgttttctggaaacccaataaaggaacagatctttgttattccacacctacaaagtcagaagatgcacagtcttttattcatgtttgaacaagcttccttcttgaacaatcaactataaagtgatgtgattctctactagaccaggaactccttgaggacagaatgagggtctaatccatattctaaatccacaccacctggcacaatacatgttgcatggttagggtcaactaagagttggttgaattaatcaataacacacagcaagagaattcacaaagagaggggagtaatcccccagcctcaatcactcggcaagtggaatcgctgggcactgattccagctctgtctcagtgcttgagacagagctgaatgtaatgtgaacatttcaaatgaacaggaaaactagactcacggataagcagtgtagtcatcaagacaacactgtcttggaggtttttctgaagttaaaaccatgctacataagcaataaattatgaaggctgagcatgtgaataaaatttaatgttgtcataaattttataacaaagttaatctgacacatttaatgacatgcataatcattagtatgcagcactgtaatcagacattgataataagcagttcacaccagtgactgtaagagtctttacttgtgttcagccaagccaactgcttggtatatttttctcccttcttagtcgttagttttccatacctacaataactatcagtggtgatgggcttctctgaccatgtgaataatttaatcctcaatgcacagatacagaaacccttgctgaagacagtgtggagcagagaaggctgtctccactccttccacctgaaacacctctgcagatggatatgggagctctgcctacagcccttggacctaaccacttcagtgtgttccagtgagtgtctggacctcggcctgaaagatttttccgaaactaaagaaaatttctctgacctaaagaccttaacctccaccccagaagctctcaccaaggactacagggaactggtggggaaaatccttatcccttactcctcaaggcacagggcagtaatgctgaggcttgtgcgccacacttgctcccagaggtccccagcgggctacctgcggtggtgaatgacctcctaacacgccccttgacggccttcctttccttgcctcacttctccactctcctaccagcattgcagggttcacatcccaaatataccactggcacttgaatcctggtctccaggtctgtttctggaaaaacccaagtaagacattgccccagtaatggggctagatgtctgaggcttcctcaagtatctacctcgaaagctcttactgctgtacacacatgcacatacacacacgtgcgtacaaccagtcacatctaagcaccccgaataccagcctgttgaaggtagcagagagctgcactataagccaaggctgctcccaagagccgctccatcactgaattggcgccccagcaagatgaaggaatgtaatcattggaaggatggagaatgttctctgaatcactgacaaattggaaggggtggagggcaagagtccacctggtggagagatggaaagagcgagagagcctggaatgataatgccattgcttagaaaaggctgctccagatgccatatctacagaaattgtacagcccaaacatctctgagcaataggtctctggtagtcttgatgtctagaccaacaattcccagttcattcttctcagggaaggagccaggatagtccagagactctcattctgctgttagattgaaagggttaggcacaacagccttggcaaagtcacaagggcaaattcacactaaagtgtaaatgacccacaactcctcttctatttttaggttggggaggtgctttagaacataaggaggaactaaagaatattcctgttacatacaaggcagagaaaagggaaactagtggtgacaagacaaatcatccctttgacatttggctggctctacctattacagctctgggggtgaggtgggaacaaaaagatgctgtgtaaagaagtatcttatgccatccctactgtagtgaggtgcagtttagaggggacactgatcaagcagagacccagagtgtttcgttccaagccagaaacagaaatgtataaaacacagcctttccagcatcagaaatgagtagtggtagtggagaactacccaaaacaggaaagaggaccacgtgaggtagagtgtcaaggccctacattccagtgcctctgctcatgactgtaattttgggtaggtcacttaaagtctctggacctcagttttgccatctgtgaaatagggataatactatccagcataaaattggttatgaggctcatgtagggcctgcctgggatgatgtgttgctaatggttaagaacacaacttctggggtctgactggacaggctgaaatccctgcttaacacgttccagcagagccctgggcgatctatttaacttttgttttctcacctgtaagctgagacgaaagtacccactttataagattattccaataattagttgaaataatgcatgcagagaattaagcatggtacttgttatttgttaaactagctattaaaatgtgtaaaatataaagtattgtatggattttaggacaatgcaaagactctttgcttgctgcaatagttcggggccctttcagatggctaaaggcagaatttgtatgtgtaaatatggtgtgcttgtctctgctctggatactgagggcttaccctgttattaaacttatttagtaaatattgaactgtcatgaggcctaacatttagttccagttattagataaaacatttgctttgaatggtatttgaattgccaggttctagattattctggttgacaaactcttcgtattttataaagaggctaaaattggtaagctatcacagaacagatgtgccattttcaaggtatattaaaccatgattcactgtaacattgttcctactggcaacaaattcagagcaggctggactttatttggtgaagaaacattgagtggaagagaaatgacattattttatgtatttacattttcaaattactgtggcttaaacctgttcagccaacattacccaccttcagtctgctaaataaatgattcagtacatttctaatttacagaattttttaacaaaagaaaatgtaatttgatagccaaatcaacgttaaacattatacatttaaaaaaccacaggcaaagacacaaacatgatgacactaacttttgttaaagtatgcttacctatggtttcctctgaggcacgttctttcatgctaagcttccaacataatatgaaaatgaaggagatgcattttgcaaagcaaaacagaccttaagcaaaatattatacttctcaaattaacactgttacaaagttttagaatttaataagttcattaatttaaaagtttggatgtctgagtccttctatcccaaaacaagatcttggagggtcttccacagccatgtaataccatggtcacatgaccctttccaaaattattaatctgaatttactatatgaggataaatctatctttttgaaaatatttaggaaaatgagcttggtatttataaaatgaagctctctttgggtggtatcctaagacacgtcaagccaatcagcctgtaactgtgaaaaaaacattggtaggtacaaaagtggggtgggagaggagtgacttaactttgttaagtgatgggaaagaaacactaatagcattatctcaataaaatgtgatttaaaaaaatttaaaatactaaatcattgaactgacaaagaaatataaatcattcagaaataaactcattaggtcatcaaatcctgttaaatctgcaattaggaagagcaaggtgtacaatccatacatttaaactcacaggctcactttgcacaacgtcaatttactccttaatatgttattaatacgcattttccaaaaggatgtattagtaaatggtacacatctacttcttggcaacatcatataacctggtacaacataagcattcttcttatagttaagaaatgtggatggtatcaaaattagaaaaataaatgccctattatgttgtggtcaggtttaaggcatgtgaattttatcttcatacaaaagattaaaatctagatattaaaaagtagtgcagtatcagtgatgctgcctcagttcccaaaatgtcacatcacaaaaatatcccataattgcctgtagtttattccttggctttcctcttttctctctgcatctttgtaacaattttttaaaagtggaaatataattgttggcaatgctaacagctgtagaaatgattacaagatgtggaaaagcataacaggaatgtcaagaatctgtttctggcagtaatatatatggaacattgttcaggacaaaagaggagaaggaagaaaaaaaggagaggggtttatcatctctaagaattttcaaactaaacctcattgcttaataggaaaaaaagattccatatttaaagttaagtcacctctaactactagctaaagcatgacatcaccagcactggagtcagcggaagtgtgtttttgaaggacagtgttgcaggagaatctggacaggttttagagccaggagagagaaaataattctacctctgacagttgaaggaccttaggcaaatcagtttacctctgctagactacactccaaaatttggacattcaaaaatttgatattaataaccacatgaaagtctcgtgttgaggtgaatatgtatttgttggtgaaagatatgttggtttttaaacagacagcactctgcaattgtaggctattgttttgttttgccagttgtcaaattctatccagctatacacacttgtgtggcctcctaatggtgtttttccagtggctaaaggtttatgaataagacacttttcctaatggaattaacccgatgcttttcttaaacatgtaaccttgagttcaccgcaaaaaacaatgcttcgattagagcaatgcatataataaaggttaccctcgtttcttagacactagacatcattcacaaaaagagaactgcttttgaaagggatgtatttgcactggaaagaatagttttctacttctaattataaatgatttattggtgaaagcaaaacaacagcctgtctgagaggcacttctatgagcatcctcacgtgtgatttgcaaggttgaagaagagggaaaaatgcctcaattgtaccaatggtgagaaaacacccaaagtacaaagcaggtttcaaaaaaaccatactcataaccaaggacaataataaagcaatgtgttgacatatactctataagtcttcctccataaatagtttatagaaattttgtaatttctgtaaatgcatcctataataattttgcatcttgctttttttttacatttaatatcaagtagatttctaaagggcaattatttgaaaattatcccaaatacatggggaaatatacatcaagtgaaaaaatgcagtgggtgatagagatatcaggaagcgcctcaaatatttctcatctcgttggagaaaaacaaacatgttctcatttagaatgagtgggagttacctaattgatttaggcctctatatttaacttctagtcaaaaaaggtagttctatctagcaacaatattatggggaacaaaagaaaaaattaactctctaaatttgcagtagggtcttttcttcagaagtaccaaatcccatctattaccagctccatgcttcaggcctaaaatggatctccctgaagcaatgacagaatttttgccaagtgactaggatataaacaccactttggttgcacagtgagacatatgctccaaagaaaactggttcaaaaacaggcaagtgggtttctacagaataaatgagagccctgtcaatggcttcatcttcagggctttgtgtctgtgcttgcgtggtggctcttgtttcatctatggataatggtggcacacagttttcataattccttacattaatgaactgctataaatttgtttttggtattctagagagtcctaacttcagcttctgggcaatgctgaggaggcaccctatattctagacttaccttttgcaaggtgtactctcagcattgtgggcgatttccatgggagaatattctatttaaagaactactgtcccagcataaaacaaaaaatcatttatgaagatgcaggagactcggaaagctctcaattattgtttgcacaagcacaatgtcacagcctcctttccccattccacaagggggtcaggaagagagtactcagctgtgagaaaagacatacagaagaattcatgtggtcatgagagcgaggacatggccgatcccccaaggaggatgtgtcatacacttcatgagcccaagagtgtgctgtagggtctgaagggcaagatgctggttcactgatgtaaaggagagggaaaaaagcttcaaccaactagaaaaacagtctctatgcatgctatttttgattttaaacacaggtatcaattccttctctcagagagtccattttaaaataggatacatttttaaaggaatatttaaaggacacattcattaaaatttattttaaaaacttttcaaaagaaacaaaaggtatgaattttatttaatccttgaggaaatggttcttttctcacacacataaatcactcattttgtttttctttatctcctttattaatctacattagaaaaataaacttttcatacactaagaacaaggaaaccactctcaattgacaaaatgttccaatccaacacaatgattactttcacctttaatttacaggcagccagattcaaaatccttaaagttgcttaaacttaaaaatgacaatgacaacctaaaaggtataatgttgattggaacagacatttaattggaaaattgatgattttccatttccaattaaatctctagatagaaatgaaaaaaattaaaaatcgtatttaagaaaagccaaatcttgggttgtgaggtatctttttaaggatgtttcagcagaaaaaaacaaaggctctcacaattgtgtagctgcctagattaagtgggtatcctgatcaaggagatgggggatgatttggctttagtattccaatgataaagtttataatgagaataacatgttgctacaaaatccagtctcttcctcagatgccttccacagagggcaggaagctttgtcagttttgtttgctgatgatgcctggttccgtcaacaaataacacctgtcacacggtgggtagtcaatatacatttgttgaataaatatgaaaaaaagaaatgtacaatatgtttgtgaagccaactgtgtgtgcattgctattgaggtacacaaaaagtctttgttttaaatttgagaatgaggactttcaatggaatatatctataaaaatgaaaaaaagacattactgtctggacttttgtacagcaagagaagaaaaaccactagccaagagccaactcacctgataggcctggatcaagcatgcagctgtggagaacacccctgggactctaactctggcactctgcaagctgggtacttgggcaggacagcagcagcactcatgaactgggcagcacctgttggtgagggctgatcacatggattctctcatcccagccttacaatcagtccttcaggtacatactttttctgactttgctgatgaggaaactctcttcaagtggtatttaaatttcttctttcattttccttctggtaacaaagaagtctgtggctcaaaagatgtttctctaagaccccatcctattaggtctctgagctgtgggaagtatttatacaattgcttgtgaatataagatccaggaatttccctaagatccctaacaaaattggtgataagtagtcccacatgttaatccagccacccacggatgacagcacttaccatttctttgataaatgtcaaatgcatttgaagtacctacctgaaatatttgtttaaatgctatctaatctattaattttatatatgtgtgagtctgttttgtataccttctgattataggataaatgtaaataaatccaaagagtaatcaaagctaccactttcaagaagccttctttgtagaaccggaagagtcttaaataggcttttcaggtatgcatctcttattatcgctgaactccaagtcctgcaaggcaggcatcatgtgtgggtcacctttacagtaggcacaggccttaaaacagtgacatgcacattgcaggcactccataaatgtttgctgaattggctaaaccttggtttgttcccataatcaaccaccacaaacagcacacagataattacttcttggaaagattccaactagtgtttgatgttacctacgtggtttttctctcaagatcttaagagcagctctgtaggattacattattttctgttttttttttcctttgaccttaatgtcatctacttcaataacagcttcatacaaaattcctaccagcacataccacagcagattcaaggccttgttttaaaaatggtgccagcttctcttaatttggaagatatattgtctctcctgaacatgggctaagaaaatgtataatttggtattaacataagagctgaagacactttaaatgcattgtttcatttttataagataaaaaaaattttaagaatcaaaatgttatcaacagacttgtccttcattaaaaagtaaaactgcatttgcctacattttatgaaagtgtccaattatgaacaattttgaaatgtaacttttaaaaatgtaaacagcaaaaatgttgtatttaaaataaatctggaaaggcagaaaaacaaaaaatacccagaagacagagtttttggtgaaagttaagatatttcatctttgaacaacttagaatctttcctgcattttatagtctagttccaggcattaatttgaaataaccttggaatcctaaatctaacacccttcggaacaaagtagcttttctcttctgctttatgagcaaatggactaaatactagggaatggtactgtctgggcctttgaaccaagattgaaagagatgaaatcctatatgatatgtataaacattagagaatccattttgatttaataaaaggttgaatttgttctatatcctgtgagaaaatggttcccttttcctgaaaatgttacctcattccaacaatagaaagttggtttttttccagggtgtggtgttggcgggggacagagttgccatgaatatggcatctatgaagactgctgttatattcatttctcaaaatgcactgtggtaggaaattcagaacgcagtgagagaaaataaatgtttgacttcaaaatataaggccgcatttaaagcagaaggtaaagtatagaacagttgacagtataaattctttatctgcaatcttgcagttccctaaatctctgtaacacatcacttttaaaagcctcagataagtggttctataataatttaccaataattcaacccctcaaaagtcttagcaagttaaaccttataatcttacattttagaaatgacccaacttgatccttttattcttcagaatatctctctcaaattttcatttgtttttcattaattgatgaataatgagacattttaggtacctgtccacaaagaaatgaaattttcactttccaggaacctaacaaatgaaaagatagaaatcaattccaacagaatattaccaaagaaatcttttagaatggactgttaaaattatttatttgtatttatctggctctactatttgtggtacatttccacttcaaagctaaacctcaaataacatcatagtgagtggttgacttcatgtttaactgagatcttgaagactgaaaaagaccacgacaaacacacatctattttcttggctactgcatccgtgttcatcaccattctgatagtctgcaatgtattgcagctcaccctttgggaaggactaaagtagacatctgtttgttctgcttactcagcattcctaccctaattttcctttggagaacccctttattctagaccacgtgaagctaatgccaaaccccattccaggggatgcacctgaatccaacctccatcatctaaacagtgccttctccacgttcagagaagagcaagtgactcaaactgccctcataagaacagacctgggacttctgctgcaaatattgaagagtaagtactcttttttcttgctaggactaagctggtagtaccttctatgaggctatcatatggaaacaacttgtctgaaaatgaagccacaactagaaaacagatcctggtaacccggattgatggatccagccctaccttaaatggcaagacctaacccgaggctttttgcatcaaccaataaagtccttaagccagtttgagttggttttgtcacttgcagctaaaagaattctgactctaacaatgtgacaatagcaaaaataaacataactgcttttgaggtttctaatggattttcctccctatatacatgatttcatttaatcctcacaattcaggaaagcacatatctattaacattaaattaatattcattattttgaacacatgctatgtggataagggatgaggaaagccaaggaagtaatcaacgtgaaatctcacttatatgggagggaagtggaggttacatatctcagggcacttaacagatatcatcaaatgaaagaataaacagtgtgtgggagaggcagtaggtgattcttcatcaattcctggatgaaaaattaggagataatgaactccgaacaggcagcctaatgagaatggctcaagcaacaggacatagagagggagttaggttagacatggggttcttgggaattttcacctcgtgggggggcgggggggtcgtgcagctgttgtcagtgggaaagggaaaaaggaaaaggctgagtttggaaggcagggagggaggagacaatgtgagtcagtgaaaaagggcccttagaatgacaagtctggaccagagagaggctaagactgaaaatacaagttgggtaaccactggcatacagatggcagttcaggcttgggcactgcccaccagagcctcagcatgaagagaagagggggaggctggccaccacctccctctaggtaatcgtcatcctgatgctgagctcctgaaaacaggctctttcactcgccccatctcttgctcttgattgcaacccggcattcaggaggcaccctgtaatatctgtggagtgaccgacaacacagcgccagggcactgagaagatcccagggcgccagggactggttctacaagggtgcccctcccggtcccctccagcgcgccgccagagctgccagtcttggctgctacacgggaggcagcctcattatgcagctctcacctcttaaattagttcatgctctcacattaggtgtaatcacagcttgcaacgctttctggggatgtctcagaaagatctgagttgaaaaaatatttttgtgtcattttaatttaaagtaaaattgctgcttcttccccgcccctttctttcctcctggcccacccagcgaccctggccggccgtgctcaacgggggcgggggtcggaggtgagatttcctccacataattccttaaacagctatcaactaagtctcaaagaaaaaaaaaagagatctagaagcagagacgtggctgctggcgatcccaaagctggtgttcgctcttgggggagagcgtaccctgggggaggccgggaggccgggccagaggctagcccagaggcagagggcaggagcgctcagccggcgccccgcgtctctccagctcccgacgctgcgctggctccgctgagcacgccaggatcaaggtcgcctggtggggaccggagcgccaggagcctgtgggaagcgttccagccggcctctgactgggatccggcgccgcgtttctgctttggacttgactgacaggtccccccgccctcccgccgccctactaccagcctgggttcatccttcagggctacgtctaccgcacccgggctggaaagcctggagcgcgcccttcctctcctcatcttctcagctctcctttctccctgccacttggcaaagctgcattttgactttcacgttttggactacgtgtgtgtagttccaagtccatgcgtggcacgaaaatccacttagggtaaaaattattctcgaaaaatcgcccatctcaggatctggtgtctacactcaaggctaggaggtgcaggtacgggtgcgtaaagcatgccgtaagggtgcacagtaaataaaaagtacggatgcaaaatgtaaattttaagtgcaaaacagaaaagcagtactcgttgccgccccgcacgctgggttttaaggggcacgaaggtgggcctcggctgcttttgctcagccccgcgtcctcagcgcccggcccagtacccggtactccgtaggggttcaatgatctcccctgaataagtgaacgaattaacaaatgaatgaatgaccgctcgatccgacctccgcggccggcagagcagtcgctggagaggcgggagagagcgagaggccaagctccaccatcgcggccgccggctggggcagagggacacggagacactcggcgccccggctccgcaccgagtccccg

SEQ ID NO: 12761 - RNA, 15386 nt, Homo sapiens
  source 1..15386: mol_type = other RNA
gatctcactttgttgcccaggctggtcttaaactcctggcctcaagtgatccccttgtttcagccccgcaaagtgctgggattacaggtgtgagccaccatgcccgtgcccagccacctcatgagtcttgatggggggcagagaccaacaactccacagaagccagatgcttgctttcccagcctctcttgcagctagggcttgggcatgtgatccaggctcagccaatcagatggcactgactcttggcatgacatgggctaaggaggggctgcagggaatccatttgggctggggtggcagctgcactgggagcgacatcagtttccagagggagcagcagaatctggcatcaggcttggggcgtggtaggtgcaaccagactctgcacccagcagcagtggcagaatgggttctctgtggagagtctgtgtattgctccttccgctgaggccaccagcatctgcctccatgaacccctcagagcctgtgagcaactcaacagccttgaattttttcccttcctgtttgaatgagccagggttgtttcactgcttgaactaagagccgttcctgacatgaaaactaagccacatctttttgacccaaagattctggcatcctaaaatacccatctcattttaagttaaaaataaatccatgtttgagcatctactgtttcagttactgtgctaggtgttacaaagctaactaagagtgacaagtaaataactatcatcaccatgataaacagagaatggaaccctggtttttggaatacagacacaaaatgattaattctgcctggaagcgttttggaacatttcagagaggtagtgagctgggccaagagaagagcatacgcaaggaatggtggcatgaagttgcctggtgtgtcctgagaagaaagatgggctaagaaggactggggtagggcagagaagggggtcactggaggtgaggctgggaaagtgagccaaggctcaaatgcaaactgtctgaacttcattttctgtgcaagcaggagaagccgctgacatgggtttggaagatggactgaagccggagaaaaatggaagcaagaaaccctctcacaagaggccataaccacaaccaagtccatgagattgaaaaggaaggcagatatttgaaaaatatttaaagagatgtgaggggtaggacaggcacagtggctcatgcctgtagtcccagcactttgggaggccgaggtgggcagatccacgaggtcaggagatcaagaccatcctaacatggtaaaaccccatctctactaacaatacaaaaaattagtcaggtgtggtggcacgtgcctgtagtcccagctactcaggaggctgaggcaggagaatcgcttgaacctgggaggcggaggttgcagtgagccgagattgtgccactgcaccctagcctaggcaacagagcaagactctgtctcaaaaaaaataaaaaaaaaaaaaagagagaaagagagagagagatgaggagttgctgcactgctgggtgtggagagccgaggaggattcaaagatggtcctgaagtcccagctggaagaagtaggcggcagcaatgtttttaatactgtaaattcatcacgtagcacaggtttggggtggagaaagaaaaattgcattggcttcagggcatgcccagatctttcctcatcttaggcgtttgctaatacatgcattttctaagctgatgtcttgcgtttaatcactgctccattcaaaagagagaaggaggttgtttcaaacctagttgatatcatttgacttccatgctattcacagggctattttatttgaaacaggtataccacagccttaaattgcaagttaatccaggatgttcctaggttggcagttaggaacatgtaattctttggaagggctaaaagtcagctctttaaattatctccatatgaaccttctctccaccttagggtggatccacttatttagtccactgccagtaccacactagaacccgggtggtcactggactccagaaacaacagtagccctctctctgttctgtctctttttgactatctctattctgttcctgaccctgatttctcctgccaagctcaattttgacagctgacaacggcaagccatggcttcccaaaacattattttcaggtcaacttataaatttcaagaacacatttggctccgcttcctgtggtactaagcctacttcttgacagcatttgcctttgttgtaaatagcaaagttcttctagttggatttttgctaagaagtgtgtggatgtggcatgtgacgacatctttagcttggattctagaaaggcactaccattgtgcatttggctaaaggaaacacattttacccgtgaatgccttctatttacaaatgctcagctagcacacaaagctaagtacaagcaataagtactatcctacaatgttactcatttctgaaagcacaaaatgatgactggtatagctttggagatgttttctggaaacccaataaaggaacagatctttgttattccacacctacaaagtcagaagatgcacagtcttttattcatgtttgaacaagcttccttcttgaacaatcaactataaagtgatgtgattctctactagaccaggaactccttgaggacagaatgagggtctaatccatattctaaatccacaccacctggcacaatacatgttgcatggttagggtcaactaagagttggttgaattaatcaataacacacagcaagagaattcacaaagagaggggagtaatcccccagcctcaatcactcggcaagtggaatcgctgggcactgattccagctctgtctcagtgcttgagacagagctgaatgtaatgtgaacatttcaaatgaacaggaaaactagactcacggataagcagtgtagtcatcaagacaacactgtcttggaggtttttctgaagttaaaaccatgctacataagcaataaattatgaaggctgagcatgtgaataaaatttaatgttgtcataaattttataacaaagttaatctgacacatttaatgacatgcataatcattagtatgcagcactgtaatcagacattgataataagcagttcacaccagtgactgtaagagtctttacttgtgttcagccaagccaactgcttggtatatttttctcccttcttagtcgttagttttccatacctacaataactatcagtggtgatgggcttctctgaccatgtgaataatttaatcctcaatgcacagatacagaaacccttgctgaagacagtgtggagcagagaaggctgtctccactccttccacctgaaacacctctgcagatggatatgggagctctgcctacagcccttggacctaaccacttcagtgtgttccagtgagtgtctggacctcggcctgaaagatttttccgaaactaaagaaaatttctctgacctaaagaccttaacctccaccccagaagctctcaccaaggactacagggaactggtggggaaaatccttatcccttactcctcaaggcacagggcagtaatgctgaggcttgtgcgccacacttgctcccagaggtccccagcgggctacctgcggtggtgaatgacctcctaacacgccccttgacggccttcctttccttgcctcacttctccactctcctaccagcattgcagggttcacatcccaaatataccactggcacttgaatcctggtctccaggtctgtttctggaaaaacccaagtaagacattgccccagtaatggggctagatgtctgaggcttcctcaagtatctacctcgaaagctcttactgctgtacacacatgcacatacacacacgtgcgtacaaccagtcacatctaagcaccccgaataccagcctgttgaaggtagcagagagctgcactataagccaaggctgctcccaagagccgctccatcactgaattggcgccccagcaagatgaaggaatgtaatcattggaaggatggagaatgttctctgaatcactgacaaattggaaggggtggagggcaagagtccacctggtggagagatggaaagagcgagagagcctggaatgataatgccattgcttagaaaaggctgctccagatgccatatctacagaaattgtacagcccaaacatctctgagcaataggtctctggtagtcttgatgtctagaccaacaattcccagttcattcttctcagggaaggagccaggatagtccagagactctcattctgctgttagattgaaagggttaggcacaacagccttggcaaagtcacaagggcaaattcacactaaagtgtaaatgacccacaactcctcttctatttttaggttggggaggtgctttagaacataaggaggaactaaagaatattcctgttacatacaaggcagagaaaagggaaactagtggtgacaagacaaatcatccctttgacatttggctggctctacctattacagctctgggggtgaggtgggaacaaaaagatgctgtgtaaagaagtatcttatgccatccctactgtagtgaggtgcagtttagaggggacactgatcaagcagagacccagagtgtttcgttccaagccagaaacagaaatgtataaaacacagcctttccagcatcagaaatgagtagtggtagtggagaactacccaaaacaggaaagaggaccacgtgaggtagagtgtcaaggccctacattccagtgcctctgctcatgactgtaattttgggtaggtcacttaaagtctctggacctcagttttgccatctgtgaaatagggataatactatccagcataaaattggttatgaggctcatgtagggcctgcctgggatgatgtgttgctaatggttaagaacacaacttctggggtctgactggacaggctgaaatccctgcttaacacgttccagcagagccctgggcgatctatttaacttttgttttctcacctgtaagctgagacgaaagtacccactttataagattattccaataattagttgaaataatgcatgcagagaattaagcatggtacttgttatttgttaaactagctattaaaatgtgtaaaatataaagtattgtatggattttaggacaatgcaaagactctttgcttgctgcaatagttcggggccctttcagatggctaaaggcagaatttgtatgtgtaaatatggtgtgcttgtctctgctctggatactgagggcttaccctgttattaaacttatttagtaaatattgaactgtcatgaggcctaacatttagttccagttattagataaaacatttgctttgaatggtatttgaattgccaggttctagattattctggttgacaaactcttcgtattttataaagaggctaaaattggtaagctatcacagaacagatgtgccattttcaaggtatattaaaccatgattcactgtaacattgttcctactggcaacaaattcagagcaggctggactttatttggtgaagaaacattgagtggaagagaaatgacattattttatgtatttacattttcaaattactgtggcttaaacctgttcagccaacattacccaccttcagtctgctaaataaatgattcagtacatttctaatttacagaattttttaacaaaagaaaatgtaatttgatagccaaatcaacgttaaacattatacatttaaaaaaccacaggcaaagacacaaacatgatgacactaacttttgttaaagtatgcttacctatggtttcctctgaggcacgttctttcatgctaagcttccaacataatatgaaaatgaaggagatgcattttgcaaagcaaaacagaccttaagcaaaatattatacttctcaaattaacactgttacaaagttttagaatttaataagttcattaatttaaaagtttggatgtctgagtccttctatcccaaaacaagatcttggagggtcttccacagccatgtaataccatggtcacatgaccctttccaaaattattaatctgaatttactatatgaggataaatctatctttttgaaaatatttaggaaaatgagcttggtatttataaaatgaagctctctttgggtggtatcctaagacacgtcaagccaatcagcctgtaactgtgaaaaaaacattggtaggtacaaaagtggggtgggagaggagtgacttaactttgttaagtgatgggaaagaaacactaatagcattatctcaataaaatgtgatttaaaaaaatttaaaatactaaatcattgaactgacaaagaaatataaatcattcagaaataaactcattaggtcatcaaatcctgttaaatctgcaattaggaagagcaaggtgtacaatccatacatttaaactcacaggctcactttgcacaacgtcaatttactccttaatatgttattaatacgcattttccaaaaggatgtattagtaaatggtacacatctacttcttggcaacatcatataacctggtacaacataagcattcttcttatagttaagaaatgtggatggtatcaaaattagaaaaataaatgccctattatgttgtggtcaggtttaaggcatgtgaattttatcttcatacaaaagattaaaatctagatattaaaaagtagtgcagtatcagtgatgctgcctcagttcccaaaatgtcacatcacaaaaatatcccataattgcctgtagtttattccttggctttcctcttttctctctgcatctttgtaacaattttttaaaagtggaaatataattgttggcaatgctaacagctgtagaaatgattacaagatgtggaaaagcataacaggaatgtcaagaatctgtttctggcagtaatatatatggaacattgttcaggacaaaagaggagaaggaagaaaaaaaggagaggggtttatcatctctaagaattttcaaactaaacctcattgcttaataggaaaaaaagattccatatttaaagttaagtcacctctaactactagctaaagcatgacatcaccagcactggagtcagcggaagtgtgtttttgaaggacagtgttgcaggagaatctggacaggttttagagccaggagagagaaaataattctacctctgacagttgaaggaccttaggcaaatcagtttacctctgctagactacactccaaaatttggacattcaaaaatttgatattaataaccacatgaaagtctcgtgttgaggtgaatatgtatttgttggtgaaagatatgttggtttttaaacagacagcactctgcaattgtaggctattgttttgttttgccagttgtcaaattctatccagctatacacacttgtgtggcctcctaatggtgtttttccagtggctaaaggtttatgaataagacacttttcctaatggaattaacccgatgcttttcttaaacatgtaaccttgagttcaccgcaaaaaacaatgcttcgattagagcaatgcatataataaaggttaccctcgtttcttagacactagacatcattcacaaaaagagaactgcttttgaaagggatgtatttgcactggaaagaatagttttctacttctaattataaatgatttattggtgaaagcaaaacaacagcctgtctgagaggcacttctatgagcatcctcacgtgtgatttgcaaggttgaagaagagggaaaaatgcctcaattgtaccaatggtgagaaaacacccaaagtacaaagcaggtttcaaaaaaaccatactcataaccaaggacaataataaagcaatgtgttgacatatactctataagtcttcctccataaatagtttatagaaattttgtaatttctgtaaatgcatcctataataattttgcatcttgctttttttttacatttaatatcaagtagatttctaaagggcaattatttgaaaattatcccaaatacatggggaaatatacatcaagtgaaaaaatgcagtgggtgatagagatatcaggaagcgcctcaaatatttctcatctcgttggagaaaaacaaacatgttctcatttagaatgagtgggagttacctaattgatttaggcctctatatttaacttctagtcaaaaaaggtagttctatctagcaacaatattatggggaacaaaagaaaaaattaactctctaaatttgcagtagggtcttttcttcagaagtaccaaatcccatctattaccagctccatgcttcaggcctaaaatggatctccctgaagcaatgacagaatttttgccaagtgactaggatataaacaccactttggttgcacagtgagacatatgctccaaagaaaactggttcaaaaacaggcaagtgggtttctacagaataaatgagagccctgtcaatggcttcatcttcagggctttgtgtctgtgcttgcgtggtggctcttgtttcatctatggataatggtggcacacagttttcataattccttacattaatgaactgctataaatttgtttttggtattctagagagtcctaacttcagcttctgggcaatgctgaggaggcaccctatattctagacttaccttttgcaaggtgtactctcagcattgtgggcgatttccatgggagaatattctatttaaagaactactgtcccagcataaaacaaaaaatcatttatgaagatgcaggagactcggaaagctctcaattattgtttgcacaagcacaatgtcacagcctcctttccccattccacaagggggtcaggaagagagtactcagctgtgagaaaagacatacagaagaattcatgtggtcatgagagcgaggacatggccgatcccccaaggaggatgtgtcatacacttcatgagcccaagagtgtgctgtagggtctgaagggcaagatgctggttcactgatgtaaaggagagggaaaaaagcttcaaccaactagaaaaacagtctctatgcatgctatttttgattttaaacacaggtatcaattccttctctcagagagtccattttaaaataggatacatttttaaaggaatatttaaaggacacattcattaaaatttattttaaaaacttttcaaaagaaacaaaaggtatgaattttatttaatccttgaggaaatggttcttttctcacacacataaatcactcattttgtttttctttatctcctttattaatctacattagaaaaataaacttttcatacactaagaacaaggaaaccactctcaattgacaaaatgttccaatccaacacaatgattactttcacctttaatttacaggcagccagattcaaaatccttaaagttgcttaaacttaaaaatgacaatgacaacctaaaaggtataatgttgattggaacagacatttaattggaaaattgatgattttccatttccaattaaatctctagatagaaatgaaaaaaattaaaaatcgtatttaagaaaagccaaatcttgggttgtgaggtatctttttaaggatgtttcagcagaaaaaaacaaaggctctcacaattgtgtagctgcctagattaagtgggtatcctgatcaaggagatgggggatgatttggctttagtattccaatgataaagtttataatgagaataacatgttgctacaaaatccagtctcttcctcagatgccttccacagagggcaggaagctttgtcagttttgtttgctgatgatgcctggttccgtcaacaaataacacctgtcacacggtgggtagtcaatatacatttgttgaataaatatgaaaaaaagaaatgtacaatatgtttgtgaagccaactgtgtgtgcattgctattgaggtacacaaaaagtctttgttttaaatttgagaatgaggactttcaatggaatatatctgataggcctggatcaagcatgcagctgtggagaacacccctgggactctaactctggcactctgcaagctgggtacttgggcaggacagcagcagcactcatgaactgggcagcaccgactggcaaacctccccctgaagatggagaaggaggaaggagtgttactggaatgagagcttgagtccaggggaggaggatgggctgctgaggaggcgacaccatcctgaaagaagaatcctctgccagaggcttttcagggtcatttcttcacactctctgcagggaagcacggagacagcaggaagaaatatcctaacctcactctcttccctctacaggtgcttccattggccaaatccacccagaggccagttggtggcgatcagctctcttcaagtggtatttaaatttcttctttcattttccttctggtaacaaagaagtctgtggctcaaaagatgtttctctaagaccccatcctattaggtctctgagctgtgggaagtatttatacaattgcttgtgaatataagatccaggaatttccctaagatccctaacaaaattggtgataagtagtcccacatgttaatccagccacccacggatgacagcacttaccatttctttgataaatgtcaaatgcatttgaagtacctacctgaaatatttgtttaaatgctatctaatctattaattttatatatgtgtgagtctgttttgtataccttctgattataggataaatgtaaataaatccaaagagtaatcaaagctaccactttcaagaagccttctttgtagaaccggaagagtcttaaataggcttttcaggtatgcatctcttattatcgctgaactccaagtcctgcaaggcaggcatcatgtgtgggtcacctttacagtaggcacaggccttaaaacagtgacatgcacattgcaggcactccataaatgtttgctgaattggctaaaccttggtttgttcccataatcaaccaccacaaacagcacacagataattacttcttggaaagattccaactagtgtttgatgttacctacgtggtttttctctcaagatcttaagagcagctctgtaggattacattattttctgttttttttttcctttgaccttaatgtcatctacttcaataacagcttcatacaaaattcctaccagcacataccacagcagattcaaggccttgttttaaaaatggtgccagcttctcttaatttggaagatatattgtctctcctgaacatgggctaagaaaatgtataatttggtattaacataagagctgaagacactttaaatgcattgtttcatttttataagataaaaaaaattttaagaatcaaaatgttatcaacagacttgtccttcattaaaaagtaaaactgcatttgcctacattttatgaaagtgtccaattatgaacaattttgaaatgtaacttttaaaaatgtaaacagcaaaaatgttgtatttaaaataaatctggaaaggcagaaaaacaaaaaatacccagaagacagagtttttggtgaaagttaagatatttcatctttgaacaacttagaatctttcctgcattttatagtctagttccaggcattaatttgaaataaccttggaatcctaaatctaacacccttcggaacaaagtagcttttctcttctgctttatgagcaaatggactaaatactagggaatggtactgtctgggcctttgaaccaagattgaaagagatgaaatcctatatgatatgtataaacattagagaatccattttgatttaataaaaggttgaatttgttctatatcctgtgagaaaatggttcccttttcctgaaaatgttacctcattccaacaatagaaagttggtttttttccagggtgtggtgttggcgggggacagagttgccatgaatatggcatctatgaagactgctgttatattcatttctcaaaatgcactgtggtaggaaattcagaacgcagtgagagaaaataaatgtttgacttcaaaatataaggccgcatttaaagcagaaggtaaagtatagaacagttgacagtataaattctttatctgcaatcttgcagttccctaaatctctgtaacacatcacttttaaaagcctcagataagtggttctataataatttaccaataattcaacccctcaaaagtcttagcaagttaaaccttataatcttacattttagaaatgacccaacttgatccttttattcttcagaatatctctctcaaattttcatttgtttttcattaattgatgaataatgagacattttaggtacctgtccacaaagaaatgaaattttcactttccaggaacctaacaaatgaaaagatagaaatcaattccaacagaatattaccaaagaaatcttttagaatggactgttaaaattatttatttgtatttatctggctctactatttgtggtacatttccacttcaaagctaaacctcaaataacatcatagtgagtggttgacttcatgtttaactgagatcttgaagactgaaaaagaccacgacaaacacacatctattttcttggctactgcatccgtgttcatcaccattctgatagtctgcaatgtattgcagctcaccctttgggaaggactaaagtagacatctgtttgttctgcttactcagcattcctaccctaattttcctttggagaacccctttattctagaccacgtgaagctaatgccaaaccccattccaggggatgcacctgaatccaacctccatcatctaaacagtgccttctccacgttcagagaagagcaagtgactcaaactgccctcataagaacagacctgggacttctgctgcaaatattgaagagtaagtactcttttttcttgctaggactaagctggtagtaccttctatgaggctatcatatggaaacaacttgtctgaaaatgaagccacaactagaaaacagatcctggtaacccggattgatggatccagccctaccttaaatggcaagacctaacccgaggctttttgcatcaaccaataaagtccttaagccagtttgagttggttttgtcacttgcagctaaaagaattctgactctaacaatgtgacaatagcaaaaataaacataactgcttttgaggtttctaatggattttcctccctatatacatgatttcatttaatcctcacaattcaggaaagcacatatctattaacattaaattaatattcattattttgaacacatgctatgtggataagggatgaggaaagccaaggaagtaatcaacgtgaaatctcacttatatgggagggaagtggaggttacatatctcagggcacttaacagatatcatcaaatgaaagaataaacagtgtgtgggagaggcagtaggtgattcttcatcaattcctggatgaaaaattaggagataatgaactccgaacaggcagcctaatgagaatggctcaagcaacaggacatagagagggagttaggttagacatggggttcttgggaattttcacctcgtgggggggcgggggggtcgtgcagctgttgtcagtgggaaagggaaaaaggaaaaggctgagtttggaaggcagggagggaggagacaatgtgagtcagtgaaaaagggcccttagaatgacaagtctggaccagagagaggctaagactgaaaatacaagttgggtaaccactggcatacagatggcagttcaggcttgggcactgcccaccagagcctcagcatgaagagaagagggggaggctggccaccacctccctctaggtaatcgtcatcctgatgctgagctcctgaaaacaggctctttcactcgccccatctcttgctcttgattgcaacccggcattcaggaggcaccctgtaatatctgtggagtgaccgacaacacagcgccagggcactgagaagatcccagggcgccagggactggttctacaagggtgcccctcccggtcccctccagcgcgccgccagagctgccagtcttggctgctacacgggaggcagcctcattatgcagctctcacctcttaaattagttcatgctctcacattaggtgtaatcacagcttgcaacgctttctggggatgtctcagaaagatctgagttgaaaaaatatttttgtgtcattttaatttaaagtaaaattgctgcttcttccccgcccctttctttcctcctggcccacccagcgaccctggccggccgtgctcaacgggggcgggggtcggaggtgagatttcctccacataattccttaaacagctatcaactaagtctcaaagaaaaaaaaaagagatctagaagcagagacgtggctgctggcgatcccaaagctggtgttcgctcttgggggagagcgtaccctgggggaggccgggaggccgggccagaggctagcccagaggcagagggcaggagcgctcagccggcgccccgcgtctctccagctcccgacgctgcgctggctccgctgagcacgccaggatcaaggtcgcctggtggggaccggagcgccaggagcctgtgggaagcgttccagccggcctctgactgggatccggcgccgcgtttctgctttggacttgactgacaggtccccccgccctcccgccgccctactaccagcctgggttcatccttcagggctacgtctaccgcacccgggctggaaagcctggagcgcgcccttcctctcctcatcttctcagctctcctttctccctgccacttggcaaagctgcattttgactttcacgttttggactacgtgtgtgtagttccaagtccatgcgtggcacgaaaatccacttagggtaaaaattattctcgaaaaatcgcccatctcaggatctggtgtctacactcaaggctaggaggtgcaggtacgggtgcgtaaagcatgccgtaagggtgcacagtaaataaaaagtacggatgcaaaatgtaaattttaagtgcaaaacagaaaagcagtactcgttgccgccccgcacgctgggttttaaggggcacgaaggtgggcctcggctgcttttgctcagccccgcgtcctcagcgcccggcccagtacccggtactccgtaggggttcaatgatctcccctgaataagtgaacgaattaacaaatgaatgaatgaccgctcgatccgacctccgcggccggcagagcagtcgctggagaggcgggagagagcgagaggccaagctccaccatcgcggccgccggctggggcagagggacacggagacactcggcgccccggctccgcaccgagtccccg

SEQ ID NO: 12762 - RNA, 15116 nt, Homo sapiens
  source 1..15116: mol_type = other RNA
gatctcactttgttgcccaggctggtcttaaactcctggcctcaagtgatccccttgtttcagccccgcaaagtgctgggattacaggtgtgagccaccatgcccgtgcccagccacctcatgagtcttgatggggggcagagaccaacaactccacagaagccagatgcttgctttcccagcctctcttgcagctagggcttgggcatgtgatccaggctcagccaatcagatggcactgactcttggcatgacatgggctaaggaggggctgcagggaatccatttgggctggggtggcagctgcactgggagcgacatcagtttccagagggagcagcagaatctggcatcaggcttggggcgtggtaggtgcaaccagactctgcacccagcagcagtggcagaatgggttctctgtggagagtctgtgtattgctccttccgctgaggccaccagcatctgcctccatgaacccctcagagcctgtgagcaactcaacagccttgaattttttcccttcctgtttgaatgagccagggttgtttcactgcttgaactaagagccgttcctgacatgaaaactaagccacatctttttgacccaaagattctggcatcctaaaatacccatctcattttaagttaaaaataaatccatgtttgagcatctactgtttcagttactgtgctaggtgttacaaagctaactaagagtgacaagtaaataactatcatcaccatgataaacagagaatggaaccctggtttttggaatacagacacaaaatgattaattctgcctggaagcgttttggaacatttcagagaggtagtgagctgggccaagagaagagcatacgcaaggaatggtggcatgaagttgcctggtgtgtcctgagaagaaagatgggctaagaaggactggggtagggcagagaagggggtcactggaggtgaggctgggaaagtgagccaaggctcaaatgcaaactgtctgaacttcattttctgtgcaagcaggagaagccgctgacatgggtttggaagatggactgaagccggagaaaaatggaagcaagaaaccctctcacaagaggccataaccacaaccaagtccatgagattgaaaaggaaggcagatatttgaaaaatatttaaagagatgtgaggggtaggacaggcacagtggctcatgcctgtagtcccagcactttgggaggccgaggtgggcagatccacgaggtcaggagatcaagaccatcctaacatggtaaaaccccatctctactaacaatacaaaaaattagtcaggtgtggtggcacgtgcctgtagtcccagctactcaggaggctgaggcaggagaatcgcttgaacctgggaggcggaggttgcagtgagccgagattgtgccactgcaccctagcctaggcaacagagcaagactctgtctcaaaaaaaataaaaaaaaaaaaaagagagaaagagagagagagatgaggagttgctgcactgctgggtgtggagagccgaggaggattcaaagatggtcctgaagtcccagctggaagaagtaggcggcagcaatgtttttaatactgtaaattcatcacgtagcacaggtttggggtggagaaagaaaaattgcattggcttcagggcatgcccagatctttcctcatcttaggcgtttgctaatacatgcattttctaagctgatgtcttgcgtttaatcactgctccattcaaaagagagaaggaggttgtttcaaacctagttgatatcatttgacttccatgctattcacagggctattttatttgaaacaggtataccacagccttaaattgcaagttaatccaggatgttcctaggttggcagttaggaacatgtaattctttggaagggctaaaagtcagctctttaaattatctccatatgaaccttctctccaccttagggtggatccacttatttagtccactgccagtaccacactagaacccgggtggtcactggactccagaaacaacagtagccctctctctgttctgtctctttttgactatctctattctgttcctgaccctgatttctcctgccaagctcaattttgacagctgacaacggcaagccatggcttcccaaaacattattttcaggtcaacttataaatttcaagaacacatttggctccgcttcctgtggtactaagcctacttcttgacagcatttgcctttgttgtaaatagcaaagttcttctagttggatttttgctaagaagtgtgtggatgtggcatgtgacgacatctttagcttggattctagaaaggcactaccattgtgcatttggctaaaggaaacacattttacccgtgaatgccttctatttacaaatgctcagctagcacacaaagctaagtacaagcaataagtactatcctacaatgttactcatttctgaaagcacaaaatgatgactggtatagctttggagatgttttctggaaacccaataaaggaacagatctttgttattccacacctacaaagtcagaagatgcacagtcttttattcatgtttgaacaagcttccttcttgaacaatcaactataaagtgatgtgattctctactagaccaggaactccttgaggacagaatgagggtctaatccatattctaaatccacaccacctggcacaatacatgttgcatggttagggtcaactaagagttggttgaattaatcaataacacacagcaagagaattcacaaagagaggggagtaatcccccagcctcaatcactcggcaagtggaatcgctgggcactgattccagctctgtctcagtgcttgagacagagctgaatgtaatgtgaacatttcaaatgaacaggaaaactagactcacggataagcagtgtagtcatcaagacaacactgtcttggaggtttttctgaagttaaaaccatgctacataagcaataaattatgaaggctgagcatgtgaataaaatttaatgttgtcataaattttataacaaagttaatctgacacatttaatgacatgcataatcattagtatgcagcactgtaatcagacattgataataagcagttcacaccagtgactgtaagagtctttacttgtgttcagccaagccaactgcttggtatatttttctcccttcttagtcgttagttttccatacctacaataactatcagtggtgatgggcttctctgaccatgtgaataatttaatcctcaatgcacagatacagaaacccttgctgaagacagtgtggagcagagaaggctgtctccactccttccacctgaaacacctctgcagatggatatgggagctctgcctacagcccttggacctaaccacttcagtgtgttccagtgagtgtctggacctcggcctgaaagatttttccgaaactaaagaaaatttctctgacctaaagaccttaacctccaccccagaagctctcaccaaggactacagggaactggtggggaaaatccttatcccttactcctcaaggcacagggcagtaatgctgaggcttgtgcgccacacttgctcccagaggtccccagcgggctacctgcggtggtgaatgacctcctaacacgccccttgacggccttcctttccttgcctcacttctccactctcctaccagcattgcagggttcacatcccaaatataccactggcacttgaatcctggtctccaggtctgtttctggaaaaacccaagtaagacattgccccagtaatggggctagatgtctgaggcttcctcaagtatctacctcgaaagctcttactgctgtacacacatgcacatacacacacgtgcgtacaaccagtcacatctaagcaccccgaataccagcctgttgaaggtagcagagagctgcactataagccaaggctgctcccaagagccgctccatcactgaattggcgccccagcaagatgaaggaatgtaatcattggaaggatggagaatgttctctgaatcactgacaaattggaaggggtggagggcaagagtccacctggtggagagatggaaagagcgagagagcctggaatgataatgccattgcttagaaaaggctgctccagatgccatatctacagaaattgtacagcccaaacatctctgagcaataggtctctggtagtcttgatgtctagaccaacaattcccagttcattcttctcagggaaggagccaggatagtccagagactctcattctgctgttagattgaaagggttaggcacaacagccttggcaaagtcacaagggcaaattcacactaaagtgtaaatgacccacaactcctcttctatttttaggttggggaggtgctttagaacataaggaggaactaaagaatattcctgttacatacaaggcagagaaaagggaaactagtggtgacaagacaaatcatccctttgacatttggctggctctacctattacagctctgggggtgaggtgggaacaaaaagatgctgtgtaaagaagtatcttatgccatccctactgtagtgaggtgcagtttagaggggacactgatcaagcagagacccagagtgtttcgttccaagccagaaacagaaatgtataaaacacagcctttccagcatcagaaatgagtagtggtagtggagaactacccaaaacaggaaagaggaccacgtgaggtagagtgtcaaggccctacattccagtgcctctgctcatgactgtaattttgggtaggtcacttaaagtctctggacctcagttttgccatctgtgaaatagggataatactatccagcataaaattggttatgaggctcatgtagggcctgcctgggatgatgtgttgctaatggttaagaacacaacttctggggtctgactggacaggctgaaatccctgcttaacacgttccagcagagccctgggcgatctatttaacttttgttttctcacctgtaagctgagacgaaagtacccactttataagattattccaataattagttgaaataatgcatgcagagaattaagcatggtacttgttatttgttaaactagctattaaaatgtgtaaaatataaagtattgtatggattttaggacaatgcaaagactctttgcttgctgcaatagttcggggccctttcagatggctaaaggcagaatttgtatgtgtaaatatggtgtgcttgtctctgctctggatactgagggcttaccctgttattaaacttatttagtaaatattgaactgtcatgaggcctaacatttagttccagttattagataaaacatttgctttgaatggtatttgaattgccaggttctagattattctggttgacaaactcttcgtattttataaagaggctaaaattggtaagctatcacagaacagatgtgccattttcaaggtatattaaaccatgattcactgtaacattgttcctactggcaacaaattcagagcaggctggactttatttggtgaagaaacattgagtggaagagaaatgacattattttatgtatttacattttcaaattactgtggcttaaacctgttcagccaacattacccaccttcagtctgctaaataaatgattcagtacatttctaatttacagaattttttaacaaaagaaaatgtaatttgatagccaaatcaacgttaaacattatacatttaaaaaaccacaggcaaagacacaaacatgatgacactaacttttgttaaagtatgcttacctatggtttcctctgaggcacgttctttcatgctaagcttccaacataatatgaaaatgaaggagatgcattttgcaaagcaaaacagaccttaagcaaaatattatacttctcaaattaacactgttacaaagttttagaatttaataagttcattaatttaaaagtttggatgtctgagtccttctatcccaaaacaagatcttggagggtcttccacagccatgtaataccatggtcacatgaccctttccaaaattattaatctgaatttactatatgaggataaatctatctttttgaaaatatttaggaaaatgagcttggtatttataaaatgaagctctctttgggtggtatcctaagacacgtcaagccaatcagcctgtaactgtgaaaaaaacattggtaggtacaaaagtggggtgggagaggagtgacttaactttgttaagtgatgggaaagaaacactaatagcattatctcaataaaatgtgatttaaaaaaatttaaaatactaaatcattgaactgacaaagaaatataaatcattcagaaataaactcattaggtcatcaaatcctgttaaatctgcaattaggaagagcaaggtgtacaatccatacatttaaactcacaggctcactttgcacaacgtcaatttactccttaatatgttattaatacgcattttccaaaaggatgtattagtaaatggtacacatctacttcttggcaacatcatataacctggtacaacataagcattcttcttatagttaagaaatgtggatggtatcaaaattagaaaaataaatgccctattatgttgtggtcaggtttaaggcatgtgaattttatcttcatacaaaagattaaaatctagatattaaaaagtagtgcagtatcagtgatgctgcctcagttcccaaaatgtcacatcacaaaaatatcccataattgcctgtagtttattccttggctttcctcttttctctctgcatctttgtaacaattttttaaaagtggaaatataattgttggcaatgctaacagctgtagaaatgattacaagatgtggaaaagcataacaggaatgtcaagaatctgtttctggcagtaatatatatggaacattgttcaggacaaaagaggagaaggaagaaaaaaaggagaggggtttatcatctctaagaattttcaaactaaacctcattgcttaataggaaaaaaagattccatatttaaagttaagtcacctctaactactagctaaagcatgacatcaccagcactggagtcagcggaagtgtgtttttgaaggacagtgttgcaggagaatctggacaggttttagagccaggagagagaaaataattctacctctgacagttgaaggaccttaggcaaatcagtttacctctgctagactacactccaaaatttggacattcaaaaatttgatattaataaccacatgaaagtctcgtgttgaggtgaatatgtatttgttggtgaaagatatgttggtttttaaacagacagcactctgcaattgtaggctattgttttgttttgccagttgtcaaattctatccagctatacacacttgtgtggcctcctaatggtgtttttccagtggctaaaggtttatgaataagacacttttcctaatggaattaacccgatgcttttcttaaacatgtaaccttgagttcaccgcaaaaaacaatgcttcgattagagcaatgcatataataaaggttaccctcgtttcttagacactagacatcattcacaaaaagagaactgcttttgaaagggatgtatttgcactggaaagaatagttttctacttctaattataaatgatttattggtgaaagcaaaacaacagcctgtctgagaggcacttctatgagcatcctcacgtgtgatttgcaaggttgaagaagagggaaaaatgcctcaattgtaccaatggtgagaaaacacccaaagtacaaagcaggtttcaaaaaaaccatactcataaccaaggacaataataaagcaatgtgttgacatatactctataagtcttcctccataaatagtttatagaaattttgtaatttctgtaaatgcatcctataataattttgcatcttgctttttttttacatttaatatcaagtagatttctaaagggcaattatttgaaaattatcccaaatacatggggaaatatacatcaagtgaaaaaatgcagtgggtgatagagatatcaggaagcgcctcaaatatttctcatctcgttggagaaaaacaaacatgttctcatttagaatgagtgggagttacctaattgatttaggcctctatatttaacttctagtcaaaaaaggtagttctatctagcaacaatattatggggaacaaaagaaaaaattaactctctaaatttgcagtagggtcttttcttcagaagtaccaaatcccatctattaccagctccatgcttcaggcctaaaatggatctccctgaagcaatgacagaatttttgccaagtgactaggatataaacaccactttggttgcacagtgagacatatgctccaaagaaaactggttcaaaaacaggcaagtgggtttctacagaataaatgagagccctgtcaatggcttcatcttcagggctttgtgtctgtgcttgcgtggtggctcttgtttcatctatggataatggtggcacacagttttcataattccttacattaatgaactgctataaatttgtttttggtattctagagagtcctaacttcagcttctgggcaatgctgaggaggcaccctatattctagacttaccttttgcaaggtgtactctcagcattgtgggcgatttccatgggagaatattctatttaaagaactactgtcccagcataaaacaaaaaatcatttatgaagatgcaggagactcggaaagctctcaattattgtttgcacaagcacaatgtcacagcctcctttccccattccacaagggggtcaggaagagagtactcagctgtgagaaaagacatacagaagaattcatgtggtcatgagagcgaggacatggccgatcccccaaggaggatgtgtcatacacttcatgagcccaagagtgtgctgtagggtctgaagggcaagatgctggttcactgatgtaaaggagagggaaaaaagcttcaaccaactagaaaaacagtctctatgcatgctatttttgattttaaacacaggtatcaattccttctctcagagagtccattttaaaataggatacatttttaaaggaatatttaaaggacacattcattaaaatttattttaaaaacttttcaaaagaaacaaaaggtatgaattttatttaatccttgaggaaatggttcttttctcacacacataaatcactcattttgtttttctttatctcctttattaatctacattagaaaaataaacttttcatacactaagaacaaggaaaccactctcaattgacaaaatgttccaatccaacacaatgattactttcacctttaatttacaggcagccagattcaaaatccttaaagttgcttaaacttaaaaatgacaatgacaacctaaaaggtataatgttgattggaacagacatttaattggaaaattgatgattttccatttccaattaaatctctagatagaaatgaaaaaaattaaaaatcgtatttaagaaaagccaaatcttgggttgtgaggtatctttttaaggatgtttcagcagaaaaaaacaaaggctctcacaattgtgtagctgcctagattaagtgggtatcctgatcaaggagatgggggatgatttggctttagtattccaatgataaagtttataatgagaataacatgttgctacaaaatccagtctcttcctcagatgccttccacagagggcaggaagctttgtcagttttgtttgctgatgatgcctggttccgtcaacaaataacacctgtcacacggtgggtagtcaatatacatttgttgaataaatatgaaaaaaagaaatgtacaatatgtttgtgaagccaactgtgtgtgcattgctattgaggtacacaaaaagtctttgttttaaatttgagaatgaggactttcaatggaatatatctgataggcctggatcaagcatgcagctgtggagaacacccctgggactctaactctggcactctgcaagctgggtacttgggcaggacagcagcagcactcatgaactgggcagcacctctcttcaagtggtatttaaatttcttctttcattttccttctggtaacaaagaagtctgtggctcaaaagatgtttctctaagaccccatcctattaggtctctgagctgtgggaagtatttatacaattgcttgtgaatataagatccaggaatttccctaagatccctaacaaaattggtgataagtagtcccacatgttaatccagccacccacggatgacagcacttaccatttctttgataaatgtcaaatgcatttgaagtacctacctgaaatatttgtttaaatgctatctaatctattaattttatatatgtgtgagtctgttttgtataccttctgattataggataaatgtaaataaatccaaagagtaatcaaagctaccactttcaagaagccttctttgtagaaccggaagagtcttaaataggcttttcaggtatgcatctcttattatcgctgaactccaagtcctgcaaggcaggcatcatgtgtgggtcacctttacagtaggcacaggccttaaaacagtgacatgcacattgcaggcactccataaatgtttgctgaattggctaaaccttggtttgttcccataatcaaccaccacaaacagcacacagataattacttcttggaaagattccaactagtgtttgatgttacctacgtggtttttctctcaagatcttaagagcagctctgtaggattacattattttctgttttttttttcctttgaccttaatgtcatctacttcaataacagcttcatacaaaattcctaccagcacataccacagcagattcaaggccttgttttaaaaatggtgccagcttctcttaatttggaagatatattgtctctcctgaacatgggctaagaaaatgtataatttggtattaacataagagctgaagacactttaaatgcattgtttcatttttataagataaaaaaaattttaagaatcaaaatgttatcaacagacttgtccttcattaaaaagtaaaactgcatttgcctacattttatgaaagtgtccaattatgaacaattttgaaatgtaacttttaaaaatgtaaacagcaaaaatgttgtatttaaaataaatctggaaaggcagaaaaacaaaaaatacccagaagacagagtttttggtgaaagttaagatatttcatctttgaacaacttagaatctttcctgcattttatagtctagttccaggcattaatttgaaataaccttggaatcctaaatctaacacccttcggaacaaagtagcttttctcttctgctttatgagcaaatggactaaatactagggaatggtactgtctgggcctttgaaccaagattgaaagagatgaaatcctatatgatatgtataaacattagagaatccattttgatttaataaaaggttgaatttgttctatatcctgtgagaaaatggttcccttttcctgaaaatgttacctcattccaacaatagaaagttggtttttttccagggtgtggtgttggcgggggacagagttgccatgaatatggcatctatgaagactgctgttatattcatttctcaaaatgcactgtggtaggaaattcagaacgcagtgagagaaaataaatgtttgacttcaaaatataaggccgcatttaaagcagaaggtaaagtatagaacagttgacagtataaattctttatctgcaatcttgcagttccctaaatctctgtaacacatcacttttaaaagcctcagataagtggttctataataatttaccaataattcaacccctcaaaagtcttagcaagttaaaccttataatcttacattttagaaatgacccaacttgatccttttattcttcagaatatctctctcaaattttcatttgtttttcattaattgatgaataatgagacattttaggtacctgtccacaaagaaatgaaattttcactttccaggaacctaacaaatgaaaagatagaaatcaattccaacagaatattaccaaagaaatcttttagaatggactgttaaaattatttatttgtatttatctggctctactatttgtggtacatttccacttcaaagctaaacctcaaataacatcatagtgagtggttgacttcatgtttaactgagatcttgaagactgaaaaagaccacgacaaacacacatctattttcttggctactgcatccgtgttcatcaccattctgatagtctgcaatgtattgcagctcaccctttgggaaggactaaagtagacatctgtttgttctgcttactcagcattcctaccctaattttcctttggagaacccctttattctagaccacgtgaagctaatgccaaaccccattccaggggatgcacctgaatccaacctccatcatctaaacagtgccttctccacgttcagagaagagcaagtgactcaaactgccctcataagaacagacctgggacttctgctgcaaatattgaagagtaagtactcttttttcttgctaggactaagctggtagtaccttctatgaggctatcatatggaaacaacttgtctgaaaatgaagccacaactagaaaacagatcctggtaacccggattgatggatccagccctaccttaaatggcaagacctaacccgaggctttttgcatcaaccaataaagtccttaagccagtttgagttggttttgtcacttgcagctaaaagaattctgactctaacaatgtgacaatagcaaaaataaacataactgcttttgaggtttctaatggattttcctccctatatacatgatttcatttaatcctcacaattcaggaaagcacatatctattaacattaaattaatattcattattttgaacacatgctatgtggataagggatgaggaaagccaaggaagtaatcaacgtgaaatctcacttatatgggagggaagtggaggttacatatctcagggcacttaacagatatcatcaaatgaaagaataaacagtgtgtgggagaggcagtaggtgattcttcatcaattcctggatgaaaaattaggagataatgaactccgaacaggcagcctaatgagaatggctcaagcaacaggacatagagagggagttaggttagacatggggttcttgggaattttcacctcgtgggggggcgggggggtcgtgcagctgttgtcagtgggaaagggaaaaaggaaaaggctgagtttggaaggcagggagggaggagacaatgtgagtcagtgaaaaagggcccttagaatgacaagtctggaccagagagaggctaagactgaaaatacaagttgggtaaccactggcatacagatggcagttcaggcttgggcactgcccaccagagcctcagcatgaagagaagagggggaggctggccaccacctccctctaggtaatcgtcatcctgatgctgagctcctgaaaacaggctctttcactcgccccatctcttgctcttgattgcaacccggcattcaggaggcaccctgtaatatctgtggagtgaccgacaacacagcgccagggcactgagaagatcccagggcgccagggactggttctacaagggtgcccctcccggtcccctccagcgcgccgccagagctgccagtcttggctgctacacgggaggcagcctcattatgcagctctcacctcttaaattagttcatgctctcacattaggtgtaatcacagcttgcaacgctttctggggatgtctcagaaagatctgagttgaaaaaatatttttgtgtcattttaatttaaagtaaaattgctgcttcttccccgcccctttctttcctcctggcccacccagcgaccctggccggccgtgctcaacgggggcgggggtcggaggtgagatttcctccacataattccttaaacagctatcaactaagtctcaaagaaaaaaaaaagagatctagaagcagagacgtggctgctggcgatcccaaagctggtgttcgctcttgggggagagcgtaccctgggggaggccgggaggccgggccagaggctagcccagaggcagagggcaggagcgctcagccggcgccccgcgtctctccagctcccgacgctgcgctggctccgctgagcacgccaggatcaaggtcgcctggtggggaccggagcgccaggagcctgtgggaagcgttccagccggcctctgactgggatccggcgccgcgtttctgctttggacttgactgacaggtccccccgccctcccgccgccctactaccagcctgggttcatccttcagggctacgtctaccgcacccgggctggaaagcctggagcgcgcccttcctctcctcatcttctcagctctcctttctccctgccacttggcaaagctgcattttgactttcacgttttggactacgtgtgtgtagttccaagtccatgcgtggcacgaaaatccacttagggtaaaaattattctcgaaaaatcgcccatctcaggatctggtgtctacactcaaggctaggaggtgcaggtacgggtgcgtaaagcatgccgtaagggtgcacagtaaataaaaagtacggatgcaaaatgtaaattttaagtgcaaaacagaaaagcagtactcgttgccgccccgcacgctgggttttaaggggcacgaaggtgggcctcggctgcttttgctcagccccgcgtcctcagcgcccggcccagtacccggtactccgtaggggttcaatgatctcccctgaataagtgaacgaattaacaaatgaatgaatgaccgctcgatccgacctccgcggccggcagagcagtcgctggagaggcgggagagagcgagaggccaagctccaccatcgcggccgccggctggggcagagggacacggagacactcggcgccccggctccgcaccgagtccccg

SEQ ID NO: 12763 - RNA, 16824 nt, Homo sapiens
  source 1..16824: mol_type = other RNA
gatctcactttgttgcccaggctggtcttaaactcctggcctcaagtgatccccttgtttcagccccgcaaagtgctgggattacaggtgtgagccaccatgcccgtgcccagccacctcatgagtcttgatggggggcagagaccaacaactccacagaagccagatgcttgctttcccagcctctcttgcagctagggcttgggcatgtgatccaggctcagccaatcagatggcactgactcttggcatgacatgggctaaggaggggctgcagggaatccatttgggctggggtggcagctgcactgggagcgacatcagtttccagagggagcagcagaatctggcatcaggcttggggcgtggtaggtgcaaccagactctgcacccagcagcagtggcagaatgggttctctgtggagagtctgtgtattgctccttccgctgaggccaccagcatctgcctccatgaacccctcagagcctgtgagcaactcaacagccttgaattttttcccttcctgtttgaatgagccagggttgtttcactgcttgaactaagagccgttcctgacatgaaaactaagccacatctttttgacccaaagattctggcatcctaaaatacccatctcattttaagttaaaaataaatccatgtttgagcatctactgtttcagttactgtgctaggtgttacaaagctaactaagagtgacaagtaaataactatcatcaccatgataaacagagaatggaaccctggtttttggaatacagacacaaaatgattaattctgcctggaagcgttttggaacatttcagagaggtagtgagctgggccaagagaagagcatacgcaaggaatggtggcatgaagttgcctggtgtgtcctgagaagaaagatgggctaagaaggactggggtagggcagagaagggggtcactggaggtgaggctgggaaagtgagccaaggctcaaatgcaaactgtctgaacttcattttctgtgcaagcaggagaagccgctgacatgggtttggaagatggactgaagccggagaaaaatggaagcaagaaaccctctcacaagaggccataaccacaaccaagtccatgagattgaaaaggaaggcagatatttgaaaaatatttaaagagatgtgaggggtaggacaggcacagtggctcatgcctgtagtcccagcactttgggaggccgaggtgggcagatccacgaggtcaggagatcaagaccatcctaacatggtaaaaccccatctctactaacaatacaaaaaattagtcaggtgtggtggcacgtgcctgtagtcccagctactcaggaggctgaggcaggagaatcgcttgaacctgggaggcggaggttgcagtgagccgagattgtgccactgcaccctagcctaggcaacagagcaagactctgtctcaaaaaaaataaaaaaaaaaaaaagagagaaagagagagagagatgaggagttgctgcactgctgggtgtggagagccgaggaggattcaaagatggtcctgaagtcccagctggaagaagtaggcggcagcaatgtttttaatactgtaaattcatcacgtagcacaggtttggggtggagaaagaaaaattgcattggcttcagggcatgcccagatctttcctcatcttaggcgtttgctaatacatgcattttctaagctgatgtcttgcgtttaatcactgctccattcaaaagagagaaggaggttgtttcaaacctagttgatatcatttgacttccatgctattcacagggctattttatttgaaacaggtataccacagccttaaattgcaagttaatccaggatgttcctaggttggcagttaggaacatgtaattctttggaagggctaaaagtcagctctttaaattatctccatatgaaccttctctccaccttagggtggatccacttatttagtccactgccagtaccacactagaacccgggtggtcactggactccagaaacaacagtagccctctctctgttctgtctctttttgactatctctattctgttcctgaccctgatttctcctgccaagctcaattttgacagctgacaacggcaagccatggcttcccaaaacattattttcaggtcaacttataaatttcaagaacacatttggctccgcttcctgtggtactaagcctacttcttgacagcatttgcctttgttgtaaatagcaaagttcttctagttggatttttgctaagaagtgtgtggatgtggcatgtgacgacatctttagcttggattctagaaaggcactaccattgtgcatttggctaaaggaaacacattttacccgtgaatgccttctatttacaaatgctcagctagcacacaaagctaagtacaagcaataagtactatcctacaatgttactcatttctgaaagcacaaaatgatgactggtatagctttggagatgttttctggaaacccaataaaggaacagatctttgttattccacacctacaaagtcagaagatgcacagtcttttattcatgtttgaacaagcttccttcttgaacaatcaactataaagtgatgtgattctctactagaccaggaactccttgaggacagaatgagggtctaatccatattctaaatccacaccacctggcacaatacatgttgcatggttagggtcaactaagagttggttgaattaatcaataacacacagcaagagaattcacaaagagaggggagtaatcccccagcctcaatcactcggcaagtggaatcgctgggcactgattccagctctgtctcagtgcttgagacagagctgaatgtaatgtgaacatttcaaatgaacaggaaaactagactcacggataagcagtgtagtcatcaagacaacactgtcttggaggtttttctgaagttaaaaccatgctacataagcaataaattatgaaggctgagcatgtgaataaaatttaatgttgtcataaattttataacaaagttaatctgacacatttaatgacatgcataatcattagtatgcagcactgtaatcagacattgataataagcagttcacaccagtgactgtaagagtctttacttgtgttcagccaagccaactgcttggtatatttttctcccttcttagtcgttagttttccatacctacaataactatcagtggtgatgggcttctctgaccatgtgaataatttaatcctcaatgcacagatacagaaacccttgctgaagacagtgtggagcagagaaggctgtctccactccttccacctgaaacacctctgcagatggatatgggagctctgcctacagcccttggacctaaccacttcagtgtgttccagtgagtgtctggacctcggcctgaaagatttttccgaaactaaagaaaatttctctgacctaaagaccttaacctccaccccagaagctctcaccaaggactacagggaactggtggggaaaatccttatcccttactcctcaaggcacagggcagtaatgctgaggcttgtgcgccacacttgctcccagaggtccccagcgggctacctgcggtggtgaatgacctcctaacacgccccttgacggccttcctttccttgcctcacttctccactctcctaccagcattgcagggttcacatcccaaatataccactggcacttgaatcctggtctccaggtctgtttctggaaaaacccaagtaagacattgccccagtaatggggctagatgtctgaggcttcctcaagtatctacctcgaaagctcttactgctgtacacacatgcacatacacacacgtgcgtacaaccagtcacatctaagcaccccgaataccagcctgttgaaggtagcagagagctgcactataagccaaggctgctcccaagagccgctccatcactgaattggcgccccagcaagatgaaggaatgtaatcattggaaggatggagaatgttctctgaatcactgacaaattggaaggggtggagggcaagagtccacctggtggagagatggaaagagcgagagagcctggaatgataatgccattgcttagaaaaggctgctccagatgccatatctacagaaattgtacagcccaaacatctctgagcaataggtctctggtagtcttgatgtctagaccaacaattcccagttcattcttctcagggaaggagccaggatagtccagagactctcattctgctgttagattgaaagggttaggcacaacagccttggcaaagtcacaagggcaaattcacactaaagtgtaaatgacccacaactcctcttctatttttaggttggggaggtgctttagaacataaggaggaactaaagaatattcctgttacatacaaggcagagaaaagggaaactagtggtgacaagacaaatcatccctttgacatttggctggctctacctattacagctctgggggtgaggtgggaacaaaaagatgctgtgtaaagaagtatcttatgccatccctactgtagtgaggtgcagtttagaggggacactgatcaagcagagacccagagtgtttcgttccaagccagaaacagaaatgtataaaacacagcctttccagcatcagaaatgagtagtggtagtggagaactacccaaaacaggaaagaggaccacgtgaggtagagtgtcaaggccctacattccagtgcctctgctcatgactgtaattttgggtaggtcacttaaagtctctggacctcagttttgccatctgtgaaatagggataatactatccagcataaaattggttatgaggctcatgtagggcctgcctgggatgatgtgttgctaatggttaagaacacaacttctggggtctgactggacaggctgaaatccctgcttaacacgttccagcagagccctgggcgatctatttaacttttgttttctcacctgtaagctgagacgaaagtacccactttataagattattccaataattagttgaaataatgcatgcagagaattaagcatggtacttgttatttgttaaactagctattaaaatgtgtaaaatataaagtattgtatggattttaggacaatgcaaagactctttgcttgctgcaatagttcggggccctttcagatggctaaaggcagaatttgtatgtgtaaatatggtgtgcttgtctctgctctggatactgagggcttaccctgttattaaacttatttagtaaatattgaactgtcatgaggcctaacatttagttccagttattagataaaacatttgctttgaatggtatttgaattgccaggttctagattattctggttgacaaactcttcgtattttataaagaggctaaaattggtaagctatcacagaacagatgtgccattttcaaggtatattaaaccatgattcactgtaacattgttcctactggcaacaaattcagagcaggctggactttatttggtgaagaaacattgagtggaagagaaatgacattattttatgtatttacattttcaaattactgtggcttaaacctgttcagccaacattacccaccttcagtctgctaaataaatgattcagtacatttctaatttacagaattttttaacaaaagaaaatgtaatttgatagccaaatcaacgttaaacattatacatttaaaaaaccacaggcaaagacacaaacatgatgacactaacttttgttaaagtatgcttacctatggtttcctctgaggcacgttctttcatgctaagcttccaacataatatgaaaatgaaggagatgcattttgcaaagcaaaacagaccttaagcaaaatattatacttctcaaattaacactgttacaaagttttagaatttaataagttcattaatttaaaagtttggatgtctgagtccttctatcccaaaacaagatcttggagggtcttccacagccatgtaataccatggtcacatgaccctttccaaaattattaatctgaatttactatatgaggataaatctatctttttgaaaatatttaggaaaatgagcttggtatttataaaatgaagctctctttgggtggtatcctaagacacgtcaagccaatcagcctgtaactgtgaaaaaaacattggtaggtacaaaagtggggtgggagaggagtgacttaactttgttaagtgatgggaaagaaacactaatagcattatctcaataaaatgtgatttaaaaaaatttaaaatactaaatcattgaactgacaaagaaatataaatcattcagaaataaactcattaggtcatcaaatcctgttaaatctgcaattaggaagagcaaggtgtacaatccatacatttaaactcacaggctcactttgcacaacgtcaatttactccttaatatgttattaatacgcattttccaaaaggatgtattagtaaatggtacacatctacttcttggcaacatcatataacctggtacaacataagcattcttcttatagttaagaaatgtggatggtatcaaaattagaaaaataaatgccctattatgttgtggtcaggtttaaggcatgtgaattttatcttcatacaaaagattaaaatctagatattaaaaagtagtgcagtatcagtgatgctgcctcagttcccaaaatgtcacatcacaaaaatatcccataattgcctgtagtttattccttggctttcctcttttctctctgcatctttgtaacaattttttaaaagtggaaatataattgttggcaatgctaacagctgtagaaatgattacaagatgtggaaaagcataacaggaatgtcaagaatctgtttctggcagtaatatatatggaacattgttcaggacaaaagaggagaaggaagaaaaaaaggagaggggtttatcatctctaagaattttcaaactaaacctcattgcttaataggaaaaaaagattccatatttaaagttaagtcacctctaactactagctaaagcatgacatcaccagcactggagtcagcggaagtgtgtttttgaaggacagtgttgcaggagaatctggacaggttttagagccaggagagagaaaataattctacctctgacagttgaaggaccttaggcaaatcagtttacctctgctagactacactccaaaatttggacattcaaaaatttgatattaataaccacatgaaagtctcgtgttgaggtgaatatgtatttgttggtgaaagatatgttggtttttaaacagacagcactctgcaattgtaggctattgttttgttttgccagttgtcaaattctatccagctatacacacttgtgtggcctcctaatggtgtttttccagtggctaaaggtttatgaataagacacttttcctaatggaattaacccgatgcttttcttaaacatgtaaccttgagttcaccgcaaaaaacaatgcttcgattagagcaatgcatataataaaggttaccctcgtttcttagacactagacatcattcacaaaaagagaactgcttttgaaagggatgtatttgcactggaaagaatagttttctacttctaattataaatgatttattggtgaaagcaaaacaacagcctgtctgagaggcacttctatgagcatcctcacgtgtgatttgcaaggttgaagaagagggaaaaatgcctcaattgtaccaatggtgagaaaacacccaaagtacaaagcaggtttcaaaaaaaccatactcataaccaaggacaataataaagcaatgtgttgacatatactctataagtcttcctccataaatagtttatagaaattttgtaatttctgtaaatgcatcctataataattttgcatcttgctttttttttacatttaatatcaagtagatttctaaagggcaattatttgaaaattatcccaaatacatggggaaatatacatcaagtgaaaaaatgcagtgggtgatagagatatcaggaagcgcctcaaatatttctcatctcgttggagaaaaacaaacatgttctcatttagaatgagtgggagttacctaattgatttaggcctctatatttaacttctagtcaaaaaaggtagttctatctagcaacaatattatggggaacaaaagaaaaaattaactctctaaatttgcagtagggtcttttcttcagaagtaccaaatcccatctattaccagctccatgcttcaggcctaaaatggatctccctgaagcaatgacagaatttttgccaagtgactaggatataaacaccactttggttgcacagtgagacatatgctccaaagaaaactggttcaaaaacaggcaagtgggtttctacagaataaatgagagccctgtcaatggcttcatcttcagggctttgtgtctgtgcttgcgtggtggctcttgtttcatctatggataatggtggcacacagttttcataattccttacattaatgaactgctataaatttgtttttggtattctagagagtcctaacttcagcttctgggcaatgctgaggaggcaccctatattctagacttaccttttgcaaggtgtactctcagcattgtgggcgatttccatgggagaatattctatttaaagaactactgtcccagcataaaacaaaaaatcatttatgaagatgcaggagactcggaaagctctcaattattgtttgcacaagcacaatgtcacagcctcctttccccattccacaagggggtcaggaagagagtactcagctgtgagaaaagacatacagaagaattcatgtggtcatgagagcgaggacatggccgatcccccaaggaggatgtgtcatacacttcatgagcccaagagtgtgctgtagggtctgaagggcaagatgctggttcactgatgtaaaggagagggaaaaaagcttcaaccaactagaaaaacagtctctatgcatgctatttttgattttaaacacaggtatcaattccttctctcagagagtccattttaaaataggatacatttttaaaggaatatttaaaggacacattcattaaaatttattttaaaaacttttcaaaagaaacaaaaggtatgaattttatttaatccttgaggaaatggttcttttctcacacacataaatcactcattttgtttttctttatctcctttattaatctacattagaaaaataaacttttcatacactaagaacaaggaaaccactctcaattgacaaaatgttccaatccaacacaatgattactttcacctttaatttacaggcagccagattcaaaatccttaaagttgcttaaacttaaaaatgacaatgacaacctaaaaggtataatgttgattggaacagacatttaattggaaaattgatgattttccatttccaattaaatctctagatagaaatgaaaaaaattaaaaatcgtatttaagaaaagccaaatcttgggttgtgaggtatctttttaaggatgtttcagcagaaaaaaacaaaggctctcacaattgtgtagctgcctagattaagtgggtatcctgatcaaggagatgggggatgatttggctttagtattccaatgataaagtttataatgagaataacatgttgctacaaaatccagtctcttcctcagatgccttccacagagggcaggaagctttgtcagttttgtttgctgatgatgcctggttccgtcaacaaataacacctgtcacacggtgggtagtcaatatacatttgttgaataaatatgaaaaaaagaaatgtacaatatgtttgtgaagccaactgtgtgtgcattgctattgaggtacacaaaaagtctttgttttaaatttgagaatgaggactttcaatggaatatatctgataggcctggatcaagcatgcagctgtggagaacacccctgggactctaactctggcactctgcaagctgggtacttgggcaggacagcagcagcactcatgaactgggcagcacctgttggtgagggctgatcacatggattctctcatcccagccttacaatcagtccttcaggtacatactttttctgactttgctgatgaggaaactatgcacagaggttacacagcttaacaaagggttctcacctaatgaacaatgaaatgggattttagcctttctttgcatctggtcttagagccaatacccaagaagcactgtactgtatgcattgtctcagagaaacttactcttcctgggcctcagtctttaaaaggtgggcagttgacttaataagaattaaagatcaatgattaaggttcaaggcactccaaaattctggtctttattgaaaaggctacagaagtctcaccttaataataccctatagacttgatattcttggttaattaaatattggaaaccaatttcatagtaattgaggtcagaaaaaagtactcatgacattttagaatatgatgacaaagccatagataaatttcaatgcacctgtaattacttaaaactgttatagcatgcaatgtgttaccacaacagccagagaaatactaatttactcagcctattcttctagaccagtaaacactaggattaaatagatattttcattgaatttgttctacccttcattgccatttatagatagcttacttgtcatagattactttctaattgttttatgtttcctaactagcctgcaatactttggcaaggacctcaaacaatagtagacagtaggtgtaaaatagatggctacattgaacagatgactaaaaggatgcctcctaagtacctatatcttgaaatatatattattgtgccttgctttcaatttgtgattttaaaatctagaaatcacctgttttatgtaataacaataaaatccttctttgttgaaaacatgcacaaataaagtttacaagctcaaaaaattaaacagcagtaacggtcaagctttccaacaataaaatacattttggtaaggttttcattttacaaaaactcaaaatagctttatgagttcacaaaataatatgatatttttcaagatattaacatattcttataccggaagagcatagaataaaatttacttggagattgagcatttgcttctttaagaaatacttcttttagtatttttactttaatattatgaaagctacataattacattcagattcattaactactccagtagttaatttttaaaacttatgatgaatagttttgtttaaaatatataacattggtaatatgcaaatctgaatctgtaataaagaaggatttgcattcctgatttttttttctgatacaaccaatgacaaaataactaatggttccacagaggataaaatgtctcaaatctgttggttctgaaggtgaagcgagatttttgtactgataccgtgtatcactgagataccaggaggaaatggaattaaactcagatagttcaaatggagagattttaatgaagggacgacctacagaggtgtcggcagggttggggggaatcagcgagatatgcttagaacccaccgactggcaaacctccccctgaagatggagaaggaggaaggagtgttactggaatgagagcttgagtccaggggaggaggatgggctgctgaggaggcgacaccatcctgaaagaagaatcctctgccagaggcttttcagggtcatttcttcacactctctctcttcaagtggtatttaaatttcttctttcattttccttctggtaacaaagaagtctgtggctcaaaagatgtttctctaagaccccatcctattaggtctctgagctgtgggaagtatttatacaattgcttgtgaatataagatccaggaatttccctaagatccctaacaaaattggtgataagtagtcccacatgttaatccagccacccacggatgacagcacttaccatttctttgataaatgtcaaatgcatttgaagtacctacctgaaatatttgtttaaatgctatctaatctattaattttatatatgtgtgagtctgttttgtataccttctgattataggataaatgtaaataaatccaaagagtaatcaaagctaccactttcaagaagccttctttgtagaaccggaagagtcttaaataggcttttcaggtatgcatctcttattatcgctgaactccaagtcctgcaaggcaggcatcatgtgtgggtcacctttacagtaggcacaggccttaaaacagtgacatgcacattgcaggcactccataaatgtttgctgaattggctaaaccttggtttgttcccataatcaaccaccacaaacagcacacagataattacttcttggaaagattccaactagtgtttgatgttacctacgtggtttttctctcaagatcttaagagcagctctgtaggattacattattttctgttttttttttcctttgaccttaatgtcatctacttcaataacagcttcatacaaaattcctaccagcacataccacagcagattcaaggccttgttttaaaaatggtgccagcttctcttaatttggaagatatattgtctctcctgaacatgggctaagaaaatgtataatttggtattaacataagagctgaagacactttaaatgcattgtttcatttttataagataaaaaaaattttaagaatcaaaatgttatcaacagacttgtccttcattaaaaagtaaaactgcatttgcctacattttatgaaagtgtccaattatgaacaattttgaaatgtaacttttaaaaatgtaaacagcaaaaatgttgtatttaaaataaatctggaaaggcagaaaaacaaaaaatacccagaagacagagtttttggtgaaagttaagatatttcatctttgaacaacttagaatctttcctgcattttatagtctagttccaggcattaatttgaaataaccttggaatcctaaatctaacacccttcggaacaaagtagcttttctcttctgctttatgagcaaatggactaaatactagggaatggtactgtctgggcctttgaaccaagattgaaagagatgaaatcctatatgatatgtataaacattagagaatccattttgatttaataaaaggttgaatttgttctatatcctgtgagaaaatggttcccttttcctgaaaatgttacctcattccaacaatagaaagttggtttttttccagggtgtggtgttggcgggggacagagttgccatgaatatggcatctatgaagactgctgttatattcatttctcaaaatgcactgtggtaggaaattcagaacgcagtgagagaaaataaatgtttgacttcaaaatataaggccgcatttaaagcagaaggtaaagtatagaacagttgacagtataaattctttatctgcaatcttgcagttccctaaatctctgtaacacatcacttttaaaagcctcagataagtggttctataataatttaccaataattcaacccctcaaaagtcttagcaagttaaaccttataatcttacattttagaaatgacccaacttgatccttttattcttcagaatatctctctcaaattttcatttgtttttcattaattgatgaataatgagacattttaggtacctgtccacaaagaaatgaaattttcactttccaggaacctaacaaatgaaaagatagaaatcaattccaacagaatattaccaaagaaatcttttagaatggactgttaaaattatttatttgtatttatctggctctactatttgtggtacatttccacttcaaagctaaacctcaaataacatcatagtgagtggttgacttcatgtttaactgagatcttgaagactgaaaaagaccacgacaaacacacatctattttcttggctactgcatccgtgttcatcaccattctgatagtctgcaatgtattgcagctcaccctttgggaaggactaaagtagacatctgtttgttctgcttactcagcattcctaccctaattttcctttggagaacccctttattctagaccacgtgaagctaatgccaaaccccattccaggggatgcacctgaatccaacctccatcatctaaacagtgccttctccacgttcagagaagagcaagtgactcaaactgccctcataagaacagacctgggacttctgctgcaaatattgaagagtaagtactcttttttcttgctaggactaagctggtagtaccttctatgaggctatcatatggaaacaacttgtctgaaaatgaagccacaactagaaaacagatcctggtaacccggattgatggatccagccctaccttaaatggcaagacctaacccgaggctttttgcatcaaccaataaagtccttaagccagtttgagttggttttgtcacttgcagctaaaagaattctgactctaacaatgtgacaatagcaaaaataaacataactgcttttgaggtttctaatggattttcctccctatatacatgatttcatttaatcctcacaattcaggaaagcacatatctattaacattaaattaatattcattattttgaacacatgctatgtggataagggatgaggaaagccaaggaagtaatcaacgtgaaatctcacttatatgggagggaagtggaggttacatatctcagggcacttaacagatatcatcaaatgaaagaataaacagtgtgtgggagaggcagtaggtgattcttcatcaattcctggatgaaaaattaggagataatgaactccgaacaggcagcctaatgagaatggctcaagcaacaggacatagagagggagttaggttagacatggggttcttgggaattttcacctcgtgggggggcgggggggtcgtgcagctgttgtcagtgggaaagggaaaaaggaaaaggctgagtttggaaggcagggagggaggagacaatgtgagtcagtgaaaaagggcccttagaatgacaagtctggaccagagagaggctaagactgaaaatacaagttgggtaaccactggcatacagatggcagttcaggcttgggcactgcccaccagagcctcagcatgaagagaagagggggaggctggccaccacctccctctaggtaatcgtcatcctgatgctgagctcctgaaaacaggctctttcactcgccccatctcttgctcttgattgcaacccggcattcaggaggcaccctgtaatatctgtggagtgaccgacaacacagcgccagggcactgagaagatcccagggcgccagggactggttctacaagggtgcccctcccggtcccctccagcgcgccgccagagctgccagtcttggctgctacacgggaggcagcctcattatgcagctctcacctcttaaattagttcatgctctcacattaggtgtaatcacagcttgcaacgctttctggggatgtctcagaaagatctgagttgaaaaaatatttttgtgtcattttaatttaaagtaaaattgctgcttcttccccgcccctttctttcctcctggcccacccagcgaccctggccggccgtgctcaacgggggcgggggtcggaggtgagatttcctccacataattccttaaacagctatcaactaagtctcaaagaaaaaaaaaagagatctagaagcagagacgtggctgctggcgatcccaaagctggtgttcgctcttgggggagagcgtaccctgggggaggccgggaggccgggccagaggctagcccagaggcagagggcaggagcgctcagccggcgccccgcgtctctccagctcccgacgctgcgctggctccgctgagcacgccaggatcaaggtcgcctggtggggaccggagcgccaggagcctgtgggaagcgttccagccggcctctgactgggatccggcgccgcgtttctgctttggacttgactgacaggtccccccgccctcccgccgccctactaccagcctgggttcatccttcagggctacgtctaccgcacccgggctggaaagcctggagcgcgcccttcctctcctcatcttctcagctctcctttctccctgccacttggcaaagctgcattttgactttcacgttttggactacgtgtgtgtagttccaagtccatgcgtggcacgaaaatccacttagggtaaaaattattctcgaaaaatcgcccatctcaggatctggtgtctacactcaaggctaggaggtgcaggtacgggtgcgtaaagcatgccgtaagggtgcacagtaaataaaaagtacggatgcaaaatgtaaattttaagtgcaaaacagaaaagcagtactcgttgccgccccgcacgctgggttttaaggggcacgaaggtgggcctcggctgcttttgctcagccccgcgtcctcagcgcccggcccagtacccggtactccgtaggggttcaatgatctcccctgaataagtgaacgaattaacaaatgaatgaatgaccgctcgatccgacctccgcggccggcagagcagtcgctggagaggcgggagagagcgagaggccaagctccaccatcgcggccgccggctggggcagagggacacggagacactcggcgccccggctccgcaccgagtccccg

SEQ ID NO: 12764 - RNA, 12253 nt, Homo sapiens
  source 1..12253: mol_type = other RNA
gatctcactttgttgcccaggctggtcttaaactcctggcctcaagtgatccccttgtttcagccccgcaaagtgctgggattacaggtgtgagccaccatgcccgtgcccagccacctcatgagtcttgatggggggcagagaccaacaactccacagaagccagatgcttgctttcccagcctctcttgcagctagggcttgggcatgtgatccaggctcagccaatcagatggcactgactcttggcatgacatgggctaaggaggggctgcagggaatccatttgggctggggtggcagctgcactgggagcgacatcagtttccagagggagcagcagaatctggcatcaggcttggggcgtggtaggtgcaaccagactctgcacccagcagcagtggcagaatgggttctctgtggagagtctgtgtattgctccttccgctgaggccaccagcatctgcctccatgaacccctcagagcctgtgagcaactcaacagccttgaattttttcccttcctgtttgaatgagccagggttgtttcactgcttgaactaagagccgttcctgacatgaaaactaagccacatctttttgacccaaagattctggcatcctaaaatacccatctcattttaagttaaaaataaatccatgtttgagcatctactgtttcagttactgtgctaggtgttacaaagctaactaagagtgacaagtaaataactatcatcaccatgataaacagagaatggaaccctggtttttggaatacagacacaaaatgattaattctgcctggaagcgttttggaacatttcagagaggtagtgagctgggccaagagaagagcatacgcaaggaatggtggcatgaagttgcctggtgtgtcctgagaagaaagatgggctaagaaggactggggtagggcagagaagggggtcactggaggtgaggctgggaaagtgagccaaggctcaaatgcaaactgtctgaacttcattttctgtgcaagcaggagaagccgctgacatgggtttggaagatggactgaagccggagaaaaatggaagcaagaaaccctctcacaagaggccataaccacaaccaagtccatgagattgaaaaggaaggcagatatttgaaaaatatttaaagagatgtgaggggtaggacaggcacagtggctcatgcctgtagtcccagcactttgggaggccgaggtgggcagatccacgaggtcaggagatcaagaccatcctaacatggtaaaaccccatctctactaacaatacaaaaaattagtcaggtgtggtggcacgtgcctgtagtcccagctactcaggaggctgaggcaggagaatcgcttgaacctgggaggcggaggttgcagtgagccgagattgtgccactgcaccctagcctaggcaacagagcaagactctgtctcaaaaaaaataaaaaaaaaaaaaagagagaaagagagagagagatgaggagttgctgcactgctgggtgtggagagccgaggaggattcaaagatggtcctgaagtcccagctggaagaagtaggcggcagcaatgtttttaatactgtaaattcatcacgtagcacaggtttggggtggagaaagaaaaattgcattggcttcagggcatgcccagatctttcctcatcttaggcgtttgctaatacatgcattttctaagctgatgtcttgcgtttaatcactgctccattcaaaagagagaaggaggttgtttcaaacctagttgatatcatttgacttccatgctattcacagggctattttatttgaaacaggtataccacagccttaaattgcaagttaatccaggatgttcctaggttggcagttaggaacatgtaattctttggaagggctaaaagtcagctctttaaattatctccatatgaaccttctctccaccttagggtggatccacttatttagtccactgccagtaccacactagaacccgggtggtcactggactccagaaacaacagtagccctctctctgttctgtctctttttgactatctctattctgttcctgaccctgatttctcctgccaagctcaattttgacagctgacaacggcaagccatggcttcccaaaacattattttcaggtcaacttataaatttcaagaacacatttggctccgcttcctgtggtactaagcctacttcttgacagcatttgcctttgttgtaaatagcaaagttcttctagttggatttttgctaagaagtgtgtggatgtggcatgtgacgacatctttagcttggattctagaaaggcactaccattgtgcatttggctaaaggaaacacattttacccgtgaatgccttctatttacaaatgctcagctagcacacaaagctaagtacaagcaataagtactatcctacaatgttactcatttctgaaagcacaaaatgatgactggtatagctttggagatgttttctggaaacccaataaaggaacagatctttgttattccacacctacaaagtcagaagatgcacagtcttttattcatgtttgaacaagcttccttcttgaacaatcaactataaagtgatgtgattctctactagaccaggaactccttgaggacagaatgagggtctaatccatattctaaatccacaccacctggcacaatacatgttgcatggttagggtcaactaagagttggttgaattaatcaataacacacagcaagagaattcacaaagagaggggagtaatcccccagcctcaatcactcggcaagtggaatcgctgggcactgattccagctctgtctcagtgcttgagacagagctgaatgtaatgtgaacatttcaaatgaacaggaaaactagactcacggataagcagtgtagtcatcaagacaacactgtcttggaggtttttctgaagttaaaaccatgctacataagcaataaattatgaaggctgagcatgtgaataaaatttaatgttgtcataaattttataacaaagttaatctgacacatttaatgacatgcataatcattagtatgcagcactgtaatcagacattgataataagcagttcacaccagtgactgtaagagtctttacttgtgttcagccaagccaactgcttggtatatttttctcccttcttagtcgttagttttccatacctacaataactatcagtggtgatgggcttctctgaccatgtgaataatttaatcctcaatgcacagatacagaaacccttgctgaagacagtgtggagcagagaaggctgtctccactccttccacctgaaacacctctgcagatggatatgggagctctgcctacagcccttggacctaaccacttcagtgtgttccagtgagtgtctggacctcggcctgaaagatttttccgaaactaaagaaaatttctctgacctaaagaccttaacctccaccccagaagctctcaccaaggactacagggaactggtggggaaaatccttatcccttactcctcaaggcacagggcagtaatgctgaggcttgtgcgccacacttgctcccagaggtccccagcgggctacctgcggtggtgaatgacctcctaacacgccccttgacggccttcctttccttgcctcacttctccactctcctaccagcattgcagggttcacatcccaaatataccactggcacttgaatcctggtctccaggtctgtttctggaaaaacccaagtaagacattgccccagtaatggggctagatgtctgaggcttcctcaagtatctacctcgaaagctcttactgctgtacacacatgcacatacacacacgtgcgtacaaccagtcacatctaagcaccccgaataccagcctgttgaaggtagcagagagctgcactataagccaaggctgctcccaagagccgctccatcactgaattggcgccccagcaagatgaaggaatgtaatcattggaaggatggagaatgttctctgaatcactgacaaattggaaggggtggagggcaagagtccacctggtggagagatggaaagagcgagagagcctggaatgataatgccattgcttagaaaaggctgctccagatgccatatctacagaaattgtacagcccaaacatctctgagcaataggtctctggtagtcttgatgtctagaccaacaattcccagttcattcttctcagggaaggagccaggatagtccagagactctcattctgctgttagattgaaagggttaggcacaacagccttggcaaagtcacaagggcaaattcacactaaagtgtaaatgacccacaactcctcttctatttttaggttggggaggtgctttagaacataaggaggaactaaagaatattcctgttacatacaaggcagagaaaagggaaactagtggtgacaagacaaatcatccctttgacatttggctggctctacctattacagctctgggggtgaggtgggaacaaaaagatgctgtgtaaagaagtatcttatgccatccctactgtagtgaggtgcagtttagaggggacactgatcaagcagagacccagagtgtttcgttccaagccagaaacagaaatgtataaaacacagcctttccagcatcagaaatgagtagtggtagtggagaactacccaaaacaggaaagaggaccacgtgaggtagagtgtcaaggccctacattccagtgcctctgctcatgactgtaattttgggtaggtcacttaaagtctctggacctcagttttgccatctgtgaaatagggataatactatccagcataaaattggttatgaggctcatgtagggcctgcctgggatgatgtgttgctaatggttaagaacacaacttctggggtctgactggacaggctgaaatccctgcttaacacgttccagcagagccctgggcgatctatttaacttttgttttctcacctgtaagctgagacgaaagtacccactttataagattattccaataattagttgaaataatgcatgcagagaattaagcatggtacttgttatttgttaaactagctattaaaatgtgtaaaatataaagtattgtatggattttaggacaatgcaaagactctttgcttgctgcaatagttcggggccctttcagatggctaaaggcagaatttgtatgtgtaaatatggtgtgcttgtctctgctctggatactgagggcttaccctgttattaaacttatttagtaaatattgaactgtcatgaggcctaacatttagttccagttattagataaaacatttgctttgaatggtatttgaattgccaggttctagattattctggttgacaaactcttcgtattttataaagaggctaaaattggtaagctatcacagaacagatgtgccattttcaaggtatattaaaccatgattcactgtaacattgttcctactggcaacaaattcagagcaggctggactttatttggtgaagaaacattgagtggaagagaaatgacattattttatgtatttacattttcaaattactgtggcttaaacctgttcagccaacattacccaccttcagtctgctaaataaatgattcagtacatttctaatttacagaattttttaacaaaagaaaatgtaatttgatagccaaatcaacgttaaacattatacatttaaaaaaccacaggcaaagacacaaacatgatgacactaacttttgttaaagtatgcttacctatggtttcctctgaggcacgttctttcatgctaagcttccaacataatatgaaaatgaaggagatgcattttgcaaagcaaaacagaccttaagcaaaatattatacttctcaaattaacactgttacaaagttttagaatttaataagttcattaatttaaaagtttggatgtctgagtccttctatcccaaaacaagatcttggagggtcttccacagccatgtaataccatggtcacatgaccctttccaaaattattaatctgaatttactatatgaggataaatctatctttttgaaaatatttaggaaaatgagcttggtatttataaaatgaagctctctttgggtggtatcctaagacacgtcaagccaatcagcctgtaactgtgaaaaaaacattggtaggtacaaaagtggggtgggagaggagtgacttaactttgttaagtgatgggaaagaaacactaatagcattatctcaataaaatgtgatttaaaaaaatttaaaatactaaatcattgaactgacaaagaaatataaatcattcagaaataaactcattaggtcatcaaatcctgttaaatctgcaattaggaagagcaaggtgtacaatccatacatttaaactcacaggctcactttgcacaacgtcaatttactccttaatatgttattaatacgcattttccaaaaggatgtattagtaaatggtacacatctacttcttggcaacatcatataacctggtacaacataagcattcttcttatagttaagaaatgtggatggtatcaaaattagaaaaataaatgccctattatgttgtggtcaggtttaaggcatgtgaattttatcttcatacaaaagattaaaatctagatattaaaaagtagtgcagtatcagtgatgctgcctcagttcccaaaatgtcacatcacaaaaatatcccataattgcctgtagtttattccttggctttcctcttttctctctgcatctttgtaacaattttttaaaagtggaaatataattgttggcaatgctaacagctgtagaaatgattacaagatgtggaaaagcataacaggaatgtcaagaatctgtttctggcagtaatatatatggaacattgttcaggacaaaagaggagaaggaagaaaaaaaggagaggggtttatcatctctaagaattttcaaactaaacctcattgcttaataggaaaaaaagattccatatttaaagttaagtcacctctaactactagctaaagcatgacatcaccagcactggagtcagcggaagtgtgtttttgaaggacagtgttgcaggagaatctggacaggttttagagccaggagagagaaaataattctacctctgacagttgaaggaccttaggcaaatcagtttacctctgctagactacactccaaaatttggacattcaaaaatttgatattaataaccacatgaaagtctcgtgttgaggtgaatatgtatttgttggtgaaagatatgttggtttttaaacagacagcactctgcaattgtaggctattgttttgttttgccagttgtcaaattctatccagctatacacacttgtgtggcctcctaatggtgtttttccagtggctaaaggtttatgaataagacacttttcctaatggaattaacccgatgcttttcttaaacatgtaaccttgagttcaccgcaaaaaacaatgcttcgattagagcaatgcatataataaaggttaccctcgtttcttagacactagacatcattcacaaaaagagaactgcttttgaaagggatgtatttgcactggaaagaatagttttctacttctaattataaatgatttattggtgaaagcaaaacaacagcctgtctgagaggcacttctatgagcatcctcacgtgtgatttgcaaggttgaagaagagggaaaaatgcctcaattgtaccaatggtgagaaaacacccaaagtacaaagcaggtttcaaaaaaaccatactcataaccaaggacaataataaagcaatgtgttgacatatactctataagtcttcctccataaatagtttatagaaattttgtaatttctgtaaatgcatcctataataattttgcatcttgctttttttttacatttaatatcaagtagatttctaaagggcaattatttgaaaattatcccaaatacatggggaaatatacatcaagtgaaaaaatgcagtgggtgatagagatatcaggaagcgcctcaaatatttctcatctcgttggagaaaaacaaacatgttctcatttagaatgagtgggagttacctaattgatttaggcctctatatttaacttctagtcaaaaaaggtagttctatctagcaacaatattatggggaacaaaagaaaaaattaactctctaaatttgcagtagggtcttttcttcagaagtaccaaatcccatctattaccagctccatgcttcaggcctaaaatggatctccctgaagcaatgacagaatttttgccaagtgactaggatataaacaccactttggttgcacagtgagacatatgctccaaagaaaactggttcaaaaacaggcaagtgggtttctacagaataaatgagagccctgtcaatggcttcatcttcagggctttgtgtctgtgcttgcgtggtggctcttgtttcatctatggataatggtggcacacagttttcataattccttacattaatgaactgctataaatttgtttttggtattctagagagtcctaacttcagcttctgggcaatgctgaggaggcaccctatattctagacttaccttttgcaaggtgtactctcagcattgtgggcgatttccatgggagaatattctatttaaagaactactgtcccagcataaaacaaaaaatcatttatgaagatgcaggagactcggaaagctctcaattattgtttgcacaagcacaatgtcacagcctcctttccccattccacaagggggtcaggaagagagtactcagctgtgagaaaagacatacagaagaattcatgtggtcatgagagcgaggacatggccgatcccccaaggaggatgtgtcatacacttcatgagcccaagagtgtgctgtagggtctgaagggcaagatgctggttcactgatgtaaaggagagggaaaaaagcttcaaccaactagaaaaacagtctctatgcatgctatttttgattttaaacacaggtatcaattccttctctcagagagtccattttaaaataggatacatttttaaaggaatatttaaaggacacattcattaaaatttattttaaaaacttttcaaaagaaacaaaaggtatgaattttatttaatccttgaggaaatggttcttttctcacacacataaatcactcattttgtttttctttatctcctttattaatctacattagaaaaataaacttttcatacactaagaacaaggaaaccactctcaattgacaaaatgttccaatccaacacaatgattactttcacctttaatttacaggcagccagattcaaaatccttaaagttgcttaaacttaaaaatgacaatgacaacctaaaaggtataatgttgattggaacagacatttaattggaaaattgatgattttccatttccaattaaatctctagatagaaatgaaaaaaattaaaaatcgtatttaagaaaagccaaatcttgggttgtgaggtatctttttaaggatgtttcagcagaaaaaaacaaaggctctcacaattgtgtagctgcctagattaagtgggtatcctgatcaaggagatgggggatgatttggctttagtattccaatgataaagtttataatgagaataacatgttgctacaaaatccagtctcttcctcagatgccttccacagagggcaggaagctttgtcagttttgtttgctgatgatgcctggttccgtcaacaaataacacctgtcacacggtgggtagtcaatatacatttgttgaataaatatgaaaaaaagaaatgtacaatatgtttgtgaagccaactgtgtgtgcattgctattgaggtacacaaaaagtctttgttttaaatttgagaatgaggactttcaatggaatatatctgataggcctggatcaagcatgcagctgtggagaacacccctgggactctaactctggcactctgcaagctgggtacttgggcaggacagcagcagcactcatgaactgggcagcacctgttggtgagggctgatcacatggattctctcatcccagccttacaatcagtccttcaggtacatactttttctgactttgctgatgaggaaactatgcacagaggttacacagcttaacaaagggttctcacctaatgaacaatgaaatgggattttagcctttctttgcatctggtcttagagccaatacccaagaagcactgtactgtatgcattgtctcagagaaacttactcttcctgggcctcagtctttaaaaggtgggcagttgacttaataagaattaaagatcaatgattaaggttcaaggcactccaaaattctggtctttattgaaaaggctacagaagtctcaccttaataataccctatagacttgatattcttggttaattaaatattggaaaccaatttcatagtaattgaggtcagaaaaaagtactcatgacattttagaatatgatgacaaagccatagataaatttcaatgcacctgtaattacttaaaactgttatagcatgcaatgtgttaccacaacagccagagaaatactaatttactcagcctattcttctagaccagtaaacactaggattaaatagatattttcattgaatttgttctacccttcattgccatttatagatagcttacttgtcatagattactttctaattgttttatgtttcctaactagcctgcaatactttggcaaggacctcaaacaatagtagacagtaggtgtaaaatagatggctacattgaacagatgactaaaaggatgcctcctaagtacctatatcttgaaatatatattattgtgccttgctttcaatttgtgattttaaaatctagaaatcacctgttttatgtaataacaataaaatccttctttgttgaaaacatgcacaaataaagtttacaagctcaaaaaattaaacagcagtaacggtcaagctttccaacaataaaatacattttggtaaggttttcattttacaaaaactcaaaatagctttatgagttcacaaaataatatgatatttttcaagatattaacatattcttataccggaagagcatagaataaaatttacttggagattgagcatttgcttctttaagaaatacttcttttagtatttttactttaatattatgaaagctacataattacattcagattcattaactactccagtagttaatttttaaaacttatgatgaatagttttgtttaaaatatataacattggtaatatgcaaatctgaatctgtaataaagaaggatttgcattcctgatttttttttctgatacaaccaatgacaaaataactaatggttccacagaggataaaatgtctcaaatctgttggttctgaaggtgaagcgagatttttgtactgataccgtgtatcactgagataccaggaggaaatggaattaaactcagatagttcaaatggagagattttaatgaagggacgacctacagaggtgtcggcagggttggggggaatcagcgagatatgcttagaacccaccgactggcaaacctccccctgaagatggagaaggaggaaggagtgttactggaatgagagcttgagtccaggggaggaggatgggctgctgaggaggcgacaccatcctgaaagaagaatcctctgccagaggcttttcagggtcatttcttcacactctctgcagggaagcacggagacagcaggaagaaatatcctaacctcactctcttccctctacaggtgcttccattggccaaatccacccagaggccagttggtggcgatcagctctcttcaagtggtatttaaatttcttctttcattttccttctggtaacaaagaagtctgtggctcaaaagatgtttctctaagaccccatcctattaggtctctgagctgagggccgacgagtgggggcgggcaggagggccgagggaggcggaacaggatcgaggcgcgaggcgggagtcgagaaagcgagcggccgaggcgactctcagtgcgcggacgcgggcgcgcgcccgcgctcccttcgtcgactcacggcgagagcccaaccctgctgccgcgcgccacccgcctcgccgcgcct

SEQ ID NO: 12765 - RNA, 16934 nt, Homo sapiens
  source 1..16934: mol_type = other RNA
gatctcactttgttgcccaggctggtcttaaactcctggcctcaagtgatccccttgtttcagccccgcaaagtgctgggattacaggtgtgagccaccatgcccgtgcccagccacctcatgagtcttgatggggggcagagaccaacaactccacagaagccagatgcttgctttcccagcctctcttgcagctagggcttgggcatgtgatccaggctcagccaatcagatggcactgactcttggcatgacatgggctaaggaggggctgcagggaatccatttgggctggggtggcagctgcactgggagcgacatcagtttccagagggagcagcagaatctggcatcaggcttggggcgtggtaggtgcaaccagactctgcacccagcagcagtggcagaatgggttctctgtggagagtctgtgtattgctccttccgctgaggccaccagcatctgcctccatgaacccctcagagcctgtgagcaactcaacagccttgaattttttcccttcctgtttgaatgagccagggttgtttcactgcttgaactaagagccgttcctgacatgaaaactaagccacatctttttgacccaaagattctggcatcctaaaatacccatctcattttaagttaaaaataaatccatgtttgagcatctactgtttcagttactgtgctaggtgttacaaagctaactaagagtgacaagtaaataactatcatcaccatgataaacagagaatggaaccctggtttttggaatacagacacaaaatgattaattctgcctggaagcgttttggaacatttcagagaggtagtgagctgggccaagagaagagcatacgcaaggaatggtggcatgaagttgcctggtgtgtcctgagaagaaagatgggctaagaaggactggggtagggcagagaagggggtcactggaggtgaggctgggaaagtgagccaaggctcaaatgcaaactgtctgaacttcattttctgtgcaagcaggagaagccgctgacatgggtttggaagatggactgaagccggagaaaaatggaagcaagaaaccctctcacaagaggccataaccacaaccaagtccatgagattgaaaaggaaggcagatatttgaaaaatatttaaagagatgtgaggggtaggacaggcacagtggctcatgcctgtagtcccagcactttgggaggccgaggtgggcagatccacgaggtcaggagatcaagaccatcctaacatggtaaaaccccatctctactaacaatacaaaaaattagtcaggtgtggtggcacgtgcctgtagtcccagctactcaggaggctgaggcaggagaatcgcttgaacctgggaggcggaggttgcagtgagccgagattgtgccactgcaccctagcctaggcaacagagcaagactctgtctcaaaaaaaataaaaaaaaaaaaaagagagaaagagagagagagatgaggagttgctgcactgctgggtgtggagagccgaggaggattcaaagatggtcctgaagtcccagctggaagaagtaggcggcagcaatgtttttaatactgtaaattcatcacgtagcacaggtttggggtggagaaagaaaaattgcattggcttcagggcatgcccagatctttcctcatcttaggcgtttgctaatacatgcattttctaagctgatgtcttgcgtttaatcactgctccattcaaaagagagaaggaggttgtttcaaacctagttgatatcatttgacttccatgctattcacagggctattttatttgaaacaggtataccacagccttaaattgcaagttaatccaggatgttcctaggttggcagttaggaacatgtaattctttggaagggctaaaagtcagctctttaaattatctccatatgaaccttctctccaccttagggtggatccacttatttagtccactgccagtaccacactagaacccgggtggtcactggactccagaaacaacagtagccctctctctgttctgtctctttttgactatctctattctgttcctgaccctgatttctcctgccaagctcaattttgacagctgacaacggcaagccatggcttcccaaaacattattttcaggtcaacttataaatttcaagaacacatttggctccgcttcctgtggtactaagcctacttcttgacagcatttgcctttgttgtaaatagcaaagttcttctagttggatttttgctaagaagtgtgtggatgtggcatgtgacgacatctttagcttggattctagaaaggcactaccattgtgcatttggctaaaggaaacacattttacccgtgaatgccttctatttacaaatgctcagctagcacacaaagctaagtacaagcaataagtactatcctacaatgttactcatttctgaaagcacaaaatgatgactggtatagctttggagatgttttctggaaacccaataaaggaacagatctttgttattccacacctacaaagtcagaagatgcacagtcttttattcatgtttgaacaagcttccttcttgaacaatcaactataaagtgatgtgattctctactagaccaggaactccttgaggacagaatgagggtctaatccatattctaaatccacaccacctggcacaatacatgttgcatggttagggtcaactaagagttggttgaattaatcaataacacacagcaagagaattcacaaagagaggggagtaatcccccagcctcaatcactcggcaagtggaatcgctgggcactgattccagctctgtctcagtgcttgagacagagctgaatgtaatgtgaacatttcaaatgaacaggaaaactagactcacggataagcagtgtagtcatcaagacaacactgtcttggaggtttttctgaagttaaaaccatgctacataagcaataaattatgaaggctgagcatgtgaataaaatttaatgttgtcataaattttataacaaagttaatctgacacatttaatgacatgcataatcattagtatgcagcactgtaatcagacattgataataagcagttcacaccagtgactgtaagagtctttacttgtgttcagccaagccaactgcttggtatatttttctcccttcttagtcgttagttttccatacctacaataactatcagtggtgatgggcttctctgaccatgtgaataatttaatcctcaatgcacagatacagaaacccttgctgaagacagtgtggagcagagaaggctgtctccactccttccacctgaaacacctctgcagatggatatgggagctctgcctacagcccttggacctaaccacttcagtgtgttccagtgagtgtctggacctcggcctgaaagatttttccgaaactaaagaaaatttctctgacctaaagaccttaacctccaccccagaagctctcaccaaggactacagggaactggtggggaaaatccttatcccttactcctcaaggcacagggcagtaatgctgaggcttgtgcgccacacttgctcccagaggtccccagcgggctacctgcggtggtgaatgacctcctaacacgccccttgacggccttcctttccttgcctcacttctccactctcctaccagcattgcagggttcacatcccaaatataccactggcacttgaatcctggtctccaggtctgtttctggaaaaacccaagtaagacattgccccagtaatggggctagatgtctgaggcttcctcaagtatctacctcgaaagctcttactgctgtacacacatgcacatacacacacgtgcgtacaaccagtcacatctaagcaccccgaataccagcctgttgaaggtagcagagagctgcactataagccaaggctgctcccaagagccgctccatcactgaattggcgccccagcaagatgaaggaatgtaatcattggaaggatggagaatgttctctgaatcactgacaaattggaaggggtggagggcaagagtccacctggtggagagatggaaagagcgagagagcctggaatgataatgccattgcttagaaaaggctgctccagatgccatatctacagaaattgtacagcccaaacatctctgagcaataggtctctggtagtcttgatgtctagaccaacaattcccagttcattcttctcagggaaggagccaggatagtccagagactctcattctgctgttagattgaaagggttaggcacaacagccttggcaaagtcacaagggcaaattcacactaaagtgtaaatgacccacaactcctcttctatttttaggttggggaggtgctttagaacataaggaggaactaaagaatattcctgttacatacaaggcagagaaaagggaaactagtggtgacaagacaaatcatccctttgacatttggctggctctacctattacagctctgggggtgaggtgggaacaaaaagatgctgtgtaaagaagtatcttatgccatccctactgtagtgaggtgcagtttagaggggacactgatcaagcagagacccagagtgtttcgttccaagccagaaacagaaatgtataaaacacagcctttccagcatcagaaatgagtagtggtagtggagaactacccaaaacaggaaagaggaccacgtgaggtagagtgtcaaggccctacattccagtgcctctgctcatgactgtaattttgggtaggtcacttaaagtctctggacctcagttttgccatctgtgaaatagggataatactatccagcataaaattggttatgaggctcatgtagggcctgcctgggatgatgtgttgctaatggttaagaacacaacttctggggtctgactggacaggctgaaatccctgcttaacacgttccagcagagccctgggcgatctatttaacttttgttttctcacctgtaagctgagacgaaagtacccactttataagattattccaataattagttgaaataatgcatgcagagaattaagcatggtacttgttatttgttaaactagctattaaaatgtgtaaaatataaagtattgtatggattttaggacaatgcaaagactctttgcttgctgcaatagttcggggccctttcagatggctaaaggcagaatttgtatgtgtaaatatggtgtgcttgtctctgctctggatactgagggcttaccctgttattaaacttatttagtaaatattgaactgtcatgaggcctaacatttagttccagttattagataaaacatttgctttgaatggtatttgaattgccaggttctagattattctggttgacaaactcttcgtattttataaagaggctaaaattggtaagctatcacagaacagatgtgccattttcaaggtatattaaaccatgattcactgtaacattgttcctactggcaacaaattcagagcaggctggactttatttggtgaagaaacattgagtggaagagaaatgacattattttatgtatttacattttcaaattactgtggcttaaacctgttcagccaacattacccaccttcagtctgctaaataaatgattcagtacatttctaatttacagaattttttaacaaaagaaaatgtaatttgatagccaaatcaacgttaaacattatacatttaaaaaaccacaggcaaagacacaaacatgatgacactaacttttgttaaagtatgcttacctatggtttcctctgaggcacgttctttcatgctaagcttccaacataatatgaaaatgaaggagatgcattttgcaaagcaaaacagaccttaagcaaaatattatacttctcaaattaacactgttacaaagttttagaatttaataagttcattaatttaaaagtttggatgtctgagtccttctatcccaaaacaagatcttggagggtcttccacagccatgtaataccatggtcacatgaccctttccaaaattattaatctgaatttactatatgaggataaatctatctttttgaaaatatttaggaaaatgagcttggtatttataaaatgaagctctctttgggtggtatcctaagacacgtcaagccaatcagcctgtaactgtgaaaaaaacattggtaggtacaaaagtggggtgggagaggagtgacttaactttgttaagtgatgggaaagaaacactaatagcattatctcaataaaatgtgatttaaaaaaatttaaaatactaaatcattgaactgacaaagaaatataaatcattcagaaataaactcattaggtcatcaaatcctgttaaatctgcaattaggaagagcaaggtgtacaatccatacatttaaactcacaggctcactttgcacaacgtcaatttactccttaatatgttattaatacgcattttccaaaaggatgtattagtaaatggtacacatctacttcttggcaacatcatataacctggtacaacataagcattcttcttatagttaagaaatgtggatggtatcaaaattagaaaaataaatgccctattatgttgtggtcaggtttaaggcatgtgaattttatcttcatacaaaagattaaaatctagatattaaaaagtagtgcagtatcagtgatgctgcctcagttcccaaaatgtcacatcacaaaaatatcccataattgcctgtagtttattccttggctttcctcttttctctctgcatctttgtaacaattttttaaaagtggaaatataattgttggcaatgctaacagctgtagaaatgattacaagatgtggaaaagcataacaggaatgtcaagaatctgtttctggcagtaatatatatggaacattgttcaggacaaaagaggagaaggaagaaaaaaaggagaggggtttatcatctctaagaattttcaaactaaacctcattgcttaataggaaaaaaagattccatatttaaagttaagtcacctctaactactagctaaagcatgacatcaccagcactggagtcagcggaagtgtgtttttgaaggacagtgttgcaggagaatctggacaggttttagagccaggagagagaaaataattctacctctgacagttgaaggaccttaggcaaatcagtttacctctgctagactacactccaaaatttggacattcaaaaatttgatattaataaccacatgaaagtctcgtgttgaggtgaatatgtatttgttggtgaaagatatgttggtttttaaacagacagcactctgcaattgtaggctattgttttgttttgccagttgtcaaattctatccagctatacacacttgtgtggcctcctaatggtgtttttccagtggctaaaggtttatgaataagacacttttcctaatggaattaacccgatgcttttcttaaacatgtaaccttgagttcaccgcaaaaaacaatgcttcgattagagcaatgcatataataaaggttaccctcgtttcttagacactagacatcattcacaaaaagagaactgcttttgaaagggatgtatttgcactggaaagaatagttttctacttctaattataaatgatttattggtgaaagcaaaacaacagcctgtctgagaggcacttctatgagcatcctcacgtgtgatttgcaaggttgaagaagagggaaaaatgcctcaattgtaccaatggtgagaaaacacccaaagtacaaagcaggtttcaaaaaaaccatactcataaccaaggacaataataaagcaatgtgttgacatatactctataagtcttcctccataaatagtttatagaaattttgtaatttctgtaaatgcatcctataataattttgcatcttgctttttttttacatttaatatcaagtagatttctaaagggcaattatttgaaaattatcccaaatacatggggaaatatacatcaagtgaaaaaatgcagtgggtgatagagatatcaggaagcgcctcaaatatttctcatctcgttggagaaaaacaaacatgttctcatttagaatgagtgggagttacctaattgatttaggcctctatatttaacttctagtcaaaaaaggtagttctatctagcaacaatattatggggaacaaaagaaaaaattaactctctaaatttgcagtagggtcttttcttcagaagtaccaaatcccatctattaccagctccatgcttcaggcctaaaatggatctccctgaagcaatgacagaatttttgccaagtgactaggatataaacaccactttggttgcacagtgagacatatgctccaaagaaaactggttcaaaaacaggcaagtgggtttctacagaataaatgagagccctgtcaatggcttcatcttcagggctttgtgtctgtgcttgcgtggtggctcttgtttcatctatggataatggtggcacacagttttcataattccttacattaatgaactgctataaatttgtttttggtattctagagagtcctaacttcagcttctgggcaatgctgaggaggcaccctatattctagacttaccttttgcaaggtgtactctcagcattgtgggcgatttccatgggagaatattctatttaaagaactactgtcccagcataaaacaaaaaatcatttatgaagatgcaggagactcggaaagctctcaattattgtttgcacaagcacaatgtcacagcctcctttccccattccacaagggggtcaggaagagagtactcagctgtgagaaaagacatacagaagaattcatgtggtcatgagagcgaggacatggccgatcccccaaggaggatgtgtcatacacttcatgagcccaagagtgtgctgtagggtctgaagggcaagatgctggttcactgatgtaaaggagagggaaaaaagcttcaaccaactagaaaaacagtctctatgcatgctatttttgattttaaacacaggtatcaattccttctctcagagagtccattttaaaataggatacatttttaaaggaatatttaaaggacacattcattaaaatttattttaaaaacttttcaaaagaaacaaaaggtatgaattttatttaatccttgaggaaatggttcttttctcacacacataaatcactcattttgtttttctttatctcctttattaatctacattagaaaaataaacttttcatacactaagaacaaggaaaccactctcaattgacaaaatgttccaatccaacacaatgattactttcacctttaatttacaggcagccagattcaaaatccttaaagttgcttaaacttaaaaatgacaatgacaacctaaaaggtataatgttgattggaacagacatttaattggaaaattgatgattttccatttccaattaaatctctagatagaaatgaaaaaaattaaaaatcgtatttaagaaaagccaaatcttgggttgtgaggtatctttttaaggatgtttcagcagaaaaaaacaaaggctctcacaattgtgtagctgcctagattaagtgggtatcctgatcaaggagatgggggatgatttggctttagtattccaatgataaagtttataatgagaataacatgttgctacaaaatccagtctcttcctcagatgccttccacagagggcaggaagctttgtcagttttgtttgctgatgatgcctggttccgtcaacaaataacacctgtcacacggtgggtagtcaatatacatttgttgaataaatatgaaaaaaagaaatgtacaatatgtttgtgaagccaactgtgtgtgcattgctattgaggtacacaaaaagtctttgttttaaatttgagaatgaggactttcaatggaatatatctgataggcctggatcaagcatgcagctgtggagaacacccctgggactctaactctggcactctgcaagctgggtacttgggcaggacagcagcagcactcatgaactgggcagcacctgttggtgagggctgatcacatggattctctcatcccagccttacaatcagtccttcaggtacatactttttctgactttgctgatgaggaaactatgcacagaggttacacagcttaacaaagggttctcacctaatgaacaatgaaatgggattttagcctttctttgcatctggtcttagagccaatacccaagaagcactgtactgtatgcattgtctcagagaaacttactcttcctgggcctcagtctttaaaaggtgggcagttgacttaataagaattaaagatcaatgattaaggttcaaggcactccaaaattctggtctttattgaaaaggctacagaagtctcaccttaataataccctatagacttgatattcttggttaattaaatattggaaaccaatttcatagtaattgaggtcagaaaaaagtactcatgacattttagaatatgatgacaaagccatagataaatttcaatgcacctgtaattacttaaaactgttatagcatgcaatgtgttaccacaacagccagagaaatactaatttactcagcctattcttctagaccagtaaacactaggattaaatagatattttcattgaatttgttctacccttcattgccatttatagatagcttacttgtcatagattactttctaattgttttatgtttcctaactagcctgcaatactttggcaaggacctcaaacaatagtagacagtaggtgtaaaatagatggctacattgaacagatgactaaaaggatgcctcctaagtacctatatcttgaaatatatattattgtgccttgctttcaatttgtgattttaaaatctagaaatcacctgttttatgtaataacaataaaatccttctttgttgaaaacatgcacaaataaagtttacaagctcaaaaaattaaacagcagtaacggtcaagctttccaacaataaaatacattttggtaaggttttcattttacaaaaactcaaaatagctttatgagttcacaaaataatatgatatttttcaagatattaacatattcttataccggaagagcatagaataaaatttacttggagattgagcatttgcttctttaagaaatacttcttttagtatttttactttaatattatgaaagctacataattacattcagattcattaactactccagtagttaatttttaaaacttatgatgaatagttttgtttaaaatatataacattggtaatatgcaaatctgaatctgtaataaagaaggatttgcattcctgatttttttttctgatacaaccaatgacaaaataactaatggttccacagaggataaaatgtctcaaatctgttggttctgaaggtgaagcgagatttttgtactgataccgtgtatcactgagataccaggaggaaatggaattaaactcagatagttcaaatggagagattttaatgaagggacgacctacagaggtgtcggcagggttggggggaatcagcgagatatgcttagaacccaccgactggcaaacctccccctgaagatggagaaggaggaaggagtgttactggaatgagagcttgagtccaggggaggaggatgggctgctgaggaggcgacaccatcctgaaagaagaatcctctgccagaggcttttcagggtcatttcttcacactctctgcagggaagcacggagacagcaggaagaaatatcctaacctcactctcttccctctacaggtgcttccattggccaaatccacccagaggccagttggtggcgatcagctctcttcaagtggtatttaaatttcttctttcattttccttctggtaacaaagaagtctgtggctcaaaagatgtttctctaagaccccatcctattaggtctctgagctgtgggaagtatttatacaattgcttgtgaatataagatccaggaatttccctaagatccctaacaaaattggtgataagtagtcccacatgttaatccagccacccacggatgacagcacttaccatttctttgataaatgtcaaatgcatttgaagtacctacctgaaatatttgtttaaatgctatctaatctattaattttatatatgtgtgagtctgttttgtataccttctgattataggataaatgtaaataaatccaaagagtaatcaaagctaccactttcaagaagccttctttgtagaaccggaagagtcttaaataggcttttcaggtatgcatctcttattatcgctgaactccaagtcctgcaaggcaggcatcatgtgtgggtcacctttacagtaggcacaggccttaaaacagtgacatgcacattgcaggcactccataaatgtttgctgaattggctaaaccttggtttgttcccataatcaaccaccacaaacagcacacagataattacttcttggaaagattccaactagtgtttgatgttacctacgtggtttttctctcaagatcttaagagcagctctgtaggattacattattttctgttttttttttcctttgaccttaatgtcatctacttcaataacagcttcatacaaaattcctaccagcacataccacagcagattcaaggccttgttttaaaaatggtgccagcttctcttaatttggaagatatattgtctctcctgaacatgggctaagaaaatgtataatttggtattaacataagagctgaagacactttaaatgcattgtttcatttttataagataaaaaaaattttaagaatcaaaatgttatcaacagacttgtccttcattaaaaagtaaaactgcatttgcctacattttatgaaagtgtccaattatgaacaattttgaaatgtaacttttaaaaatgtaaacagcaaaaatgttgtatttaaaataaatctggaaaggcagaaaaacaaaaaatacccagaagacagagtttttggtgaaagttaagatatttcatctttgaacaacttagaatctttcctgcattttatagtctagttccaggcattaatttgaaataaccttggaatcctaaatctaacacccttcggaacaaagtagcttttctcttctgctttatgagcaaatggactaaatactagggaatggtactgtctgggcctttgaaccaagattgaaagagatgaaatcctatatgatatgtataaacattagagaatccattttgatttaataaaaggttgaatttgttctatatcctgtgagaaaatggttcccttttcctgaaaatgttacctcattccaacaatagaaagttggtttttttccagggtgtggtgttggcgggggacagagttgccatgaatatggcatctatgaagactgctgttatattcatttctcaaaatgcactgtggtaggaaattcagaacgcagtgagagaaaataaatgtttgacttcaaaatataaggccgcatttaaagcagaaggtaaagtatagaacagttgacagtataaattctttatctgcaatcttgcagttccctaaatctctgtaacacatcacttttaaaagcctcagataagtggttctataataatttaccaataattcaacccctcaaaagtcttagcaagttaaaccttataatcttacattttagaaatgacccaacttgatccttttattcttcagaatatctctctcaaattttcatttgtttttcattaattgatgaataatgagacattttaggtacctgtccacaaagaaatgaaattttcactttccaggaacctaacaaatgaaaagatagaaatcaattccaacagaatattaccaaagaaatcttttagaatggactgttaaaattatttatttgtatttatctggctctactatttgtggtacatttccacttcaaagctaaacctcaaataacatcatagtgagtggttgacttcatgtttaactgagatcttgaagactgaaaaagaccacgacaaacacacatctattttcttggctactgcatccgtgttcatcaccattctgatagtctgcaatgtattgcagctcaccctttgggaaggactaaagtagacatctgtttgttctgcttactcagcattcctaccctaattttcctttggagaacccctttattctagaccacgtgaagctaatgccaaaccccattccaggggatgcacctgaatccaacctccatcatctaaacagtgccttctccacgttcagagaagagcaagtgactcaaactgccctcataagaacagacctgggacttctgctgcaaatattgaagagtaagtactcttttttcttgctaggactaagctggtagtaccttctatgaggctatcatatggaaacaacttgtctgaaaatgaagccacaactagaaaacagatcctggtaacccggattgatggatccagccctaccttaaatggcaagacctaacccgaggctttttgcatcaaccaataaagtccttaagccagtttgagttggttttgtcacttgcagctaaaagaattctgactctaacaatgtgacaatagcaaaaataaacataactgcttttgaggtttctaatggattttcctccctatatacatgatttcatttaatcctcacaattcaggaaagcacatatctattaacattaaattaatattcattattttgaacacatgctatgtggataagggatgaggaaagccaaggaagtaatcaacgtgaaatctcacttatatgggagggaagtggaggttacatatctcagggcacttaacagatatcatcaaatgaaagaataaacagtgtgtgggagaggcagtaggtgattcttcatcaattcctggatgaaaaattaggagataatgaactccgaacaggcagcctaatgagaatggctcaagcaacaggacatagagagggagttaggttagacatggggttcttgggaattttcacctcgtgggggggcgggggggtcgtgcagctgttgtcagtgggaaagggaaaaaggaaaaggctgagtttggaaggcagggagggaggagacaatgtgagtcagtgaaaaagggcccttagaatgacaagtctggaccagagagaggctaagactgaaaatacaagttgggtaaccactggcatacagatggcagttcaggcttgggcactgcccaccagagcctcagcatgaagagaagagggggaggctggccaccacctccctctaggtaatcgtcatcctgatgctgagctcctgaaaacaggctctttcactcgccccatctcttgctcttgattgcaacccggcattcaggaggcaccctgtaatatctgtggagtgaccgacaacacagcgccagggcactgagaagatcccagggcgccagggactggttctacaagggtgcccctcccggtcccctccagcgcgccgccagagctgccagtcttggctgctacacgggaggcagcctcattatgcagctctcacctcttaaattagttcatgctctcacattaggtgtaatcacagcttgcaacgctttctggggatgtctcagaaagatctgagttgaaaaaatatttttgtgtcattttaatttaaagtaaaattgctgcttcttccccgcccctttctttcctcctggcccacccagcgaccctggccggccgtgctcaacgggggcgggggtcggaggtgagatttcctccacataattccttaaacagctatcaactaagtctcaaagaaaaaaaaaagagatctagaagcagagacgtggctgctggcgatcccaaagctggtgttcgctcttgggggagagcgtaccctgggggaggccgggaggccgggccagaggctagcccagaggcagagggcaggagcgctcagccggcgccccgcgtctctccagctcccgacgctgcgctggctccgctgagcacgccaggatcaaggtcgcctggtggggaccggagcgccaggagcctgtgggaagcgttccagccggcctctgactgggatccggcgccgcgtttctgctttggacttgactgacaggtccccccgccctcccgccgccctactaccagcctgggttcatccttcagggctacgtctaccgcacccgggctggaaagcctggagcgcgcccttcctctcctcatcttctcagctctcctttctccctgccacttggcaaagctgcattttgactttcacgttttggactacgtgtgtgtagttccaagtccatgcgtggcacgaaaatccacttagggtaaaaattattctcgaaaaatcgcccatctcaggatctggtgtctacactcaaggctaggaggtgcaggtacgggtgcgtaaagcatgccgtaagggtgcacagtaaataaaaagtacggatgcaaaatgtaaattttaagtgcaaaacagaaaagcagtactcgttgccgccccgcacgctgggttttaaggggcacgaaggtgggcctcggctgcttttgctcagccccgcgtcctcagcgcccggcccagtacccggtactccgtaggggttcaatgatctcccctgaataagtgaacgaattaacaaatgaatgaatgaccgctcgatccgacctccgcggccggcagagcagtcgctggagaggcgggagagagcgagaggccaagctccaccatcgcggccgccggctggggcagagggacacggagacactcggcgccccggctccgcaccgagtccccg

SEQ ID NO: 12766 - RNA, 13505 nt, Homo sapiens
  source 1..13505: mol_type = other RNA
gatctcactttgttgcccaggctggtcttaaactcctggcctcaagtgatccccttgtttcagccccgcaaagtgctgggattacaggtgtgagccaccatgcccgtgcccagccacctcatgagtcttgatggggggcagagaccaacaactccacagaagccagatgcttgctttcccagcctctcttgcagctagggcttgggcatgtgatccaggctcagccaatcagatggcactgactcttggcatgacatgggctaaggaggggctgcagggaatccatttgggctggggtggcagctgcactgggagcgacatcagtttccagagggagcagcagaatctggcatcaggcttggggcgtggtaggtgcaaccagactctgcacccagcagcagtggcagaatgggttctctgtggagagtctgtgtattgctccttccgctgaggccaccagcatctgcctccatgaacccctcagagcctgtgagcaactcaacagccttgaattttttcccttcctgtttgaatgagccagggttgtttcactgcttgaactaagagccgttcctgacatgaaaactaagccacatctttttgacccaaagattctggcatcctaaaatacccatctcattttaagttaaaaataaatccatgtttgagcatctactgtttcagttactgtgctaggtgttacaaagctaactaagagtgacaagtaaataactatcatcaccatgataaacagagaatggaaccctggtttttggaatacagacacaaaatgattaattctgcctggaagcgttttggaacatttcagagaggtagtgagctgggccaagagaagagcatacgcaaggaatggtggcatgaagttgcctggtgtgtcctgagaagaaagatgggctaagaaggactggggtagggcagagaagggggtcactggaggtgaggctgggaaagtgagccaaggctcaaatgcaaactgtctgaacttcattttctgtgcaagcaggagaagccgctgacatgggtttggaagatggactgaagccggagaaaaatggaagcaagaaaccctctcacaagaggccataaccacaaccaagtccatgagattgaaaaggaaggcagatatttgaaaaatatttaaagagatgtgaggggtaggacaggcacagtggctcatgcctgtagtcccagcactttgggaggccgaggtgggcagatccacgaggtcaggagatcaagaccatcctaacatggtaaaaccccatctctactaacaatacaaaaaattagtcaggtgtggtggcacgtgcctgtagtcccagctactcaggaggctgaggcaggagaatcgcttgaacctgggaggcggaggttgcagtgagccgagattgtgccactgcaccctagcctaggcaacagagcaagactctgtctcaaaaaaaataaaaaaaaaaaaaagagagaaagagagagagagatgaggagttgctgcactgctgggtgtggagagccgaggaggattcaaagatggtcctgaagtcccagctggaagaagtaggcggcagcaatgtttttaatactgtaaattcatcacgtagcacaggtttggggtggagaaagaaaaattgcattggcttcagggcatgcccagatctttcctcatcttaggcgtttgctaatacatgcattttctaagctgatgtcttgcgtttaatcactgctccattcaaaagagagaaggaggttgtttcaaacctagttgatatcatttgacttccatgctattcacagggctattttatttgaaacaggtataccacagccttaaattgcaagttaatccaggatgttcctaggttggcagttaggaacatgtaattctttggaagggctaaaagtcagctctttaaattatctccatatgaaccttctctccaccttagggtggatccacttatttagtccactgccagtaccacactagaacccgggtggtcactggactccagaaacaacagtagccctctctctgttctgtctctttttgactatctctattctgttcctgaccctgatttctcctgccaagctcaattttgacagctgacaacggcaagccatggcttcccaaaacattattttcaggtcaacttataaatttcaagaacacatttggctccgcttcctgtggtactaagcctacttcttgacagcatttgcctttgttgtaaatagcaaagttcttctagttggatttttgctaagaagtgtgtggatgtggcatgtgacgacatctttagcttggattctagaaaggcactaccattgtgcatttggctaaaggaaacacattttacccgtgaatgccttctatttacaaatgctcagctagcacacaaagctaagtacaagcaataagtactatcctacaatgttactcatttctgaaagcacaaaatgatgactggtatagctttggagatgttttctggaaacccaataaaggaacagatctttgttattccacacctacaaagtcagaagatgcacagtcttttattcatgtttgaacaagcttccttcttgaacaatcaactataaagtgatgtgattctctactagaccaggaactccttgaggacagaatgagggtctaatccatattctaaatccacaccacctggcacaatacatgttgcatggttagggtcaactaagagttggttgaattaatcaataacacacagcaagagaattcacaaagagaggggagtaatcccccagcctcaatcactcggcaagtggaatcgctgggcactgattccagctctgtctcagtgcttgagacagagctgaatgtaatgtgaacatttcaaatgaacaggaaaactagactcacggataagcagtgtagtcatcaagacaacactgtcttggaggtttttctgaagttaaaaccatgctacataagcaataaattatgaaggctgagcatgtgaataaaatttaatgttgtcataaattttataacaaagttaatctgacacatttaatgacatgcataatcattagtatgcagcactgtaatcagacattgataataagcagttcacaccagtgactgtaagagtctttacttgtgttcagccaagccaactgcttggtatatttttctcccttcttagtcgttagttttccatacctacaataactatcagtggtgatgggcttctctgaccatgtgaataatttaatcctcaatgcacagatacagaaacccttgctgaagacagtgtggagcagagaaggctgtctccactccttccacctgaaacacctctgcagatggatatgggagctctgcctacagcccttggacctaaccacttcagtgtgttccagtgagtgtctggacctcggcctgaaagatttttccgaaactaaagaaaatttctctgacctaaagaccttaacctccaccccagaagctctcaccaaggactacagggaactggtggggaaaatccttatcccttactcctcaaggcacagggcagtaatgctgaggcttgtgcgccacacttgctcccagaggtccccagcgggctacctgcggtggtgaatgacctcctaacacgccccttgacggccttcctttccttgcctcacttctccactctcctaccagcattgcagggttcacatcccaaatataccactggcacttgaatcctggtctccaggtctgtttctggaaaaacccaagtaagacattgccccagtaatggggctagatgtctgaggcttcctcaagtatctacctcgaaagctcttactgctgtacacacatgcacatacacacacgtgcgtacaaccagtcacatctaagcaccccgaataccagcctgttgaaggtagcagagagctgcactataagccaaggctgctcccaagagccgctccatcactgaattggcgccccagcaagatgaaggaatgtaatcattggaaggatggagaatgttctctgaatcactgacaaattggaaggggtggagggcaagagtccacctggtggagagatggaaagagcgagagagcctggaatgataatgccattgcttagaaaaggctgctccagatgccatatctacagaaattgtacagcccaaacatctctgagcaataggtctctggtagtcttgatgtctagaccaacaattcccagttcattcttctcagggaaggagccaggatagtccagagactctcattctgctgttagattgaaagggttaggcacaacagccttggcaaagtcacaagggcaaattcacactaaagtgtaaatgacccacaactcctcttctatttttaggttggggaggtgctttagaacataaggaggaactaaagaatattcctgttacatacaaggcagagaaaagggaaactagtggtgacaagacaaatcatccctttgacatttggctggctctacctattacagctctgggggtgaggtgggaacaaaaagatgctgtgtaaagaagtatcttatgccatccctactgtagtgaggtgcagtttagaggggacactgatcaagcagagacccagagtgtttcgttccaagccagaaacagaaatgtataaaacacagcctttccagcatcagaaatgagtagtggtagtggagaactacccaaaacaggaaagaggaccacgtgaggtagagtgtcaaggccctacattccagtgcctctgctcatgactgtaattttgggtaggtcacttaaagtctctggacctcagttttgccatctgtgaaatagggataatactatccagcataaaattggttatgaggctcatgtagggcctgcctgggatgatgtgttgctaatggttaagaacacaacttctggggtctgactggacaggctgaaatccctgcttaacacgttccagcagagccctgggcgatctatttaacttttgttttctcacctgtaagctgagacgaaagtacccactttataagattattccaataattagttgaaataatgcatgcagagaattaagcatggtacttgttatttgttaaactagctattaaaatgtgtaaaatataaagtattgtatggattttaggacaatgcaaagactctttgcttgctgcaatagttcggggccctttcagatggctaaaggcagaatttgtatgtgtaaatatggtgtgcttgtctctgctctggatactgagggcttaccctgttattaaacttatttagtaaatattgaactgtcatgaggcctaacatttagttccagttattagataaaacatttgctttgaatggtatttgaattgccaggttctagattattctggttgacaaactcttcgtattttataaagaggctaaaattggtaagctatcacagaacagatgtgccattttcaaggtatattaaaccatgattcactgtaacattgttcctactggcaacaaattcagagcaggctggactttatttggtgaagaaacattgagtggaagagaaatgacattattttatgtatttacattttcaaattactgtggcttaaacctgttcagccaacattacccaccttcagtctgctaaataaatgattcagtacatttctaatttacagaattttttaacaaaagaaaatgtaatttgatagccaaatcaacgttaaacattatacatttaaaaaaccacaggcaaagacacaaacatgatgacactaacttttgttaaagtatgcttacctatggtttcctctgaggcacgttctttcatgctaagcttccaacataatatgaaaatgaaggagatgcattttgcaaagcaaaacagaccttaagcaaaatattatacttctcaaattaacactgttacaaagttttagaatttaataagttcattaatttaaaagtttggatgtctgagtccttctatcccaaaacaagatcttggagggtcttccacagccatgtaataccatggtcacatgaccctttccaaaattattaatctgaatttactatatgaggataaatctatctttttgaaaatatttaggaaaatgagcttggtatttataaaatgaagctctctttgggtggtatcctaagacacgtcaagccaatcagcctgtaactgtgaaaaaaacattggtaggtacaaaagtggggtgggagaggagtgacttaactttgttaagtgatgggaaagaaacactaatagcattatctcaataaaatgtgatttaaaaaaatttaaaatactaaatcattgaactgacaaagaaatataaatcattcagaaataaactcattaggtcatcaaatcctgttaaatctgcaattaggaagagcaaggtgtacaatccatacatttaaactcacaggctcactttgcacaacgtcaatttactccttaatatgttattaatacgcattttccaaaaggatgtattagtaaatggtacacatctacttcttggcaacatcatataacctggtacaacataagcattcttcttatagttaagaaatgtggatggtatcaaaattagaaaaataaatgccctattatgttgtggtcaggtttaaggcatgtgaattttatcttcatacaaaagattaaaatctagatattaaaaagtagtgcagtatcagtgatgctgcctcagttcccaaaatgtcacatcacaaaaatatcccataattgcctgtagtttattccttggctttcctcttttctctctgcatctttgtaacaattttttaaaagtggaaatataattgttggcaatgctaacagctgtagaaatgattacaagatgtggaaaagcataacaggaatgtcaagaatctgtttctggcagtaatatatatggaacattgttcaggacaaaagaggagaaggaagaaaaaaaggagaggggtttatcatctctaagaattttcaaactaaacctcattgcttaataggaaaaaaagattccatatttaaagttaagtcacctctaactactagctaaagcatgacatcaccagcactggagtcagcggaagtgtgtttttgaaggacagtgttgcaggagaatctggacaggttttagagccaggagagagaaaataattctacctctgacagttgaaggaccttaggcaaatcagtttacctctgctagactacactccaaaatttggacattcaaaaatttgatattaataaccacatgaaagtctcgtgttgaggtgaatatgtatttgttggtgaaagatatgttggtttttaaacagacagcactctgcaattgtaggctattgttttgttttgccagttgtcaaattctatccagctatacacacttgtgtggcctcctaatggtgtttttccagtggctaaaggtttatgaataagacacttttcctaatggaattaacccgatgcttttcttaaacatgtaaccttgagttcaccgcaaaaaacaatgcttcgattagagcaatgcatataataaaggttaccctcgtttcttagacactagacatcattcacaaaaagagaactgcttttgaaagggatgtatttgcactggaaagaatagttttctacttctaattataaatgatttattggtgaaagcaaaacaacagcctgtctgagaggcacttctatgagcatcctcacgtgtgatttgcaaggttgaagaagagggaaaaatgcctcaattgtaccaatggtgagaaaacacccaaagtacaaagcaggtttcaaaaaaaccatactcataaccaaggacaataataaagcaatgtgttgacatatactctataagtcttcctccataaatagtttatagaaattttgtaatttctgtaaatgcatcctataataattttgcatcttgctttttttttacatttaatatcaagtagatttctaaagggcaattatttgaaaattatcccaaatacatggggaaatatacatcaagtgaaaaaatgcagtgggtgatagagatatcaggaagcgcctcaaatatttctcatctcgttggagaaaaacaaacatgttctcatttagaatgagtgggagttacctaattgatttaggcctctatatttaacttctagtcaaaaaaggtagttctatctagcaacaatattatggggaacaaaagaaaaaattaactctctaaatttgcagtagggtcttttcttcagaagtaccaaatcccatctattaccagctccatgcttcaggcctaaaatggatctccctgaagcaatgacagaatttttgccaagtgactaggatataaacaccactttggttgcacagtgagacatatgctccaaagaaaactggttcaaaaacaggcaagtgggtttctacagaataaatgagagccctgtcaatggcttcatcttcagggctttgtgtctgtgcttgcgtggtggctcttgtttcatctatggataatggtggcacacagttttcataattccttacattaatgaactgctataaatttgtttttggtattctagagagtcctaacttcagcttctgggcaatgctgaggaggcaccctatattctagacttaccttttgcaaggtgtactctcagcattgtgggcgatttccatgggagaatattctatttaaagaactactgtcccagcataaaacaaaaaatcatttatgaagatgcaggagactcggaaagctctcaattattgtttgcacaagcacaatgtcacagcctcctttccccattccacaagggggtcaggaagagagtactcagctgtgagaaaagacatacagaagaattcatgtggtcatgagagcgaggacatggccgatcccccaaggaggatgtgtcatacacttcatgagcccaagagtgtgctgtagggtctgaagggcaagatgctggttcactgatgtaaaggagagggaaaaaagcttcaaccaactagaaaaacagtctctatgcatgctatttttgattttaaacacaggtatcaattccttctctcagagagtccattttaaaataggatacatttttaaaggaatatttaaaggacacattcattaaaatttattttaaaaacttttcaaaagaaacaaaaggtatgaattttatttaatccttgaggaaatggttcttttctcacacacataaatcactcattttgtttttctttatctcctttattaatctacattagaaaaataaacttttcatacactaagaacaaggaaaccactctcaattgacaaaatgttccaatccaacacaatgattactttcacctttaatttacaggcagccagattcaaaatccttaaagttgcttaaacttaaaaatgacaatgacaacctaaaaggtataatgttgattggaacagacatttaattggaaaattgatgattttccatttccaattaaatctctagatagaaatgaaaaaaattaaaaatcgtatttaagaaaagccaaatcttgggttgtgaggtatctttttaaggatgtttcagcagaaaaaaacaaaggctctcacaattgtgtagctgcctagattaagtgggtatcctgatcaaggagatgggggatgatttggctttagtattccaatgataaagtttataatgagaataacatgttgctacaaaatccagtctcttcctcagatgccttccacagagggcaggaagctttgtcagttttgtttgctgatgatgcctggttccgtcaacaaataacacctgtcacacggtgggtagtcaatatacatttgttgaataaatatgaaaaaaagaaatgtacaatatgtttgtgaagccaactgtgtgtgcattgctattgaggtacacaaaaagtctttgttttaaatttgagaatgaggactttcaatggaatatatctgataggcctggatcaagcatgcagctgtggagaacacccctgggactctaactctggcactctgcaagctgggtacttgggcaggacagcagcagcactcatgaactgggcagcacctgttggtgagggctgatcacatggattctctcatcccagccttacaatcagtccttcaggtacatactttttctgactttgctgatgaggaaactatgcacagaggttacacagcttaacaaagggttctcacctctcttcaagtggtatttaaatttcttctttcattttccttctggtaacaaagaagtctgtggctcaaaagatgtttctctaagaccccatcctattaggtctctgagattttagaaatgacccaacttgatccttttattcttcagaatatctctctcaaattttcatttgtttttcattaattgatgaataatgagacattttaggtacctgtccacaaagaaatgaaattttcactttccaggaacctaacaaatgaaaagatagaaatcaattccaacagaatattaccaaagaaatcttttagaatggactgttaaaattatttatttgtatttatctggctctactatttgtggtacatttccacttcaaagctaaacctcaaataacatcatagtgagtggttgacttcatgtttaactgagatcttgaagactgaaaaagaccacgacaaacacacatctattttcttggctactgcatccgtgttcatcaccattctgatagtctgcaatgtattgcagctcaccctttgggaaggactaaagtagacatctgtttgttctgcttactcagcattcctaccctaattttcctttggagaacccctttattctagaccacgtgaagctaatgccaaaccccattccaggggatgcacctgaatccaacctccatcatctaaacagtgccttctccacgttcagagaagagcaagtgactcaaactgccctcataagaacagacctgggacttctgctgcaaatattgaagagtaagtactcttttttcttgctaggactaagctggtagtaccttctatgaggctatcatatggaaacaacttgtctgaaaatgaagccacaactagaaaacagatcctggtaacccggattgatggatccagccctaccttaaatggcaagacctaacccgaggctttttgcatcaaccaataaagtccttaagccagtttgagttggttttgtcacttgcagctaaaagaattctgactctaacaatgtgacaatagcaaaaataaacataactgcttttgaggtttctaatggattttcctccctatatacatgatttcatttaatcctcacaattcaggaaagcacatatctattaacattaaattaatattcattattttgaacacatgctatgtggataagggatgaggaaagccaaggaagtaatcaacgtgaaatctcacttatatgggagggaagtggaggttacatatctcagggcacttaacagatatcatcaaatgaaagaataaacagtgtgtgggagaggcagtaggtgattcttcatcaattcctggatgaaaaattaggagataatgaactccgaacaggcagcctaatgagaatggctcaagcaacaggacatagagagggagttaggttagacatggggttcttgggaattttcacctcgtgggggggcgggggggtcgtgcagctgttgtcagtgggaaagggaaaaaggaaaaggctgagtttggaaggcagggagggaggagacaatgtgagtcagtgaaaaagggcccttagaatgacaagtctggaccagagagaggctaagactgaaaatacaagttgggtaaccactggcatacagatggcagttcaggcttgggcactgcccaccagagcctcagcatgaagagaagagggggaggctggccaccacctccctctaggtaatcgtcatcctgatgctgagctcctgaaaacaggctctttcactcgccccatctcttgctcttgattgcaacccggcattcaggaggcaccctgtaatatctgtggagtgaccgacaacacagcgccagggcactgagaagatcccagggcgccagggactggttctacaagggtgcccctcccggtcccctccagcgcgccgccagagctgccagtcttggctgctacacgggaggcagcctcattatgcagctctcacctcttaaattagttcatgctctcacattaggtgtaatcacagcttgcaacgctttctggggatgtctcagaaagatctgagttgaaaaaatatttttgtgtcattttaatttaaagtaaaattgctgcttcttccccgcccctttctttcctcctggcccacccagcgaccctggccggccgtgctcaacgggggcgggggtcggaggtgagatttcctccacataattccttaaacagctatcaactaagtctcaaagaaaaaaaaaagagatctagaagcagagacgtggctgctggcgatcccaaagctggtgttcgctcttgggggagagcgtaccctgggggaggccgggaggccgggccagaggctagcccagaggcagagggcaggagcgctcagccggcgccccgcgtctctccagctcccgacgctgcgctggctccgctgagcacgccaggatcaaggtcgcctggtggggaccggagcgccaggagcctgtgggaagcgttccagccggcctctgactgggatccggcgccgcgtttctgctttggacttgactgacaggtccccccgccctcccgccgccctactaccagcctgggttcatccttcagggctacgtctaccgcacccgggctggaaagcctggagcgcgcccttcctctcctcatcttctcagctctcctttctccctgccacttggcaaagctgcattttgactttcacgttttggactacgtgtgtgtagttccaagtccatgcgtggcacgaaaatccacttagggtaaaaattattctcgaaaaatcgcccatctcaggatctggtgtctacactcaaggctaggaggtgcaggtacgggtgcgtaaagcatgccgtaagggtgcacagtaaataaaaagtacggatgcaaaatgtaaattttaagtgcaaaacagaaaagcagtactcgttgccgccccgcacgctgggttttaaggggcacgaaggtgggcctcggctgcttttgctcagccccgcgtcctcagcgcccggcccagtacccggtactccgtaggggttcaatgatctcccctgaataagtgaacgaattaacaaatgaatgaatgaccgctcgatccgacctccgcggccggcagagcagtcgctggagaggcgggagagagcgagaggccaagctccaccatcgcggccgccggctggggcagagggacacggagacactcggcgccccggctccgcaccgagtccc

SEQ ID NO: 12767 - RNA, 15247 nt, Homo sapiens
  source 1..15247: mol_type = other RNA
gatctcactttgttgcccaggctggtcttaaactcctggcctcaagtgatccccttgtttcagccccgcaaagtgctgggattacaggtgtgagccaccatgcccgtgcccagccacctcatgagtcttgatggggggcagagaccaacaactccacagaagccagatgcttgctttcccagcctctcttgcagctagggcttgggcatgtgatccaggctcagccaatcagatggcactgactcttggcatgacatgggctaaggaggggctgcagggaatccatttgggctggggtggcagctgcactgggagcgacatcagtttccagagggagcagcagaatctggcatcaggcttggggcgtggtaggtgcaaccagactctgcacccagcagcagtggcagaatgggttctctgtggagagtctgtgtattgctccttccgctgaggccaccagcatctgcctccatgaacccctcagagcctgtgagcaactcaacagccttgaattttttcccttcctgtttgaatgagccagggttgtttcactgcttgaactaagagccgttcctgacatgaaaactaagccacatctttttgacccaaagattctggcatcctaaaatacccatctcattttaagttaaaaataaatccatgtttgagcatctactgtttcagttactgtgctaggtgttacaaagctaactaagagtgacaagtaaataactatcatcaccatgataaacagagaatggaaccctggtttttggaatacagacacaaaatgattaattctgcctggaagcgttttggaacatttcagagaggtagtgagctgggccaagagaagagcatacgcaaggaatggtggcatgaagttgcctggtgtgtcctgagaagaaagatgggctaagaaggactggggtagggcagagaagggggtcactggaggtgaggctgggaaagtgagccaaggctcaaatgcaaactgtctgaacttcattttctgtgcaagcaggagaagccgctgacatgggtttggaagatggactgaagccggagaaaaatggaagcaagaaaccctctcacaagaggccataaccacaaccaagtccatgagattgaaaaggaaggcagatatttgaaaaatatttaaagagatgtgaggggtaggacaggcacagtggctcatgcctgtagtcccagcactttgggaggccgaggtgggcagatccacgaggtcaggagatcaagaccatcctaacatggtaaaaccccatctctactaacaatacaaaaaattagtcaggtgtggtggcacgtgcctgtagtcccagctactcaggaggctgaggcaggagaatcgcttgaacctgggaggcggaggttgcagtgagccgagattgtgccactgcaccctagcctaggcaacagagcaagactctgtctcaaaaaaaataaaaaaaaaaaaaagagagaaagagagagagagatgaggagttgctgcactgctgggtgtggagagccgaggaggattcaaagatggtcctgaagtcccagctggaagaagtaggcggcagcaatgtttttaatactgtaaattcatcacgtagcacaggtttggggtggagaaagaaaaattgcattggcttcagggcatgcccagatctttcctcatcttaggcgtttgctaatacatgcattttctaagctgatgtcttgcgtttaatcactgctccattcaaaagagagaaggaggttgtttcaaacctagttgatatcatttgacttccatgctattcacagggctattttatttgaaacaggtataccacagccttaaattgcaagttaatccaggatgttcctaggttggcagttaggaacatgtaattctttggaagggctaaaagtcagctctttaaattatctccatatgaaccttctctccaccttagggtggatccacttatttagtccactgccagtaccacactagaacccgggtggtcactggactccagaaacaacagtagccctctctctgttctgtctctttttgactatctctattctgttcctgaccctgatttctcctgccaagctcaattttgacagctgacaacggcaagccatggcttcccaaaacattattttcaggtcaacttataaatttcaagaacacatttggctccgcttcctgtggtactaagcctacttcttgacagcatttgcctttgttgtaaatagcaaagttcttctagttggatttttgctaagaagtgtgtggatgtggcatgtgacgacatctttagcttggattctagaaaggcactaccattgtgcatttggctaaaggaaacacattttacccgtgaatgccttctatttacaaatgctcagctagcacacaaagctaagtacaagcaataagtactatcctacaatgttactcatttctgaaagcacaaaatgatgactggtatagctttggagatgttttctggaaacccaataaaggaacagatctttgttattccacacctacaaagtcagaagatgcacagtcttttattcatgtttgaacaagcttccttcttgaacaatcaactataaagtgatgtgattctctactagaccaggaactccttgaggacagaatgagggtctaatccatattctaaatccacaccacctggcacaatacatgttgcatggttagggtcaactaagagttggttgaattaatcaataacacacagcaagagaattcacaaagagaggggagtaatcccccagcctcaatcactcggcaagtggaatcgctgggcactgattccagctctgtctcagtgcttgagacagagctgaatgtaatgtgaacatttcaaatgaacaggaaaactagactcacggataagcagtgtagtcatcaagacaacactgtcttggaggtttttctgaagttaaaaccatgctacataagcaataaattatgaaggctgagcatgtgaataaaatttaatgttgtcataaattttataacaaagttaatctgacacatttaatgacatgcataatcattagtatgcagcactgtaatcagacattgataataagcagttcacaccagtgactgtaagagtctttacttgtgttcagccaagccaactgcttggtatatttttctcccttcttagtcgttagttttccatacctacaataactatcagtggtgatgggcttctctgaccatgtgaataatttaatcctcaatgcacagatacagaaacccttgctgaagacagtgtggagcagagaaggctgtctccactccttccacctgaaacacctctgcagatggatatgggagctctgcctacagcccttggacctaaccacttcagtgtgttccagtgagtgtctggacctcggcctgaaagatttttccgaaactaaagaaaatttctctgacctaaagaccttaacctccaccccagaagctctcaccaaggactacagggaactggtggggaaaatccttatcccttactcctcaaggcacagggcagtaatgctgaggcttgtgcgccacacttgctcccagaggtccccagcgggctacctgcggtggtgaatgacctcctaacacgccccttgacggccttcctttccttgcctcacttctccactctcctaccagcattgcagggttcacatcccaaatataccactggcacttgaatcctggtctccaggtctgtttctggaaaaacccaagtaagacattgccccagtaatggggctagatgtctgaggcttcctcaagtatctacctcgaaagctcttactgctgtacacacatgcacatacacacacgtgcgtacaaccagtcacatctaagcaccccgaataccagcctgttgaaggtagcagagagctgcactataagccaaggctgctcccaagagccgctccatcactgaattggcgccccagcaagatgaaggaatgtaatcattggaaggatggagaatgttctctgaatcactgacaaattggaaggggtggagggcaagagtccacctggtggagagatggaaagagcgagagagcctggaatgataatgccattgcttagaaaaggctgctccagatgccatatctacagaaattgtacagcccaaacatctctgagcaataggtctctggtagtcttgatgtctagaccaacaattcccagttcattcttctcagggaaggagccaggatagtccagagactctcattctgctgttagattgaaagggttaggcacaacagccttggcaaagtcacaagggcaaattcacactaaagtgtaaatgacccacaactcctcttctatttttaggttggggaggtgctttagaacataaggaggaactaaagaatattcctgttacatacaaggcagagaaaagggaaactagtggtgacaagacaaatcatccctttgacatttggctggctctacctattacagctctgggggtgaggtgggaacaaaaagatgctgtgtaaagaagtatcttatgccatccctactgtagtgaggtgcagtttagaggggacactgatcaagcagagacccagagtgtttcgttccaagccagaaacagaaatgtataaaacacagcctttccagcatcagaaatgagtagtggtagtggagaactacccaaaacaggaaagaggaccacgtgaggtagagtgtcaaggccctacattccagtgcctctgctcatgactgtaattttgggtaggtcacttaaagtctctggacctcagttttgccatctgtgaaatagggataatactatccagcataaaattggttatgaggctcatgtagggcctgcctgggatgatgtgttgctaatggttaagaacacaacttctggggtctgactggacaggctgaaatccctgcttaacacgttccagcagagccctgggcgatctatttaacttttgttttctcacctgtaagctgagacgaaagtacccactttataagattattccaataattagttgaaataatgcatgcagagaattaagcatggtacttgttatttgttaaactagctattaaaatgtgtaaaatataaagtattgtatggattttaggacaatgcaaagactctttgcttgctgcaatagttcggggccctttcagatggctaaaggcagaatttgtatgtgtaaatatggtgtgcttgtctctgctctggatactgagggcttaccctgttattaaacttatttagtaaatattgaactgtcatgaggcctaacatttagttccagttattagataaaacatttgctttgaatggtatttgaattgccaggttctagattattctggttgacaaactcttcgtattttataaagaggctaaaattggtaagctatcacagaacagatgtgccattttcaaggtatattaaaccatgattcactgtaacattgttcctactggcaacaaattcagagcaggctggactttatttggtgaagaaacattgagtggaagagaaatgacattattttatgtatttacattttcaaattactgtggcttaaacctgttcagccaacattacccaccttcagtctgctaaataaatgattcagtacatttctaatttacagaattttttaacaaaagaaaatgtaatttgatagccaaatcaacgttaaacattatacatttaaaaaaccacaggcaaagacacaaacatgatgacactaacttttgttaaagtatgcttacctatggtttcctctgaggcacgttctttcatgctaagcttccaacataatatgaaaatgaaggagatgcattttgcaaagcaaaacagaccttaagcaaaatattatacttctcaaattaacactgttacaaagttttagaatttaataagttcattaatttaaaagtttggatgtctgagtccttctatcccaaaacaagatcttggagggtcttccacagccatgtaataccatggtcacatgaccctttccaaaattattaatctgaatttactatatgaggataaatctatctttttgaaaatatttaggaaaatgagcttggtatttataaaatgaagctctctttgggtggtatcctaagacacgtcaagccaatcagcctgtaactgtgaaaaaaacattggtaggtacaaaagtggggtgggagaggagtgacttaactttgttaagtgatgggaaagaaacactaatagcattatctcaataaaatgtgatttaaaaaaatttaaaatactaaatcattgaactgacaaagaaatataaatcattcagaaataaactcattaggtcatcaaatcctgttaaatctgcaattaggaagagcaaggtgtacaatccatacatttaaactcacaggctcactttgcacaacgtcaatttactccttaatatgttattaatacgcattttccaaaaggatgtattagtaaatggtacacatctacttcttggcaacatcatataacctggtacaacataagcattcttcttatagttaagaaatgtggatggtatcaaaattagaaaaataaatgccctattatgttgtggtcaggtttaaggcatgtgaattttatcttcatacaaaagattaaaatctagatattaaaaagtagtgcagtatcagtgatgctgcctcagttcccaaaatgtcacatcacaaaaatatcccataattgcctgtagtttattccttggctttcctcttttctctctgcatctttgtaacaattttttaaaagtggaaatataattgttggcaatgctaacagctgtagaaatgattacaagatgtggaaaagcataacaggaatgtcaagaatctgtttctggcagtaatatatatggaacattgttcaggacaaaagaggagaaggaagaaaaaaaggagaggggtttatcatctctaagaattttcaaactaaacctcattgcttaataggaaaaaaagattccatatttaaagttaagtcacctctaactactagctaaagcatgacatcaccagcactggagtcagcggaagtgtgtttttgaaggacagtgttgcaggagaatctggacaggttttagagccaggagagagaaaataattctacctctgacagttgaaggaccttaggcaaatcagtttacctctgctagactacactccaaaatttggacattcaaaaatttgatattaataaccacatgaaagtctcgtgttgaggtgaatatgtatttgttggtgaaagatatgttggtttttaaacagacagcactctgcaattgtaggctattgttttgttttgccagttgtcaaattctatccagctatacacacttgtgtggcctcctaatggtgtttttccagtggctaaaggtttatgaataagacacttttcctaatggaattaacccgatgcttttcttaaacatgtaaccttgagttcaccgcaaaaaacaatgcttcgattagagcaatgcatataataaaggttaccctcgtttcttagacactagacatcattcacaaaaagagaactgcttttgaaagggatgtatttgcactggaaagaatagttttctacttctaattataaatgatttattggtgaaagcaaaacaacagcctgtctgagaggcacttctatgagcatcctcacgtgtgatttgcaaggttgaagaagagggaaaaatgcctcaattgtaccaatggtgagaaaacacccaaagtacaaagcaggtttcaaaaaaaccatactcataaccaaggacaataataaagcaatgtgttgacatatactctataagtcttcctccataaatagtttatagaaattttgtaatttctgtaaatgcatcctataataattttgcatcttgctttttttttacatttaatatcaagtagatttctaaagggcaattatttgaaaattatcccaaatacatggggaaatatacatcaagtgaaaaaatgcagtgggtgatagagatatcaggaagcgcctcaaatatttctcatctcgttggagaaaaacaaacatgttctcatttagaatgagtgggagttacctaattgatttaggcctctatatttaacttctagtcaaaaaaggtagttctatctagcaacaatattatggggaacaaaagaaaaaattaactctctaaatttgcagtagggtcttttcttcagaagtaccaaatcccatctattaccagctccatgcttcaggcctaaaatggatctccctgaagcaatgacagaatttttgccaagtgactaggatataaacaccactttggttgcacagtgagacatatgctccaaagaaaactggttcaaaaacaggcaagtgggtttctacagaataaatgagagccctgtcaatggcttcatcttcagggctttgtgtctgtgcttgcgtggtggctcttgtttcatctatggataatggtggcacacagttttcataattccttacattaatgaactgctataaatttgtttttggtattctagagagtcctaacttcagcttctgggcaatgctgaggaggcaccctatattctagacttaccttttgcaaggtgtactctcagcattgtgggcgatttccatgggagaatattctatttaaagaactactgtcccagcataaaacaaaaaatcatttatgaagatgcaggagactcggaaagctctcaattattgtttgcacaagcacaatgtcacagcctcctttccccattccacaagggggtcaggaagagagtactcagctgtgagaaaagacatacagaagaattcatgtggtcatgagagcgaggacatggccgatcccccaaggaggatgtgtcatacacttcatgagcccaagagtgtgctgtagggtctgaagggcaagatgctggttcactgatgtaaaggagagggaaaaaagcttcaaccaactagaaaaacagtctctatgcatgctatttttgattttaaacacaggtatcaattccttctctcagagagtccattttaaaataggatacatttttaaaggaatatttaaaggacacattcattaaaatttattttaaaaacttttcaaaagaaacaaaaggtatgaattttatttaatccttgaggaaatggttcttttctcacacacataaatcactcattttgtttttctttatctcctttattaatctacattagaaaaataaacttttcatacactaagaacaaggaaaccactctcaattgacaaaatgttccaatccaacacaatgattactttcacctttaatttacaggcagccagattcaaaatccttaaagttgcttaaacttaaaaatgacaatgacaacctaaaaggtataatgttgattggaacagacatttaattggaaaattgatgattttccatttccaattaaatctctagatagaaatgaaaaaaattaaaaatcgtatttaagaaaagccaaatcttgggttgtgaggtatctttttaaggatgtttcagcagaaaaaaacaaaggctctcacaattgtgtagctgcctagattaagtgggtatcctgatcaaggagatgggggatgatttggctttagtattccaatgataaagtttataatgagaataacatgttgctacaaaatccagtctcttcctcagatgccttccacagagggcaggaagctttgtcagttttgtttgctgatgatgcctggttccgtcaacaaataacacctgtcacacggtgggtagtcaatatacatttgttgaataaatatgaaaaaaagaaatgtacaatatgtttgtgaagccaactgtgtgtgcattgctattgaggtacacaaaaagtctttgttttaaatttgagaatgaggactttcaatggaatatatctgataggcctggatcaagcatgcagctgtggagaacacccctgggactctaactctggcactctgcaagctgggtacttgggcaggacagcagcagcactcatgaactgggcagcacctgttggtgagggctgatcacatggattctctcatcccagccttacaatcagtccttcaggtacatactttttctgactttgctgatgaggaaactatgcacagaggttacacagcttaacaaagggttctcacctctcttcaagtggtatttaaatttcttctttcattttccttctggtaacaaagaagtctgtggctcaaaagatgtttctctaagaccccatcctattaggtctctgagctgtgggaagtatttatacaattgcttgtgaatataagatccaggaatttccctaagatccctaacaaaattggtgataagtagtcccacatgttaatccagccacccacggatgacagcacttaccatttctttgataaatgtcaaatgcatttgaagtacctacctgaaatatttgtttaaatgctatctaatctattaattttatatatgtgtgagtctgttttgtataccttctgattataggataaatgtaaataaatccaaagagtaatcaaagctaccactttcaagaagccttctttgtagaaccggaagagtcttaaataggcttttcaggtatgcatctcttattatcgctgaactccaagtcctgcaaggcaggcatcatgtgtgggtcacctttacagtaggcacaggccttaaaacagtgacatgcacattgcaggcactccataaatgtttgctgaattggctaaaccttggtttgttcccataatcaaccaccacaaacagcacacagataattacttcttggaaagattccaactagtgtttgatgttacctacgtggtttttctctcaagatcttaagagcagctctgtaggattacattattttctgttttttttttcctttgaccttaatgtcatctacttcaataacagcttcatacaaaattcctaccagcacataccacagcagattcaaggccttgttttaaaaatggtgccagcttctcttaatttggaagatatattgtctctcctgaacatgggctaagaaaatgtataatttggtattaacataagagctgaagacactttaaatgcattgtttcatttttataagataaaaaaaattttaagaatcaaaatgttatcaacagacttgtccttcattaaaaagtaaaactgcatttgcctacattttatgaaagtgtccaattatgaacaattttgaaatgtaacttttaaaaatgtaaacagcaaaaatgttgtatttaaaataaatctggaaaggcagaaaaacaaaaaatacccagaagacagagtttttggtgaaagttaagatatttcatctttgaacaacttagaatctttcctgcattttatagtctagttccaggcattaatttgaaataaccttggaatcctaaatctaacacccttcggaacaaagtagcttttctcttctgctttatgagcaaatggactaaatactagggaatggtactgtctgggcctttgaaccaagattgaaagagatgaaatcctatatgatatgtataaacattagagaatccattttgatttaataaaaggttgaatttgttctatatcctgtgagaaaatggttcccttttcctgaaaatgttacctcattccaacaatagaaagttggtttttttccagggtgtggtgttggcgggggacagagttgccatgaatatggcatctatgaagactgctgttatattcatttctcaaaatgcactgtggtaggaaattcagaacgcagtgagagaaaataaatgtttgacttcaaaatataaggccgcatttaaagcagaaggtaaagtatagaacagttgacagtataaattctttatctgcaatcttgcagttccctaaatctctgtaacacatcacttttaaaagcctcagataagtggttctataataatttaccaataattcaacccctcaaaagtcttagcaagttaaaccttataatcttacattttagaaatgacccaacttgatccttttattcttcagaatatctctctcaaattttcatttgtttttcattaattgatgaataatgagacattttaggtacctgtccacaaagaaatgaaattttcactttccaggaacctaacaaatgaaaagatagaaatcaattccaacagaatattaccaaagaaatcttttagaatggactgttaaaattatttatttgtatttatctggctctactatttgtggtacatttccacttcaaagctaaacctcaaataacatcatagtgagtggttgacttcatgtttaactgagatcttgaagactgaaaaagaccacgacaaacacacatctattttcttggctactgcatccgtgttcatcaccattctgatagtctgcaatgtattgcagctcaccctttgggaaggactaaagtagacatctgtttgttctgcttactcagcattcctaccctaattttcctttggagaacccctttattctagaccacgtgaagctaatgccaaaccccattccaggggatgcacctgaatccaacctccatcatctaaacagtgccttctccacgttcagagaagagcaagtgactcaaactgccctcataagaacagacctgggacttctgctgcaaatattgaagagtaagtactcttttttcttgctaggactaagctggtagtaccttctatgaggctatcatatggaaacaacttgtctgaaaatgaagccacaactagaaaacagatcctggtaacccggattgatggatccagccctaccttaaatggcaagacctaacccgaggctttttgcatcaaccaataaagtccttaagccagtttgagttggttttgtcacttgcagctaaaagaattctgactctaacaatgtgacaatagcaaaaataaacataactgcttttgaggtttctaatggattttcctccctatatacatgatttcatttaatcctcacaattcaggaaagcacatatctattaacattaaattaatattcattattttgaacacatgctatgtggataagggatgaggaaagccaaggaagtaatcaacgtgaaatctcacttatatgggagggaagtggaggttacatatctcagggcacttaacagatatcatcaaatgaaagaataaacagtgtgtgggagaggcagtaggtgattcttcatcaattcctggatgaaaaattaggagataatgaactccgaacaggcagcctaatgagaatggctcaagcaacaggacatagagagggagttaggttagacatggggttcttgggaattttcacctcgtgggggggcgggggggtcgtgcagctgttgtcagtgggaaagggaaaaaggaaaaggctgagtttggaaggcagggagggaggagacaatgtgagtcagtgaaaaagggcccttagaatgacaagtctggaccagagagaggctaagactgaaaatacaagttgggtaaccactggcatacagatggcagttcaggcttgggcactgcccaccagagcctcagcatgaagagaagagggggaggctggccaccacctccctctaggtaatcgtcatcctgatgctgagctcctgaaaacaggctctttcactcgccccatctcttgctcttgattgcaacccggcattcaggaggcaccctgtaatatctgtggagtgaccgacaacacagcgccagggcactgagaagatcccagggcgccagggactggttctacaagggtgcccctcccggtcccctccagcgcgccgccagagctgccagtcttggctgctacacgggaggcagcctcattatgcagctctcacctcttaaattagttcatgctctcacattaggtgtaatcacagcttgcaacgctttctggggatgtctcagaaagatctgagttgaaaaaatatttttgtgtcattttaatttaaagtaaaattgctgcttcttccccgcccctttctttcctcctggcccacccagcgaccctggccggccgtgctcaacgggggcgggggtcggaggtgagatttcctccacataattccttaaacagctatcaactaagtctcaaagaaaaaaaaaagagatctagaagcagagacgtggctgctggcgatcccaaagctggtgttcgctcttgggggagagcgtaccctgggggaggccgggaggccgggccagaggctagcccagaggcagagggcaggagcgctcagccggcgccccgcgtctctccagctcccgacgctgcgctggctccgctgagcacgccaggatcaaggtcgcctggtggggaccggagcgccaggagcctgtgggaagcgttccagccggcctctgactgggatccggcgccgcgtttctgctttggacttgactgacaggtccccccgccctcccgccgccctactaccagcctgggttcatccttcagggctacgtctaccgcacccgggctggaaagcctggagcgcgcccttcctctcctcatcttctcagctctcctttctccctgccacttggcaaagctgcattttgactttcacgttttggactacgtgtgtgtagttccaagtccatgcgtggcacgaaaatccacttagggtaaaaattattctcgaaaaatcgcccatctcaggatctggtgtctacactcaaggctaggaggtgcaggtacgggtgcgtaaagcatgccgtaagggtgcacagtaaataaaaagtacggatgcaaaatgtaaattttaagtgcaaaacagaaaagcagtactcgttgccgccccgcacgctgggttttaaggggcacgaaggtgggcctcggctgcttttgctcagccccgcgtcctcagcgcccggcccagtacccggtactccgtaggggttcaatgatctcccctgaataagtgaacgaattaacaaatgaatgaatgaccgctcgatccgacctccgcggccggcagagcagtcgctggagaggcgggagagagcgagaggccaagctccaccatcgcggccgccggctggggcagagggacacggagacactcggcgccccggctccgcaccgagtcc

SEQ ID NO: 12768 - RNA, 15207 nt, Homo sapiens
  source 1..15207: mol_type = other RNA
gatctcactttgttgcccaggctggtcttaaactcctggcctcaagtgatccccttgtttcagccccgcaaagtgctgggattacaggtgtgagccaccatgcccgtgcccagccacctcatgagtcttgatggggggcagagaccaacaactccacagaagccagatgcttgctttcccagcctctcttgcagctagggcttgggcatgtgatccaggctcagccaatcagatggcactgactcttggcatgacatgggctaaggaggggctgcagggaatccatttgggctggggtggcagctgcactgggagcgacatcagtttccagagggagcagcagaatctggcatcaggcttggggcgtggtaggtgcaaccagactctgcacccagcagcagtggcagaatgggttctctgtggagagtctgtgtattgctccttccgctgaggccaccagcatctgcctccatgaacccctcagagcctgtgagcaactcaacagccttgaattttttcccttcctgtttgaatgagccagggttgtttcactgcttgaactaagagccgttcctgacatgaaaactaagccacatctttttgacccaaagattctggcatcctaaaatacccatctcattttaagttaaaaataaatccatgtttgagcatctactgtttcagttactgtgctaggtgttacaaagctaactaagagtgacaagtaaataactatcatcaccatgataaacagagaatggaaccctggtttttggaatacagacacaaaatgattaattctgcctggaagcgttttggaacatttcagagaggtagtgagctgggccaagagaagagcatacgcaaggaatggtggcatgaagttgcctggtgtgtcctgagaagaaagatgggctaagaaggactggggtagggcagagaagggggtcactggaggtgaggctgggaaagtgagccaaggctcaaatgcaaactgtctgaacttcattttctgtgcaagcaggagaagccgctgacatgggtttggaagatggactgaagccggagaaaaatggaagcaagaaaccctctcacaagaggccataaccacaaccaagtccatgagattgaaaaggaaggcagatatttgaaaaatatttaaagagatgtgaggggtaggacaggcacagtggctcatgcctgtagtcccagcactttgggaggccgaggtgggcagatccacgaggtcaggagatcaagaccatcctaacatggtaaaaccccatctctactaacaatacaaaaaattagtcaggtgtggtggcacgtgcctgtagtcccagctactcaggaggctgaggcaggagaatcgcttgaacctgggaggcggaggttgcagtgagccgagattgtgccactgcaccctagcctaggcaacagagcaagactctgtctcaaaaaaaataaaaaaaaaaaaaagagagaaagagagagagagatgaggagttgctgcactgctgggtgtggagagccgaggaggattcaaagatggtcctgaagtcccagctggaagaagtaggcggcagcaatgtttttaatactgtaaattcatcacgtagcacaggtttggggtggagaaagaaaaattgcattggcttcagggcatgcccagatctttcctcatcttaggcgtttgctaatacatgcattttctaagctgatgtcttgcgtttaatcactgctccattcaaaagagagaaggaggttgtttcaaacctagttgatatcatttgacttccatgctattcacagggctattttatttgaaacaggtataccacagccttaaattgcaagttaatccaggatgttcctaggttggcagttaggaacatgtaattctttggaagggctaaaagtcagctctttaaattatctccatatgaaccttctctccaccttagggtggatccacttatttagtccactgccagtaccacactagaacccgggtggtcactggactccagaaacaacagtagccctctctctgttctgtctctttttgactatctctattctgttcctgaccctgatttctcctgccaagctcaattttgacagctgacaacggcaagccatggcttcccaaaacattattttcaggtcaacttataaatttcaagaacacatttggctccgcttcctgtggtactaagcctacttcttgacagcatttgcctttgttgtaaatagcaaagttcttctagttggatttttgctaagaagtgtgtggatgtggcatgtgacgacatctttagcttggattctagaaaggcactaccattgtgcatttggctaaaggaaacacattttacccgtgaatgccttctatttacaaatgctcagctagcacacaaagctaagtacaagcaataagtactatcctacaatgttactcatttctgaaagcacaaaatgatgactggtatagctttggagatgttttctggaaacccaataaaggaacagatctttgttattccacacctacaaagtcagaagatgcacagtcttttattcatgtttgaacaagcttccttcttgaacaatcaactataaagtgatgtgattctctactagaccaggaactccttgaggacagaatgagggtctaatccatattctaaatccacaccacctggcacaatacatgttgcatggttagggtcaactaagagttggttgaattaatcaataacacacagcaagagaattcacaaagagaggggagtaatcccccagcctcaatcactcggcaagtggaatcgctgggcactgattccagctctgtctcagtgcttgagacagagctgaatgtaatgtgaacatttcaaatgaacaggaaaactagactcacggataagcagtgtagtcatcaagacaacactgtcttggaggtttttctgaagttaaaaccatgctacataagcaataaattatgaaggctgagcatgtgaataaaatttaatgttgtcataaattttataacaaagttaatctgacacatttaatgacatgcataatcattagtatgcagcactgtaatcagacattgataataagcagttcacaccagtgactgtaagagtctttacttgtgttcagccaagccaactgcttggtatatttttctcccttcttagtcgttagttttccatacctacaataactatcagtggtgatgggcttctctgaccatgtgaataatttaatcctcaatgcacagatacagaaacccttgctgaagacagtgtggagcagagaaggctgtctccactccttccacctgaaacacctctgcagatggatatgggagctctgcctacagcccttggacctaaccacttcagtgtgttccagtgagtgtctggacctcggcctgaaagatttttccgaaactaaagaaaatttctctgacctaaagaccttaacctccaccccagaagctctcaccaaggactacagggaactggtggggaaaatccttatcccttactcctcaaggcacagggcagtaatgctgaggcttgtgcgccacacttgctcccagaggtccccagcgggctacctgcggtggtgaatgacctcctaacacgccccttgacggccttcctttccttgcctcacttctccactctcctaccagcattgcagggttcacatcccaaatataccactggcacttgaatcctggtctccaggtctgtttctggaaaaacccaagtaagacattgccccagtaatggggctagatgtctgaggcttcctcaagtatctacctcgaaagctcttactgctgtacacacatgcacatacacacacgtgcgtacaaccagtcacatctaagcaccccgaataccagcctgttgaaggtagcagagagctgcactataagccaaggctgctcccaagagccgctccatcactgaattggcgccccagcaagatgaaggaatgtaatcattggaaggatggagaatgttctctgaatcactgacaaattggaaggggtggagggcaagagtccacctggtggagagatggaaagagcgagagagcctggaatgataatgccattgcttagaaaaggctgctccagatgccatatctacagaaattgtacagcccaaacatctctgagcaataggtctctggtagtcttgatgtctagaccaacaattcccagttcattcttctcagggaaggagccaggatagtccagagactctcattctgctgttagattgaaagggttaggcacaacagccttggcaaagtcacaagggcaaattcacactaaagtgtaaatgacccacaactcctcttctatttttaggttggggaggtgctttagaacataaggaggaactaaagaatattcctgttacatacaaggcagagaaaagggaaactagtggtgacaagacaaatcatccctttgacatttggctggctctacctattacagctctgggggtgaggtgggaacaaaaagatgctgtgtaaagaagtatcttatgccatccctactgtagtgaggtgcagtttagaggggacactgatcaagcagagacccagagtgtttcgttccaagccagaaacagaaatgtataaaacacagcctttccagcatcagaaatgagtagtggtagtggagaactacccaaaacaggaaagaggaccacgtgaggtagagtgtcaaggccctacattccagtgcctctgctcatgactgtaattttgggtaggtcacttaaagtctctggacctcagttttgccatctgtgaaatagggataatactatccagcataaaattggttatgaggctcatgtagggcctgcctgggatgatgtgttgctaatggttaagaacacaacttctggggtctgactggacaggctgaaatccctgcttaacacgttccagcagagccctgggcgatctatttaacttttgttttctcacctgtaagctgagacgaaagtacccactttataagattattccaataattagttgaaataatgcatgcagagaattaagcatggtacttgttatttgttaaactagctattaaaatgtgtaaaatataaagtattgtatggattttaggacaatgcaaagactctttgcttgctgcaatagttcggggccctttcagatggctaaaggcagaatttgtatgtgtaaatatggtgtgcttgtctctgctctggatactgagggcttaccctgttattaaacttatttagtaaatattgaactgtcatgaggcctaacatttagttccagttattagataaaacatttgctttgaatggtatttgaattgccaggttctagattattctggttgacaaactcttcgtattttataaagaggctaaaattggtaagctatcacagaacagatgtgccattttcaaggtatattaaaccatgattcactgtaacattgttcctactggcaacaaattcagagcaggctggactttatttggtgaagaaacattgagtggaagagaaatgacattattttatgtatttacattttcaaattactgtggcttaaacctgttcagccaacattacccaccttcagtctgctaaataaatgattcagtacatttctaatttacagaattttttaacaaaagaaaatgtaatttgatagccaaatcaacgttaaacattatacatttaaaaaaccacaggcaaagacacaaacatgatgacactaacttttgttaaagtatgcttacctatggtttcctctgaggcacgttctttcatgctaagcttccaacataatatgaaaatgaaggagatgcattttgcaaagcaaaacagaccttaagcaaaatattatacttctcaaattaacactgttacaaagttttagaatttaataagttcattaatttaaaagtttggatgtctgagtccttctatcccaaaacaagatcttggagggtcttccacagccatgtaataccatggtcacatgaccctttccaaaattattaatctgaatttactatatgaggataaatctatctttttgaaaatatttaggaaaatgagcttggtatttataaaatgaagctctctttgggtggtatcctaagacacgtcaagccaatcagcctgtaactgtgaaaaaaacattggtaggtacaaaagtggggtgggagaggagtgacttaactttgttaagtgatgggaaagaaacactaatagcattatctcaataaaatgtgatttaaaaaaatttaaaatactaaatcattgaactgacaaagaaatataaatcattcagaaataaactcattaggtcatcaaatcctgttaaatctgcaattaggaagagcaaggtgtacaatccatacatttaaactcacaggctcactttgcacaacgtcaatttactccttaatatgttattaatacgcattttccaaaaggatgtattagtaaatggtacacatctacttcttggcaacatcatataacctggtacaacataagcattcttcttatagttaagaaatgtggatggtatcaaaattagaaaaataaatgccctattatgttgtggtcaggtttaaggcatgtgaattttatcttcatacaaaagattaaaatctagatattaaaaagtagtgcagtatcagtgatgctgcctcagttcccaaaatgtcacatcacaaaaatatcccataattgcctgtagtttattccttggctttcctcttttctctctgcatctttgtaacaattttttaaaagtggaaatataattgttggcaatgctaacagctgtagaaatgattacaagatgtggaaaagcataacaggaatgtcaagaatctgtttctggcagtaatatatatggaacattgttcaggacaaaagaggagaaggaagaaaaaaaggagaggggtttatcatctctaagaattttcaaactaaacctcattgcttaataggaaaaaaagattccatatttaaagttaagtcacctctaactactagctaaagcatgacatcaccagcactggagtcagcggaagtgtgtttttgaaggacagtgttgcaggagaatctggacaggttttagagccaggagagagaaaataattctacctctgacagttgaaggaccttaggcaaatcagtttacctctgctagactacactccaaaatttggacattcaaaaatttgatattaataaccacatgaaagtctcgtgttgaggtgaatatgtatttgttggtgaaagatatgttggtttttaaacagacagcactctgcaattgtaggctattgttttgttttgccagttgtcaaattctatccagctatacacacttgtgtggcctcctaatggtgtttttccagtggctaaaggtttatgaataagacacttttcctaatggaattaacccgatgcttttcttaaacatgtaaccttgagttcaccgcaaaaaacaatgcttcgattagagcaatgcatataataaaggttaccctcgtttcttagacactagacatcattcacaaaaagagaactgcttttgaaagggatgtatttgcactggaaagaatagttttctacttctaattataaatgatttattggtgaaagcaaaacaacagcctgtctgagaggcacttctatgagcatcctcacgtgtgatttgcaaggttgaagaagagggaaaaatgcctcaattgtaccaatggtgagaaaacacccaaagtacaaagcaggtttcaaaaaaaccatactcataaccaaggacaataataaagcaatgtgttgacatatactctataagtcttcctccataaatagtttatagaaattttgtaatttctgtaaatgcatcctataataattttgcatcttgctttttttttacatttaatatcaagtagatttctaaagggcaattatttgaaaattatcccaaatacatggggaaatatacatcaagtgaaaaaatgcagtgggtgatagagatatcaggaagcgcctcaaatatttctcatctcgttggagaaaaacaaacatgttctcatttagaatgagtgggagttacctaattgatttaggcctctatatttaacttctagtcaaaaaaggtagttctatctagcaacaatattatggggaacaaaagaaaaaattaactctctaaatttgcagtagggtcttttcttcagaagtaccaaatcccatctattaccagctccatgcttcaggcctaaaatggatctccctgaagcaatgacagaatttttgccaagtgactaggatataaacaccactttggttgcacagtgagacatatgctccaaagaaaactggttcaaaaacaggcaagtgggtttctacagaataaatgagagccctgtcaatggcttcatcttcagggctttgtgtctgtgcttgcgtggtggctcttgtttcatctatggataatggtggcacacagttttcataattccttacattaatgaactgctataaatttgtttttggtattctagagagtcctaacttcagcttctgggcaatgctgaggaggcaccctatattctagacttaccttttgcaaggtgtactctcagcattgtgggcgatttccatgggagaatattctatttaaagaactactgtcccagcataaaacaaaaaatcatttatgaagatgcaggagactcggaaagctctcaattattgtttgcacaagcacaatgtcacagcctcctttccccattccacaagggggtcaggaagagagtactcagctgtgagaaaagacatacagaagaattcatgtggtcatgagagcgaggacatggccgatcccccaaggaggatgtgtcatacacttcatgagcccaagagtgtgctgtagggtctgaagggcaagatgctggttcactgatgtaaaggagagggaaaaaagcttcaaccaactagaaaaacagtctctatgcatgctatttttgattttaaacacaggtatcaattccttctctcagagagtccattttaaaataggatacatttttaaaggaatatttaaaggacacattcattaaaatttattttaaaaacttttcaaaagaaacaaaaggtatgaattttatttaatccttgaggaaatggttcttttctcacacacataaatcactcattttgtttttctttatctcctttattaatctacattagaaaaataaacttttcatacactaagaacaaggaaaccactctcaattgacaaaatgttccaatccaacacaatgattactttcacctttaatttacaggcagccagattcaaaatccttaaagttgcttaaacttaaaaatgacaatgacaacctaaaaggtataatgttgattggaacagacatttaattggaaaattgatgattttccatttccaattaaatctctagatagaaatgaaaaaaattaaaaatcgtatttaagaaaagccaaatcttgggttgtgaggtatctttttaaggatgtttcagcagaaaaaaacaaaggctctcacaattgtgtagctgcctagattaagtgggtatcctgatcaaggagatgggggatgatttggctttagtattccaatgataaagtttataatgagaataacatgttgctacaaaatccagtctcttcctcagatgccttccacagagggcaggaagctttgtcagttttgtttgctgatgatgcctggttccgtcaacaaataacacctgtcacacggtgggtagtcaatatacatttgttgaataaatatgaaaaaaagaaatgtacaatatgtttgtgaagccaactgtgtgtgcattgctattgaggtacacaaaaagtctttgttttaaatttgagaatgaggactttcaatggaatatatctgataggcctggatcaagcatgcagctgtggagaacacccctgggactctaactctggcactctgcaagctgggtacttgggcaggacagcagcagcactcatgaactgggcagcacctgttggtgagggctgatcacatggattctctcatcccagccttacaatcagtccttcaggtacatactttttctgactttgctgatgaggaaactctcttcaagtggtatttaaatttcttctttcattttccttctggtaacaaagaagtctgtggctcaaaagatgtttctctaagaccccatcctattaggtctctgagctgtgggaagtatttatacaattgcttgtgaatataagatccaggaatttccctaagatccctaacaaaattggtgataagtagtcccacatgttaatccagccacccacggatgacagcacttaccatttctttgataaatgtcaaatgcatttgaagtacctacctgaaatatttgtttaaatgctatctaatctattaattttatatatgtgtgagtctgttttgtataccttctgattataggataaatgtaaataaatccaaagagtaatcaaagctaccactttcaagaagccttctttgtagaaccggaagagtcttaaataggcttttcaggtatgcatctcttattatcgctgaactccaagtcctgcaaggcaggcatcatgtgtgggtcacctttacagtaggcacaggccttaaaacagtgacatgcacattgcaggcactccataaatgtttgctgaattggctaaaccttggtttgttcccataatcaaccaccacaaacagcacacagataattacttcttggaaagattccaactagtgtttgatgttacctacgtggtttttctctcaagatcttaagagcagctctgtaggattacattattttctgttttttttttcctttgaccttaatgtcatctacttcaataacagcttcatacaaaattcctaccagcacataccacagcagattcaaggccttgttttaaaaatggtgccagcttctcttaatttggaagatatattgtctctcctgaacatgggctaagaaaatgtataatttggtattaacataagagctgaagacactttaaatgcattgtttcatttttataagataaaaaaaattttaagaatcaaaatgttatcaacagacttgtccttcattaaaaagtaaaactgcatttgcctacattttatgaaagtgtccaattatgaacaattttgaaatgtaacttttaaaaatgtaaacagcaaaaatgttgtatttaaaataaatctggaaaggcagaaaaacaaaaaatacccagaagacagagtttttggtgaaagttaagatatttcatctttgaacaacttagaatctttcctgcattttatagtctagttccaggcattaatttgaaataaccttggaatcctaaatctaacacccttcggaacaaagtagcttttctcttctgctttatgagcaaatggactaaatactagggaatggtactgtctgggcctttgaaccaagattgaaagagatgaaatcctatatgatatgtataaacattagagaatccattttgatttaataaaaggttgaatttgttctatatcctgtgagaaaatggttcccttttcctgaaaatgttacctcattccaacaatagaaagttggtttttttccagggtgtggtgttggcgggggacagagttgccatgaatatggcatctatgaagactgctgttatattcatttctcaaaatgcactgtggtaggaaattcagaacgcagtgagagaaaataaatgtttgacttcaaaatataaggccgcatttaaagcagaaggtaaagtatagaacagttgacagtataaattctttatctgcaatcttgcagttccctaaatctctgtaacacatcacttttaaaagcctcagataagtggttctataataatttaccaataattcaacccctcaaaagtcttagcaagttaaaccttataatcttacattttagaaatgacccaacttgatccttttattcttcagaatatctctctcaaattttcatttgtttttcattaattgatgaataatgagacattttaggtacctgtccacaaagaaatgaaattttcactttccaggaacctaacaaatgaaaagatagaaatcaattccaacagaatattaccaaagaaatcttttagaatggactgttaaaattatttatttgtatttatctggctctactatttgtggtacatttccacttcaaagctaaacctcaaataacatcatagtgagtggttgacttcatgtttaactgagatcttgaagactgaaaaagaccacgacaaacacacatctattttcttggctactgcatccgtgttcatcaccattctgatagtctgcaatgtattgcagctcaccctttgggaaggactaaagtagacatctgtttgttctgcttactcagcattcctaccctaattttcctttggagaacccctttattctagaccacgtgaagctaatgccaaaccccattccaggggatgcacctgaatccaacctccatcatctaaacagtgccttctccacgttcagagaagagcaagtgactcaaactgccctcataagaacagacctgggacttctgctgcaaatattgaagagtaagtactcttttttcttgctaggactaagctggtagtaccttctatgaggctatcatatggaaacaacttgtctgaaaatgaagccacaactagaaaacagatcctggtaacccggattgatggatccagccctaccttaaatggcaagacctaacccgaggctttttgcatcaaccaataaagtccttaagccagtttgagttggttttgtcacttgcagctaaaagaattctgactctaacaatgtgacaatagcaaaaataaacataactgcttttgaggtttctaatggattttcctccctatatacatgatttcatttaatcctcacaattcaggaaagcacatatctattaacattaaattaatattcattattttgaacacatgctatgtggataagggatgaggaaagccaaggaagtaatcaacgtgaaatctcacttatatgggagggaagtggaggttacatatctcagggcacttaacagatatcatcaaatgaaagaataaacagtgtgtgggagaggcagtaggtgattcttcatcaattcctggatgaaaaattaggagataatgaactccgaacaggcagcctaatgagaatggctcaagcaacaggacatagagagggagttaggttagacatggggttcttgggaattttcacctcgtgggggggcgggggggtcgtgcagctgttgtcagtgggaaagggaaaaaggaaaaggctgagtttggaaggcagggagggaggagacaatgtgagtcagtgaaaaagggcccttagaatgacaagtctggaccagagagaggctaagactgaaaatacaagttgggtaaccactggcatacagatggcagttcaggcttgggcactgcccaccagagcctcagcatgaagagaagagggggaggctggccaccacctccctctaggtaatcgtcatcctgatgctgagctcctgaaaacaggctctttcactcgccccatctcttgctcttgattgcaacccggcattcaggaggcaccctgtaatatctgtggagtgaccgacaacacagcgccagggcactgagaagatcccagggcgccagggactggttctacaagggtgcccctcccggtcccctccagcgcgccgccagagctgccagtcttggctgctacacgggaggcagcctcattatgcagctctcacctcttaaattagttcatgctctcacattaggtgtaatcacagcttgcaacgctttctggggatgtctcagaaagatctgagttgaaaaaatatttttgtgtcattttaatttaaagtaaaattgctgcttcttccccgcccctttctttcctcctggcccacccagcgaccctggccggccgtgctcaacgggggcgggggtcggaggtgagatttcctccacataattccttaaacagctatcaactaagtctcaaagaaaaaaaaaagagatctagaagcagagacgtggctgctggcgatcccaaagctggtgttcgctcttgggggagagcgtaccctgggggaggccgggaggccgggccagaggctagcccagaggcagagggcaggagcgctcagccggcgccccgcgtctctccagctcccgacgctgcgctggctccgctgagcacgccaggatcaaggtcgcctggtggggaccggagcgccaggagcctgtgggaagcgttccagccggcctctgactgggatccggcgccgcgtttctgctttggacttgactgacaggtccccccgccctcccgccgccctactaccagcctgggttcatccttcagggctacgtctaccgcacccgggctggaaagcctggagcgcgcccttcctctcctcatcttctcagctctcctttctccctgccacttggcaaagctgcattttgactttcacgttttggactacgtgtgtgtagttccaagtccatgcgtggcacgaaaatccacttagggtaaaaattattctcgaaaaatcgcccatctcaggatctggtgtctacactcaaggctaggaggtgcaggtacgggtgcgtaaagcatgccgtaagggtgcacagtaaataaaaagtacggatgcaaaatgtaaattttaagtgcaaaacagaaaagcagtactcgttgccgccccgcacgctgggttttaaggggcacgaaggtgggcctcggctgcttttgctcagccccgcgtcctcagcgcccggcccagtacccggtactccgtaggggttcaatgatctcccctgaataagtgaacgaattaacaaatgaatgaatgaccgctcgatccgacctccgcggccggcagagcagtcgctggagaggcgggagagagcgagaggccaagctccaccatcgcggccgccggctggggcagagggacacggagacactcggcgccccggctccgcaccgagtcc

SEQ ID NO: 12769 - RNA, 2600 nt, Homo sapiens
  source 1..2600: mol_type = other RNA
gatctcactttgttgcccaggctggtcttgaactcctggactccagtgatcctcctgtcacggcctccccaaattttggaattacaggtgtgaggcactgtgcctggcccaatttaatatttgaatgtgacacactctttcgtattaacacgtctactaaaaaacacagaaatactacagccagtttggccaaactcataaggtgtatccctaattctctgacactgggtgattcctcctaaacccatagagacagcatatttctagttctgggctcactccattggtgctagctagaatgtgtctcttgttttcaatccagctcttcctccctttctggaacagactgacttcccctcttcacaggccctgagaaatgtgtacttcttatccccagctctaatttaaagaataggttcaattctagcttttccatgtcagtgacaagacctttggctaattaacttaatctcttcataacttagcttcctcatcttcagaatagaacttggccggtgtcacggctcatgcctgtaatcccagcatttggggaggccgagatggcaggattgcttgaggccaggagttcaagactagcctgggcaacatcgtgagatcctgtcgctacaaaaaatacaaagttacccttgtggtggcatgcatctgcagtgctagcttctctggaggctgaggtgggagaattgcttgagcccagaagttgacgctgcacttagccatgattggactactgcactccagcctgggcaacagagcaagaccgtgtataaaaccaaccaactaacgaacaaacaaaatggagttagtaatcctatcttccctgtgaagtaaaataactcacatgtgttaagcacctaaagcctgtcattagtcattggggaaatgcaaatcaaaaccccaataagaaaccactgggatgtctacagtaaaaaagtcagggctgggtgtggtgactcacgcctgtgatcccagcactttgggaggctgaggtgggcataatgcctgaggtcaggagttcgagaccagcctggccaacatggtgaaaccccgtctctactacaaatacaaaaattagccaggcatggtggtgtgtgcctgtaatcccagctagtcgggaggctgaggcaggagaatcgcttgaacccaggaggtggaggttgcagtgagccgagattgtgccaacgcactccaacctgggtgacagaacgagactcagtcaaaacaaaaacaaaaacaaaaacaaaagaacaaggagggagaaagagagtgacagagacagagaggtatagaaacagaaagagacagagagaagggaaagagggaagtaggcagagaagaaggaagggggagggagggagggaggaaggatggaaggaaggcaaggaggaggggggagggagggtggactgtaggtcagagaaggagggaggaaaggagggagggaggaaggaaagaaggaaggaagggagggagggaggaaaggagggagggaggaaaggaaaagaaataaaggaggaagactaaagtgttcccattcgctacatctcttgagagaaagtcagccatttcagcagttctgtggaaagagtttggtgaagcaagtcttcttcatggcgaccttcagctccttgttcctgaggctgaagatgatggggctgaggaagggtgtgaggaccgtgtaggtgatgcccatcaaggtgtctccttccggagactggggacctttgggcttcaggtaaatgacggaggcaaagccatagtgcacgaccaccacagtgaggtgagaggcacaggtggagaaggccttgttccgaccttcagcagaagggatcttcaagatggcggccacgatgaaggcataggagaggaggatgaggagaaaacagcccagcagggccgtgatacacaccaagcccacgcctttggccaccaccagcacatcatctccacaggccaacttcaacagaggtggcacgtggcagaagaaatggtggatctccttgtgtccacagaaggcgaggtggaaaatggccgaggtcaccaccatccccatgaccaagccaccagcccaggagcagcccacccggcaggtgcagccccgcaggctcatgagcacgttgtaacgcagggggtggcagatggccacgtagcggtcgtagcccatgacagtgagcaggaaggagtgggtgaagccgaagctgaaggagaagaacatctgactggcacaggccaggaaggcgatggagcgctgggtggacagcaggtcggccagcatgcgcgggatgatggccacggtgtagaggatctcggtgatggagagggcacacaggaagaggtacatgggcatgtggaggctgcgctcgctccagacagtggccatgatgagcaggttgcccagcagcgtgaacaggtacatcagcaggaacagcaggaagagcatcagctggaggtgggggaaggcagagaagccaacgaggatgaattcagacacggaggtgtggtttagcccctgcatggcggccaccccttcatcagagacctttagggacgccttgcagccaggcctgtaatggccctgggca

SEQ ID NO: 12770 - RNA, 3210 nt, Homo sapiens
  source 1..3210: mol_type = other RNA
gatctcactttgttgcccaggctggtcttgaactcctgggctcaagcagtcctcctgcctctgcctccaaagtgctagaactaaaggcatgagccaccatgcccagccctcttgaatgttttatagttttcgttatacaagtcttatacttattttgttaaatttattcctaagtatttaattctctttggtgatattgtgaacacaattttctttatttcatttttggagttttctgaacagaaaaatacaattgattttctgtatattgatctagcctgtgaccttgctgaacttgattaattctattacactatgattttttgttgtggttagacccttacacaatcaaatgaggttaaaaaaaattgtcagagtggccccagaccaacaacaggatgacagtagcctttgcccatacagagataaaatttagtttttgcagtcctttcccatagagattgtatggcagtagccaattctatggcctactgccatacaacctgaactgaagtccagaaagtttaggtgactgggccacagagctaattactggtggagccaagaagagaaattatatccctacctccttgcccactaagctccccattccagtgggctgctttctggtccttttccatgattgggctttagtagctgtcatttcctccagtgtccaagagtattttcttggccttccagtaaagctccccaagttgtctgtgttccgcctcaactgctaacttgcctacctgataaacattttgaaaagcaatctaaattctagaaattgtctctcctgcaaacaaactacagattccatttaaagcatttccttgagtccagaaagttctgagattttcctgttttggactagacttccaaagggcttcatcttaaattgtatgtatttattgacctaattgtttactgatctttagaatttagagtttaggttgggaggtcaaaatcataactttctcaatttttttggcaaactgatatgatggctggaaatcatccagaaaaagtagagatcattatattttcttgaatattcattcaagtttcaatttaatacttaaacattcattttcgaataaaaatactatgtcttgtactagggatacaaagacttggttattcttgttggagtaatgattctcctctatctggggaggtcatcctctgcagttggggactgaaggactgggagatgggagattgaaacttaaagaggtaaaggtatgtcttggaataaaactagttatcagtcaccaccagaccatcatggcggctagaattccagaaacggtgaatagaagttcatcttctattttgtcttcatggaatatatcactctggtaaacagctggttctaaatatgatggttagactttcaaggtcttcattttttagatgtaattcttcaaggagggtgtctagaaaccgtgtaaacaccataccttcctgagaatgtttctgaatgccaagaattggggtcagtaatgacagcaacaccatagcaattaaagtccattccgcaggtttgtgtataatatttctatttgttaacctgaaagttcgaacaagatttttaagttgtgtgtaaatatctcccaatgtaatctgaagaggaaccagaagcccaggcaacactttactcaacttttcaagtacgatgcgttttctaatctggttctgggaacttgagtctatcagtggaaaggtggaatcatgctcttctgagtcttgtgatttggtggtttcttcacccaaaacataccgtcctctgtaaaactccctgatcctcagatttaacttttcagtttcttttttcaaattctcgtaacttggcagtggtttaatggctgtacctgagcccctaaaaggtaaagactcatccaagctgttctgagattccctccaggcagggaaatgactatctggatctgagattatgtcatcttcatcaagttcttctttaaccagagaggcttcgggtttcagacacacagaagcataattctggccatacaaaaacctcaatgtttcttctgtcttccactcaatcaaagtctccttcaaaactttaagtaagtttctctttccaacttcaggacacacctgcactgaactagacactgacctagacacttggtttgatttggcaaattttctcttaaaatgctctgcacttttcttacttatgcctactagagttatttctgacctactgtattcactttcagaattttctgacgcttttaatctttcaggcaaagtgctatttgaagaactctgagtatttactttctgtaaaggaagttcacatgtagcatctttctcctgactatctaatttgcaatcgcctaactgctcagtgacatctactactgtctgttctttgtctttgtgtttggagttagctttgtgaccagctttctttttcattatgcttttttggtgcagctgtggtctaatatttgttgaatttggtctgtttcctggtagaatggaggaaacaaagtcttgctcattgtcactgctactatcactgtgagtgctagaagaactagattcatattgcttttcaaagtggctaggattgtcgatatctgatgttttaatggctttactgcataactgtacttcttctccagaatggccactttgttcttcctttagcagttgaaaatcaggatgcctctcttcttctcgaacccatactggagttttgggaatttgtgcttcaaaaaacttagatgcttgataacaaaaattgctgcaaaaagactttctttcagtaatatcatagactttattggttttggtagaaattttatatttctgttttggtacaattcccagcttcttctgacataaaggataaccacagagtttgacaatagaacgttcatccacgacatcactgtagtgagcaggtgtaatgaacctcccacactccattaggaactcttctgtaatattctcctctaaaagctgttcaacaatatgtagagcttttctctcaaattcaatcttctttctcacagctgcttctagttcagctttccttttagaagcatcttcttgtttcaaagtacttgtctgtttagtacctgcggcttttcgagagcagcggggagccccggccttgcggccggcagaagacggcccagcgaagtccgccatgggggagagtagtct

SEQ ID NO: 12771 - RNA, 1560 nt, Homo sapiens
  source 1..1560: mol_type = other RNA
gatctcactttgttgcccaggctggttttgaactcctggcctcaagtgatcctcccgccttggtctctcaacgtactgggattacaggtgggagtccccgcgcccggcaaagcctatattaaacccttttatgcacactcggcggtactgcagagagggcagggaggaagcagaggtgccctggcatcttcagctggaggtgagcagggcgctgagggtgggagaggcccggcgcctggggatgggaggcaggactgcaccttcacagggacgcttccaccctaccccggaggtcagggcctctcgcccagctctggctctgaggtcctggagggagggagatgctgttgcgactcagaagattgggggagggccacccccattcgagaagagtgaaaatcctgagcctgaagaagtggaaccggttggagccgaggctttagaggatggcgttcgaaagagggtctggcgccgccctgtggactgttcgggctcgcagggccgaaggctccgaagactgagaccttttgtgttctggaaaaaatgctgccacagaggtctgattttgaagtggctgccaacatcccagacaccgaaggtgttatttttatattctactgtctccacacagaaacctactgtagggacggcaggcacagtctcccccagcttcaatttatacaagatggtggtttttccagctgtatccaaactcaatataagaatccgcatcttttttttcccaagtagacttttaaagagcttttcaaaaatgtttcccattgtaatttaatcgaattctgttgccactcaaggtaccgctacctacaacaccgccgactccgcggcctttaggatttcagctcagttcagctaaaccacgacaggcgtgggggcaggaacagcaaccaaccaatcacccaccgcctcctggagcttttgcaccaatgagctcgaagttttgtgagtgacgacatatctggccaatgcaaagaagagtaagggcctgggagggagggagcgccgtaggcgacgccatgaagctctggcaataccatgttcatcttcaaatcacagttaaacgaattctggcgagacacgcccacgtcccccacccccgatgccatgtgcgaccaatcagaaaagcaaaaggattgtctatttgcacggccaatcagctgggaaaatcgccgaggtttgagctaacctcggagcgttcacaccaaccgggaggggacatgtgggccgggccaagttaatagtgccatggaaggaaatttaccgcggttgagttaaacgtagacattagtttggggcggtgttccgcgtaggaaataccacacactgacactgaaattaggcataaggaagttttcctattccgcctgaggctagactgccctcccacctctacacagattttcaagttggggaaaatactggccacccgcacctcgttaagacgtcgcagaaccagtcctcgtttccgagaaatgctttctatagtcagttccctaaatgcccaacttgttagctaaaaaggttacaaacgcctgtaaa

SEQ ID NO: 12772 - RNA, 1272 nt, Homo sapiens
  source 1..1272: mol_type = other RNA
gatctcactttgttgcccaggcttgagctagctagcttgcttgcttgcttgctttctctctcttcctctctctctctctttcttttttttttcagagtcttgctctgttgcctaggctggagtgcactggtgagatctcggctcattgcaacctccacctctcgggttcaagtgactctcctgcctcagccttctgaatagctgggattattggcacatgccaccacacccagctactttttgtatttttagtagagacaggctttcaccatgttggccaggctggtctcgaactcctggcctcaagtgatctgcctgcctccccctcccaaagtgctgggattacaggtgtgagccactgtgcccggccaagcatgtttctaagaaaagggcaaacaattctcaaagaggcccctaatatctaaaattggtttagaatccctgccctaggtgaatacaggaaacactatcaaaactaaaagggaacttgtagggcatcttaatcaatcaaccaagataggtaccaaggcccaaaaccatgtagaggcttgtgcaagatcacaagcagaggtgcaatttgaagctagattctcccactcttaaactagtgccggacagacgaaggcctagcacatgggctacggagccctagtagattccagtccccacactgagccaggaggggtcgctgcccagggatacctacagccatactcgagctggacaaggcgcacgctctttgtggaagcaaacacgtccaccaccgcgtagaggggctgcgcagctggcagtccccgggcgctcgggcccatgtcctcgccgttgatgatgatgtgcatgtcggccgtgccatcggggcgcgggcaaaagaggacacccaggcggctacggcgcgcggtcggaggcagcacgttcagctcatagagctggtccaagagatggctgtagagccctggccggctgcggcccaccaggcggtcccggggaatgcgaaactgctcaatgcgcagatatggttccacgaggagggttggaggtcggctgggggccgctgcctccgcctccgggcggccctcccggggcacgcggttgtggtggcgcgtgatggcgaagacccaggtgtggcccaggttgaccagatcgggcagagaaaactcgggaacgggggccagactggcggggtccagcgcggtcagaccgagacgcagatgtccgcaccagcccagctctttctcctcgatctcgaccaggaagacctggcccggggccagc

SEQ ID NO: 12773 - RNA, 896 nt, Homo sapiens
  source 1..896: mol_type = other RNA
gatctcactttgttgcccaggggctggctctggttgtcaattttcatttccaccagagaagtgttgtatgggagggcttctaccaggcgcagaatcccagctccagaaatgaagttggattccacattcagtgtcttcaacaccttgttctccttgagcatctcagcaagggcatacgccacggggtcattactccgtgtccccacgatgctgaacttcttcacatatgagttttctttcagggcttctgcatatgccttgagggtggggatggggatattccggatattattgaggttaacttcttcaagttttgggtcgttgttctttatccgttccagcgtttcctctacgtctgttgaatttggttcttcgtcgggcacaggcttgtattgtgtgggtttaatcacgctgttgagcccctccttgttcatgatggagctgctgctcagggcctggtagtactgctggttactcatgagcgtgtgcatgcccaggatcgctgcaatgtcacagagttctgcatctgaagcatttgccaaggcttcctccagctccggttccagcgtcacactttccagcacaggatccagtggcttctgcttaggaacccagacctttcatcagggtccagctcatccagctcattttccagggtcctcagctcttcctctgttagggctccaaggatttcatcttcatccaggtcacggtatttctctagttctcgtctgtacgacatcgtggaagaacttgtctgtgtctcctgaatttctgtgctgagtaatacccggacgcagagctgtggggccggcgcggacgcgggctgcggaacaggcgcgggcggcgggcagatggacgcgggcggaggccgcggtgctccggcgggcagcggg

SEQ ID NO: 12774 - RNA, 1085 nt, Homo sapiens
  source 1..1085: mol_type = other RNA
gatctcactttgttgcccaggggctggctctggttgtcaattttcatttccaccagagaagtgttgtatgggagggcttctaccaggcgcagaatcccagctccagaaatgaagttggattccacattcagtgtcttcaacaccttgttctccttgagcatctcagcaagggcatacgccacggggtcattactccgtgtccccacgatgctgaacttcttcacatatgagttttctttcagggcttctgcatatgccttgagggtggggatggggatattccggatattattgaggttaacttcttcaagttttgggtcgttgttctttatccgttccagcgtttcctctacgtctgttgaatttggttcttcgtcgggcacaggcttgtattgtgtgggtttaatcacgctgttgagcccctccttgttcatgatggagctgctgctcagggcctggtagtactgctggttactcatgagcgtgtgcatgcccaggatcgctgcaatgtcacagagttctgcatctgaagcatttgccaaggcttcctccagctccggttccagcgtcacactttccagcacaggatccagtggcttctgcttaggaacccagacctttcctcgtttttcccctgtgtaggggaccagatcttctcggtccttaaactcctttgcttgcttttccaagtgatccaagagctcctctcttttaaaggggcccgtgggcgccttggtggtctgatccttctgcctcaggcctgcaggcagcagtgcattatcagggtccagctcatccagctcattttccagggtcctcagctcttcctctgttagggctccaaggatttcatcttcatccaggtcacggtatttctctagttctcgtctgtacgacatcgtggaagaacttgtctgtgtctcctgaatttctgtgctgagtaatacccggacgcagagctgtggggccggcgcggacgcgggctgcggaacaggcgcgggcggcgggcagatggacgcgggcggaggccgcggtgctccggcgggcagcgggcgggcgagcgcagcgcggggctggacgagctc

SEQ ID NO: 12775 - RNA, 1035 nt, Homo sapiens
  source 1..1035: mol_type = other RNA
gatctcactttgttgcccaggggctggctctggttgtcaattttcatttccaccagagaagtgttgtatgggagggcttctaccaggcgcagaatcccagctccagaaatgaagttggattccacattcagtgtcttcaacaccttgttctccttgagcatctcagcaagggcatacgccacggggtcattactccgtgtccccacgatgctgaacttcttcacatatgagttttctttcagggcttctgcatatgccttgagggtggggatggggatattccggatattattgaggttaacttcttcaagttttgggtcgttgttctttatccgttccagcgtttcctctacgtctgttgaatttggttcttcgtcgggcacaggcttgtattgtgtgggtttaatcacgctgttgagcccctccttgttcatgatggagctgctgctcagggcctggtagtactgctggttactcatgagcgtgtgcatgcccaggatcgctgcaatgtcacagagttctgcatctgaagcatttgccaaggcttcctccagctccggttccagcgtcacactttccagcacaggatccagtggcttctgcttaggaacccagacctttcctcgtttttcccctgtgtaggggaccagatcttctcggtccttaaactcctttgcttgcttttccaagtgatccaagagctcctctcttttaaaggggcccgtgggcgccttggtggtctgatccttctgcctcaggcctgcaggcagcagtgcattatcagggtccagctcatccagctcattttccagggtcctcagctcttcctctgttagggctccaaggatttcatcttcatccaggtcacggtatttctctagttctcgtctgtacgacatcgtggaagaacttgtctgtgtctcctgaatttctgtgctgagtaatacctctgattgaagcgccgctccgtccgtttcccagcagcgcggccaggtgggctctgagccgcaagctttaaccgcgatcgttttgtct

SEQ ID NO: 12776 - RNA, 4019 nt, Homo sapiens
  source 1..4019: mol_type = other RNA
gatctcactttgttgcccaggttggtctccaattcctgggctcaagcgatcctcctgccttggcctcccagagtgctggcgtgaaccattgcaccagacctgtaattacactttaaagagcattccagtcacctggggaacagttagctctgtatcttccccagtccacctcctgagggtctgacccaagaggaggttcttggtatggggggtagggagccctccagcccctaggcaatcctgattcagagggtgaggttgctttagagcagtggttctcacacttgcaaatgtgtcagaatgccctgtaagacttctccgaatacagattgctagactccagccttagagattctgaatcagtaggcttggcgtggccttggggaggctgtatttctaacatgctagagtgctaaaggtgcctgtcctgggaccacactttgagacacattaggccagagaacagctagaagatatcttcttccatgtgcatctgcttccttggaagggaatttctgttaacagacagggatcagacacccttccaggaccatgcatcatgatgacacccctgctgcggttcgtggcctctgcatgccacccctttgtctctggagggggagaaacagtaatataaacattgctaaaacgtgtcgtgtctcgtcagtgaaaactccatttgactaggcttattaaaaagacatcactattgcaaaatgatttaagtgcttcatttgtgaaggagcagaagaggagatgaggagcctctaagaatctggctataaatactcttcaagcatgcaaaatgtgccttgatgcaaactggggtttttttattttcataagaaggcagtgctggccttcttgttggaagcacctgtaaggttttgggaccacatgggatataaaatgaggtggggtgtttttccacccctctctggaataggttctggattttccccccaagaccttatttatggcaaaagacaggcccatgcactcctcatttctggcctcattagcctgagaggtttcgcttttggtaagaaattgtggagacaatccactgacggggactgcagatgtatgtaggtcagaaagtctatttgcaaagtgctgagggagtttgatcatgggtcatgagtgtggcttccagcttgtctctagcaggaggtaggaaagtgacttgttggggtcacatggtcactggtaactgagcccagaccacatcccaggtctcctgactcctcgctccatagtcctgccacagcatcatgcttctgtgaggaactggactggtagctccctaatccccgggggaaattagacagcctggtttcttatctgtcttaggctattaggatctgttgagccttcactgttgggacatgctagggagtatctcctggtggacagtggaagagacatggtggtcatattcatagatggtcctggtggaagaaactaaggcctctcagctaaagaacagctggtgtattctttctgactgtgtgcctcagtttgcccatacaaaaccgagtccataatctcttctctacctgccttgtaacacagatgaataatctgggcactgtacaaggtaaggaatgaatgcagtgacctgaccttgtatgtccagtttggaggggcagagggtcgagccagcttgagttccagatggctgactctgtaccttcattgctacaagattgtgggcaaattcttcaagtctcttagcctttgtttcatcatcagtaaaatggcaatggtaatcattacttcatcttgataagccattattatgaggaatgatgagatcacagttcatccttatagcaacctgtggaacagaaactactgctctccccattcaaagagggtaaagctgtgtcaggcgcacaacagttaccaaatggcgagaaggcgagaggactcttggttttacccagggatattatacatttgttcagtagtgccaggagtttctggaggtgtccttcttatacagtttcctggagacctcgtgattggatggcatggtgacatctttgccaccttgtcaccgtgcctcttactctccccagcctaatggagttgggtgagaaggatatccagtgggtcagcttctataaaatgtcagcattattccctccgtgtgtccagagaatttgtgcccttgagatgtccaggggaatggagatcaggggtccctgcagtggggaaaatggcttggctccatcttggccacctgctgtgtgtccttggcaaataacaccacctctctgggccagagagtgactgatggttcagatggtgcagaagtctcagtttaacaggtcatctgatctggaagaatggctctgacatatacccctgtctgtgaaacaagaggttgggactccatcattccccaagtttctcccagctgtgaccctcttggcccccaactatgggttctactcctgttctgagaggcctaactgagggtttcaactctctgatgagtaaggggccagcctctggagtttgtgcagccagaaaattccatctgtctggtctttccttttccctttggacagaatccctcattccaggcacttatgaatctccccaggataccccccaagcaaagttcctatttcttcatatttgcatgccctcctctcaaaacttagctttcttgtgatgccctctgctctgttaccatctctaggcagaagctaatttatgttttgatgccaattgcagatagcaggcattacctttccaggtagattagcattttatgtctcagtctaactgtggaagttcaggcagaatgactatggtgaagggaaaatttagaagtcagtaatacttccttgcatctctcgatgcttaatcgaaatgtagatgcagctgcctcctgagtttgctgggcccaggatagagtgatgcctccacattggtagagttctctgtttcccgctttggcttctaagttcagagtggcctgggatggtttcattttggttggattgtttgtggcatgattaccctatgggtcacaaagcttggttctgagggctgatgaaattccgggtaagccctgtgctagactcactgattcccacactcaagggtggctggacccaaggccctttcttaacagattgaaggttgtgtgcaaacctatctggcctcaggcaattggctggtcagtgtgggctgtttgctaggagctggtgtttgtagtagctattctttggcatcaagtggcctgttaagtcaaggactcctctgcaccatcagttactgtctggtccctactgtcttacctcacctgtcccaggaatggacaggtagatgggggactagctaagacattagggaagcccaagtccatttctaccactttggaatttggggctgaatcactcctcctctccgagtgatttcagtttcctcctcagtgaatggatcgaataacatgtttcttgctgaactgttgtaaggacgacatggatcccagcccaggacctgacacactgggactgctggatcatcaccctcatcacaatgcttccattcagaggcagcaaatagtgccccttgaatgatgtcaccaacagccaatcagaaagctcctgagctgttccaacaggagggctccattatgattgggtctctcagaagtctgagactttgaatgatagtctagtattaaggaacactggatagtcttataataagcgagactttcttgccaccaaaggccaaaccccatgcccacttctgccatatcaagatctctggaacaatgggacttcctgtttgggccaaggggaagtgactgaaagtcacaccttactgaggcttggcaaagccttctctatcggtttcctcacctgtgatactgccaggaggctgagacaactgaacagagtgacataacatccaggaggggcttctcacccagtggtcatcacagaagggcaggagggcccctaacaaggcattaattccctggatgactttca

SEQ ID NO: 12777 - RNA, 567 nt, Homo sapiens
  source 1..567: mol_type = other RNA
gatctcactttgttgcccaggttgttcgccagctcttggcttcaagtaatcttcctgccgcagcctctcaaagtgttgggattacagatgtgaggcactgtgcccagccaagcttggtattctcacatggagagttgaacccaggctgcctgggtcagatgtattcttaagtctttcattcatacattactcgggggtcctcagccatctctgccttcaggtggcaccaacaggatcaaatgttaattttttctcatggctcaatgaccactttttcccaggctacttggctttcttgtggcttcccacgtttcttatctgcatctgataagaacagatagagtttctcatcaattttgtgagcatagctggacaggtcagagaatatcagagctggaaaagacacatcttttcacaactcctctctttagagattaaaaaaccaaaaagtatgtaaaacagtagtttacaacaactggtaatttagccctcaggaaacaagtggcgatgtctggagacattttttattttcacagttgagggtgctactggcatcgcactggaaga

SEQ ID NO: 12778 - RNA, 1168 nt, Homo sapiens
  source 1..1168: mol_type = other RNA
gatgatgctgctgatgctgcctcggcgggagccatggacactgttgggtgactggctggggctggtgtgggtgctcagggactccttgctggcactggtgagcttgtttgccaagggaaggctgatgagctccatacacttcttgcacataatagacccgcagaggcggcagtggtggcggcggttccggatgctgaacttattcccacagtctggacagaaagggacatcctggtcgttgacccaaggcaccacagacttttctattgctcgaatctttgcagactcagtatttgttctgtcaaatgcagtgagctgattattagtttattgacttccacaacatagtggtcaattctagcagctcggtgttttttgaagtcggaaagatggcttctcacagcaccaagctcctggggttcccacatgtaaggatcaacccctccatagctgaaagactcatatccttgggtccctgactctgctcgatcatccccttctcgtttcaacaacctgtcctttgcttttttagccttctggacaagacttttaatttgccctttgacatcacggtcttcccctgagtgttcttcctcgtaatgtgagtgaagctgatagaaagactgcagatccttcaggcacagagggcagaggaagccctccctcacttcccctgggtcgtccagagaagccatggcagtgccgctctcaaccctaggaaggcaggaatctcatgccaagagtcagcttgattcctcccaaggaaccatggttcccgcagcattagcttaagcagcacacagatggtgaggaagtggcttcatggccctggatgaggtttcctctctggagtaggaggagcccttggcaattctcttacattcattccaaatgatccaacttcataattcatatgccacttcagccactgggggaatgtctgaagtacttatcaacaagcagaagtttttacttgatgctctttaccttgattgtttattcaaccacatatagtaagttcttgatacttgtaagacaccctgccgggctcctgcgggcacccaggtttgtcccccccttcaggcccgggctctgggcctccaccgtccgtcactcagccgcagccgccatctccatcggtcgctcggaactcggcaggtgcgcctgc

SEQ ID NO: 12779 - RNA, 1311 nt, Homo sapiens
  source 1..1311: mol_type = other RNA
gatgatgctgctgatgctgcctcggcgggagccatggacactgttgggtgactggctggggctggtgtgggtgctcagggactccttgctggcactggtgagcttgtttgccaagggaaggctgatgagctccatacacttcttgcacataatagacccgcagaggcggcagtggtggcggcggttccggatgctgaacttattcccacagtctggacagaaagggacatcctggtcgttgacccaaggcaccacagacttttctattgctcgaatctttgcagactcagtatttgttctgtcaaatgcagtgagcttctctaacctgattattagtttattgacttccacaacatagtggtcaattctagcagctcggtgttttttgaagtcggaaagatggcttctcacagcaccaagctcctggggttcccacatgtaaggatcaacccctccatagctgaaagactcatatccttgggtccctgactctgctcgatcatccccttctcgtttcaacaacctgtcctttgcttttttagccttctggacaagacctccaggatgggattcagctaaacctccatccgtggactggtgttccccataggcttaactggacacagagttcttgcttccccactactgcccacgcacttattgaatgcatgtgagaatacttgcaaaaagcttcaagaaacagatataacatttttaatttgccctttgacatcacggtcttcccctgagtgttcttcctcgtaatgtgagtgaagctgatagaaagactgcagatccttcaggcacagagggcagaggaagccctccctcacttcccctgggtcgtccagagaagccatggcagtgccgctctcaaccctaggaaggcaggaatctcatgccaagagtcagcttgattcctcccaaggaaccatggttcccgcagcattagcttaagcagcacacagatggtgaggaagtggcttcatggccctggatgaggtttcctctctggagtaggaggagcccttggcaattctcttacattcattccaaatgatccaacttcataattcatatgccacttcagccactgggggaatgtctgaagtacttatcaacaagcagaagtttttacttgatgctctttaccttgattgtttattcaaccacatatagtaagttcttgatacttgtaagacaccctgccgggctcctgcgggcacccaggtttgtcccccccttcaggcccgggctctgggcctccaccgtccgtcactcagccgcagccgccatctccatcggtcgctc

SEQ ID NO: 12780 - RNA, 1483 nt, Homo sapiens
  source 1..1483: mol_type = other RNA
gatgatgctgctgatgctgcctcggcgggagccatggacactgttgggtgactggctggggctggtgtgggtgctcagggactccttgctggcactggtgagcttgtttgccaagggaaggctgatgagctccatacacttcttgcacataatagacccgcagaggcggcagtggtggcggcggttccggatgctgaacttattcccacagtctggacagaaagggacatcctggtcgttgacccaaggcaccacagacttttctattgctcgaatctttgcagactcagtatttgttctgtcaaatgcagtgagcttctctaacctgattattagtttattgacttccacaacatagtggtcaattctagcagctcggtgttttttgaagtcggaaagatggcttctcacagcaccaagctcctggggttcccacatgtaaggatcaacccctccatagctgaaagactcatatccttgggtccctgactctgctcgatcatccccttctcgtttcaacaacctgtcctttgcttttttagccttctggacaagacctccaggatgggattcagctaaacctccatccgtggactggtgttccccataggcttaactggacacagagttcttgcttccccactactgcccacgcacttattgaatgcatgtgagaatacttgcaaaaagcttcaagaaacagatataacatttttaatttgccctttgacatcacggtcttcccctgagtgttcttcctcgtaatgtgagtgaagctgatagaaagactgcagatccttcaggcacagagggcagaggaagccctccctcacttcccctgggtcgtccagagaagccatggcagtgccgctctcaaccctaggaaggcaggaatctcatgccaagagtcagcttgattcctcccaaggaaccatggttcccgcagcattagcttaagcagcacacagatggtgaggaagtggcttcatggccctggatgaggtttcctctctggagtaggaggagcccttggcaattctcttacattcattccaaatgatccaacttcataattcatatgccacttcagccactgggggaatgtctgaagtacttatcaacaagcagaagtttttacttgatgctctttaccttgattgtttattcaaccacatatagtaagttcttgatacttgtaagacactcagagcatcagaatggacttctccttcacagcactcatctcaatttataaccgcaggtacatacgtgaagtgaccaagtaagactgtaaaatctgggagggcacagactctatatgttttccacttcgccgtctccccagggtttagcacagtaccctgccgggctcctgcgggcacccaggtttgtcccccccttcaggcccgggctctgggcctccaccgtccgtcactcagccgcagccgccatctccatcggtcgctcggaactcggcaggtgc

SEQ ID NO: 12781 - RNA, 1146 nt, Homo sapiens
  source 1..1146: mol_type = other RNA
gatgatgctgctgatgctgcctcggcgggagccatggacactgttgggtgactggctggggctggtgtgggtgctcagggactccttgctggcactggtgagcttgtttgccaagggaaggctgatgagctccatacacttcttgcacataatagacccgcagaggcggcagtggtggcggcggttccggatgctgaacttattcccacagtctggacagaaagggacatcctggtcgttgacccaaggcaccacagacttttctattgctcgaatctttgcagactcagtatttgttctgtcaaatgcagtgagcttctctaacctgattattagtttattgacttccacaacatagtggtcaattctagcagctcggtgttttttgaagtcggaaagatggcttctcacagcaccaagctcctggggttcccacatgtaaggatcaacccctccatagctgaaagactcatatccttgggtccctgactctgctcgatcatccccttctcgtttcaacaacctgtcctttgcttttttagccttctggacaagacttttaatttgccctttgacatcacggtcttcccctgagtgttcttcctcgtaatgtgagtgaagctgatagaaagactgcagatccttcaggcacagagggcagaggaagccctccctcacttcccctgggtcgtccagagaagccatggcagtgccgctctcaaccctaggaaggcaggaatctcatgccaagagtcagcttgattcctcccaaggaaccatggttcccgcagcattagcttaagcagcacacagatggtgaggaagtggcttcatggccctggatgaggtttcctctctggagtaggaggagccattcattccaaatgatccaacttcataattcatatgccacttcagccactgggggaatgtctgaagtacttatcaacaagcagaagtttttacttgatgctctttaccttgattgtttattcaaccacatatagtaagttcttgatacttgtaagacaccctgccgggctcctgcgggcacccaggtttgtcccccccttcaggcccgggctctgggcctccaccgtccgtcactcagccgcagccgccatctccatcggtcgctcggaactc

SEQ ID NO: 12782 - RNA, 1291 nt, Homo sapiens
  source 1..1291: mol_type = other RNA
gatgatgctgctgatgctgcctcggcgggagccatggacactgttgggtgactggctggggctggtgtgggtgctcagggactccttgctggcactggtgagcttgtttgccaagggaaggctgatgagctccatacacttcttgcacataatagacccgcagaggcggcagtggtggcggcggttccggatgctgaacttattcccacagtctggacagaaagggacatcctggtcgttgacccaaggcaccacagacttttctattgctcgaatctttgcagactcagtatttgttctgtcaaatgcagtgagcttctctaacctgattattagtttattgacttccacaacatagtggtcaattctagcagctcggtgttttttgaagtcggaaagatggcttctcacagcaccaagctcctggggttcccacatgtaaggatcaacccctccatagctgaaagactcatatccttgggtccctgactctgctcgatcatccccttctcgtttcaacaacctgtcctttgcttttttagccttctggacaagacttttaatttgccctttgacatcacggtcttcccctgagtgttcttcctcgtaatgtgagtgaagctgatagaaagactgcagatccttcaggcacagagggcagaggaagccctccctcacttcccctgggtcgtccagagaagccatggcagtgccgctctcaaccctaggaaggcaggaatctcatgccaagagtcagcttgattcctcccaaggaaccatggttcccgcagcattagcttaagcagcacacagatggtgaggaagtggcttcatggccctggatgaggtttcctctctggagtaggaggagccattcattccaaatgatccaacttcataattcatatgccacttcagccactgggggaatgtctgaagtacttatcaacaagcagaagtttttacttgatgctctttaccttgattgtttattcaaccacatatagtaagttcttgatacttgtaagacactcagagcatcagaatggacttctccttcacagcactcatctcaatttataaccgcaggtacatacgtgaagtgaccaagtaagactgtaaaatctgggagggcacagactctatatgttttccacttcgccgtctccccagggtttagcacagtaccctgccgggctcctgcgggcacccaggtttgtcccccccttcaggcccgggctctgggcctccaccgtccgtcactcagccgcagccgccatctccatcggtc

SEQ ID NO: 12783 - RNA, 1164 nt, Homo sapiens
  source 1..1164: mol_type = other RNA
gatgatgctgctgatgctgcctcggcgggagccatggacactgttgggtgactggctggggctggtgtgggtgctcagggactccttgctggcactggtgagcttgtttgccaagggaaggctgatgagctccatacacttcttgcacataatagacccgcagaggcggcagtggtggcggcggttccggatgctgaacttattcccacagtctggacagaaagggacatcctggtcgttgacccaaggcaccacagacttttctattgctcgaatctttgcagactcagtatttgttctgtcaaatgcagtgagcttctctaacctgattattagtttattgacttccacaacatagtggtcaattctagcagctcggtgttttttgaagtcggaaagatggcttctcacagcaccaagctcctggggttcccacatgtaaggatcaacccctccatagctgaaagactcatatccttgggtccctgactctgctcgatcatccccttctcgtttcaacaacctgtcctttgcttttttagccttctggacaagacttttaatttgccctttgacatcacggtcttcccctgagtgttcttcctcgtaatgtgagtgaagctgatagaaagactgcagatccttcaggcacagagggcagaggaagccctccctcacttcccctgggtcgtccagagaagccatggcagtgccgctctcaaccctaggaaggcaggaatctcatgccaagagtcagcttgattcctcccaaggaaccatggttcccgcagcattagcttaagcagcacacagatggtgaggaagtggcttcatggccctggatgaggtttcctctctggagtaggaggagcccttggcaattctcttacattcattccaaatgatccaacttcataattcatatgccacttcagccactgggggaatgtctgaagtacttatcaacaagcagaagtttttacttgatgctctttaccttgattgtttattcaaccacatatagtaagttcttgatacttgtaagacaccctctgtatgtaccctgccgggctcctgcgggcacccaggtttgtcccccccttcaggcccgggctctgggcctccaccgtccgtcactcagccgcagccgccatctccatcggt

SEQ ID NO: 12784 - RNA, 1163 nt, Homo sapiens
  source 1..1163: mol_type = other RNA
gatgatgctgctgatgctgcctcggcgggagccatggacactgttgggtgactggctggggctggtgtgggtgctcagggactccttgctggcactggtgagcttgtttgccaagggaaggctgatgagctccatacacttcttgcacataatagacccgcagaggcggcagtggtggcggcggttccggatgctgaacttattcccacagtctggacagaaagggacatcctggtcgttgacccaaggcaccacagacttttctattgctcgaatctttgcagactcagtatttgttctgtcaaatgcagtgagcttctctaacctgattattagtttattgacttccacaacatagtggtcaattctagcagctcggtgttttttgaagtcggaaagatggcttctcacagcaccaagctcctggggttcccacatgtaaggatcaacccctccatagctgaaagactcatatccttgggtccctgactctgctcgatcatccccttctcgtttcaacaacctgtcctttgcttttttagccttctggacaagacttttaatttgccctttgacatcacggtcttcccctgagtgttcttcctcgtaatgtgagtgaagctgatagaaagactgcagatccttcaggcacagagggcagaggaagccctccctcacttcccctgggtcgtccagagaagccatggcagtgccgctctcaaccctaggaaggcaggaatctcatgccaagagtcagcttgattcctcccaaggaaccatggttcccgcagcattagcttaagcagcacacagatggtgaggaagtggcttcatggccctggatgaggtttcctctctggagtaggaggagcccttggcaattctcttacattcattccaaatgatccaacttcataattcatatgccacttcagccactgggggaatgtctgaagtacttatcaacaagcagaagtttttacttgatgctctttaccttgattgtttattcaaccacatatagtaagttcttgatacttgtaagacaccctgccgggctcctgcgggcacccaggtttgtcccccccttcaggcccgggctctgggcctccaccgtccgtcactcagccgcagccgccatctccatcggtcgctcggaactc

SEQ ID NO: 12785 - RNA, 1319 nt, Homo sapiens
  source 1..1319: mol_type = other RNA
gatgatgctgctgatgctgcctcggcgggagccatggacactgttgggtgactggctggggctggtgtgggtgctcagggactccttgctggcactggtgagcttgtttgccaagggaaggctgatgagctccatacacttcttgcacataatagacccgcagaggcggcagtggtggcggcggttccggatgctgaacttattcccacagtctggacagaaagggacatcctggtcgttgacccaaggcaccacagacttttctattgctcgaatctttgcagactcagtatttgttctgtcaaatgcagtgagcttctctaacctgattattagtttattgacttccacaacatagtggtcaattctagcagctcggtgttttttgaagtcggaaagatggcttctcacagcaccaagctcctggggttcccacatgtaaggatcaacccctccatagctgaaagactcatatccttgggtccctgactctgctcgatcatccccttctcgtttcaacaacctgtcctttgcttttttagccttctggacaagacttttaatttgccctttgacatcacggtcttcccctgagtgttcttcctcgtaatgtgagtgaagctgatagaaagactgcagatccttcaggcacagagggcagaggaagccctccctcacttcccctgggtcgtccagagaagccatggcagtgccgctctcaaccctaggaaggcaggaatctcatgccaagagtcagcttgattcctcccaaggaaccatggttcccgcagcattagcttaagcagcacacagatggtgaggaagtggcttcatggccctggatgaggtttcctctctggagtaggaggagcccttggcaattctcttacattcattccaaatgatccaacttcataattcatatgccacttcagccactgggggaatgtctgaagtacttatcaacaagcagaagtttttacttgatgctctttaccttgattgtttattcaaccacatatagtaagttcttgatacttgtaagacactcagagcatcagaatggacttctccttcacagcactcatctcaatttataaccgcaggtacatacgtgaagtgaccaagtaagactgtaaaatctgggagggcacagactctatatgttttccacttcgccgtctccccagggtttagcacagtaccctgccgggctcctgcgggcacccaggtttgtcccccccttcaggcccgggctctgggcctccaccgtccgtcactcagccgcagccgccatctccatcggtcgctcggaactc

SEQ ID NO: 12786 - RNA, 668 nt, Homo sapiens
  source 1..668: mol_type = other RNA
gatgatgctgctgatgctgcctcggcgggagccatggacactgttgggtgactggctggggctggtgtgggtgctcagggactccttgctggcactggtgagcttgtttgccaagggaaggctgatgagctccatacacttcttgcacataatagacccgcagaggcggcagtggtggcggcggttccggatgctgaacttattcccacagtctggacagaaagggacatcctggtcgttgacccaaggcaccacagacttttctattgctcgaatctttgcagactcagtatttgttctgtcaaatgcagtgagcttctctaacctgattattagtttattgacttccacaacatagtggtcaattctagcagctcggtgttttttgaagtcggaaagatggcttctcacagcactgtttgtccctgggcaggttctcatgaggtgcagtgaagatctaacaagaccatgggtataaggcacttaatgtagtgcctaacacaaagtggatgctcagctggttctcttccattttcttcccccagcaagggcataaggtccatgagaagcttagaccattatggtttactgatgcctcctcagccaactcttaaaactttacctagaacatagcagatgctcaataaccacttgctgaatgaataaat

SEQ ID NO: 12787 - RNA, 491 nt, Homo sapiens
  source 1..491: mol_type = other RNA
gatgatgctgctgatgctgctggttggaggtccatactttgagaaccactgtgtaatcacccaaggggcttttcctgcctcctgcatgaacaaaatcagttcactgagaccatgttattgcagtaaagaaaaaagtttaattgacacaaggccagccatgcagtagatggagttattactcaactccatctccccaaaagctcagaggctagggtttttatggacaacttggtgggcaaggggctatggaaagggtactgctgaataattggggatgaaatcacaggagtgtgggaaatggtcctcgtgtgctgagtccacttctgggtagggccacaggaccagctgagtccatgagtcatgagtccagtggggtcagtcatagcatggcagttagaaacttagattctggagccacacttcagtccccaacttaacctctctgtgcctcagatatgcctcatacagacttcagacagggactacatgca

SEQ ID NO: 12788 - RNA, 94 nt, Homo sapiens
  source 1..94: mol_type = other RNA
gatgtactgaactgggtcagaccaggagagaggattcctggatcctggcccagtggccaatccgccctgggcttctcaccccccagactcctct

SEQ ID NO: 12789 - RNA, 35 nt, Homo sapiens
  source 1..35: mol_type = other RNA
gcagagaacaaaggactcagtaaatggtgctcagg

SEQ ID NO: 12790 - RNA, 472 nt, Homo sapiens
  source 1..472: mol_type = other RNA
gcagagtgcaaacaattttgacccggtcccagcgcttctcggcggctgcccggaccagcttgtcaggcccaaacatgcgaacgcggttggggtttgagccactgcggctctcggaaggggacatgaaagatgaggtgaccagaaggacctcatagtcttgctccccagcgcctccagctgaactgcccaccagcacctccacgaaagctgagccatcattcccaatgtccacactgtgtatctgctcctccttctccaactgtaggaccacagagatggtcttctcgcctgccttggctgcccgccattttcggtaagtgtctgccttgagaagattttctgcacagtgagtcgagtcctggctgctgcaggacacgacatggcggaggcggatctccggcatgtcaacgtcgtgggcttcgcctggccagaaggatgaggtagagtatggggtccgaggggcagggagagt

SEQ ID NO: 12791 - RNA, 1224 nt, Homo sapiens
  source 1..1224: mol_type = other RNA
gcagcccagctgaggcctctgaactgtgactccgccccgtggccgcatgcgtcggaactcctacctgccctttgcccttctcgaggccggtgcttgactggaggagggctggcagcagaagtgcagctgaccgggttgcgttttcgtacggctgactaaagcggataccggtggcgactcatttctcgttttatttttcaacgatttggcggagaagctcctcttgtgaatggactttggatttcttggagctgcgctgcgggtcccacagtgtggctttcggcccgtgctgtgctggcgcctgcacttcctctggcggggcacggggtggcgctccctggtaaagcagcggccagggggagccgtgagtgaggcgctgcctctcccgctgaagcgggttccaaggccaccgtgagggggaccatccatccaggtaaaacgtgttctttccttgttcctttgcgaatcgatggggatcaggcttccccaggtggtgaagtgaggaacagggaccgcggggctcgcctgaccagtggggtctccatccttgtccgtgctgacaaaagacaagaacagacagcgcctgaaatcttcccgcctccgtgagggaagcctgcgtctgggaacgcgccgcagggaagtgatccctgagtgagggaggaggtgccggggcatcattaatcagacctcaatgccgggaaggttctttgtttaaagaaacactcatgtttaaagagcacttggtgcggacttgctgtggccatcgccctcaacagctcatctttaggaggtgcaggctgaattcacgcctcggtgtcgtccatgtctgcctgccgcgcagaggagacagcgagaggccttcccaccgcacggcttttacgggaagctcttcgcattggctacaggggtgtggtttggtttatagccacaccaagtaattttaatagaactcaataactgtgttgccttgcaggctccgagtgctacaggcagacccgagtccgagtcttcctacggttcattgtccccccctggatttcctagggactccagatacgatggcatcgatgtcagttaacttggcacttcttaaaatagatctatgatcaaatcttaagtttttccgaataagactcatttaaaggaagcaatcttcaggcttttacaggatattgatctcttgggaatgtcagcaggggcacaaggagagcagtcgatgcgtct

SEQ ID NO: 12792 - RNA, 989 nt, Homo sapiens
  source 1..989: mol_type = other RNA
gcagcccagctgaggcctctgcagcctctgttgtcacctctggtgactcttcagcaggtggtacttcttgacctaccagttgttcaagaaccgcctttcctgcctcgttttcagaggtaactaccttctcctctggctcgtccccacccacatccactggcttgactgtcgggtctaaagactctgcttctacctccactgcagtgccctgcttttctagagtcaccacaggctgctcttctgaaacttcttttggcttctcctctatgctcacaattacctctccctgcttctcctgacctcctttttctctgcactcttcttggacatcagttccagaaactgatttttcttcctcagcatctggtacttcctgttctggcttcccagaagtgacctcagcttcattcggtccttctggtgctgctcctccttttgcctcttcagaggtttcagttaaccaatctagagtcaagtcaactttttcctgtggctcctctgcagatttacttatatccatatcttctcttccacccttctccatttcactgtcctgttctttatcagtttcaggctttgccaaagacttgtcttctgtttttttggcttcttctttttctcccatggcgtcataaacctgttctctcaactcttcccttgcttcctcatctatgttatcattattttctaccagagattcatcttctgttttttctccttcttcctcttccacatgcacaccttccaaggcgtttcccaacacaccattctccattctctccactttatctgcagatgtagaaggagcaggaacatcttcaattttgtcggcagaaaccagctccgcggcgacggcggcagtggctgtggactccatggccatcgttcccctgaggtggcgaaccagcgaacggaatagagcctgcgagaaaaacaggcaatttgggacgccagagactcactcagggacagaaaatggcagattagag

SEQ ID NO: 12793 - RNA, 1181 nt, Homo sapiens
  source 1..1181: mol_type = other RNA
gcagcccagctgaggcctctgcagcctctgttgtcacctctggtgactcttcagcaggtggtacttcttgacctaccagttgttcaagaaccgcctttcctgcctcgttttcagaggtaactaccttctcctctggctcgtccccacccacatccactggcttgactgtcgggtctaaagactctgcttctacctccactgcagtgccctgcttttctagagtcaccacaggctgctcttctgaaacttcttttggcttctcctctatgctcacaattacctctccctgcttctcctgacctcctttttctctgcactcttcttggacatcagttccagaaactgatttttcttcctcagcatctggtacttcctgttctggcttcccagaagtgacctcagcttcattcggtccttctggtgctgctcctccttttgcctcttcagaggtttcagttaaccaatctagagtcaagtcaactttttcctgtggctcctctgcagatttacttatatccatatcttctcttccacccttctccatttcactgtcctgttctttatcagtttcaggctttgccaaagacttgtcttctgtttttttggcttcttctttttctcccatggcgtcataaacctgttctctcaactcttcccttgcttcctcatctatgttatcattattttctaccagagattcatcttctgttttttctccttcttcctcttccacatgcacaccttccaaggcgtttcccaacacaccattctccattcttgccaactccagaagtgatttcccatagaaaaagaaggcttctccacactcattagctgtctctccatacttcttacctaaaagactagctgcttcctggaatgcattgacagctgctggaatatcccccatcaccagatgtttctgtcctaaacccaatagtttcttagcttcactatccacatccagactctccactttatctgcagatgtagaaggagcaggaacatcttcaattttgtcggcagaaaccagctccgcggcgacggcggcagtggctgtggactccatggccatcgttcccctgaggtggcgaaccagcgaacggaatagagcctgcgagaaaaacaggcaatttgggacgccagagactcactcagggacagaaaatggcagattagag

SEQ ID NO: 12794 - RNA, 1251 nt, Homo sapiens
  source 1..1251: mol_type = other RNA
gcagcccagctgaggcctctgcagcctctgttgtcacctctggtgactcttcagcaggtggtacttcttgacctaccagttgttcaagaaccgcctttcctgcctcgttttcagaggtaactaccttctcctctggctcgtccccacccacatccactggcttgactgtcgggtctaaagactctgcttctacctccactgcagtgccctgcttttctagagtcaccacaggctgctcttctgaaacttcttttggcttctcctctatgctcacaattacctctccctgcttctcctgacctcctttttctctgcactcttcttggacatcagttccagaaactgatttttcttcctcagcatctggtacttcctgttctggcttcccagaagtgacctcagcttcattcggtccttctggtgctgctcctccttttgcctcttcagaggtttcagttaaccaatctagagtcaagtcaactttttcctgtggctcctctgcagatttacttatatccatatcttctcttccacccttctccatttcactgtcctgttctttatcagtttcaggctttgccaaagacttgtcttctgtttttttggcttcttctttttctcccatggcgtcataaacctgttctctcaactcttcccttgcttcctcatctatgttatcattattttctaccagagattcatcttctgttttttctccttcttcctcttccacatgcacaccttccaaggcgtttcccaacacaccattctccattcttgccaactccagaagtgatttcccatagaaaaagaaggcttctccacactcattagctgtctctccatacttcttacctaaaagactagctgcttcctggaatgcattgacagctgctggaatatcccccatcaccagatgtttctgtcctaaacccaatagtttcttagcttcactatccacatccagatgtatgattctatttagataatattctacaaaatgcaacccatcttcagtgacagaaagcagattaatggttgctctccactttatctgcagatgtagaaggagcaggaacatcttcaattttgtcggcagaaaccagctccgcggcgacggcggcagtggctgtggactccatggccatcgttcccctgaggtggcgaaccagcgaacggaatagagcctgcgagaaaaacaggcaatttgggacgccagagactcactcagggacagaaaatggcagatta

SEQ ID NO: 12795 - RNA, 2776 nt, Homo sapiens
  source 1..2776: mol_type = other RNA
gcaggcacagacagccctggcacaaggccacctggcccttgcggaagtcgcggcaggggcagagccggcggtacttggtgttggagccggcgcagctgaagagcagaggctccttctgcaggtagcactcctggccaggctgggcgaacgccgggtacaggtggttcatctccgactcggtgctgtcacagggcacctgcagcttgaggaaggcgtcctggctgttcaggaaggggaagaaggagggctcacagattagcccgtggtccaggcaggtgtcggtgcaggccctcccaggcacggccagccaggcccgcagggcgtgcgcggggggccaggccccaggagccaagctggtgttccgagcccactcgaggtgggtggcattgggggccaggacaaaggggctctgcggggcgtgggcctctggtagggcagggtctggagctctgcagaagtcctggtgctggatgtaggcgtggatccgctccagcatcccctcgcaggtgtactcgtagggtaggtaggggtctacctgagttctcataatggccttgatggctgcttcaaactcctctgagttgttgtagtcgactgtccacacgtggggcttgccgatgaagttctccgcgtagggatgctgggagaacacctctctggaggtgggcttgcctcggaagaactcgtggttgagggagctgtggggcgggctgaagcgggactgcaggaagatgcaaccattggcgatggcctccaggggggcggggccctcgtaggggaagccaaacccgatgaagagtttggccttgcgcagcagctgctgaaactcaggctgcggtaagaggccgtggttcttcacaaaggctggcacctcggggggccgctggctctcgtagtacacggtgccatggatctccatgtatttgttcaggatgcccaggaacttctccttcccctggagcttccagatgctcgcctccttgccgtacaccacggccatgttgctggccttgccgcctttgatgagccgcttctccgtctcgttgagctcctcggacacgaagcccatgaaggagttgtcgggggtatgaggaaacatggtcatgaactgcttggggttgaggttccagtagccccagttggtccggtagccgtgcagcgtggcgtactcctcgtggttgtacgcaggttccgtcccgaaggtgtcgatgaccctgattcggcaccggtacttcttgaaggagagtcccatgtgccgcttcatctgctgcaggccgtggtagtcggtgtagatgaggtcgaagggcaggggcatggtgagcgggcagcttccccggcctggcggtacccctaagttactctgcagctccttcagggagactgtgacccgcaggccatggcccaggacatagagtgcagtcagaatgtccgcccactgcaccatctcccctaggggcccgcccttcaggacccgagggctgaacacgtccccggactcctccgtcaggaagccgatgtggaccaggatctgcttctggtccctctgggtggcccccagcttctgtgccaggcgctgggcagccagcgcccactgggctgtgagcctcttggtccgcttcttcatgaagatcagggactccttcccgctgcccatcaggtccagaaggtgggacaggttgcttcggaaaactgcctggactttggggaggggcttgggtgccctctgggcagccgtctggttcctccagggcagcggggggcagaaccactcgacctcactgaggtagatgaggaaggagcactcggtgccgtccaccccaaagaaggcgtagcaggggtcagaggtccagcgggcacgcatccactccaccttccctgagcagtcagggaacttggggtcactgggtgcctcacactggtcccgccggccttctgacaccttgctgtgcaggagcagactgtggcgcaggatctggtccaccttcacagcgatgtcggagacgttctgggcaatagcctggatccgctccatgaggccggccccagggggcatcctgtctgcgggaaagtgcaggtcgccgccggcccggtgcagctcactgctgttctccagcctggccagtgcgtccatgcgcttcaccatcagctccagcaggtcgctcatcttgcgcaggacgccgcgggactcggggccccccatcacttctgtgcggatggtgaatggcgagtcccccaggcgccgggccgagaactggcctcccagagacgtcatcaggaagcagagagtgaagaagccgatgcccaggacaaaaagcacttaggcatgaggcaggcgggctctagcctccaggcagagctggttcattaacagctgcagtcctgaaagtgcagtccccagacgagcagtcagcatcacctgagactccttagaaatgccaatgccgggcccagaccccaaattactgaatcagatactctggggtggagcaagcaagctgttttagcaaagtctcctgaagattccactgcatgctaaagtttgagaaccagtgatggacacagcagggcctgaggccagccagaccccatcaatcactcaggccagccttggtgcagtgtgcagaggccttgctgcagcagtcatgagcttgtttgaacacccccctccacttccaccactagatggtaagatgtccagggcagagccacacggcccatgcccaggctccccccaacacacatctcccctaggcaggcacgcccagggtcatcagcc

SEQ ID NO: 12796 - RNA, 3009 nt, Homo sapiens
  source 1..3009: mol_type = other RNA
gcaggcacagacagccctggcacaaggccacctggcccttgcggaagtcgcggcaggggcagagccggcggtacttggtgttggagccggcgcagctgaagagcagaggctccttctgcaggtagcactcctggccaggctgggcgaacgccgggtacaggtggttcatctccgactcggtgctgtcacagggcacctgcagcttgaggaaggcgtcctggctgttcaggaaggggaagaaggagggctcacagattagcccgtggtccaggcaggtgtcggtgcaggccctcccaggcacggccagccaggcccgcagggcgtgcgcggggggccaggccccaggagccaagctggtgttccgagcccactcgaggtgggtggcattgggggccaggacaaaggggctctgcggggcgtgggcctctggtagggcagggtctggagctctgcagaagtcctggtgctggatgtaggcgtggatccgctccagcatcccctcgcaggtgtactcgtagggtaggtaggggtctacctgagttctcataatggccttgatggctgcttcaaactcctctgagttgttgtagtcgactgtccacacgtggggcttgccgatgaagttctccgcgtagggatgctgggagaacacctctctggaggtgggcttgcctcggaagaactcgtggttgagggagctgtggggcgggctgaagcgggactgcaggaagatgcaaccattggcgatggcctccaggggggcggggccctcgtaggggaagccaaacccgatgaagagtttggccttgcgcagcagctgctgaaactcaggctgcggtaagaggccgtggttcttcacaaaggctggcacctcggggggccgctggctctcgtagtacacggtgccatggatctccatgtatttgttcaggatgcccaggaacttctccttcccctggagcttccagatgctcgcctccttgccgtacaccacggccatgttgctggccttgccgcctttgatgagccgcttctccgtctcgttgagctcctcggacacgaagcccatgaaggagttgtcgggggtatgaggaaacatggtcatgaactgcttggggttgaggttccagtagccccagttggtccggtagccgtgcagcgtggcgtactcctcgtggttgtacgcaggttccgtcccgaaggtgtcgatgaccctgattcggcaccggtacttcttgaaggagagtcccatgtgccgcttcatctgctgcaggccgtggtagtcggtgtagatgaggtcgaagggcaggggcatggtgagcgggcagcttccccggcctggcggtacccctaagttactctgcagctccttcagggagactgtgacccgcaggccatggcccaggacatagagtgcagtcagaatgtccgcccactgcaccatctcccctaggggcccgcccttcaggacccgagggctgaacacgtccccggactcctccgtcaggaagccgatgtggaccaggatctgcttctggtccctctgggtggcccccagcttctgtgccaggcgctgggcagccagcgcccactgggctgtgagcctcttggtccgcttcttcatgaagatcagggactccttcccgctgcccatcaggtccagaaggtgggacaggttgcttcggaaaactgcctggactttggggaggggcttgggtgccctctgggcagccgtctggttcctccagggcagcggggggcagaaccactcgacctcactgaggtagatgaggaaggagcactcggtgccgtccaccccaaagaaggcgtagcaggggtcagaggtccagcgggcacgcatccactccaccttccctgagcagtcagggaacttggggtcactgggtgcctcacactggtcccgccggccttctgacaccttgctgtgcaggagcagactgtggcgcaggatctggtccaccttcacagcgatgtcggagacgttctgggcaatagcctggatccgctccatgaggccggccccagggggcatcctgtctgcgggaaagtgcaggtcgccgccggcccggtgcagctcactgctgttctccagcctggccagtgcgtccatgcgcttcaccatcagctccagcaggtcgctcatcttgcgcaggacgccgcgggactcggggccccccatcacttctgtgcggatggtgaatggcgagtcccccaggcgccgggccgagaactggcctcccagagacgtcatcaggaagcagagagtgaagaagccgatgcccaggacaaaaagccgaaagggtctcagggtgaccaggcatcttctgaccattatcttcccatcggggttgacggtgatcattgttcaaacttgttggtgcgagcagccgcgggcgaggccggacgcaccgtcctgggcccagctctcgccgcgtccgggccacgaaccctctgcgggccgaagccgcgtccgagcgaagctgggagcgcgcggcccggtggcctcgctgctcaggcctgggcgtgcagcggagggagcggcgcggctgccggagggcggcgagggcgcccggccgggccgtctctgcgtctccgccctccccgcttcacattttggggaccgggaggcggcgcgcccccagaccgccggccgcgcgtctgcctgctcgggctcgctcgctgggcgggaaggtgccgcggcgcgcagacgggctccccgcggcgggcgccctcatccccggccccgcgccctcggtgccggctaaaggcggccccgggcccgcgccccggtccccagcgcctccgggccgcgccgatcctcagccccgcgccgcgccgcgcccatggctctcgacgagggcaacccgcgcccgccgcgcgctctctcgcccgctggctccgccgcccgcgctctggtgtccggcgtccggccccgcgcgacgctacgcccggaggcgccgcattgttcctcggaggaggcggccgagc

SEQ ID NO: 12797 - RNA, 2767 nt, Homo sapiens
  source 1..2767: mol_type = other RNA
gcaggcacagacagccctggcacaaggccacctggcccttgcggaagtcgcggcaggggcagagccggcggtacttggtgttggagccggcgcagctgaagagcagaggctccttctgcaggtagcactcctggccaggctgggcgaacgccgggtacaggtggttcatctccgactcggtgctgtcacagggcacctgcagcttgaggaaggcgtcctggctgttcaggaaggggaagaaggagggctcacagattagcccgtggtccaggcaggtgtcggtgcaggccctcccaggcacggccagccaggcccgcagggcgtgcgcggggggccaggccccaggagccaagctggtgttccgagcccactcgaggtgggtggcattgggggccaggacaaaggggctctgcggggcgtgggcctctggtagggcagggtctggagctctgcagaagtcctggtgctggatgtaggcgtggatccgctccagcatcccctcgcaggtgtactcgtagggtaggtaggggtctacctgagttctcataatggccttgatggctgcttcaaactcctctgagttgttgtagtcgactgtccacacgtggggcttgccgatgaagttctccgcgtagggatgctgggagaacacctctctggaggtgggcttgcctcggaagaactcgtggttgagggagctgtggggcgggctgaagcgggactgcaggaagatgcaaccattggcgatggcctccaggggggcggggccctcgtaggggaagccaaacccgatgaagagtttggccttgcgcagcagctgctgaaactcaggctgcggtaagaggccgtggttcttcacaaaggctggcacctcggggggccgctggctctcgtagtacacggtgccatggatctccatgtatttgttcaggatgcccaggaacttctccttcccctggagcttccagatgctcgcctccttgccgtacaccacggccatgttgctggccttgccgcctttgatgagccgcttctccgtctcgttgagctcctcggacacgaagcccatgaaggagttgtcgggggtatgaggaaacatggtcatgaactgcttggggttgaggttccagtagccccagttggtccggtagccgtgcagcgtggcgtactcctcgtggttgtacgcaggttccgtcccgaaggtgtcgatgaccctgattcggcaccggtacttcttgaaggagagtcccatgtgccgcttcatctgctgcaggccgtggtagtcggtgtagatgaggtcgaagggcaggggcatggtgagcgggcagcttccccggcctggcggtacccctaagttactctgcagctccttcagggagactgtgacccgcaggccatggcccaggacatagagtgcagtcagaatgtccgcccactgcaccatctcccctaggggcccgcccttcaggacccgagggctgaacacgtccccggactcctccgtcaggaagccgatgtggaccaggatctgcttctggtccctctgggtggcccccagcttctgtgccaggcgctgggcagccagcgcccactgggctgtgagcctcttggtccgcttcttcatgaagatcagggactccttcccgctgcccatcaggtccagaaggtgggacaggttgcttcggaaaactgcctggactttggggaggggcttgggtgccctctgggcagccgtctggttcctccagggcagcggggggcagaaccactcgacctcactgaggtagatgaggaaggagcactcggtgccgtccaccccaaagaaggcgtagcaggggtcagaggtccagcgggcacgcatccactccaccttccctgagcagtcagggaacttggggtcactgggtgcctcacactggtcccgccggccttctgacaccttgctgtgcaggagcagactgtggcgcaggatctggtccaccttcacagcgatgtcggagacgttctgggcaatagcctggatccgctccatgaggccggccccagggggcatccttctgtgcggatggtgaatggcgagtcccccaggcgccgggccgagaactggcctcccagagacgtcatcaggaagcagagagtgaagaagccgatgcccaggacaaaaagccgaaagggtctcagggtgaccaggcatcttctgaccattatcttcccatcggggttgacggtgatcattgttcaaacttgttggtgcgagcagccgcgggcgaggccggacgcaccgtcctgggcccagctctcgccgcgtccgggccacgaaccctctgcgggccgaagccgcgtccgagcgaagctgggagcgcgcggcccggtggcctcgctgctcaggcctgggcgtgcagcggagggagcggcgcggctgccggagggcggcgagggcgcccggccgggccgtctctgcgtctccgccctccccgcttcacattttggggaccgggaggcggcgcgcccccagaccgccggccgcgcgtctgcctgctcgggctcgctcgctgggcgggaaggtgccgcggcgcgcagacgggctccccgcggcgggcgccctcatccccggccccgcgccctcggtgccggctaaaggcggccccgggcccgcgccccggtccccagcgcctccgggccgcgccgatcctcagccccgcgccgcgccgcgcccatggctctcgacgagggcaacccgcgcccgccgcgcgctctctcgcccgct

SEQ ID NO: 12798 - RNA, 3003 nt, Homo sapiens
  source 1..3003: mol_type = other RNA
gcaggcacagacagccctggcacaaggccacctggcccttgcggaagtcgcggcaggggcagagccggcggtacttggtgttggagccggcgcagctgaagagcagaggctccttctgcaggtagcactcctggccaggctgggcgaacgccgggtacaggtggttcatctccgactcggtgctgtcacagggcacctgcagcttgaggaaggcgtcctggctgttcaggaaggggaagaaggagggctcacagattagcccgtggtccaggcaggtgtcggtgcaggccctcccaggcacggccagccaggcccgcagggcgtgcgcggggggccaggccccaggagccaagctggtgttccgagcccactcgaggtgggtggcattgggggccaggacaaaggggctctgcggggcgtgggcctctggtagggcagggtctggagctctgcagaagtcctggtgctggatgtaggcgtggatccgctccagcatcccctcgcaggtgtactcgtagggtaggtaggggtctacctgagttctcataatggccttgatggctgcttcaaactcctctgagttgttgtagtcgactgtccacacgtggggcttgccgatgaagttctccgcgtagggatgctgggagaacacctctctggaggtgggcttgcctcggaagaactcgtggttgagggagctgtggggcgggctgaagcgggactgcaggaagatgcaaccattggcgatggcctccaggggggcggggccctcgtaggggaagccaaacccgatgaagagtttggccttgcgcagcagctgctgaaactcaggctgcggtaagaggccgtggttcttcacaaaggctggcacctcggggggccgctggctctcgtagtacacggtgccatggatctccatgtatttgttcaggatgcccaggaacttctccttccccttccagatgctcgcctccttgccgtacaccacggccatgttgctggccttgccgcctttgatgagccgcttctccgtctcgttgagctcctcggacacgaagcccatgaaggagttgtcgggggtatgaggaaacatggtcatgaactgcttggggttgaggttccagtagccccagttggtccggtagccgtgcagcgtggcgtactcctcgtggttgtacgcaggttccgtcccgaaggtgtcgatgaccctgattcggcaccggtacttcttgaaggagagtcccatgtgccgcttcatctgctgcaggccgtggtagtcggtgtagatgaggtcgaagggcaggggcatggtgagcgggcagcttccccggcctggcggtacccctaagttactctgcagctccttcagggagactgtgacccgcaggccatggcccaggacatagagtgcagtcagaatgtccgcccactgcaccatctcccctaggggcccgcccttcaggacccgagggctgaacacgtccccggactcctccgtcaggaagccgatgtggaccaggatctgcttctggtccctctgggtggcccccagcttctgtgccaggcgctgggcagccagcgcccactgggctgtgagcctcttggtccgcttcttcatgaagatcagggactccttcccgctgcccatcaggtccagaaggtgggacaggttgcttcggaaaactgcctggactttggggaggggcttgggtgccctctgggcagccgtctggttcctccagggcagcggggggcagaaccactcgacctcactgaggtagatgaggaaggagcactcggtgccgtccaccccaaagaaggcgtagcaggggtcagaggtccagcgggcacgcatccactccaccttccctgagcagtcagggaacttggggtcactgggtgcctcacactggtcccgccggccttctgacaccttgctgtgcaggagcagactgtggcgcaggatctggtccaccttcacagcgatgtcggagacgttctgggcaatagcctggatccgctccatgaggccggccccagggggcatcctgtctgcgggaaagtgcaggtcgccgccggcccggtgcagctcactgctgttctccagcctggccagtgcgtccatgcgcttcaccatcagctccagcaggtcgctcatcttgcgcaggacgccgcgggactcggggccccccatcacttctgtgcggatggtgaatggcgagtcccccaggcgccgggccgagaactggcctcccagagacgtcatcaggaagcagagagtgaagaagccgatgcccaggacaaaaagccgaaagggtctcagggtgaccaggcatcttctgaccattatcttcccatcggggttgacggtgatcattgttcaaacttgttggtgcgagcagccgcgggcgaggccggacgcaccgtcctgggcccagctctcgccgcgtccgggccacgaaccctctgcgggccgaagccgcgtccgagcgaagctgggagcgcgcggcccggtggcctcgctgctcaggcctgggcgtgcagcggagggagcggcgcggctgccggagggcggcgagggcgcccggccgggccgtctctgcgtctccgccctccccgcttcacattttggggaccgggaggcggcgcgcccccagaccgccggccgcgcgtctgcctgctcgggctcgctcgctgggcgggaaggtgccgcggcgcgcagacgggctccccgcggcgggcgccctcatccccggccccgcgccctcggtgccggctaaaggcggccccgggcccgcgccccggtccccagcgcctccgggccgcgccgatcctcagccccgcgccgcgccgcgcccatggctctcgacgagggcaacccgcgcccgccgcgcgctctctcgcccgctggctccgccgcccgcgctctggtgtccggcgtccggccccgcgcgacgctacgcccggaggcgccgcattgttcctcggaggaggcggccgagc

SEQ ID NO: 12799 - RNA, 2513 nt, Homo sapiens
  source 1..2513: mol_type = other RNA
gcaggcacagacagccctggcacaaggccacctggcccttgcggaagtcgcggcaggggcagagccggcggtacttggtgttggagccggcgcagctgaagagcagaggctccttctgcaggtagcactcctggccaggctgggcgaacgccgggtacaggtggttcatctccgactcggtgctgtcacagggcacctgcagcttgaggaaggcgtcctggctgttcaggaaggggaagaaggagggctcacagattagcccgtggtccaggcaggtgtcggtgcaggccctcccaggcacggccagccaggcccgcagggcgtgcgcggggggccaggccccaggagccaagctggtgttccgagcccactcgaggtgggtggcattgggggccaggacaaaggggctctgcggggcgtgggcctctggtagggcagggtctggagctctgcagaagtcctggtgctggatgtaggcgtggatccgctccagcatcccctcgcaggtgtactcgtagggtaggtaggggtctacctgagttctcataatggccttgatggctgcttcaaactcctctgagttgttgtagtcgactgtccacacgtggggcttgccgatgaagttctccgcgtagggatgctgggagaacacctctctggaggtgggcttgcctcggaagaactcgtggttgagggagctgtggggcgggctgaagcgggactgcaggaagatgcaaccattggcgatggcctccaggggggcggggccctcgtaggggaagccaaacccgatgaagagtttggccttgcgcagcagctgctgaaactcaggctgcggtaagaggccgtggttcttcacaaaggctggcacctcggggggccgctggctctcgtagtacacggtgccatggatctccatgtatttgttcaggatgcccaggaacttctccttccccttccagatgctcgcctccttgccgtacaccacggccatgttgctggccttgccgcctttgatgagccgcttctccgtctcgttgagctcctcggacacgaagcccatgaaggagttgtcgggggtatgaggaaacatggtcatgaactgcttggggttgaggttccagtagccccagttggtccggtagccgtgcagcgtggcgtactcctcgtggttgtacgcaggttccgtcccgaaggtgtcgatgaccctgattcggcaccggtacttcttgaaggagagtcccatgtgccgcttcatctgctgcaggccgtggtagtcggtgtagatgaggtcgaagggcaggggcatggtgagcgggcagcttccccggcctggcggtacccctaagttactctgcagctccttcagggagactgtgacccgcaggccatggcccaggacatagagtgcagtcagaatgtccgcccactgcaccatctcccctaggggcccgcccttcaggacccgagggctgaacacgtccccggactcctccgtcaggaagccgatgtggaccaggatctgcttctggtccctctgggtggcccccagcttctgtgccaggcgctgggcagccagcgcccactgggctgtgagcctcttggtccgcttcttcatgaagatcagggactccttcccgctgcccatcaggtccagaaggtgggacaggttgcttcggaaaactgcctggactttggggaggggcttgggtgccctctgggcagccgtctggttcctccagggcagcggggggcagaaccactcgacctcactgaggtagatgaggaaggagcactcggtgccgtccaccccaaagaaggcgtagcaggggtcagaggtccagcgggcacgcatccactccaccttccctgagcagtcagggaacttggggtcactgggtgcctcacactggtcccgccggccttctgacaccttgctgtgcaggagcagactgtggcgcaggatctggtccaccttcacagcgatgtcggagacgttctgggcaatagcctggatccgctccatgaggccggccccagggggcatcctgtctgcgggaaagtgcaggtcgccgccggcccggtgcagctcactgctgttctccagcctggccagtgcgtccatgcgcttcaccatcagctccagcaggtcgctcatcttgcgcaggacgccgcgggactcggggccccccatcacttctgtgcggatggtgaatggcgagtcccccaggcgccgggccgagaactggcctcccagagacgtcatcaggaagcagagagtgaagaagccgatgcccaggacaaaaagcctgcggagaggaaggaggcgggtcaggagggcaggaagggccatcgtgccctgacgctccaccacgtaccggctgcacaaatgttttacgaatgagtgcatgagtgaaggaagcaagggagaatgaaaggatgggggctgagctccagacccaggagggcccccccactataggataaagagagctcaactacaagatgctggc

SEQ ID NO: 12800 - RNA, 2779 nt, Homo sapiens
  source 1..2779: mol_type = other RNA
gcaggcacagacagccctggcacaaggccacctggcccttgcggaagtcgcggcaggggcagagccggcggtacttggtgttggagccggcgcagctgaagagcagaggctccttctgcaggtagcactcctggccaggctgggcgaacgccgggtacaggtggttcatctccgactcggtgctgtcacagggcacctgcagcttgaggaaggcgtcctggctgttcaggaaggggaagaaggagggctcacagattagcccgtggtccaggcaggtgtcggtgcaggccctcccaggcacggccagccaggcccgcagggcgtgcgcggggggccaggccccaggagccaagctggtgttccgagcccactcgaggtgggtggcattgggggccaggacaaaggggctctgcggggcgtgggcctctggtagggcagggtctggagctctgcagaagtcctggtgctggatgtaggcgtggatccgctccagcatcccctcgcaggtgtactcgtagggtaggtaggggtctacctgagttctcataatggccttgatggctgcttcaaactcctctgagttgttgtagtcgactgtccacacgtggggcttgccgatgaagttctccgcgtagggatgctgggagaacacctctctggaggtgggcttgcctcggaagaactcgtggttgagggagctgtggggcgggctgaagcgggactgcaggaagatgcaaccattggcgatggcctccaggggggcggggccctcgtaggggaagccaaacccgatgaagagtttggccttgcgcagcagctgctgaaactcaggctgcggtaagaggccgtggttcttcacaaaggctggcacctcggggggccgctggctctcgtagtacacggtgccatggatctccatgtatttgttcaggatgcccaggaacttctccttcccgaaacatggtcatgaactgcttggggttgaggttccagtagccccagttggtccggtagccgtgcagcgtggcgtactcctcgtggttgtacgcaggttccgtcccgaaggtgtcgatgaccctgattcggcaccggtacttcttgaaggagagtcccatgtgccgcttcatctgctgcaggccgtggtagtcggtgtagatgaggtcgaagggcaggggcatggtgagcgggcagcttccccggcctggcggtacccctaagttactctgcagctccttcagggagactgtgacccgcaggccatggcccaggacatagagtgcagtcagaatgtccgcccactgcaccatctcccctaggggcccgcccttcaggacccgagggctgaacacgtccccggactcctccgtcaggaagccgatgtggaccaggatctgcttctggtccctctgggtggcccccagcttctgtgccaggcgctgggcagccagcgcccactgggctgtgagcctcttggtccgcttcttcatgaagatcagggactccttcccgctgcccatcaggtccagaaggtgggacaggttgcttcggaaaactgcctggactttggggaggggcttgggtgccctctgggcagccgtctggttcctccagggcagcggggggcagaaccactcgacctcactgaggtagatgaggaaggagcactcggtgccgtccaccccaaagaaggcgtagcaggggtcagaggtccagcgggcacgcatccactccaccttccctgagcagtcagggaacttggggtcactgggtgcctcacactggtcccgccggccttctgacaccttgctgtgcaggagcagactgtggcgcaggatctggtccaccttcacagcgatgtcggagacgttctgggcaatagcctggatccgctccatgaggccggccccagggggcatcctgtctgcgggaaagtgcaggtcgccgccggcccggtgcagctcactgctgttctccagcctggccagtgcgtccatgcgcttcaccatcagctccagcaggtcgctcatcttgcgcaggacgccgcgggactcggggccccccatcacttctgtgcggatggtgaatggcgagtcccccaggcgccgggccgagaactggcctcccagagacgtcatcaggaagcagagagtgaagaagccgatgcccaggacaaaaagccgaaagggtctcagggtgaccaggcatcttctgaccattatcttcccatcggggttgacggtgatcattgttcaaacttgttggtgcgagcagccgcgggcgaggccggacgcaccgtcctgggcccagctctcgccgcgtccgggccacgaaccctctgcgggccgaagccgcgtccgagcgaagctgggagcgcgcggcccggtggcctcgctgctcaggcctgggcgtgcagcggagggagcggcgcggctgccggagggcggcgagggcgcccggccgggccgtctctgcgtctccgccctccccgcttcacattttggggaccgggaggcggcgcgcccccagaccgccggccgcgcgtctgcctgctcgggctcgctcgctgggcgggaaggtgccgcggcgcgcagacgggctccccgcggcgggcgccctcatccccggccccgcgccctcggtgccggctaaaggcggccccgggcccgcgccccggtccccagcgcctccgggccgcgccgatcctcagccccgcgccgcgccgcgcccatggctctcgacgagggcaacccgcgcccgccgcgcgctctctcgcccgctg

SEQ ID NO: 12801 - RNA, 3476 nt, Homo sapiens
  source 1..3476: mol_type = other RNA
gcagggacagcaaaggggtgccacaatcacttggcaaggatggatggcacagggaacagggaatgatttataaatccttctgagagcagaaagccgtcttcccatcatctttatagctgactcccccggctcttagagacctgtgatagcagcatcattaccacttccctgcatccatctcttgcacttttgtaatatgggaaagagagattaattgtatggtgaaactcttcaacaatttgctgaacctctgcattcctgacattaatctttccccaagtgccctatcattaacttgaaaaatcaaccgggcaaaaccttagagtaggttcatgcaaatgaaaatacataaatagtgtgcggggatggtgcagggatggagacggggagggctgtcggctgccagagaacctatagcaaaatgatacattaagctgttttcctaaatgcttcacccatgaaacatgtcgtttatccacaaccctgtactatttcattagaatcgtttactttgggcctggacctgctactagcaagaaaaccacttccgccttcaagttttcaaagtatgcaaataaaaaaatcacttctcttcctctgtctccaaaagaaaatctctattctctcttcattcgtgcgattcagcaactagccgccttttcctaggttttcttcaatttgaaaagaaaataaaacacacttgttttgagattttcccacatcataaatgttctcattatgccaaatttgactactactcttatcaaatataaaattggctagagaaatatattcacttttgaagttttgaattcattttttaaataagacccctccacatgtagatttgttcttatgtaagaggaggtcttgatctgtgctcacaacatcattataaccagatagagaaacagagattctatcaaggagaaaatggcccttgagtagagttcataagtgtggattttgcccatgaggtgccccttggtggcagaagccaatgtgtggctttgccctggccaatcctctgttttctctctttgtagccccaactgtgatttaagtcttatgctacatcatgaatcagagttcaatcatgaatgttagtagtttaggaatgaaaagtaagaatgcacccatttttctactgactacttttgaactagatctttaaaaaaaaaaaatcggcactaagctgaatctccccagaatggagcgtcatctacttccccatccataaccactggtcacctgagtcaggcagagggaagaatgcatgattcaaatcaaaccaggttaaatgaacagacagaattagagagtcctcaaaagggaaactcagcgattttctaagatggttttctagatttagttgaaagttaaatacataaatcttataaaatctgcaatgtttgtgctaggaacaaaatgtaaagtggaatttaaaatgaaaagtgattcaccacttattatactttttcctttgtaaattgtaagtgattgtaggatcaagaaagttaaaacttagcaaaggcttggatttaagtaaaaaggcagtcagggtttttttcaattattcattcaattaatatttattgagaggctttagcgtgcacatctcactcaaggcaaacagttgagaagcttataatttagacagcacaagacaaatacttgagtaatagataatataattacatataaacaggtcacatgtagaatctcccagagcaaaccttcttttctcgagtttgctgatgtctgtagctaggaagaacaaaaacaaatgattagagtcttcatgattacggatttgtttggactttgattactaactaaattaataatttatttttataagctaacttcagcttaaaatcatttgagcttatgtgcaaggtaaatatgtttgaatttttaacactttctatgtaatactagggaaccccatttgacaaatttagtagaaccatcattaatctacatagattattttattgaactaaaagcaattattaatattcgttaagtgccaggcagtttacacacacacacacacaatttatccctctaaccttatgaagggcatactatcatcatctgcataaaagctaacaaagtttatgatgcattgcagtgaaagtgtaaacagaatttttcttttgcaaggaatttaggggattacggtgctccacagttacacatttatcatttacttattgcacggtaagccgtcgggatataaagatgatcgagacctgatacttcctctgcagcttaccttctaaagagagagatggacatgtaaacaggggcgctgaaggaggtgaagacactgtgctggaaatcttaaaggtggagtggggcagggagttccacccggagccttcacggagcagtgacacatggactttcttggtttgatctttatctagaaggcagcctggacaagttgaagccatgtctaagcattccccaagttttaacagtgtacttgaggcaatgtggttattattgttgtgatctcacaaccagacagagtggtgatctacagtacccttagcaagtaagaaagtgcattgccagtttcattgcatctactgtaaagatcttggccagtaccgtaaagatcttggccatgtactgcaaagatcttggaagcagagaatagcaacaacatcctcatgttaaaagcagaagacactagaggtctctggagatagaataaaacctccttctatttgcctcttattctatccaacaaataaaatccatcagcaacctttcatgacatcgactcaatacccagagtacattttgagggactaaccacaccaggacctactaagcacttcatgacagcagtttgttgggaataagaattatggatggtgcagtccaataacatgagtatgtgcatgtgatttaacagcttcaaatagcagtgtgtagtgaatacatgccaacataacttacctaggactcaacctaaactcttaagatgcaacacgcattcacacacatacttgtttctaaagttattacattctatagttgttcacttctgctagctctagaatgagtaaggctgaattctttccccaaagcatactgtaaattatcatatcatagacttttgatagaatttcaagtatttgtgaatcattaataattgtcctaactttaaaaaggtgtctaccttgaacatgatattcaaatcatgaattcctgaaggctcgttgagttggttgttcttggccatcatcttgaagcatactgtgcatcttaattttccctaaggaatatgttgttgcctccatcggcttgatgaaatcagtgctcagaaccgttttaggcttgaattctccttacaacattccttcgcgacgtctccaattccctaggactcttcctttctggttcttctttggctaaaaagtcctttgcgttgtcctttatacttttgtaactccagc

SEQ ID NO: 12802 - RNA, 3424 nt, Homo sapiens
  source 1..3424: mol_type = other RNA
gcagggacagcaaaggggtgccacaatcacttggcaaggatggatggcacagggaacagggaatgatttataaatccttctgagagcagaaagccgtcttcccatcatctttatagctgactcccccggctcttagagacctgtgatagcagcatcattaccacttccctgcatccatctcttgcacttttgtaatatgggaaagagagattaattgtatggtgaaactcttcaacaatttgctgaacctctgcattcctgacattaatctttccccaagtgccctatcattaacttgaaaaatcaaccgggcaaaaccttagagtaggttcatgcaaatgaaaatacataaatagtgtgcggggatggtgcagggatggagacggggagggctgtcggctgccagagaacctatagcaaaatgatacattaagctgttttcctaaatgcttcacccatgaaacatgtcgtttatccacaaccctgtactatttcattagaatcgtttactttgggcctggacctgctactagcaagaaaaccacttccgccttcaagttttcaaagtatgcaaataaaaaaatcacttctcttcctctgtctccaaaagaaaatctctattctctcttcattcgtgcgattcagcaactagccgccttttcctaggttttcttcaatttgaaaagaaaataaaacacacttgttttgagattttcccacatcataaatgttctcattatgccaaatttgactactactcttatcaaatataaaattggctagagaaatatattcacttttgaagttttgaattcattttttaaataagacccctccacatgtagatttgttcttatgtaagaggaggtcttgatctgtgctcacaacatcattataaccagatagagaaacagagattctatcaaggagaaaatggcccttgagtagagttcataagtgtggattttgcccatgaggtgccccttggtggcagaagccaatgtgtggctttgccctggccaatcctctgttttctctctttgtagccccaactgtgatttaagtcttatgctacatcatgaatcagagttcaatcatgaatgttagtagtttaggaatgaaaagtaagaatgcacccatttttctactgactacttttgaactagatctttaaaaaaaaaaaatcggcactaagctgaatctccccagaatggagcgtcatctacttccccatccataaccactggtcacctgagtcaggcagagggaagaatgcatgattcaaatcaaaccaggttaaatgaacagacagaattagagagtcctcaaaagggaaactcagcgattttctaagatggttttctagatttagttgaaagttaaatacataaatcttataaaatctgcaatgtttgtgctaggaacaaaatgtaaagtggaatttaaaatgaaaagtgattcaccacttattatactttttcctttgtaaattgtaagtgattgtaggatcaagaaagttaaaacttagcaaaggcttggatttaagtaaaaaggcagtcagggtttttttcaattattcattcaattaatatttattgagaggctttagcgtgcacatctcactcaaggcaaacagttgagaagcttataatttagacagcacaagacaaatacttgagtaatagataatataattacatataaacaggtcacatgtagaatctcccagagcaaaccttcttttctcgagtttgctgatgtctgtagctaggaagaacaaaaacaaatgattagagtcttcatgattacggatttgtttggactttgattactaactaaattaataatttatttttataagctaacttcagcttaaaatcatttgagcttatgtgcaaggtaaatatgtttgaatttttaacactttctatgtaatactagggaaccccatttgacaaatttagtagaaccatcattaatctacatagattattttattgaactaaaagcaattattaatattcgttaagtgccaggcagtttacacacacacacacacaatttatccctctaaccttatgaagggcatactatcatcatctgcataaaagctaacaaagtttatgatgcattgcagtgaaagtgtaaacagaatttttcttttgcaaggaatttaggggattacggtgctccacagttacacatttatcatttacttattgcacggtaagccgtcgggatataaagatgatcgagacctgatacttcctctgcagcttaccttctaaagagagagatggacatgtaaacaggggcgctgaaggaggtgaagacactgtgctggaaatcttaaaggtggagtggggcagggagttccacccggagccttcacggagcagtgacacatggactttcttggtttgatctttatctagaaggcagcctggacaagttgaagccatgtctaagcattccccaagttttaacagtgtacttgaggcaatgtggttattattgttgtgatctcacaaccagacagagtggtgatctacagtacccttagcaagtaagaaagtgcattgccagtttcattgcatctactgtaaagatcttggccagtaccgtaaagatcttggccatgtactgcaaagatcttggaagcagagaatagcaacaacatcctcatgttaaaagcagaagacactagaggtctctggagatagaataaaacctccttctatttgcctcttattctatccaacaaataaaatccatcagcaacctttcatgacatcgactcaatacccagagtacattttgagggactaaccacaccaggacctactaagcacttcatgacagcagtttgttgggaataagaattatggatggtgcagtccaataacatgagtatgtgcatgtgatttaacagcttcaaatagcagtgtgtagtgaatacatgccaacataacttacctaggactcaacctaaactcttaagatgcaacacgcattcacacacatacttgtttctaaagttattacattctatagttgttcacttctgctagctctagaatgagtaaggctgaattctttccccaaagcatactgtaaattatcatatcatagacttttgatagaatttcaagtatttgtgaatcattaataattgtcctaactttaaaaaggtgtctaccttgaacatgatattcaaatcatgaattcctgaaggctcgttgagttggttgttcttggccatcatcttgaagcatactgtgcatcttaattttccctaaggaatatgttgttgcctccatcggcttgatgaaatcagtgctcagaacctttctggttcttctttggctaaaaagtcctttgcgttgtcctttatacttttgtaactccagcactttggaacttg

SEQ ID NO: 12803 - RNA, 2658 nt, Homo sapiens
  source 1..2658: mol_type = other RNA
gcagggacagcaaaggggtgccacaatcacttggcaaggatggatggcacagggaacagggaatgatttataaatccttctgagagcagaaagccgtcttcccatcatctttatagctgactcccccggctcttagagacctgtgatagcagcatcattaccacttccctgcatccatctcttgcacttttgtaatatgggaaagagagattaattgtatggtgaaactcttcaacaatttgctgaacctctgcattcctgacattaatctttccccaagtgccctatcattaacttgaaaaatcaaccgggcaaaaccttagagtaggttcatgcaaatgaaaatacataaatagtgtgcggggatggtgcagggatggagacggggagggctgtcggctgccagagaacctatagcaaaatgatacattaagctgttttcctaaatgcttcacccatgaaacatgtcgtttatccacaaccctgtactatttcattagaatcgtttactttgggcctggacctgctactagcaagaaaaccacttccgccttcaagttttcaaagtatgcaaataaaaaaatcacttctcttcctctgtctccaaaagaaaatctctattctctcttcattcgtgcgattcagcaactagccgccttttcctaggttttcttcaatttgaaaagaaaataaaacacacttgttttgagattttcccacatcataaatgttctcattatgccaaatttgactactactcttatcaaatataaaattggctagagaaatatattcacttttgaagttttgaattcattttttaaataagacccctccacatgtagatttgttcttatgtaagaggaggtcttgatctgtgctcacaacatcattataaccagatagagaaacagagattctatcaaggagaaaatggcccttgagtagagttcataagtgtggattttgcccatgaggtgccccttggtggcagaagccaatgtgtggctttgccctggccaatcctctgttttctctctttgtagccccaactgtgatttaagtcttatgctacatcatgaatcagagttcaatcatgaatgttagtagtttaggaatgaaaagtaagaatgcacccatttttctactgactacttttgaactagatctttaaaaaaaaaaaatcggcactaagctgaatctccccagaatggagcgtcatctacttccccatccataaccactggtcacctgagtcaggcagagggaagaatgcatgattcaaatcaaaccaggttaaatgaacagacagaattagagagtcctcaaaagggaaactcagcgattttctaagatggttttctagatttagttgaaagttaaatacataaatcttataaaatctgcaatgtttgtgctaggaacaaaatgtaaagtggaatttaaaatgaaaagtgattcaccacttattatactttttcctttgtaaattgtaagtgattgtaggatcaagaaagttaaaacttagcaaaggcttggatttaagtaaaaaggcagtcagggtttttttcaattattcattcaattaatatttattgagaggctttagcgtgcacatctcactcaaggcaaacagttgagaagcttataatttagacagcacaagacaaatacttgagtaatagataatataattacatataaacaggtcacatgtagaatctcccagagcaaaccttcttttctcgagtttgctgatgtctgtagctaggaagaacaaaaacaaatgattagagtcttcatgattacggatttgtttggactttgattactaactaaattaataatttatttttataagctaacttcagcttaaaatcatttgagcttatgtgcaaggtaaatatgtttgaatttttaacactttctatgtaatactagggaaccccatttgacaaatttagtagaaccatcattaatctacatagattattttattgaactaaaagcaattattaatattcgttaagtgccaggcagtttacacacacacacacacaatttatccctctaaccttatgaagggcatactatcatcatctgcataaaagctaacaaagtttatgatgcattgcagtgaaagtgtaaacagaatttttcttttgcaaggaatttaggggattacggtgctccacagttacacatttatcatttacttattgcacggtaagccgtcgggatataaagatgatcgagacctgatacttcctctgcagcttaccttctaaagagagagatggacatgtaaacaggggcgctgaaggaggtgaagacactgtgctggaaatcttaaaggtggagtggggcagggagttccacccggagccttcacggagcagtgacacatggactttcttggtttgatctttatctagaaggcagccttgaacatgatattcaaatcatgaattcctgaaggctcgttgagttggttgttcttggccatcatcttgaagcatactgtgcatcttaattttccctaaggaatatgttgttgcctccatcggcttgatgaaatcagtgctcagaaccgttttaggcttgaattctccttacaacattccttcgcgacgtctccaattccctaggactcttcct

SEQ ID NO: 12804 - RNA, 2900 nt, Homo sapiens
  source 1..2900: mol_type = other RNA
gcagggacagcaaaggggtgccacaatcacttggcaaggatggatggcacagggaacagggaatgatttataaatccttctgagagcagaaagccgtcttcccatcatctttatagctgactcccccggctcttagagacctgtgatagcagcatcattaccacttccctgcatccatctcttgcacttttgtaatatgggaaagagagattaattgtatggtgaaactcttcaacaatttgctgaacctctgcattcctgacattaatctttccccaagtgccctatcattaacttgaaaaatcaaccgggcaaaaccttagagtaggttcatgcaaatgaaaatacataaatagtgtgcggggatggtgcagggatggagacggggagggctgtcggctgccagagaacctatagcaaaatgatacattaagctgttttcctaaatgcttcacccatgaaacatgtcgtttatccacaaccctgtactatttcattagaatcgtttactttgggcctggacctgctactagcaagaaaaccacttccgccttcaagttttcaaagtatgcaaataaaaaaatcacttctcttcctctgtctccaaaagaaaatctctattctctcttcattcgtgcgattcagcaactagccgccttttcctaggttttcttcaatttgaaaagaaaataaaacacacttgttttgagattttcccacatcataaatgttctcattatgccaaatttgactactactcttatcaaatataaaattggctagagaaatatattcacttttgaagttttgaattcattttttaaataagacccctccacatgtagatttgttcttatgtaagaggaggtcttgatctgtgctcacaacatcattataaccagatagagaaacagagattctatcaaggagaaaatggcccttgagtagagttcataagtgtggattttgcccatgaggtgccccttggtggcagaagccaatgtgtggctttgccctggccaatcctctgttttctctctttgtagccccaactgtgatttaagtcttatgctacatcatgaatcagagttcaatcatgaatgttagtagtttaggaatgaaaagtaagaatgcacccatttttctactgactacttttgaactagatctttaaaaaaaaaaaatcggcactaagctgaatctccccagaatggagcgtcatctacttccccatccataaccactggtcacctgagtcaggcagagggaagaatgcatgattcaaatcaaaccaggttaaatgaacagacagaattagagagtcctcaaaagggaaactcagcgattttctaagatggttttctagatttagttgaaagttaaatacataaatcttataaaatctgcaatgtttgtgctaggaacaaaatgtaaagtggaatttaaaatgaaaagtgattcaccacttattatactttttcctttgtaaattgtaagtgattgtaggatcaagaaagttaaaacttagcaaaggcttggatttaagtaaaaaggcagtcagggtttttttcaattattcattcaattaatatttattgagaggctttagcgtgcacatctcactcaaggcaaacagttgagaagcttataatttagacagcacaagacaaatacttgagtaatagataatataattacatataaacaggtcacatgtagaatctcccagagcaaaccttcttttctcgagtttgctgatgtctgtagcttctaaagagagagatggacatgtaaacaggggcgctgaaggaggtgaagacactgtgctggaaatcttaaaggtggagtggggcagggagttccacccggagccttcacggagcagtgacacatggactttcttggtttgatctttatctagaaggcagcctggacaagttgaagccatgtctaagcattccccaagttttaacagtgtacttgaggcaatgtggttattattgttgtgatctcacaaccagacagagtggtgatctacagtacccttagcaagtaagaaagtgcattgccagtttcattgcatctactgtaaagatcttggccagtaccgtaaagatcttggccatgtactgcaaagatcttggaagcagagaatagcaacaacatcctcatgttaaaagcagaagacactagaggtctctggagatagaataaaacctccttctatttgcctcttattctatccaacaaataaaatccatcagcaacctttcatgacatcgactcaatacccagagtacattttgagggactaaccacaccaggacctactaagcacttcatgacagcagtttgttgggaataagaattatggatggtgcagtccaataacatgagtatgtgcatgtgatttaacagcttcaaatagcagtgtgtagtgaatacatgccaacataacttacctaggactcaacctaaactcttaagatgcaacacgcattcacacacatacttgtttctaaagttattacattctatagttgttcacttctgctagctctagaatgagtaaggctgaattctttccccaaagcatactgtaaattatcatatcatagacttttgatagaatttcaagtatttgtgaatcattaataattgtcctaactttaaaaaggtgtctaccttgaacatgatattcaaatcatgaattcctgaaggctcgttgagttggttgttcttggccatcatcttgaagcatactgtgcatcttaattttccctaaggaatatgttgttgcctccatcggcttgatgaaatcagtgctcagaaccgttttaggcttgaattctccttacaacattccttcgcgacgtctccaattccctaggactcttcct

SEQ ID NO: 12805 - RNA, 1982 nt, Homo sapiens
  source 1..1982: mol_type = other RNA
gcagggacagcaaaggggtgccacaatcacttggcaaggatggatggcacagggaacagggaatgatttataaatccttctgagagcagaaagccgtcttcccatcatctttatagctgactcccccggctcttagagacctgtgatagcagcatcattaccacttccctgcatccatctcttgcacttttgtaatatgggaaagagagattaattgtatggtgaaactcttcaacaatttgctgaacctctgcattcctgacattaatctttccccaagtgccctatcattaacttgaaaaatcaaccgggcaaaaccttagagtaggttcatgcaaatgaaaatacataaatagtgtgcggggatggtgcagggatggagacggggagggctgtcggctgccagagaacctatagcaaaatgatacattaagctgttttcctaaatgcttcacccatgaaacatgtcgtttatccacaaccctgtactatttcattagaatcgtttactttgggcctggacctgctactagcaagaaaaccacttccgccttcaagttttcaaagtatgcaaataaaaaaatcacttctcttcctctgtctccaaaagaaaatctctattctctcttcattcgtgcgattcagcaactagccgccttttcctaggttttcttcaatttgaaaagaaaataaaacacacttgttttgagattttcccacatcataaatgttctcattatgccaaatttgactactactcttatcaaatataaaattggctagagaaatatattcacttttgaagttttgaattcattttttaaataagacccctccacatgtagatttgttcttatgtaagaggaggtcttgatctgtgctcacaacatcattataaccagatagagaaacagagattctatcaaggagaaaatggcccttgagtagagttcataagtgtggattttgcccatgaggtgccccttggtggcagaagccaatgtgtggctttgccctggccaatcctctgttttctctctttgtagccccaactgtgatttaagtcttatgctacatcatgaatcagagttcaatcatgaatgttagtagtttaggaatgaaaagtaagaatgcacccatttttctactgactacttttgaactagatctttaaaaaaaaaaaatcggcactaagctgaatctccccagaatggagcgtcatctacttccccatccataaccactggtcacctgagtcaggcagagggaagaatgcatgattcaaatcaaaccaggttaaatgaacagacagaattagagagtcctcaaaagggaaactcagcgattttctaagatggttttctagatttagttgaaagttaaatacataaatcttataaaatctgcaatgtttgtgctaggaacaaaatgtaaagtggaatttaaaatgaaaagtgattcaccacttattatactttttcctttgtaaattgtaagtgattgtaggatcaagaaagttaaaacttagcaaaggcttggatttaagtaaaaaggcagtcagggtttttttcaattattcattcaattaatatttattgagaggctttagcgtgcacatctcactcaaggcaaacagttgagaagcttataatttagacagcacaagacaaatacttgagtaatagataatataattacatataaacaggtcacatgtagaatctcccagagcaaaccttcttttctcgagtttgctgatgtctgtagcttgaacatgatattcaaatcatgaattcctgaaggctcgttgagttggttgttcttggccatcatcttgaagcatactgtgcatcttaattttccctaaggaatatgttgttgcctccatcggcttgatgaaatcagtgctcagaaccgttttaggcttgaattctccttacaacattccttcgcgacgtctccaattccctaggactcttcct

SEQ ID NO: 12806 - RNA, 206 nt, Homo sapiens
  source 1..206: mol_type = other RNA
gccctgtggactcagttctggtaaagagtttactgttggcatgtaaaaaatgcacattatgacaaaagagatcccaactctaaagacattgaagccggaaaacattatcagctgcagttgtatctgagcggattttgtctgttttttcactgctgtgttctgtttcctaagacaacacttccatgctgtcctctgtatctgctgtt

SEQ ID NO: 12807 - RNA, 476 nt, Homo sapiens
  source 1..476: mol_type = other RNA
gccctgtggactcagttctggtaaagagtttactgttggcatgtaaaaaatgcacattatgacaaaagagatcccaactctaaagacattgaagccggaaaacattatcagctgcagttgtatctgagcggattttgtctgttttttcactgctgtgttctgtttcctaagacaacacttccatgctgtcctctgtatctgctgttaattctttattttctattttgctactttcaaatttttcttgaacaacttcaagaagttttctactgatgatctatgttatctgcccgggacctgcgggcggggacctgggccgttcccgaggccgcgcggccaacagttcccgccgccacgcgacggaggaggaggcagaagacggggccgtgccagactagccgggtagcctggaaccacttcgccaacctgcaaaggcgtagcacttctccctcccagcctgcagccgccaccgactc

SEQ ID NO: 12808 - RNA, 534 nt, Homo sapiens
  source 1..534: mol_type = other RNA
gccctgtggactcagttctggtaaagagtttactgttggcatgtaaaaaatgcacattatgacaaaagagatcccaactctaaagacattgaagccggaaaacattatcagctgcagttgtatctgagcggattttgtctgttttttcactgctgtgttctgtttcctaagacaacacttccatgctgtcctctgtatctgctgttaattctttattttctattttgctactttcaaatttttcttgaacaacttcaagaagttttctactgatgatctatgttatctgcccgggacctgcgggcggggacctgggccgttcccgaggccgcgcggccaacagttcccgccgccacgcgacggaggaggaggcagaagacggggccgtgccagactagccgggtagcctggaaccacttcgccaacctgcaaaggcgtagcacttctccctcccagcctgcagccgccaccgactcggcggagtcggcctcctgggaaaaaacaacctgcgaagctcctccttctcctcgtgct

SEQ ID NO: 12809 - RNA, 2702 nt, Homo sapiens
  source 1..2702: mol_type = other RNA
gcctctctcggagtcgctcggactttagcaaggaaagggaaggctgtgagccagatgctggggtcactcaggaaagcaagaaagtgttagaaacagtgctatatggagtccaacaccagcaaagctcttggataataatcacaaaacagtggtcgagagaagtactggagagaacggaaaagccgatcccactttcgttcagttaagggacaggaataagagaaagatacgttgagaagattacaagagaaatggtgtcttcagagaaaaggcaatggtcacctaatggtagaagcagaggtacaaataattttttgataagatctgtgcaggtttttaaaatatagagtctcaaggaataggtcgtacaggttcaagttagacaaacgtaagacaagaggttaagactctctggatacggatgaaaataagggcctaggtgcagggagagtggtatctgagatttaagactttgattttaatgaccagggcttgggaagaagaggatggaggagggacttgtgagcaactaacaaaagaggaatgtaaattaggcagaaatcaatgaatgtaggaagtgttgggtttacatgatgaccactgtggggagctccagcccattcctcccttaggagcacaggttccggagctcggcagaggagttcaaattttcaatctcttcactagttatggaacaagccacttaaattgtgttggaggattagccgcttaatctttccgtcaaatggaagtcatgaaatggggataattacagttgcgagaattaaatgagctattacatatcacgtgtttttgcgtcatcagcccagaggttgtgtagttacaccaggcaacagtaccaagaccgtgagtgcagctgagcaatggtgctcagggcttgaggcttagtatgacaagataaactgttagcaggtgttgactcttcctttaggacaatgtgctctttggggattgtctttttctccagcactgccacgcgacccatatagtaaaaacaaggtgaaggtgcctccaattgtcttttccaggaagaaccaattgacacgaagtccaggaccaggagccctggcctccctcggactttgaatgaaatctgctccttctctgaggtgtgcatctcctcccttgtctcttctcgcagtagagtggtgggatgctgggattgtggtgaggatctgggcaacaaagccaggggcacacatcagcccgcttcagacctggccttggggcttgggagggctcatggctcactcgtggtccaagaccgccatgggcgcacaggcctggagcgcagtaggctatgaagacagtgcgatgacaccaaagggaccgcccactctagcgggagacgggaggagagaagaaactcctccactctctgtttccattcctggaacatgtctctggacacacaatctctcagcttttgctgggctgtctccacacatattgctttgggataagaatacgggctgccgggcaccaccaccaagggctggacaagcatcaggaagtttcctcgaagtatctacttgcagtggtgcccttgtgcgggtcctgggcctcctcattatcattttattgcatttctcttctttgcaccctgaggactttttcgaggaagattgttctttccaagtccacttgtctcatcttctccctgagctacagacctcacagcagaattcagtcatctaggactccttggctcccaagagcaatgccagtattaaactacacgatgacaggggctttcattcatcactcttttctctgcagtaatcatgggatcaggatgccagaggcttcaagcgttcactaccttgaatgtaatagtcacaggtagaatggaagtcagcctcaagtacagccagctcttttgtgcctgagccatcaccaagctctaagttttgtagccaactctaaaggcaacctgtgttcctttgtgaagcaggccccgctctcctgatagctcccatatgatacaccctgattagcaaggcagcatcaggcagaacaaaagctccattaaccagggctggtgggcgggaaggcaaaaccaggggccctgttggctctctgatgggaaatgctggccatgtagctcttgggttttctcagcactgctggattcagattgctcctcttccactgaatccccagggtgcgtgcacagcccagctggaaacgggacaccagagggctccgagtgaacacaagagccaagggcaaatccacatgatgcccaacaggcaggccttgcactggctttctccatcttccttttagagtggatgcttgatgctcattctttaaaaggacctctcttcttggagaatacctttcttttttctttcctttttctttcaggatctactttgtgctacaggccaacagcccggataagcatctgggtccccagcaagcgctctgtgctttttttaaaaacacgcacacatgttctgcctcttatttcctgagcagtcccaacacctggagtggtcacagtccaaaaaagtcaggccaggaaattgagttcttcttgactcctggctgggacatttagccagggacattatgaatgtgttttgtaactaaccctctacaagagaagaccaggtccctgccaaggaattcacgagaccctggagttcgcaaagagggaaaagaagagaaacctc

SEQ ID NO: 12810 - RNA, 1782 nt, Homo sapiens
  source 1..1782: mol_type = other RNA
gcggaaggcggagcggcggagggcagggcggcgaaggtcaggaggccaggccccccagcccgcgcaggtgagccttgctgtctacctcttcctcctccatctcgaaggctgagtggtcttggctgtcgaaacaggaggcgctgaggaagacagggggagccggcggggactggggtggggtccccggagagggcggctcttccttaatgtttgcgaggggcagcgggagcccttcttcctcctgctcggccttcaggggcggcgggggcggtggcggcgacgtcggggcctgggcctgcagtgcctgcagcgcggcggccctctccagctctgcgcggtggcagcgctggtggcgcaggaggctgtaggcgcgcgagaagcggcgcgggcagcgggggcacgggtgcggggctgggccccccgcgtgcacctgtgcgtggcgcgccaggtcggccaggcgcttgaactcccgctggcagcgcacgcactggaaggggcgcgctcccgagtgggtcaccccgtgctgccgcaggtgcgcccggcgcctgaaacctttgccgcactctgggcaccagaagcggggctccccggcggggggccgagccggggcggcgtcgcctccgttctgcccttctcccccttccgaggcacccccgcactccgccccctcgcccccctccggccccttggctgagttccgtgcacccgaggccttgtcgtccttcttgcccgccgcgggcagcggggccagcaggctgagggggccgtggacgcggcggtgctggcggaggtaggaggcgaggcggaaggccaggccgcagtctgggcacacgaaagggcggtcggtggagtggaccagccggtggcgcgacagggaccagggcctggcgaaggccttgaggcagatggagcactggtgtcgcttggggcgtggcgggggccccccttccccttcctgttcgccctcggggcgcagacacgggtgcgccttgagctcgcccttggtggcgaaggcttcgcggcagcgcagacacagcagcgtccagtctgcctggagcaggacctgtttctcctcctgccgcccggccgccagcgccagctcggccctcagctctgctgccccggcctcggcctcctccgactccgactcccggggctccgcggcgctggtgggcgcagccagcgtggaaggctcccccgcaggccacgtctcaggccacgctgcgaccgcctcctcctccgtggcccctgctgcagcggtggtgggcggctccgagccctcgtcctgcgggccccagctgggttcggccgtctccttggccaccctctcgatggccagctcgacctcgccgcccgcgtgctcctgagccaggtggcgcctgagctgggccggttctgggaaggtgcgggggcaggcggcgcagcgcagcgggggctggggcccgtggccgcgcaggtggcgggaaaggtgggccggccggcggaaggccttggggcacagcgggcaggcgtggggccggagccccgagtggctcagccggtgccgggagaggtagtaggggaaacggaagaggcggccgcaggtggggcagggcaggggcgccctaggggctccagcgccccccctgccacggccacggccccgaccacggcctcggccacggccccggcctcggccacggtgaggtgggctgccctgggcgggtggaggaggctgcggatccatgcctcgcctccttggctcctttcttccttccccacggccggccaaacgcggacggt

SEQ ID NO: 12811 - RNA, 4432 nt, Homo sapiens
  source 1..4432: mol_type = other RNA
gcggagagagaatggggagctgactctgtgggtcatcatccccaccaatgcccaacatcctaggacaggccttagctgcagactagggtttctgacatgcctcctccttcctggcatctgacaacagatgcccctgcactacagaaatagcatttataagactaaaaagctctacgcaaaagtgttactggaaaaattcatgccatgtaaaggattctgattttttacaacaaaatgcaaaaagaggcaactgtataaaaaaagcactggcgcagaatcaagcaaccttggaaaagccactccccttctctggacctgtttcttccatagtaaaatgaacagatttggccaggctagtggctttcaagcagtagaccagagctggcactgaagctgcccttgagaagtgagtaaaaggacaacccaactactaggacttggagtcttctattcctccttcaaccaagccaaccctgctcttttttctatttaatatttagggattctatgtaaggtttggtttgaagaaagaattcttctgttagagaaaagtctgaaaatccttggactaaatgtaatccctaaggccctcttcagcaatggcattctgtaactctgtgataatattccccatccctcccaaaagacccagagatcccaattccttggccatccatcatcctctctattgcttaagcagctctgaggtccgggtcctaagaagaaacctcaaagaagaatctatgcatagagtaaggccatctgcctgattgccatttcattgcacaagcaagcatcaaattaactctccccacagccttttcctctcatcatgatcacactggaagcagctactattggggaagaaaaggcatatgatgtgcctcctctttcctggcatctgacaagaagctcagtgagaacatcagttgggttgggctctgggttcagtgccaacaggccctggcagctgcctggctgcagtggaataacagcagttacaacttaactagaggcagaggatggaaagacattaaattcagttgggagggaagagcaaatggaagctagacaaaagcggctcattaggacgctgcacgggcatgggctctctgggagatgctgctggtctcaccaggctgcccttgaacctgtaaaccttcctgactagctctatgtagaccctgttgatgagctctatgcctataagtctaatgaacagaagtaacacggcccacagagtgtatgagtgtgggtggagggggtgtgggcagggggtagaatctgggagagaaaagttacccttcaaaaaacttttacctgtttttggtaatttccctttcctctccattcttactacctctacccctattcataccctcaccgtcagcttcactgtcctaaactgtgactttaattatggcactttcctgttgaagaacctaaaatacctctcattttttttccccaaggtaaaatccaccttcctcagttttgaaatttaaaaaatgcttctatttcactaagtatgcttactatacgtcagtccatgtgctaagtgctttatatacattctacattttaatcctcataataaccccaatgaggttggtataatcttaattttccaggcttgaaagctgaggttcagtgaagttaaataatttgagcaaggttcaatagccagaacaaactgtaatctgtcttcaatctacccatccaacatcaactccctttattttcttcttcagattcatctgctctaatccaatgagatactctctgtttagggtagagtattagtcttcaaatcagctatatggccataagcaagctacttaatccttctgggcctcaaatgaggataacaccagccacacaggttgttgtaggctaacaggcaatatatttacagatatttggtaccatgtagacactttaaaaaaatactaatatagctccaaatccactgacctctgcccttcagctcccagaatgtccttttccttaaatgtttcctatgcctctcacctgttggaattggaccagatcttcaagatccaaattaaattcttagcctctgggaagccagccaaccctgcaatcctagactccagtgaccctggcctctacttagaaccacactaatctgcagctttcatatgacaaggaatacgcttcttcattctatgacttgccatgtcatatcaccccaaccagactagcttctcactcttctttacatccctcagcattaggccttgctcacagcaggcatttaataaatttcagttgactgattgataccacaaatacagattccagcctctcaggaaataaaacatttaggctgaatactgacctaagtcaagtgggtagatggggccagtgaagccatttgttttgcttactctatggccaaagggaggctgggagttttcccaggctggcgcactgcctctgtttatataactattctgtagcttctttgtgccaatgagtgagggtctgagtcacaatgtgcccctggctcctctacacctctagccaaccaggcagattcggaagaggttctccagagtcttgactatctatatacctgtaggggaaacagccagaaaccgagccttcagcgaagaagcaatatctggcaaggttgggtaaatgagatttgaatatttcatcctgttccaagaagaatcccaataagtacaggaagcacattattttgctcacagtggggacaaagcaggctttccatggcttctgatgagttctgtggccacgctggactcccctggccatttctgggttatataaatgtttgatgaaaaatctctcaggggaaatcaaatttttgtaagaagttaatgacagcccatccagatgtatgatgacttgagttgatagctcattaaccctttcccagctgatatcttcacccagagactccacaaggcatcaataaggtcagataggtcatggatgtagtacttgaagacagatgcattggttgcctccaaagccagcaagtactcattccgggctttgatggccttcagcttattctccgtgtacttggcttggcgcttctccttcatcttctcaatcttcttcactgagctcctccggacatgtttctcctcaatgcgaacgttggccgtggagtcaggggagcgtggggtctgccggtcctcctgctttaccgatttaccaatttgcttctcctcctgcttctccgcctcctttagtttgctctgagcactgatgctgtcggcattgtacatgtgatatgtcttcatgaccgagtagagctcgttcaggaccttcatcaaatcatcttggagctgctggccgacttctttactctttttaaagagtcttcctgagtcctcgctgacttgtacaaatcgaggaatgatattattcaggtagatgtcactcagggtggtatggtccctgctttcccgcttcacctggtttaagaggagattccagcagttgactggagagagaacattctgatccttcttgaattgctggtccttggtgctgcatgtcttggccaggaagcgttctgccagcttctccaggttgcgggagtagtccatctcaatctctgccttctttcggaagaagtcctggaggtcctgcaacagttgcacccgaagctcacactgctggtccaggcatttcatctgctctgtgagctgagcacggatctctttgacctgagtatcgtactctgctatgatctccttatcctttttgaatttggctggagacgtcatgttttccttctttcttccaaattcgaattgtgaattgatagatccacggaaaaaatccaaccacctaaatcaatacctccaagaccgcttctctcgagggcagaaggggccccccacggtggtctccagcgctccgtggagcgcgggctgcgggctgggcagacggctacggcgggcacatgcagacggtgggcgctgaggccgggtgcggcggcggctggtgcctgtgctagagccggagccgcagcctcagcattagccgggagaactgcagcgcccggaggctggcctggggtctgacatcaacgacacaggcggggagtggaagtccttccgcacaacatggtgtggggctgcgggggtgtggacgcgcccagctgtgtccccgggagggagtgggtgcttttcggggtgccgggggagggctgggcgtgcttcgcggttttttgtcgtagaggctcaaagatgctgcaaatcaaatcccaaacgggagccgcaacagcgcagactggatcggaagtcgtttgctccggttcacttgcctggctctgacgcgacgggtcccaggcccccggctccgcttcccactcagagctctcctcccctctcttccccgccacccgtttctacgcagatctgtg

SEQ ID NO: 12812 - RNA, 173 nt, Homo sapiens
  source 1..173: mol_type = other RNA
gcggggctgggcgcgcgcgtacgagtggtaggcggtcagcaccacgccgcccgagtcctccacctccatcgtcagccgcgcatgtctcggcgccggccccagaacaaagaccgggaccagcatggaccggcgcgccgggaggctgtcagcagctgggcggcgcggcccgaggt

SEQ ID NO: 12813 - RNA, 175 nt, Homo sapiens
  source 1..175: mol_type = other RNA
gcggggctgggcgcgcgcgtacgagtggtaggcggtcagcaccacgccgcccgagtcctccacctccatcgtcagccgcgcatgtctcggcgccggccccagaacaaagaccgggaccagcatggaccggcgcgccgggaggctgtcagcagctgggcggcgcggcccgaggtgc

SEQ ID NO: 12814 - RNA, 903 nt, Homo sapiens
  source 1..903: mol_type = other RNA
gcggggctgggcgcgcgctcgtgtgtctgcgccagctccagccgccggctggtctcccggagcgtgtgctcgacgcgcgggttgcgcacgggcgcgcgcggcgacagcggctgcatcaggagccccgagggcgcgccctgggagagtatgcccggtgctccaccgtcgtcactggccagggactcgctggatgtccaggcgcctgggctacgtgcgcccgcgaggccgggccggggcgcgcggggacggcgcgaggtcgggggtcccggggcgcggcgggcagcggggccacgctccagctcctctatgtacttgaggaagtccaggtccaggtggaagccgtagggcgtctccaccgagtagggcgagctcgggctgcgtgcgcccccggcggcggggaccgggcacaggcgggggccgcccaggtcgggcaggttctgattcagggcaaacttggccatgtttcctgcagcagctgtcagaggcacccaaggtcagttgtgaaactcttgcaggaatgatggggaattgcgggctggatgcaccaaagatccaaatcaacaaatcaacggatacttgtctccctggaatgtcgctagcggagtgtcacaggcttgatccttggcttgtaagagtttgtaatgcaaacacaaaacacctgggttgtcagagctgtgactattcatggggctgcctgggaaagtgactgtttggatgacatgatggaggctgtaagaaagtgaggaagattgggccacatataataatgtgatatttaacaaggacaaatattgaatccagaactttggttcaaaaagcacagggtgaaatctcagcactctgggaagccaaagcagaaggatcgcttgagcctaggagtcaagacccacctgcgcaacatag

SEQ ID NO: 12815 - RNA, 527 nt, Homo sapiens
  source 1..527: mol_type = other RNA
gcggggctgggcgcgcgctcgtgtgtctgcgccagctccagccgccggctggtctcccggagcgtgtgctcgacgcgcgggttgcgcacgggcgcgcgcggcgacagcggctgcatcaggagccccgagggcgcgccctgggagagtatgcccggtgctccaccgtcgtcactggccagggactcgctggatgtccaggcgcctgggctacgtgcgcccgcgaggccgggccggggcgcgcggggacggcgcgaggtcgggggtcccggggcgcggcgggcagcggggccacgctccagctcctctatgtacttgaggaagtccaggtccaggtggaagccgtagggcgtctccaccgagtagggcgagctcgggctgcgtgcgcccccggcggcggggaccgggcacaggcgggggccgcccaggtcgggcaggttctgattcagggcaaacttggccatgtttcctgcagcagctgtcagaggcaccctgaagccgcagccccagccgcgcccgcacccgagccc

SEQ ID NO: 12816 - RNA, 664 nt, Homo sapiens
  source 1..664: mol_type = other RNA
gcggggctgggcgcgcgctcgtgtgtctgcgccagctccagccgccggctggtctcccggagcgtgtgctcgacgcgcgggttgcgcacgggcgcgcgcggcgacagcggctgcatcaggagccccgagggcgcgccctgggagagtatgcccggtgctccaccgtcgtcactggccagggactcgctggatgtccaggcgcctgggctacgtgcgcccgcgaggccgggccggggcgcgcggggacggcgcgaggtcgggggtcccggggcgcggcgggcagcggggccacgctccagctcctctatgtacttgaggaagtccaggtccaggtggaagccgtagggcgtctccaccgagtagggcgagctcgggctgcgtgcgcccccggcggcggggaccgggcacaggcgggggccgcccaggtcgggcaggttctgattcagggcaaacttggccatgtttcctgcagcagctgtcagaggcaccctgcaaaaggggtgaaggtggggctgggcgctgtccctctggctggagcctctggggcctgcctttgagtctaagcaaacaggacccaagagctctcctccacccagccacctccctccacacatggcctctccttcctcttccctaaagaaaccttgaaacttttttttttttt

SEQ ID NO: 12817 - RNA, 672 nt, Homo sapiens
  source 1..672: mol_type = other RNA
gcggggctgggcgcgcgctcgtgtgtctgcgccagctccagccgccggctggtctcccggagcgtgtgctcgacgcgcgggttgcgcacgggcgcgcgcggcgacagcggctgcatcaggagccccgagggcgcgccctgggagagtatgcccggtgctccaccgtcgtcactggccagggactcgctggatgtccaggcgcctgggctacgtgcgcccgcgaggccgggccggggcgcgcggggacggcgcgaggtcgggggtcccggggcgcggcgggcagcggggccacgctccagctcctctatgtacttgaggaagtccaggtccaggtggaagccgtagggcgtctccaccgagtagggcgagctcgggctgcgtgcgcccccggcggcggggaccgggcacaggcgggggccgcccaggtcgggcaggttctgattcagggcaaacttggccatgtttcctgcagcagctgtcagaggcaccctgcaaaaggggtgaaggtggggctgggcgctgtccctctggctggagcctctggggcctgcctttgagtctaagcaaacaggacccaagagctctcctccacccagccacctccctccacacatggcctctccttcctcttccctaaagaaaccttgaaacttttttttttttttttttttt

SEQ ID NO: 12818 - RNA, 647 nt, Homo sapiens
  source 1..647: mol_type = other RNA
gcggggctgggcgcgcgctcgtgtgtctgcgccagctccagccgccggctggtctcccggagcgtgtgctcgacgcgcgggttgcgcacgggcgcgcgcggcgacagcggctgcatcaggagccccgagggcgcgccctgggagagtatgcccggtgctccaccgtcgtcactggccagggactcgctggatgtccaggcgcctgggctacgtgcgcccgcgaggccgggccggggcgcgcggggacggcgcgaggtcgggggtcccggggcgcggcgggcagcggggccacgctccagctcctctatgtacttgaggaagtccaggtccaggtggaagccgtagggcgtctccaccgagtagggcgagctcgggctgcgtgcgcccccggcggcggggaccgggcacaggcgggggccgcccaggtcgggcaggttctgattcagggcaaacttggccatgtttcctgcagcagctgtcagaggcaccctgggacttccaatgtgggaggggtcccggccagaggacacgacgcccgccccgtcgcagcgggcagagccctcagtggggctggaaacgcagcgcagcgccgggtcccggtgcgtccccgaatccacccacccaggggtcccccatccgtgtccccg

SEQ ID NO: 12819 - RNA, 648 nt, Homo sapiens
  source 1..648: mol_type = other RNA
gcggggctgggcgcgcggggtcgggggctctccgcggctgagtgcccaggactagtgggtgccacagggcgaggagaggaggtcctcgggggtcgcgatgccggggtctctgtctccgtggtccgggtctctcctagcttggtcagcagtcggacccgttagtcgccggccagtgcccgactcctcccaccgcgcgggccccgccggaccctggaggggactggtctgcagagacgctggggctcgcgggccggcaccggctccgggagggctaagatgctgcctttgctttcccctatgcttgttagatttccacaggtcggacgcctgtgaggttaagaaggaggtgacccctgtggaaatcaccgcccccttctcccaacacccccagactcagcgacttctagcttcccatttcctgggggaagctaggcccagggtaaggagacgcagagcgtccctcccagatagaagtgtctggcagaggtccagctgatgtcaacagagagaaagcagaacctgaagctgggagaggttgagagtagaacaccgaatttgaattccccccaccatcatcaccctccttcctcttggagcttggacccagaaacagccccattaacctccttgctcgtgtaggtttgttct

SEQ ID NO: 12820 - RNA, 302 nt, Homo sapiens
  source 1..302: mol_type = other RNA
gcggggctgggcgcgcggggtcgggggctctccgcggctgagtgcccaggactagtgggtgccacagggcgaggagaggaggtcctcgggggtcgcgatgccggggtctctgtctccgtggtccgggtctctcctagcttggtcagcagtcggacccgttagtcgccggccagtgcccgactcctcccaccgcgcgggccccgccggaccctggaggggactggtctgcagagacgctggggctcgcgggccggcaccggctccgggagggctgcgtgcgcagagctgacactgacaacacc

SEQ ID NO: 12821 - RNA, 894 nt, Homo sapiens
  source 1..894: mol_type = other RNA
gcggggctgggcgcgcggggtcgggggctctccgcggctgagtgcccaggactagtgggtgccacagggcgaggagaggaggtcctcgggggtcgcgatgccggggtctctgtctccgtggtccgggtctctcctagcttggtcagcagtcggacccgttagtcgccggccagtgcccgactcctcccaccgcgcgggccccgccggaccctggaggggactggtctgcagagacgctggggctcgcgggccggcaccggctccgggagggctgcgtgcgcagagctgacactgacaacaccgccggcgccccgcccccacccgcccttaaaggagccgcacccgcgccgggcggggccaggacagcctggcgctccctcgctggaggagggcgggagggctagcagcgagcggaggaggttccggggttgaaaataggcgggatctttgatcacctcgccccatcttgcaatcgcggtgctcccacactcagctcaaggcaagagtaacttcacttacctaagatgctgcctttgctttcccctatgcttgttagatttccacaggtcggacgcctgtgaggttaagaaggaggtgacccctgtggaaatcaccgcccccttctcccaacacccccagactcagcgacttctagcttcccatttcctgggggaagctaggcccagggtaaggagacgcagagcgtccctcccagatagaagtgtctggcagaggtccagctgatgtcaacagagagaaagcagaacctgaagctgggagaggttgagagtagaacaccgaatttgaattccccccaccatcatcaccctccttcctcttggagcttggacccagaaacagccccattaacctccttgctcgtgtaggtttgtt

SEQ ID NO: 12822 - RNA, 1793 nt, Homo sapiens
  source 1..1793: mol_type = other RNA
gctatttcacgacaccagggttcaaatcccagcccaacctctttctggctgggtgatcttgtacaagtcctgaacctctctgcacctcagtttcctcattcgtaccacaggggaccggcaccagcacacagcattaccccaggattggacgaattgtcacatctgcaagtctccactggtgttattacgttatcaggcacaaaccccctccagacacctgagcctcccccacaggctcccagtgaggagccatcacatgcccaggccagccgaggggccctcaggcatggggatctgggcaatggcagcaagctgggcggggggtgcagccaggatgacagcagatctgcagggcggggtcctcgccccgggccacctggctggggccgaaggtcacagctgcgtctaactgggccttgagcagctgaagctgtttcagggcttgcagcacctctggggtggccccggccacaccccccagcaggttgtagttctcaccagggtccttggacaggtcatagagcagcgggggctcatgagcagtcagagagctggaggcgtggcaggcagggtctgcagtggtatcactgtgggcagagccctgggtgaagaagtgagccttgtactttccagtccgcacagcaaaaaccccacggacctcgtctgggtaggacgggtagaagaagagagactgccgagggctcttgcctgtgcccagcagcagggggctgaggtcaaagccatccaaggtgacattgggcagtggggccccagccagggctgccagggtaggcagcaggtccagggagctggccagctcgtgggtcacgccgggagcgatatgacctggccagaaggccaaggcaggctctcggacaccgccctcgtaggtcgttccctttccacaccgcaagagaccggagcagccgcctcgggacatacgcatggtctcaggtccattgtctgcagtgaagatgaccagcgtctcttcaagcagccccaggtcccctatggctgtcatcagggtccccacagctgcatccagctccatcagggagtccccaaatggcccgcggcctgaacgctctgcaaagctctgcccactgaactgagggtagtgggtgtggtgagaggcatagtacaggaagaaggggcgatcctggcgctgggcgtcggccatgaggtcatgggcgaaagccatgtagcgggcctctagtccgggcagccaggggggctgcgcctccacggacaggttggccaacagtgggatggggaccaggccctggtcacagccaccgtcgcaaggagtggccggcgggaagcaggtcaggttctggcaggggccctggtcgtgggagtacgggatgcctagaaatcgatggaagccctgatgggggggcaggaaggccccctcaggccccaccccaaggtgccacttgccggccattcctgtgaggtagcctcgggcagccaggacttcggccacggtcacctcctccaggggcaggcccccccgggagctgggcaccaggacgccagggtacatgcccatccgaaccgggagccggccggtcaggagggcggcccgggagaccgcgggctgggacggaactcctccaggaccagggcaccttcagattctcgagcggagatctgatcctcctcgcctagcggtccgggctcagggtcgggggcgtaagtcacttggcgctgaccagcggagtcgggccggggggaaggcgctagagggagcccaggaggagccggtaccgggctgcgggcgcttccgcctc

SEQ ID NO: 12823 - RNA, 2078 nt, Homo sapiens
  source 1..2078: mol_type = other RNA
gctatttcacgacaccagggttcaaatcccagcccaacctctttctggctgggtgatcttgtacaagtcctgaacctctctgcacctcagtttcctcattcgtaccacaggggaccggcaccagcacacagcattaccccaggattggacgaattgtcacatctgcaagtctccactggtgttattacgttatcaggcacaaaccccctccagacacctgagcctcccccacaggctcccagtgaggagccatcacatgcccaggccagccgaggggccctcaggcatggggatctgggcaatggcagcaagctgggcggggggtgcagccaggatgacagcagatctgcagggcggggtcctcgccccgggccacctggctggggccgaaggtcacagctgcgtctaactgggccttgagcagctgaagctgtttcagggcttgcagcacctctggggtggccccggccacaccccccagcaggttgtagttctcaccagggtccttggacaggtcatagagcagcgggggctcatgagcagtcagagagctggaggcgtggcaggcagggtctgcagtggtatcactgtgggcagagccctgggtgaagaagtgagccttgtactttccagtccgcacagcaaaaaccccacggacctcgtctgggtaggacgggtagaagaagagagactgccgagggctcttgcctgtgcccagcagcagggggctgaggtcaaagccatccaaggtgacattgggcagtggggccccagccagggctgccagggtaggcagcaggtccagggagctggccagctcgtgggtcacgccgggagcgatatgacctggccagaaggccaaggcaggctctcggacaccgccctcgtaggtcgttccctttccacaccgcaagagaccggagcagccgcctcgggacatacgcatggtctcaggtccattgtctgcagtgaagatgaccagcgtctcttcaagcagccccaggtcccctatggctgtcatcagggtccccacagctgcatccagctccatcagggagtccccaaatggcccgcggcctgaacgctctgcaaagctctgcccactgaactgagggtagtgggtgtggtgagaggcatagtacaggaagaaggggcgatcctggcgctgggcgtcggccatgaggtcatgggcgaaagccatgtagcgggcctctagtccgggcagccaggggggctgcgcctccacggacaggttggccaacagtgggatggggaccaggccctggtcacagccaccgtcgcaaggagtggccggcgggaagcaggtcaggttctggcaggggccctggtcgtgggagtacgggatgcctagaaatcgatggaagccctgatgggggggcaggaaggccccctcaggccccaccccaaggtgccacttgccggccattcctgtgaggtagcctcgggcagccaggacttcggccacggtcacctcctccaggggcaggcccccccgggagctgggcaccaggacgccagggtacatgcccatccgaaccgggagccggccggtcaggagggcggccctagagggtgtgcacagagacacaggcacgtagaagtctgtgaaccgcagccctcccgccgccagctggtccaggttgggagtggtagagctggggtgcccatagcagcccaggtccccatagccgaggtcgtcggcaaagatcagcacgatgttgggcggacgggcaacggccaggccagcagccagggccaggaggagggaccgcggtgcccccatggacatgggaccgaggggtcctgacggccgcctcctgaagctccagagggccggggcccgacagtaccgggagaccgcgggctgggacggaactcctccaggaccagggcaccttcagattctcgagcggagatctgatcctcctcgcctagcggtccgggctcagggtcgggggcgtaagtcacttggcgctgaccagcggagtcgggccggggggaaggcgctagagggagcccaggaggagccggtaccgggctgcgggcgcttccgcctc

SEQ ID NO: 12824 - RNA, 2030 nt, Homo sapiens
  source 1..2030: mol_type = other RNA
gctatttcacgacaccagggttcaaatcccagcccaacctctttctggctgggtgatcttgtacaagtcctgaacctctctgcacctcagtttcctcattcgtaccacaggggaccggcaccagcacacagcattaccccaggattggacgaattgtcacatctgcaagtctccactggtgttattacgttatcaggcacaaaccccctccagacacctgagcctcccccacaggctcccagtgaggagccatcacatgcccaggccagccgaggggccctcaggcatggggatctgggcaatggcagcaagctgggcggggggtgcagccaggatgacagcagatctgcagggcggggtcctcgccccgggccacctggctggggccgaaggtcacagctgcgtctaactgggccttgagcagctgaagctgtttcagggcttgcagcacctctggggtggccccggccacaccccccagcaggttgtagttctcaccagggtccttggacaggtcatagagcagcgggggctcatgagcagtcagagagctggaggcgtggcaggcagggtctgcagtggtatcactgtgggcagagccctgggtgaagaagtgagccttgtactttccagtccgcacagcaaaaaccccacggacctcgtctgggtaggacgggtagaagaagagagactgccgagggctcttgcctgtgcccagcagcagggggctgaggtcaaagccatccaaggtgacattgggcagtggggccccagccagggctgccagggtaggcagcaggtccagggagctggccagctcgtgggtcacgccgggagcgatatgacctggccagaaggccaaggcaggctctcggacaccgccctcgtaggtcgttccctttccacaccgcaagagaccggagcagccgcctcgggacatacgcatggtctcaggtccattgtctgcagtgaagatgaccagcgtctcttcaagcagccccaggtcccctatggctgtcatcagggtccccacagctgcatccagctccatcagggagtccccaaatggcccgcggcctgaacgctctgcaaagctctgcccactgaactgagggtagtgggtgtggtgagaggcatagtacaggaagaaggggcgatcctggcgctgggcgtcggccatgaggtcatgggcgaaagccatgtagcgggcctctagtccgggcagccaggggggctgcgcctccacggacaggttggccaacagtgggatggggaccaggccctggtcacagccaccgtcgcaaggagtggccggcgggaagcaggtcaggttctggcaggggccctggtcgtgggagtacgggatgcctagaaatcgatggaagccctgatgggggggcaggaaggccccctcaggccccaccccaaggtgccacttgccggccattcctgtgaggtagcctcgggcagccaggacttcggccacggtcacctcctccaggggcaggcccccccgggagctgggcaccaggacgccagggtacatgcccatccgaaccgggagccggccggtcaggagggcggccctagagggtgtgcacagagacacaggcacgtagaagtctgtgaaccgcagccctcccgccgccagctggtccaggttgggagtggtagagctggggtgcccatagcagcccaggtccccatagccgaggtcgtcggcaaagatcagcacgatgttgggcggacgggcaacggccaggccagcagccagggccaggaggagggaccgcggtgcccccatggacatgggaccgaggggtcgggagaccgcgggctgggacggaactcctccaggaccagggcaccttcagattctcgagcggagatctgatcctcctcgcctagcggtccgggctcagggtcgggggcgtaagtcacttggcgctgaccagcggagtcgggccggggggaaggcgctagagggagcccaggaggagccggtaccgggctgcgggcgcttccgcctc

SEQ ID NO: 12825 - RNA, 2183 nt, Homo sapiens
  source 1..2183: mol_type = other RNA
gctatttcacgacaccagggttcaaatcccagcccaacctctttctggctgggtgatcttgtacaagtcctgaacctctctgcacctcagtttcctcattcgtaccacaggggaccggcaccagcacacagcattaccccaggattggacgaattgtcacatctgcaagtctccactggtgttattacgttatcaggcacaaaccccctccagacacctgagcctcccccacaggctcccagtgaggagccatcacatgcccaggccagccgaggggccctcaggcatggggatctgggcaatggcagcaagctgggcggggggtgcagccaggatgacagcagatctgcagggcggggtcctcgccccgggccacctggctggggccgaaggtcacagctgcgtctaactgggccttgagcagctgaagctgtttcagggcttgcagcacctctggggtggccccggccacaccccccagcaggttgtagttctcaccagggtccttggacaggtcatagagcagcgggggctcatgagcagtcagagagctggaggcgtggcaggcagggtctgcagtggtatcactgtgggcagagccctgggtgaagaagtgagccttgtactttccagtccgcacagcaaaaaccccacggacctcgtctgggtaggacgggtagaagaagagagactgccgagggctcttgcctgtgcccagcagcagggggctgaggtcaaagccatccaaggtgacattgggcagtggggccccagccagggctgccagggtaggcagcaggtccagggagctggccagctcgtgggtcacgccgggagcgatatgacctggccagaaggccaaggcaggctctcggacaccgccctcgtaggtcgttccctttccacaccgcaagagaccggagcagccgcctcgggacatacgcatggtctcaggtccattgtctgcagtgaagatgaccagcgtctcttcaagcagccccaggtcccctatggctgtcatcagggtccccacagctgcatccagctccatcagggagtccccaaatggcccgcggcctgaacgctctgcaaagctctgcccactgaactgagggtagtgggtgtggtgagaggcatagtacaggaagaaggggcgatcctggcgctgggcgtcggccatgaggtcatgggcgaaagccatgtagcgggcctctagtccgggcagccaggggggctgcgcctccacggacaggttggccaacagtgggatggggaccaggccctggtcacagccaccgtcgcaaggagtggccggcgggaagcaggtcaggttctggcaggggccctggtcgtgggagtacgggatgcctagaaatcgatggaagccctgatgggggggcaggaaggccccctcaggccccaccccaaggtgccacttgccggccattcctgtgaggtagcctcgggcagccaggacttcggccacggtcacctcctccaggggcaggcccccccgggagctgggcaccaggacgccagggtacatgcccatccgaaccgggagccggccggtcaggagggcggccctagagggtgtgcacagagacacaggcacgtagaagtctgtgaaccgcagccctcccgccgccagctggtccaggttgggagtggtagagctggggtgcccatagcagcccaggtccccatagccgaggtcgtcggcaaagatcagcacgatgttgggcggacgggcaacggccaggccagcagccagggccaggaggagggaccgcggtgcccccatggacatgggaccgaggggtctgtcccaagagagggagggctacttggctccagcaggctctttccgataccgcagacccaggcgccgcccttccctgagaccccggacccaaatactccccgaccctgacggccgcctcctgaagctccagagggccggggcccgacagtaccgggagaccgcgggctgggacggaactcctccaggaccagggcaccttcagattctcgagcggagatctgatcctcctcgcctagcggtccgggctcagggtcgggggcgtaagtcacttggcgctgaccagcggagtcgggccggggggaaggcgctagagggagcccaggaggagccggtaccgggctgcgggcgcttccgcctc

SEQ ID NO: 12826 - RNA, 1985 nt, Homo sapiens
  source 1..1985: mol_type = other RNA
gctatttcacgacaccagggttcaaatcccagcccaacctctttctggctgggtgatcttgtacaagtcctgaacctctctgcacctcagtttcctcattcgtaccacaggggaccggcaccagcacacagcattaccccaggattggacgaattgtcacatctgcaagtctccactggtgttattacgttatcaggcacaaaccccctccagacacctgagcctcccccacaggctcccagtgaggagccatcacatgcccaggccagccgaggggccctcaggcatggggatctgggcaatggcagcaagctgggcggggggtgcagccaggatgacagcagatctgcagggcggggtcctcgccccgggccacctggctggggccgaaggtcacagctgcgtctaactgggccttgagcagctgaagctgtttcagggcttgcagcacctctggggtggccccggccacaccccccagcaggttgtagttctcaccagggtccttggacaggtcatagagcagcgggggctcatgagcagtcagagagctggaggcgtggcaggcagggtctgcagtggtatcactgtgggcagagccctgggtgaagaagtgagccttgtactttccagtccgcacagcaaaaaccccacggacctcgtctgggtaggacgggtagaagaagagagactgccgagggctcttgcctgtgcccagcagcagggggctgaggtcaaagccatccaaggtgacattgggcagtggggccccagccagggctgccagggtaggcagcaggtccagggagctggccagctcgtgggtcacgccgggagcgatatgacctggccagaaggccaaggcaggctctcggacaccgccctcgtaggtcgttccctttccacaccgcaagagaccggagcagccgcctcgggacatacgcatggtctcaggtccattgtctgcagtgaagatgaccagcgtctcttcaagcagccccaggtcccctatggctgtcatcagggtccccacagctgcatccagctccatcagggagtccccaaatggcccgcggcctgaacgctctgcaaagctctgcccactgaactgagggtagtgggtgtggtgagaggcatagtacaggaagaaggggcgatcctggcgctgggcgtcggccatgaggtcatgggcgaaagccatgtagcgggcctctagtccgggcagccaggggggctgcgcctccacggacaggttggccaacagtgggatggggaccaggccctggtcacagccaccgtcgcaaggagtggccggcgggaagcaggtcaggttctggcaggggccctggtcgtgggagtacgggatgcctagaaatcgatggaagccctgatgggggggcaggaaggccccctcaggccccaccccaaggtgccacttgccggccattcctgtgaggtagcctcgggcagccaggacttcggccacggtcacctcctccaggggcaggcccccccgggagctgggcaccaggacgccagggtacatgcccatccgaaccgggagccggccggtcaggagggcggccctagagggtgtgcacagagacacaggcacgtagaagtctgtgaaccgcagccctcccgccgccagctggtccaggttgggagtggtagagctggggtgcccatagcagcccaggtccccatagccgaggtcgtcggcaaagatcagcacgatgttgggcggacgggcaacggccaggccagcagccagggccaggaggagggaccgcggtgcccccatggacatgggaccgaggggtcttcagattctcgagcggagatctgatcctcctcgcctagcggtccgggctcagggtcgggggcgtaagtcacttggcgctgaccagcggagtcgggccggggggaaggcgctagagggagcccaggaggagccggtaccgggctgcgggcgcttccgcctc

SEQ ID NO: 12827 - RNA, 1748 nt, Homo sapiens
  source 1..1748: mol_type = other RNA
gctatttcacgacaccagggttcaaatcccagcccaacctctttctggctgggtgatcttgtacaagtcctgaacctctctgcacctcagtttcctcattcgtaccacaggggaccggcaccagcacacagcattaccccaggattggacgaattgtcacatctgcaagtctccactggtgttattacgttatcaggcacaaaccccctccagacacctgagcctcccccacaggctcccagtgaggagccatcacatgcccaggccagccgaggggccctcaggcatggggatctgggcaatggcagcaagctgggcggggggtgcagccaggatgacagcagatctgcagggcggggtcctcgccccgggccacctggctggggccgaaggtcacagctgcgtctaactgggccttgagcagctgaagctgtttcagggcttgcagcacctctggggtggccccggccacaccccccagcaggttgtagttctcaccagggtccttggacaggtcatagagcagcgggggctcatgagcagtcagagagctggaggcgtggcaggcagggtctgcagtggtatcactgtgggcagagccctgggtgaagaagtgagccttgtactttccagtccgcacagcaaaaaccccacggacctcgtctgggtaggacgggtagaagaagagagactgccgagggctcttgcctgtgcccagcagcagggggctgaggtcaaagccatccaaggtgacattgggcagtggggccccagccagggctgccagggtaggcagcaggtccagggagctggccagctcgtgggtcacgccgggagcgatatgacctggccagaaggccaaggcaggctctcggacaccgccctcgtaggtcgttccctttccacaccgcaagagaccggagcagccgcctcgggacatacgcatggtctcaggtccattgtctgcagtgaagatgaccagcgtctcttcaagcagccccaggtcccctatggctgtcatcagggtccccacagctgcatccagctccatcagggagtccccaaatggcccgcggcctgaacgctctgcaaagctctgcccactgaactgagggtagtgggtgtggtgagaggcatagtacaggaagaaggggcgatcctggcgctgggcgtcggccatgaggtcatgggcgaaagccatgtagcgggcctctagtccgggcagccaggggggctgcgcctccacggacaggttggccaacagtgggatggggaccaggccctggtcacagccaccgtcgcaaggagtggccggcgggaagcaggtcaggttctggcaggggccctggtcgtgggagtacgggatgcctagaaatcgatggaagccctgatgggggggcaggaaggccccctcaggccccaccccaaggtgccacttgccggccattcctgtgaggtagcctcgggcagccaggacttcggccacggtcacctcctccaggggcaggcccccccgggagctgggcaccaggacgccagggtacatgcccatccgaaccgggagccggccggtcaggagggcggcccttcagattctcgagcggagatctgatcctcctcgcctagcggtccgggctcagggtcgggggcgtaagtcacttggcgctgaccagcggagtcgggccggggggaaggcgctagagggagcccaggaggagccggtaccgggctgcgggcgcttccgcctc

SEQ ID NO: 12828 - RNA, 628 nt, Homo sapiens
  source 1..628: mol_type = other RNA
gctcagggatgataactgtgctgagaaaccacagagtcaatcagattcaaaatgttaaaatccttcctgcttggagttttccgtcttcacatcaaagcatttcatgcccgtcagcaactttttaatgcatttgctcctcgtttgcacaatttccatttaaagactttccttggctgacttctctgatgaggtttcctgcttgccaggagagcacgctaatgcagaaattacaaagggggcttcacgtcccttttccggaggacctgatatttcagataatttccagcttcagttttggagaaacgactgttctttgcaccaggggaaaataaactgattttcagtgtaagcaacctttctgcaagtagaatggggactgttgggaatggagatgaagacttcacttcatgttattcatttcctctgtgtgtagatgttcctttaactggagtgtaggttgagtataatccatagacttctttccaggagcttaccaggaacagggttcacggcttatgtggatgatctcattttgtcctcacagcatcctcctcacagagggtgggtgctattattagcaccattttaaagaggaggaatctgagtcccagaggccaagtagttgggc

SEQ ID NO: 12829 - RNA, 560 nt, Homo sapiens
  source 1..560: mol_type = other RNA
gctcagggatgataactgtgctgagaaaccacagagtcaatcagattcaaaatgttaaaatccttcctgcttggagttttccgtcttcacatcaaagcatttcatgcccgtcagcaactttttaatgcatttgctcctcgtttgcacaatttccatttaaagactttccttggctgacttctctgatgaggtttcctgcttgccaggagagcacgctaatgcagaaattacaaagggggcttcacgtcccttttccggaggacctgatatttcagataatttccagcttcagttttggagaaacgactgttctttgcaccaggggaaaataaactgattttcagtgtaagcaacctttctgcaagtagaatggggactgttgggaatggagatgaagacttcacttcatgttattcatttccttaccaggaacagggttcacggcttatgtggatgatctcattttgtcctcacagcatcctcctcacagagggtgggtgctattattagcaccattttaaagaggaggaatctgagtcccagaggccaagtagttgggc

SEQ ID NO: 12830 - RNA, 3841 nt, Homo sapiens
  source 1..3841: mol_type = other RNA
gctcggactgagcaggtggggaggggggaaaccgatcatcaccgctgcagcactctctgggagagcaagtggctacctgcgctctgaaagaagggagcaaagtaggtggatctgagaactattggaaggcagagtcaagtccctgggatttagagtgtgatgactgggctgagagacagggaggacccaggaagactgagaatctccctctgtccttaaacctgtgcactctggggacatctaaaaagtttctgactcagcgcctaggaccgtgggccccccatcttagaaactgaaaggaatgttcatctacctttaagcaaaggcttgtgtttttaagtgaaatcatctcagatccaggagagagggctgggaagacagtgtgcagaggacttgggtgaactcctgggtctctggtgtctttcccagtaatgtctgctgtgtctgcagagcaggagtttctgctgcttcttctgatcccaactccttgcgtccctcgagtcatttctattctgaatcccacctgtgcccttcaccccagggccgacactttcaaacgaggctccacttgtcagggcagatcccagctcattctctggcacagagctgtcctcatctggggcgctgatgggttgaaggccactccagtgacagtgtctgtgtgcccagccagccggtgagaaaacgtgcttgagcccatttcatacacgtaagcgtgtctgtcctcggccccacaagccgcgaatcgtccacaaggactgaaagcgattccacatggatagccgcgggttggatgcccttcaaagtggcgctcacacctcagggttctcaggtcccacagtctcatcccatcgccaatggccgtggtcaggaaaaggttataagcctgaggctgttgggttgtaaatgatgaacctttattttggcagatttgatggacaggccgtgagtgggcttccgctatcaccgctgcactgcagccggcgttgaggtcaaacacttccacggtcctgttccggccagctgcgagtacgatgtgggaataaaagtcgttgactgccgataaactggtcatgtctactgcacccgtcgtggagagcctgcaaatcagcttggacttgctcttctgtttatatctcttaatctcatctttgcaagtgtcaatgtgatacctcagtagctgaaattcagggccagaagataacaatataaaggcatctatataatagaactgtgcagactgtataggtttagaaaacatgtctttgcccagaagcagtgcgagctctgccccacgagccgaccacattcgcagggtcccgtcccgggccgcagagagcagccacctccggtcctggctccagcacacggcattcactgccccgtcgtgacctgaaaacacagcaggtgtcccagtcaggctggcatcaaaaacgagtaacagatggttggccaacccacaggccagccactgcccatctcctgagtactggatgcagcatacacgtgtgcaggtgggggcggcagcgacctgggggccgggcttggtgggcacagcgcactccacggggtatgcctcccgtgcgcagctgctcctgctccttgaagatcctttcccctcactcttgatgttggtctttggtgaaaacatagttacatgtggtgctgacgcataaccagatgacctaactttactatggaaaaccaggcgttggtccttcatgacgttccgtgcagcacgtcgctgttcactagcagccttggtactcttctccttggcaattcccagatacagtggagaggtcggtaggacacaggagctggctggcaccgagaggctctgccccatgctggggcactgctgagccctgactagcgcggccgggttgatctccaacacggcaatcttcccgccaaagagggaggccagcaagcacagcaccttttgatccgcagtgcggttcctcagggcacacgatccggccagcaggatgctgaggctctggaaatccttgtaatacaaagcagcttccacttccaggtttgccaggttaaatacgaataagcccactgagcttccgatccacacacatcgggtgttctcagaagaaagacatccacatgcagaatttgggatgagtgagagatcacagggtgcaagtctcagtacaggaaatgttacttcaacctgctctccttttcccagagcacttgtagagggaagctggctttcttctggctggctgcacagcccagacttaacccttcttgtggagaaagtctctgtcttcttccttaggtcaacccgtgccacacgacgataatggtgtccatccatcaaactgaagatccaaagctggccgtcagcacacccggtgaccagctgcctgctttctgcatcaatgaataaactgagaagaggatatgctgataacacagatgaactgtatattaatgatcctgtacaatggtcccagaccttaaagcctctgtcctcagacgccgagatgagggtgcctgctcgccagggacagaactccaccgcagtcaccgggcccaggtggccctgcagctcggcccgaacagcctgagtctgagagaatgtgtgcaggaaggtcggtggtgggactttgtggcggttattaacatcaggacgttctatgtatgtcacagaaaatcgctgctcaatatccagcatgaatattttgtttccagcacacacggcaacaacatgatcatccaggctcaactgtaaacacagcacctttcccaaaagcgagcccatgacagtccctcgagggaccagcccttgaagtactttctctctacattcatccaggttccacattataacataatccagtgatgctgagcagattagaagtgggttcactttatttccaaaagccatagcagtaattggctgatggtgtcctcgtaggattagaagctgatgagaaggatccttagtgttccatatacaaagttcagttccatccaaagggaaagcacagtcctgcatgctgcaagcaagctgaacatgagacacagactccttggattcaaccaggtatttttctataactatatcacttagacagccaccattacttgagaaaatgtcttggggattttccatcttcaatctatttattcacctctcctcatcccaagaaaaaagaagagaaattgccgaaaactctggagcttccacattctcaactgctccattcttctcacgggctttccagttaagcaaaccttgactcaaataccactattcccacttcacagagcctgcttaggcttcctcgatcagcttccacaactgagcccttttcctccgaactccacatgcgctcagttctcaaagcgccgatctcaagcggccgcccggatgctccggcccgacttgtgccccgaattcccctggagaccctcgcactagcacggcgtcaggaggaggcttcgggtgacgagacagcgggcaacggctctggtccagagcgcgcgtgtccgccgttggaagcggtcacggcggaaccctcaaatcgccccctttcctagagacctcagcggagccgcgagcaaccgcgcagcccccgcgctccagccctgcgccctaggcacacgccccagagcagcagctcgggttcggcgccgactccgcgccgagaccagcccgctaggggaggactcacagcacccagctcccaggagggcacgcagaggactaccgagccacactccgccccacgctcgccgctatggttacttgccagccgacccacgcgagccgctatggttactagcccgccgcccctcgcgcccacgccccttt

SEQ ID NO: 12831 - RNA, 6352 nt, Homo sapiens
  source 1..6352: mol_type = other RNA
gctcggactgagcaggtggggaggggggaaaccgatcatcaccgctgcagcactctctgggagagcaagtggctacctgcgctctgaaagaagggagcaaagtaggtggatctgagaactattggaaggcagagtcaagtccctgggatttagagtgtgatgactgggctgagagacagggaggacccaggaagactgagaatctccctctgtccttaaacctgtgcactctggggacatctaaaaagtttctgactcagcgcctaggaccgtgggccccccatcttagaaactgaaaggaatgttcatctacctttaagcaaaggcttgtgtttttaagtgaaatcatctcagatccaggagagagggctgggaagacagtgtgcagaggacttgggtgaactcctgggtctctggtgtctttcccagtaatgtctgctgtgtctgcagagcaggagtttctgctgcttcttctgatcccaactccttgcgtccctcgagtcatttctattctgaatcccacctgtgcccttcaccccagggcctgtgtggagaaacaagggtgtcaaaaatgaatgagacaggacaaggggcagcccctgtcttattttgcttctttggaacaagtgaagacaaacaacaaccaaaaaaaaaaaaaaaaaccatttccaggcgaattccctggattattttagcaaactccacagcttttgataaacttgggccgagcataaggaagcaaagagtcgtacatctttttcacatccttgctcctttcacagcaggctttcagcgggaggggaggaggcgaggccccagaggggtcccggagaaagcagaagaaagcggcgtcgacattttctgaaatgccaaaggtcccgtctccactttcaatctccgcagttacaaaacagagggctgagtcatcactcccatgaagtcaggggaggggagccattcagaaggcagttgtaatttttactttatcttttactaaatattgaggatggaaacccccagcctttcccacatgcattttctccagtggagagctagaagactgggccgtctctcttgccctgctttttgtcttctctgaggtcttttgaactttcccctaagtgggctcaaaagggatgattcagtctccaagaagcccagcaagtactttcagaaaagttagggaaacgttttcagccatttcagaaagtttagagtggttttagttatggaatcttaacacagttctaaatttgttatgtattcattatctgttcttaaacagatatattttccaaagtgaatgccacaattttctgtgaacatattaacgaatgtttcagaaaacaaaattaattagtggtctaaagtatttgggaaaccacgggttaaatcaaacagctttcttagctgctctgtgggggtgggacggtggcgggggggaggggggggttctactcctttgatagccgaatctgcaccacagagctctacaagggaggcacatttcccaaaggcagcagagcctgcagtgaagtgcctgctgtgcggggagggcccgccctcctattaagaggggcaggtggctggcgtcagggtgagggtgagcccttgccttcacagaagatgtccacgtggtggttctggactagcctcttcctttctctgagccgctcctcttcccgtgaaggaagtcttcgtcccacttctcaaggctgccttgagctcagaggaggatgcctggcttgtaaggtgctctcggcagccacggttgtcctcactggaaatggagcttgcaccacacagtgagtggggcagacacaggcgtcccagacaaaactcccaggcagaaagcagagagtaggaagcagcatcattggtcccaagaaatgatggatcttgccctcagcagcccctctcctgcagccagaggggagcgtccttcacccttgttttccagccccaggctcctctctcccgaggctcgtgttctctgtggccgcatcacacggcgctgggcggctttggctttgtcctgtccacaggcctgaggacccaggggcacttttacacttcacagtcacaagcagtctaggctttacttgctgacacaagcccttgacagctgcgtgggctcctggttggtttgcttcagccgcccccgtgccaaggagcccaccggatggcttctgtccttgactcccttgcacaggcatttgtgaaaagaccacactcttcatctcatgtctgcaacaagactgagtcctttttttttttttttcccaactgagaagtcttagtttgtcattgaaagacttttaaaattttatttctgattgtctggaatctagaagtgatgaatgaattctcccaacacttcaagacctcacattactggactctttctattttctgtcacttctagttggaaaccagcgaattccatcctggcctcctttctttcttatcccgctttgctaaagcacaaactaaacccagcacacatgggagcaggcatttcaactttgtcgggcaccacagtcatctgaagggttattaaaacacagatttctgcaacccacaatttctgacctggggtctgaagtgggcccaaaactttgcatttttaattttccaggtaacaccgatgctgctggtctggggactacagttgaggtgccctggcctacgagctgtgggtttaggtggtagtgtcctatttccaagcaatttcagatgacagttttaccaggtatttgccacggtgtggtatgggtccaaacacgttttccagatgagtgatttcccttcgagttgtgtttccaggccaaggcccctcatgtctcctggttccaccatcttcaagggcctcaaggtcactgggctcatctgctctgagctgcagaagggcacagggcatggggctgtgtcttggaggctttagaagttggccctaagagtggcacacgtcaaacccaccatatgtcacggcccaaactccatcatgcagccacaccaggttgcaagggaaactttggttcagacacagagcctgttacactttcaaacgaggctccacttgtcagggcagatcccagctcattctctggcacagagctgtcctcatctggggcgctgatgggttgaaggccactccagtgacagtgtctgtgtgcccagccagccggtgagaaaacgtgcttgagcccatttcatacacgtaagcgtgtctgtcctcggccccacaagccgcgaatcgtccacaaggactgaaagcgattccacatggatagccgcgggttggatgcccttcaaagtggcgctcacacctcagggttctcaggtcccacagtctcatcccatcgccaatggccgtggtcaggaaaaggttataagcctgaggctgttgggttgtaaatgatgaacctttattttggcagatttgatggacaggccgtgagtgggcttccgctatcaccgctgcactgcagccggcgttgaggtcaaacacttccacggtcctgttccggccagctgcgagtacgatgtgggaataaaagtcgttgactgccgataaactggtcatgtctactgcacccgtcgtggagagcctgcaaatcagcttggacttgctcttctgtttatatctcttaatctcatctttgcaagtgtcaatgtgatacctcagtagctgaaattcagggccagaagataacaatataaaggcatctatataatagaactgtgcagactgtataggtttagaaaacatgtctttgcccagaagcagtgcgagctctgccccacgagccgaccacattcgcagggtcccgtcccgggccgcagagagcagccacctccggtcctggctccagcacacggcattcactgccccgtcgtgacctgaaaacacagcaggtgtcccagtcaggctggcatcaaaaacgagtaacagatggttggccaacccacaggccagccactgcccatctcctgagtactggatgcagcatacacgtgtgcaggtgggggcggcagcgacctgggggccgggcttggtgggcacagcgcactccacggggtatgcctcccgtgcgcagctgctcctgctccttgaagatcctttcccctcactcttgatgttggtctttggtgaaaacatagttacatgtggtgctgacgcataaccagatgacctaactttactatggaaaaccaggcgttggtccttcatgacgttccgtgcagcacgtcgctgttcactagcagccttggtactcttctccttggcaattcccagatacagtggagaggtcggtaggacacaggagctggctggcaccgagaggctctgccccatgctggggcactgctgagccctgactagcgcggccgggttgatctccaacacggcaatcttcccgccaaagagggaggccagcaagcacagcaccttttgatccgcagtgcggttcctcagggcacacgatccggccagcaggatgctgaggctctggaaatccttgtaatacaaagcagcttccacttccaggtttgccaggttaaatacgaataagcccactgagcttccgatccacacacatcgggtgttctcagaagaaagacatccacatgcagaatttgggatgagtgagagatcacagggtgcaagtctcagtacaggaaatgttacttcaacctgctctccttttcccagagcacttgtagagggaagctggctttcttctggctggctgcacagcccagacttaacccttcttgtggagaaagtctctgtcttcttccttaggtcaacccgtgccacacgacgataatggtgtccatccatcaaactgaagatccaaagctggccgtcagcacacccggtgaccagctgcctgctttctgcatcaatgaataaactgagaagaggatatgctgataacacagatgaactgtatattaatgatcctgtacaatggtcccagaccttaaagcctctgtcctcagacgccgagatgagggtgcctgctcgccagggacagaactccaccgcagtcaccgggcccaggtggccctgcagctcggcccgaacagcctgagtctgagagaatgtgtgcaggaaggtcggtggtgggactttgtggcggttattaacatcaggacgttctatgtatgtcacagaaaatcgctgctcaatatccagcatgaatattttgtttccagcacacacggcaacaacatgatcatccaggctcaactgtaaacacagcacctttcccaaaagcgagcccatgacagtccctcgagggaccagcccttgaagtactttctctctacattcatccaggttccacattataacataatccagtgatgctgagcagattagaagtgggttcactttatttccaaaagccatagcagtaattggctgatggtgtcctcgtaggattagaagctgatgagaaggatccttagtgttccatatacaaagttcagttccatccaaagggaaagcacagtcctgcatgctgcaagcaagctgaacatgagacacagactccttggattcaaccaggtatttttctataactatatcacttagacagccaccattacttgagaaaatgtcttggggattttccatcttcaatctatttattcacctctcctcatcccaagaaaaaagaagagaaattgccgaaaactctggagcttccacattctcaactgctccattcttctcacgggctttccagttaagcaaaccttgactcaaataccactattcccacttcacagagcctgcttaggcttcctcgatcagcttccacaactgagcccttttcctccgaactccacatgcgctcagttctcaaagcgccgatctcaagcggccgcccggatgctccggcccgacttgtgccccgaattcccctggagaccctcgcactagcacggcgtcaggaggaggcttcgggtgacgagacagcgggcaacggctctggtccagagcgcgcgtgtccgccgttggaagcggtcacggcggaaccctcaaatcgccccctttcctagagacctcagcggagccgcgagcaaccgcgcagcccccgcgctccagccctgcgccctaggcacacgccccagagcagcagctcgggttcggcgccgactccgcgccgagaccagcccgctaggggaggactcacagcacccagctcccaggagggcacgcagaggactaccgagccacactccgccccacgctcgccgctatggttacttgccagccgacccacgcgagccgctatggttactagcccgccgcccctcgcgcccacgccccttt

SEQ ID NO: 12832 - RNA, 6356 nt, Homo sapiens
  source 1..6356: mol_type = other RNA
gctcggactgagcaggtggggaggggggaaaccgatcatcaccgctgcagcactctctgggagagcaagtggctacctgcgctctgaaagaagggagcaaagtaggtggatctgagaactattggaaggcagagtcaagtccctgggatttagagtgtgatgactgggctgagagacagggaggacccaggaagactgagaatctccctctgtccttaaacctgtgcactctggggacatctaaaaagtttctgactcagcgcctaggaccgtgggccccccatcttagaaactgaaaggaatgttcatctacctttaagcaaaggcttgtgtttttaagtgaaatcatctcagatccaggagagagggctgggaagacagtgtgcagaggacttgggtgaactcctgggtctctggtgtctttcccagtaatgtctgctgtgtctgcagagcaggagtttctgctgcttcttctgatcccaactccttgcgtccctcgagtcatttctattctgaatcccacctgtgcccttcaccccagggcctgtgtggagaaacaagggtgtcaaaaatgaatgagacaggacaaggggcagcccctgtcttattttgcttctttggaacaagtgaagacaaacaacaaccaaaaaaaaaaaaaaaaaccatttccaggcgaattccctggattattttagcaaactccacagcttttgataaacttgggccgagcataaggaagcaaagagtcgtacatctttttcacatccttgctcctttcacagcaggctttcagcgggaggggaggaggcgaggccccagaggggtcccggagaaagcagaagaaagcggcgtcgacattttctgaaatgccaaaggtcccgtctccactttcaatctccgcagttacaaaacagagggctgagtcatcactcccatgaagtcaggggaggggagccattcagaaggcagttgtaatttttactttatcttttactaaatattgaggatggaaacccccagcctttcccacatgcattttctccagtggagagctagaagactgggccgtctctcttgccctgctttttgtcttctctgaggtcttttgaactttcccctaagtgggctcaaaagggatgattcagtctccaagaagcccagcaagtactttcagaaaagttagggaaacgttttcagccatttcagaaagtttagagtggttttagttatggaatcttaacacagttctaaatttgttatgtattcattatctgttcttaaacagatatattttccaaagtgaatgccacaattttctgtgaacatattaacgaatgtttcagaaaacaaaattaattagtggtctaaagtatttgggaaaccacgggttaaatcaaacagctttcttagctgctctgtgggggtgggacggtggcgggggggaggggggggttctactcctttgatagccgaatctgcaccacagagctctacaagggaggcacatttcccaaaggcagcagagcctgcagtgaagtgcctgctgtgcggggagggcccgccctcctattaagaggggcaggtggctggcgtcagggtgagggtgagcccttgccttcacagaagatgtccacgtggtggttctggactagcctcttcctttctctgagccgctcctcttcccgtgaaggaagtcttcgtcccacttctcaaggctgccttgagctcagaggaggatgcctggcttgtaaggtgctctcggcagccacggttgtcctcactggaaatggagcttgcaccacacagtgagtggggcagacacaggcgtcccagacaaaactcccaggcagaaagcagagagtaggaagcagcatcattggtcccaagaaatgatggatcttgccctcagcagcccctctcctgcagccagaggggagcgtccttcacccttgttttccagccccaggctcctctctcccgaggctcgtgttctctgtggccgcatcacacggcgctgggcggctttggctttgtcctgtccacaggcctgaggacccaggggcacttttacacttcacagtcacaagcagtctaggctttacttgctgacacaagcccttgacagctgcgtgggctcctggttggtttgcttcagccgcccccgtgccaaggagcccaccggatggcttctgtccttgactcccttgcacaggcatttgtgaaaagaccacactcttcatctcatgtctgcaacaagactgagtcctttttttttttttttcccaactgagaagtcttagtttgtcattgaaagacttttaaaattttatttctgattgtctggaatctagaagtgatgaatgaattctcccaacacttcaagacctcacattactggactctttctattttctgtcacttctagttggaaaccagcgaattccatcctggcctcctttctttcttatcccgctttgctaaagcacaaactaaacccagcacacatgggagcaggcatttcaactttgtcgggcaccacagtcatctgaagggttattaaaacacagatttctgcaacccacaatttctgacctggggtctgaagtgggcccaaaactttgcatttttaattttccaggtaacaccgatgctgctggtctggggactacagttgaggtgccctggcctacgagctgtgggtttaggtggtagtgtcctatttccaagcaatttcagatgacagttttaccaggtatttgccacggtgtggtatgggtccaaacacgttttccagatgagtgatttcccttcgagttgtgtttccaggccaaggcccctcatgtctcctggttccaccatcttcaagggcctcaaggtcactgggctcatctgctctgagctgcagaagggcacagggcatggggctgtgtcttggaggctttagaagttggccctaagagtggcacacgtcaaacccaccatatgtcacggcccaaactccatcatgcagccacaccaggttgcaagggaaactttggttcagacacagagcctgttaccgacactttcaaacgaggctccacttgtcagggcagatcccagctcattctctggcacagagctgtcctcatctggggcgctgatgggttgaaggccactccagtgacagtgtctgtgtgcccagccagccggtgagaaaacgtgcttgagcccatttcatacacgtaagcgtgtctgtcctcggccccacaagccgcgaatcgtccacaaggactgaaagcgattccacatggatagccgcgggttggatgcccttcaaagtggcgctcacacctcagggttctcaggtcccacagtctcatcccatcgccaatggccgtggtcaggaaaaggttataagcctgaggctgttgggttgtaaatgatgaacctttattttggcagatttgatggacaggccgtgagtgggcttccgctatcaccgctgcactgcagccggcgttgaggtcaaacacttccacggtcctgttccggccagctgcgagtacgatgtgggaataaaagtcgttgactgccgataaactggtcatgtctactgcacccgtcgtggagagcctgcaaatcagcttggacttgctcttctgtttatatctcttaatctcatctttgcaagtgtcaatgtgatacctcagtagctgaaattcagggccagaagataacaatataaaggcatctatataatagaactgtgcagactgtataggtttagaaaacatgtctttgcccagaagcagtgcgagctctgccccacgagccgaccacattcgcagggtcccgtcccgggccgcagagagcagccacctccggtcctggctccagcacacggcattcactgccccgtcgtgacctgaaaacacagcaggtgtcccagtcaggctggcatcaaaaacgagtaacagatggttggccaacccacaggccagccactgcccatctcctgagtactggatgcagcatacacgtgtgcaggtgggggcggcagcgacctgggggccgggcttggtgggcacagcgcactccacggggtatgcctcccgtgcgcagctgctcctgctccttgaagatcctttcccctcactcttgatgttggtctttggtgaaaacatagttacatgtggtgctgacgcataaccagatgacctaactttactatggaaaaccaggcgttggtccttcatgacgttccgtgcagcacgtcgctgttcactagcagccttggtactcttctccttggcaattcccagatacagtggagaggtcggtaggacacaggagctggctggcaccgagaggctctgccccatgctggggcactgctgagccctgactagcgcggccgggttgatctccaacacggcaatcttcccgccaaagagggaggccagcaagcacagcaccttttgatccgcagtgcggttcctcagggcacacgatccggccagcaggatgctgaggctctggaaatccttgtaatacaaagcagcttccacttccaggtttgccaggttaaatacgaataagcccactgagcttccgatccacacacatcgggtgttctcagaagaaagacatccacatgcagaatttgggatgagtgagagatcacagggtgcaagtctcagtacaggaaatgttacttcaacctgctctccttttcccagagcacttgtagagggaagctggctttcttctggctggctgcacagcccagacttaacccttcttgtggagaaagtctctgtcttcttccttaggtcaacccgtgccacacgacgataatggtgtccatccatcaaactgaagatccaaagctggccgtcagcacacccggtgaccagctgcctgctttctgcatcaatgaataaactgagaagaggatatgctgataacacagatgaactgtatattaatgatcctgtacaatggtcccagaccttaaagcctctgtcctcagacgccgagatgagggtgcctgctcgccagggacagaactccaccgcagtcaccgggcccaggtggccctgcagctcggcccgaacagcctgagtctgagagaatgtgtgcaggaaggtcggtggtgggactttgtggcggttattaacatcaggacgttctatgtatgtcacagaaaatcgctgctcaatatccagcatgaatattttgtttccagcacacacggcaacaacatgatcatccaggctcaactgtaaacacagcacctttcccaaaagcgagcccatgacagtccctcgagggaccagcccttgaagtactttctctctacattcatccaggttccacattataacataatccagtgatgctgagcagattagaagtgggttcactttatttccaaaagccatagcagtaattggctgatggtgtcctcgtaggattagaagctgatgagaaggatccttagtgttccatatacaaagttcagttccatccaaagggaaagcacagtcctgcatgctgcaagcaagctgaacatgagacacagactccttggattcaaccaggtatttttctataactatatcacttagacagccaccattacttgagaaaatgtcttggggattttccatcttcaatctatttattcacctctcctcatcccaagaaaaaagaagagaaattgccgaaaactctggagcttccacattctcaactgctccattcttctcacgggctttccagttaagcaaaccttgactcaaataccactattcccacttcacagagcctgcttaggcttcctcgatcagcttccacaactgagcccttttcctccgaactccacatgcgctcagttctcaaagcgccgatctcaagcggccgcccggatgctccggcccgacttgtgccccgaattcccctggagaccctcgcactagcacggcgtcaggaggaggcttcgggtgacgagacagcgggcaacggctctggtccagagcgcgcgtgtccgccgttggaagcggtcacggcggaaccctcaaatcgccccctttcctagagacctcagcggagccgcgagcaaccgcgcagcccccgcgctccagccctgcgccctaggcacacgccccagagcagcagctcgggttcggcgccgactccgcgccgagaccagcccgctaggggaggactcacagcacccagctcccaggagggcacgcagaggactaccgagccacactccgccccacgctcgccgctatggttacttgccagccgacccacgcgagccgctatggttactagcccgccgcccctcgcgcccacgccccttt

SEQ ID NO: 12833 - RNA, 3606 nt, Homo sapiens
  source 1..3606: mol_type = other RNA
gctgaactgggctgagctgggccacctggcaggtgtggcgcttgccctctcccggcctctcccaggtgacctgtcgggggatttcaggtcatgtcacacatacttcccggtaggcatcctcccgactcacagccaagccagaggagggcctatggctccatcctgtcccagagagtgtgtcaggtgggaacacctaccggcaggcagacagagagcctctggggctgctcctggagagggtgggtggtctcaggggaagaggcagatactgaggccaacaacttcgggcccctgtgttttggagtctggtgcagagctgccttcccatggcccatccggtggccaggcacgaccaccaccccttgctggccttatcttttgtgggactgcccagcgggcccaggcctgcccagccaataggggccacttctgaggcatccagaatctcaggcccagtgtgcctgtgttcctggggcggtggcccaggtctgcgacgtttacttaagagctcgggtgtggcctcttggaaaacagcacccgctcacatcccgtccatccaggcctggcgcacctcttactcaagaggagaattaatccatgggcctcaggtgaaataccagcttccacccccgggactcatgtgtgcggctcccagatgtgtgagcacctgctgcgtgcagatgctgggccagctgcaaggacactgcagggtcatgcccaggggctctcctggagggggcacagtgtcttaggggggccaaacagcaggagcagaaaccacaggagcacttgaacccagatggaaaccccccccggaggctttctgccagagggggcaccggggcgaggtggaggcaccagggtaaggtggaggctgttgtagcagctctgggatctgcgccttccctgagaataaaaacacggcacacggcatttggagaacgcttgtggtttatacagcgcttgcaccgccagactctcctgggtgccccgctgggcccctgagatgggttttctggtcccagcagactcatgaatgccggtctcgggggaaaggggctccagaacgtctctgtgaattgtctcaacattcttgtgaggcaggtatgatcatccccattctacagattagaaaactgaggctcagacagctggagggctgtgttcaccgtctttgccctcgctgctccacatcccggtggccaccccagactcctccggcttttcccgggagcttttgcctggcatattttgctctcctgactttgagcacaccccaagactttccttctgctcattaccagggcagcggagggtctggggtgcaaggagagagagggaccctgtagtggctgagacatggggggggactgctccgaagcccagcagcccttggagaatgtgaccaaagccccagacctctccccggaaatgtccagggatacgtgcttgtcatacacacctttggcagccacccccagggactccaggttgagaagctctggcctgagcgagacccagactcccacccccggctgttggcaagaggtaatgaccctactagtgatgggccctcgaagcctccgtccacccctgcctccgctcaccccggccatgaccccagcctggctcacagccagatgtccatccagcagaaggtaaaggggcacctgagcccatgggcaggctctcatgggaccaccggcaacatctcagccttggagatgagagggcagccttggctgggtcagggagcggggcacatgagtgtgttccggtccagtagagatgctttcaagggcaaagctgtgcggcaccgttgttaagagagaggctttcgggatcaggaatacttggttttgaacttcagctctgctccttcccagcctccctcctcagagcttcagtttttcatttgtgaaatggggatggggaaagcacccacctcatgggcctcgctagcaggctctgggtctctggcagccacggtcacgcgtgttccccagcgtggaggtgcatctctttccatacatgcttctggcagtgttgcacagcgttgcacagcttggcggcctcctggctcctgcaccagaagcttgggcccagggcacactggtcggtgcccagcagtggggtcctggggccgtggcaggcccccaccttcttgcacacagccacggggtccatcatgtccttgagactctcaatgagcacgggctcgtactgggtgacgaagtgcttgcactggatcatatagggcagcggcaggatgctgcagccacccttgaaggccaccaggatgtctcgcttggtgctcttgctctccaagttgtgggaggacaccgtgagcagcctcttgcacccattgcagaagctgccctggttctccgcgtcccactctggggacggcacgatggcataggcatcatggactgcccgggcccgcctccggttgccacacagacggatgaacttgcacaccttctctggggtgattttggccacaagctgcaccaaggaggggctgtaggtgtccaccaagatgatgcactccttcgtgatagaggcaggcattaccgagcacacgcgctccagggcatgggtgatcatgagctcagagctgttggacatgagccagtggtccagcttctgcaccacgttcatgcacacctcacaggtcacaccggccttcatctgcatctcgctctgtttccttggcaaccccagctccagggaggggaccccgtccatggccactacttgagtcaaacgggcaggtgcccctagctcctcacagaatccccccttcctgcagagctcctgcggggggagaagcctcagtgcttggtcagcagggacaaaaaactggaagaggtagttcttgcagaggacggccaggccaggccccaaggactcacactgctcctggatgttcaagtcggccaaggtcaagttggaccggacagcctcctggagtcgggagacctgccgtacacagtcttggcacagagctccttcaggcgcctggcgggggtggaaggtaaggggcccattggccatgaacggagccacagcctcaaaggtgtcctctttggagagtggcctcagggtggccaggtgcctctgcagcggctcacagaggctgagcgctgtgcacacctgtgccggggcactgtccggggccccacggagcatgctcaggatggccgaactgtgggcatccaccatccacttgcatccggctgaagactcctggctggggagccactcacaggtcttcatcaccaaagccaggatgtcagactccgtggcgtcagggttcagcccattgccagcggcggctgctatgtcctggcatacgtcgcagggcagagacttcgcggtgggtttgttccatacggccccttggcagtaccccacagccccgcacctggcagctgtctgcagatcctgacaccacaccgtggagccctttgcacactcctgggggcctgaggtggggctggccctggtggcccccaggaggctgggcaggaggagcagggcacacagcatgctgcccagggactctctggctccagagtacccagcagtggctgctgctat

SEQ ID NO: 12834 - RNA, 2831 nt, Homo sapiens
  source 1..2831: mol_type = other RNA
gctgaactgggctgagctgggccgagacgactggacccactgggccgagctgggccaagaggactggacccactgggccacgctgagccgagacaactggacccactgggccacgctggccgagacgactggacccactgggccgagctgagccgagacgactggacccactgggccgagctggacaagatgactggacccactgggccacgctggccgagacgactggacccactgggccgagctgggccgagactactggacccactgggccgagctggacaagatgactggacccactgggccacgctggccgagacgactggacccacatggcagcggacttgacctgggtttcaccggtgacctaattatatgctcatcaacacacaaatcacactcggcagtgccatgacagttccaggaacacacatatttggtgtaaaaaagggtggcaccacagttcctagaaatcttcacctttttccagaaatctttatgaatattccactccttggttaaagaaacccattaaaggtaggggccccaaaccctgcctcacgactcactttcttgagaacacccatactcccctttcttctttgacttttttttctatttgcttgtttatttttatgaggcagggtctcactatgttgcccaggctgatctcgaactcctgcctcagcctcccaatgtgttaggattacaggcgtgagccttcacacccagccacactctgctttctggagggtgtactttttgctttgcaataaatctctactttcattattttttaactcatccttgaattcgttttgtgatggtgttaagaggcaggacactggcctgggtcaaggtcccattcgcatttggggacctcccctggccaccagtatcaaaagtacttccttgttaattttcagggttttttttgagacagattctcactcactctgtcacccaggctggagtgcagtggcatgatcttggctactgcaacctctgcctcccgggatccagcgattctcgtgactcagcctcctgagtagctgggaataccggcatgtgccaccatacctggctaatttttgaatttttagtagggatggggtttcaccattttggccgggctggtcttgaactcctgggctcaagtgatccacccgccttggcctcccaaagtgctgggattacaggtgtcagccaccgtgcccggcttacttatcagttacaaagggcaaagtggtaactttactgtgagaagcttgtggatgccagtttaaccagaggatcaaaggtaccgttgccgctggtgggcagccagcgtcccgagtgctgggaaggatgcctggctcttggtgccaatctgttcatgcagaaatgtcaggaacgctcaatgcggggacaatctacaaaacaaccggtttgcattcttcaaaagtttcagtgtcataaaagatttttaaaaagacaggcccaatgtatataccgtgaaaatagtaaaacaataaaatataaaagtaaaaagactgaagtaaccttgtctttgtattgatgtggagtcaaccgctgcttccagttgcgggggagtagctgctgccaggtacgtctccctccagaaacgactctgagaccagacaaaattcgtgcgctgctctcttcaggcagtggggtgaggacagcacaagaccgagagggtgcttggaggcgcccacactcccggctctccttggccataaccccacaagcagggctccaggcagagcacggcagtccccctgggatgagaggcagagactggagtgaggggcttaggtgtgcatgttgctggtggggagtgcttgggacctctgcaagcctgtggctgagggtgaggaggtgccggaggctcaccagagagcagtgactataggccctgtgctgttatccgtcactgcataaccaatcaacaccgatttagtagctttaaaaaacatgcatttattctcagttttggggggtcaggagcccacacacaattccgctgggtggctcggggtttcaagagtgccaccaaggtgttggtatttctttctgaagcttgaggtcctctttgaaggccacgtggttgttggcagaattcagttccttgtggctgtaggactgaggtccctgctttcttgttggctggcagcctggggccactcactggttccctgatacgaggcccctcccatgccttccaacagccatatcttcacagacagcaggggtgtcttgctgctccgtcccccaggacagagcctggaatgatgcagccaatcacagagtgacttatcacctttctgtgttctatgggcaaggtagcaggacttgggaaacactttgggctttcgacatcgacactgacaaagcatgagaacaagtccacagggcccagcagtgaaccaacctgctctggggccaggccagggctgaggtcatcctgtgacactgggggccagagagcggccttggccttgctccccaccctgcctccaagcccctgtctgcctctgggctgccagcctccacctgcctgcgacggtggccccggggtgatggcctggctgtgccccatgcacaggtggttcgttaggcactcggcggctattattaacccagcagtgacgtcaccggcagccaatgggaggcaggtttatttccagggctgacagcttgatagcggttaattttagctgcatcttctttcccgaggctcgtgaaaccctagccagccaaagaaggggttgcctgtgtctccccaaacagctcagggatgggtcctgggggctctgggaggcggcaag

SEQ ID NO: 12835 - RNA, 931 nt, Homo sapiens
  source 1..931: mol_type = other RNA
gctgaactgggctgagctgggctctgtttctaccaccatgttgccttttctaggacttgctgactgtctttggagtgggctggggaatgcccttgaggtttctctctcctctgtccttgcagaccagggtttggagccacctcctctctcctgaccttctgcattttcaaaccaacagcttacatgggaatactgctgcccctgctgtttccaatgccctgggctagaattccctggatggaagtgattttctgcacataagcccaggaagatctgaagtacatgttgactgaggaactgctgacaggagaaggccagaaggcaggaggaacaagtgtagatttctggctttggttccaatgagagaagattcctgtaattctccagcatcacttctttgtatagattcctctgctctggactcagtctcttccattctgcttctgtgaagatcacagtcacatccctgaatgtaactggtaccactatttgggcctttccctcctttttctgggggcagtcagtatcattagaaggcaagcctttcgctttatgattttgggtcaatttcttcatagtctctacattttccccattctttggaagcaaaatctcttcccagtattgatctcccagtgctgaaggataaggcaacatcatggcgccagagtcagcccagtgtgtgccttgaaattctgccagaggtccaggtagatgttatttcatctcaagatggagttctgctgcctgtggtgacttcttccaaccttaattataaaaagcccagcttgtttccctgcagccaggacctgataggaagttctcgggagcacagaagtctttcctttctcaagagatcgtcctctcccagcaggcagggattggagaaggtggaccagagccagcgtgcccgggatctcggccaccgacc

SEQ ID NO: 12836 - RNA, 892 nt, Homo sapiens
  source 1..892: mol_type = other RNA
gctgaactgggctgagctgggctctgtttctaccaccatgttgccttttctaggacttgctgactgtctttggagtgggctggggaatgcccttgaggtttctctctcctctgtccttgcagaccagggtttggagccacctcctctctcctgaccttctgcattttcaaaccaacagcttacatgggaatactgctgcccctgctgtttccaatgccctgggctagaattccctggatggaagtgattttctgcacataagcccaggaagatctgaagtacatgttgactgaggaactgctgacaggagaaggccagaaggcaggaggaacaagtgtagatttctggctttggttctgccaatgagagaagattcctgtaattctccagcatcacttctttgtatagattcctctgctctggactcagtctcttccattctgcttctgtgaagatcacagtcacatccctgaatgtaactggtaccactatttgggcctttccctcctttttctgggggcagtcagtatcattagaaggcaagcctttcgctttatgattttgggtcaatttcttcatagtctctacattttccccattctttggaagcaaaatctcttcccagtattgatctcccagtgctgaaggataaggcaacatcatggcgccagagtcagcccagtgtgtgccttgaaattctgccagaggtccaggtagatgttatttcatctcaagatggagttctgctgcctgtggtgacttcttccaacctgataggaagttctcgggagcacagaagtctttcctttctcaagagatcgtcctctcccagcaggcagggattggagaaggtggaccagagccagcgtgcccgggatctcggccaccgacc

SEQ ID NO: 12837 - RNA, 934 nt, Homo sapiens
  source 1..934: mol_type = other RNA
gctgaactgggctgagctgggctctgtttctaccaccatgttgccttttctaggacttgctgactgtctttggagtgggctggggaatgcccttgaggtttctctctcctctgtccttgcagaccagggtttggagccacctcctctctcctgaccttctgcattttcaaaccaacagcttacatgggaatactgctgcccctgctgtttccaatgccctgggctagaattccctggatggaagtgattttctgcacataagcccaggaagatctgaagtacatgttgactgaggaactgctgacaggagaaggccagaaggcaggaggaacaagtgtagatttctggctttggttctgccaatgagagaagattcctgtaattctccagcatcacttctttgtatagattcctctgctctggactcagtctcttccattctgcttctgtgaagatcacagtcacatccctgaatgtaactggtaccactatttgggcctttccctcctttttctgggggcagtcagtatcattagaaggcaagcctttcgctttatgattttgggtcaatttcttcatagtctctacattttccccattctttggaagcaaaatctcttcccagtattgatctcccagtgctgaaggataaggcaacatcatggcgccagagtcagcccagtgtgtgccttgaaattctgccagaggtccaggtagatgttatttcatctcaagatggagttctgctgcctgtggtgacttcttccaaccttaattataaaaagcccagcttgtttccctgcagccaggacctgataggaagttctcgggagcacagaagtctttcctttctcaagagatcgtcctctcccagcaggcagggattggagaaggtggaccagagccagcgtgcccgggatctcggccaccgacc

SEQ ID NO: 12838 - RNA, 1015 nt, Homo sapiens
  source 1..1015: mol_type = other RNA
gctgaactgggctgagctgggctctgtttctaccaccatgttgccttttctaggacttgctgactgtctttggagtgggctggggaatgcccttgaggtttctctctcctctgtccttgcagaccagggtttggagccacctcctctctcctgaccttctgcattttcaaaccaacagcttacatgggaatactgctgcccctgctgtttccaatgccctgggctagaattccctggatggaagtgattttctgcacataagcccaggaagatctgaagtacatgttgactgaggaactgctgacaggagaaggccagaaggcaggaggaacaagtgtagatttctggctttggttctgccaatgagagaagattcctgtaattctccagcatcacttctttgtatagattcctctgctctggactcagtctcttccattctgcttctgtgaagatcacagtcacatccctgaatgtaactggtaccactatttgggcctttccctcctttttctgggggcagtcagtatcattagaaggcaagcctttcgctttatgattttgggtcaatttcttcatagtctctacattttccccattctttggaagcaaaatctcttcccagtattgatctcccagtgctgaaggataaggcaacatcatggcgccagagtcagcccagtgtgtgccttgaaattctgccagaggtccaggtagatgttatttcatctcaagatggagttctgctgcctgtggtgacttcttccaaccttaattataaaaagcccagcttgtttccctgcagccaggacctgataggaagttctcgggagcacagaagtctttcctttctcaagagatcgtcctctcccagcaggcagggattggagaaggtggacctacgctcggcctttcccgaccctcctttccccacgagagagggcatcctggggccaaggagccgcggaggccgcgctcaccagagccagcgtgcccgggatctcggccaccgacc

SEQ ID NO: 12839 - RNA, 1077 nt, Homo sapiens
  source 1..1077: mol_type = other RNA
gctgaactgggctgagctgggctctgtttctaccaccatgttgccttttctaggacttgctgactgtctttggagtgggctggggaatgcccttgaggtttctctctcctctgtccttgcagaccagggtttggagccacctcctctctcctgaccttctgcattttcaaaccaacagcttacatgggaatactgctgcccctgctgtttccaatgccctgggctagaattccctggatggaagtgattttctgcacataagcccaggaagatctgaagtacatgttgactgaggaactgctgacaggagaaggccagaaggcaggaggaacaagtgtagatttctggctttggttctgccaatgagagaagattcctgtaattctccagcatcacttctttgtatagattcctctgctctggactcagtctcttccattctgcttctgtgaagatcacagtcacatccctgaatgtaactggtaccactatttgggcctttccctcctttttctgggggcagtcagtatcattagaaggcaagcctttcgctttatgattttgggtcaatttcttcatagtctctacattttccccattctttggaagcaaaatctcttcccagtattgatctcccagtgctgaaggataaggcaacatcatggcgccagagtcagcccagtgtgtgccttgaaattctgccagaggtccaggtagatgttatttcatctcaagatggagttctgctgcctgtggtgacttcttccaaccttaattataaaaagcccagcttgtttccctgcagccaggaccttggaaaatgaatgtgagtgaaagcgacgatgccatttctaagcattgcataattccaccatttcttttgttctgagaacagcatgtccgaagagggactgtggttctactgataggaagttctcgggagcacagaagtctttcctttctcaagagatcgtcctctcccagcaggcagggattggagaaggtggaccgtgaggctgggtttcgcgttctggttccaggctgtccccccactgcctgcccctgccccgaatcgca

SEQ ID NO: 12840 - RNA, 608 nt, Homo sapiens
  source 1..608: mol_type = other RNA
gctgaactgggctgagctgggctctgtttctaccaccatgttgccttttctaggacttgctgactgtctttggagtgggctggggaatgcccttgaggtttctctctcctctgtccttgcagaccagggtttggagccacctcctctctcctgaccttctgcattttcaaaccaacagcttacatgggaatactgctgcccctgctgtttccaatgccctgggctagaattccctggatggaagtgattttctgcacataagcccaggaagatctgaagtacatgttgactgaggaactgctgacaggagaaggccagaaggcaggaggaacaagtgtagatttctggctttggttctgccaatgagagaagattcctgtaattctccagcatcacttctttgtatagattcctctgctctggactcagtctcttccattctgcttctgtgaagatcacagtcacatccctgaatgtaactggtacctgataggaagttctcgggagcacagaagtctttcctttctcaagagatcgtcctctcccagcaggcagggattggagaaggtggaccagagccagcgtgcccgggatctcggccaccgacc

SEQ ID NO: 12841 - RNA, 1057 nt, Homo sapiens
  source 1..1057: mol_type = other RNA
gctgaactgggctgagctgggctctgtttctaccaccatgttgccttttctaggacttgctgactgtctttggagtgggctggggaatgcccttgaggtttctctctcctctgtccttgcagaccagggtttggagccacctcctctctcctgaccttctgcattttcaaaccaacagcttacatgggaatactgctgcccctgctgtttccaatgccctgggctagaattccctggatggaagtgattttctgcacataagcccaggaagatctgaagtacatgttgactgaggaactgctgacaggagaaggccagaaggcaggaggaacaagtgtagatttctggctttggttctgctgtaatcccaactactcgagaggctgtggcaggagaattgcttgaacccgggaggcaaaggttgtggtgagccgagattgcacgattgcactctagcctgggcaacaagagcgaaactccatccaatgagagaagattcctgtaattctccagcatcacttctttgtatagattcctctgctctggactcagtctcttccattctgcttctgtgaagatcacagtcacatccctgaatgtaactggtaccactatttgggcctttccctcctttttctgggggcagtcagtatcattagaaggcaagcctttcgctttatgattttgggtcaatttcttcatagtctctacattttccccattctttggaagcaaaatctcttcccagtattgatctcccagtgctgaaggataaggcaacatcatggcgccagagtcagcccagtgtgtgccttgaaattctgccagaggtccaggtagatgttatttcatctcaagatggagttctgctgcctgtggtgacttcttccaaccttaattataaaaagcccagcttgtttccctgcagccaggacctgataggaagttctcgggagcacagaagtctttcctttctcaagagatcgtcctctcccagcaggcagggattggagaaggtggaccagagccagcgtgcccgggatctcggccaccgacc

SEQ ID NO: 12842 - RNA, 1138 nt, Homo sapiens
  source 1..1138: mol_type = other RNA
gctgaactgggctgagctgggctctgtttctaccaccatgttgccttttctaggacttgctgactgtctttggagtgggctggggaatgcccttgaggtttctctctcctctgtccttgcagaccagggtttggagccacctcctctctcctgaccttctgcattttcaaaccaacagcttacatgggaatactgctgcccctgctgtttccaatgccctgggctagaattccctggatggaagtgattttctgcacataagcccaggaagatctgaagtacatgttgactgaggaactgctgacaggagaaggccagaaggcaggaggaacaagtgtagatttctggctttggttctgctgtaatcccaactactcgagaggctgtggcaggagaattgcttgaacccgggaggcaaaggttgtggtgagccgagattgcacgattgcactctagcctgggcaacaagagcgaaactccatccaatgagagaagattcctgtaattctccagcatcacttctttgtatagattcctctgctctggactcagtctcttccattctgcttctgtgaagatcacagtcacatccctgaatgtaactggtaccactatttgggcctttccctcctttttctgggggcagtcagtatcattagaaggcaagcctttcgctttatgattttgggtcaatttcttcatagtctctacattttccccattctttggaagcaaaatctcttcccagtattgatctcccagtgctgaaggataaggcaacatcatggcgccagagtcagcccagtgtgtgccttgaaattctgccagaggtccaggtagatgttatttcatctcaagatggagttctgctgcctgtggtgacttcttccaaccttaattataaaaagcccagcttgtttccctgcagccaggacctgataggaagttctcgggagcacagaagtctttcctttctcaagagatcgtcctctcccagcaggcagggattggagaaggtggacctacgctcggcctttcccgaccctcctttccccacgagagagggcatcctggggccaaggagccgcggaggccgcgctcaccagagccagcgtgcccgggatctcggccaccgacc

SEQ ID NO: 12843 - RNA, 1054 nt, Homo sapiens
  source 1..1054: mol_type = other RNA
gctgaactgggctgagctgggctctgtttctaccaccatgttgccttttctaggacttgctgactgtctttggagtgggctggggaatgcccttgaggtttctctctcctctgtccttgcagaccagggtttggagccacctcctctctcctgaccttctgcattttcaaaccaacagcttacatgggaatactgctgcccctgctgtttccaatgccctgggctagaattccctggatggaagtgattttctgcacataagcccaggaagatctgaagtacatgttgactgaggaactgctgacaggagaaggccagaaggcaggaggaacaagtgtagatttctggctttggttctgtaatcccaactactcgagaggctgtggcaggagaattgcttgaacccgggaggcaaaggttgtggtgagccgagattgcacgattgcactctagcctgggcaacaagagcgaaactccatccaatgagagaagattcctgtaattctccagcatcacttctttgtatagattcctctgctctggactcagtctcttccattctgcttctgtgaagatcacagtcacatccctgaatgtaactggtaccactatttgggcctttccctcctttttctgggggcagtcagtatcattagaaggcaagcctttcgctttatgattttgggtcaatttcttcatagtctctacattttccccattctttggaagcaaaatctcttcccagtattgatctcccagtgctgaaggataaggcaacatcatggcgccagagtcagcccagtgtgtgccttgaaattctgccagaggtccaggtagatgttatttcatctcaagatggagttctgctgcctgtggtgacttcttccaaccttaattataaaaagcccagcttgtttccctgcagccaggacctgataggaagttctcgggagcacagaagtctttcctttctcaagagatcgtcctctcccagcaggcagggattggagaaggtggaccagagccagcgtgcccgggatctcggccaccgacc

SEQ ID NO: 12844 - RNA, 1135 nt, Homo sapiens
  source 1..1135: mol_type = other RNA
gctgaactgggctgagctgggctctgtttctaccaccatgttgccttttctaggacttgctgactgtctttggagtgggctggggaatgcccttgaggtttctctctcctctgtccttgcagaccagggtttggagccacctcctctctcctgaccttctgcattttcaaaccaacagcttacatgggaatactgctgcccctgctgtttccaatgccctgggctagaattccctggatggaagtgattttctgcacataagcccaggaagatctgaagtacatgttgactgaggaactgctgacaggagaaggccagaaggcaggaggaacaagtgtagatttctggctttggttctgtaatcccaactactcgagaggctgtggcaggagaattgcttgaacccgggaggcaaaggttgtggtgagccgagattgcacgattgcactctagcctgggcaacaagagcgaaactccatccaatgagagaagattcctgtaattctccagcatcacttctttgtatagattcctctgctctggactcagtctcttccattctgcttctgtgaagatcacagtcacatccctgaatgtaactggtaccactatttgggcctttccctcctttttctgggggcagtcagtatcattagaaggcaagcctttcgctttatgattttgggtcaatttcttcatagtctctacattttccccattctttggaagcaaaatctcttcccagtattgatctcccagtgctgaaggataaggcaacatcatggcgccagagtcagcccagtgtgtgccttgaaattctgccagaggtccaggtagatgttatttcatctcaagatggagttctgctgcctgtggtgacttcttccaaccttaattataaaaagcccagcttgtttccctgcagccaggacctgataggaagttctcgggagcacagaagtctttcctttctcaagagatcgtcctctcccagcaggcagggattggagaaggtggacctacgctcggcctttcccgaccctcctttccccacgagagagggcatcctggggccaaggagccgcggaggccgcgctcaccagagccagcgtgcccgggatctcggccaccgacc

SEQ ID NO: 12845 - RNA, 158 nt, Homo sapiens
  source 1..158: mol_type = other RNA
gctgaactgggctgagctgggctgggatgggatactgagttcgcatctgcttttgtcccaacttccctccccgagggtcagcagcacaaccaagcgagatcaacacaactagtgtgtggtggctaagtgcaccacagcggcgatacggctagaagaaa

SEQ ID NO: 12846 - RNA, 326 nt, Homo sapiens
  source 1..326: mol_type = other RNA
gctgaactgggctgagctgggctgggatgggatactgagttcgcatctgcttttgtcccaacttccctccccgagggtcagcagcacaaccaagcgagatcaacacaactagtgtgtggtggctaagtgcaccacagcggcgatacggctagaagaaacgcgccattctcgctgctcttcatcagacagccggcaagcgacgaaaagatgtagccgtggcgggtgtaggtgccgctgcccgggctgccctcctccaagttacacagacgttcgccggggatgcagtatctcacaggtggcgccatgattgccgctgtcccaaaacc

SEQ ID NO: 12847 - RNA, 440 nt, Homo sapiens
  source 1..440: mol_type = other RNA
gctgaactgggctgagctgggctgggatgggatactgagttcgcatctgcttttgtcccaacttccctccccgagggtcagcagcacaaccaagcgagatcaacacaactagtgtgtggtggctaagtgcaccacagcggcgatacggctagaagaaactaagagaccaacattgtaccactgaggcactaaagacgcgtccgcagtgcccatgcctaaggactggaactcaagggcagcctaagggaaaaacagaggggagatggcatgccgcttcctttaccgcgccattctcgctgctcttcatcagacagccggcaagcgacgaaaagatgtagccgtggcgggtgtaggtgccgctgcccgggctgccctcctccaagttacacagacgttcgccggggatgcagtatctcacaggtggcgccatgattgccgct

SEQ ID NO: 12848 - RNA, 1008 nt, Homo sapiens
  source 1..1008: mol_type = other RNA
gctgacagcagggctggccgctcacggagacgcgtcaccagcccgctcccagcatcccgctccgtgaaggccgaccgctccgtgactgggtcctcaggttctgagcgggccctgaacggagagtgcatgctgcccagcttcatgaagagccggtgctgcaggtccagaggtgtctctttaaagaaagatgcgggcttgtcgtagacggtcacagccctgatgtgccagttatccgccaggtcttctcgcatagcattggtaacacacaggttcaggtgggacaggcgcccaaagaacttctcgtaccacttggccagcagaacgaggggatggttggggccatgcaccagacccatgatggagtagccatagttgtgccagtcaatgacgagcttgcttccacaaaggcagcccacgaaccagcagacagcaatgctaggcagacctggggggttctggagaaagatataggcacctggctccctccacatcaacttccacagcaagtacatagcctgaagtacaactttgactccgtactggaaaactcggggcccaactgcaagactctgaagttctgtcaaccccacaatctgaattctgttgttctgcaagagctcatcatggggtttggagtccaggaaaggctggggcagaaccgctcgtctaatctcggagagctgcccaaaggcggcgactaaaggagcacttccgcctcgactccccggggcggttagaaccgaggatcaacggctgagagagcatcgtccctcccagacccttggccactcactgcagaaccccaggagggtcaccgagaagccgtgcatggccaacgacagcgcgtggtactgcatacgggggctgcggcccacgtcgcccagcaccaccgctactacatgccgggccgcccgcccccggcgccagcgcttccatcctcccagcagcagcagcggcagcagcagacacagcgccagcaggaccaagcatgaggccgccatcttggct

SEQ ID NO: 12849 - RNA, 693 nt, Homo sapiens
  source 1..693: mol_type = other RNA
gctgacagcagggctggccgctcacggagacgcgtcaccagcccgctcccagcatcccgctccgtgaaggccgaccgctccgtgactgggtcctcaggttctgagcgggccctgaacggagagtgcatgctgcccagcttcatgaagagccggtgctgcaggtccagaggtgtctctttaaagaaagatgcgggcttgtcgtagacggtcacagccctgatgtgccagttatccgccaggtcttctcgcatagcattggtaacacacaggttcaggtgggacaggcgcccaaagaacttctcgtaccacttggccagcagaacgaggggatggttggggccatgcaccagacccatgatggagtagccatagttgtgccagtcaatgacgagcttgcttccacaaaggcagcccacgaaccagcagacagcaatgctaggcagacctggggggttctggagaaagatataggcacctggctccctccacatcaacttccacagcaagtacatagcctgaagtacaactttgactccgtactggaaaactcggggcccaactgcaagactctgaagttctgtcaaccccacaatctgaattctgttgttctgcaagagctcatcatggggtttggagttaggagaattacgtgagaccacgcaatggattcacttaacacacttctgacacgtg

SEQ ID NO: 12850 - RNA, 852 nt, Homo sapiens
  source 1..852: mol_type = other RNA
gctgacagcagggctggccgctcacggagacgcgtcaccagcccgctcccagcatcccgctccgtgaaggccgaccgctccgtgactgggtcctcaggttctgagcgggccctgaacggagagtgcatgctgcccagcttcatgaagagccggtgctgcaggtccagaggtgtctctttaaagaaagatgcgggcttgtcgtagacggtcacagccctgatgtgccagttatccgccaggtcttctcgcatagcattggtaacacacaggttcaggtgggacaggcgcccaaagaacttctcgtaccacttggccagcagaacgaggggatggttggggccatgcaccagacccatgatggagtagccatagttgtgccagtcaatgacgagcttgcttccacaaaggcagcccacgaaccagcagacagcaatgctaggcagacctggggggttctggagaaagatataggcacctggctccctccacatcaacttccacagcaagtacatagcctgaagtacaactttgactccgtactggaaaactcggggcccaactgcaagactctgaagttctgtcaaccccacaatctgaattctgttgttctgcaagagctcatcatggggtttggagttgcagaaccccaggagggtcaccgagaagccgtgcatggccaacgacagcgcgtggtactgcatacgggggctgcggcccacgtcgcccagcaccaccgctactacatgccgggccgcccgcccccggcgccagcgcttccatcctcccagcagcagcagcggcagcagcagacacagcgccagcaggaccaagcatgaggccgccatcttggct

SEQ ID NO: 12851 - RNA, 870 nt, Homo sapiens
  source 1..870: mol_type = other RNA
gctgacagcagggctggccgctcacggagacgcgtcaccagcccgctcccagcatcccgctccgtgaaggccgaccgctccgtgactgggtcctcaggttctgagcgggccctgaacggagagtgcatgctgcccagcttcatgaagagccggtgctgcaggtccagaggtgtctctttaaagaaagatgcgggcttgtcgtagacggtcacagccctgatgtgccagttatccgccaggtcttctcgcatagcattggtaacacacaggttcaggtgggacaggcgcccaaagaacttctcgtaccacttggccagcagaacgaggggatggttggggccatgcaccagacccatgatggagtagccatagttgtgccagtcaatgacgagcttgcttccacaaaggcagcccacgaaccagcagacagcaatgctaggcagacctggggggttctggagaaagatataggcacctggctccctccacatcaacttccacagcaagtacatagcctgaagtacaactttgactccgtactggaaaactcggggcccaactgcaagactctgaagttctgtcaaccccacaatctgaattctgttgttctgcaagagctcatcatggggtttggagttgcagaaccccaggagggtcaccgagaagccgtgcatggccaacgacagcgcgtggtactgcatacgggggctgcggcccacgtcgcccagcaccaccgctactacatgccgggccgcccgcccccggcgccagcgcttccatcctcccagcagcagcagcggcagcagcagacacagcgccagcaggaccaagcatgaggccgccatcttggctggcccgcagcagtcacgt

SEQ ID NO: 12852 - RNA, 496 nt, Homo sapiens
  source 1..496: mol_type = other RNA
gctgacagcagggctggccgctcgcggaggcgcatcaccagcccgctcccagcatcccgctccatgaaggccgaccgctccgtgtctgggtcctcaggttcaggccctgaacggagagtgcgtgccgcccagcttcatgaagagttggtgctgcaggtccagaggtctcttgaaagaaagatgctggcttgtcatagacggtcacagcccttcctcgggtgctcgcatggggctgccactgacgacgaactgctgcagctccttggtgatctggccctggtcatgggacaggaactgtagggtcaggaccataaggagcttcaccacctgtttacgtggaagatcatttttgtcataattagtagtgggatcaatttcactgttattgtatatacagctctgtgcctcaaacagttccacatggctggggaggcctcagaatcatgacgggaggcaaaaggcacttctttcgtggtggcggcaagagaaaaatgag

SEQ ID NO: 12853 - RNA, 422 nt, Homo sapiens
  source 1..422: mol_type = other RNA
gctgacagcagggctggccgctcgtggagacgcgtcaccagcccgctcccagaatcccgctccgtgaaggccgaccgctctgtgtctgggtcctcaggttctgagcgggccctgaacggagagtgcgtgctgcccagcttcatgaagagccggtgctgcaggtccagaggtgcctctttaaagaaagatgccggcttgtcgtagacggtcacagcccagcctgcagtagctcccatgtcccttcaggttaaaattcagacttcttagcaaggaactgcttatttctccagcctctgtgacagcctcacaccctacaatcgagctctgctgatcctggagaagctccctctgagcctttgcacacctgtctctgctacttgagggtgatttccacctggttacctcctggtgtcacctcccac

SEQ ID NO: 12854 - RNA, 32 nt, Homo sapiens
  source 1..32: mol_type = other RNA
gctgcaccggagactgggtaagacatgacaag

SEQ ID NO: 12855 - RNA, 183 nt, Homo sapiens
  source 1..183: mol_type = other RNA
gctgcgggctgcggtcagggcgttctcccgttgcaccagcgcgaggttacggtgaggcctgagagcctgcattgcaaccaggactcagggggtgcactggcccgtgaccacccacccccccggagtggtgaggcaccagtatttggtcgtgctgccatctccctggcagaacctcgttgcgtt

SEQ ID NO: 12856 - RNA, 352 nt, Homo sapiens
  source 1..352: mol_type = other RNA
gctgggattacaggcatgagccaacacgctcggcattggccagccttggcaaggtgacaggcgggtatggtaatagcaatctcaggagggctcttctgttgctgtgtagaaaatgaaccaagtagcatagaatcgtgaccagctttccacacctggctggagcactcctggggccttcagtagggacagttactatcggttgtgatgcgcaggtaacagagagctcaattcatcatgacaaccagtcagacaggggctgtgagcagcctttggacagaactttcgcatagccgttaaaagagctttccaaacttgggggtcccgccgcctcggctaggcctcatctgctcat

SEQ ID NO: 12857 - RNA, 8393 nt, Homo sapiens
  source 1..8393: mol_type = other RNA
gctgggattacaggcatgagccaacatgcccagccttgtatgccgtttcttttttttctttttttttttttttgagacagggtcttactctgtcacccgggctggagtgcagtcgtagaatcagatcactacagcctttaactgctgggctcaagcaatcctcctgcctcaccctcctgagtagctagaactacaggtgtgaaccaccttgccctgctgttatatgccagtttcttataaaatactataaatatcagcaaatgtgcaacaaatgtttaatagggaggccaccttagttttcctttctgttgtatgtagtaggagcaaactgcctttctgttgtatgtagtatcagagcaggtctcttctaatattaacctgaacaaaatccatcctatttcaggatgcagttgtctatctaaacataagtagagataaatgaaggatttttttaaattttattattttattttttttgagacaaggtctcattctgtcacccaggctagagtgtagtggcacgaccacagctcactgtagccttcacctcccagactcaagcagtcttaccacctcagcctcctgagtagctagggctacaggcatgtgccaccacacccagctttttaaaatttttggtagagacagggtctcactatgttgccagggctagtcccaaactcctgggctcgtgcgatcctcccaccttggcctctcaaagtgttgggatgctttttgatgcagaatattgatttataaaatactgtatctttactgtcccttcagagttcagctaaagaaacgtgcttttaggttttaaaaacagtcccgataattgcatcctccagtggtcctacttaaactgaaaacaaggtattgtcttctttttcacagcaagaccacacaacacagaggtgttggatgaaaacagcaagcccttttcaatgcagcagtccatagaatgcctctgtcagaatcaaagactaagcttaagagttcctcgcatatatcgttgtgcacaggatcaacatgatggtgactgggaaaaaattacttcaagtaacatgcttagctttccctccttaatgtgaaaaatcaagggcttactgacataggaacaacagaaatgctcctggaacttcaagttgctgaattataagtttattttttatcaataaatatttttatacttacattgagtgatgtgtttaacaacaaattgtgacagagctgagtgctcctatcttacagggtcaatgaactacttattaagccttactggtagcactgaatttagcagttctgagaacatgtgaaactatgttaaaactgaaggcactatatatttttacataaaagcttgaacatacagatgaattataacctatgtgaagaaatcttagatataaaactaacttttcaaagatacaaaagaaattaaacaggtttcctgaaattttagttcttggtctgttcacctctgtggggaaaattcttagttccagtgataactgttctagttactacttttaagtatgtaaatactagaaaggtagtactagtgacatcatcacgtgtattgttatctatggggcaaatgtgtggtgcccagaataaaatatacctcatgcctagggtagggacatcctttccagctcaaacgtgggtagggatgtgggagaataagaatgtgggagaaccaagagaaaaagtggggctgggagagtggagttcccgtagggcataggcctgtgaagtaacactggggcagatatgtatgttatatacaactatttttttaaaaaacttatatccatgttgggagtagatgggtatataacagtttggaaatactatctttggagaatgtatttttgtatttataaatcaacttttaaaaactgtctcattcaaaagggaataaagacctgtgttatcaatgtgtcattttcttctttcctccataactgtaccttgaaaccttactgctgacctgcagaaaatgtgccgcgttatgtacctggctcatcttcaacacactaaccatgaacactaatagccattaggggacatggctacagatactacattggaaagttgtctttaatcacacaggtgttaaactcaatataaatttacctaaaaacaattgctatacctaaaaggagttctgggtactaagggtagaagcctcactggctacagttttttaatagtacaaaagtcaagaaataacacaatagtgactataacctgtattcaaatccctactctgtcactacttgatctgggctgatatggtatggctctgtgtcctcacccaaatctaaccttgaattgtagcaatccccacgtgtcaagggtgggaccaggtggaggtaactggatcatgggggcggtttcctccatgctgttcctgtgatagtgagccggtctcatgagatctgaaggttttataagcgtctggcatttccactgctggcagtcattttcatcctgccgccctgtgaaaaaggtgcctgcttctcctttttctgccatgattgtgtaagtgtcctgaggcctcaccagcaatgcggaactgagtccattaaacctctttcctttataataattacccagtttggggtatttcttcgtagcagtgtgagaacagaccataaacctccattttctcatctgttaaatggagataacagtcctggcttaacagggctttttgagttaagtgatatattccacgtaacctgcttagcataagaactggcactagaaacagaacattttagattatggaatagaacttaggggaaaatagcaaagtctctgatcatcttgaactactcaattgggacttatccctgaattaaacctttctagtagctgaagcacaagaaaataaacttggaaagaaaaaacctaaggccagtcatgcactgccctacttccctttcttctctattgcaggttaactatggcctgtaggcagtttttcttctctttttttttttttgagacagtcttgttctgtcacccaggctggagtgcagtggcgcgatcttggctcactgcaacctctgcctcccaggttcaagcgattctcctgcctcagcctcctgaggtgggattaaaggcacttgccaccacacctggctaattttcttttctttttttttttttttttttgcgatggagtctcactctcatcatccaggctgaactgcagtggtgcaatctcggctcactgcaacttccgcctcccaggttcaagcgattctcctgcctcagcctcccaagtagctgggattacaggcatccgccgttacacccagctaagtttttgtatttttagtagagacggcgttttaccatgttggccaggctggtctcaaactcctgacatcgagtgatccacccgcctcgtcctcccaaaatgctaggattacaggcatgagccaccgcacctagccggcaaacttttttaaatggttggcgggggtgggggaaatcaaatgagtaatgttttgtgacacatcaaaattataatgatgtgctgcataacttttggtcaacaatggccaaatatacgatgatgatcccgtaagattacaatggagctgaaaaattcctattgcctggggacacagccatggtaacatcatagtgaaattactttatgtagcctaagtatatagtgtttataaaagtctacagtagtgcacagtaatatcatggccttcacattcactaaccacttactgactcacccagagccagcttccagtcctgccaacttgttcatggtaaatgtcctaaataggtgtaccattttatatcttatatatatctatatatatatttttactgtaccttttctatgtttagatatgtttagatacacaaatacttagcactgtgttacaaccgcctacagtaatcagtacagtaatatgccatacaggtttgtaggttaggagcaataggctatcccatataggataccatagggtataccatctaggtttgtgtaactacatcatgattttcacacaatgatgaaattgccaagtgacatgtctcagaacatatccctgtcattaagtgacatatgactatatatgaaacttaacaaatcaggccttgttgaaacacagtcatgttgatttgtttacatattgtatatggctccttacacactatcaacggcagagttgtgtactatagttgcaatacagaccatagccaacaaagtctaaaatgttctagcacttcacagaaaaggttttttgactcctactctactgtttcagtgtcactgacccattttacctggaccaaagactactcaagtctattttcctccaactgacacaagtttctgcctcagtgtatggaggttttcctcagtaataggaaactggaaaaattagtcaacatttattgagtgcctaaatgactacctatttagtatacctgctgatttacttggcaggcttttctcactatactgcaagctccttgaaggcagagataatttacttgagtggaacctggcacaacgtaagtgctttagaaattgaataagccaagtaaaatgttttaaggcaaccctatcccaaaatattcctgaagatattaatttaatcattactaatctctgtgattagcaagggaagtagtcagtctggcacaccaaattttattaataatacttattttaatctgttccctttagtatgtctttatacagttcccctcgtgtatatacactgatataactacaatttaaaagccactaattaatctgttttttattttgtaagtaacaagatatagacatttgaatgccaatgtcttattctggagagacactggagctgaagttcaacaatgatcacacttattacctggcaataaaaacacaaccatctttccagtcaggtcaaaatatcctactttttgcctttctaccaattcccaaacattcacagtttttcaaggaccactaataaaatacaggaagcttttaaagacagtaagagaacacctagtgtaagttaggtgaattaaagatggcaaaggagattacatcctcaacactgacagcttccaagacttagaaaagagattgttccttgcttctaaaattgttctattttcctctgtaggaaaatgaaagttttttcttacaaatattaaataatcaaagtacttacgcaaaattaatctgctcctcaatgagatgagcactccatttaaatgatctttacagatccctgaagttgctgtcctgtcactgtatttaagtgatggatattcaattgaattattctgcataaataattctgttcaacccagaagtatagtagtatgatgggtcagatacagtcaactgttcaataaaaatgcagatgtctgaaattattaaaatgtacttaaaagtaacaaactgtatcacacacttaggcttagaagtgttctttcaagttttttcttttaaaaaagaaaccagtctttgaagatttttgttgaatatagctattttccaagcttcatcttctttttctttggtccattaaggtccatgtttgaagtatcagtaggaatgcttattcctggtatctgtggttctaccagggacattcggatcttctgatgttgaagattagatgagtctaacatgattttcactttaactttatcaaatacatggaacactgtatcttctattttaagtgagggtatctcatcatcataaataagctgtgggtttggtttgtccttttcttcaaaaaagactgtcccttctaaaccatactttggaattaataccacaatggcattctttcttacaaataaaatataggcttcttcacttactattcctttgcttttgaagaataactgggtatgaaaagccactgatgcacgttgggcatattgagccattttgtgccggaaatttagatttttacatatatctgcaagcttgtgtttgtctgtcaactctggataagtacagtcagccccaatagccacagccaaaagccgatgaacaatgacatctgcgtatcttctaatgggtgaagtaaaatgtgtgtatattggagacgctaagccatagtgatgaaaatcattatccattccagaacagaagtacacagcttgcatcatacagcgagtggctaatattctcaacagagtgtttagatatggaaaagtaggagattcggcctgatccaaagactcagccaaagacttggctgtatcagtcttaatttccaaattccttgacctggctgccttaacaagaatttcataatttgatggaggtggagcaggatgttttcgaagcagagcatgttcagaaaattcctcatgaattttttttgcaacagaaatattggcaagtaacataaattcttcaaccatggaatttgtttccctaagttccttggtctgcagatctataggatcgtgagtttcactgtccatgtggaatcgaacttcaggagaggatagagtcaaagcccctttttcaatccttcttttcttcagaattttggctagtttattcagtccacggagactagtggtaatatcatcattcatgtttgctgaatcaattctcaactgagcttcagcatacgtcagagatgcctttgaattaataacacttttggtaaacttcgtttttaagatttcagcattgtgattcatttcccaaatacatgaaaatgccagcctgtccacgtcacattttaaggaacacaagttagagctaagcaactctggaaccatgtcaatcctcttttcacaaagatacacagttgttcctcttctggctgattcttgatccaaggcatttcctggcctaataaaatggctcacatcagcaatatgaacaccaacctccaaatttccattttcgagttctcgacaatgtagagcatcgtctatatcagtacatcctggtgggtctacactacaaatacacagatgcctcaggtcttctcggtttttcatgtccttttcagtaatgctccagggcatctttggcagaaaactaagaacagcctgtgaaaaaggctgatggggaacatcgtgttcaagtaacaaaacttctgtttcagtctctttctctccaacatcacctaaatttctcacaaagtgtccatttggatatctggaatttctgggccaaccatcaatagcaacaataattctccgtccttctaatgtggaagcctgtctggtttctatgcgaattcgagggattctcttatcagcaggtgtaaagagatgtcttcttgactccttaatgtcagacttggaaagcatgccacaatatggtctccaattcctttttattattcctacaactctacctgtaggcttcaacattttctcgcttacagcagtcttaagcattcgttctgtctcttcttctttctccacatcttcttcattttgaccttcatcatgtaaaaccacagaagatggtgctacccactgactcttggggagaagctccacagccacaatatcttcgtgaacagctctgtttaaatgtttaagtccctgtaagattatctctttattttcttcattgtcgccatgaatccatactgtagcttccaagtaattttccctgctagctctaaatgttccttgaaggtatgtaccagattttatgccttgctgtagcttacttaagggaagatgctctgaaaatattatttttccactttctatttcattcccttcttcagacaaacaagcaagacgatctatgagttcggggttagcagttaggctctttacatattcttcacaagtgaaagctggtattccttcttctatggctttctctttgtttctcctgtcatttgttatgaagataacttgcagctggttgtctgctgacatttttttcaaatgttcattgtaccattttgctgctactcgaatcgctctatcattcctgtcattagcattttctccctgttcttgttctacataggtttctaagctgcctgggagtcgcaggctggaggccacagaagcccaggtccccggcctccaggcacttacaatctggtgcagtaacacattagtgtcgggcagcaagtagtgcggttgcgggcagacgctgctcgccgggtcctggggctgcggctccagggccggcccctcgtgcgcccctccacacgctgcgcacccgggcgcaccgcagccgatgtcgtctcgcaggtagtgctcgcgcacgatcttcatcacgccgcccgcccgggtcttttttaagaacgtcttggacttgagcatcttgcctcgccgcgcagaatcctaaccccagcagcgctcttccagcaaaaggcgtcaatctagaatac

SEQ ID NO: 12858 - RNA, 8551 nt, Homo sapiens
  source 1..8551: mol_type = other RNA
gctgggattacaggcatgagccaacatgcccagccttgtatgccgtttcttttttttctttttttttttttttgagacagggtcttactctgtcacccgggctggagtgcagtcgtagaatcagatcactacagcctttaactgctgggctcaagcaatcctcctgcctcaccctcctgagtagctagaactacaggtgtgaaccaccttgccctgctgttatatgccagtttcttataaaatactataaatatcagcaaatgtgcaacaaatgtttaatagggaggccaccttagttttcctttctgttgtatgtagtaggagcaaactgcctttctgttgtatgtagtatcagagcaggtctcttctaatattaacctgaacaaaatccatcctatttcaggatgcagttgtctatctaaacataagtagagataaatgaaggatttttttaaattttattattttattttttttgagacaaggtctcattctgtcacccaggctagagtgtagtggcacgaccacagctcactgtagccttcacctcccagactcaagcagtcttaccacctcagcctcctgagtagctagggctacaggcatgtgccaccacacccagctttttaaaatttttggtagagacagggtctcactatgttgccagggctagtcccaaactcctgggctcgtgcgatcctcccaccttggcctctcaaagtgttgggatgctttttgatgcagaatattgatttataaaatactgtatctttactgtcccttcagagttcagctaaagaaacgtgcttttaggttttaaaaacagtcccgataattgcatcctccagtggtcctacttaaactgaaaacaaggtattgtcttctttttcacagcaagaccacacaacacagaggtgttggatgaaaacagcaagcccttttcaatgcagcagtccatagaatgcctctgtcagaatcaaagactaagcttaagagttcctcgcatatatcgttgtgcacaggatcaacatgatggtgactgggaaaaaattacttcaagtaacatgcttagctttccctccttaatgtgaaaaatcaagggcttactgacataggaacaacagaaatgctcctggaacttcaagttgctgaattataagtttattttttatcaataaatatttttatacttacattgagtgatgtgtttaacaacaaattgtgacagagctgagtgctcctatcttacagggtcaatgaactacttattaagccttactggtagcactgaatttagcagttctgagaacatgtgaaactatgttaaaactgaaggcactatatatttttacataaaagcttgaacatacagatgaattataacctatgtgaagaaatcttagatataaaactaacttttcaaagatacaaaagaaattaaacaggtttcctgaaattttagttcttggtctgttcacctctgtggggaaaattcttagttccagtgataactgttctagttactacttttaagtatgtaaatactagaaaggtagtactagtgacatcatcacgtgtattgttatctatggggcaaatgtgtggtgcccagaataaaatatacctcatgcctagggtagggacatcctttccagctcaaacgtgggtagggatgtgggagaataagaatgtgggagaaccaagagaaaaagtggggctgggagagtggagttcccgtagggcataggcctgtgaagtaacactggggcagatatgtatgttatatacaactatttttttaaaaaacttatatccatgttgggagtagatgggtatataacagtttggaaatactatctttggagaatgtatttttgtatttataaatcaacttttaaaaactgtctcattcaaaagggaataaagacctgtgttatcaatgtgtcattttcttctttcctccataactgtaccttgaaaccttactgctgacctgcagaaaatgtgccgcgttatgtacctggctcatcttcaacacactaaccatgaacactaatagccattaggggacatggctacagatactacattggaaagttgtctttaatcacacaggtgttaaactcaatataaatttacctaaaaacaattgctatacctaaaaggagttctgggtactaagggtagaagcctcactggctacagttttttaatagtacaaaagtcaagaaataacacaatagtgactataacctgtattcaaatccctactctgtcactacttgatctgggctgatatggtatggctctgtgtcctcacccaaatctaaccttgaattgtagcaatccccacgtgtcaagggtgggaccaggtggaggtaactggatcatgggggcggtttcctccatgctgttcctgtgatagtgagccggtctcatgagatctgaaggttttataagcgtctggcatttccactgctggcagtcattttcatcctgccgccctgtgaaaaaggtgcctgcttctcctttttctgccatgattgtgtaagtgtcctgaggcctcaccagcaatgcggaactgagtccattaaacctctttcctttataataattacccagtttggggtatttcttcgtagcagtgtgagaacagaccataaacctccattttctcatctgttaaatggagataacagtcctggcttaacagggctttttgagttaagtgatatattccacgtaacctgcttagcataagaactggcactagaaacagaacattttagattatggaatagaacttaggggaaaatagcaaagtctctgatcatcttgaactactcaattgggacttatccctgaattaaacctttctagtagctgaagcacaagaaaataaacttggaaagaaaaaacctaaggccagtcatgcactgccctacttccctttcttctctattgcaggttaactatggcctgtaggcagtttttcttctctttttttttttttgagacagtcttgttctgtcacccaggctggagtgcagtggcgcgatcttggctcactgcaacctctgcctcccaggttcaagcgattctcctgcctcagcctcctgaggtgggattaaaggcacttgccaccacacctggctaattttcttttctttttttttttttttttttgcgatggagtctcactctcatcatccaggctgaactgcagtggtgcaatctcggctcactgcaacttccgcctcccaggttcaagcgattctcctgcctcagcctcccaagtagctgggattacaggcatccgccgttacacccagctaagtttttgtatttttagtagagacggcgttttaccatgttggccaggctggtctcaaactcctgacatcgagtgatccacccgcctcgtcctcccaaaatgctaggattacaggcatgagccaccgcacctagccggcaaacttttttaaatggttggcgggggtgggggaaatcaaatgagtaatgttttgtgacacatcaaaattataatgatgtgctgcataacttttggtcaacaatggccaaatatacgatgatgatcccgtaagattacaatggagctgaaaaattcctattgcctggggacacagccatggtaacatcatagtgaaattactttatgtagcctaagtatatagtgtttataaaagtctacagtagtgcacagtaatatcatggccttcacattcactaaccacttactgactcacccagagccagcttccagtcctgccaacttgttcatggtaaatgtcctaaataggtgtaccattttatatcttatatatatctatatatatatttttactgtaccttttctatgtttagatatgtttagatacacaaatacttagcactgtgttacaaccgcctacagtaatcagtacagtaatatgccatacaggtttgtaggttaggagcaataggctatcccatataggataccatagggtataccatctaggtttgtgtaactacatcatgattttcacacaatgatgaaattgccaagtgacatgtctcagaacatatccctgtcattaagtgacatatgactatatatgaaacttaacaaatcaggccttgttgaaacacagtcatgttgatttgtttacatattgtatatggctccttacacactatcaacggcagagttgtgtactatagttgcaatacagaccatagccaacaaagtctaaaatgttctagcacttcacagaaaaggttttttgactcctactctactgtttcagtgtcactgacccattttacctggaccaaagactactcaagtctattttcctccaactgacacaagtttctgcctcagtgtatggaggttttcctcagtaataggaaactggaaaaattagtcaacatttattgagtgcctaaatgactacctatttagtatacctgctgatttacttggcaggcttttctcactatactgcaagctccttgaaggcagagataatttacttgagtggaacctggcacaacgtaagtgctttagaaattgaataagccaagtaaaatgttttaaggcaaccctatcccaaaatattcctgaagatattaatttaatcattactaatctctgtgattagcaagggaagtagtcagtctggcacaccaaattttattaataatacttattttaatctgttccctttagtatgtctttatacagttcccctcgtgtatatacactgatataactacaatttaaaagccactaattaatctgttttttattttgtaagtaacaagatatagacatttgaatgccaatgtcttattctggagagacactggagctgaagttcaacaatgatcacacttattacctggcaataaaaacacaaccatctttccagtcaggtcaaaatatcctactttttgcctttctaccaattcccaaacattcacagtttttcaaggaccactaataaaatacaggaagcttttaaagacagtaagagaacacctagtgtaagttaggtgaattaaagatggcaaaggagattacatcctcaacactgacagcttccaagacttagaaaagagattgttccttgcttctaaaattgttctattttcctctgtaggaaaatgaaagttttttcttacaaatattaaataatcaaagtacttacgcaaaattaatctgctcctcaatgagatgagcactccatttaaatgatctttacagatccctgaagttgctgtcctgtcactgtatttaagtgatggatattcaattgaattattctgcataaataattctgttcaacccagaagtatagtagtatgatgggtcagatacagtcaactgttcaataaaaatgcagatgtctgaaattattaaaatgtacttaaaagtaacaaactgtatcacacacttaggcttagaagtgttctttcaagttttttcttttaaaaaagaaaccagtctttgaagatttttgttgaatatagctattttccaagcttcatcttctttttctttggtccattaaggtccatgtttgaagtatcagtaggaatgcttattcctggtatctgtggttctaccagggacattcggatcttctgatgttgaagattagatgagtctaacatgattttcactttaactttatcaaatacatggaacactgtatcttctattttaagtgagggtatctcatcatcataaataagctgtgggtttggtttgtccttttcttcaaaaaagactgtcccttctaaaccatactttggaattaataccacaatggcattctttcttacaaataaaatataggcttcttcacttactattcctttgcttttgaagaataactgggtatgaaaagccactgatgcacgttgggcatattgagccattttgtgccggaaatttagatttttacatatatctgcaagcttgtgtttgtctgtcaactctggataagtacagtcagccccaatagccacagccaaaagccgatgaacaatgacatctgcgtatcttctaatgggtgaagtaaaatgtgtgtatattggagacgctaagccatagtgatgaaaatcattatccattccagaacagaagtacacagcttgcatcatacagcgagtggctaatattctcaacagagtgtttagatatggaaaagtaggagattcggcctgatccaaagactcagccaaagacttggctgtatcagtcttaatttccaaattccttgacctggctgccttaacaagaatttcataatttgatggaggtggagcaggatgttttcgaagcagagcatgttcagaaaattcctcatgaattttttttgcaacagaaatattggcaagtaacataaattcttcaaccatggaatttgtttccctaagttccttggtctgcagatctataggatcgtgagtttcactgtccatgtggaatcgaacttcaggagaggatagagtcaaagcccctttttcaatccttcttttcttcagaattttggctagtttattcagtccacggagactagtggtaatatcatcattcatgtttgctgaatcaattctcaactgagcttcagcatacgtcagagatgcctttgaattaataacacttttggtaaacttcgtttttaagatttcagcattgtgattcatttcccaaatacatgaaaatgccagcctgtccacgtcacattttaaggaacacaagttagagctaagcaactctggaaccatgtcaatcctcttttcacaaagatacacagttgttcctcttctggctgattcttgatccaaggcatttcctggcctaataaaatggctcacatcagcaatatgaacaccaacctccaaatttccattttcgagttctcgacaatgtagagcatcgtctatatcagtacatcctggtgggtctacactacaaatacacagatgcctcaggtcttctcggtttttcatgtccttttcagtaatgctccagggcatctttggcagaaaactaagaacagcctgtgaaaaaggctgatggggaacatcgtgttcaagtaacaaaacttctgtttcagtctctttctctccaacatcacctaaatttctcacaaagtgtccatttggatatctggaatttctgggccaaccatcaatagcaacaataattctccgtccttctaatgtggaagcctgtctggtttctatgcgaattcgagggattctcttatcagcaggtgtaaagagatgtcttcttgactccttaatgtcagacttggaaagcatgccacaatatggtctccaattcctttttattattcctacaactctacctgtaggcttcaacattttctcgcttacagcagtcttaagcattcgttctgtctcttcttctttctccacatcttcttcattttgaccttcatcatgtaaaaccacagaagatggtgctacccactgactcttggggagaagctccacagccacaatatcttcgtgaacagctctgtttaaatgtttaagtccctgtaagattatctctttattttcttcattgtcgccatgaatccatactgtagcttccaagtaattttccctgctagctctaaatgttccttgaaggtatgtaccagattttatgccttgctgtagcttacttaagggaagatgctctgaaaatattatttttccactttctatttcattcccttcttcagacaaacaagcaagacgatctatgagttcggggttagcagttaggctctttacatattcttcacaagtgaaagctggtattccttcttctatggctttctctttgtttctcctgtcatttgttatgaagataacttgcagctggttgtctgctgacatttttttcaaatgttcattgtaccattttgctgctactcgaatcgctctatcattcctgtcattagcattttctccctgttcttgttctacataggtttctctatggtgctcattagtgaaagtatagaaatgcttctcttggttattagtcacatctcggatgcgtttatatacgggggcactgcgatttctcacttcttgaagaactgtttgtagcacaattacattcctgatggcagggtcctcaagaacatcaataagctgcctgggagtcgcaggctggaggccacagaagcccaggtccccggcctccaggcacttacaatctggtgcagtaacacattagtgtcgggcagcaagtagtgcggttgcgggcagacgctgctcgccgggtcctggggctgcggctccagggccggcccctcgtgcgcccctccacacgctgcgcacccgggcgcaccgcagccgatgtcgtctcgcaggtagtgctcgcgcacgatcttcatcacgccgcccgcccgggtcttttttaagaacgtcttggacttgagcatcttgcctcgccgcgcagaatcctaaccccagcagcgctcttccagcaaaaggcgtcaatctagaatac

SEQ ID NO: 12859 - RNA, 8483 nt, Homo sapiens
  source 1..8483: mol_type = other RNA
gctgggattacaggcatgagccaacatgcccagccttgtatgccgtttcttttttttctttttttttttttttgagacagggtcttactctgtcacccgggctggagtgcagtcgtagaatcagatcactacagcctttaactgctgggctcaagcaatcctcctgcctcaccctcctgagtagctagaactacaggtgtgaaccaccttgccctgctgttatatgccagtttcttataaaatactataaatatcagcaaatgtgcaacaaatgtttaatagggaggccaccttagttttcctttctgttgtatgtagtaggagcaaactgcctttctgttgtatgtagtatcagagcaggtctcttctaatattaacctgaacaaaatccatcctatttcaggatgcagttgtctatctaaacataagtagagataaatgaaggatttttttaaattttattattttattttttttgagacaaggtctcattctgtcacccaggctagagtgtagtggcacgaccacagctcactgtagccttcacctcccagactcaagcagtcttaccacctcagcctcctgagtagctagggctacaggcatgtgccaccacacccagctttttaaaatttttggtagagacagggtctcactatgttgccagggctagtcccaaactcctgggctcgtgcgatcctcccaccttggcctctcaaagtgttgggatgctttttgatgcagaatattgatttataaaatactgtatctttactgtcccttcagagttcagctaaagaaacgtgcttttaggttttaaaaacagtcccgataattgcatcctccagtggtcctacttaaactgaaaacaaggtattgtcttctttttcacagcaagaccacacaacacagaggtgttggatgaaaacagcaagcccttttcaatgcagcagtccatagaatgcctctgtcagaatcaaagactaagcttaagagttcctcgcatatatcgttgtgcacaggatcaacatgatggtgactgggaaaaaattacttcaagtaacatgcttagctttccctccttaatgtgaaaaatcaagggcttactgacataggaacaacagaaatgctcctggaacttcaagttgctgaattataagtttattttttatcaataaatatttttatacttacattgagtgatgtgtttaacaacaaattgtgacagagctgagtgctcctatcttacagggtcaatgaactacttattaagccttactggtagcactgaatttagcagttctgagaacatgtgaaactatgttaaaactgaaggcactatatatttttacataaaagcttgaacatacagatgaattataacctatgtgaagaaatcttagatataaaactaacttttcaaagatacaaaagaaattaaacaggtttcctgaaattttagttcttggtctgttcacctctgtggggaaaattcttagttccagtgataactgttctagttactacttttaagtatgtaaatactagaaaggtagtactagtgacatcatcacgtgtattgttatctatggggcaaatgtgtggtgcccagaataaaatatacctcatgcctagggtagggacatcctttccagctcaaacgtgggtagggatgtgggagaataagaatgtgggagaaccaagagaaaaagtggggctgggagagtggagttcccgtagggcataggcctgtgaagtaacactggggcagatatgtatgttatatacaactatttttttaaaaaacttatatccatgttgggagtagatgggtatataacagtttggaaatactatctttggagaatgtatttttgtatttataaatcaacttttaaaaactgtctcattcaaaagggaataaagacctgtgttatcaatgtgtcattttcttctttcctccataactgtaccttgaaaccttactgctgacctgcagaaaatgtgccgcgttatgtacctggctcatcttcaacacactaaccatgaacactaatagccattaggggacatggctacagatactacattggaaagttgtctttaatcacacaggtgttaaactcaatataaatttacctaaaaacaattgctatacctaaaaggagttctgggtactaagggtagaagcctcactggctacagttttttaatagtacaaaagtcaagaaataacacaatagtgactataacctgtattcaaatccctactctgtcactacttgatctgggctgatatggtatggctctgtgtcctcacccaaatctaaccttgaattgtagcaatccccacgtgtcaagggtgggaccaggtggaggtaactggatcatgggggcggtttcctccatgctgttcctgtgatagtgagccggtctcatgagatctgaaggttttataagcgtctggcatttccactgctggcagtcattttcatcctgccgccctgtgaaaaaggtgcctgcttctcctttttctgccatgattgtgtaagtgtcctgaggcctcaccagcaatgcggaactgagtccattaaacctctttcctttataataattacccagtttggggtatttcttcgtagcagtgtgagaacagaccataaacctccattttctcatctgttaaatggagataacagtcctggcttaacagggctttttgagttaagtgatatattccacgtaacctgcttagcataagaactggcactagaaacagaacattttagattatggaatagaacttaggggaaaatagcaaagtctctgatcatcttgaactactcaattgggacttatccctgaattaaacctttctagtagctgaagcacaagaaaataaacttggaaagaaaaaacctaaggccagtcatgcactgccctacttccctttcttctctattgcaggttaactatggcctgtaggcagtttttcttctctttttttttttttgagacagtcttgttctgtcacccaggctggagtgcagtggcgcgatcttggctcactgcaacctctgcctcccaggttcaagcgattctcctgcctcagcctcctgaggtgggattaaaggcacttgccaccacacctggctaattttcttttctttttttttttttttttttgcgatggagtctcactctcatcatccaggctgaactgcagtggtgcaatctcggctcactgcaacttccgcctcccaggttcaagcgattctcctgcctcagcctcccaagtagctgggattacaggcatccgccgttacacccagctaagtttttgtatttttagtagagacggcgttttaccatgttggccaggctggtctcaaactcctgacatcgagtgatccacccgcctcgtcctcccaaaatgctaggattacaggcatgagccaccgcacctagccggcaaacttttttaaatggttggcgggggtgggggaaatcaaatgagtaatgttttgtgacacatcaaaattataatgatgtgctgcataacttttggtcaacaatggccaaatatacgatgatgatcccgtaagattacaatggagctgaaaaattcctattgcctggggacacagccatggtaacatcatagtgaaattactttatgtagcctaagtatatagtgtttataaaagtctacagtagtgcacagtaatatcatggccttcacattcactaaccacttactgactcacccagagccagcttccagtcctgccaacttgttcatggtaaatgtcctaaataggtgtaccattttatatcttatatatatctatatatatatttttactgtaccttttctatgtttagatatgtttagatacacaaatacttagcactgtgttacaaccgcctacagtaatcagtacagtaatatgccatacaggtttgtaggttaggagcaataggctatcccatataggataccatagggtataccatctaggtttgtgtaactacatcatgattttcacacaatgatgaaattgccaagtgacatgtctcagaacatatccctgtcattaagtgacatatgactatatatgaaacttaacaaatcaggccttgttgaaacacagtcatgttgatttgtttacatattgtatatggctccttacacactatcaacggcagagttgtgtactatagttgcaatacagaccatagccaacaaagtctaaaatgttctagcacttcacagaaaaggttttttgactcctactctactgtttcagtgtcactgacccattttacctggaccaaagactactcaagtctattttcctccaactgacacaagtttctgcctcagtgtatggaggttttcctcagtaataggaaactggaaaaattagtcaacatttattgagtgcctaaatgactacctatttagtatacctgctgatttacttggcaggcttttctcactatactgcaagctccttgaaggcagagataatttacttgagtggaacctggcacaacgtaagtgctttagaaattgaataagccaagtaaaatgttttaaggcaaccctatcccaaaatattcctgaagatattaatttaatcattactaatctctgtgattagcaagggaagtagtcagtctggcacaccaaattttattaataatacttattttaatctgttccctttagtatgtctttatacagttcccctcgtgtatatacactgatataactacaatttaaaagccactaattaatctgttttttattttgtaagtaacaagatatagacatttgaatgccaatgtcttattctggagagacactggagctgaagttcaacaatgatcacacttattacctggcaataaaaacacaaccatctttccagtcaggtcaaaatatcctactttttgcctttctaccaattcccaaacattcacagtttttcaaggaccactaataaaatacaggaagcttttaaagacagtaagagaacacctagtgtaagttaggtgaattaaagatggcaaaggagattacatcctcaacactgacagcttccaagacttagaaaagagattgttccttgcttctaaaattgttctattttcctctgtaggaaaatgaaagttttttcttacaaatattaaataatcaaagtacttacgcaaaattaatctgctcctcaatgagatgagcactccatttaaatgatctttacagatccctgaagttgctgtcctgtcactgtatttaagtgatggatattcaattgaattattctgcataaataattctgttcaacccagaagtatagtagtatgatgggtcagatacagtcaactgttcaataaaaatgcagatgtctgaaattattaaaatgtacttaaaagtaacaaactgtatcacacacttaggcttagaagtgttctttcaagttttttcttttaaaaaagaaaccagtctttgaagatttttgttgaatatagctattttccaagcttcatcttctttttctttggtccattaaggtccatgtttgaagtatcagtaggaatgcttattcctggtatctgtggttctaccagggacattcggatcttctgatgttgaagattagatgagtctaacatgattttcactttaactttatcaaatacatggaacactgtatcttctattttaagtgagggtatctcatcatcataaataagctgtgggtttggtttgtccttttcttcaaaaaagactgtcccttctaaaccatactttggaattaataccacaatggcattctttcttacaaataaaatataggcttcttcacttactattcctttgcttttgaagaataactgggtatgaaaagccactgatgcacgttgggcatattgagccattttgtgccggaaatttagatttttacatatatctgcaagcttgtgtttgtctgtcaactctggataagtacagtcagccccaatagccacagccaaaagccgatgaacaatgacatctgcgtatcttctaatgggtgaagtaaaatgtgtgtatattggagacgctaagccatagtgatgaaaatcattatccattccagaacagaagtacacagcttgcatcatacagcgagtggctaatattctcaacagagtgtttagatatggaaaagtaggagattcggcctgatccaaagactcagccaaagacttggctgtatcagtcttaatttccaaattccttgacctggctgccttaacaagaatttcataatttgatggaggtggagcaggatgttttcgaagcagagcatgttcagaaaattcctcatgaattttttttgcaacagaaatattggcaagtaacataaattcttcaaccatggaatttgtttccctaagttccttggtctgcagatctataggatcgtgagtttcactgtccatgtggaatcgaacttcaggagaggatagagtcaaagcccctttttcaatccttcttttcttcagaattttggctagtttattcagtccacggagactagtggtaatatcatcattcatgtttgctgaatcaattctcaactgagcttcagcatacgtcagagatgcctttgaattaataacacttttggtaaacttcgtttttaagatttcagcattgtgattcatttcccaaatacatgaaaatgccagcctgtccacgtcacattttaaggaacacaagttagagctaagcaactctggaaccatgtcaatcctcttttcacaaagatacacagttgttcctcttctggctgattcttgatccaaggcatttcctggcctaataaaatggctcacatcagcaatatgaacaccaacctccaaatttccattttcgagttctcgacaatgtagagcatcgtctatatcagtacatcctggtgggtctacactacaaatacacagatgcctcaggtcttctcggtttttcatgtccttttcagtaatgctccagggcatctttggcagaaaactaagaacagcctgtgaaaaaggctgatggggaacatcgtgttcaagtaacaaaacttctgtttcagtctctttctctccaacatcacctaaatttctcacaaagtgtccatttggatatctggaatttctgggccaaccatcaatagcaacaataattctccgtccttctaatgtggaagcctgtctggtttctatgcgaattcgagggattctcttatcagcaggtgtaaagagatgtcttcttgactccttaatgtcagacttggaaagcatgccacaatatggtctccaattcctttttattattcctacaactctacctgtaggcttcaacattttctcgcttacagcagtcttaagcattcgttctgtctcttcttctttctccacatcttcttcattttgaccttcatcatgtaaaaccacagaagatggtgctacccactgactcttggggagaagctccacagccacaatatcttcgtgaacagctctgtttaaatgtttaagtccctgtaagattatctctttattttcttcattgtcgccatgaatccatactgtagcttccaagtaattttccctgctagctctaaatgttccttgaaggtatgtaccagattttatgccttgctgtagcttacttaagggaagatgctctgaaaatattatttttccactttctatttcattcccttcttcagacaaacaagcaagacgatctatgagttcggggttagcagttaggctctttacatattcttcacaagtgaaagctggtattccttcttctatggctttctctttgtttctcctgtcatttgttatgaagataacttgcagctggttgtctgctgacatttttttcaaatgttcattgtaccattttgctgctactcgaatcgctctatcattcctgtcattagcattttctccctgttcttgttctacataggtttctctatggtgctcattagtgaaagtatagaaatgcttctcttggttattagtcacatctcggatgcgtttatatacgggggcactgcgatttctcacttcttgaagaactgtttgtagcacaattacattcctgatggcagggtcctcaagaacatcaatctggtgcagtaacacattagtgtcgggcagcaagtagtgcggttgcgggcagacgctgctcgccgggtcctggggctgcggctccagggccggcccctcgtgcgcccctccacacgctgcgcacccgggcgcaccgcagccgatgtcgtctcgcaggtagtgctcgcgcacgatcttcatcacgccgcccgcccgggtcttttttaagaacgtcttggacttgagcatcttgcctcgccgcgcagaatcctaaccccagcagcgctcttccagcaaaaggcgtcaatctagaatac

SEQ ID NO: 12860 - RNA, 8325 nt, Homo sapiens
  source 1..8325: mol_type = other RNA
gctgggattacaggcatgagccaacatgcccagccttgtatgccgtttcttttttttctttttttttttttttgagacagggtcttactctgtcacccgggctggagtgcagtcgtagaatcagatcactacagcctttaactgctgggctcaagcaatcctcctgcctcaccctcctgagtagctagaactacaggtgtgaaccaccttgccctgctgttatatgccagtttcttataaaatactataaatatcagcaaatgtgcaacaaatgtttaatagggaggccaccttagttttcctttctgttgtatgtagtaggagcaaactgcctttctgttgtatgtagtatcagagcaggtctcttctaatattaacctgaacaaaatccatcctatttcaggatgcagttgtctatctaaacataagtagagataaatgaaggatttttttaaattttattattttattttttttgagacaaggtctcattctgtcacccaggctagagtgtagtggcacgaccacagctcactgtagccttcacctcccagactcaagcagtcttaccacctcagcctcctgagtagctagggctacaggcatgtgccaccacacccagctttttaaaatttttggtagagacagggtctcactatgttgccagggctagtcccaaactcctgggctcgtgcgatcctcccaccttggcctctcaaagtgttgggatgctttttgatgcagaatattgatttataaaatactgtatctttactgtcccttcagagttcagctaaagaaacgtgcttttaggttttaaaaacagtcccgataattgcatcctccagtggtcctacttaaactgaaaacaaggtattgtcttctttttcacagcaagaccacacaacacagaggtgttggatgaaaacagcaagcccttttcaatgcagcagtccatagaatgcctctgtcagaatcaaagactaagcttaagagttcctcgcatatatcgttgtgcacaggatcaacatgatggtgactgggaaaaaattacttcaagtaacatgcttagctttccctccttaatgtgaaaaatcaagggcttactgacataggaacaacagaaatgctcctggaacttcaagttgctgaattataagtttattttttatcaataaatatttttatacttacattgagtgatgtgtttaacaacaaattgtgacagagctgagtgctcctatcttacagggtcaatgaactacttattaagccttactggtagcactgaatttagcagttctgagaacatgtgaaactatgttaaaactgaaggcactatatatttttacataaaagcttgaacatacagatgaattataacctatgtgaagaaatcttagatataaaactaacttttcaaagatacaaaagaaattaaacaggtttcctgaaattttagttcttggtctgttcacctctgtggggaaaattcttagttccagtgataactgttctagttactacttttaagtatgtaaatactagaaaggtagtactagtgacatcatcacgtgtattgttatctatggggcaaatgtgtggtgcccagaataaaatatacctcatgcctagggtagggacatcctttccagctcaaacgtgggtagggatgtgggagaataagaatgtgggagaaccaagagaaaaagtggggctgggagagtggagttcccgtagggcataggcctgtgaagtaacactggggcagatatgtatgttatatacaactatttttttaaaaaacttatatccatgttgggagtagatgggtatataacagtttggaaatactatctttggagaatgtatttttgtatttataaatcaacttttaaaaactgtctcattcaaaagggaataaagacctgtgttatcaatgtgtcattttcttctttcctccataactgtaccttgaaaccttactgctgacctgcagaaaatgtgccgcgttatgtacctggctcatcttcaacacactaaccatgaacactaatagccattaggggacatggctacagatactacattggaaagttgtctttaatcacacaggtgttaaactcaatataaatttacctaaaaacaattgctatacctaaaaggagttctgggtactaagggtagaagcctcactggctacagttttttaatagtacaaaagtcaagaaataacacaatagtgactataacctgtattcaaatccctactctgtcactacttgatctgggctgatatggtatggctctgtgtcctcacccaaatctaaccttgaattgtagcaatccccacgtgtcaagggtgggaccaggtggaggtaactggatcatgggggcggtttcctccatgctgttcctgtgatagtgagccggtctcatgagatctgaaggttttataagcgtctggcatttccactgctggcagtcattttcatcctgccgccctgtgaaaaaggtgcctgcttctcctttttctgccatgattgtgtaagtgtcctgaggcctcaccagcaatgcggaactgagtccattaaacctctttcctttataataattacccagtttggggtatttcttcgtagcagtgtgagaacagaccataaacctccattttctcatctgttaaatggagataacagtcctggcttaacagggctttttgagttaagtgatatattccacgtaacctgcttagcataagaactggcactagaaacagaacattttagattatggaatagaacttaggggaaaatagcaaagtctctgatcatcttgaactactcaattgggacttatccctgaattaaacctttctagtagctgaagcacaagaaaataaacttggaaagaaaaaacctaaggccagtcatgcactgccctacttccctttcttctctattgcaggttaactatggcctgtaggcagtttttcttctctttttttttttttgagacagtcttgttctgtcacccaggctggagtgcagtggcgcgatcttggctcactgcaacctctgcctcccaggttcaagcgattctcctgcctcagcctcctgaggtgggattaaaggcacttgccaccacacctggctaattttcttttctttttttttttttttttttgcgatggagtctcactctcatcatccaggctgaactgcagtggtgcaatctcggctcactgcaacttccgcctcccaggttcaagcgattctcctgcctcagcctcccaagtagctgggattacaggcatccgccgttacacccagctaagtttttgtatttttagtagagacggcgttttaccatgttggccaggctggtctcaaactcctgacatcgagtgatccacccgcctcgtcctcccaaaatgctaggattacaggcatgagccaccgcacctagccggcaaacttttttaaatggttggcgggggtgggggaaatcaaatgagtaatgttttgtgacacatcaaaattataatgatgtgctgcataacttttggtcaacaatggccaaatatacgatgatgatcccgtaagattacaatggagctgaaaaattcctattgcctggggacacagccatggtaacatcatagtgaaattactttatgtagcctaagtatatagtgtttataaaagtctacagtagtgcacagtaatatcatggccttcacattcactaaccacttactgactcacccagagccagcttccagtcctgccaacttgttcatggtaaatgtcctaaataggtgtaccattttatatcttatatatatctatatatatatttttactgtaccttttctatgtttagatatgtttagatacacaaatacttagcactgtgttacaaccgcctacagtaatcagtacagtaatatgccatacaggtttgtaggttaggagcaataggctatcccatataggataccatagggtataccatctaggtttgtgtaactacatcatgattttcacacaatgatgaaattgccaagtgacatgtctcagaacatatccctgtcattaagtgacatatgactatatatgaaacttaacaaatcaggccttgttgaaacacagtcatgttgatttgtttacatattgtatatggctccttacacactatcaacggcagagttgtgtactatagttgcaatacagaccatagccaacaaagtctaaaatgttctagcacttcacagaaaaggttttttgactcctactctactgtttcagtgtcactgacccattttacctggaccaaagactactcaagtctattttcctccaactgacacaagtttctgcctcagtgtatggaggttttcctcagtaataggaaactggaaaaattagtcaacatttattgagtgcctaaatgactacctatttagtatacctgctgatttacttggcaggcttttctcactatactgcaagctccttgaaggcagagataatttacttgagtggaacctggcacaacgtaagtgctttagaaattgaataagccaagtaaaatgttttaaggcaaccctatcccaaaatattcctgaagatattaatttaatcattactaatctctgtgattagcaagggaagtagtcagtctggcacaccaaattttattaataatacttattttaatctgttccctttagtatgtctttatacagttcccctcgtgtatatacactgatataactacaatttaaaagccactaattaatctgttttttattttgtaagtaacaagatatagacatttgaatgccaatgtcttattctggagagacactggagctgaagttcaacaatgatcacacttattacctggcaataaaaacacaaccatctttccagtcaggtcaaaatatcctactttttgcctttctaccaattcccaaacattcacagtttttcaaggaccactaataaaatacaggaagcttttaaagacagtaagagaacacctagtgtaagttaggtgaattaaagatggcaaaggagattacatcctcaacactgacagcttccaagacttagaaaagagattgttccttgcttctaaaattgttctattttcctctgtaggaaaatgaaagttttttcttacaaatattaaataatcaaagtacttacgcaaaattaatctgctcctcaatgagatgagcactccatttaaatgatctttacagatccctgaagttgctgtcctgtcactgtatttaagtgatggatattcaattgaattattctgcataaataattctgttcaacccagaagtatagtagtatgatgggtcagatacagtcaactgttcaataaaaatgcagatgtctgaaattattaaaatgtacttaaaagtaacaaactgtatcacacacttaggcttagaagtgttctttcaagttttttcttttaaaaaagaaaccagtctttgaagatttttgttgaatatagctattttccaagcttcatcttctttttctttggtccattaaggtccatgtttgaagtatcagtaggaatgcttattcctggtatctgtggttctaccagggacattcggatcttctgatgttgaagattagatgagtctaacatgattttcactttaactttatcaaatacatggaacactgtatcttctattttaagtgagggtatctcatcatcataaataagctgtgggtttggtttgtccttttcttcaaaaaagactgtcccttctaaaccatactttggaattaataccacaatggcattctttcttacaaataaaatataggcttcttcacttactattcctttgcttttgaagaataactgggtatgaaaagccactgatgcacgttgggcatattgagccattttgtgccggaaatttagatttttacatatatctgcaagcttgtgtttgtctgtcaactctggataagtacagtcagccccaatagccacagccaaaagccgatgaacaatgacatctgcgtatcttctaatgggtgaagtaaaatgtgtgtatattggagacgctaagccatagtgatgaaaatcattatccattccagaacagaagtacacagcttgcatcatacagcgagtggctaatattctcaacagagtgtttagatatggaaaagtaggagattcggcctgatccaaagactcagccaaagacttggctgtatcagtcttaatttccaaattccttgacctggctgccttaacaagaatttcataatttgatggaggtggagcaggatgttttcgaagcagagcatgttcagaaaattcctcatgaattttttttgcaacagaaatattggcaagtaacataaattcttcaaccatggaatttgtttccctaagttccttggtctgcagatctataggatcgtgagtttcactgtccatgtggaatcgaacttcaggagaggatagagtcaaagcccctttttcaatccttcttttcttcagaattttggctagtttattcagtccacggagactagtggtaatatcatcattcatgtttgctgaatcaattctcaactgagcttcagcatacgtcagagatgcctttgaattaataacacttttggtaaacttcgtttttaagatttcagcattgtgattcatttcccaaatacatgaaaatgccagcctgtccacgtcacattttaaggaacacaagttagagctaagcaactctggaaccatgtcaatcctcttttcacaaagatacacagttgttcctcttctggctgattcttgatccaaggcatttcctggcctaataaaatggctcacatcagcaatatgaacaccaacctccaaatttccattttcgagttctcgacaatgtagagcatcgtctatatcagtacatcctggtgggtctacactacaaatacacagatgcctcaggtcttctcggtttttcatgtccttttcagtaatgctccagggcatctttggcagaaaactaagaacagcctgtgaaaaaggctgatggggaacatcgtgttcaagtaacaaaacttctgtttcagtctctttctctccaacatcacctaaatttctcacaaagtgtccatttggatatctggaatttctgggccaaccatcaatagcaacaataattctccgtccttctaatgtggaagcctgtctggtttctatgcgaattcgagggattctcttatcagcaggtgtaaagagatgtcttcttgactccttaatgtcagacttggaaagcatgccacaatatggtctccaattcctttttattattcctacaactctacctgtaggcttcaacattttctcgcttacagcagtcttaagcattcgttctgtctcttcttctttctccacatcttcttcattttgaccttcatcatgtaaaaccacagaagatggtgctacccactgactcttggggagaagctccacagccacaatatcttcgtgaacagctctgtttaaatgtttaagtccctgtaagattatctctttattttcttcattgtcgccatgaatccatactgtagcttccaagtaattttccctgctagctctaaatgttccttgaaggtatgtaccagattttatgccttgctgtagcttacttaagggaagatgctctgaaaatattatttttccactttctatttcattcccttcttcagacaaacaagcaagacgatctatgagttcggggttagcagttaggctctttacatattcttcacaagtgaaagctggtattccttcttctatggctttctctttgtttctcctgtcatttgttatgaagataacttgcagctggttgtctgctgacatttttttcaaatgttcattgtaccattttgctgctactcgaatcgctctatcattcctgtcattagcattttctccctgttcttgttctacataggtttctctggtgcagtaacacattagtgtcgggcagcaagtagtgcggttgcgggcagacgctgctcgccgggtcctggggctgcggctccagggccggcccctcgtgcgcccctccacacgctgcgcacccgggcgcaccgcagccgatgtcgtctcgcaggtagtgctcgcgcacgatcttcatcacgccgcccgcccgggtcttttttaagaacgtcttggacttgagcatcttgcctcgccgcgcagaatcctaaccccagcagcgctcttccagcaaaaggcgtcaatctagaatac

SEQ ID NO: 12861 - RNA, 949 nt, Homo sapiens
  source 1..949: mol_type = other RNA
gctgggattacaggcatgagccaacatgcctggcctgctgttggttagaataataccacagagcatcagtctagtccactcctagatatagactcacaaagaagaaagccaggtggcacagtgatttctgtcacattctcaggagcgacctcttacgaacgcatgtctcttcaaagtgcatttctgggttgaaaatccactcgcaatgcagttcttgtgtttggaacttcagttttctgatcaggtagctgtgatgacagtaacaggatctacctctgggtggctcttctgacttcatgccactgctctttctctttcaggcaaggtcttcaggccagtgagggttggtgtcatttgtgggacagaagagcccaaatcaagctgagttgaggcaataaatatgctctcctgcttccagatcaaagtccttatttaaaatgcatatgccatgtgtagtaaggcaaagcctgccacctccaatgcttctcctgttcccccagcagtgctgtgagagaggtggcagatgtggcatggtggcccgcatacacatttgcaagcttgagttctgatgtcagctctgctccttatcttctgtatatccttaggcaaatgtctgcacctctgagtttccactgtttcctcccctacaaaatgggcagaagaagaactaagcttccttgttcggaggatccacaggtgcagagcaaggcaaagtagacactcagtaatggtggccaattatcccccaattcatgctctgcctttagggagttgccagtctcctaaagagaatagaagtagctcacagatggttgaagtacaagtggaatcaaagcacctgcaaaaaaggcacaagctaaaagatgtgagaggtcttaggagggaataatcctagtttggagaaaggttctaagcttccaggaggaggtggtgcaagtgttggctcttg

SEQ ID NO: 12862 - RNA, 1185 nt, Homo sapiens
  source 1..1185: mol_type = other RNA
gctgggattacaggcatgagccaacatgcctggcctgctgttggttagaataataccacagagcatcagtctagtccactcctagatatagactcacaaagaagaaagccaggtggcacagtgatttctgtcacattctcaggagcgacctcttacgaacgcatgtctcttcaaagtgcatttctgggttgaaaatccactcgcaatgcagttcttgtgtttggaacttcagttttctgatcaggtagctgtgatgacagtaacaggatctacctctgggtggctgtgaggatttgggatatgcattaatgtacccgttccactgcctgccctggggcaaactcagtgaatcttcactgctgatgtctatctagtacccaatctgagctagggtttttacacgtgctgcttccaaattctcatagcaaaaccattactgaagtgcgattcctgaggctcagggagagaacacagacagaggcaaagctggcaggtaaacgcacctcttctgacttcatgccactgctctttctctttcaggcaaggtcttcaggccagtgagggttggtgtcatttgtgggacagaagagcccaaatcaagctgagttgaggcaataaatatgctctcctgcttccagatcaaagtccttatttaaaatgcatatgccatgtgtagtaaggcaaagcctgccacctccaatgcttctcctgttcccccagcagtgctgtgagagaggtggcagatgtggcatggtggcccgcatacacatttgcaagcttgagttctgatgtcagctctgctccttatcttctgtatatccttaggcaaatgtctgcacctctgagtttccactgtttcctcccctacaaaatgggcagaagaagaactaagcttccttgttcggaggatccacaggtgcagagcaaggcaaagtagacactcagtaatggtggccaattatcccccaattcatgctctgcctttagggagttgccagtctcctaaagagaatagaagtagctcacagatggttgaagtacaagtggaatcaaagcacctgcaaaaaaggcacaagctaaaagatgtgagaggtcttaggagggaataatcctagtttggagaaaggttctaagcttccaggaggaggtggtgcaagtgttggctcttgaatgagcaaggttgga

SEQ ID NO: 12863 - RNA, 1074 nt, Homo sapiens
  source 1..1074: mol_type = other RNA
gctgggattacaggcatgagccaacatgcctggcctgctgttggttagaataataccacagagcatcagtctagtccactcctagatatagactcacaaagaagaaagccaggtggcacagtgatttctgtcacattctcaggagcgacctcttacgaacgcatgtctcttcaaagtgcatttctgggttgaaaatccactcgcaatgcagttcttgtgtttggaacttcagttttctgatcaggtagctgtgatgacagtaacaggatctacctctgggtggctgtgaggatttgggatatgcattaatgtacccgttccactgcctgccctggggcaaactcagtgaatcttcactgctgatgtctatctagtacccaatctgagctagggtttttacacgtgctgcttccaaattctcatagcaaaaccattactgaagtgcgattcctgaggctcagggagagaacacagacagaggcaaagctggcaggtaaacgcacctcttctgacttcatgccactgctctttctctttcaggcaaggtcttcaggccagtgagggttggtgtcatttgtgggacagaagagcccaaatcaagctgagttgaggcaataaatatgctctcctgcttccagatcaaagtccttatttaaaatgcatatgccatgtgtagtaaggcaaagcctgccacctccaatgcttctcctgttcccccagcagtgctgtgagagaggtggcagatgtggcatggtggcccgcatacacatttgcaagcttgagttctgatgtcagctctgctccttatcttctgtatatccttaggcaaatgtctgcacctctgagtttccactgtttcctcccctctgcctttagggagttgccagtctcctaaagagaatagaagtagctcacagatggttgaagtacaagtggaatcaaagcacctgcaaaaaaggcacaagctaaaagatgtgagaggtcttaggagggaataatcctagtttggagaaaggttctaagcttccaggaggaggtggtgcaagtgttggctcttgaatgagcaaggttgga

SEQ ID NO: 12864 - RNA, 1038 nt, Homo sapiens
  source 1..1038: mol_type = other RNA
gctgggattacaggcatgagccaacatgctcagcctgaaatggtacattttttttttacaaaaggaaaacagatattaatattatgggagattatattttccttaaatgactgcaataatatctctacttaatctctcattccacatgctcttcttataatgtgactaacactcctcccaattagtgtcccctttacttaaatgtggtgtttttgtagctgcttcaacaagtagagtacagtggaagtgacgctgtacaacctctgagattaggtcataaaaatcaatgcaagctggtctgagtctgagtgcagtggtgtttacaactaattgatcacaactactttacagatttctttgttccttctccactcccactgcttcacttggctaaccaggatcatccttggggcaaccaaggaataactgtagttttaatcaattctcgagttgttgtccttggtcccagtcacataatcaacatgtcaaagtcttctaccatgtacctcacttattaaaaagaaacgagtttccataaagtcgaccacgcatctttgttctctttatcccagatcctctctctgcatccgtagtttcctctcccacttggcatctctttaccatttcttcttgtttacttgactatcccagctcccaacattttctgtcccggaatccactaagcctgggttatactgtgtacatgttagaaatgatattcaataaaaaggcccaggaaaccatgcactgagttcctatatttcatttttcttaaatgctccagctacacccaaggactgactgaggggccgggagactgggctccgtgcccaggtggcaggggcgtgtaattctaacaccgcaggcagcccctgctgacgagatacagaggagtaacgacagttaatagtaaacgaagcgaagccccgggaggtgtagcgagcatgtccacgacagccagtcactgatcctccggcctcccacgcttccagccgagacagtcacgctccgcggggccaagatggcgccctccccgcg

SEQ ID NO: 12865 - RNA, 1066 nt, Homo sapiens
  source 1..1066: mol_type = other RNA
gctgggattacaggcatgagccaacatgctcagcctgaaatggtacattttttttttacaaaaggaaaacagatattaatattatgggagattatattttccttaaatgactgcaataatatctctacttaatctctcattccacatgctcttcttataatgtgactaacactcctcccaattagtgtcccctttacttaaatgtggtgtttttgtagctgcttcaacaagtagagtacagtggaagtgacgctgtacaacctctgagattaggtcataaaaatcaatgcaagctggtctgagtctgagtgcagtggtgtttacaactaattgatcacaactactttacagatttctttgttccttctccactcccactgcttcacttggctaaccagtgaaaaggaaatagccatattgtaccaggatcatccttggggcaaccaaggaataactgtagttttaatcaattctcgagttgttgtccttggtcccagtcacataatcaacatgtcaaagtcttctaccatgtacctcacttattaaaaagaaacgagtttccataaagtcgaccacgcatctttgttctctttatcccagatcctctctctgcatccgtagtttcctctcccacttggcatctctttaccatttcttcttgtttacttgactatcccagctcccaacattttctgtcccggaatccactaagcctgggttatactgtgtacatgttagaaatgatattcaataaaaaggcccaggaaaccatgcactgagttcctatatttcatttttcttaaatgctccagctacacccaaggactgactgaggggccgggagactgggctccgtgcccaggtggcaggggcgtgtaattctaacaccgcaggcagcccctgctgacgagatacagaggagtaacgacagttaatagtaaacgaagcgaagccccgggaggtgtagcgagcatgtccacgacagccagtcactgatcctccggcctcccacgcttccagccgagacagtcacgctccgcggggccaagatggcgccctccccgcg

SEQ ID NO: 12866 - RNA, 1875 nt, Homo sapiens
  source 1..1875: mol_type = other RNA
gctgggattacaggcatgagccaaccgcacccagccaggaattctttttgagtgctttaatttttggtctttagaattctagtgctcaagttatgaaatggaggagaatgtctatttttacactgagtaactcacacattccttctcaatgagggaaaaaacatacttgtctaaaaagatatatactaattcattatatgtgttaataatgaaaatagtagaacatgtctgagaatgccttttcaaggcctgcatagggatggaaatctgaattaagctttggaattgcaaacgtcagaattgagactgcattgataagcagaaaagcaaataatgctgacctgagatcttcaaccttctctcctgtggctttcatgagtcttgaaaggagactggtgcttactaagaccactgatttgtactaaggagcgtttgcatctggtgtcttcccttgtgctgaaatagctctgagtaaatgctttgattccctcatgatacttatgggactttttttctaatgtgtcttttcctatgtctaaaaagatttgagctctgactaaaggctttgccacagtcatgacacttgtagggcttctcaccagtatgggttcgtcgatgctgaatcagaattgcgcttcggctgaatgcctttgcacactcgtcacatgcataaggtttctttccactgtggattctctgatgtaaaataagggctgagctctgactaaagattttgccacattcatcacatttctgttgttttttccaagaagggtttccttgtctcttttcaaacctaccatcttgttcataggttcctctatatgtggaactctgggagccattcatatgaaggatattggaaacattgcaatgcagttctatgcctaaagaagtcttttgccttgaagcagatttcacatttgtagttttgatgtcttcatcatgtggtcttaaggactgaagctcccatgatgctccctggagctgcttcttcacgggcatgagctggctacttggcaattcctcagtgatttctgaaggtgctagcttctctgcaatcatgtccttccttcgtccaaaaaagatctgctttggtccatcaagctctctctccacatcctccagcatagtcacagtttcctctccattctctggatgatgcttctgcacccaggcctgaagctcttttgggaggatggccaggaactgctccagcaccagcagctccaggatctgctccttggtgtgcacttccggcctcagccagagatgacaaagttcccagagccggctcagagcctcatggggcccaggtgaatcctggtagccaaactgcctgaattgctggcggaaggtctctgggctgtagctgctgctccagtggaggctagagtctggatcacaggtctgctcttcctcttccatcttctctgtcagaatcccattacactcctctgaagtttgtgttaggagtgatgatgactttcccaattttgcagacattttgacagacaaatagctcagtactgttaggctttaatcctcaaggaggtgaagctgtcctgatggacactcccccatgttgtagacggggaagcagtcacagcaaagccaggtactctggccaagggcaaagctggggtctgaacccaggccgtccacatttatccatggtgctgtgtggttagaggccataggcagcaggggcccttgtggtgacccctgcgcgttgtctcagcgcagaggaggaagtggcggcaggcagccgcgctcccagatgaagcggggccagaagagtctggggaacaagacctcccgacgccgtcggggagaaaccggggaactgccagctgcgcaacaacttccggttct

SEQ ID NO: 12867 - RNA, 2253 nt, Homo sapiens
  source 1..2253: mol_type = other RNA
gctgggattacaggcatgagccaaccgcacccagccaggaattctttttgagtgctttaatttttggtctttagaattctagtgctcaagttatgaaatggaggagaatgtctatttttacactgagtaactcacacattccttctcaatgagggaaaaaacatacttgtctaaaaagatatatactaattcattatatgtgttaataatgaaaatagtagaacatgtctgagaatgccttttcaaggcctgcatagggatggaaatctgaattaagctttggaattgcaaacgtcagaattgagactgcattgataagcagaaaagcaaataatgctgacctgagatcttcaaccttctctcctgtggctttcatgagtcttgaaaggagactggtgcttactaagaccactgatttgtactaaggagcgtttgcatctggtgtcttcccttgtgctgaaatagctctgagtaaatgctttgattccctcatgatacttatgggactttttttctaatgtgtcttttcctatgtctaaaaagatttgagctctgactaaaggctttgccacagtcatgacacttgtagggcttctcaccagtatgggttcgtcgatgctgaatcagaattgcgcttcggctgaatgcctttgcacactcgtcacatgcataaggtttctttccactgtggattctctgatgtaaaataagggctgagctctgactaaagattttgccacattcatcacatttctgttgttttttccaagaagggtttccttgtctcttttcaaacctaccatcttgttcataggttcctctatatgtggaactctgggagccattcatatgaaggatattggaaacattgcaatgcagttctatgcctaaagaagtcttttgccttgaagcagatttcacatttgtagttttgatgtcttcatcatgtggtcttaaggactgaagctcccatgatgctccctggagctgcttcttcacgggcatgagctggctacttggcaattcctcagtgatttctgaaggtgctagcttctctgcaatcatgtccttccttcgtccaaaaaagatctgctttggtccatcaagctctctctccacatcctccagcatagtcacagtttcctctccattctctggatgatgcttctgcacccaggcctgaagctcttttgggaggatggccaggaactgctccagcaccagcagctccaggatctgctccttggtgtgcacttccggcctcagccagagatgacaaagttcccagagccggctcagagcctcatggggcccaggtgaatcctggtagccaaactgcctgaattgctggcggaaggtctctgggctgtagctgctgctccagtggaggctagagtctggatcacaggtctgctcttcctcttccatcttctctgtcagaatcccattacactcctctgaagtttgtgttaggagtgatgatgactttcccaattttgcagacattttgacagacaaatagctcagtactgttaggctttaatcctcaaggaggtgaagctgtcctgatggacactcccccatgttgtagacggggaagcagtcacagcaaagccaggtactctggccaagggcaaagctggggtctgaacccaggccgtccacatttatccatggtgctgtgtggttagaggccataggcagcaggggcccttgtggtgacccctgcgcgttgtctcagcgcagaggaggaagtggcggcaggcagccgcgctcccagatgaagcggggccagaagagtctggggaacaagacctgagaggtgggaagggttgaggccaccggtttggagccgtcaggtaccctaagggatatatgagggaccccggggctaaagcagcctctggaagagagtggccgccctgtcacttcagcaccaggcgcagaatctgtgctaaacctgaggtgagggtaaggaacccccgacaccgcacgacaaccagaaagaacgtccctggaggggaggcttcgatcaaagcctgggacgcaggggtctttctgcaggggacgccgctctcggctctaccctgctgtggtgggccggctctgggagggctggcttccgaccatctcccgacctcccgcgcccaccgcgccgcgccgcgcgcctcccaggctgggaaccgccggggcgaagcggcaggtggcgcgggttcacctggcagggcaggcgcccggggtccgccggggaag

SEQ ID NO: 12868 - RNA, 1638 nt, Homo sapiens
  source 1..1638: mol_type = other RNA
gctgggattacaggcatgagccaaccgcacccagccaggaattctttttgagtgctttaatttttggtctttagaattctagtgctcaagttatgaaatggaggagaatgtctatttttacactgagtaactcacacattccttctcaatgagggaaaaaacatacttgtctaaaaagatatatactaattcattatatgtgttaataatgaaaatagtagaacatgtctgagaatgccttttcaaggcctgcatagggatggaaatctgaattaagctttggaattgcaaacgtcagaattgagactgcattgataagcagaaaagcaaataatgctgacctgagatcttcaaccttctctcctgtggctttcatgagtcttgaaaggagactggtgcttactaagaccactgatttgtactaaggagcgtttgcatctggtgtcttcccttgtgctgaaatagctctgagtaaatgctttgattccctcatgatacttatgggactttttttctaatgtgtcttttcctatgtctaaaaagatttgagctctgactaaaggctttgccacagtcatgacacttgtagggcttctcaccagtatgggttcgtcgatgctgaatcagaattgcgcttcggctgaatgcctttgcacactcgtcacatgcataaggtttctttccactgtggattctctgatgtaaaataagggctgagctctgactaaagattttgccacattcatcacatttctgttgttttttccaagaagggtttccttgtctcttttcaaacctaccatcttgttcataggttcctctatatgtggaactctgggagccattcatatgaaggatattggaaacattgcaatgcagttctatgcctaaagaagtcttttgccttgaagcagatttcacatttgtagttttgatgtcttcatcatgtggtcttaaggactgaagctcccatgatgctccctggagctgcttcttcacgggcatgagctggctacttggcaattcctcagtgatttctgaaggtgctagcttctctgcaatcatgtccttccttcgtccaaaaaagatctgctttggtccatcaagctctctctccacatcctccagcatagtcacagtttcctctccattctctggatgatgcttctgcacccaggcctgaagctcttttgggaggatggccaggaactgctccagcaccagcagctccaggatctgctccttggtgtgcacttccggcctcagccagagatgacaaagttcccagagccggctcagagcctcatggggcccaggtgaatcctggtagccaaactgcctgaattgctggcggaaggtctctgggctgtagctgctgctccagtggaggctagagtctggatcacaggtctgctcttcctcttccatcttctctgtcagaatcccattacactcctctgaagtttgtgttaggagtgatgatgactttcccaattttgcagacattttgacagacaaatagctcagtactgttaggctttaatcctcaaggaggtgaagctgtcctgatggacactcctcccgacgccgtcggggagaaaccggggaactgccagctgcgcaacaacttccggttct

SEQ ID NO: 12869 - RNA, 2418 nt, Homo sapiens
  source 1..2418: mol_type = other RNA
gctgggattacaggcatgagccaaccgcacccagccaggaattctttttgagtgctttaatttttggtctttagaattctagtgctcaagttatgaaatggaggagaatgtctatttttacactgagtaactcacacattccttctcaatgagggaaaaaacatacttgtctaaaaagatatatactaattcattatatgtgttaataatgaaaatagtagaacatgtctgagaatgccttttcaaggcctgcatagggatggaaatctgaattaagctttggaattgcaaacgtcagaattgagactgcattgataagcagaaaagcaaataatgctgacctgagatcttcaaccttctctcctgtggctttcatgagtcttgaaaggagactggtgcttactaagaccactgatttgtactaaggagcgtttgcatctggtgtcttcccttgtgctgaaatagctctgagtaaatgctttgattccctcatgatacttatgggactttttttctaatgtgtcttttcctatgtctaaaaagatttgagctctgactaaaggctttgccacagtcatgacacttgtagggcttctcaccagtatgggttcgtcgatgctgaatcagaattgcgcttcggctgaatgcctttgcacactcgtcacatgcataaggtttctttccactgtggattctctgatgtaaaataagggctgagctctgactaaagattttgccacattcatcacatttctgttgttttttccaagaagggtttccttgtctcttttcaaacctaccatcttgttcataggttcctctatatgtggaactctgggagccattcatatgaaggatattggaaacattgcaatgcagttctatgcctaaagaagtcttttgccttgaagcagatttcacatttgtagttttgatgtcttcatcatgtggtcttaaggactgaagctcccatgatgctccctggagctgcttcttcacgggcatgagctggctacttggcaattcctcagtgatttctgaaggtgctagcttctctgcaatcatgtccttccttcgtccaaaaaagatctgctttggtccatcaagctctctctccacatcctccagcatagtcacagtttcctctccattctctggatgatgcttctgcacccaggcctgaagctcttttgggaggatggccaggaactgctccagcaccagcagctccaggatctgctccttggtgtgcacttccggcctcagccagagatgacaaagttcccagagccggctcagagcctcatggggcccaggtgaatcctggtagccaaactgcctgaattgctggcggaaggtctctgggctgtagctgctgctccagtggaggctagagtctggatcacaggtctgctcttcctcttccatcttctctgtcagaatcccattacactcctctgaagtttgtgttaggagtgatgatgactttcccaattttgcagacattttgacagacaaatagctcagtactgttaggctttaatcctcaaggaggtgaagctgtcctgatggacactcgtgcgcctccgtcttccatcgttatgtatcctgccatttgacttattttctcacttcaccaagtattgttctaggccctgtataaagcctgtgagttcataaagttgttaccaaataaatgatacaactttacacaatgatgtgccccatgttgtagacggggaagcagtcacagcaaagccaggtactctggccaagggcaaagctggggtctgaacccaggccgtccacatttatccatggtgctgtgtggttagaggccataggcagcaggggcccttgtggtgacccctgcgcgttgtctcagcgcagaggaggaagtggcggcaggcagccgcgctcccagatgaagcggggccagaagagtctggggaacaagacctgagaggtgggaagggttgaggccaccggtttggagccgtcaggtaccctaagggatatatgagggaccccggggctaaagcagcctctggaagagagtggccgccctgtcacttcagcaccaggcgcagaatctgtgctaaacctgaggtgagggtaaggaacccccgacaccgcacgacaaccagaaagaacgtccctggaggggaggcttcgatcaaagcctgggacgcaggggtctttctgcaggggacgccgctctcggctctaccctgctgtggtgggccggctctgggagggctggcttccgaccatctcccgacctcccgcgcccaccgcgccgcgccgcgcgcctcccaggctgggaaccgccggggcgaagcggcaggtggcgcgggttcacctggcagggcaggcgcccggggtccgccggggaaggacgaggggaaggggtgcgcg

SEQ ID NO: 12870 - RNA, 2366 nt, Homo sapiens
  source 1..2366: mol_type = other RNA
gctgggattacaggcatgagccaaccgcacccagccaggaattctttttgagtgctttaatttttggtctttagaattctagtgctcaagttatgaaatggaggagaatgtctatttttacactgagtaactcacacattccttctcaatgagggaaaaaacatacttgtctaaaaagatatatactaattcattatatgtgttaataatgaaaatagtagaacatgtctgagaatgccttttcaaggcctgcatagggatggaaatctgaattaagctttggaattgcaaacgtcagaattgagactgcattgataagcagaaaagcaaataatgctgacctgagatcttcaaccttctctcctgtggctttcatgagtcttgaaaggagactggtgcttactaagaccactgatttgtactaaggagcgtttgcatctggtgtcttcccttgtgctgaaatagctctgagtaaatgctttgattccctcatgatacttatgggactttttttctaatgtgtcttttcctatgtctaaaaagatttgagctctgactaaaggctttgccacagtcatgacacttgtagggcttctcaccagtatgggttcgtcgatgctgaatcagaattgcgcttcggctgaatgcctttgcacactcgtcacatgcataaggtttctttccactgtggattctctgatgtaaaataagggctgagctctgactaaagattttgccacattcatcacatttctgttgttttttccaagaagggtttccttgtctcttttcaaacctaccatcttgttcataggttcctctatatgtggaactctgggagccattcatatgaaggatattggaaacattgcaatgcagttctatgcctaaagaagtcttttgccttgaagcagatttcacatttgtagttttgatgtcttcatcatgtggtcttaaggactgaagctcccatgatgctccctggagctgcttcttcacgggcatgagctggctacttggcaattcctcagtgatttctgaaggtgctagcttctctgcaatcatgtccttccttcgtccaaaaaagatctgctttggtccatcaagctctctctccacatcctccagcatagtcacagtttcctctccattctctggatgatgcttctgcacccaggcctgaagctcttttgggaggatggccaggaactgctccagcaccagcagctccaggatctgctccttggtgtgcacttccggcctcagccagagatgacaaagttcccagagccggctcagagcctcatggggcccaggtgaatcctggtagccaaactgcctgaattgctggcggaaggtctctgggctgtagctgctgctccagtggaggctagagtctggatcacaggtctgctcttcctcttccatcttctctgtcagaatcccattacactcctctgaagtttgtgttaggagtgatgatgactttcccaattttgcagacattttgacagacaaatagctcagtactgttaggctttaatcctcaaggaggtgaagctgtcctgatggacactcgtgcgcctccgtcttccatcgttatgtatcctgccatttgacttattttctcacttcaccaagtattgttctaggccctgtataaagcctgtgagttcataaagttgttaccaaataaatgatacaactttacacaatgatgtgctatgaaacaaacaatagcagacacacatattaacagaatttactatgtgccaagcactgttttgaacaccttagtaaaaataaacaaaggttaaatcctcataaaagccctagattatttttacccccatgttgtagacggggaagcagtcacagcaaagccaggtactctggccaagggcaaagctggggtctgaacccaggccgtccacatttatccatggtgctgtgtggttagaggccataggcagcaggggcccttgtggtgacccctgcgcgttgtctcagcgcagaggaggaagtggcggcaggcagccgcgctcccagatgaagcggggccagaagagtctggggaacaagacctgagaggtgggaagggttgaggccaccggtttggagccgtcaggtaccctaagggatatatgagggaccccggggctaaagcagcctctggaagagagtggccgccctgtcacttcagcaccaggcgcagaatctgtgctaaacctgaggtgagggtaaggaacccccgacaccgcacgacaaccagaaagaacgtccctggaggggaggcttcgatcaaagcctgggacgcaggggtctttctgcaggggacgccgctctcggctctaccctgctgtggt

SEQ ID NO: 12871 - RNA, 3583 nt, Homo sapiens
  source 1..3583: mol_type = other RNA
gctgggattacaggcatgagccaacgcgtccggcagaatggtaaatgtttaatatggaaaagggaacatttagtctggacagagaggacaataaataattatggctaccatttgtcaccacctttcctggcatttacttatttatttatttattgagatggagtttcgctcttgttgcccaggctggagtgcaatggcacaatctcggctcaccgcaacctccgcctcctgggttcaagcgattctcccgcctcaggctccccaggtagctgggattacaggcatgcaccaccacgcctggctaatttttgtatttttagtagagacggggtttctccatgttggtcaggctggtctcaaactcctgacctcaggtgatcctcctgcctcggcctcccaaagtgctgggattacaggtttgagccactgcgcctggcctttcctggcatttaaaatagctatgtccagtcttcagaacagccctgtggcgaggtatgatcatgaaacccacgttataaagtgaagaggaaacagattttataacttgcccaagatcatccagctaaatggagaagtggagattcaaagtcgggtctgactctttgtactagcttaagaacagactctcagctggatgtggtggctcatacctgtaatctcaacacttaaggaggccgaggcagatggatcacttgagcccaggagttttagaccacacaaacacacaaaaaattagccaggtgtggtggtgcatgcctgcagtcccagctactcaggaggctaaggagggaggattgattgagccctggtgattgaggctgcagttagccatgatcacaccaagagagggaagaaggaaggtggctgtcagtcactggtatcagagacaagcagaggacagagaagacaaatgcaaaatctttctttggctgggacttgtcagaaagggaatctccagtgttggtgatggtgtcaccaacagcctcatgtgccttatgtgtgggcatctctgaaggcagaaagaactccattttccctggaggaaaatggaccagtgagcatgaggctgaggtctgactcctgggggccacacaggcaggcctgagcaccttgcccctcctcactgaagggggcttaatgtctggggcacagttgactccatccctctcttttttcctgtatgtggttttttgtttttttttttttcaagacaaggtctcattctgtcacacagactggagtgcagtggcacaatctcagctcactgcaaactctgcctcccaggttcaagtgattctcccatctcagcctcccgagtagctgggactacaggcacgcacgtacaggctggtcttgaactcctgacctaaagtgatctgcctgcctcgtttttcctgtatgttctaatgttatttcagggatcccctttgcctcactctggccattccaaaacatatatatgtttcatttatataaatccaaatgaaaatattaaaattgcaagtgagatatttttggccttaatctttgaatttcaatgttttcttatctgtagagctggtgtgctaactcctgtaattctgggcaatgcccatgtggttcttggctgcttcaagccatctcaggtctgattttcacacaagctcagcagcactgggctagaagggtaccgccctcccactctgctgccactttgaatagaagtccaagctttcgctttcttgccctgactttgattcttcacattgctgaggagcagtgattgaagcttaatctcattgtctacagtccgtctcctctatggagctgcactattctttcccatctcaattatttctgatgtaaccaaaacactctctctccccactgccttttttcttttgtaaagacttgcaaagggtcagttccagaggctcgagccctgtgttctgactttcacagacagaggcctgccactcttacatttacaggtcatcattctgagcaatacactttttttgaagagtagtcctaaaagctcactaaaaagttgcatttgtatttaacttaaatagagaaccttatgtgtagtccatgtttctggactctatacctgattttgaatcactggacttaaattattggacttacaacactgatacatcttgtaaatgaacctaagcaaagaataccagccctacatcccactcccctcaagataactgggaaagacacaaagccatgctgaggaggagccatggtttgatattgtccagtgagtgtctcttggcctcagaatgctgccacttcctgcagttccagcccttggctgtggtccattctgagtaagtgaattcctctgttaaaacttgcacacaataaggagatggcgtcaccaacagccagagaagtcaagggtcctgatccatccagagacaaggtgaaaaggcaggctccagtatcttggttccaaatcttcaccttgcaatcatgtgatgaggtagcaattaaaggcatcaaggccaatgctcttggtagaaagacgcaggatgcgacagtctggaaatgccccttatactcacatattctgtttcgagtctgtcttaggtcccacaacgtggcttcacagccttctcctccaaagccattgctgcaggagatacacttgtgtccatccacactgacttcacagtaggtctgaatgtgctgctttgcaggaaacatatgagctacctgcagcccccgactgtcccataatctcacaagaaacactttcacagctgctcagtaagcccacctgagggttttatcttcagaggtctgtagtatgtatggttctctggggacccagcacaggtgagtgaccacgttcctggagacagatgctctttccacactctgtcctgtcaccacatcccacagaagcagggtgttgtcccgagagccagtgcacagctgtgatgagtctggactcacagccaatccggtgaccaccatggcatggccacacaattgctgccttggttgtgaggaaccgtgcaagtcccacatcatgaccatcctgtcacgagaggcactgaagaactggctggatttgggaatacaggctaccttggtgatctcatgttcatgtcctttgaaccttttcaccacatttccagttttccaattataggccacaactgtcttatctttccctccagagacacaaaggtctgagttcaaagcagccacgacagagacggtatccatgtgagctgggctatactcttgaaaagctttagtttgaattctctcttctataatttcatcaggcctgcttctgtggaggagcttgtttcagttggcacctgagtagcagcatcccttgtggctgctggaagttgtgttccccccaaaccaataggatcttcttggttagctgccctattcaataatttgtaatgtgtatcctttggaaaatagttcaggcagccacttcttaatctctgtaattagtgggaagccactgaagttaatctcttctctgtctaagcatgtttgcacggtgggctgcggggctggagctggggccggcgggaacgcggagcctgggggtgggaac

SEQ ID NO: 12872 - RNA, 3482 nt, Homo sapiens
  source 1..3482: mol_type = other RNA
gctgggattacaggcatgagccaacgcgtccggcagaatggtaaatgtttaatatggaaaagggaacatttagtctggacagagaggacaataaataattatggctaccatttgtcaccacctttcctggcatttacttatttatttatttattgagatggagtttcgctcttgttgcccaggctggagtgcaatggcacaatctcggctcaccgcaacctccgcctcctgggttcaagcgattctcccgcctcaggctccccaggtagctgggattacaggcatgcaccaccacgcctggctaatttttgtatttttagtagagacggggtttctccatgttggtcaggctggtctcaaactcctgacctcaggtgatcctcctgcctcggcctcccaaagtgctgggattacaggtttgagccactgcgcctggcctttcctggcatttaaaatagctatgtccagtcttcagaacagccctgtggcgaggtatgatcatgaaacccacgttataaagtgaagaggaaacagattttataacttgcccaagatcatccagctaaatggagaagtggagattcaaagtcgggtctgactctttgtactagcttaagaacagactctcagctggatgtggtggctcatacctgtaatctcaacacttaaggaggccgaggcagatggatcacttgagcccaggagttttagaccacacaaacacacaaaaaattagccaggtgtggtggtgcatgcctgcagtcccagctactcaggaggctaaggagggaggattgattgagccctggtgattgaggctgcagttagccatgatcacaccaagagagggaagaaggaaggtggctgtcagtcactggtatcagagacaagcagaggacagagaagacaaatgcaaaatctttctttggctgggacttgtcagaaagggaatctccagtgttggtgatggtgtcaccaacagcctcatgtgccttatgtgtgggcatctctgaaggcagaaagaactccattttccctggaggaaaatggaccagtgagcatgaggctgaggtctgactcctgggggccacacaggcaggcctgagcaccttgcccctcctcactgaagggggcttaatgtctggggcacagttgactccatccctctcttttttcctgtatgtggttttttgtttttttttttttcaagacaaggtctcattctgtcacacagactggagtgcagtggcacaatctcagctcactgcaaactctgcctcccaggttcaagtgattctcccatctcagcctcccgagtagctgggactacaggcacgcacgtacaggctggtcttgaactcctgacctaaagtgatctgcctgcctcgtttttcctgtatgttctaatgttatttcagggatcccctttgcctcactctggccattccaaaacatatatatgtttcatttatataaatccaaatgaaaatattaaaattgcaagtgagatatttttggccttaatctttgaatttcaatgttttcttatctgtagagctggtgtgctaactcctgtaattctgggcaatgcccatgtggttcttggctgcttcaagccatctcaggtctgattttcacacaagctcagcagcactgggctagaagggtaccgccctcccactctgctgccactttgaatagaagtccaagctttcgctttcttgccctgactttgattcttcacattgctgaggagcagtgattgaagcttaatctcattgtctacagtccgtctcctctatggagctgcactattctttcccatctcaattatttctgatgtaaccaaaacactctctctccccactgccttttttcttttgtaaagacttgcaaagggtcagttccagaggctcgagccctgtgttctgactttcacagacagaggcctgccactcttacatttacaggtcatcattctgagcaatacactttttttgaagagtagtcctaaaagctcactaaaaagttgcatttgtatttaacttaaatagagaaccttatgtgtagtccatgtttctggactctatacctgattttgaatcactggacttaaattattggacttacaacactgatacatcttgtaaatgaacctaagcaaagaataccagccctacatcccactcccctcaagataactgggaaagacacaaagccatgctgaggaggagccatggtttgatattgtccagtgagtgtctcttggcctcagaatgctgccacttcctgcagttccagcccttggctgtggtccattctgagtaagtgaattcctctgttaaaacttgcacacaataaggagatggcgtcaccaacagccagagaagtcaagggtcctgatccatccagagacaaggtgaaaaggcaggctccagtatcttggttccaaatcttcaccttgcaatcatgtgatgaggtagcaattaaaggcatcaaggccaatgctcttggtagaaagacgcaggatgcgacagtctggaaatgccccttatactcacatattctgtttcgagtctgtcttaggtcccacaacgtggcttcacagccttctcctccaaagccattgctgcaggagatacacttgtgtccatccacactgacttcacagtaggtctgaatgtgctgctttgcaggaaacatatgagctacctgcagcccccgactgtcccataatctgagggttttatcttcagaggtctgtagtatgtatggttctctggggacccagcacaggtgagtgaccacgttcctggagacagatgctctttccacactctgtcctgtcaccacatcccacagaagcagggtgttgtcccgagagccagtgcacagctgtgatgagtctggactcacagccaatccggtgaccaccatggcatggccacacaattgctgccttggttgtgaggaaccgtgcaagtcccacatcatgaccatcctgtcacgagaggcactgaagaactggctggatttgggaatacaggctaccttggtgatctcatgttcatgtcctttgaaccttttcaccacatttccagttttccaattataggccacaactgtccgtatttataagtgctgtgtttgagtttgctttgctgtttccccatcacgacacaaaacctaaacgaaaccttctgtggaggagcttgtttcagttggcacctgagtagcagcatcccttgtggctgctggaagttgtgttccccccaaaccaataggatcttcttggttagctgccctattcaataatttgtaatgtgtatcctttggaaaatagttcaggcagccacttcttaatctctgtaattagtgggaagccactgaagttaatctcttctctgtctaagcatgtttgcacggtgggctgcggggctggagctggggccggcgggaacgcggagcctgggggtgggaac

SEQ ID NO: 12873 - RNA, 3612 nt, Homo sapiens
  source 1..3612: mol_type = other RNA
gctgggattacaggcatgagccaacgcgtccggcagaatggtaaatgtttaatatggaaaagggaacatttagtctggacagagaggacaataaataattatggctaccatttgtcaccacctttcctggcatttacttatttatttatttattgagatggagtttcgctcttgttgcccaggctggagtgcaatggcacaatctcggctcaccgcaacctccgcctcctgggttcaagcgattctcccgcctcaggctccccaggtagctgggattacaggcatgcaccaccacgcctggctaatttttgtatttttagtagagacggggtttctccatgttggtcaggctggtctcaaactcctgacctcaggtgatcctcctgcctcggcctcccaaagtgctgggattacaggtttgagccactgcgcctggcctttcctggcatttaaaatagctatgtccagtcttcagaacagccctgtggcgaggtatgatcatgaaacccacgttataaagtgaagaggaaacagattttataacttgcccaagatcatccagctaaatggagaagtggagattcaaagtcgggtctgactctttgtactagcttaagaacagactctcagctggatgtggtggctcatacctgtaatctcaacacttaaggaggccgaggcagatggatcacttgagcccaggagttttagaccacacaaacacacaaaaaattagccaggtgtggtggtgcatgcctgcagtcccagctactcaggaggctaaggagggaggattgattgagccctggtgattgaggctgcagttagccatgatcacaccaagagagggaagaaggaaggtggctgtcagtcactggtatcagagacaagcagaggacagagaagacaaatgcaaaatctttctttggctgggacttgtcagaaagggaatctccagtgttggtgatggtgtcaccaacagcctcatgtgccttatgtgtgggcatctctgaaggcagaaagaactccattttccctggaggaaaatggaccagtgagcatgaggctgaggtctgactcctgggggccacacaggcaggcctgagcaccttgcccctcctcactgaagggggcttaatgtctggggcacagttgactccatccctctcttttttcctgtatgtggttttttgtttttttttttttcaagacaaggtctcattctgtcacacagactggagtgcagtggcacaatctcagctcactgcaaactctgcctcccaggttcaagtgattctcccatctcagcctcccgagtagctgggactacaggcacgcacgtacaggctggtcttgaactcctgacctaaagtgatctgcctgcctcgtttttcctgtatgttctaatgttatttcagggatcccctttgcctcactctggccattccaaaacatatatatgtttcatttatataaatccaaatgaaaatattaaaattgcaagtgagatatttttggccttaatctttgaatttcaatgttttcttatctgtagagctggtgtgctaactcctgtaattctgggcaatgcccatgtggttcttggctgcttcaagccatctcaggtctgattttcacacaagctcagcagcactgggctagaagggtaccgccctcccactctgctgccactttgaatagaagtccaagctttcgctttcttgccctgactttgattcttcacattgctgaggagcagtgattgaagcttaatctcattgtctacagtccgtctcctctatggagctgcactattctttcccatctcaattatttctgatgtaaccaaaacactctctctccccactgccttttttcttttgtaaagacttgcaaagggtcagttccagaggctcgagccctgtgttctgactttcacagacagaggcctgccactcttacatttacaggtcatcattctgagcaatacactttttttgaagagtagtcctaaaagctcactaaaaagttgcatttgtatttaacttaaatagagaaccttatgtgtagtccatgtttctggactctatacctgattttgaatcactggacttaaattattggacttacaacactgatacatcttgtaaatgaacctaagcaaagaataccagccctacatcccactcccctcaagataactgggaaagacacaaagccatgctgaggaggagccatggtttgatattgtccagtgagtgtctcttggcctcagaatgctgccacttcctgcagttccagcccttggctgtggtccattctgagtaagtgaattcctctgttaaaacttgcacacaataaggagatggcgtcaccaacagccagagaagtcaagggtcctgatccatccagagacaaggtgaaaaggcaggctccagtatcttggttccaaatcttcaccttgcaatcatgtgatgaggtagcaattaaaggcatcaaggccaatgctcttggtagaaagacgcaggatgcgacagtctggaaatgccccttatactcacatattctgtttcgagtctgtcttaggtcccacaacgtggcttcacagccttctcctccaaagccattgctgcaggagatacacttgtgtccatccacactgacttcacagtaggtctgaatgtgctgctttgcaggaaacatatgagctacctgcagcccccgactgtcccataatctgagggttttatcttcagaggtctgtagtatgtatggttctctggggacccagcacaggtgagtgaccacgttcctggagacagatgctctttccacactctgtcctgtcaccacatcccacagaagcagggtgttgtcccgagagccagtgcacagctgtgatgagtctggactcacagccaatccggtgaccaccatggcatggccacacaattgctgccttggttgtgaggaaccgtgcaagtcccacatcatgaccatcctgtcacgagaggcactgaagaactggctggatttgggaatacaggctaccttggtgatctcatgttcatgtcctttgaaccttttcaccacatttccagttttccaattataggccacaactgtcttatctttccctccagagacacaaaggtctgagttcaaagcagccacgacagagacggtatccatgtgagctgggctatactcttgaaaagctttagtttgaattctctcttctataatttcatcaggcccgtatttataagtgctgtgtttgagtttgctttgctgtttccccatcacgacacaaaacctaaacgaaaccttctgtggaggagcttgtttcagttggcacctgagtagcagcatcccttgtggctgctggaagttgtgttccccccaaaccaataggatcttcttggttagctgccctattcaataatttgtaatgtgtatcctttggaaaatagttcaggcagccacttcttaatctctgtaattagtgggaagccactgaagttaatctcttctctgtctaagcatgtttgcacggtgggctgcggggctggagctggggccggcgggaacgcggagcctgggggtgggaac

SEQ ID NO: 12874 - RNA, 3615 nt, Homo sapiens
  source 1..3615: mol_type = other RNA
gctgggattacaggcatgagccaacgcgtccggcagaatggtaaatgtttaatatggaaaagggaacatttagtctggacagagaggacaataaataattatggctaccatttgtcaccacctttcctggcatttacttatttatttatttattgagatggagtttcgctcttgttgcccaggctggagtgcaatggcacaatctcggctcaccgcaacctccgcctcctgggttcaagcgattctcccgcctcaggctccccaggtagctgggattacaggcatgcaccaccacgcctggctaatttttgtatttttagtagagacggggtttctccatgttggtcaggctggtctcaaactcctgacctcaggtgatcctcctgcctcggcctcccaaagtgctgggattacaggtttgagccactgcgcctggcctttcctggcatttaaaatagctatgtccagtcttcagaacagccctgtggcgaggtatgatcatgaaacccacgttataaagtgaagaggaaacagattttataacttgcccaagatcatccagctaaatggagaagtggagattcaaagtcgggtctgactctttgtactagcttaagaacagactctcagctggatgtggtggctcatacctgtaatctcaacacttaaggaggccgaggcagatggatcacttgagcccaggagttttagaccacacaaacacacaaaaaattagccaggtgtggtggtgcatgcctgcagtcccagctactcaggaggctaaggagggaggattgattgagccctggtgattgaggctgcagttagccatgatcacaccaagagagggaagaaggaaggtggctgtcagtcactggtatcagagacaagcagaggacagagaagacaaatgcaaaatctttctttggctgggacttgtcagaaagggaatctccagtgttggtgatggtgtcaccaacagcctcatgtgccttatgtgtgggcatctctgaaggcagaaagaactccattttccctggaggaaaatggaccagtgagcatgaggctgaggtctgactcctgggggccacacaggcaggcctgagcaccttgcccctcctcactgaagggggcttaatgtctggggcacagttgactccatccctctcttttttcctgtatgtggttttttgtttttttttttttcaagacaaggtctcattctgtcacacagactggagtgcagtggcacaatctcagctcactgcaaactctgcctcccaggttcaagtgattctcccatctcagcctcccgagtagctgggactacaggcacgcacgtacaggctggtcttgaactcctgacctaaagtgatctgcctgcctcgtttttcctgtatgttctaatgttatttcagggatcccctttgcctcactctggccattccaaaacatatatatgtttcatttatataaatccaaatgaaaatattaaaattgcaagtgagatatttttggccttaatctttgaatttcaatgttttcttatctgtagagctggtgtgctaactcctgtaattctgggcaatgcccatgtggttcttggctgcttcaagccatctcaggtctgattttcacacaagctcagcagcactgggctagaagggtaccgccctcccactctgctgccactttgaatagaagtccaagctttcgctttcttgccctgactttgattcttcacattgctgaggagcagtgattgaagcttaatctcattgtctacagtccgtctcctctatggagctgcactattctttcccatctcaattatttctgatgtaaccaaaacactctctctccccactgccttttttcttttgtaaagacttgcaaagggtcagttccagaggctcgagccctgtgttctgactttcacagacagaggcctgccactcttacatttacaggtcatcattctgagcaatacactttttttgaagagtagtcctaaaagctcactaaaaagttgcatttgtatttaacttaaatagagaaccttatgtgtagtccatgtttctggactctatacctgattttgaatcactggacttaaattattggacttacaacactgatacatcttgtaaatgaacctaagcaaagaataccagccctacatcccactcccctcaagataactgggaaagacacaaagccatgctgaggaggagccatggtttgatattgtccagtgagtgtctcttggcctcagaatgctgccacttcctgcagttccagcccttggctgtggtccattctgagtaagtgaattcctctgttaaaacttgcacacaataaggagatggcgtcaccaacagccagagaagtcaagggtcctgatccatccagagacaaggtgaaaaggcaggctccagtatcttggttccaaatcttcaccttgcaatcatgtgatgaggtagcaattaaaggcatcaaggccaatgctcttggtagaaagacgcaggatgcgacagtctggaaatgccccttatactcacatattctgtttcgagtctgtcttaggtcccacaacgtggcttcacagccttctcctccaaagccattgctgcaggagatacacttgtgtccatccacactgacttcacagtaggtctgaatgtgctgctttgcaggaaacatatgagctacctgcagcccccgactgtcccataatctgagggttttatcttcagaggtctgtagtatgtatggttctctggggacccagcacaggtgagtgaccacgttcctggagacagatgctctttccacactctgtcctgtcaccacatcccacagaagcagggtgttgtcccgagagccagtgcacagctgtgatgagtctggactcacagccaatccggtgaccaccatggcatggccacacaattgctgccttggttgtgaggaaccgtgcaagtcccacatcatgaccatcctgtcacgagaggcactgaagaactggctggatttgggaatacaggctaccttggtgatctcatgttcatgtcctttgaaccttttcaccacatttccagttttccaattataggccacaactgtcttatctttccctccagagacacaaaggtctgagttcaaagcagccacgacagagacggtatccatgtgagctgggctatactcttgaaaagctttagtttgaattctctcttctataatttcatcaggcctgccgtatttataagtgctgtgtttgagtttgctttgctgtttccccatcacgacacaaaacctaaacgaaaccttctgtggaggagcttgtttcagttggcacctgagtagcagcatcccttgtggctgctggaagttgtgttccccccaaaccaataggatcttcttggttagctgccctattcaataatttgtaatgtgtatcctttggaaaatagttcaggcagccacttcttaatctctgtaattagtgggaagccactgaagttaatctcttctctgtctaagcatgtttgcacggtgggctgcggggctggagctggggccggcgggaacgcggagcctgggggtgggaac

SEQ ID NO: 12875 - RNA, 1616 nt, Homo sapiens
  source 1..1616: mol_type = other RNA
gctgggattacaggcatgagccaacgtgccaccagacgtaattctttaagacaaaaaagggagtctctgaagaaaagccacaaatgttcatccacctcatctattttgttccattagaaaatgcttagaggttagaacaggttagaatatgttaaaaaaaaataccagttgggatttggaataggtctaagggcaaccacatttaacataataacctctcctttgtatttgaaaatgacctcacattagcaggtgataaatctcaagctctttccagtaagagtggtggactctaccattctaaccccactcttgtcctgtatccctggacatgtccataggaggtgggcaggaaggtctttatgtgcacctgtgaaatggaactaagtttactggctccaaaaggttttgaatccatcacgtgggagagaatttactctcaaaatgacctgttctggatgagattcccctctttttttattgtgaagttgaagataagagtccgttttcggggtgggtaatcccaaagtgagcttgtttttttccacaaaatgttgtttggatttccttcgccgagggccacgtgatcccggcaggaaaacctcgttatgtgaacttgagctcttcacgtacggagaaaggctgctcgacttctcctccaggtcactgtcgctcagctctgaaaacggcttgctgcgacgggcaccatgctcatagtttgggcttaaaaattcactaccaagtaaagaagctgcactctgtggactctctttctgctcgccttttcccccggagagttccattgacgtctcctgggaagggtagaggggagccaaaggcagattttctaaagagctgtccgtggactccggcaacgcttccacagacagcagctgcccttcctccttcttactcttccagttcgggtcatagcggaggtctgaatatttgtcttctattggttgttgcctgttattggcgccctggtcccaggtatggtggttttgctcgcgagccatctgagctgcttttccacttgcttcctcttccatctcgtgcaggcttccccatcgagggctttcctcctcgtctaagctgtcgggctccataccgttgccccggattcgatcatcaaactcagaatggcacataatctcttgcgtgaggctttctgaatcagattccaaggagtcttttgaaatccgatgtaagtcttctttcttcaaaggtgggtgtgtggactggacatttaagttggtatgaaggacaggagattgaatagagagcttgggaattagtttacgtttactcatcttgaaaaatgcaaaaaattaacaggggatactcgtgttgataggagcagctggctgatatttaaagttgtggttcacaaaagcgttacctgcccggcgctcctccgcggccgcgacccggacgggccccgcatcctcccgcgccgccgccgccgccgcccgggcccccgcccgccccggcgctgccctggagaccgcagacaacacagacgccggcgccacatgggcggggcaggacccgacctaggatcccgcgtcccgaaccgcacccccggccctggcacggaggctgcaaacggccgt

SEQ ID NO: 12876 - RNA, 12597 nt, Homo sapiens
  source 1..12597: mol_type = other RNA
gctgggattacaggcatgagccaactgtgcccagccagccttagtatttatagacctggtttcctcaggtccaaatccctctccttcaatcaaatgttatacaactgcaactgtcctccacgtcgcctccatttatagagcattctatgaccttacctccccaccattaacttttccctggctaatttgaaactgcctgtacgagctttaaatgagttctttgtggacttcggaaagtgcttacattctcagcagttcctgtaatcctgtaaccaaagaagcgttgttgatggccaaggcttattcttcctacaaatatgattgagttctgacacctggtataatgttttctttaaaatgagagccaatgtaataaaattctttatggaatagtctgcaaaatgctttaatatattaataaaattaaaacaattttcacagaaaattttaataattttttctaacttcttttctgattgcacagttaattttaccatctagttacttcaataatattttctctgcctacagagcaaatataagggtaaattatacagaccctgctttagaaaggctcacaattcaagctggtctaacacgatgagtcaatgctatggaaaaacagaagagaccagttaattctattcagagtaagatcaaggaggacctcatatggatgaccttgggacttactggggtaactagaccgagaaggatgagtccattatcaggatttaagaatccagaactaagtgctaagtaaggggtttaaggaaagcatcagcaaaaattcactaattgttttcttttttttttttttttgagacggagtctcgctctgtctcccaggctggagtgcagtggcgcaatctcggctcactgcaagttgcgcctcccgggttcacgccattctcctgcctcaacctcccgagtagctgggactacaggcgcccgccaccacgcccggctaatttttttttttttatatttttagtagagacggggtttcaccgtgttagccaggatggtctcgatctcctgaccttgtgatccacctgcctcagcctcccaaagtgctgggattacaggcgtgacccaccgcgcccggcctcactaattgttagtttaaattaccacctacatgaagtcttataccctggctttgtattttatgttggctaaagagaatgattcaataagactataggataaaggcaccattaaaggtgcttcagtggcattctttcattgaggagaaatctgcagaagggtagcactttctagtaaaacatagtactctaaacacggttagcttacatgttcttccatttatttaagtgccttaaaaacaaaaggagaagcaaaaccctgaaagatcttggtttaattcttttcttctctaaaagtaggtttctgttttttggaggggatttaattgctcatctgatctgaatgcccatgaccagctcttgtttatcattggcatggccatgaacacaaacaatataaaatgccaatttaaccaatccaccatgcttgttttttcttttttcctaggaattaacagtggcaggccctggaaatagatgggtaagagcaaatctgtggtcatcaactaggtgcacagtccagtgggtgtgtgagatgcatgcacagggcagacagtagagcctgcaactgtgatggaattaacagggtaggccctgcaaacagatgagtaaaagcaaatctgcggccatcactaggtgcacagtgcagtgggggtgtgtgagatgcacagggcagacagtacagcctgcaactgtgatggaattaacagggtaggccctggaagatgagtaaaagcaaatctgcggccatcactaggtgcacagtgcagtgggggtgtgtgagatgcacagggcagacagtacagcctgcaactgtggcgcaggcgcagaacaggattgaatttcgctaaaaagacaaaggaagaaaaagtatggtctctgtcctcagggcattgcaacccattaggctgaatcatatgaactgcagattatgcaggtaaaatatggccacatatccacaccttcacagggctctgcctgacacacggaggacacaatcacaagagccaaagcagggaaggggcagggaaaaagtggacacaaccccaccccagtccagtggtgcggatcaataaatcgagacttacggccaatctgaaatagattctattcatgaaagtccttccagaaacaacattcaggatgacggcatcagtgttagccaagtgtctgagtggtctgggtgtcacatctgtgtgtgtgcccaaatggatgaaatttatgcacaaccaataagccccacaaaagtgattgttatgctgagccgaacaaccattttttacttccctttgtctctcccatagcttctctttccttttcacttcctggacctaccaaagccttggccttgggtggggaggcatccagtgactgtccttttcagcttcaacaatggcaacacaatctcttggctttgtatttgtgtaagagttccttttcacgatgagaatgtccaaaatagataccattctacattattcctttatttaaaaccacaggaaacatagaaacgagtttgaggaataccacttcaagatgggaatgggaggcaaaaataattcagccaactaggaggtgggcaaaatgctccgattccctttgttttcatatacgatttcattgaaggaagtggaagggatttaatagaaaagatatgatgatgacaaatcaagtcaatattgaaagaatactctaggcggggcgcagtggctcacgcctgtaatcccaacactttgggaggctgaggtgagcggatcacctgaggtcgggagttcgagaccagcctgaccaacacgaagaaaccccatctactaaaaatacaaaattagccgggtgtggtggcacatgcctgtaatcccagctacttgggagtctgaggcaggagaatcacttgaacccagtaggcggaagttgcggtgagccaagatcgtaccattgcactccagcctgggcaacaagactgaaactccgtctcaaaaaaaaaaaaaaaagtgtgtccaatcacagacttttgtcatttcttgagttctgaatcggctaaaacatccgagtgagttttctaacagtaaaagctgcatctctaggccactgaccacactgcagccctctgacagtgtcacactggcattattttgctgcttatggacaaaagaatgagcaatttcctgttggccagctctgaataccttattcactagaggctgagatggagtcagtactgctactacaggaacacgagtcaacatctcttaaatgctgtgtgccagactatgcgaagaaagggccttaaaaacattatctcatttaatcaccataagccttcgaagtagatgctagtattatccccatttcatagataactgaggagtggagaggtcagtcacctgcttcaagtcacagatcccataagtggcaaagtgagacagctggatgatccaacttcaaaagctgagcccccgcctgcttctatctgcttgatgcaaattcccaaaagtcaaaggcttctaaattcgcgctaattcctcaaatccctcctcttatcctggtgcagcctcagttggagtgacaggaagtttagatatgagtaagaaaacggaacctgacactgagttaaaaggacaatttcttccttcagagacaatcttactttatattaaacttcatttctgaagctccctgattctctaaaataatcaaaatgttcagcccaagatatgtcaaaatggtgaagaaatatcttaaaatccagttttcacccctctaacaataaagttaaatcctcccctttaatgggtctagtcagtggaagaacatttctctcattttaatcatttttctcctgatattttctctccttttaatcatttcttcacaaacatctgaatgtttatgctccaggcaagaggagagaaaatgatgagaatatccttatccctgggtgtgaggagtaattactctactgcccttttaaatacctttgaggtttatttcttaatttttttcctccaacttcagtttcacaacttcttcatgaaacaaggagcttggtaaaggaggccagcaagtaacaggttggctgtgagcgtgacatgaatgctcaggctgtaaactgtcttcctcagagagcagtgactccaatggtcagtgacatgcaggaggaaacgcaggattaggaccgactttccttaggtgtagcctcacgttttaatccctgaggtatgttgtaaatgggcagcgcatgaacaggtgatcaactcagaagacgagcttcataaaggttgccatagaactttagaatatgcctatggatggccaagtcacaaccagaattgagtccttaatcactgaccccatgtgtatttctatggaaggggagtgcagtatgtggcccaaaggttctgaaaaactgtgtgtgacagtctcctggctgtgtagcattttttgttgcttatagacaaaatttctctcctctatccaaatcagtaggccataggccattatttaagacaaacttttgagtataaaaaatttgtcttttacatacacaaatgcacacatatatagggtttgggacagactccacacccctaaaactagaggaaaaacaaggccctctagcaggtctgaacatgatgtaatcactttttcctttacttatgtaaaaggtaccctttgtcaaattagcacacttctggcaataattctggccccaaataaatagaaactttaagttgaaacttggcaattgtgaaatttccaaataattaaaaggtaaattttacagtaaagagactaatttttttctaattccatatgctataggctacaaaatatatatttaaattcccttaggtattaccaaatgtgtgttgaggtcctcaactggggttgagggaccctaactaggggttaatacatcatgcaaaattttccacgtattggaagaaacatcagaaatcagcttttgtgtgctccttaagccagttttaaaatagattttaaaatattcaccttccagctgattagcatgaaaggtttgaaaaatatacaaaagcagagtgctatggattgcatgtttatgtcctcccaaaattcatctgttgaaaccctaatctccaaagcaatggtattaggaggcggagctaataccataagtgggcctttgggaagtgagtaggtcctgagggtggagccctcatgaatattagcgccctcacaagaagggaaaggagagcttgcttgcttcctttctctctctctgccatgtaaggatgcaatgggaagatgatggctatcagcaaaccagggtaagggtgctcaccaggaactcaccttgatcttggacttcccagcctccagaacggtgagaaatttctgtcatttaagctacccagtgtatggtattttgttattgcagcctgagctgattaagacacagagtaactcacaaaataaataacatcaagtatcactggccaagccaatgagcagtcataccaaaagtagtttacttttaagatgtccatcttccacagaatctccaaggaagtagcttgcagtagtctcatccccacggaaatgatgcagtgattttatgcacaagggtaggagcaaaatgtgaactaatggtctacaaaactaatctcatctacaatagaagaaaacaagtcaggcctacttctccataccattcatgcctatggtggcaaaaggcagcatgagtctcatgctttgctggtgacattcaaatgtcagacagatttacttactcgagctctttggcggatgaaaagttttgtgtcaatacctcagggtttgctgcaatactaacaacctaaagaggaatgttcatggtcttccagggaaaaaattaaaaaaagaaagcccacaaaatagattctgaaatttcaggtttggtggggaaagaactgagagagaagcagagataggaaatggacaaatatatagactgaaatactacttaaggaggatacaggatttcttttaaaatacttgttctgaaagagatggtaccctcccccacctccgcccaagaggcagttctggaaatgtgagcatgttaggggtgccactgatgggcggccactactgagatttaacctgttggagcatgcgtgatacacaagccctgcagcttacagccctcacaacaaagagctgactcatcaacacaactttcaattgccccgcccaatattcatatagatgggaactcagtttacaataacaaatctatgatctcatttcattttatatataaacacacagaattttcagcccagttttaatatgctttggatttttcaagaatgcaatgagagaattctataaatggaaggaagcctatatactgagtgattatgagcaagaaagccagagccaggctgctttcattttaatcccagctctgccattattagcacataaccaggatgactagcacataacctgggtaactccctcatatgcaaaacgggactaacagcagtactcacctcatagatttattagaaaggtattagaacaatgccaggcacacagcaagcactatatgagtgaagccattacagactaggtatgcctagaactttatctaaagaattggccacattttagaaaatcatactgctgacatcgacccctttcctggtattgaactgccaatgcagcaggtctgaattggtaactaccacattcatggtgatttttcacatatttatatttatacacacacatacaaagtatgtgccctgcttagtagtttaattacatcttgtaatataaccatgctagaatatgtacatatgaaaataattatttcattataaaatatcttatctgtttcagttagaacgtcactgatgggtatgttttagaggctagttatattacctgctagtttcatttcagaatagtaaatggagtgatgtttttatgagtgaaggtaagcttcatcatccatgattttcatttgaagattgaaaagtgatgctataaaatattataataggggtaggtgttgagttgtgtctgggagagttttaacaatcactcttgtaaagtatcctgtcaaggagttcaagatcagcctggccaacatggtgaaactccatctctactaaaaatacaaaaattagccaggtgtggtggcgggcacctgtaatcccagctacttgggaggctgaggcaggagaattgcctgaacctgggaggcagaggctgcagtgagttgagattgtaccactgcactctagcctgggtgacagagtgagaatctgtctcagaaaaaaaaaaaaattttttttaaagaaataaaaataaagaatcctgtcaaaaagcatcatcaagcaacttcatatgtgaacacacgtccacaattaaacctggattactactgaggcaagcagtttccattaatttctaagaaatccatattaaactattatttatgtatgtccatagtagaggtttacaaaggttttttttttttagcagcaatatatttttcaaacacaattcaggagaaaacctcaaataaaaagaaagatgaagctgtggagggtgactgcaagtagaggagccaggaacttctctcgcgggtcctgggactccagggaacaaaggctgaaaagcaccaatctggttggccactgcctataatgaagactgactgccgaatattcacttaaaggatggctgttcaattcacaagtggcattttccccacagaaaaagagctcaccagccagctaaggcctccagagtgatttaactcatcatccagtggaactacagctcttagagttctccccacaatctggggagtaagaggagatgttgccacccacttcctgggcataaagccagctcaagacaagagtaaaacaggcagggctggctcgcccctcgtacacagctccctcctcatcaccagtgccctacacgagacctccccagcccacaccccaccctcctagtgtgttgaacaccctgtggtcacacactgcaagcctcttctctccatctgccaaacacccttgggtctccatgtctccatgaaataccagatctttttctttttgttttttttttgagacagagtctccttctgtcacccaggctggagtgcagtggcctgatcttggctcactacaacctccgcctccagggttcaagtgattctcctgcctcagcctcccgagtagctgggactacaggtgcccaccaccatgcgaagctgatttttagtagagacagggtttcaccatgttggccaggctggtcttgaactcctgaccccaggtaatccacccaccttggccccccaaagttctggaattacaggcatgagccactgcgccaggccgaaataccagatcttcatggcagttgtcttagaggtagagaagaaaacagccagactgagccgggtgtggtggctcatgcctgtaatcccagcactttgggaggctgaggccggcagatcagttgaggttgggagtttgagaccagcctggccaacgtagtgaaaccccgtctccactaaaaatacaaaaattagccaggcatggtggcgggcacctataatcccagctacatgggaggctgaggcaggagaatcgcttgaacctggaaggtggaggttgcagtgagctgagattgcgccactgcactccagcctgggtgacagattgagactccatctcaaaaacaaacaaacaaacaaaaaaaaccagcctgactgaattcagtcacagtaattatacatgagtggttgctagttcctttaaccacaccagaagcattttaaagggaagatgtttcctaactccagtgattttcatgggctgaattccaggcagttcagcaaactcaacaattccggtggtatgagaaagggcattttggagtaggagatttcggctctgcctaggaagatacctcagaaaattcccctcgtgcaatttcactttgcatatgcttctcctgttcttccatttctaatccataaaatcccaaaatgcttgggagggtttattttgattttttttaacaatactgccctgctggcaacagccacgatagtcacttgctcatctgaaaatgccttgcactttctttttcactagcttcgtgtatgacgcaaaacagaaatatttcaattacaggtgactaagagtaagaaaaatatacaactatatttaaaatacttaaattaacaagatagtacttttccattctaacaaaatatcatacattcagtttaaacaagagttaatatccagacacacgttttcaaaatacctgatgctagttgaaaattagtgaccatgaggctttccaagatatttctaattagcaaactgtgtacaattttgaagaagtgtacacaccgtgctggaagacagacactgaacaggtcaaaatgcaaactcatgtatctttcatcaacctaaatcttgttgcttcacttttctaaatgatactttggctgtcagcgaatcttatagcttcttttcccttaaagacaataatatataacaacaccaccccacacaaataaccataaacttctttgtgtgaaataagccctatcaaaatgtgttcatgtatttctgtaccaactgatctatactgagactgtcatgaaaaaggtatcaaacaagtgtaacaggcctacacttaaacctctgcctcaaaggagaaatcagatacttgccacgttattgcaaagtcaaagctgctacacttaaaatatggtagatagtttagaaaaatcaaatcaaaaatgttttctcactggctttttcagataaagaagttggaccacaaaccaacacatctgtgtgaaaacagccaccaatttgagtccccccagcccctcaaaaaggaacaatgccaccagtccctcacaatgaccataacgtctctggccaggactgcgatttctagcgcgtgtcttcacattctatctctggggaagcaagacaaacaggctctacccatttccctccttttgtctccacaagccagcacctaagatcctctgaatttgttcccatccaatcctgcaaacttccaagaagggcagtagataacttttcaaaagaaaaagaaattgcataaggtccctacataatactgaggctgaaacgagaagaggctgtccactgtaaaagcaaggcacttggggcaggagccaggcaggtggcctgagcagggtccctctcagtgagtcaacagtttgaggcgcgtaaaccagctgaccaggagggacggttctgtggacgaggacttcgtagctgaggagccagatttctttttggtcccttcctcctggaatggaatcgtggcgctgctgtggagatctgagttgatgtagcacctgcttcctcggatgtagtccgcaccccggaccagatgccgctcggtcgtgggtctggagaaccggtatgggggagaggagctctcttcaatgatcggaggaatccgctcgttactgaaataccggcaaagggcatcctcccctttcctgccatgacctcgaggtctggcaaaagggtccacaatccccatccagttcccatcagcaggcatggacaaaggccgtggcttgccataagatggtgttttctctctcatttttgtgggcagaatgttggtttccaccgagtacccaggcaactgatccgagtctgcaatggtgaatcttcgtctccggctttcctggtccaagaaggaattcggggactctgaacccttaggaccaggcaatggttgtttgcacttactggaccctccataaacaaaactgccattctcatcccggggagagtagggaacagcaggcggaggaggaatataaagatccaggatggctgacttctccttcttcagtgaggtatccatagtgctttcaggggactgggttgtcgcgggtggaggtgaggtctgtacaagaggtggcttccaccgtaggtttttcaggggagcaggagtaaagttgaaagacccggtggggcgcttcttaagcagtaacacaactccggtgggattctctctcaatttcttcaccagatttttcagctgccatcccaccacagtttgctgattaacttgaatgacttcgtcaccagcatgaatcttctgagatctgtctgcaggagaattttctgtggttccagtaatcacgtgtaacccatcataggttgatttgatgtacatgcccaggccttccccaggtttaatgtttggtaagtgaacttcctccagacatgcacactggctcatcacaggatctgtggtagatcggattgttttgtcacagatgccatttaaaaccttgaccacagttaaaactttatcctccatttccgctacaaagcaatccttctggactgtagtggtcaggtccaagcaaagctggataattttgttcttcgtgactgagaaatcagtgatccctgtaaacggagcccggtccagccacgccagcagggccttggcggcgccgatgagctccaccaccgaggtcaggaactcattgggggccttgcgggaggtgttgccatcgtaagcgggacttttccgtcggctacttatgtaattctgtaaattgtgggaagatgctctcagtttcagaaccaagttcttcatgttatcagtttcgaggccataattcagtgcacagagaaggtccacagcctccaacacaagctcctggtgtccaatccgtgtgacccccagctcctccaggtcctgatgggaaatctgcagcagctgctcgccgttgatcttctctcgttcaaacttgtggacatattgttgcaggcagtcatccaaccctctagtccagtccaccacttgtttggggctccacttggtcacgggttccatggtaaaccgcttcgcctctcgctgggctggagagtcgcagataaagtgctgctgcctgcgctccggtgccccttcccgggagggcgcgcccgcggctgctcccctgcgcccgagcgactccgtcaagactgcatggccgcggtcagccagtcgtcccagcgcggctccgccaggggagcccggccctctccctccagctgccacagtccagctgcagctcctccttcccccgccgccgccgggatcccgggcacagctgctgctcccgagcgacggcagctgcaggcacgccgggctgcgaccccagacccctggcctcggctcggcacgggagcctcccggcccgcgaccacttcctcggatctctcgaggcgcgatcggctctccctcggccggtcttctcgcctgctggctctccggggtccccgctccgcgtgcgctggcgtcccggagccttcccggcgcaggtcccacctcctgcgccgccctcccgtgccgccctggcagggccgagcgcagagcgtgcgcgctcgggttgcaaagtttcagctccggttgctgcaaaccgaat

SEQ ID NO: 12877 - RNA, 3249 nt, Homo sapiens
  source 1..3249: mol_type = other RNA
gctgggattacaggcatgagccaagtgttgtcagtttctatcgtggaacctacacatattcagatatgcggcaatggtgacagacaacagtaaataaaccatgtgtacataataagcatgaaaatgtgaaatttcctttgacaatcaaatcttccctccaaagaacttagttttttttccccttaagtttcactaggtgtttacccttacaaaactcatcaattgcagttggacagactttttttctgtatttttcttggtctcctccccaaccctcttacttaggacagtattattctgctaggactgccataacaaaatgccacagactggatggcttcaacaacagcagtttatcaaccgaagtttattttctcacacctttgggggctgaaagcccaagatcaaggtgattgcagggttggtttctcctgaggccccctcctcggcttgcagacggccaccttctcactgtgtcctcacgtggcctctctgtgtgccttccacctaagtgtctcttcctcttcttaggacaccagtcctaggccaggtgcagtggctcatgcctgtaatcccagcactctgggaggccgaggcaggtggatcacctgaggtcaggagtttgagaccagcctggccaacatggtgaaaccccgcctctactaaaaatacaaaaacttagccaggcgttgtggtgcacgcctgtaatcccagctactcaggaggctgaggcatgaaaagtgctcgaacctgggaggcgggggttgcagtgagctgagatcacgccactgcactccagcatgagtgacagagcaaggctccatctcaaaaaaaaaaaaaaaaagggaaaaaaaggacaccagtcctacaggattagggttgcattcttatgacttcatttaaccttaatcacttctttaaaggtcttatttccaattacagtcacattaggggttagagctccaacatatgaatttgacgcaattcagtccacaacaggtaccacctgtattctatctctttcttcactctccccaccaccactctgtctctattctcaggcaggagtattatagacgcatttccattacttgtaaacatgtacacatttgttaaagggttagatgcatttaagttgggcatcaagccgcaggccaggaaagaactctagtctctaccactaggcaaagtcatagatctcaggagagaaaaagaattggaattcccaggttacacagatcggaaagcaagcagcaggataatgtgatgagattataattttaaatccagagatagaaaagtaaaggaagtttctttcattttcctgtcatgcatatgaccctttctttattcaaaagtatcaaaaagataggctgggtacggtggttcacacctgtaatcccagtgctttaggaggctgaggtgggaggattgcttgaggccaggagtttgagaccagcctgggcaatgtggcaagaccccacctctactaaaacatacaaaataagccaggtgtggggggtgtgaacctgtagtctcagctacttgggaggctgaggtgggaggagatcatttgagcccaggaggttgagaatacagtgaactatgatcataccactgcaccctagcctgggtaagagactgagaccttcatctccaaaaaacaaaacaaaacaaaacaaaacaaccacaaaaacaattatatgtacatataagataactgaagagaaatgccagattcttgttatgaagtctcctcaagtttctcatggagatttatttggatgggcatagcctacctcccagagtaaagtttgggtctctctctcaggtaggcatttccgatgccctagaatccattcccagtggtctggcattgggtaaagagggggtgccgcctggagtgctgccagcgggccacagcatcaccccaatgctccaggccaaaactctccatcacaggctggtgtcgaccagctgcccaggctgttgaagcacctgcttcctcctgttgatagcattcagaactttcttcctgggacccagctgcatttgtatgctctgaaggtcctcatcagagcagagcagcagagcttctagatcaatctgctctctcttgaagataggcaggaattcttccaggtgctgagacagcaagaacacttccaggggcgtggcatcgaccacatcttcctcccactccacttcatcgtcatcccacggcagatcatctttgaggccgttttcctctccctcttcatcagctgcaccctcatcagcctctgatgctccttgtctttgaagcaattcactgggcagtttaaaaccaaactctctcttgctatctgagatgtcttcaggactcgatatcctgttccttctaaaaacaatacttcctagacctggacgattgagaatggattcatggtgcacactgccgtcctcctctgctgacaactggagcttctctttgaagtcccctgagaacgagtcttcctcttcctctctgaacacttccatcacgttcctctgcccacttctgccttccttccccacctgttctgctgtatctttgttcttcttgaacttgatcttgaaagtgtctttaatgcccttagatagtgacccgaatgtgccaggagcagaagcatttgaaggggatgatctggagaaggtacccttggaagaagagagagtcccggattcctccttgctgtaggtgtgggccatcttattttggtgcttctcctggagcctctcacactctttgatctgcctcctggcattcttctgagcctgctccttcagcctggtgaccttcttggggttcatgatgttctgtgcagtggcagccttgtccaggagagcaacacattcattctgctccctgctggcagcagcatccagtggagtctgtaagtcattatccagggcaaagatgttggcaccaaagttgaccaggaatgagacgcagtgggcatggccattggaggctgcaaaatgtagaggagtgtttccccagatgtcacacctatcagggtcccctcctctactgcagattatctctagggcttccaagttcccatggtaggctgccaagagagtaggagtcatgccgtcttcatccgaaagatttagatctcgcttggtagcctcttttagaagttccaggtaactatcactagcagcttggtggtaacgagtagacatttttcctgctcaccagaacttggccagatgtctctccag

SEQ ID NO: 12878 - RNA, 3160 nt, Homo sapiens
  source 1..3160: mol_type = other RNA
gctgggattacaggcatgagccaatgccccggcctgacagacactttttaaaataagacatttatgtggccaacaaacatatgaaaaaaagctcatcatcactggttatcagagaaatgtgaatcaaaaccataatgagataccatctcatgccagttagaatggctatcattaaaaaggcaggaaacaacagatgctagagaggacgtggagaaacaggaacacttttacactgttggtgggactgtaaactagttcaaccattgtggaaacagtgtggcgattcctcaaggatctagaaccaaaaataccatttgacccaggaatccctttacagggtatatacccaaaggattataaatcattctactataaagacacatgcacacgtatgtttattgtggcactgttcacaatagcaaagacttgaaaccaacccaaatgcccatcaataatacactggataaagaaaaggtggcacatatacacccatggaatactatggaatactatgcagccataaaaaagatgatttcatgtcctttgcagggacatggatgaagctggaaaccatcattctcagcaaactaacacaagaacataaaactaaacattgcatgttctcactcataagtaggagctgaacaatgagaacacatggacacaggtaggggaacatcacacactggggcctgtttgggggtgagggggtaagggagggatagcattaggagaaatacctaacgtagttgacaggttgatgggtgcagcaaaccaccatggcatgtatatacctacgtaacaaacctgcaagttctgcacatgtaccccagagcttaaagtatataaaaaaaagaaaaaatctcatgtggcagattaaagaaaaaaaacttactaaggtatatgcatatgtagatattataaccattaattcaaaaaagtcctataaaaacattccccattactgagcaattgcttattccctttgtcattaaaacatgcactttgatttacttcaaaactgaggggactagtccagttttgtactcttgtaaattatgagtctttcttgaagaaatctgcagcattacacaaaattgaatcagatattcagattcacaagatttgtgcctccttatctcacacattcataagttggaactcttcatttgcagtttatctatattctgtttcatggaactagggagcatcccctgcctaactctgtaaaaccaatttgtcaaactcttgtacagatcagaaaagtaaaggaattaatataaatacctccagtaatagggatgcacaagggtgatgacaattttattaatagattatagtagtatatgcttatatttatagattatacacatcacacacacacataaacatacacactcacatttgggtaataatgcatttgccatcagtaaggaacataaatgaccttattgtttgagtcagacaaatattaatttgaatcagagcttaactaccatttatttgagaaatctcaggaaaattaactaatccttcctaaatttattgttcctattggcaaaatggggacaatatgttatagctagaagagttgttttcttgagtcaaaaaaatgtatatatataaagcacttgatacttactaggggctgaataaattgttgaaatcaccactgtaataatagtaaaagaacttaatatgaatacttaatatggatagaaaactaggaggcccactggaaataccatatatgcaccataatattaacccagttagcttcatctatctccaaccttatttgttaataacaagttttaaattatacaggccagactccaaactaattgtctttctccttcatttcagaaaaattttccaaagatgacttaaaataacacttgaattggagggaggaaggaaagctaatattattagagcacaacatcttaaattttaaagaattatatttgagaggaatatatacaatagacagcttggaagagcattctgggtagaaataagattcacctctcttccaatctgaaacataataacaatgcctttcatttgtatggttcttcagagtttaaacatggcttttaagcacatttttctctgaggaagctcttcctttgacagcatcttcctcagtgctgccttcatggaatcattccgtaagctataaatgactggattgagtgttggaggtatcacagtatagaatacggagaatacaaggtccacagtcgatgaggaatcagaaggcagtctgagaaactcaaagcctgcagctgaaagaaagaaggtggctacaaataggtgtggtaggcaggtggagaagaccttggtccggccctcagctgatgggattctcagcactgtagagaagatgcgaatgtaggagagcacaatggagatcaaacagataaatgctgcagacgttgtgaatgcagccagtgcaatctcattaatgaattcataagaacaggctagtttcagcatctgaggaacatcacagaagaattggtgaatgactctcttcccacagagaggtatggagaagttaatggcagcatgcatgagcccagagaggcccccagcaatccacacagctatcactgcatgcctacaggcacggggatccataatagtctcataatgaagtggttgacagattgctgcgtacctgtcataagacatcactgtgagaatggccacttctgatgaggccagagctatgaagaagaaaacctgaagaatgcactgaacaagagaaatgtaaccgttgcccataagtgaatttgcaatggactgggggactgtgacagagatgaagcagaggtccagaagagagaggtgctttaaaaagtaatacatgggggaatggagacgacggtccacggtaatgatggtgataatgaggaggttgcctgtcaaggccagcaggtatgtcaccagaaataccaatgcatgtaaaatctgaagcttacgctcatcagaaaaccccataagaaggaatccactcattgaagtcaaattgaccatagtctctctgaagataccaagtgtgactcagagtggatctctcggtagaaacaaatctcaattgatcctgagactgagcatctttgttctagaatcaagctggtgtttcagtcag

SEQ ID NO: 12879 - RNA, 1522 nt, Homo sapiens
  source 1..1522: mol_type = other RNA
gctgggattacaggcatgagccaatgcgctcagcctaaacacatacaattctaaacactcagaaatgcacacaattcttataaacatgatctacccagcacctgttcatggtgaagattttgaatgttattggagcgaggttttcatgtgatcatcaaatgttggcccactcggtggctggactgaaacacgaaaactcccgaaagctctgcctgtgacccatcaccagtcagcttcctgacagccggggaatgagtgccttcactctgaagcagcatctgagagcacaccatatcatctgctacagaagttgtctgaaaacgaagggcacgcctgtttcagatctgagctggcactaggatgtatccttcgcctctggaatctggagcccgcaccgactccacaggcggggcagaggccaaaagtcaggcctggaggctgatttctaagcagacagcccagctctcagcagaacacctaatccatcacagtgatccagagacacggctccactggggttttatcccatgtaagaggagagggaacagggatgggtgccccaggtcacaccagcagactgagggatcctttgactccccattttttccagcactccagaatattgagaataaatgacacatttactgagaccattcattcaaggtggttgcatgcaaatgaagttattgtggcttacatgtgtgagttattacgagttcaaggccatgtgtctgaatataagctgggatgccttttcttctcacctaggagacaatagaatgttccatgaggatcaaagagccatgagggccaggccaatgtgggagaaggagtgtggagagaggtgtctgggaaaagagaaaatcggcagtaccactaggcgcattagaatagagtaaggagctgccagaagacgtgagctgggagtggacagcccccacaggtgcaacgtctcagccagcagcaccaggcaagagatggtgaggaagaaggagttgattcagatcaagtccaggaaccaatgggaactgtctccaggctggccagagcaatcctctgcttccacgactgcctgagagagtccagtcactgcacactcatgtcctcactgcaggatcaacactgtggctctggaagacctgactgaatgagtatccttggtgacctcccaggagaagtcactgaggggatcagagtgcgtaacccactggctgcacccagggcctctgaccaaacaggaaagatggagagcaagcagttggctggcccaggacactcaggccagatgcaggaagggttgttgcatttaataaaaatgagtgttaaatcatgatctgggagaaattggaagcttcatcaccactggtgggaatgcaaaatgatgcaggtgcagccaccatggaaaacagttcggtggttcatcaagttaagcacagaattaccgcttgacccagcaattccactcctaggtatataccaaaaagaactgaaagcagatgttcaaacaaaaatgtatgcagaa

SEQ ID NO: 12880 - RNA, 2796 nt, Homo sapiens
  source 1..2796: mol_type = other RNA
gctgggattacaggcatgagccacaacgcccaacctttttttttttaaactttaattaaatgctactttctcatagacttccctagactggtttgcaatctaaggtaataggaaacaaggcattgggcattttgaagaaactgcaggttaagctatggtgccaagcagaagactaaacactgatttgagtgtcaaatctccagcacattctgggatagaggcaggttctcaaatgtttcctagtgttctttccttttcactaattaaattttcccttctctggcgaatccagtgcagtatacaaccccctgattgcctctcttggtcaaatagttgttagaagggaacctgtcaggcacctgtggcttcggcttagattggaaaggtgacagactagctctgattcacctcctcctgagacagcctggacagtggagggatcaactggaaggccgaaacctggtaacagctgcctctgattcctggtggaaatgaccaaccagattcaatccatatcactgggaaagatcaaggaaaaaaaatagcttcccctccaaaaatggtaaagaggaaataaggagacaagaaaccaaaaatacttagaatggcacaaaaagtgatacgcataaacttctttttgttattacatctaactgtaagtttcctaaagtccagttatcaagttgaattgtgtggatagaggagagaggccaactggattttctctcaagagttcacggcttcagtctgagaggtcctgggtttgcgctgggggagcccctttttgaatgaaggcgtgggagggctgggctccatgctgactccagttccattggtccctgcagagtgagtctggcctctttcaatggtgtttcctggtgcctgagatggagcactctgatacctggaaccagatgaataccacgagctgtttctgtaacgacccatactgtcatgccgcccttggttcatggggtcattggacttttggccttgtggcctatagccctgtcctcctcgtctgttccctggcaatacctcccgaagtggctggtagggctggccactggagtttgctatggctgcaggagtctctcccggtgcaaagtttttcttgttagcacttgtaaggctgggaggagaggcacaggtggaagaggaagcagcagaggcatcacttgggctactcaaggacacagatgtaactgagctacatcgggatctggtcgaatagctgttctttggatgagacacttgtccaaatgaatcaatgctcttctttagggtctctacatcacaggtgaaccgggctactcgtcccagatcctcatcatatttacgttcactaacaaagtgcttgatatcagctctgagctcaaccaattgctgctctgacatttgaacagccacatgagtcatcttctttagaagttcagccttcttttgtcggctgagcaaaatttccattgcttcagctttcactttgtccatttcagcaagcaacgccacttctcgatccattaaacagctctccaattcagcaaaggcttgtttcattttcttaatggaggcatccatctcttctttaactacaactcgataccgtgcaagagacactgtgcagcgctggaggtcttttacagatttttcaatattggaacttagctttttactggtggcgaggggaacatcttccatccccatatttgaaaactgagtttctgtggtaggtcttgagagagatttggcagcattcctgggttgttgagaattgtgaatagagtgcatagtcaaagacttggtctcaaaatcagagacaccattctgcagcatggatcctgttctatccagcgtatctagcatggcagactcgggatcctccaattctctggcatctattgaaagtgtctccaaaccttcactgagtgagtccacagactcagtgtcattgatggcaccattgacatggtagccattcataccacctttctctgaggaaggcgcagactgttcctcttgaatggaaactgatttactggaatctgggatgccgttacttggttctgcggcaggtttcggtttgtttttcttctttttgttctttttcttgcctgttactgtccattctttgagtacttcactggcactaccttccatgaatgcttgtactgttttgtccacacagttatcaaagtgctgcaaaaccaggataatttcattgttgctcttattaggaactattgcacgtaccgcatttatcttctctttcatgttctcaaaagctcctccctgggccagtacggtattggactgcaaatcaaaaatgaatcctgatgaatccttctggttctgtttcctggacattgtcgtttcttcgatctcaaaaaatatacaagaaaagtatccttttgccttgtctgggttttgagtgtaggtatctctgatttaaaagtgggcaacggaagtgtgcagttggaagcaaaaaatacgaaatcctgctgttcgaaattctgctcactagctgttaatctcctttccttttcttgtatcaacttcttgtcaggaagtatcattgcagacattcatgtctccttttccagggagattatatgaggtaaccagggtagtcacattcatagagacagaaagtagaatattggtagccagcagctagcccaggcccccgcaatcgcctcgtcgccccagctccgggctccgcgtcccggacgctcccgggtctgagaagaggaaaggagatcctccacctccccttctagagccaccgccgccgtcgcc

SEQ ID NO: 12881 - RNA, 2720 nt, Homo sapiens
  source 1..2720: mol_type = other RNA
gctgggattacaggcatgagccacaacgcccaacctttttttttttaaactttaattaaatgctactttctcatagacttccctagactggtttgcaatctaaggtaataggaaacaaggcattgggcattttgaagaaactgcaggttaagctatggtgccaagcagaagactaaacactgatttgagtgtcaaatctccagcacattctgggatagaggcaggttctcaaatgtttcctagtgttctttccttttcactaattaaattttcccttctctggcgaatccagtgcagtatacaaccccctgattgcctctcttggtcaaatagttgttagaagggaacctgtcaggcacctgtggcttcggcttagattggaaaggtgacagactagctctgattcacctcctcctgagacagcctggacagtggagggatcaactggaaggccgaaacctggtaacagctgcctctgattcctggtggaaatgaccaaccagattcaatccatatcactgggaaagatcaaggaaaaaaaatagcttcccctccaaaaatggtaaagaggaaataaggagacaagaaaccaaaaatacttagaatggcacaaaaagtgatacgcataaacttctttttgttattacatctaactgtaagtttcctaaagtccagttatcaagttgaattgtgtggatagaggagagaggccaactggattttctctcaagagttcacggcttcagtctgagaggtcctgggtttgcgctgggggagcccctttttgaatgaaggcgtgggagggctgggctccatgctgactccagttccattggtccctgcagagtgagtctggcctctttcaatggtgtttcctggtgcctgagatggagcactctgatacctggaaccagatgaataccacgagctgtttctgtaacgacccatactgtcatgccgcccttggttcatggggtcattggacttttggccttgtggcctatagccctgtcctcctcgtctgttccctggcaatacctcccgaagtggctggtagggctggccactggagtttgctatggctgcaggagtctctcccggtgcaaagtttttcttgttagcacttgtaaggctgggaggagaggcacaggtggaagaggaagcagcagaggcatcacttgggctactcaaggacacagatgtaactgagctacatcgggatctggtcgaatagctgttctttggatgagacacttgtccaaatgaatcaatgctcttctttagggtctctacatcacaggtgaaccgggctactcgtcccagatcctcatcatatttacgttcactaacaaagtgcttgatatcagctctgagctcaaccaattgctgctctgacatttgaacagccacatgagtcatcttctttagaagttcagccttcttttgtcggctgagcaaaatttccattgcttcagctttcactttgtccatttcagcaagcaacgccacttctcgatccattaaacagctctccaattcagcaaaggcttgtttcattttcttaatggaggcatccatctcttctttaactacaactcgataccgtgcaagagacactgtgcagcgctggaggtcttttacagatttttcaatattggaacttagctttttactggtggcgaggggaacatcttccatccccatatttgaaaactgagtttctgtggtaggtcttgagagagatttggcagcattcctgggttgttgagaattgtgaatagagtgcatagtcaaagacttggtctcaaaatcagagacaccattctgcagcatggatcctgttctatccagcgtatctagcatggcagactcgggatcctccaattctctggcatctattgaaagtgtctccaaaccttcactgagtgagtccacagactcagtgtcattgatggcaccattgacatggtagccattcataccacctttctctgaggaaggcgcagactgttcctcttgaatggaaactgatttactggaatctgggatgccgttacttggttctgcggcaggtttcggtttgtttttcttctttttgttctttttcttgcctgttactgtccattctttgagtacttcactggcactaccttccatgaatgcttgtactgttttgtccacacagttatcaaagtgctgcaaaaccaggataatttcattgttgctcttattaggaactattgcacgtaccgcatttatcttctctttcatgttctcaaaagctcctccctgggccagtacggtattggactgcaaatcaaaaatgaatcctgatgaatccttctggttctgtttcctggacattgtcgtttcttcgatctcaaaaaatatacaagaaaagtatccttttgccttgtctgggttttgagtgtaggtatctctgatttaaaagtgggcaacggaagtgtgcagttggaagcaaaaaatacgaaatcctgctgttcgaaattctgctcactagctgttaatctcctttccttttcttgtatcaacttcttgtcaggaagtatcattgcagacattcatgtctccttttccagggagattcggggaaaggaagagactcggggagagggttggggacaaagtagatggaaggggaaaacgggtgggacgcgagctcgcgtccgcgtgcagcacagctcgtacccggcggcatc

SEQ ID NO: 12882 - RNA, 2733 nt, Homo sapiens
  source 1..2733: mol_type = other RNA
gctgggattacaggcatgagccacaacgcccaacctttttttttttaaactttaattaaatgctactttctcatagacttccctagactggtttgcaatctaaggtaataggaaacaaggcattgggcattttgaagaaactgcaggttaagctatggtgccaagcagaagactaaacactgatttgagtgtcaaatctccagcacattctgggatagaggcaggttctcaaatgtttcctagtgttctttccttttcactaattaaattttcccttctctggcgaatccagtgcagtatacaaccccctgattgcctctcttggtcaaatagttgttagaagggaacctgtcaggcacctgtggcttcggcttagattggaaaggtgacagactagctctgattcacctcctcctgagacagcctggacagtggagggatcaactggaaggccgaaacctggtaacagctgcctctgattcctggtggaaatgaccaaccagattcaatccatatcactgggaaagatcaaggaaaaaaaatagcttcccctccaaaaatggtaaagaggaaataaggagacaagaaaccaaaaatacttagaatggcacaaaaagtgatacgcataaacttctttttgttattacatctaactgtaagtttcctaaagtccagttatcaagttgaattgtgtggatagaggagagaggccaactggattttctctcaagagttcacggcttcagtctgagaggtcctgggtttgcgctgggggagcccctttttgaatgaaggcgtgggagggctgggctccatgctgactccagttccattggtccctgcagagtgagtctggcctctttcaatggtgtttcctggtgcctgagatggagcactctgatacctggaaccagatgaataccacgagctgtttctgtaacgacccatactgtcatgccgcccttggttcatggggtcattggacttttggccttgtggcctatagccctgtcctcctcgtctgttccctggcaatacctcccgaagtggctggtagggctggccactggagtttgctatggctgcaggagtctctcccggtgcaaagtttttcttgttagcacttgtaaggctgggaggagaggcacaggtggaagaggaagcagcagaggcatcacttgggctactcaaggacacagatgtaactgagctacatcgggatctggtcgaatagctgttctttggatgagacacttgtccaaatgaatcaatgctcttctttagggtctctacatcacaggtgaaccgggctactcgtcccagatcctcatcatatttacgttcactaacaaagtgcttgatatcagctctgagctcaaccaattgctgctctgacatttgaacagccacatgagtcatcttctttagaagttcagccttcttttgtcggctgagcaaaatttccattgcttcagctttcactttgtccatttcagcaagcaacgccacttctcgatccattaaacagctctccaattcagcaaaggcttgtttcattttcttaatggaggcatccatctcttctttaactacaactcgataccgtgcaagagacactgtgcagcgctggaggtcttttacagatttttcaatattggaacttagctttttactggtggcgaggggaacatcttccatccccatatttgaaaactgagtttctgtggtaggtcttgagagagatttggcagcattcctgggttgttgagaattgtgaatagagtgcatagtcaaagacttggtctcaaaatcagagacaccattctgcagcatggatcctgttctatccagcgtatctagcatggcagactcgggatcctccaattctctggcatctattgaaagtgtctccaaaccttcactgagtgagtccacagactcagtgtcattgatggcaccattgacatggtagccattcataccacctttctctgaggaaggcgcagactgttcctcttgaatggaaactgatttactggaatctgggatgccgttacttggttctgcggcaggtttcggtttgtttttcttctttttgttctttttcttgcctgttactgtccattctttgagtacttcactggcactaccttccatgaatgcttgtactgttttgtccacacagttatcaaagtgctgcaaaaccaggataatttcattgttgctcttattaggaactattgcacgtaccgcatttatcttctctttcatgttctcaaaagctcctccctgggccagtacggtattggactgcaaatcaaaaatgaatcctgatgaatccttctggttctgtttcctggacattgtcgtttcttcgatctcaaaaaatatacaagaaaagtatccttttgccttgtctgggttttgagtgtaggtatctctgatttaaaagtgggcaacggaagtgtgcagttggaagcaaaaaatacgaaatcctgctgttcgaaattctgctcactagctgttaatctcctttccttttcttgtatcaacttcttgtcaggaagtatcattgcagacattcatgtctccttttccagggagattctagcccaggcccccgcaatcgcctcgtcgccccagctccgggctccgcgtcccggacgctcccgggtctgagaagaggaaaggagatcctccacctccccttctagagccaccgccgccgtcgcc

SEQ ID NO: 12883 - RNA, 2880 nt, Homo sapiens
  source 1..2880: mol_type = other RNA
gctgggattacaggcatgagccacaacgcccaacctttttttttttaaactttaattaaatgctactttctcatagacttccctagactggtttgcaatctaaggtaataggaaacaaggcattgggcattttgaagaaactgcaggttaagctatggtgccaagcagaagactaaacactgatttgagtgtcaaatctccagcacattctgggatagaggcaggttctcaaatgtttcctagtgttctttccttttcactaattaaattttcccttctctggcgaatccagtgcagtatacaaccccctgattgcctctcttggtcaaatagttgttagaagggaacctgtcaggcacctgtggcttcggcttagattggaaaggtgacagactagctctgattcacctcctcctgagacagcctggacagtggagggatcaactggaaggccgaaacctggtaacagctgcctctgattcctggtggaaatgaccaaccagattcaatccatatcactgggaaagatcaaggaaaaaaaatagcttcccctccaaaaatggtaaagaggaaataaggagacaagaaaccaaaaatacttagaatggcacaaaaagtgatacgcataaacttctttttgttattacatctaactgtaagtttcctaaagtccagttatcaagttgaattgtgtggatagaggagagaggccaactggattttctctcaagagttcacggcttcagtctgagaggtcctgggtttgcgctgggggagcccctttttgaatgaaggcgtgggagggctgggctccatgctgactccagttccattggtccctgcagagtgagtctggcctctttcaatggtgtttcctggtgcctgagatggagcactctgatacctggaaccagatgaataccacgagctgtttctgtaacgacccatactgtcatgccgcccttggttcatggggtcattggacttttggccttgtggcctatagccctgtcctcctcgtctgttccctggcaatacctcccgaagtggctggtagggctggccactggagtttgctatggctgcaggagtctctcccggtgcaaagtttttcttgttagcacttgtaaggctgggaggagaggcacaggtggaagaggaagcagcagaggcatcacttgggctactcaaggacacagatgtaactgagctacatcgggatctggtcgaatagctgttctttggatgagacacttgtccaaatgaatcaatgctcttctttagggtctctacatcacaggtgaaccgggctactcgtcccagatcctcatcatatttacgttcactaacaaagtgcttgatatcagctctgagctcaaccaattgctgctctgacatttgaacagccacatgagtcatcttctttagaagttcagccttcttttgtcggctgagcaaaatttccattgcttcagctttcactttgtccatttcagcaagcaacgccacttctcgatccattaaacagctctccaattcagcaaaggcttgtttcattttcttaatggaggcatccatctcttctttaactacaactcgataccgtgcaagagacactgtgcagcgctggaggtcttttacagatttttcaatattggaacttagctttttactggtggcgaggggaacatcttccatccccatatttgaaaactgagtttctgtggtaggtcttgagagagatttggcagcattcctgggttgttgagaattgtgaatagagtgcatagtcaaagacttggtctcaaaatcagagacaccattctgcagcatggatcctgttctatccagcgtatctagcatggcagactcgggatcctccaattctctggcatctattgaaagtgtctccaaaccttcactgagtgagtccacagactcagtgtcattgatggcaccattgacatggtagccattcataccacctttctctgaggaaggcgcagactgttcctcttgaatggaaactgatttactggaatctgggatgccgttacttggttctgcggcaggtttcggtttgtttttcttctttttgttctttttcttgcctgttactgtccattctttgagtacttcactggcactaccttccatgaatgcttgtactgttttgtccacacagttatcaaagtgctgcaaaaccaggataatttcattgttgctcttattaggaactattgcacgtaccgcatttatcttctctttcatgttctcaaaagctcctccctgggccagtacggtattggactgcaaatcaaaaatgaatcctgatgaatccttctggttctgtttcctggacattgtcgtttcttcgatctcaaaaaatatacaagaaaagtatccttttgccttgtctgggttttgagtgtaggtatctctgatttaaaagtgggcaacggaagtgtgcagttggaagcaaaaaatacgaaatcctgctgttcgaaattctgctcactagctgttaatctcctttccttttcttgtatcaacttcttgtcaggaagtatcattgcagacattcatgtctccttttccagggagattctctcataccactggacctgggggtgagtaagtgtcctctttgctcctcacagatgtttccaaatcagtctccctccttattccatatgaggtaaccagggtagtcacattcatagagacagaaagtagaatattggtagccagcagctagcccaggcccccgcaatcgcctcgtcgccccagctccgggctccgcgtcccggacgctcccgggtctgagaagaggaaaggagatcctccacctccccttctagagccaccgccgccgtcgcc

SEQ ID NO: 12884 - RNA, 4383 nt, Homo sapiens
  source 1..4383: mol_type = other RNA
gctgggattacaggcatgagccacaacgcccaacctttttttttttaaactttaattaaatgctactttctcatagacttccctagactggtttgcaatctaaggtaataggaaacaaggcattgggcattttgaagaaactgcaggttaagctatggtgccaagcagaagactaaacactgatttgagtgtcaaatctccagcacattctgggatagaggcaggttctcaaatgtttcctagtgttctttccttttcactaattaaattttcccttctctggcgaatccagtgcagtatacaaccccctgattgcctctcttggtcaaatagttgttagaagggaacctgtcaggcacctgtggcttcggcttagattggaaaggtgacagactagctctgattcacctcctcctgagacagcctggacagtggagggatcaactggaaggccgaaacctggtaacagctgcctctgattcctggtggaaatgaccaaccagattcaatccatatcactgggaaagatcaaggaaaaaaaatagcttcccctccaaaaatggtaaagaggaaataaggagacaagaaaccaaaaatacttagaatggcacaaaaagtgatacgcataaacttctttttgttattacatctaactgtaagtttcctaaagtccagttatcaagttgaattgtgtggatagaggagagaggccaactggattttctctcaagagttcacggcttcagtctgagaggtcctgggtttgcgctgggggagcccctttttgaatgaaggcgtgggagggctgggctccatgctgactccagttccattggtccctgcagagtgagtctggcctctttcaatggtgtttcctggtgcctgagatggagcactctgatacctggaaccagatgaataccacgagctgtttctgtaacgacccatactgtcatgccgcccttggttcatggggtcattggacttttggccttgtggcctatagccctgtcctcctcgtctgttccctggcaatacctcccgaagtggctggtagggctggccactggagtttgctatggctgcaggagtctctcccggtgcaaagtttttcttgttagcacttgtaaggctgggaggagaggcacaggtggaagaggaagcagcagaggcatcacttgggctactcaaggacacagatgtaactgagctacatcgggatctggtcgaatagctgttctttggatgagacacttgtccaaatgaatcaatgctcttctttagggtctctacatcacaggtgaaccgggctactcgtcccagatcctcatcatatttacgttcactaacaaagtgcttgatatcagctctgagctcaaccaattgctgctctgacatttgaacagccacatgagtcatcttctttagaagttcagccttcttttgtcggctgagcaaaatttccattgcttcagctttcactttgtccatttcagcaagcaacgccacttctcgatccattaaactaggaaaagatgacaaaggaataaaaagtttgatcagaaactcaaatacaaaattagcacattattaatagtaaagaaagaccagtgagtttgtttgctaaaagcatactaaaaaataatattgtatggatcacatacaaattctgatgtcttactctcaacaaagaatattttaagattttcccataaataaaataaatagacccaattcccttttatattgcaatattggtacattgcagcagtacaccaattgtagacgtctaagagttgagaaccagcagatggcagtagcaagctacaaaacacattttttagtaagctgtgctaaagcaaaagtccgtgtggaaattacttacttaaccatgtatgtactcacatacttttttttttttttttgagacggagtctcgctgtctcctaggctggagtgcagtggcgcgatcttggctcactgcaagctccgccttccgggttcacgccattctcctgcctcagcctcccgagtagcttggactacaggcgcccgccaccacgctcgtctattttttttgtatttttagtagagatggggtttcaccgtgtcagccagaatggtctcgatctcctgacctcgtgatccgcccgcctcggcctcccaaagtgctgggattacaggtgtgagccaccgcgcccggcctgtactcatactttttatatttatattttggtctataaaatttgatggccttgcatctaattaatttttaccaagcaatatccccactagggcatagtaaatttatccatgattaggacttgtatgtcttcaacagctgaccatggttgcaccaagtccacttacattttagtacttagaatgcaaagtagtcaaaagatagacatatagtgtgctagtttctgagaaacacataatagtaactaggaaggatggaattacagatttctggtaggctttttacagaaaaagaacattaaataggcaattagaattttttccactgcaaatataaatggtttataggcacataaagcttttccatgttgttataaaagagcccacagccttcaatgtataaggagacagtagtaccctagtattcaacctctggatgaaaataattttccttaccatatcggttttgctttgtggtggcaaaaagaaaaaaaaatctagaatgttaatacttgcacaaacatgcaatgttccaactttcttcaaatttggagttcattctgatttctccttttgaaggggaatataactacagggtaaataaaagttccactcttgtttctggttgtaatcacactcaaacacacacacacacacacacacacactctttctctctcgctctaattcaatttagctcaatacatagttatgttagcacaaagtagttaatgtggagactatagtgtgagacatacaaaaatgtctaaggcagggtcatttcctcaaggagcaaatcttttatagggaagtgccagagaacataggtttgataatcgttacgcatgatgttaataaacagacttgtaactaaacaaatttggttgacatattaatccaaaagcatcaaactggagagaagatacaattattgtggggtagcaatactttgctaagaaagcatttcccaaaccttggcaatattttgctccaagaactctagcagcattggaataccagctctccaattcagcaaaggcttgtttcattttcttaatggaggcatccatctcttctttaactacaactcgataccgtgcaagagacactgtgcagcgctggaggtcttttacagatttttcaatattggaacttagctttttactggtggcgaggggaacatcttccatccccatatttgaaaactgagtttctgtggtaggtcttgagagagatttggcagcattcctgggttgttgagaattgtgaatagagtgcatagtcaaagacttggtctcaaaatcagagacaccattctgcagcatggatcctgttctatccagcgtatctagcatggcagactcgggatcctccaattctctggcatctattgaaagtgtctccaaaccttcactgagtgagtccacagactcagtgtcattgatggcaccattgacatggtagccattcataccacctttctctgaggaaggcgcagactgttcctcttgaatggaaactgatttactggaatctgggatgccgttacttggttctgcggcaggtttcggtttgtttttcttctttttgttctttttcttgcctgttactgtccattctttgagtacttcactggcactaccttccatgaatgcttgtactgttttgtccacacagttatcaaagtgctgcaaaaccaggataatttcattgttgctcttattaggaactattgcacgtaccgcatttatcttctctttcatgttctcaaaagctcctccctgggccagtacggtattggactgcaaatcaaaaatgaatcctgatgaatccttctggttctgtttcctggacattgtcgtttcttcgatctcaaaaaatatacaagaaaagtatccttttgccttgtctgggttttgagtgtaggtatctctgatttaaaagtgggcaacggaagtgtgcagttggaagcaaaaaatacgaaatcctgctgttcgaaattctgctcactagctgttaatctcctttccttttcttgtatcaacttcttgtcaggaagtatcattgcagacattcatgtctccttttccagggagattctagcccaggcccccgcaatcgcctcgtcgccccagctccgggctccgcgtcccggacgctcccgggtctgagaagaggaaag

SEQ ID NO: 12885 - RNA, 2840 nt, Homo sapiens
  source 1..2840: mol_type = other RNA
gctgggattacaggcatgagccacaacgcccaacctttttttttttaaactttaattaaatgctactttctcatagacttccctagactggtttgcaatctaaggtaataggaaacaaggcattgggcattttgaagaaactgcaggttaagctatggtgccaagcagaagactaaacactgatttgagtgtcaaatctccagcacattctgggatagaggcaggttctcaaatgtttcctagtgttctttccttttcactaattaaattttcccttctctggcgaatccagtgcagtatacaaccccctgattgcctctcttggtcaaatagttgttagaagggaacctgtcaggcacctgtggcttcggcttagattggaaaggtgacagactagctctgattcacctcctcctgagacagcctggacagtggagggatcaactggaaggccgaaacctggtaacagctgcctctgattcctggtggaaatgaccaaccagattcaatccatatcactgggaaagatcaaggaaaaaaaatagcttcccctccaaaaatggtaaagaggaaataaggagacaagaaaccaaaaatacttagaatggcacaaaaagtgatacgcataaacttctttttgttattacatctaactgtaagtttcctaaagtccagttatcaagttgaattgtgtggatagaggagagaggccaactggattttctctcaagagttcacggcttcagtctgagaggtcctgggtttgcgctgggggagcccctttttgaatgaaggcgtgggagggctgggctccatgctgactccagttccattggtccctgcagagtgagtctggcctctttcaatggtgtttcctggtgcctgagatggagcactctgatacctggaaccagatgaataccacgagctgtttctgtaacgacccatactgtcatgccgcccttggttcatggggtcattggacttttggccttgtggcctatagccctgtcctcctcgtctgttccctggcaatacctcccgaagtggctggtagggctggccactggagtttgctatggctgcaggagtctctcccggtgcaaagtttttcttgttagcacttgtaaggctgggaggagaggcacaggtggaagaggaagcagcagaggcatcacttgggctactcaaggacacagatgtaactgagctacatcgggatctggtcgaatagctgttctttggatgagacacttgtccaaatgaatcaatgctcttctttagggtctctacatcacaggtgaaccgggctactcgtcccagatcctcatcatatttacgttcactaacaaagtgcttgatatcagctctgagctcaaccaattgctgctctgacatttgaacagccacatgagtcatcttctttagaagttcagccttcttttgtcggctgagcaaaatttccattgcttcagctttcactttgtccatttcagcaagcaacgccacttctcgatccattaaacttggcaatattttgctccaagaactctagcagcattggaataccagctctccaattcagcaaaggcttgtttcattttcttaatggaggcatccatctcttctttaactacaactcgataccgtgcaagagacactgtgcagcgctggaggtcttttacagatttttcaatattggaacttagctttttactggtggcgaggggaacatcttccatccccatatttgaaaactgagtttctgtggtaggtcttgagagagatttggcagcattcctgggttgttgagaattgtgaatagagtgcatagtcaaagacttggtctcaaaatcagagacaccattctgcagcatggatcctgttctatccagcgtatctagcatggcagactcgggatcctccaattctctggcatctattgaaagtgtctccaaaccttcactgagtgagtccacagactcagtgtcattgatggcaccattgacatggtagccattcataccacctttctctgaggaaggcgcagactgttcctcttgaatggaaactgatttactggaatctgggatgccgttacttggttctgcggcaggtttcggtttgtttttcttctttttgttctttttcttgcctgttactgtccattctttgagtacttcactggcactaccttccatgaatgcttgtactgttttgtccacacagttatcaaagtgctgcaaaaccaggataatttcattgttgctcttattaggaactattgcacgtaccgcatttatcttctctttcatgttctcaaaagctcctccctgggccagtacggtattggactgcaaatcaaaaatgaatcctgatgaatccttctggttctgtttcctggacattgtcgtttcttcgatctcaaaaaatatacaagaaaagtatccttttgccttgtctgggttttgagtgtaggtatctctgatttaaaagtgggcaacggaagtgtgcagttggaagcaaaaaatacgaaatcctgctgttcgaaattctgctcactagctgttaatctcctttccttttcttgtatcaacttcttgtcaggaagtatcattgcagacattcatgtctccttttccagggagattatatgaggtaaccagggtagtcacattcatagagacagaaagtagaatattggtagccagcagctagcccaggcccccgcaatcgcctcgtcgccccagctccgggctccgcgtcccggacgctcccgggtctgagaagaggaaaggagatcctccacctccccttctagagccaccgccgccgtcgcc

SEQ ID NO: 12886 - RNA, 6900 nt, Homo sapiens
  source 1..6900: mol_type = other RNA
gctgggattacaggcatgagccacaatgcccagccaagaatctaataatttttggatcttgaaaattgtatttcttattagaaaaagtaaagaatcacaggcttacatcctatgatcacagatctaagtgttctggttgaaagaggaagaagaggcaacatacaaactacacttctgtggacaccaagtgtagtgtggcaggaaaacataaagtttgcatgtataaaaccttaaaagttgaatgcctacaatgtacttgtctgtggcaggtatgagagatcgaaaccttacaatgtcaatgggatcagacaagggctctattttgatcctggaaagcatcaccagctgtatacattgtattctatgcattctattttaaacccctggagcagctcagtggctcgctggctgaatactgagacactgacattactgcaggctaggatttccccctataggacagccacttgtgatacttaccccatcaaagttttcctccatcttactgtgacagaacctacatgagattcattcgggaaattctcaacaagaggactctatcctataagtcgtccccaatccccagatctccaatggattattcttgtaaacagcacttttaccttccgatcgctctaccacagaggccaaaaagggttttcccctaacatccaaatacctattcagataccagccctgctccttctcttaaaatctgtcttctcacctgggcgtggtggctaatgcctgtaatcccagcactttgggatgctgaggtcggtgatcacttgacatcaggagttcgagaccagcctgggcaacatggcaaaaccccatctctactaaaaatacaaaaattagctgggcatggtggcacgtgcctgtaatcccagctacttgggaggctgaggcaagagaatcgcttgaacccaggagcgggaggttgcagtgacctgagatcacgccactgcactccagcctgggcgaaagagtgagattgtgtctcaaaaaaataaaaatgtgtcttccacttcttaaaccccaaagctgttttgttgttgttgtcatttaaaacagacacagactatgcttccctcctgatttattaagaccgacatatttaatttgcatttcttgagggaatagcacctggaaaccagggagaaagaagctgaagcatgcaggtcatgaattattcaatttggtgtcaataatttgtcagaaaaattaaaaaaaatcaatagataaccgtattgtagttcaactgattataatatagaagcaacggataatgaacaccctttcctcaaagtcatttattctcaacctttggaaatgattacgtttttacctccagtgaatcccttcatcacagagaataacagggtaccagcccaagccaacagtgccccataccagagaactcagggaaacaaagaccctaaaggttatgtacaatgagagaatcagactgtgaggctccagctctcttctgtatccctgctcactttacctcagtgcacaccatatcccttcttcctccattgtgaaatgtgcatacacgtgtttgtctgtgaatatataaatatctctatttacacatatatacatatataaaaatgtgcaatacaaagacataagcaaggagtttttcctaataactatttaatcagagactgattggagaaaaaacaagttcttcccctcaaattttccttctaacttgagaaccaattcctggaccaattcctgctcaaagaaaacatttaagaagcacctgtcggctgggagtgctagctcacacctgtaatcccagcactttgggaggccgaggcgggtggtcacttgaggtcaggagtttgaaaacagcctgaccaacatggtgaaccacttctcatagagacacattattaacttggtgaaacttaattgggatgaggagcactctgtatacatgtatcatttctgtttttcctcattgtgatggttaatcttatgtgtcaacttgactaggccacatgatgcccagatatttggtcatacagtattctgggtgtgtctgtgaaggtgtttttggaagagactaacatttcagtcagtagactgaatacagcacatggccctccctaatgtaagtggccctcatccaatcagttgaaggtctgaatagaacaagtaagggagaagtcctcctgcctgactgcttgaactaagacctcagtcttttcctgcctctgaactggaacagaaacatcagctcttctagggtatccaagctggccttcagactggaactacaccatcagctctcctggatctctagctggcccactgcagatcttgggatttctcaaactccattattgtgtgaaccaattccttataataaatctcaggctgggcatggtggctcccgtctgtaatcccagcactttgggaggccacgactggcagatcacctgaggtctagagttcaagaccagcctggccaacaaggtaaaaccttgtctctactaaacatataaaaaattagctgggcatggtggcaggtgcctgtaatcccagctgcttgggaggctaaggcagaagaatcgctggaacccaggaggtggaggttgcagtgagctgagattgcaccactgcactccagcctaggcgacagagcaagcctccatctcaaaaaataaataaataaataaataaataaataaataataataataataataataaatccctgaagaatcctaactcctcaacataaattaacctggacatctgaggtgcctgccattataagaagaaacacaacagatccattaagtgggacaggtctgggaaacagtaaaatgagtctcacatcctctatccaccagagcaaaaaaagtgaagaaaacttcatgtaactttgtctgatgctgtttgctatactgtgtataaaaaggcagacccctatccagtactttgtttccaccctttttaaaggtactcagatcctttctagttctctaggcattggttctctatctgtacgtaaaactacaactgcctgtcctggcatctccagacactgacaagcaaatatgtccaggctgtcatgatttttctgagacaactgatattgtgtacttgaaaactgcaatgtgtcccaagttcaacatagccttcctccatctaagtagtggccaaatattcataatacacctctaatttccttccatcctcctccccaattcaaaaccagtgtgtattctcaagctacatttcaggggcaacgcacagtaagtagatctcattccccaaataaacaatcactacagaggtgtaatatgggaggtatatgaaaaaacatattttattccctctgggcccaaatgaatcatactttctggtcacaacttttagaggcaggctattatttcagcaggccactctctcactttttctgttccctctctgactccttcatcctttaccaaagtacagagaaacgttatctctagcccccttccgtcacccacaaatcagcgtatgatagtcaacaaaaactgaggaaagacttctagccaagaaaaagacccattaaagagtggtgtttttgttctgatcattctaaactgatcattctgatcattgttgtgtgacaatacaaatggtgcccctctgtacctttttttggtacaccaacagttgttctatgtccccatcatttccttttgagaccttgaagtttcaacaacattcttgaccttcttaatttatccaatgttaaacacttgaatgctacaaagagcatgtgcatgggacactactaggctgaaaaaataaggcctacctcttccaggccaagctgttttggacatgatcacactgatcagtttgagtccaagtatagccagaaccaaggagaaaaggaaagtttcagagatgaaaaataggcttaaaaattaaaatgtgacaatgtaaaatcttaactcctgaagaccaatgaattaccaaaaacagtgaactggctgcagacacttactgtctctatttctgtgaggcaaattattttaagattactaggaaaaaagacagtaaacaatgagttgagcactttgagaggttgaggcaggcagatcacttgagcccaggagtttgagaccagcctgggcaacacggcaaaaccctatctctacaaaaatacaaaaattacccaggcatggtggcacacgcctgtagtcccagccacttggtaggctgaggtgggaggatcacttgagcctgggaggtcgaggctgtggtgagctgagatcgtgccactgcactccagcctaggcgacagaaacaaacaaaaaaagcagtgagttggggattttttttttttttttgagatggagtttcgctcttgttgcccagactggagtgcattggtatgatccggctcaccgcaacctccacctcctgggttcaagcgattctcccacctcagcctcatgagtagctgggattacaggcatgcaccaccacgcccagctaattttatatttttagtagagacaaggttttaccttgttggccaggctggtcttgatctcttgaccttgtgatccgcctgcctcggcctcccaaagtgctgggattacaggcgtgagccaccgcgcccagcggtaatcattttttaaaatctcagaagcaaaggtctcaaacatctgtctttctgtgcctgtatgctgcccaactcattcccaaaaaggaatgggaatcagattcctatcaacataaggctcccaatatatgttatgtaggtttcttgggaaactgcatcaactgaagtagtctttaaaaattaaaataagaggccaggcgcagtggctcacgcctgtaatcccagcactttgggaggctgaggcaggcggagcacaaggtcaggagattgagaccatcctggctaacacggtgaaaccccatctctactaaatatacaaaaaattagctgggcatggtaacaaatgcctgtggtcccagctactccggaggctgaggtaggagaatcgcttgaactcaggaggcagagtttgcaatgagccaagatcgtgccactgcacttcagcctaggcgacagagcgagactccatctcaaaaaaaaaaaacaaaaaaaattaaaataagaaaaccaaagcacacaatgataaaccacttttctcttcttgctgtaatttttctttgatttgctctctggggatcaagacaaaacaaaatcattagtcttagatacctgaatttgacctcgcctcatagctaatgtgatcaagagtagttttttttttttttaaatacaattaagacaaaaggactttatatcagcaggactttagggctgtggttccactgtttttatagtaaaatacactaatggtggggtagaggttggagaaggaggtggaaacatccgttacaaggcaacatgacagacagcaggaccctaactagactttaaggaattaattctattcagacggggggagccctacataattaagtttcacacttataaaattatcactctgaattcagggataagaggcatttggttgtagatacaattccatctgtagatactaactttaaatttaaagaagaaaaacattcattgcatttatattatgtgttgagtttcttacatattcctaaatccatctactaattttttgttttgatacaatttacagctatggtaagatgattaccacagccctgattcaggtgtggtctttagcttcagaaagtccatcggtcatgtagctgactgtcattgctaaatctgttgcttgcagaggcctcagtgctctggctttgccgagtagagtcctcaccatttaagctcttcctacatacaggacatgtgtcatgcagttctagccacggcacaatacaactgctgtgaaagaagtgattgcaaggtaactgccggacttcctcttcaactgtgtaatcttctttgcatactggacactctaaacccatatcaacttgttcctgagttactgtcactgttggaagagatgtgatcttttccttgtcagctgggggagggcctgtgttttccagttgtcctaaaagctgggttacaatggcatcaagccctgtctgaccccaggcatagtccccagggttggagtgcagcatcccgctccaggaaaaagggtgtggagatccaggaatggcagaatttgcaaagaatcctgcaaagatgtgttgtagtattccttcaatagctggagatctgtcaggacgagaacttcctcgagatctgtatctccgacccaatggcaaccgtggaggtcttgctccccagaagtcagtgtgagtctggtgacccctttcattggctctattatcttggtccagtggactgctacttagaaagggtctaaaatcttgaaaaaacatcgtgtgatccaaatggccccaaagctctgcaaaatgtgttgttgtggtattgtctatccgactgccgccaccacctaaaaaactggaatcatctgtcacttcttcaataaagcctgattcacatctgggacatatatattccggtagtttggggctgacctcgcccttgcaaaagtggcagaaaaaccggtgggcggctacagcggcgcccgagtccgccccggccgccgaagcctccgccatttttgccctccgccgcggccgtccgagagggcagccggcccgtccctcgccaggccgctacctcccgagctgcagtcgtcgccgccgccgccgcctcggtgcggcccaccgcttcagagcccgcgtcggtcacgtgagttggccaggcccagaaacgcggcggcgccaacagctaccctgcggcccgcctcccagcaccaaagaggcgcaggaaggagagac

SEQ ID NO: 12887 - RNA, 3555 nt, Homo sapiens
  source 1..3555: mol_type = other RNA
gctgggattacaggcatgagccacaatgcctaactactgatgcacgatttctaaattaagaatttataatataccataacttatattcttttatggttatcttttatggtttttttttttcctgcttccagtttaagaagttcttcctaaagggagtaggatcaggaagataatcacattttctaaatatgtttcaatcacattttaatctataattccacatatagtttctacatcaagtcgtcatcctgttgcattaattttaaagagcatgcttctagtgtataaggttgaaaagcattcttccccttatagattactaaagatttattattaatgggtatactgattttctttagtcttactttttatttatcctttttaagtcatcaacaaactttttctgagtatttgattacctttctttcaaaccgtacagtatctcctggatttgtttctctttttatttaggtactttctccaaaagtgattttagtttgtacggaaaatcttctgaagctttgatggtacatattcttattaatgccctcacattagaataactattttcagaacataaaattgtaggttcaaagtttttttcaggttcaatttcacattcttgagctaggcatggtactgatggttttcaccataacatacaccaatgtccttttgtctgtgggctcccatccagcctggtggctgaagtcatctacaggtaagattgaccaaacctctgaacaggactgaaaaaaatgttatcttcagaaaaccagccctcttgtacactgctgctgtgaatacaaattgattaacttttctggatggcaatctagcaatgcagatcaaacatttaaaaatacatatatatctcgacacaattttatctccaggcatccacatgaaagaactccacaatgttcagaagtgtacagataaggatactcgtcacagcattataatatgaaaaataaactgaaaaccacctcatctccaaacacaattaaattatgttaaaattctataaacagggattaggatgtgtaggtttacccaagggaaaatatatttaatgtttaggtttaaaaagcaaaaaaaaagcctactttttgtttcaaaaatatgcatatgtaagtagaaaatatctgaaagctgaaaggctactatccaaaaatattaacagcagctttctctaaacagaaactaaagcagtttctcttttctttttgcttttctatacttattacatgtctaccacaaacctctttgttataatttctccagttgagtcagttttacaatttggaatgcagagatcaagtggttctataatcagcatatacttcgcacgtaccattcattcaatccacacccctttaaacccctttgacacacgtcaaactcatttacatctatgtccctccaatgacaatatagtggtcaacacatataaaacatgaatacactatatcaagacactcaggaatacatctctgggataaaatctgactgccttctattatattttaatgaataaccaaaataaagggattctttcagttacagagagcagaataattaaaatagtaactttcaaactttgtagcagcagaagtatttcttcaaataaaatcttttttgaaacccaatatagaaaacagataaaaataaagccattctagaggtgggggccttggaaagtgagtactatccactcagacttctttcttgcctctcacaaggaaggaagctactgtgtagtttgaaaattactatttaatacattctgctaaccctaaatgccatgtcagagctagaagagaaaatgtacacacattcaatctaacatttatttatttcaggttttttttttttttggcaactataaattacattcactagtacacctggaattcttcatagtgtgttcaactaaagaataagcaaacacagcatagatcagtttaaaagaaatcatggtacttcttagagcaatttgcaaaaggggaaaaaagtcttaggctcactccttggaaataaatatcaagtaaccataaaaatattcagccatttttcagttattcggggagttcaggcatggtcccacgcagagcatcagagttcctctttgaaataacccagctttgccaatgacatctcttttctcaactgcataacctcccaaaacatctgatcaacatcctgctgtttcacgagtccctgctgaatgtatcgaatgtatgtaaaaaagttacatacagaagtgatcctgtatctgcaaaaaggagaaatataataatagttgcttgagtcccctaatttaattctgtgtttacaggacttactctggccagtgagagcacattttctcactttttgagaatgttaaacatggaaagatatcttcctggtagattttgtctaagaaaggacacgtcctgtccattgtgggctcatccttccacaatcggaattcattatacaaggataagtcagcctctttgcagtcttttacaattggctgtatcacactgaggtcctgatgactgccactcatagcactgcttgtgcttttatttcttgtatgcccctttttaaaaggtgtctttccacctggcaaaggctcctgcgtaggtgatgttggagaactggacaatacaagtgtcttcaatgcagctacttcagcttgaagtacatcaatttttccttgtgcttcttttagctgtttttctgctgttgcctgcttgatatttgcttctctcaccattttatgagcttcctcaaatagactagctgtgagttcttccaattcctgtccaagttgatctcgcacttttgaaagcctctcacattcttcatcttttaacttcagttccctctgagcttttgcgagttcttcttttaatcgttcatagcccttttctctaacttccaaaacagatgggcttcgtaaacgagacagactatcagtactcaacccaaaaatatcatcactgccatcgcaagcctctgttatagtagcaccctgtaaaaactctctctctgcattatagttgtcctttcttgtagttaatttagttaatccagctgtgactccagaggtagagcaaggggctgggtctgtaacatgaaagctgatactagatatttccgcacaatttaaacgtctgggggatgaatacacgggttgtgtaggaagttcagaaacatctaatgcatttgcctggataggtacagaggataaagctgaagggtgtggccggtagatgacacttggtgaggtagtctgctcttgagttcctgattcatacacaccaagaaggtccggagaagtaggtgaagcaaggtttacttcatggaagccttccaagggatcattagccatagcaaaagcctcatcataagataacctgagactccgcggccatatacaccttacgacgtgtgtgtgtgtggcgggagatgggaggggaggaatcctgtagaacccagatcccatcattccagcaactgccagagcgttcgagaatgtcatgtctgtacctgtcttct

SEQ ID NO: 12888 - RNA, 3773 nt, Homo sapiens
  source 1..3773: mol_type = other RNA
gctgggattacaggcatgagccacaatgcctaactactgatgcacgatttctaaattaagaatttataatataccataacttatattcttttatggttatcttttatggtttttttttttcctgcttccagtttaagaagttcttcctaaagggagtaggatcaggaagataatcacattttctaaatatgtttcaatcacattttaatctataattccacatatagtttctacatcaagtcgtcatcctgttgcattaattttaaagagcatgcttctagtgtataaggttgaaaagcattcttccccttatagattactaaagatttattattaatgggtatactgattttctttagtcttactttttatttatcctttttaagtcatcaacaaactttttctgagtatttgattacctttctttcaaaccgtacagtatctcctggatttgtttctctttttatttaggtactttctccaaaagtgattttagtttgtacggaaaatcttctgaagctttgatggtacatattcttattaatgccctcacattagaataactattttcagaacataaaattgtaggttcaaagtttttttcaggttcaatttcacattcttgagctaggcatggtactgatggttttcaccataacatacaccaatgtccttttgtctgtgggctcccatccagcctggtggctgaagtcatctacaggtaagattgaccaaacctctgaacaggactgaaaaaaatgttatcttcagaaaaccagccctcttgtacactgctgctgtgaatacaaattgattaacttttctggatggcaatctagcaatgcagatcaaacatttaaaaatacatatatatctcgacacaattttatctccaggcatccacatgaaagaactccacaatgttcagaagtgtacagataaggatactcgtcacagcattataatatgaaaaataaactgaaaaccacctcatctccaaacacaattaaattatgttaaaattctataaacagggattaggatgtgtaggtttacccaagggaaaatatatttaatgtttaggtttaaaaagcaaaaaaaaagcctactttttgtttcaaaaatatgcatatgtaagtagaaaatatctgaaagctgaaaggctactatccaaaaatattaacagcagctttctctaaacagaaactaaagcagtttctcttttctttttgcttttctatacttattacatgtctaccacaaacctctttgttataatttctccagttgagtcagttttacaatttggaatgcagagatcaagtggttctataatcagcatatacttcgcacgtaccattcattcaatccacacccctttaaacccctttgacacacgtcaaactcatttacatctatgtccctccaatgacaatatagtggtcaacacatataaaacatgaatacactatatcaagacactcaggaatacatctctgggataaaatctgactgccttctattatattttaatgaataaccaaaataaagggattctttcagttacagagagcagaataattaaaatagtaactttcaaactttgtagcagcagaagtatttcttcaaataaaatcttttttgaaacccaatatagaaaacagataaaaataaagccattctagaggtgggggccttggaaagtgagtactatccactcagacttctttcttgcctctcacaaggaaggaagctactgtgtagtttgaaaattactatttaatacattctgctaaccctaaatgccatgtcagagctagaagagaaaatgtacacacattcaatctaacatttatttatttcaggttttttttttttttggcaactataaattacattcactagtacacctggaattcttcatagtgtgttcaactaaagaataagcaaacacagcatagatcagtttaaaagaaatcatggtacttcttagagcaatttgcaaaaggggaaaaaagtcttaggctcactccttggaaataaatatcaagtaaccataaaaatattcagccatttttcagttattcggggagttcaggcatggtcccacgcagagcatcagagttcctctttgaaataacccagctttgccaatgacatctcttttctcaactgcataacctcccaaaacatctgatcaacatcctgctgtttcacgagtccctgctgaatgtatcgaatgtatgtaaaaaagttacatacagaagtgatcctgtatctgcaaaaaggagaaatataataatagttgcttgagtcccctaatttaattctgtgtttacaggacttactctggccagtgagagcacattttctctttgcagtcttttacaattggctgtatcacactgaggtcctgatgactgccactcatagcactgcttgtgcttttatttcttgtatgcccctttttaaaaggtgtctttccacctggcaaaggctcctgcgtaggtgatgttggagaactggacaatacaagtgtcttcaatgcagctacttcagcttgaagtacatcaatttttccttgtgcttcttttagctgtttttctgctgttgcctgcttgatatttgcttctctcaccattttatgagcttcctcaaatagactagctgtgagttcttccaattcctgtccaagttgatctcgcacttttgaaagcctctcacattcttcatcttttaacttcagttccctctgagcttttgcgagttcttcttttaatcgttcatagcccttttctctaacttccaaaacagatgggcttcgtaaacgagacagactatcagtactcaacccaaaaatatcatcactgccatcgcaagcctctgttatagtagcaccctgtaaaaactctctctctgcattatagttgtcctttcttgtagttaatttagttaatccagctgtgactccagaggtagagcaaggggctgggtctgtaacatgaaagctgatactagatatttccgcacaatttaaacgtctgggggatgaatacacgggttgtgtaggaagttcagaaacatctaatgcatttgcctggataggtacagaggataaagctgaagggtgtggccggtagatgacacttggtgaggtagtctgctcttgagttcctgattcatacacaccaagaaggtccggagaagtaggtgaagcaaggtttacttcatggaagccttccaagggatcattagccatagcaaaagcctcatcataagataaccctttcatcttttttaatcccataacaaccggcaactcttcacatgctgcgacttccacccagcatcatcacttctggagccagtaagctcgcgcttcctgggcggtcggggcgagttgtcaacgctgggagggcagagccatgcaatcccacccgtgcagttcgtctcaactcccccgaacacaagtctggcggcacggagctgcctacttgggcgcgactccgggcgcctgcccggaatttcccaccaggtttcaccgaaacctcccgagggtgacctctacgcctcagcacggtgcctcgcgcgtagtttcctaagactgggacacgaaaccaccccaggtccacagccctgccgcgcggcgtccggtgttgtgagctgcttccgacttgttcgggaactctctcttcatcctcttcgcgaccgcggccctccgctcccggccgcgcccgcccgccgccaggtaacccgctggactcgggctccct

SEQ ID NO: 12889 - RNA, 3456 nt, Homo sapiens
  source 1..3456: mol_type = other RNA
gctgggattacaggcatgagccacaatgcctaactactgatgcacgatttctaaattaagaatttataatataccataacttatattcttttatggttatcttttatggtttttttttttcctgcttccagtttaagaagttcttcctaaagggagtaggatcaggaagataatcacattttctaaatatgtttcaatcacattttaatctataattccacatatagtttctacatcaagtcgtcatcctgttgcattaattttaaagagcatgcttctagtgtataaggttgaaaagcattcttccccttatagattactaaagatttattattaatgggtatactgattttctttagtcttactttttatttatcctttttaagtcatcaacaaactttttctgagtatttgattacctttctttcaaaccgtacagtatctcctggatttgtttctctttttatttaggtactttctccaaaagtgattttagtttgtacggaaaatcttctgaagctttgatggtacatattcttattaatgccctcacattagaataactattttcagaacataaaattgtaggttcaaagtttttttcaggttcaatttcacattcttgagctaggcatggtactgatggttttcaccataacatacaccaatgtccttttgtctgtgggctcccatccagcctggtggctgaagtcatctacaggtaagattgaccaaacctctgaacaggactgaaaaaaatgttatcttcagaaaaccagccctcttgtacactgctgctgtgaatacaaattgattaacttttctggatggcaatctagcaatgcagatcaaacatttaaaaatacatatatatctcgacacaattttatctccaggcatccacatgaaagaactccacaatgttcagaagtgtacagataaggatactcgtcacagcattataatatgaaaaataaactgaaaaccacctcatctccaaacacaattaaattatgttaaaattctataaacagggattaggatgtgtaggtttacccaagggaaaatatatttaatgtttaggtttaaaaagcaaaaaaaaagcctactttttgtttcaaaaatatgcatatgtaagtagaaaatatctgaaagctgaaaggctactatccaaaaatattaacagcagctttctctaaacagaaactaaagcagtttctcttttctttttgcttttctatacttattacatgtctaccacaaacctctttgttataatttctccagttgagtcagttttacaatttggaatgcagagatcaagtggttctataatcagcatatacttcgcacgtaccattcattcaatccacacccctttaaacccctttgacacacgtcaaactcatttacatctatgtccctccaatgacaatatagtggtcaacacatataaaacatgaatacactatatcaagacactcaggaatacatctctgggataaaatctgactgccttctattatattttaatgaataaccaaaataaagggattctttcagttacagagagcagaataattaaaatagtaactttcaaactttgtagcagcagaagtatttcttcaaataaaatcttttttgaaacccaatatagaaaacagataaaaataaagccattctagaggtgggggccttggaaagtgagtactatccactcagacttctttcttgcctctcacaaggaaggaagctactgtgtagtttgaaaattactatttaatacattctgctaaccctaaatgccatgtcagagctagaagagaaaatgtacacacattcaatctaacatttatttatttcaggttttttttttttttggcaactataaattacattcactagtacacctggaattcttcatagtgtgttcaactaaagaataagcaaacacagcatagatcagtttaaaagaaatcatggtacttcttagagcaatttgcaaaaggggaaaaaagtcttaggctcactccttggaaataaatatcaagtaaccataaaaatattcagccatttttcagttattcggggagttcaggcatggtcccacgcagagcatcagagttcctctttgaaataacccagctttgccaatgacatctcttttctcaactgcataacctcccaaaacatctgatcaacatcctgctgtttcacgagtccctgctgaatgtatcgaatgtatgtaaaaaagttacatacagaagtgatcctgtatctgcaaaaaggagaaatataataatagttgcttgagtcccctaatttaattctgtgtttacaggacttactctggccagtgagagcacattttctctttgcagtcttttacaattggctgtatcacactgaggtcctgatgactgccactcatagcactgcttgtgcttttatttcttgtatgcccctttttaaaaggtgtctttccacctggcaaaggctcctgcgtaggtgatgttggagaactggacaatacaagtgtcttcaatgcagctacttcagcttgaagtacatcaatttttccttgtgcttcttttagctgtttttctgctgttgcctgcttgatatttgcttctctcaccattttatgagcttcctcaaatagactagctgtgagttcttccaattcctgtccaagttgatctcgcacttttgaaagcctctcacattcttcatcttttaacttcagttccctctgagcttttgcgagttcttcttttaatcgttcatagcccttttctctaacttccaaaacagatgggcttcgtaaacgagacagactatcagtactcaacccaaaaatatcatcactgccatcgcaagcctctgttatagtagcaccctgtaaaaactctctctctgcattatagttgtcctttcttgtagttaatttagttaatccagctgtgactccagaggtagagcaaggggctgggtctgtaacatgaaagctgatactagatatttccgcacaatttaaacgtctgggggatgaatacacgggttgtgtaggaagttcagaaacatctaatgcatttgcctggataggtacagaggataaagctgaagggtgtggccggtagatgacacttggtgaggtagtctgctcttgagttcctgattcatacacaccaagaaggtccggagaagtaggtgaagcaaggtttacttcatggaagccttccaagggatcattagccatagcaaaagcctcatcataagataacctgaagaacccaccgcggccgctgccggcgctcaggggcgctcacagagccgcagagagcgcgtcccgaagcagcgagaaacggaggaggacggcgagccctttccgctacactccacggcggcgggctcactacgccggcagccgccgagggaacgcgggactgcgcctgc

SEQ ID NO: 12890 - RNA, 3426 nt, Homo sapiens
  source 1..3426: mol_type = other RNA
gctgggattacaggcatgagccacaatgcctaactactgatgcacgatttctaaattaagaatttataatataccataacttatattcttttatggttatcttttatggtttttttttttcctgcttccagtttaagaagttcttcctaaagggagtaggatcaggaagataatcacattttctaaatatgtttcaatcacattttaatctataattccacatatagtttctacatcaagtcgtcatcctgttgcattaattttaaagagcatgcttctagtgtataaggttgaaaagcattcttccccttatagattactaaagatttattattaatgggtatactgattttctttagtcttactttttatttatcctttttaagtcatcaacaaactttttctgagtatttgattacctttctttcaaaccgtacagtatctcctggatttgtttctctttttatttaggtactttctccaaaagtgattttagtttgtacggaaaatcttctgaagctttgatggtacatattcttattaatgccctcacattagaataactattttcagaacataaaattgtaggttcaaagtttttttcaggttcaatttcacattcttgagctaggcatggtactgatggttttcaccataacatacaccaatgtccttttgtctgtgggctcccatccagcctggtggctgaagtcatctacaggtaagattgaccaaacctctgaacaggactgaaaaaaatgttatcttcagaaaaccagccctcttgtacactgctgctgtgaatacaaattgattaacttttctggatggcaatctagcaatgcagatcaaacatttaaaaatacatatatatctcgacacaattttatctccaggcatccacatgaaagaactccacaatgttcagaagtgtacagataaggatactcgtcacagcattataatatgaaaaataaactgaaaaccacctcatctccaaacacaattaaattatgttaaaattctataaacagggattaggatgtgtaggtttacccaagggaaaatatatttaatgtttaggtttaaaaagcaaaaaaaaagcctactttttgtttcaaaaatatgcatatgtaagtagaaaatatctgaaagctgaaaggctactatccaaaaatattaacagcagctttctctaaacagaaactaaagcagtttctcttttctttttgcttttctatacttattacatgtctaccacaaacctctttgttataatttctccagttgagtcagttttacaatttggaatgcagagatcaagtggttctataatcagcatatacttcgcacgtaccattcattcaatccacacccctttaaacccctttgacacacgtcaaactcatttacatctatgtccctccaatgacaatatagtggtcaacacatataaaacatgaatacactatatcaagacactcaggaatacatctctgggataaaatctgactgccttctattatattttaatgaataaccaaaataaagggattctttcagttacagagagcagaataattaaaatagtaactttcaaactttgtagcagcagaagtatttcttcaaataaaatcttttttgaaacccaatatagaaaacagataaaaataaagccattctagaggtgggggccttggaaagtgagtactatccactcagacttctttcttgcctctcacaaggaaggaagctactgtgtagtttgaaaattactatttaatacattctgctaaccctaaatgccatgtcagagctagaagagaaaatgtacacacattcaatctaacatttatttatttcaggttttttttttttttggcaactataaattacattcactagtacacctggaattcttcatagtgtgttcaactaaagaataagcaaacacagcatagatcagtttaaaagaaatcatggtacttcttagagcaatttgcaaaaggggaaaaaagtcttaggctcactccttggaaataaatatcaagtaaccataaaaatattcagccatttttcagttattcggggagttcaggcatggtcccacgcagagcatcagagttcctctttgaaataacccagctttgccaatgacatctcttttctcaactgcataacctcccaaaacatctgatcaacatcctgctgtttcacgagtccctgctgaatgtatcgaatgtatgtaaaaaagttacatacagaagtgatcctgtatctgcaaaaaggagaaatataataatagttgcttgagtcccctaatttaattctgtgtttacaggacttactctggccagtgagagcacattttctctttgcagtcttttacaattggctgtatcacactgaggtcctgatgactgccactcatagcactgcttgtgcttttatttcttgtatgcccctttttaaaaggtgtctttccacctggcaaaggctcctgcgtaggtgatgttggagaactggacaatacaagtgtcttcaatgcagctacttcagcttgaagtacatcaatttttccttgtgcttcttttagctgtttttctgctgttgcctgcttgatatttgcttctctcaccattttatgagcttcctcaaatagactagctgtgagttcttccaattcctgtccaagttgatctcgcacttttgaaagcctctcacattcttcatcttttaacttcagttccctctgagcttttgcgagttcttcttttaatcgttcatagcccttttctctaacttccaaaacagatgggcttcgtaaacgagacagactatcagtactcaacccaaaaatatcatcactgccatcgcaagcctctgttatagtagcaccctgtaaaaactctctctctgcattatagttgtcctttcttgtagttaatttagttaatccagctgtgactccagaggtagagcaaggggctgggtctgtaacatgaaagctgatactagatatttccgcacaatttaaacgtctgggggatgaatacacgggttgtgtaggaagttcagaaacatctaatgcatttgcctggataggtacagaggataaagctgaagggtgtggccggtagatgacacttggtgaggtagtctgctcttgagttcctgattcatacacaccaagaaggtccggagaagtaggtgaagcaaggtttacttcatggaagccttccaagggatcattagccatagcaaaagcctcatcataagataacctgagactccgcggccatatacaccttacgacgtgtgtgtgtgtggcgggagatgggaggggaggaatcctgtagaacccagatcccatcattccagcaactgccagagcgttcgagaatgtcatgtctgtacctgtcttct

SEQ ID NO: 12891 - RNA, 3835 nt, Homo sapiens
  source 1..3835: mol_type = other RNA
gctgggattacaggcatgagccacaatgcctaactactgatgcacgatttctaaattaagaatttataatataccataacttatattcttttatggttatcttttatggtttttttttttcctgcttccagtttaagaagttcttcctaaagggagtaggatcaggaagataatcacattttctaaatatgtttcaatcacattttaatctataattccacatatagtttctacatcaagtcgtcatcctgttgcattaattttaaagagcatgcttctagtgtataaggttgaaaagcattcttccccttatagattactaaagatttattattaatgggtatactgattttctttagtcttactttttatttatcctttttaagtcatcaacaaactttttctgagtatttgattacctttctttcaaaccgtacagtatctcctggatttgtttctctttttatttaggtactttctccaaaagtgattttagtttgtacggaaaatcttctgaagctttgatggtacatattcttattaatgccctcacattagaataactattttcagaacataaaattgtaggttcaaagtttttttcaggttcaatttcacattcttgagctaggcatggtactgatggttttcaccataacatacaccaatgtccttttgtctgtgggctcccatccagcctggtggctgaagtcatctacaggtaagattgaccaaacctctgaacaggactgaaaaaaatgttatcttcagaaaaccagccctcttgtacactgctgctgtgaatacaaattgattaacttttctggatggcaatctagcaatgcagatcaaacatttaaaaatacatatatatctcgacacaattttatctccaggcatccacatgaaagaactccacaatgttcagaagtgtacagataaggatactcgtcacagcattataatatgaaaaataaactgaaaaccacctcatctccaaacacaattaaattatgttaaaattctataaacagggattaggatgtgtaggtttacccaagggaaaatatatttaatgtttaggtttaaaaagcaaaaaaaaagcctactttttgtttcaaaaatatgcatatgtaagtagaaaatatctgaaagctgaaaggctactatccaaaaatattaacagcagctttctctaaacagaaactaaagcagtttctcttttctttttgcttttctatacttattacatgtctaccacaaacctctttgttataatttctccagttgagtcagttttacaatttggaatgcagagatcaagtggttctataatcagcatatacttcgcacgtaccattcattcaatccacacccctttaaacccctttgacacacgtcaaactcatttacatctatgtccctccaatgacaatatagtggtcaacacatataaaacatgaatacactatatcaagacactcaggaatacatctctgggataaaatctgactgccttctattatattttaatgaataaccaaaataaagggattctttcagttacagagagcagaataattaaaatagtaactttcaaactttgtagcagcagaagtatttcttcaaataaaatcttttttgaaacccaatatagaaaacagataaaaataaagccattctagaggtgggggccttggaaagtgagtactatccactcagacttctttcttgcctctcacaaggaaggaagctactgtgtagtttgaaaattactatttaatacattctgctaaccctaaatgccatgtcagagctagaagagaaaatgtacacacattcaatctaacatttatttatttcaggttttttttttttttggcaactataaattacattcactagtacacctggaattcttcatagtgtgttcaactaaagaataagcaaacacagcatagatcagtttaaaagaaatcatggtacttcttagagcaatttgcaaaaggggaaaaaagtcttaggctcactccttggaaataaatatcaagtaaccataaaaatattcagccatttttcagttattcggggagttcaggcatggtcccacgcagagcatcagagttcctctttgaaataacccagctttgccaatgacatctcttttctcaactgcataacctcccaaaacatctgatcaacatcctgctgtttcacgagtccctgctgaatgtatcgaatgtatgtaaaaaagttacatacagaagtgatcctgtatctgcaaaaaggagaaatataataatagttgcttgagtcccctaatttaattctgtgtttacaggacttactctggccagtgagagcacatttttttggtcctccgcattcaactgcagaagctttcacaaaccggataggttgtaatcccactggttcaatgcttagagtattgttttccacagcctccagaacagctgaagccaactcactttttgagaatgttaaacatggaaagatatcttcctggtagattttgtctaagaaaggacacgtcctgtccattgtgggctcatccttccacaatcggaattcattatacaaggataagtcagccagcatcatttttattgataattcgtcaaaatgcaattcaattaaaacaggttaacattggttattccatttaataaactcctggcttccatacaaaaatttaacaagcacacacatttcttcaagattaatgatggacttgaatttaacaatgtaaaagatggcttctctttgcagtcttttacaattggctgtatcacactgaggtcctgatgactgccactcatagcactgcttgtgcttttatttcttgtatgcccctttttaaaaggtgtctttccacctggcaaaggctcctgcgtaggtgatgttggagaactggacaatacaagtgtcttcaatgcagctacttcagcttgaagtacatcaatttttccttgtgcttcttttagctgtttttctgctgttgcctgcttgatatttgcttctctcaccattttatgagcttcctcaaatagactagctgtgagttcttccaattcctgtccaagttgatctcgcacttttgaaagcctctcacattcttcatcttttaacttcagttccctctgagcttttgcgagttcttcttttaatcgttcatagcccttttctctaacttccaaaacagatgggcttcgtaaacgagacagactatcagtactcaacccaaaaatatcatcactgccatcgcaagcctctgttatagtagcaccctgtaaaaactctctctctgcattatagttgtcctttcttgtagttaatttagttaatccagctgtgactccagaggtagagcaaggggctgggtctgtaacatgaaagctgatactagatatttccgcacaatttaaacgtctgggggatgaatacacgggttgtgtaggaagttcagaaacatctaatgcatttgcctggataggtacagaggataaagctgaagggtgtggccggtagatgacacttggtgaggtagtctgctcttgagttcctgattcatacacaccaagaaggtccggagaagtaggtgaagcaaggtttacttcatggaagccttccaagggatcattagccatagcaaaagcctcatcataagataacctgagactccgcggccatatacaccttacgacgtgtgtgtgtgtggcgggagatgggaggggaggaatcctgtagaacccagatcccatcattccagcaactgccagagcgttcgagaatgtcatgtctgtacctgtcttct

SEQ ID NO: 12892 - RNA, 6161 nt, Homo sapiens
  source 1..6161: mol_type = other RNA
gctgggattacaggcatgagccacaatgcctaactactgatgcacgatttctaaattaagaatttataatataccataacttatattcttttatggttatcttttatggtttttttttttcctgcttccagtttaagaagttcttcctaaagggagtaggatcaggaagataatcacattttctaaatatgtttcaatcacattttaatctataattccacatatagtttctacatcaagtcgtcatcctgttgcattaattttaaagagcatgcttctagtgtataaggttgaaaagcattcttccccttatagattactaaagatttattattaatgggtatactgattttctttagtcttactttttatttatcctttttaagtcatcaacaaactttttctgagtatttgattacctttctttcaaaccgtacagtatctcctggatttgtttctctttttatttaggtactttctccaaaagtgattttagtttgtacggaaaatcttctgaagctttgatggtacatattcttattaatgccctcacattagaataactattttcagaacataaaattgtaggttcaaagtttttttcaggttcaatttcacattcttgagctaggcatggtactgatggttttcaccataacatacaccaatgtccttttgtctgtgggctcccatccagcctggtggctgaagtcatctacaggtaagattgaccaaacctctgaacaggactgaaaaaaatgttatcttcagaaaaccagccctcttgtacactgctgctgtgaatacaaattgattaacttttctggatggcaatctagcaatgcagatcaaacatttaaaaatacatatatatctcgacacaattttatctccaggcatccacatgaaagaactccacaatgttcagaagtgtacagataaggatactcgtcacagcattataatatgaaaaataaactgaaaaccacctcatctccaaacacaattaaattatgttaaaattctataaacagggattaggatgtgtaggtttacccaagggaaaatatatttaatgtttaggtttaaaaagcaaaaaaaaagcctactttttgtttcaaaaatatgcatatgtaagtagaaaatatctgaaagctgaaaggctactatccaaaaatattaacagcagctttctctaaacagaaactaaagcagtttctcttttctttttgcttttctatacttattacatgtctaccacaaacctctttgttataatttctccagttgagtcagttttacaatttggaatgcagagatcaagtggttctataatcagcatatacttcgcacgtaccattcattcaatccacacccctttaaacccctttgacacacgtcaaactcatttacatctatgtccctccaatgacaatatagtggtcaacacatataaaacatgaatacactatatcaagacactcaggaatacatctctgggataaaatctgactgccttctattatattttaatgaataaccaaaataaagggattctttcagttacagagagcagaataattaaaatagtaactttcaaactttgtagcagcagaagtatttcttcaaataaaatcttttttgaaacccaatatagaaaacagataaaaataaagccattctagaggtgggggccttggaaagtgagtactatccactcagacttctttcttgcctctcacaaggaaggaagctactgtgtagtttgaaaattactatttaatacattctgctaaccctaaatgccatgtcagagctagaagagaaaatgtacacacattcaatctaacatttatttatttcaggttttttttttttttggcaactataaattacattcactagtacacctggaattcttcatagtgtgttcaactaaagaataagcaaacacagcatagatcagtttaaaagaaatcatggtacttcttagagcaatttgcaaaaggggaaaaaagtcttaggctcactccttggaaataaatatcaagtaaccataaaaatattcagccatttttcagttattcggggagttcaggcatggtcccacgcagagcatcagagttcctctttgaaataacccagctttgccaatgacatctcttttctcaactgcataacctcccaaaacatctgatcaacatcctgctgtttcacgagtccctgctgaatgtatcgaatgtatgtaaaaaagttacatacagaagtgatcctgtatctgcaaaaaggagaaatataataatagttgcttgagtcccctaatttaattctgtgtttacaggacttactctggccagtgagagcacatttttttggtcctccgcattcaactgcagaagctttcacaaaccggataggttgtaatcccactggttcaatgcttagagtattgttttccacagcctccagaacagctgaagccaactcactttttgagaatgttaaacatggaaagatatcttcctggtagattttgtctaagaaaggacacgtcctgtccattgtgggctcatccttccacaatcggaattcattatacaaggataagtcagcctctttgcagtcttttacaattggctgtatcacactgaggtcctgatgactgccactcatagcactgcttgtgcttttatttcttgtatgcccctttttaaaaggtgtctttccacctggcaaaggctcctgcgtaggtgatgttggagaactggacaatacaagtgtcttcaatgcagctacttcagcttgaagtacatcaatttttccttgtgcttcttttagctgtttttctgctgttgcctgcttgatatttgcttctctcaccattttatgagcttccattgtatcacaagtgccaacagtattcagtatagtaacatgttgtacaggtttgtagcccaggagcaataagcaatatcatatagccaaggtgtgtaataggctgtaccatctaggttttaccacatcttggtttgtgtaagtatattctaccgatttctgcacgatgaaatcaaaactgtgcatattgagtttattcagaataatctttaattcctaaaaagatatgcaaacacacacatataaagtgcaaaaaaagaatcttttcataagacaatggtaaacagatcatgaaggcacaattaagaccaaataaaaactttgagcgctttttccacgattcataaataattggttcgaatacaactttcttcattaccaaaatcatctttaatcaatgtactttgttttccagaaagtagccacagtgtcaatgctaacagccaccactgggttagaaaaggttagagactccaaactatattttttagatatgctttttcacttattgcctattgcctaagctgcatttctggcccttcacatcctgctacttacagggagaagtttctttctgttttttctacttctatttcatgtaacagaacatacatacatgtgcagatgggtgaaactaagcagggctagctaaattaaatgcaagtagtcaggaaatcaaaattaacataaatagcttaatatatttgctttcttacctaatatccatatcactacaaaattttcttccagtcagacaatactggaagaaaaatctaatgcttctgtataaccttctattcagaaatgtaacaagtcacatagcttctattctagctctttaactttccactcttcctatccttaaatttattctcctctcatctctgatgactagctagctaaataaataaacagattaattttaaaatgttcatgaaagaaaatgaccccaaaaagacagaaaagaaggcaaaggggtatggagcagagaaggcatggaaagccctacatgtctaaagacattcagggcaatgttacttgtaatgataaaagttgtggaacaggcacctagtagattatgactatcgttacaattagtgatggtgcagcaacattaaaaatgttatttagaaaaacacaaaatattaaattacaactaagtaagaatacatacatacctgagactgtgaaatagattatgaataaataataacaaaaggtgatggaatttccacccccccaagtttattataataaaagttttaagaacaaatctttaggaaaaaaacatatatatatcgttaaatgataatggcattagccattccagtaacacatcaatgtttttgttaaggaacttctaaagactcaaggtcttaacccaaaggagacactttacagcaacagttcttactcatggaagtactaccctcacctcacccccaggggtatctgtatgctgtcaaaatgaccgggggtattaccagcacttttctgagcaaagcctattataatggtttattgtgtacgtcaacttgactgaatcaaagggtgctcgaatatgtagtcaaacattatcctgaatgtttctggataagaataacatttacattggtagactgagtaaagtagactgccctctagaatgtgggtgaccctcatccaatcagttgatggcctgaatagaacaaaaaagggtgccgctccctcaaggaagagattttttttctgccttcagactcaaactgaaacatttgctcttcccagttctcagaccttcaaagttggactggaagtgcaccatcagccctcctgggcctccagtttgctgactcccactgcagctccctgggacttgccagcctccataacagcaagagccaactccctataataatgagtgcctctgtccctctctctccctctctgtatctctctatacatgtatatgtatataggctctgtttttctggagaaccctgactaaaacaccaaggacactaaacgtcctacagtgttagtggcacccctatggagaaacactgctccagttaggtagaaatttttcctggtggcgggctggatataaaaagtatgccttcttacaagtagatgtgccttctaacatttctcaaatcatcccatgtaagatgactatctcaaagagtttgccctcttagttgtacagtcatatgtagttaatctaaagtagcccgtaaatacttggtaaaataaaaatcaatactaaaatttgcctcctttctttgcacacatacatttttaaataatctgatactggtggcccatagatgttttttatttcttttcacatcatcttaagttgtaaactctacattgcttaaagatttctcttttgcttagaggacttataaatatacatgaagctaagcaaatatttttcaagattccctcaaaatacaattttgtcaatatataaaagtcaagatgttgctgttggccaagatgtaaatagaccaacctcaaatagactagctgtgagttcttccaattcctgtccaagttgatctcgcacttttgaaagcctctcacattcttcatcttttaacttcagttccctctgagcttttgcgagttcttcttttaatcgttcatagcccttttctctaacttccaaaacagatgggcttcgtaaacgagacagactatcagtactcaacccaaaaatatcatcactgccatcgcaagcctctgttatagtagcaccctgtaaaaactctctctctgcattatagttgtcctttcttgtagttaatttagttaatccagctgtgactccagaggtagagcaaggggctgggtctgtaacatgaaagctgatactagatatttccgcacaatttaaacgtctgggggatgaatacacgggttgtgtaggaagttcagaaacatctaatgcatttgcctggataggtacagaggataaagctgaagggtgtggccggtagatgacacttggtgaggtagtctgctcttgagttcctgattcatacacaccaagaaggtccggagaagtaggtgaagcaaggtttacttcatggaagccttccaagggatcattagccatagcaaaagcctcatcataagataacctgaagaacccaccgcggccgctgccggcgctcaggggcgctcacagagccgcagagagcgcgtcccgaagcagcgagaaacggaggaggacggcgagccctttccgctacactccacggcggcgggctcactac

SEQ ID NO: 12893 - RNA, 3776 nt, Homo sapiens
  source 1..3776: mol_type = other RNA
gctgggattacaggcatgagccacaatgcctaactactgatgcacgatttctaaattaagaatttataatataccataacttatattcttttatggttatcttttatggtttttttttttcctgcttccagtttaagaagttcttcctaaagggagtaggatcaggaagataatcacattttctaaatatgtttcaatcacattttaatctataattccacatatagtttctacatcaagtcgtcatcctgttgcattaattttaaagagcatgcttctagtgtataaggttgaaaagcattcttccccttatagattactaaagatttattattaatgggtatactgattttctttagtcttactttttatttatcctttttaagtcatcaacaaactttttctgagtatttgattacctttctttcaaaccgtacagtatctcctggatttgtttctctttttatttaggtactttctccaaaagtgattttagtttgtacggaaaatcttctgaagctttgatggtacatattcttattaatgccctcacattagaataactattttcagaacataaaattgtaggttcaaagtttttttcaggttcaatttcacattcttgagctaggcatggtactgatggttttcaccataacatacaccaatgtccttttgtctgtgggctcccatccagcctggtggctgaagtcatctacaggtaagattgaccaaacctctgaacaggactgaaaaaaatgttatcttcagaaaaccagccctcttgtacactgctgctgtgaatacaaattgattaacttttctggatggcaatctagcaatgcagatcaaacatttaaaaatacatatatatctcgacacaattttatctccaggcatccacatgaaagaactccacaatgttcagaagtgtacagataaggatactcgtcacagcattataatatgaaaaataaactgaaaaccacctcatctccaaacacaattaaattatgttaaaattctataaacagggattaggatgtgtaggtttacccaagggaaaatatatttaatgtttaggtttaaaaagcaaaaaaaaagcctactttttgtttcaaaaatatgcatatgtaagtagaaaatatctgaaagctgaaaggctactatccaaaaatattaacagcagctttctctaaacagaaactaaagcagtttctcttttctttttgcttttctatacttattacatgtctaccacaaacctctttgttataatttctccagttgagtcagttttacaatttggaatgcagagatcaagtggttctataatcagcatatacttcgcacgtaccattcattcaatccacacccctttaaacccctttgacacacgtcaaactcatttacatctatgtccctccaatgacaatatagtggtcaacacatataaaacatgaatacactatatcaagacactcaggaatacatctctgggataaaatctgactgccttctattatattttaatgaataaccaaaataaagggattctttcagttacagagagcagaataattaaaatagtaactttcaaactttgtagcagcagaagtatttcttcaaataaaatcttttttgaaacccaatatagaaaacagataaaaataaagccattctagaggtgggggccttggaaagtgagtactatccactcagacttctttcttgcctctcacaaggaaggaagctactgtgtagtttgaaaattactatttaatacattctgctaaccctaaatgccatgtcagagctagaagagaaaatgtacacacattcaatctaacatttatttatttcaggttttttttttttttggcaactataaattacattcactagtacacctggaattcttcatagtgtgttcaactaaagaataagcaaacacagcatagatcagtttaaaagaaatcatggtacttcttagagcaatttgcaaaaggggaaaaaagtcttaggctcactccttggaaataaatatcaagtaaccataaaaatattcagccatttttcagttattcggggagttcaggcatggtcccacgcagagcatcagagttcctctttgaaataacccagctttgccaatgacatctcttttctcaactgcataacctcccaaaacatctgatcaacatcctgctgtttcacgagtccctgctgaatgtatcgaatgtatgtaaaaaagttacatacagaagtgatcctgtatctgcaaaaaggagaaatataataatagttgcttgagtcccctaatttaattctgtgtttacaggacttactctggccagtgagagcacatttttttggtcctccgcattcaactgcagaagctttcacaaaccggataggttgtaatcccactggttcaatgcttagagtattgttttccacagcctccagaacagctgaagccaactcactttttgagaatgttaaacatggaaagatatcttcctggtagattttgtctaagaaaggacacgtcctgtccattgtgggctcatccttccacaatcggaattcattatacaaggataagtcagcctctttgcagtcttttacaattggctgtatcacactgaggtcctgatgactgccactcatagcactgcttgtgcttttatttcttgtatgcccctttttaaaaggtgtctttccacctggcaaaggctcctgcgtaggtgatgttggagaactggacaatacaagtgtcttcaatgcagctacttcagcttgaagtacatcaatttttccttgtgcttcttttagctgtttttctgctgttgcctgcttgatatttgcttctctcaccattttatgagcttccattgtatcacaagtgccaacagtattcagtatagtaacatgttgtacaggtttgtagcccaggagcaataagcaatatcatatagccaaggtgtgtaataggctgtaccatctaggttttaccacatcttggtttgtgtaagtatattctaccgatttctgcacgatgaaatctcaaatagactagctgtgagttcttccaattcctgtccaagttgatctcgcacttttgaaagcctctcacattcttcatcttttaacttcagttccctctgagcttttgcgagttcttcttttaatcgttcatagcccttttctctaacttccaaaacagatgggcttcgtaaacgagacagactatcagtactcaacccaaaaatatcatcactgccatcgcaagcctctgttatagtagcaccctgtaaaaactctctctctgcattatagttgtcctttcttgtagttaatttagttaatccagctgtgactccagaggtagagcaaggggctgggtctgtaacatgaaagctgatactagatatttccgcacaatttaaacgtctgggggatgaatacacgggttgtgtaggaagttcagaaacatctaatgcatttgccaagaaggtccggagaagtaggtgaagcaaggtttacttcatggaagccttccaagggatcattagccatagcaaaagcctcatcataagataacctgaagaacccaccgcggccgctgccggcgctcaggggcgctcacagagccgcagagagcgcgtcccgaagcagcgagaaacggaggaggacggcgagccctttccgctacactccacggcggcgggctcactacgccggcagccgccgagggaacgcgggactgcgcc

SEQ ID NO: 12894 - RNA, 3914 nt, Homo sapiens
  source 1..3914: mol_type = other RNA
gctgggattacaggcatgagccacaatgcctaactactgatgcacgatttctaaattaagaatttataatataccataacttatattcttttatggttatcttttatggtttttttttttcctgcttccagtttaagaagttcttcctaaagggagtaggatcaggaagataatcacattttctaaatatgtttcaatcacattttaatctataattccacatatagtttctacatcaagtcgtcatcctgttgcattaattttaaagagcatgcttctagtgtataaggttgaaaagcattcttccccttatagattactaaagatttattattaatgggtatactgattttctttagtcttactttttatttatcctttttaagtcatcaacaaactttttctgagtatttgattacctttctttcaaaccgtacagtatctcctggatttgtttctctttttatttaggtactttctccaaaagtgattttagtttgtacggaaaatcttctgaagctttgatggtacatattcttattaatgccctcacattagaataactattttcagaacataaaattgtaggttcaaagtttttttcaggttcaatttcacattcttgagctaggcatggtactgatggttttcaccataacatacaccaatgtccttttgtctgtgggctcccatccagcctggtggctgaagtcatctacaggtaagattgaccaaacctctgaacaggactgaaaaaaatgttatcttcagaaaaccagccctcttgtacactgctgctgtgaatacaaattgattaacttttctggatggcaatctagcaatgcagatcaaacatttaaaaatacatatatatctcgacacaattttatctccaggcatccacatgaaagaactccacaatgttcagaagtgtacagataaggatactcgtcacagcattataatatgaaaaataaactgaaaaccacctcatctccaaacacaattaaattatgttaaaattctataaacagggattaggatgtgtaggtttacccaagggaaaatatatttaatgtttaggtttaaaaagcaaaaaaaaagcctactttttgtttcaaaaatatgcatatgtaagtagaaaatatctgaaagctgaaaggctactatccaaaaatattaacagcagctttctctaaacagaaactaaagcagtttctcttttctttttgcttttctatacttattacatgtctaccacaaacctctttgttataatttctccagttgagtcagttttacaatttggaatgcagagatcaagtggttctataatcagcatatacttcgcacgtaccattcattcaatccacacccctttaaacccctttgacacacgtcaaactcatttacatctatgtccctccaatgacaatatagtggtcaacacatataaaacatgaatacactatatcaagacactcaggaatacatctctgggataaaatctgactgccttctattatattttaatgaataaccaaaataaagggattctttcagttacagagagcagaataattaaaatagtaactttcaaactttgtagcagcagaagtatttcttcaaataaaatcttttttgaaacccaatatagaaaacagataaaaataaagccattctagaggtgggggccttggaaagtgagtactatccactcagacttctttcttgcctctcacaaggaaggaagctactgtgtagtttgaaaattactatttaatacattctgctaaccctaaatgccatgtcagagctagaagagaaaatgtacacacattcaatctaacatttatttatttcaggttttttttttttttggcaactataaattacattcactagtacacctggaattcttcatagtgtgttcaactaaagaataagcaaacacagcatagatcagtttaaaagaaatcatggtacttcttagagcaatttgcaaaaggggaaaaaagtcttaggctcactccttggaaataaatatcaagtaaccataaaaatattcagccatttttcagttattcggggagttcaggcatggtcccacgcagagcatcagagttcctctttgaaataacccagctttgccaatgacatctcttttctcaactgcataacctcccaaaacatctgatcaacatcctgctgtttcacgagtccctgctgaatgtatcgaatgtatgtaaaaaagttacatacagaagtgatcctgtatctgcaaaaaggagaaatataataatagttgcttgagtcccctaatttaattctgtgtttacaggacttactctggccagtgagagcacatttttttggtcctccgcattcaactgcagaagctttcacaaaccggataggttgtaatcccactggttcaatgcttagagtattgttttccacagcctccagaacagctgaagccaactcactttttgagaatgttaaacatggaaagatatcttcctggtagattttgtctaagaaaggacacgtcctgtccattgtgggctcatccttccacaatcggaattcattatacaaggataagtcagcctctttgcagtcttttacaattggctgtatcacactgaggtcctgatgactgccactcatagcactgcttgtgcttttatttcttgtatgcccctttttaaaaggtgtctttccacctggcaaaggctcctgcgtaggtgatgttggagaactggacaatacaagtgtcttcaatgcagctacttcagcttgaagtacatcaatttttccttgtgcttcttttagctgtttttctgctgttgcctgcttgatatttgcttctctcaccattttatgagcttcctcaaatagactagctgtgagttcttccaattcctgtccaagttgatctcgcacttttgaaagcctctcacattcttcatcttttaacttcagttccctctgagcttttgcgagttcttcttttaatcgttcatagcccttttctctaacttccaaaacagatgggcttcgtaaacgagacagactatcagtactcaacccaaaaatatcatcactgccatcgcaagcctctgttatagtagcaccctgtaaaaactctctctctgcattatagttgtcctttcttgtagttaatttagttaatccagctgtgactccagaggtagagcaaggggctgggtctgtaacatgaaagctgatactagatatttccgcacaatttaaacgtctgggggatgaatacacgggttgtgtaggaagttcagaaacatctaatgcatttgccaagaaggtccggagaagtaggtgaagcaaggtttacttcatggaagccttccaagggatcattagccatagcaaaagcctcatcataagataaccctttcatcttttttaatcccataacaaccggcaactcttcacatgctgcgacttccacccagcatcatcacttctggagccagtaagctcgcgcttcctgggcggtcggggcgagttgtcaacgctgggagggcagagccatgcaatcccacccgtgcagttcgtctcaactcccccgaacacaagtctggcggcacggagctgcctacttgggcgcgactccgggcgcctgcccggaatttcccaccaggtttcaccgaaacctcccgagggtgacctctacgcctcagcacggtgcctcgcgcgtagtttcctaagactgggacacgaaaccaccccaggtccacagccctgccgcgcggcgtccggtgttgtgagctgcttccgacttgttcgggaactctctcttcatcctcttcgcgaccgcggccctccgctcccggccgcgcccgcccgccgccaggtaacccgctggactc

SEQ ID NO: 12895 - RNA, 4015 nt, Homo sapiens
  source 1..4015: mol_type = other RNA
gctgggattacaggcatgagccacaatgcctaactactgatgcacgatttctaaattaagaatttataatataccataacttatattcttttatggttatcttttatggtttttttttttcctgcttccagtttaagaagttcttcctaaagggagtaggatcaggaagataatcacattttctaaatatgtttcaatcacattttaatctataattccacatatagtttctacatcaagtcgtcatcctgttgcattaattttaaagagcatgcttctagtgtataaggttgaaaagcattcttccccttatagattactaaagatttattattaatgggtatactgattttctttagtcttactttttatttatcctttttaagtcatcaacaaactttttctgagtatttgattacctttctttcaaaccgtacagtatctcctggatttgtttctctttttatttaggtactttctccaaaagtgattttagtttgtacggaaaatcttctgaagctttgatggtacatattcttattaatgccctcacattagaataactattttcagaacataaaattgtaggttcaaagtttttttcaggttcaatttcacattcttgagctaggcatggtactgatggttttcaccataacatacaccaatgtccttttgtctgtgggctcccatccagcctggtggctgaagtcatctacaggtaagattgaccaaacctctgaacaggactgaaaaaaatgttatcttcagaaaaccagccctcttgtacactgctgctgtgaatacaaattgattaacttttctggatggcaatctagcaatgcagatcaaacatttaaaaatacatatatatctcgacacaattttatctccaggcatccacatgaaagaactccacaatgttcagaagtgtacagataaggatactcgtcacagcattataatatgaaaaataaactgaaaaccacctcatctccaaacacaattaaattatgttaaaattctataaacagggattaggatgtgtaggtttacccaagggaaaatatatttaatgtttaggtttaaaaagcaaaaaaaaagcctactttttgtttcaaaaatatgcatatgtaagtagaaaatatctgaaagctgaaaggctactatccaaaaatattaacagcagctttctctaaacagaaactaaagcagtttctcttttctttttgcttttctatacttattacatgtctaccacaaacctctttgttataatttctccagttgagtcagttttacaatttggaatgcagagatcaagtggttctataatcagcatatacttcgcacgtaccattcattcaatccacacccctttaaacccctttgacacacgtcaaactcatttacatctatgtccctccaatgacaatatagtggtcaacacatataaaacatgaatacactatatcaagacactcaggaatacatctctgggataaaatctgactgccttctattatattttaatgaataaccaaaataaagggattctttcagttacagagagcagaataattaaaatagtaactttcaaactttgtagcagcagaagtatttcttcaaataaaatcttttttgaaacccaatatagaaaacagataaaaataaagccattctagaggtgggggccttggaaagtgagtactatccactcagacttctttcttgcctctcacaaggaaggaagctactgtgtagtttgaaaattactatttaatacattctgctaaccctaaatgccatgtcagagctagaagagaaaatgtacacacattcaatctaacatttatttatttcaggttttttttttttttggcaactataaattacattcactagtacacctggaattcttcatagtgtgttcaactaaagaataagcaaacacagcatagatcagtttaaaagaaatcatggtacttcttagagcaatttgcaaaaggggaaaaaagtcttaggctcactccttggaaataaatatcaagtaaccataaaaatattcagccatttttcagttattcggggagttcaggcatggtcccacgcagagcatcagagttcctctttgaaataacccagctttgccaatgacatctcttttctcaactgcataacctcccaaaacatctgatcaacatcctgctgtttcacgagtccctgctgaatgtatcgaatgtatgtaaaaaagttacatacagaagtgatcctgtatctgcaaaaaggagaaatataataatagttgcttgagtcccctaatttaattctgtgtttacaggacttactctggccagtgagagcacatttttttggtcctccgcattcaactgcagaagctttcacaaaccggataggttgtaatcccactggttcaatgcttagagtattgttttccacagcctccagaacagctgaagccaactcactttttgagaatgttaaacatggaaagatatcttcctggtagattttgtctaagaaaggacacgtcctgtccattgtgggctcatccttccacaatcggaattcattatacaaggataagtcagcctctttgcagtcttttacaattggctgtatcacactgaggtcctgatgactgccactcatagcactgcttgtgcttttatttcttgtatgcccctttttaaaaggtgtctttccacctggcaaaggctcctgcgtaggtgatgttggagaactggacaatacaagtgtcttcaatgcagctacttcagcttgaagtacatcaatttttccttgtgcttcttttagctgtttttctgctgttgcctgcttgatatttgcttctctcaccattttatgagcttcctcaaatagactagctgtgagttcttccaattcctgtccaagttgatctcgcacttttgaaagcctctcacattcttcatcttttaacttcagttccctctgagcttttgcgagttcttcttttaatcgttcatagcccttttctctaacttccaaaacagatgggcttcgtaaacgagacagactatcagtactcaacccaaaaatatcatcactgccatcgcaagcctctgttatagtagcaccctgtaaaaactctctctctgcattatagttgtcctttcttgtagttaatttagttaatccagctgtgactccagaggtagagcaaggggctgggtctgtaacatgaaagctgatactagatatttccgcacaatttaaacgtctgggggatgaatacacgggttgtgtaggaagttcagaaacatctaatgcatttgcctggataggtacagaggataaagctgaagggtgtggccggtagatgacacttggtgaggtagtctgctcttgagttcctgattcatacacaccaagaaggtccggagaagtaggtgaagcaaggtttacttcatggaagccttccaagggatcattagccatagcaaaagcctcatcataagataaccctttcatcttttttaatcccataacaaccggcaactcttcacatgctgcgacttccacccagcatcatcacttctggagccagtaagctcgcgcttcctgggcggtcggggcgagttgtcaacgctgggagggcagagccatgcaatcccacccgtgcagttcgtctcaactcccccgaacacaagtctggcggcacggagctgcctacttgggcgcgactccgggcgcctgcccggaatttcccaccaggtttcaccgaaacctcccgagggtgacctctacgcctcagcacggtgcctcgcgcgtagtttcctaagactgggacacgaaaccaccccaggtccacagccctgccgcgcggcgtccggtgttgtgagctgcttccgacttgttcgggaactctctcttcatcctcttcgcgaccgcggccctccgctcccggccgcgcccgcccgccgccaggtaacccgctggactcgggctccct

SEQ ID NO: 12896 - RNA, 3630 nt, Homo sapiens
  source 1..3630: mol_type = other RNA
gctgggattacaggcatgagccacaatgcctaactactgatgcacgatttctaaattaagaatttataatataccataacttatattcttttatggttatcttttatggtttttttttttcctgcttccagtttaagaagttcttcctaaagggagtaggatcaggaagataatcacattttctaaatatgtttcaatcacattttaatctataattccacatatagtttctacatcaagtcgtcatcctgttgcattaattttaaagagcatgcttctagtgtataaggttgaaaagcattcttccccttatagattactaaagatttattattaatgggtatactgattttctttagtcttactttttatttatcctttttaagtcatcaacaaactttttctgagtatttgattacctttctttcaaaccgtacagtatctcctggatttgtttctctttttatttaggtactttctccaaaagtgattttagtttgtacggaaaatcttctgaagctttgatggtacatattcttattaatgccctcacattagaataactattttcagaacataaaattgtaggttcaaagtttttttcaggttcaatttcacattcttgagctaggcatggtactgatggttttcaccataacatacaccaatgtccttttgtctgtgggctcccatccagcctggtggctgaagtcatctacaggtaagattgaccaaacctctgaacaggactgaaaaaaatgttatcttcagaaaaccagccctcttgtacactgctgctgtgaatacaaattgattaacttttctggatggcaatctagcaatgcagatcaaacatttaaaaatacatatatatctcgacacaattttatctccaggcatccacatgaaagaactccacaatgttcagaagtgtacagataaggatactcgtcacagcattataatatgaaaaataaactgaaaaccacctcatctccaaacacaattaaattatgttaaaattctataaacagggattaggatgtgtaggtttacccaagggaaaatatatttaatgtttaggtttaaaaagcaaaaaaaaagcctactttttgtttcaaaaatatgcatatgtaagtagaaaatatctgaaagctgaaaggctactatccaaaaatattaacagcagctttctctaaacagaaactaaagcagtttctcttttctttttgcttttctatacttattacatgtctaccacaaacctctttgttataatttctccagttgagtcagttttacaatttggaatgcagagatcaagtggttctataatcagcatatacttcgcacgtaccattcattcaatccacacccctttaaacccctttgacacacgtcaaactcatttacatctatgtccctccaatgacaatatagtggtcaacacatataaaacatgaatacactatatcaagacactcaggaatacatctctgggataaaatctgactgccttctattatattttaatgaataaccaaaataaagggattctttcagttacagagagcagaataattaaaatagtaactttcaaactttgtagcagcagaagtatttcttcaaataaaatcttttttgaaacccaatatagaaaacagataaaaataaagccattctagaggtgggggccttggaaagtgagtactatccactcagacttctttcttgcctctcacaaggaaggaagctactgtgtagtttgaaaattactatttaatacattctgctaaccctaaatgccatgtcagagctagaagagaaaatgtacacacattcaatctaacatttatttatttcaggttttttttttttttggcaactataaattacattcactagtacacctggaattcttcatagtgtgttcaactaaagaataagcaaacacagcatagatcagtttaaaagaaatcatggtacttcttagagcaatttgcaaaaggggaaaaaagtcttaggctcactccttggaaataaatatcaagtaaccataaaaatattcagccatttttcagttattcggggagttcaggcatggtcccacgcagagcatcagagttcctctttgaaataacccagctttgccaatgacatctcttttctcaactgcataacctcccaaaacatctgatcaacatcctgctgtttcacgagtccctgctgaatgtatcgaatgtatgtaaaaaagttacatacagaagtgatcctgtatctgcaaaaaggagaaatataataatagttgcttgagtcccctaatttaattctgtgtttacaggacttactctggccagtgagagcacatttttttggtcctccgcattcaactgcagaagctttcacaaaccggataggttgtaatcccactggttcaatgcttagagtattgttttccacagcctccagaacagctgaagccaactcactttttgagaatgttaaacatggaaagatatcttcctggtagattttgtctaagaaaggacacgtcctgtccattgtgggctcatccttccacaatcggaattcattatacaaggataagtcagcctctttgcagtcttttacaattggctgtatcacactgaggtcctgatgactgccactcatagcactgcttgtgcttttatttcttgtatgcccctttttaaaaggtgtctttccacctggcaaaggctcctgcgtaggtgatgttggagaactggacaatacaagtgtcttcaatgcagctacttcagcttgaagtacatcaatttttccttgtgcttcttttagctgtttttctgctgttgcctgcttgatatttgcttctctcaccattttatgagcttcctcaaatagactagctgtgagttcttccaattcctgtccaagttgatctcgcacttttgaaagcctctcacattcttcatcttttaacttcagttccctctgagcttttgcgagttcttcttttaatcgttcatagcccttttctctaacttccaaaacagatgggcttcgtaaacgagacagactatcagtactcaacccaaaaatatcatcactgccatcgcaagcctctgttatagtagcaccctgtaaaaactctctctctgcattatagttgtcctttcttgtagttaatttagttaatccagctgtgactccagaggtagagcaaggggctgggtctgtaacatgaaagctgatactagatatttccgcacaatttaaacgtctgggggatgaatacacgggttgtgtaggaagttcagaaacatctaatgcatttgcctggataggtacagaggataaagctgaagggtgtggccggtagatgacacttggtgaggtagtctgctcttgagttcctgattcatacacaccaagaaggtccggagaagtaggtgaagcaaggtttacttcatggaagccttccaagggatcattagccatagcaaaagcctcatcataagataacctgaactcactgatcacatcttgtcacaaaaacggagacaatcaaacattatgtatattatgtggcaaataagaaatgaacatcactgccattaataaagcatt

SEQ ID NO: 12897 - RNA, 3698 nt, Homo sapiens
  source 1..3698: mol_type = other RNA
gctgggattacaggcatgagccacaatgcctaactactgatgcacgatttctaaattaagaatttataatataccataacttatattcttttatggttatcttttatggtttttttttttcctgcttccagtttaagaagttcttcctaaagggagtaggatcaggaagataatcacattttctaaatatgtttcaatcacattttaatctataattccacatatagtttctacatcaagtcgtcatcctgttgcattaattttaaagagcatgcttctagtgtataaggttgaaaagcattcttccccttatagattactaaagatttattattaatgggtatactgattttctttagtcttactttttatttatcctttttaagtcatcaacaaactttttctgagtatttgattacctttctttcaaaccgtacagtatctcctggatttgtttctctttttatttaggtactttctccaaaagtgattttagtttgtacggaaaatcttctgaagctttgatggtacatattcttattaatgccctcacattagaataactattttcagaacataaaattgtaggttcaaagtttttttcaggttcaatttcacattcttgagctaggcatggtactgatggttttcaccataacatacaccaatgtccttttgtctgtgggctcccatccagcctggtggctgaagtcatctacaggtaagattgaccaaacctctgaacaggactgaaaaaaatgttatcttcagaaaaccagccctcttgtacactgctgctgtgaatacaaattgattaacttttctggatggcaatctagcaatgcagatcaaacatttaaaaatacatatatatctcgacacaattttatctccaggcatccacatgaaagaactccacaatgttcagaagtgtacagataaggatactcgtcacagcattataatatgaaaaataaactgaaaaccacctcatctccaaacacaattaaattatgttaaaattctataaacagggattaggatgtgtaggtttacccaagggaaaatatatttaatgtttaggtttaaaaagcaaaaaaaaagcctactttttgtttcaaaaatatgcatatgtaagtagaaaatatctgaaagctgaaaggctactatccaaaaatattaacagcagctttctctaaacagaaactaaagcagtttctcttttctttttgcttttctatacttattacatgtctaccacaaacctctttgttataatttctccagttgagtcagttttacaatttggaatgcagagatcaagtggttctataatcagcatatacttcgcacgtaccattcattcaatccacacccctttaaacccctttgacacacgtcaaactcatttacatctatgtccctccaatgacaatatagtggtcaacacatataaaacatgaatacactatatcaagacactcaggaatacatctctgggataaaatctgactgccttctattatattttaatgaataaccaaaataaagggattctttcagttacagagagcagaataattaaaatagtaactttcaaactttgtagcagcagaagtatttcttcaaataaaatcttttttgaaacccaatatagaaaacagataaaaataaagccattctagaggtgggggccttggaaagtgagtactatccactcagacttctttcttgcctctcacaaggaaggaagctactgtgtagtttgaaaattactatttaatacattctgctaaccctaaatgccatgtcagagctagaagagaaaatgtacacacattcaatctaacatttatttatttcaggttttttttttttttggcaactataaattacattcactagtacacctggaattcttcatagtgtgttcaactaaagaataagcaaacacagcatagatcagtttaaaagaaatcatggtacttcttagagcaatttgcaaaaggggaaaaaagtcttaggctcactccttggaaataaatatcaagtaaccataaaaatattcagccatttttcagttattcggggagttcaggcatggtcccacgcagagcatcagagttcctctttgaaataacccagctttgccaatgacatctcttttctcaactgcataacctcccaaaacatctgatcaacatcctgctgtttcacgagtccctgctgaatgtatcgaatgtatgtaaaaaagttacatacagaagtgatcctgtatctgcaaaaaggagaaatataataatagttgcttgagtcccctaatttaattctgtgtttacaggacttactctggccagtgagagcacatttttttggtcctccgcattcaactgcagaagctttcacaaaccggataggttgtaatcccactggttcaatgcttagagtattgttttccacagcctccagaacagctgaagccaactcactttttgagaatgttaaacatggaaagatatcttcctggtagattttgtctaagaaaggacacgtcctgtccattgtgggctcatccttccacaatcggaattcattatacaaggataagtcagcctctttgcagtcttttacaattggctgtatcacactgaggtcctgatgactgccactcatagcactgcttgtgcttttatttcttgtatgcccctttttaaaaggtgtctttccacctggcaaaggctcctgcgtaggtgatgttggagaactggacaatacaagtgtcttcaatgcagctacttcagcttgaagtacatcaatttttccttgtgcttcttttagctgtttttctgctgttgcctgcttgatatttgcttctctcaccattttatgagcttcctcaaatagactagctgtgagttcttccaattcctgtccaagttgatctcgcacttttgaaagcctctcacattcttcatcttttaacttcagttccctctgagcttttgcgagttcttcttttaatcgttcatagcccttttctctaacttccaaaacagatgggcttcgtaaacgagacagactatcagtactcaacccaaaaatatcatcactgccatcgcaagcctctgttatagtagcaccctgtaaaaactctctctctgcattatagttgtcctttcttgtagttaatttagttaatccagctgtgactccagaggtagagcaaggggctgggtctgtaacatgaaagctgatactagatatttccgcacaatttaaacgtctgggggatgaatacacgggttgtgtaggaagttcagaaacatctaatgcatttgcctggataggtacagaggataaagctgaagggtgtggccggtagatgacacttggtgaggtagtctgctcttgagttcctgattcatacacaccaagaaggtccggagaagtaggtgaagcaaggtttacttcatggaagccttccaagggatcattagccatagcaaaagcctcatcataagataacctgaagaacccaccgcggccgctgccggcgctcaggggcgctcacagagccgcagagagcgcgtcccgaagcagcgagaaacggaggaggacggcgagccctttccgctacactccacggcggcgggctcactacgccggcagccgccgagggaacgcgggactgcgcctgc

SEQ ID NO: 12898 - RNA, 3995 nt, Homo sapiens
  source 1..3995: mol_type = other RNA
gctgggattacaggcatgagccacaatgcctaactactgatgcacgatttctaaattaagaatttataatataccataacttatattcttttatggttatcttttatggtttttttttttcctgcttccagtttaagaagttcttcctaaagggagtaggatcaggaagataatcacattttctaaatatgtttcaatcacattttaatctataattccacatatagtttctacatcaagtcgtcatcctgttgcattaattttaaagagcatgcttctagtgtataaggttgaaaagcattcttccccttatagattactaaagatttattattaatgggtatactgattttctttagtcttactttttatttatcctttttaagtcatcaacaaactttttctgagtatttgattacctttctttcaaaccgtacagtatctcctggatttgtttctctttttatttaggtactttctccaaaagtgattttagtttgtacggaaaatcttctgaagctttgatggtacatattcttattaatgccctcacattagaataactattttcagaacataaaattgtaggttcaaagtttttttcaggttcaatttcacattcttgagctaggcatggtactgatggttttcaccataacatacaccaatgtccttttgtctgtgggctcccatccagcctggtggctgaagtcatctacaggtaagattgaccaaacctctgaacaggactgaaaaaaatgttatcttcagaaaaccagccctcttgtacactgctgctgtgaatacaaattgattaacttttctggatggcaatctagcaatgcagatcaaacatttaaaaatacatatatatctcgacacaattttatctccaggcatccacatgaaagaactccacaatgttcagaagtgtacagataaggatactcgtcacagcattataatatgaaaaataaactgaaaaccacctcatctccaaacacaattaaattatgttaaaattctataaacagggattaggatgtgtaggtttacccaagggaaaatatatttaatgtttaggtttaaaaagcaaaaaaaaagcctactttttgtttcaaaaatatgcatatgtaagtagaaaatatctgaaagctgaaaggctactatccaaaaatattaacagcagctttctctaaacagaaactaaagcagtttctcttttctttttgcttttctatacttattacatgtctaccacaaacctctttgttataatttctccagttgagtcagttttacaatttggaatgcagagatcaagtggttctataatcagcatatacttcgcacgtaccattcattcaatccacacccctttaaacccctttgacacacgtcaaactcatttacatctatgtccctccaatgacaatatagtggtcaacacatataaaacatgaatacactatatcaagacactcaggaatacatctctgggataaaatctgactgccttctattatattttaatgaataaccaaaataaagggattctttcagttacagagagcagaataattaaaatagtaactttcaaactttgtagcagcagaagtatttcttcaaataaaatcttttttgaaacccaatatagaaaacagataaaaataaagccattctagaggtgggggccttggaaagtgagtactatccactcagacttctttcttgcctctcacaaggaaggaagctactgtgtagtttgaaaattactatttaatacattctgctaaccctaaatgccatgtcagagctagaagagaaaatgtacacacattcaatctaacatttatttatttcaggttttttttttttttggcaactataaattacattcactagtacacctggaattcttcatagtgtgttcaactaaagaataagcaaacacagcatagatcagtttaaaagaaatcatggtacttcttagagcaatttgcaaaaggggaaaaaagtcttaggctcactccttggaaataaatatcaagtaaccataaaaatattcagccatttttcagttattcggggagttcaggcatggtcccacgcagagcatcagagttcctctttgaaataacccagctttgccaatgacatctcttttctcaactgcataacctcccaaaacatctgatcaacatcctgctgtttcacgagtccctgctgaatgtatcgaatgtatgtaaaaaagttacatacagaagtgatcctgtatctgcaaaaaggagaaatataataatagttgcttgagtcccctaatttaattctgtgtttacaggacttactctggccagtgagagcacatttttttggtcctccgcattcaactgcagaagctttcacaaaccggataggttgtaatcccactggttcaatgcttagagtattgttttccacagcctccagaacagctgaagccaactcactttttgagaatgttaaacatggaaagatatcttcctggtagattttgtctaagaaaggacacgtcctgtccattgtgggctcatccttccacaatcggaattcattatacaaggataagtcagcctctttgcagtcttttacaattggctgtatcacactgaggtcctgatgactgccactcatagcactgcttgtgcttttatttcttgtatgcccctttttaaaaggtgtctttccacctggcaaaggctcctgcgtaggtgatgttggagaactggacaatacaagtgtcttcaatgcagctacttcagcttgaagtacatcaatttttccttgtgcttcttttagctgtttttctgctgttgcctgcttgatatttgcttctctcaccattttatgagcttcctcaaatagactagctgtgagttcttccaattcctgtccaagttgatctcgcacttttgaaagcctctcacattcttcatcttttaacttcagttccctctgagcttttgcgagttcttcttttaatcgttcatagcccttttctctaacttccaaaacagatgggcttcgtaaacgagacagactatcagtactcaacccaaaaatatcatcactgccatcgcaagcctctgttatagtagcaccctgtaaaaactctctctctgcattatagttgtcctttcttgtagttaatttagttaatccagctgtgactccagaggtagagcaaggggctgggtctgtaacatgaaagctgatactagatatttccgcacaatttaaacgtctgggggatgaatacacgggttgtgtaggaagttcagaaacatctaatgcatttgcctggataggtacagaggataaagctgaagggtgtggccggtagatgacacttggtgaggtagtctgctcttgagttcctgattcatacacaccaagaaggtccggagaagtaggtgaagcaaggtttacttcatggaagccttccaagggatcattagccatagcaaaagcctcatcataagataacctgagactccgcggccatatacaccttacgacgtgtgtgtgtgtggcgggagatgggaggggaggaatcctgtagaacccagatcccatcattccagcaactgccagagcgttcgagaatgtcatgtctgtacctgtcttctctcatcttttgtgccaactgttttatcaaacttctaccccactttaggtcttccaggtaggaaaaatacagaaagagccaagatcccaaaaatcaaaaaaaaataataataatagaggtagtcatagtatgtgtctctatgtttagcaaaagagaaacgtgcatttgtgtgatacacttattgaataggaccatcattctgggtattaatctcatctattagaggcagtaaagaaaagtagactatatgtatggttgttggagtcagaattactgggcttgagcctgccacctgctagctgagtgaccttaggcaaatgaatctctc

SEQ ID NO: 12899 - RNA, 3221 nt, Homo sapiens
  source 1..3221: mol_type = other RNA
gctgggattacaggcatgagccacaatgcctaactactgatgcacgatttctaaattaagaatttataatataccataacttatattcttttatggttatcttttatggtttttttttttcctgcttccagtttaagaagttcttcctaaagggagtaggatcaggaagataatcacattttctaaatatgtttcaatcacattttaatctataattccacatatagtttctacatcaagtcgtcatcctgttgcattaattttaaagagcatgcttctagtgtataaggttgaaaagcattcttccccttatagattactaaagatttattattaatgggtatactgattttctttagtcttactttttatttatcctttttaagtcatcaacaaactttttctgagtatttgattacctttctttcaaaccgtacagtatctcctggatttgtttctctttttatttaggtactttctccaaaagtgattttagtttgtacggaaaatcttctgaagctttgatggtacatattcttattaatgccctcacattagaataactattttcagaacataaaattgtaggttcaaagtttttttcaggttcaatttcacattcttgagctaggcatggtactgatggttttcaccataacatacaccaatgtccttttgtctgtgggctcccatccagcctggtggctgaagtcatctacaggtaagattgaccaaacctctgaacaggactgaaaaaaatgttatcttcagaaaaccagccctcttgtacactgctgctgtgaatacaaattgattaacttttctggatggcaatctagcaatgcagatcaaacatttaaaaatacatatatatctcgacacaattttatctccaggcatccacatgaaagaactccacaatgttcagaagtgtacagataaggatactcgtcacagcattataatatgaaaaataaactgaaaaccacctcatctccaaacacaattaaattatgttaaaattctataaacagggattaggatgtgtaggtttacccaagggaaaatatatttaatgtttaggtttaaaaagcaaaaaaaaagcctactttttgtttcaaaaatatgcatatgtaagtagaaaatatctgaaagctgaaaggctactatccaaaaatattaacagcagctttctctaaacagaaactaaagcagtttctcttttctttttgcttttctatacttattacatgtctaccacaaacctctttgttataatttctccagttgagtcagttttacaatttggaatgcagagatcaagtggttctataatcagcatatacttcgcacgtaccattcattcaatccacacccctttaaacccctttgacacacgtcaaactcatttacatctatgtccctccaatgacaatatagtggtcaacacatataaaacatgaatacactatatcaagacactcaggaatacatctctgggataaaatctgactgccttctattatattttaatgaataaccaaaataaagggattctttcagttacagagagcagaataattaaaatagtaactttcaaactttgtagcagcagaagtatttcttcaaataaaatcttttttgaaacccaatatagaaaacagataaaaataaagccattctagaggtgggggccttggaaagtgagtactatccactcagacttctttcttgcctctcacaaggaaggaagctactgtgtagtttgaaaattactatttaatacattctgctaaccctaaatgccatgtcagagctagaagagaaaatgtacacacattcaatctaacatttatttatttcaggttttttttttttttggcaactataaattacattcactagtacacctggaattcttcatagtgtgttcaactaaagaataagcaaacacagcatagatcagtttaaaagaaatcatggtacttcttagagcaatttgcaaaaggggaaaaaagtcttaggctcactccttggaaataaatatcaagtaaccataaaaatattcagccatttttcagttattcggggagttcaggcatggtcccacgcagagcatcagagttcctctttgaaataacccagctttgccaatgacatctcttttctcaactgcataacctcccaaaacatctgatcaacatcctgctgtttcacgagtccctgctgaatgtatcgaatgtatgtaaaaaagttacatacagaagtgatcctgtatctgcaaaaaggagaaatataataatagttgcttgagtcccctaatttaattctgtgtttacaggacttactctggccagtgagagcacatttttttggtcctccgcattcaactgcagaagctttcacaaaccggataggttgtaatcccactggttcaatgcttagagtattgttttccacagcctccagaacagctgaagccaactcactttttgagaatgttaaacatggaaagatatcttcctggtagattttgtctaagaaaggacacgtcctgtccattgtgggctcatccttccacaatcggaattcattatacaaggataagtcagcctctttgcagtcttttacaattggctgtatcacactgaggtcctgatgactgccactcatagcactgcttgtgcttttatttcttgtatgcccctttttaaaaggtgtctttccacctggcaaaggctcctgcgtaggtgatgttggagaactggacaatacaagtgtcttcaatgcagctacttcagcttgaagtacatcaatttttccttgtgcttcttttagctgtttttctgctgttgcctgcttgatatttgcttctctcaccattttatgagcttcctcaaatagactagctgtgagttcttccaattcctgtccaagttgatctcgcacttttgaaagcctctcacattcttcatcttttaacttcagttcctggaaaatcgggtcactcccatccgaatattgcgcttttcagaccggcttaagaaacggcgcaccacgagactatatcccacacctggctcagagggtcctacgcccacggaatctcgctgattgctagcacagcagtctgagatcaaactgcaaggcggcaacgaggctgggggagggacgcccgccattgcccaggcttgcttaggtaaacaaagcagccgggaagc

SEQ ID NO: 12900 - RNA, 3136 nt, Homo sapiens
  source 1..3136: mol_type = other RNA
gctgggattacaggcatgagccacaatgcctaactactgatgcacgatttctaaattaagaatttataatataccataacttatattcttttatggttatcttttatggtttttttttttcctgcttccagtttaagaagttcttcctaaagggagtaggatcaggaagataatcacattttctaaatatgtttcaatcacattttaatctataattccacatatagtttctacatcaagtcgtcatcctgttgcattaattttaaagagcatgcttctagtgtataaggttgaaaagcattcttccccttatagattactaaagatttattattaatgggtatactgattttctttagtcttactttttatttatcctttttaagtcatcaacaaactttttctgagtatttgattacctttctttcaaaccgtacagtatctcctggatttgtttctctttttatttaggtactttctccaaaagtgattttagtttgtacggaaaatcttctgaagctttgatggtacatattcttattaatgccctcacattagaataactattttcagaacataaaattgtaggttcaaagtttttttcaggttcaatttcacattcttgagctaggcatggtactgatggttttcaccataacatacaccaatgtccttttgtctgtgggctcccatccagcctggtggctgaagtcatctacaggtaagattgaccaaacctctgaacaggactgaaaaaaatgttatcttcagaaaaccagccctcttgtacactgctgctgtgaatacaaattgattaacttttctggatggcaatctagcaatgcagatcaaacatttaaaaatacatatatatctcgacacaattttatctccaggcatccacatgaaagaactccacaatgttcagaagtgtacagataaggatactcgtcacagcattataatatgaaaaataaactgaaaaccacctcatctccaaacacaattaaattatgttaaaattctataaacagggattaggatgtgtaggtttacccaagggaaaatatatttaatgtttaggtttaaaaagcaaaaaaaaagcctactttttgtttcaaaaatatgcatatgtaagtagaaaatatctgaaagctgaaaggctactatccaaaaatattaacagcagctttctctaaacagaaactaaagcagtttctcttttctttttgcttttctatacttattacatgtctaccacaaacctctttgttataatttctccagttgagtcagttttacaatttggaatgcagagatcaagtggttctataatcagcatatacttcgcacgtaccattcattcaatccacacccctttaaacccctttgacacacgtcaaactcatttacatctatgtccctccaatgacaatatagtggtcaacacatataaaacatgaatacactatatcaagacactcaggaatacatctctgggataaaatctgactgccttctattatattttaatgaataaccaaaataaagggattctttcagttacagagagcagaataattaaaatagtaactttcaaactttgtagcagcagaagtatttcttcaaataaaatcttttttgaaacccaatatagaaaacagataaaaataaagccattctagaggtgggggccttggaaagtgagtactatccactcagacttctttcttgcctctcacaaggaaggaagctactgtgtagtttgaaaattactatttaatacattctgctaaccctaaatgccatgtcagagctagaagagaaaatgtacacacattcaatctaacatttatttatttcaggttttttttttttttggcaactataaattacattcactagtacacctggaattcttcatagtgtgttcaactaaagaataagcaaacacagcatagatcagtttaaaagaaatcatggtacttcttagagcaatttgcaaaaggggaaaaaagtcttaggctcactccttggaaataaatatcaagtaaccataaaaatattcagccatttttcagttattcggggagttcaggcatggtcccacgcagagcatcagagttcctctttgaaataacccagctttgccaatgacatctcttttctcaactgcataacctcccaaaacatctgatcaacatcctgctgtttcacgagtccctgctgaatgtatcgaatgtatgtaaaaaagttacatacagaagtgatcctgtatctgcaaaaaggagaaatataataatagttgcttgagtcccctaatttaattctgtgtttacaggacttactctggccagtgagagcacatttttttggtcctccgcattcaactgcagaagctttcacaaaccggataggttgtaatcccactggttcaatgcttagagtattgttttccacagcctccagaacagctgaagccaactcactttttgagaatgttaaacatggaaagatatcttcctggtagattttgtctaagaaaggacacgtcctgtccattgtgggctcatccttccacaatcggaattcattatacaaggataagtcagcctctttgcagtcttttacaattggctgtatcacactgaggtcctgatgactgccactcatagcactgcttgtgcttttatttcttgtatgcccctttttaaaaggtgtctttccacctggcaaaggctcctgcgtaggtgatgttggagaactggacaatacaagtgtcttcaatgcagctacttcagcttgaagtacatcaatttttccttgtgcttcttttagctgtttttctgctgttgcctgcttgatatttgcttctctcaccattttatgagcttcctcaaatagactagctgtgagttcttccaattcctgtccaagttgatctcgcacttttgaaagcctctcacattcttcatcttttaacttcagttcctggctcagagggtcctacgcccacggaatctcgctgattgctagcacagcagtctgagatcaaactgcaaggcggcaacgaggctgggggagggacgcccgccattgcccaggcttgcttaggtaaacaaagcagccgggaagc

SEQ ID NO: 12901 - RNA, 3693 nt, Homo sapiens
  source 1..3693: mol_type = other RNA
gctgggattacaggcatgagccacaatgcctaactactgatgcacgatttctaaattaagaatttataatataccataacttatattcttttatggttatcttttatggtttttttttttcctgcttccagtttaagaagttcttcctaaagggagtaggatcaggaagataatcacattttctaaatatgtttcaatcacattttaatctataattccacatatagtttctacatcaagtcgtcatcctgttgcattaattttaaagagcatgcttctagtgtataaggttgaaaagcattcttccccttatagattactaaagatttattattaatgggtatactgattttctttagtcttactttttatttatcctttttaagtcatcaacaaactttttctgagtatttgattacctttctttcaaaccgtacagtatctcctggatttgtttctctttttatttaggtactttctccaaaagtgattttagtttgtacggaaaatcttctgaagctttgatggtacatattcttattaatgccctcacattagaataactattttcagaacataaaattgtaggttcaaagtttttttcaggttcaatttcacattcttgagctaggcatggtactgatggttttcaccataacatacaccaatgtccttttgtctgtgggctcccatccagcctggtggctgaagtcatctacaggtaagattgaccaaacctctgaacaggactgaaaaaaatgttatcttcagaaaaccagccctcttgtacactgctgctgtgaatacaaattgattaacttttctggatggcaatctagcaatgcagatcaaacatttaaaaatacatatatatctcgacacaattttatctccaggcatccacatgaaagaactccacaatgttcagaagtgtacagataaggatactcgtcacagcattataatatgaaaaataaactgaaaaccacctcatctccaaacacaattaaattatgttaaaattctataaacagggattaggatgtgtaggtttacccaagggaaaatatatttaatgtttaggtttaaaaagcaaaaaaaaagcctactttttgtttcaaaaatatgcatatgtaagtagaaaatatctgaaagctgaaaggctactatccaaaaatattaacagcagctttctctaaacagaaactaaagcagtttctcttttctttttgcttttctatacttattacatgtctaccacaaacctctttgttataatttctccagttgagtcagttttacaatttggaatgcagagatcaagtggttctataatcagcatatacttcgcacgtaccattcattcaatccacacccctttaaacccctttgacacacgtcaaactcatttacatctatgtccctccaatgacaatatagtggtcaacacatataaaacatgaatacactatatcaagacactcaggaatacatctctgggataaaatctgactgccttctattatattttaatgaataaccaaaataaagggattctttcagttacagagagcagaataattaaaatagtaactttcaaactttgtagcagcagaagtatttcttcaaataaaatcttttttgaaacccaatatagaaaacagataaaaataaagccattctagaggtgggggccttggaaagtgagtactatccactcagacttctttcttgcctctcacaaggaaggaagctactgtgtagtttgaaaattactatttaatacattctgctaaccctaaatgccatgtcagagctagaagagaaaatgtacacacattcaatctaacatttatttatttcaggttttttttttttttggcaactataaattacattcactagtacacctggaattcttcatagtgtgttcaactaaagaataagcaaacacagcatagatcagtttaaaagaaatcatggtacttcttagagcaatttgcaaaaggggaaaaaagtcttaggctcactccttggaaataaatatcaagtaaccataaaaatattcagccatttttcagttattcggggagttcaggcatggtcccacgcagagcatcagagttcctctttgaaataacccagctttgccaatgacatctcttttctcaactgcataacctcccaaaacatctgatcaacatcctgctgtttcacgagtccctgctgaatgtatcgaatgtatgtaaaaaagttacatacagaagtgatcctgtatctgcaaaaaggagaaatataataatagttgcttgagtcccctaatttaattctgtgtttacaggacttactctggccagtgagagcacatttttttggtcctccgcattcaactgcagaagctttcacaaaccggataggttgtaatcccactggttcaatgcttagagtattgttttccacagcctccagaacagctgaagccaatttttgagaatgttaaacatggaaagatatcttcctggtagattttgtctaagaaaggacacgtcctgtccattgtgggctcatccttccacaatcggaattcattatacaaggataagtcagcctctttgcagtcttttacaattggctgtatcacactgaggtcctgatgactgccactcatagcactgcttgtgcttttatttcttgtatgcccctttttaaaaggtgtctttccacctggcaaaggctcctgcgtaggtgatgttggagaactggacaatacaagtgtcttcaatgcagctacttcagcttgaagtacatcaatttttccttgtgcttcttttagctgtttttctgctgttgcctgcttgatatttgcttctctcaccattttatgagcttcctcaaatagactagctgtgagttcttccaattcctgtccaagttgatctcgcacttttgaaagcctctcacattcttcatcttttaacttcagttccctctgagcttttgcgagttcttcttttaatcgttcatagcccttttctctaacttccaaaacagatgggcttcgtaaacgagacagactatcagtactcaacccaaaaatatcatcactgccatcgcaagcctctgttatagtagcaccctgtaaaaactctctctctgcattatagttgtcctttcttgtagttaatttagttaatccagctgtgactccagaggtagagcaaggggctgggtctgtaacatgaaagctgatactagatatttccgcacaatttaaacgtctgggggatgaatacacgggttgtgtaggaagttcagaaacatctaatgcatttgcctggataggtacagaggataaagctgaagggtgtggccggtagatgacacttggtgaggtagtctgctcttgagttcctgattcatacacaccaagaaggtccggagaagtaggtgaagcaaggtttacttcatggaagccttccaagggatcattagccatagcaaaagcctcatcataagataacctgaagaacccaccgcggccgctgccggcgctcaggggcgctcacagagccgcagagagcgcgtcccgaagcagcgagaaacggaggaggacggcgagccctttccgctacactccacggcggcgggctcactacgccggcagccgccgagggaacgcgggactgcgcctgc

SEQ ID NO: 12902 - RNA, 3663 nt, Homo sapiens
  source 1..3663: mol_type = other RNA
gctgggattacaggcatgagccacaatgcctaactactgatgcacgatttctaaattaagaatttataatataccataacttatattcttttatggttatcttttatggtttttttttttcctgcttccagtttaagaagttcttcctaaagggagtaggatcaggaagataatcacattttctaaatatgtttcaatcacattttaatctataattccacatatagtttctacatcaagtcgtcatcctgttgcattaattttaaagagcatgcttctagtgtataaggttgaaaagcattcttccccttatagattactaaagatttattattaatgggtatactgattttctttagtcttactttttatttatcctttttaagtcatcaacaaactttttctgagtatttgattacctttctttcaaaccgtacagtatctcctggatttgtttctctttttatttaggtactttctccaaaagtgattttagtttgtacggaaaatcttctgaagctttgatggtacatattcttattaatgccctcacattagaataactattttcagaacataaaattgtaggttcaaagtttttttcaggttcaatttcacattcttgagctaggcatggtactgatggttttcaccataacatacaccaatgtccttttgtctgtgggctcccatccagcctggtggctgaagtcatctacaggtaagattgaccaaacctctgaacaggactgaaaaaaatgttatcttcagaaaaccagccctcttgtacactgctgctgtgaatacaaattgattaacttttctggatggcaatctagcaatgcagatcaaacatttaaaaatacatatatatctcgacacaattttatctccaggcatccacatgaaagaactccacaatgttcagaagtgtacagataaggatactcgtcacagcattataatatgaaaaataaactgaaaaccacctcatctccaaacacaattaaattatgttaaaattctataaacagggattaggatgtgtaggtttacccaagggaaaatatatttaatgtttaggtttaaaaagcaaaaaaaaagcctactttttgtttcaaaaatatgcatatgtaagtagaaaatatctgaaagctgaaaggctactatccaaaaatattaacagcagctttctctaaacagaaactaaagcagtttctcttttctttttgcttttctatacttattacatgtctaccacaaacctctttgttataatttctccagttgagtcagttttacaatttggaatgcagagatcaagtggttctataatcagcatatacttcgcacgtaccattcattcaatccacacccctttaaacccctttgacacacgtcaaactcatttacatctatgtccctccaatgacaatatagtggtcaacacatataaaacatgaatacactatatcaagacactcaggaatacatctctgggataaaatctgactgccttctattatattttaatgaataaccaaaataaagggattctttcagttacagagagcagaataattaaaatagtaactttcaaactttgtagcagcagaagtatttcttcaaataaaatcttttttgaaacccaatatagaaaacagataaaaataaagccattctagaggtgggggccttggaaagtgagtactatccactcagacttctttcttgcctctcacaaggaaggaagctactgtgtagtttgaaaattactatttaatacattctgctaaccctaaatgccatgtcagagctagaagagaaaatgtacacacattcaatctaacatttatttatttcaggttttttttttttttggcaactataaattacattcactagtacacctggaattcttcatagtgtgttcaactaaagaataagcaaacacagcatagatcagtttaaaagaaatcatggtacttcttagagcaatttgcaaaaggggaaaaaagtcttaggctcactccttggaaataaatatcaagtaaccataaaaatattcagccatttttcagttattcggggagttcaggcatggtcccacgcagagcatcagagttcctctttgaaataacccagctttgccaatgacatctcttttctcaactgcataacctcccaaaacatctgatcaacatcctgctgtttcacgagtccctgctgaatgtatcgaatgtatgtaaaaaagttacatacagaagtgatcctgtatctgcaaaaaggagaaatataataatagttgcttgagtcccctaatttaattctgtgtttacaggacttactctggccagtgagagcacatttttttggtcctccgcattcaactgcagaagctttcacaaaccggataggttgtaatcccactggttcaatgcttagagtattgttttccacagcctccagaacagctgaagccaatttttgagaatgttaaacatggaaagatatcttcctggtagattttgtctaagaaaggacacgtcctgtccattgtgggctcatccttccacaatcggaattcattatacaaggataagtcagcctctttgcagtcttttacaattggctgtatcacactgaggtcctgatgactgccactcatagcactgcttgtgcttttatttcttgtatgcccctttttaaaaggtgtctttccacctggcaaaggctcctgcgtaggtgatgttggagaactggacaatacaagtgtcttcaatgcagctacttcagcttgaagtacatcaatttttccttgtgcttcttttagctgtttttctgctgttgcctgcttgatatttgcttctctcaccattttatgagcttcctcaaatagactagctgtgagttcttccaattcctgtccaagttgatctcgcacttttgaaagcctctcacattcttcatcttttaacttcagttccctctgagcttttgcgagttcttcttttaatcgttcatagcccttttctctaacttccaaaacagatgggcttcgtaaacgagacagactatcagtactcaacccaaaaatatcatcactgccatcgcaagcctctgttatagtagcaccctgtaaaaactctctctctgcattatagttgtcctttcttgtagttaatttagttaatccagctgtgactccagaggtagagcaaggggctgggtctgtaacatgaaagctgatactagatatttccgcacaatttaaacgtctgggggatgaatacacgggttgtgtaggaagttcagaaacatctaatgcatttgcctggataggtacagaggataaagctgaagggtgtggccggtagatgacacttggtgaggtagtctgctcttgagttcctgattcatacacaccaagaaggtccggagaagtaggtgaagcaaggtttacttcatggaagccttccaagggatcattagccatagcaaaagcctcatcataagataacctgagactccgcggccatatacaccttacgacgtgtgtgtgtgtggcgggagatgggaggggaggaatcctgtagaacccagatcccatcattccagcaactgccagagcgttcgagaatgtcatgtctgtacctgtcttct

SEQ ID NO: 12903 - RNA, 3550 nt, Homo sapiens
  source 1..3550: mol_type = other RNA
gctgggattacaggcatgagccacaatgcctaactactgatgcacgatttctaaattaagaatttataatataccataacttatattcttttatggttatcttttatggtttttttttttcctgcttccagtttaagaagttcttcctaaagggagtaggatcaggaagataatcacattttctaaatatgtttcaatcacattttaatctataattccacatatagtttctacatcaagtcgtcatcctgttgcattaattttaaagagcatgcttctagtgtataaggttgaaaagcattcttccccttatagattactaaagatttattattaatgggtatactgattttctttagtcttactttttatttatcctttttaagtcatcaacaaactttttctgagtatttgattacctttctttcaaaccgtacagtatctcctggatttgtttctctttttatttaggtactttctccaaaagtgattttagtttgtacggaaaatcttctgaagctttgatggtacatattcttattaatgccctcacattagaataactattttcagaacataaaattgtaggttcaaagtttttttcaggttcaatttcacattcttgagctaggcatggtactgatggttttcaccataacatacaccaatgtccttttgtctgtgggctcccatccagcctggtggctgaagtcatctacaggtaagattgaccaaacctctgaacaggactgaaaaaaatgttatcttcagaaaaccagccctcttgtacactgctgctgtgaatacaaattgattaacttttctggatggcaatctagcaatgcagatcaaacatttaaaaatacatatatatctcgacacaattttatctccaggcatccacatgaaagaactccacaatgttcagaagtgtacagataaggatactcgtcacagcattataatatgaaaaataaactgaaaaccacctcatctccaaacacaattaaattatgttaaaattctataaacagggattaggatgtgtaggtttacccaagggaaaatatatttaatgtttaggtttaaaaagcaaaaaaaaagcctactttttgtttcaaaaatatgcatatgtaagtagaaaatatctgaaagctgaaaggctactatccaaaaatattaacagcagctttctctaaacagaaactaaagcagtttctcttttctttttgcttttctatacttattacatgtctaccacaaacctctttgttataatttctccagttgagtcagttttacaatttggaatgcagagatcaagtggttctataatcagcatatacttcgcacgtaccattcattcaatccacacccctttaaacccctttgacacacgtcaaactcatttacatctatgtccctccaatgacaatatagtggtcaacacatataaaacatgaatacactatatcaagacactcaggaatacatctctgggataaaatctgactgccttctattatattttaatgaataaccaaaataaagggattctttcagttacagagagcagaataattaaaatagtaactttcaaactttgtagcagcagaagtatttcttcaaataaaatcttttttgaaacccaatatagaaaacagataaaaataaagccattctagaggtgggggccttggaaagtgagtactatccactcagacttctttcttgcctctcacaaggaaggaagctactgtgtagtttgaaaattactatttaatacattctgctaaccctaaatgccatgtcagagctagaagagaaaatgtacacacattcaatctaacatttatttatttcaggttttttttttttttggcaactataaattacattcactagtacacctggaattcttcatagtgtgttcaactaaagaataagcaaacacagcatagatcagtttaaaagaaatcatggtacttcttagagcaatttgcaaaaggggaaaaaagtcttaggctcactccttggaaataaatatcaagtaaccataaaaatattcagccatttttcagttattcggggagttcaggcatggtcccacgcagagcatcagagttcctctttgaaataacccagctttgccaatgacatctcttttctcaactgcataacctcccaaaacatctgatcaacatcctgctgtttcacgagtccctgctgaatgtatcgaatgtatgtaaaaaagttacatacagaagtgatcctgtatctgcaaaaaggagaaatataataatagttgcttgagtcccctaatttaattctgtgtttacaggacttactctggccagtgagagcacatttttttttgagaatgttaaacatggaaagatatcttcctggtagattttgtctaagaaaggacacgtcctgtccattgtgggctcatccttccacaatcggaattcattatacaaggataagtcagcctctttgcagtcttttacaattggctgtatcacactgaggtcctgatgactgccactcatagcactgcttgtgcttttatttcttgtatgcccctttttaaaaggtgtctttccacctggcaaaggctcctgcgtaggtgatgttggagaactggacaatacaagtgtcttcaatgcagctacttcagcttgaagtacatcaatttttccttgtgcttcttttagctgtttttctgctgttgcctgcttgatatttgcttctctcaccattttatgagcttcctcaaatagactagctgtgagttcttccaattcctgtccaagttgatctcgcacttttgaaagcctctcacattcttcatcttttaacttcagttccctctgagcttttgcgagttcttcttttaatcgttcatagcccttttctctaacttccaaaacagatgggcttcgtaaacgagacagactatcagtactcaacccaaaaatatcatcactgccatcgcaagcctctgttatagtagcaccctgtaaaaactctctctctgcattatagttgtcctttcttgtagttaatttagttaatccagctgtgactccagaggtagagcaaggggctgggtctgtaacatgaaagctgatactagatatttccgcacaatttaaacgtctgggggatgaatacacgggttgtgtaggaagttcagaaacatctaatgcatttgcctggataggtacagaggataaagctgaagggtgtggccggtagatgacacttggtgaggtagtctgctcttgagttcctgattcatacacaccaagaaggtccggagaagtaggtgaagcaaggtttacttcatggaagccttccaagggatcattagccatagcaaaagcctcatcataagataacctgagactccgcggccatatacaccttacgacgtgtgtgtgtgtggcgggagatgggaggggaggaatcctgtagaacccagatcccatcattccagcaactgccagagcgttcgagaatgtcatgtctgtacctgtcttct

SEQ ID NO: 12904 - RNA, 3915 nt, Homo sapiens
  source 1..3915: mol_type = other RNA
gctgggattacaggcatgagccacaatgcctaactactgatgcacgatttctaaattaagaatttataatataccataacttatattcttttatggttatcttttatggtttttttttttcctgcttccagtttaagaagttcttcctaaagggagtaggatcaggaagataatcacattttctaaatatgtttcaatcacattttaatctataattccacatatagtttctacatcaagtcgtcatcctgttgcattaattttaaagagcatgcttctagtgtataaggttgaaaagcattcttccccttatagattactaaagatttattattaatgggtatactgattttctttagtcttactttttatttatcctttttaagtcatcaacaaactttttctgagtatttgattacctttctttcaaaccgtacagtatctcctggatttgtttctctttttatttaggtactttctccaaaagtgattttagtttgtacggaaaatcttctgaagctttgatggtacatattcttattaatgccctcacattagaataactattttcagaacataaaattgtaggttcaaagtttttttcaggttcaatttcacattcttgagctaggcatggtactgatggttttcaccataacatacaccaatgtccttttgtctgtgggctcccatccagcctggtggctgaagtcatctacaggtaagattgaccaaacctctgaacaggactgaaaaaaatgttatcttcagaaaaccagccctcttgtacactgctgctgtgaatacaaattgattaacttttctggatggcaatctagcaatgcagatcaaacatttaaaaatacatatatatctcgacacaattttatctccaggcatccacatgaaagaactccacaatgttcagaagtgtacagataaggatactcgtcacagcattataatatgaaaaataaactgaaaaccacctcatctccaaacacaattaaattatgttaaaattctataaacagggattaggatgtgtaggtttacccaagggaaaatatatttaatgtttaggtttaaaaagcaaaaaaaaagcctactttttgtttcaaaaatatgcatatgtaagtagaaaatatctgaaagctgaaaggctactatccaaaaatattaacagcagctttctctaaacagaaactaaagcagtttctcttttctttttgcttttctatacttattacatgtctaccacaaacctctttgttataatttctccagttgagtcagttttacaatttggaatgcagagatcaagtggttctataatcagcatatacttcgcacgtaccattcattcaatccacacccctttaaacccctttgacacacgtcaaactcatttacatctatgtccctccaatgacaatatagtggtcaacacatataaaacatgaatacactatatcaagacactcaggaatacatctctgggataaaatctgactgccttctattatattttaatgaataaccaaaataaagggattctttcagttacagagagcagaataattaaaatagtaactttcaaactttgtagcagcagaagtatttcttcaaataaaatcttttttgaaacccaatatagaaaacagataaaaataaagccattctagaggtgggggccttggaaagtgagtactatccactcagacttctttcttgcctctcacaaggaaggaagctactgtgtagtttgaaaattactatttaatacattctgctaaccctaaatgccatgtcagagctagaagagaaaatgtacacacattcaatctaacatttatttatttcaggttttttttttttttggcaactataaattacattcactagtacacctggaattcttcatagtgtgttcaactaaagaataagcaaacacagcatagatcagtttaaaagaaatcatggtacttcttagagcaatttgcaaaaggggaaaaaagtcttaggctcactccttggaaataaatatcaagtaaccataaaaatattcagccatttttcagttattcggggagttcaggcatggtcccacgcagagcatcagagttcctctttgaaataacccagctttgccaatgacatctcttttctcaactgcataacctcccaaaacatctgatcaacatcctgctgtttcacgagtccctgctgaatgtatcgaatgtatgtaaaaaagttacatacagaagtgattttggtcctccgcattcaactgcagaagctttcacaaaccggataggttgtaatcccactggttcaatgcttagagtattgttttccacagcctccagaacagctgaagccaactcactttttgagaatgttaaacatggaaagatatcttcctggtagattttgtctaagaaaggacacgtcctgtccattgtgggctcatccttccacaatcggaattcattatacaaggataagtcagcctctttgcagtcttttacaattggctgtatcacactgaggtcctgatgactgccactcatagcactgcttgtgcttttatttcttgtatgcccctttttaaaaggtgtctttccacctggcaaaggctcctgcgtaggtgatgttggagaactggacaatacaagtgtcttcaatgcagctacttcagcttgaagtacatcaatttttccttgtgcttcttttagctgtttttctgctgttgcctgcttgatatttgcttctctcaccattttatgagcttcctcaaatagactagctgtgagttcttccaattcctgtccaagttgatctcgcacttttgaaagcctctcacattcttcatcttttaacttcagttccctctgagcttttgcgagttcttcttttaatcgttcatagcccttttctctaacttccaaaacagatgggcttcgtaaacgagacagactatcagtactcaacccaaaaatatcatcactgccatcgcaagcctctgttatagtagcaccctgtaaaaactctctctctgcattatagttgtcctttcttgtagttaatttagttaatccagctgtgactccagaggtagagcaaggggctgggtctgtaacatgaaagctgatactagatatttccgcacaatttaaacgtctgggggatgaatacacgggttgtgtaggaagttcagaaacatctaatgcatttgcctggataggtacagaggataaagctgaagggtgtggccggtagatgacacttggtgaggtagtctgctcttgagttcctgattcatacacaccaagaaggtccggagaagtaggtgaagcaaggtttacttcatggaagccttccaagggatcattagccatagcaaaagcctcatcataagataaccctttcatcttttttaatcccataacaaccggcaactcttcacatgctgcgacttccacccagcatcatcacttctggagccagtaagctcgcgcttcctgggcggtcggggcgagttgtcaacgctgggagggcagagccatgcaatcccacccgtgcagttcgtctcaactcccccgaacacaagtctggcggcacggagctgcctacttgggcgcgactccgggcgcctgcccggaatttcccaccaggtttcaccgaaacctcccgagggtgacctctacgcctcagcacggtgcctcgcgcgtagtttcctaagactgggacacgaaaccaccccaggtccacagccctgccgcgcggcgtccggtgttgtgagctgcttccgacttgttcgggaactctctcttcatcctcttcgcgaccgcggccctccgctcccggccgcgcccgcccgccgccaggtaacccgctggactcgggctccct

SEQ ID NO: 12905 - RNA, 3598 nt, Homo sapiens
  source 1..3598: mol_type = other RNA
gctgggattacaggcatgagccacaatgcctaactactgatgcacgatttctaaattaagaatttataatataccataacttatattcttttatggttatcttttatggtttttttttttcctgcttccagtttaagaagttcttcctaaagggagtaggatcaggaagataatcacattttctaaatatgtttcaatcacattttaatctataattccacatatagtttctacatcaagtcgtcatcctgttgcattaattttaaagagcatgcttctagtgtataaggttgaaaagcattcttccccttatagattactaaagatttattattaatgggtatactgattttctttagtcttactttttatttatcctttttaagtcatcaacaaactttttctgagtatttgattacctttctttcaaaccgtacagtatctcctggatttgtttctctttttatttaggtactttctccaaaagtgattttagtttgtacggaaaatcttctgaagctttgatggtacatattcttattaatgccctcacattagaataactattttcagaacataaaattgtaggttcaaagtttttttcaggttcaatttcacattcttgagctaggcatggtactgatggttttcaccataacatacaccaatgtccttttgtctgtgggctcccatccagcctggtggctgaagtcatctacaggtaagattgaccaaacctctgaacaggactgaaaaaaatgttatcttcagaaaaccagccctcttgtacactgctgctgtgaatacaaattgattaacttttctggatggcaatctagcaatgcagatcaaacatttaaaaatacatatatatctcgacacaattttatctccaggcatccacatgaaagaactccacaatgttcagaagtgtacagataaggatactcgtcacagcattataatatgaaaaataaactgaaaaccacctcatctccaaacacaattaaattatgttaaaattctataaacagggattaggatgtgtaggtttacccaagggaaaatatatttaatgtttaggtttaaaaagcaaaaaaaaagcctactttttgtttcaaaaatatgcatatgtaagtagaaaatatctgaaagctgaaaggctactatccaaaaatattaacagcagctttctctaaacagaaactaaagcagtttctcttttctttttgcttttctatacttattacatgtctaccacaaacctctttgttataatttctccagttgagtcagttttacaatttggaatgcagagatcaagtggttctataatcagcatatacttcgcacgtaccattcattcaatccacacccctttaaacccctttgacacacgtcaaactcatttacatctatgtccctccaatgacaatatagtggtcaacacatataaaacatgaatacactatatcaagacactcaggaatacatctctgggataaaatctgactgccttctattatattttaatgaataaccaaaataaagggattctttcagttacagagagcagaataattaaaatagtaactttcaaactttgtagcagcagaagtatttcttcaaataaaatcttttttgaaacccaatatagaaaacagataaaaataaagccattctagaggtgggggccttggaaagtgagtactatccactcagacttctttcttgcctctcacaaggaaggaagctactgtgtagtttgaaaattactatttaatacattctgctaaccctaaatgccatgtcagagctagaagagaaaatgtacacacattcaatctaacatttatttatttcaggttttttttttttttggcaactataaattacattcactagtacacctggaattcttcatagtgtgttcaactaaagaataagcaaacacagcatagatcagtttaaaagaaatcatggtacttcttagagcaatttgcaaaaggggaaaaaagtcttaggctcactccttggaaataaatatcaagtaaccataaaaatattcagccatttttcagttattcggggagttcaggcatggtcccacgcagagcatcagagttcctctttgaaataacccagctttgccaatgacatctcttttctcaactgcataacctcccaaaacatctgatcaacatcctgctgtttcacgagtccctgctgaatgtatcgaatgtatgtaaaaaagttacatacagaagtgattttggtcctccgcattcaactgcagaagctttcacaaaccggataggttgtaatcccactggttcaatgcttagagtattgttttccacagcctccagaacagctgaagccaactcactttttgagaatgttaaacatggaaagatatcttcctggtagattttgtctaagaaaggacacgtcctgtccattgtgggctcatccttccacaatcggaattcattatacaaggataagtcagcctctttgcagtcttttacaattggctgtatcacactgaggtcctgatgactgccactcatagcactgcttgtgcttttatttcttgtatgcccctttttaaaaggtgtctttccacctggcaaaggctcctgcgtaggtgatgttggagaactggacaatacaagtgtcttcaatgcagctacttcagcttgaagtacatcaatttttccttgtgcttcttttagctgtttttctgctgttgcctgcttgatatttgcttctctcaccattttatgagcttcctcaaatagactagctgtgagttcttccaattcctgtccaagttgatctcgcacttttgaaagcctctcacattcttcatcttttaacttcagttccctctgagcttttgcgagttcttcttttaatcgttcatagcccttttctctaacttccaaaacagatgggcttcgtaaacgagacagactatcagtactcaacccaaaaatatcatcactgccatcgcaagcctctgttatagtagcaccctgtaaaaactctctctctgcattatagttgtcctttcttgtagttaatttagttaatccagctgtgactccagaggtagagcaaggggctgggtctgtaacatgaaagctgatactagatatttccgcacaatttaaacgtctgggggatgaatacacgggttgtgtaggaagttcagaaacatctaatgcatttgcctggataggtacagaggataaagctgaagggtgtggccggtagatgacacttggtgaggtagtctgctcttgagttcctgattcatacacaccaagaaggtccggagaagtaggtgaagcaaggtttacttcatggaagccttccaagggatcattagccatagcaaaagcctcatcataagataacctgaagaacccaccgcggccgctgccggcgctcaggggcgctcacagagccgcagagagcgcgtcccgaagcagcgagaaacggaggaggacggcgagccctttccgctacactccacggcggcgggctcactacgccggcagccgccgagggaacgcgggactgcgcctgc

SEQ ID NO: 12906 - RNA, 3568 nt, Homo sapiens
  source 1..3568: mol_type = other RNA
gctgggattacaggcatgagccacaatgcctaactactgatgcacgatttctaaattaagaatttataatataccataacttatattcttttatggttatcttttatggtttttttttttcctgcttccagtttaagaagttcttcctaaagggagtaggatcaggaagataatcacattttctaaatatgtttcaatcacattttaatctataattccacatatagtttctacatcaagtcgtcatcctgttgcattaattttaaagagcatgcttctagtgtataaggttgaaaagcattcttccccttatagattactaaagatttattattaatgggtatactgattttctttagtcttactttttatttatcctttttaagtcatcaacaaactttttctgagtatttgattacctttctttcaaaccgtacagtatctcctggatttgtttctctttttatttaggtactttctccaaaagtgattttagtttgtacggaaaatcttctgaagctttgatggtacatattcttattaatgccctcacattagaataactattttcagaacataaaattgtaggttcaaagtttttttcaggttcaatttcacattcttgagctaggcatggtactgatggttttcaccataacatacaccaatgtccttttgtctgtgggctcccatccagcctggtggctgaagtcatctacaggtaagattgaccaaacctctgaacaggactgaaaaaaatgttatcttcagaaaaccagccctcttgtacactgctgctgtgaatacaaattgattaacttttctggatggcaatctagcaatgcagatcaaacatttaaaaatacatatatatctcgacacaattttatctccaggcatccacatgaaagaactccacaatgttcagaagtgtacagataaggatactcgtcacagcattataatatgaaaaataaactgaaaaccacctcatctccaaacacaattaaattatgttaaaattctataaacagggattaggatgtgtaggtttacccaagggaaaatatatttaatgtttaggtttaaaaagcaaaaaaaaagcctactttttgtttcaaaaatatgcatatgtaagtagaaaatatctgaaagctgaaaggctactatccaaaaatattaacagcagctttctctaaacagaaactaaagcagtttctcttttctttttgcttttctatacttattacatgtctaccacaaacctctttgttataatttctccagttgagtcagttttacaatttggaatgcagagatcaagtggttctataatcagcatatacttcgcacgtaccattcattcaatccacacccctttaaacccctttgacacacgtcaaactcatttacatctatgtccctccaatgacaatatagtggtcaacacatataaaacatgaatacactatatcaagacactcaggaatacatctctgggataaaatctgactgccttctattatattttaatgaataaccaaaataaagggattctttcagttacagagagcagaataattaaaatagtaactttcaaactttgtagcagcagaagtatttcttcaaataaaatcttttttgaaacccaatatagaaaacagataaaaataaagccattctagaggtgggggccttggaaagtgagtactatccactcagacttctttcttgcctctcacaaggaaggaagctactgtgtagtttgaaaattactatttaatacattctgctaaccctaaatgccatgtcagagctagaagagaaaatgtacacacattcaatctaacatttatttatttcaggttttttttttttttggcaactataaattacattcactagtacacctggaattcttcatagtgtgttcaactaaagaataagcaaacacagcatagatcagtttaaaagaaatcatggtacttcttagagcaatttgcaaaaggggaaaaaagtcttaggctcactccttggaaataaatatcaagtaaccataaaaatattcagccatttttcagttattcggggagttcaggcatggtcccacgcagagcatcagagttcctctttgaaataacccagctttgccaatgacatctcttttctcaactgcataacctcccaaaacatctgatcaacatcctgctgtttcacgagtccctgctgaatgtatcgaatgtatgtaaaaaagttacatacagaagtgattttggtcctccgcattcaactgcagaagctttcacaaaccggataggttgtaatcccactggttcaatgcttagagtattgttttccacagcctccagaacagctgaagccaactcactttttgagaatgttaaacatggaaagatatcttcctggtagattttgtctaagaaaggacacgtcctgtccattgtgggctcatccttccacaatcggaattcattatacaaggataagtcagcctctttgcagtcttttacaattggctgtatcacactgaggtcctgatgactgccactcatagcactgcttgtgcttttatttcttgtatgcccctttttaaaaggtgtctttccacctggcaaaggctcctgcgtaggtgatgttggagaactggacaatacaagtgtcttcaatgcagctacttcagcttgaagtacatcaatttttccttgtgcttcttttagctgtttttctgctgttgcctgcttgatatttgcttctctcaccattttatgagcttcctcaaatagactagctgtgagttcttccaattcctgtccaagttgatctcgcacttttgaaagcctctcacattcttcatcttttaacttcagttccctctgagcttttgcgagttcttcttttaatcgttcatagcccttttctctaacttccaaaacagatgggcttcgtaaacgagacagactatcagtactcaacccaaaaatatcatcactgccatcgcaagcctctgttatagtagcaccctgtaaaaactctctctctgcattatagttgtcctttcttgtagttaatttagttaatccagctgtgactccagaggtagagcaaggggctgggtctgtaacatgaaagctgatactagatatttccgcacaatttaaacgtctgggggatgaatacacgggttgtgtaggaagttcagaaacatctaatgcatttgcctggataggtacagaggataaagctgaagggtgtggccggtagatgacacttggtgaggtagtctgctcttgagttcctgattcatacacaccaagaaggtccggagaagtaggtgaagcaaggtttacttcatggaagccttccaagggatcattagccatagcaaaagcctcatcataagataacctgagactccgcggccatatacaccttacgacgtgtgtgtgtgtggcgggagatgggaggggaggaatcctgtagaacccagatcccatcattccagcaactgccagagcgttcgagaatgtcatgtctgtacctgtcttct

SEQ ID NO: 12907 - RNA, 3563 nt, Homo sapiens
  source 1..3563: mol_type = other RNA
gctgggattacaggcatgagccacaatgcctaactactgatgcacgatttctaaattaagaatttataatataccataacttatattcttttatggttatcttttatggtttttttttttcctgcttccagtttaagaagttcttcctaaagggagtaggatcaggaagataatcacattttctaaatatgtttcaatcacattttaatctataattccacatatagtttctacatcaagtcgtcatcctgttgcattaattttaaagagcatgcttctagtgtataaggttgaaaagcattcttccccttatagattactaaagatttattattaatgggtatactgattttctttagtcttactttttatttatcctttttaagtcatcaacaaactttttctgagtatttgattacctttctttcaaaccgtacagtatctcctggatttgtttctctttttatttaggtactttctccaaaagtgattttagtttgtacggaaaatcttctgaagctttgatggtacatattcttattaatgccctcacattagaataactattttcagaacataaaattgtaggttcaaagtttttttcaggttcaatttcacattcttgagctaggcatggtactgatggttttcaccataacatacaccaatgtccttttgtctgtgggctcccatccagcctggtggctgaagtcatctacaggtaagattgaccaaacctctgaacaggactgaaaaaaatgttatcttcagaaaaccagccctcttgtacactgctgctgtgaatacaaattgattaacttttctggatggcaatctagcaatgcagatcaaacatttaaaaatacatatatatctcgacacaattttatctccaggcatccacatgaaagaactccacaatgttcagaagtgtacagataaggatactcgtcacagcattataatatgaaaaataaactgaaaaccacctcatctccaaacacaattaaattatgttaaaattctataaacagggattaggatgtgtaggtttacccaagggaaaatatatttaatgtttaggtttaaaaagcaaaaaaaaagcctactttttgtttcaaaaatatgcatatgtaagtagaaaatatctgaaagctgaaaggctactatccaaaaatattaacagcagctttctctaaacagaaactaaagcagtttctcttttctttttgcttttctatacttattacatgtctaccacaaacctctttgttataatttctccagttgagtcagttttacaatttggaatgcagagatcaagtggttctataatcagcatatacttcgcacgtaccattcattcaatccacacccctttaaacccctttgacacacgtcaaactcatttacatctatgtccctccaatgacaatatagtggtcaacacatataaaacatgaatacactatatcaagacactcaggaatacatctctgggataaaatctgactgccttctattatattttaatgaataaccaaaataaagggattctttcagttacagagagcagaataattaaaatagtaactttcaaactttgtagcagcagaagtatttcttcaaataaaatcttttttgaaacccaatatagaaaacagataaaaataaagccattctagaggtgggggccttggaaagtgagtactatccactcagacttctttcttgcctctcacaaggaaggaagctactgtgtagtttgaaaattactatttaatacattctgctaaccctaaatgccatgtcagagctagaagagaaaatgtacacacattcaatctaacatttatttatttcaggttttttttttttttggcaactataaattacattcactagtacacctggaattcttcatagtgtgttcaactaaagaataagcaaacacagcatagatcagtttaaaagaaatcatggtacttcttagagcaatttgcaaaaggggaaaaaagtcttaggctcactccttggaaataaatatcaagtaaccataaaaatattcagccatttttcagttattcggggagttcaggcatggtcccacgcagagcatcagagttcctctttgaaataacccagctttgccaatgacatctcttttctcaactgcataacctcccaaaacatctgatcaacatcctgctgtttcacgagtccctgctgaatgtatcgaatgtatgtaaaaaagttacatacagaagtgattttggtcctccgcattcaactgcagaagctttcacaaaccggataggttgtaatcccactggttcaatgcttagagtattgttttccacagcctccagaacagctgaagccaatttttgagaatgttaaacatggaaagatatcttcctggtagattttgtctaagaaaggacacgtcctgtccattgtgggctcatccttccacaatcggaattcattatacaaggataagtcagcctctttgcagtcttttacaattggctgtatcacactgaggtcctgatgactgccactcatagcactgcttgtgcttttatttcttgtatgcccctttttaaaaggtgtctttccacctggcaaaggctcctgcgtaggtgatgttggagaactggacaatacaagtgtcttcaatgcagctacttcagcttgaagtacatcaatttttccttgtgcttcttttagctgtttttctgctgttgcctgcttgatatttgcttctctcaccattttatgagcttcctcaaatagactagctgtgagttcttccaattcctgtccaagttgatctcgcacttttgaaagcctctcacattcttcatcttttaacttcagttccctctgagcttttgcgagttcttcttttaatcgttcatagcccttttctctaacttccaaaacagatgggcttcgtaaacgagacagactatcagtactcaacccaaaaatatcatcactgccatcgcaagcctctgttatagtagcaccctgtaaaaactctctctctgcattatagttgtcctttcttgtagttaatttagttaatccagctgtgactccagaggtagagcaaggggctgggtctgtaacatgaaagctgatactagatatttccgcacaatttaaacgtctgggggatgaatacacgggttgtgtaggaagttcagaaacatctaatgcatttgcctggataggtacagaggataaagctgaagggtgtggccggtagatgacacttggtgaggtagtctgctcttgagttcctgattcatacacaccaagaaggtccggagaagtaggtgaagcaaggtttacttcatggaagccttccaagggatcattagccatagcaaaagcctcatcataagataacctgagactccgcggccatatacaccttacgacgtgtgtgtgtgtggcgggagatgggaggggaggaatcctgtagaacccagatcccatcattccagcaactgccagagcgttcgagaatgtcatgtctgtacctgtcttct

SEQ ID NO: 12908 - RNA, 8058 nt, Homo sapiens
  source 1..8058: mol_type = other RNA
gctgggattacaggcatgagccacacctagcccaatttagtgaattttaagaagcattttaaaaaaatgaaaactaaaacatagaggatatccgaggttctaaggttaagaatttctttatgaaacctgcttggaacacagttgtaaacaaatggactgatttatgatggaaggcacgtttcttgctgcagatcatggtctgaagtttgaaagccaccagcctagagggttctgaaaacttctccttcctaacacagctgaaggaaaaggggtgggtaggggcggaggcacagggacatctccaggtttggacttttccaacatgatttgcagaaggcacttgattctggaaagtagacctttggcatttcgaccctcacccacactcccacacccactctgcacagatcggtggtgcatccgaggcagggctgagttagaacaggacatcctagactcggcggcagtgactattattcagaaatggcacatcaagggccggcctgcccttcatcctgcaggggtacttgggcatgtggaggcccctttctccctggtgttgcaactggagaggagtcggttcctgaagaacagatgggagagtgctggggccaggtaccctgggagagaggagggaaatgaaatccggcacaggggctgcggggataggggcagtcaggaggcggcagtgcggtgcaagggcccccccacgcggccagctgtggaacttccaccacgactccctgtcctctcctgagcccgcccatcacgtgtagaagctcagatgctgggcgccaggagggcggcttcctggctctgggcaccgtggttctgtcctaacgaggggcgctctctgggtgtaaaaacagatgttctggctgggcgcggtggctcacgcctgtaatcccagcactttgggaggctgaggtgggtagactgcctgagctcaggagttcgagaccagcctgggcaacatggtgaaaccctgtctctactaaaatacaaaaattagacaggcatgctggccggcgcctgtagtcgcagctactcgggaggcttaggcacgagaattgcctgaacccgggaggtggaggttgtagtgagccaagatctcgccactgggctccagcctgggcgacagagactctgtctcaaaaaaaaaaaaaagagatgctctgtctggcctgggttgttgttggtggccagagtaagtggtgtgaacaagagccccggcttgggaacatgtctcagactggcattgaaaatgaaagccaggattcctctaaatccaccgccttgaagtgtaaacagtccagagagaaaccgactttgccatgctccctcacccaagaaagccctctctcaaaatgcgctagaaagtttatatctgcctgatccagagagcaagtggaaggtgcggagaagccagacagaaaaatcgaccttaaccaagagttccatctcccagccttaagttgtgggatactgaacaaacaaaactacacatgtcctgggaattttgctttgtggtgtttttaaaaagaatgtcagagccctccttgggggcttcagaaaagcaggtattgctggcccatggcttctcaagatcacagtccccaacctatgctcactgagaagatacccgcttacttccccagtctcaggcagagagttcgtggtgaagtgataagtagcaggagaggccagcagacaggaagccacggggtcaccaaggggcagggagagaaggcctggctgcggccccgtcacccgccaagcgagcccctgaaaaggctgtgggcagcccccctgccagtgaggcctagctcctgtctggtgggagcagagccgcctggatggcccagtgtcactcgatgctccatctctctccccgctaatgagctgtcacctcagtgggtgatttaactggatctttcctggtaaaacaagaggggctattgagagcggaaacacccatccgggagtcccctgagatggaaatgaccctcttaaattggggatctctggaatgtcctgattatctgcacccagtgtgcttcctggaggaaggctagcaggacagaggagcagcggagggcaggggtcctccctgaggaagttgggggaatgagaccccacctccccacgcagagcaagtcatcaaatgagaaatggagctccaaacagcactgagatttctggggctgggcgcagtagctcacacctgtaatcccagcactctgggaggctgagatgggaggatcgcttgagcccaggagtttgagaccagcctgggcaacatagcaagagctcatctctgcaaatattttttttaattaaaaaagaaaaaagatttctggaaccctttccacagtctagtctttgccactgtattcctgttatcagccctcattctctataaatggagtctgaagaacagcaaagacacagggaggagcctggaattcctactgcacagccaggatggaggagacagggatggcaagcgggagcaggtggaggcagtgaagaggagggccagaggctagatgtgcagaggttctagaaggaggggcagctggggaaggaggggcttgaccccctcagggtctcaagacagtccccaatgcccctgctttgcacggggcaatgtactcccctgggcgcctctgcacccttctgtctaccaatcatgctctgaatgttccccgggagccagttcaaggatcacctcccccaggaaaccttccctgattaacctcagcccaccacgtcacgtctcctcttgtgaacgccggagtttgggcgccatcccgtgttgtgctggttgatatgaatgtgtaactgctggaggtcttttcttaagacttctctcctggcctgaatttgaagcttctcaggagcagactccatttcttccttgtttctgcatctatccaccaatacacagagctgccggtcaaaggcatcgggacaaggcttgtcctgccctctctggggcctgactgtgggatagaaggttctggagagccagggcacgctgggcaggtggcggggccgagaagggagggaagacacgggcgaaggaaagcacaggagcgaagcgggcaaggggcacaggcgccctcatcccaggaaggcgtcgtagtccatgtaccacaccagctggccggagtgcggcaggacacccgagatgggccacttcttgggctcatggcccacccggctcaccagcgtggtgatctcacgcttcatcctgcccatgaccaggactgccaccttcttggcgcggttgatgagaggcaggctaaggctcatgcggcggtgtggctgggaggggctcgtggtcagcacgaccagctgctcgccatccaggccagtgggtgactgtgggaagagggaggctgtgtgcccgtcggcacccatgcccagcagcaccaggtcgaagctgctgttggccaccagggctgagatctccctggcatagatctgggcgccctggtcctcctcggcgcagagccgctgctgcaggtgcacaggcatggggtggatgttgtagtaggggatccggacgtgctgcagcaggtgggcctgcaggccctggaagttggactccgggtctgagagtgggacgcagcgctcgtcaaccagccacaggtgcgtgtgggcccaggggaagccatagtgcgccgtggccagctgctggaacagggccacggggctcgagccccccgacagtgccaggtggaactggccaaagcgccgcacggctcgcacagcggtggcctcgatgtcattagccagcttagagatcagctcctcggaccaggcggagaccagcgggctctctcggtacttggccctgaggacctggaagtcactgggcattggggccggccctggccctggcaccagctgctccggctgctgctgggaaaagaacaaccggccgctactgaactcaaagtccaacagacggccattctcagctcctccagggtagaggcgtggggccttatgggccaggctctccagcagaggggtccagaagttccaggaggccagcaagttctctgtggtgatgaagaaattcttccggccatggaagatatgggataagaggacggagtgggcgtcccgctcccgcacagggctgtaggcgtagtaatcggacagagggctgccgaaaaggcggagcccaggtggtccctccatttccttccagctggagggcagggagggcctgaacaggttcctgctgaccagcacggcagggctgcccaggtcgccatggccgatgtggaagacgagctgccggggcaggcactggctctgcgccgcggcccagtgcttttcgctctgcacacagcaggcctggttcttgaacaagatccgagcgtagcccactctctcgtccaaggctttgccagacatcaggatgaaaggcacgccctcccagcgaaggttgtcaatgtgcactaggacggctgcgaaggtcggcgtcaggctgtggaagctgtctggcttctgcagctctctgcgcacctgctcactgtaagactggtactggcccacgacggcactgcccctctgcaggccccgcagcgcctggaagacctgaagcttgtgccgcagcacagcctccgcactgctgacattgtggggcagctccatggccacgagggtgaggacctccgtcagatggttctggaggacgtcgcgaatgacaccgtactcctcatagaagctggtgcggccttcagcatccacggtctctttcatgatgatctccacccgctccacatggtgccggttccagaggccgtccaaagccttgcggttctggtctcggaaaggcaggatctgcgccacagcctgcttgcctaagtaatggtccacccggtacatctcctcctcctggaaaaaggtcccgagttctgtggccagctgctgggctgagaagtggtcatggccaaagggtttctcaaggacaacccgcagccaggcgcccgggcctggccggcagctactgttgatgttgcgggcaatgtcttcataggcgaagggtggcactgagaagtagaagatcctgccagcctcccggaggcctgcgtgctggagctgtgcctcgatgtccttgttcagggcctgatagtcctcggccgtcttcagttggcggtactggctcagctgcaggaactgatccttgtgctctgcacagtgactgggtgccatgtccttggggcaggagagggattccagggccttggccatgagctcttgaccctgcttgggggctgtcagagcagctccatggaagctaaaactgtgacccctccccgcttcatccaggtacagctggaacagtccctgccataagtacttcttagccaggtccccagttgctcccagcaggattatggagacatgtccctggagctcctgggcttgcaggcagcccagaagggccaagcacatcgccactatgagcatattccacatgccagttaaaaggctctgctaacatcccagaaggtgggggccagggggtttggatcagaatccaggttccggcctttgttctcacacaagcggaagaggcgtgcagctgtccccatacagacccggcacagcagacccagcctgtgctgaagctctagccgcagagcgttttctggtaaaccacaggaggaagcagttctaatcctctatgcccagcagacaaggggtgggagagaggagcgggaggtaaaggtcaatgtctgctgctgccctgttccctttcccagcttttgacgttaccttctgtgcgccaggcaggaggaagggaaattttcttcaaatcatgacccatgagtttggaattttttaaaaagaacatgtgggagtaaaacaaaagttcaaactaaagatcatttgaaactaaagcacaaggtgatgtgcctagtctttttacaatagccaacccaaggtttttgtttttgttgttttttgtctgttttttgcaatcttcctgttctggtccatttatgctgaacccatcaatgcagataaaaatcaagcctgctatcaatgacctctgatctgcattcactgccctaagggccagaatggggacaaaagcttccagatcgggctctggggtccttgttcctctctcatctcagagaatcctcatcccatctttaggcacctgtcctgtaatcccagcactttgggagactgagacgggaggactacttgagcccaggagattgagaccagcctgggcaacatggcaaaaacccgtttctactaaaaatacaaaagttagctgggtgtggtggcgggtgcctgtaatcccagctacttgggaggctgaggcagaataattgcttgaacccaggaggcggaggctgcagtgagcagagattgcaccactgcactccagcctgggtgacagagtgagactctgtctcaaaaaaaaaaaccattaaattaaaaagaaaggtaataaatactcaaaactcattacttcctaatcatctgactacatttcactaatatctatgctcttgatattatttatatccactgcatctatgaggtgaagatattctattatagtgtatttgaagttggccaacgtcagaatatttacaccacagatataggcaaaggctataaatcaggttccccactaccaaccccacccctcacagagtcagttggtaaacattaccagcacacaactgcctatccgtccaagtctttatttacagcccgaacttcccctaaactccagactcatgcagtcaattgctattctgagagcatgagtgggatgtttgccagacttaatatgtacaaaactgaactgatttctctcccaatctgcttccaatgtagctttccccattatcagtaaatgacaactctatctttccaggtgttcagacccagaaaccttgaggtcatcgtatctgtcagcaaatcctgtagtttctatcttcaaaatttatctagaatacaactgcttctcaccaccttccaccactccactccagtgccagccaccgtcatctccgtctggattactacaggaacttcctaattggcctcctctgtctacctggaccctctatggctgagcctcaacacggcagtcagagtgacctttttatagctccagctggatcatgccattcctctgtgcagatgtctgcagagtctacacattctggcctcccacccattacctctttgatctcttctcttaccatcctgcctgtctaggctctggccgcccagcctcctgcctcagggcctttgcacttgttctctccgcctggccaactcccccatgtcccccaccaggtccacgtggtttactccctcactaatttttctttgctaaaatgtcatcttctcagtgaggcttactcagaccactctaaaattgtaaaccgcccacccccatcctcctctcctgctttatttctccccacagtacatcgctttctaatatactgtatgataattacattcattttgcctattgtctgccattccttttcccaagagtgtgcgtgccaatgaggacagggacttttgtttgttttgttctccgcagtacctccagtatccaaaacaaggcctggcatacagaaggcgctctataaatatctgctaaatgaacaaataaatcccatttgcacaggaccactgtcatttctgcatttgaaatacggcacaaaggaatatacctctaatggtgacttcaagcactgtgacacagcacacagcagcagcttactacttggaacaacacttttaataataaaagagctatttatggagtatttaactatatgccaaatgctaggctatcggtgtgacatgcatcacaccatttaaatcttgccacaaccatatgaggtaggtaacatgattatccccatcttagcagggagtagagaggaaactaaggcaaagagaagtcaaataacatggccaggcgcagtggcttacgcctataatcccagcactttgggaggctgaggcaggaggatcattgga

SEQ ID NO: 12909 - RNA, 8451 nt, Homo sapiens
  source 1..8451: mol_type = other RNA
gctgggattacaggcatgagccacacctagcccaatttagtgaattttaagaagcattttaaaaaaatgaaaactaaaacatagaggatatccgaggttctaaggttaagaatttctttatgaaacctgcttggaacacagttgtaaacaaatggactgatttatgatggaaggcacgtttcttgctgcagatcatggtctgaagtttgaaagccaccagcctagagggttctgaaaacttctccttcctaacacagctgaaggaaaaggggtgggtaggggcggaggcacagggacatctccaggtttggacttttccaacatgatttgcagaaggcacttgattctggaaagtagacctttggcatttcgaccctcacccacactcccacacccactctgcacagatcggtggtgcatccgaggcagggctgagttagaacaggacatcctagactcggcggcagtgactattattcagaaatggcacatcaagggccggcctgcccttcatcctgcaggggtacttgggcatgtggaggcccctttctccctggtgttgcaactggagaggagtcggttcctgaagaacagatgggagagtgctggggccaggtaccctgggagagaggagggaaatgaaatccggcacaggggctgcggggataggggcagtcaggaggcggcagtgcggtgcaagggcccccccacgcggccagctgtggaacttccaccacgactccctgtcctctcctgagcccgcccatcacgtgtagaagctcagatgctgggcgccaggagggcggcttcctggctctgggcaccgtggttctgtcctaacgaggggcgctctctgggtgtaaaaacagatgttctggctgggcgcggtggctcacgcctgtaatcccagcactttgggaggctgaggtgggtagactgcctgagctcaggagttcgagaccagcctgggcaacatggtgaaaccctgtctctactaaaatacaaaaattagacaggcatgctggccggcgcctgtagtcgcagctactcgggaggcttaggcacgagaattgcctgaacccgggaggtggaggttgtagtgagccaagatctcgccactgggctccagcctgggcgacagagactctgtctcaaaaaaaaaaaaaagagatgctctgtctggcctgggttgttgttggtggccagagtaagtggtgtgaacaagagccccggcttgggaacatgtctcagactggcattgaaaatgaaagccaggattcctctaaatccaccgccttgaagtgtaaacagtccagagagaaaccgactttgccatgctccctcacccaagaaagccctctctcaaaatgcgctagaaagtttatatctgcctgatccagagagcaagtggaaggtgcggagaagccagacagaaaaatcgaccttaaccaagagttccatctcccagccttaagttgtgggatactgaacaaacaaaactacacatgtcctgggaattttgctttgtggtgtttttaaaaagaatgtcagagccctccttgggggcttcagaaaagcaggtattgctggcccatggcttctcaagatcacagtccccaacctatgctcactgagaagatacccgcttacttccccagtctcaggcagagagttcgtggtgaagtgataagtagcaggagaggccagcagacaggaagccacggggtcaccaaggggcagggagagaaggcctggctgcggccccgtcacccgccaagcgagcccctgaaaaggctgtgggcagcccccctgccagtgaggcctagctcctgtctggtgggagcagagccgcctggatggcccagtgtcactcgatgctccatctctctccccgctaatgagctgtcacctcagtgggtgatttaactggatctttcctggtaaaacaagaggggctattgagagcggaaacacccatccgggagtcccctgagatggaaatgaccctcttaaattggggatctctggaatgtcctgattatctgcacccagtgtgcttcctggaggaaggctagcaggacagaggagcagcggagggcaggggtcctccctgaggaagttgggggaatgagaccccacctccccacgcagagcaagtcatcaaatgagaaatggagctccaaacagcactgagatttctggggctgggcgcagtagctcacacctgtaatcccagcactctgggaggctgagatgggaggatcgcttgagcccaggagtttgagaccagcctgggcaacatagcaagagctcatctctgcaaatattttttttaattaaaaaagaaaaaagatttctggaaccctttccacagtctagtctttgccactgtattcctgttatcagccctcattctctataaatggagtctgaagaacagcaaagacacagggaggagcctggaattcctactgcacagccaggatggaggagacagggatggcaagcgggagcaggtggaggcagtgaagaggagggccagaggctagatgtgcagaggttctagaaggaggggcagctggggaaggaggggcttgaccccctcagggtctcaagacagtccccaatgcccctgctttgcacggggcaatgtactcccctgggcgcctctgcacccttctgtctaccaatcatgctctgaatgttccccgggagccagttcaaggatcacctcccccaggaaaccttccctgattaacctcagcccaccacgtcacgtctcctcttgtgaacgccggagtttgggcgccatcccgtgttgtgctggttgatatgaatgtgtaactgctggaggtcttttcttaagacttctctcctggcctgaatttgaagcttctcaggagcagactccatttcttccttgtttctgcatctatccaccaatacacagagctgccggtcaaaggcatcgggacaaggcttgtcctgccctctctggggcctgactgtgggatagaaggttctggagagccagggcacgctgggcaggtggcggggccgagaagggagggaagacacgggcgaaggaaagcacaggagcgaagcgggcaaggggcacaggcgccctcatcccaggaaggcgtcgtagtccatgtaccacaccagctggccggagtgcggcaggacacccgagatgggccacttcttgggctcatggcccacccggctcaccagcgtggtgatctcacgcttcatcctgcccatgaccaggactgccaccttcttggcgcggttgatgagaggcaggctaaggctcatgcggcggtgtggctgggaggggctcgtggtcagcacgaccagctgctcgccatccaggccagtgggtgactgtgggaagagggaggctgtgtgcccgtcggcacccatgcccagcagcaccaggtcgaagctgctgttggccaccagggctgagatctccctggcatagatctgggcgccctggtcctcctcggcgcagagccgctgctgcaggtgcacaggcatggggtggatgttgtagtaggggatccggacgtgctgcagcaggtgggcctgcaggccctggaagttggactccgggtctgagagtgggacgcagcgctcgtcaaccagccacaggtgcgtgtgggcccaggggaagccatagtgcgccgtggccagctgctggaacagggccacggggctcgagccccccgacagtgccaggtggaactggccaaagcgccgcacggctcgcacagcggtggcctcgatgtcattagccagcttagagatcagctcctcggaccaggcggagaccagcgggctctctcggtacttggccctgaggacctggaagtcactgggcattggggccggccctggccctggcaccagctgctccggctgctgctgggaaaagaacaaccggccgctactgaactcaaagtccaacagacggccattctcagctcctccagggtagaggcgtggggccttatgggccaggctctccagcagaggggtccagaagttccaggaggccagcaagttctctgtggtgatgaagaaattcttccggccatggaagatatgggataagaggacggagtgggcgtcccgctcccgcacagggctgtaggcgtagtaatcggacagagggctgccgaaaaggcggagcccaggtggtccctccatttccttccagctggagggcagggagggcctgaacaggttcctgctgaccagcacggcagggctgcccaggtcgccatggccgatgtggaagacgagctgccggggcaggcactggctctgcgccgcggcccagtgcttttcgctctgcacacagcaggcctggttcttgaacaagatccgagcgtagcccactctctcgtccaaggctttgccagacatcaggatgaaaggcacgccctcccagcgaaggttgtcaatgtgcactaggacggctgcgaaggtcggcgtcaggctgtggaagctgtctggcttctgcagctctctgcgcacctgctcactgtaagactggtactggcccacgacggcactgcccctctgcaggccccgcagcgcctggaagacctgaagcttgtgccgcagcacagcctccgcactgctgacattgtggggcagctccatggccacgagggtgaggacctccgtcagatggttctggaggacgtcgcgaatgacaccgtactcctcatagaagctggtgcggccttcagcatccacggtctctttcatgatgatctccacccgctccacatggtgccggttccagaggccgtccaaagccttgcggttctggtctcggaaaggcaggatctgcgccacagcctgcttgcctaagtaatggtccacccggtacatctcctcctcctggaaaaaggtcccgagttctgtggccagctgctgggctgagaagtggtcatggccaaagggtttctcaaggacaacccgcagccaggcgcccgggcctggccggcagctactgttgatgttgcgggcaatgtcttcataggcgaagggtggcactgagaagtagaagatcctgccagcctcccggaggcctgcgtgctggagctgtgcctcgatgtccttgttcagggcctgatagtcctcggccgtcttcagttggcggtactggctcagctgcaggaactgatccttgtgctctgcacagtgactgggtgccatgtccttggggcaggagagggattccagggccttggccatgagctcttgaccctgcttgggggctgtcagagcagctccatggaagctaaaactgtgacccctccccgcttcatccaggtacagctggaacagtccctgccataagtacttcttagccaggtccccagttgctcccagcaggattatggagacatgtccctggagctcctgggcttgcaggcagcccagaagggccaagcacatcgccactatgagcatattccacatgcctgggtgcacggaccacaggaccattctgctttttcctcctgctttccagtccctgtccttggcccttcaagcgttttttcctcaaccggcaatcgctcgtctggagagaaggagaagctgcaaggtcagtgcaggagagaggcagcaagaaatctgaagcccagagaacagcctggagaaggaggagccgccagctggcaggctgcgcttcagagctgctgatcggatcctggtagccagggctctggacgtgcctggtacaaagggaggagctaagcctccagagtcctggcatgggcaggtgggggagccccaagggccagcacctctgcccccaccccagaagactgcagacagctgtgacggatggccacctggcctgaactgactcctggccctctctttaatcctgttctgactctgaggtttgccacagtcctccctgaccagtcctgttgtgggtccccggttctgaggttggcctcccttatctgttatgttgccagcactcctttaaacaaatccaagatattgggtattacaacatgattgcttactctgtggttgcaaaacaactaaaaaacaactctttcctaaatgggtgggggtagtatgtgtgggtatttttttttttatgtttttttaacctttacagtgtttctcaaactttaatgagcatttgaatttcctggggatctttttaaaaggacattctgatgcagaaggaagaggacctgaagtgctgacagctggtccaagagcacactttgagtagtgagactccggaatactgagcagcgagcaccagagcagcagttctcatcaaaggagggcatcagaacaaacacgcggtcctcgcctcctgctccctttctcaagacagagacattctgatccagtaggtgtagggtgggtcctaacacaggtgtttcgaaacagtctcaaatggtttcatgcgcccatccccttgtaaaaactggttgttcctgaatccaataataatacctatgttaaccaagtagtcggcgtgtgccagatgacttaaacgcacctttccaatcattcctcacaacagtcttgtggaggaggttctgtgaggagtctcattctacagacgaggaaactgggaggtgaaggaaactgtcaagccacaaagcctggaccctcagtcacgatgctaaacagcttcctttgtcaagcagaagaaggaagcattggggtccaaggacctgggctcaagaccactgcctaacttcgtgatctaattaagtcagctaattaggccaggcacagtggctcatgcctataatcccggcactctgggaggccaaggcaggaggatcacttgagcccaggacttccagaccagcctgggcaacacagcgagacccccatctctacaaaaaatatttaaaaactagctgggcgtggtggcacatgtctgtagtctcagctactcaggaggctgaggactgcttgagcccgagaggtccaggctgcagtgagccatgatcgcaccactgcactccagcctggtgacagagcaagatcctgtctcaaaaaaagtaaataaataaaataaataaataaatcagctaattaaatcagggagatgccctccacctttccataagggtgggtaggtgattagagccttagcatccacatttcttcatctacaaaacagggcaaataccatcaacccaaggtgggggtggggggaggggcagtgaagactgagatgatacatttgacaaaaatgctatacaaatgttaattaattaattaaatgcaaagttcctcctggcccccaagggtagtataccattgctctcaggaaaaacattgtgaacctccctcctctcctggggctacagagccaggccctgcagacagcactggagaaccaaccctggttcctaactcaacactcccgactagtctggaagcagcaggaggaaggctggcttggtcatcctccctgctgccctgacagggaaagaagcaggcccagagaagcccagttaagtcaaagtcagggacagggggaccccagcctctggagcagaggcacccacggctccaacacatctcctgggctccaagcctcctcctcatgctgcacggctctgcttcagaaggttttcttctgaagcacttctcccctctgcctccttgcctgctctgagaggaatgggctgtgaaataaaccttccgaaattacatacttgaagttagccaaagagcatggaagtagccttccaaaagcttatccaactacgaatcacttctgctcaaaaaattaacaaatcaatgagaaaatctttagtgaaaagtttgagcagctgtaaggggagggggcattacactgggaacccgaatgtgtggtggctcttgcctgcgccctgcctctaaacaaccacataaccttaaacaagtcatttagcctggctgggcctcagtttcctcatcgaggaaatgggagggtgagataaaggatctgtgtgatcttttagtgtccctaagtcctgttttccgaggaaaggtgatccgcaccctattatccgggaactgccctccacttttctataaggcaaatgagtgcttcgagccttgacctctgcagccaggcagggaaacagagaactaaaatatgaagccaagagctgagaactgtgcgtcattcagcagttaagacaaaaactcttgaagctatgacttacgtgtgtggaggatgcaatttcatttacaattcttatttaagatacttgccagaaatacactcactacgaaacaaaatgctgtgggggcatcctgtagggaggtggaaaaggccttcttctgatggctcatcttagagccagggcggactgcaggcacgtgaacccagtcctgggcacccttcactgtctccaactctaatcctgagaggctcctacgagtcat

SEQ ID NO: 12910 - RNA, 5684 nt, Homo sapiens
  source 1..5684: mol_type = other RNA
gctgggattacaggcatgagccacacctagcccaatttagtgaattttaagaagcattttaaaaaaatgaaaactaaaacatagaggatatccgaggttctaaggttaagaatttctttatgaaacctgcttggaacacagttgtaaacaaatggactgatttatgatggaaggcacgtttcttgctgcagatcatggtctgaagtttgaaagccaccagcctagagggttctgaaaacttctccttcctaacacagctgaaggaaaaggggtgggtaggggcggaggcacagggacatctccaggtttggacttttccaacatgatttgcagaaggcacttgattctggaaagtagacctttggcatttcgaccctcacccacactcccacacccactctgcacagatcggtggtgcatccgaggcagggctgagttagaacaggacatcctagactcggcggcagtgactattattcagaaatggcacatcaagggccggcctgcccttcatcctgcaggggtacttgggcatgtggaggcccctttctccctggtgttgcaactggagaggagtcggttcctgaagaacagatgggagagtgctggggccaggtaccctgggagagaggagggaaatgaaatccggcacaggggctgcggggataggggcagtcaggaggcggcagtgcggtgcaagggcccccccacgcggccagctgtggaacttccaccacgactccctgtcctctcctgagcccgcccatcacgtgtagaagctcagatgctgggcgccaggagggcggcttcctggctctgggcaccgtggttctgtcctaacgaggggcgctctctgggtgtaaaaacagatgttctggctgggcgcggtggctcacgcctgtaatcccagcactttgggaggctgaggtgggtagactgcctgagctcaggagttcgagaccagcctgggcaacatggtgaaaccctgtctctactaaaatacaaaaattagacaggcatgctggccggcgcctgtagtcgcagctactcgggaggcttaggcacgagaattgcctgaacccgggaggtggaggttgtagtgagccaagatctcgccactgggctccagcctgggcgacagagactctgtctcaaaaaaaaaaaaaagagatgctctgtctggcctgggttgttgttggtggccagagtaagtggtgtgaacaagagccccggcttgggaacatgtctcagactggcattgaaaatgaaagccaggattcctctaaatccaccgccttgaagtgtaaacagtccagagagaaaccgactttgccatgctccctcacccaagaaagccctctctcaaaatgcgctagaaagtttatatctgcctgatccagagagcaagtggaaggtgcggagaagccagacagaaaaatcgaccttaaccaagagttccatctcccagccttaagttgtgggatactgaacaaacaaaactacacatgtcctgggaattttgctttgtggtgtttttaaaaagaatgtcagagccctccttgggggcttcagaaaagcaggtattgctggcccatggcttctcaagatcacagtccccaacctatgctcactgagaagatacccgcttacttccccagtctcaggcagagagttcgtggtgaagtgataagtagcaggagaggccagcagacaggaagccacggggtcaccaaggggcagggagagaaggcctggctgcggccccgtcacccgccaagcgagcccctgaaaaggctgtgggcagcccccctgccagtgaggcctagctcctgtctggtgggagcagagccgcctggatggcccagtgtcactcgatgctccatctctctccccgctaatgagctgtcacctcagtgggtgatttaactggatctttcctggtaaaacaagaggggctattgagagcggaaacacccatccgggagtcccctgagatggaaatgaccctcttaaattggggatctctggaatgtcctgattatctgcacccagtgtgcttcctggaggaaggctagcaggacagaggagcagcggagggcaggggtcctccctgaggaagttgggggaatgagaccccacctccccacgcagagcaagtcatcaaatgagaaatggagctccaaacagcactgagatttctggggctgggcgcagtagctcacacctgtaatcccagcactctgggaggctgagatgggaggatcgcttgagcccaggagtttgagaccagcctgggcaacatagcaagagctcatctctgcaaatattttttttaattaaaaaagaaaaaagatttctggaaccctttccacagtctagtctttgccactgtattcctgttatcagccctcattctctataaatggagtctgaagaacagcaaagacacagggaggagcctggaattcctactgcacagccaggatggaggagacagggatggcaagcgggagcaggtggaggcagtgaagaggagggccagaggctagatgtgcagaggttctagaaggaggggcagctggggaaggaggggcttgaccccctcagggtctcaagacagtccccaatgcccctgctttgcacggggcaatgtactcccctgggcgcctctgcacccttctgtctaccaatcatgctctgaatgttccccgggagccagttcaaggatcacctcccccaggaaaccttccctgattaacctcagcccaccacgtcacgtctcctcttgtgaacgccggagtttgggcgccatcccgtgttgtgctggttgatatgaatgtgtaactgctggaggtcttttcttaagacttctctcctggcctgaatttgaagcttctcaggagcagactccatttcttccttgtttctgcatctatccaccaatacacagagctgccggtcaaaggcatcgggacaaggcttgtcctgccctctctggggcctgactgtgggatagaaggttctggagagccagggcacgctgggcaggtggcggggccgagaagggagggaagacacgggcgaaggaaagcacaggagcgaagcgggcaaggggcacaggcgccctcatcccaggaaggcgtcgtagtccatgtaccacaccagctggccggagtgcggcaggacacccgagatgggccacttcttgggctcatggcccacccggctcaccagcgtggtgatctcacgcttcatcctgcccatgaccaggactgccaccttcttggcgcggttgatgagaggcaggctaaggctcatgcggcggtgtggctgggaggggctcgtggtcagcacgaccagctgctcgccatccaggccagtgggtgactgtgggaagagggaggctgtgtgcccgtcggcacccatgcccagcagcaccaggtcgaagctgctgttggccaccagggctgagatctccctggcatagatctgggcgccctggtcctcctcggcgcagagccgctgctgcaggtgcacaggcatggggtggatgttgtagtaggggatccggacgtgctgcagcaggtgggcctgcaggccctggaagttggactccgggtctgagagtgggacgcagcgctcgtcaaccagccacaggtgcgtgtgggcccaggggaagccatagtgcgccgtggccagctgctggaacagggccacggggctcgagccccccgacagtgccaggtggaactggccaaagcgccgcacggctcgcacagcggtggcctcgatgtcattagccagcttagagatcagctcctcggaccaggcggagaccagcgggctctctcggtacttggccctgaggacctggaagtcactgggcattggggccggccctggccctggcaccagctgctccggctgctgctgggaaaagaacaaccggccgctactgaactcaaagtccaacagacggccattctcagctcctccagggtagaggcgtggggccttatgggccaggctctccagcagaggggtccagaagttccaggaggccagcaagttctctgtggtgatgaagaaattcttccggccatggaagatatgggataagaggacggagtgggcgtcccgctcccgcacagggctgtaggcgtagtaatcggacagagggctgccgaaaaggcggagcccaggtggtccctccatttccttccagctggagggcagggagggcctgaacaggttcctgctgaccagcacggcagggctgcccaggtcgccatggccgatgtggaagacgagctgccggggcaggcactggctctgcgccgcggcccagtgcttttcgctctgcacacagcaggcctggttcttgaacaagatccgagcgtagcccactctctcgtccaaggctttgccagacatcaggatgaaaggcacgccctcccagcgaaggttgtcaatgtgcactaggacggctgcgaaggtcggcgtcaggctgtggaagctgtctggcttctgcagctctctgcgcacctgctcactgtaagactggtactggcccacgacggcactgcccctctgcaggccccgcagcgcctggaagacctgaagcttgtgccgcagcacagcctccgcactgctgacattgtggggcagctccatggccacgagggtgaggacctccgtcagatggttctggaggacgtcgcgaatgacaccgtactcctcatagaagctggtgcggccttcagcatccacggtctctttcatgatgatctccacccgctccacatggtgccggttccagaggccgtccaaagccttgcggttctggtctcggaaaggcaggatctgcgccacagcctgcttgcctaagtaatggtccacccggtacatctcctcctcctggaaaaaggtcccgagttctgtggccagctgctgggctgagaagtggtcatggccaaagggtttctcaaggacaacccgcagccaggcgcccgggcctggccggcagctactgttgatgttgcgggcaatgtcttcataggcgaagggtggcactgagaagtagaagatcctgccagcctcccggaggcctgcgtgctggagctgtgcctcgatgtccttgttcagggcctgatagtcctcggccgtcttcagttggcggtactggctcagctgcaggaactgatccttgtgctctgcacagtgactgggtgccatgtccttggggcaggagagggattccagggccttggccatgagctcttgaccctgcttgggggctgtcagagcagctccatggaagctaaaactgtgacccctccccgcttcatccaggtacagctggaacagtccctgccataagtacttcttagccaggtccccagttgctcccagcaggattatggagacatgtccctggagctcctgggcttgcaggcagcccagaagggccaagcacatcgccactatgagcatattccacatgcctgggtgccagttaaaaggctctgctaacatcccagaaggtgggggccagggggtttggatcagaatccaggttccggcctttgttctcacacaagcggaagaggcgtgcagctgtccccatacagacccggcacagcagacccagcctgtgctgaagctctagccgcagagcgttttct

SEQ ID NO: 12911 - RNA, 5805 nt, Homo sapiens
  source 1..5805: mol_type = other RNA
gctgggattacaggcatgagccacacctagcccaatttagtgaattttaagaagcattttaaaaaaatgaaaactaaaacatagaggatatccgaggttctaaggttaagaatttctttatgaaacctgcttggaacacagttgtaaacaaatggactgatttatgatggaaggcacgtttcttgctgcagatcatggtctgaagtttgaaagccaccagcctagagggttctgaaaacttctccttcctaacacagctgaaggaaaaggggtgggtaggggcggaggcacagggacatctccaggtttggacttttccaacatgatttgcagaaggcacttgattctggaaagtagacctttggcatttcgaccctcacccacactcccacacccactctgcacagatcggtggtgcatccgaggcagggctgagttagaacaggacatcctagactcggcggcagtgactattattcagaaatggcacatcaagggccggcctgcccttcatcctgcaggggtacttgggcatgtggaggcccctttctccctggtgttgcaactggagaggagtcggttcctgaagaacagatgggagagtgctggggccaggtaccctgggagagaggagggaaatgaaatccggcacaggggctgcggggataggggcagtcaggaggcggcagtgcggtgcaagggcccccccacgcggccagctgtggaacttccaccacgactccctgtcctctcctgagcccgcccatcacgtgtagaagctcagatgctgggcgccaggagggcggcttcctggctctgggcaccgtggttctgtcctaacgaggggcgctctctgggtgtaaaaacagatgttctggctgggcgcggtggctcacgcctgtaatcccagcactttgggaggctgaggtgggtagactgcctgagctcaggagttcgagaccagcctgggcaacatggtgaaaccctgtctctactaaaatacaaaaattagacaggcatgctggccggcgcctgtagtcgcagctactcgggaggcttaggcacgagaattgcctgaacccgggaggtggaggttgtagtgagccaagatctcgccactgggctccagcctgggcgacagagactctgtctcaaaaaaaaaaaaaagagatgctctgtctggcctgggttgttgttggtggccagagtaagtggtgtgaacaagagccccggcttgggaacatgtctcagactggcattgaaaatgaaagccaggattcctctaaatccaccgccttgaagtgtaaacagtccagagagaaaccgactttgccatgctccctcacccaagaaagccctctctcaaaatgcgctagaaagtttatatctgcctgatccagagagcaagtggaaggtgcggagaagccagacagaaaaatcgaccttaaccaagagttccatctcccagccttaagttgtgggatactgaacaaacaaaactacacatgtcctgggaattttgctttgtggtgtttttaaaaagaatgtcagagccctccttgggggcttcagaaaagcaggtattgctggcccatggcttctcaagatcacagtccccaacctatgctcactgagaagatacccgcttacttccccagtctcaggcagagagttcgtggtgaagtgataagtagcaggagaggccagcagacaggaagccacggggtcaccaaggggcagggagagaaggcctggctgcggccccgtcacccgccaagcgagcccctgaaaaggctgtgggcagcccccctgccagtgaggcctagctcctgtctggtgggagcagagccgcctggatggcccagtgtcactcgatgctccatctctctccccgctaatgagctgtcacctcagtgggtgatttaactggatctttcctggtaaaacaagaggggctattgagagcggaaacacccatccgggagtcccctgagatggaaatgaccctcttaaattggggatctctggaatgtcctgattatctgcacccagtgtgcttcctggaggaaggctagcaggacagaggagcagcggagggcaggggtcctccctgaggaagttgggggaatgagaccccacctccccacgcagagcaagtcatcaaatgagaaatggagctccaaacagcactgagatttctggggctgggcgcagtagctcacacctgtaatcccagcactctgggaggctgagatgggaggatcgcttgagcccaggagtttgagaccagcctgggcaacatagcaagagctcatctctgcaaatattttttttaattaaaaaagaaaaaagatttctggaaccctttccacagtctagtctttgccactgtattcctgttatcagccctcattctctataaatggagtctgaagaacagcaaagacacagggaggagcctggaattcctactgcacagccaggatggaggagacagggatggcaagcgggagcaggtggaggcagtgaagaggagggccagaggctagatgtgcagaggttctagaaggaggggcagctggggaaggaggggcttgaccccctcagggtctcaagacagtccccaatgcccctgctttgcacggggcaatgtactcccctgggcgcctctgcacccttctgtctaccaatcatgctctgaatgttccccgggagccagttcaaggatcacctcccccaggaaaccttccctgattaacctcagcccaccacgtcacgtctcctcttgtgaacgccggagtttgggcgccatcccgtgttgtgctggttgatatgaatgtgtaactgctggaggtcttttcttaagacttctctcctggcctgaatttgaagcttctcaggagcagactccatttcttccttgtttctgcatctatccaccaatacacagagctgccggtcaaaggcatcgggacaaggcttgtcctgccctctctggggcctgactgtgggatagaaggttctggagagccagggcacgctgggcaggtggcggggccgagaagggagggaagacacgggcgaaggaaagcacaggagcgaagcgggcaaggggcacaggcgccctcatcccaggaaggcgtcgtagtccatgtaccacaccagctggccggagtgcggcaggacacccgagatgggccacttcttgggctcatggcccacccggctcaccagcgtggtgatctcacgcttcatcctgcccatgaccaggactgccaccttcttggcgcggttgatgagaggcaggctaaggctcatgcggcggtgtggctgggaggggctcgtggtcagcacgaccagctgctcgccatccaggccagtgggtgactgtgggaagagggaggctgtgtgcccgtcggcacccatgcccagcagcaccaggtcgaagctgctgttggccaccagggctgagatctccctggcatagatctgggcgccctggtcctcctcggcgcagagccgctgctgcaggtgcacaggcatggggtggatgttgtagtaggggatccggacgtgctgcagcaggtgggcctgcaggccctggaagttggactccgggtctgagagtgggacgcagcgctcgtcaaccagccacaggtgcgtgtgggcccaggggaagccatagtgcgccgtggccagctgctggaacagggccacggggctcgagccccccgacagtgccaggtggaactggccaaagcgccgcacggctcgcacagcggtggcctcgatgtcattagccagcttagagatcagctcctcggaccaggcggagaccagcgggctctctcggtacttggccctgaggacctggaagtcactgggcattggggccggccctggccctggcaccagctgctccggctgctgctgggaaaagaacaaccggccgctactgaactcaaagtccaacagacggccattctcagctcctccagggtagaggcgtggggccttatgggccaggctctccagcagaggggtccagaagttccaggaggccagcaagttctctgtggtgatgaagaaattcttccggccatggaagatatgggataagaggacggagtgggcgtcccgctcccgcacagggctgtaggcgtagtaatcggacagagggctgccgaaaaggcggagcccaggtggtccctccatttccttccagctggagggcagggagggcctgaacaggttcctgctgaccagcacggcagggctgcccaggtcgccatggccgatgtggaagacgagctgccggggcaggcactggctctgcgccgcggcccagtgcttttcgctctgcacacagcaggcctggttcttgaacaagatccgagcgtagcccactctctcgtccaaggctttgccagacatcaggatgaaaggcacgccctcccagcgaaggttgtcaatgtgcactaggacggctgcgaaggtcggcgtcaggctgtggaagctgtctggcttctgcagctctctgcgcacctgctcactgtaagactggtactggcccacgacggcactgcccctctgcaggccccgcagcgcctggaagacctgaagcttgtgccgcagcacagcctccgcactgctgacattgtggggcagctccatggccacgagggtgaggacctccgtcagatggttctggaggacgtcgcgaatgacaccgtactcctcatagaagctggtgcggccttcagcatccacggtctctttcatgatgatctccacccgctccacatggtgccggttccagaggccgtccaaagccttgcggttctggtctcggaaaggcaggatctgcgccacagcctgcttgcctaagtaatggtccacccggtacatctcctcctcctggaaaaaggtcccgagttctgtggccagctgctgggctgagaagtggtcatggccaaagggtttctcaaggacaacccgcagccaggcgcccgggcctggccggcagctactgttgatgttgcgggcaatgtcttcataggcgaagggtggcactgagaagtagaagatcctgccagcctcccggaggcctgcgtgctggagctgtgcctcgatgtccttgttcagggcctgatagtcctcggccgtcttcagttggcggtactggctcagctgcaggaactgatccttgtgctctgcacagtgactgggtgccatgtccttggggcaggagagggattccagggccttggccatgagctcttgaccctgcttgggggctgtcagagcagctccatggaagctaaaactgtgacccctccccgcttcatccaggtacagctggaacagtccctgccataagtacttcttagccaggtccccagttgctcccagcaggattatggagacatgtccctggagctcctgggcttgcaggcagcccagaagggccaagcacatcgccactatgagcatattccacatgcctgggtgcttcctctcgcgcggcggcgcaggccgctcctccgggacacggccggggcggcgctgagggccgggcccgctcccgagggctcccctgcgccctgggccgcacctcctcttccgcagggcccgtcactccgacaagtgcgcgtgtcacgcggccacgcgccgcacgacactccgataccgcccgcggagcccgcggcggccgcaggggaaggcgcgaggccaaggccagcccggccgccaccccgccccaggcctcaggcctcaggcctccaccgccttgcgctcagcaagact

SEQ ID NO: 12912 - RNA, 5804 nt, Homo sapiens
  source 1..5804: mol_type = other RNA
gctgggattacaggcatgagccacacctagcccaatttagtgaattttaagaagcattttaaaaaaatgaaaactaaaacatagaggatatccgaggttctaaggttaagaatttctttatgaaacctgcttggaacacagttgtaaacaaatggactgatttatgatggaaggcacgtttcttgctgcagatcatggtctgaagtttgaaagccaccagcctagagggttctgaaaacttctccttcctaacacagctgaaggaaaaggggtgggtaggggcggaggcacagggacatctccaggtttggacttttccaacatgatttgcagaaggcacttgattctggaaagtagacctttggcatttcgaccctcacccacactcccacacccactctgcacagatcggtggtgcatccgaggcagggctgagttagaacaggacatcctagactcggcggcagtgactattattcagaaatggcacatcaagggccggcctgcccttcatcctgcaggggtacttgggcatgtggaggcccctttctccctggtgttgcaactggagaggagtcggttcctgaagaacagatgggagagtgctggggccaggtaccctgggagagaggagggaaatgaaatccggcacaggggctgcggggataggggcagtcaggaggcggcagtgcggtgcaagggcccccccacgcggccagctgtggaacttccaccacgactccctgtcctctcctgagcccgcccatcacgtgtagaagctcagatgctgggcgccaggagggcggcttcctggctctgggcaccgtggttctgtcctaacgaggggcgctctctgggtgtaaaaacagatgttctggctgggcgcggtggctcacgcctgtaatcccagcactttgggaggctgaggtgggtagactgcctgagctcaggagttcgagaccagcctgggcaacatggtgaaaccctgtctctactaaaatacaaaaattagacaggcatgctggccggcgcctgtagtcgcagctactcgggaggcttaggcacgagaattgcctgaacccgggaggtggaggttgtagtgagccaagatctcgccactgggctccagcctgggcgacagagactctgtctcaaaaaaaaaaaaaagagatgctctgtctggcctgggttgttgttggtggccagagtaagtggtgtgaacaagagccccggcttgggaacatgtctcagactggcattgaaaatgaaagccaggattcctctaaatccaccgccttgaagtgtaaacagtccagagagaaaccgactttgccatgctccctcacccaagaaagccctctctcaaaatgcgctagaaagtttatatctgcctgatccagagagcaagtggaaggtgcggagaagccagacagaaaaatcgaccttaaccaagagttccatctcccagccttaagttgtgggatactgaacaaacaaaactacacatgtcctgggaattttgctttgtggtgtttttaaaaagaatgtcagagccctccttgggggcttcagaaaagcaggtattgctggcccatggcttctcaagatcacagtccccaacctatgctcactgagaagatacccgcttacttccccagtctcaggcagagagttcgtggtgaagtgataagtagcaggagaggccagcagacaggaagccacggggtcaccaaggggcagggagagaaggcctggctgcggccccgtcacccgccaagcgagcccctgaaaaggctgtgggcagcccccctgccagtgaggcctagctcctgtctggtgggagcagagccgcctggatggcccagtgtcactcgatgctccatctctctccccgctaatgagctgtcacctcagtgggtgatttaactggatctttcctggtaaaacaagaggggctattgagagcggaaacacccatccgggagtcccctgagatggaaatgaccctcttaaattggggatctctggaatgtcctgattatctgcacccagtgtgcttcctggaggaaggctagcaggacagaggagcagcggagggcaggggtcctccctgaggaagttgggggaatgagaccccacctccccacgcagagcaagtcatcaaatgagaaatggagctccaaacagcactgagatttctggggctgggcgcagtagctcacacctgtaatcccagcactctgggaggctgagatgggaggatcgcttgagcccaggagtttgagaccagcctgggcaacatagcaagagctcatctctgcaaatattttttttaattaaaaaagaaaaaagatttctggaaccctttccacagtctagtctttgccactgtattcctgttatcagccctcattctctataaatggagtctgaagaacagcaaagacacagggaggagcctggaattcctactgcacagccaggatggaggagacagggatggcaagcgggagcaggtggaggcagtgaagaggagggccagaggctagatgtgcagaggttctagaaggaggggcagctggggaaggaggggcttgaccccctcagggtctcaagacagtccccaatgcccctgctttgcacggggcaatgtactcccctgggcgcctctgcacccttctgtctaccaatcatgctctgaatgttccccgggagccagttcaaggatcacctcccccaggaaaccttccctgattaacctcagcccaccacgtcacgtctcctcttgtgaacgccggagtttgggcgccatcccgtgttgtgctggttgatatgaatgtgtaactgctggaggtcttttcttaagacttctctcctggcctgaatttgaagcttctcaggagcagactccatttcttccttgtttctgcatctatccaccaatacacagagctgccggtcaaaggcatcgggacaaggcttgtcctgccctctctggggcctgactgtgggatagaaggttctggagagccagggcacgctgggcaggtggcggggccgagaagggagggaagacacgggcgaaggaaagcacaggagcgaagcgggcaaggggcacaggcgccctcatcccaggaaggcgtcgtagtccatgtaccacaccagctggccggagtgcggcaggacacccgagatgggccacttcttgggctcatggcccacccggctcaccagcgtggtgatctcacgcttcatcctgcccatgaccaggactgccaccttcttggcgcggttgatgagaggcaggctaaggctcatgcggcggtgtggctgggaggggctcgtggtcagcacgaccagctgctcgccatccaggccagtgggtgactgtgggaagagggaggctgtgtgcccgtcggcacccatgcccagcagcaccaggtcgaagctgctgttggccaccagggctgagatctccctggcatagatctgggcgccctggtcctcctcggcgcagagccgctgctgcaggtgcacaggcatggggtggatgttgtagtaggggatccggacgtgctgcagcaggtgggcctgcaggccctggaagttggactccgggtctgagagtgggacgcagcgctcgtcaaccagccacaggtgcgtgtgggcccaggggaagccatagtgcgccgtggccagctgctggaacagggccacggggctcgagccccccgacagtgccaggtggaactggccaaagcgccgcacggctcgcacagcggtggcctcgatgtcattagccagcttagagatcagctcctcggaccaggcggagaccagcgggctctctcggtacttggccctgaggacctggaagtcactgggcattggggccggccctggccctggcaccagctgctccggctgctgctgggaaaagaacaaccggccgctactgaactcaaagtccaacagacggccattctcagctcctccagggtagaggcgtggggccttatgggccaggctctccagcagaggggtccagaagttccaggaggccagcaagttctctgtggtgatgaagaaattcttccggccatggaagatatgggataagaggacggagtgggcgtcccgctcccgcacagggctgtaggcgtagtaatcggacagagggctgccgaaaaggcggagcccaggtggtccctccatttccttccagctggagggcagggagggcctgaacaggttcctgctgaccagcacggcagggctgcccaggtcgccatggccgatgtggaagacgagctgccggggcaggcactggctctgcgccgcggcccagtgcttttcgctctgcacacagcaggcctggttcttgaacaagatccgagcgtagcccactctctcgtccaaggctttgccagacatcaggatgaaaggcacgccctcccagcgaaggttgtcaatgtgcactaggacggctgcgaaggtcggcgtcaggctgtggaagctgtctggcttctgcagctctctgcgcacctgctcactgtaagactggtactggcccacgacggcactgcccctctgcaggccccgcagcgcctggaagacctgaagcttgtgccgcagcacagcctccgcactgctgacattgtggggcagctccatggccacgagggtgaggacctccgtcagatggttctggaggacgtcgcgaatgacaccgtactcctcatagaagctggtgcggccttcagcatccacggtctctttcatgatgatctccacccgctccacatggtgccggttccagaggccgtccaaagccttgcggttctggtctcggaaaggcaggatctgcgccacagcctgcttgcctaagtaatggtccacccggtacatctcctcctcctggaaaaaggtcccgagttctgtggccagctgctgggctgagaagtggtcatggccaaagggtttctcaaggacaacccgcagccaggcgcccgggcctggccggcagctactgttgatgttgcgggcaatgtcttcataggcgaagggtggcactgagaagtagaagatcctgccagcctcccggaggcctgcgtgctggagctgtgcctcgatgtccttgttcagggcctgatagtcctcggccgtcttcagttggcggtactggctcagctgcaggaactgatccttgtgctctgcacagtgactgggtgccatgtccttggggcaggagagggattccagggccttggccatgagctcttgaccctgcttgggggctgtcagagcagctccatggaagctaaaactgtgacccctccccgcttcatccaggtacagctggaacagtccctgccataagtacttcttagccaggtccccagttgctcccagcaggattatggagacatgtccctggagctcctgggcttgcaggcagcccagaagggccaagcacatcgccactatgagcatattccacatgcttcctctcgcgcggcggcgcaggccgctcctccgggacacggccggggcggcgctgagggccgggcccgctcccgagggctcccctgcgccctgggccgcacctcctcttccgcagggcccgtcactccgacaagtgcgcgtgtcacgcggccacgcgccgcacgacactccgataccgcccgcggagcccgcggcggccgcaggggaaggcgcgaggccaaggccagcccggccgccaccccgccccaggcctcaggcctcaggcctccaccgccttgcgctcagcaagactggggccc

SEQ ID NO: 12913 - RNA, 5142 nt, Homo sapiens
  source 1..5142: mol_type = other RNA
gctgggattacaggcatgagccacacctagcccaatttagtgaattttaagaagcattttaaaaaaatgaaaactaaaacatagaggatatccgaggttctaaggttaagaatttctttatgaaacctgcttggaacacagttgtaaacaaatggactgatttatgatggaaggcacgtttcttgctgcagatcatggtctgaagtttgaaagccaccagcctagagggttctgaaaacttctccttcctaacacagctgaaggaaaaggggtgggtaggggcggaggcacagggacatctccaggtttggacttttccaacatgatttgcagaaggcacttgattctggaaagtagacctttggcatttcgaccctcacccacactcccacacccactctgcacagatcggtggtgcatccgaggcagggctgagttagaacaggacatcctagactcggcggcagtgactattattcagaaatggcacatcaagggccggcctgcccttcatcctgcaggggtacttgggcatgtggaggcccctttctccctggtgttgcaactggagaggagtcggttcctgaagaacagatgggagagtgctggggccaggtaccctgggagagaggagggaaatgaaatccggcacaggggctgcggggataggggcagtcaggaggcggcagtgcggtgcaagggcccccccacgcggccagctgtggaacttccaccacgactccctgtcctctcctgagcccgcccatcacgtgtagaagctcagatgctgggcgccaggagggcggcttcctggctctgggcaccgtggttctgtcctaacgaggggcgctctctgggtgtaaaaacagatgttctggctgggcgcggtggctcacgcctgtaatcccagcactttgggaggctgaggtgggtagactgcctgagctcaggagttcgagaccagcctgggcaacatggtgaaaccctgtctctactaaaatacaaaaattagacaggcatgctggccggcgcctgtagtcgcagctactcgggaggcttaggcacgagaattgcctgaacccgggaggtggaggttgtagtgagccaagatctcgccactgggctccagcctgggcgacagagactctgtctcaaaaaaaaaaaaaagagatgctctgtctggcctgggttgttgttggtggccagagtaagtggtgtgaacaagagccccggcttgggaacatgtctcagactggcattgaaaatgaaagccaggattcctctaaatccaccgccttgaagtgtaaacagtccagagagaaaccgactttgccatgctccctcacccaagaaagccctctctcaaaatgcgctagaaagtttatatctgcctgatccagagagcaagtggaaggtgcggagaagccagacagaaaaatcgaccttaaccaagagttccatctcccagccttaagttgtgggatactgaacaaacaaaactacacatgtcctgggaattttgctttgtggtgtttttaaaaagaatgtcagagccctccttgggggcttcagaaaagcaggtattgctggcccatggcttctcaagatcacagtccccaacctatgctcactgagaagatacccgcttacttccccagtctcaggcagagagttcgtggtgaagtgataagtagcaggagaggccagcagacaggaagccacggggtcaccaaggggcagggagagaaggcctggctgcggccccgtcacccgccaagcgagcccctgaaaaggctgtgggcagcccccctgccagtgaggcctagctcctgtctggtgggagcagagccgcctggatggcccagtgtcactcgatgctccatctctctccccgctaatgagctgtcacctcagtgggtgatttaactggatctttcctggtaaaacaagaggggctattgagagcggaaacacccatccgggagtcccctgagatggaaatgaccctcttaaattggggatctctggaatgtcctgattatctgcacccagtgtgcttcctggaggaaggctagcaggacagaggagcagcggagggcaggggtcctccctgaggaagttgggggaatgagaccccacctccccacgcagagcaagtcatcaaatgagaaatggagctccaaacagcactgagatttctggggctgggcgcagtagctcacacctgtaatcccagcactctgggaggctgagatgggaggatcgcttgagcccaggagtttgagaccagcctgggcaacatagcaagagctcatctctgcaaatattttttttaattaaaaaagaaaaaagatttctggaaccctttccacagtctagtctttgccactgtattcctgttatcagccctcattctctataaatggagtctgaagaacagcaaagacacagggaggagcctggaattcctactgcacagccaggatggaggagacagggatggcaagcgggagcaggtggaggcagtgaagaggagggccagaggctagatgtgcagaggttctagaaggaggggcagctggggaaggaggggcttgaccccctcagggtctcaagacagtccccaatgcccctgctttgcacggggcaatgtactcccctgggcgcctctgcacccttctgtctaccaatcatgctctgaatgttccccgggagccagttcaaggatcacctcccccaggaaaccttccctgattaacctcagcccaccacgtcacgtctcctcttgtgaacgccggagtttgggcgccatcccgtgttgtgctggttgatatgaatgtgtaactgctggaggtcttttcttaagacttctctcctggcctgaatttgaagcttctcaggagcagactccatttcttccttgtttctgcatctatccaccaatacacagagctgccggtcaaaggcatcgggacaaggcttgtcctgccctctctggggcctgactgtgggatagaaggttctggagagccagggcacgctgggcaggtggcggggccgagaagggagggaagacacgggcgaaggaaagcacaggagcgaagcgggcaaggggcacaggcgccctcatcccaggaaggcgtcgtagtccatgtaccacaccagctggccggagtgcggcaggacacccgagatgggccacttcttgggctcatggcccacccggctcaccagcgtggtgatctcacgcttcatcctgcccatgaccaggactgccaccttcttggcgcggttgatgagaggcaggctaaggctcatgcggcggtgtggctgggaggggctcgtggtcagcacgaccagctgctcgccatccaggccagtgggtgactgtgggaagagggaggctgtgtgcccgtcggcacccatgcccagcagcaccaggtcgaagctgctgttggccaccagggctgagatctccctggcatagatctgggcgccctggtcctcctcggcgcagagccgctgctgcaggtgcacaggcatggggtggatgttgtagtaggggatccggacgtgctgcagcaggtgggcctgcaggccctggaagttggactccgggtctgagagtgggacgcagcgctcgtcaaccagccacaggtgcgtgtgggcccaggggaagccatagtgcgccgtggccagctgctggaacagggccacggggctcgagccccccgacagtgccaggtggaactggccaaagcgccgcacggctcgcacagcggtggcctcgatgtcattagccagcttagagatcagctcctcggaccaggcggagaccagcgggctctctcggtacttggccctgaggacctggaagtcactgggcattggggccggccctggccctggcaccagctgctccggctgctgctgggaaaagaacaaccggccgctactgaactcaaagtccaacagacggccattctcagctcctccagggtagaggcgtggggccttatgggccaggctctccagcagaggggtccagaagttccaggaggccagcaagttctctgtggtgatgaagaaattcttccggccatggaagatatgggataagaggacggagtgggcgtcccgctcccgcacagggctgtaggcgtagtaatcggacagagggctgccgaaaaggcggagcccaggtggtccctccatttccttccagctggagggcagggagggcctgaacaggttcctgctgaccagcacggcagggctgcccaggtcgccatggccgatgtggaagacgagctgccggggcaggcactggctctgcgccgcggcccagtgcttttcgctctgcacacagcaggcctggttcttgaacaagatccgagcgtagcccactctctcgtccaaggctttgccagacatcaggatgaaaggcacgccctcccagcgaaggttgtcaatgtgcactaggacggctgctcactgtaagactggtactggcccacgacggcactgcccctctgcaggccccgcagcgcctggaagacctgaagcttgtgccgcagcacagcctccgcactgctgacattgtggggcagctccatggccacgagggtgaggacctccgtcagatggttctggaggacgtcgcgaatgacaccgtactcctcatagaagctggtgcggccttcagcatccacggtctctttcatgatgatctccacccgctccacatggtgccggttccagaggccgtccaaagccttgcggttctggtctcggaaaggcaggatctgcgccacagcctgcttgcctaagtaatggtccacccggtacatctcctcctcctggaaaaaggtcccgagttctgtggccagctgctgggctgagaagtggtcatggccaaagggtttctcaaggacaacccgcagccaggcgcccgggcctggccggcagctactgttgatgttgcgggcaatgtcttcataggcgaagggtggcactgagaagtagaagatcctgccagcctcccggaggcctgcgtgctggagctgtgcctcgatgtccttgttcagggcctgatagtcctcggccgtcttcagttggcggtactggctcagctgcaggaac

SEQ ID NO: 12914 - RNA, 874 nt, Homo sapiens
  source 1..874: mol_type = other RNA
gctgggattacaggcatgagccacagcacacagccggtaacagcttttgaacataagcacctccacagacccctggtgccttcttgttggtatatatcgataaagcttccaatcatgctcccttggaacaagcttccttgagcctgcattcgaatctttagaacatcggtgggattggctatagtggaagatatcactcctgacactaccccacagatcatattaattaaaagagtttcatcttctaaacgttctacgaataagcgcttcaagctttggtaaatcccaattttaatggtgccatatgatgcttgtcttagcaacgcaggagcaattcctgaatagagagccaatacaccttcctctttacagatgcgaaacagcgcatggaacatccctctatattttatctctttgaaacgggcatcaatgctttggccttgaacctgaagtcgtgttttggtaaggtccacagggaaagtcccaaactcagccacgatagaggcaaggccgccatatacaaagggtttccaattcagaccagacatctcatgacttacagtggtacttttctggtgaatcacggccgccgttgcaaacttcacccttagaaaaattaggattattccgggaaagatacccattcaccctctgggtagcaggatcttgccagttcctcagctgtcagagcgagctcgtggagagaagggaggcgcctgaagaaggcggcctcccaggggggtcgaggaagcagggttcaatcgaagaagtaaaaccaccgatgccagaagagtgaaagacagggaagggactcagctgctcgggctcatcggacgactgggaagctgaggctcccacagtcggaaacgccact

SEQ ID NO: 12915 - RNA, 848 nt, Homo sapiens
  source 1..848: mol_type = other RNA
gctgggattacaggcatgagccacagcacacagccggtaacagcttttgaacataagcacctccacagacccctggtgccttcttgttggtatatatcgataaagcttccaatcatgctcccttggaacaagcttccttgagcctgcattcgaatctttagaacatcggtgggattggctatagtggaagatatcactcctgacactaccccacagatcatattaattaaaagagtttcatcttctaaacgttctacgaataagcgcttcaagctttggtaaatcccaattttaatggtgccatatgatgcttgtcttagcaacgcaggagcaattcctgaatagagagccaatacaccttcctctttacagatgcgaaacagcgcatggaacatccctctatattttatctctttgaaacgggcatcaatgctttggccttgaacctgaagtcgtgttttggtaaggtccacagggaaagtcccaaactcagccacgatagaggcaaggccgccatatacaaagggtttccaattcagaccagacatctcatgacttacagtggtacttttctggtgtccgcttacaatcacggccgccgttgcaaacttcacccttagaaaaattaggattattccgggaaagatacccattcaccctctgggtagcaggatcttgccagttcctcagctgtcagagcgagctcgtggagagaagggaggcgcctgaagaaggcggcctcccaggggggtcgaggaagcagggttcaatcgaagaagtaaaaccaccgatgccagaagagtgaaagacagggaagggactcagctgctcgggctcatcggacgact

SEQ ID NO: 12916 - RNA, 2718 nt, Homo sapiens
  source 1..2718: mol_type = other RNA
gctgggattacaggcatgagccacagcacccagccttgcatagcagtttcttaggttacagcatgtgggcaagatgtgatttctgctcggagttactgaaggcgtgcaggcaggagggaatccgactccgggacaaagccagtgtgcagcaggatttctccctccttgcctgaaaagcagtggattcttgaggatgcgtaagttgctctgcactgaggaccctgatgaaggtgacagatgcatcttctttctctccactttgcttgcaggaagaggaaccttgcaggatgacatttgcactaccagttagcatctgtgtggacacagacgatgccagggaacaccgtggtcagccccacggcagctgtaggtcccccagtattacagaagagagtaagagctcaatttctaagtgtgaccagacacgtgcagcattgtgtcaaccccgtcttgacggcatccttgaaaatcaaatgcagaagtgatcctctaacctcatcactccttaggaactgcaaagccctggatgctgtgtttggacctgcagcaggcacttgctcatcatcagcaggggtggcttcagctgctgcctaatcactcgctttagagcatggtaccgggtcccacatctgggccatctcatagtgggtcacgggtgtttctgtgtaggataaagctttgtgtcatgaccgtctcctcccttccacaaaggcagctgggtctccaaagactgaaggtgattccaagaccttctctccttcattgatccctaaaaggaagtttttatcactgggtccaagaaactttccctggattgaagcacacaagaaacaaagacagttcttctcttgacacccagctccatggaagcacagcctcctgttttcatttccggaagggggtgagcctgttgaaggtgtgccagaagagcgaggacttcctcttgggttccgccaggccaaagacctgctgctgggggacgcttgtgggcatagtgatgtggcgctggtggatggggtgcaggccctggtgcggtggggccacagggcacctgttgtagccttttgactttccatgtcctgccttttgagcatttaacatggcaagtttcttctggttttctgaaatttccattcccatctccttgtcctcttgcacccgcctcctttcatctgcacaggcctgcagccacctcgccttgtcttcttgttttttggcacaaaacaaataaacctcgtctgtggtcctactgacgagcttgaaggcatttttcacgctgaggttgcagtccttgtcgcgcccatcccccaggtccacaagctccatctcatccatgtccagccggcccttgtagtacagcatgtccctgcgcagcaggtccttcttgcaggacaccagctggtggtcaaacaggaagaacgtccgctgctggcttttgccttgcttagtgattttggtcagctccccagaatgaatcaattctgagcttcggtctaagatatccagtccctcccagcccacgatagacacctgccagcgagctatcttgtcgatgctctccagcttgcgcttgcgctcgttgatcagacaggccacattcttcatggcctcatatgctgcctttatgttgctgtaatcaccgtgttcctgtgtggtatacttgagcagctcggccagctgcagcgggtatttgcagatcttctgcactggtgtgagcaggaacccgtcgatggcgatgtcaatcatctgctgcagcaggcggcaggcttcaaagaaatgtctgtacttgccctgcttcatgaggttggcgagctccaggcaggcgcccgggtggttgttgcagtactcggaatagatggcaaagccctcttgattttgaagaaagcaagatcctatttcacttaagtgaggttcctctttgttgtactgtttctcaaggtctttcagaaactttctttggaatttgtaaatatcttcaatgtttccaaaaatagtggctagctgcgcaacggtgaacattcctgtgtgcttgcggcactgtcggatatagccctcacagatgtccctgaggtgtttgatgtacacccgctcggtgtccatgatctcccggatgacgttggtccgcatctgctgcttgttctcacagtgtctgtggcggctctggctggcctcctcgtcctgctcctcactgggggtgctgctggagttttccgacagctcttcctgattcactcgcaatctgacgaagctcgcggggaaccaggcttccttatcttcactgcggccccaccaccagtccttgttggaggcttccagaacctggatgacatccccggctttgaagcccagttcctggtcatccatggtcacatggtcccacagggcttctgcgcagaccacgttgccatcactgatcagctcattgatggccagctgctccccgccgggctgcaggtaccgagggctggcctggcagaggtcttcatagctgaagtcctcctcactaccgttgtcatccactaaggcagagggctcagtacctccatctgaagaaaccaagtgaaggctttccagactccagaatcttgctatctcccctctagctaccatccttctgtttggaaaacggcaaccttcagagcaggactggggtgtgaccgaggagccggtccccaagcatcacagaggactgcacaggctggcagctacgggaactgc

SEQ ID NO: 12917 - RNA, 5195 nt, Homo sapiens
  source 1..5195: mol_type = other RNA
gctgggattacaggcatgagccacagcacccagccttgcatagcagtttcttaggttacagcatgtgggcaagatgtgatttctgctcggagttactgaaggcgtgcaggcaggagggaatccgactccgggacaaagccagtgtgcagcaggatttctccctccttgcctgaaaagcagtggattcttgaggatgcgtaagttgctctgcactgaggaccctgatgaaggtgacagatgcatcttctttctctccactttgcttgcaggaagaggaaccttgcaggatgacatttgcactaccagttagcatctgtgtggacacagacgatgccagggaacaccgtggtcagccccacggcagctgtaggtcccccagtattacagaagagagtaagagctcaatttctaagtgtgaccagacacgtgcagcattgtgtcaaccccgtcttgacggcatccttgaaaatcaaatgcagaagtgatcctctaacctcatcactccttaggaactgcaaagccctggatgctgtgtttggacctgcagcaggcacttgctcatcatcagcaggggtggcttcagctgctgcctaatcactcgctttagagcatggtaccgggtcccacatctgggccatctcatagtgggtcacgggtgtttctgtgtaggataaagctttgtgtcatgaccgtctcctcccttccacaaaggcagctgggtctccaaagactgaaggtgattccaagaccttctctccttcattgatccctaaaaggaagtttttatcactgggtccaagaaactttccctggattgaagcacacaagaaacaaagacagttcttctcttgacacccagctccatggaagcacagcctcctgttttcatttccggaagggggtgagcctgttgaaggtgtgccagaagagcgaggacttcctcttgggttccgccaggccaaagacctgctgctgggggacgcttgtgggcatagtgatgtggcgctggtggatggggtgcaggccctggtgcggtggggccacagggcacctgttgtagccttttgactttccatgtcctgccttttgagcatttaacatggcaagtttcttctggttttctgaaatttccattcccatctccttgtcctcttgcacccgcctcctttcatctgcacaggcctgcagccacctcgccttgtcttcttgttttttggcacaaaacaaataaacctcgtctgtggtcctactgacgagcttgaaggcatttttcacgctgaggttgcagtccttgtcgcgcccatcccccaggtccacaagctccatctcatccatgtccagccggcccttgtagtacagcatgtccctgcgcagcaggtccttcttgcaggacaccagctggtggtcaaacaggaagaacgtccgctgctggcttttgccttgcttagtgattttggtcagctccccagaatgaatcaattctgagcttcggtctaagatatccagtccctcccagcccacgatagacacctgccagcgagctatcttgtcgatgctctccagcttgcgcttgcgctcgttgatcagacaggccacattcttcatggcctcatatgctgcctttatgttgctgtaatcaccgtgttcctgtgtggtatacttgagcagctcggccagctgcagcgggtatttgcagatcttctgcactggtgtgagcaggaacccgtcgatggcgatgtcaatcatctgctgcagcaggcggcaggcttcaaagaaatgtctgtacttgccctgcttcatgaggttggcgagctccaggcaggcgcccgggtggttgttgcagtactcggaatagatggcaaagccctcttgattttgaagaaagcaagatcctatttcacttaagtgaggttcctctttgttgtactgtttctcaaggtctttcagaaactttctttggaatttgtaaatatcttcaatgtttccaaaaatagtggctagctgcgcaacggtgaacattcctgtgtgcttgcggcactgtcggatatagccctcacagatgtccctgaggtgtttgatgtacacccgctcggtgtccatgatctcccggatgacgttggtccgcatctgctgcttgttctcacagtgtctgtggcggctctggctggcctcctcgtcctgctcctcactgggggtgctgctggagttttccgacagctcttcctgattcactcgcaatctgacgaagctcgcggggaaccaggcttccttatcttcactgcggccccaccaccagtccttgttggaggcttccagaacctggatgacatccccggctttgaagcccagttcctggtcatccatggtcacatggtcccacagggcttctgcgcagaccacgttgccatcactgatcagctcattgatggccagctgctccccgccgggctgcaggtaccgagggctggcctggcagaggtcttcatagctgaagtcctcctcactaccgttgtcatccactaaggcagagggctcagtacctccatctgaagaaacgttggatgctctcatctgccgccggcgtcccacacggtccaacccaatgggggtgctctgggagaatgtgaagggccggaaccgggccgacacagccttgtagggtggcacctggtgagcaggcatgggcggcctggaagccggttgggtcagaagattgtccagttcctccgtctggttggtcccatacaagctgaccccacctatcacggaaatggggcgccttctccgggctcctttggggcagcccactggagcattctggtcttcagggctggcagaagtcatgcttgcctgggggtcctcgtccacacggtcttccttctgggggtctgcagcaaccgagtcttcaggaatagacaaactgcggctggccagctggccgtagtcagagaatggccgaggccttggccgtctcccagagccccatctcctcttgggggttctctgtgcctctgtcctttcctcatcctgtgatgagcttcgcctccaggggccatcagggacgacctcctccttctccttttcttctgggccggctgccacaccaatgttcaccagaaggtccttgctgccctcatcaccatgtgtggcttccaggggatcctgcaaggacacaggccctggctctctctgagcaggctcttctgcccttccttcactttcctctgaattcgcggacagggcactgtgattgctgtgacagctggcacttcctgccccggggctctgggggctctgagggctctggggcttgggtgtggtgggccttagaggggtgggaggctgctcagggtcaaatgtcaactggctgccagcgtttgggtcacaggagtctttgctcaacacatcctggacaatcgggcttggcaaagagctgcaagtgcaggaactgtcgctttccaccgcccaggaacttttggtttcaagaggaaatacggcagtgtcagcgtctaggtggggccccttagaggtggctgagccgaaaccgggggccacggtgcaggttgcagtggtcccatgcatgaccgccccgccccgcctgctgtcctgctcagtgctcctggagacgcggcgggagtagtcgtcatgcagccggctgtgtgcctgaagtctcaggctggcctctccaggggatggggccccactcctaggactctccctcctccaggcagcctcagtcacattgctcacaagtttgaagactctgtcaaagtccttggcccttatcgggctcctccagcgtttggtccttcctgacccaagcttttgggagtcagtggaggaactgctcagggtcctctgtggtacccgtgcgtcatgggccgtcctgaggtctgcaagattggaggtggacttccgcttaaaggagctcttcttcagaaaggcaagattgtccgtgctcttgctcctcctgtagcccatgctgttgttttcagggtccctcacgagaatctcacacacggcgggcacctggccagtggctatcgtgggtgtcgcatggttctggggcgcatccagcaggcagatgcggcccaggccgtaggctctgcggaggctgcgggagcggtgtgtgctccgctggaaggcatcgtccgtgtcctcgaggtcggagccatccaatgtgccccactctgctggcctgagggcaccacatgctggtcccggtgctaagggggagcccctgcttgcctgggctcctgggacagcgccatttgggatggactttcccaggccatgctccgaagcctctccctttgaacaggcatttgacccctctcggctctgaattcctttcaggactgaggacttcagtttcttaaaggatcccattttccggaaggaggcgagggtgttccatgtggaggagttccccaccaggaccatggagtggggccgctcggggtgggcacccgtcctcttccgactggtggaaaagaggcgcacaagcttggctgggctgagtttggcttcctgggtgtccgtgtcgccaccagggctgcagccacagactccatttccacacgcaagggaggtcaccatcttggcgtctttcaggtccgagcctgcacagggggctgcggggcctggcccgaggccgtttggggcagtggtcatgttctccaggcagggtgcccagggccgcacggcagcctgggtcatggccacgggcactgccgagtccgcagaccgcagctccaggccttcatctccaggaatgccgtcctggcactcacacctgccttgcacatcgggctcctgggtggccacgggcgagtttctgcaccagctactcttgaagacaagctcttcacggccaggatgtttgtgaggcctacgctttgccatctgcacggtgttgccatttcattttcatcaggcctgtggtgctgcacaggcagcgaatatgactcccatcactctgcagctcaaaaaatgcagatagacaggtcacccctagctggaactaggcttcatcttcccttgtcagagcttgacaaggtttgaagctggccctgtctcagcatccctcctacgtcctcagagggtccttggagggatcccagcatcccgctccgagctggaagggggaggaaggtcacggagaagccgactggaaactgtcccgggtgcgcgcc

SEQ ID NO: 12918 - RNA, 5043 nt, Homo sapiens
  source 1..5043: mol_type = other RNA
gctgggattacaggcatgagccacagcacccagccttgcatagcagtttcttaggttacagcatgtgggcaagatgtgatttctgctcggagttactgaaggcgtgcaggcaggagggaatccgactccgggacaaagccagtgtgcagcaggatttctccctccttgcctgaaaagcagtggattcttgaggatgcgtaagttgctctgcactgaggaccctgatgaaggtgacagatgcatcttctttctctccactttgcttgcaggaagaggaaccttgcaggatgacatttgcactaccagttagcatctgtgtggacacagacgatgccagggaacaccgtggtcagccccacggcagctgtaggtcccccagtattacagaagagagtaagagctcaatttctaagtgtgaccagacacgtgcagcattgtgtcaaccccgtcttgacggcatccttgaaaatcaaatgcagaagtgatcctctaacctcatcactccttaggaactgcaaagccctggatgctgtgtttggacctgcagcaggcacttgctcatcatcagcaggggtggcttcagctgctgcctaatcactcgctttagagcatggtaccgggtcccacatctgggccatctcatagtgggtcacgggtgtttctgtgtaggataaagctttgtgtcatgaccgtctcctcccttccacaaaggcagctgggtctccaaagactgaaggtgattccaagaccttctctccttcattgatccctaaaaggaagtttttatcactgggtccaagaaactttccctggattgaagcacacaagaaacaaagacagttcttctcttgacacccagctccatggaagcacagcctcctgttttcatttccggaagggggtgagcctgttgaaggtgtgccagaagagcgaggacttcctcttgggttccgccaggccaaagacctgctgctgggggacgcttgtgggcatagtgatgtggcgctggtggatggggtgcaggccctggtgcggtggggccacagggcacctgttgtagccttttgactttccatgtcctgccttttgagcatttaacatggcaagtttcttctggttttctgaaatttccattcccatctccttgtcctcttgcacccgcctcctttcatctgcacaggcctgcagccacctcgccttgtcttcttgttttttggcacaaaacaaataaacctcgtctgtggtcctactgacgagcttgaaggcatttttcacgctgaggttgcagtccttgtcgcgcccatcccccaggtccacaagctccatctcatccatgtccagccggcccttgtagtacagcatgtccctgcgcagcaggtccttcttgcaggacaccagctggtggtcaaacaggaagaacgtccgctgctggcttttgccttgcttagtgattttggtcagctccccagaatgaatcaattctgagcttcggtctaagatatccagtccctcccagcccacgatagacacctgccagcgagctatcttgtcgatgctctccagcttgcgcttgcgctcgttgatcagacaggccacattcttcatggcctcatatgctgcctttatgttgctgtaatcaccgtgttcctgtgtggtatacttgagcagctcggccagctgcagcgggtatttgcagatcttctgcactggtgtgagcaggaacccgtcgatggcgatgtcaatcatctgctgcagcaggcggcaggcttcaaagaaatgtctgtacttgccctgcttcatgaggttggcgagctccaggcaggcgcccgggtggttgttgcagtactcggaatagatggcaaagccctcttgattttgaagaaagcaagatcctatttcacttaagtgaggttcctctttgttgtactgtttctcaaggtctttcagaaactttctttggaatttgtaaatatcttcaatgtttccaaaaatagtggctagctgcgcaacggtgaacattcctgtgtgcttgcggcactgtcggatatagccctcacagatgtccctgaggtgtttgatgtacacccgctcggtgtccatgatctcccggatgacgttggtccgcatctgctgcttgttctcacagtgtctgtggcggctctggctggcctcctcgtcctgctcctcactgggggtgctgctggagttttccgacagctcttcctgattcactcgcaatctgacgaagctcgcggggaaccaggcttccttatcttcactgcggccccaccaccagtccttgttggaggcttccagaacctggatgacatccccggctttgaagcccagttcctggtcatccatggtcacatggtcccacagggcttctgcgcagaccacgttgccatcactgatcagctcattgatggccagctgctccccgccgggctgcaggtaccgagggctggcctggcagaggtcttcatagctgaagtcctcctcactaccgttgtcatccactaaggcagagggctcagtacctccatctgaagaaacgttggatgctctcatctgccgccggcgtcccacacggtccaacccaatgggggtgctctgggagaatgtgaagggccggaaccgggccgacacagccttgtagggtggcacctggtgagcaggcatgggcggcctggaagccggttgggtcagaagattgtccagttcctccgtctggttggtcccatacaagctgaccccacctatcacggaaatggggcgccttctccgggctcctttggggcagcccactggagcattctggtcttcagggctggcagaagtcatgcttgcctgggggtcctcgtccacacggtcttccttctgggggtctgcagcaaccgagtcttcaggaatagacaaactgcggctggccagctggccgtagtcagagaatggccgaggccttggccgtctcccagagccccatctcctcttgggggttctctgtgcctctgtcctttcctcatcctgtgatgagcttcgcctccaggggccatcagggacgacctcctccttctccttttcttctgggccggctgccacaccaatgttcaccagaaggtccttgctgccctcatcaccatgtgtggcttccaggggatcctgcaaggacacaggccctggctctctctgagcaggctcttctgcccttccttcactttcctctgaattcgcggacagggcactgtgattgctgtgacagctggcacttcctgccccggggctctgggggctctgagggctctggggcttgggtgtggtgggccttagaggggtgggaggctgctcagggtcaaatgtcaactggctgccagcgtttgggtcacaggagtctttgctcaacacatcctggacaatcgggcttggcaaagagctgcaagtgcaggaactgtcgctttccaccgcccaggaacttttggtttcaagaggaaatacggcagtgtcagcgtctaggtggggccccttagaggtggctgagccgaaaccgggggccacggtgcaggttgcagtggtcccatgcatgaccgccccgccccgcctgctgtcctgctcagtgctcctggagacgcggcgggagtagtcgtcatgcagccggctgtgtgcctgaagtctcaggctggcctctccaggggatggggccccactcctaggactctccctcctccaggcagcctcagtcacattgctcacaagtttgaagactctgtcaaagtccttggcccttatcgggctcctccagcgtttggtccttcctgacccaagcttttgggagtcagtggaggaactgctcagggtcctctgtggtacccgtgcgtcatgggccgtcctgaggtctgcaagattggaggtggacttccgcttaaaggagctcttcttcagaaaggcaagattgtccgtgctcttgctcctcctgtagcccatgctgttgttttcagggtccctcacgagaatctcacacacggcgggcacctggccagtggctatcgtgggtgtcgcatggttctggggcgcatccagcaggcagatgcggcccaggccgtaggctctgcggaggctgcgggagcggtgtgtgctccgctggaaggcatcgtccgtgtcctcgaggtcggagccatccaatgtgccccactctgctggcctgagggcaccacatgctggtcccggtgctaagggggagcccctgcttgcctgggctcctgggacagcgccatttgggatggactttcccaggccatgctccgaagcctctccctttgaacaggcatttgacccctctcggctctgaattcctttcaggactgaggacttcagtttcttaaaggatcccattttccggaaggaggcgagggtgttccatgtggaggagttccccaccaggaccatggagtggggccgctcggggtgggcacccgtcctcttccgactggtggaaaagaggcgcacaagcttggctgggctgagtttggcttcctgggtgtccgtgtcgccaccagggctgcagccacagactccatttccacacgcaagggaggtcaccatcttggcgtctttcaggtccgagcctgcacagggggctgcggggcctggcccgaggccgtttggggcagtggtcatgttctccaggcagggtgcccagggccgcacggcagcctgggtcatggccacgggcactgccgagtccgcagaccgcagctccaggccttcatctccaggaatgccgtcctggcactcacacctgccttgcacatcgggctcctgggtggccacgggctcctgcggcgcctcttggcggagcctacaaagtcagcgtgtccaacacgtccctgccctcagagccacctccggtgccggcggagccccgaggtcgccgcactctcggaggagcctgggatccagtgcgcgccctcggagctagcgaccggcagggcgatcgcgggagaaagcgcaacgcacactctcctcccgcgccgcggcagcacactc

SEQ ID NO: 12919 - RNA, 3279 nt, Homo sapiens
  source 1..3279: mol_type = other RNA
gctgggattacaggcatgagccacagcacccagccttgcatagcagtttcttaggttacagcatgtgggcaagatgtgatttctgctcggagttactgaaggcgtgcaggcaggagggaatccgactccgggacaaagccagtgtgcagcaggatttctccctccttgcctgaaaagcagtggattcttgaggatgcgtaagttgctctgcactgaggaccctgatgaaggtgacagatgcatcttctttctctccactttgcttgcaggaagaggaaccttgcaggatgacatttgcactaccagttagcatctgtgtggacacagacgatgccagggaacaccgtggtcagccccacggcagctgtaggtcccccagtattacagaagagagtaagagctcaatttctaagtgtgaccagacacgtgcagcattgtgtcaaccccgtcttgacggcatccttgaaaatcaaatgcagaagtgatcctctaacctcatcactccttaggaactgcaaagccctggatgctgtgtttggacctgcagcaggcacttgctcatcatcagcaggggtggcttcagctgctgcctaatcactcgctttagagcatggtaccgggtcccacatctgggccatctcatagtgggtcacgggtgtttctgtgtaggataaagctttgtgtcatgaccgtctcctcccttccacaaaggcagctgggtctccaaagactgaaggtgattccaagaccttctctccttcattgatccctaaaaggaagtttttatcactgggtccaagaaactttccctggattgaagcacacaagaaacaaagacagttcttctcttgacacccagctccatggaagcacagcctcctgttttcatttccggaagggggtgagcctgttgaaggtgtgccagaagagcgaggacttcctcttgggttccgccaggccaaagacctgctgctgggggacgcttgtgggcatagtgatgtggcgctggtggatggggtgcaggccctggtgcggtggggccacagggcacctgttgtagccttttgactttccatgtcctgccttttgagcatttaacatggcaagtttcttctggttttctgaaatttccattcccatctccttgtcctcttgcacccgcctcctttcatctgcacaggcctgcagccacctcgccttgtcttcttgttttttggcacaaaacaaataaacctcgtctgtggtcctactgacgagcttgaaggcatttttcacgctgaggttgcagtccttgtcgcgcccatcccccaggtccacaagctccatctcatccatgtccagccggcccttgtagtacagcatgtccctgcgcagcaggtccttcttgcaggacaccagctggtggtcaaacaggaagaacgtccgctgctggcttttgccttgcttagtgattttggtcagctccccagaatgaatcaattctgagcttcggtctaagatatccagtccctcccagcccacgatagacacctgccagcgagctatcttgtcgatgctctccagcttgcgcttgcgctcgttgatcagacaggccacattcttcatggcctcatatgctgcctttatgttgctgtaatcaccgtgttcctgtgtggtatacttgagcagctcggccagctgcagcgggtatttgcagatcttctgcactggtgtgagcaggaacccgtcgatggcgatgtcaatcatctgctgcagcaggcggcaggcttcaaagaaatgtctgtacttgccctgcttcatgaggttggcgagctccaggcaggcgcccgggtggttgttgcagtactcggaatagatggcaaagccctcttgattttgaagaaagcaagatcctatttcacttaagtgaggttcctctttgttgtactgtttctcaaggtctttcagaaactttctttggaatttgtaaatatcttcaatgtttccaaaaatagtggctagctgcgcaacggtgaacattcctgtgtgcttgcggcactgtcggatatagccctcacagatgtccctgaggtgtttgatgtacacccgctcggtgtccatgatctcccggatgacgttggtccgcatctgctgcttgttctcacagtgtctgtggcggctctggctggcctcctcgtcctgctcctcactgggggtgctgctggagttttccgacagctcttcctgattcactcgcaatctgacgaagctcgcggggaaccaggcttccttatcttcactgcggccccaccaccagtccttgttggaggcttccagaacctggatgacatccccggctttgaagcccagttcctggtcatccatggtcacatggtcccacagggcttctgcgcagaccacgttgccatcactgatcagctcattgatggccagctgctccccgccgggctgcaggtaccgagggctggcctggcagaggtcttcatagctgaagtcctcctcactaccgttgtcatccactaaggcagagggctcagtacctccatctgaagaaacgttggatgctctcatctgccgccggcgtcccacacggtccaacccaatgggggtgctctgggagaatgtgaagggccggaaccgggccgacacagccttgtagggtggcacctggtgagcaggcatgggcggcctggaagccggttgggtcagaagattgtccagttcctccgtctggttggtcccatacaagctgaccccacctatcacggaaatggggcgccttctccgggctcctttggggcagcccactggagcattctggtcttcagggctggcagaagtcatgcttgcctgggggtcctcgtccacacggtcttccttctgggggtctgcagcaaccgagtcttcaggaatagacaaactgcggctggccagctggccgtagtcagagaatggccgaggccttggccgtctcccagagccccatctcctcttgggggttctctgtgcctctgtcctttcctcatcctgtgatgagcttcgcctccaggggccatcagggacgacctcctgcggcgcctcttggcggagcctacaaagtcagcgtgtccaacacgtccctgccctcagagccacctccggtgccggcggagccccgaggtcgccgcactctcggaggagcctgggatccagtgcgcgccctcggagctagcgaccggcagggcgatcgcgggagaaagcgcaacgcacactctcctcccgcgccgcggcagcacactc

SEQ ID NO: 12920 - RNA, 2926 nt, Homo sapiens
  source 1..2926: mol_type = other RNA
gctgggattacaggcatgagccacagcacccagccttgcatagcagtttcttaggttacagcatgtgggcaagatgtgatttctgctcggagttactgaaggcgtgcaggcaggagggaatccgactccgggacaaagccagtgtgcagcaggatttctccctccttgcctgaaaagcagtggattcttgaggatgcgtaagttgctctgcactgaggaccctgatgaaggtgacagatgcatcttctttctctccactttgcttgcaggaagaggaaccttgcaggatgacatttgcactaccagttagcatctgtgtggacacagacgatgccagggaacaccgtggtcagccccacggcagctgtaggtcccccagtattacagaagagagtaagagctcaatttctaagtgtgaccagacacgtgcagcattgtgtcaaccccgtcttgacggcatccttgaaaatcaaatgcagaagtgatcctctaacctcatcactccttaggaactgcaaagccctggatgctgtgtttggacctgcagcaggcacttgctcatcatcagcaggggtggcttcagctgctgcctaatcactcgctttagagcatggtaccgggtcccacatctgggccatctcatagtgggtcacgggtgtttctgtgtaggataaagctttgtgtcatgaccgtctcctcccttccacaaaggcagctgggtctccaaagactgaaggtgattccaagaccttctctccttcattgatccctaaaaggaagtttttatcactgggtccaagaaactttccctggattgaagcacacaagaaacaaagacagttcttctcttgacacccagctccatggaagcacagcctcctgttttcatttccggaagggggtgagcctgttgaaggtgtgccagaagagcgaggacttcctcttgggttccgccaggccaaagacctgctgctgggggacgcttgtgggcatagtgatgtggcgctggtggatggggtgcaggccctggtgcggtggggccacagggcacctgttgtagccttttgactttccatgtcctgccttttgagcatttaacatggcaagtttcttctggttttctgaaatttccattcccatctccttgtcctcttgcacccgcctcctttcatctgcacaggcctgcagccacctcgccttgtcttcttgttttttggcacaaaacaaataaacctcgtctgtggtcctactgacgagcttgaaggcatttttcacgctgaggttgcagtccttgtcgcgcccatcccccaggtccacaagctccatctcatccatgtccagccggcccttgtagtacagcatgtccctgcgcagcaggtccttcttgcaggacaccagctggtggtcaaacaggaagaacgtccgctgctggcttttgccttgcttagtgattttggtcagctccccagaatgaatcaattctgagcttcggtctaagatatccagtccctcccagcccacgatagacacctgccagcgagctatcttgtcgatgctctccagcttgcgcttgcgctcgttgatcagacaggccacattcttcatggcctcatatgctgcctttatgttgctgtaatcaccgtgttcctgtgtggtatacttgagcagctcggccagctgcagcgggtatttgcagatcttctgcactggtgtgagcaggaacccgtcgatggcgatgtcaatcatctgctgcagcaggcggcaggcttcaaagaaatgtctgtacttgccctgcttcatgaggttggcgagctccaggcaggcgcccgggtggttgttgcagtactcggaatagatggcaaagccctcttgattttgaagaaagcaagatcctatttcacttaagtgaggttcctctttgttgtactgtttctcaaggtctttcagaaactttctttggaatttgtaaatatcttcaatgtttccaaaaatagtggctagctgcgcaacggtgaacattcctgtgtgcttgcggcactgtcggatatagccctcacagatgtccctgaggtgtttgatgtacacccgctcggtgtccatgatctcccggatgacgttggtccgcatctgctgcttgttctcacagtgtctgtggcggctctggctggcctcctcgtcctgctcctcactgggggtgctgctggagttttccgacagctcttcctgattcactcgcaatctgacgaagctcgcggggaaccaggcttccttatcttcactgcggccccaccaccagtccttgttggaggcttccagaacctggatgacatccccggctttgaagcccagttcctggtcatccatggtcacatggtcccacagggcttctgcgcagaccacgttgccatcactgatcagctcattgatggccagctgctccccgccgggctgcaggtaccgagggctggcctggcagaggtcttcatagctgaagtcctcctcactaccgttgtcatccactaaggcagagggctcagtacctccatctgaagaaacttcaaatgatagcgatgcacattttttttcttttctatatttttcttttttgagtatgagtccttggtcaagtttctttctttgttttttcacctgttgaatgtggatgataaaacccatctctcagggttgtttatacattctgaacaagtacttgttattggtgtgctttgagcctcaagtggaatgatgatacatgaaagcaccccaagtgaaggctttccagactccagaatcttgctatctcccctctagctaccatccttctgtttggaaaacggcaaccttcagagcaggactggggtgtgaccgaggagccggtccccaagcatcacagaggactgcacaggctggcagctacgggaactgc

SEQ ID NO: 12921 - RNA, 2532 nt, Homo sapiens
  source 1..2532: mol_type = other RNA
gctgggattacaggcatgagccacagcacccagccttgcatagcagtttcttaggttacagcatgtgggcaagatgtgatttctgctcggagttactgaaggcgtgcaggcaggagggaatccgactccgggacaaagccagtgtgcagcaggatttctccctccttgcctgaaaagcagtggattcttgaggatgcgtaagttgctctgcactgaggaccctgatgaaggtgacagatgcatcttctttctctccactttgcttgcaggaagaggaaccttgcaggatgacatttgcactaccagttagcatctgtgtggacacagacgatgccagggaacaccgtggtcagccccacggcagctgtaggtcccccagtattacagaagagagtaagagctcaatttctaagtgtgaccagacacgtgcagcattgtgtcaaccccgtcttgacggcatccttgaaaatcaaatgcagaagtgatcctctaacctcatcactccttaggaactgcaaagccctggatgctgtgtttggacctgcagcaggcacttgctcatcatcagcaggggtggcttcagctgctgcctaatcactcgctttagagcatggtaccgggtcccacatctgggccatctcatagtgggtcacgggtgtttctgtgtaggataaagctttgtgtcatgaccgtctcctcccttccacaaaggcagctgggtctccaaagactgaaggtgattccaagaccttctctccttcattgatccctaaaaggaagtttttatcactgggtccaagaaactttccctggattgaagcacacaagaaacaaagacagttcttctcttgacacccagctccatggaagcacagcctcctgttttcatttccggaagggggtgagcctgttgaaggtgtgccagaagagcgaggacttcctcttgggttccgccaggccaaagacctgctgctgggggacgcttgtgggcatagtgatgtggcgctggtggatggggtgcaggccctggtgcggtggggccacagggcacctgttgtagccttttgactttccatgtcctgccttttgagcatttaacatggcaagtttcttctggttttctgaaatttccattcccatctccttgtcctcttgcacccgcctcctttcatctgcacaggcctgcagccacctcgccttgtcttcttgttttttggcacaaaacaaataaacctcgtctgtggtcctactgacgagcttgaaggcatttttcacgctgaggttgcagtccttgtcgcgcccatcccccaggtccacaagctccatctcatccatgtccagccggcccttgtagtacagcatgtccctgcgcagcaggtccttcttgcaggacaccagctggtggtcaaacaggaagaacgtccgctgctggcttttgccttgcttagtgattttggtcagctccccagaatgaatcaattctgagcttcggtctaagatatccagtccctcccagcccacgatagacacctgccagcgagctatcttgtcgatgctctccagcttgcgcttgcgctcgttgatcagacaggccacattcttcatggcctcatatgctgcctttatgttgctgtaatcaccgtgttcctgtgtggtatacttgagcagctcggccagctgcagcgggtatttgcagatcttctgcactggtgtgagcaggaacccgtcgatggcgatgtcaatcatctgctgcagcaggcggcaggcttcaaagaaatgtctgtacttgccctgcttcatgaggttggcgagctccaggcaggcgcccgggtggttgttgcagtactcggaatagatggcaaagccctcttgattttgaagaaagcaagatcctatttcacttaagtgaggttcctctttgttgtactgtttctcaaggtctttcagaaactttctttggaatttgtaaatatcttcaatgtttccaaaaatagtggctagctgcgcaacggtgaacattcctgtgtgcttgcggcactgtcggatatagcctctgacgaagctcgcggggaaccaggcttccttatcttcactgcggccccaccaccagtccttgttggaggcttccagaacctggatgacatccccggctttgaagcccagttcctggtcatccatggtcacatggtcccacagggcttctgcgcagaccacgttgccatcactgatcagctcattgatggccagctgctccccgccgggctgcaggtaccgagggctggcctggcagaggtcttcatagctgaagtcctcctcactaccgttgtcatccactaaggcagagggctcagtacctccatctgaagaaaccaagtgaaggctttccagactccagaatcttgctatctcccctctagctaccatccttctgtttggaaaacggcaaccttcagagcaggactggggtgtgaccgaggagccggtccccaagcatcacagaggactgcacaggctggcagctacgggaactgc

SEQ ID NO: 12922 - RNA, 4463 nt, Homo sapiens
  source 1..4463: mol_type = other RNA
gctgggattacaggcatgagccacagcacccggccgagaagtctcatttttaaaattaaaataaaataggtagatggatggatagataaaacaaaaaatatatgaacttccttgtctcagaggcaaatttgtgttcttaaaagttctgcaggcagaaggacactagatcacagtcacattgcatccccgacttccttagtccatcgcttcccccaaaaatggattaggaatgggcagtctgcgagggaagcatgttggctagggtgggcaaggcagaaagagaaggaaagactcttaaaaagaaaagaaggataaatatcgccagggagtcaagcacaagcaatctttcttattccctcctttccatctgtagcacaaaccccagttaatcaattactttcttgaagagaattactgttacgtggaaagcgacctaagaaagcatttgttgtcagcattatgcactgcaggccttatcacaatcaggccaaaaaagtaccattacagagccaaaggagatcatctaatttcatagaatcccttcttgtgaaagtatgttattggatatgcctgatgctgtcaaagtggggtggaggaaggctgagcagtactaagaatacggctttttttgtggttgttcaaagaagaactatagcaattcttcctttccagtgtttttataatttggtttagaatcagccaagacaaaacaagagaagggctggaaaccttccctccaagaagttggaatcaatatattttcctgaaatattttgttagtgtggtaattaagatagagtttcactcagaactttatgcatttgactatttcctcattaaaaaaaaaaggtcagtgtgctaataaagataaatacattctattttcctttcaggattttaattctctcaaccctatcatagtactcaagagcaagcttacctgatgtccttacaaaatcctggttctaatgctctacagcaaaatcacctgtgcaaatatgtgtgcacactgtgtgtgtgtgtgtgtgtgtgtgtgtgtgtgtcagagtgagagagaatgcattgagcactggcatgtgcatctgaaaagttttagtcttaattcctcattctttatttttggtagcatcattaacattacaaaaacagtaaactggtataggtttcaaacatgcaaacttgctaatagtattctgcagagggacaattccaggatcagagagaatacttcttgctccaaacacaattttacattttgaaatatgatttactttctggattgcagccaggcaattaccattcacaaatatttcaagtgagagagagaaagtggttgctactagtcccataatttggaattgctgctaacagattttacatatcatctacttttctgccattctctttcagaaaatacaattaaaccttaatatttctgcattttaagtcttactgtcagcttcgtcactgcttgaaacaaaagtgtgtaagtggctccctctggtgctgccactagtattaatttttctattcgcaaccacagatgtaacccagagaagcaggaaaaagtaggtagaagccctcataactggaaatgtctcttggcacacaatcccacatggaataatattagataagagatgagggggtttggagggcggggtaggaatagatgcttaatatcttccgtggccttttttcctcacttcatatacacaaaaggaaattgcaaaagctttaagaaaagtcatgtttactaaaccccagccaaaatcccccattcttgttgcctaatactaatgacctaagaaagtacttaagtactacttctaatggaccttgacagggccatcagtcaccagcccagcactccacttgacctggggcctacatagccatgattagagcaaaagtgggatcataaaaagtctcttccaagtggcaaccgagggctccagaacagcacctctgaatggcagtggtgaaggaagctggcaaaacttccttctgtggctgtggtccatagttctctctgatgaccactctttcaatgtaagtcctactcacagacagacaatgtttgaaatttagactccgtaagggaatgatctgacttctaggtcagccaccacagtgtacagtcccaatgattagtttatagcaatctgcaggctctctcatgctgatcttgccctcttttctgccaaagaggcagcacatcttccctgctatatttctctaaagcacagcacagcctccaccaccagccagaatgttaatgcattatcactctgtacactgagaaaacaagtgaccatatgtagcctatgccagcggagctgtaactgtgaagaacaatggctctgagtcaacaacagaattaaactactccctcttgtgaagctcttctgaatattttaagtgttgccttgaaagtgtgggattatgtgcaagcataaacattagcttaatgcaattttttggtacagaatatgccagagtttaaaaatcagaattgaaatgcagaaaataactttgggataaatttaatttttttatgtgtgattaaaacatgattgaagtggcatactttatgtataattaaagttgctttgtaattaagagatttaaacatgtatagaaaatgatacagcctagtttggagattttacaaaggcacctattaaatactcacccctagcaagcctatgactcaaatgttttcacattctaatgctgatagagttcttgaattttctaaagctgccaatttcaccatttctaaatgctttatccctccttccatgtgctagtgaaataaaagcagcccaatctcccctgcattaacaaaaacatggatgtagaacaccatatcttaacttcaaaaactccaggtgaataaagaaggactgtcacaattgaggtagcgtttgactcatctttgccttctccattgtgcctagcaccatgtcccacccagtgcttaggaaatacgtgataaatggctattagtaggtgagcacagtgtgtccgtgtttatgtatggagggttctcatgataatgcaaacacttctgaacatttttatgtgccaggcaaaagtgctatgttattttgtttattcccataacggccctatactttttagagttttagaatagcctggtgaaggaatgacactcaaaatagactagcaggactactctcagtgtattttttacagacagaaaaactaaatcaaagagaggtgaagtccacacagaatcatgaattttagtactaacttagcagcagtaccacctattaagctaaagaattatgcagaacaagtttggttgttttcccccttatcttgctcatttgtgtcacccctttcccagacccaaattcctcaatctcccaccctctccagagattgcctcttggcccccctacaggtccctaaaacatccttctagtaagcacctggcattaacctaggcttgttctcactagcaatgatcttggtttaaactgatcttcctggccttccccatcaatacttgtcttttttatgtttcattctttttagccaagtatcacatggcggagggaaatagtcagacaaacttattcatattagagtgttggttgctgatatttgcatttagaaggcttttgcaacatttcaaaagcacaatggaaaatcctgaatttgggttctggatttaggtacagaaaggatgccatgtaagagacgtgtgtaagagacattgttgactggatacagggatcaggagacaggaaatcaggagttggaaatgggggaaagaaataatattcatgaagataagcaaaaaaatatatggactgatagatgaatgctagatttattttcctgggggccagtgacacgttttctaggggccagtgacacgttttctagtgtttttccacattcccgtctacagtacatatggaatatgaacagttttttccaagaaaagtgattgtttcttctcaggctttctcatatcaatcattcaactataattttcaattaataaagataaacagaggtagatagatacacatttacatattgatatatatgtatacatatggcagttttgcaaacctgagtgtagcaggataaataaaagatattgcaatgttaaagatggctctttatactctttctaacactctaacaaattattccatttccagtgattataccttcgttctcccctatagcagcaccacccatactcttgtttttctcagatttctatggtagagtgtcccacgagaggctgttctgtgagatctcaggcttcctaggggttctagagaaggctcgtgaagaaatgacattcaaaatagcataccaggactattcccagcgtattttgagttacaactggcagagttgtaatgcacctattcttttttttttttttttgagacagagtctcgctctgt

SEQ ID NO: 12923 - RNA, 2387 nt, Homo sapiens
  source 1..2387: mol_type = other RNA
gctgggattacaggcatgagccacagcaccctgccagttcacacagttaataaacatttattaagcaccttctatgtgccaggctctgtgtgaggccccagagaagaaaagacagtagacaagtctttccttttaagaatgtataggctagaagagacattcacgtcagtgtactcctttgctttggtactaacacagaacattttagggtcaaggtgaaaaaagaaggccagaattttgggccttcataatccagggcaccaacatacctacaaataacaggtctgagctgagcagtattacagggctccaacattcagagtttagtcctatcacttatttggtgagtatgagacaaactgagtgctctctcttgtctcatttatagatgcaaagaatagccctttctcttcccaagagtcagcgagggattgaagacaatatctctttgagggaccttgcagatcacctgtggttcaagcaggctatgccttctccccattgtgaggccatttgagtatggcacacgtcacaaatcccctcccccctagaatgcctcctccgtaccatgccccaggccaatcagttatcagtatactagctaacatttatcaagtacttactatgtactgggaattgggccaagtattttgtatttctaattccatttaatctacttaataagtatatacagcacaccttattactgtgaatattttacaactgagaaaatggaagcttacaatgataaaaaaactggtagctgataaatggtcaagctgggactttcacgcctagactgactgcaaatcacgtgcttagtcttaaccactctgttgggaactccccatccctcccaattgttattcaaggaactttgtggctgagaacttacaagggttcttagtgaaggtgttcaagcaggaacctgaggaatcagacccaaaggagagtcaggaacatggaagcagaagttccatgttttttattgtgattggtgggaaaaggaagttcttgggtggacatgggatgtgggtgaatcggagggtataatgattccttgagggtctaagatcaggttttctgaatggagaatggcacaactacagaatgatccagagggattcagagggacatagtgacaaccatggagtacaggattagtatatgtttctcaatgactctccaatagtcataatcaaaatacaatgaaattggaagtgaccctggagatcctctagtccaaacatttcacatgtgagggccctgagctggaaaggtgaacacactcgtacagtgaagcacagcttgttcatgtatgtactaagctcgaacccatgttctgggcccaccagctactggtgatctcaggaatggattctgaagaccattcagggtaatgtcataccatcctcagagccatcattctgggaggtggtggggtggagatcggaaaaaggcagattccctggaacaatgggcctttcagctaaaccttggataaatggcttcagtcccaggaggagagaaggtgagtttccacattttaccttctgggaaaatcctaccttgtcttctcttgaacaaacggaacaaaaacactgaagacagaatgagaacaagcagaaagaacatagccagcacgctcagcaacccggtgtggtgagtacggaagcccattgcgatgtctgcacagagctgccgggcagagatggagtcagaattgttgctgacagggttctgggctgtacacgtgtaagtcagctcttggtcctcaggagtctggaagatttgaaggacattaccctcttctcccaggggactccaattgtatgtcacattcttttcttctttctctacagagcatgtcagtgtgacattacaggtgctgttcacagatgccattaaactctgtgtaatttttggtttcccaagccgacgatagatttgcaggttgtagcgcttggtggtggtgtagggatcagcctgtgtatttatgtctgctttgtagtctcctgcgtcttccatcctcagatcgctaatgaccagattgtagttcggacctaaggcatgtatccgttcataataatttctgtgggtcacagtaactacgggtgctgtttctgagtctcctggtgttacataagcaacagatgttttagaagtccaagcaatgattttaacttgccgtggttcttggatatttacagggaaagtgactgactctcccagaatcccattcactgtgaagatttctgagtcttttccagctgcttccggccaggtttgcaggcaaaggagcaagatccataggtggtgctgagccatctctttcagggtctaaccttctgtggaaaagcacggcactgttctagcagagtcagttt

SEQ ID NO: 12924 - RNA, 4757 nt, Homo sapiens
  source 1..4757: mol_type = other RNA
gctgggattacaggcatgagccacagcacctggccgtaaatgagagtttttatgtgcaagtaaaggcagttaaataactttcagtaataaaatgcatcacaatatttcacaggtttaaaacacaacctggttacctttttgaataaaataacatttggaagaaggcatagctacttttaaaagctattctatgctttccttgtgtttgaaatttcaagaaaaaataaaatgataaatcacaaaattaaaaatgccaaattcaagttaattcctataattcttccattttgttatgaatattctgtaatatcaaacattcatttttaatgtgctaaaaatatgggtttacaaaatatgaacaggtaatttttaaagagtaaattatgttaagaactttattattttcgattcattttatagggtagtaaaataatacttcttcaaaatcatttaaatgttattgatgccattgcaaaatcattataaataaattttctccattatccaatcacatctagataacattgaatatgtacaggtttctctggataggtaccaaaaggtaccacattttatacagacttaattgtgaaagctgggtgaaataaattttcagatcaaaattttttttaagtttaaatcattcactctttaaatttcagacagtgtcagtgtgactcttacttttaaaggaaaaaaattagtttaaaatttaatagccacagatttaataattttttactttaacacttaatgtacattttcatgagcagtaattaagatatgttgaaattttaaatgtgaaagatttcaaagtttcagtatgttaacattactcttcaaatgttcttaatatatatataaacacttacaaattatagatacaactagttgtatatctacaatacatatatgaacaccattcttcttctctagccatatttatatgaggataaagtaataaatctctgtgctattcaaggaaaaaaaatgaatgctttaaaaaataaatctttaaagaatagtttcaaaaataaagttcaaatattgcacaaaataatttaactgtaaatattactacatagtgtaaaacaattttaaaaaaatttttacactctacagtaaatcccactttctaattctataaaagaatttattggaagtccacattaaatgtttagatattaaatgcttacattcagtttgatgggaattcaattttcacaagttaactgagactttgtcttaaaagttcatctatttgagttttgtacatattttttacatcttcgagatctaatcgaagttcttctgcctcttctgctttttctccatacatctgcagaatagtgttgtacctttgatccaaatctcttagctgagttctaagtttgggtatctccttcaccttctcttcaagttcatcattttgatttgttaatttaactagttcttcagccattattgatcgagttttttctagattgccaatttctagctgtaaatgagtgatttccccttcccttagctttagctgagactgtaggttttcaattatgcttgatcctgctcccatccttacagcatcataaagattgcttccatttgctgatataggcattggtccaaatgagtgatcatgagactcatcctgagacagaaaagatgtctgtagtcctgccatatcaacaccacttattgaacttgagcgtgacatggtgggagtgctagaaacagaaaatggcttgcgttccttttcttttattgtttcttgagtaaaaatggctttcttcctttcttgttcaactttcattctttccatttctaactgactattcaacaatgtcttttctttcctcgtctcttcaagtgttcttacatattcatcttttaggttttccaattcaacctggtacctattgttctcatcctccagtttacacagcctatttttctctgattctagctgggcttgaaatctactgttttcctgtcttaaaagagaattctgtgactccatggaagacatctgaattttgttagcaaggagttcttctgtagctgcacgttctctctcaactgctgctgccagcaaggtctgggattcaccaagcctatcagaaagattcttctctaatttctcccacgacgatgtctgggatcccagggttgcttgcaaattttctatttgtcgaagcaatggtcttgttgttgatgaaacactttgactcagttcctggtttcgattctctgcttcctggagtctctgctgaagttcaccgatctcatggcgtaaataatcctcctttctggcagccgcttgttctgtacgctgcaatgcaagcctaaggtcccccacttgaatggctaatgtttcttgctgctgacgggcttcttcttgggccttctctaatgctgcagaaagttcttctttagctttcatttcacggctcagagcagcttcctgtgcctcactatcctttgcagcattggctttgtgaagatcagtaagttctttgtatgcactatccagggcagcctgaatacttcggttcttttcttcaagttcatccatgtctacctgaagacggccaagatctttctcttggcgttctaccatggaatttagttttttaatattttctctatgttgtttctcaacctcttctttgccatcaaggacctgtttcaaatgctgcaactcctcttctagctctttaacttttttgttcagctttgcaaccatattttcattctccttgtctttagctcttaatttcttgatgatgttagaattgtgcagctgctgttttgaaagtttttctccttcttccattaaccctcggatctgctcatctttctctttcaaaaggtctgcagtttcactactatttaatctagtggcaagttcttcttttatgtttttgatttcctttttagcagcatctctctctttgcaggctagttgaactttcttttctgcttctgcaattctttgagtaaactcatctttcaaggaagaaatgctactgctttcttctttcactctgaacatttcatctttcaggttatcaaaagcttcttctagaagtgctttttccttactaagagataataactgagcctcccttttttccagcttttcattcagaaattcaactgtcttgcaaacatcttccttctcagaaagtgcttctggctgactttcagcaggttcacactgctcagccaccttgtctaacacagtctgtccttcatttattggtgtggaagaaaccaagatatcaggctgttcacagttaacaggagttgcacttcgtccactttcttccatttctgcttcctcagtgggtataactaatgtttcatttacttcttcagattttccttcagcagattcaactgttttagactttggagttgaagaattaactataataggcactaaagcatatcccttgcctgacaattcatcatctgaattgatttcacttacactccggctatctaatgactgtacactaaatgagtctattctttcaaaagcatcagatgaacagcaactctcagtgagtttttggaaatcatctaaacgattatattcaggacaagcagatgcagagagaagctgaaaagatgtctgcatcaagtgaagacttgattttgaatctgtagtctcttgtctcgagctcgctgagctctcacttattacactttcatgatctaaaacttcaatatcactggtggtagaagtacctgatgaaaaggtactaacaggaggagaaggtgtattgctctgcctgtcttcatgtttttgttccttaggttccaaagctatgtcctttgtttctgctgtgagagactgcgtagacgtattagatatactttccatagttgttttcacatcaattacactttcagatactttcaaacttacagttggcaccttcatatccgattctttattaacagtttcttcgtgcttgccttcagttttaggtgatgaagtacctgctgccagagtttcccctgaaacacacaaagaagagtcttttacttgtgattcagttgtttcaggagttcttgactggccaatgtgcaaggattcatgtaagctgcttttcacttcttcttctggtcgttgtgattttgctggaggttttgataccactggactcttctgaatggtctggacatcagttggcgagagaaaggcactgaagaaattttcagattcatcgaccacagtcctccgaactggctttgtgattgctttaggagaggctattggtggactctgaggttcagtgtttgatttcaacccccaggttgaagtatcccatcctccactgacaggggaacttattcccggctctccatacggaatggtctcggcccagatgctcggctcctcttcctggatgtccagaaccctgtcaatagacttctgggcctgggacagggcctgcttagcgaagctggagagctgggaggcgttgaaccaactcatcgcccctcctcagccggcagtggcggcggcagcaccaagcgggaaggcctcaggcctggggaagggtgcagaggaacggcttcgctccccttttccactcggctggttctgtcagcgtgtggccattaccccgacagcctcccgcgagcccgggatgttaccctcggccgttcccgcacagctgagacgaagggggcccatgtgcgcatgcgcttgcttcttccacgtacacagcaaccaaatctac

SEQ ID NO: 12925 - RNA, 4766 nt, Homo sapiens
  source 1..4766: mol_type = other RNA
gctgggattacaggcatgagccacagcacctggccgtaaatgagagtttttatgtgcaagtaaaggcagttaaataactttcagtaataaaatgcatcacaatatttcacaggtttaaaacacaacctggttacctttttgaataaaataacatttggaagaaggcatagctacttttaaaagctattctatgctttccttgtgtttgaaatttcaagaaaaaataaaatgataaatcacaaaattaaaaatgccaaattcaagttaattcctataattcttccattttgttatgaatattctgtaatatcaaacattcatttttaatgtgctaaaaatatgggtttacaaaatatgaacaggtaatttttaaagagtaaattatgttaagaactttattattttcgattcattttatagggtagtaaaataatacttcttcaaaatcatttaaatgttattgatgccattgcaaaatcattataaataaattttctccattatccaatcacatctagataacattgaatatgtacaggtttctctggataggtaccaaaaggtaccacattttatacagacttaattgtgaaagctgggtgaaataaattttcagatcaaaattttttttaagtttaaatcattcactctttaaatttcagacagtgtcagtgtgactcttacttttaaaggaaaaaaattagtttaaaatttaatagccacagatttaataattttttactttaacacttaatgtacattttcatgagcagtaattaagatatgttgaaattttaaatgtgaaagatttcaaagtttcagtatgttaacattactcttcaaatgttcttaatatatatataaacacttacaaattatagatacaactagttgtatatctacaatacatatatgaacaccattcttcttctctagccatatttatatgaggataaagtaataaatctctgtgctattcaaggaaaaaaaatgaatgctttaaaaaataaatctttaaagaatagtttcaaaaataaagttcaaatattgcacaaaataatttaactgtaaatattactacatagtgtaaaacaattttaaaaaaatttttacactctacagtaaatcccactttctaattctataaaagaatttattggaagtccacattaaatgtttagatattaaatgcttacattcagtttgatgggaattcaattttcacaagttaactgagactttgtcttaaaagttcatctatttgagttttgtacatattttttacatcttcgagatctaatcgaagttcttctgcctcttctgctttttctccatacatctgcagaatagtgttgtacctttgatccaaatctcttagctgagttctaagtttgggtatctccttcaccttctcttcaagttcatcattttgatttgttaatttaactagttcttcagccattattgatcgagttttttctagattgccaatttctagctgtaaatgagtgatttccccttcccttagctttagctgagactgtaggttttcaattatgcttgatcctgctcccatccttacagcatcataaagattgcttccatttgctgatataggcattggtccaaatgagtgatcatgagactcatcctgagacagaaaagatgtctgtagtcctgccatatcaacaccacttattgaacttgagcgtgacatggtgggagtgctagaaacagaaaatggcttgcgttccttttcttttattgtttcttgagtaaaaatggctttcttcctttcttgttcaactttcattctttccatttctaactgactattcaacaatgtcttttctttcctcgtctcttcaagtgttcttacatattcatcttttaggttttccaattcaacctggtacctattgttctcatcctccagtttacacagcctatttttctctgattctagctgggcttgaaatctactgttttcctgtcttaaaagagaattctgtgactccatggaagacatctgaattttgttagcaaggagttcttctgtagctgcacgttctctctcaactgctgctgccagcaaggtctgggattcaccaagcctatcagaaagattcttctctaatttctcccacgacgatgtctgggatcccagggttgcttgcaaattttctatttgtcgaagcaatggtcttgttgttgatgaaacactttgactcagttcctggtttcgattctctgcttcctggagtctctgctgaagttcaccgatctcatggcgtaaataatcctcctttctggcagccgcttgttctgtacgctgcaatgcaagcctaaggtcccccacttgaatggctaatgtttcttgctgctgacgggcttcttcttgggccttctctaatgctgcagaaagttcttctttagctttcatttcacggctcagagcagcttcctgtgcctcactatcctttgcagcattggctttgtgaagatcagtaagttctttgtatgcactatccagggcagcctgaatacttcggttcttttcttcaagttcatccatgtctacctgaagacggccaagatctttctcttggcgttctaccatggaatttagttttttaatattttctctatgttgtttctcaacctcttctttgccatcaaggacctgtttcaaatgctgcaactcctcttctagctctttaacttttttgttcagctttgcaaccatattttcattctccttgtctttagctcttaatttcttgatgatgttagaattgtgcagctgctgttttgaaagtttttctccttcttccattaaccctcggatctgctcatctttctctttcaaaaggtctgcagtttcactactatttaatctagtggcaagttcttcttttatgtttttgatttcctttttagcagcatctctctctttgcaggctagttgaactttcttttctgcttctgcaattctttgagtaaactcatctttcaaggaagaaatgctactgctttcttctttcactctgaacatttcatctttcaggttatcaaaagcttcttctagaagtgctttttccttactaagagataataactgagcctcccttttttccagcttttcattcagaaattcaactgttagagttaccttgcaaacatcttccttctcagaaagtgcttctggctgactttcagcaggttcacactgctcagccaccttgtctaacacagtctgtccttcatttattggtgtggaagaaaccaagatatcaggctgttcacagttaacaggagttgcacttcgtccactttcttccatttctgcttcctcagtgggtataactaatgtttcatttacttcttcagattttccttcagcagattcaactgttttagactttggagttgaagaattaactataataggcactaaagcatatcccttgcctgacaattcatcatctgaattgatttcacttacactccggctatctaatgactgtacactaaatgagtctattctttcaaaagcatcagatgaacagcaactctcagtgagtttttggaaatcatctaaacgattatattcaggacaagcagatgcagagagaagctgaaaagatgtctgcatcaagtgaagacttgattttgaatctgtagtctcttgtctcgagctcgctgagctctcacttattacactttcatgatctaaaacttcaatatcactggtggtagaagtacctgatgaaaaggtactaacaggaggagaaggtgtattgctctgcctgtcttcatgtttttgttccttaggttccaaagctatgtcctttgtttctgctgtgagagactgcgtagacgtattagatatactttccatagttgttttcacatcaattacactttcagatactttcaaacttacagttggcaccttcatatccgattctttattaacagtttcttcgtgcttgccttcagttttaggtgatgaagtacctgctgccagagtttcccctgaaacacacaaagaagagtcttttacttgtgattcagttgtttcaggagttcttgactggccaatgtgcaaggattcatgtaagctgcttttcacttcttcttctggtcgttgtgattttgctggaggttttgataccactggactcttctgaatggtctggacatcagttggcgagagaaaggcactgaagaaattttcagattcatcgaccacagtcctccgaactggctttgtgattgctttaggagaggctattggtggactctgaggttcagtgtttgatttcaacccccaggttgaagtatcccatcctccactgacaggggaacttattcccggctctccatacggaatggtctcggcccagatgctcggctcctcttcctggatgtccagaaccctgtcaatagacttctgggcctgggacagggcctgcttagcgaagctggagagctgggaggcgttgaaccaactcatcgcccctcctcagccggcagtggcggcggcagcaccaagcgggaaggcctcaggcctggggaagggtgcagaggaacggcttcgctccccttttccactcggctggttctgtcagcgtgtggccattaccccgacagcctcccgcgagcccgggatgttaccctcggccgttcccgcacagctgagacgaagggggcccatgtgcgcatgcgcttgcttcttccacgtacacagcaaccaaatctac

SEQ ID NO: 12926 - RNA, 2201 nt, Homo sapiens
  source 1..2201: mol_type = other RNA
gctgggattacaggcatgagccacagcacgcagccctaaatttcattctggttaaattgcacgtttagagtgtccaattagaataatctgtaatccatttccacgtggccatcagttgctaaatcttaaatctgtgtcattggacaagtttttgatttccctaaacccatttgttcttgcgtaaactgaggataatattggcagggattttgtaattagagtaatgctaagatcttagcacagagcctggaacacagaaaaagcccaccaaatggtagctagtatcatttcgtgttatgagttgaaactaattagttctagagtcatcacatctcagaccagaagggaccttcctggtctcccagtccaaccgcgactctccaacacgcagccaagcagtcgtgtctgtgcaggacagcttccaagatactcagcatttgacataaaactcttccattgggactattgccaatagcggtgaggaggagggaaagtggtgtgaaggcatatttgccagaacgggctgtatgaaaatataacctgacttttcttgcacagttggatttctgagcacagaagtgttgcaagttatcctactggaatggaatgtaaactacagtctaaggtgttactttgtgaaaggcactttgaaaacaaaccccctctcatatctcttataaaccacagctgttaaaatccagaggtacccagttaggtagtacagatttctttccaacacaactaataaatgagagactgctctgaaaacctcggcatgcatcacttaagcctgggagctgcacagtgacactcagctggtgcctggcaccagcagagattatcattgaagcattgaaggttacgccaggaatcacaacattgccacctgcattctggctgggaatcacaagcctgccaggaaaagtcgatgcaagccctccatgtccttcctcagtgccaggggctggaggacactgttagggatcagcttcaccccccacctgcaattcgaccttgttcttgagtcattgtcctccccgagcctaaggtgttcactcaccaacaggtgacaattgtgagcacctgccttccctacctgattattaagggctttaatgaatttcattttcataaagtgttttcatatccttgacagaacatttctatcccagtgtaggggaaaagccattatcattattgacctcagagtcaaaagagagatactttttcagccttccttactaataaaattgtagtatcaaatgtttatataatgcttttcatcatagacacaaacacaaaattttaaagttcacaattttggaatatgaatttgctgcattattcaaggttgccagttacagtagagttgctctaatgattccaagtgcagatggccagagctggcctcagattctcagttcattaaacagtccttcctttgaccaacagccctctcattgtaaggccgcctgggtctcagctgatgtcaaaagccccattctaccctgggtggattgttcacataaaggatccccatacatattctgctgcagatagggatggggctggctctgcagatgtcgctgcctccagcactgtcacttttgctcatcacacgatcttgggtctctttccagagacttgcacaaagctcaattcagagtttgcctgtgactgatgcacacttggcctgcagatggacagaggaggaggaaaaggcatcccagtgttcttccccgtttgcctgggaaagcttgggaattcttggcctctttaacagcttcgactcaggctggtgtctgttatgatgtcttatgtattcccaacatttttttcatttctttgaggaacaatatcttgtttccagaaagtgcacattaaaaacaaatctgttgtcaaattgaatggcagtccacaaagtaaatgtcctgtactctggtaactggcccaactcgtcctgtcacccaaaacggggtagatagggatccaaggaagcatggcagagacacgcgcagggtgacagggctgaggtggctctgcacccagctccccctgcagttcccacacacgggcttcccattcatcccggtgattgatgctcctggaagcgcctggaaactctgcctgtgagctaattattatggggaatgacctgcgtcctggtcaggagtgagtagggagatcattaggtgagagct

SEQ ID NO: 12927 - RNA, 3484 nt, Homo sapiens
  source 1..3484: mol_type = other RNA
gctgggattacaggcatgagccacagcactgcgcctggcctttttttttttttttttttttttttttttttttagtagagatggggttttaccatgttggccaggctggtcttgaactcctgacctcaggtgatccacacgcttcagcctcccaaagtgctgggattacaggcgtgagccaccacgcccagcctaaatatttctttatagcaatgcaaggatggcctaacacactgcctaaatcaaaattgctattcacttcaagggtattcattacctgactagcttttttgggtgcatatgaacataatgtaaattttatggctgatcaaatgtcattactatgaagatactccctatgagctcacagagtcaggacatcaacaatatttaaactctcactgtaaacatgacacagtggtaggcactgtggaaatatatttggtcctattttccctacctgagcatgtaaaagagcagactattctaacagtgtgatgactctgcagtgaagaaaagaatccactctcccggcacactgatagagcatgtacctgggcatagtattcctcaaaggagaatggtcataaaaatgatactgcagaattcaaatagcattcaagaggtctccactaaatggggacatgtaggctatctgaagttattatagatttccttatttcaggaatcttcaaggcaaaatatacgatgtgatacatgaaatcatgaaatagccagtaacatacatgatgaaattatcttactagaaagttacacatcaggaaaaaaaaaaaaagagagtttaaaagaaaaaaaaggcaatgggtacaaaactactctatctcaagttggagtgaaaaaatacagcgttagcatttatccatgatagaaaggcagcacagaaaagaactcaagacagaatgaacctgtaaccaggctccttaattagaacataattctaagaccaaagtctgggtagaatctgtacacagaatagtttttatagccattgactgcatgtgttaaaaagtactttgtaacaagagtacaataaatgggaaaaatcttagaggtcatctgaaagcctgatcccaatgctgtcctttgtgggtgagtagtgtcatgttggtatgttgtactcaaactgaagtggcttgaacagctggtcagcacagtgaaaaaggcagccaattaggaatatattgtacatttagttccactggatactttaatatataaactgcatgaactattatatcttatggggactgaacaccccatattatcactttaaaaagtattctaagcttccattttctacaaaaaagaaaaacatcgacttttaaaaagtaaacgtcaagaagcttactttcagatacaatatgagactaaaaaccggatactaattagataaacagtagtgttaacatgatgtaaacagaagaattttaagaaaatttcccttaatttaacaattaagcaaaataataattatgcatttagagttcatatggtaattttcaagtaagtgtgtttattcccccaccacatacaaacccagccttggtgctcacatctctctccaaggatgatcacattgtccccaattactacaggacagtaactttgcctttctcttcaaattgctgattctgactgcttggacaacataaccgtttttggttcttggtctgtgggactgtcagctggtatagctttaacatcaacatttgtaattcctatatttatgttgtgtcttcgcagatcagacttgattaatgctgttaatatgatgcctataaacatccagacacagagaaaaatgttccctgccttaggaccatagtctgatgtgagctttccttgagccaatgtgaacaaaattccaaatatctgtgcagaagcattaagaagaccagatgaagtaccttcagattcagggtaagtgatttcaacagcaaattcaaaacccaaagggaggtaaccagtcatgaagaagccaagcacccctccagtaacaaacacgatgataatatatctaaggtccaatgtgaaagtaaagataaccattccaataaaagacaaaatataaactatcagagtagtctgtttgtatgttttagtataatccagccataagccacaaagaatagagcccaccattccagctactactagcgttagcccaatccttccagcattgacttcttctccctcataatatgtcaatatcatttgatttaataacgttgagactgaataaaaggcaccagtcatgataccataagtgatcaacagaaggacaaaaggaatgtttttaaacaggtttcttattgatttcttataggagtactcttcagggggactgtcttgaagagctgcttgagcctgacttggtggataccgaggtttttctttgaaggcaattgctgttaaaataaataaaagtgtggcaacagctgatgttccataaaacatggtgctgatattacaagccaggagatttgtgtcattctgtgtgttgggtactaaaactggtggtagcaaaaagccaactgcagttccaagctgattgcccagcacggcggtggcacaagctgtggacacctctttgggcccaaaccacactgaggcgatgcgggagggcaagcccaggatgaacacctgggccaccgagcacaagcactggcccaacatggtgacccagaagagatgctgctgcacactgccgcacttgatccaggcacccaggcagttgaggccggagcccagcagggcggtgagccgcaggcctctggtgtccagcagccaggtggccgggaagatgaggggcacgtaggccagcatgtacaccatggacagccagtcgatgtgcagcaaggtgacaccgtagaagccctcgaagacgttgctaatgatgctgtactggatccactgaaaggcgttgaccagcgagtacaggctgaagatcaggagcaccacgaagcgccgcggggagagcgccgtaaggggcagcgggctgctctcggcccccggggtctcagctcccgcgcccgcaggcagcagccgggcctgggtctcctcttctggggccagtggagtctgaggcccgcccagaactcccgaggcggcagcgaggctgtcccggggggccccattcaccgggaaggtgcccgctttgggcccgttctgcagctccacgctctccttcccaacgggcgcgcccctcggcaacgggaggtatcctttcgcgagcgggtgtccgggcgccaccgccgccccctcctcatcgtctggccgcgccatatcccaggctccccggcgccacctcgctcccccgccccactccccgactccgctctcccggcccacagcccgaggtcctcctggggccccacctccaacccctcggcccaccgctccttccccggtggcgcgcgccgcgaaccgcaatccgcgctaccgcgtgaacagatgaaggtct

SEQ ID NO: 12928 - RNA, 3659 nt, Homo sapiens
  source 1..3659: mol_type = other RNA
gctgggattacaggcatgagccacagcatctggctccttagaataatttttaactaatttctgtttattccctgtattcatccagtcactaaatcttatcagatctcctttgatatgcctcttgaatctgtgtattaaccccatgctgactgtgatcatcctggacaggatcctggaaacctactgtgaggagatatcttatctcacatgttctctttaaagcaactcatttgatccttgtcaaacccctgtaagacagggagaggaggcgctgatgtaaaaatggtcctattttataactggagaaattgaggaacagagacataaaggatagtgctcaaagtcatgataaaagcaaactgctcaaggggggtatgatgagatatcctccattgcccagcgatatctattctcctgagtcctttaatttgcaataaagctttcctcagatcaatttctcatccagggcttttatacttatgaactagaatacaaagtatagttcctaatcttacaattttaggaccagctataccccttgccctaataagattttaatctctgtgttgctataaatacctgaggctgtgaaatttataaagaaaagagggtttatttggttcactcttcagcaggctatatacaaaagaagcatggcaccagcatctgcttagcttctagtgagggctcaggaaacttagaatcatggcagaaggcaaagggcgagcaggcgagtcacacagtgagagagagcttagcagttttcaaatttttaagtctcaggatccctttatattcttaaaaattgagagcctcaaagagcctttgtttatttggtctgttactattagtatctcccatactagacattaaaactaaaaaaaaaaaaattaaatagttctccactaatttaaaaataaaaaataaataaaagtgaaacttctatgaaaaatctattttccgaaatgagaagagtggcattgttttgtattttcaaatgtctttccatatctggcttactagaaaatagttgagttgtcatatctggctctgtatttaatctgctgtgatatgttgttttgactgaagtatgttctgggaaaccagaatatgctaccccaaaataggaaggattgttctactgaaggtagttttgaaggagcagatgcaagaaacctctctgccttccacttgcctaaatcaagacatagatttgcaaagacaaaaggtatcctgcccacctctctactaggagaaacaaaggttaaccactgaagacaactttagcctggaaaagaatctgtgttaataagcttcaccaactagcctctacccgccatattgatttgcccttccaaaatttactacggctacagattcaaagtccttttcctcagtcttgtattctctaaaaacttactgttctttgttgaaaatgctctattcaaagccaccttgaaaactactaattccatgggtgtctcccatgtatatataaaatatacatgtcaataaacttctgtcttttgttataggtatccatatccaatgaagaatctatgagggttgaaaaaaagtatttttcccctatggtatgaagattatctggcattacacagttatgcagttgaaaaagaaaacagtaattcaattgctttttaccatacctatggaaactgttcttttacactaggccaaaattaacaggtgatagtttcctaaaagttagttacaatgtaaaatctaaaattggtctctcttggacagtaaatgaaattttcactcatgcataattttgtaacataatgaatgggtcatgtggaaaatactggttcaccgagttttattttgtgtgtacagtacttcccgtttcatcatacagaatattcaaagacatgtactagagtattgaggcttaataaaattatttttattgcttcaagaacattcctaagtgaaactaactagctttttaaaaaaactacaggcatgtagaaataacatatagaatattattagtaaggtttcatgtaattgccttcattcattctaaggagccagaacttttactccttactccttatcatcagtggaaatgtcaacacattgaaaaaggtaaataacttcttagtattactagcaacacagatttgaccttgaagaaagggacactgaaaggaaccagggactcccagaggtacacagaccacacgatgagaactaccattgtaggctgttggctagtatataaagaaagagtacataaagctgcacaacacttggcatgtgtttttgacaatctggggaaaaaaacaaagatccatgacctatcataatttataaattctgctgactcatgaatctgaatggcaggttctacaaggctgctgtttggaagctagtaaccagtcagaaatggcattttatcctaatttcatcaggtaaatgctggaaacaatgtagaatgcttattaaaacgtcacctactaatgttgatctgaagaagtcaattaaaaatatctgttggaagaaaatacatgttacatggaaagaagtaaagaaaaatctgttatagtgataatcattaatttaggattttgcaaagacctcaggacaattccctcagcactgttaagaatctgtggctgggcaaagctcattcacttattttctcatttcttgcactctagaacctaccacaagtcatctatagtcccattttgataaagtgaatcaagacaaagagctaaaaccaaatgataggttactcatggtctcccaaagggctgatagagcactatgatgctcatccattgatatctactcaattatttataatctttcctgccaaagtagctcatttcaaatgctcagtgttggcaaatattaaaatacagtagccttccattatcggtgggttcatgttccacagtttcagttacccgtagtcagctgtagtccaaaaatattatatgaaaattccagaaataaacaattcttaagttttaaactgcacgccattctgagtagcatgatgaaatcttgcactgtccccatgaggatgtgaatcatgcctttgtccagtgtatccatgctatataccttatctacctgtaagtcacctagtagccatctgggttatcagattaactgttaaggtatcacaatgcttgtgttcaaggtcagtagtagcctaatactacatcacaatgcttacaatgcctacattattcaccttacttcatctcataatttcacatcaacacaagaagggtgagtacagtgccacattcacattaactgacattatgctatactgttataattgttctatcttgttgttctcttattgtgcctaatttataatttaaactttatcatagggatgtatgtatgtataggaaaaaacaatgcatacagggttcagtactatctgcagttttagacatccactgggaatgctggaatgtattccctaaagataagggtagactacagtataaacatcccaagaggctcttctgatactagttataaggcatcagcagtggcagcaatgtgagtagtattagtgattatttgaaccatcaatttacatgcataccatatgttacagatttccaagaacaggttgagtatccctaattcaaaaatccaaa

SEQ ID NO: 12929 - RNA, 2872 nt, Homo sapiens
  source 1..2872: mol_type = other RNA
gctgggattacaggcatgagccacagcgcacccagcctttgttagctatttctactgggactttaaagtattatattttatcatatttcttattacttcaatagtacctgggaacttgtctcaaacatgagacccagcttttttccagagatggtacctactggagaattctagattgaagtaagaaaggaaattaggatataaaacaaggaggattggctgaagcttagcttcagaaaaagagaggtctaatatctccctgggacaatagagaaactagtagctcaattaagtatttaaaaccatgattttataactgactgattacagtaacatgtatggcctatggcaaaaataagcttctcattgtttcctaatgttcatactgcattgatatcaatacttgtccattttaactcttacagcagaacagatctttgttgcatgtactctatcttagagtatcacagatagagtaaaaaatacctatgcaccctcacatattttgaatccttgtattacagatttttctttcactttaaactgacctcagaagctataattgttggaccataattgattcttaaacgttttctaaaaatattgttattttagtgtttctcaatgatgaatacatgtcaaatgtagaaaatcaaagctaaacccctcagttatctcgaactcatgcaacatgaattctcatcgattatcttgttttatcaataaggaaagaaatgggatcttgttatgcaggagtaatccgttccaatgtgatgttctgatgtctgaggagcacgtctgcctttcagaacagatcctgcactctgctagtgcatttctccagcactccacggggcttttacccaacaatgcagcttcacacacagacaccacactggtatatggcacaagctggcctaatatgcagggaaaggatggtctctacccacacagccagacagtgctttctactttattaaacatcaaagcccaaatagatgttccctgtggaggaggacttaaggacactaggggaggagaaagggacacctgggaagagaatcacaccacagagaccaatcttcacaaaaagggtccaacattgatttctagggaggagcagggcatggtcagctcaaatttggtgataacgtcaggatgaaggaccccaagcttcccgacgctttgacccctggcaaagatctctgcacatcgcccggggaagaaagcaggcccttctgatgctttgatcacatatccccccttgtcttcaccaggaggcacatcgagcaactgcataattctgtccagcagcccatgaatgatctcaaacccaggattcttgttgtaataaacagcacagagatgtctgtagttttttgcacctacatctgtattagaatcttttattacaatgtcagagatttcaaacagtttcagtggaaggggcatcttacgatttgctgctatggtcttcaggaggccaggaagaagggtagtgcgtgccacctgaaattcagctgttttaggattacttatgtggactgcctttgttgcagagatatccacacctagtttatcagcaatatcttcttgggagcacagggcaaaggtaagtgcttcagtgaagccagcggctgccatgtcatgtcggagaagttcagtgagcttattaagaggaaattgattagctatggtgtaagttttcgggagagtcatctgaatgttgttatatccataagcaatagctgcatcttctacaatatcacatgcatggataatgtcagctctggttggagggatttcaatctcaatctgattcccatcacctatgacttctgattttaaatacatcctggtcagaagtttggcaagattttctggagtttctctgattccaacttttttgttaattaggtcagctctcaccatctcctttcggtaagctaattctggaaaggtatgtgattttccattaggaaaaaccacttcagcagcttcgaccgtaaattgattctcacaatattcactgaacatggtgacaataatatcaagaactatttttgccttagtaaagtcagttcccgtgcattcaataaaaatatttctagtatttactgttattctggaatgatccccattgatgatgggaggcattgaaaggacgacaccattgctatcatagataactggatacaggggtttgttttcaatgatatgtaaataatgtttcaggtgattgtcagtcttgtatatgttcatcagttcacaggctgtatactccttggtcttatttagaggcttgaatttgatatctgaaggacgctttgcagtataagtaaatgggcccgacaaagtgtccaaatcatgggtaccaatggcaaccagtgctcttttcctgcaaatattctgatgtaatttctcctgaagttcaatgaagctgtcatatcgatctttagtaaactttatattacggagaactgctgctaccgcaaaaggacgtatcttagctgtctcttctgtgataatcaatttctggatttttccatcaggcattacccgtttatacactggagcctttatcctttctttgaagacctgaagtcctcgaaccaatccttccagacacaggagatcatatctattggcagggacgtcaattttgtaaagaacaacatcagaggctcctgctgcctttacattaccttgttctttacttattatttccttctcagatgtaatttcatcaagctccagaccaaattcaaaacatagttcatcaaattcttcgtcagtgtaggtgcggcccagggcttggaagagcagatcacgcttcacgctgacagtcggcatggtgtgtcgaactcactgc

SEQ ID NO: 12930 - RNA, 3068 nt, Homo sapiens
  source 1..3068: mol_type = other RNA
gctgggattacaggcatgagccacagcgcacccagcctttgttagctatttctactgggactttaaagtattatattttatcatatttcttattacttcaatagtacctgggaacttgtctcaaacatgagacccagcttttttccagagatggtacctactggagaattctagattgaagtaagaaaggaaattaggatataaaacaaggaggattggctgaagcttagcttcagaaaaagagaggtctaatatctccctgggacaatagagaaactagtagctcaattaagtatttaaaaccatgattttataactgactgattacagtaacatgtatggcctatggcaaaaataagcttctcattgtttcctaatgttcatactgcattgatatcaatacttgtccattttaactcttacagcagaacagatctttgttgcatgtactctatcttagagtatcacagatagagtaaaaaatacctatgcaccctcacatattttgaatccttgtattacagatttttctttcactttaaactgacctcagaagctataattgttggaccataattgattcttaaacgttttctaaaaatattgttattttagtgtttctcaatgatgaatacatgtcaaatgtagaaaatcaaagctaaacccctcagttatctcgaactcatgcaacatgaattctcatcgattatcttgttttatcaataaggaaagaaatgggatcttgttatgcaggagtaatccgttccaatgtgatgttctgatgtctgaggagcacgtctgcctttcagaacagatcctgcactctgctagtgcatttctccagcactccacggggcttttacccaacaatgcagcttcacacacagacaccacactggtatatggcacaagctggcctaatatgcagggaaaggatggtctctacccacacagccagacagtgctttctactttattaaacatcaaagcccaaatagatgttccctgtggaggaggacttaaggacactaggggaggagaaagggacacctgggaagagaatcacaccacagagaccaatcttcacaaaaagggtccaacattgatttctagggaggagcagggcatggtcagctcaaatttggtgataacgtcaggatgaaggaccccaagcttcccgacgctttgacccctggcaaagatctctgcacatcgcccggggaagaaagcaggcccttctgatgctttgatcacatatccccccttgtcttcaccaggaggcacatcgagcaactgcataattctgtccagcagcccatgaatgatctcaaacccaggattcttgttgtaataaacagcacagagatgtctgtagttttttgcacctacatctgtattagaatcttttattacaatgtcagagatttcaaacagtttcagtggaaggggcatcttacgatttgctgctatggtcttcaggaggccaggaagaagggtagtgcgtgccacctgaaattcagctgttttaggattacttatgtggactgcctttgttgcagagatatccacacctagtttatcagcaatatcttcttgggagcacagggcaaaggtaagtgcttcagtgaagccagcggctgccatgtcatgtcggagaagttcagtgagcttattaagaggaaattgattagctatggtgtaagttttcgggagagtcatctgaatgttgttatatccataagcaatagctgcatcttctacaatatcacatgcatggataatgtcagctctggttggagggatttcaatctcaatctgattcccatcacctatgacttctgattttaaatacatcctggtcagaagtttggcaagattttctggagtttctctgattccaacttttttgttaattaggtcagctctcaccatctcctttcggtaagctaattctggaaaggtatgtgattttccattaggaaaaaccacttcagcagcttcgaccgtaaattgattctcacaatattcactgaacatggtgacaataatatcaagaactatttttgccttagtaaagtcagttcccgtgcattcaataaaaatatttctagtatttactgttattctggaatgatccccattgatgatgggaggcattgaaaggacgacaccattgctatcatagataactggatacaggggtttgttttcaatgatatgtaaataatgtttcaggtgattgtcagtcttgtatatgttcatcagttcacaggctgtatactccttggtcttatttagaggcttgaatttgatatctgaaggacgctttgcagtataagtaaatgggcccgacaaagtgtccaaatcatgggtaccaatggcaaccagtgctcttttcctgcaaatattctgatgtaatttctcctgaagttcaatgaagctgtcatatcgatctttagtaaactttatattacggagaactgctgctaccgcaaaaggacgtatcttagctgtctcttctgtgataatcaatttctggatttttccatcaggcattacccgtttatacactggagcctttatcctttctttgaagacctgaagtcctcgaaccaatccttccagacacaggagatcatatctattggcagggacgtcaattttgtaaagaacaacatcagaggctcctgctgcctttacattaccttgttctttacttattatttccttctcagatgtctttttcttcagttccagtgattttctggtttgtatagttatgactttttcaattagttccactctctccttccacggtgcattgtattgctccagttttttcctgataggaggcagccttctttatgggccaaacacagcgatgctggtgatcagtggacaaactgcaccttggacataaaagctctaggtctttaatttcatcaagctccagaccaaattcaaaacatagttcatcaaattcttcgtcagtgtaggtgcggcccagggcttggaagagcagatcacgcttcacgctgacagtcggcatggtgtgtcgaactcactgc

SEQ ID NO: 12931 - RNA, 506 nt, Homo sapiens
  source 1..506: mol_type = other RNA
gctgggattacaggcatgagccacagcgccaagccaaaaatgtcggtgaattttcagagactagatccattcagtgaacacagccagggctagttctggagcttagaagtccaaatcaggtggtggtagggttgcttccttctgagcactctgaatcttttccgtgcgtttttccttgcttctgatggttcctggaaatctttcacatttcttggcatcactccagtctctgccttcatattcacatgcccttacaaaacttactctctgttgctaggagcgtgtttgctaaggaaatgcttgctaaagatatttttaagagcatttctcttaaaggcattaatgttcaagatattgtcacagataagttttggtaccaatgcaattaccaagagtgttgatgttatggccctgttgcaaaggaaacttgttgttaagggtgttgcaagactcttgtgttaatatcgttgtaaagaaagttgttgttaaggatgctgttcctaact

SEQ ID NO: 12932 - RNA, 3158 nt, Homo sapiens
  source 1..3158: mol_type = other RNA
gctgggattacaggcatgagccacagcgcccggccaattagtcttttgataagggttctataaggcctaatcatctgcattattactcatttaattgtatattacttcctggccaggcacagtggctcacacctctaatcccagcactttgaggggccaagatgggcagatcacttgaggtcaggagttcgagaccagcctggccgatacggtggaactctctccattaaaaacaaaaattagcggccaggcacggtggctcacgcctgtaatcccagcatttgggaggccaaggcaggcggatcacgaggtcaagagattgagacaatcctggcaaacatggtgaaaccccgtctctactaaaaatacaaaaattagctgggcatggtgacacgtgcctgtaatcccagctactcaggaggctgaggcaggagaatcacttgaacccgggaggcagaggttgcagtgagccgcgattgcgccactgcactccagcctggcgacagagagagactccatctcaagaaaaaaaaaaaaaaaattagctgggcgtggtggtgggcgcccgtaatcccagctacttgggagcttaaggctcgagaatcacttgaatccaggaggtggaggttgcagtgagctgacattgcaacaccactctagcctggcaaaagagtaagactccatctcaaaaaaaccccacaaaatttatattacttcctttttcagttttccctcgtaaaacttgtgaagtcattacatgtcagcaccaatttcattattaataaacaaaaaatatactctagttggaattaaactctcatcatcaatgtagttagacccatgcaattaatacctaatgccccttttctccactaactaatatggcatctaatttataataaaatattttaagtctcctgttatatttaaattgcatcaaatttaaattatgttaattataagactggcatgccaagccaaattatcacagaagattacatgaacaagcaatgttagtgatagatgctttttgttatccatcaaataattactaagttttctttttaaaaaaaatcagtgtttatgggcacacaattaaataccatttagaaaatccttaacttaggaccaggtcactggcttagttaaagtatatttatatttgatagtttccaaggtaaggttaccattggggaaattgtgataattaagtcaaacagttgtaccactgacctaaccagtacattaaggatttctaaatgtatcttattgtgtatttagcataagtggccatgctaatattatcaataccaaactgcagacaagattagttaagaactatgcagaaaacctgagcatcctacctttactttctatacattcgcattaccaattttttcttttcaaaacatcccttgcatcaagtgctactttctaacagctcttaagattctctgttcaccagaacaagcaacattaaagataacattggttcccatgttatatattcattactaatagcacttatcaaagctaaacctagataatattccttctttcctgacatactgctcagtggcaagtacacttcttctcaaccagcataggaaacctttcctttgggtcatttcccttctcaaaaaactttgcttaagggaaattggagctaaagagcttaccaacaaatagccctactagagttcaataaatatgctttgctattaagtctaatatacaaatatgatagaagtttgaaaatggaaccttatcccagtgctatattggcacgtaacatggctagtgatcatttcaaaaggagtcatgttatgttttgagtttgtttgtgataaacctattgtctaaacagatttattctttaagaatatacacaagaggttttcctccattattttcacacatcagatatggtgtttggttttttgaaggagggagggggtactatctacaacaaatacttcattcatagccataaaccatttgtatcttgggcttgagcccctggttaaatcaggaatgctcttcagcgctgctgctgaatgatctgctccggatgtgatttctcagttgctctataagttcaggattttgttgctgtatctgctgagcaaactgctgtcccgcttggatgaggcttgacaggtcagttaggcccccaactccagcagcaggtcccccaatggcatttgtcatcattcctgacattagctgttgaacttgagggttctgcattaaacttgccgccatactaatgaaggctggattatttatcaagctagccatgtcaaagctcagtccagttcctgtaggactggatacctctcttaacttctgttctgctattttcagatttgacttataggaatcattttcagggtcaagatctaatgccttttgataacttgtaactgcttcttcaaatttattcaaggcagtgagggccagccccattctcccataggccttgctgtactttgaatcaattgctattgctttttcacaatcctttatcgcatctgtgtagtgacctaatttgctctgagcagcagccctgttgcaatagtaaactgcattattgggatccaattctattgcctgtgtgtaacaatccactgcagcagcataattttcttctttcatgtggttattgccttcatcttttaattggtcagcttttcccacatcttcaggcactgagtttgaaaggggcagaacgtcattcttacagaaggaactggtaaacatttctgtcaaaggctgtgaaactgctaggtgtgtatcttctgggctgatcttaaaaactgtctccaagcactgaattgcaacttccaaactttcttgttcatccgaggtgtaagtgtccatctgactttgttcccgtaagaaacgaataactgcataaaccaggtgcttgatagatgacattttagaagcttaaacacttttccaagcaggaggacgcgagacgactgctgctggcccgcggggttccgtaggcaggcccgcccgacccctggtcctcggggctggagcccggctcgggatcgcagcactggtcgcggcggcgcaaacttccccggcccctaggccgtagaccccagaacccaccaggctgtgctctctctcaggcggcagggtct

SEQ ID NO: 12933 - RNA, 3030 nt, Homo sapiens
  source 1..3030: mol_type = other RNA
gctgggattacaggcatgagccacagcgcccggccaattagtcttttgataagggttctataaggcctaatcatctgcattattactcatttaattgtatattacttcctggccaggcacagtggctcacacctctaatcccagcactttgaggggccaagatgggcagatcacttgaggtcaggagttcgagaccagcctggccgatacggtggaactctctccattaaaaacaaaaattagcggccaggcacggtggctcacgcctgtaatcccagcatttgggaggccaaggcaggcggatcacgaggtcaagagattgagacaatcctggcaaacatggtgaaaccccgtctctactaaaaatacaaaaattagctgggcatggtgacacgtgcctgtaatcccagctactcaggaggctgaggcaggagaatcacttgaacccgggaggcagaggttgcagtgagccgcgattgcgccactgcactccagcctggcgacagagagagactccatctcaagaaaaaaaaaaaaaaaattagctgggcgtggtggtgggcgcccgtaatcccagctacttgggagcttaaggctcgagaatcacttgaatccaggaggtggaggttgcagtgagctgacattgcaacaccactctagcctggcaaaagagtaagactccatctcaaaaaaaccccacaaaatttatattacttcctttttcagttttccctcgtaaaacttgtgaagtcattacatgtcagcaccaatttcattattaataaacaaaaaatatactctagttggaattaaactctcatcatcaatgtagttagacccatgcaattaatacctaatgccccttttctccactaactaatatggcatctaatttataataaaatattttaagtctcctgttatatttaaattgcatcaaatttaaattatgttaattataagactggcatgccaagccaaattatcacagaagattacatgaacaagcaatgttagtgatagatgctttttgttatccatcaaataattactaagttttctttttaaaaaaaatcagtgtttatgggcacacaattaaataccatttagaaaatccttaacttaggaccaggtcactggcttagttaaagtatatttatatttgatagtttccaaggtaaggttaccattggggaaattgtgataattaagtcaaacagttgtaccactgacctaaccagtacattaaggatttctaaatgtatcttattgtgtatttagcataagtggccatgctaatattatcaataccaaactgcagacaagattagttaagaactatgcagaaaacctgagcatcctacctttactttctatacattcgcattaccaattttttcttttcaaaacatcccttgcatcaagtgctactttctaacagctcttaagattctctgttcaccagaacaagcaacattaaagataacattggttcccatgttatatattcattactaatagcacttatcaaagctaaacctagataatattccttctttcctgacatactgctcagtggcaagtacacttcttctcaaccagcataggaaacctttcctttgggtcatttcccttctcaaaaaactttgcttaagggaaattggagctaaagagcttaccaacaaatagccctactagagttcaataaatatgctttgctattaagtctaatatacaaatatgatagaagtttgaaaatggaaccttatcccagtgctatattggcacgtaacatggctagtgatcatttcaaaaggagtcatgttatgttttgagtttgtttgtgataaacctattgtctaaacagatttattctttaagaatatacacaagaggttttcctccattattttcacacatcagatatggtgtttggttttttgaaggagggagggggtactatctacaacaaatacttcattcatagccataaaccatttgtatcttgggcttgagcccctggttaaatcaggaatgctcttcagcgctgctgctgaatgatctgctccggatgtgatttctcagttgctctataagttcaggattttgttgctgtatctgctgagcaaactgctgtcccgcttggatgaggcttgacaggtcagttaggcccccaactccagcagcaggtcccccaatggcatttgtcatcattcctgacattagctgttgaacttgagggttctgcattaaacttgccgccatactaatgaaggctggattatttatcaagctagccatgtcaaagctcagtccagttcctgtaggactggatacctctcttaacttctgttctgctattttcagatttgacttataggaatcattttcagggtcaagatctaatgccttttgataacttgtaactgcttcttcaaatttattcaaggcagtgagggccagccccattctcccataggccttgctgtactttgaatcaattgctattgctttttcacaatcctttatcgcatctgtgtagtgacctaatttgctctgagcagcagccctgttgcaatagtaaactgcattattgggatccaattctattgcctgtgtgtaacaatccactgcagcagcataattttcttctttcatgtggttattgccttcatcttttaattggtcagcttttcccacatcttcaggcactgagtttgaaaggggcagaacgtcattcttacagaaggaactggtaaacatttctgtcaaaggctgtgaaactgctaggtgtgtatcttctgggctgatcttaaaaactgtctccaagcactgaattgcaacttccaaactttcttgttcatccgaggtgtaagtgtccatctgactttgttcccgtaagaaacgaataactgcataaaccaggtgcttgatagatgacattttagaagcttaaacacttttcctgtcattaaaagtgccgcagctgtggactcagaacaattgtgtttgctcctcgcgcccattatt

SEQ ID NO: 12934 - RNA, 3299 nt, Homo sapiens
  source 1..3299: mol_type = other RNA
gctgggattacaggcatgagccacagcgcccggccaattagtcttttgataagggttctataaggcctaatcatctgcattattactcatttaattgtatattacttcctggccaggcacagtggctcacacctctaatcccagcactttgaggggccaagatgggcagatcacttgaggtcaggagttcgagaccagcctggccgatacggtggaactctctccattaaaaacaaaaattagcggccaggcacggtggctcacgcctgtaatcccagcatttgggaggccaaggcaggcggatcacgaggtcaagagattgagacaatcctggcaaacatggtgaaaccccgtctctactaaaaatacaaaaattagctgggcatggtgacacgtgcctgtaatcccagctactcaggaggctgaggcaggagaatcacttgaacccgggaggcagaggttgcagtgagccgcgattgcgccactgcactccagcctggcgacagagagagactccatctcaagaaaaaaaaaaaaaaaattagctgggcgtggtggtgggcgcccgtaatcccagctacttgggagcttaaggctcgagaatcacttgaatccaggaggtggaggttgcagtgagctgacattgcaacaccactctagcctggcaaaagagtaagactccatctcaaaaaaaccccacaaaatttatattacttcctttttcagttttccctcgtaaaacttgtgaagtcattacatgtcagcaccaatttcattattaataaacaaaaaatatactctagttggaattaaactctcatcatcaatgtagttagacccatgcaattaatacctaatgccccttttctccactaactaatatggcatctaatttataataaaatattttaagtctcctgttatatttaaattgcatcaaatttaaattatgttaattataagactggcatgccaagccaaattatcacagaagattacatgaacaagcaatgttagtgatagatgctttttgttatccatcaaataattactaagttttctttttaaaaaaaatcagtgtttatgggcacacaattaaataccatttagaaaatccttaacttaggaccaggtcactggcttagttaaagtatatttatatttgatagtttccaaggtaaggttaccattggggaaattgtgataattaagtcaaacagttgtaccactgacctaaccagtacattaaggatttctaaatgtatcttattgtgtatttagcataagtggccatgctaatattatcaataccaaactgcagacaagattagttaagaactatgcagaaaacctgagcatcctacctttactttctatacattcgcattaccaattttttcttttcaaaacatcccttgcatcaagtgctactttctaacagctcttaagattctctgttcaccagaacaagcaacattaaagataacattggttcccatgttatatattcattactaatagcacttatcaaagctaaacctagataatattccttctttcctgacatactgctcagtggcaagtacacttcttctcaaccagcataggaaacctttcctttgggtcatttcccttctcaaaaaactttgcttaagggaaattggagctaaagagcttaccaacaaatagccctactagagttcaataaatatgctttgctattaagtctaatatacaaatatgatagaagtttgaaaatggaaccttatcccagtgctatattggcacgtaacatggctagtgatcatttcaaaaggagtcatgttatgttttgagtttgtttgtgataaacctattgtctaaacagatttattctttaagaatatacacaagaggttttcctccattattttcacacatcagatatggtgtttggttttttgaaggagggagggggtactatctacaacaaatacttcattcatagccataaaccatttgtatcttgggcttgagcccctggttaaatcaggaatgctcttcagcgctgctgctgaatgatctgctccggatgtgatttctcagttgctctataagttcaggattttgttgctgtatctgctgagcaaactgctgtcccgcttggatgaggcttgacaggtcagttaggcccccaactccagcagcaggtcccccaatggcatttgtcatcattcctgacattagctgttgaacttgagggttctgcattaaacttgccgccatactaatgaaggctggattatttatcaagctagccatgtcaaagctcagtccagttcctgtaggactggatacctctcttaacttctgttctgctattttcagatttgacttataggaatcattttcagggtcaagatctaatgccttttgataacttgtaactgcttcttcaaatttattcaaggcagtgagggccagccccattctcccataggccttgctgtactttgaatcaattgctattgctttttcacaatcctttatcgcatctgtgtagtgacctaatttgctctgagcagcagccctgttgcaatagtaaactgcattattgggatccaattctattgcctgtgtgtaacaatccactgcagcagcataattttcttctttcatgtggttattgccttccttatcttcatctctctcctcccttttagagctgccccagcccgttccagatgcaacaccctccctaatcaccatctcaatctggacctggtcttccactctttcccttcatcttttaattggtcagcttttcccacatcttcaggcactgagtttgaaaggggcagaacgtcattcttacagaaggaactggtaaacatttctgtcaaaggctgtgaaactgctaggtgtgtatcttctgggctgatcttaaaaactgtctccaagcactgaattgcaacttccaaactttcttgttcatccgaggtgtaagtgtccatctgactttgttcccgtaagaaacgaataactgcataaaccaggtgcttgatagatgacattttagaagcttaaacacttttccaagcaggaggacgcgagacgactgctgctggcccgcggggttccgtaggcaggcccgcccgacccctggtcctcggggctggagcccggctcgggatcgcagcactggtcgcggcggcgcaaacttccccggcccctaggccgtagaccccagaacccaccaggctgtgctctctctcaggcggcagggtctggccagcaccgcccctggggcggggccggac

SEQ ID NO: 12935 - RNA, 844 nt, Homo sapiens
  source 1..844: mol_type = other RNA
gctgggattacaggcatgagccacagcgcccggccagcctttgcctttttaatctctccctgtttctgcttctctgccccattttgtcctgtgtgtttctgccctctggcaatctctctcttgtcccttggcctcccgctggccatggcttgttttgtggcctgggcagaaggtgctgtatcaggcagggtcacgacgggaaacgaagtttacccccaactggttcaagtgaagagacctcgtgatgtattagtgaggacccaaggacaaaatgtctgggaggccaaaagcatctctcagacagtctctacaggactcttccaggtcccggaagcccgagcgagcttcctggaggaggtggctggggagagtggaggagccggtaggggtcgctgtgcttgcgcgcgcccgtccaggaactcgccggggctgtggggagggggcgccggcccattcctcctgatctgggcagcctccgggccccaactccagccagccgacccctttcctccactttcgggggtctctctgggacagatgtggctttagaggaagcctttgcaaagtggcagctttggggcgggtttgggattctggaagcttctgagcatagtgtgagtgtgtgcgaggggatgggggaaggcccagcatgtggaaaagtcattttcatgcttgagttgggagcagacagagatcaggggagacgagggagtcctcgctttcggagggggtgtaaagtaaactaaccagggaggagcctcccacagccactctggtctgagacagcgcctgcccagaatccctctccacagctcttctaacaactgaggatccctggggccag

SEQ ID NO: 12936 - RNA, 1280 nt, Homo sapiens
  source 1..1280: mol_type = other RNA
gctgggattacaggcatgagccacagcgcccggcctacagcaaaacttatggaaagaatggtcagttatctgtctccactttctcttctctcattatctgtgagcacattttaattaggcttttgcccacatcgctctgctgaaactgctcttttcaaagtagtcagtgactttcatattaaattaaacggtcatttctcaggccttactcttcacttatcattgtattggttatctgttgctatgtaacaattaccctcaaatttagtgactcgaaacaagaagcaattatctcatagtttctatgggtcagaaatccaggaatagcttagctatgtgattctggattaggttctcttatgaagtttcattcaaggtgttggcaggggttgtagtcatgtcaagtcttagaaggttggaggatccacttccaatatactcactcacatgtctggcaaattagtgtttgtttttgatagtaggccttagttcttcaccatgtagacctcttcataaggttgcttgagcatcctcacaatatggcaactggcttctcctccagcaatcccaagtggattcccacagcactttgataccacctccaagtggccacttcctggaactctcacaatgtgtccatgtttgtttcctccaccagagcaaagtttctttttcccttccttctggggtttcttttaccagtctcttgacccgagtgtgagtgtccaccccgttcagctgttcctacggctgtctcagtgatcacgagcacttgataggaaccttcccagcttgggtggagattgtcttccttccaagtcttaattagcaccaagtcgccaggctggaagtggtgacagtcccattttcccaccgtggttcgtgcacgaggttgtctggttgccgcggtgcctgcttttcttcctgtgtcacttttgttatctcctgaatcatggtctccggtttgtctgtggcttctgtggggagccgggacatccagacagagcgggccacataaatcaagtggggcacgtctcccctctccatgcaggcacagagatccccgtatggccaccagattgtgaaaaacaaactcacccttccaaacccaaagaatggattcagagactcggagaacagcaaaagtgagacttttaatggtggtcttgcaagattgggtgtctgataggcaggcacgcccagtatagttttgtttgtttgtttgtttgcttttggagacagagtcttgctctgtcacccaggcttgagtgcagtggcac

SEQ ID NO: 12937 - RNA, 2683 nt, Homo sapiens
  source 1..2683: mol_type = other RNA
gctgggattacaggcatgagccacagcgcccggcctacagcaaaacttatggaaagaatggtcagttatctgtctccactttctcttctctcattatctgtgagcacattttaattaggcttttgcccacatcgctctgctgaaactgctcttttcaaagtagtcagtgactttcatattaaattaaacggtcatttctcaggccttactcttcacttatcattgtattggttatctgttgctatgtaacaattaccctcaaatttagtgactcgaaacaagaagcaattatctcatagtttctatgggtcagaaatccaggaatagcttagctatgtgattctggattaggttctcttatgaagtttcattcaaggtgttggcaggggttgtagtcatgtcaagtcttagaaggttggaggatccacttccaatatactcactcacatgtctggcaaattagtgtttgtttttgatagtaggccttagttcttcaccatgtagacctcttcataaggttgcttgagcatcctcacaatatggcaactggcttctcctctccaagtggccagctcctggtactatcacaatgtgtccatgtttgtctcctccaccagagcaaagttcctgaaagtaataacagagtctctttcacagagtgggtgggaagattaaatgagacaacgtattcaaaagatctagcaaattgcctggaatatattagttgcttaataactcttactattattattataccatttttcagatgaaaaaacaccagtgatgtggctggactccagggtgaatggccatgtcagaccccagagatgctgcatccttaaccttattctcccagcctcaaagattccctaggcatggcaggctatgaagcagagacacgaatcaaggtgatgagggctggggcattaaatggtaacctggatggacagtagactaggaggctcctctaatgccatatcactgcaggagtcgcagaacgttggcacaattcagggaagtccccctaagttgaattgacagccattttgatgggatagagactaaaggttgaagttaatttgatttccagaatatgaagaaattagatgttttgggcatgtataagtttatgaactgagattcaaactcacaatatcaatagtacaaagcactgtgtaataaagccaagcaatcagcgcaatggcttttcctggaattcagaggagagagatcattgagagcaatcaagaaaggtttcctggaggatgggacctggaacaataatagtactactaataactatttatggagggcttgattctttatatattattgatatggtttggctgtatccccacccaaatctcatcttgtagtttccataatccccacctgtcgtgggagggacccagtgggaggtaattgaatcgtgggggtagttacctccatgctgttctcatgatagtgagttctcacgagatatgatggttttaaaaggggcttttcccttttcactcattcttcttctccctgctgccatgtgaagaaggacacgtttgcttccctttctgccatgatagtaagtttcctgagacctccccagccatgctgaattgagtcaattaaacctctttcctttataaattacccagtctcgtgtatgtattcacagcagcaaaaaatggactaatacaattacttcttttaaagtattcacaataaactagcaatatatgtaaatgttatcatctccatttcacagataaggaaactgaagctcagagagtgtaagtaactttctcattatcataaagctaataagtagtttgagtcaggatttgaacctaggtctatctctggtcctatggaaacatgcccatggcccatccctttccacacttgagtgcctgtcttgaaggatcaagctgaaactcagctccctccccttgacagtgacatacccagcaatcccaagtggattcccacagcactttgataccacctccaagtggccacttcctggaactctcacaatgtgtccatgtttgtttcctccaccagagcaaagtttctttttcccttccttctggggtttcttttaccagtctcttgacccgagtgtgagtgtccaccccgttcagctgttcctacggctgtctcagtgatcacgagcacttgataggaaccttcccagcttgggtggagattgtcttccttccaagtcttaattagcaccaagtcgccaggctggaagtggtgacagtcccattttcccaccgtggttcgtgcacgaggttgtctggttgccgcggtgcctgcttttcttcctgtgtcacttttgttatctcctgaatcatggtctccggtttgtctgtggcttctgtggggagccgggacatccagacagagcgggccacataaatcaagtggggcacgtctcccctctccatgcaggcacagagatccccgtatggccaccagattgtgaaaaacaaactcacccttccaaacccaaagaatggattcagagactcggagaacagcaaaagtgagacttttaatggtggtcttgcaagattgggtgtctgataggcaggcacgcccagtatagttttgtttgtttgtttgtttgcttttggagacagagtcttgctctgtcacccaggcttgagtgcagtggcac

SEQ ID NO: 12938 - RNA, 1170 nt, Homo sapiens
  source 1..1170: mol_type = other RNA
gctgggattacaggcatgagccacagcgcccggcctacagcaaaacttatggaaagaatggtcagttatctgtctccactttctcttctctcattatctgtgagcacattttaattaggcttttgcccacatcgctctgctgaaactgctcttttcaaagtagtcagtgactttcatattaaattaaacggtcatttctcaggccttactcttcacttatcattgtattggttatctgttgctatgtaacaattaccctcaaatttagtgactcgaaacaagaagcaattatctcatagtttctatgggtcagaaatccaggaatagcttagctatgtgattctggattaggttctcttatgaagtttcattcaaggtgttggcaggggttgtagtcatgtcaagtcttagaaggttggaggatccacttccaatatactcactcacatgtctggcaaattagtgtttgtttttgatagtaggccttagttcttcaccatgtagacctcttcataaggttgcttgagcatcctcacaatatggcaactggcttctcctctttttcccttccttctggggtttcttttaccagtctcttgacccgagtgtgagtgtccaccccgttcagctgttcctacggctgtctcagtgatcacgagcacttgataggaaccttcccagcttgggtggagattgtcttccttccaagtcttaattagcaccaagtcgccaggctggaagtggtgacagtcccattttcccaccgtggttcgtgcacgaggttgtctggttgccgcggtgcctgcttttcttcctgtgtcacttttgttatctcctgaatcatggtctccggtttgtctgtggcttctgtggggagccgggacatccagacagagcgggccacataaatcaagtggggcacgtctcccctctccatgcaggcacagagatccccgtatggccaccagattgtgaaaaacaaactcacccttccaaacccaaagaatggattcagagactcggagaacagcaaaagtgagacttttaatggtggtcttgcaagattgggtgtctgataggcaggcacgcccagtatagttttgtttgtttgtttgtttgcttttggagacagagtcttgctctgtcacccaggcttgagtgcagtggcac

SEQ ID NO: 12939 - RNA, 1238 nt, Homo sapiens
  source 1..1238: mol_type = other RNA
gctgggattacaggcatgagccacagcgcccggcctagcatttggtaatatcttgatgttgctagttttgttttaggaatgtgtttccctcatgaattccaggagcacaggtggttggaagggctctcttgacagtgattttatagctcaccatcagatcacagcataagactgaaggcttgactcatctttcttctcttgtccttagtttgtccatttgtaaaaggagagagattttgctggaggatatttgaggactcttttatctctaacatcccatgaattgcaaacattattaactactgttacctttcatgacagcaggtagttgaatccaaattgcattctcttttctagttaatgtgtttcagccttctgcgattttgtattagacaagaaatatatgggaccctctttttcctgacatgagggaatacagctggtaatttgcatctctcttggggacctagatatactttcacatcatctgctttcttctgaagacttgaggtgtctgaacaggatagtactaaagtcactgttaagtcaagaccaggccgagaaaaacttcctttgtatcagaaccaaatatcttggcaaagtggcttcaacttcttctactatggcatcagtatattttatattgtatctaaattgcttgaaacactgtcctgatatccacatcagcatttatggctttggttgaaaccttttccaggaaacctccccagatcccttctgatttaggtaccgtcctctgtgctccctgtgattaaatcagcctctacacatattacacaatcactatgctctgatttccgtttacttgtttctcttttgcaatctgtgtcatattcctctttttatccgccgtgccaagtatggagcctgtcacatagcaggcctcataaatacttattgaaagaattaataatagacgtagaaccaacgggcttagtaagcccctggagaaaggaatcaaagatgtttctgaggcctctatatcaggaagtgcggaaatttcatggtttgagaatgggcaggaaagatcatttgtgagctgtatttaatgcaaaagttgctcccccatcctgatttcttagctcactgggccaatcggcggaaggacaggtggggctcaaattaggagaaaaaaaccacacttcccgtcatgcctctgggcaccgctcccgtttccccctctttgtcaccgcctcttccccacggaaatgaaagga

SEQ ID NO: 12940 - RNA, 45 nt, Homo sapiens
  source 1..45: mol_type = other RNA
gctgggattacaggcatgagccacagcgccggccgaaaggcatgt

SEQ ID NO: 12941 - RNA, 3448 nt, Homo sapiens
  source 1..3448: mol_type = other RNA
gctgggattacaggcatgagccacagcgcctggcctgggacacacatttttggacaaaaacaatgataaattctgatgctaccaaattgccttcttatgaaaaaggaatgtggcagataagacagtagctctagaacaaaccctcatgttgacaataactgggcctagggaaaaggaggcggccccttacaactcaatccatgccttcagttgtccttatcctggttcccacacttaaccacagttgacacgggcgtgatcagacatattttgttcttgttttcaagctaagcacccttgagcccctctgaaatgtcagctgcctcaaggataagggactttactgtcaacatgatgggttgggtgagggggaaggggaacaattatccaatgtttcaacaaatctcagtagtaccccaagacatagtatttttggatagccttttaactagaacagtgagcatcaaggctagtagaatagataacaccttgatgaacacacttcctggtgatgataaaagttaggagagactctccattataaatgtgttggtgccactcagaatgaaagctattgagcagaggacttggtaccctggaacaccacacttggctctgagccataccttagccaccaaggagccttcaatcgctccctgattggaagcccaggtaatgtgttaccatgataatttcattttaactcgacattcagaagtccagcttgacttgaggatggagttttacttctatccatgagggctggctttggaatgcctcccctgtgagcacagaaggatttttaacagcatctcatgcccagcgtttttgtactttccgccatccgtgctaagtagaaggcaagttctgaatgagagtgctgacagttcctcttcctgagtgggagaaagcaccacttcagtggcagagtaggacttcccaaaatagactaagaagtagctgtaggtaaatgaattatgtgttcattcacagctttattgtttcatgccaggtccaagaatacttcaagaagtacatttttaagagttcttgagacagttgtattcaaatataaggaggcctgtgaattctctttaacaaatctacaaatatgggagagaatatgtgtgtgacatcaataaatggttaagattcctagtatagagggtgctatgtttacatttttcatctctagagttcaggtaatttttatacattaaatttggggtaagacaaaaattttgtagcctttttaatttaggggaaagtagctgttcagggtgactattatttcataaaaagtttgtgttaacctagctagtaagactctggcaggatctggcatttgctctcaggagaacaatctttgcatagcaatctcaggggtatcccagctaactgaagcctctgttaggtttggacatgcctggcataacgagatgaaaactgatcaacgtgggcatgaaatcagcgggtgtggagactgagcctttctggtgaaacagaacctgggtaccaatagcttctgtttcctacacagaaattgaatcttttggctagggtttggccaggtgccaacaaatagaaagtagaagaatgtctcaaggggaagggagatggagggggccaagaagggagataatatcgtggctgtgtttcatgggaacatagagcatttacaaagggaatgtgatttactcaaatctctatatagccccatgttcacataagcttagtgcctcatagctaactggtactcaatgagtttttgttgaatcaaactaaaccacccccattccccaaaagaaatgctacaaaagcaaacacccctgagttgtgtccagtcctattagagtcctggttaaattctattccgggggacttcgcaagtggctaaaacagcaacgatcctagaaactaagggagtcccactctttgctagctgaaacagggtctgcaatctacacgatggttttaacaccgtgttctgaaagttacagagaactcttgagtgaaggatggggcaactgccccagcagaatcataccttcttcgtgggctgctgggccttcaggacatggttgggctgattatatagggatgcttccaagacggcacctgcggctctcagccttctttaacacagccgttttgtttgggatctcttccagcccctgcccacaactactgtctggctactcacttcccaattttctagtcattggtgttcactccaggttacgagagaggagggaaggtggcaaaagagaattgctatttccaaaactttggtctgagtgggaggataaactgagtgtaaatttgtgaatttgagagaaaggcagactgcatgggttatgtaaacagcaagacaagagaagagggagacaaaaggtaagactttcttcatgtgttattcctgcaacttcctggatattaaattttggtttaatgctaaagagcaggaaccattcccaagctatgtaatcactatgaagccagatctcttttaatattatggacagtacactaatagtttccattttagaaacttcagaatgatagtgaataacattttaaaagtgtttactcttcatatccattaaaacatacacaacaatttccaactaactcttggcagctcattcaccaatagagttatctgattttttttctggcatggtatcaattctccatcaactctaacaaactgcccccaaatcacagccgtcttgtgtcaaacacctgttaatactggcaagcaccatggagtccatgtcaaagagagctaaagaagatgccaaaatatctaagctatttctacaaaaaggtggtaataattttgtatgtgaacatgttagataaaaatcactggaatcagaaacgacttcaaagcttgtatgacaatgacttgattcataggatacatacaaatgaaaccaagactgctggttagaagtgctttgatcacaatctatgtgtctctactttgcccatttcctgaacctcatcttggaagaaaaagcaggatagtaaggcatgtaaaaacacatccaacctacatttctattcttcacactgctttgtgctctctgattttaaataaaaatgcaatagctgtagggtactgggatacattaaaataattgttctgctattactcaactgagcaaaggattttaaataaggataagcataaagtatctgccaacaaccatcagtcaaggctgctaacagggcttttttcaatcttctaaagcagactaaaagttgacttgctagcaagttattaaataaaagcagagaatcctacagatagatttggaaagaccacaacaaatgcatgaggtccatgactcaacaagccctcaataaagagttaaatttaaaaaaaattgtctaaggtcttcatgacttctgtgctttacattttctcgatatttaagtg

SEQ ID NO: 12942 - RNA, 1737 nt, Homo sapiens
  source 1..1737: mol_type = other RNA
gctgggattacaggcatgagccacagctatgtttattttcagtgatctaaagatacaggattaaggcttgtagttcataaagaatccagtggttggcaaacacaaaccattttttactttctcagacatcagaaattataaaagagccttttatgaatgctgctctcaggcaatttgtagctgaaatatatgatgatttctagaaatgtcaaaatctttcattaaagagagactccaacataaagggtatttgttgatttcagctatccaggatccatttcttaccttcttgaagcaacccagatttttgaggattccctcattccacaccactctcaggtcatgtggtctggacagagctccaaccccagctctagggataagcaggtaatcaagttctaggccaatcagtgcatctcatgtccttggtttagaggtaagcactgagaacacaagccatgctcttggaatgaacctggagacattcccgttggggtcaggggttttctccctcttttttttctgctggaattgaacctgtatccagccatgtcgggaatctcaacagctctgggttgtttatgggagctaatacatcttcttttttggtttaactcaattggagccccattttcttctcctgaatgttatataggggttgcctcggcgcattaacttccctcagcagacgaccagatatgtcccttagctctaaaagtctgcatgcaagctgaggatgcagaagtttggccactgatttggaggatctggatatgctgtttaatccacgaattaatgttgctcgattaatcttagctaaagcaatagccatcctgattttggatgttttctgcgcaggttctcttttctgattagactgtgataatcttaggatggtgggaaattcatctttaaactcatctacaaggtccatgattgctttctggatcccctcgattcttccagaaaagttcttcaacacctgcccacatatccacccaacaggtttgattggcatggtgagttcttgcttgggttcctagtccttaacaagcttgcaggcctgggtaatgcttgtcctagtctgccattagtgaaagatgagggtagccttccacttgggaaagccagcaaggacagaactcacagctcactgctggaattctttgttactgtacaataggcttccgagaacctgctacagaatcttctgacatcactctggcagtgagaggaagaggagtgtgtttggaggcataagggaaggagtgaggggattgaataataaagtacactaaggagttctatgatataagttgaaatttgtcccaaattctgcagtgataccacaaataatggatcatctgagaacaaaaggtccctttgaaaaaaaatggcatgtgctttaaaagaaatgctttatatatgatgccaaatagaaaagaaacaccagcagtgaattcagaaagacttctgaatagattgtttttgcttcaccaatgaggatcactaggtcaaactcgggcaaaactgtaaagtctttggtttctctgctttataatctcaatctcttttcttcatcttttaccctcctagtaccctcacatgtcagatgaccattagttcccccgatcaaatatgggaagaacttgataccatgcagacttgattgactgcctagttttatatatatatagtttgtttgtttgtttgttttttgagatggagtcttgccct

SEQ ID NO: 12943 - RNA, 3387 nt, Homo sapiens
  source 1..3387: mol_type = other RNA
gctgggattacaggcatgagccacagtctctggccgcagcctcttttgaaaggaagacccttcaggtggacactgctcacgactcagaacgattttacgtggcccctccagacctgggcccattgcacactcagcccctcccccatcatcaaacaagctggttaattggtcacatttcagtctgagacctttccaagtctcttccacacacaaaaggcagtcgccagaagtcacaaacgtccctcaagccccctttcagactcaatgcaaatgcatccagaatgtctctggggaagtggaaaagctgctgctttccatcttgaaaggccgtggccttcgccgtccaaaggatgctctagtaaaggcctctgctgggcattactgtgtcaacaacattctggcgagcattgattgtgtgcaaaggaacgtcaggccgctaaatttaagtcttcaggaccccttgtttatcctcaagggaaaggtggcagatgacatagcctcaacaaggcacagcaggtacagaaagtgggtatttacttacacatcaaaacttttcaacaacatcgtttgtgggtgacatcagctgctttcttgtctctaagcagcatggctgcagttgggacatcctcctccctcagtgagaatagtggtcctggccacggcgggaagcagacattctaaggacctggggcacagacattccagaaggtaggcaccatttcagtgcccaggccttctctgtagttgctgggaggggtacggctgctgccctcctgcacgggagccatgtgcctcaggggcgtctcaagaatcggttctcgcagtgggggccctcccagccatcccgacacttgcagcggtagctcccattctgcaggacgcagctgccctcattcatgcacgggctgggtttgcagaggttgactggctgcttggcttctccacacagccactcaatgagcacgtcctggtggtaccgcaggtcggcgtaagctgccacgtggatcagggaatcccggggacctgcaagcctccgcagaccctcacttaggacaggccccacgcccacgaccaagacagagatgccattgttcctcagcttctgggcaggaacggctgcatcctctgcgcctctcccgcctgtgagcaccaccacagctttggggacaccaggccgggcacccctctggacggtcatcactttgtcatagatgtgcagcagggcggtgccggctgagcccaccccacctaggtagggggcctggctaatggcccgcagcatcgcagcccgggtgggtttggtgtccagcccgaaggcagtctgcacctggctgccatacaccaccaggccgacctgtgtcacgtcagggttcacctcaaactggagggcacagcttctcacaaagctctgcatctgagcaaaattctcgggccctactgaggcagaggtgtccaacatgaagacgaggtccagggcttgtgtccggcaccctggccgctgccggctgcacagcttcccctgcagctcagggatttggttgaacagatcctgaggatccgagtagaccatcacatgctttgggctgcctgtgatctcctccagctctgcccgcacggcctcactgcctacacccagcaggagcagctctcgcgcccttgcgtgacgcgctgggcccgcaacctcatcctcggagtgtgactcagtgagcaaaaccaccactctacgtggccggtcctggcctgtcctggtggcgctcccgaagccacgctctgccgcctgccgcaaggcactgcccgtcagggtggggccaccacggaagggaatgccatcgaggctccagaccaggtcaggcacatcctggtactcccccacaggcaccgccaccagcagctccctgctgtatgtggccacacccactcgggcccgagagtcctcgctcagcacggcccgcacaaaccgcttcacgaagactttggcccgcaggaagccgtccagagtggtgcccgcagagctgtccagcaggaagaggaggtcgaccctgcattccaggctcagcttcagggcacagttagcctcccctccaaaggccagcgggcagaggcactggtagccgtccagtccttctggaacacatgtgcctccattctggcagggctgcgagtcacaggggcctgggcaggtggtcctgtagcaggtggcagggtgggttaggaacactctcttccagctgtagaagggacagtgtgcagccagcaccgcaagggtccgccgcgatcctctccagcatggggcattgccagcgaactcccggaccatctccagcgtcctgtgctcacaggggtgagcctcgaccctgcagtctggcgtggcgctggagcagatggccgagctgctgagggtgctgaagaggccgttggtggcatcctccacctgctcagccaacagcacgtgctgccctctaggctcgctggccagtgcatgcagctcctcccacctgggaaacctgacccccacagcaaacacagtgacacccctttccttcagctgcttggatggcagtgccacatccccctgggacttcccatcagtgacgatgatgaggatctggggcacagaagcatttctgcctccaggcaaccctctgtgcagaaggtatttcagagcaagttccgtctccgtgcgccctcctttgaaaaccatcctcttgattcttgccttcacttcctgttgggttgaaaatgaatccaaggggaattccagatgaggagtggaactgaactggaatgctcccactctgaccctctcggggctgatgtccagaccgtcacagactgtgatggcaaagtgcttggacctttcaaagctccctttcccgacgctgttagacccatctaacagaaacatgatgtccactgcagccgagcaccacatcattttgctggcagctgaaatcttcccgatggtttctttgcttacatggacttcctggagagggagagatgggggcactctggaaaacaggaaaacacagacggcttccagcaacaggaaagggggcatgttgatataacggaaggagagcggcgaccagcgctcggtgcccgggcggctctactcacagacccgggcgcggctcgggccagggggcgctacgggatcacaggaggggcgcccggggcgcggctgccacgtgggacacctgtttgtctctcctgggagagggcggcacgacccgacccggctgaggtcggaggaactaccgccagggaggtgcatagagcccctcgcgttttttaaagcggcatcggcccaggtctgcaaataaaaaagtacttcacttctacgcgggtcacccagcctccgagcggtgcagccgcgaacactgt

SEQ ID NO: 12944 - RNA, 3329 nt, Homo sapiens
  source 1..3329: mol_type = other RNA
gctgggattacaggcatgagccacagtctctggccgcagcctcttttgaaaggaagacccttcaggtggacactgctcacgactcagaacgattttacgtggcccctccagacctgggcccattgcacactcagcccctcccccatcatcaaacaagctggttaattggtcacatttcagtctgagacctttccaagtctcttccacacacaaaaggcagtcgccagaagtcacaaacgtccctcaagccccctttcagactcaatgcaaatgcatccagaatgtctctggggaagtggaaaagctgctgctttccatcttgaaaggccgtggccttcgccgtccaaaggatgctctagtaaaggcctctgctgggcattactgtgtcaacaacattctggcgagcattgattgtgtgcaaaggaacgtcaggccgctaaatttaagtcttcaggaccccttgtttatcctcaagggaaaggtggcagatgacatagcctcaacaaggcacagcaggtacagaaagtgggtatttacttacacatcaaaacttttcaacaacatcgtttgtgggtgacatcagctgctttcttgtctctaagcagcatggctgcagttgggacatcctcctccctcagtgagaatagtggtcctggccacggcgggaagcagacattctaaggacctggggcacagacattccagaaggtaggcaccatttcagtgcccaggccttctctgtagttgctgggaggggtacggctgctgccctcctgcacgggagccatgtgcctcaggggcgtctcaagaatcggttctcgcagtgggggccctcccagccatcccgacacttgcagcggtagctcccattctgcaggacgcagctgccctcattcatgcacgggctgggtttgcagaggttgactggctgcttggcttctccacacagccactcaatgagcacgtcctggtggtaccgcaggtcggcgtaagctgccacgtggatcagggaatcccggggacctgcaagcctccgcagaccctcacttaggacaggccccacgcccacgaccaagacagagatgccattgttcctcagcttctgggcaggaacggctgcatcctctgcgcctctcccgcctgtgagcaccaccacagctttggggacaccaggccgggcacccctctggacggtcatcactttgtcatagatgtgcagcagggcggtgccggctgagcccaccccacctaggtagggggcctggctaatggcccgcagcatcgcagcccgggtgggtttggtgtccagcccgaaggcagtctgcacctggctgccatacaccaccaggccgacctgtgtcacgtcagggttcacctcaaactggagggcacagcttctcacaaagctctgcatctgagcaaaattctcgggccctactgaggcagaggtgtccaacatgaagacgaggtccagggcttgtgtccggcaccctggccgctgccggctgcacagcttcccctgcagctcagggatttggttgaacagatcctgaggatccgagtagaccatcacatgctttgggctgcctgtgatctcctccagctctgcccgcacggcctcactgcctacacccagcaggagcagctctcgcgcccttgcgtgacgcgctgggcccgcaacctcatcctcggagtgtgactcagtgagcaaaaccaccactctacgtggccggtcctggcctgtcctggtggcgctcccgaagccacgctctgccgcctgccgcaaggcactgcccgtcagggtggggccaccacggaagggaatgccatcgaggctccagaccaggtcaggcacatcctggtactcccccacaggcaccgccaccagcagctccctgctgtatgtggccacacccactcgggcccgagagtcctcgctcagcacggcccgcacaaaccgcttcacgaagactttggcccgcaggaagccgtccagagtggtgcccgcagagctgtccagcaggaagaggaggtcgaccctgcattccaggctcagcttcagggcacagttagcctcccctccaaaggccagcgggcagaggcactggtagccgtccagtccttctggaacacatgtgcctccattctggcagggctgcgagtcacaggggcctgggcaggtggtcctgtagcaggtggcagggtgggttaggaacactctcttccagctgtagaagggacagtgtgcagccagcaccgcaagggtccgccgcgatcctctccagcatggggcattgccagcgaactcccggaccatctccagcgtcctgtgctcacaggggtgagcctcgaccctgcagtctggcgtggcgctggagcagatggccgagctgctgagggtgctgaagaggccgttggtggcatcctccacctgctcagccaacagcacgtgctgccctctaggctcgctggccagtgcatgcagctcctcccacctgggaaacctgacccccacagcaaacacagtgacacccctttccttcagctgcttggatggcagtgccacatccccctgggacttcccatcagtgacgatgatgaggatctggggcacagaagcatttctgcctccaggcaaccctctgtgcagaaggtatttcagagcaagttccgtctccgtgcgccctcctttgaaaaccatcctcttgattcttgccttcacttcctgttgggttgaaaatgaatccaaggggaattccagatgaggagtggaactgaactggaatgctcccactctgaccctctcggggctgatgtccagaccgtcacagactgtgatggcaaagtgcttggacctttcaaagctccctttcccgacgctgttagacccatctaacagaaacatgatgtccactgcagccgagcaccacatcattttgctggcagctgaaatcttcccgatggtttctttgcttacatggacttcctggagagggagagatgggggcactctggaaaacaggaaaacacagacggcttccagcaacaggaaagggggcatgttgatataactgctgaccgcacccctcccaaaaccccgccagctcgcccgggacggaccgcgagtggccacgagggaggcgcgcgccaggtgcgctcttcccccgacgccgccgtgccaggaaggccgcgctcaggtgcgcgcagacaatgcgaacaaagcccgcaccctcggcggggccgcgcagcccgggtgctctgggtaggggtggctgggcagagggggccccagtaccgggagcgtgaatcggtcatcggcagccggcact

SEQ ID NO: 12945 - RNA, 4789 nt, Homo sapiens
  source 1..4789: mol_type = other RNA
gctgggattacaggcatgagccacagtgcccaatcaggaaacacatttaagtgccttatactaccatatgtggaatgaatccagtagccataccaagttattgaccagttatcttaagcagacattcttctgatcacatccaaaattgatgtctacatcagctaactttcctacaagattatcaaattttacacagtatttttctgtatttaatgactgccatggtctgcaaaattatgtgattagacaatgaatgacgcttaaagaatgatgacctattttctaaagtacactcaaaatattaaactttagagacaaagcaaaatctatcataaagttggcttctgttgatagaaacagagaggtaggttaataatcactgtcctaagataagcaagaatgcttagaaataaaagttgagaccctgcttcaaaaaagagaagttgaaccttccagccctgagtttctaatattacatgaaaattatgaaaatgagcattaagccagtcgcagtggctcacgtctgtaatcccagcactttgggaggctgaggcaggcggatcacgaggtcaggagtttgagaccagcctggccaatatggtgaaacgccgtctgtactaaaaatacaaaaattagccaggcatggtggcgcgtgcctgtagtcccagctacttgggaggcggaggcagaagaattgcttgaacccgggagacggaggttgcagtgagctgagattgcgccactgcactccagcctaggtaacagagcgagactctgtctcaaaaaaaaaaaaaaatgagcattacaaaaaataccagtgaccatttctttccatccatgattactgaatacatcaccttctctcatataacaattcaagtggcacatggctacagactgaaaataaatggaccctggacacaagtgatgttggtataaaaagtacaactaagggagaatttgttcccaccctcctacccaagggacagatggcaatgtctggagatatctttgttgtcatggctgaggagggggtctactggaatctagtgggtagaggccagggctgcagctgaacatcctaagcacacaggacagcccccaacaacaatgaattatcaatcccaaaatgttaatagttccaaggttgatcctctggtttaaaggaacaaattcttattaacagagaacaacacaaaaaccttttaaggcctgtctaggtaatacagccctaatcttagagttagggaacatagaaaagttaaactccttggtagactaaaatcaaatttgctgtgaaaaactaaaatactggactgattccagagttttaccatcacttacaagaatagaagaaatttggccaggcacggtggctcatgcctgtaatcccagcactttgggaggccgatgtgggcaggtcatctgaagttaggagttcaagacaagcctggccaacatggtgaaaccccatctctactaaaaatacaaaaataggccaggcatgatggcacgtgcctgtggtcccagctactcgggagtgagactctgtttaaaacaaacaaacaaacaaacaaaaaaaaacagaatagaaaaaatttaaatgatccactaaaatggcgtaatgtcttaaaccggaagcacagagataatctattccacataggtcaaatatctgatccaagaggcataaaccaaaggcagttttatcagctaaatttgcagcagtaaaggataatttagggaatgatttgagagaatatcctacatttcttcatacatcccaactgccattttctaatggcatgggttccatgaacagggatgcatagaagtcattcaaagatttgttgaatgatactgaatatgaattttgcatgaaatggacagagaaaagtatcttacatttgtctgagaactacctgtaattaaaagtcattgagaaacaaggagaaagagaaccagtttctatattacagaattcagaaaaaacaaacaccaaaactctaagccattttacaaataaattcaatatgaaatcacttacttcctattatattcacttccagggttacttttagaaaacatatccatatcaacatggcttcaagcttgcctactgaaggaagtgcaaactttaagaagatcatcttccctctcagtttatggaacttaaaacatcaccaaggagaatgaaggctcattgcctatggttcataaaagaaatgtccaaaggctttgaatgcataaaccagctagagtagaataaggtttcttcctatcagattgaaaagaagagagaaaagaaaactaaaagggtgttagaccaagttttcctcttttttttttttttttttttttaaatatggagtctcgctctattgcccaggctggagtgcaatggcgcaatctcggctcactgcaacctccgcctcccgggttcaaatgattctcctgcctcagcctcccgagtagttgggactacaggcgcccaccaccaggactggctaatttttgtatttttagtagagacggggtttcaccatgttggtcaggctggtcttgaactcctgatctcagatgatccgcccgcctcggcctcccaaagtgctgggatgacaggcatgagccaccacgcctggcctcttgtttgtatttagagttgattgtcaaagcagtggtcccttttgatcagagtaacttagaaaaatcaagtaattcctatgtaaatgatagctgaaatcttctgaaacccaggactacttatgcaatcactttttaaagatgattcttccctctttcactgtgattttatgcaagtaaaatcacacaagtagatggggaaaccagaatcaacagtctctgagggactttaggcacaatttggcagagggcccctgacttcttttctgcaatctaatagtgatccagccatggcctcctatgacctcatctgcttactgactacaatgtcttacattttcctgaaggattttttgtttacatgataaattctaacctctgcatctaactattgctttgcaattttgaggttaaatcacctacactgctttatgtaggagacaatcctcaaacatattgccatttgcctgggatctcataatgaaacatctcccttccctccacaaccacgtacataatacattttaagagctgtttaacttagaacttctcaaaaaatatattttgaaatactaagtttcattatacccttacttataaccatggtagtcacttttcccaacaatgagggtcaccagaccaaataattagggtaaattttgacatacatcaatggccagcatttagtctaggaattcaaatataactaatgctttaaacacataaggaactataaaaccaaaatgtgtgcttaaggcgaggtccacatgagtaacattgccacattatcagtcaaagaaatgatcatgacagtcattttaaccactaactgagatcacagaatgactgtacacaatgactcaagtggccatgcatataaaaacaacctaaattccagttgacaatgtgcacatttttggaaaaacaaataagtataatatagactagaaggtctctgagatactactttttccttttttcaccatatcttttccaatggaactttggagtcttggttccggacctgctgtatttctaagaggaactcttcccatcaccatgctgccttctgagctaaaggcatgtgcttctgaattgtacagagacagaccttcaggaaaaatgttctgaattttcaaatgtacatcttttaaaatgtctaacctaaaaaaaatgaacaaactgaaaaaaacatttgttcctttgttattaaaaatgactggtctacaaaggttttgttttagtagatggggctacacagtacgtaactgagactgaagacaaaaatcgaaaatttgtggtttctaaaaagagaaataggatatataaggttggcattaccagttttggggagaaacactgaataagttaaaggaaaaaaaaagatgagaatgagtgatctgttttatcttaagaaacttttgtcccatacagaatctttaaaatagacaattatataaaatttatctattgttcttatgacatttaaataagttaacacacagtggaaagcgtggcattagttgtcttcttcctcatcccctttaattactggagtaccatccagctttttcagtttgggcactctcttggttgcttcttcaatccagttattctcagcagaatgtttctcttccaagggattgcctacaaacaccaggtcttcgaggcatggcagttctgccagcttcacaaactcagcccagtcttttaccaggttattagacatgtagagaatcttcaatttcttcattatgtggatccctttcaacttctcaataaaattgtaggagatccacagttcttctaatgtgtcccctactgcctccagtccatttaagttctttatgttgtttcttcctaaagataatatcctcaagttttttaagccattcaggttggcaattttttcaatgcagtttgtagacagtgaaagcttctcgcaattagcaagcatggacaaggatgcatccatcttctctatagggggaatctgggcataaagttttatctctttggcttcagatggcctctggccagttttctcttcccatctcgctaaggcttctttgattgttgttgctttcgccattccggcggttgctactgtcactgctctggttgctagggcccgcggggtcagtgc

SEQ ID NO: 12946 - RNA, 4835 nt, Homo sapiens
  source 1..4835: mol_type = other RNA
gctgggattacaggcatgagccacagtgcccaatcaggaaacacatttaagtgccttatactaccatatgtggaatgaatccagtagccataccaagttattgaccagttatcttaagcagacattcttctgatcacatccaaaattgatgtctacatcagctaactttcctacaagattatcaaattttacacagtatttttctgtatttaatgactgccatggtctgcaaaattatgtgattagacaatgaatgacgcttaaagaatgatgacctattttctaaagtacactcaaaatattaaactttagagacaaagcaaaatctatcataaagttggcttctgttgatagaaacagagaggtaggttaataatcactgtcctaagataagcaagaatgcttagaaataaaagttgagaccctgcttcaaaaaagagaagttgaaccttccagccctgagtttctaatattacatgaaaattatgaaaatgagcattaagccagtcgcagtggctcacgtctgtaatcccagcactttgggaggctgaggcaggcggatcacgaggtcaggagtttgagaccagcctggccaatatggtgaaacgccgtctgtactaaaaatacaaaaattagccaggcatggtggcgcgtgcctgtagtcccagctacttgggaggcggaggcagaagaattgcttgaacccgggagacggaggttgcagtgagctgagattgcgccactgcactccagcctaggtaacagagcgagactctgtctcaaaaaaaaaaaaaaatgagcattacaaaaaataccagtgaccatttctttccatccatgattactgaatacatcaccttctctcatataacaattcaagtggcacatggctacagactgaaaataaatggaccctggacacaagtgatgttggtataaaaagtacaactaagggagaatttgttcccaccctcctacccaagggacagatggcaatgtctggagatatctttgttgtcatggctgaggagggggtctactggaatctagtgggtagaggccagggctgcagctgaacatcctaagcacacaggacagcccccaacaacaatgaattatcaatcccaaaatgttaatagttccaaggttgatcctctggtttaaaggaacaaattcttattaacagagaacaacacaaaaaccttttaaggcctgtctaggtaatacagccctaatcttagagttagggaacatagaaaagttaaactccttggtagactaaaatcaaatttgctgtgaaaaactaaaatactggactgattccagagttttaccatcacttacaagaatagaagaaatttggccaggcacggtggctcatgcctgtaatcccagcactttgggaggccgatgtgggcaggtcatctgaagttaggagttcaagacaagcctggccaacatggtgaaaccccatctctactaaaaatacaaaaataggccaggcatgatggcacgtgcctgtggtcccagctactcgggagtgagactctgtttaaaacaaacaaacaaacaaacaaaaaaaaacagaatagaaaaaatttaaatgatccactaaaatggcgtaatgtcttaaaccggaagcacagagataatctattccacataggtcaaatatctgatccaagaggcataaaccaaaggcagttttatcagctaaatttgcagcagtaaaggataatttagggaatgatttgagagaatatcctacatttcttcatacatcccaactgccattttctaatggcatgggttccatgaacagggatgcatagaagtcattcaaagatttgttgaatgatactgaatatgaattttgcatgaaatggacagagaaaagtatcttacatttgtctgagaactacctgtaattaaaagtcattgagaaacaaggagaaagagaaccagtttctatattacagaattcagaaaaaacaaacaccaaaactctaagccattttacaaataaattcaatatgaaatcacttacttcctattatattcacttccagggttacttttagaaaacatatccatatcaacatggcttcaagcttgcctactgaaggaagtgcaaactttaagaagatcatcttccctctcagtttatggaacttaaaacatcaccaaggagaatgaaggctcattgcctatggttcataaaagaaatgtccaaaggctttgaatgcataaaccagctagagtagaataaggtttcttcctatcagattgaaaagaagagagaaaagaaaactaaaagggtgttagaccaagttttcctcttttttttttttttttttttttaaatatggagtctcgctctattgcccaggctggagtgcaatggcgcaatctcggctcactgcaacctccgcctcccgggttcaaatgattctcctgcctcagcctcccgagtagttgggactacaggcgcccaccaccaggactggctaatttttgtatttttagtagagacggggtttcaccatgttggtcaggctggtcttgaactcctgatctcagatgatccgcccgcctcggcctcccaaagtgctgggatgacaggcatgagccaccacgcctggcctcttgtttgtatttagagttgattgtcaaagcagtggtcccttttgatcagagtaacttagaaaaatcaagtaattcctatgtaaatgatagctgaaatcttctgaaacccaggactacttatgcaatcactttttaaagatgattcttccctctttcactgtgattttatgcaagtaaaatcacacaagtagatggggaaaccagaatcaacagtctctgagggactttaggcacaatttggcagagggcccctgacttcttttctgcaatctaatagtgatccagccatggcctcctatgacctcatctgcttactgactacaatgtcttacattttcctgaaggattttttgtttacatgataaattctaacctctgcatctaactattgctttgcaattttgaggttaaatcacctacactgctttatgtaggagacaatcctcaaacatattgccatttgcctgggatctcataatgaaacatctcccttccctccacaaccacgtacataatacattttaagagctgtttaacttagaacttctcaaaaaatatattttgaaatactaagtttcattatacccttacttataaccatggtagtcacttttcccaacaatgagggtcaccagaccaaataattagggtaaattttgacatacatcaatggccagcatttagtctaggaattcaaatataactaatgctttaaacacataaggaactataaaaccaaaatgtgtgcttaaggcgaggtccacatgagtaacattgccacattatcagtcaaagaaatgatcatgacagtcattttaaccactaactgagatcacagaatgactgtacacaatgactcaagtggccatgcatataaaaacaacctaaattccagttgacaatgtgcacatttttggaaaaacaaataagtataatatagactagaaggtctctgagatactactttttccttttttcaccatatcttttccaatggaactttggagtcttggttccggacctgctgtatttctaagaggaactcttcccatcaccatgctgccttctgagctaaaggcatgtgcttctgaattgtacagagacagaccttcaggaaaaatgttctgaattttcaaatgtacatcttttaaaatgtctaacctaaaaaaaatgaacaaactgaaaaaaacatttgttcctttgttattaaaaatgactggtctacaaaggttttgttttagtagatggggctacacagtacgtaactgagactgaagacaaaaatcgaaaatttgtggtttctaaaaagagaaataggatatataaggttggcattaccagttttggggagaaacactgaataagttaaaggaaaaaaaaagatgagaatgagtgatctgttttatcttaagaaacttttgtcccatacagaatctttaaaatagacaattatataaaatttatctattgttcttatgacatttaaataagttaacacacagtggaaagcgtggcattagttgtcttcttcctcatcccctttaattactggagtaccatccagctttttcagtttgggcactctcttggttgcttcttcaatccagttattctcagcagaatgtttctcttccaagggattgcctacaaacaccaggtcttcgaggcatggcagttctgccagcttcacaaactcagcccagtcttttaccaggttattagacatgtagagaatcttcaatttcttcattatgtggatccctttcaacttctcaataaaattgtaggagatccacagttcttctaatgtgtcccctactgcctccagtccatttaagttctttatgttgtttcttcctaaagataatatcctcaagttttttaagccattcaggttggcaattttttcaatgcagtttgtagacagtgaaagcttctcgcaattagcaagcatggacaaggatgcatccatcttctctatagggggaatctgggcataaagttttatctctttggcttcagatggcctctggccagttttctcttcccatctcgctaaggcttctttgattgttgttgctttcgcctgaatcaaccaatcagctcacttgactcaaccaatcaaggcccagcattccggcggttgctactgtcactgctctggttgctagggcccgcggggtcagtgc

SEQ ID NO: 12947 - RNA, 4863 nt, Homo sapiens
  source 1..4863: mol_type = other RNA
gctgggattacaggcatgagccacagtgcccaatcaggaaacacatttaagtgccttatactaccatatgtggaatgaatccagtagccataccaagttattgaccagttatcttaagcagacattcttctgatcacatccaaaattgatgtctacatcagctaactttcctacaagattatcaaattttacacagtatttttctgtatttaatgactgccatggtctgcaaaattatgtgattagacaatgaatgacgcttaaagaatgatgacctattttctaaagtacactcaaaatattaaactttagagacaaagcaaaatctatcataaagttggcttctgttgatagaaacagagaggtaggttaataatcactgtcctaagataagcaagaatgcttagaaataaaagttgagaccctgcttcaaaaaagagaagttgaaccttccagccctgagtttctaatattacatgaaaattatgaaaatgagcattaagccagtcgcagtggctcacgtctgtaatcccagcactttgggaggctgaggcaggcggatcacgaggtcaggagtttgagaccagcctggccaatatggtgaaacgccgtctgtactaaaaatacaaaaattagccaggcatggtggcgcgtgcctgtagtcccagctacttgggaggcggaggcagaagaattgcttgaacccgggagacggaggttgcagtgagctgagattgcgccactgcactccagcctaggtaacagagcgagactctgtctcaaaaaaaaaaaaaaatgagcattacaaaaaataccagtgaccatttctttccatccatgattactgaatacatcaccttctctcatataacaattcaagtggcacatggctacagactgaaaataaatggaccctggacacaagtgatgttggtataaaaagtacaactaagggagaatttgttcccaccctcctacccaagggacagatggcaatgtctggagatatctttgttgtcatggctgaggagggggtctactggaatctagtgggtagaggccagggctgcagctgaacatcctaagcacacaggacagcccccaacaacaatgaattatcaatcccaaaatgttaatagttccaaggttgatcctctggtttaaaggaacaaattcttattaacagagaacaacacaaaaaccttttaaggcctgtctaggtaatacagccctaatcttagagttagggaacatagaaaagttaaactccttggtagactaaaatcaaatttgctgtgaaaaactaaaatactggactgattccagagttttaccatcacttacaagaatagaagaaatttggccaggcacggtggctcatgcctgtaatcccagcactttgggaggccgatgtgggcaggtcatctgaagttaggagttcaagacaagcctggccaacatggtgaaaccccatctctactaaaaatacaaaaataggccaggcatgatggcacgtgcctgtggtcccagctactcgggagtgagactctgtttaaaacaaacaaacaaacaaacaaaaaaaaacagaatagaaaaaatttaaatgatccactaaaatggcgtaatgtcttaaaccggaagcacagagataatctattccacataggtcaaatatctgatccaagaggcataaaccaaaggcagttttatcagctaaatttgcagcagtaaaggataatttagggaatgatttgagagaatatcctacatttcttcatacatcccaactgccattttctaatggcatgggttccatgaacagggatgcatagaagtcattcaaagatttgttgaatgatactgaatatgaattttgcatgaaatggacagagaaaagtatcttacatttgtctgagaactacctgtaattaaaagtcattgagaaacaaggagaaagagaaccagtttctatattacagaattcagaaaaaacaaacaccaaaactctaagccattttacaaataaattcaatatgaaatcacttacttcctattatattcacttccagggttacttttagaaaacatatccatatcaacatggcttcaagcttgcctactgaaggaagtgcaaactttaagaagatcatcttccctctcagtttatggaacttaaaacatcaccaaggagaatgaaggctcattgcctatggttcataaaagaaatgtccaaaggctttgaatgcataaaccagctagagtagaataaggtttcttcctatcagattgaaaagaagagagaaaagaaaactaaaagggtgttagaccaagttttcctcttttttttttttttttttttttaaatatggagtctcgctctattgcccaggctggagtgcaatggcgcaatctcggctcactgcaacctccgcctcccgggttcaaatgattctcctgcctcagcctcccgagtagttgggactacaggcgcccaccaccaggactggctaatttttgtatttttagtagagacggggtttcaccatgttggtcaggctggtcttgaactcctgatctcagatgatccgcccgcctcggcctcccaaagtgctgggatgacaggcatgagccaccacgcctggcctcttgtttgtatttagagttgattgtcaaagcagtggtcccttttgatcagagtaacttagaaaaatcaagtaattcctatgtaaatgatagctgaaatcttctgaaacccaggactacttatgcaatcactttttaaagatgattcttccctctttcactgtgattttatgcaagtaaaatcacacaagtagatggggaaaccagaatcaacagtctctgagggactttaggcacaatttggcagagggcccctgacttcttttctgcaatctaatagtgatccagccatggcctcctatgacctcatctgcttactgactacaatgtcttacattttcctgaaggattttttgtttacatgataaattctaacctctgcatctaactattgctttgcaattttgaggttaaatcacctacactgctttatgtaggagacaatcctcaaacatattgccatttgcctgggatctcataatgaaacatctcccttccctccacaaccacgtacataatacattttaagagctgtttaacttagaacttctcaaaaaatatattttgaaatactaagtttcattatacccttacttataaccatggtagtcacttttcccaacaatgagggtcaccagaccaaataattagggtaaattttgacatacatcaatggccagcatttagtctaggaattcaaatataactaatgctttaaacacataaggaactataaaaccaaaatgtgtgcttaaggcgaggtccacatgagtaacattgccacattatcagtcaaagaaatgatcatgacagtcattttaaccactaactgagatcacagaatgactgtacacaatgactcaagtggccatgcatataaaaacaacctaaattccagttgacaatgtgcacatttttggaaaaacaaataagtataatatagactagaaggtctctgagatactactttttccttttttcaccatatcttttccaatggaactttggagtcttggttccggacctgctgtatttctaagaggaactcttcccatcaccatgctgccttctgagctaaaggcatgtgcttctgaattgtacagagacagaccttcaggaaaaatgttctgaattttcaaatgtacatcttttaaaatgtctaacctaaaaaaaatgaacaaactgaaaaaaacatttgttcctttgttattaaaaatgactggtctacaaaggttttgttttagtagatggggctacacagtacgtaactgagactgaagacaaaaatcgaaaatttgtggtttctaaaaagagaaataggatatataaggttggcattaccagttttggggagaaacactgaataagttaaaggaaaaaaaaagatgagaatgagtgatctgttttatcttaagaaacttttgtcccatacagaatctttaaaatagacaattatataaaatttatctattgttcttatgacatttaaataagttaacacacagtggaaagcgtggcattagttgtcttcttcctcatcccctttaattactggagtaccatccagctttttcagtttgggcactctcttggttgcttcttcaatccagttattctcagcagaatgtttctcttccaagggattgcctacaaacaccaggtcttcgaggcatggcagttctgccagcttcacaaactcagcccagtcttttaccaggttattagacatgtagagaatcttcaatttcttcattatgtggatccctttcaacttctcaataaaattgtaggagatccacagttcttctaatgtgtcccctactgcctccagtccatttaagttctttatgttgtttcttcctaaagataatatcctcaagttttttaagccattcaggttggcaattttttcaatgcagtttgtagacagtgaaagcttctcgcaattagcaagcatggacaaggatgcatccatcttctctatagggggaatctgggcataaagttttatctctttggcttcagatggcctctggccagttttctcttcccatctcgctaaggcttctttgattgttgttgctttcgcctgaatcaaccaatcagctcacttgactcaaccaatcaaggcccagccttttccactcccaatcttctctcagctttggctacgcggcccgaaaggtactcaccattccggcggttgctactgtcactgct

SEQ ID NO: 12948 - RNA, 4934 nt, Homo sapiens
  source 1..4934: mol_type = other RNA
gctgggattacaggcatgagccacagtgcccaatcaggaaacacatttaagtgccttatactaccatatgtggaatgaatccagtagccataccaagttattgaccagttatcttaagcagacattcttctgatcacatccaaaattgatgtctacatcagctaactttcctacaagattatcaaattttacacagtatttttctgtatttaatgactgccatggtctgcaaaattatgtgattagacaatgaatgacgcttaaagaatgatgacctattttctaaagtacactcaaaatattaaactttagagacaaagcaaaatctatcataaagttggcttctgttgatagaaacagagaggtaggttaataatcactgtcctaagataagcaagaatgcttagaaataaaagttgagaccctgcttcaaaaaagagaagttgaaccttccagccctgagtttctaatattacatgaaaattatgaaaatgagcattaagccagtcgcagtggctcacgtctgtaatcccagcactttgggaggctgaggcaggcggatcacgaggtcaggagtttgagaccagcctggccaatatggtgaaacgccgtctgtactaaaaatacaaaaattagccaggcatggtggcgcgtgcctgtagtcccagctacttgggaggcggaggcagaagaattgcttgaacccgggagacggaggttgcagtgagctgagattgcgccactgcactccagcctaggtaacagagcgagactctgtctcaaaaaaaaaaaaaaatgagcattacaaaaaataccagtgaccatttctttccatccatgattactgaatacatcaccttctctcatataacaattcaagtggcacatggctacagactgaaaataaatggaccctggacacaagtgatgttggtataaaaagtacaactaagggagaatttgttcccaccctcctacccaagggacagatggcaatgtctggagatatctttgttgtcatggctgaggagggggtctactggaatctagtgggtagaggccagggctgcagctgaacatcctaagcacacaggacagcccccaacaacaatgaattatcaatcccaaaatgttaatagttccaaggttgatcctctggtttaaaggaacaaattcttattaacagagaacaacacaaaaaccttttaaggcctgtctaggtaatacagccctaatcttagagttagggaacatagaaaagttaaactccttggtagactaaaatcaaatttgctgtgaaaaactaaaatactggactgattccagagttttaccatcacttacaagaatagaagaaatttggccaggcacggtggctcatgcctgtaatcccagcactttgggaggccgatgtgggcaggtcatctgaagttaggagttcaagacaagcctggccaacatggtgaaaccccatctctactaaaaatacaaaaataggccaggcatgatggcacgtgcctgtggtcccagctactcgggagtgagactctgtttaaaacaaacaaacaaacaaacaaaaaaaaacagaatagaaaaaatttaaatgatccactaaaatggcgtaatgtcttaaaccggaagcacagagataatctattccacataggtcaaatatctgatccaagaggcataaaccaaaggcagttttatcagctaaatttgcagcagtaaaggataatttagggaatgatttgagagaatatcctacatttcttcatacatcccaactgccattttctaatggcatgggttccatgaacagggatgcatagaagtcattcaaagatttgttgaatgatactgaatatgaattttgcatgaaatggacagagaaaagtatcttacatttgtctgagaactacctgtaattaaaagtcattgagaaacaaggagaaagagaaccagtttctatattacagaattcagaaaaaacaaacaccaaaactctaagccattttacaaataaattcaatatgaaatcacttacttcctattatattcacttccagggttacttttagaaaacatatccatatcaacatggcttcaagcttgcctactgaaggaagtgcaaactttaagaagatcatcttccctctcagtttatggaacttaaaacatcaccaaggagaatgaaggctcattgcctatggttcataaaagaaatgtccaaaggctttgaatgcataaaccagctagagtagaataaggtttcttcctatcagattgaaaagaagagagaaaagaaaactaaaagggtgttagaccaagttttcctcttttttttttttttttttttttaaatatggagtctcgctctattgcccaggctggagtgcaatggcgcaatctcggctcactgcaacctccgcctcccgggttcaaatgattctcctgcctcagcctcccgagtagttgggactacaggcgcccaccaccaggactggctaatttttgtatttttagtagagacggggtttcaccatgttggtcaggctggtcttgaactcctgatctcagatgatccgcccgcctcggcctcccaaagtgctgggatgacaggcatgagccaccacgcctggcctcttgtttgtatttagagttgattgtcaaagcagtggtcccttttgatcagagtaacttagaaaaatcaagtaattcctatgtaaatgatagctgaaatcttctgaaacccaggactacttatgcaatcactttttaaagatgattcttccctctttcactgtgattttatgcaagtaaaatcacacaagtagatggggaaaccagaatcaacagtctctgagggactttaggcacaatttggcagagggcccctgacttcttttctgcaatctaatagtgatccagccatggcctcctatgacctcatctgcttactgactacaatgtcttacattttcctgaaggattttttgtttacatgataaattctaacctctgcatctaactattgctttgcaattttgaggttaaatcacctacactgctttatgtaggagacaatcctcaaacatattgccatttgcctgggatctcataatgaaacatctcccttccctccacaaccacgtacataatacattttaagagctgtttaacttagaacttctcaaaaaatatattttgaaatactaagtttcattatacccttacttataaccatggtagtcacttttcccaacaatgagggtcaccagaccaaataattagggtaaattttgacatacatcaatggccagcatttagtctaggaattcaaatataactaatgctttaaacacataaggaactataaaaccaaaatgtgtgcttaaggcgaggtccacatgagtaacattgccacattatcagtcaaagaaatgatcatgacagtcattttaaccactaactgagatcacagaatgactgtacacaatgactcaagtggccatgcatataaaaacaacctaaattccagttgacaatgtgcacatttttggaaaaacaaataagtataatatagactagaaggtctctgagatactactttttccttttttcaccatatcttttccaatggaactttggagtcttggttccggacctgctgtatttctaagaggaactcttcccatcaccatgctgccttctgagctaaaggcatgtgcttctgaattgtacagagacagaccttcaggaaaaatgttctgaattttcaaatgtacatcttttaaaatgtctaacctaaaaaaaatgaacaaactgaaaaaaacatttgttcctttgttattaaaaatgactggtctacaaaggttttgttttagtagatggggctacacagtacgtaactgagactgaagacaaaaatcgaaaatttgtggtttctaaaaagagaaataggatatataaggttggcattaccagttttggggagaaacactgaataagttaaaggaaaaaaaaagatgagaatgagtgatctgttttatcttaagaaacttttgtcccatacagaatctttaaaatagacaattatataaaatttatctattgttcttatgacatttaaataagttaacacacagtggaaagcgtggcattagttgtcttcttcctcatcccctttaattactggagtaccatccagctttttcagtttgggcactctcttggttgcttcttcaatccagttattctcagcagaatgtttctcttccaagggattgcctacaaacaccaggtcttcgaggcatggcagttctgccagcttcacaaactcagcccagtcttttaccaggttattagacatgtagagaatcttcaatttcttcattatgtggatccctttcaacttctcaataaaattgtaggagatccacagttcttctaatgtgtcccctactgcctccagtccatttaagttctttatgttgtttcttcctaaagataatatcctcaagttttttaagccattcaggttggcaattttttcaatgcagtttgtagacagtgaaagcttctcgcaattagcaagcatggacaaggatgcatccatcttctctatagggggaatctgggcataaagttttatctctttggcttcagatggcctctggccagttttctcttcccatctcgctaaggcttctttgattgttgttgctttcgcctgaatcaaccaatcagctcacttgactcaaccaatcaaggcccagttttcaacatggatttgaaaatcctagatacaatattatatcttcaagctggacatggtggctcatgcctgcaatcccagcactatgggaagccaaggctggaggatcacttgaggccaggagtttgagaccagcctggacaacacagcaagaccc

SEQ ID NO: 12949 - RNA, 2998 nt, Homo sapiens
  source 1..2998: mol_type = other RNA
gctgggattacaggcatgagccacagtgcccagccagggacaaatgtttgcattaaatctcccctgttcagcttactggtgaggcttcatttcctgtctcagattttccacacatctgtaagtgtccattctgtacaacttgaatcagctcgtggtcctgagcactcaagtacgtcatgtattttctttcaactggcttgtggttcccactcagtccttcctgctttgctactattatcaaaagcttttcgatttccacataaaagtaaatggttacacgaaaataaatttcagtaagacacaggcagcgccagtcctctcgacccgcagggctgtcggagagaagccaggtgtgttttgcagtgtctggcacagcagctgccccactcctctgcaggaacccactgctttcccaagctgaagccctggggacctgcaagaggcgtgttcgtgctaggaattcactcgaattgagggtgaggaactcggttctcgcagggatagctcgcaaaggaggctcgtgctcctcaaacacctggggcaagaaccacttcccttttcaaacgttcaacctgtctcacactgacagtgcgggtctgaactccattccatgagatgactgatcacgtctgggtgttgccatcatagctatggaaacctccagcagctccgattcccagtttggtcctctctcctcacagacgtcgcagaccccacactgagcagccacggaacggcagtcagaggcggtcagcccaccggtcacccgtcaccaaaactcatctcccgttcctactgacggtcgggaccatgagtttcaccagaggtggtgctgcagatccacacctctccgcagagcccctgctgcgctgaaagcacggctgtccctccacagccacgggcggcagcagccctccggcccacagtcagcggctggagctcagcccccatgaggctggggctaggctgagcccaccacacccaggctgcgaggacgcgctccacggcgtactcgaagttgagagtgtgcacggaagtgtgtccctcccgcgccgcgtgcagcgcagcctcattgcagatgttggcgatgtcagccccactgaatcctggtgtcagctctgccagacgctgggagtaaaaggtgctggactgggtcagcttcaggctcttcaggtgctgctcaaaaatctcccgcctctcctgggagatggtggttgcagtgagccgagatcgcgccgctgcactccagcctgggggatagagtgagactgtctcaaaaaaaaaaaaaagagaacgctcttggaaggagaggtgggtggggatcacttgaggccaggggtttgacaccagccttggcaacacagcgagactctgttaaaaattaaccagcacggcggcgcacgcccatagtagtcctagctcctcagcttgagccctgaaggttgaggccgcagtgagtggtgatcgcagcactgcactccagcctgggtgacagcgcaacaccctttctctgcagcgtggggagatcaatgaagacgtgccggtccagtcggcctggcctcatcagagcaccgtccaaaatgtcagctcggttcgtggacgccaggacgatgacatggtctgtggtacccattccatccatttctaccagaagctggttgagcgtctgctcctcctccgtgttggagaagccggacatggtggtggagcgcttcttgcccaccgcgtcgatctcatcgatgtagacgatgcagggggcccgggctcgggcttccttaaagaggctccgcacacgggcagcgccgaggcctccaatgacctccacgaactctgggccggccatcgccaggaagggcacctgagcctccgtggccaccgccttggccagcagcgtcttcccacagccgggggggccgagcagcagtgcgccctttgggaccttggcgccaagctggaggaagcgttctgggctcttcagataatccacaaactcgcggacttccagtttggcttcgtgcattcctgccacgtctttgaagctgactcctttccccatcttcccatccacaatggtgaaacgagccattttaagctgattaaaagcactgaatccaccttcccttccagtcatcccggccagacggaaaacataccacaggatggccaggcccactgccgtcatccccacagagtacagggcatttccaaagaatcctgttcgcttgtaggaaactgggatcctgtccttggcctcgatattcagctcatcttcagctgctcgaagcttctcttcaaacttgtcaatatttgcaacctgcattcggtacatcaaggctagccgaggccgcccaaacaccacggctccagggtgcaggtagacttccaccacgtcgctctcaggcaccacctggacgcgctgcacctcgcccttggccagcatctcgtggacaaagtcgttccaggaaatgctgcctccgctggtgctgagagcattcaggaggctcatgacaaccgcgatgaccagcaaggtgcgcagccgctctcggtacatctggtcgtcccgctcacggcgtctcctctcctcttcgtcctcttcaggcgccttccccttcgacttatccttctccttattcttctgcttcaaccttgaggtgttaaaatagaaagtaccacctaaaagttgccagagtctgactggattctgaactaaatgttgtttcaacaacaatccgttgatcccttcaaaggtaggggttagcagtctcaattgtaagctctgcagagctcggcctccagcctcggcgaggtcccccggaggcctgctggccatgtacggccgccccctcccgggcctggcggggaaccctggactccaggccgggcctgggccccacagcggccgaggacccgggcctggaccccggcggagggcacggagcagcagcagcagcacggccatgttggcctgaaagccgcgcctgcgtgatccgcggggcgc

SEQ ID NO: 12950 - RNA, 15283 nt, Homo sapiens
  source 1..15283: mol_type = other RNA
gctgggattacaggcatgagccacagtgcctgcctggccacaaataattttaaagagttatcttccatatatctcaattctacataatctgactcattgtttttatttattagggcaagtcagtgtaggtatgatatgctgatccagaaaagtcattatagagaatttagcattgcagtccaatgctatttatacctcctctaaaccagagatgatgctaaactcattagaagtacttttgtgtacatctagaattttggctatgatttttaaattctaatttaagcagtttctgaacttttgtaaagattcttaatagtgaatcataatgatacagctcctcaaaacagaaggacttaaatgttaaaaactggagtaaataggagtaggtactgatccatgtttctgtccctcttttacaggatgcagactcttcttattttaaaatctttaagacaaaacatgactgaaaagagcacctgtacttttcaagccactggagggagaaatggaaaacatgaaaacagcaatcttcttatgcttctgaataatcaaagactaatttgtgattttactttttaatagatatgactttgcttccaacatggaatgaaataaaaaataaataataaaagattgccatgaatcttgcaaaaaaggtattaactcatactatattcttggataaaataaccttttaaaatactttagcacatatgcttaaaatctaagttaacagatttgtcttagtccatttgtgctgctataacaaaataccacagatttggtaatttataaacaacagaaatctgtttttcctggctcttgaggctgggaattccaagaccaatgcaccagcagaattagtgtctggtgaaggctgatctctgcttccaagatggcacctcattgctgcatcctccacagtggaggaatgtatgtcctcacatggtggaagggacagaagggaaagaggagcaaaatgctttcaaaagagcatttaatctcattcattactcagtcacctcttaaaggccacatcctttaatactgttgctttggggattaagtttcgacatgaattttggaggggacaaaaacatccaaaccatagcaacataaatgtatagaatatttcacacaaagcagagtgctgggtaatgaccagatataaagaagtatttgaaatgaccttacctccaagatgcttatactcttagaaaagttgacaggtacagatggctgtaatttgaagcagcaggtaggattcattgcacctattattcattaaacacctgttgtatgtcttctactgtactggagtgcttagtattagttaattaactcattcctcataacagcccactaagatagatggtattacctaccttgatagatgaagaaagaccaacaaggttttacttttccaaggtcaaggtcacaaagctagtaaggggtaaagccatgattagattcagctcaggaagattccactggcaactccttacttctactattattaattttactttaacatttaacaccttacagcagaaaacatgcacaggcactaataggaaatcagcaggagtaacaggtaaagaaaaacatggtccttatctacaagcagttcacaattgagctggagccaaagtaacatacataaaataactgtagaatagttgttgggcaagttggaagccacccaagtggctgtccttggaaaagggggaagatgacatgtggtagaggtacacgatgaggtatagcgggtagaagcaatggaataaatgcatacataacaacatggatatgtactagaggcatagtcataagtgaagaaataaagaagcaacgctaacacaatactgttcacatacacaaatatatgtgcacagaagatagtgctcattttgcaagaaaacatacaacctaattagatatatatttaggtatggtaatagttacttaggatggggaggaaacggggtgaactatggggataaaatataataaagagaggactcttgcgtgaccagtgatgaaaactggaataacaacattatttattgaatacaacacaccaattataagaatgaaaagattggaataattctagaatgccacaaaataacatatgtcatgtggcctggtacagactataagcataatagttcagaaaagggagatttgcagatagaatcatgtggaagcccttcctgatgaaggtgtcacttgcactgggccttgaaagaaaggaatttagacagatgaagagaagcttcaggaggccaggttccaggtcagttttgttttattcatcactgaatctccagtgcctgcctagcattgtgcctgctgatgtctgttcaactactccagccaatgaatggtagaagaggtatatataaattaaaatctttaaagattcatctgtatggcatttttttctttctttctttctttcttttggagatggagtcttactgtgtcgcccaggctagagtacagtggcactatctcagttcaccgcaatctctgcctcctgggttcaagcgatcctcctgcctcaacctcccaagtagctgggactacaggtgtgcaccaccatgcccggctaagttttgtatttttagtagagacgggggtttcaccatgttggccaggctggtctcaaactcctgacctcaaatgatccacccgccctggcctcccaaagtgccaccgctcccggcctgtgtatggtatttttctatggcatgtaattttctgtacacaccctctttctttcttaggcttttttgtcagcagcccaagatggaaaaggcagctttatgtcaaggttcgccaaagacagtcaagagctgtgaaagccaaatgttcacatttaactttttttaaagtatttattactcggcatcaatgtatttcttaatcattatcctgagtggacttttaagtaggaagaaaatggtgtgttcattactccaaagctgaaacacagttggggttgtgtaaggtgacagcaggtgagttggtaaaagagttagcagaagtgacggctttcgtttcctcaactactggattcaccagtaagccacatgagacctcagtcacaatcggtaattcaaaggtagatttaaatataaatatcctgttatttctgacacctttactgaggtataattgatgtatgataaactgcatatatttaaagtgtacaatttgttaagttttgccatatggctacacttgtgaaccataaccacaatcaagagagtaaacacatatatcagccccagaagtttccctttgcccttttgtaatcatttcccctcgcccaccccattccaggcaaccaatgatgtgcttgcattattatagattagtttgcattttatagttttacataaatgtaattatacattttgtacacataaactgctggcgggaatgtcaaaaggtacaattaacttgaaaaagacttttagcagttccttaaaaatttaaatatacacttatcatatgatttagccatcccagtcctaggtatttgcccaagagaaatgaaagcttatgtccacataaagacttgtaaatgaatgctcatagcagctttacataatagcccaaaactggaaccaacaaatgtccatcaacaggtgaatggtataaacaaactgttatattctataccatgcagcactactcagcgataaaaaataatgaatgattgatacataaaacaacatggaagaacctcaaagaagccagggcatctgggtctggagatttcttttatcaggagattttaaattatgaatttaattctttaatggttataggatattcagattatttcatcttggttgagttttaatagtttgtggttttcaagaatcagattatttcttctaagttgtcatgtgtataagccgaaagttacagtatttcctcattatctttttaatgactgcctgatttatagtgatactcttcatttcattcttgataataatgatttgtgttttttctttttgtcagtctttctacaggtttatggattttcttgattgttttttgaagaaccagttttttgtttatgtatttttctatttgcagtttcattgatttctgcttttggttatttcctttcttttgcctgctttgggcttattttgctattctttttcttgtttcttgtggtgggaacttaggttattgtgctgagacctttcctcatttctaatatgctatcttcctaggtattccctgggatgtaggagacagctcttggagacacatggggttggctatctggcttttggagagactttgtctaccacaagaatagagtaaaagcagactctttcaggaagggaagaggatggctgcctctttcatctttataagtagggaaaattaattttccctgtcccttgcctatgcagtatttggccacttacatagccaaaatcccatgagtttcttatcaggttgctctgggggatatggacgagtgcaaaggtgggcaggtgcacttgtttaccctgagtaataagaaatctatctctgactctgaacatcttatgtgcatactcaagataagaaaaataaagatgaatattaaaaagcaaactttttatgagtggatactggtttatcaaatactttttctggatctactgaaatattatttttctcctttcattctgttaatgtgttgaatcatattgattgatttgcaactatcacaccaacctcactttttcaggaagaaacccaacttgattgtgattattctgtgtgtgtaggggtgtgtgtgtgtgtgtgtatgtgtgtagtttagtttgctagtattttgtttgggatttttgcattgatgttggggggaatgaaataggtccctttctcataaagtttttgccaggttttggtatctaggttttctggcatcataaaatgagttggggagggttcctgcatttctactgctctttgtaagaatttaagattgtctttccattgacgaatcaatccatctaggcttgttgtttcactatggaaaagcaaataaagtaactataggttccacttctttagcagatagggaactactcgaattttctattttttcatttgtcaattttggctcttccatagtttaaagaatttattcacttcatctaaaatttccaactaattggcatgaagttgtgcacatattttgtcagatgactctaggatttgtaatatcctttcattcctgatattggttgtttgtgtttcttcctttttcagtctaccagacacttatcaattatcttttcaaagaatcaacttttggcttagttgatccactttatcttcattttctactccattaattcttgttctttattatttcctttattttcttcaggtttaatttgctattcttagaatattttaactactaggttcattttcaatcttttttttttaatgtgcgtttaagactataaatttccttctaagcatggctttaggcgtctaccataagttttgacatgtagcactttcactactcagttcaaatatattctaattttcattgtaatttattgtctgatccatgagttatttaaaagtgtatttcttaatttatgaacttaatagaatttttctatttttgaaattattattgatttctaagtgaatgatacatggccaaagaatatattccattcctatgacttggaatatggtcagttttgataaatattctatctgcatttgaaaataatgtgtattttgcagttgttgggtattctgtttcatatatgccaattaggttaagttttaaagtattattccaatctttacatatttacgtatttttgcatggctgctgttctgttactgagtatattaaaatctgggaatgcagacttgtcttttctcattttagttctgttcatttctgcttatatatttgaggctatattgttaaatcattaaaatattagacctgttgaaactttctggtgaatcaaatcttttatcattacaaattgtctctctttgtaatacttttcaccttaaggtctacattgaataatgttgcaatagccaccatagtcccctgccctatcgtttttgttttttgtatttcatattataatttttccattcttgtttacttcaaacctttgtattcctatacttaagacatctcttgcataaaggtactttgtgggttttctttcttttcactttgatgatctttgcatttaattggtacactgtctattcatatgaatgttgtaactgatatttaaacctcctaatctactgtttgatttctatttgtcctatttgttctatattttctctacctttttgccttattattccactttagccctgtattagctttgtagttctacgattgttttattttgctttttgctgttcttttagtggttaccctatagatgacacagcagtcttatttatactttaatcttctttctgataattctgaccttagaattcctgcaccaaatttgtatattattgtcacattttaacattatttattttaacctcgaagactattttatatagttaatattcacttaaactgtatatatatatttttaaattactgttcattcctacctttatctctaacctttttctgggatctttttccttctgtctgaagaataccctttactatcacctttaatgacaatctgctattaaatttgttgcgtttgaaagtgtctttgccttcattcttaagaattgtttttggggaaaggctgggtattgaattctaaaattgcagatattttctttcagtaacctgaaaatatcatgccattgatttctgcttcccatattttctgttgagaagttagctgtcagtttaataaaattgtgcctcctttaaaagtaatgtcttttatcattgtctggctcctttaatgattttctttttgtgttttattttttcttaggatgtgctaagttgtaattttgtttttatttatcatgctttgatcttgcaggtcttcatgtcttaaaaacttggagaattctcagtcattatctcctcacaggttgcttctgccatattctctcttctcctggaaatccagttacgtgtatgttagatcttctcaagttaactctatgtctcttatactctctactatattttctattcttttgtctcttagtttttcacatctggtatttacttctgacataacttctagttcactaattcttacttcactgtatgcactttctatcaaatctattcactgaatcctttttttttttttttctttttgagatggagtctcgctctgtcgcccaggctggagtgcagtggcatgatcttggctcactgaaacctctgcctcccgggttcaagtgattctcctgcctcagcctcctgagtagctgggactacaggcacccaccaccacacccggttatttttttttttatttttactacagatggggtttcattgtgttagccaggatggtctcgatctcctgacctcatgatccacccgcctcagcctcccaaagtgctgggattacaggcgtgagccaccgcgcccggcctattcactgaattcttaaacttgattaatgtacttttaagttggggacttgttgattgattcttctatatagtttctgattttctgctgaaattctcaatcttgtgttttagatctttaaacacactaaacatagtaattttagaccctgtgttgtatagctcattatctgggtcccctgtggctctgtcccatcatctgtcgcttctttcggattttcatcatgttgtcttgtttcctcagataccttaaataactttccaacactaaacatgaaaagttataaaaataactcaaaagatcagtccagagaggatttacatttgctctgggtagcggctgcagcaaagggtcacctgaatccagttttgggaagtgagaagatcctaactgcatctggtttttcttcacccttacaatttggatatggtccttggggtcacaacccaatgtatggtcagttaactaggattcctttcccctcccctacttccttggagagtcttggtctccagtttttgtccctctaactcagcagcaaggctgttataagtgttacttagcgtctcagactctcaaccaccttatcctgaattggcatgtctcctataagaaaagcagcccaaatgctgagctcaggtctctaagtttcattctgtcttagatcttagtgatgttattcttcactgtcttttggttctctaatgcctttaagcagattttaaaatactattttgcctggcattgctagttctctgaaatagttggtatgaatgcaccactaaaagttagaagtagaaaagtaggttttagggaaaattcagtaacgttagtgttagtccaaactgcaccattttgtaagctccccgctattttgcagaccttgatcaaagtaaaacatttcacaggggttcgggcagtgagaaacatgctgcctaaccacctgaccacaaggcggaaaaaggcccaacctaagaaatatccctatcatatcttgctgggcaaagttccaaggaatactatgatgacatcccaccacaacaagggccagaaccacctcatcatgggagcatcttatcaatatcctgccgagcagcaagccatactgcccagacccctctcacccatgcctataagtacgcccagcctgtaagcagcggtgggctctggcattaagctggtcccccacttctgtaggttttatgctagacataaagtctgcatttgctgtcaagctgccctctgtgtgtctttctttaactctcaccttcccttcaaaatctaacagtcagtttttaatataccaagtgaagataccaaataagtgatatatataggttcagtgtaagaagagaggttgggttaggtacatatatttgatcatcatcaatttattgatgatatttcaagtcttgaagtagatgagattatctatggtgattgcagaaacacaaaggggggcctagaatcaattgttgagaaattctaaaatttagaggtcaggtagaagaggagaggcagcaaagatgtttgaggagttgctaggaagataagaagaaaacaaagataatgtagtgtcaggaaagttcaaaagaaaacacaaaagctgcttcaaggaatggtcaaatgtgtcaattactactagctggtttgacaataaaaaggtcaatagtgaccttaataaaaactttttttttttttaatttgggagagtcatggagatgggatccagattggaatgatttgacaagtaaatgaaagagaaaacctggctatgaatgaaatggagatatgggagcactttgaggaggatgcaaggttaagcgaaggcatagcttgacattattatcacagtgaaaatctctaaacaacttaaaattcacattatttgggggacagtagtccaataaataatatctatcaatggaattttatgctgtcattaaaagtgataattatggctgggcacggtggctcacgcctgtaatcccagcactttgggaggctgaggcgggcggagcatgaggtcaagagttcgagaccagcctggccaacatggtgaaactctgtctctactaaaaatacaaaaattagccggcgtggtggcatgcgcctttaatcccagctactcaggaggctgagccaggagaatcgcttgaacccagaaggcggaggttgcagtgagctgagatcgtgccactgcaccccagcctgggtgacagagcgagattccatctcggaaaaaaaaaaaagctgataattacaagtacttttaacgacatgagaaaatatttctacatgacaaagatataaaggtgtacagctagcaaatctcaatcatgtaaattaaatcataagtctgagatgtaaactcagagtaatacaaaatcctatcttagtaactgtactatattacctccaaaaaaagaataacatacaaatctcttgaattcattaactgaaaattggtccaaaaagtttatcctttaacattgttagagtgaactcgtccacatactaaataaatggaatactaataacaacttaactggtacatttcatataatttgaatgatttctaaggagaatacattattataaatctagggggctcctactgatttcattggaaattaagtaagaattagaggaaactgatctctcaactgatgtggattcattattaatcccccttacatgtatctgtaaaacgttcctaagcaagaagagaatgaaaataaaattcagatcgtattataaaaattttcttccatctccttctgactttagttcatataccttaagacactagtaactggtagtcctgttgggtaaatcatttttcagaagcagtaaattcagttgaaagaaatacataatgagtcagatatatgctttagtagtcatatgcagattaccctaacattgctcttcctgtgaatattcacatgatgaatgggatgaaccccgctcctttcacatatattagaaggatatttgaaaaggaaggaaaatattttattaaaagttttttaaagtttatgaattgaagtctatgaaaacaaactacttgatacaaaaacattcagatattagatgtcaaaataaatcagcacatttgaaaatactataaattatatttcaaacaaatatatacacattatgttaaccttcaacaggatccattatcactacttagaacactgatatgtttatctcttaagtatgtaaaaattacatagctgttaactttgtatggcaattcacctataacacatttaagaaagcattacaaaattcattatatgataattctacaaaagttttctcacatttaccaaagcctactaaagtccagagggcacaaatattggccaaatagttcttttatcttagacataaagatgtttttgctgttttttagaaccattaagatggctaagagaaccaactttacggagcttagctgttctcaggcatctgaatgggggtgtggagaagtcctcaagttacaagaatcacagttacttttttaggatgaaaaaataaaaacattgcatttgatgacattacagtcaaaatgagctctaatacaaatgtatgtggagaggttttgaagaataaatcggatatcccaggggaggttctgctgcttgtaccgtaagatttcttaaaagtagtggatgagcttgtatactataacgttcttcatcatcgtttgtggcataaagtaattcccatgaaagattggcccactgacctctaacagcttcaggatttaactttcccacttggatcaataattcttgaaggctaagcactctcccagtgtaaattcccatattagaatcataccccagagaaaacaagtatggcttttcttgtaaaattgcttccttccacttttcatcagataccaaaccaatgtaccagtcacgttcatattcttcaaggtacttaatcagttctctaaagtcttctattggacctaaacttgctttatcaatcattagtttcagagtatacctgaatgctttcagtgctagttgaaacagttctggcttttctgtgagccagtccaaagcaacagaccaaggcaaaacaccaccgtaaactctcaatatatgaccaggactaggagccatattgtctattccaaataaactaaaataacaagtcattactgtatgaacataaaagtcttttaaaactttgtccttggcaatttcttccagtacatttgaggccttctcttctgaatgataacattccaactgccttagaacaaattggtaccagtcttctggaaataacgagctcatctccttcattttggaactgggcatacagctagtcctccactctgcgggtaagcatactaagtgagaatgtgaacaactgaactccatgagaggaatatatggcatgtcctcttgttttcctttgtcaacagcagggtatcctaatagaactgctttgtaaagatcgttttcaggaacagtgcctgtagaatgatcaccaaccctctgtgattctactgatcctggaataaacaaatttgtacctggcaaatctttcaactgatgtttttcttctattacttttttgatagttggctcatcatcaaaaatattatcatcagaccagtcattaaaagtttctgaatttaaactgtctatgtcttctggggatttgggaggtggcaaagtgttcaaagcaggcaacattagaggtgctttccctttattttcagtgttgtgaacattctctttcatgccaggccttttggagcagtattgaacaagtatccacacaagtactttaatgaggtcacctttaaattcttttaagttttcatgagaatcaattatgcctgatagaacattcctggcatcagaatacaatttcacaggcaaaacagtacagggtgtcaagacatttccaaagtgttcattaagggaacatactcttgtgtattcttgctcaaaagcatcttcaaaaacttcatcaactctgcgagcttctgcagtatgacaggatgtttcctgcaattctaaccccttaatgttaatagagcagtaagtatagccacattccagaatcattatccacattaaacgatcctgaaaacggcccaagtaatgagatccaggtaggaggagacctaaacttccagctgccattgcagtctgcagtacagcagtcaacctgggcaccatttggtagtagtacactgtatctgcacacacacaggctgtggtgcctgctgctcctggccaactctgaataggtcggggaaaccccaccaagaacacaggaagggtgaaaagagggagtaagggagaagagagtagtgtagaaaaaactatgatgaccaacacgaatggagaaaagacaatgttgagtatacataaagtggcagttgtttttcgacgttgttttttctctgtccatgatgtcaaaagcacagtcacggcaaactgcaatttagagatgaactgaatcaaacgatcacgtatgataccaaccagtaagagtctgagtcctgtatccaggcttctgttccaccatatgtctgtactggagatcaagtgtactgttgatacaatgactgtctccaataaagcattttctgtattctgccataccattctaaaggctcttgtgaatccaatacagacagacactgagtggagcccttgtaaggaactgtccaatgaaagaaatgctatcatggcaaaaggtgatactaaagttagcaaaatccgtctgacaataccaatcttcatgagcctagtttgcttctcaaagaatacagtcacagtttgcacatccttcggataaaagggatttcggaaaattccaatgatatatacgctttgaatttctctaagtatccacagtattataagtaatatcatcaaaccatagcccacaatagcctgggaattgcttttagaaatctgtgagaagccagcaaagtgatgaagcaagctagtttctaaaagagccaagactaatataatgatgtagaaaaggcattccttccatgaaaaatgtttttccggaccactgggtaaatccttagatttggttccaattttgtgacccatatcacttaagttcagactcagcaagaaaccaaatccagtcatgaaaagaaccacaccaacagtgcttggaatgaaatatgatgctatagctgttccagcagacatgatgaacattactaataaccgtaagtgggttgacatagatgagcctccaaggccgaactctaaaacctgctccattgcccataagagaagtgcatcgggtgggggcagagtcccaagtgcccacagaaagggtaaaaatacaaacaagatgtgtaaaatctgattcatgtgttctagagctggcatatttaccacaaacctgtgtgccagatccacagaaacaaagaaaaaaatataaagaggtctcataagaggaataatttcataagtatcctgtgtttggaaagtcgcagtctctgtagctgtgtttacaattaaagaatattctgctatacatagtgtcatccatccaaagaagaatagtagagcagtgcctcctgtactgccatacagcaaggttattctatttgggagcagataccatgttccaagaccacacgctaatccagcaagaatagaatgaaaaactgtattggctacatatttcttgccaggaatgagaaatttgacagtctcagcaccagtacaactggtaaattcatgctcatcctcctctgctaagatatccgtggttagtattctttctactgttgttgatttgtttttggcgtataaacttgtgaactggatgacaaatgcagtaaaaagcattaatccacctgaaagtgctgctgtataatagtctttcaggatgcctaactggtataaaagtgttccgactccaccccaaacccatggcattagaaaaagaataatttgattaacatatatgtaaggaggggcacaatagcctaatttgaatcgagggcctccaagaacagtctgtggaaagcgcttcagaaagaagtcctgcttgtaatcattcagtagaggcacatctggactcatcctcactcgggattattctgaaagtcacatgcttttctgtaacacagcagtttctcaagtcacccgagggaagagaagacgcgaaggcatcccagggaccgcatttttgcaggtaaactcgggctgggcgctcccgccgggaggttggttagtgcccgaatgcggaggcagaaaagctgcggcggccgaataacgagctcaccgcggccccgcccgggccagctctcggtttccatggctaacgtctactccggcggccgccacccggagctgaacggagcgcgtgcgcgttcggggacctcgtcggcgcctggctggcctcgctgccccggtctgtgctcgctcccgaggcgggccctgccgtaaagcaggcttggcctagaggaagcagggaaatagcgcgcttcgttcgcgccaggactaggccaacatctgcctggccggggacgacgggagtcgctcgtgctctggtctcgcactgggcctagcagaagcagcagcggggaaagccgagacgccctgaacgttcccttgggccgggcctttacgc

SEQ ID NO: 12951 - RNA, 6635 nt, Homo sapiens
  source 1..6635: mol_type = other RNA
gctgggattacaggcatgagccacagtgcctggactcatttattgattcaatcatttatttatatcggtgtgggctcgaggatatttattttattctttgggttgtgatccaacactgctttattttgttgctcacactgtttcagcttcagccactgggaacatcttccctctgcatgcccatctcacatcactgtatgtataaagttctgccttgctctctgactctacaagatgctccaggctcatcttgtatactttctgccctagttttagaatcagctatttctccagcgatccctggttcgttttattggagaatggtgttagcaaccaagatcttggagctaggtatacattactcgtaaatgaaaaaaacccactataattctcaatagggaaaacagtgcttcctatggagcccacactcaaaaatgttggcactgccagtgatcgctcggctggggctttcaggacgtaaatgatgctttcatacatatcagtgtaaaaagctctgctcgtgaattctcatgtccgctcattttacacaatgagcaagctgacaggacaatacacaactatgagcataattaagaaaggttttttttttttttccttttataggaacacttcgtgctctgattctgaaaccgcctttgcaaaattgtaactgaggtggggaaagagatctgacctaaccaactccatcttgcttctaacctccaagctgtccttgttcattcctgggtgtaggctcaactaactttgggagaaacttagtttagtttatagtttaaaacaaagatgataacagccctttcccaagacaaacccccttcttgtctggggactagatttcctttgtaggactaacaaattagcctcaagattagaaattatggttcaggagtcatgtagctggaagctacaagattctgaccctccctaaactgctcctatgtcggtgctcgagatattttgcagacctgcactcgacggatcagctggcaccacccagatcgattaactggctcatctgatctcgtggcccccaccctggaactgacttagcacaaaaggacacctcaattccttatgatttcatctccgacccaaccaatcaacacccttgactcactggccttccccctcccaccaaattatccttaaaaactctgatccccgaatgctcagggagatcgatttgagtactaataagactccagtctcctgcacaagcagctctgtgtactcttcctctattgcaattcctgtcttgataaatcggctctgtgtaggcggcggaagaggtgaacctgttgggcggttaccacctctgtcgtgtgtgacagttgttttgaatctctaattgctcagtacagatcccacatgcaggttaagtaagatgctttgaagaaaatggaaagtcttaagtgattgcttccaagaaatcaaacctacatttatctaggtaacaacggactttacgtatcacaaatgaagagactgacaaagtaaatcaacttggccttttcttaggtatgtcaagtcagttttttttttcctaaggtgttgaaatggaaattcttccatttcactaattagcattcctttttggatgtttcgaaaataaaaaataaatctaaaatatgtaataaacggcaagtacaaaaagggcttgacagaaaaataacatgttacttttaccagatctaacatgaacatcttctaaggtaaattcgttttcagaatttgtctaaactattcttaggctattcatctaccccgcaacaggacaatgtctgctctgttttagctttctcaatagattgtaagcaaatctctttgcggcacatatttaaaacagaaagacaacatttgatcttatctgatgccagagccttcttgatcttacggaagatgtgaacgagttttcctggaactgtaacacactgccatctggctgatacacactggaagacaccatcaatttaaaagtgttatcatgattttagaggaaaatgtggtgtggagaaaggcctgtctttgaatggatgaaataggttaataaaaaacatcactgtttaaaaactagaacactgaaaaattctaggaaagcttattttcccttatatttttatggtactttcaacacttaataacactatttcaattaagttttctcctagagtttatagtatatcagtacattcttttctgtggatgcaataatatagaatcttattccaaatcttactggcaggttctcttaaattcttcaacggctgccatagtgattaaccaaaattagttatgatttctgcctatctgtgtgagaacttacaggggaaattgttctaaacctgaggaacatgaagtaactgtactgcacactccaaatgatgacagtcattttatatcaccttcaattacccaacagcttttaatagtctggccataagtttctttgcacgagcatttgttaaataactaccattcagtcaaagaaggtaagggaagtcctgtttaaagaatcctaagtaatcctaatcctaagaattataaataattattaattttatacaagtatcaacaaaaacttacccagtagtttgtctataaatttggtatgtactcaagcacacctcagtgtgtatgcatgtaaatgggtaattcccatttactgggtatttgtgtctaatacatgtgcacattagcagggcagtggaaaggaaagggaaaaattgcaaacattcacaggaatgctctacatataaaaaattggtacaaatacatacaattctttttttacagtcaagtttaaattcttacaaacaaacttaccttttctggaatattttgagtaataatgtctaaatgtgataaaactgctaaaaacgtacaaatgcttgttttaagattttcttcaccataagaaaaacaatcccagaactttggaagaaattgagggaatttatgaagaatcaatataataatccattctataaaatattttatggatgcttgattgttggtgaaaccagcctggaaaatcctgtcaataattccattcaagaaattctggtcaagtctagggaaaagtaccagcagagtctgccacactcggtttttcactctgtgctgtagagaattcacatagtagcgttttttggacttggacactaattcatctttatctaatagcttgattgcaagatcctcaataaacaacttgtgggacatattggagccatctaataaacacaggaatttgacagcacaaattctcacataatggtcttctctcttagtactttgatcacgcctaaacacagttccaaatatacaagcctcaaggataagttcgctataatttttagcacttgataaagatccttgggacacatttgaagcagacactatccaagactgacagcagtaacttatcagtgtattgaagactccagtctttatagcagacatttcaattatcttgtacataatctcttttattttgaaatatgcctggcccttgattttggcagcaatggtaagaactttgttatcaaaaacaaactgaacaaaagcttttaaattagcccagaatatcagctgagtgttgcttaaagaagatataattttccacgccatgtcaaaagactctatgcagagtgattcagaggaagtcagaagcttgggaaccaacactttcaagcaatggaacactggtaaaacttgatcagaagaaagaactgtgagggcttctagtgcagactgcaaagtccttattggcatctgaacggcaggtagaaacggttccagaatttcactccctgtggttggtataagggtgtgatattttttcaacaggaaagagaggcacacccattgatcatgaatatattgtgcaactatttttccccatccttgggaagatgacgattcttccaaaacactgctgcactccaaggggtgagcataactgctctgctcctctgcgtggggcttctgcagcgtctgattgagctgaagagaggaaaggaagctttccaggggcccagcatggagagagtccagctgcagctcaggcttctggtctatggcctcacacaccatggccaaggcagccatgctcactactctctgaatctgacttccaactgttggctcctgtccactgtccatctcttgaagatgctgaatggatgcatttttcaaaagagaaataactctccagatagggttaccccttttccacccaaccttcaaatgcagatttataagctcagttaacaccatcaggtataaatggcaacgatccagatctgaaacactatttagctcattcatagtaagtcttctgagaataaattcagaaatgctctctgtagtagacatgaaaaagttctgaagaacagtagacacctcatcatcttgggcactggaacctttcaacctgcatgtgttcaacagcttcaacagcagctggaggcatctgtcagtcttcagcaagggcatgtaggcattggtactaaacttcataagcacatccagaagagggtctaagaatatccgcaatacattctctgttctctgctttccgctatactgagtcttcattccttccacatccacagccagcaagaccatcagagaaacaagcttggcttcaaaccaatcaggcataaagcagttttctcctgtttcccaagcagatgacttaacatactcttgaacaatgctctttacataagcatttaaagatgtcttgtgaagtccaatggagctacacgtaggggatggcttaaaatagctttcattaacacgtagccagtcacacagctctgtccacaatgaagttcctcgtcctaaggattcctcttgtctcagagacatgagaaaagttgagacatcagaaagtgacactttctccacatctagcaaattcatagctgtttgaagaaggtagcattgggctgcccctctcaggagaatctgatgtgtgatcatagtgcaatgaataacatccctgagagcaagaagcccatctatacccagggccttatgtcttgggacatttgccaaagccttagatagaaacaaaatgggaacagcacaccaatgcctacttgtcatcttccgaataaacttcaataggaagctactctttatttcttctggaagaagagaaatataagtgactaaaaacttctgtaatttcagtcccaatggagaacagcttcctattggctggcctggggacctgctatacagagagctctctgaaagcgcatccattaatggtccaataataaactcagaaaattctggtgaaaatggaagaatctttgtttcatacagctccaaaaaatggataacaccttctttggacaggattttgttttcactttcaaacattcttttataaatacacatatgccaggatgggtgaaagagccaacatccattttcctctgacaccgcatattcaaacagattgtttagctttggtaaaactggctttataacatgtatctgatttccttctaaagtctccataattaaaatataattttcccaaaactttagaagctcatcttttttcctctcagaccaccaaaacagacttgggccgtttccttcctggggcccgcaggtgcagtcggcccccagctccgccgacacctccaccgccctctgcagcaggtagcgcgctcgcttgcgcgtcagggcgtccgcctggcccagccccgcctgcaccgtcctccagaagcgccagcagcgccgggcgtccgggcccgcctcgcgcgcgccgcgggcgcggtcgccgccgggctcgggcaacagcttctcggccagggcgctcaggaccagcagcttctcctctacgcggccggaccccagggacgccccaggcgcggccagcccgccccacacggcccgcagcgccgccccgccacattggaccagcactggcagcagtcgcccggccaccagcgccgccgcgtcctcggcaggcccggcctcatccccgtccccgcccccgcccagcgccagggcgacggcggtccccgccacgcgctccagtagcggcccgtcctcgcggggccgcaaacatggcccgacggctgctagcacttccacggcagcctcggcgccaggcgcgcgccacccggcgagcagatcgcgcagcgcctcctcagccagcgcggccgccagctgcggacgcccggccaggcggacgcacgagcgcagggccgcgcccgccgccctcagcacgcgccggcggtggcgaggctgcagactggggtccgggccgcccgcggggcgtccgcgcaggctccgcagcagtggcacgaggtaccctgcagccacctcgcgcgccgcctccgggagcgcgcctgcgcccccgctgccgcgcgcctcctcgtcctcgagccgctgcagaaggaagcgcagcgtctccacgcgctccgcggatgcctccccttggcacagcgccccaagcagggcccgggggtcccggctctgcgagagcagcgcttccgcgagcacccactccatttgccgagcgcccgcgccaccggcccgggctcccaaaggaaggcgccggcgtgtgcgatgcgtgcgcacag

SEQ ID NO: 12952 - RNA, 6703 nt, Homo sapiens
  source 1..6703: mol_type = other RNA
gctgggattacaggcatgagccacagtgcctggactcatttattgattcaatcatttatttatatcggtgtgggctcgaggatatttattttattctttgggttgtgatccaacactgctttattttgttgctcacactgtttcagcttcagccactgggaacatcttccctctgcatgcccatctcacatcactgtatgtataaagttctgccttgctctctgactctacaagatgctccaggctcatcttgtatactttctgccctagttttagaatcagctatttctccagcgatccctggttcgttttattggagaatggtgttagcaaccaagatcttggagctaggtatacattactcgtaaatgaaaaaaacccactataattctcaatagggaaaacagtgcttcctatggagcccacactcaaaaatgttggcactgccagtgatcgctcggctggggctttcaggacgtaaatgatgctttcatacatatcagtgtaaaaagctctgctcgtgaattctcatgtccgctcattttacacaatgagcaagctgacaggacaatacacaactatgagcataattaagaaaggttttttttttttttccttttataggaacacttcgtgctctgattctgaaaccgcctttgcaaaattgtaactgaggtggggaaagagatctgacctaaccaactccatcttgcttctaacctccaagctgtccttgttcattcctgggtgtaggctcaactaactttgggagaaacttagtttagtttatagtttaaaacaaagatgataacagccctttcccaagacaaacccccttcttgtctggggactagatttcctttgtaggactaacaaattagcctcaagattagaaattatggttcaggagtcatgtagctggaagctacaagattctgaccctccctaaactgctcctatgtcggtgctcgagatattttgcagacctgcactcgacggatcagctggcaccacccagatcgattaactggctcatctgatctcgtggcccccaccctggaactgacttagcacaaaaggacacctcaattccttatgatttcatctccgacccaaccaatcaacacccttgactcactggccttccccctcccaccaaattatccttaaaaactctgatccccgaatgctcagggagatcgatttgagtactaataagactccagtctcctgcacaagcagctctgtgtactcttcctctattgcaattcctgtcttgataaatcggctctgtgtaggcggcggaagaggtgaacctgttgggcggttaccacctctgtcgtgtgtgacagttgttttgaatctctaattgctcagtacagatcccacatgcaggttaagtaagatgctttgaagaaaatggaaagtcttaagtgattgcttccaagaaatcaaacctacatttatctaggtaacaacggactttacgtatcacaaatgaagagactgacaaagtaaatcaacttggccttttcttaggtatgtcaagtcagttttttttttcctaaggtgttgaaatggaaattcttccatttcactaattagcattcctttttggatgtttcgaaaataaaaaataaatctaaaatatgtaataaacggcaagtacaaaaagggcttgacagaaaaataacatgttacttttaccagatctaacatgaacatcttctaaggtaaattcgttttcagaatttgtctaaactattcttaggctattcatctaccccgcaacaggacaatgtctgctctgttttagctttctcaatagattgtaagcaaatctctttgcggcacatatttaaaacagaaagacaacatttgatcttatctgatgccagagccttcttgatcttacggaagatgtgaacgagttttcctggaactgtaacacactgccatctggctgatacacactggaagacaccatcaatttaaaagtgttatcatgattttagaggaaaatgtggtgtggagaaaggcctgtctttgaatggatgaaataggttaataaaaaacatcactgtttaaaaactagaacactgaaaaattctaggaaagcttattttcccttatatttttatggtactttcaacacttaataacactatttcaattaagttttctcctagagtttatagtatatcagtacattcttttctgtggatgcaataatatagaatcttattccaaatcttactggcaggttctcttaaattcttcaacggctgccatagtgattaaccaaaattagttatgatttctgcctatctgtgtgagaacttacaggggaaattgttctaaacctgaggaacatgaagtaactgtactgcacactccaaatgatgacagtcattttatatcaccttcaattacccaacagcttttaatagtctggccataagtttctttgcacgagcatttgttaaataactaccattcagtcaaagaaggtaagggaagtcctgtttaaagaatcctaagtaatcctaatcctaagaattataaataattattaattttatacaagtatcaacaaaaacttacccagtagtttgtctataaatttggtatgtactcaagcacacctcagtgtgtatgcatgtaaatgggtaattcccatttactgggtatttgtgtctaatacatgtgcacattagcagggcagtggaaaggaaagggaaaaattgcaaacattcacaggaatgctctacatataaaaaattggtacaaatacatacaattctttttttacagtcaagtttaaattcttacaaacaaacttaccttttctggaatattttgagtaataatgtctaaatgtgataaaactgctaaaaacgtacaaatgcttgttttaagattttcttcaccataagaaaaacaatcccagaactttggaagaaattgagggaatttatgaagaatcaatataataatccattctataaaatattttatggatgcttgattgttggtgaaaccagcctggaaaatcctgtcaataattccattcaagaaattctggtcaagtctagggaaaagtaccagcagagtctgccacactcggtttttcactctgtgctgtagagaattcacatagtagcgttttttggacttggacactaattcatctttatctaatagcttgattgcaagatcctcaataaacaacttgtgggacatattggagccatctaataaacacaggaatttgacagcacaaattctcacataatggtcttctctcttagtattttccataacaatatttgccgcacagtcatgtccaaggttttctatgaaggtctgtacatcctgaacaagtctttgatcacgcctaaacacagttccaaatatacaagcctcaaggataagttcgctataatttttagcacttgataaagatccttgggacacatttgaagcagacactatccaagactgacagcagtaacttatcagtgtattgaagactccagtctttatagcagacatttcaattatcttgtacataatctcttttattttgaaatatgcctggcccttgattttggcagcaatggtaagaactttgttatcaaaaacaaactgaacaaaagcttttaaattagcccagaatatcagctgagtgttgcttaaagaagatataattttccacgccatgtcaaaagactctatgcagagtgattcagaggaagtcagaagcttgggaaccaacactttcaagcaatggaacactggtaaaacttgatcagaagaaagaactgtgagggcttctagtgcagactgcaaagtccttattggcatctgaacggcaggtagaaacggttccagaatttcactccctgtggttggtataagggtgtgatattttttcaacaggaaagagaggcacacccattgatcatgaatatattgtgcaactatttttccccatccttgggaagatgacgattcttccaaaacactgctgcactccaaggggtgagcataactgctctgctcctctgcgtggggcttctgcagcgtctgattgagctgaagagaggaaaggaagctttccaggggcccagcatggagagagtccagctgcagctcaggcttctggtctatggcctcacacaccatggccaaggcagccatgctcactactctctgaatctgacttccaactgttggctcctgtccactgtccatctcttgaagatgctgaatggatgcatttttcaaaagagaaataactctccagatagggttaccccttttccacccaaccttcaaatgcagatttataagctcagttaacaccatcaggtataaatggcaacgatccagatctgaaacactatttagctcattcatagtaagtcttctgagaataaattcagaaatgctctctgtagtagacatgaaaaagttctgaagaacagtagacacctcatcatcttgggcactggaacctttcaacctgcatgtgttcaacagcttcaacagcagctggaggcatctgtcagtcttcagcaagggcatgtaggcattggtactaaacttcataagcacatccagaagagggtctaagaatatccgcaatacattctctgttctctgctttccgctatactgagtcttcattccttccacatccacagccagcaagaccatcagagaaacaagcttggcttcaaaccaatcaggcataaagcagttttctctttcccaagcagatgacttaacatactcttgaacaatgctctttacataagcatttaaagatgtcttgtgaagtccaatggagctacacgtaggggatggcttaaaatagctttcattaacacgtagccagtcacacagctctgtccacaatgaagttcctcgtcctaaggattcctcttgtctcagagacatgagaaaagttgagacatcagaaagtgacactttctccacatctagcaaattcatagctgtttgaagaaggtagcattgggctgcccctctcaggagaatctgatgtgtgatcatagtgcaatgaataacatccctgagagcaagaagcccatctatacccagggccttatgtcttgggacatttgccaaagccttagatagaaacaaaatgggaacagcacaccaatgcctacttgtcatcttccgaataaacttcaataggaagctactctttatttcttctggaagaagagaaatataagtgactaaaaacttctgtaatttcagtcccaatggagaacagcttcctattggctggcctggggacctgctatacagagagctctctgaaagcgcatccattaatggtccaataataaactcagaaaattctggtgaaaatggaagaatctttgtttcatacagctccaaaaaatggataacaccttctttggacaggattttgttttcactttcaaacattcttttataaatacacatatgccaggatgggtgaaagagccaacatccattttcctctgacaccgcatattcaaacagattgtttagctttggtaaaactggctttataacatgtatctgatttccttctaaagtctccataattaaaatataattttcccaaaactttagaagctcatcttttttcctctcagaccaccaaaacagacttgggccgtttccttcctggggcccgcaggtgcagtcggcccccagctccgccgacacctccaccgccctctgcagcaggtagcgcgctcgcttgcgcgtcagggcgtccgcctggcccagccccgcctgcaccgtcctccagaagcgccagcagcgccgggcgtccgggcccgcctcgcgcgcgccgcgggcgcggtcgccgccgggctcgggcaacagcttctcggccagggcgctcaggaccagcagcttctcctctacgcggccggaccccagggacgccccaggcgcggccagcccgccccacacggcccgcagcgccgccccgccacattggaccagcactggcagcagtcgcccggccaccagcgccgccgcgtcctcggcaggcccggcctcatccccgtccccgcccccgcccagcgccagggcgacggcggtccccgccacgcgctccagtagcggcccgtcctcgcggggccgcaaacatggcccgacggctgctagcacttccacggcagcctcggcgccaggcgcgcgccacccggcgagcagatcgcgcagcgcctcctcagccagcgcggccgccagctgcggacgcccggccaggcggacgcacgagcgcagggccgcgcccgccgccctcagcacgcgccggcggtggcgaggctgcagactggggtccgggccgcccgcggggcgtccgcgcaggctccgcagcagtggcacgaggtaccctgcagccacctcgcgcgccgcctccgggagcgcgcctgcgcccccgctgccgcgcgcctcctcgtcctcgagccgctgcagaaggaagcgcagcgtctccacgcgctccgcggatgcctccccttggcacagcgccccaagcagggcccgggggtcccggctctgcgagagcagcgcttccgcgagcacccactccatttgccgagcgcccgcgccaccggcccgggctcccaaaggaaggcgccggcgtgtgcgatgcgtgcgcaca

SEQ ID NO: 12953 - RNA, 5836 nt, Homo sapiens
  source 1..5836: mol_type = other RNA
gctgggattacaggcatgagccacagtgcctggactcatttattgattcaatcatttatttatatcggtgtgggctcgaggatatttattttattctttgggttgtgatccaacactgctttattttgttgctcacactgtttcagcttcagccactgggaacatcttccctctgcatgcccatctcacatcactgtatgtataaagttctgccttgctctctgactctacaagatgctccaggctcatcttgtatactttctgccctagttttagaatcagctatttctccagcgatccctggttcgttttattggagaatggtgttagcaaccaagatcttggagctaggtatacattactcgtaaatgaaaaaaacccactataattctcaatagggaaaacagtgcttcctatggagcccacactcaaaaatgttggcactgccagtgatcgctcggctggggctttcaggacgtaaatgatgctttcatacatatcagtgtaaaaagctctgctcgtgaattctcatgtccgctcattttacacaatgagcaagctgacaggacaatacacaactatgagcataattaagaaaggttttttttttttttccttttataggaacacttcgtgctctgattctgaaaccgcctttgcaaaattgtaactgaggtggggaaagagatctgacctaaccaactccatcttgcttctaacctccaagctgtccttgttcattcctgggtgtaggctcaactaactttgggagaaacttagtttagtttatagtttaaaacaaagatgataacagccctttcccaagacaaacccccttcttgtctggggactagatttcctttgtaggactaacaaattagcctcaagattagaaattatggttcaggagtcatgtagctggaagctacaagattctgaccctccctaaactgctcctatgtcggtgctcgagatattttgcagacctgcactcgacggatcagctggcaccacccagatcgattaactggctcatctgatctcgtggcccccaccctggaactgacttagcacaaaaggacacctcaattccttatgatttcatctccgacccaaccaatcaacacccttgactcactggccttccccctcccaccaaattatccttaaaaactctgatccccgaatgctcagggagatcgatttgagtactaataagactccagtctcctgcacaagcagctctgtgtactcttcctctattgcaattcctgtcttgataaatcggctctgtgtaggcggcggaagaggtgaacctgttgggcggttaccacctctgtcgtgtgtgacagttgttttgaatctctaattgctcagtacagatcccacatgcaggttaagtaagatgctttgaagaaaatggaaagtcttaagtgattgcttccaagaaatcaaacctacatttatctaggtaacaacggactttacgtatcacaaatgaagagactgacaaagtaaatcaacttggccttttcttaggtatgtcaagtcagttttttttttcctaaggtgttgaaatggaaattcttccatttcactaattagcattcctttttggatgtttcgaaaataaaaaataaatctaaaatatgtaataaacggcaagtacaaaaagggcttgacagaaaaataacatgttacttttaccagatctaacatgaacatcttctaaggtaaattcgttttcagaatttgtctaaactattcttaggctattcatctaccccgcaacaggacaatgtctgctctgttttagctttctcaatagattgtaagcaaatctctttgcggcacatatttaaaacagaaagacaacatttgatcttatctgatgccagagccttcttgatcttacggaagatgtgaacgagttttcctggaactgtaacacactgccatctggctgatacacacttttctggaatattttgagtaataatgtctaaatgtgataaaactgctaaaaacgtacaaatgcttgttttaagattttcttcaccataagaaaaacaatcccagaactttggaagaaattgagggaatttatgaagaatcaatataataatccattctataaaatattttatggatgcttgattgttggtgaaaccagcctggaaaatcctgtcaataattccattcaagaaattctggtcaagtctagggaaaagtaccagcagagtctgccacactcggtttttcactctgtgctgtagagaattcacatagtagcgttttttggacttggacactaattcatctttatctaatagcttgattgcaagatcctcaataaacaacttgtgggacatattggagccatctaataaacacaggaatttgacagcacaaattctcacataatggtcttctctcttagtattttccataacaatatttgccgcacagtcatgtccaaggttttctatgaaggtctgtacatcctgaacaagtctttgatcacgcctaaacacagttccaaatatacaagcctcaaggataagttcgctataatttttagcacttgataaagatccttgggacacatttgaagcagacactatccaagactgacagcagtaacttatcagtgtattgaagactccagtctttatagcagacatttcaattatcttgtacataatctcttttattttgaaatatgcctggcccttgattttggcagcaatggtaagaactttgttatcaaaaacaaactgaacaaaagcttttaaattagcccagaatatcagctgagtgttgcttaaagaagatataattttccacgccatgtcaaaagactctatgcagagtgattcagaggaagtcagaagcttgggaaccaacactttcaagcaatggaacactggtaaaacttgatcagaagaaagaactgtgagggcttctagtgcagactgcaaagtccttattggcatctgaacggcaggtagaaacggttccagaatttcactccctgtggttggtataagggtgtgatattttttcaacaggaaagagaggcacacccattgatcatgaatatattgtgcaactatttttccccatccttgggaagatgacgattcttccaaaacactgctgcactccaaggggtgagcataactgctctgctcctctgcgtggggcttctgcagcgtctgattgagctgaagagaggaaaggaagctttccaggggcccagcatggagagagtccagctgcagctcaggcttctggtctatggcctcacacaccatggccaaggcagccatgctcactactctctgaatctgacttccaactgttggctcctgtccactgtccatctcttgaagatgctgaatggatgcatttttcaaaagagaaataactctccagatagggttaccccttttccacccaaccttcaaatgcagatttataagctcagttaacaccatcaggtataaatggcaacgatccagatctgaaacactatttagctcattcatagtaagtcttctgagaataaattcagaaatgctctctgtagtagacatgaaaaagttctgaagaacagtagacacctcatcatcttgggcactggaacctttcaacctgcatgtgttcaacagcttcaacagcagctggaggcatctgtcagtcttcagcaagggcatgtaggcattggtactaaacttcataagcacatccagaagagggtctaagaatatccgcaatacattctctgttctctgctttccgctatactgagtcttcattccttccacatccacagccagcaagaccatcagagaaacaagcttggcttcaaaccaatcaggcataaagcagttttctcctgtttcccaagcagatgacttaacatactcttgaacaatgctctttacataagcatttaaagatgtcttgtgaagtccaatggagctacacgtaggggatggcttaaaatagctttcattaacacgtagccagtcacacagctctgtccacaatgaagttcctcgtcctaaggattcctcttgtctcagagacatgagaaaagttgagacatcagaaagtgacactttctccacatctagcaaattcatagctgtttgaagaaggtagcattgggctgcccctctcaggagaatctgatgtgtgatcatagtgcaatgaataacatccctgagagcaagaagcccatctatacccagggccttatgtcttgggacatttgccaaagccttagatagaaacaaaatgggaacagcacaccaatgcctacttgtcatcttccgaataaacttcaataggaagctactctttatttcttctggaagaagagaaatataagtgactaaaaacttctgtaatttcagtcccaatggagaacagcttcctattggctggcctggggacctgctatacagagagctctctgaaagcgcatccattaatggtccaataataaactcagaaaattctggtgaaaatggaagaatctttgtttcatacagctccaaaaaatggataacaccttctttggacaggattttgttttcactttcaaacattcttttataaatacacatatgccaggatgggtgaaagagccaacatccattttcctctgacaccgcatattcaaacagattgtttagctttggtaaaactggctttataacatgtatctgatttccttctaaagtctccataattaaaatataattttcccaaaactttagaagctcatcttttttcctctcagaccaccaaaacagacttgggccgtttccttcctggggcccgcaggtgcagtcggcccccagctccgccgacacctccaccgccctctgcagcaggtagcgcgctcgcttgcgcgtcagggcgtccgcctggcccagccccgcctgcaccgtcctccagaagcgccagcagcgccgggcgtccgggcccgcctcgcgcgcgccgcgggcgcggtcgccgccgggctcgggcaacagcttctcggccagggcgctcaggaccagcagcttctcctctacgcggccggaccccagggacgccccaggcgcggccagcccgccccacacggcccgcagcgccgccccgccacattggaccagcactggcagcagtcgcccggccaccagcgccgccgcgtcctcggcaggcccggcctcatccccgtccccgcccccgcccagcgccagggcgacggcggtccccgccacgcgctccagtagcggcccgtcctcgcggggccgcaaacatggcccgacggctgctagcacttccacggcagcctcggcgccaggcgcgcgccacccggcgagcagatcgcgcagcgcctcctcagccagcgcggccgccagctgcggacgcccggccaggcggacgcacgagcgcagggccgcgcccgccgccctcagcacgcgccggcggtggcgaggctgcagactggggtccgggccgcccgcggggcgtccgcgcaggctccgcagcagtggcacgaggtaccctgcagccacctcgcgcgccgcctccgggagcgcgcctgcgcccccgctgccgcgcgcctcctcgtcctcgagccgctgcagaaggaagcgcagcgtctccacgcgctccgcggatgcctccccttggcacagcgccccaagcagggcccgggggtcccggctctgcgagagcagcgcttccgcgagcacccactccatttgccgagcgcccgcgccaccggcccgggctcccaaaggaaggcgccggcgtgtgcgatgcgtgcgcacag

SEQ ID NO: 12954 - RNA, 1838 nt, Homo sapiens
  source 1..1838: mol_type = other RNA
gctgggattacaggcatgagccacagtgcctggccacaattcactttaattctcttaataaaaagactattttaatctcattttatagatgaggaaagtgaggcactgcaaggttatataacttgcctaatgagaaacagctaataagtggcagagtctgaatttgaaaatggagtgatctttgtagcttaaaaaaatttttttttggattgctgggatgaacagaaatgctggacagctgttctctggcccctgaggccagagtggagtctagcaaacagctatacccacatggcagcctgaacagcggcagaggccagggtttggtagcctctccagggagaaggcaagagttaaagaataggagaagcccattcctgggagagaaggagccagcagtgcccccttaggaaactaatagtgagtaactgcagacacttctctgtaggcaggtacgggcttgagccgccataactagatgtttagggaagtgaggtcttcttttgtaagcacaggcaatgaagactggaatactaattgctcatctttgggtcccatagcaccaacatttgtgtgcagcaccaagtaagtggtcaatggattgcttgtagactgacctctctagtcccgtcctagatgaaccattgggccccaaccactgagcctctactcagcacatgacttggcagttagaaacaaggactaaagtcaactggacaggtcaaaggaattgctttaattgaggtcacaggcatcacaggggtctgctcagcttcctcgccaccagggagaaaagtccttcgttgttggccatggtggaagaataactttgcgagatcacctcaaaccattcgattgtgtagccagcctctttcacagcagcctctactgcctcccggcccagggggaggctggagaacttctgctcaccaatcatgtagtagctgctcttgagcgcatccatgatcaccaggaagccccctggcttcagtaggctgccgaggttcctgagcgccctgcagtaggtggggaggtctgggcaggcggcatccagacacagtgtgctgagcacgcagtcagccgggggtaaggggacggcccccagtggctggctctgagtcacatcacacttcagcacctgcttgaccgcctgtctcaacttctcctccttctctggacccttgactctgttcccttcaagatcacacacataggtcaccactggggaccagtcaaaggcctctggctctttcttcagccacttctccagctcctgcaggttctggtctgagtagtcagtgacgacgatctccttaaaggattcacaagcagagaggagctgatagatagtggggccagagccgatgtcaatcagcaggtctcccttcacaccgtctaggcagaatatcttgaaaagatttttcagaaggtgcttaagaatctggctttctgcagagtgcctagaaccaaacttgtaatatttttctaggtaatcccgagggttaaaatggcttagataggtgtccttggaggtgaagcctgattccattatgtctcacttctgtaccactggagcactgccctccttctctttcctccagaagccagggagtgaccctgcagaagttgtcttcctgagtctcaggctaacagcattccttccatcagttcagcccttcttgtccattggacgagccgtcctgatgcacttcctctttccctccagctcgtgtcactagaagctcactctatgctgaagaccacactcctctcccccagcgcccgcgccgccgcgaccccagcacagcgcctaagccccagctttgatgtccaagaac

SEQ ID NO: 12955 - RNA, 1707 nt, Homo sapiens
  source 1..1707: mol_type = other RNA
gctgggattacaggcatgagccacagtgcctggccacaattcactttaattctcttaataaaaagactattttaatctcattttatagatgaggaaagtgaggcactgcaaggttatataacttgcctaatgagaaacagctaataagtggcagagtctgaatttgaaaatggagtgatctttgtagcttaaaaaaatttttttttggattgctgggatgaacagaaatgctggacagctgttctctggcccctgaggccagagtggagtctagcaaacagctatacccacatggcagcctgaacagcggcagaggccagggtttggtagcctctccagggagaaggcaagagttaaagaataggagaagcccattcctgggagagaaggagccagcagtgcccccttaggaaactaatagtgagtaactgcagacacttctctgtaggcaggtacgggcttgagccgccataactagatgtttagggaagtgaggtcttcttttgtaagcacaggcaatgaagactggaatactaattgctcatctttgggtcccatagcaccaacatttgtgtgcagcaccaagtaagtggtcaatggattgcttgtagactgacctctctagtcccgtcctagatgaaccattgggccccaaccactgagcctctactcagcacatgacttggcagttagaaacaaggactaaagtcaactggacaggtcaaaggaattgctttaattgaggtcacaggcatcacaggggtctgctcagcttcctcgccaccagggagaaaagtccttcgttgttggccatggtggaagaataactttgcgagatcacctcaaaccattcgattgtgtagccagcctctttcacagcagcctctactgcctcccggcccagggggaggctggagaacttctgctcaccaatcatgtagtagctgctcttgagcgcatccatgatcaccaggaagccccctggcttcagtaggctgccgaggttcctgagcgccctgcagtaggtggggaggtctgggcaggcggcatccagacacagtgtgctgagcacgcagtcagccgggggtaaggggacggcccccagtggctggctctgagtcacatcacacttcagcacctgcttgaccgcctgtctcaacttctcctccttctctggacccttgactctgttcccttcaagatcacacacataggtcaccactggggaccagtcaaaggcctctggctctttcttcagccacttctccagctcctgcaggttctggtctgagtagtcagtgacgacgatctccttaaaggattcacaagcagagaggagctgatagatagtggggccagagccgatgtcaatcagcaggtctcccttcacaccgtctaggcagaatatcttgaaaagatttttcagaaggtgcttaagaatctggctttctgcagagtgcctagaaccaaacttgtaatatttttctaggtaatcccgagggttaaaatggcttagataggtgtccttggaggtgaagcctgattccattatgtctcacttctgtaccactggagcactgccctccttctctttcctccagaagccagggagtgaccctgcagaagttgtcttcctgagtctcaggctaacagcattccttccatcagttcagcccttcttttagaacagatggttggttaaacact

SEQ ID NO: 12956 - RNA, 1731 nt, Homo sapiens
  source 1..1731: mol_type = other RNA
gctgggattacaggcatgagccacagtgcctggccacaattcactttaattctcttaataaaaagactattttaatctcattttatagatgaggaaagtgaggcactgcaaggttatataacttgcctaatgagaaacagctaataagtggcagagtctgaatttgaaaatggagtgatctttgtagcttaaaaaaatttttttttggattgctgggatgaacagaaatgctggacagctgttctctggcccctgaggccagagtggagtctagcaaacagctatacccacatggcagcctgaacagcggcagaggccagggtttggtagcctctccagggagaaggcaagagttaaagaataggagaagcccattcctgggagagaaggagccagcagtgcccccttaggaaactaatagtgagtaactgcagacacttctctgtaggcaggtacgggcttgagccgccataactagatgtttagggaagtgaggtcttcttttgtaagcacaggcaatgaagactggaatactaattgctcatctttgggtcccatagcaccaacatttgtgtgcagcaccaagtaagtggtcaatggattgcttgtagactgacctctctagtcccgtcctagatgaaccattgggccccaaccactgagcctctactcagcacatgacttggcagttagaaacaaggactaaagtcaactggacaggtcaaaggaattgctttaattgaggtcacaggcatcacaggggtctgctcagcttcctcgccaccagggagaaaagtccttcgttgttggccatggtggaagaataactttgcgagatcacctcaaaccattcgattgtgtagccagcctctttcacagcagcctctactgcctcccggcccagggggaggctggagaacttctgctcaccaatcatgtagtagctgctcttgagcgcatccatgatcaccaggaagccccctggcttcagtaggctgccgaggttcctgagcgccctgcagtaggtggggaggtctgggcaggcggcatccagacacagtgtgctgagcacgcagtcagccgggggtaaggggacggcccccagtggctggctctgagtcacatcacacttcagcacctgcttgaccgcctgtctcaacttctcctccttctctggacccttgactctgttcccttcaagatcacacacataggtcaccactggggaccagtcaaaggcctctggctctttcttcagccacttctccagctcctgcaggttctggtctgagtagtcagtgacgacgatctccttaaaggattcacaagcagagaggagctgatagatagtggggccagagccgatgtcaatcagcaggtctcccttcacaccgtctaggcagaatatcttgaaaagatttttcagaaggtgcttaagaatctggctttctgcagagtgcctagaaccaaacttgtaatatttttctaggtaatcccgagggttaaaatggcttagataggtgtccttggaggtgaagcctgattccattatgtctcacttctgtaccactggagcactgccctccttctctttcctccagaagccagggagtgaccctgcagaagttgtcttcctgagtctcaggctaacagcattccttccatcagttcagcccttgggaaggaatgctgaataattgatttacagccttgttgccactggccagacca

SEQ ID NO: 12957 - RNA, 1730 nt, Homo sapiens
  source 1..1730: mol_type = other RNA
gctgggattacaggcatgagccacagtgcctggccacaattcactttaattctcttaataaaaagactattttaatctcattttatagatgaggaaagtgaggcactgcaaggttatataacttgcctaatgagaaacagctaataagtggcagagtctgaatttgaaaatggagtgatctttgtagcttaaaaaaatttttttttggattgctgggatgaacagaaatgctggacagctgttctctggcccctgaggccagagtggagtctagcaaacagctatacccacatggcagcctgaacagcggcagaggccagggtttggtagcctctccagggagaaggcaagagttaaagaataggagaagcccattcctgggagagaaggagccagcagtgcccccttaggaaactaatagtgagtaactgcagacacttctctgtaggcaggtacgggcttgagccgccataactagatgtttagggaagtgaggtcttcttttgtaagcacaggcaatgaagactggaatactaattgctcatctttgggtcccatagcaccaacatttgtgtgcagcaccaagtaagtggtcaatggattgcttgtagactgacctctctagtcccgtcctagatgaaccattgggccccaaccactgagcctctactcagcacatgacttggcagttagaaacaaggactaaagtcaactggacaggtcaaaggaattgctttaattgaggtcacaggcatcacaggggtctgctcagcttcctcgccaccagggagaaaagtccttcgttgttggccatggtggaagaataactttgcgagatcacctcaaaccattcgattgtgtagccagcctctttcacagcagcctctactgcctcccggcccagggggaggctggagaacttctgctcaccaatcatgtagtagctgctcttgagcgcatccatgatcaccaggaagccccctggcttcagtaggctgccgaggttcctgagcgccctgcagtaggtggggaggtctgggcaggcggcatccagacacagtgtgctgagcacgcagtcagccgggggtaaggggacggcccccagtggctggctctgagtcacatcacacttcagcacctgcttgaccgcctgtctcaacttctcctccttctctggacccttgactctgttcccttcaagatcacacacataggtcaccactggggaccagtcaaaggcctctggctctttcttcagccacttctccagctcctgcaggttctggtctgagtagtcagtgacgacgatctccttaaaggattcacaagcagagaggagctgatagatagtggggccagagccgatgtcaatcagcaggtctcccttcacaccgtctaggcagaatatcttgaaaagatttttcagaaggtgcttaagaatctggctttctgcagagtgcctagaaccaaacttgtaatatttttctaggtaatcccgagggttaaaatggcttagataggtgtccttggaggtgaagcctgattccattatgtctcacttctgtaccactggagcactgccctccttctctttcctccagaagccagggagtgaccctgcagaagttgtcttcctgagtctcaggctaacagcattccttccatcagttcagccctttttgagacagagtagggatggggcttggcttcagctcactccccgctaaagc

SEQ ID NO: 12958 - RNA, 1768 nt, Homo sapiens
  source 1..1768: mol_type = other RNA
gctgggattacaggcatgagccacagtgcctggccacaattcactttaattctcttaataaaaagactattttaatctcattttatagatgaggaaagtgaggcactgcaaggttatataacttgcctaatgagaaacagctaataagtggcagagtctgaatttgaaaatggagtgatctttgtagcttaaaaaaatttttttttggattgctgggatgaacagaaatgctggacagctgttctctggcccctgaggccagagtggagtctagcaaacagctatacccacatggcagcctgaacagcggcagaggccagggtttggtagcctctccagggagaaggcaagagttaaagaataggagaagcccattcctgggagagaaggagccagcagtgcccccttaggaaactaatagtgagtaactgcagacacttctctgtaggcaggtacgggcttgagccgccataactagatgtttagggaagtgaggtcttcttttgtaagcacaggcaatgaagactggaatactaattgctcatctttgggtcccatagcaccaacatttgtgtgcagcaccaagtaagtggtcaatggattgcttgtagactgacctctctagtcccgtcctagatgaaccattgggccccaaccactgagcctctactcagcacatgacttggcagttagaaacaaggactaaagtcaactggacaggtcaaaggaattgctttaattgaggtcacaggcatcacaggggtctgctcagcttcctcgccaccagggagaaaagtccttcgttgttggccatggtggaagaataactttgcgagatcacctcaaaccattcgattgtgtagccagcctctttcacagcagcctctactgcctcccggcccagggggaggctggagaacttctgctcaccaatcatgtagtagctgctcttgagcgcatccatgatcaccaggaagccccctggcttcagtaggctgccgaggttcctgagcgccctgcagtaggtggggaggtctgggcaggcggcatccagacacagtgtgctgagcacgcagtcagccgggggtaaggggacggcccccagtggctggctctgagtcacatcacacttcagcacctgcttgaccgcctgtctcaacttctcctccttctctggacccttgactctgttcccttcaagatcacacacataggtcaccactggggaccagtcaaaggcctctggctctttcttcagccacttctccagctcctgcaggttctggtctgagtagtcagtgacgacgatctccttaaaggattcacaagcagagaggagctgatagatagtggggccagagccgatgtcaatcagcaggtctcccttcacaccgtcttgtccattggacgagccgtcctgatgcacttcctctttccctccagctcgtgtcactagaagctcactctatgctgaagaccacagtttatagcatcgtggtgtttagaaagctgattcacgtcgttactctagttggcttcacaattgtcctgaggatgggtgggctaggtatttgctgaccccagtcttagggttgaggaagtgaggccttcgggagcctttgagatacagtgaaggtcacgcggtgcacagcagagctggcctcaaacccaggtcccctcgactgaatcccagattctgccaaatctcagctgcccctcttcctctagggtgcaccgcacggcagccaccaagctatttggcatcaga

SEQ ID NO: 12959 - RNA, 5223 nt, Homo sapiens
  source 1..5223: mol_type = other RNA
gctgggattacaggcatgagccacagtgcctggccctatgttctcttatattttttcaccaatgttgaatttaagtggattaggtaaaacagcccagcccagcccatcaaacagcatgtcttattgaatcaagttgatttacccagaaaagcctcacttctttaggtttgtgggaatactacagctgttgacaaacgtccctgatgggttctcttcccctgcctgggtaccagtacctcattaatcctgatgagaaaatggcttgtttttctcctcctgctataaccaccacgacttcttatttcctgcagcatcctatggctctactttgagacgggtacctgggtgtatcctgtgtttgccaaactcagcctcttgggtctagcagctttcttctctctcagctacgtcttcatcgccagcatctacctacttggagagaagctcaaccactggaaatggggtcagtgtatttctttcttagctacagatgcgcttcttccgtgtctgcctctccccttcacctggaaacagaaagaaaaactagccgcaaacagaagcaatgatgcttactgtctttgtccaaagtactcagacaggtcctgccaagaggtcctgccaaggcaagaggacagcgttgggggtggggcactcttttaaaggaccccatcaaaggatctcccctcctcccccaaacaatgtgtcatttaactttagagctaaaaataatcttctttagaaagcccaggacctagagaacaaggtattaccatccctagcatgaataaataaaatcaggggtctccccctaacccaagtgagggctccagggacacaagctttgaaaatatcaaggtttcattttgagggaagtgagtccagatagccctctcagctcctcccacctcctcccaactcagcagtacctcattaggctgctcctcagccttccataagacatttaccagatgaaatcacatcctagacttgagattgaaatcctcattcagacagagtcttcagcaatgagaatatgtcagtaagttaagctttctcgttataggtgggtacaatcctgttgcttcttcctaagaaaaaaaaatcatcttaacttagttaattttaaaatggaagatttcattctccttcctgcttcctctctccccaccccaccccagaatatttttttattgttggaaaagtaactaccagaaagtcaggctgtaaaacacccatgacttgcttccctaccccaggagaagcgcaggaactctaccctgattctgtatataaggatggcaaagagtcacacccagtcccccacatcactcgcccacatgccattctgttctatcaaaatagagatggcagaagtgccatcttccgcccaatctatgaactggtgtgaaaacataagcccgtgtatgcaaaaaaaacctgacagtttcagaaggttcagtaccagagtgtgcgtttctgagaggaagctgagaccctggagaaataagcacgcaacttggatgtatcacatgttttctactcttggagaatttgactggtttaagaaactctcaagggcaaaattctctttgaaagcaaacacttaaaaaaatggaatactaaaaattacttcccaatcaggattccaaatcacagaaaattatcgcaaaaaaaaaaatgtgttgacatttcagatgtgttgacatataattctaactagttttggctccttgaagttctgggtaaagatttctgatgcctccccaaatctctctctctctatatatatttaaagaagctttaagatataggaagtacagagaaaaacttgattacttagagcttagagaacaataacttttaaaatcaattgtattgagttcaataatgtattgagttaatttttaaattgttactctatggtgaattttaaacatccattgaattaaaaaacaaaattatcatcatatttattattattgaaattactattctcaatacaacgttcttaacaagcctcattgtttaagtactgcatccaatttttaactataattaggtctcaataaacagataagctggcatcatatggaccctcaactacctcatgtacatgcaagttttcaagtagaaagagacgattgtaaatgactgtacttacctctcgaggtctttctagatttttaactttttaaagaagagaaagggtaaaaggtcctatttaacatcagaataagatcagaaatgtattaaatcttgaacagatctttattaattataaataatttaatacgaattaaagaaaaattagatttgttaaagttgcaatgcagtgaacacttttacattgctgaaagctaaataacctatgtgaacacatttccccatgtcctattctactgaaaacactttctaaggcttcccccaattgactgaagaaagtccacacccttggaatgacacacaagggcctctgtgacccagtccctgctttggcttttgctcttctatatgtgtgccccagtggcaccaaactgctggttttccctccacgttgatgttgtttcttacgtccacgggattctgtgtctcctccagtctttgcctggttcatactcatgcatttcaacactcgcctcttccaggaagccttccctggtcagcccaggttggacttcatgcccttcccagtgcttccccctttacctcccagtcaccagacttaccattttatcatgactgcggttttactactgctttagggatttgtttttccactagacctcgggtgtcttacgaattaggggtatgtcttgttcatctcaagatccactatttccattagctttctcgttgcctcaatcagtgcagacaatagaatatccaagggccttttttcagcaaataggaggtcaggctattggaggctagaatctgttggaatctctgcttctgaaatcctgagacacaactggaatctctgcttccagtggcccaatttgaagtcaccagccaagcaccaagcggtcaagaacatcaggcgaagtatcagtcaagacccattcaatgtgacagtagctctctagcagtagttctccaccttggctttttacatcacagaaacactagggaagtttaaaaaataataattcccaggcctgccttagaccaattagatccatatctctagagatggtgactcgacatgggtattttttaaagcttcccagttattttaacttgcaatcgggatccggaaccgctgttacagagcaacgcttctcaaacctgtataggcctctgatgctcatcaaaatgaggatcttggggaacccggagatcttgttaaagtgtggattctgatttagtggatctggggtgcagtttgagattctgcccttctaacgcatactccagacatactgatgctgctggtctgaggacaaggctctattacatctcaggaccctggactcctcccaatgtggataattctgtctacggcatccttgtgcagtgtggtgctctcctgagtgggctgctggactgagaagggtgttggtggtgatggtcacaatagctgaacatctactcactttctccctcctcctgtgccacatcagtgggtgaatatggacaagagagcaagaaggacagcaataagaaaccatactgggaatcacatgttaaattggaaagtgtatgatgaggtcctcccagggcactcagttgcagggaactggctttgagcgtcaaggaggcaagtgttgtcatggcccacaggaaggtccttcaagaatgcactgaggctcaaaaagctcacaagaggttcctcagggccacctggcctgacctgtcaccatctcactccctgccctgggctagcctttctgtgtcatgaggcagagggttgggcaagcacagagtcagttactgggaccagtcatcccccaagaaagattcaatttctactttttgggaggagttagatggaatgttaacttcaaaccatgatagaagcagatgggggaagctgtctctggcaagacattgagagcttggctcaccatgaccatgactgaacacccaggcatgcccagggcaggttctcttccacattgactgggggcaagaggcaatcaggacatcctatcaaaggctcccttctctgccccttatgtgcttaattttcttttttttctttgatgattgatagcacacaaggatgctgacaccagcacacaagctcctcaggaagagaaaatcatcccacaagagatatggggcacagaaaggggctaaacacctccaggcccaaatggcagggcctctgctatgtgggggtggttggagagacagtcagcttatccagggcctgtgacccctctccctatgccccttgatggacacatgccaggagtcaggctgtcctttgtcagggcccctaagaccataggtccttctcatcctaaggacagactgtaagctgaaaattccagcctggccaagtggcgctgggagtgtgtcctggacagaatgacatggaaactttcttttaatattatttgccataaaccaggttttttaaaaggcagattttcttgatgaaagctgcctagaggccatctaatccacctccttgttttattcatgaaggaattagatgaggtttgtcttattaactctgcttattccatagcaaaagaattttatcatgcgatgactccacaggtacttctaaagcatggtcccactggggcagcatttagtcaatggcaaaaatttatctccattttgcctttcttgtcctaacttcatctccctaaactcaaaaagagcccgctgtggattaccctccctgcctcttcctcagcctctttcccacaggagtttctccagccagccctcagttccctgtcctccctggacttctgcagtgtgaacacaggactatcagtgctcagatctcatttctctaacacctgctatccccccaaccatcaattttcttgcccttttctgagtcagcccactgaaactaggcaaatgttcttcaaattttcaatgcctggcattcatttttgtggttgtagatacataggtgtaaatctttgagaatactatgtttttatttatcctgatttctaactattggaataataaggcatataattatatatggtatctatggtgatgttgattgaaacaataatttcttggcca

SEQ ID NO: 12960 - RNA, 4658 nt, Homo sapiens
  source 1..4658: mol_type = other RNA
gctgggattacaggcatgagccacagtgcctggcctaaaatactcttaaatgatgcaccctccatacatagaaaatcttcctagaagtaatatcatcctatataatgagatgagggttaagctggtgataaagttaggcataagtagggcatcaccctaaatcccgagttaagaggagtttgctgtagtttggggagcatattgaaaacacattgttggctgtgggcggcaagccatccaggtgctgaggcaagagaccgagggcacgagctgttccagtataataaaatatataaaacaacaagagttatactagatctagatcacagacatgattatatatgaatatcattaatcattagttatccggaggcctaaccgtctccctgtggtgctgtgcttcagtggtcacgctcctagtctgccttcatgttccatcctgtacacctggctctgccttttagataacagtagcaaaattagtgaaagtactaaaagtctctgatacgcagaaataatggcgtaagctgtctctctctctccctgtctatctctgccttggctgccaggcagggaagggccccctgtccagtggacacgtgacccacgtgaccttacctgtcattggagatgactcacactctttaccctgccccttttgctttgtatccaataaataacagtgcagccagacattcggggcctctaccggtctccgcctcttggtggtagtggtcccccaagcccagctgtcttttcttttacctctttgtcttgtgtctttatttctacaatctctcgtctccgcacatggggagaaaaacccaccgaccctgtggggctggtccctacagttggccgggcacggtggctcacacttgtaatcccagtactctgggaggcagaggtgggtggattacctgaggtcaggccttcaacaccagcctggccaacatggcaaaaccccgtctctactaaaaatacaaaaattagccaggcatggtggcgcacacctgtaatcccagctactcaggaggctgaggcaggagaattgctccaacccaggaggcagaggttgcagtgagccaagatcacgtcactgcactccagcctgggcgacagaccgagactcagtctcaaaaaaaaaagaagaaaaaaaaaaagaaaatacattgtcaagactcaaatcacagagtggtgtttcacatgatggtagagactgctgattgccctcttgaacccagcttccatttcttctttttcttatttatttatattttgagacggagtttctctcttgttgcccaggctggagtacaatggagcaatcttggctcactgcaacctctgcctcccaggttcaagcaattctcctgcctcagcctcctgagtagctgggattacaggcatgagccaccatgcccggctagtttttttttttttttttgtattttcagtagagatggggtttctccctgttggtcaggctggtctcgaactcccaacctcaggtgacccacccaccttggcctcccaaagtgctggaattataggcgtgagccactgtgcccggcctttgccaggtatcttgactagaggaagatagtgttctgggtgggagactcaagaggtctggttactgaagatacagatctcacttaaagtaagtaaattgacatctggtttccaaatcaatctattatgaaattggcccatgtcactttcatttggcctgatcaagtttttactgagaactgaattgggcacagtggctcacacctgtaatcccagcaccttaggaggctaaggcgggaggatcacttgagtccaggagtttgaaaacagcctgggcaacataacaaagtcccatctccacaaaaaatacaaacattagcccaggaagctgaagcaggaggatcatttgagcccaggaggtcgaggcagcagtgagctatgatcgtgccactgcactccagcctggatggcagagcaagaccctgtctcaaaaaaaaaaaaaaaaaaaatttgagaacattggacattcagtatctctcccctctcttgggcatcatgtttaggttctgtctctagagcacatctcagagcctgctacaggtaaacaggccagaagttaaatgcatgaaacaaattaaatgcatgaaacattcaagcacattcttattggtgtaattaaaataaaaaagtaaatgcatgaaacagaagctgtttacccacagcagaggaggggcagaaatcatatccagtgtgccatatcattactgcctgccagcatttccttaggctatttcatttatttactttttttgagatggagtctcgctctgactcccaggctggagtgcagtggcatgatctccactcactgcaacctccacctcccaggttcaaccaattttcctgcctcagcctcccaagtagctgggattacaggtgccagccaccatgactgcctaatttgtgtatttttagtgagagacagggtttcactacgttggccaggctggtctcaaactcctgacctcgagtgatccacccgcctcggcttcccaaagtgctgggattacaggcgtgagccaccatgcccaccttcctttggttattgagatggacaaagagttacccagtaagttaagagcagctagtttttaatgaatcttagcccagaatacaaagcagggtgtagcagttgccttaatggtgatataattgtaaacaatagctttttcttcccctataaactcgagttataggaagcgtttcagagagaggataacacatttgaatctattttttaaaaatcatcctgaaagctagcagtattgttgtcgtttaaaaggttcctcatatactcttaccctcagccaacccaccatgtttatcaattcaaattctagaactttcttgacccaagagattttgtaggaaaaatttctcttttcagatattcagcacgcaaggatcatttttcttggttttgttgctgatcttgctgaactttccatcaatggctgagggaggaagcttgcatgattcttatgagttcttctgaggcactttgactgtgacagttttcacttcagtgtatgcctgcagcccgtactcgcccaactcccggccactccccgacatcttgtagccaccaaagggtgactgggctccaaacacatcatagcagttgacccacacagtgcccgcctggagggcctgggacaggtaattggccttgtccaaatcctttgtgaagacagctgcggccagcccgtacgtggaattgttggctctcccaacaacctcctctatggtcttgaacttcaggatctgcatcactggcccgaagatctcctccttggcgatggtcatgccatcctgcacatctccaaacacagtgggctggatgaagtaaccacggtcagcagcaatgcccccaccacacagcagcttcgccccctcttgcttccccgtgttgatgtagccgaggatcttcttaaactgagtttcatccacctgcggcccctgctcggtcttgctatcaaaggggttcccgaccacccgagacttggcccgggcaacgctccgctccacaaactcatcatagatgtcctcctgcacgaaggtccgggagccggcacagcagcactggccctggttgaagaacagggcgaagtgggcctgttccacggcccaatccatatcggcatctgacatgatgatgttggggctcttcccccccagctccaaggtcactctcttgaggttgctgctcccagcagcaacctggattacgcggccaatctcagtggagcctgtgaatgccactttgtccacatcctcatgggaggcaatggcggccccagccgtggggccaaatccaggcacaatgttgaccacaccagggggaaagccagcctccttgatcaggttggccacatagagggcggtgaggggtgtctgctcagctaccttcatcacaaccacgtttccagttgccaaggctgggcccagcttccatgcttgcatcaggagcgggaaattccacggaatgatctgcccgcacacccccacaggttcatggcgtgtgtagctgaagaagtctccgtcaatggggatggttttcccgtggtacttatcagcccagccggcataataccggagacatttgaggaccatgtccaaatccaccaggtaggagatgacatagggcttgccattgtccagggtctccaaggccgccaggtaggtccggtcccgctcgatcagatcggccaggcggttcagcagccggcccctgtgtgatgcgtccatgcggcgccaaggtgagcccagctggaaggcggcccgggcggccttcactgccttgtccacatcttccttgtccccttcagctacctgacagatgacctctccagtggacggattgacggtggggaatgttttcctgctgacggcatcgtgccattcattgtttatgaaaatctggttgcagaagacctcgggctgctggttgggggcaggcacggcctgggtggcggcggctgacaagaggcggcggcccaggcggggcccgaagcgggcggcagcgcgcaacatcgcagcgggctagcggacagcgagcggaccgagagcagagctagggtctc

SEQ ID NO: 12961 - RNA, 4517 nt, Homo sapiens
  source 1..4517: mol_type = other RNA
gctgggattacaggcatgagccacagtgcctggcctaaaatactcttaaatgatgcaccctccatacatagaaaatcttcctagaagtaatatcatcctatataatgagatgagggttaagctggtgataaagttaggcataagtagggcatcaccctaaatcccgagttaagaggagtttgctgtagtttggggagcatattgaaaacacattgttggctgtgggcggcaagccatccaggtgctgaggcaagagaccgagggcacgagctgttccagtataataaaatatataaaacaacaagagttatactagatctagatcacagacatgattatatatgaatatcattaatcattagttatccggaggcctaaccgtctccctgtggtgctgtgcttcagtggtcacgctcctagtctgccttcatgttccatcctgtacacctggctctgccttttagataacagtagcaaaattagtgaaagtactaaaagtctctgatacgcagaaataatggcgtaagctgtctctctctctccctgtctatctctgccttggctgccaggcagggaagggccccctgtccagtggacacgtgacccacgtgaccttacctgtcattggagatgactcacactctttaccctgccccttttgctttgtatccaataaataacagtgcagccagacattcggggcctctaccggtctccgcctcttggtggtagtggtcccccaagcccagctgtcttttcttttacctctttgtcttgtgtctttatttctacaatctctcgtctccgcacatggggagaaaaacccaccgaccctgtggggctggtccctacagttggccgggcacggtggctcacacttgtaatcccagtactctgggaggcagaggtgggtggattacctgaggtcaggccttcaacaccagcctggccaacatggcaaaaccccgtctctactaaaaatacaaaaattagccaggcatggtggcgcacacctgtaatcccagctactcaggaggctgaggcaggagaattgctccaacccaggaggcagaggttgcagtgagccaagatcacgtcactgcactccagcctgggcgacagaccgagactcagtctcaaaaaaaaaagaagaaaaaaaaaaagaaaatacattgtcaagactcaaatcacagagtggtgtttcacatgatggtagagactgctgattgccctcttgaacccagcttccatttcttctttttcttatttatttatattttgagacggagtttctctcttgttgcccaggctggagtacaatggagcaatcttggctcactgcaacctctgcctcccaggttcaagcaattctcctgcctcagcctcctgagtagctgggattacaggcatgagccaccatgcccggctagtttttttttttttttttgtattttcagtagagatggggtttctccctgttggtcaggctggtctcgaactcccaacctcaggtgacccacccaccttggcctcccaaagtgctggaattataggcgtgagccactgtgcccggcctttgccaggtatcttgactagaggaagatagtgttctgggtgggagactcaagaggtctggttactgaagatacagatctcacttaaagtaagtaaattgacatctggtttccaaatcaatctattatgaaattggcccatgtcactttcatttggcctgatcaagtttttactgagaactgaattgggcacagtggctcacacctgtaatcccagcaccttaggaggctaaggcgggaggatcacttgagtccaggagtttgaaaacagcctgggcaacataacaaagtcccatctccacaaaaaatacaaacattagcccaggaagctgaagcaggaggatcatttgagcccaggaggtcgaggcagcagtgagctatgatcgtgccactgcactccagcctggatggcagagcaagaccctgtctcaaaaaaaaaaaaaaaaaaaatttgagaacattggacattcagtatctctcccctctcttgggcatcatgtttaggttctgtctctagagcacatctcagagcctgctacaggtaaacaggccagaagttaaatgcatgaaacaaattaaatgcatgaaacattcaagcacattcttattggtgtaattaaaataaaaaagtaaatgcatgaaacagaagctgtttacccacagcagaggaggggcagaaatcatatccagtgtgccatatcattactgcctgccagcatttccttaggctatttcatttatttactttttttgagatggagtctcgctctgactcccaggctggagtgcagtggcatgatctccactcactgcaacctccacctcccaggttcaaccaattttcctgcctcagcctcccaagtagctgggattacaggtgccagccaccatgactgcctaatttgtgtatttttagtgagagacagggtttcactacgttggccaggctggtctcaaactcctgacctcgagtgatccacccgcctcggcttcccaaagtgctgggattacaggcgtgagccaccatgcccaccttcctttggttattgagatggacaaagagttacccagtaagttaagagcagctagtttttaatgaatcttagcccagaatacaaagcagggtgtagcagttgccttaatggtgatataattgtaaacaatagctttttcttcccctataaactcgagttataggaagcgtttcagagagaggataacacatttgaatctattttttaaaaatcatcctgaaagctagcagtattgttgtcgtttaaaaggttcctcatatactcttaccctcagccaacccaccatgtttatcaattcaaattctagaactttcttgacccaagagattttgtaggaaaaatttctcttttcagatattcagcacgcaaggatcatttttcttggttttgttgctgatcttgctgaactttccatcaatggctgagggaggaagcttgcatgattcttatgagttcttctgaggcactttgactgtgacagttttcacttcagtgtatgcctgcagcccgtactcgcccaactcccggccactccccgacatcttgtagccaccaaagggtgactgggctccaaacacatcatagcagttgacccacacagtgcccgcctggagggcctgggacaggtaattggccttgtccaaatcctttgtgaagacagctgcggccagcccgtacgtggaattgttggctctcccaacaacctcctctatggtcttgaacttcaggatctgcatcactggcccgaagatctcctccttggcgatggtcatgccatcctgcacatctccaaacacagtgggctggatgaagtaaccacggtcagcagcaatgcccccaccacacagcagcttcgccccctcttgcttccccgtgttgatgtagccgaggatcttcttaaactgagtttcatccacctgcggcccctgctcggtcttgctatcaaaggggttcccgaccacccgagacttggcccgggcaacgctccgctccacaaactcatcatagatgtcctcctgcacgaaggtccgggagccggcacagcagcactggccctggttgaagaacagggcgaagtgggcctgttccacggcccaatccatatcggcatctgacatgatgatgttggggctcttcccccccagctccaaggtcactctcttgaggttgctgctcccagcagcaacctggattacgcggccaatctcagtggagcctgtgaatgccactttgtccacatcctcatgggaggcaatggcggccccagccgtggggccaaatccaggcacaatgttgaccacaccagggggaaagccagcctccttgatcaggttggccacatagagggcggtgaggggtgtctgctcagctaccttcatcacaaccacgtttccagttgccaaggctgggcccagcttccatgcttgcatcaggagcgggaaattccacggaatgatctgcccgcacacccccacaggttcatggcgtgtgtagctgaagaagtctccgtcaatggggatggttttcccgtggtacttatcagcccagccggcataataccggagacatttgaggaccatgtccaaatccaccaggtaggagatgacatagggcttgccattgtccagggtctccaaggccttgtccccttcagctacctgacagatgacctctccagtggacggattgacggtggggaatgttttcctgctgacggcatcgtgccattcattgtttatgaaaatctggttgcagaagacctcgggctgctggttgggggcaggcacggcctgggtggcggcggctgacaagaggcggcggcccaggcggggcccgaagcgggcggcagcgcgcaacatcgcagcgggctagcggacagcgagcggaccgagagcagagctagggtctc

SEQ ID NO: 12962 - RNA, 6864 nt, Homo sapiens
  source 1..6864: mol_type = other RNA
gctgggattacaggcatgagccaccaaacctggcccaatatgtaaatatcaatgtaaccaccagcctagatcaagatgtagaatgttttaaattgattataagttgcagaagcaatgcatgaacacactctccttgtaaagcattaaaacatgagctgtgagccgacccctcccagtgtcccgcctacacacacaaggccccactgttatatgtaattgattgtgtgtccggaagcaggggcttccccctaggcattcccaggcctctaggcagctgagcagcctgacccaacaggtttagggtctttctccttgaacattctcttctgcccattcccttcccccacccaaatcctccaacagagaaagagcctgtggatttggataacacaactgcctcgctgagcttcctccctccccatccttacaactgaaagcggtctgactcggacgcttctaagctgtggctgcagagaacacaaagagcagccttcggcgcgcggacgcaccatcgatgtactgggttggggcgggggggacgccaaccggccccaaagcacatcgaagccagaaactgcccgaactagttacattccagcaagattagcacaaggccgggcctgctcctgcgcccacccctcctcccctcctgagccatgaataggatttttaactatttccctcccacttgctgtccagcctcacacatggacaatgctccccgctgtttgcacattaacctcccatttgccaggcagcttctcaggggctgcagattaacatccaccaactcagacaatcatccccggggaggggtgcaaggggctcagacaaaagctacagacactgagcccagtcaatcaccgcacagtgaccactggccaacagtgcaagggactcctggactccagacacacaggaatcaccacaggcggctcattcctggctctgggcacctgccccacgtgggaccagagaggatactcccctaatgcaggcctacagcaaccagaagacatcctccccaccccatctaatctgggacattctggcctaggaggggcccgaaaggatcagggactgaagggctgggaaggcagagggcagccttaggcaggcctcgcagacccagcccaccctgtttaggcttctcctttctcccggcaaagcggagctctcaggggacagaacaggaagcaggtgcctcaggcccctgccctggggctccctgggaaagctgcctggtctctcagcaagaagggcccctgactgaagcagcttgtagacatgattccatacatcaaagccattttcctattcccttgtgtgcaggtgtgcacacaggcatgaacttggaaacacaacagcatgtaggggggagggaatggggagacagctggactgtgaggtatgggaatggtccttctatgtcctaggccagcagctcagcccctgcatttgtattaaaaatctcctccaggtgatgctcatgcaccctggtcctgaaccagaggccctggaagtgaacaatcgcatgcattagctgaggatcctgttaagatgcagtctgggtcaagaggtgtgtcgtggggcccaggatggtaagtttctaaccagctcaagacacactcttgaggccatctcagtgaggcctcagactgggcgcatcatcagaagggcgatctctctgtatgctgcttcaccaagtagttgtctggctacagtttccacccttctcgagaaaggtcaccacctctcaagacagccagttgcagctgcggacagctctgtttgagtccttcctcatattaagacatccaacagtgacaatctgaagtctttcttctcttgacctggtagttccagaccctcagaagaccttgtggcttccactcgtgttttccccacatacctgtgcctcctcatctaggccagtgaggctgtttttctgagcttcattctcttcttagtactaatgccagacagggtgggggcaggggagcagatctcagtgcagattggcgaggctatttgggtaggagtgagaatagagcccccaacggaaacagaaaccagagttctagcctggagcagttaacatacaagaaacttaaggacaattaaaaagcaacaaccacaattaacgtggtttacacaggcaaaactcattaatgtggatcggggtgctggagtttacctttgctaggcaaaccctttttacagacagtacagattaattgcaagcaagactccaaggggaatatctaaatggctatgaaacaaccttcaagcccccccaatgcaggaaaaagcaccactgacctacaagggacacacagaggacttcgtccagggagcccccttgccagtctggcttcaattcctggtgaagttcagaagcaataaacctgtgctccttttgaaaggttttataattcagaagaccccctaattcacactaacatccaccccaagtctgaattaattgtgttacccagcagttctgctaaggaatcacttcatcatcactgctgcagggaaaatttgagcggggccgatggtttgcagtggcagcaagtctacaaatgattatccctaatgagatgatgcgagagcagcctcaaataaggcactcctccagctgccccgtgcccagctgggcttcctgccctcccacccgctccaggccatgagcccttcatggggctctcatggcaagaggggcctggatcttccaaaggtgaaaccatcccaaagacccaagggctcccactcagtctcctgctgccactccctgccccactgcaaggtcacacatgacagtggggtctggctgagctaggactgaatcctgactgtaccccttaccagttgttaccttgatctaaagttaatctttctgagcctcagctcccacatgttgaaaaggtattagtataatccagttcctaagattgtgtggtggtttaactgagtgaacgcttagcatgcacagggcctggagtaggtaaactcttacgatggtagtaaaaaggaggaagatttcttttaaggacagggagatggcccctctttctttgaggctccaaagctcactgttcttctgttgtgacactaacctttccctgccttgagatcagttccactacttgtgttgttgctctggtggaccaggaaacagacagttcctatataaggtcatggccccactcatcttttacttacctactgcaacgttcaacccaatccttgcaattagtaggaacctgatcaatatttctgcattgacttgccagcatgaaccagcctactcaggacaaagcatggaggtcgtaaccaaatgggtcaaacagccaacagaccagacctccccgcccccgcccctgtgagcaggtttctgaccttacgaacaacagcagttgcgtttaggtaaaacgacaatcacacttctgactggctgtcaaactattcatgaaaatggccaccaacttcctattttttaaatcaaacactaagccatatgtctgctacacaatgaaaaatcccaaacctatgtggtttaataggctttccaacatttcttcagaagcctagatctctaacgtttacatttaaggtgacactggctcacggtctgttgttccatagtcttattgcactgtttacacatcctacctcatttttacagaaatgggtcattaggccagggaccaccttcttccatgtcatgacatgctttggttgggagtggcgaaggtctaattttaggccgtctgagaaagggcctaaaatttcctgaatagatgctctggtctggtctctctccttcagctcttatatccagctggtcccttctgtcctgaagaggtaaacagcctcaagcggggcccagagacttgggttctaactcgaccccaattagcagtgtgatgactttaggcaggtcctttccccttgctgatcacagctgctagaaaaagcctctctggctgctccttctcagtctcctttgccagttcttgctcttctctccagtgtgcaaaagctgtagtgcccacggctcagcccttgacctctttttttctcagcttcagtctcagggatctcctccagtctcatggcttgaagtaccatcaacatgctgatgactaaagtctctgtctctaacctagacctcatccctgacttctagacccaattaccccacctatcactctccccactggatgtccaaaaagtatctccaatacaacatgtcccaaacagagctcctaattatttcctcccaaacctgcccctcccacagtcttctccatttctgtcaatgacactttcttctttcccactgcccaggagacattcctaactcttcttcctcttgctccccacatttgttccatcagcaaatcctgtcactcctccttcaaaatgggtccagaatctgagaactttccccatttctactgccaccatccaggccccactggcccaacaacttgtctctgattttctacccttgaccccttcggtctatgattatatcatggcagccatggcgctacgttaaaacaaaggttggatcacgtcacctttctgctcaagacccctctctactccccatctcagtcaaaaggcttcatcatgggctgcatgcccctgtgaccagccccctgtcccctttctgactgtgcctccttcagtgctgccccccagccttgcccactctgctccagccactctgttctgcccgctcctggaacctaccaagcgccatcccctttgcacctgctgttccctctgcctggcgtgctcttcccccgtgtatgtgtctatagagtttgtcacctccctgtgaggccttcaataaatattgaataaatgaatgaacaagcaaactgaaggctttaccctgaaccctccctggcaggccgggatcccacagtttgcctgttcgttctttccctgtggctggatcctgaactccgcccaccacatctcccacccccagggggtgctgttcacaatgtggtccgtggctagcagggcagctcccaacgtcaactctgcagggagccgtgtgaagtcacaatatgaatacccggccctttctaaggtgcctggcacgtagtggatggctcagcgtatatctcctgaacgaagtttcacctctcaccctgagccagaatcctgcccactcagaacccaagacccatgcctggggctgcctctggccaggaagctctctctcctcagcccatccccagccttctcctcctggcccagctcccccttcccttgctgagtttctagcacctcttatgctgttcacacccagacaattccgaaaacactggatcccctgtgaatggtgtggaaatgcaacttccccacgtggagtcgctgggcatgttccccttcccttcccctcgaaccctgcacagagggggccattatgtcacacaaggccacttcacgagtaagggacaaaacagcccttttgaaactcaaaacaaagcttaagagccgcacctgagttactaaagcttccactcagcctcacccattcctagcaataagctgcagcagccggatctgctcccacctctgggtgacggctgggaacaccaggctgttacctttcatcaaaaacacaaagggacagcaagggacctcaggcatgtaatggcgccgaggagtagccataacatgttattacagaattagttctttcgaaactgcgtgccaactgattattaataaactgcaaaaatgagttaagggcggaataattggggctgaatgcctaccaatcctgcacatgttaaccaagacatatgaggttcaactagaagccaattgaacagttacttattgttaactactatgtgccaagatgtcggtgcgtcgagatctttaagacttgctggaggccccactgccagaggtgtgtaatctaaatggggaaaggaaaggaaaacatgccctttcattcaatagtttttaaaacagtacagtgtactaggaaaggctgaggtaaaacatctgcttcaatagggaggcagagaaaaggggatatagaggccctggggagatttcttgaaggagacagaaaactggagatctgcaaagagaagaaacaggaggaagcaacacatcccgtgtggaaggggagaaagtgggtgctgtgagcaggagtgacaaagtcttcaggaagactgagcctggggacaaggctggcctcaacatttgccttctatacagggtgtgcacaaacctcaatgccaagccccattcaaggaaaaggaggaaggctgcagatggacctcactgactctccctacagcagaagcgggcacagccgggtgcagcgtctaggtcaggagaggtggtgtttgcattcatgctgtcataacggctgtggtcaggcttggatgaggacgtcaagctgacaaaacctcaaggtgatggaggaccattccttccattatttgagccatcccagaaagaagggaggtaattcttaagcgcgacatgttcacaaatggaaaagtgtggatttggcctggatgttggcattttacttgggccggggctttatgtgacgtgggttctatgttggcagcccagaggcagccaagtgacccagggaagccagcaaccatagggtttccagcctcatggtatcaatggaagaattatgagatcacaaatgtcagagcccctggggccttgtaggtaaatgcttggtttgattttaagtgatccagataatagaagaagttctcactggcttctttaagatggtcccttagacttacagatgtttttaggttctcatgattcaaaaatctattcttgcccccc

SEQ ID NO: 12963 - RNA, 2189 nt, Homo sapiens
  source 1..2189: mol_type = other RNA
gctgggattacaggcatgagccaccaaatctggcccaaattgagtttaataaagagcttgagtgatgctcagattagggagggagtgaccgggaatgctggggtctggaactgggggcccagctgagctctgaatcagagagcagtgagacctaagggtccctgatctcagagggtccctcctgtctcagggtgaggacctgaagggtgtgggtcccggggagggtgaggaggccattgtaggagatttactgagatggtatcgggatgccccaagcaccacgtagggggattacatctgggtttctgggaacgaagagctgagttaggggagagaacccgaaagatctcagtggggaaaggactaggggtgcagggtgtttcacagaaacaatcaaggggcctcgatttcacagaaatcatcaagagggctccttgtgggtagaagaggggtatcacagcaccccaaatattggggcctgttcacccctctgcagccattctggggttttaatgtaaaaccccaatggcaggatattccacatacattatcatgggtttgcaacattagcatacgctggctgtcccgcaggacggtggggactggaaaatcagtccagggtctgggtttgagtcctaagaggacaggcctggcggcgccacacggctcctcttcaacagctgccggagcccctcagggcccggcccgggccgcagcaggtgaacgggctgctcattctccaggttgcgcagtgtggggtccgccccagctgccaacaggtgccgcacgatggcctcctgggccggcccagggggcagggcagccgccatgtggagggctgtgttcccgtgggccttcatgttgacaaaggtccgcaggtctccccggggcagctccagcagcagctgaaccagagtggggttggcagcctgcacggccaagtgcagaactgtcttgttgctcttgatctcctggctggtgtgattagcacccatttgcagcaacatgtggacacaatccagcctgtctcgggcctgtgtgctcagcacccggggacagaggtcggaagggcgcatagcaacgttaagggccaggatggccgtgtggagcggggtgaggccctcgaagtctctggcttccaggtcaacctggaccccagagttaagcacagccaagagaactcctgggagcccgtaggtagcggccacgtgcaagaccgaacgtccctgatggtcagcggcattgggctctgctcccaggttcaacagatcctccacaatcaggggctggttggcagcagccgccaccaggagaggggtcttgcccttatgctcacgaatgtcaagacgccggtacacctggagcacctcagccgcagcatatgccgcccagcgcagcccccgagccgcaaacaggtgaaggagcctccatgccctggggaaatgggcacggctgccctgggtccgagggtgggtagaagtcaggaggcaggaaattttcggcagcagaagcagggcaagagtaggggctgtcagtgtaggcagcatgcgtgttggggtcccagtctggaaagcccaggctgctaggtccagaacccacagtctccgagtgtgcagtcacagcctcattcacagatggggtcaggggctgctctgggggagggagaaattgtccctgcaccccgccagcgtcgggctgctgctgctggcggcgcctctgctcttccagaagcttcttcacggtttgcgttgggcagtggctgcgctcacccctgctcactgtgcgggagaggagagggggaagtcatcaagggtccttaagtcacctaaatgccgcgggggtggcgcgcggggagtgggtttgggcaccctcctcgccctcccgcgcggaaaaactggcacatagatgccgcctgactcctccaaagccattagaagatttggggtggggcatccgcctccgccgtttccttccttttgctccgcactttccctctgacccaactttccaccaccgtcgcggaaagtgaggaagggggaggagggcacccctctgcagcaaccaccccacttccgtaaaaaaattccacccccagatatccaagttttgaagtcagcgggttggtggggggccggcgccaggcgtcactccctagactcacatccaggttcccaacatttttttcccta

SEQ ID NO: 12964 - RNA, 1895 nt, Homo sapiens
  source 1..1895: mol_type = other RNA
gctgggattacaggcatgagccaccaaatctggcccaaattgagtttaataaagagcttgagtgatgctcagattagggagggagtgaccgggaatgctggggtctggaactgggggcccagctgagctctgaatcagagagcagtgagacctaagggtccctgatctcagagggtccctcctgtctcagggtgaggacctgaagggtgtgggtcccggggagggtgaggaggccattgtaggagatttactgagatggtatcgggatgccccaagcaccacgtagggggattacatctgggtttctgggaacgaagagctgagttaggggagagaacccgaaagatctcagtggggaaaggactaggggtgcagggtgtttcacagaaacaatcaaggggcctcgatttcacagaaatcatcaagagggctccttgtgggtagaagaggggtatcacagcaccccaaatattggggcctgttcacccctctgcagccattctggggttttaatgtaaaaccccaatggcaggatattccacatacattatcatgggtttgcaacattagcatacgctggctgtcccgcaggacggtggggactggaaaatcagtccagggtctgggtttgagtcctaagaggacaggcctggcggcgccacacggctcctcttcaacagctgccggagcccctcagggcccggcccgggccgcagcaggtgaacgggctgctcattctccaggttgcgcagtgtggggtccgccccagctgccaacaggtgccgcacgatggcctcctgggccggcccagggggcagggcagccgccatgtggagggctgtgttcccgtgggccttcatgttgacaaaggtccgcaggtctccccggggcagctccagcagcagctgaaccagagtggggttggcagcctgcacggccaagtgcagaactgtcttgttgctcttgatctcctggctggtgtgattagcacccatttgcagcaacatgtggacacaatccagcctgtctcgggcctgtgtgctcagcacccggggacagaggtcggaagggcgcatagcaacgttaagggccaggatggccgtgtggagcggggtgaggccctcgaagtctctggcttccaggtcaacctggaccccagagttaagcacagccaagagaactcctgggagcccgtaggtagcggccacgtgcaagaccgaacgtccctgatggtcagcggcattgggctctgctcccaggttcaacagatcctccacaatcaggggctggttggcagcagccgccaccaggagaggggtcttgcccttatgctcacgaatgtcaagacgccggtacacctggagcacctcagccgcagcatatgccgcccagcgcagcccccgagccgcaaacaggtgaaggagcctccatgccctggggaaatgggcacggctgccctgggtccgagggtgggtagaagtcaggaggcaggaaattttcggcagcagaagcagggcaagagtaggggctgtcagtgtaggcagcatgcgtgttggggtcccagtctggaaagcccaggctgctaggtccagaacccacagtctccgagtgtgctgggaagggagggtggccagtcacagcctcattcacagatggggtcaggggctgctctgggggagggagaaattgtccctgcaccccgccagcgtcgggctgctgctgctggcggcgcctctgctcttccagaagcttcttcacggtttgcgttgggcagtggctgcgctcacccctgctcactcggggattccgtggcgtggattgcgggcccccagggccgcggcctcggcgctgcgccagcctcgctgtttcccccgcggagccgccgccgggtcccc

SEQ ID NO: 12965 - RNA, 2206 nt, Homo sapiens
  source 1..2206: mol_type = other RNA
gctgggattacaggcatgagccaccaaatctggcccaaattgagtttaataaagagcttgagtgatgctcagattagggagggagtgaccgggaatgctggggtctggaactgggggcccagctgagctctgaatcagagagcagtgagacctaagggtccctgatctcagagggtccctcctgtctcagggtgaggacctgaagggtgtgggtcccggggagggtgaggaggccattgtaggagatttactgagatggtatcgggatgccccaagcaccacgtagggggattacatctgggtttctgggaacgaagagctgagttaggggagagaacccgaaagatctcagtggggaaaggactaggggtgcagggtgtttcacagaaacaatcaaggggcctcgatttcacagaaatcatcaagagggctccttgtgggtagaagaggggtatcacagcaccccaaatattggggcctgttcacccctctgcagccattctggggttttaatgtaaaaccccaatggcaggatattccacatacattatcatgggtttgcaacattagcatacgctggctgtcccgcaggacggtggggactggaaaatcagtccagggtctgggtttgagtcctaagaggacaggcctggcggcgccacacggctcctcttcaacagctgccggagcccctcagggcccggcccgggccgcagcaggtgaacgggctgctcattctccaggttgcgcagtgtggggtccgccccagctgccaacaggtgccgcacgatggcctcctgggccggcccagggggcagggcagccgccatgtggagggctgtgttcccgtgggccttcatgttgacaaaggtccgcaggtctccccggggcagctccagcagcagctgaaccagagtggggttggcagcctgcacggccaagtgcagaactgtcttgttgctcttgatctcctggctggtgtgattagcacccatttgcagcaacatgtggacacaatccagcctgtctcgggcctgtgtgctcagcacccggggacagaggtcggaagggcgcatagcaacgttaagggccaggatggccgtgtggagcggggtgaggccctcgaagtctctggcttccaggtcaacctggaccccagagttaagcacagccaagagaactcctgggagcccgtaggtagcggccacgtgcaagaccgaacgtccctgatggtcagcggcattgggctctgctcccaggttcaacagatcctccacaatcaggggctggttggcagcagccgccaccaggagaggggtcttgcccttatgctcacgaatgtcaagacgccggtacacctggagcacctcagccgcagcatatgccgcccagcgcagcccccgagccgcaaacaggtgaaggagcctccatgccctggggaaatgggcacggctgccctgggtccgagggtgggtagaagtcaggaggcaggaaattttcggcagcagaagcagggcaagagtaggggctgtcagtgtaggcagcatgcgtgttggggtcccagtctggaaagcccaggctgctaggtccagaacccacagtctccgagtgtgctgggaagggagggtggccagtcacagcctcattcacagatggggtcaggggctgctctgggggagggagaaattgtccctgcaccccgccagcgtcgggctgctgctgctggcggcgcctctgctcttccagaagcttcttcacggtttgcgttgggcagtggctgcgctcacccctgctcactgtgcgggagaggagagggggaagtcatcaagggtccttaagtcacctaaatgccgcgggggtggcgcgcggggagtgggtttgggcaccctcctcgccctcccgcgcggaaaaactggcacatagatgccgcctgactcctccaaagccattagaagatttggggtggggcatccgcctccgccgtttccttccttttgctccgcactttccctctgacccaactttccaccaccgtcgcggaaagtgaggaagggggaggagggcacccctctgcagcaaccaccccacttccgtaaaaaaattccacccccagatatccaagttttgaagtcagcgggttggtggggggccggcgccaggcgtcactccctagactcacatccaggttcccaacatttttttccct

SEQ ID NO: 12966 - RNA, 2146 nt, Homo sapiens
  source 1..2146: mol_type = other RNA
gctgggattacaggcatgagccaccaaatctggcccaaattgagtttaataaagagcttgagtgatgctcagattagggagggagtgaccgggaatgctggggtctggaactgggggcccagctgagctctgaatcagagagcagtgagacctaagggtccctgatctcagagggtccctcctgtctcagggtgaggacctgaagggtgtgggtcccggggagggtgaggaggccattgtaggagatttactgagatggtatcgggatgccccaagcaccacgtagggggattacatctgggtttctgggaacgaagagctgagttaggggagagaacccgaaagatctcagtggggaaaggactaggggtgcagggtgtttcacagaaacaatcaaggggcctcgatttcacagaaatcatcaagagggctccttgtgggtagaagaggggtatcacagcaccccaaatattggggcctgttcacccctctgcagccattctggggttttaatgtaaaaccccaatggcaggatattccacatacattatcatgggtttgcaacattagcatacgctggctgtcccgcaggacggtggggactggaaaatcagtccagggtctgggtttgagtcctaagaggacaggcctggcggcgccacacggctcctcttcaacagctgccggagcccctcagggcccggcccgggccgcagcaggtgaacgggctgctcattctccaggttgcgcagtgtggggtccgccccagctgccaacaggtgccgcacgatggcctcctgggccggcccagggggcagggcagccgccatgtggagggctgtgttcccgtgggccttcatgttgacaaaggtccgcaggtctccccggggcagctccagcagcagctgaaccagagtggggttggcagcctgcacggccaagtgcagaactgtcttgttgctcttgatctcctggctggtgtgattagcacccatttgcagcaacatgtggacacaatccagcctgtctcgggcctgtgtgctcagcacccggggacagaggtcggaagggcgcatagcaacgttaagggccaggatggccgtgtggagcggggtgaggccctcgaagtctctggcttccaggtcaacctggaccccagagttaagcacagccaagagaactcctgggagcccgtaggtagcggccacgtgcaagaccgaacgtccctgatggtcagcggcattgggctctgctcccaggttcaacagatcctccacaatcaggggctggttggcagcagccgccaccaggagaggggtcttgcccttatgctcacgaatgtcaagacgccggtacacctggagcacctcagccgcagcatatgccgcccagcgcagcccccgagccgcaaacaggtgaaggagcgtgtccccctcctcatcctgggccagcagctgctgtggccccaaagccagcatgtgagctcgggccacctccagcgatggtccagggaccacagcggggaactgtgggggtcctgaagggggtgcagaaactctccagggtccagccagtcacagcctcattcacagatggggtcaggggctgctctgggggagggagaaattgtccctgcaccccgccagcgtcgggctgctgctgctggcggcgcctctgctcttccagaagcttcttcacggtttgcgttgggcagtggctgcgctcacccctgctcactgtgcgggagaggagagggggaagtcatcaagggtccttaagtcacctaaatgccgcgggggtggcgcgcggggagtgggtttgggcaccctcctcgccctcccgcgcggaaaaactggcacatagatgccgcctgactcctccaaagccattagaagatttggggtggggcatccgcctccgccgtttccttccttttgctccgcactttccctctgacccaactttccaccaccgtcgcggaaagtgaggaagggggaggagggcacccctctgcagcaaccaccccacttccgtaaaaaaattccacccccagatatccaagttttgaagtcagcgggttggtggggggccggcgccaggcgtcactccctagactcacatccaggttcccaacatttttttccct

SEQ ID NO: 12967 - RNA, 2314 nt, Homo sapiens
  source 1..2314: mol_type = other RNA
gctgggattacaggcatgagccaccaaatctggcccaaattgagtttaataaagagcttgagtgatgctcagattagggagggagtgaccgggaatgctggggtctggaactgggggcccagctgagctctgaatcagagagcagtgagacctaagggtccctgatctcagagggtccctcctgtctcagggtgaggacctgaagggtgtgggtcccggggagggtgaggaggccattgtaggagatttactgagatggtatcgggatgccccaagcaccacgtagggggattacatctgggtttctgggaacgaagagctgagttaggggagagaacccgaaagatctcagtggggaaaggactaggggtgcagggtgtttcacagaaacaatcaaggggcctcgatttcacagaaatcatcaagagggctccttgtgggtagaagaggggtatcacagcaccccaaatattggggcctgttcacccctctgcagccattctggggttttaatgtaaaaccccaatggcaggatattccacatacattatcatgggtttgcaacattagcatacgctggctgtcccgcaggacggtggggactggaaaatcagtccagggtctgggtttgagtcctaagaggacaggcctggcggcgccacacggctcctcttcaacagctgccggagcccctcagggcccggcccgggccgcagcaggtgaacgggctgctcattctccaggttgcgcagtgtggggtccgccccagctgccaacaggtgccgcacgatggcctcctgggccggcccagggggcagggcagccgccatgtggagggctgtgttcccgtgggccttcatgttgacaaaggtccgcaggtctccccggggcagctccagcagcagctgaaccagagtggggttggcagcctgcacggccaagtgcagaactgtcttgttgctcttgatctcctggctggtgtgattagcacccatttgcagcaacatgtggacacaatccagcctgtctcgggcctgtgtgctcagcacccggggacagaggtcggaagggcgcatagcaacgttaagggccaggatggccgtgtggagcggggtgaggccctcgaagtctctggcttccaggtcaacctggaccccagagttaagcacagccaagagaactcctgggagcccgtaggtagcggccacgtgcaagaccgaacgtccctgatggtcagcggcattgggctctgctcccaggttcaacagatcctccacaatcaggggctggttggcagcagccgccaccaggagaggggtcttgcccttatgctcacgaatgtcaagacgccggtacacctggagcacctcagccgcagcatatgccgcccagcgcagcccccgagccgcaaacaggtgaaggagcgtgtccccctcctcatcctgggccagcagctgctgtggccccaaagccagcatgtgagctcgggccacctccagcgatggtccagggaccacagcggggaactgtgggggtcctgaagggggtgcagaaactctccagggtccagcctccatgccctggggaaatgggcacggctgccctgggtccgagggtgggtagaagtcaggaggcaggaaattttcggcagcagaagcagggcaagagtaggggctgtcagtgtaggcagcatgcgtgttggggtcccagtctggaaagcccaggctgctaggtccagaacccacagtctccgagtgtgcagtcacagcctcattcacagatggggtcaggggctgctctgggggagggagaaattgtccctgcaccccgccagcgtcgggctgctgctgctggcggcgcctctgctcttccagaagcttcttcacggtttgcgttgggcagtggctgcgctcacccctgctcactcggggattccgtggcgtggattgcgggcccccagggccgcggcctcggcgctgcgccagcctcgctgtttcccccgcggagccgccgccgggtccccgatcttgggtccggtacccgcgagtttttaaactaggggttatggcaccgcccagtcctgggcagggcccgcccacaggcctgggagtccccgggtcgcgctccggcgaacgcagtccctgaatgggcgcggcggacttgggaggcggactactcagtccccccgggaaggagggagctggggtccagatctttgctctgaaggagcctagggcaccgggctccaagaggagggagaaaccggggggcctggatttcttttcttttctttttcttttttttcttttctttt

SEQ ID NO: 12968 - RNA, 1958 nt, Homo sapiens
  source 1..1958: mol_type = other RNA
gctgggattacaggcatgagccaccaaatctggcccaaattgagtttaataaagagcttgagtgatgctcagattagggagggagtgaccgggaatgctggggtctggaactgggggcccagctgagctctgaatcagagagcagtgagacctaagggtccctgatctcagagggtccctcctgtctcagggtgaggacctgaagggtgtgggtcccggggagggtgaggaggccattgtaggagatttactgagatggtatcgggatgccccaagcaccacgtagggggattacatctgggtttctgggaacgaagagctgagttaggggagagaacccgaaagatctcagtggggaaaggactaggggtgcagggtgtttcacagaaacaatcaaggggcctcgatttcacagaaatcatcaagagggctccttgtgggtagaagaggggtatcacagcaccccaaatattggggcctgttcacccctctgcagccattctggggttttaatgtaaaaccccaatggcaggatattccacatacattatcatgggtttgcaacattagcatacgctggctgtcccgcaggacggtggggactggaaaatcagtccagggtctgggtttgagtcctaagaggacaggcctggcggcgccacacggctcctcttcaacagctgccggagcccctcagggcccggcccgggccgcagcaggtgaacgggctgctcattctccaggttgcgcagtgtggggtccgccccagctgccaacaggtgccgcacgatggcctcctgggccggcccagggggcagggcagccgccatgtggagggctgtgttcccgtgggccttcatgttgacaaaggtccgcaggtctccccggggcagctccagcagcagctgaaccagagtggggttggcagcctgcacggccaagtgcagaactgtcttgttgctcttgatctcctggctggtgtgattagcacccatttgcagcaacatgtggacacaatccagcctgtctcgggcctgtgtgctcagcacccggggacagaggtcggaagggcgcatagcaacgttaagggccaggatggccgtgtggagcggggtgaggccctcgaagtctctggcttccaggtcaacctggaccccagagttaagcacagccaagagaactcctgggagcccgtaggtagcggccacgtgcaagaccgaacgtccctgatggtcagcggcattgggctctgctcccaggttcaacagatcctccacaatcaggggctggttggcagcagccgccaccaggagaggggtcttgcccttatgctcacgaatgtcaagacgccggtacacctggagcacctcagccgcagcatatgccgcccagcgcagcccccgagccgcaaacaggtgaaggagcgtgtccccctcctcatcctgggccagcagctgctgtggccccaaagccagcatgtgagctcgggccacctccagcgatggtccagggaccacagcggggaactgtgggggtcctgaagggggtgcagaaactctccagggtccagcctccatgccctggggaaatgggcacggctgccctgggtccgagggtgggtagaagtcaggaggcaggaaattttcggcagcagaagcagggcaagagtaggggctgtcagtgtaggcagcatgcgtgttggggtcccagtctggaaagcccaggctgctaggtccagaacccacagtctccgagtgtgctgggaagggagggtggccagtcacagcctcattcacagatggggtcaggggctgctctgggggagggagaaattgtccctgcaccccgccagcgtcgggctgctgctgctggcggcgcctctgctcttccagaagcttcttcacggtttgcgttgggcagtggctgcgctcacccctgctcacccgggccgggagcgg

SEQ ID NO: 12969 - RNA, 1959 nt, Homo sapiens
  source 1..1959: mol_type = other RNA
gctgggattacaggcatgagccaccaaatctggcccaaattgagtttaataaagagcttgagtgatgctcagattagggagggagtgaccgggaatgctggggtctggaactgggggcccagctgagctctgaatcagagagcagtgagacctaagggtccctgatctcagagggtccctcctgtctcagggtgaggacctgaagggtgtgggtcccggggagggtgaggaggccattgtaggagatttactgagatggtatcgggatgccccaagcaccacgtagggggattacatctgggtttctgggaacgaagagctgagttaggggagagaacccgaaagatctcagtggggaaaggactaggggtgcagggtgtttcacagaaacaatcaaggggcctcgatttcacagaaatcatcaagagggctccttgtgggtagaagaggggtatcacagcaccccaaatattggggcctgttcacccctctgcagccattctggggttttaatgtaaaaccccaatggcaggatattccacatacattatcatgggtttgcaacattagcatacgctggctgtcccgcaggacggtggggactggaaaatcagtccagggtctgggtttgagtcctaagaggacaggcctggcggcgccacacggctcctcttcaacagctgccggagcccctcagggcccggcccgggccgcagcaggtgaacgggctgctcattctccaggttgcgcagtgtggggtccgccccagctgccaacaggtgccgcacgatggcctcctgggccggcccagggggcagggcagccgccatgtggagggctgtgttcccgtgggccttcatgttgacaaaggtccgcaggtctccccggggcagctccagcagcagctgaaccagagtggggttggcagcctgcacggccaagtgcagaactgtcttgttgctcttgatctcctggctggtgtgattagcacccatttgcagcaacatgtggacacaatccagcctgtctcgggcctgtgtgctcagcacccggggacagaggtcggaagggcgcatagcaacgttaagggccaggatggccgtgtggagcggggtgaggccctcgaagtctctggcttccaggtcaacctggaccccagagttaagcacagccaagagaactcctgggagcccgtaggtagcggccacgtgcaagaccgaacgtccctgatggtcagcggcattgggctctgctcccaggttcaacagatcctccacaatcaggggctggttggcagcagccgccaccaggagaggggtcttgcccttatgctcacgaatgtcaagacgccggtacacctggagcacctcagccgcagcatatgccgcccagcgcagcccccgagccgcaaacaggtgaaggagcgtgtccccctcctcatcctgggccagcagctgctgtggccccaaagccagcatgtgagctcgggccacctccagcgatggtccagggaccacagcggggaactgtgggggtcctgaagggggtgcagaaactctccagggtccagcctccatgccctggggaaatgggcacggctgccctgggtccgagggtgggtagaagtcaggaggcaggaaattttcggcagcagaagcagggcaagagtaggggctgtcagtgtaggcagcatgcgtgttggggtcccagtctggaaagcccaggctgctaggtccagaacccacagtctccgagtgtgctgggaagggagggtggccagtcacagcctcattcacagatggggtcaggggctgctctgggggagggagaaattgtccctgcaccccgccagcgtcgggctgctgctgctggcggcgcctctgctcttccagaagcttcttcacggtttgcgttgggcagtggctgcgctcacccctgctcaccggaaatcaggagtcc

SEQ ID NO: 12970 - RNA, 2361 nt, Homo sapiens
  source 1..2361: mol_type = other RNA
gctgggattacaggcatgagccaccaaatctggcccaaattgagtttaataaagagcttgagtgatgctcagattagggagggagtgaccgggaatgctggggtctggaactgggggcccagctgagctctgaatcagagagcagtgagacctaagggtccctgatctcagagggtccctcctgtctcagggtgaggacctgaagggtgtgggtcccggggagggtgaggaggccattgtaggagatttactgagatggtatcgggatgccccaagcaccacgtagggggattacatctgggtttctgggaacgaagagctgagttaggggagagaacccgaaagatctcagtggggaaaggactaggggtgcagggtgtttcacagaaacaatcaaggggcctcgatttcacagaaatcatcaagagggctccttgtgggtagaagaggggtatcacagcaccccaaatattggggcctgttcacccctctgcagccattctggggttttaatgtaaaaccccaatggcaggatattccacatacattatcatgggtttgcaacattagcatacgctggctgtcccgcaggacggtggggactggaaaatcagtccagggtctgggtttgagtcctaagaggacaggcctggcggcgccacacggctcctcttcaacagctgccggagcccctcagggcccggcccgggccgcagcaggtgaacgggctgctcattctccaggttgcgcagtgtggggtccgccccagctgccaacaggtgccgcacgatggcctcctgggccggcccagggggcagggcagccgccatgtggagggctgtgttcccgtgggccttcatgttgacaaaggtccgcaggtctccccggggcagctccagcagcagctgaaccagagtggggttggcagcctgcacggccaagtgcagaactgtcttgttgctcttgatctcctggctggtgtgattagcacccatttgcagcaacatgtggacacaatccagcctgtctcgggcctgtgtgctcagcacccggggacagaggtcggaagggcgcatagcaacgttaagggccaggatggccgtgtggagcggggtgaggccctcgaagtctctggcttccaggtcaacctggaccccagagttaagcacagccaagagaactcctgggagcccgtaggtagcggccacgtgcaagaccgaacgtccctgatggtcagcggcattgggctctgctcccaggttcaacagatcctccacaatcaggggctggttggcagcagccgccaccaggagaggggtcttgcccttatgctcacgaatgtcaagacgccggtacacctggagcacctcagccgcagcatatgccgcccagcgcagcccccgagccgcaaacaggtgaaggagcgtgtccccctcctcatcctgggccagcagctgctgtggccccaaagccagcatgtgagctcgggccacctccagcgatggtccagggaccacagcggggaactgtgggggtcctgaagggggtgcagaaactctccagggtccagcctgtggcagagaagatcctacatagaactgggtgtctggggggtcctccatgccctggggaaatgggcacggctgccctgggtccgagggtgggtagaagtcaggaggcaggaaattttcggcagcagaagcagggcaagagtaggggctgtcagtgtaggcagcatgcgtgttggggtcccagtctggaaagcccaggctgctaggtccagaacccacagtctccgagtgtgcagtcacagcctcattcacagatggggtcaggggctgctctgggggagggagaaattgtccctgcaccccgccagcgtcgggctgctgctgctggcggcgcctctgctcttccagaagcttcttcacggtttgcgttgggcagtggctgcgctcacccctgctcactcggggattccgtggcgtggattgcgggcccccagggccgcggcctcggcgctgcgccagcctcgctgtttcccccgcggagccgccgccgggtccccgatcttgggtccggtacccgcgagtttttaaactaggggttatggcaccgcccagtcctgggcagggcccgcccacaggcctgggagtccccgggtcgcgctccggcgaacgcagtccctgaatgggcgcggcggacttgggaggcggactactcagtccccccgggaaggagggagctggggtccagatctttgctctgaaggagcctagggcaccgggctccaagaggagggagaaaccggggggcctggatttcttttcttttctttttcttttttttcttttctttttt

SEQ ID NO: 12971 - RNA, 2005 nt, Homo sapiens
  source 1..2005: mol_type = other RNA
gctgggattacaggcatgagccaccaaatctggcccaaattgagtttaataaagagcttgagtgatgctcagattagggagggagtgaccgggaatgctggggtctggaactgggggcccagctgagctctgaatcagagagcagtgagacctaagggtccctgatctcagagggtccctcctgtctcagggtgaggacctgaagggtgtgggtcccggggagggtgaggaggccattgtaggagatttactgagatggtatcgggatgccccaagcaccacgtagggggattacatctgggtttctgggaacgaagagctgagttaggggagagaacccgaaagatctcagtggggaaaggactaggggtgcagggtgtttcacagaaacaatcaaggggcctcgatttcacagaaatcatcaagagggctccttgtgggtagaagaggggtatcacagcaccccaaatattggggcctgttcacccctctgcagccattctggggttttaatgtaaaaccccaatggcaggatattccacatacattatcatgggtttgcaacattagcatacgctggctgtcccgcaggacggtggggactggaaaatcagtccagggtctgggtttgagtcctaagaggacaggcctggcggcgccacacggctcctcttcaacagctgccggagcccctcagggcccggcccgggccgcagcaggtgaacgggctgctcattctccaggttgcgcagtgtggggtccgccccagctgccaacaggtgccgcacgatggcctcctgggccggcccagggggcagggcagccgccatgtggagggctgtgttcccgtgggccttcatgttgacaaaggtccgcaggtctccccggggcagctccagcagcagctgaaccagagtggggttggcagcctgcacggccaagtgcagaactgtcttgttgctcttgatctcctggctggtgtgattagcacccatttgcagcaacatgtggacacaatccagcctgtctcgggcctgtgtgctcagcacccggggacagaggtcggaagggcgcatagcaacgttaagggccaggatggccgtgtggagcggggtgaggccctcgaagtctctggcttccaggtcaacctggaccccagagttaagcacagccaagagaactcctgggagcccgtaggtagcggccacgtgcaagaccgaacgtccctgatggtcagcggcattgggctctgctcccaggttcaacagatcctccacaatcaggggctggttggcagcagccgccaccaggagaggggtcttgcccttatgctcacgaatgtcaagacgccggtacacctggagcacctcagccgcagcatatgccgcccagcgcagcccccgagccgcaaacaggtgaaggagcgtgtccccctcctcatcctgggccagcagctgctgtggccccaaagccagcatgtgagctcgggccacctccagcgatggtccagggaccacagcggggaactgtgggggtcctgaagggggtgcagaaactctccagggtccagcctgtggcagagaagatcctacatagaactgggtgtctggggggtcctccatgccctggggaaatgggcacggctgccctgggtccgagggtgggtagaagtcaggaggcaggaaattttcggcagcagaagcagggcaagagtaggggctgtcagtgtaggcagcatgcgtgttggggtcccagtctggaaagcccaggctgctaggtccagaacccacagtctccgagtgtgctgggaagggagggtggccagtcacagcctcattcacagatggggtcaggggctgctctgggggagggagaaattgtccctgcaccccgccagcgtcgggctgctgctgctggcggcgcctctgctcttccagaagcttcttcacggtttgcgttgggcagtggctgcgctcacccctgctcacccgggccgggagcggtg

SEQ ID NO: 12972 - RNA, 2062 nt, Homo sapiens
  source 1..2062: mol_type = other RNA
gctgggattacaggcatgagccaccaaatctggcccaaattgagtttaataaagagcttgagtgatgctcagattagggagggagtgaccgggaatgctggggtctggaactgggggcccagctgagctctgaatcagagagcagtgagacctaagggtccctgatctcagagggtccctcctgtctcagggtgaggacctgaagggtgtgggtcccggggagggtgaggaggccattgtaggagatttactgagatggtatcgggatgccccaagcaccacgtagggggattacatctgggtttctgggaacgaagagctgagttaggggagagaacccgaaagatctcagtggggaaaggactaggggtgcagggtgtttcacagaaacaatcaaggggcctcgatttcacagaaatcatcaagagggctccttgtgggtagaagaggggtatcacagcaccccaaatattggggcctgttcacccctctgcagccattctggggttttaatgtaaaaccccaatggcaggatattccacatacattatcatgggtttgcaacattagcatacgctggctgtcccgcaggacggtggggactggaaaatcagtccagggtctgggtttgagtcctaagaggacaggcctggcggcgccacacggctcctcttcaacagctgccggagcccctcagggcccggcccgggccgcagcaggtgaacgggctgctcattctccaggttgcgcagtgtggggtccgccccagctgccaacaggtgccgcacgatggcctcctgggccggcccagggggcagggcagccgccatgtggagggctgtgttcccgtgggccttcatgttgacaaaggtccgcaggtctccccggggcagctccagcagcagctgaaccagagtggggttggcagcctgcacggccaagtgcagaactgtcttgttgctcttgatctcctggctggtgtgattagcacccatttgcagcaacatgtggacacaatccagcctgtctcgggcctgtgtgctcagcacccggggacagaggtcggaagggcgcatagcaacgttaagggccaggatggccgtgtggagcggggtgaggccctcgaagtctctggcttccaggtcaacctggaccccagagttaagcacagccaagagaactcctgggagcccgtaggtagcggccacgtgcaagaccgaacgtccctgatggtcagcggcattgggctctgctcccaggttcaacagatcctccacaatcaggggctggttggcagcagccgccaccaggagaggggtcttgcccttatgctcacgaatgtcaagacgccggtacacctggagcacctcagccgcagcatatgccgcccagcgcagcccccgagccgcaaacaggtgaaggagcgtgtccccctcctcatcctgggccagcagctgctgtggccccaaagccagcatgtgagctcgggccacctccagcgatggtccagggaccacagcggggaactgtgggggtcctgaagggggtgcagaaactctccagggtccagcctgtggcagagaagatcctacatagaactgggtgtctggggggtcctccatgccctggggaaatgggcacggctgccctgggtccgagggtgggtagaagtcaggaggcaggaaattttcggcagcagaagcagggcaagagtaggggctgtcagtgtaggcagcatgcgtgttggggtcccagtctggaaagcccaggctgctaggtccagaacccacagtctccgagtgtgctgggaagggagggtggccagtcacagcctcattcacagatggggtcaggggctgctctgggggagggagaaattgtccctgcaccccgccagcgtcgggctgctgctgctggcggcgcctctgctcttccagaagcttcttcacggtttgcgttgggcagtggctgcgctcacccctgctcaccttccgagcctgggttccggcggaggaagggttaagtggggattgcgcggggcgggggcgggaggaggtggctc

SEQ ID NO: 12973 - RNA, 2379 nt, Homo sapiens
  source 1..2379: mol_type = other RNA
gctgggattacaggcatgagccaccaaatctggcccaaattgagtttaataaagagcttgagtgatgctcagattagggagggagtgaccgggaatgctggggtctggaactgggggcccagctgagctctgaatcagagagcagtgagacctaagggtccctgatctcagagggtccctcctgtctcagggtgaggacctgaagggtgtgggtcccggggagggtgaggaggccattgtaggagatttactgagatggtatcgggatgccccaagcaccacgtagggggattacatctgggtttctgggaacgaagagctgagttaggggagagaacccgaaagatctcagtggggaaaggactaggggtgcagggtgtttcacagaaacaatcaaggggcctcgatttcacagaaatcatcaagagggctccttgtgggtagaagaggggtatcacagcaccccaaatattggggcctgttcacccctctgcagccattctggggttttaatgtaaaaccccaatggcaggatattccacatacattatcatgggtttgcaacattagcatacgctggctgtcccgcaggacggtggggactggaaaatcagtccagggtctgggtttgagtcctaagaggacaggcctggcggcgccacacggctcctcttcaacagctgccggagcccctcagggcccggcccgggccgcagcaggtgaacgggctgctcattctccaggttgcgcagtgtggggtccgccccagctgccaacaggtgccgcacgatggcctcctgggccggcccagggggcagggcagccgccatgtggagggctgtgttcccgtgggccttcatgttgacaaaggtccgcaggtctccccggggcagctccagcagcagctgaaccagagtggggttggcagcctgcacggccaagtgcagaactgtcttgttgctcttgatctcctggctggtgtgattagcacccatttgcagcaacatgtggacacaatccagcctgtctcgggcctgtgtgctcagcacccggggacagaggtcggaagggcgcatagcaacgttaagggccaggatggccgtgtggagcggggtgaggccctcgaagtctctggcttccaggtcaacctggaccccagagttaagcacagccaagagaactcctgggagcccgtaggtagcggccacgtgcaagaccgaacgtccctgatggtcagcggcattgggctctgctcccaggttcaacagatcctccacaatcaggggctggttggcagcagccgccaccaggagaggggtcttgcccttatgctcacgaatgtcaagacgccggtacacctggagcacctcagccgcagcatatgccgcccagcgcagcccccgagccgcaaacaggtgaaggagcgtgtccccctcctcatcctgggccagcagctgctgtggccccaaagccagcatgtgagctcgggccacctccagcgatggtccagggaccacagcggggaactgtgggggtcctgaagggggtgcagaaactctccagggtccagcctgtggcagagaagatcctacatagaactgggtgtctggggggtcctccatgccctggggaaatgggcacggctgccctgggtccgagggtgggtagaagtcaggaggcaggaaattttcggcagcagaagcagggcaagagtaggggctgtcagtgtaggcagcatgcgtgttggggtcccagtctggaaagcccaggctgctaggtccagaacccacagtctccgagtgtgctgggaagggagggtggccagtcacagcctcattcacagatggggtcaggggctgctctgggggagggagaaattgtccctgcaccccgccagcgtcgggctgctgctgctggcggcgcctctgctcttccagaagcttcttcacggtttgcgttgggcagtggctgcgctcacccctgctcactcggggattccgtggcgtggattgcgggcccccagggccgcggcctcggcgctgcgccagcctcgctgtttcccccgcggagccgccgccgggtccccgatcttgggtccggtacccgcgagtttttaaactaggggttatggcaccgcccagtcctgggcagggcccgcccacaggcctgggagtccccgggtcgcgctccggcgaacgcagtccctgaatgggcgcggcggacttgggaggcggactactcagtccccccgggaaggagggagctggggtccagatctttgctctgaaggagcctagggcaccgggctccaagaggagggagaaaccggggggcctggatttcttttcttttctttttcttttttttcttttctttttt

SEQ ID NO: 12974 - RNA, 2022 nt, Homo sapiens
  source 1..2022: mol_type = other RNA
gctgggattacaggcatgagccaccaaatctggcccaaattgagtttaataaagagcttgagtgatgctcagattagggagggagtgaccgggaatgctggggtctggaactgggggcccagctgagctctgaatcagagagcagtgagacctaagggtccctgatctcagagggtccctcctgtctcagggtgaggacctgaagggtgtgggtcccggggagggtgaggaggccattgtaggagatttactgagatggtatcgggatgccccaagcaccacgtagggggattacatctgggtttctgggaacgaagagctgagttaggggagagaacccgaaagatctcagtggggaaaggactaggggtgcagggtgtttcacagaaacaatcaaggggcctcgatttcacagaaatcatcaagagggctccttgtgggtagaagaggggtatcacagcaccccaaatattggggcctgttcacccctctgcagccattctggggttttaatgtaaaaccccaatggcaggatattccacatacattatcatgggtttgcaacattagcatacgctggctgtcccgcaggacggtggggactggaaaatcagtccagggtctgggtttgagtcctaagaggacaggcctggcggcgccacacggctcctcttcaacagctgccggagcccctcagggcccggcccgggccgcagcaggtgaacgggctgctcattctccaggttgcgcagtgtggggtccgccccagctgccaacaggtgccgcacgatggcctcctgggccggcccagggggcagggcagccgccatgtggagggctgtgttcccgtgggccttcatgttgacaaaggtccgcaggtctccccggggcagctccagcagcagctgaaccagagtggggttggcagcctgcacggccaagtgcagaactgtcttgttgctcttgatctcctggctggtgtgattagcacccatttgcagcaacatgtggacacaatccagcctgtctcgggcctgtgtgctcagcacccggggacagaggtcggaagggcgcatagcaacgttaagggccaggatggccgtgtggagcggggtgaggcctgcagaatggagacagtgagggacccgcatctgcacccacctcgcccagccacaccaaccacaccagccctgcccacacccaacttaccctcgaagtctctggcttccaggtcaacctggaccccagagttaagcacagcctgggaggaagagaaggcagactgctgggtaagggtatcccctggcctcctggccctggaagccaaaatctgggcaaccagtctaccccccagacaaacccctgcctgccagctggccataccaagagaactcctgggagcccgtaggtagcggccacgtgcaagaccgaacgtccctgatggtcagcggcattgggctctgctcccaggttcaacagatcctccacaatcaggggctggttggcagcagccgccaccaggagaggggtcttgcccttatgctcacgaatgtcaagacgccggtacacctggagcacctcagccgcagcatatgccgcccagcgcagcccccgagccgcaaacaggtgaaggagcgtgtccccctcctcatcctgggccagcagctgctgtggccccaaagccagcatgtgagctcgggccacctccagcgatggtccagggaccacagcggggaactgtgggggtcctgaagggggtgcagaaactctccagggtccagccagtcacagcctcattcacagatggggtcaggggctgctctgggggagggagaaattgtccctgcaccccgccagcgtcgggctgctgctgctggcggcgcctctgctcttccagaagcttcttcacggtttgcgttgggcagtggctgcgctcacccctgctcaccttccgagcctgggttccggcggaggaagggttaagtggggattgcgcggggcgggggcgggaggaggtggctc

SEQ ID NO: 12975 - RNA, 4961 nt, Homo sapiens
  source 1..4961: mol_type = other RNA
gctgggattacaggcatgagccaccaagactggcctgaactccacgtctttaaatactcaggagacaaagggcagcaaggtgaagagaaagaatgaatcataccagctcagccctggtgggtacatcaaggacactggccagcttttaattcctgttcctatcatgccacagagcacctcccattgactcctctctcttttcccttctcattgatgggcatcttatgcttgactctctgcccctagtaactaactttccaggggttttcttgatctagcccggtaggggagatcctgagaccatcacaacatgccgtcaagacaattggcagctacagcatcaatgctgtaaaatggcagcaaaacaatgcctctaagagacccctattgtgtgacttgtaataggttttgaaaaaggttgatggatagatgacagaagtatcagaagtattggaaagctggcagatttgcagctttgtttcttttgcgcctaagttactctgcttgagttacctgtggtttttggagtccctctctttaacaaacacctatatacaaagttctgatgggtgtaaattactctataacatatatagttcttttaaaaacatgattatcaatgaagtccttacataaagaggaaaaggcacctgttattgttgatcattttaaacctggggaaactgaggctgaaaaaggtaacatggctagccaaggaatgtacatctaatcacccagtcagaatttgaacccaaatccagtgttttttgagccacattattgacaccctctttcactaaagtcctatgatttccatctagatatagtaatagtaataacaaatagatacagctatcaggttgctttctgtgtaaagtgattgtgcttgaagagttgcatctgacatccctttcacccctttactttctggctcagtatctccctaagtatttataaataaataaatgactaaacaagcttggaattcagaccacctcttcctctttggtccaacagtagagagagaggagttaacagttagttatcacatttgtgtcttcattatccctatacccagtaccccttacctgggcaccaaaagggaactaacagcaatgttttctttattcactacatatcttccagccttttcggtcctcgggtataggctaataaataattcatatctagttattgtccttgaggagctactaaaccattctgagagacatctatctatttactcatgtattcatccatccagtaatccattcatccatccatccatccacccatccctgcatccattaatctattcatacactccaaaaagaattactaagcattgacaaaacactaagtgctgttcttggtgctgaagacagtaatgaacaaaacaaaaggccctacattatggaagctccattctattaaggccatgaacaaagttaacaaattagtgtgtaatataataaaagtgagagataagtgacataaagttaaagcaaggaaaggaaatagagatctggtgatggagacaaaggtgaagagcactgtggtagagcaggtgcaaagggaagccttcaccaacgtgactctgtcttggtgatagatcagcaatccctgaccatgaccctcacccacaccaactcccctaacccccacccatgatttctaaagaagccagcatcagacccactatgctgccagctcccttcagaagctccctccccatatgaaacttatttttcatgtattagtgttgaccaggctctcactggcctccaccttcctctcttttccctacttctgacctcagaaggctttgttgttggcacagtattttaaggttggcacaatattagggatctcacatcagccctgtgaatctgcaacacattcccagggaataatgtactgagcaaaggatgaaggctcttcattctgccgactctccagacacaccgaacatttcaagatgattgtagcagcatgcagcagacaaacaggattctggagccaaatgtgtgtcctgtcactgacttttcagccttgaagggcaaaacccctcttgaaaggctcacttttgtcatctaagctgctaccatgttttagatgatgcctcctgagttctttagaagcccagcctgggatgtctgtttcagtagtcagtggcacgatgagccccagaatactggaaatctgctttgaccaagttcttgcaataaaacttgaatctcattaagccatttgtaattaatcctgagtagaagatggatggaaggattgattaggctaggatactgttgctgctgctgctgacaacagctgatttctaccactcttctgggaacttgccatgaattgtgtcatttatacctcacaataaccctatgaggtgtgtactaatgttatccctactgtacagaggaggagaccaaagcaaagaggggttaagtaacttgctcaaggtaacacagctggagtatggctgagtcaggtgaaaactccaacatgagagctattgtagtaagatgcagagctgggatttgaactcactacaccacactgaggttcgtaatccttgggacggcaatgagctcttaaaagcttagggagagctaatgcacagcaaccatgggcttgcttcactcacaaatctgggaataaaaaataggtaatcaacatgtgttccctgaagaaggaagctgttacacagtaattctgagctcctaaattggcagaaggaactttgcagcagggagatcctattgtttgggagtgtttcgagtggtccccaagggtgcagggaactcatgtttggtgtcaatagatcactctagggtgtcagaaacagagaagctgtttgttaactcacccttctgacaccccctgtgaatgtcatgtaaatttcatctttgtgtagcatttcatgaattttcagagctctttcagagtcaacaccttattcaatgtcttatcttggtgttcaagcttcttcacaatgaggctctagcctaagtttccagactcctcgccttcacccctgcttcccaccctatgaccgtccattcctcttcaagccacatcaatcttcctgacatccccacaattacctcatcctcacatacctacttattggtcttcctgcttttatcccatcctcttcctcccttctccacactgcagccactctgttgtgatcactccagtcacaacagtcccaacttaaagttgccctccatgctccagacacaatggcctcttctctgttcttcagacttgctaaccttcttctcctatgccctttgtatgtgccatgattatctttgcctggaaaactaccctctttccttccccaatctgtcagggcatggatggctctctctcatcattctgatctcagtttaaatctcatttcttcagacaaacctcttttctctatgtgagttcctctcttttgtcttctgtcaactttactatttgttcttgtaatagtactttttattatttggatttgttaagtattttaattatcttagtaggctgaaggttccatgagatcagtaccaagtttgttctgtgcttaaaacaatccctggcacatagcaggtgttaataaatatgctgggtcagtggatagaggaataaatgagtgaatgaatgaatgaatgaatgaatggactgatggatattttagtctttccactgattggtaacctctatgtgttctttgtcttttctctgcactggacaaatcttgtttagcattttcaagtcaatgatttgttgaatctttgcatctatctcataaagaatgtattatccttatcaaaatctagatatcatctcaaatttatacaactacaaataatggaaccagaatttgaacccagctttatctgatacccaagtccaagcatgtgctggagataacacaacatgtattactcctgtccatttatatgagcaggagaggaaagacattagcttagatgtcagcaagctaagtctcttagagctatgtttatccacaacgttgaacagcagacataatcaaaactatgttttatacagtgagcctgcacatattcacgtgtgaatgtgtgtgcgcacatctctaaaataagttttgcaaaataatacacattgtcattacatgggaccatgttctgatagcttctattcttttgatggcatttttgtaatgctgatggagccactgaattgatttcacagtttgagagtgggtcataaccttaagtttaaaaacctctttcttagaggagctaataaagtgccagaggccacagtgggaacaggtgcatgacaactggatctgaggtggcttgcaggagacatttctttcccagagatctgaaggatgaagataattcaagggcttcagtttgaggggttggtggaggaactggaaatggtacctgagccaggcaaggcccacatgagggttttaggtcttacccctgccatttctatggccagccacttgtgtcttttacccaaccctataggccactgggcccatcatttccacatttgctcttatgaaatgtgctcaacctgccctttcttgtgccttgtgcctcagatcttatcttatttctgtacgatgctctatcttccctggggaaaggaaaaacaacaacaacaacaacaccctgccctctgctccctgcatgggaattactgcccatctttaagccatactctgttctgaggccccagatgccagttttcagagagcctggggaactcccttactaacagcagctcccatttgactgtgccttgagggtgctgccaggagcacgtgcagggcaaggggaagatagaatgggcagaattgttttaacaaaagcaagactgctttaaagtggttgcatgtgggattatttttgaaacataggccctctaggatgaaaagaagaaaaatttggaaa

SEQ ID NO: 12976 - RNA, 1808 nt, Homo sapiens
  source 1..1808: mol_type = other RNA
gctgggattacaggcatgagccaccaagccagtcctaccccacgcttgtcagtattctgggagatcccccagttcccagccccctgggccctggcaacccgctccccacccttctcccgtcagacccgaccaaggagacctaagcttcaacccaggcccccgcgcccctccactacccgtccggcggctcaggcctcggcgccttcgggacccacgagcagcagcggctgggcattcttgcccttgtcgtgccagcacacgtcgaagaaggggtacacgggcctgggcaggcgctcgtggaaggcaaaaagcggcacgagcgcgtcggcgtcgctggcatcgtagaaggagaggacgccgtcgccgaagctcaggtaaaggccaatgcgcgtgggccgcctctcggggctgcgcagagcgcgcggctccttggcctccacgtgtgcctccaggatcttgccctcgcgcagccccagcagccacaggccctgcgagggcaccgcgtgcaggcgcccgcggcggggggcctcggccgcgatcacgcccagcgcccagcgcggcttgtcgccaacatccacctcccagtagtgctcgccctcggagagctgctggtgcgccaccaccgccaccgccttgtcgaactggcgcgggtcctccccggccggcggcgccttctgctccgagcactccacgcggcggccagaggaagacaccaccaggctcgggtgcgcagagctcgggtcaaaggtcagctcctccagcgctggcatcagagcccggaacatcttcctccacacctggaatttgaagtcatctgagataattggcagctggatgtccagacgggcgggtgggggagactctgccaggatcttctgcagcctgctggtcaccaggcagtatttcatgaggaactcagtctgcggcttgtccgccacctcctccaggaccttctccatctgccgcagctgctccaggtaagagttcaggctccccagctcccggcgcaaggcgacccctgcctcaccccgtacacgctctgcctcgcggtccaaggagccctccagtgcagccaggaacacccgcatcttgcccagctgctcccccacggccccccggaactgacgcactgtctcctccacctccaccagctgatgctccagcacagccacactcttctccttgcgcatgcatgcctcctgcagctgcagtttctgctgtggcagctgtgtcttgaggcgtgcgtgggcctcggcggcaggcaggaggcgatgaccgcggtgcgagccgagtgaggcgcacactccgcacaccagcgcgcggtcctgctcgcagtagatgctcagcgggtccaggtgctcctcgcagtggccctgcggcacctgggccagcccctccaccaggcgcgccagctgcaggttggtgctgagtgcctgcggccgcgtgggggcctggcagcaggggcagagaacggtgccatccgccgccggctccccggccacgcggcctaggcaggcgcggcagaaactgtggccgcactcggctgtcacgggcgcgtcgaacagctgcaggcacagcgggcaggacagctcctggtgcaggaggccgggcgcagccgacatggcgggcaggtctggttggagatcttaggctgaaagagtctcgaaggaggaccggtcagggttgagcttagctggactggggtcagggctgggtccaaggatctgagacaagcagcaggctccaagcaaggacagggactcacaggggcagctggcagtggacaccacgcgtgatgggcacacagt

SEQ ID NO: 12977 - RNA, 1442 nt, Homo sapiens
  source 1..1442: mol_type = other RNA
gctgggattacaggcatgagccaccaagccagtcctaccccacgcttgtcagtattctgggagatcccccagttcccagccccctgggccctggcaacccgctccccacccttctcccgtcagacccgaccaaggagacctaagcttcaacccaggcccccgcgcccctccactacccgtccggcggctcaggcctcggcgccttcgggacccacgagcagcagcggctgggcattcttgcccttgtcgtgccagcacacgtcgaagaaggggtacacgggcctgggcaggcgctcgtggaaggcaaaaagcggcacgagcgcgtcggcgtcgctggcatcgtagaaggagaggacgccgtcgccgaagctcaggtaaaggccaatgcgcgtgggccgcctctcggggctgcgcagagcgcgcggctccttggcctccacgtgtgcctccaggatcttgccctcgcgcagccccagcagccacaggccctgcgagggcaccgcgtgcaggcgcccgcggcggggggcctcggccgcgatcacgcccagcgcccagcgcggcttgtcgccaacatccacctcccagtagtgctcgccctcggagagctgctggtgcgccaccaccgccaccgccttgtcgaactggcgcgggtcctccccggccggcggcgccttctgctccgagcactccacgcggcggccagaggaagacaccaccaggctcgggtgcgcagagctcgggtcaaaggtcagctcctccagcgctggcatcagagcccggaacatcttcctccacacctggaatttgaagtcatctgagataattggcagctggatgtccagacgggcgggtgggggagactctgccaggatcttctgcagcctgctggtcaccaggcagtatttcatgaggaactcagtctgcggcttgtccgccacctcctccaggaccttctccatctgccgcagctgctccaggtaagagttcaggctccccagctcccggcgcaaggcgacccctgcctcaccccgtacacgctctgcctcgcggtccaaggagccctccagtgcagccaggaacacccgcatcttgcccagctgctcccccacggccccccggaactgacgcactgtctcctccacctccaccagctgatgctccagcacagccacactcttctccttgcgcatgcatgcctcctgcagctgcagtttctgctgtggcagctgtgtgtttgctcagcgcccttatcgccaggctccatccctgcgcggctttcctctgccagccccgccttaagctcctcagaccctctttcctggctgcttcgccccgcccccgccccccgcaactccaggagctcgtgagcctctctagagactcagaatccaaatcactgcagcgacctccccatcggccccgtgccaccgaacagcccctcc

SEQ ID NO: 12978 - RNA, 1997 nt, Homo sapiens
  source 1..1997: mol_type = other RNA
gctgggattacaggcatgagccaccaagcccagccctctgaggaatttttcatcactcctttctccttcctgtcattttttctccagcctcaggcaatttcctgcctcgattttgttttcttcctttaaggaatgttctatttttatttggcagataaaatgaggttacttagagatcatcttgagtctctcaaggcttatttttaagctttcttaaaattggtatacattagcctttagtctagctccagtttggatctcttatgaaagtacaacctttctgagtctctactcaatgccccacatgttcaagatctttccactttaactggttggcattcaaacttctcccagctcagtgtgagctctgagagtttttcctcttataactccctggcagtttttcttttcacctaatgcaacacatatgcatctacgtctatttaattataagttaataaacttttcattttaaaaggcttatatgtatattttcagaagcagcaaggtagacaaaaaacactggtgaaaattgtatctgatcctaaagtcagtcttttggagaagacaatttcattagatgggtgctgacagccatcgagagaaaaggaaagcagactgagtttctggggactactgcaagaagaaaaagagaacatagagagctggcctcatcctcaaaagtgatcccacatctaaccaaattaaaaaatccacatgaggtttctcaatacctactgtaaacaatttatcaagatacctggttagcacttcgtgtacaaagtgataaccagacgtcatttttcttggaaaaatcggggttggaaccacagctttgacttcattatcaatatatttaaccaacaatctgggctcctctatggaagtggcttaaatgccttgcagattaaccatggactaagaactttctttgatcttgaatactgttccaaaacacacaaccccagggctccatttctcacccaatataatcattcctgagcagagcattatcaaatagtatcaagccaggaaactggcttagggtactaaggtgaaaggatttagccaagtagcaacccaaatatgaacaaggaaatgagcttaagacacattaagcatttagaataagccccacctgactgatgaccatggtggattaagcttcatctttaattattgatattaatgatctactgtgagcaagatgatctctaaggtactttctaattgtgaaatattattctgtcttatgtatcagacataactgatagcctatcactacatgtgctttactgactacatttctgtcggtcttactaaaagtaaagagctcaactgttgtcatcatctaaaggtgccaccacttttatttgtttaccagatcaccagatgatactggtccattacccttgacctagtcagaccttgacaaaagacttaatggtgctatttaggatgcatttccttgctgctttgtgcaggtggctttctcgttgttgcataaacagtgacgggaacatcagttattgtcaggcaatgacttccagggcacctccggagttgcctggttggtgacatctccttcccattacaggcagcactggagctcagcccaggttccagctcaattgaagaatctcctccttccactggaaacctccttggctgggttccaaattgaaaaggcatacttcactgaaaaccaaaagaggctgagtctgattcctgtagaggtgaataaatcaatgctttctactggcctttccacagaaggctggaattgccaaaggaatgatgatcaaatgttccggtgacacccggaaattatgacatcaggagattctttcacatagtttcctacctgctgccagttaccccggcctccggagctgccgatgctcgaagatgttgacaaggcagctaggatatacagtccagaagcccagtcgctacggtaacggtgacacgcaagtgcacttgcgcggccttctgac

SEQ ID NO: 12979 - RNA, 3358 nt, Homo sapiens
  source 1..3358: mol_type = other RNA
gctgggattacaggcatgagccaccaagcccggcctattaactttcttctatatgctactcatttgtctagtaaagagtaaataataaactttttccttagaagaaatatatatcatttgtccaacagttacttaagtaggcagggattctattccattttacatatgacactagattttctgaatctcaatcttggactcattggtgttttgtagccaagagaattcctcaatggtatggattttctgttgaagatgaaggttggaagtctgagagaattctttttcagacacatcacattcacaaggtttttcatctgtgtggattttctgatgtacagtaaggttttttctttgcctaaaaactttactacaatcattacacccatagggtttctcccctgtgtgaattctctggtggccaactaaattcctcttagaagtaaaggatttcctacacttgtcacactcataaggtttttccccagtgtgcattctctgatgtacaacaaggtttttattctgactaaagtcttttccacactcattacatttataaggtttctctccagtatggattctttgatgtaccataagatttctactagaggtaaggactttcctacatacatgacattcgtaggttttttctccactgtgaattctttgatgttcaatcaggtttctgttgtacgtaaaaccttttccacactcactacacgcatagggcttctcaccagtatggatcctctgatgggctataaggtttgagcggtaactgaagaccttcccacagtcattgcatttataagatttttccctcgtgtgaattctctgatgtccaatgaggcttttcttcagaatgaagcatttgccacactcatcacactcatagggtttctcaccactgtggattctcttatgctcaatgaggtttctgtttgaactgaaagctcttccacactcactgcattcaaagggtttttctccggtgtggattctccgatgtacaagcaggcttgaattgtaactgaaagccttcccacaatcctcacatttgtaggctttctcttgtgtatggagtttctgatggaccataaaacttttgctcataataaaggttttcccacactctcgacattcatatggcttctccccattgtggagtctctcatggtcaatgaggtttctgtttgaaccgaagaccttaccacaatctttacattcatagagattctctccagtgtggaacctttgatgtaaaatgaggctcttcttcagaataaaaactttcccacattcattacattcatagggcttctccccattgtggagtctctggtggtcaaaaaggtaagcactttgagtaaaggctttcccacattcagtgcatttgtaaggtttctctctgctgtgcatcctcttatggtcaatgaagtttgacttagaactgaaaatcttcccacactttttacaaccaaaggttttcttttctgtgtggactctctgatgtaagaggaggcttttgcttcgaatgaaaacttttccacattctttacacttgtaagggttctctgcactgtggagtcgctgatggtcaataagataagtggtctgagcaaaggtctttccacattcatcacatttatagggtttttccccagagtggattctctggtgcagaatgaggctcttcttcagaatgaaagctttctgacacttattacatttataaggttcttcccctttgtggagcctctgatggtcaatgaggtaagcattctgagagaagactttcccacattcattacacttataaggtctctcccctgaatggcgccttagatgtataattaggcctgagtgcctatagaagccctttccacactccttacacttataaggtttctccccagtgtggatcctctgatggtttagaaggtaagcactttgagaaaatgctttcccacattcattacatttataaggtttctcccctgaatggttccgtaaatgcattagaaggctcgaacgctgaataaagccttttccacattccttacatttatgaggtttctcaccagtgtggattctccgatggtttataagatgggagattttattaaaatgtttacaacacatatcacatttataaaacttctttccttcagtacctattaaactttcagaaatagctgaaccgaaagtcaagctgtctcctaattccttccacttttggccttgtttctctggtggagtccttttcttcttgtctcgttcacaaagggaaactttcttcactgtatctgccctttcatctgtttcatttccccactgacttgccaaaacttgccattcacactcttcttcaaaatcaaggacctggggaacacttccttgaagtctttttgatgttcctttatgagagtctgctctttgagaactacttggctttgatgtcacctcctcattctcggtcatggtctcccattctagggaggtcacatttccataattctccagcatcacatcccagtacaaggccctctggattgggcccagacatgcccattcctctgaagtgaagcatactgacacctcctcgaacatcaccaactccatgctgaggatcctggaggttgaatgccactaggtcagtaggaggatgcgggcaaatttcagctgctatgtggctgccaggaagtacaggaggaagtgttgttcctggggcactcaccaccttctggagagtgtcctgatccttgacaaggactggaacttgtattgctggtccatcaaggtctttctgcagctcctctaccagggccacagcctcctcgccacttccagggtgatggagctgtacccaggtccgaatctccccaggcaggatgctcagaaactgctccagcaccagcagctccaggatctgtgccttggtgcgtgcttctggtctcagccaccggcgacagagttccctgagccggctcagggcttcctggggtccagatgtctcatggtaacgtaattgtctaaagtgtaggtgggaggtctcccaaacagaggagctacttccttggaagctggttccccatttccaggtatcatccttccccttcacaaggccctcttgtctcagagcattgtgggctacattttctcttgtcattgttgttttttgaaaaaggctcctctccagtccaggtctccttaatccttgacttcttccttacagcttggagagtatcatcgggggctcccgctgcggctccagccttgcgtaccgccgcctcggcgccaggccgctaggagatgacacaggaacgagcccttccggcagccgaggcacagaataatg

SEQ ID NO: 12980 - RNA, 3628 nt, Homo sapiens
  source 1..3628: mol_type = other RNA
gctgggattacaggcatgagccaccaagcccggcctattaactttcttctatatgctactcatttgtctagtaaagagtaaataataaactttttccttagaagaaatatatatcatttgtccaacagttacttaagtaggcagggattctattccattttacatatgacactagattttctgaatctcaatcttggactcattggtgttttgtagccaagagaattcctcaatggtatggattttctgttgaagatgaaggttggaagtctgagagaattctttttcagacacatcacattcacaaggtttttcatctgtgtggattttctgatgtacagtaaggttttttctttgcctaaaaactttactacaatcattacacccatagggtttctcccctgtgtgaattctctggtggccaactaaattcctcttagaagtaaaggatttcctacacttgtcacactcataaggtttttccccagtgtgcattctctgatgtacaacaaggtttttattctgactaaagtcttttccacactcattacatttataaggtttctctccagtatggattctttgatgtaccataagatttctactagaggtaaggactttcctacatacatgacattcgtaggttttttctccactgtgaattctttgatgttcaatcaggtttctgttgtacgtaaaaccttttccacactcactacacgcatagggcttctcaccagtatggatcctctgatgggctataaggtttgagcggtaactgaagaccttcccacagtcattgcatttataagatttttccctcgtgtgaattctctgatgtccaatgaggcttttcttcagaatgaagcatttgccacactcatcacactcatagggtttctcaccactgtggattctcttatgctcaatgaggtttctgtttgaactgaaagctcttccacactcactgcattcaaagggtttttctccggtgtggattctccgatgtacaagcaggcttgaattgtaactgaaagccttcccacaatcctcacatttgtaggctttctcttgtgtatggagtttctgatggaccataaaacttttgctcataataaaggttttcccacactctcgacattcatatggcttctccccattgtggagtctctcatggtcaatgaggtttctgtttgaaccgaagaccttaccacaatctttacattcatagagattctctccagtgtggaacctttgatgtaaaatgaggctcttcttcagaataaaaactttcccacattcattacattcatagggcttctccccattgtggagtctctggtggtcaaaaaggtaagcactttgagtaaaggctttcccacattcagtgcatttgtaaggtttctctctgctgtgcatcctcttatggtcaatgaagtttgacttagaactgaaaatcttcccacactttttacaaccaaaggttttcttttctgtgtggactctctgatgtaagaggaggcttttgcttcgaatgaaaacttttccacattctttacacttgtaagggttctctgcactgtggagtcgctgatggtcaataagataagtggtctgagcaaaggtctttccacattcatcacatttatagggtttttccccagagtggattctctggtgcagaatgaggctcttcttcagaatgaaagctttctgacacttattacatttataaggttcttcccctttgtggagcctctgatggtcaatgaggtaagcattctgagagaagactttcccacattcattacacttataaggtctctcccctgaatggcgccttagatgtataattaggcctgagtgcctatagaagccctttccacactccttacacttataaggtttctccccagtgtggatcctctgatggtttagaaggtaagcactttgagaaaatgctttcccacattcattacatttataaggtttctcccctgaatggttccgtaaatgcattagaaggctcgaacgctgaataaagccttttccacattccttacatttatgaggtttctcaccagtgtggattctccgatggtttataagatgggagattttattaaaatgtttacaacacatatcacatttataaaacttctttccttcagtacctattaaactttcagaaatagctgaaccgaaagtcaagctgtctcctaattccttccacttttggccttgtttctctggtggagtccttttcttcttgtctcgttcacaaagggaaactttcttcactgtatctgccctttcatctgtttcatttccccactgacttgccaaaacttgccattcacactcttcttcaaaatcaaggacctggggaacacttccttgaagtctttttgatgttcctttatgagagtctgctctttgagaactacttggctttgatgtcacctcctcattctcggtcatggtctcccattctagggaggtcacatttccataattctccagcatcacatcccagtacaaggccctctggattgggcccagacatgcccattcctctgaagtgaagcatactgacacctcctcgaacatcaccaactcctggggctgggctgttaggagcataagtgccattaattgatttcttgggttctcttcctgggaaagggcagaagcttcaggggcaggagaatcatgctgaggatcctggaggttgaatgccactaggtcagtaggaggatgcgggcaaatttcagctgctatgtggctgccaggaagtacaggaggaagtgttgttcctggggcactcaccaccttctggagagtgtcctgatccttgacaaggactggaacctcaagtatggagcatcaaaacagcagtaaagctttgcattgagaacaatggagctgccctcgagccccactcatggcactggtgacctctcccagaggagactgtacacaacggtgggaacagaagccagacttgtattgctggtccatcaaggtctttctgcagctcctctaccagggccacagcctcctcgccacttccagggtgatggagctgtacccaggtccgaatctccccaggcaggatgctcagaaactgctccagcaccagcagctccaggatctgtgccttggtgcgtgcttctggtctcagccaccggcgacagagttccctgagccggctcagggcttcctggggtccagatgtctcatggtaacgtaattgtctaaagtgtaggtgggaggtctcccaaacagaggagctacttccttggaagctggttccccatttccaggtatcatccttccccttcacaaggccctcttgtctcagagcattgtgggctacattttctcttgtcattgttgttttttgaaaaaggctcctctccagtccaggtctccttaatccttgacttcttccttacagcttggagagtatcatccatattcctgtgcacagcagcctcaatccaaaggatctgcacagcacagatcttgcctgatctcctccttgagttcagtgaagaagttcctaagagggtcttgagtcacgaaagcgccagacccacatcttgaacaaagcgcagaaggaact

SEQ ID NO: 12981 - RNA, 3583 nt, Homo sapiens
  source 1..3583: mol_type = other RNA
gctgggattacaggcatgagccaccaagcccggcctattaactttcttctatatgctactcatttgtctagtaaagagtaaataataaactttttccttagaagaaatatatatcatttgtccaacagttacttaagtaggcagggattctattccattttacatatgacactagattttctgaatctcaatcttggactcattggtgttttgtagccaagagaattcctcaatggtatggattttctgttgaagatgaaggttggaagtctgagagaattctttttcagacacatcacattcacaaggtttttcatctgtgtggattttctgatgtacagtaaggttttttctttgcctaaaaactttactacaatcattacacccatagggtttctcccctgtgtgaattctctggtggccaactaaattcctcttagaagtaaaggatttcctacacttgtcacactcataaggtttttccccagtgtgcattctctgatgtacaacaaggtttttattctgactaaagtcttttccacactcattacatttataaggtttctctccagtatggattctttgatgtaccataagatttctactagaggtaaggactttcctacatacatgacattcgtaggttttttctccactgtgaattctttgatgttcaatcaggtttctgttgtacgtaaaaccttttccacactcactacacgcatagggcttctcaccagtatggatcctctgatgggctataaggtttgagcggtaactgaagaccttcccacagtcattgcatttataagatttttccctcgtgtgaattctctgatgtccaatgaggcttttcttcagaatgaagcatttgccacactcatcacactcatagggtttctcaccactgtggattctcttatgctcaatgaggtttctgtttgaactgaaagctcttccacactcactgcattcaaagggtttttctccggtgtggattctccgatgtacaagcaggcttgaattgtaactgaaagccttcccacaatcctcacatttgtaggctttctcttgtgtatggagtttctgatggaccataaaacttttgctcataataaaggttttcccacactctcgacattcatatggcttctccccattgtggagtctctcatggtcaatgaggtttctgtttgaaccgaagaccttaccacaatctttacattcatagagattctctccagtgtggaacctttgatgtaaaatgaggctcttcttcagaataaaaactttcccacattcattacattcatagggcttctccccattgtggagtctctggtggtcaaaaaggtaagcactttgagtaaaggctttcccacattcagtgcatttgtaaggtttctctctgctgtgcatcctcttatggtcaatgaagtttgacttagaactgaaaatcttcccacactttttacaaccaaaggttttcttttctgtgtggactctctgatgtaagaggaggcttttgcttcgaatgaaaacttttccacattctttacacttgtaagggttctctgcactgtggagtcgctgatggtcaataagataagtggtctgagcaaaggtctttccacattcatcacatttatagggtttttccccagagtggattctctggtgcagaatgaggctcttcttcagaatgaaagctttctgacacttattacatttataaggttcttcccctttgtggagcctctgatggtcaatgaggtaagcattctgagagaagactttcccacattcattacacttataaggtctctcccctgaatggcgccttagatgtataattaggcctgagtgcctatagaagccctttccacactccttacacttataaggtttctccccagtgtggatcctctgatggtttagaaggtaagcactttgagaaaatgctttcccacattcattacatttataaggtttctcccctgaatggttccgtaaatgcattagaaggctcgaacgctgaataaagccttttccacattccttacatttatgaggtttctcaccagtgtggattctccgatggtttataagatgggagattttattaaaatgtttacaacacatatcacatttataaaacttctttccttcagtacctattaaactttcagaaatagctgaaccgaaagtcaagctgtctcctaattccttccacttttggccttgtttctctggtggagtccttttcttcttgtctcgttcacaaagggaaactttcttcactgtatctgccctttcatctgtttcatttccccactgacttgccaaaacttgccattcacactcttcttcaaaatcaaggacctggggaacacttccttgaagtctttttgatgttcctttatgagagtctgctctttgagaactacttggctttgatgtcacctcctcattctcggtcatggtctcccattctagggaggtcacatttccataattctccagcatcacatcccagtacaaggccctctggattgggcccagacatgcccattcctctgaagtgaagcatactgacacctcctcgaacatcaccaactcctggggctgggctgttaggagcataagtgccattaattgatttcttgggttctcttcctgggaaagggcagaagcttcaggggcaggagaatcatgctgaggatcctggaggttgaatgccactaggtcagtaggaggatgcgggcaaatttcagctgctatgtggctgccaggaagtacaggaggaagtgttgttcctggggcactcaccaccttctggagagtgtcctgatccttgacaaggactggaacctcaagtatggagcatcaaaacagcagtaaagctttgcattgagaacaatggagctgccctcgagccccactcatggcactggtgacctctcccagaggagactgtacacaacggtgggaacagaagccagacttgtattgctggtccatcaaggtctttctgcagctcctctaccagggccacagcctcctcgccacttccagggtgatggagctgtacccaggtccgaatctccccaggcaggatgctcagaaactgctccagcaccagcagctccaggatctgtgccttggtgcgtgcttctggtctcagccaccggcgacagagttccctgagccggctcagggcttcctggggtccagatgtctcatggtaacgtaattgtctaaagtgtaggtgggaggtctcccaaacagaggagctacttccttggaagctggttccccatttccaggtatcatccttccccttcacaaggccctcttgtctcagagcattgtgggctacattttctcttgtcattgttgttttttgaaaaaggctcctctccagtccaggtctccttaatccttgacttcttccttacagcttggagagtatcatcgggggctcccgctgcggctccagccttgcgtaccgccgcctcggcgccaggccgctaggagatgacacaggaacgagcccttccggcagccgaggcacagaataatg

SEQ ID NO: 12982 - RNA, 3495 nt, Homo sapiens
  source 1..3495: mol_type = other RNA
gctgggattacaggcatgagccaccaagcccggcctattaactttcttctatatgctactcatttgtctagtaaagagtaaataataaactttttccttagaagaaatatatatcatttgtccaacagttacttaagtaggcagggattctattccattttacatatgacactagattttctgaatctcaatcttggactcattggtgttttgtagccaagagaattcctcaatggtatggattttctgttgaagatgaaggttggaagtctgagagaattctttttcagacacatcacattcacaaggtttttcatctgtgtggattttctgatgtacagtaaggttttttctttgcctaaaaactttactacaatcattacacccatagggtttctcccctgtgtgaattctctggtggccaactaaattcctcttagaagtaaaggatttcctacacttgtcacactcataaggtttttccccagtgtgcattctctgatgtacaacaaggtttttattctgactaaagtcttttccacactcattacatttataaggtttctctccagtatggattctttgatgtaccataagatttctactagaggtaaggactttcctacatacatgacattcgtaggttttttctccactgtgaattctttgatgttcaatcaggtttctgttgtacgtaaaaccttttccacactcactacacgcatagggcttctcaccagtatggatcctctgatgggctataaggtttgagcggtaactgaagaccttcccacagtcattgcatttataagatttttccctcgtgtgaattctctgatgtccaatgaggcttttcttcagaatgaagcatttgccacactcatcacactcatagggtttctcaccactgtggattctcttatgctcaatgaggtttctgtttgaactgaaagctcttccacactcactgcattcaaagggtttttctccggtgtggattctccgatgtacaagcaggcttgaattgtaactgaaagccttcccacaatcctcacatttgtaggctttctcttgtgtatggagtttctgatggaccataaaacttttgctcataataaaggttttcccacactctcgacattcatatggcttctccccattgtggagtctctcatggtcaatgaggtttctgtttgaaccgaagaccttaccacaatctttacattcatagagattctctccagtgtggaacctttgatgtaaaatgaggctcttcttcagaataaaaactttcccacattcattacattcatagggcttctccccattgtggagtctctggtggtcaaaaaggtaagcactttgagtaaaggctttcccacattcagtgcatttgtaaggtttctctctgctgtgcatcctcttatggtcaatgaagtttgacttagaactgaaaatcttcccacactttttacaaccaaaggttttcttttctgtgtggactctctgatgtaagaggaggcttttgcttcgaatgaaaacttttccacattctttacacttgtaagggttctctgcactgtggagtcgctgatggtcaataagataagtggtctgagcaaaggtctttccacattcatcacatttatagggtttttccccagagtggattctctggtgcagaatgaggctcttcttcagaatgaaagctttctgacacttattacatttataaggttcttcccctttgtggagcctctgatggtcaatgaggtaagcattctgagagaagactttcccacattcattacacttataaggtctctcccctgaatggcgccttagatgtataattaggcctgagtgcctatagaagccctttccacactccttacacttataaggtttctccccagtgtggatcctctgatggtttagaaggtaagcactttgagaaaatgctttcccacattcattacatttataaggtttctcccctgaatggttccgtaaatgcattagaaggctcgaacgctgaataaagccttttccacattccttacatttatgaggtttctcaccagtgtggattctccgatggtttataagatgggagattttattaaaatgtttacaacacatatcacatttataaaacttctttccttcagtacctattaaactttcagaaatagctgaaccgaaagtcaagctgtctcctaattccttccacttttggccttgtttctctggtggagtccttttcttcttgtctcgttcacaaagggaaactttcttcactgtatctgccctttcatctgtttcatttccccactgacttgccaaaacttgccattcacactcttcttcaaaatcaaggacctggggaacacttccttgaagtctttttgatgttcctttatgagagtctgctctttgagaactacttggctttgatgtcacctcctcattctcggtcatggtctcccattctagggaggtcacatttccataattctccagcatcacatcccagtacaaggccctctggattgggcccagacatgcccattcctctgaagtgaagcatactgacacctcctcgaacatcaccaactcctggggctgggctgttaggagcataagtgccattaattgatttcttgggttctcttcctgggaaagggcagaagcttcaggggcaggagaatcatgctgaggatcctggaggttgaatgccactaggtcagtaggaggatgcgggcaaatttcagctgctatgtggctgccaggaagtacaggaggaagtgttgttcctggggcactcaccaccttctggagagtgtcctgatccttgacaaggactggaacttgtattgctggtccatcaaggtctttctgcagctcctctaccagggccacagcctcctcgccacttccagggtgatggagctgtacccaggtccgaatctccccaggcaggatgctcagaaactgctccagcaccagcagctccaggatctgtgccttggtgcgtgcttctggtctcagccaccggcgacagagttccctgagccggctcagggcttcctggggtccagatgtctcatggtaacgtaattgtctaaagtgtaggtgggaggtctcccaaacagaggagctacttccttggaagctggttccccatttccaggtatcatccttccccttcacaaggccctcttgtctcagagcattgtgggctacattttctcttgtcattgttgttttttgaaaaaggctcctctccagtccaggtctccttaatccttgacttcttccttacagcttggagagtatcatccatattcctgtgcacagcagcctcaatccaaaggatctgcacagcacagatcttgcctgatctcctccttgagttcagtgaagaagttcctaagagggtcttgagtcacgaaagcgccagacccacatcttgaacaaagcgcagaaggaact

SEQ ID NO: 12983 - RNA, 3450 nt, Homo sapiens
  source 1..3450: mol_type = other RNA
gctgggattacaggcatgagccaccaagcccggcctattaactttcttctatatgctactcatttgtctagtaaagagtaaataataaactttttccttagaagaaatatatatcatttgtccaacagttacttaagtaggcagggattctattccattttacatatgacactagattttctgaatctcaatcttggactcattggtgttttgtagccaagagaattcctcaatggtatggattttctgttgaagatgaaggttggaagtctgagagaattctttttcagacacatcacattcacaaggtttttcatctgtgtggattttctgatgtacagtaaggttttttctttgcctaaaaactttactacaatcattacacccatagggtttctcccctgtgtgaattctctggtggccaactaaattcctcttagaagtaaaggatttcctacacttgtcacactcataaggtttttccccagtgtgcattctctgatgtacaacaaggtttttattctgactaaagtcttttccacactcattacatttataaggtttctctccagtatggattctttgatgtaccataagatttctactagaggtaaggactttcctacatacatgacattcgtaggttttttctccactgtgaattctttgatgttcaatcaggtttctgttgtacgtaaaaccttttccacactcactacacgcatagggcttctcaccagtatggatcctctgatgggctataaggtttgagcggtaactgaagaccttcccacagtcattgcatttataagatttttccctcgtgtgaattctctgatgtccaatgaggcttttcttcagaatgaagcatttgccacactcatcacactcatagggtttctcaccactgtggattctcttatgctcaatgaggtttctgtttgaactgaaagctcttccacactcactgcattcaaagggtttttctccggtgtggattctccgatgtacaagcaggcttgaattgtaactgaaagccttcccacaatcctcacatttgtaggctttctcttgtgtatggagtttctgatggaccataaaacttttgctcataataaaggttttcccacactctcgacattcatatggcttctccccattgtggagtctctcatggtcaatgaggtttctgtttgaaccgaagaccttaccacaatctttacattcatagagattctctccagtgtggaacctttgatgtaaaatgaggctcttcttcagaataaaaactttcccacattcattacattcatagggcttctccccattgtggagtctctggtggtcaaaaaggtaagcactttgagtaaaggctttcccacattcagtgcatttgtaaggtttctctctgctgtgcatcctcttatggtcaatgaagtttgacttagaactgaaaatcttcccacactttttacaaccaaaggttttcttttctgtgtggactctctgatgtaagaggaggcttttgcttcgaatgaaaacttttccacattctttacacttgtaagggttctctgcactgtggagtcgctgatggtcaataagataagtggtctgagcaaaggtctttccacattcatcacatttatagggtttttccccagagtggattctctggtgcagaatgaggctcttcttcagaatgaaagctttctgacacttattacatttataaggttcttcccctttgtggagcctctgatggtcaatgaggtaagcattctgagagaagactttcccacattcattacacttataaggtctctcccctgaatggcgccttagatgtataattaggcctgagtgcctatagaagccctttccacactccttacacttataaggtttctccccagtgtggatcctctgatggtttagaaggtaagcactttgagaaaatgctttcccacattcattacatttataaggtttctcccctgaatggttccgtaaatgcattagaaggctcgaacgctgaataaagccttttccacattccttacatttatgaggtttctcaccagtgtggattctccgatggtttataagatgggagattttattaaaatgtttacaacacatatcacatttataaaacttctttccttcagtacctattaaactttcagaaatagctgaaccgaaagtcaagctgtctcctaattccttccacttttggccttgtttctctggtggagtccttttcttcttgtctcgttcacaaagggaaactttcttcactgtatctgccctttcatctgtttcatttccccactgacttgccaaaacttgccattcacactcttcttcaaaatcaaggacctggggaacacttccttgaagtctttttgatgttcctttatgagagtctgctctttgagaactacttggctttgatgtcacctcctcattctcggtcatggtctcccattctagggaggtcacatttccataattctccagcatcacatcccagtacaaggccctctggattgggcccagacatgcccattcctctgaagtgaagcatactgacacctcctcgaacatcaccaactcctggggctgggctgttaggagcataagtgccattaattgatttcttgggttctcttcctgggaaagggcagaagcttcaggggcaggagaatcatgctgaggatcctggaggttgaatgccactaggtcagtaggaggatgcgggcaaatttcagctgctatgtggctgccaggaagtacaggaggaagtgttgttcctggggcactcaccaccttctggagagtgtcctgatccttgacaaggactggaacttgtattgctggtccatcaaggtctttctgcagctcctctaccagggccacagcctcctcgccacttccagggtgatggagctgtacccaggtccgaatctccccaggcaggatgctcagaaactgctccagcaccagcagctccaggatctgtgccttggtgcgtgcttctggtctcagccaccggcgacagagttccctgagccggctcagggcttcctggggtccagatgtctcatggtaacgtaattgtctaaagtgtaggtgggaggtctcccaaacagaggagctacttccttggaagctggttccccatttccaggtatcatccttccccttcacaaggccctcttgtctcagagcattgtgggctacattttctcttgtcattgttgttttttgaaaaaggctcctctccagtccaggtctccttaatccttgacttcttccttacagcttggagagtatcatcgggggctcccgctgcggctccagccttgcgtaccgccgcctcggcgccaggccgctaggagatgacacaggaacgagcccttccggcagccgaggcacagaataatg

SEQ ID NO: 12984 - RNA, 3504 nt, Homo sapiens
  source 1..3504: mol_type = other RNA
gctgggattacaggcatgagccaccaagcccggcctattaactttcttctatatgctactcatttgtctagtaaagagtaaataataaactttttccttagaagaaatatatatcatttgtccaacagttacttaagtaggcagggattctattccattttacatatgacactagattttctgaatctcaatcttggactcattggtgttttgtagccaagagaattcctcaatggtatggattttctgttgaagatgaaggttggaagtctgagagaattctttttcagacacatcacattcacaaggtttttcatctgtgtggattttctgatgtacagtaaggttttttctttgcctaaaaactttactacaatcattacacccatagggtttctcccctgtgtgaattctctggtggccaactaaattcctcttagaagtaaaggatttcctacacttgtcacactcataaggtttttccccagtgtgcattctctgatgtacaacaaggtttttattctgactaaagtcttttccacactcattacatttataaggtttctctccagtatggattctttgatgtaccataagatttctactagaggtaaggactttcctacatacatgacattcgtaggttttttctccactgtgaattctttgatgttcaatcaggtttctgttgtacgtaaaaccttttccacactcactacacgcatagggcttctcaccagtatggatcctctgatgggctataaggtttgagcggtaactgaagaccttcccacagtcattgcatttataagatttttccctcgtgtgaattctctgatgtccaatgaggcttttcttcagaatgaagcatttgccacactcatcacactcatagggtttctcaccactgtggattctcttatgctcaatgaggtttctgtttgaactgaaagctcttccacactcactgcattcaaagggtttttctccggtgtggattctccgatgtacaagcaggcttgaattgtaactgaaagccttcccacaatcctcacatttgtaggctttctcttgtgtatggagtttctgatggaccataaaacttttgctcataataaaggttttcccacactctcgacattcatatggcttctccccattgtggagtctctcatggtcaatgaggtttctgtttgaaccgaagaccttaccacaatctttacattcatagagattctctccagtgtggaacctttgatgtaaaatgaggctcttcttcagaataaaaactttcccacattcattacattcatagggcttctccccattgtggagtctctggtggtcaaaaaggtaagcactttgagtaaaggctttcccacattcagtgcatttgtaaggtttctctctgctgtgcatcctcttatggtcaatgaagtttgacttagaactgaaaatcttcccacactttttacaaccaaaggttttcttttctgtgtggactctctgatgtaagaggaggcttttgcttcgaatgaaaacttttccacattctttacacttgtaagggttctctgcactgtggagtcgctgatggtcaataagataagtggtctgagcaaaggtctttccacattcatcacatttatagggtttttccccagagtggattctctggtgcagaatgaggctcttcttcagaatgaaagctttctgacacttattacatttataaggttcttcccctttgtggagcctctgatggtcaatgaggtaagcattctgagagaagactttcccacattcattacacttataaggtctctcccctgaatggcgccttagatgtataattaggcctgagtgcctatagaagccctttccacactccttacacttataaggtttctccccagtgtggatcctctgatggtttagaaggtaagcactttgagaaaatgctttcccacattcattacatttataaggtttctcccctgaatggttccgtaaatgcattagaaggctcgaacgctgaataaagccttttccacattccttacatttatgaggtttctcaccagtgtggattctccgatggtttataagatgggagattttattaaaatgtttacaacacatatcacatttataaaacttctttccttcagtacctattaaactttcagaaatagctgaaccgaaagtcaagctgtctcctaattccttccacttttggccttgtttctctggtggagtccttttcttcttgtctcgttcacaaagggaaactttcttcactgtatctgccctttcatctgtttcatttccccactgacttgccaaaacttgccattcacactcttcttcaaaatcaaggacctggggaacacttccttgaagtctttttgatgttcctttatgagagtctgctctttgagaactacttggctttgatgtcacctcctcattctcggtcatggtctcccattctagggaggtcacatttccataattctccagcatcacatcccagtacaaggccctctggattgggcccagacatgcccattcctctgaagtgaagcatactgacacctcctcgaacatcaccaactcctggggctgggctgttaggagcataagtgccattaattgatttcttgggttctcttcctgggaaagggcagaagcttcaggggcaggagaatcatgctgaggatcctggaggttgaatgccactaggtcagtaggaggatgcgggcaaatttcagctgctatgtggctgccaggaagtacaggaggaagtgttgttcctggggcactcaccaccttctggagagtgtcctgatccttgacaaggactggaacttgtattgctggtccatcaaggtctttctgcagctcctctaccagggccacagcctcctcgccacttccagggtgatggagctgtacccaggtccgaatctccccaggcaggatgctcagaaactgctccagcaccagcagctccaggatctgtgccttggtgcgtgcttctggtctcagccaccggcgacagagttccctgagccggctcagggcttcctggggtccagatgtctcatggtaacgtaattgtctaaagtgtaggtgggaggtctcccaaacagaggagctacttccttggaagctggttccccatttccaggtatcatccttccccttcacaaggccctcttgtctcagagcattgtgggctacattttctcttgtcattgttgttttttgaaaaaggctcctctccagtccaggtctccttaatccttgacttcttccttacagcttggagagtatcatctacaagacccatattcctgtgcacagcagcctcaatccaaaggatctgcacagcacagatcttgcctgatctcctccttgagttcagtgaagaagttcctaagagggtcttgagtcacgaaagcgccagacccacatcttgaacaaagcgcagaaggaact

SEQ ID NO: 12985 - RNA, 3459 nt, Homo sapiens
  source 1..3459: mol_type = other RNA
gctgggattacaggcatgagccaccaagcccggcctattaactttcttctatatgctactcatttgtctagtaaagagtaaataataaactttttccttagaagaaatatatatcatttgtccaacagttacttaagtaggcagggattctattccattttacatatgacactagattttctgaatctcaatcttggactcattggtgttttgtagccaagagaattcctcaatggtatggattttctgttgaagatgaaggttggaagtctgagagaattctttttcagacacatcacattcacaaggtttttcatctgtgtggattttctgatgtacagtaaggttttttctttgcctaaaaactttactacaatcattacacccatagggtttctcccctgtgtgaattctctggtggccaactaaattcctcttagaagtaaaggatttcctacacttgtcacactcataaggtttttccccagtgtgcattctctgatgtacaacaaggtttttattctgactaaagtcttttccacactcattacatttataaggtttctctccagtatggattctttgatgtaccataagatttctactagaggtaaggactttcctacatacatgacattcgtaggttttttctccactgtgaattctttgatgttcaatcaggtttctgttgtacgtaaaaccttttccacactcactacacgcatagggcttctcaccagtatggatcctctgatgggctataaggtttgagcggtaactgaagaccttcccacagtcattgcatttataagatttttccctcgtgtgaattctctgatgtccaatgaggcttttcttcagaatgaagcatttgccacactcatcacactcatagggtttctcaccactgtggattctcttatgctcaatgaggtttctgtttgaactgaaagctcttccacactcactgcattcaaagggtttttctccggtgtggattctccgatgtacaagcaggcttgaattgtaactgaaagccttcccacaatcctcacatttgtaggctttctcttgtgtatggagtttctgatggaccataaaacttttgctcataataaaggttttcccacactctcgacattcatatggcttctccccattgtggagtctctcatggtcaatgaggtttctgtttgaaccgaagaccttaccacaatctttacattcatagagattctctccagtgtggaacctttgatgtaaaatgaggctcttcttcagaataaaaactttcccacattcattacattcatagggcttctccccattgtggagtctctggtggtcaaaaaggtaagcactttgagtaaaggctttcccacattcagtgcatttgtaaggtttctctctgctgtgcatcctcttatggtcaatgaagtttgacttagaactgaaaatcttcccacactttttacaaccaaaggttttcttttctgtgtggactctctgatgtaagaggaggcttttgcttcgaatgaaaacttttccacattctttacacttgtaagggttctctgcactgtggagtcgctgatggtcaataagataagtggtctgagcaaaggtctttccacattcatcacatttatagggtttttccccagagtggattctctggtgcagaatgaggctcttcttcagaatgaaagctttctgacacttattacatttataaggttcttcccctttgtggagcctctgatggtcaatgaggtaagcattctgagagaagactttcccacattcattacacttataaggtctctcccctgaatggcgccttagatgtataattaggcctgagtgcctatagaagccctttccacactccttacacttataaggtttctccccagtgtggatcctctgatggtttagaaggtaagcactttgagaaaatgctttcccacattcattacatttataaggtttctcccctgaatggttccgtaaatgcattagaaggctcgaacgctgaataaagccttttccacattccttacatttatgaggtttctcaccagtgtggattctccgatggtttataagatgggagattttattaaaatgtttacaacacatatcacatttataaaacttctttccttcagtacctattaaactttcagaaatagctgaaccgaaagtcaagctgtctcctaattccttccacttttggccttgtttctctggtggagtccttttcttcttgtctcgttcacaaagggaaactttcttcactgtatctgccctttcatctgtttcatttccccactgacttgccaaaacttgccattcacactcttcttcaaaatcaaggacctggggaacacttccttgaagtctttttgatgttcctttatgagagtctgctctttgagaactacttggctttgatgtcacctcctcattctcggtcatggtctcccattctagggaggtcacatttccataattctccagcatcacatcccagtacaaggccctctggattgggcccagacatgcccattcctctgaagtgaagcatactgacacctcctcgaacatcaccaactcctggggctgggctgttaggagcataagtgccattaattgatttcttgggttctcttcctgggaaagggcagaagcttcaggggcaggagaatcatgctgaggatcctggaggttgaatgccactaggtcagtaggaggatgcgggcaaatttcagctgctatgtggctgccaggaagtacaggaggaagtgttgttcctggggcactcaccaccttctggagagtgtcctgatccttgacaaggactggaacttgtattgctggtccatcaaggtctttctgcagctcctctaccagggccacagcctcctcgccacttccagggtgatggagctgtacccaggtccgaatctccccaggcaggatgctcagaaactgctccagcaccagcagctccaggatctgtgccttggtgcgtgcttctggtctcagccaccggcgacagagttccctgagccggctcagggcttcctggggtccagatgtctcatggtaacgtaattgtctaaagtgtaggtgggaggtctcccaaacagaggagctacttccttggaagctggttccccatttccaggtatcatccttccccttcacaaggccctcttgtctcagagcattgtgggctacattttctcttgtcattgttgttttttgaaaaaggctcctctccagtccaggtctccttaatccttgacttcttccttacagcttggagagtatcatctacaagaccgggggctcccgctgcggctccagccttgcgtaccgccgcctcggcgccaggccgctaggagatgacacaggaacgagcccttccggcagccgaggcacagaataatg

SEQ ID NO: 12986 - RNA, 3077 nt, Homo sapiens
  source 1..3077: mol_type = other RNA
gctgggattacaggcatgagccaccaagcccggcctatttgtatttttaatagagaaagggtttcaccatgttgcctaggctggtcttgaactcctgacctcaggtgatttgcccacctcggcctcccaaagtactgggattacagacgtgagccaccgcgcctggccctgttactgtctttaaacagtcttgcttttttctttagctgattgtcaacagcctgtagatacttcacaattgaaagaaaattacagaacaccaatatattagagataattagtctaaggacaacacatcatttagacacattaactattttgtaactccaactctgaatacatttcatctgactttctcaagggagaaattaaagaacttggcacaagatgttaaaagtctaaactccttaaatttctcaagatacactgaatgttttaatgaactttctccatctaaagtttgcagttttaagacagaaggattcctttaaccagtgagttaaaaggttaagttttaagtgtgcaccatacccatacaccaagttggtaggtagagagacaattacctcatccttaggaaaataaggtctgatagtataaactttggaggtaggagtcagtggaggtggctgaaaaaagagatcatttgccccatcaattggcagcaaacgctaaccactgtacaaaagacttcaccatagacattatactcttgatatcccaaacataggagtacatgtcataaagaattgtcctgttggcacaattggagagccgagtgaacattcccatcactagtccacacatctcttcaaacttggctgctcgtgaccgccattcttcaattttttcagagtcttttcctttgcaattgacactgacaacactactatttgctcgaagccattgaaattcccgtaacatctgtgctcctttgggtccatgctcgtaaggaaggtagaatagatcagcaagtaactgcaaatcctccagggtcactggttccgcagtgtacaaaggcttttcatttggacctggcacaaactgctccttgtttgtctgttcatcagtttgcatgggggcaatgtcactaatacaatcttcttgcatggacatctctggggattttgattcagctatgctctctttatcagtgtccattggtttcaattcctctgccattttcgcttcaacaatttcactcagtatttgattgtcattcttgtggtccgtttcttcttgtttttccaccaccatgtccatgggttcttcatcaggctgtttcttttcttcttccttggtcagagtagtaggctcaccactcaaggctgctccctggctcataatgggctcctgataaactgttgttactacggttgtggcatttaaagagggtgctgcaactaaaggagtcccatcaactacacttgctttagctccactgtgtgcaacttgcctactgctgtattgatgaggcacaccaaactcttgcaaccattctgttaatgctagctttagagccatctgtggactatagagtacatcagtttcaatatcttcatcactgccttcattttctaattttatctggatggacacagtactatcttcactgtcagtcatcactacatcttttctcactccattcatgtttgatttgtaccaggtggcaagggtgtggatagcaacgtagttggcttcaaattcacaatttggattagtgaggactccttttaaccgtgggatgagttctgtggatcttcctttgtacgggcccagaaacagtctcttctgatcataatcattagcatgaatgttatcccagattactggagctctcttaataatcttagaaacctcttcgatggactctactggaatttctttagaaacaactttgggacctgtccaaagcacttcaattccaggtagaagcttttcacccacagtccttaaatatggagactgagacacatttggataacagaaagtgccacagtattctgtgggacagaagaggaaagtttctggctctcctaggtactgatagatttcatttgtgatggagacttgggcatgagcaaaagaactgaatacctctttgtctgctgcacacatattatggtctatatcatcaaaaagcaaagcaaatgatctgcacccaaactgagaaacctggtccaatttacgtttcaatgtggatacttccttggggttagaaaaagtgatatccaatccaggtgagatcgcatagatgaactctatctcatattctcgtgcagcagagatgagagtcataagttgctcagcttcctccactgaatacatctctcgccaaaacatcctatgtttgtagtcatcttttggggcatacaagtatgtatttaattcccatttctggagccttctaaagagttcttttctctgttccataacccaaggtcttccataaaatccttccaccacaccgcagaggaaccgccgagcccctcctgcagccccggccaccgccgctcccccagccccggcggggttgtcttctccgggtgccggagctgccggcggctccagcgatgcccccgcagaggcggcagggttggagctgagctcgctctcccgctcctccaacgtcgcttgactctccttctgcaccatcctcctgcccccggccgctgccacctctgcgggtcctcctcgacctctgtccgttggggcaccggcccggagccctggagagggcttcagctccaagtgtgcgcccctccggctccttcccctccccctctgcccttccccctccctctccgcagggacccgaatgcccggatgagaagggcggcggcaccggcgcgagccctttgtcagccgcagcctcggctttaagctggggcgccagaagcctaagcggagagcgaggctgtgacctctcgttccctggaagaagacggccaagggtcctgtcctcgttctctgcctctgctgccctcccgataatcttaggtcttccgctgtttcccctccaagccccgagctctccctctgctgctgcctccaccgcccgcttcctgtttatccgc

SEQ ID NO: 12987 - RNA, 3353 nt, Homo sapiens
  source 1..3353: mol_type = other RNA
gctgggattacaggcatgagccaccaagcccggcctttttttttttttttttttttttttaatgagacagagtctccctctgttgcctaggctggagtgcagtagcgcaatctaggctccccccgcaggttaaagtaattctcctgcctcagcctcctgagtagctgggattacaggtgtgtgccaacacgcccagctaatttttgtatttttagtagagacagggtttcaccatgttggtcaggctggtctcgatctcctgaccttgtgatctccccgcctcagcctcccaaagtgctgggattagaggcgtgggctaccacacccggccaagagggattttctttaagcaagctttcacagtagtggagttaaatgatgtgggctaaaaggtggaggcaaaaaagccaaaaagaaatgggaaaggacatggcaggatgggaaattccaacatgagctaatatgagtgtgagaacgatcatttgcaggagagtgaaaatctcccgcaaaggtagataaagagccactttgtgtgtccagtgagaaagtggactgtgagtaacctataagctgctcattggaaacaagagggccctcaacaacgttacaaaggagcagatcatccttctggtctcttgctcctggtgcttctgaatccacagcaaaccttggcaggaacatgcttccctttgccacccagaggtgctctgagaaaacactctaactcactaggaggtggagatatagacctttttctgaactgcttctcacatgcaggggaaaataaatcaaagagaaggcctaaaagaactggaacttggactaaattaaagaaaattaagaaaaaatgagaataggaaggaagtttttgcaaacaaggaaaaccactatttttttttctccccatccaagataactttcaatagtgtattactctcaatatgttggtggcaagcttggttggctccagacaaaaacttgtaatacccaaggagaaaaaatttacctaccgctgctgatggcattagtgaggtcagcccaagccagcaacctccttgcagacttcagccccactgtatattggttcagcctggatcatggcacctaatggtaccttctgggcacctgctcagaaccaggaattctgcacctctctctaagctcagccagtttattgaacaaataatctatatttatagagcagactccactgttgattaaacagctttaaaatattatagcaaacgagagcccattgttttaatgtgaatccaggcatttcactttgtttttttgaaaagagagtttaatcttcttccctaaataggatacttacagataagcatggcatgaaaccttaagcaccgtatttgaattttagaatgtggcaatctatataacagtaaatatatgactgtgattcttttctatcttctctaaacgccattcaattctctcctctctttaattgaatttgggaaacaaggtttgacaaagggatacaatatttaaagtctactagaagcacaaggaaaaaattctccaccaaagcacatcgacacgtttgtcctccccacccctttttaactgaagagccccaattttgatactagaggagttatggtctattgtgaacacacatcttagaagtagcctcacattttcttagagctcactttgtcattttcccccttttgatactctgccaaatttaacttcaagaatttatgatttaagacactgtgagagtacttaaatccaaagttcctggaaaaataggatgtaaaagaaaagttacaatgcaaaccaccccaatggactcttagtgagaagcaggtaaatcaatcattcactccctcatgtctgcaggcctaggaggggactctgaaaatagcatcgtatttggaagaagaggagtggagagacgtcaggagaagagaagagaaaaatgtatgttttctaggtctccagtggtctttcttctctttagatggtttaactgcaggtgagttgatctttctcttcctttggcgtgacggtgttgggatgtgctatgggtagaagtctctgggggctctcaagtctcttgtctcagttcttcttggatggtcatctccagagcccaggtccatggcttctgggtagctgggaaattcctgaggtaaagggaactcctctgctgaagagtgagtccggtgcccgaacaccttttcctgcagctcagtgatgtcattgcggatgtcagccagcataagtagcaggaagtcgaaagaaccagggggtcctggagaccctctgggcccaggcgctcctctctcccccttagaaccatctcttcctggtgcccctggtggacccacagggcccctccggccttgcttaatgtgggacagatcaggagatggtcccatgggtcccattgagccccgtgggccgggctgcccaggagggcctggcataccggggaagcctgggcttccctttggtcctggtgagccgggagggccctggcccccaggcaggccaggaggtcctggaaggtaggtgtttgaggccagcaccttgtcaccagtgatatacttgcccaggtcagctgcattgttggggagcagagcaatcttttgcttcagctgcagcacggtctgcttcatctggtagaactccttgcatgtggcacagcaagttccggctttcaccatgttctcagacttctcatggccagtgtcattgggatatttgtctcccctggtacatgtcttcccatcatcttcccggatgtagccttcccggcactcgcagcggtagctgcccaaggtattgatgcagatgtgggcacacagcgtcccattgctgctggcacactcatcaatatccagacagtatggcttctcccgcttccggtgtctctcccggtcatatcggtatcccggataacaagtacacagcactcggccaaagttgtccgtgcactgctgttcacagggagcctcggcacaaacgtcgtaatcttctgggatgcattgtccaagaacaaatttatatcctttgcagcactttttcctgtagcatgtggtgagctcgcctgaagacttcagacacgggtatttagtcgtcgcgattttgctctctgagcagatttctctgtcgccgtcctccggctcctctctgtaggtccacgtgtgtcccaacgccaggagcagcagcagcggacccaggctcctgcccagctggcccctggcagctcctccccggctcggaggcggcggcaccatcagggaagctcccggcttcttcccagcgccgagctccgtccggaccaagcgtcctgctcctccgcggccgccgccgccttc

SEQ ID NO: 12988 - RNA, 4000 nt, Homo sapiens
  source 1..4000: mol_type = other RNA
gctgggattacaggcatgagccaccaagcccggcctttttttttttttttttttttttttaatgagacagagtctccctctgttgcctaggctggagtgcagtagcgcaatctaggctccccccgcaggttaaagtaattctcctgcctcagcctcctgagtagctgggattacaggtgtgtgccaacacgcccagctaatttttgtatttttagtagagacagggtttcaccatgttggtcaggctggtctcgatctcctgaccttgtgatctccccgcctcagcctcccaaagtgctgggattagaggcgtgggctaccacacccggccaagagggattttctttaagcaagctttcacagtagtggagttaaatgatgtgggctaaaaggtggaggcaaaaaagccaaaaagaaatgggaaaggacatggcaggatgggaaattccaacatgagctaatatgagtgtgagaacgatcatttgcaggagagtgaaaatctcccgcaaaggtagataaagagccactttgtgtgtccagtgagaaagtggactgtgagtaacctataagctgctcattggaaacaagagggccctcaacaacgttacaaaggagcagatcatccttctggtctcttgctcctggtgcttctgaatccacagcaaaccttggcaggaacatgcttccctttgccacccagaggtgctctgagaaaacactctaactcactaggaggtggagatatagacctttttctgaactgcttctcacatgcaggggaaaataaatcaaagagaaggcctaaaagaactggaacttggactaaattaaagaaaattaagaaaaaatgagaataggaaggaagtttttgcaaacaaggaaaaccactatttttttttctccccatccaagataactttcaatagtgtattactctcaatatgttggtggcaagcttggttggctccagacaaaaacttgtaatacccaaggagaaaaaatttacctaccgctgctgatggcattagtgaggtcagcccaagccagcaacctccttgcagacttcagccccactgtatattggttcagcctggatcatggcacctaatggtaccttctgggcacctgctcagaaccaggaattctgcacctctctctaagctcagccagtttattgaacaaataatctatatttatagagcagactccactgttgattaaacagctttaaaatattatagcaaacgagagcccattgttttaatgtgaatccaggcatttcactttgtttttttgaaaagagagtttaatcttcttccctaaataggatacttacagataagcatggcatgaaaccttaagcaccgtatttgaattttagaatgtggcaatctatataacagtaaatatatgactgtgattcttttctatcttctctaaacgccattcaattctctcctctctttaattgaatttgggaaacaaggtttgacaaagggatacaatatttaaagtctactagaagcacaaggaaaaaattctccaccaaagcacatcgacacgtttgtcctccccacccctttttaactgaagagccccaattttgatactagaggagttatggtctattgtgaacacacatcttagaagtagcctcacattttcttagagctcactttgtcattttcccccttttgatactctgccaaatttaacttcaagaatttatgatttaagacactgtgagagtacttaaatccaaagttcctggaaaaataggatgtaaaagaaaagttacaatgcaaaccaccccaatggactcttagtgagaagcaggtaaatcaatcattcactccctcatgtctgcaggcctaggaggggactctgaaaatagcatcgtatttggaagaagaggagtggagagacgtcaggagaagagaagagaaaaatgtatgttttctaggtctccagtggtctttcttctctttagatggtttaactgcaggtgagttgatctttctcttcctttggcgtgacggtgttgggatgtgctatgggtagaagtctctgggggctctcaagtctcttgtctcagttcttcttggatggtcatctccagagcccaggtccatggcttctgggtagctgggaaattcctgaggtaaagggaactcctctgctgaagagtgagtccggtgcccgaacaccttttcctgcagctcagtgatgtcattgcggatgtcagccagcataagtagcaggaagtcgaaagaaccagggggtcctggagaccctctgggcccaggcgctcctctctcccccttagaaccatctcttcctggtgcccctggtggacccacagggcccctccggccttgcttaatgtgggacagatcaggagatggtcccatgggtcccattgagccccgtgggccgggctgcccaggagggcctggcataccggggaagcctgggcttccctttggtcctggtgagccgggagggccctggcccccaggcaggccaggaggtcctggaaggtaggtgtttgaggccagcaccttgtcaccagtgatatacttgcccaggtcagctgcattgttggggagcagagcaatcttttgcttcagctgcagcacggtctgcttcatctggtagaactccttgcatgtggcacagcaagttccggctttcaccatgttctcagacttctcatggccagtgtcattgggatatttgtctcccctggtacatgtcttcccatcatcttcccggatgtagccttcccggcactcgcagcggtagctgcccaaggtattgatgcagatgtgggcacacagcgtcccattgctgctggcacactcatcaatatccagacagtatggcttctcccgcttccggtgtctctcccggtcatatcggtatcccggataacaagtacacagcactcggccaaagttgtccgtgcactgctgttcacagggagcctcggcacaaacgtcgtaatcttctgggatgcattgtccaagaacaaatttatatcctttgcagcactttttcctgtagcatgtggtgagctcgcctgaagacttcagacacgggtatttagtcgtcgcgattttgctctctgagcagatttctctgtcgccgtcctccggctcctctctgtaggtccacgtgtgtcccaacgccaggagcagcagcagcggacccaggctcctgcccagctggcccctggcagctcctccccggctcggaggcggcggcaccatcagggaagctcccggcttcttcccagcgccgagctccgtccggaccaagcgtcctgctcctccgcggccgccgccgccttccctcttcccggcagggggcgccggagagcaggggcgtttgcaccacctgcggtgtccggctggcgcgagggccctgaggttcaagttgtctcgtcgggacgttcacgtccgattgacagacttgctggactcggcttggggctgcgccctcgcctcttccctctccctcctctgggagaagcgcgcagggtggggaaagcgggcggttgtttgcattttgcaccagggtctcacgaccgggaggaggaggagctgattctccaccggggagaagagggagggggaagagaggggttaataagcttccttcctgttgtccatgggtttctaaagcccagggtcaggccagtgttcgtctttcctccgtgaggacctaccctgagatttgcaactatcttagtcttcttttctcttagattatgtgaggaaggaggagttgaaaggctacaacgggcctctcaaattgttcaaacctgaaatagcgctatttatatagtgtaatcactcttccttaaaacctttagaagaaagttctctggttgtttcattggtcaataaaccatgcgctgtcttcttcataactcgagttcggaacaagtaaggaggtctttctgggagccttacatctccttgtcctgagcggcttt

SEQ ID NO: 12989 - RNA, 2767 nt, Homo sapiens
  source 1..2767: mol_type = other RNA
gctgggattacaggcatgagccaccaagcctggccaattttgataattttcatccacatcaaataagaataaatatagcttattggccgggcatagtggctgcgcatgcctgtagtcccagctactcaggaggctgaggcaggagaatttttaacctgggtggcggaggttgcagtgagccaagattgcaccactggactccagcctgggtgtgtctcaaaaaaaaaaaaaatgaagtaggccaaatgtggactaataatgagaatgtgtaataaatcacatattatgaataacctacttttgtccaaagaatttatgaaatttacatgaaatattcccgttagaataaaaggaaactgatagcagttgttgcatctgtggaaagtgagtggctacagaactggatgttaggggagaattaattttcacatttttggtaatttttgaatttttataatgtgtgcttttattaaacaaaaaatttagaagattttaaaaaataaatgtaatgtcaaaatatatacgccagatactctttaatcccactgttgggaatctgcacaatagaaacaaaagaaggtaaaattagagttctaggtgaacattagaaacaacttcaatgtctgtagtaggtaatggcccaaaatacggacatacattccattctagaaatattctgaaccttacaaagaatgggttacatctttacgtactgacctggaaaagtattcatgattattatgaaaaggacaagacgctgtcaaatgtctgtatgggggtaaaagctcctccaaacacatgcaaaaaatgctttctgtgtacaggttgtttgagcataaaggaagaagaaatacacatactggttatctcagagatttgagggaagggaggaaattgttttcattttatttcactgtttcagtgaaatatttcactggtttcagtgaaacatgtaattttagaaaatttattctcaataaaaaaatttattctcaataatggttaatacaataactcagaaacagcattaaaatgagaccaaaatttacactttagttatccactttctcacttaaaaacatttgattttcaaggattatttaaataaataaatactaatgaaactggtggcttaccaactttttccttaaataaaacaaagacaatgtatatttccatcaacaaatttcatgatgctagactaggatggggagggaggagaggaaacctgactggcttctcgccagtatgaagagtctgatgtaagttaagttgtaatctatgattaaacgccttcccgcattgataaggtttctttccagaatgaattctctgatggtgtgagaagcttgaatgatagctaaaggccttcccacattccttacattcatagggtttctcaccagtatgaattctttgatgttgaataaggtgtgaatgaagtctaaaggccttaccacatatcatgcattcatgaggtttctcaccagtatgaattctctgatgtcttttgaggtgtgaacactgtctaaaagtcttcccacattccttacactcatagggtttctcaccagtatgaatcctctgatgtagggttagttgtaagccatcacaaaaagccttcccacattcatgacattcataaggtttcttgccagaatgaattttctgatggtgtgagaagcttgagtgatagctaaaggccttcccacattcccgacattcatagggtttctcaccagtatgaattctctgatgtatagtaagatgtgagcgatgcctaaaagtctttccacattctttacattcataaggtttctctccagtatggagtcgcaggtgttcagtaagttgaaagccacgaataaaagccttcccacattgcttacattcatagggtttttcaccagtatgaagtctctgatgttgagtaagctgtgatcgctgtctaaaggccttcccacattctttacattcataaggtttctcaccagtgtgaattctttgatgtagagtaagttctgagccataattaaaggccttcccacattcgttacattcatagcgtttttcaccattatgaattcttagatgtttaagttgtgagcaatgaacaaaggccttccaacattctttacactcattgcatttgtcaccattttgaattgtctgttgtttaaaaaggcatggtgtattaacaatttctgtgcattctttacattcagaaagttctttagaatgagttcttttgtggtgactaaaaaataaatggtaactgaagatttttctacactttttacattcagagattttctctctatcataaaattcttgagtgagtaaagtatgttggctaaaaatgggcatgttttcatggttaatcataagttgtctaaaataaccctcctcttgtccctgatgttgctcaaaatgacagttgccttcccagatagcgctgaaaattgatctctcaggactatggcttttaaattcttccatgttaacccactgggataattctgtttcataaatatccctttttggagataacttctggggctcatctctggatgccaagtcactggacaggagagattctgagagactactagaagtgtgataacgtcacattctgaaatctaacagaatgcgtgattatgtatttctgtgtgttctagaagtttctagagtagtaggtttggggaataaacatgtactttcagaaattagctgactttgttaccagtacttctactgtactcttaaa

SEQ ID NO: 12990 - RNA, 3108 nt, Homo sapiens
  source 1..3108: mol_type = other RNA
gctgggattacaggcatgagccaccaagcctggccaattttgataattttcatccacatcaaataagaataaatatagcttattggccgggcatagtggctgcgcatgcctgtagtcccagctactcaggaggctgaggcaggagaatttttaacctgggtggcggaggttgcagtgagccaagattgcaccactggactccagcctgggtgtgtctcaaaaaaaaaaaaaatgaagtaggccaaatgtggactaataatgagaatgtgtaataaatcacatattatgaataacctacttttgtccaaagaatttatgaaatttacatgaaatattcccgttagaataaaaggaaactgatagcagttgttgcatctgtggaaagtgagtggctacagaactggatgttaggggagaattaattttcacatttttggtaatttttgaatttttataatgtgtgcttttattaaacaaaaaatttagaagattttaaaaaataaatgtaatgtcaaaatatatacgccagatactctttaatcccactgttgggaatctgcacaatagaaacaaaagaaggtaaaattagagttctaggtgaacattagaaacaacttcaatgtctgtagtaggtaatggcccaaaatacggacatacattccattctagaaatattctgaaccttacaaagaatgggttacatctttacgtactgacctggaaaagtattcatgattattatgaaaaggacaagacgctgtcaaatgtctgtatgggggtaaaagctcctccaaacacatgcaaaaaatgctttctgtgtacaggttgtttgagcataaaggaagaagaaatacacatactggttatctcagagatttgagggaagggaggaaattgttttcattttatttcactgtttcagtgaaatatttcactggtttcagtgaaacatgtaattttagaaaatttattctcaataaaaaaatttattctcaataatggttaatacaataactcagaaacagcattaaaatgagaccaaaatttacactttagttatccactttctcacttaaaaacatttgattttcaaggattatttaaataaataaatactaatgaaactggtggcttaccaactttttccttaaataaaacaaagacaatgtatatttccatcaacaaatttcatgatgctagactaggatggggagggaggagaggaaacctgactggcttctcgccagtatgaagagtctgatgtaagttaagttgtaatctatgattaaacgccttcccgcattgataaggtttctttccagaatgaattctctgatggtgtgagaagcttgaatgatagctaaaggccttcccacattccttacattcatagggtttctcaccagtatgaattctttgatgttgaataaggtgtgaatgaagtctaaaggccttaccacatatcatgcattcatgaggtttctcaccagtatgaattctctgatgtcttttgaggtgtgaacactgtctaaaagtcttcccacattccttacactcatagggtttctcaccagtatgaatcctctgatgtagggttagttgtaagccatcacaaaaagccttcccacattcatgacattcataaggtttcttgccagaatgaattttctgatggtgtgagaagcttgagtgatagctaaaggccttcccacattcccgacattcatagggtttctcaccagtatgaattctctgatgtatagtaagatgtgagcgatgcctaaaagtctttccacattctttacattcataaggtttctctccagtatggagtcgcaggtgttcagtaagttgaaagccacgaataaaagccttcccacattgcttacattcatagggtttttcaccagtatgaagtctctgatgttgagtaagctgtgatcgctgtctaaaggccttcccacattctttacattcataaggtttctcaccagtgtgaattctttgatgtagagtaagttctgagccataattaaaggccttcccacattcgttacattcatagcgtttttcaccattatgaattcttagatgtttaagttgtgagcaatgaacaaaggccttccaacattctttacactcattgcatttgtcaccattttgaattgtctgttgtttaaaaaggcatggtgtattaacaatttctgtgcattctttacattcagaaagttctttagaatgagttcttttgtggtgactaaaaaataaatggtaactgaagatttttctacactttttacattcagagattttctctctatcataaaattcttgagtgagtaaagtatgttggctaaaaatgggcatgttttcatggttaatcataagttgtctaaaataaccctcctcttgtccctgatgttgctcaaaatgacagttgccttcccagatagcgctgaaaattgatctctcaggactatggcttttaaattcttccatgttaacccactgggataattctgtttcataaatatccctttttggagataacttctggggctcatctctggatgccaagtctgcatttatgtctgtagcctcattattgtccaagaaattattgtgaaatccccaagttttccatgtacctgggcaccatcttcctgtctcttccctcacaaccatccagggctccttcccttgctccaatgaggagattacggctggcttagaaacagaaagtccaagtgacaccaagttgctataattctccaacatcacctccttgtacaaattcctctgcgctgggttcaggcattcccattcctcctgagagacatctatagccacatctctgaacatcaccaactcatgggccatgtcttattttagaattgaatgtattatttaatcctcttcttcgttccctctggaagaaactcaatccaaagaaggtgttgcttcagcattctcagggaaggctctggtccaagctctgattcggattccaagcgaagccacacgcccagctcttccttctccaccggcccgggacatccttacctgcctctacccggagaccattcctgcgaggctcctaccggaagt

SEQ ID NO: 12991 - RNA, 3129 nt, Homo sapiens
  source 1..3129: mol_type = other RNA
gctgggattacaggcatgagccaccaagcctggccaattttgataattttcatccacatcaaataagaataaatatagcttattggccgggcatagtggctgcgcatgcctgtagtcccagctactcaggaggctgaggcaggagaatttttaacctgggtggcggaggttgcagtgagccaagattgcaccactggactccagcctgggtgtgtctcaaaaaaaaaaaaaatgaagtaggccaaatgtggactaataatgagaatgtgtaataaatcacatattatgaataacctacttttgtccaaagaatttatgaaatttacatgaaatattcccgttagaataaaaggaaactgatagcagttgttgcatctgtggaaagtgagtggctacagaactggatgttaggggagaattaattttcacatttttggtaatttttgaatttttataatgtgtgcttttattaaacaaaaaatttagaagattttaaaaaataaatgtaatgtcaaaatatatacgccagatactctttaatcccactgttgggaatctgcacaatagaaacaaaagaaggtaaaattagagttctaggtgaacattagaaacaacttcaatgtctgtagtaggtaatggcccaaaatacggacatacattccattctagaaatattctgaaccttacaaagaatgggttacatctttacgtactgacctggaaaagtattcatgattattatgaaaaggacaagacgctgtcaaatgtctgtatgggggtaaaagctcctccaaacacatgcaaaaaatgctttctgtgtacaggttgtttgagcataaaggaagaagaaatacacatactggttatctcagagatttgagggaagggaggaaattgttttcattttatttcactgtttcagtgaaatatttcactggtttcagtgaaacatgtaattttagaaaatttattctcaataaaaaaatttattctcaataatggttaatacaataactcagaaacagcattaaaatgagaccaaaatttacactttagttatccactttctcacttaaaaacatttgattttcaaggattatttaaataaataaatactaatgaaactggtggcttaccaactttttccttaaataaaacaaagacaatgtatatttccatcaacaaatttcatgatgctagactaggatggggagggaggagaggaaacctgactggcttctcgccagtatgaagagtctgatgtaagttaagttgtaatctatgattaaacgccttcccgcattgataaggtttctttccagaatgaattctctgatggtgtgagaagcttgaatgatagctaaaggccttcccacattccttacattcatagggtttctcaccagtatgaattctttgatgttgaataaggtgtgaatgaagtctaaaggccttaccacatatcatgcattcatgaggtttctcaccagtatgaattctctgatgtcttttgaggtgtgaacactgtctaaaagtcttcccacattccttacactcatagggtttctcaccagtatgaatcctctgatgtagggttagttgtaagccatcacaaaaagccttcccacattcatgacattcataaggtttcttgccagaatgaattttctgatggtgtgagaagcttgagtgatagctaaaggccttcccacattcccgacattcatagggtttctcaccagtatgaattctctgatgtatagtaagatgtgagcgatgcctaaaagtctttccacattctttacattcataaggtttctctccagtatggagtcgcaggtgttcagtaagttgaaagccacgaataaaagccttcccacattgcttacattcatagggtttttcaccagtatgaagtctctgatgttgagtaagctgtgatcgctgtctaaaggccttcccacattctttacattcataaggtttctcaccagtgtgaattctttgatgtagagtaagttctgagccataattaaaggccttcccacattcgttacattcatagcgtttttcaccattatgaattcttagatgtttaagttgtgagcaatgaacaaaggccttccaacattctttacactcattgcatttgtcaccattttgaattgtctgttgtttaaaaaggcatggtgtattaacaatttctgtgcattctttacattcagaaagttctttagaatgagttcttttgtggtgactaaaaaataaatggtaactgaagatttttctacactttttacattcagagattttctctctatcataaaattcttgagtgagtaaagtatgttggctaaaaatgggcatgttttcatggttaatcataagttgtctaaaataaccctcctcttgtccctgatgttgctcaaaatgacagttgccttcccagatagcgctgaaaattgatctctcaggactatggcttttaaattcttccatgttaacccactgggataattctgtttcataaatatccctttttggagataacttctggggctcatctctggatgccaagtctgcatttatgtctgtagcctcattattgtccaagaaattattgtgaaatccccaagttttccatgtacctgggcaccatcttcctgtctcttccctcacaaccatccagggctccttcccttgctccaatgaggagattacggctggcttagaaacagaaagtccaagtgacaccaagttgctataattctccaacatcacctccttgtacaaattcctctgcgctgggttcaggcattcccattcctcctgagagacatctatagccacatctctgaacatcaccaactcctaaaatgacaaataatagtaatgggccatgtcttattttagaattgaatgtattatttaatcctcttcttcgttccctctggaagaaactcaatccaaagaaggtgttgcttcagcattctcagggaaggctctggtccaagctctgattcggattccaagcgaagccacacgcccagctcttccttctccaccggcccgggacatccttacctgcctctacccggagaccattcctgcgaggctcctaccggaagt

SEQ ID NO: 12992 - RNA, 3071 nt, Homo sapiens
  source 1..3071: mol_type = other RNA
gctgggattacaggcatgagccaccaagcctggccaattttgataattttcatccacatcaaataagaataaatatagcttattggccgggcatagtggctgcgcatgcctgtagtcccagctactcaggaggctgaggcaggagaatttttaacctgggtggcggaggttgcagtgagccaagattgcaccactggactccagcctgggtgtgtctcaaaaaaaaaaaaaatgaagtaggccaaatgtggactaataatgagaatgtgtaataaatcacatattatgaataacctacttttgtccaaagaatttatgaaatttacatgaaatattcccgttagaataaaaggaaactgatagcagttgttgcatctgtggaaagtgagtggctacagaactggatgttaggggagaattaattttcacatttttggtaatttttgaatttttataatgtgtgcttttattaaacaaaaaatttagaagattttaaaaaataaatgtaatgtcaaaatatatacgccagatactctttaatcccactgttgggaatctgcacaatagaaacaaaagaaggtaaaattagagttctaggtgaacattagaaacaacttcaatgtctgtagtaggtaatggcccaaaatacggacatacattccattctagaaatattctgaaccttacaaagaatgggttacatctttacgtactgacctggaaaagtattcatgattattatgaaaaggacaagacgctgtcaaatgtctgtatgggggtaaaagctcctccaaacacatgcaaaaaatgctttctgtgtacaggttgtttgagcataaaggaagaagaaatacacatactggttatctcagagatttgagggaagggaggaaattgttttcattttatttcactgtttcagtgaaatatttcactggtttcagtgaaacatgtaattttagaaaatttattctcaataaaaaaatttattctcaataatggttaatacaataactcagaaacagcattaaaatgagaccaaaatttacactttagttatccactttctcacttaaaaacatttgattttcaaggattatttaaataaataaatactaatgaaactggtggcttaccaactttttccttaaataaaacaaagacaatgtatatttccatcaacaaatttcatgatgctagactaggatggggagggaggagaggaaacctgactggcttctcgccagtatgaagagtctgatgtaagttaagttgtaatctatgattaaacgccttcccgcattgataaggtttctttccagaatgaattctctgatggtgtgagaagcttgaatgatagctaaaggccttcccacattccttacattcatagggtttctcaccagtatgaattctttgatgttgaataaggtgtgaatgaagtctaaaggccttaccacatatcatgcattcatgaggtttctcaccagtatgaattctctgatgtcttttgaggtgtgaacactgtctaaaagtcttcccacattccttacactcatagggtttctcaccagtatgaatcctctgatgtagggttagttgtaagccatcacaaaaagccttcccacattcatgacattcataaggtttcttgccagaatgaattttctgatggtgtgagaagcttgagtgatagctaaaggccttcccacattcccgacattcatagggtttctcaccagtatgaattctctgatgtatagtaagatgtgagcgatgcctaaaagtctttccacattctttacattcataaggtttctctccagtatggagtcgcaggtgttcagtaagttgaaagccacgaataaaagccttcccacattgcttacattcatagggtttttcaccagtatgaagtctctgatgttgagtaagctgtgatcgctgtctaaaggccttcccacattctttacattcataaggtttctcaccagtgtgaattctttgatgtagagtaagttctgagccataattaaaggccttcccacattcgttacattcatagcgtttttcaccattatgaattcttagatgtttaagttgtgagcaatgaacaaaggccttccaacattctttacactcattgcatttgtcaccattttgaattgtctgttgtttaaaaaggcatggtgtattaacaatttctgtgcattctttacattcagaaagttctttagaatgagttcttttgtggtgactaaaaaataaatggtaactgaagatttttctacactttttacattcagagattttctctctatcataaaattcttgagtgagtaaagtatgttggctaaaaatgggcatgttttcatggttaatcataagttgtctaaaataaccctcctcttgtccctgatgttgctcaaaatgacagttgccttcccagatagcgctgaaaattgatctctcaggactatggcttttaaattcttccatgttaacccactgggataattctgtttcataaatatccctttttggagataacttctggggctcatctctggatgccaagtctgcatttatgtctgtagcctcattattgtccaagaaattattgtgaaatccccaagttttccatgtacctgggcaccatcttcctgtctcttccctcacaaccatccagggctccttcccttgctccaatgaggagattacggctggcttagaaacagaaagtcctccttgtacaaattcctctgcgctgggttcaggcattcccattcctcctgagagacatctatagccacatctctgaacatcaccaactcatgggccatgtcttattttagaattgaatgtattatttaatcctcttcttcgttccctctggaagaaactcaatccaaagaaggtgttgcttcagcattctcagggaaggctctggtccaagctctgattcggattccaagcgaagccacacgcccagctcttccttctccaccggcccgggacatccttacctgcctctacccggagaccattcctgcgaggctcctaccggaagt

SEQ ID NO: 12993 - RNA, 3092 nt, Homo sapiens
  source 1..3092: mol_type = other RNA
gctgggattacaggcatgagccaccaagcctggccaattttgataattttcatccacatcaaataagaataaatatagcttattggccgggcatagtggctgcgcatgcctgtagtcccagctactcaggaggctgaggcaggagaatttttaacctgggtggcggaggttgcagtgagccaagattgcaccactggactccagcctgggtgtgtctcaaaaaaaaaaaaaatgaagtaggccaaatgtggactaataatgagaatgtgtaataaatcacatattatgaataacctacttttgtccaaagaatttatgaaatttacatgaaatattcccgttagaataaaaggaaactgatagcagttgttgcatctgtggaaagtgagtggctacagaactggatgttaggggagaattaattttcacatttttggtaatttttgaatttttataatgtgtgcttttattaaacaaaaaatttagaagattttaaaaaataaatgtaatgtcaaaatatatacgccagatactctttaatcccactgttgggaatctgcacaatagaaacaaaagaaggtaaaattagagttctaggtgaacattagaaacaacttcaatgtctgtagtaggtaatggcccaaaatacggacatacattccattctagaaatattctgaaccttacaaagaatgggttacatctttacgtactgacctggaaaagtattcatgattattatgaaaaggacaagacgctgtcaaatgtctgtatgggggtaaaagctcctccaaacacatgcaaaaaatgctttctgtgtacaggttgtttgagcataaaggaagaagaaatacacatactggttatctcagagatttgagggaagggaggaaattgttttcattttatttcactgtttcagtgaaatatttcactggtttcagtgaaacatgtaattttagaaaatttattctcaataaaaaaatttattctcaataatggttaatacaataactcagaaacagcattaaaatgagaccaaaatttacactttagttatccactttctcacttaaaaacatttgattttcaaggattatttaaataaataaatactaatgaaactggtggcttaccaactttttccttaaataaaacaaagacaatgtatatttccatcaacaaatttcatgatgctagactaggatggggagggaggagaggaaacctgactggcttctcgccagtatgaagagtctgatgtaagttaagttgtaatctatgattaaacgccttcccgcattgataaggtttctttccagaatgaattctctgatggtgtgagaagcttgaatgatagctaaaggccttcccacattccttacattcatagggtttctcaccagtatgaattctttgatgttgaataaggtgtgaatgaagtctaaaggccttaccacatatcatgcattcatgaggtttctcaccagtatgaattctctgatgtcttttgaggtgtgaacactgtctaaaagtcttcccacattccttacactcatagggtttctcaccagtatgaatcctctgatgtagggttagttgtaagccatcacaaaaagccttcccacattcatgacattcataaggtttcttgccagaatgaattttctgatggtgtgagaagcttgagtgatagctaaaggccttcccacattcccgacattcatagggtttctcaccagtatgaattctctgatgtatagtaagatgtgagcgatgcctaaaagtctttccacattctttacattcataaggtttctctccagtatggagtcgcaggtgttcagtaagttgaaagccacgaataaaagccttcccacattgcttacattcatagggtttttcaccagtatgaagtctctgatgttgagtaagctgtgatcgctgtctaaaggccttcccacattctttacattcataaggtttctcaccagtgtgaattctttgatgtagagtaagttctgagccataattaaaggccttcccacattcgttacattcatagcgtttttcaccattatgaattcttagatgtttaagttgtgagcaatgaacaaaggccttccaacattctttacactcattgcatttgtcaccattttgaattgtctgttgtttaaaaaggcatggtgtattaacaatttctgtgcattctttacattcagaaagttctttagaatgagttcttttgtggtgactaaaaaataaatggtaactgaagatttttctacactttttacattcagagattttctctctatcataaaattcttgagtgagtaaagtatgttggctaaaaatgggcatgttttcatggttaatcataagttgtctaaaataaccctcctcttgtccctgatgttgctcaaaatgacagttgccttcccagatagcgctgaaaattgatctctcaggactatggcttttaaattcttccatgttaacccactgggataattctgtttcataaatatccctttttggagataacttctggggctcatctctggatgccaagtctgcatttatgtctgtagcctcattattgtccaagaaattattgtgaaatccccaagttttccatgtacctgggcaccatcttcctgtctcttccctcacaaccatccagggctccttcccttgctccaatgaggagattacggctggcttagaaacagaaagtcctccttgtacaaattcctctgcgctgggttcaggcattcccattcctcctgagagacatctatagccacatctctgaacatcaccaactcctaaaatgacaaataatagtaatgggccatgtcttattttagaattgaatgtattatttaatcctcttcttcgttccctctggaagaaactcaatccaaagaaggtgttgcttcagcattctcagggaaggctctggtccaagctctgattcggattccaagcgaagccacacgcccagctcttccttctccaccggcccgggacatccttacctgcctctacccggagaccattcctgcgaggctcctaccggaagt

SEQ ID NO: 12994 - RNA, 3362 nt, Homo sapiens
  source 1..3362: mol_type = other RNA
gctgggattacaggcatgagccaccaagcctggccaattttgataattttcatccacatcaaataagaataaatatagcttattggccgggcatagtggctgcgcatgcctgtagtcccagctactcaggaggctgaggcaggagaatttttaacctgggtggcggaggttgcagtgagccaagattgcaccactggactccagcctgggtgtgtctcaaaaaaaaaaaaaatgaagtaggccaaatgtggactaataatgagaatgtgtaataaatcacatattatgaataacctacttttgtccaaagaatttatgaaatttacatgaaatattcccgttagaataaaaggaaactgatagcagttgttgcatctgtggaaagtgagtggctacagaactggatgttaggggagaattaattttcacatttttggtaatttttgaatttttataatgtgtgcttttattaaacaaaaaatttagaagattttaaaaaataaatgtaatgtcaaaatatatacgccagatactctttaatcccactgttgggaatctgcacaatagaaacaaaagaaggtaaaattagagttctaggtgaacattagaaacaacttcaatgtctgtagtaggtaatggcccaaaatacggacatacattccattctagaaatattctgaaccttacaaagaatgggttacatctttacgtactgacctggaaaagtattcatgattattatgaaaaggacaagacgctgtcaaatgtctgtatgggggtaaaagctcctccaaacacatgcaaaaaatgctttctgtgtacaggttgtttgagcataaaggaagaagaaatacacatactggttatctcagagatttgagggaagggaggaaattgttttcattttatttcactgtttcagtgaaatatttcactggtttcagtgaaacatgtaattttagaaaatttattctcaataaaaaaatttattctcaataatggttaatacaataactcagaaacagcattaaaatgagaccaaaatttacactttagttatccactttctcacttaaaaacatttgattttcaaggattatttaaataaataaatactaatgaaactggtggcttaccaactttttccttaaataaaacaaagacaatgtatatttccatcaacaaatttcatgatgctagactaggatggggagggaggagaggaaacctgactggcttctcgccagtatgaagagtctgatgtaagttaagttgtaatctatgattaaacgccttcccgcattgataaggtttctttccagaatgaattctctgatggtgtgagaagcttgaatgatagctaaaggccttcccacattccttacattcatagggtttctcaccagtatgaattctttgatgttgaataaggtgtgaatgaagtctaaaggccttaccacatatcatgcattcatgaggtttctcaccagtatgaattctctgatgtcttttgaggtgtgaacactgtctaaaagtcttcccacattccttacactcatagggtttctcaccagtatgaatcctctgatgtagggttagttgtaagccatcacaaaaagccttcccacattcatgacattcataaggtttcttgccagaatgaattttctgatggtgtgagaagcttgagtgatagctaaaggccttcccacattcccgacattcatagggtttctcaccagtatgaattctctgatgtatagtaagatgtgagcgatgcctaaaagtctttccacattctttacattcataaggtttctctccagtatggagtcgcaggtgttcagtaagttgaaagccacgaataaaagccttcccacattgcttacattcatagggtttttcaccagtatgaagtctctgatgttgagtaagctgtgatcgctgtctaaaggccttcccacattctttacattcataaggtttctcaccagtgtgaattctttgatgtagagtaagttctgagccataattaaaggccttcccacattcgttacattcatagcgtttttcaccattatgaattcttagatgtttaagttgtgagcaatgaacaaaggccttccaacattctttacactcattgcatttgtcaccattttgaattgtctgttgtttaaaaaggcatggtgtattaacaatttctgtgcattctttacattcagaaagttctttagaatgagttcttttgtggtgactaaaaaataaatggtaactgaagatttttctacactttttacattcagagattttctctctatcataaaattcttgagtgagtaaagtatgttggctaaaaatgggcatgttttcatggttaatcataagttgtctaaaataaccctcctcttgtccctgatgttgctcaaaatgacagttgccttcccagatagcgctgaaaattgatctctcaggactatggcttttaaattcttccatgttaacccactgggataattctgtttcataaatatccctttttggagataacttctggggctcatctctggatgccaagtctgcatttatgtctgtagcctcattattgtccaagaaattattgtgaaatccccaagttttccatgtacctgtggtcccagctacttgggaggctgaggtgggaagattgcttgagcctgagaggtccaggctgcagtgagctgtgatcactccactgcactccagcatgggtaacagagtgagaccctgtctcaacaacaacaaaaaagatctgttgtataaccctgtgcccacactggacaatactgcattgtacacctaaaattccattaagagggtagatctcatgtaaagtatttacaacacaagaaaattttttaaagtgtttacatatttaataaatacttttttctatttcttagcatacagcaccaatgtaaataaatattaattatagcatccacagttaaatttctcaatatttgtttttgagaaacactgagtattttttgagaaacactttatttcccactttattgagggaaaattgacaattaaaatttatatatttaaaggatacaacctgatgatttgatatacatttacattgtgaaataatcaccacagtcagctaactaacctattcatcaccttacatagttaactgttttcttttttttgtggtaacaaaaaaacatgtaccttcagcacgtttcaaatatacaatacagtactgcaaactagagtcataatattctggagtctgaatgtggatattcagaatccactcatcttgcataactgaagctttattttatttatttttttgagatggagtctag

SEQ ID NO: 12995 - RNA, 3039 nt, Homo sapiens
  source 1..3039: mol_type = other RNA
gctgggattacaggcatgagccaccaagcctggccaattttgataattttcatccacatcaaataagaataaatatagcttattggccgggcatagtggctgcgcatgcctgtagtcccagctactcaggaggctgaggcaggagaatttttaacctgggtggcggaggttgcagtgagccaagattgcaccactggactccagcctgggtgtgtctcaaaaaaaaaaaaaatgaagtaggccaaatgtggactaataatgagaatgtgtaataaatcacatattatgaataacctacttttgtccaaagaatttatgaaatttacatgaaatattcccgttagaataaaaggaaactgatagcagttgttgcatctgtggaaagtgagtggctacagaactggatgttaggggagaattaattttcacatttttggtaatttttgaatttttataatgtgtgcttttattaaacaaaaaatttagaagattttaaaaaataaatgtaatgtcaaaatatatacgccagatactctttaatcccactgttgggaatctgcacaatagaaacaaaagaaggtaaaattagagttctaggtgaacattagaaacaacttcaatgtctgtagtaggtaatggcccaaaatacggacatacattccattctagaaatattctgaaccttacaaagaatgggttacatctttacgtactgacctggaaaagtattcatgattattatgaaaaggacaagacgctgtcaaatgtctgtatgggggtaaaagctcctccaaacacatgcaaaaaatgctttctgtgtacaggttgtttgagcataaaggaagaagaaatacacatactggttatctcagagatttgagggaagggaggaaattgttttcattttatttcactgtttcagtgaaatatttcactggtttcagtgaaacatgtaattttagaaaatttattctcaataaaaaaatttattctcaataatggttaatacaataactcagaaacagcattaaaatgagaccaaaatttacactttagttatccactttctcacttaaaaacatttgattttcaaggattatttaaataaataaatactaatgaaactggtggcttaccaactttttccttaaataaaacaaagacaatgtatatttccatcaacaaatttcatgatgctagactaggatggggagggaggagaggaaacctgactggcttctcgccagtatgaagagtctgatgtaagttaagttgtaatctatgattaaacgccttcccgcattgataaggtttctttccagaatgaattctctgatggtgtgagaagcttgaatgatagctaaaggccttcccacattccttacattcatagggtttctcaccagtatgaattctttgatgttgaataaggtgtgaatgaagtctaaaggccttaccacatatcatgcattcatgaggtttctcaccagtatgaattctctgatgtcttttgaggtgtgaacactgtctaaaagtcttcccacattccttacactcatagggtttctcaccagtatgaatcctctgatgtagggttagttgtaagccatcacaaaaagccttcccacattcatgacattcataaggtttcttgccagaatgaattttctgatggtgtgagaagcttgagtgatagctaaaggccttcccacattcccgacattcatagggtttctcaccagtatgaattctctgatgtatagtaagatgtgagcgatgcctaaaagtctttccacattctttacattcataaggtttctctccagtatggagtcgcaggtgttcagtaagttgaaagccacgaataaaagccttcccacattgcttacattcatagggtttttcaccagtatgaagtctctgatgttgagtaagctgtgatcgctgtctaaaggccttcccacattctttacattcataaggtttctcaccagtgtgaattctttgatgtagagtaagttctgagccataattaaaggccttcccacattcgttacattcatagcgtttttcaccattatgaattcttagatgtttaagttgtgagcaatgaacaaaggccttccaacattctttacactcattgcatttgtcaccattttgaattgtctgttgtttaaaaaggcatggtgtattaacaatttctgtgcattctttacattcagaaagttctttagaatgagttcttttgtggtgactaaaaaataaatggtaactgaagatttttctacactttttacattcagagattttctctctatcataaaattcttgagtgagtaaagtatgttggctaaaaatgggcatgttttcatggttaatcataagttgtctaaaataaccctcctcttgtccctgatgttgctcaaaatgacagttgccttcccagatagcgctgaaaattgatctctcaggactatggcttttaaattcttccatgttaacccactgggataattctgtttcataaatatccctttttggagataacttctggggctcatctctggatgccaagtctgggcaccatcttcctgtctcttccctcacaaccatccagggctccttcccttgctccaatgaggagattacggctggcttagaaacagaaagtccaagtgacaccaagttgctataattctccaacatcacctccttgtacaaattcctctgcgctgggttcaggcattcccattcctcctgagagacatctatagccacatctctgaacatcaccaactcatgggccatgtcttattttagaattgaatgtattatttaatcctcttcttcgttccctctggaagaaactcaatccaaagaaggtgttgcttcagcattctcagggaaggctctggtccaagctctgattcggattccaagcgaagccacacgcccagctcttccttctccaccggcccgggacatccttacctgcctctacccggagaccattcctgcgaggctcctaccggaagt

SEQ ID NO: 12996 - RNA, 3002 nt, Homo sapiens
  source 1..3002: mol_type = other RNA
gctgggattacaggcatgagccaccaagcctggccaattttgataattttcatccacatcaaataagaataaatatagcttattggccgggcatagtggctgcgcatgcctgtagtcccagctactcaggaggctgaggcaggagaatttttaacctgggtggcggaggttgcagtgagccaagattgcaccactggactccagcctgggtgtgtctcaaaaaaaaaaaaaatgaagtaggccaaatgtggactaataatgagaatgtgtaataaatcacatattatgaataacctacttttgtccaaagaatttatgaaatttacatgaaatattcccgttagaataaaaggaaactgatagcagttgttgcatctgtggaaagtgagtggctacagaactggatgttaggggagaattaattttcacatttttggtaatttttgaatttttataatgtgtgcttttattaaacaaaaaatttagaagattttaaaaaataaatgtaatgtcaaaatatatacgccagatactctttaatcccactgttgggaatctgcacaatagaaacaaaagaaggtaaaattagagttctaggtgaacattagaaacaacttcaatgtctgtagtaggtaatggcccaaaatacggacatacattccattctagaaatattctgaaccttacaaagaatgggttacatctttacgtactgacctggaaaagtattcatgattattatgaaaaggacaagacgctgtcaaatgtctgtatgggggtaaaagctcctccaaacacatgcaaaaaatgctttctgtgtacaggttgtttgagcataaaggaagaagaaatacacatactggttatctcagagatttgagggaagggaggaaattgttttcattttatttcactgtttcagtgaaatatttcactggtttcagtgaaacatgtaattttagaaaatttattctcaataaaaaaatttattctcaataatggttaatacaataactcagaaacagcattaaaatgagaccaaaatttacactttagttatccactttctcacttaaaaacatttgattttcaaggattatttaaataaataaatactaatgaaactggtggcttaccaactttttccttaaataaaacaaagacaatgtatatttccatcaacaaatttcatgatgctagactaggatggggagggaggagaggaaacctgactggcttctcgccagtatgaagagtctgatgtaagttaagttgtaatctatgattaaacgccttcccgcattgataaggtttctttccagaatgaattctctgatggtgtgagaagcttgaatgatagctaaaggccttcccacattccttacattcatagggtttctcaccagtatgaattctttgatgttgaataaggtgtgaatgaagtctaaaggccttaccacatatcatgcattcatgaggtttctcaccagtatgaattctctgatgtcttttgaggtgtgaacactgtctaaaagtcttcccacattccttacactcatagggtttctcaccagtatgaatcctctgatgtagggttagttgtaagccatcacaaaaagccttcccacattcatgacattcataaggtttcttgccagaatgaattttctgatggtgtgagaagcttgagtgatagctaaaggccttcccacattcccgacattcatagggtttctcaccagtatgaattctctgatgtatagtaagatgtgagcgatgcctaaaagtctttccacattctttacattcataaggtttctctccagtatggagtcgcaggtgttcagtaagttgaaagccacgaataaaagccttcccacattgcttacattcatagggtttttcaccagtatgaagtctctgatgttgagtaagctgtgatcgctgtctaaaggccttcccacattctttacattcataaggtttctcaccagtgtgaattctttgatgtagagtaagttctgagccataattaaaggccttcccacattcgttacattcatagcgtttttcaccattatgaattcttagatgtttaagttgtgagcaatgaacaaaggccttccaacattctttacactcattgcatttgtcaccattttgaattgtctgttgtttaaaaaggcatggtgtattaacaatttctgtgcattctttacattcagaaagttctttagaatgagttcttttgtggtgactaaaaaataaatggtaactgaagatttttctacactttttacattcagagattttctctctatcataaaattcttgagtgagtaaagtatgttggctaaaaatgggcatgttttcatggttaatcataagttgtctaaaataaccctcctcttgtccctgatgttgctcaaaatgacagttgccttcccagatagcgctgaaaattgatctctcaggactatggcttttaaattcttccatgttaacccactgggataattctgtttcataaatatccctttttggagataacttctggggctcatctctggatgccaagtctgggcaccatcttcctgtctcttccctcacaaccatccagggctccttcccttgctccaatgaggagattacggctggcttagaaacagaaagtcctccttgtacaaattcctctgcgctgggttcaggcattcccattcctcctgagagacatctatagccacatctctgaacatcaccaactcatgggccatgtcttattttagaattgaatgtattatttaatcctcttcttcgttccctctggaagaaactcaatccaaagaaggtgttgcttcagcattctcagggaaggctctggtccaagctctgattcggattccaagcgaagccacacgcccagctcttccttctccaccggcccgggacatccttacctgcctctacccggagaccattcctgcgaggctcctaccggaagt

SEQ ID NO: 12997 - RNA, 3023 nt, Homo sapiens
  source 1..3023: mol_type = other RNA
gctgggattacaggcatgagccaccaagcctggccaattttgataattttcatccacatcaaataagaataaatatagcttattggccgggcatagtggctgcgcatgcctgtagtcccagctactcaggaggctgaggcaggagaatttttaacctgggtggcggaggttgcagtgagccaagattgcaccactggactccagcctgggtgtgtctcaaaaaaaaaaaaaatgaagtaggccaaatgtggactaataatgagaatgtgtaataaatcacatattatgaataacctacttttgtccaaagaatttatgaaatttacatgaaatattcccgttagaataaaaggaaactgatagcagttgttgcatctgtggaaagtgagtggctacagaactggatgttaggggagaattaattttcacatttttggtaatttttgaatttttataatgtgtgcttttattaaacaaaaaatttagaagattttaaaaaataaatgtaatgtcaaaatatatacgccagatactctttaatcccactgttgggaatctgcacaatagaaacaaaagaaggtaaaattagagttctaggtgaacattagaaacaacttcaatgtctgtagtaggtaatggcccaaaatacggacatacattccattctagaaatattctgaaccttacaaagaatgggttacatctttacgtactgacctggaaaagtattcatgattattatgaaaaggacaagacgctgtcaaatgtctgtatgggggtaaaagctcctccaaacacatgcaaaaaatgctttctgtgtacaggttgtttgagcataaaggaagaagaaatacacatactggttatctcagagatttgagggaagggaggaaattgttttcattttatttcactgtttcagtgaaatatttcactggtttcagtgaaacatgtaattttagaaaatttattctcaataaaaaaatttattctcaataatggttaatacaataactcagaaacagcattaaaatgagaccaaaatttacactttagttatccactttctcacttaaaaacatttgattttcaaggattatttaaataaataaatactaatgaaactggtggcttaccaactttttccttaaataaaacaaagacaatgtatatttccatcaacaaatttcatgatgctagactaggatggggagggaggagaggaaacctgactggcttctcgccagtatgaagagtctgatgtaagttaagttgtaatctatgattaaacgccttcccgcattgataaggtttctttccagaatgaattctctgatggtgtgagaagcttgaatgatagctaaaggccttcccacattccttacattcatagggtttctcaccagtatgaattctttgatgttgaataaggtgtgaatgaagtctaaaggccttaccacatatcatgcattcatgaggtttctcaccagtatgaattctctgatgtcttttgaggtgtgaacactgtctaaaagtcttcccacattccttacactcatagggtttctcaccagtatgaatcctctgatgtagggttagttgtaagccatcacaaaaagccttcccacattcatgacattcataaggtttcttgccagaatgaattttctgatggtgtgagaagcttgagtgatagctaaaggccttcccacattcccgacattcatagggtttctcaccagtatgaattctctgatgtatagtaagatgtgagcgatgcctaaaagtctttccacattctttacattcataaggtttctctccagtatggagtcgcaggtgttcagtaagttgaaagccacgaataaaagccttcccacattgcttacattcatagggtttttcaccagtatgaagtctctgatgttgagtaagctgtgatcgctgtctaaaggccttcccacattctttacattcataaggtttctcaccagtgtgaattctttgatgtagagtaagttctgagccataattaaaggccttcccacattcgttacattcatagcgtttttcaccattatgaattcttagatgtttaagttgtgagcaatgaacaaaggccttccaacattctttacactcattgcatttgtcaccattttgaattgtctgttgtttaaaaaggcatggtgtattaacaatttctgtgcattctttacattcagaaagttctttagaatgagttcttttgtggtgactaaaaaataaatggtaactgaagatttttctacactttttacattcagagattttctctctatcataaaattcttgagtgagtaaagtatgttggctaaaaatgggcatgttttcatggttaatcataagttgtctaaaataaccctcctcttgtccctgatgttgctcaaaatgacagttgccttcccagatagcgctgaaaattgatctctcaggactatggcttttaaattcttccatgttaacccactgggataattctgtttcataaatatccctttttggagataacttctggggctcatctctggatgccaagtctgggcaccatcttcctgtctcttccctcacaaccatccagggctccttcccttgctccaatgaggagattacggctggcttagaaacagaaagtcctccttgtacaaattcctctgcgctgggttcaggcattcccattcctcctgagagacatctatagccacatctctgaacatcaccaactcctaaaatgacaaataatagtaatgggccatgtcttattttagaattgaatgtattatttaatcctcttcttcgttccctctggaagaaactcaatccaaagaaggtgttgcttcagcattctcagggaaggctctggtccaagctctgattcggattccaagcgaagccacacgcccagctcttccttctccaccggcccgggacatccttacctgcctctacccggagaccattcctgcgaggctcctaccggaagt

SEQ ID NO: 12998 - RNA, 3137 nt, Homo sapiens
  source 1..3137: mol_type = other RNA
gctgggattacaggcatgagccaccaagcctggccaattttgataattttcatccacatcaaataagaataaatatagcttattggccgggcatagtggctgcgcatgcctgtagtcccagctactcaggaggctgaggcaggagaatttttaacctgggtggcggaggttgcagtgagccaagattgcaccactggactccagcctgggtgtgtctcaaaaaaaaaaaaaatgaagtaggccaaatgtggactaataatgagaatgtgtaataaatcacatattatgaataacctacttttgtccaaagaatttatgaaatttacatgaaatattcccgttagaataaaaggaaactgatagcagttgttgcatctgtggaaagtgagtggctacagaactggatgttaggggagaattaattttcacatttttggtaatttttgaatttttataatgtgtgcttttattaaacaaaaaatttagaagattttaaaaaataaatgtaatgtcaaaatatatacgccagatactctttaatcccactgttgggaatctgcacaatagaaacaaaagaaggtaaaattagagttctaggtgaacattagaaacaacttcaatgtctgtagtaggtaatggcccaaaatacggacatacattccattctagaaatattctgaaccttacaaagaatgggttacatctttacgtactgacctggaaaagtattcatgattattatgaaaaggacaagacgctgtcaaatgtctgtatgggggtaaaagctcctccaaacacatgcaaaaaatgctttctgtgtacaggttgtttgagcataaaggaagaagaaatacacatactggttatctcagagatttgagggaagggaggaaattgttttcattttatttcactgtttcagtgaaatatttcactggtttcagtgaaacatgtaattttagaaaatttattctcaataaaaaaatttattctcaataatggttaatacaataactcagaaacagcattaaaatgagaccaaaatttacactttagttatccactttctcacttaaaaacatttgattttcaaggattatttaaataaataaatactaatgaaactggtggcttaccaactttttccttaaataaaacaaagacaatgtatatttccatcaacaaatttcatgatgctagactaggatggggagggaggagaggaaacctgactggcttctcgccagtatgaagagtctgatgtaagttaagttgtaatctatgattaaacgccttcccgcattgataaggtttctttccagaatgaattctctgatggtgtgagaagcttgaatgatagctaaaggccttcccacattccttacattcatagggtttctcaccagtatgaattctttgatgttgaataaggtgtgaatgaagtctaaaggccttaccacatatcatgcattcatgaggtttctcaccagtatgaattctctgatgtcttttgaggtgtgaacactgtctaaaagtcttcccacattccttacactcatagggtttctcaccagtatgaatcctctgatgtagggttagttgtaagccatcacaaaaagccttcccacattcatgacattcataaggtttcttgccagaatgaattttctgatggtgtgagaagcttgagtgatagctaaaggccttcccacattcccgacattcatagggtttctcaccagtatgaattctctgatgtatagtaagatgtgagcgatgcctaaaagtctttccacattctttacattcataaggtttctctccagtatggagtcgcaggtgttcagtaagttgaaagccacgaataaaagccttcccacattgcttacattcatagggtttttcaccagtatgaagtctctgatgttgagtaagctgtgatcgctgtctaaaggccttcccacattctttacattcataaggtttctcaccagtgtgaattctttgatgtagagtaagttctgagccataattaaaggccttcccacattcgttacattcatagcgtttttcaccattatgaattcttagatgtttaagttgtgagcaatgaacaaaggccttccaacattctttacactcattgcatttgtcaccattttgaattgtctgttgtttaaaaaggcatggtgtattaacaatttctgtgcattctttacattcagaaagttctttagaatgagttcttttgtggtgactaaaaaataaatggtaactgaagatttttctacactttttacattcagagattttctctctatcataaaattcttgagtgagtaaagtatgttggctaaaaatgggcatgttttcatggttaatcataagttgtctaaaataaccctcctcttgtccctgatgttgctcaaaatgacagttgccttcccagatagcgctgaaaattgatctctcaggactatggcttttaaattcttccatgttaacccactgggataattctgtttcataaatatccctttttggagataacttctggggctcatctctggatgccaagtctgggcaccatcttcctgtctcttccctcacaaccatccagggctccttcccttgctccaatgaggagattacggctggcttagaaacagaaagtcctgtaatcacagctactcgggaggctgaggcaggagaattgcttgaagctgggaggcagaggttgtggtgagccgagatcacgccattgcactctagccaagtgacaccaagttgctataattctccaacatcacctccttgtacaaattcctctgcgctgggttcaggcattcccattcctcctgagagacatctatagccacatctctgaacatcaccaactcatgggccatgtcttattttagaattgaatgtattatttaatcctcttcttcgttccctctggaagaaactcaatccaaagaaggtgttgcttcagcattctcagggaaggctctggtccaagctctgattcggattccaagcgaagccacacgcccagctcttccttctccaccggcccgggacatccttacctgcctctacccggagaccattcctgcgaggctcctaccggaagt

SEQ ID NO: 12999 - RNA, 3624 nt, Homo sapiens
  source 1..3624: mol_type = other RNA
gctgggattacaggcatgagccaccaagcctggccgggattccttttcaaagtctggctgcacctagagccagtttgcttctgcttggcctcatggggcctcagagaaagccacaaaggaggatgggtctttcctgggttcatttaactgccatttataacactttttcctctaaacagcttaatggacttcctactacttgtatagtttgattttcaggactctgttcagcaagaatacctactttacaaaactcagcataaaaatgaggtgaaacagtttaactaaaactggagtttggctgggtagtgtggctcacaactgatcccagcactttgggaggccgaggcaggaggattgcctgagaccaggaatttgaggccagcctgggcaacatagtaagacccccgtctctatcttaaaaaaaaaataaaagaataaaacaagttccttcacctcttgacaagacaaagctgacactttttttttttgagacagagaaaaaaagaaaactctacagccagaatcatacttttgagtctcgctctgtcgcccaggctggatggagtgcagtggcgtgatctcagctcactgtaacctccgcctcctgggttcaagtaattctctgccttggcttcacgagtagctgggattacaggtgctcgccaccacgcccggctaatttttgtatctttagtagagacagggtttcaccatcttggccaggctggtcttgagctcctgacctcgtgatccacccgccccgccctcccaaagtgctgggattacaggcgtgaaccactgcacctggccactttcttaaacctacacattggttgctgtgatattaattctatttttacaaaataagtgtataaccaggaagtactaatcctgctttctatgcccaattgttaacaggaaagggctcagtgcacttctcaattgtcacccctgcccccagccctgatccacggcctctaccccaagaatgagccaagaaccagctgctctagggatctcagcagcaaaatcctgcccaaggctgttaaaatgtgtgggcactcatttacactcgtgctgtcatgaaacacatccttgaacagggactattctctttcatttccataagcaaactggcgtctaaggccacaagccctccgtaaaaataagaactcggcacaaatggccagtcacatgcttacctgcatttttaaagacagctttcaggtatttggggactacattattaccaaaccttggctttgggagattatacaggtccgaggaactcgtgtctactgcagacgaatgcaattaccccaccttcctccatacagaattgttaggaaatgtccactcctttgggggtgatttttctcctcaagttgtagccaacattttgtccgtaactgatttcagggcaaacatttctgacatcttcctccagctcagtctgccatgccttggcaatccagtttcctgtcatatgcgagccatccaagttgatgccaagtaagatttgcccagctcaaagtgaaagtgtttgcgtcttggtatccggaatcctcagccccagtagcaaagctttagtcattcaccttcatccaatagacgtttgtgaacgtcctgctgtccattttgtcaataaacaggcagccctgcaggtggtccatctcgtgctggatgatgcgggctgcccacccgctcgcctgccacaccacctgttctccattggggtccagcccgcgttctggaggcaggggacgccggctagggccccacgctgggcggttcggcctgcgtctccgctcgccctccctccgggcaggctgggcccgcgggctccaggcgtggctcctcggcgggaggctctggtgctggagctgtgagctcgggccccagcgcctggtcatccagggtgaaaagcgtctctctctttggcaggataaaggcgaggggctcctgaatggcgccgatgttcacatgccctaggttaccgtacttggagagctgagtgggaggaatgcctaaagtctgtgctatctgagctggtggaaaaaggacttggagacagcgatttaaatacggaacaaggtcttccaggaagacagtgcagaactggacaaagagctcttgctccccgctgctgaaggcagcctcttcagcgcgatggaaggccaggattattttagttaccttggcaagggcatcttccaaggccccagtcacatcctgcgccagggccacagggcagcagaggcgcagatcattgaaggcaaccagaatattgttgagaaagcaggcgaggggtgggaaatctaggagcaccatgggtggctgcagcgtccccggctgggtggctggcacagcagcaggcatgttactggtgcccaggatggctggagccgagatgagcatgtaggagttcatttcttcctggaatttctccactgtttcctgaattgctttctggaaagtgctgatggccacccgctggaaaacaggagccaactgaccccggaaatcagctcccacccggctgaaggacagcccaaagtacatgcactggcccagcagagagtccaggtggccgcctatgccccggtaaaggtcggtctccagcacctgcaggaattgtgagaccttctgtagcacccagccatggaagatggcactctcattcacagtgtgctcacccatggcagggggcagcagtgggtcctcgtctgagaagatggcacggtactgggtgatgatatcaaagagatggacacgggaggcctcgatggtttttgtaatatggaaatagggatcatcattaggaatggcagtcaggatggaccggagccaagcatctcgggcctgaagaaacttcaccctcaactcagcctcagtgaagacgtccatgcgccgcaggtagccaatgacacggaggcaggcaggaagctggatgttggtcctcagttgctggatcagctggctcagcatcagctgcatggactggcgcacttcgttcacgatgccctggatgacagggatggaagagtatttcctctccagtcggcgtacgtaggctgcaagctccagggcctcttcataataactgttccggacacaggtgtccatgagctgaggaatctccagtatttccaaaatttctgtgtgccggtttagggtcaggctattcatccggcggttggagctgatctcctcggcttccttcacaaagttcctgcagctctgctggaagctgggcaaacggtcgagcaggcggccgagcgacgcctccacgtcgccaaacaggcggtggatgcgctcggtgcactcggcgccgcggatgaaggtcttgtagttagcgaaggccaagtcgcgcgtctgctgcagcagctgcgcccgctcctccgccaggcgctcgggctcgcgccgcagccgctccagccccgagccgctcaactcccggaggtagcggcccacatcgggccgctcgcgccactgggcctcggggaagcggtcccggaacagcgacgccaggagcccttcatcctccacctcgccgagagccgctgctgtggccgtggctaccgatgggatagtcgccgcggtcgccatcttcccagcaac

SEQ ID NO: 13000 - RNA, 3663 nt, Homo sapiens
  source 1..3663: mol_type = other RNA
gctgggattacaggcatgagccaccaagcctggccgggattccttttcaaagtctggctgcacctagagccagtttgcttctgcttggcctcatggggcctcagagaaagccacaaaggaggatgggtctttcctgggttcatttaactgccatttataacactttttcctctaaacagcttaatggacttcctactacttgtatagtttgattttcaggactctgttcagcaagaatacctactttacaaaactcagcataaaaatgaggtgaaacagtttaactaaaactggagtttggctgggtagtgtggctcacaactgatcccagcactttgggaggccgaggcaggaggattgcctgagaccaggaatttgaggccagcctgggcaacatagtaagacccccgtctctatcttaaaaaaaaaataaaagaataaaacaagttccttcacctcttgacaagacaaagctgacactttttttttttgagacagagaaaaaaagaaaactctacagccagaatcatacttttgagtctcgctctgtcgcccaggctggatggagtgcagtggcgtgatctcagctcactgtaacctccgcctcctgggttcaagtaattctctgccttggcttcacgagtagctgggattacaggtgctcgccaccacgcccggctaatttttgtatctttagtagagacagggtttcaccatcttggccaggctggtcttgagctcctgacctcgtgatccacccgccccgccctcccaaagtgctgggattacaggcgtgaaccactgcacctggccactttcttaaacctacacattggttgctgtgatattaattctatttttacaaaataagtgtataaccaggaagtactaatcctgctttctatgcccaattgttaacaggaaagggctcagtgcacttctcaattgtcacccctgcccccagccctgatccacggcctctaccccaagaatgagccaagaaccagctgctctagggatctcagcagcaaaatcctgcccaaggctgttaaaatgtgtgggcactcatttacactcgtgctgtcatgaaacacatccttgaacagggactattctctttcatttccataagcaaactggcgtctaaggccacaagccctccgtaaaaataagaactcggcacaaatggccagtcacatgcttacctgcatttttaaagacagctttcaggtatttggggactacattattaccaaaccttggctttgggagattatacaggtccgaggaactcgtgtctactgcagacgaatgcaattaccccaccttcctccatacagaattgttaggaaatgtccactcctttgggggtgatttttctcctcaagttgtagccaacattttgtccgtaactgatttcagggcaaacatttctgacatcttcctccagctcagtctgccatgccttggcaatccagtttcctgtcatatgcgagccatccaagttgatgccaagtaagatttgcccagctcaaagtgaaagtgtttgcgtcttggtatccggaatcctcagccccagtagcaaagctttagtcattcaccttcatccaatagacgtttgtgaacgtcctgctgtccattttgtcaataaacaggcagccctgcaggtggtccatctcgtgctggatgatgcgggctgcccacccgctcgcctgccacaccacctgttctccattggggtccagcccgcgttctggaggcaggggacgccggctagggccccacgctgggcggttcggcctgcgtctccgctcgccctccctccgggcaggctgggcccgcgggctccaggcgtggctcctcggcgggaggctctggtgctggagctgtgagctcgggccccagcgcctggtcatccagggtgaaaagcgtctctctctttggcaggataaaggcgaggggctcctgaatggcgccgatgttcacatgccctaggttaccgtacttggagagctgagtgggaggaatgcctaacccagacgtggggaaagcaaaatggaaaacagttactaaagtctgtgctatctgagctggtggaaaaaggacttggagacagcgatttaaatacggaacaaggtcttccaggaagacagtgcagaactggacaaagagctcttgctccccgctgctgaaggcagcctcttcagcgcgatggaaggccaggattattttagttaccttggcaagggcatcttccaaggccccagtcacatcctgcgccagggccacagggcagcagaggcgcagatcattgaaggcaaccagaatattgttgagaaagcaggcgaggggtgggaaatctaggagcaccatgggtggctgcagcgtccccggctgggtggctggcacagcagcaggcatgttactggtgcccaggatggctggagccgagatgagcatgtaggagttcatttcttcctggaatttctccactgtttcctgaattgctttctggaaagtgctgatggccacccgctggaaaacaggagccaactgaccccggaaatcagctcccacccggctgaaggacagcccaaagtacatgcactggcccagcagagagtccaggtggccgcctatgccccggtaaaggtcggtctccagcacctgcaggaattgtgagaccttctgtagcacccagccatggaagatggcactctcattcacagtgtgctcacccatggcagggggcagcagtgggtcctcgtctgagaagatggcacggtactgggtgatgatatcaaagagatggacacgggaggcctcgatggtttttgtaatatggaaatagggatcatcattaggaatggcagtcaggatggaccggagccaagcatctcgggcctgaagaaacttcaccctcaactcagcctcagtgaagacgtccatgcgccgcaggtagccaatgacacggaggcaggcaggaagctggatgttggtcctcagttgctggatcagctggctcagcatcagctgcatggactggcgcacttcgttcacgatgccctggatgacagggatggaagagtatttcctctccagtcggcgtacgtaggctgcaagctccagggcctcttcataataactgttccggacacaggtgtccatgagctgaggaatctccagtatttccaaaatttctgtgtgccggtttagggtcaggctattcatccggcggttggagctgatctcctcggcttccttcacaaagttcctgcagctctgctggaagctgggcaaacggtcgagcaggcggccgagcgacgcctccacgtcgccaaacaggcggtggatgcgctcggtgcactcggcgccgcggatgaaggtcttgtagttagcgaaggccaagtcgcgcgtctgctgcagcagctgcgcccgctcctccgccaggcgctcgggctcgcgccgcagccgctccagccccgagccgctcaactcccggaggtagcggcccacatcgggccgctcgcgccactgggcctcggggaagcggtcccggaacagcgacgccaggagcccttcatcctccacctcgccgagagccgctgctgtggccgtggctaccgatgggatagtcgccgcggtcgccatcttcccagcaac

SEQ ID NO: 13001 - RNA, 3765 nt, Homo sapiens
  source 1..3765: mol_type = other RNA
gctgggattacaggcatgagccaccaagcctggccgggattccttttcaaagtctggctgcacctagagccagtttgcttctgcttggcctcatggggcctcagagaaagccacaaaggaggatgggtctttcctgggttcatttaactgccatttataacactttttcctctaaacagcttaatggacttcctactacttgtatagtttgattttcaggactctgttcagcaagaatacctactttacaaaactcagcataaaaatgaggtgaaacagtttaactaaaactggagtttggctgggtagtgtggctcacaactgatcccagcactttgggaggccgaggcaggaggattgcctgagaccaggaatttgaggccagcctgggcaacatagtaagacccccgtctctatcttaaaaaaaaaataaaagaataaaacaagttccttcacctcttgacaagacaaagctgacactttttttttttgagacagagaaaaaaagaaaactctacagccagaatcatacttttgagtctcgctctgtcgcccaggctggatggagtgcagtggcgtgatctcagctcactgtaacctccgcctcctgggttcaagtaattctctgccttggcttcacgagtagctgggattacaggtgctcgccaccacgcccggctaatttttgtatctttagtagagacagggtttcaccatcttggccaggctggtcttgagctcctgacctcgtgatccacccgccccgccctcccaaagtgctgggattacaggcgtgaaccactgcacctggccactttcttaaacctacacattggttgctgtgatattaattctatttttacaaaataagtgtataaccaggaagtactaatcctgctttctatgcccaattgttaacaggaaagggctcagtgcacttctcaattgtcacccctgcccccagccctgatccacggcctctaccccaagaatgagccaagaaccagctgctctagggatctcagcagcaaaatcctgcccaaggctgttaaaatgtgtgggcactcatttacactcgtgctgtcatgaaacacatccttgaacagggactattctctttcatttccataagcaaactggcgtctaaggccacaagccctccgtaaaaataagaactcggcacaaatggccagtcacatgcttacctgcatttttaaagacagctttcaggtatttggggactacattattaccaaaccttggctttgggagattatacaggtccgaggaactcgtgtctactgcagacgaatgcaattaccccaccttcctccatacagaattgttaggaaatgtccactcctttgggggtgatttttctcctcaagttgtagccaacattttgtccgtaactgatttcagggcaaacatttctgacatcttcctccagctcagtctgccatgccttggcaatccagtttcctgtcatatgcgagccatccaagttgatgccaagtaagatttgcccagctcaaagtgaaagtgtttgcgtcttggtatccggaatcctcagccccagtagcaaagctttagtcattcaccttcatccaatagacgtttgtgaacgtcctgctgtccattttgtcaataaacaggcagccctgcaggtggtccatctcgtgctggatgatgcgggctgcccacccgctcgcctgccacaccacctgttctccattggggtccagcccgcgttctggaggcaggggacgccggctagggccccacgctgggcggttcggcctgcgtctccgctcgccctccctccgggcaggctgggcccgcgggctccaggcgtggctcctcggcgggaggctctggtgctggagctgtgagctcgggccccagcgcctggtcatccagggtgaaaagcgtctctctctttggcaggataaaggcgaggggctcctgaatggcgccgatgttcacatgccctaggttaccgtacttggagagctgagtgggaggaatgcctgaggtcaggaattcgagaccagcctgacccacacggagaaatcccatctctcttaaaaatacaacattagccgggcttggtggcgcaggcctgtaatcccagctacttgggaaggctaaggcaggagaatcgcttgaacctaaagtctgtgctatctgagctggtggaaaaaggacttggagacagcgatttaaatacggaacaaggtcttccaggaagacagtgcagaactggacaaagagctcttgctccccgctgctgaaggcagcctcttcagcgcgatggaaggccaggattattttagttaccttggcaagggcatcttccaaggccccagtcacatcctgcgccagggccacagggcagcagaggcgcagatcattgaaggcaaccagaatattgttgagaaagcaggcgaggggtgggaaatctaggagcaccatgggtggctgcagcgtccccggctgggtggctggcacagcagcaggcatgttactggtgcccaggatggctggagccgagatgagcatgtaggagttcatttcttcctggaatttctccactgtttcctgaattgctttctggaaagtgctgatggccacccgctggaaaacaggagccaactgaccccggaaatcagctcccacccggctgaaggacagcccaaagtacatgcactggcccagcagagagtccaggtggccgcctatgccccggtaaaggtcggtctccagcacctgcaggaattgtgagaccttctgtagcacccagccatggaagatggcactctcattcacagtgtgctcacccatggcagggggcagcagtgggtcctcgtctgagaagatggcacggtactgggtgatgatatcaaagagatggacacgggaggcctcgatggtttttgtaatatggaaatagggatcatcattaggaatggcagtcaggatggaccggagccaagcatctcgggcctgaagaaacttcaccctcaactcagcctcagtgaagacgtccatgcgccgcaggtagccaatgacacggaggcaggcaggaagctggatgttggtcctcagttgctggatcagctggctcagcatcagctgcatggactggcgcacttcgttcacgatgccctggatgacagggatggaagagtatttcctctccagtcggcgtacgtaggctgcaagctccagggcctcttcataataactgttccggacacaggtgtccatgagctgaggaatctccagtatttccaaaatttctgtgtgccggtttagggtcaggctattcatccggcggttggagctgatctcctcggcttccttcacaaagttcctgcagctctgctggaagctgggcaaacggtcgagcaggcggccgagcgacgcctccacgtcgccaaacaggcggtggatgcgctcggtgcactcggcgccgcggatgaaggtcttgtagttagcgaaggccaagtcgcgcgtctgctgcagcagctgcgcccgctcctccgccaggcgctcgggctcgcgccgcagccgctccagccccgagccgctcaactcccggaggtagcggcccacatcgggccgctcgcgccactgggcctcggggaagcggtcccggaacagcgacgccaggagcccttcatcctccacctcgccgagagccgctgctgtggccgtggctaccgatgggatagtcgccgcggtcgccatcttcccagcaac

SEQ ID NO: 13002 - RNA, 3341 nt, Homo sapiens
  source 1..3341: mol_type = other RNA
gctgggattacaggcatgagccaccaagcctggccgggattccttttcaaagtctggctgcacctagagccagtttgcttctgcttggcctcatggggcctcagagaaagccacaaaggaggatgggtctttcctgggttcatttaactgccatttataacactttttcctctaaacagcttaatggacttcctactacttgtatagtttgattttcaggactctgttcagcaagaatacctactttacaaaactcagcataaaaatgaggtgaaacagtttaactaaaactggagtttggctgggtagtgtggctcacaactgatcccagcactttgggaggccgaggcaggaggattgcctgagaccaggaatttgaggccagcctgggcaacatagtaagacccccgtctctatcttaaaaaaaaaataaaagaataaaacaagttccttcacctcttgacaagacaaagctgacactttttttttttgagacagagaaaaaaagaaaactctacagccagaatcatacttttgagtctcgctctgtcgcccaggctggatggagtgcagtggcgtgatctcagctcactgtaacctccgcctcctgggttcaagtaattctctgccttggcttcacgagtagctgggattacaggtgctcgccaccacgcccggctaatttttgtatctttagtagagacagggtttcaccatcttggccaggctggtcttgagctcctgacctcgtgatccacccgccccgccctcccaaagtgctgggattacaggcgtgaaccactgcacctggccactttcttaaacctacacattggttgctgtgatattaattctatttttacaaaataagtgtataaccaggaagtactaatcctgctttctatgcccaattgttaacaggaaagggctcagtgcacttctcaattgtcacccctgcccccagccctgatccacggcctctaccccaagaatgagccaagaaccagctgctctagggatctcagcagcaaaatcctgcccaaggctgttaaaatgtgtgggcactcatttacactcgtgctgtcatgaaacacatccttgaacagggactattctctttcatttccataagcaaactggcgtctaaggccacaagccctccgtaaaaataagaactcggcacaaatggccagtcacatgcttacctgcatttttaaagacagctttcaggtatttggggactacattattaccaaaccttggctttgggagattatacaggtccgaggaactcgtgtctactgcagacgaatgcaattaccccaccttcctccatacagaattgttaggaaatgtccactcctttgggggtgatttttctcctcaagttgtagccaacattttgtccgtaactgatttcagggcaaacatttctgacatcttcctccagctcagtctgccatgccttggcaatccagtttcctgtcatatgcgagccatccaagttgatgccaagtaagatttgcccagctcaaagtgaaagtgtttgcgtcttggtatccggaatcctcagccccagtagcaaagctttagtcattcaccttcatccaatagacgtttgtgaacgtcctgctgtccattttgtcaataaacaggcagccctgcaggtggtccatctcgtgctggatgatgcgggctgcccacccgctcgcctgccacaccacctgttctccattggggtccagccctaaagtctgtgctatctgagctggtggaaaaaggacttggagacagcgatttaaatacggaacaaggtcttccaggaagacagtgcagaactggacaaagagctcttgctccccgctgctgaaggcagcctcttcagcgcgatggaaggccaggattattttagttaccttggcaagggcatcttccaaggccccagtcacatcctgcgccagggccacagggcagcagaggcgcagatcattgaaggcaaccagaatattgttgagaaagcaggcgaggggtgggaaatctaggagcaccatgggtggctgcagcgtccccggctgggtggctggcacagcagcaggcatgttactggtgcccaggatggctggagccgagatgagcatgtaggagttcatttcttcctggaatttctccactgtttcctgaattgctttctggaaagtgctgatggccacccgctggaaaacaggagccaactgaccccggaaatcagctcccacccggctgaaggacagcccaaagtacatgcactggcccagcagagagtccaggtggccgcctatgccccggtaaaggtcggtctccagcacctgcaggaattgtgagaccttctgtagcacccagccatggaagatggcactctcattcacagtgtgctcacccatggcagggggcagcagtgggtcctcgtctgagaagatggcacggtactgggtgatgatatcaaagagatggacacgggaggcctcgatggtttttgtaatatggaaatagggatcatcattaggaatggcagtcaggatggaccggagccaagcatctcgggcctgaagaaacttcaccctcaactcagcctcagtgaagacgtccatgcgccgcaggtagccaatgacacggaggcaggcaggaagctggatgttggtcctcagttgctggatcagctggctcagcatcagctgcatggactggcgcacttcgttcacgatgccctggatgacagggatggaagagtatttcctctccagtcggcgtacgtaggctgcaagctccagggcctcttcataataactgttccggacacaggtgtccatgagctgaggaatctccagtatttccaaaatttctgtgtgccggtttagggtcaggctattcatccggcggttggagctgatctcctcggcttccttcacaaagttcctgcagctctgctggaagctgggcaaacggtcgagcaggcggccgagcgacgcctccacgtcgccaaacaggcggtggatgcgctcggtgcactcggcgccgcggatgaaggtcttgtagttagcgaaggccaagtcgcgcgtctgctgcagcagctgcgcccgctcctccgccaggcgctcgggctcgcgccgcagccgctccagccccgagccgctcaactcccggaggtagcggcccacatcgggccgctcgcgccactgggcctcggggaagcggtcccggaacagcgacgccaggagcccttcatcctccacctcgccgagagccgctgctgtggccgtggctaccgatgggatagtcgccgcggtcgccatcttcccagcaac

SEQ ID NO: 13003 - RNA, 2339 nt, Homo sapiens
  source 1..2339: mol_type = other RNA
gctgggattacaggcatgagccaccaagcctggccgggattccttttcaaagtctggctgcacctagagccagtttgcttctgcttggcctcatggggcctcagagaaagccacaaaggaggatgggtctttcctgggttcatttaactgccatttataacactttttcctctaaacagcttaatggacttcctactacttgtatagtttgattttcaggactctgttcagcaagaatacctactttacaaaactcagcataaaaatgaggtgaaacagtttaactaaaactggagtttggctgggtagtgtggctcacaactgatcccagcactttgggaggccgaggcaggaggattgcctgagaccaggaatttgaggccagcctgggcaacatagtaagacccccgtctctatcttaaaaaaaaaataaaagaataaaacaagttccttcacctcttgacaagacaaagctgacactttttttttttgagacagagaaaaaaagaaaactctacagccagaatcatacttttgagtctcgctctgtcgcccaggctggatggagtgcagtggcgtgatctcagctcactgtaacctccgcctcctgggttcaagtaattctctgccttggcttcacgagtagctgggattacaggtgctcgccaccacgcccggctaatttttgtatctttagtagagacagggtttcaccatcttggccaggctggtcttgagctcctgacctcgtgatccacccgccccgccctcccaaagtgctgggattacaggcgtgaaccactgcacctggccactttcttaaacctacacattggttgctgtgatattaattctatttttacaaaataagtgtataaccaggaagtactaatcctgctttctatgcccaattgttaacaggaaagggctcagtgcacttctcaattgtcacccctgcccccagccctgatccacggcctctaccccaagaatgagccaagaaccagctgctctagggatctcagcagcaaaatcctgcccaaggctgttaaaatgtgtgggcactcatttacactcgtgctgtcatgaaacacatccttgaacagggactattctctttcatttccataagcaaactggcgtctaaggccacaagccctccgtaaaaataagaactcggcacaaatggccagtcacatgcttacctgcatttttaaagacagctttcaggtatttggggactacattattaccaaaccttggctttgggagattatacaggtccgaggaactcgtgtctactgcagacgaatgcaattaccccaccttcctccatacagaattgttaggaaatgtccactcctttgggggtgatttttctcctcaagttgtagccaacattttgtccgtaactgatttcagggcaaacatttctgacatcttcctccagctcagtctgccatgccttggcaatccagtttcctgtcatatgcgagccatccaagttgatgccaagtaagatttgcccagctcaaagtgaaagtgtttgcgtcttggtatccggaatcctcagccccagtagcaaagctttagtcattcaccttcatccaatagacgtttgtgaacgtcctgctgtccattttgtcaataaacaggcagccctgcaggtggtccatctcgtgctggatgatgcgggctgcccacccgctcgcctgccacaccacctgttctccattggggtccagccctgagatctgcaccgcctggaagcggggcacgcaggccaggaagccggcgacgctctcgcagccctcgggaaaggtgaccaggcggctgtcaagcactcgcaggctggggttcacgaacacgcgcagggggaagggctccatttggcggagcgcgcgctggcggggcgggcactcccgacacagcgcctcggggagctccagcgccagcacctgccgcggcacccccagctgcggcgcgcttaggcccacgcagcgccgccgccgcatcacctggaccagccgttgcgtcagccgctgcagctcgggcccgcctagctgcgcccgctccaccggggccgccacgccgcgcagcaccgggtccccgacttggcacacgtgcgagaacggcggttcgggaggacccagcaccagacgcctcaggtggcgccaataggagcgccgcagcgccgggccctcgacgccgtccggggcggccgtggagctgcaagcccggacaccgacggctgccgccccgccccacggcacggccgcccacagtggccaaagactcagcgcgccccacagccgggccatggcggcccccttaacagt

SEQ ID NO: 13004 - RNA, 3172 nt, Homo sapiens
  source 1..3172: mol_type = other RNA
gctgggattacaggcatgagccaccaagcctggccgggattccttttcaaagtctggctgcacctagagccagtttgcttctgcttggcctcatggggcctcagagaaagccacaaaggaggatgggtctttcctgggttcatttaactgccatttataacactttttcctctaaacagcttaatggacttcctactacttgtatagtttgattttcaggactctgttcagcaagaatacctactttacaaaactcagcataaaaatgaggtgaaacagtttaactaaaactggagtttggctgggtagtgtggctcacaactgatcccagcactttgggaggccgaggcaggaggattgcctgagaccaggaatttgaggccagcctgggcaacatagtaagacccccgtctctatcttaaaaaaaaaataaaagaataaaacaagttccttcacctcttgacaagacaaagctgacactttttttttttgagacagagaaaaaaagaaaactctacagccagaatcatacttttgagtctcgctctgtcgcccaggctggatggagtgcagtggcgtgatctcagctcactgtaacctccgcctcctgggttcaagtaattctctgccttggcttcacgagtagctgggattacaggtgctcgccaccacgcccggctaatttttgtatctttagtagagacagggtttcaccatcttggccaggctggtcttgagctcctgacctcgtgatccacccgccccgccctcccaaagtgctgggattacaggcgtgaaccactgcacctggccactttcttaaacctacacattggttgctgtgatattaattctatttttacaaaataagtgtataaccaggaagtactaatcctgctttctatgcccaattgttaacaggaaagggctcagtgcacttctcaattgtcacccctgcccccagccctgatccacggcctctaccccaagaatgagccaagaaccagctgctctagggatctcagcagcaaaatcctgcccaaggctgttaaaatgtgtgggcactcatttacactcgtgctgtcatgaaacacatccttgaacagggactattctctttcatttccataagcaaactggcgtctaaggccacaagccctccgtaaaaataagaactcggcacaaatggccagtcacatgcttacctgcatttttaaagacagctttcaggtatttggggactacattattaccaaaccttggctttgggagattatacaggtccgaggaactcgtgtctactgcagacgaatgcaattaccccaccttcctccatacagaattgttaggaaatgtccactcctttgggggtgatttttctcctcaagttgtagccaacattttgtccgtaactgatttcagggcaaacatttctgacatcttcctccagctcagtctgccatgccttggcaatccagtttcctgtcatatgcgagccatccaagttgatgccaagtaagatttgcccagctcaaagtgaaagtgtttgcgtcttggtatccggaatcctcagccccagtagcaaagctttagtcattcaccttcatccaatagacgtttgtgaacgtcctgctgtccattttgtcaataaacaggcagccctgcaggtggtccatctcgtgctggatgatgcgggctgcccacccgctcgcctgccacaccacctgttctccattggggtccagcccttggcaagggcatcttccaaggccccagtcacatcctgcgccagggccacagggcagcagaggcgcagatcattgaaggcaaccagaatattgttgagaaagcaggcgaggggtgggaaatctaggagcaccatgggtggctgcagcgtccccggctgggtggctggcacagcagcaggcatgttactggtgcccaggatggctggagccgagatgagcatgtaggagttcatttcttcctggaatttctccactgtttcctgaattgctttctggaaagtgctgatggccacccgctggaaaacaggagccaactgaccccggaaatcagctcccacccggctgaaggacagcccaaagtacatgcactggcccagcagagagtccaggtggccgcctatgccccggtaaaggtcggtctccagcacctgcaggaattgtgagaccttctgtagcacccagccatggaagatggcactctcattcacagtgtgctcacccatggcagggggcagcagtgggtcctcgtctgagaagatggcacggtactgggtgatgatatcaaagagatggacacgggaggcctcgatggtttttgtaatatggaaatagggatcatcattaggaatggcagtcaggatggaccggagccaagcatctcgggcctgaagaaacttcaccctcaactcagcctcagtgaagacgtccatgcgccgcaggtagccaatgacacggaggcaggcaggaagctggatgttggtcctcagttgctggatcagctggctcagcatcagctgcatggactggcgcacttcgttcacgatgccctggatgacagggatggaagagtatttcctctccagtcggcgtacgtaggctgcaagctccagggcctcttcataataactgttccggacacaggtgtccatgagctgaggaatctccagtatttccaaaatttctgtgtgccggtttagggtcaggctattcatccggcggttggagctgatctcctcggcttccttcacaaagttcctgcagctctgctggaagctgggcaaacggtcgagcaggcggccgagcgacgcctccacgtcgccaaacaggcggtggatgcgctcggtgcactcggcgccgcggatgaaggtcttgtagttagcgaaggccaagtcgcgcgtctgctgcagcagctgcgcccgctcctccgccaggcgctcgggctcgcgccgcagccgctccagccccgagccgctcaactcccggaggtagcggcccacatcgggccgctcgcgccactgggcctcggggaagcggtcccggaacagcgacgccaggagcccttcatcctccacctcgccgagagccgctgctgtggccgtggctaccgatgggatagtcgccgcggtcgccatcttcccagcaac

SEQ ID NO: 13005 - RNA, 3518 nt, Homo sapiens
  source 1..3518: mol_type = other RNA
gctgggattacaggcatgagccaccaagcctggccgggattccttttcaaagtctggctgcacctagagccagtttgcttctgcttggcctcatggggcctcagagaaagccacaaaggaggatgggtctttcctgggttcatttaactgccatttataacactttttcctctaaacagcttaatggacttcctactacttgtatagtttgattttcaggactctgttcagcaagaatacctactttacaaaactcagcataaaaatgaggtgaaacagtttaactaaaactggagtttggctgggtagtgtggctcacaactgatcccagcactttgggaggccgaggcaggaggattgcctgagaccaggaatttgaggccagcctgggcaacatagtaagacccccgtctctatcttaaaaaaaaaataaaagaataaaacaagttccttcacctcttgacaagacaaagctgacactttttttttttgagacagagaaaaaaagaaaactctacagccagaatcatacttttgagtctcgctctgtcgcccaggctggatggagtgcagtggcgtgatctcagctcactgtaacctccgcctcctgggttcaagtaattctctgccttggcttcacgagtagctgggattacaggtgctcgccaccacgcccggctaatttttgtatctttagtagagacagggtttcaccatcttggccaggctggtcttgagctcctgacctcgtgatccacccgccccgccctcccaaagtgctgggattacaggcgtgaaccactgcacctggccactttcttaaacctacacattggttgctgtgatattaattctatttttacaaaataagtgtataaccaggaagtactaatcctgctttctatgcccaattgttaacaggaaagggctcagtgcacttctcaattgtcacccctgcccccagccctgatccacggcctctaccccaagaatgagccaagaaccagctgctctagggatctcagcagcaaaatcctgcccaaggctgttaaaatgtgtgggcactcatttacactcgtgctgtcatgaaacacatccttgaacagggactattctctttcatttccataagcaaactggcgtctaaggccacaagccctccgtaaaaataagaactcggcacaaatggccagtcacatgcttacctgcatttttaaagacagctttcaggtatttggggactacattattaccaaaccttggctttgggagattatacaggtccgaggaactcgtgtctactgcagacgaatgcaattaccccaccttcctccatacagaattgttaggaaatgtccactcctttgggggtgatttttctcctcaagttgtagccaacattttgtccgtaactgatttcagggcaaacatttctgacatcttcctccagctcagtctgccatgccttggcaatccagtttcctgtcatatgcgagccatccaagttgatgccaagtaagatttgcccagctcaaagtgaaagtgtttgcgtcttggtatccggaatcctcagccccagtagcaaagctttagtcattcaccttcatccaatagacgtttgtgaacgtcctgctgtccattttgtcaataaacaggcagccctgcaggtggtccatctcgtgctggatgatgcgggctgcccacccgctcgcctgccacaccacctgttctccattggggtccagccgtggctcctcggcgggaggctctggtgctggagctgtgagctcgggccccagcgcctggtcatccagggtgaaaagcgtctctctctttggcaggataaaggcgaggggctcctgaatggcgccgatgttcacatgccctaggttaccgtacttggagagctgagtgggaggaatgcctaaagtctgtgctatctgagctggtggaaaaaggacttggagacagcgatttaaatacggaacaaggtcttccaggaagacagtgcagaactggacaaagagctcttgctccccgctgctgaaggcagcctcttcagcgcgatggaaggccaggattattttagttaccttggcaagggcatcttccaaggccccagtcacatcctgcgccagggccacagggcagcagaggcgcagatcattgaaggcaaccagaatattgttgagaaagcaggcgaggggtgggaaatctaggagcaccatgggtggctgcagcgtccccggctgggtggctggcacagcagcaggcatgttactggtgcccaggatggctggagccgagatgagcatgtaggagttcatttcttcctggaatttctccactgtttcctgaattgctttctggaaagtgctgatggccacccgctggaaaacaggagccaactgaccccggaaatcagctcccacccggctgaaggacagcccaaagtacatgcactggcccagcagagagtccaggtggccgcctatgccccggtaaaggtcggtctccagcacctgcaggaattgtgagaccttctgtagcacccagccatggaagatggcactctcattcacagtgtgctcacccatggcagggggcagcagtgggtcctcgtctgagaagatggcacggtactgggtgatgatatcaaagagatggacacgggaggcctcgatggtttttgtaatatggaaatagggatcatcattaggaatggcagtcaggatggaccggagccaagcatctcgggcctgaagaaacttcaccctcaactcagcctcagtgaagacgtccatgcgccgcaggtagccaatgacacggaggcaggcaggaagctggatgttggtcctcagttgctggatcagctggctcagcatcagctgcatggactggcgcacttcgttcacgatgccctggatgacagggatggaagagtatttcctctccagtcggcgtacgtaggctgcaagctccagggcctcttcataataactgttccggacacaggtgtccatgagctgaggaatctccagtatttccaaaatttctgtgtgccggtttagggtcaggctattcatccggcggttggagctgatctcctcggcttccttcacaaagttcctgcagctctgctggaagctgggcaaacggtcgagcaggcggccgagcgacgcctccacgtcgccaaacaggcggtggatgcgctcggtgcactcggcgccgcggatgaaggtcttgtagttagcgaaggccaagtcgcgcgtctgctgcagcagctgcgcccgctcctccgccaggcgctcgggctcgcgccgcagccgctccagccccgagccgctcaactcccggaggtagcggcccacatcgggccgctcgcgccactgggcctcggggaagcggtcccggaacagcgacgccaggagcccttcatcctccacctcgccgagagccgctgctgtggccgtggctaccgatgggatagtcgccgcggtcgccatcttcccagcaac

SEQ ID NO: 13006 - RNA, 3621 nt, Homo sapiens
  source 1..3621: mol_type = other RNA
gctgggattacaggcatgagccaccaagcctggccgggattccttttcaaagtctggctgcacctagagccagtttgcttctgcttggcctcatggggcctcagagaaagccacaaaggaggatgggtctttcctgggttcatttaactgccatttataacactttttcctctaaacagcttaatggacttcctactacttgtatagtttgattttcaggactctgttcagcaagaatacctactttacaaaactcagcataaaaatgaggtgaaacagtttaactaaaactggagtttggctgggtagtgtggctcacaactgatcccagcactttgggaggccgaggcaggaggattgcctgagaccaggaatttgaggccagcctgggcaacatagtaagacccccgtctctatcttaaaaaaaaaataaaagaataaaacaagttccttcacctcttgacaagacaaagctgacactttttttttttgagacagagaaaaaaagaaaactctacagccagaatcatacttttgagtctcgctctgtcgcccaggctggatggagtgcagtggcgtgatctcagctcactgtaacctccgcctcctgggttcaagtaattctctgccttggcttcacgagtagctgggattacaggtgctcgccaccacgcccggctaatttttgtatctttagtagagacagggtttcaccatcttggccaggctggtcttgagctcctgacctcgtgatccacccgccccgccctcccaaagtgctgggattacaggcgtgaaccactgcacctggccactttcttaaacctacacattggttgctgtgatattaattctatttttacaaaataagtgtataaccaggaagtactaatcctgctttctatgcccaattgttaacaggaaagggctcagtgcacttctcaattgtcacccctgcccccagccctgatccacggcctctaccccaagaatgagccaagaaccagctgctctagggatctcagcagcaaaatcctgcccaaggctgttaaaatgtgtgggcactcatttacactcgtgctgtcatgaaacacatccttgaacagggactattctctttcatttccataagcaaactggcgtctaaggccacaagccctccgtaaaaataagaactcggcacaaatggccagtcacatgcttacctgcatttttaaagacagctttcaggtatttggggactacattattaccaaaccttggctttgggagattatacaggtccgaggaactcgtgtctactgcagacgaatgcaattaccccaccttcctccatacagaattgttaggaaatgtccactcctttgggggtgatttttctcctcaagttgtagccaacattttgtccgtaactgatttcagggcaaacatttctgacatcttcctccagctcagtctgccatgccttggcaatccagtttcctgtcatatgcgagccatccaagttgatgccaagtaagatttgcccagctcaaagtgaaagtgtttgcgtcttggtatccggaatcctcagccccagtagcaaagctttagtcattcaccttcatccaatagacgtttgtgaacgtcctgctgtccattttgtcaataaacaggcagccctgcaggtggtccatctcgtgctggatgatgcgggctgcccacccgctcgcctgccacaccacctgttctccattggggtccagccgttctggaggcaggggacgccggctagggccccacgctgggcggttcggcctgcgtctccgctcgccctccctccgggcaggctgggcccgcgggctccaggcgtggctcctcggcgggaggctctggtgctggagctgtgagctcgggccccagcgcctggtcatccagggtgaaaagcgtctctctctttggcaggataaaggcgaggggctcctgaatggcgccgatgttcacatgccctaggttaccgtacttggagagctgagtgggaggaatgcctaaagtctgtgctatctgagctggtggaaaaaggacttggagacagcgatttaaatacggaacaaggtcttccaggaagacagtgcagaactggacaaagagctcttgctccccgctgctgaaggcagcctcttcagcgcgatggaaggccaggattattttagttaccttggcaagggcatcttccaaggccccagtcacatcctgcgccagggccacagggcagcagaggcgcagatcattgaaggcaaccagaatattgttgagaaagcaggcgaggggtgggaaatctaggagcaccatgggtggctgcagcgtccccggctgggtggctggcacagcagcaggcatgttactggtgcccaggatggctggagccgagatgagcatgtaggagttcatttcttcctggaatttctccactgtttcctgaattgctttctggaaagtgctgatggccacccgctggaaaacaggagccaactgaccccggaaatcagctcccacccggctgaaggacagcccaaagtacatgcactggcccagcagagagtccaggtggccgcctatgccccggtaaaggtcggtctccagcacctgcaggaattgtgagaccttctgtagcacccagccatggaagatggcactctcattcacagtgtgctcacccatggcagggggcagcagtgggtcctcgtctgagaagatggcacggtactgggtgatgatatcaaagagatggacacgggaggcctcgatggtttttgtaatatggaaatagggatcatcattaggaatggcagtcaggatggaccggagccaagcatctcgggcctgaagaaacttcaccctcaactcagcctcagtgaagacgtccatgcgccgcaggtagccaatgacacggaggcaggcaggaagctggatgttggtcctcagttgctggatcagctggctcagcatcagctgcatggactggcgcacttcgttcacgatgccctggatgacagggatggaagagtatttcctctccagtcggcgtacgtaggctgcaagctccagggcctcttcataataactgttccggacacaggtgtccatgagctgaggaatctccagtatttccaaaatttctgtgtgccggtttagggtcaggctattcatccggcggttggagctgatctcctcggcttccttcacaaagttcctgcagctctgctggaagctgggcaaacggtcgagcaggcggccgagcgacgcctccacgtcgccaaacaggcggtggatgcgctcggtgcactcggcgccgcggatgaaggtcttgtagttagcgaaggccaagtcgcgcgtctgctgcagcagctgcgcccgctcctccgccaggcgctcgggctcgcgccgcagccgctccagccccgagccgctcaactcccggaggtagcggcccacatcgggccgctcgcgccactgggcctcggggaagcggtcccggaacagcgacgccaggagcccttcatcctccacctcgccgagagccgctgctgtggccgtggctaccgatgggatagtcgccgcggtcgccatcttcccagcaac

SEQ ID NO: 13007 - RNA, 2147 nt, Homo sapiens
  source 1..2147: mol_type = other RNA
gctgggattacaggcatgagccaccaagcctggcctcatcatggatttttgcattaattttgatttttaaaaaatactgctgtaaggtcaggcacagtggctcatgcctgtagtcccagcactttgggaggctgaggcagggggatcatttgagtcaggagttcgagaccagcctggccaacatggtgaaatcatgtctctactaaaaatagaaaaattagctgggcatggtggcgcatgcctgtaatcccagctactcaggaggctgtggcaggagaatcgcttgaaccggggaggcacaggtttcagtgagctgagatctcgcctctacattccagcctgggtaacgagtgatacttgatctcaaaaaaaaaaaacccaaaacaaaatattgctttaaaatattttttatcttggttgctgagcttttttggtgtcctcttaaaattctgccctggagatgtcaccctagctccagccctgaccttaagagggaggtactagtattatccacatttattttttatttttttaattaaataattaattaattatatttatttttgagacggagtctcgctctgttgcccaggctggagtgcagtggcgctatctcggctcactgcaagctctgcctcccagtttcacgccattctcctgcctcagcctcccaagtagctgggactgcaggtgcccaccaccacacccggctaattttttgtatttttagtagagatggggtttcaccatgttagccaggatggtctcaatctcctgatcttgtgatccacctgcctcggcctcccaaagtgctgggattacaggtgtgagccactgcgcccggcctgttatccacattttataaatgaggaaaccaaggcacagagaggtgaagtgacttgcccaagatcatacagtgggaaaagtggcggagtcaggatttgaatctgggcagcctggctctaggtgctgggctctagatggaaggccctgtctgagctccctgcactaggaacaagtgtggtcaggggctggacggtcagcttttgggtagccattcaagaaatgtattgaaaaacctagagaggcaggctagggagagctgagttggttacatctggggtccatctagggttccatccctggaagagatggtggtggttagggctgtccggagctcctcaggggcaaagacccccagttctgtgatgatgccaccagtgatgaggtcgtggggggtgacatcgaaggcaggattccaaactccaatcccaggtgctgcaatccggaccccattaacatcggtcagctcctggcccggtcgctcttcaataatgatctccttgccggtctccagacggaggtcacatgaagagctgggggcagccacgtagaagggaatgccatggtgcttggcgacaatggccagctggtaggtgcccaccttgttggctgtgtcgccgttggcaaccacgcggtcagctcccacgaccacagctgacacgcccctatgggccatggcagcagccaccatgctgtcggtgataagggtggcggggatctgctcatagaccagctcaaaggccgtcagccgggctccctggttgtagggccgggtctcgagcacagtcccgcccaggggccctcgcagtggcagttccctctgcctggtatgctcttcccaatgctcgcatagctccgtttcacgtctctcccggaccgcctcttccgtagcgccctcccgttcggcctcccgggctgcaacatcagccaggtcgcgggcggcgcgggccatgttgacagcggtgggccgggcggtgacgaggaagctcagcttgtcgcgcacgaaggccacgagcgcggcgagtcccggtcccccggcgcccgcctgcagctccacggcgaggctgagacagcccaccagggctatggccggggcgccccgcaccttcatggcgcggatggcctcccaggcctggtgcaccgagcccaccgcctcgtagcggctctgcttgggcagcagcagctggtctaggatctgcagggagccccgcgagtagcggatcgcctccagggtcatggtgcagcagccaagcccagcgcaactcagagggagctaggggtccgcgcgcacttgggagcggggc

SEQ ID NO: 13008 - RNA, 2201 nt, Homo sapiens
  source 1..2201: mol_type = other RNA
gctgggattacaggcatgagccaccaagcctggcctcatcatggatttttgcattaattttgatttttaaaaaatactgctgtaaggtcaggcacagtggctcatgcctgtagtcccagcactttgggaggctgaggcagggggatcatttgagtcaggagttcgagaccagcctggccaacatggtgaaatcatgtctctactaaaaatagaaaaattagctgggcatggtggcgcatgcctgtaatcccagctactcaggaggctgtggcaggagaatcgcttgaaccggggaggcacaggtttcagtgagctgagatctcgcctctacattccagcctgggtaacgagtgatacttgatctcaaaaaaaaaaaacccaaaacaaaatattgctttaaaatattttttatcttggttgctgagcttttttggtgtcctcttaaaattctgccctggagatgtcaccctagctccagccctgaccttaagagggaggtactagtattatccacatttattttttatttttttaattaaataattaattaattatatttatttttgagacggagtctcgctctgttgcccaggctggagtgcagtggcgctatctcggctcactgcaagctctgcctcccagtttcacgccattctcctgcctcagcctcccaagtagctgggactgcaggtgcccaccaccacacccggctaattttttgtatttttagtagagatggggtttcaccatgttagccaggatggtctcaatctcctgatcttgtgatccacctgcctcggcctcccaaagtgctgggattacaggtgtgagccactgcgcccggcctgttatccacattttataaatgaggaaaccaaggcacagagaggtgaagtgacttgcccaagatcatacagtgggaaaagtggcggagtcaggatttgaatctgggcagcctggctctaggtgctgggctctagatggaaggccctgtctgagctccctgcactaggaacaagtgtggtcaggggctggacggtcagcttttgggtagccattcaagaaatgtattgaaaaacctagagaggcaggctagggagagctgagttggttacatctggggtccatctagggttccatccctggaagagatggtggtggttagggctgtccggagctcctcaggggcaaagacccccagttctgtgatgatgccaccagtgatgaggtcgtggggggtgacatcgaaggcaggattccaaactccaatcccaggtgctgcaatccggaccccattaacatcggtcagctcctggcccggtcgctcttcaataatgatctccttgccggtctccagacggaggtcacatgaagagctgggggcagccacgtagaagggaatgccatggtgcttggcgacaatggccagctggtaggtgcccaccttgttggctgtgtcgccgttggcaaccacgcggtcagctcccacgaccacagctgacacgcccctatgggccatggcagcagccaccatgctgtcggtgataagggtggcggggatctgctcatagaccagctcaaaggccgtcagccgggctccctggttgtagggccgggtctctgtgcagaaggcatgctccaggcggcccaggctgtgcagtgagcgaatcacaccgagcacagtcccgcccaggggccctcgcagtggcagttccctctgcctggtatgctcttcccaatgctcgcatagctccgtttcacgtctctcccggaccgcctcttccgtagcgccctcccgttcggcctcccgggctgcaacatcagccaggtcgcgggcggcgcgggccatgttgacagcggtgggccgggcggtgacgaggaagctcagcttgtcgcgcacgaaggccacgagcgcggcgagtcccggtcccccggcgcccgcctgcagctccacggcgaggctgagacagcccaccagggctatggccggggcgccccgcaccttcatggcgcggatggcctcccaggcctggtgcaccgagcccaccgcctcgtagcggctctgcttgggcagcagcagctggtctaggatctgcagggagccccgcgagtagcggatcgcctccagggtcatggtgcagcagccaagcccagcgcaactcagagggagctaggggtccgcgcgcacttgggagcggggc

SEQ ID NO: 13009 - RNA, 2313 nt, Homo sapiens
  source 1..2313: mol_type = other RNA
gctgggattacaggcatgagccaccaagcctggcctcatcatggatttttgcattaattttgatttttaaaaaatactgctgtaaggtcaggcacagtggctcatgcctgtagtcccagcactttgggaggctgaggcagggggatcatttgagtcaggagttcgagaccagcctggccaacatggtgaaatcatgtctctactaaaaatagaaaaattagctgggcatggtggcgcatgcctgtaatcccagctactcaggaggctgtggcaggagaatcgcttgaaccggggaggcacaggtttcagtgagctgagatctcgcctctacattccagcctgggtaacgagtgatacttgatctcaaaaaaaaaaaacccaaaacaaaatattgctttaaaatattttttatcttggttgctgagcttttttggtgtcctcttaaaattctgccctggagatgtcaccctagctccagccctgaccttaagagggaggtactagtattatccacatttattttttatttttttaattaaataattaattaattatatttatttttgagacggagtctcgctctgttgcccaggctggagtgcagtggcgctatctcggctcactgcaagctctgcctcccagtttcacgccattctcctgcctcagcctcccaagtagctgggactgcaggtgcccaccaccacacccggctaattttttgtatttttagtagagatggggtttcaccatgttagccaggatggtctcaatctcctgatcttgtgatccacctgcctcggcctcccaaagtgctgggattacaggtgtgagccactgcgcccggcctgttatccacattttataaatgaggaaaccaaggcacagagaggtgaagtgacttgcccaagatcatacagtgggaaaagtggcggagtcaggatttgaatctgggcagcctggctctaggtgctgggctctagatggaaggccctgtctgagctccctgcactaggaacaagtgtggtcaggggctggacggtcagcttttgggtagccattcaagaaatgtattgaaaaacctagagaggcaggctagggagagctgagttggttacatctggggtccatctagggttccatccctggaagagatggtggtggttagggctgtccggagctcctcaggggcaaagacccccagttctgtgatgatgccaccagtgatgaggtcgtggggggtgacatcgaaggcaggattccaaactccaatcccaggtgctgcaatccggaccccattaacatcggtcagctcctggcccggtcgctcttcaataatgatctccttgccggtctccagacggaggtcacatgaagagctgggggcagccacgtagaagggaatgccatggtgcttggcgacaatggccagctggtaggtgcccaccttgttggctgtgtcgccgttggcaaccacgcggtcagctcccacgaccacagctgacacgcccctatgggccatggcagcagccaccatgctgtcggtgataagggtggcggggatctgctcatagaccagctcaaaggccgtcagccgggctccctggttgtagggccgggtctctgtgcagaaggcatgctccaggcggcccaggctgtgcagtgagcgaatcacaccgagcacagtcccgcccaggggccctcgcagtggcagttccctctgcctggtatgctcttcccaatgctcgcatagctccgtttcacgtcttgccaccgctgggggccacccgctccaggaggtggcgggctcctaggtccccaatgcttcggttgtctctgaggtctttctccagcatgtcctcggtgcagcagatcactctctcccggaccgcctcttccgtagcgccctcccgttcggcctcccgggctgcaacatcagccaggtcgcgggcggcgcgggccatgttgacagcggtgggccgggcggtgacgaggaagctcagcttgtcgcgcacgaaggccacgagcgcggcgagtcccggtcccccggcgcccgcctgcagctccacggcgaggctgagacagcccaccagggctatggccggggcgccccgcaccttcatggcgcggatggcctcccaggcctggtgcaccgagcccaccgcctcgtagcggctctgcttgggcagcagcagctggtctaggatctgcagggagccccgcgagtagcggatcgcctccagggtcatggtgcagcagccaagcccagcgcaactcagagggagctaggggtccgcgcgcacttgggagcggggc

SEQ ID NO: 13010 - RNA, 2288 nt, Homo sapiens
  source 1..2288: mol_type = other RNA
gctgggattacaggcatgagccaccaagcctggcctcatcatggatttttgcattaattttgatttttaaaaaatactgctgtaaggtcaggcacagtggctcatgcctgtagtcccagcactttgggaggctgaggcagggggatcatttgagtcaggagttcgagaccagcctggccaacatggtgaaatcatgtctctactaaaaatagaaaaattagctgggcatggtggcgcatgcctgtaatcccagctactcaggaggctgtggcaggagaatcgcttgaaccggggaggcacaggtttcagtgagctgagatctcgcctctacattccagcctgggtaacgagtgatacttgatctcaaaaaaaaaaaacccaaaacaaaatattgctttaaaatattttttatcttggttgctgagcttttttggtgtcctcttaaaattctgccctggagatgtcaccctagctccagccctgaccttaagagggaggtactagtattatccacatttattttttatttttttaattaaataattaattaattatatttatttttgagacggagtctcgctctgttgcccaggctggagtgcagtggcgctatctcggctcactgcaagctctgcctcccagtttcacgccattctcctgcctcagcctcccaagtagctgggactgcaggtgcccaccaccacacccggctaattttttgtatttttagtagagatggggtttcaccatgttagccaggatggtctcaatctcctgatcttgtgatccacctgcctcggcctcccaaagtgctgggattacaggtgtgagccactgcgcccggcctgttatccacattttataaatgaggaaaccaaggcacagagaggtgaagtgacttgcccaagatcatacagtgggaaaagtggcggagtcaggatttgaatctgggcagcctggctctaggtgctgggctctagatggaaggccctgtctgagctccctgcactaggaacaagtgtggtcaggggctggacggtcagcttttgggtagccattcaagaaatgtattgaaaaacctagagaggcaggctagggagagctgagttggttacatctggggtccatctagggttccatccctggaagagatggtggtggttagggctgtccggagctcctcaggggcaaagacccccagttctgtgatgatgccaccagtgatgaggtcgtggggggtgacatcgaaggcaggattccaaactccaatcccaggtgctgcaatccggaccccattaacatcggtcagctcctggcccggtcgctcttcaataatgatctccttgccggtctccagacggaggtcacatgaagagctgggggcagccacgtagaagggaatgccatggtgcttggcgacaatggccagctggtaggtgcccaccttgttggctgtgtcgccgttggcaaccacgcggtcagctcccacgaccacagctgacacgcccctatgggccatggcagcagccaccatgctgtcggtgataagggtggcggggatctgctcatagaccagctcaaaggccgtcagccgggctccctggttgtagggccgggtctctgtgcagaaggcatgctccaggcggcccaggctgtgcagtgagcgaatcacacctagggctgtaccatagccagcggtggccagagcaccagtgttacagtgggtcagcacagtcaccttgccaccgctgggggccacccgctccaggaggtggcgggctcctaggtccccaatgcttcggttgtctctgaggtctttctccagcatgtcctcggtgcagcagatcactctctcccggaccgcctcttccgtagcgccctcccgttcggcctcccgggctgcaacatcagccaggtcgcgggcggcgcgggccatgttgacagcggtgggccgggcggtgacgaggaagctcagcttgtcgcgcacgaaggccacgagcgcggcgagtcccggtcccccggcgcccgcctgcagctccacggcgaggctgagacagcccaccagggctatggccggggcgccccgcaccttcatggcgcggatggcctcccaggcctggtgcaccgagcccaccgcctcgtagcggctctgcttgggcagcagcagctggtctaggatctgcagggagccccgcgagtagcggatcgcctccagggtcatggtgcagcagccaagcccagcgcaactcagagggagctaggggtccgcgcgcacttgggagcggggc

SEQ ID NO: 13011 - RNA, 2731 nt, Homo sapiens
  source 1..2731: mol_type = other RNA
gctgggattacaggcatgagccaccaatcccagcctgaaaagccttttattgggatgtcttaacaagggatcataaatcagatttcaatttctaaatgtttgccctggctgcaatgtgggtaatgtttatgggggtgggtggtgggcaaggaagaggacaaaaatattcaataggacccatagtccatataaaataatgctgcctttgataaagcccctgtgacattttttattgaccttacacacataagcacactcatgtgtcacttaacaaggatacattctgagaaatgcatccttaggtgatttcaccattttctgagcatcaaagtgtacttacccaacctacatggtatagcctactacacacctatgctatatggtgtggcctattgctcctaggctccaaacctgtatagcacgtgattgaactgaaaactttaggcaatcataacacaatgggaagtatttgtgtacctaaacatatctaaatattaaataaaaaggtatagtaaaaatagggtaatcttacgggaccatcatcatatatgtggttcgttgttgaccgaaacattattacgtagtacatgactgtacctggtattttcagaatggatttatattagacagggttttccagagagacaaaacatagatggatggatggatagacagagatgagaggggattgattaggggaatcagctcacacaatttggaaactgagaagtcccatgccaggcatttgcaagctggagacccagggcagctggtagtgtggctcagtcccagctgaaggcctcagaattagggaagccgatggtgttactctcagtccaagacagcaggtctgagaacccagggaagcaacggttcagatcctggagtccaaaagctgaagaacttgggaattctgcttccaaaagcaggagaagaagggtgccccagctccagaagagagagaaaaaaattgtctctcctctgcctttttgttctatctgggccatcagccaattagatggtgccacccacactgtgtgagggcagatcttcctcactcagtccactgcttcaaatgccaatctcctccagaaacacgctcacagacacacccagaaataatgctttaccagctatctgtgtatcccctgatccagtcaagttgacacctaaaattaaccatcacaggatttctctattgcttggcagagttccaacatttcagactttctaatgtcttaaagtagtacttttaataaatggatgtatcgttttactcttctaggagctaaggactggctcaattgactataaagaatcgagaatgtcagctgaccaggcaaccaggagacgctttcctgacttccactatgcacgtgggctgcataattgtgtctgtgaagtaatgaagaacgtgcttgctctgtaacatccaaacgcgtggccaccattcacagatagtgtcctttgggaaaggtgtgggtatagatggggaatggtcagtcctatgaatatggggctataagacagcaaggctagaaagtatctgtgctttcattttttaattttatctattttttttttttttttgcactaatggtttgcattcacattgaggaactgagactgttttcagacttttggcctactgatgaccttatgttcataaaaggatagaagtataataagttgtttaatataaaacatactgaaattttattttctgtctccttggatataaagtttccacttatcttgggtttaagtacctactcctccacagagagggaccttgtgcatgtagattgatattctcaggatgaaagcagtacctactacaactaggaactcacagaacaggaagacgatgcttgttcctgatggcatgtaaatctagattcacttctagctggaaggaggcaggccagaaattcagagttgtaggtccttggcctgggtggatgtgctacaacatgaaccataaacctccatcacttatcttggcggatagaaaattggaactttggaggaaagtttcgcatcaagcactcagacccaataaatactcccactccttgcagagctaccgaacattctgcactccatttatcaggctacccaaggatgcttggaatgtgctggccggagccaccatcagcacttgctgatgactctttgtggtaccgccactcactttctgtactgtgttctttcttcttccttctcttttgttcttctgcccagcgacacacttgtgcagactgacttggtgccttggtgcctgttatggactgaatgctcgtgtcctcccacattcatatgtcaaagcacaatccccaatgtgatggtatttggagatggggcctctggggggtgatcaggtttagctgttgtaaaggtgagccctccgcgtctggattagtgcccttataaaaagagacacaagcgagctttctcattctccttccaccatgttaagatacaatgagaagacggccatctatgggggctccagttgacagccccagttgagcatccactgtcgtaggagtgaaccatcctggacagtccaacccagtcagctcccaggtgacttcggctgttccagtgcccagccacaccttgtgatgcagaatgcccagtcaactcacagaactcaatccaacgccagcgcccggcccgcacagcacggaatcccggggaaggcggagggcggggtccgaggccccgc

SEQ ID NO: 13012 - RNA, 3908 nt, Homo sapiens
  source 1..3908: mol_type = other RNA
gctgggattacaggcatgagccaccaatcccagcctgaaaagccttttattgggatgtcttaacaagggatcataaatcagatttcaatttctaaatgtttgccctggctgcaatgtgggtaatgtttatgggggtgggtggtgggcaaggaagaggacaaaaatattcaataggacccatagtccatataaaataatgctgcctttgataaagcccctgtgacattttttattgaccttacacacataagcacactcatgtgtcacttaacaaggatacattctgagaaatgcatccttaggtgatttcaccattttctgagcatcaaagtgtacttacccaacctacatggtatagcctactacacacctatgctatatggtgtggcctattgctcctaggctccaaacctgtatagcacgtgattgaactgaaaactttaggcaatcataacacaatgggaagtatttgtgtacctaaacatatctaaatattaaataaaaaggtatagtaaaaatagggtaatcttacgggaccatcatcatatatgtggttcgttgttgaccgaaacattattacgtagtacatgactgtacctggtattttcagaatggatttatattagacagggttttccagagagacaaaacatagatggatggatggatagacagagatgagaggggattgattaggggaatcagctcacacaatttggaaactgagaagtcccatgccaggcatttgcaagctggagacccagggcagctggtagtgtggctcagtcccagctgaaggcctcagaattagggaagccgatggtgttactctcagtccaagacagcaggtctgagaacccagggaagcaacggttcagatcctggagtccaaaagctgaagaacttgggaattctgcttccaaaagcaggagaagaagggtgccccagctccagaagagagagaaaaaaattgtctctcctctgcctttttgttctatctgggccatcagccaattagatggtgccacccacactgtgtgagggcagatcttcctcactcagtccactgcttcaaatgccaatctcctccagaaacacgctcacagacacacccagaaataatgctttaccagctatctgtgtatcccctgatccagtcaagttgacacctaaaattaaccatcacaggatttctctattgcttggcagagttccaacatttcagactttctaatgtcttaaagtagtacttttaataaatggatgtatcgttttactcttctaggagctaaggactggctcaattgactataaagaatcgagaatgtcagctgaccaggcaaccaggagacgctttcctgacttccactatgcacgtgggctgcataattgtgtctgtgaagtaatgaagaacgtgcttgctctgtaacatccaaacgcgtggccaccattcacagatagtgtcctttgggaaaggtgtgggtatagatggggaatggtcagtcctatgaatatggggctataagacagcaaggctagaaagtatctgtgctttcattttttaattttatctattttttttttttttttgcactaatggtttgcattcacattgaggaactgagactgttttcagacttttggcctactgatgaccttatgttcataaaaggatagaagtataataagttgtttaatataaaacatactgaaattttattttctgtctccttggatataaagtttccacttatcttgggtttaagtacctactcctccacagagagggaccttgtgcatgtagattgatattctcaggatgaaagcagtacctactacaactaggaactcacagaacaggaagacgatgcttgttcctgatggcatgtaaatctagattcacttctagctggaaggaggcaggccagaaattcagagttgtaggtccttggcctgggtggatgtgctacaacatgaaccataaacctccatcacttatcttggcggatagaaaattggaactttggaggaaagtttcgcatcaagcactcagacccaataaatactcccactccttgcagagctaccgaacattctgcactccatttatcaggctacccaaggatgcttggaatgtgctggccggagccaccatcagcacttgctgatgactctttgtggtaccgccactcactttctgtactgtgttctttcttcttccttctcttttgttcttctgcccagcgacacacttgtgcagactgacttggtgccttggtgcctgttatggactgaatgctcgtgtcctcccacattcatatgtcaaagcacaatccccaatgtgatggtatttggagatggggcctctggggggtgatcaggtttagctgttgtaaaggtgagccctccgcgtctggattagtgcccttataaaaagagacacaagcgagctttctcattctccttccaccatgttaagatacaatgagaagacggccatctggaaaacaggaagcaggccttcacctgctgtaggcaatcataacacaatgagaagtattgtgttggcactatctggtccaggagcagctggacctcccagaaagacatggggtcagcctccacctggatcctgaacttcccagcctccataagcatgagaaataaatgtctgttgcttaagccatccagcctatggtaactttttatagcagcctgaagctactaagatggtgccaagactgtgagatggcactagaagagagagaataaaaacacaggctcttaagtggttcaaatcctggctctgccacttgtccattatgtggtttttgggcaaagctgaatctttctgtgcctcagttcccaatctggaaaatgagacgtctattctatcagggtagggatgagataagatcatgtgttcaattagatgggatcaaacacatggtagaggaacttaatacatctttattgttattatagctatgtcactgaaagaattgggttaaataaaatgcaatctctcggccgggcgcagtggctcacacctgtaatcccagcactttgggaggccaaggtgggtggatcatgaggtcaggagttcgagaccagcctggccaagatggtgaaaccctgtctctactaaaaatacgaaaattagccgggcgtggcaggcacctgtaatcccagttacccgggaggctgaggcagaagaatcgcttgaacccgggagcggaggttgcagtgagccgagatcgctgcactctagcctgggtgacacagcaaaactctgtctcaaaaaaaaaaaaaaaaaaaaaaatgcaatctctcaccagaagttgaaaatctagcctgtgagataaagagacacttaattgtaatacgtggcgcttggcaaaaggtgacaaatactattatataatcagtatatggaaaaaacaccatgaaagctgcagtagatcaactagaactgcaaattccttatcactgctttcatcaagagctggagtctagttcccctcctccttgaaacagtgacctgttgacaaacagaatgaggctgaaacaactctgggtgtcttgtaaggcaaaaccatgaggaaccttgcagctgcttcctgattctcatgcggcactccctcttggaacagagctgccatgctgggagatgttacctatgggggctccagttgacagccccagttgagcatccactgtcgtaggagtgaaccatcctggacagtccaacccagtcagctcccaggtgacttcggctgttccagtgcccagccacaccttgtgatgcagaatgcccagtcaactcacagaactcaatccaacgccagcgcccggcccgcacagcacggaatcccggggaaggcggagggcggggtccgaggccccgc

SEQ ID NO: 13013 - RNA, 1498 nt, Homo sapiens
  source 1..1498: mol_type = other RNA
gctgggattacaggcatgagccaccacacacagctgtggcatgtttaatatccatagtatggtgcttcttttaaatattgcatattttacttagtcagtttatggttgtgcattttataatttttgttattgtaaaaaaacttacaacacacgcctgtaagcccagcagtttgggaggccaagaagggcggatcatttgaggtcagaagtttgagaccagcctggccaacatggtgaaaccctgtctgtactaaaaatacaaaaattagctgggtgtgttggcgtgcgcctgtaatcccagctactcgggatgcggaggcaggagaatcacttgaactcaggaggcagaggttgcaggatggtaccactgtacttcagcctgggcaacaagagcgaaactgtgtctcctgtctcaaattaaacaaaaacaaaaaaaaaacttgcaacaaaacttttgggaatacatatttttgtgggcatgcttcatttccttagtaggtaatgtctaataaattaatagaattttttggggcttcaagtaagttttgccagattgctttctcagattacataatttttgttttcaacagggaagtttgatggtgcccatttcaaaagtggtcgctttaaactgcttgtgctcgtgggcaggggctggttatcttggctctggagccagcatcctcggtggtatagaccccactgctgtggccttcgctgttttcatgctcacctcgaagctttttttctctggcacagcccttctctgcaggacctcaaagtggccagcagtcaaggcctccacagcgggctctggggattagcaccttcactttgttgcttcttaaactcctatttgcttttatgtttctttaaagaactcaaaatgagttgcagcagtgggaggcggctccaagtcactgcacgtcttccttggtgtccctgaggtctcaagagctctgtcatcaggctctgggcttctcagcgcatcgaggcccctcagcgcggcagaggggtccacagccacgggtgctgggctcggtgttgttgccaacgttggtgcagcaagaggtgaggaagggtccgttagcgtctctgcggcagatggtggtcctggctgtcgtgcgccacggtcatgtacgtgaagcactgttcttagctgcttgcccatccctggtgggcctgtgaggacctgacgcaagtgccgggggcatgggagctgggagggagccacgcaacgtgggcttcatgtgcactacaccccttactcgggggccctgtgtccttgtaggtggtaacgtggaccctgctacgctgcggttaggagtaaagcggtaatggagacagacgtggaccctgccatgtcaggactgacagtgcagtggcaggtgaggggtggtaacccggtgtggaaatggaaacacaggaaggcactggcattctgggagcaggtgatagaaggccagggaggttttctggtggaagtgacatcttggtt

SEQ ID NO: 13014 - RNA, 1544 nt, Homo sapiens
  source 1..1544: mol_type = other RNA
gctgggattacaggcatgagccaccacacatggccgaaggttcttcttaagtagacattcagactcacaaggcacatcgcagttaacatcagaatcacttctgatgataatataagtgaagaatataagacaggaggcgcatatattaataccagcagagcagctcccagtgtgtctcttcagttggaacagttgttgcagtggtctacttgctgtccagaagccttccatgatggttactgggtcctctacctgtggccgcagaatgttaggtccaaaaacggttgccagattctggacactcatcttgttgacatttgagtatgcctgaacttcatccagaaacttgcagatgtatctgagcaggttgtaatttgcctgaggaaggttgctcacttgtttagccaactccagagtgccctccccctcgtccttggtgagcagctgggcgcagctgaggaagtcctcgtacctggcgaaggggaccacgggctcggggagctcccgcaggtacagcttcagcagggaggccaccgtgtgcacgtctgttgtgctgtcaaacagtggcttctccccacagtcgaaggaatcctgcaggtccctcaccaggttggcctggcctggcatgcggaacagcccctcctcagtgagcccgcgctcccggatgaagtccacacactgctccaccagcaggggcgccaggcgggggccatacttccgctcgtggtggactgtttcctctaggcgctgcccaaagatccctccgcccagcggggcccagatgactcggcggatggcctgcacccagtcctccatgtcacgctgggagctggccatgagcaggagcgcctcggggttggccggcaccttctcccgctccccggcaccacctgggctgatctcaaagaggtgcttccctgggtcctcggggccaggaggaagttcagtcacctgtgtcccttgtagagaaataaatccctggggcttgatctcatctttgtccttgtagtagaaaagctgatccccacgcagcacaaaccagcgctgctgccagttcttcatgatgctcctctgcttcttcagccagcccgccttcagcacggggcccagcctgtgagggcacggcatccgcccagggctccggctctgctcccccatcactaggcttttggagcgggccctcctggcctgcctgatctttgggctcagcatgttcttgcagccgtccggccagccccgcagggccgttcatgctgtcatccacttgcttttgctcgtcctcgcgcctagtcgcccctcatgtcctgctcgttcggggccccgtggccgctggcgtcacccgtcaggctccctcggctacctctcctggctccggacggacggctcgccttggactacataaacctcgatgcattatttatccatcccagaattaattcccatccaagcggaccattaaagcctcagtaatcactgctgatcaatcactggaccagggcggggcagtccctccgcctggcctgggcgcacgcgtggctgtccaa

SEQ ID NO: 13015 - RNA, 1249 nt, Homo sapiens
  source 1..1249: mol_type = other RNA
gctgggattacaggcatgagccaccacacatggccgaaggttcttcttaagtagacattcagactcacaaggcacatcgcagttaacatcagaatcacttctgatgataatataagtgaagaatataagacaggaggcgcatatattaataccagcagagcagctcccagtgtgtctcttcagttggaacagttgttgcagtggtctacttgctgtccagaagccttccatgatggttactgggtcctctacctgtggccgcagaatgttaggtccaaaaacggttgccagattctggacactcatcttgttgacatttgagtatgcctgaacttcatccagaaacttgcagatgtatctgagcaggttgtaatttgcctgaggaaggttgctcacttgtttagccaactccagagtgccctccccctcgtccttggtgagcagctgggcgcagctgaggaagtcctcgtacctggcgaaggggaccacgggctcggggagctcccgcaggtacagcttcagcagggaggccaccgtgtgcacgtctgttgtgctgtcaaacagtggcttctccccacagtcgaaggaatcctgcaggtccctcaccaggttggcctggcctggcatgcggaacagcccctcctcagtgagcccgcgctcccggatgaagtccacacactgctccaccagcaggggcgccaggcgggggccatacttccgctcgtggtggactgtttcctctaggcgctgcccaaagatccctccgcccagcggggcccagatgactcggcggatggcctgcacccagtcctccatgtcacgctgggagctggccatgagcaggagcgcctcggggttggccggcaccttctcccgctccccggcaccacctgggctgatctcaaagaggtgcttccctgggtcctcggggccaggaggaagttcagtcacctgtgtcccttgtagagaaataaatccctggggcttgatctcatctttgtccttgtagtagaaaagctgatccccacgcagcacaaaccagcgctgctgccagttcttcatgatgctcctctgcttcttcagccagcccgccttcagcacggggcccagcctgtgagggcacggcatccgcccagggctccggctctgctcccccatcactaggcttttggagcgggtgaaatatctggctgcaaacgtcctccttttgctggaagctgtcggcagcataatgaagctggcagtctgt

SEQ ID NO: 13016 - RNA, 1475 nt, Homo sapiens
  source 1..1475: mol_type = other RNA
gctgggattacaggcatgagccaccacacatggccgaaggttcttcttaagtagacattcagactcacaaggcacatcgcagttaacatcagaatcacttctgatgataatataagtgaagaatataagacaggaggcgcatatattaataccagcagagcagctcccagtgtgtctcttcagttggaacagttgttgcagtggtctacttgctgtccagaagccttccatgatggttactgggtcctctacctgtggccgcagaatgttaggtccaaaaacggttgccagattctggacactcatcttgttgacatttgagtatgcctgaacttcatccagaaacttgcagatgtatctgagcaggttgtaatttgcctgaggaaggttgctcacttgtttagccaactccagagtgccctccccctcgtccttggtgagcagctgggcgcagctgaggaagtcctcgtacctggcgaaggggaccacgggctcggggagctcccgcaggtacagcttcagcagggaggccaccgtgtgcacgtctgttgtgctgtcaaacagtggcttctccccacagtcgaaggaatcctgcaggtccctcaccaggttggcctggcctggcatgcggaacagcccctcctcagtgagcccgcgctcccggatgaagtccacacactgctccaccagcaggggcgccaggcgggggccatacttccgctcgtggtggactgtttcctctaggcgctgcccaaagatccctggaggcaagggttctagagggtgggcatgcgatctacgggcagtacctccgcccagcggggcccagatgactcggcggatggcctgcacccagtcctccatgtcacgctgggagctggccatgagcaggagcgcctcggggttggccggcaccttctcccgctccccggcaccacctgggctgatctcaaagaggtgcttccctgggtcctcggggccaggaggaagttcagtcacctgtgtcccttgtagagaaataaatccctggggcttgatctcatctttgtccttgtagtagaaaagctgatccccacgcagcacaaaccagcgctgctgccagttcttcatgatgctcctctgcttcttcagccagcccgccttcagcacggggcccagcctgtgagggcacggcatccgcccagggctccggctctgctcccccatcactaggcttttggagcgggtgaaatatctggctgcaaacgtcctccttttgctggaagctgtcggcagcataatgaagctggcagtctgtgcaaatttcttctgtatcctttttataaagaaccaaccacatcctcaagcagacaagctaattcctgttttccagtaacaggagatccacatctttctttgcagcaagttcaaaggcaggtcatacaccagctaagcgggcacagctgggcacagttcccggggcctgccgggcagcg

SEQ ID NO: 13017 - RNA, 1423 nt, Homo sapiens
  source 1..1423: mol_type = other RNA
gctgggattacaggcatgagccaccacacatggccgaaggttcttcttaagtagacattcagactcacaaggcacatcgcagttaacatcagaatcacttctgatgataatataagtgaagaatataagacaggaggcgcatatattaataccagcagagcagctcccagtgtgtctcttcagttggaacagttgttgcagtggtctacttgctgtccagaagccttccatgatggttactgggtcctctacctgtggccgcagaatgttaggtccaaaaacggttgccagattctggacactcatcttgttgacatttgagtatgcctgaacttcatccagaaacttgcagatgtatctgagcaggttgtaatttgcctgaggaaggttgctcacttgtttagccaactccagagtgccctggcgaaggggaccacgggctcggggagctcccgcaggtacagcttcagcagggaggccaccgtgtgcacgtctgttgtgctgtcaaacagtggcttctccccacagtcgaaggaatcctgcaggtccctcaccaggttggcctggcctggcatgcggaacagcccctcctcagtgagcccgcgctcccggatgaagtccacacactgctccaccagcaggggcgccaggcgggggccatacttccgctcgtggtggactgtttcctctaggcgctgcccaaagatccctggaggcaagggttctagagggtgggcatgcgatctacgggcagtacctccgcccagcggggcccagatgactcggcggatggcctgcacccagtcctccatgtcacgctgggagctggccatgagcaggagcgcctcggggttggccggcaccttctcccgctccccggcaccacctgggctgatctcaaagaggtgcttccctgggtcctcggggccaggaggaagttcagtcacctgtgtcccttgtagagaaataaatccctggggcttgatctcatctttgtccttgtagtagaaaagctgatccccacgcagcacaaaccagcgctgctgccagttcttcatgatgctcctctgcttcttcagccagcccgccttcagcacggggcccagcctgtgagggcacggcatccgcccagggctccggctctgctcccccatcactaggcttttggagcgggtgaaatatctggctgcaaacgtcctccttttgctggaagctgtcggcagcataatgaagctggcagtctgtgcaaatttcttctgtatcctttttataaagaaccaaccacatcctcaagcagacaagctaattcctgttttccagtaacaggagatccacatctttctttgcagcaagttcaaaggcaggtcatacaccagctaagcgggcacagctgggcacagttcccggggcctgccgggcagcg

SEQ ID NO: 13018 - RNA, 2336 nt, Homo sapiens
  source 1..2336: mol_type = other RNA
gctgggattacaggcatgagccaccacaccaagccaatattcttagtcatatacaagagggcctgaggcagatccagatgtagggtgctcatctctgagaaggcagtgggtggaggaagttcagtactctaacccccaggagatgcagggccccccagtttcatgcccttccctttgcacaatgctttgcacttagagttgagcccagccagcttcctaggagtatggggagatgttgtgagtgggacccccgagatgactgcatggcacttcatagctggcatagctgtcctggttatctatggctgcataacaaatcaactatatacctaatggcacaaaataattttattatgtgcccagattctgtgggtcagcagttcagacagagcacagcaggagagatttgtctctattccatgatttctgggatttcaggaaaaactaaaatagctggggatgttagatggctaagctcagctgggactgttgactggagcacctagacatggcccctccatgtggcttgggcttcctcacaacatggcagcttcaggacagtgaatcttcctacttctttacatggtggctcagggctccaagagtgagtgttccagcaaacaaagtataatttgcaggggcatggtctttactcacttagggtctcttctgccataccctatgcaaagtgctggaattacaggcatgagccaccgtgcctggcctgtggccatgttttaacaccaccacaattgccatgggttgccaggcagcctggcagaggaacactgcaaggacccgtcccttcatggcagattcagaaaggctgaaaggcgttatggtcagtcagggaagacccaggagccactcaggcccacacagacctctctgtgtgccactggcctcttgcacccctcctttgactgtgacgttctcccctggagggatcaagaggtcaaaccaggcactcagaaaggcaagggccatagtagggtgaccttgagtgagccacatgatgtctgggagctttgcattccttgcctgcatcatggcagatgtttcctctctcccacggttctggggaagaacagaggagagaatgtatatgaaacccattcacccagtaggttcctggccaaagcaggtttccttccaaggggaatggggtggggcgggggtgccacaggcagggagaagatctgagggcctgactcactgggttctctcccagggacttaaccagggtggcgtgtctgcacttgaagctgcagcaggcacctctcaggcctgtggctcccagctctaattacagatttctggacatgtttcctgtttgggagctggcagtgtccccgcagaggatccacagataatgagcagctggcttcagaggctccatccatggggcactgacctgggagcaggcccaagcaggcccgcctcagacagcagaaggccctcaaaggtcatctggtctcaattcttccccacatcacactcacacaggaccaacaccgtgatcaccatgaccagtctctgcttgcacggttccagtgatgggcagctcaccacttcacagccagtctgctaatctctagacatcactcaagacagcactggaagcacttcccaaatcagtttgtcctttaacttctagctattgatccccaggtccaccaagaacaatgaaacatggaacagaagaagggcgcagaccctgggatcaagaagaactggctttggttccaatcttagtttttacgcttgcagtcttggtctctttgatcctcaatattcttctctccagagatgttaatgttctagggtggggcctgagatgttgcacttctaaccagctcccagctgtggctgaagctgttgctccacaggccacactttgagtgttgtggaagaaagcagacagtcaacttacaacaccttcaatattcaggtcaggcactaacttgctgcatggccttaaacatgtcctttctgttttctgggtcttatcttcccatctgtaaaacaaggtagatggattaggtcttgcctagagaaggaactgacattacctgagccactgatatgtttatttattaacttttctctccaaaatatttgattgagcaattcctatgaaccaggacctgatctatagcactgcacaggagagatgaaacaaagctcatgcctcgtggagctggccccatgctttgcacgaaatgcctgattcctatgatctcatttagcctttactacagtcacccacaggagttgggtgccatcatccttgctttacagataagaaaactgaggcatcggcagggtgcggtggc

SEQ ID NO: 13019 - RNA, 782 nt, Homo sapiens
  source 1..782: mol_type = other RNA
gctgggattacaggcatgagccaccacaccagctgcttctattttcttaaaggcagatagtacctaatattacaattcttctgaagcattagtctgtttgttacagcattgtctatgacaggaagatcatcaacaacaacaaaaaactgcagatgaccttgtcttcacatagcagagggcagagaaagatcacttccttggtgtctcttcttataagggaactaatcccattcatgagggctcttctcatggcccaattccttccaaaggctccactcactcgcattgtgtcaccgccaccaccgtacgtccccgctccgaggtggagggcggcgcggggtagaggagaagatagtgcgtctagcctatgtggccgcgcttgcctatgtggccgcgcttgcctggctgggtctgattgagggagccccggggcgcggcaagtcccggctcgctgcagccaggagctctgtctcctgaagatacccgcgccgagggcacagcttactccgccagacaagccaaccatggagatgttgcctggactctccatcctggttctcttagacaatgctcgggaagctggatgctccatattcttcaggagatttctccctttttcccccagctagcttgtgaggacaggggaaaggcttgaggaaaaataaatagaccattttgcattagccctttctgttaaaacttgcacctctctaattttttctccctcacctctgcagaaggcagagtacagcttccgtgacagctccaaacaattaaacttc

SEQ ID NO: 13020 - RNA, 2161 nt, Homo sapiens
  source 1..2161: mol_type = other RNA
gctgggattacaggcatgagccaccacaccaggctaatgctccttcttgacttaagtctggtcaatgggcaactgttgcttataaccaatgaattcttaaaaaattctcaaaaattctaaaaattcttggcatccccattttctctcctcctatgtaccagccctttaaatttggatgctttccccaaacaagctttcaaagctaccgaaatcctccatgccactggctccagtgggcgatcctcagcctaggtctggattcctatcgatcacctcttcctttggctttcaaccactctccagatgatgacaaaatccttgccagggtcctgtgcagggtggcccctcccaacgtcccctctgtcagtactcgccgcgctccgcctgttctgcctgctctggccccatcggctctgtctctgtctctccctcccgattgggatgcgtcctcctgccacagcacgcgcatgtgctgctcccactccctggacgttccttgctcctgactcattagtcacttttccagcaagccttccctggtaacctcttccagccccaggactcaatgctttctttagattctgctgtggcagcaagtacctcaccttcactgctcttgtcataggtgacactttctagttgtgtgattctgtagctattcatctattccctacattatagcagaagcttggggaggtgttaggtgtctgactagaatgcagagccacatagggccatgcagtgtctatgtcccctccacacggacatctggctttgagccaaaggatgacgtctgcccatttcttgtttttgccttcacttagtcacctagttttgttgtgtgaacaaatgaatcaatgagtgaattctccaggaaccaaccctggttatcaggcgctcattgtggaactgcttcaggcccacagcccacaagtgggtccacagaactcagaccctgagagacacaagacaccatcactgcccaatatggcaccaggccctggcacataggtggagtgtggtcacagacagggcactgtactggctgctagggccatgagctggagtcccagctctgccctgatcacctgctgcccttggcaaatcccttccaagccctgtgtcggtttgcctggctgtgaaactgggacgctgatcaaggtgtctcctcgcccttcctgctcagccattggtgcctcagtgattctaggagaacattagctacaaccgaccacaagagagatccctgaggattcaggagcatagagccaaggaggtgggggtgtccagccggagacgtaccagccggagacctacctcagccaagggcttgacatcacctttcttcaccagaacagaagtgagggccacgccactctcagaaatggcccggtggaagaggttcttggccaatggagacaaaacaagaacagagacactttctcctcccactgaccctccaaagatggtcacagagcctgggttccctccaaagctggcaatgttgtcctggacccagtgcagggcagccagctggtccaggtgaccccagttccccgggctgtgttcatcccctgtgctgaagaatccccagatgcccaggcgatattgaatggtcaccaccaccacgttttcatgggcagcaagggccagcccatcgtaggttgatgccgcacccaccatcagcccccctccgtggatccacaccatcaccggcagcctgtttttcttggtcaagtcagcaggagtgtaaatattgaggtaaagacagtcttcagaaagcttgagaggaatgttctcttttcagtttgtaaatagctctgagattaactgccccgccttgggatcttgggtgaacataggagggtacgaggtggcattcttcacaaagttccatggctctgcaggctgtggtagagtaaacctcaggggtccaagaggcggcttggcaaaagggattcccaggaaaacggccacaggctgtgcaaatccttctaagctgacgaacttccccaacactttgccatgcagggtgtccaccaaaggtggcgaggacagatgccctgcccaagccgcggaagcagcgagagtggccaggacaagagcagggagccacatcctggaagggcgacagttccgggggcctgcgaggtctccgtgc

SEQ ID NO: 13021 - RNA, 503 nt, Homo sapiens
  source 1..503: mol_type = other RNA
gctgggattacaggcatgagccaccacaccagtaaattttgaataccaaccctttctgtgcctgagtatcctgccaatcacaatgtgttataataagcaccctcaagcagggttcatagtgcatttgttgttttatccagattattatacaaaagtgaatctattagcaaaaagtgatacccagtggcaagtggaggactcctgtaatgcacacgatcctcacgacgatggtcccgacttcgcgactcactaccatgtcgacgatcccagctacggctacggtgacgacactgccgacctggacttcggctccgactatttctccgtctataccgatcccgatctcgactacgacagttccgggtccccgcaggggggtcccggttctctccgttcctttgagtatgttgtggggagtggagctcggatagttcctagagtctaggcaagaaaagcagcactgcaggtacagagcctcctcttcccgcaaaatggcggcagct

SEQ ID NO: 13022 - RNA, 581 nt, Homo sapiens
  source 1..581: mol_type = other RNA
gctgggattacaggcatgagccaccacaccagtaaattttgaataccaaccctttctgtgcctgagtatcctgccaatcacaatgtgttataataagcaccctcaagcagggttcatagtgcatttgttgttttatccagattattatacaaaagtgaatctattagcaaaaagtgatacccagtggcaagtggaggactcctgtaatgcacacgatcctcacgacgatggtcccgacttcgcgactcactaccatgtcgacgatcccagctacggctacggtgacgacactgccgacctggacttcggctccgactatttctccgtctataccgatcccgatctcgactacgactcttcttttttatagggagcttccagcatggcctcaatcactatgtcaaagtcatcagatgccatcctgtcagatcagttccgggtccccgcaggggggtcccggttctctccgttcctttgagtatgttgtggggagtggagctcggatagttcctagagtctaggcaagaaaagcagcactgcaggtacagagcctcctcttcccgcaaaatggcggcagctct

SEQ ID NO: 13023 - RNA, 4213 nt, Homo sapiens
  source 1..4213: mol_type = other RNA
gctgggattacaggcatgagccaccacacccaaccacggactgtgcttttaagagtcggtctccaggttccacctccatcccttgaacgtgggccctctgaactcagcagcaccttgtcctgcttgatgcctcctaaccctccccaaactccaaccatctgcattacatctactggccatcccagtaaccagagcctaagtacattttgaagaatatagtcgaggcctcacaccctggctaaggagtaagctggtttttgggctgtgcagagccacgtcctactaactgtgctttaacatcccctgcagagctaagtcttagccaccaaggacaagaccaagcaagggggggtgggggagtggggaagtggcctatttaagacgaacctatcgatacccagagttcactggttcagttacttgctttcactagtttttagctttttaataaataagtagcaatgttctgggatgactcctggcagctgcgaaccctcattttagcaatagtctgcacagctccttcagcctgttggtctggctgaaatgcctctctccccactccggcttttgtctggcttgggccctcctggtcatcttgtcctaggcagcctgtggaggtctatgaaagccacacctccagccagctgatgctgcgcccgagtcacatggcaggcgccacaggcaaccccggtgctcacagggcatcagggagcacagcagcatctgccatggaggcggcttataagttagtgacatacagttatctcacttggtggcagtcacctttaggctaaagcatccaaatcccaggaagaaaatactcacgttagttgatggatgttggaaggcattggaggaaaacaccacagttaggactgttaatgacttacacactgttggtgagactcatctcgaacatgcgcaaacattgatcgtagtaacggtggtggtggttagtgccacattcaaataaaaatagttctatacaatatgttcatttggtcatgtgctatttacagattttacaaaacacacacatacacacacatacacacttgcccttatgttctctataccaggccagcagaaacttgcataaaatgtacatcacagatgacaattagtgcctgtacattaagaatacaattcctatgactacctacacagcagagcaggagccttcttcccctcaagcagagtacaactaaagttctgagctaagaacaggttccaggtagttgcgggccacaaacttgagcgtctcatccatgagaatcacgggcaaggagattttcagcaccatcagccactgggtcacgttcagcggtgtgatctggaagatgagtggcaagggttcgacatagaggatcaggaagtggagtgacatggacaggcagatggagcccacgagccagatgttctcccaggggggcatcctcagcaaggactggttttcggacaagctgttgagggcgttacacatttctatagttactagaacagagagcgccattgtcatcgggtatggggattcaaagattgcacaatccacgccttcaaagtccgggttgtcctctttacactgtaggaaatgactcagctggtagaaggacactcttggaccaccgtcagcagcaatgaaccaccatgcagcagcacccacggtagcagcgccgacgtaacagccaatagccaagtaacggaaaaagagccacccgctgatcaatggttcctttgggttccggggaggtttattcatgatgtccagatcaggagggttgaaccccagtgcagtggcaggcaggccatctgtcaccagattgacccagagcagctgaacaggaatcaaagcctcgggaaatccaagggctgctgtcaggaaaatacagacaacttccccgacgttggacgagatgaggtagcggatgaactgtttcatgttgttgtagattgcccgcccctcctcaacggcagccacaatggtggagaagttgtcatccgccaggaccatctcagaggcggttttagccaccgcagtgccagagcccatagcaatgccaatctcggctttcttcagagcaggagcatcgttcacgccatcgccagtcatagctgtaatctcatcaaaagactgaagaaattctacgattttagacttgtgggagggttcaactcgagcaaaacagcgggcgttcaggcaggcgtctcgctgggcggaggggttgagttcatcaaactcccggcctgtgaaagcttttgacgtcacgtcctcatcctgcccgaagatgccgatgcggcgacagatggccacagcagtgcccttgttgtccccagtgatcatgatgacccggatgcctgcttgccggcacagcttcacggaggaggccacctcgattctcggaggatccagcatgcccacgcagccaacgaaggtcagattggtctcatatttaataaagttggcagagtcctcaaggtgcatttcttctcttctcagtgggttgtcatgagtggccagggccaggcatcgcagtgtgtcgctgccactaccccactctcgaatgacagacatgatcttctgtttgactccagaggtcataggaaccttagtacttccaactcgaatgtgggtgcacctgtcaatgacaccttcaggagcacccttcacaaacatcttgctcattgatgtcctgcttggtttatttggtgtacagtaaaccgacattgactttctgtcacgtgaaaactctagagtgaattcctttttcatcagctgtttaatgactgagttgcaggcatttgcacgttctattttagaaagacccttcaattcggtatcaaatacattcatcttctctactaggcaagtgagagcagtctctgtagcttctccaactttttcatacacaccctttgcctcattgtaatccaaagcagagtcattacaaagagcacaaattgttgctaattctaccagaccatcatactggtgacaattcactggtttatcatctttatgcacttctccaataggtgcataagttgatccagttatggtaaactcattaagggaacaagtatcaccttccactctgtccagaatgaacatcctgcagactgacatctggtttgttgtaagtgtaccagtcttgtctgagcagataacagaagtacaaccaagggtttccacagacgggaggcttcgaacaatggcatttttctttgccattctgcgagttccaagagccaggcaggtggtgatgactgcaggcagaccttcaggaatggctgctacagccagggccactgcaattttaaagtagtaaatagcacctctgatccaggaccctccatgaaccgggtcattgaagtgcccaatatttatgatccagactgcaatgcaaataagggagatgactttggaaagctgttccccaaattcatctagtttttgctgaaggggtgttctctcctgttctgttgccaccatttcatcccggatcttgccaatttcggtgttaactccagttgctaccaccactcccatagctttcccagcagcaatgtttgtaccagaaaacagcatgttctttttatcttggttgacagctcgtgggtcagggacgggatcagtgtgcttgatgacagagacagattcacctgtgagaattgactggtcaactcttagtgtggtagatttgatggaagttaaccttatatcagcaggaactttgtcaccaacagcaatttctacaatatcaccaggaactatgtctttagctttaatccgctgcacactctttctgtcctgtcgatacactttgcccatttcaggctcatattccttaagggcttcgatggcattttcagcatttctttcctgccatacacccacaattgcattggctactaatatgagtaaaattacaaaaggttctacaaaggctgtaattgtttcttcaccttcttcaaaccaagccaaaacaaaagatatacatgctgccagtaataaaatcctaactagcaagtcttcaaactgctcaatcacaagttccagcaaggtttttccttcttcagccggtaactcgttggagccccatctctccttaagcttcttgacctgttccaggctcagccccgtactctcgttgacgccgaagtggcccagcacctcctccaccgtcttggtgtgcgcgttctccatggcttc

SEQ ID NO: 13024 - RNA, 5821 nt, Homo sapiens
  source 1..5821: mol_type = other RNA
gctgggattacaggcatgagccaccacacccaaccacggactgtgcttttaagagtcggtctccaggttccacctccatcccttgaacgtgggccctctgaactcagcagcaccttgtcctgcttgatgcctcctaaccctccccaaactccaaccatctgcattacatctactggccatcccagtaaccagagcctaagtacattttgaagaatatagtcgaggcctcacaccctggctaaggagtaagctggtttttgggctgtgcagagccacgtcctactaactgtgctttaacatcccctgcagagctaagtcttagccaccaaggacaagaccaagcaagggggggtgggggagtggggaagtggcctatttaagacgaacctatcgatacccagagttcactggttcagttacttgctttcactagtttttagctttttaataaataagtagcaatgttctgggatgactcctggcagctgcgaaccctcattttagcaatagtctgcacagctccttcagcctgttggtctggctgaaatgcctctctccccactccggcttttgtctggcttgggccctcctggtcatcttgtcctaggcagcctgtggaggtctatgaaagccacacctccagccagctgatgctgcgcccgagtcacatggcaggcgccacaggcaaccccggtgctcacagggcatcagggagcacagcagcatctgccatggaggcggcttataagttagtgacatacagttatctcacttggtggcagtcacctttaggctaaagcatccaaatcccaggaagaaaatactcacgttagttgatggatgttggaaggcattggaggaaaacaccacagttaggactgttaatgacttacacactgttggtgagactcatctcgaacatgcgcaaacattgatcgtagtaacggtggtggtggttagtgccacattcaaataaaaatagttctatacaatatgttcatttggtcatgtgctatttacagattttacaaaacacacacatacacacacatacacacttgcccttatgttctctataccaggccagcagaaacttgcataaaatgtacatcacagatgacaattagtgcctgtacattaagaatacaattcctatgactacctacacagcagagcaggagccttcttcccctcaagcagagtacaactaaagttctgagctaagaactggagagaaagttggacatgtctgttagtcccaggtaagccacttacgagttaaagacaagacagttatttttctctgtccatttaaaatgttttatttttttaaaactagatgacgtgccactgaaataggcaatgttggcaaaacaatgtctgttacaataaaatacattagacatttaaataaataaccttaaaaactatgtgaagggacataaacccagtcgattgaatctggaacaatgttttctgcacaagcgagtacaggcatacctctcgttaaaactgatgtaaacagaacgaaccatcacaatcctaaagaagaagccaagcggggcgggggtaaggtggggagaggtggggtggggtggggtgaacggaggccaaagtgggtgagggaagtagcaaaccaaaacaatactgactgaggtagcaagactctgctcagtgcagaaaaattggcttatgaataaaaattagactgtgatatcaaattaaatccggatcatcatgcaaaagacacaatacatgctatttagttttagaaaaaaaaccacacacattcatttcctaaaatctgctgccaattaatttgctgacaatgtctgctggctcaactattttttttatacaaggatgagtattaaacagaacactgtacatgctttttcatctacaaaaaaatatttgcataaaatagtgttagttctctgtacatgtcaatggacactttaattatgtgtataaaaaaggaaaatcttgccccactggagtcagaaaaagcaaaacaaaatctagagtatgaaacctccatcaccagccagtatgttcatgtgaaaattcagcagaaatagacagttgctttaaacaataaaaaaattaattgattaagttaaacatcttctttatggaaaactgtcagtcaagaccagaacatatcgctaaagttagtgtctgtgctatagacccagatcaccaggggcattatgagcagcacaaacggccaggaaatcccatcggtgcatgccgagaacgagcaggatttggtggcaggctgcacacactctttaccaggttccaggtagttgcgggccacaaacttgagcgtctcatccatgagaatcacgggcaaggagattttcagcaccatcagccactgggtcacgttcagcggtgtgatctggaagatgagtggcaagggttcgacatagaggatcaggaagtggagtgacatggacaggcagatggagcccacgagccagatgttctcccaggggggcatcctcagcaaggactggttttcggacaagctgttgagggcgttacacatttctatagttactagaacagagagcgccattgtcatcgggtatggggattcaaagattgcacaatccacgccttcaaagtccgggttgtcctctttacactgtaggaaatgactcagctggtagaaggacactcttggaccaccgtcagcagcaatgaaccaccatgcagcagcacccacggtagcagcgccgacgtaacagccaatagccaagtaacggaaaaagagccacccgctgatcaatggttcctttgggttccggggaggtttattcatgatgtccagatcaggagggttgaaccccagtgcagtggcaggcaggccatctgtcaccagattgacccagagcagctgaacaggaatcaaagcctcgggaaatccaagggctgctgtcaggaaaatacagacaacttccccgacgttggacgagatgaggtagcggatgaactgtttcatgttgttgtagattgcccgcccctcctcaacggcagccacaatggtggagaagttgtcatccgccaggaccatctcagaggcggttttagccaccgcagtgccagagcccatagcaatgccaatctcggctttcttcagagcaggagcatcgttcacgccatcgccagtcatagctgtaatctcatcaaaagactgaagaaattctacgattttagacttgtgggagggttcaactcgagcaaaacagcgggcgttcaggcaggcgtctcgctgggcggaggggttgagttcatcaaactcccggcctgtgaaagcttttgacgtcacgtcctcatcctgcccgaagatgccgatgcggcgacagatggccacagcagtgcccttgttgtccccagtgatcatgatgacccggatgcctgcttgccggcacagcttcacggaggaggccacctcgattctcggaggatccagcatgcccacgcagccaacgaaggtcagattggtctcatatttaataaagttggcagagtcctcaaggtgcatttcttctcttctcagtgggttgtcatgagtggccagggccaggcatcgcagtgtgtcgctgccactaccccactctcgaatgacagacatgatcttctgtttgactccagaggtcataggaaccttagtacttccaactcgaatgtgggtgcacctgtcaatgacaccttcaggagcacccttcacaaacatcttgctcattgatgtcctgcttggtttatttggtgtacagtaaaccgacattgactttctgtcacgtgaaaactctagagtgaattcctttttcatcagctgtttaatgactgagttgcaggcatttgcacgttctattttagaaagacccttcaattcggtatcaaatacattcatcttctctactaggcaagtgagagcagtctctgtagcttctccaactttttcatacacaccctttgcctcattgtaatccaaagcagagtcattacaaagagcacaaattgttgctaattctaccagaccatcatactggtgacaattcactggtttatcatctttatgcacttctccaataggtgcataagttgatccagttatggtaaactcattaagggaacaagtatcaccttccactctgtccagaatgaacatcctgcagactgacatctggtttgttgtaagtgtaccagtcttgtctgagcagataacagaagtacaaccaagggtttccacagacgggaggcttcgaacaatggcatttttctttgccattctgcgagttccaagagccaggcaggtggtgatgactgcaggcagaccttcaggaatggctgctacagccagggccactgcaattttaaagtagtaaatagcacctctgatccaggaccctccatgaaccgggtcattgaagtgcccaatatttatgatccagactgcaatgcaaataagggagatgactttggaaagctgttccccaaattcatctagtttttgctgaaggggtgttctctcctgttctgttgccaccatttcatcccggatcttgccaatttcggtgttaactccagttgctaccaccactcccatagctttcccagcagcaatgtttgtaccagaaaacagcatgttctttttatcttggttgacagctcgtgggtcagggacgggatcagtgtgcttgatgacagagacagattcacctgtgagaattgactggtcaactcttagtgtggtagatttgatggaagttaaccttatatcagcaggaactttgtcaccaacagcaatttctacaatatcaccaggaactatgtctttagctttaatccgctgcacactctttctgtcctgtcgatacactttgcccatttcaggctcatattccttaagggcttcgatggcattttcagcatttctttcctgccatacacccacaattgcattggctactaatatgagtaaaattacaaaaggttctacaaaggctgtaattgtttcttcaccttcttcaaaccaagccaaaacaaaagatatacatgctgccagtaataaaatcctaactagcaagtcttcaaactgctcaatcacaagttccagcaaggtttttccttcttcagccggtaactcgttggagccccatctctccttaagcttcttgacctgttccaggctcagccccgtactctcgttgacgccgaagtggcccagcacctcctccaccgtcttggtgtgcgcgttctccatggcttcgggggcccggccggcctcgcctcccgtccccgcggcctcctcgcctccgcctcgcactccggccgcgggctcgtgccaccccgggagcccaggcgcggacgggctctcccctcctcctcttgcggccgcttccgcctcgccgggcgctgaatcaccccgcgccccctcccccagacaaccgcccctcgcgcggccccgagctccgcagggcgggttgggggctcctgacccaccctccctcccctcgccagaagggagggcctccctcgccctcagccgcccgccgggagggcaggccgcggcccccgagccccctccccgctctcttgaggcgatcagaggccccgcccgggccggaggagggggcgcccggcagaccactgagggcggaacgcggcgagggaggcgagccggcggggcggtgcgcggcgcgctcgcccgggtccctcagcgccgcacgcccgacagcggcggaggaaactgcggcgaaggaaaaggaggtggcgtcggggacggctccgcggcggctgctctaat

SEQ ID NO: 13025 - RNA, 3393 nt, Homo sapiens
  source 1..3393: mol_type = other RNA
gctgggattacaggcatgagccaccacacccagcaataattggtatctcttaaatctcattctagtttgctagaatcaagattactaaggagttgaaacaaaggtagaagaatccatactataatatcccaaattatgttttcaaagctaactcattcctttggttcaaaaagaaaaaaagttgcctccttttaaaatccaatattagtatggctgatggaaattaggccaaattataaacaaattataaacctacagtagcaaccataaaatttatgctgtactaggaaatgacagagctattcctagtttattatttagcatacagaaggtactccaaaaaatttaccggggcggggcgtggtggctcacgcctgtaatcccagcactttgggaagctgaggtgggtggattatttgaggtcaggagttagtgatcagcctggtcaacatggtgaaacctcgtctcttctaaaaatgtgaaaattagccgggcatggtggcatgagcctgtaatcccagctacttgggaggctgaggcaggagactctattgaacctggaaggcagaggttgcagcgagccaagatcccgccactgcactcctgcctgggagacagagcaaaactctgtggaaaaaagaagaaaaaaatttattgggtgaatgaaaagtgattttgcaaaattaggcatcacagaatgttagaagtcatccagtccaacttattcacaacaccccctcccctgcagtcccattttacagacaggaagctccaacctgtagtactcacagatgctgctgagattcatctccacccactcactggaagcaatcaattattttggggggggtgtgtgtgtgtgtgtgtctgtctgtctaaaaggtgtaaatgaggagtgacatttctacattgtttattctgtacttttccttggagttaatgcaacacctcctgtcgcttagattttaaaaggaaaaaggagaaatgtgtctagtcataaaggggttgccgttaggaagtcagacttcagactgtgcgtctaagagtagaatccacttctcaagagactgggaatgtaaaatgaccactcaggttagaatttccaactgacagccaggaggaaaacttactctaaagttttttttgcctagtttaaattgcattttaaatcactgtttaagctattacagtattactgtaaaaagtttcaaagtaatttttagtcattacctacactgaaatttgaaagtgaagtcaacagcatgctttattctaactgctgttaaaactcaaaactattttttttaacaaattacaatattcctcttagattttcttctggacacctatacttcttcctactgtgtccagtattctccagcacatgtacctttgtgtttctctgcccatgtacatacccctgaaagttcaacaaaaaaagctataaaatagcagagagaacccaaaatatttcttatactgccaagttccctttaaaccttgggcacttgctctactacatggttgtattaatgctcataactaagctttcgatgaattagaccaatgtgttctatgttctaaatgatatttagatatctgaatccttctgttatagccaacaataaaaaaagttattaaaaatgttgaaaagtataaaatagtaattataaattagcaaatacccaatttaaaaaagcagttttccttatacagtacaagcaacagtaatttgaatattattcactttcagccaccatttgccctagatgtactttaaagtttttaagcttgtgtttttggagtgaaaatgtatatggatacttattctaataatgtaattcaggtatcaaaaaatacatatgcatgttaaaatgtgatgacagctcatattatagcaactcataacaggtaagtattatttccagaataacattaagtcacttttgtagctctaagtcaatgctgcacaaatggacacttaagattaaggcatcattctgctctggagtagtgcttctgtgaatcccaggaactgtacaaaggctttccgttttaaaaaatatatcttctgttatacttcagttatttcattccactgatcattttcttgcaaatgaaaattgaaaataccagtctataatgttttcatacacctgatttgacgatgccttcttcagctccattctccagccactgagattcactgtccaacaagcggttttttgattcactaagtggtttgataggaaaaggttgatttgagccactactgtcatttgccaagttttctgctttctacctctgcagtttagatcttctggcatactcattctggtttgtaacagaagcttgttctggatccatccccacaaggcgagttggaaaactgcaaccatcacccaagcttgaaaatattggaagtagccaatatttcttttcatcaccaaagacttgtctccaatttttactgcatccaagagagaaaccatttccatcaggtccgtatgaaaacgtgggtgcgcggaatgattctattgttgttctattttttccaactagccagcagtggtagctgaaaagtgagaggacgctgatgaagaacattgcagacacaaagaaaagaaaaagtacgtggaattttgcacgtgtatctgtcagttcattcgtccaaaattttataaagtactctaaaactgttgcagccacgaaaaggcaatataatagggaatacaataaaaacagcaggaagaatttgtaattagaaaatcccacacagttattcacccaaggacagtgatgatccatcttaagaatacatgagtcacaggctgagcagtgatgcgcccgatcaggtttaatcagctgacatttttcacaatatctgatagtttttgaagctgatgtggtatagataggtaaagctcttgctgctcttctcaaaatttcttgttgtctttcttggctgaattctttttcataacgttccttttcagaattggacaagtagaactctttggagggggaagcgggagatgtgaaaattgtcatccaataggaccatacaaacataacaaagaacagatggaaagccacaaggtaaacaacggtctttccattttcttcatttccaaaaatagtaaacacgcagagctccaccacgtacgcgtagtaggaccagacgaccacgaaggtgatgaagagcaccggcacccagcccacgacgcgctggcagcagcgccacagcgtccagggcgccatgttccgctggcggctgccgagccccgcgtcccaccgttctggggagcgcgggagccccggcgacggtgactcggacgctccaggcggctgctggtccagctcccccgcctccgaggcaggacttgtgggagc

SEQ ID NO: 13026 - RNA, 3618 nt, Homo sapiens
  source 1..3618: mol_type = other RNA
gctgggattacaggcatgagccaccacacccagcaataattggtatctcttaaatctcattctagtttgctagaatcaagattactaaggagttgaaacaaaggtagaagaatccatactataatatcccaaattatgttttcaaagctaactcattcctttggttcaaaaagaaaaaaagttgcctccttttaaaatccaatattagtatggctgatggaaattaggccaaattataaacaaattataaacctacagtagcaaccataaaatttatgctgtactaggaaatgacagagctattcctagtttattatttagcatacagaaggtactccaaaaaatttaccggggcggggcgtggtggctcacgcctgtaatcccagcactttgggaagctgaggtgggtggattatttgaggtcaggagttagtgatcagcctggtcaacatggtgaaacctcgtctcttctaaaaatgtgaaaattagccgggcatggtggcatgagcctgtaatcccagctacttgggaggctgaggcaggagactctattgaacctggaaggcagaggttgcagcgagccaagatcccgccactgcactcctgcctgggagacagagcaaaactctgtggaaaaaagaagaaaaaaatttattgggtgaatgaaaagtgattttgcaaaattaggcatcacagaatgttagaagtcatccagtccaacttattcacaacaccccctcccctgcagtcccattttacagacaggaagctccaacctgtagtactcacagatgctgctgagattcatctccacccactcactggaagcaatcaattattttggggggggtgtgtgtgtgtgtgtgtctgtctgtctaaaaggtgtaaatgaggagtgacatttctacattgtttattctgtacttttccttggagttaatgcaacacctcctgtcgcttagattttaaaaggaaaaaggagaaatgtgtctagtcataaaggggttgccgttaggaagtcagacttcagactgtgcgtctaagagtagaatccacttctcaagagactgggaatgtaaaatgaccactcaggttagaatttccaactgacagccaggaggaaaacttactctaaagttttttttgcctagtttaaattgcattttaaatcactgtttaagctattacagtattactgtaaaaagtttcaaagtaatttttagtcattacctacactgaaatttgaaagtgaagtcaacagcatgctttattctaactgctgttaaaactcaaaactattttttttaacaaattacaatattcctcttagattttcttctggacacctatacttcttcctactgtgtccagtattctccagcacatgtacctttgtgtttctctgcccatgtacatacccctgaaagttcaacaaaaaaagctataaaatagcagagagaacccaaaatatttcttatactgccaagttccctttaaaccttgggcacttgctctactacatggttgtattaatgctcataactaagctttcgatgaattagaccaatgtgttctatgttctaaatgatatttagatatctgaatccttctgttatagccaacaataaaaaaagttattaaaaatgttgaaaagtataaaatagtaattataaattagcaaatacccaatttaaaaaagcagttttccttatacagtacaagcaacagtaatttgaatattattcactttcagccaccatttgccctagatgtactttaaagtttttaagcttgtgtttttggagtgaaaatgtatatggatacttattctaataatgtaattcaggtatcaaaaaatacatatgcatgttaaaatgtgatgacagctcatattatagcaactcataacaggtaagtattatttccagaataacattaagtcacttttgtagctctaagtcaatgctgcacaaatggacacttaagattaaggcatcattctgctctggagtagtgcttctgtgaatcccaggaactgtacaaaggctttccgttttaaaaaatatatcttctgttatacttcagttatttcattccactgatcattttcttgcaaatgaaaattgaaaataccagtctataatgttttcatacacctgatttgacgatgccttcttcagctccattctccagccactgagattcactgtccaacaagcggttttttgattcactaagtggtttgataggaaaaggttgatttgagccactactgtcatttgccaagttttctgctttctacctctgcagtttagatcttctggcatactcattctggtttgtaacagaagcttgttctggatccatccccacaaggcgagttggaaaactgcaaccatcacccaagcttgaaaatattggaagtagccaatatttcttttcatcaccaaagacttgtctccaatttttactgcatccaagagagaaaccatttccatcaggtccgtatgaaaacgtgggtgcgcggaatgattctggcagatatatggctgcagattgcaggtggattttaacttttttacaaaacactaccgtaaaaatccttattttgtgtcttggttatgttagcagatacatgaatatttcaatgataacatagcagtacttcttacatgtcaatagctcagtgagcaatgccaccattgctgtttagggaatgtttgtccaattacgtgaataccttacttttccccctattgttgttctattttttccaactagccagcagtggtagctgaaaagtgagaggacgctgatgaagaacattgcagacacaaagaaaagaaaaagtacgtggaattttgcacgtgtatctgtcagttcattcgtccaaaattttataaagtactctaaaactgttgcagccacgaaaaggcaatataatagggaatacaataaaaacagcaggaagaatttgtaattagaaaatcccacacagttattcacccaaggacagtgatgatccatcttaagaatacatgagtcacaggctgagcagtgatgcgcccgatcaggtttaatcagctgacatttttcacaatatctgatagtttttgaagctgatgtggtatagataggtaaagctcttgctgctcttctcaaaatttcttgttgtctttcttggctgaattctttttcataacgttccttttcagaattggacaagtagaactctttggagggggaagcgggagatgtgaaaattgtcatccaataggaccatacaaacataacaaagaacagatggaaagccacaaggtaaacaacggtctttccattttcttcatttccaaaaatagtaaacacgcagagctccaccacgtacgcgtagtaggaccagacgaccacgaaggtgatgaagagcaccggcacccagcccacgacgcgctggcagcagcgccacagcgtccagggcgccatgttccgctggcggctgccgagccccgcgtcccaccgttctggggagcgcgggagccccggcgacggtgactcggacgctccaggcggctgctggtccagctcccccgcctccgaggcaggacttgtgggagcaaaagt

SEQ ID NO: 13027 - RNA, 3330 nt, Homo sapiens
  source 1..3330: mol_type = other RNA
gctgggattacaggcatgagccaccacacccagcaataattggtatctcttaaatctcattctagtttgctagaatcaagattactaaggagttgaaacaaaggtagaagaatccatactataatatcccaaattatgttttcaaagctaactcattcctttggttcaaaaagaaaaaaagttgcctccttttaaaatccaatattagtatggctgatggaaattaggccaaattataaacaaattataaacctacagtagcaaccataaaatttatgctgtactaggaaatgacagagctattcctagtttattatttagcatacagaaggtactccaaaaaatttaccggggcggggcgtggtggctcacgcctgtaatcccagcactttgggaagctgaggtgggtggattatttgaggtcaggagttagtgatcagcctggtcaacatggtgaaacctcgtctcttctaaaaatgtgaaaattagccgggcatggtggcatgagcctgtaatcccagctacttgggaggctgaggcaggagactctattgaacctggaaggcagaggttgcagcgagccaagatcccgccactgcactcctgcctgggagacagagcaaaactctgtggaaaaaagaagaaaaaaatttattgggtgaatgaaaagtgattttgcaaaattaggcatcacagaatgttagaagtcatccagtccaacttattcacaacaccccctcccctgcagtcccattttacagacaggaagctccaacctgtagtactcacagatgctgctgagattcatctccacccactcactggaagcaatcaattattttggggggggtgtgtgtgtgtgtgtgtctgtctgtctaaaaggtgtaaatgaggagtgacatttctacattgtttattctgtacttttccttggagttaatgcaacacctcctgtcgcttagattttaaaaggaaaaaggagaaatgtgtctagtcataaaggggttgccgttaggaagtcagacttcagactgtgcgtctaagagtagaatccacttctcaagagactgggaatgtaaaatgaccactcaggttagaatttccaactgacagccaggaggaaaacttactctaaagttttttttgcctagtttaaattgcattttaaatcactgtttaagctattacagtattactgtaaaaagtttcaaagtaatttttagtcattacctacactgaaatttgaaagtgaagtcaacagcatgctttattctaactgctgttaaaactcaaaactattttttttaacaaattacaatattcctcttagattttcttctggacacctatacttcttcctactgtgtccagtattctccagcacatgtacctttgtgtttctctgcccatgtacatacccctgaaagttcaacaaaaaaagctataaaatagcagagagaacccaaaatatttcttatactgccaagttccctttaaaccttgggcacttgctctactacatggttgtattaatgctcataactaagctttcgatgaattagaccaatgtgttctatgttctaaatgatatttagatatctgaatccttctgttatagccaacaataaaaaaagttattaaaaatgttgaaaagtataaaatagtaattataaattagcaaatacccaatttaaaaaagcagttttccttatacagtacaagcaacagtaatttgaatattattcactttcagccaccatttgccctagatgtactttaaagtttttaagcttgtgtttttggagtgaaaatgtatatggatacttattctaataatgtaattcaggtatcaaaaaatacatatgcatgttaaaatgtgatgacagctcatattatagcaactcataacaggtaagtattatttccagaataacattaagtcacttttgtagctctaagtcaatgctgcacaaatggacacttaagattaaggcatcattctgctctggagtagtgcttctgtgaatcccaggaactgtacaaaggctttccgttttaaaaaatatatcttctgttatacttcagttatttcattccactgatcattttcttgcaaatgaaaattgaaaataccagtctataatgttttcatacacctgatttgacgatgccttcttcagctccattctccagccactgagattcactgtccaacaagcggttttttgattcactaagtggtttgataggaaaaggttgatttgagccactacttctggcatactcattctggtttgtaacagaagcttgttctggatccatccccacaaggcgagttggaaaactgcaaccatcacccaagcttgaaaatattggaagtagccaatatttcttttcatcaccaaagacttgtctccaatttttactgcatccaagagagaaaccatttccatcaggtccgtatgaaaacgtgggtgcgcggaatgattctattgttgttctattttttccaactagccagcagtggtagctgaaaagtgagaggacgctgatgaagaacattgcagacacaaagaaaagaaaaagtacgtggaattttgcacgtgtatctgtcagttcattcgtccaaaattttataaagtactctaaaactgttgcagccacgaaaaggcaatataatagggaatacaataaaaacagcaggaagaatttgtaattagaaaatcccacacagttattcacccaaggacagtgatgatccatcttaagaatacatgagtcacaggctgagcagtgatgcgcccgatcaggtttaatcagctgacatttttcacaatatctgatagtttttgaagctgatgtggtatagataggtaaagctcttgctgctcttctcaaaatttcttgttgtctttcttggctgaattctttttcataacgttccttttcagaattggacaagtagaacattttcttcatttccaaaaatagtaactaagaaagggctcaaatcaatgaccttggtttccacattaatacacgcagagctccaccacgtacgcgtagtaggaccagacgaccacgaaggtgatgaagagcaccggcacccagcccacgacgcgctggcagcagcgccacagcgtccagggcgccatgttccgctggcggctgccgagccccgcgtcccaccgttctggggagcgcgggagccccggcgacggtgactcggacgctccaggcggctgctggtccagctcccccgcctccgaggcaggacttgtgggagcaaaagtccgaggcgccgccgggactcctcccgtcccggcgccc

SEQ ID NO: 13028 - RNA, 3321 nt, Homo sapiens
  source 1..3321: mol_type = other RNA
gctgggattacaggcatgagccaccacacccagcaataattggtatctcttaaatctcattctagtttgctagaatcaagattactaaggagttgaaacaaaggtagaagaatccatactataatatcccaaattatgttttcaaagctaactcattcctttggttcaaaaagaaaaaaagttgcctccttttaaaatccaatattagtatggctgatggaaattaggccaaattataaacaaattataaacctacagtagcaaccataaaatttatgctgtactaggaaatgacagagctattcctagtttattatttagcatacagaaggtactccaaaaaatttaccggggcggggcgtggtggctcacgcctgtaatcccagcactttgggaagctgaggtgggtggattatttgaggtcaggagttagtgatcagcctggtcaacatggtgaaacctcgtctcttctaaaaatgtgaaaattagccgggcatggtggcatgagcctgtaatcccagctacttgggaggctgaggcaggagactctattgaacctggaaggcagaggttgcagcgagccaagatcccgccactgcactcctgcctgggagacagagcaaaactctgtggaaaaaagaagaaaaaaatttattgggtgaatgaaaagtgattttgcaaaattaggcatcacagaatgttagaagtcatccagtccaacttattcacaacaccccctcccctgcagtcccattttacagacaggaagctccaacctgtagtactcacagatgctgctgagattcatctccacccactcactggaagcaatcaattattttggggggggtgtgtgtgtgtgtgtgtctgtctgtctaaaaggtgtaaatgaggagtgacatttctacattgtttattctgtacttttccttggagttaatgcaacacctcctgtcgcttagattttaaaaggaaaaaggagaaatgtgtctagtcataaaggggttgccgttaggaagtcagacttcagactgtgcgtctaagagtagaatccacttctcaagagactgggaatgtaaaatgaccactcaggttagaatttccaactgacagccaggaggaaaacttactctaaagttttttttgcctagtttaaattgcattttaaatcactgtttaagctattacagtattactgtaaaaagtttcaaagtaatttttagtcattacctacactgaaatttgaaagtgaagtcaacagcatgctttattctaactgctgttaaaactcaaaactattttttttaacaaattacaatattcctcttagattttcttctggacacctatacttcttcctactgtgtccagtattctccagcacatgtacctttgtgtttctctgcccatgtacatacccctgaaagttcaacaaaaaaagctataaaatagcagagagaacccaaaatatttcttatactgccaagttccctttaaaccttgggcacttgctctactacatggttgtattaatgctcataactaagctttcgatgaattagaccaatgtgttctatgttctaaatgatatttagatatctgaatccttctgttatagccaacaataaaaaaagttattaaaaatgttgaaaagtataaaatagtaattataaattagcaaatacccaatttaaaaaagcagttttccttatacagtacaagcaacagtaatttgaatattattcactttcagccaccatttgccctagatgtactttaaagtttttaagcttgtgtttttggagtgaaaatgtatatggatacttattctaataatgtaattcaggtatcaaaaaatacatatgcatgttaaaatgtgatgacagctcatattatagcaactcataacaggtaagtattatttccagaataacattaagtcacttttgtagctctaagtcaatgctgcacaaatggacacttaagattaaggcatcattctgctctggagtagtgcttctgtgaatcccaggaactgtacaaaggctttccgttttaaaaaatatatcttctgttatacttcagttatttcattccactgatcattttcttgcaaatgaaaattgaaaataccagtctataatgttttcatacacctgatttgacgatgccttcttcagctccattctccagccactgagattcactgtccaacaagcggttttttgattcactaagtggtttgataggaaaaggttgatttgagccactacttctggcatactcattctggtttgtaacagaagcttgttctggatccatccccacaaggcgagttggaaaactgcaaccatcacccaagcttgaaaatattggaagtagccaatatttcttttcatcaccaaagacttgtctccaatttttactgcatccaagagagaaaccatttccatcaggtccgtatgaaaacgtgggtgcgcggaatgattctattgttgttctattttttccaactagccagcagtggtagctgaaaagtgagaggacgctgatgaagaacattgcagacacaaagaaaagaaaaagtacgtggaattttgcacgtgtatctgtcagttcattcgtccaaaattttataaagtactctaaaactgttgcagccacgaaaaggcaatataatagggaatacaataaaaacagcaggaagaatttgtaattagaaaatcccacacagttattcacccaaggacagtgatgatccatcttaagaatacatgagtcacaggctgagcagtgatgcgcccgatcaggtttaatcagctgacatttttcacaatatctgatagtttttgaagctgatgtggtatagataggtaaagctcttgctgctcttctcaaaatttcttgttgtctttcttggctgaattctttttcataacgttccttttcagaattggacaagtagaactctttggagggggaagcgggagatgtgaaaattgtcatccaataggaccatacaaacataacaaagaacagatggaaagccacaaggtaaacaacggtctttcacacgcagagctccaccacgtacgcgtagtaggaccagacgaccacgaaggtgatgaagagcaccggcacccagcccacgacgcgctggcagcagcgccacagcgtccagggcgccatgttccgctggcggctgccgagccccgcgtcccaccgttctggggagcgcgggagccccggcgacggtgactcggacgctccaggcggctgctggtccagctcccccgcctccgaggcaggacttgtgggagc

SEQ ID NO: 13029 - RNA, 3354 nt, Homo sapiens
  source 1..3354: mol_type = other RNA
gctgggattacaggcatgagccaccacacccagcaataattggtatctcttaaatctcattctagtttgctagaatcaagattactaaggagttgaaacaaaggtagaagaatccatactataatatcccaaattatgttttcaaagctaactcattcctttggttcaaaaagaaaaaaagttgcctccttttaaaatccaatattagtatggctgatggaaattaggccaaattataaacaaattataaacctacagtagcaaccataaaatttatgctgtactaggaaatgacagagctattcctagtttattatttagcatacagaaggtactccaaaaaatttaccggggcggggcgtggtggctcacgcctgtaatcccagcactttgggaagctgaggtgggtggattatttgaggtcaggagttagtgatcagcctggtcaacatggtgaaacctcgtctcttctaaaaatgtgaaaattagccgggcatggtggcatgagcctgtaatcccagctacttgggaggctgaggcaggagactctattgaacctggaaggcagaggttgcagcgagccaagatcccgccactgcactcctgcctgggagacagagcaaaactctgtggaaaaaagaagaaaaaaatttattgggtgaatgaaaagtgattttgcaaaattaggcatcacagaatgttagaagtcatccagtccaacttattcacaacaccccctcccctgcagtcccattttacagacaggaagctccaacctgtagtactcacagatgctgctgagattcatctccacccactcactggaagcaatcaattattttggggggggtgtgtgtgtgtgtgtgtctgtctgtctaaaaggtgtaaatgaggagtgacatttctacattgtttattctgtacttttccttggagttaatgcaacacctcctgtcgcttagattttaaaaggaaaaaggagaaatgtgtctagtcataaaggggttgccgttaggaagtcagacttcagactgtgcgtctaagagtagaatccacttctcaagagactgggaatgtaaaatgaccactcaggttagaatttccaactgacagccaggaggaaaacttactctaaagttttttttgcctagtttaaattgcattttaaatcactgtttaagctattacagtattactgtaaaaagtttcaaagtaatttttagtcattacctacactgaaatttgaaagtgaagtcaacagcatgctttattctaactgctgttaaaactcaaaactattttttttaacaaattacaatattcctcttagattttcttctggacacctatacttcttcctactgtgtccagtattctccagcacatgtacctttgtgtttctctgcccatgtacatacccctgaaagttcaacaaaaaaagctataaaatagcagagagaacccaaaatatttcttatactgccaagttccctttaaaccttgggcacttgctctactacatggttgtattaatgctcataactaagctttcgatgaattagaccaatgtgttctatgttctaaatgatatttagatatctgaatccttctgttatagccaacaataaaaaaagttattaaaaatgttgaaaagtataaaatagtaattataaattagcaaatacccaatttaaaaaagcagttttccttatacagtacaagcaacagtaatttgaatattattcactttcagccaccatttgccctagatgtactttaaagtttttaagcttgtgtttttggagtgaaaatgtatatggatacttattctaataatgtaattcaggtatcaaaaaatacatatgcatgttaaaatgtgatgacagctcatattatagcaactcataacaggtaagtattatttccagaataacattaagtcacttttgtagctctaagtcaatgctgcacaaatggacacttaagattaaggcatcattctgctctggagtagtgcttctgtgaatcccaggaactgtacaaaggctttccgttttaaaaaatatatcttctgttatacttcagttatttcattccactgatcattttcttgcaaatgaaaattgaaaataccagtctataatgttttcatacacctgatttgacgatgccttcttcagctccattctccagccactgagattcactgtccaacaagcggttttttgattcactaagtggtttgataggaaaaggttgatttgagccactacttctggcatactcattctggtttgtaacagaagcttgttctggatccatccccacaaggcgagttggaaaactgcaaccatcacccaagcttgaaaatattggaagtagccaatatttcttttcatcaccaaagacttgtctccaatttttactgcatccaagagagaaaccatttccatcaggtccgtatgaaaacgtgggtgcgcggaatgattctattgttgttctattttttccaactagccagcagtggtagctgaaaagtgagaggacgctgatgaagaacattgcagacacaaagaaaagaaaaagtacgtggaattttgcacgtgtatctgtcagttcattcgtccaaaattttataaagtactctaaaactgttgcagccacgaaaaggcaatataatagggaatacaataaaaacagcaggaagaatttgtaattagaaaatcccacacagttattcacccaaggacagtgatgatccatcttaagaatacatgagtcacaggctgagcagtgatgcgcccgatcaggtttaatcagctgacatttttcacaatatctgatagtttttgaagctgatgtggtatagataggtaaagctcttgctgctcttctcaaaatttcttgttgtctttcttggctgaattctttttcataacgttccttttcagaattggacaagtagaactctttggagggggaagcgggagatgtgaaaattgtcatccaataggaccatacaaacataacaaagaacagatggaaagccacaaggtaaacaacggtctttccattttcttcatttccaaaaatagtaaacacgcagagctccaccacgtacgcgtagtaggaccagacgaccacgaaggtgatgaagagcaccggcacccagcccacgacgcgctggcagcagcgccacagcgtccagggcgccatgttccgctggcggctgccgagccccgcgtcccaccgttctggggagcgcgggagccccggcgacggtgactcggacgctccaggcggctgctggtccagctcccccgcctccgaggcaggacttgtgggagcaaaagt

SEQ ID NO: 13030 - RNA, 3396 nt, Homo sapiens
  source 1..3396: mol_type = other RNA
gctgggattacaggcatgagccaccacacccagcaataattggtatctcttaaatctcattctagtttgctagaatcaagattactaaggagttgaaacaaaggtagaagaatccatactataatatcccaaattatgttttcaaagctaactcattcctttggttcaaaaagaaaaaaagttgcctccttttaaaatccaatattagtatggctgatggaaattaggccaaattataaacaaattataaacctacagtagcaaccataaaatttatgctgtactaggaaatgacagagctattcctagtttattatttagcatacagaaggtactccaaaaaatttaccggggcggggcgtggtggctcacgcctgtaatcccagcactttgggaagctgaggtgggtggattatttgaggtcaggagttagtgatcagcctggtcaacatggtgaaacctcgtctcttctaaaaatgtgaaaattagccgggcatggtggcatgagcctgtaatcccagctacttgggaggctgaggcaggagactctattgaacctggaaggcagaggttgcagcgagccaagatcccgccactgcactcctgcctgggagacagagcaaaactctgtggaaaaaagaagaaaaaaatttattgggtgaatgaaaagtgattttgcaaaattaggcatcacagaatgttagaagtcatccagtccaacttattcacaacaccccctcccctgcagtcccattttacagacaggaagctccaacctgtagtactcacagatgctgctgagattcatctccacccactcactggaagcaatcaattattttggggggggtgtgtgtgtgtgtgtgtctgtctgtctaaaaggtgtaaatgaggagtgacatttctacattgtttattctgtacttttccttggagttaatgcaacacctcctgtcgcttagattttaaaaggaaaaaggagaaatgtgtctagtcataaaggggttgccgttaggaagtcagacttcagactgtgcgtctaagagtagaatccacttctcaagagactgggaatgtaaaatgaccactcaggttagaatttccaactgacagccaggaggaaaacttactctaaagttttttttgcctagtttaaattgcattttaaatcactgtttaagctattacagtattactgtaaaaagtttcaaagtaatttttagtcattacctacactgaaatttgaaagtgaagtcaacagcatgctttattctaactgctgttaaaactcaaaactattttttttaacaaattacaatattcctcttagattttcttctggacacctatacttcttcctactgtgtccagtattctccagcacatgtacctttgtgtttctctgcccatgtacatacccctgaaagttcaacaaaaaaagctataaaatagcagagagaacccaaaatatttcttatactgccaagttccctttaaaccttgggcacttgctctactacatggttgtattaatgctcataactaagctttcgatgaattagaccaatgtgttctatgttctaaatgatatttagatatctgaatccttctgttatagccaacaataaaaaaagttattaaaaatgttgaaaagtataaaatagtaattataaattagcaaatacccaatttaaaaaagcagttttccttatacagtacaagcaacagtaatttgaatattattcactttcagccaccatttgccctagatgtactttaaagtttttaagcttgtgtttttggagtgaaaatgtatatggatacttattctaataatgtaattcaggtatcaaaaaatacatatgcatgttaaaatgtgatgacagctcatattatagcaactcataacaggtaagtattatttccagaataacattaagtcacttttgtagctctaagtcaatgctgcacaaatggacacttaagattaaggcatcattctgctctggagtagtgcttctgtgaatcccaggaactgtacaaaggctttccgttttaaaaaatatatcttctgttatacttcagttatttcattccactgatcattttcttgcaaatgaaaattgaaaataccagtctataatgttttcatacacctgatttgacgatgccttcttcagctccattctccagccactgagattcactgtccaacaagcggttttttgattcactaagtggtttgataggaaaaggttgatttgagccactgtcatttgccaagttttctgctttctacctctgcagtttagatcttctggcatactcattctggtttgtaacagaagcttgttctggatccatccccacaaggcgagttggaaaactgcaaccatcacccaagcttgaaaatattggaagtagccaatatttcttttcatcaccaaagacttgtctccaatttttactgcatccaagagagaaaccatttccatcaggtccgtatgaaaacgtgggtgcgcggaatgattctattgttgttctattttttccaactagccagcagtggtagctgaaaagtgagaggacgctgatgaagaacattgcagacacaaagaaaagaaaaagtacgtggaattttgcacgtgtatctgtcagttcattcgtccaaaattttataaagtactctaaaactgttgcagccacgaaaaggcaatataatagggaatacaataaaaacagcaggaagaatttgtaattagaaaatcccacacagttattcacccaaggacagtgatgatccatcttaagaatacatgagtcacaggctgagcagtgatgcgcccgatcaggtttaatcagctgacatttttcacaatatctgatagtttttgaagctgatgtggtatagataggtaaagctcttgctgctcttctcaaaatttcttgttgtctttcttggctgaattctttttcataacgttccttttcagaattggacaagtagaactctttggagggggaagcgggagatgtgaaaattgtcatccaataggaccatacaaacataacaaagaacagatggaaagccacaaggtaaacaacggtctttccattttcttcatttccaaaaatagtaaacacgcagagctccaccacgtacgcgtagtaggaccagacgaccacgaaggtgatgaagagcaccggcacccagcccacgacgcgctggcagcagcgccacagcgtccagggcgccatgttccgctggcggctgccgagccccgcgtcccaccgttctggggagcgcgggagccccggcgacggtgactcggacgctccaggcggctgctggtccagctcccccgcctccgaggcaggacttgtgggagcaaaagt

SEQ ID NO: 13031 - RNA, 3345 nt, Homo sapiens
  source 1..3345: mol_type = other RNA
gctgggattacaggcatgagccaccacacccagcaataattggtatctcttaaatctcattctagtttgctagaatcaagattactaaggagttgaaacaaaggtagaagaatccatactataatatcccaaattatgttttcaaagctaactcattcctttggttcaaaaagaaaaaaagttgcctccttttaaaatccaatattagtatggctgatggaaattaggccaaattataaacaaattataaacctacagtagcaaccataaaatttatgctgtactaggaaatgacagagctattcctagtttattatttagcatacagaaggtactccaaaaaatttaccggggcggggcgtggtggctcacgcctgtaatcccagcactttgggaagctgaggtgggtggattatttgaggtcaggagttagtgatcagcctggtcaacatggtgaaacctcgtctcttctaaaaatgtgaaaattagccgggcatggtggcatgagcctgtaatcccagctacttgggaggctgaggcaggagactctattgaacctggaaggcagaggttgcagcgagccaagatcccgccactgcactcctgcctgggagacagagcaaaactctgtggaaaaaagaagaaaaaaatttattgggtgaatgaaaagtgattttgcaaaattaggcatcacagaatgttagaagtcatccagtccaacttattcacaacaccccctcccctgcagtcccattttacagacaggaagctccaacctgtagtactcacagatgctgctgagattcatctccacccactcactggaagcaatcaattattttggggggggtgtgtgtgtgtgtgtgtctgtctgtctaaaaggtgtaaatgaggagtgacatttctacattgtttattctgtacttttccttggagttaatgcaacacctcctgtcgcttagattttaaaaggaaaaaggagaaatgtgtctagtcataaaggggttgccgttaggaagtcagacttcagactgtgcgtctaagagtagaatccacttctcaagagactgggaatgtaaaatgaccactcaggttagaatttccaactgacagccaggaggaaaacttactctaaagttttttttgcctagtttaaattgcattttaaatcactgtttaagctattacagtattactgtaaaaagtttcaaagtaatttttagtcattacctacactgaaatttgaaagtgaagtcaacagcatgctttattctaactgctgttaaaactcaaaactattttttttaacaaattacaatattcctcttagattttcttctggacacctatacttcttcctactgtgtccagtattctccagcacatgtacctttgtgtttctctgcccatgtacatacccctgaaagttcaacaaaaaaagctataaaatagcagagagaacccaaaatatttcttatactgccaagttccctttaaaccttgggcacttgctctactacatggttgtattaatgctcataactaagctttcgatgaattagaccaatgtgttctatgttctaaatgatatttagatatctgaatccttctgttatagccaacaataaaaaaagttattaaaaatgttgaaaagtataaaatagtaattataaattagcaaatacccaatttaaaaaagcagttttccttatacagtacaagcaacagtaatttgaatattattcactttcagccaccatttgccctagatgtactttaaagtttttaagcttgtgtttttggagtgaaaatgtatatggatacttattctaataatgtaattcaggtatcaaaaaatacatatgcatgttaaaatgtgatgacagctcatattatagcaactcataacaggtaagtattatttccagaataacattaagtcacttttgtagctctaagtcaatgctgcacaaatggacacttaagattaaggcatcattctgctctggagtagtgcttctgtgaatcccaggaactgtacaaaggctttccgttttaaaaaatatatcttctgttatacttcagttatttcattccactgatcattttcttgcaaatgaaaattgaaaataccagtctataatgttttcatacacctgatttgacgatgccttcttcagctccattctccagccactgagattcactgtccaacaagcggttttttgattcactaagtggtttgataggaaaaggttgatttgagccacttctggcatactcattctggtttgtaacagaagcttgttctggatccatccccacaaggcgagttggaaaactgcaaccatcacccaagcttgaaaatattggaagtagccaatatttcttttcatcaccaaagacttgtctccaatttttactgcatccaagagagaaaccatttccatcaggtccgtatgaaaacgtgggtgcgcggaatgattctattgttgttctattttttccaactagccagcagtggtagctgaaaagtgagaggacgctgatgaagaacattgcagacacaaagaaaagaaaaagtacgtggaattttgcacgtgtatctgtcagttcattcgtccaaaattttataaagtactctaaaactgttgcagccacgaaaaggcaatataatagggaatacaataaaaacagcaggaagaatttgtaattagaaaatcccacacagttattcacccaaggacagtgatgatccatcttaagaatacatgagtcacaggctgagcagtgatgcgcccgatcaggtttaatcagctgacatttttcacaatatctgatagtttttgaagctgatgtggtatagataggtaaagctcttgctgctcttctcaaaatttcttgttgtctttcttggctgaattctttttcataacgttccttttcagaattggacaagtagaactctttggagggggaagcgggagatgtgaaaattgtcatccaataggaccatacaaacataacaaagaacagatggaaagccacaaggtaaacaacggtctttccattttcttcatttccaaaaatagtaaacacgcagagctccaccacgtacgcgtagtaggaccagacgaccacgaaggtgatgaagagcaccggcacccagcccacgacgcgctggcagcagcgccacagcgtccagggcgccatgttccgctggcggctgccgagccccgcgtcccaccgttctggggagcgcgggagccccggcgacggtgactcggacgctccaggcggctgctggtccagctcccccgcctccgaggcaggacttgtgggagc

SEQ ID NO: 13032 - RNA, 3589 nt, Homo sapiens
  source 1..3589: mol_type = other RNA
gctgggattacaggcatgagccaccacacccagcaataattggtatctcttaaatctcattctagtttgctagaatcaagattactaaggagttgaaacaaaggtagaagaatccatactataatatcccaaattatgttttcaaagctaactcattcctttggttcaaaaagaaaaaaagttgcctccttttaaaatccaatattagtatggctgatggaaattaggccaaattataaacaaattataaacctacagtagcaaccataaaatttatgctgtactaggaaatgacagagctattcctagtttattatttagcatacagaaggtactccaaaaaatttaccggggcggggcgtggtggctcacgcctgtaatcccagcactttgggaagctgaggtgggtggattatttgaggtcaggagttagtgatcagcctggtcaacatggtgaaacctcgtctcttctaaaaatgtgaaaattagccgggcatggtggcatgagcctgtaatcccagctacttgggaggctgaggcaggagactctattgaacctggaaggcagaggttgcagcgagccaagatcccgccactgcactcctgcctgggagacagagcaaaactctgtggaaaaaagaagaaaaaaatttattgggtgaatgaaaagtgattttgcaaaattaggcatcacagaatgttagaagtcatccagtccaacttattcacaacaccccctcccctgcagtcccattttacagacaggaagctccaacctgtagtactcacagatgctgctgagattcatctccacccactcactggaagcaatcaattattttggggggggtgtgtgtgtgtgtgtgtctgtctgtctaaaaggtgtaaatgaggagtgacatttctacattgtttattctgtacttttccttggagttaatgcaacacctcctgtcgcttagattttaaaaggaaaaaggagaaatgtgtctagtcataaaggggttgccgttaggaagtcagacttcagactgtgcgtctaagagtagaatccacttctcaagagactgggaatgtaaaatgaccactcaggttagaatttccaactgacagccaggaggaaaacttactctaaagttttttttgcctagtttaaattgcattttaaatcactgtttaagctattacagtattactgtaaaaagtttcaaagtaatttttagtcattacctacactgaaatttgaaagtgaagtcaacagcatgctttattctaactgctgttaaaactcaaaactattttttttaacaaattacaatattcctcttagattttcttctggacacctatacttcttcctactgtgtccagtattctccagcacatgtacctttgtgtttctctgcccatgtacatacccctgaaagttcaacaaaaaaagctataaaatagcagagagaacccaaaatatttcttatactgccaagttccctttaaaccttgggcacttgctctactacatggttgtattaatgctcataactaagctttcgatgaattagaccaatgtgttctatgttctaaatgatatttagatatctgaatccttctgttatagccaacaataaaaaaagttattaaaaatgttgaaaagtataaaatagtaattataaattagcaaatacccaatttaaaaaagcagttttccttatacagtacaagcaacagtaatttgaatattattcactttcagccaccatttgccctagatgtactttaaagtttttaagcttgtgtttttggagtgaaaatgtatatggatacttattctaataatgtaattcaggtatcaaaaaatacatatgcatgttaaaatgtgatgacagctcatattatagcaactcataacaggtaagtattatttccagaataacattaagtcacttttgtagctctaagtcaatgctgcacaaatggacacttaagattaaggcatcattctgctctggagtagtgcttctgtgaatcccaggaactgtacaaaggctttccgttttaaaaaatatatcttctgttatacttcagttatttcattccactgatcattttcttgcaaatgaaaattgaaaataccagtctataatgttttcatacaccttgctcttattcaaatggttagttatgaacaagtggtactcaattttctattgccactgttacatggttatttgtccctgatttgacgatgccttcttcagctccattctccagccactgagattcactgtccaacaagcggttttttgattcactaagtggtttgataggaaaaggttgatttgagccactactgtcatttgccaagttttctgctttctacctctgcagtttagatcttctggcatactcattctggtttgtaacagaagcttgttctggatccatccccacaaggcgagttggaaaactgcaaccatcacccaagcttgaaaatattggaagtagccaatatttcttttcatcaccaaagacttgtctccaatttttactgcatccaagagagaaaccatttccatcaggtccgtatgaaaacgtgggtgcgcggaatgattctattgttgttctattttttccaactagccagcagtggtagctgaaaagtgagaggacgctgatgaagaacattgcagacacaaagaaaagaaaaagtacgtggaattttgcacgtgtatctgtcagttcattcgtccaaaattttataaagtactctaaaactgttgcagccacgaaaaggcaatataatagggaatacaataaaaacagcaggaagaatttgtaattagaaaatcccacacagttattcacccaaggacagtgatgatccatcttaagaatacatgagtcacaggctgagcagtgatgcgcccgatcaggtttaatcagctgacatttttcacaatatctgatagttggaaataaccaatcttctttctgttctttgtttccactttcttcagccttttctaaagccgacttcccctgtccagctcattggagctcctttctattttgtagactgcatgaggctttttgaagctgatgtggtatagataggtaaagctcttgctgctcttctcaaaatttcttgttgtctttcttggctgaattctttttcataacgttccttttcagaattggacaagtagaactctttggagggggaagcgggagatgtgaaaattgtcatccaataggaccatacaaacataacaaagaacagatggaaagccacaaggtaaacaacggtctttccattttcttcatttccaaaaatagtaaacacgcagagctccaccacgtacgcgtagtaggaccagacgaccacgaaggtgatgaagagcaccggcacccagcccacgacgcgctggcagcagcgccacagcgtccagggcgccatgttccgctggcggctgccgagccccgcgtcccaccgttctggggagcgcgggagccccggcgacggtgactcggacgctccaggcggctgctggtccagctcccccgcctccgaggcaggacttgtgggagc

SEQ ID NO: 13033 - RNA, 3477 nt, Homo sapiens
  source 1..3477: mol_type = other RNA
gctgggattacaggcatgagccaccacacccagcaataattggtatctcttaaatctcattctagtttgctagaatcaagattactaaggagttgaaacaaaggtagaagaatccatactataatatcccaaattatgttttcaaagctaactcattcctttggttcaaaaagaaaaaaagttgcctccttttaaaatccaatattagtatggctgatggaaattaggccaaattataaacaaattataaacctacagtagcaaccataaaatttatgctgtactaggaaatgacagagctattcctagtttattatttagcatacagaaggtactccaaaaaatttaccggggcggggcgtggtggctcacgcctgtaatcccagcactttgggaagctgaggtgggtggattatttgaggtcaggagttagtgatcagcctggtcaacatggtgaaacctcgtctcttctaaaaatgtgaaaattagccgggcatggtggcatgagcctgtaatcccagctacttgggaggctgaggcaggagactctattgaacctggaaggcagaggttgcagcgagccaagatcccgccactgcactcctgcctgggagacagagcaaaactctgtggaaaaaagaagaaaaaaatttattgggtgaatgaaaagtgattttgcaaaattaggcatcacagaatgttagaagtcatccagtccaacttattcacaacaccccctcccctgcagtcccattttacagacaggaagctccaacctgtagtactcacagatgctgctgagattcatctccacccactcactggaagcaatcaattattttggggggggtgtgtgtgtgtgtgtgtctgtctgtctaaaaggtgtaaatgaggagtgacatttctacattgtttattctgtacttttccttggagttaatgcaacacctcctgtcgcttagattttaaaaggaaaaaggagaaatgtgtctagtcataaaggggttgccgttaggaagtcagacttcagactgtgcgtctaagagtagaatccacttctcaagagactgggaatgtaaaatgaccactcaggttagaatttccaactgacagccaggaggaaaacttactctaaagttttttttgcctagtttaaattgcattttaaatcactgtttaagctattacagtattactgtaaaaagtttcaaagtaatttttagtcattacctacactgaaatttgaaagtgaagtcaacagcatgctttattctaactgctgttaaaactcaaaactattttttttaacaaattacaatattcctcttagattttcttctggacacctatacttcttcctactgtgtccagtattctccagcacatgtacctttgtgtttctctgcccatgtacatacccctgaaagttcaacaaaaaaagctataaaatagcagagagaacccaaaatatttcttatactgccaagttccctttaaaccttgggcacttgctctactacatggttgtattaatgctcataactaagctttcgatgaattagaccaatgtgttctatgttctaaatgatatttagatatctgaatccttctgttatagccaacaataaaaaaagttattaaaaatgttgaaaagtataaaatagtaattataaattagcaaatacccaatttaaaaaagcagttttccttatacagtacaagcaacagtaatttgaatattattcactttcagccaccatttgccctagatgtactttaaagtttttaagcttgtgtttttggagtgaaaatgtatatggatacttattctaataatgtaattcaggtatcaaaaaatacatatgcatgttaaaatgtgatgacagctcatattatagcaactcataacaggtaagtattatttccagaataacattaagtcacttttgtagctctaagtcaatgctgcacaaatggacacttaagattaaggcatcattctgctctggagtagtgcttctgtgaatcccaggaactgtacaaaggctttccgttttaaaaaatatatcttctgttatacttcagttatttcattccactgatcattttcttgcaaatgaaaattgaaaataccagtctataatgttttcatacaccttgctcttattcaaatggttagttatgaacaagtggtactcaattttctattgccactgttacatggttatttgtccctgatttgacgatgccttcttcagctccattctccagccactgagattcactgtccaacaagcggttttttgattcactaagtggtttgataggaaaaggttgatttgagccactactgtcatttgccaagttttctgctttctacctctgcagtttagatcttctggcatactcattctggtttgtaacagaagcttgttctggatccatccccacaaggcgagttggaaaactgcaaccatcacccaagcttgaaaatattggaagtagccaatatttcttttcatcaccaaagacttgtctccaatttttactgcatccaagagagaaaccatttccatcaggtccgtatgaaaacgtgggtgcgcggaatgattctattgttgttctattttttccaactagccagcagtggtagctgaaaagtgagaggacgctgatgaagaacattgcagacacaaagaaaagaaaaagtacgtggaattttgcacgtgtatctgtcagttcattcgtccaaaattttataaagtactctaaaactgttgcagccacgaaaaggcaatataatagggaatacaataaaaacagcaggaagaatttgtaattagaaaatcccacacagttattcacccaaggacagtgatgatccatcttaagaatacatgagtcacaggctgagcagtgatgcgcccgatcaggtttaatcagctgacatttttcacaatatctgatagtttttgaagctgatgtggtatagataggtaaagctcttgctgctcttctcaaaatttcttgttgtctttcttggctgaattctttttcataacgttccttttcagaattggacaagtagaactctttggagggggaagcgggagatgtgaaaattgtcatccaataggaccatacaaacataacaaagaacagatggaaagccacaaggtaaacaacggtctttccattttcttcatttccaaaaatagtaaacacgcagagctccaccacgtacgcgtagtaggaccagacgaccacgaaggtgatgaagagcaccggcacccagcccacgacgcgctggcagcagcgccacagcgtccagggcgccatgttccgctggcggctgccgagccccgcgtcccaccgttctggggagcgcgggagccccggcgacggtgactcggacgctccaggcggctgctggtccagctcccccgcctccgaggcaggacttgtgggagcaaaagt

SEQ ID NO: 13034 - RNA, 3125 nt, Homo sapiens
  source 1..3125: mol_type = other RNA
gctgggattacaggcatgagccaccacacccagcaataattggtatctcttaaatctcattctagtttgctagaatcaagattactaaggagttgaaacaaaggtagaagaatccatactataatatcccaaattatgttttcaaagctaactcattcctttggttcaaaaagaaaaaaagttgcctccttttaaaatccaatattagtatggctgatggaaattaggccaaattataaacaaattataaacctacagtagcaaccataaaatttatgctgtactaggaaatgacagagctattcctagtttattatttagcatacagaaggtactccaaaaaatttaccggggcggggcgtggtggctcacgcctgtaatcccagcactttgggaagctgaggtgggtggattatttgaggtcaggagttagtgatcagcctggtcaacatggtgaaacctcgtctcttctaaaaatgtgaaaattagccgggcatggtggcatgagcctgtaatcccagctacttgggaggctgaggcaggagactctattgaacctggaaggcagaggttgcagcgagccaagatcccgccactgcactcctgcctgggagacagagcaaaactctgtggaaaaaagaagaaaaaaatttattgggtgaatgaaaagtgattttgcaaaattaggcatcacagaatgttagaagtcatccagtccaacttattcacaacaccccctcccctgcagtcccattttacagacaggaagctccaacctgtagtactcacagatgctgctgagattcatctccacccactcactggaagcaatcaattattttggggggggtgtgtgtgtgtgtgtgtctgtctgtctaaaaggtgtaaatgaggagtgacatttctacattgtttattctgtacttttccttggagttaatgcaacacctcctgtcgcttagattttaaaaggaaaaaggagaaatgtgtctagtcataaaggggttgccgttaggaagtcagacttcagactgtgcgtctaagagtagaatccacttctcaagagactgggaatgtaaaatgaccactcaggttagaatttccaactgacagccaggaggaaaacttactctaaagttttttttgcctagtttaaattgcattttaaatcactgtttaagctattacagtattactgtaaaaagtttcaaagtaatttttagtcattacctacactgaaatttgaaagtgaagtcaacagcatgctttattctaactgctgttaaaactcaaaactattttttttaacaaattacaatattcctcttagattttcttctggacacctatacttcttcctactgtgtccagtattctccagcacatgtacctttgtgtttctctgcccatgtacatacccctgaaagttcaacaaaaaaagctataaaatagcagagagaacccaaaatatttcttatactgccaagttccctttaaaccttgggcacttgctctactacatggttgtattaatgctcataactaagctttcgatgaattagaccaatgtgttctatgttctaaatgatatttagatatctgaatccttctgttatagccaacaataaaaaaagttattaaaaatgttgaaaagtataaaatagtaattataaattagcaaatacccaatttaaaaaagcagttttccttatacagtacaagcaacagtaatttgaatattattcactttcagccaccatttgccctagatgtactttaaagtttttaagcttgtgtttttggagtgaaaatgtatatggatacttattctaataatgtaattcaggtatcaaaaaatacatatgcatgttaaaatgtgatgacagctcatattatagcaactcataacaggtaagtattatttccagaataacattaagtcacttttgtagctctaagtcaatgctgcacaaatggacacttaagattaaggcatcattctgctctggagtagtgcttctgtgaatcccaggaactgtacaaaggctttccgttttaaaaaatatatcttctgttatacttcagttatttcattccactgatcattttcttgcaaatgaaaattgaaaataccagtctataatgttttcatacaccttgctcttattcaaatggttagttatgaacaagtggtactcaattttctattgccactgttacatggttatttgtccctgatttgacgatgccttcttcagctccattctccagccactgagattcactgtccaacaagcggttttttgattcactaagtggtttgataggaaaaggttgatttgagccactacttctggcatactcattctggtttgtaacagaagcttgttctggatccatccccacaaggcgagttggaaaactgcaaccatcacccaagcttgaaaatattggaagtagccaatatttcttttcatcaccaaagacttgtctccaatttttactgcatccaagagagaaaccatttccatcaggtccgtatgaaaacgtgggtgcgcggaatgattctattgttgttctattttttccaactagccagcagtggtagctgaaaagtgagaggacgctgatgaagaacattgcagacacaaagaaaagaaaaagtacgtggaattttgcacgtgtatctgtcagttcattcgtccaaaattttataaagtactctaaaactgttgcagccacgaaaaggcaatataatagggaatacaataaaaacagcaggaagaatttgtaattagaaaatcccacacagttattcacccaaggacagtgatgatccatcttaagaatacatgagtcacaggctgagcagtgatgcgcccgatcaggtttaatcagctgacatttttcacaatatctgatagtttttgaagctgatgtggtatagataggtaaagctcttgctgctcttctcaaaatttcttgttgtctttcttggctgaattctttttcataacgttccttttcagaattggacaagtagaacagatgataagttctctgacagggcaaatggagcatgccacagcaaggtcactggatacaggcttgggcagtcagatgac

SEQ ID NO: 13035 - RNA, 3198 nt, Homo sapiens
  source 1..3198: mol_type = other RNA
gctgggattacaggcatgagccaccacacccagcaataattggtatctcttaaatctcattctagtttgctagaatcaagattactaaggagttgaaacaaaggtagaagaatccatactataatatcccaaattatgttttcaaagctaactcattcctttggttcaaaaagaaaaaaagttgcctccttttaaaatccaatattagtatggctgatggaaattaggccaaattataaacaaattataaacctacagtagcaaccataaaatttatgctgtactaggaaatgacagagctattcctagtttattatttagcatacagaaggtactccaaaaaatttaccggggcggggcgtggtggctcacgcctgtaatcccagcactttgggaagctgaggtgggtggattatttgaggtcaggagttagtgatcagcctggtcaacatggtgaaacctcgtctcttctaaaaatgtgaaaattagccgggcatggtggcatgagcctgtaatcccagctacttgggaggctgaggcaggagactctattgaacctggaaggcagaggttgcagcgagccaagatcccgccactgcactcctgcctgggagacagagcaaaactctgtggaaaaaagaagaaaaaaatttattgggtgaatgaaaagtgattttgcaaaattaggcatcacagaatgttagaagtcatccagtccaacttattcacaacaccccctcccctgcagtcccattttacagacaggaagctccaacctgtagtactcacagatgctgctgagattcatctccacccactcactggaagcaatcaattattttggggggggtgtgtgtgtgtgtgtgtctgtctgtctaaaaggtgtaaatgaggagtgacatttctacattgtttattctgtacttttccttggagttaatgcaacacctcctgtcgcttagattttaaaaggaaaaaggagaaatgtgtctagtcataaaggggttgccgttaggaagtcagacttcagactgtgcgtctaagagtagaatccacttctcaagagactgggaatgtaaaatgaccactcaggttagaatttccaactgacagccaggaggaaaacttactctaaagttttttttgcctagtttaaattgcattttaaatcactgtttaagctattacagtattactgtaaaaagtttcaaagtaatttttagtcattacctacactgaaatttgaaagtgaagtcaacagcatgctttattctaactgctgttaaaactcaaaactattttttttaacaaattacaatattcctcttagattttcttctggacacctatacttcttcctactgtgtccagtattctccagcacatgtacctttgtgtttctctgcccatgtacatacccctgaaagttcaacaaaaaaagctataaaatagcagagagaacccaaaatatttcttatactgccaagttccctttaaaccttgggcacttgctctactacatggttgtattaatgctcataactaagctttcgatgaattagaccaatgtgttctatgttctaaatgatatttagatatctgaatccttctgttatagccaacaataaaaaaagttattaaaaatgttgaaaagtataaaatagtaattataaattagcaaatacccaatttaaaaaagcagttttccttatacagtacaagcaacagtaatttgaatattattcactttcagccaccatttgccctagatgtactttaaagtttttaagcttgtgtttttggagtgaaaatgtatatggatacttattctaataatgtaattcaggtatcaaaaaatacatatgcatgttaaaatgtgatgacagctcatattatagcaactcataacaggtaagtattatttccagaataacattaagtcacttttgtagctctaagtcaatgctgcacaaatggacacttaagattaaggcatcattctgctctggagtagtgcttctgtgaatcccaggaactgtacaaaggctttccgttttaaaaaatatatcttctgttatacttcagttatttcattccactgatcattttcttgcaaatgaaaattgaaaataccagtctataatgttttcatacaccttgctcttattcaaatggttagttatgaacaagtggtactcaattttctattgccactgttacatggttatttgtccctgatttgacgatgccttcttcagctccattctccagccactgagattcactgtccaacaagcggttttttgattcactaagtggtttgataggaaaaggttgatttgagccactacttctggcatactcattctggtttgtaacagaagcttgttctggatccatccccacaaggcgagttggaaaactgcaaccatcacccaagcttgaaaatattggaagtagccaatatttcttttcatcaccaaagacttgtctccaatttttactgcatccaagagagaaaccatttccatcaggtccgtatgaaaacgtgggtgcgcggaatgattctattgttgttctattttttccaactagccagcagtggtagctgaaaagtgagaggacgctgatgaagaacattgcagacacaaagaaaagaaaaagtacgtggaattttgcacgtgtatctgtcagttcattcgtccaaaattttataaagtactctaaaactgttgcagccacgaaaaggcaatataatagggaatacaataaaaacagcaggaagaatttgtaattagaaaatcccacacagttattcacccaaggacagtgatgatccatcttaagaatacatgagtcacaggctgagcagtgatgcgcccgatcaggtttaatcagctgacatttttcacaatatctgatagtttttgaagctgatgtggtatagataggtaaagctcttgctgctcttctcaaaatttcttgttgtctttcttggctgaattctttttcataacgttccttttcagaattggacaagtagaacattttcttcatttccaaaaatagtaactaagaaagggctcaaatcaatgaccttggtttccacattaatctcaaaaataaccaccttgaccaaagagaagaagttattcaatccattcgtactttaaatatcaaccacacgcagagctccac

SEQ ID NO: 13036 - RNA, 3426 nt, Homo sapiens
  source 1..3426: mol_type = other RNA
gctgggattacaggcatgagccaccacacccagcaataattggtatctcttaaatctcattctagtttgctagaatcaagattactaaggagttgaaacaaaggtagaagaatccatactataatatcccaaattatgttttcaaagctaactcattcctttggttcaaaaagaaaaaaagttgcctccttttaaaatccaatattagtatggctgatggaaattaggccaaattataaacaaattataaacctacagtagcaaccataaaatttatgctgtactaggaaatgacagagctattcctagtttattatttagcatacagaaggtactccaaaaaatttaccggggcggggcgtggtggctcacgcctgtaatcccagcactttgggaagctgaggtgggtggattatttgaggtcaggagttagtgatcagcctggtcaacatggtgaaacctcgtctcttctaaaaatgtgaaaattagccgggcatggtggcatgagcctgtaatcccagctacttgggaggctgaggcaggagactctattgaacctggaaggcagaggttgcagcgagccaagatcccgccactgcactcctgcctgggagacagagcaaaactctgtggaaaaaagaagaaaaaaatttattgggtgaatgaaaagtgattttgcaaaattaggcatcacagaatgttagaagtcatccagtccaacttattcacaacaccccctcccctgcagtcccattttacagacaggaagctccaacctgtagtactcacagatgctgctgagattcatctccacccactcactggaagcaatcaattattttggggggggtgtgtgtgtgtgtgtgtctgtctgtctaaaaggtgtaaatgaggagtgacatttctacattgtttattctgtacttttccttggagttaatgcaacacctcctgtcgcttagattttaaaaggaaaaaggagaaatgtgtctagtcataaaggggttgccgttaggaagtcagacttcagactgtgcgtctaagagtagaatccacttctcaagagactgggaatgtaaaatgaccactcaggttagaatttccaactgacagccaggaggaaaacttactctaaagttttttttgcctagtttaaattgcattttaaatcactgtttaagctattacagtattactgtaaaaagtttcaaagtaatttttagtcattacctacactgaaatttgaaagtgaagtcaacagcatgctttattctaactgctgttaaaactcaaaactattttttttaacaaattacaatattcctcttagattttcttctggacacctatacttcttcctactgtgtccagtattctccagcacatgtacctttgtgtttctctgcccatgtacatacccctgaaagttcaacaaaaaaagctataaaatagcagagagaacccaaaatatttcttatactgccaagttccctttaaaccttgggcacttgctctactacatggttgtattaatgctcataactaagctttcgatgaattagaccaatgtgttctatgttctaaatgatatttagatatctgaatccttctgttatagccaacaataaaaaaagttattaaaaatgttgaaaagtataaaatagtaattataaattagcaaatacccaatttaaaaaagcagttttccttatacagtacaagcaacagtaatttgaatattattcactttcagccaccatttgccctagatgtactttaaagtttttaagcttgtgtttttggagtgaaaatgtatatggatacttattctaataatgtaattcaggtatcaaaaaatacatatgcatgttaaaatgtgatgacagctcatattatagcaactcataacaggtaagtattatttccagaataacattaagtcacttttgtagctctaagtcaatgctgcacaaatggacacttaagattaaggcatcattctgctctggagtagtgcttctgtgaatcccaggaactgtacaaaggctttccgttttaaaaaatatatcttctgttatacttcagttatttcattccactgatcattttcttgcaaatgaaaattgaaaataccagtctataatgttttcatacaccttgctcttattcaaatggttagttatgaacaagtggtactcaattttctattgccactgttacatggttatttgtccctgatttgacgatgccttcttcagctccattctccagccactgagattcactgtccaacaagcggttttttgattcactaagtggtttgataggaaaaggttgatttgagccactacttctggcatactcattctggtttgtaacagaagcttgttctggatccatccccacaaggcgagttggaaaactgcaaccatcacccaagcttgaaaatattggaagtagccaatatttcttttcatcaccaaagacttgtctccaatttttactgcatccaagagagaaaccatttccatcaggtccgtatgaaaacgtgggtgcgcggaatgattctattgttgttctattttttccaactagccagcagtggtagctgaaaagtgagaggacgctgatgaagaacattgcagacacaaagaaaagaaaaagtacgtggaattttgcacgtgtatctgtcagttcattcgtccaaaattttataaagtactctaaaactgttgcagccacgaaaaggcaatataatagggaatacaataaaaacagcaggaagaatttgtaattagaaaatcccacacagttattcacccaaggacagtgatgatccatcttaagaatacatgagtcacaggctgagcagtgatgcgcccgatcaggtttaatcagctgacatttttcacaatatctgatagtttttgaagctgatgtggtatagataggtaaagctcttgctgctcttctcaaaatttcttgttgtctttcttggctgaattctttttcataacgttccttttcagaattggacaagtagaactctttggagggggaagcgggagatgtgaaaattgtcatccaataggaccatacaaacataacaaagaacagatggaaagccacaaggtaaacaacggtctttccattttcttcatttccaaaaatagtaaacacgcagagctccaccacgtacgcgtagtaggaccagacgaccacgaaggtgatgaagagcaccggcacccagcccacgacgcgctggcagcagcgccacagcgtccagggcgccatgttccgctggcggctgccgagccccgcgtcccaccgttctggggagcgcgggagccccggcgacggtgactcggacgctccaggcggctgctggtccagctcccccgcctccgaggcaggacttgtgggagc

SEQ ID NO: 13037 - RNA, 2912 nt, Homo sapiens
  source 1..2912: mol_type = other RNA
gctgggattacaggcatgagccaccacacccagcaataattggtatctcttaaatctcattctagtttgctagaatcaagattactaaggagttgaaacaaaggtagaagaatccatactataatatcccaaattatgttttcaaagctaactcattcctttggttcaaaaagaaaaaaagttgcctccttttaaaatccaatattagtatggctgatggaaattaggccaaattataaacaaattataaacctacagtagcaaccataaaatttatgctgtactaggaaatgacagagctattcctagtttattatttagcatacagaaggtactccaaaaaatttaccggggcggggcgtggtggctcacgcctgtaatcccagcactttgggaagctgaggtgggtggattatttgaggtcaggagttagtgatcagcctggtcaacatggtgaaacctcgtctcttctaaaaatgtgaaaattagccgggcatggtggcatgagcctgtaatcccagctacttgggaggctgaggcaggagactctattgaacctggaaggcagaggttgcagcgagccaagatcccgccactgcactcctgcctgggagacagagcaaaactctgtggaaaaaagaagaaaaaaatttattgggtgaatgaaaagtgattttgcaaaattaggcatcacagaatgttagaagtcatccagtccaacttattcacaacaccccctcccctgcagtcccattttacagacaggaagctccaacctgtagtactcacagatgctgctgagattcatctccacccactcactggaagcaatcaattattttggggggggtgtgtgtgtgtgtgtgtctgtctgtctaaaaggtgtaaatgaggagtgacatttctacattgtttattctgtacttttccttggagttaatgcaacacctcctgtcgcttagattttaaaaggaaaaaggagaaatgtgtctagtcataaaggggttgccgttaggaagtcagacttcagactgtgcgtctaagagtagaatccacttctcaagagactgggaatgtaaaatgaccactcaggttagaatttccaactgacagccaggaggaaaacttactctaaagttttttttgcctagtttaaattgcattttaaatcactgtttaagctattacagtattactgtaaaaagtttcaaagtaatttttagtcattacctacactgaaatttgaaagtgaagtcaacagcatgctttattctaactgctgttaaaactcaaaactattttttttaacaaattacaatattcctcttagattttcttctggacacctatacttcttcctactgtgtccagtattctccagcacatgtacctttgtgtttctctgcccatgtacatacccctgaaagttcaacaaaaaaagctataaaatagcagagagaacccaaaatatttcttatactgccaagttccctttaaaccttgggcacttgctctactacatggttgtattaatgctcataactaagctttcgatgaattagaccaatgtgttctatgttctaaatgatatttagatatctgaatccttctgttatagccaacaataaaaaaagttattaaaaatgttgaaaagtataaaatagtaattataaattagcaaatacccaatttaaaaaagcagttttccttatacagtacaagcaacagtaatttgaatattattcactttcagccaccatttgccctagatgtactttaaagtttttaagcttgtgtttttggagtgaaaatgtatatggatacttattctaataatgtaattcaggtatcaaaaaatacatatgcatgttaaaatgtgatgacagctcatattatagcaactcataacaggtaagtattatttccagaataacattaagtcacttttgtagctctaagtcaatgctgcacaaatggacacttaagattaaggcatcattctgctctggagtagtgcttctgtgaatcccaggaactgtacaaaggctttccgttttaaaaaatatatcttctgttatacttcagttatttcattccactgatcattttcttgcaaatgaaaattgaaaataccagtctataatgttttcatacaccttgctcttattcaaatggttagttatgaacaagtggtactcaattttctattgccactgttacatggttatttgtccctgatttgacgatgccttcttcagctccattctccagccactgagattcactgtccaacaagcggttttttgattcactaagtggtttgataggaaaaggttgatttgagccactacttctggcatactcattctggtttgtaacagaagcttgttctggatccatccccacaaggcgagttggaaaactgcaaccatcacccaagcttgaaaatattggaagtagccaatatttcttttcatcaccaaagacttgtctccaatttttactgcatccaagagagaaaccatttccatcaggtccgtatgaaaacgtgggtgcgcggaatgattctattgttgttctattttttccaactagccagcagtggtagctgaaaagtgagaggacgctgatgaagaacattgcagacacaaagaaaagaaaaagtacgtggaattttgcacgtgtatctgtcagttcattctttggacaactctctgtagacttcctgcggcaaagcttgtgcaaatagagacatatattaagaaaccaatttttatgcaaaattatcctaaacactagttttataaatcctgttgaaagaacactaagatgttgctttctaatggccatctataacattttctcaagaaatacaaaagaaaaaatagacaagaacatgtagctgttcaagc

SEQ ID NO: 13038 - RNA, 3474 nt, Homo sapiens
  source 1..3474: mol_type = other RNA
gctgggattacaggcatgagccaccacacccagcaataattggtatctcttaaatctcattctagtttgctagaatcaagattactaaggagttgaaacaaaggtagaagaatccatactataatatcccaaattatgttttcaaagctaactcattcctttggttcaaaaagaaaaaaagttgcctccttttaaaatccaatattagtatggctgatggaaattaggccaaattataaacaaattataaacctacagtagcaaccataaaatttatgctgtactaggaaatgacagagctattcctagtttattatttagcatacagaaggtactccaaaaaatttaccggggcggggcgtggtggctcacgcctgtaatcccagcactttgggaagctgaggtgggtggattatttgaggtcaggagttagtgatcagcctggtcaacatggtgaaacctcgtctcttctaaaaatgtgaaaattagccgggcatggtggcatgagcctgtaatcccagctacttgggaggctgaggcaggagactctattgaacctggaaggcagaggttgcagcgagccaagatcccgccactgcactcctgcctgggagacagagcaaaactctgtggaaaaaagaagaaaaaaatttattgggtgaatgaaaagtgattttgcaaaattaggcatcacagaatgttagaagtcatccagtccaacttattcacaacaccccctcccctgcagtcccattttacagacaggaagctccaacctgtagtactcacagatgctgctgagattcatctccacccactcactggaagcaatcaattattttggggggggtgtgtgtgtgtgtgtgtctgtctgtctaaaaggtgtaaatgaggagtgacatttctacattgtttattctgtacttttccttggagttaatgcaacacctcctgtcgcttagattttaaaaggaaaaaggagaaatgtgtctagtcataaaggggttgccgttaggaagtcagacttcagactgtgcgtctaagagtagaatccacttctcaagagactgggaatgtaaaatgaccactcaggttagaatttccaactgacagccaggaggaaaacttactctaaagttttttttgcctagtttaaattgcattttaaatcactgtttaagctattacagtattactgtaaaaagtttcaaagtaatttttagtcattacctacactgaaatttgaaagtgaagtcaacagcatgctttattctaactgctgttaaaactcaaaactattttttttaacaaattacaatattcctcttagattttcttctggacacctatacttcttcctactgtgtccagtattctccagcacatgtacctttgtgtttctctgcccatgtacatacccctgaaagttcaacaaaaaaagctataaaatagcagagagaacccaaaatatttcttatactgccaagttccctttaaaccttgggcacttgctctactacatggttgtattaatgctcataactaagctttcgatgaattagaccaatgtgttctatgttctaaatgatatttagatatctgaatccttctgttatagccaacaataaaaaaagttattaaaaatgttgaaaagtataaaatagtaattataaattagcaaatacccaatttaaaaaagcagttttccttatacagtacaagcaacagtaatttgaatattattcactttcagccaccatttgccctagatgtactttaaagtttttaagcttgtgtttttggagtgaaaatgtatatggatacttattctaataatgtaattcaggtatcaaaaaatacatatgcatgttaaaatgtgatgacagctcatattatagcaactcataacaggtaagtattatttccagaataacattaagtcacttttgtagctctaagtcaatgctgcacaaatggacacttaagattaaggcatcattctgctctggagtagtgcttctgtgaatcccaggaactgtacaaaggctttccgttttaaaaaatatatcttctgttatacttcagttatttcattccactgatcattttcttgcaaatgaaaattgaaaataccagtctataatgttttcatacaccttgctcttattcaaatggttagttatgaacaagtggtactcaattttctattgccactgttacatggttatttgtccctgatttgacgatgccttcttcagctccattctccagccactgagattcactgtccaacaagcggttttttgattcactaagtggtttgataggaaaaggttgatttgagccactgtcatttgccaagttttctgctttctacctctgcagtttagatcttctggcatactcattctggtttgtaacagaagcttgttctggatccatccccacaaggcgagttggaaaactgcaaccatcacccaagcttgaaaatattggaagtagccaatatttcttttcatcaccaaagacttgtctccaatttttactgcatccaagagagaaaccatttccatcaggtccgtatgaaaacgtgggtgcgcggaatgattctattgttgttctattttttccaactagccagcagtggtagctgaaaagtgagaggacgctgatgaagaacattgcagacacaaagaaaagaaaaagtacgtggaattttgcacgtgtatctgtcagttcattcgtccaaaattttataaagtactctaaaactgttgcagccacgaaaaggcaatataatagggaatacaataaaaacagcaggaagaatttgtaattagaaaatcccacacagttattcacccaaggacagtgatgatccatcttaagaatacatgagtcacaggctgagcagtgatgcgcccgatcaggtttaatcagctgacatttttcacaatatctgatagtttttgaagctgatgtggtatagataggtaaagctcttgctgctcttctcaaaatttcttgttgtctttcttggctgaattctttttcataacgttccttttcagaattggacaagtagaactctttggagggggaagcgggagatgtgaaaattgtcatccaataggaccatacaaacataacaaagaacagatggaaagccacaaggtaaacaacggtctttccattttcttcatttccaaaaatagtaaacacgcagagctccaccacgtacgcgtagtaggaccagacgaccacgaaggtgatgaagagcaccggcacccagcccacgacgcgctggcagcagcgccacagcgtccagggcgccatgttccgctggcggctgccgagccccgcgtcccaccgttctggggagcgcgggagccccggcgacggtgactcggacgctccaggcggctgctggtccagctcccccgcctccgaggcaggacttgtgggagcaaaagt

SEQ ID NO: 13039 - RNA, 3429 nt, Homo sapiens
  source 1..3429: mol_type = other RNA
gctgggattacaggcatgagccaccacacccagcaataattggtatctcttaaatctcattctagtttgctagaatcaagattactaaggagttgaaacaaaggtagaagaatccatactataatatcccaaattatgttttcaaagctaactcattcctttggttcaaaaagaaaaaaagttgcctccttttaaaatccaatattagtatggctgatggaaattaggccaaattataaacaaattataaacctacagtagcaaccataaaatttatgctgtactaggaaatgacagagctattcctagtttattatttagcatacagaaggtactccaaaaaatttaccggggcggggcgtggtggctcacgcctgtaatcccagcactttgggaagctgaggtgggtggattatttgaggtcaggagttagtgatcagcctggtcaacatggtgaaacctcgtctcttctaaaaatgtgaaaattagccgggcatggtggcatgagcctgtaatcccagctacttgggaggctgaggcaggagactctattgaacctggaaggcagaggttgcagcgagccaagatcccgccactgcactcctgcctgggagacagagcaaaactctgtggaaaaaagaagaaaaaaatttattgggtgaatgaaaagtgattttgcaaaattaggcatcacagaatgttagaagtcatccagtccaacttattcacaacaccccctcccctgcagtcccattttacagacaggaagctccaacctgtagtactcacagatgctgctgagattcatctccacccactcactggaagcaatcaattattttggggggggtgtgtgtgtgtgtgtgtctgtctgtctaaaaggtgtaaatgaggagtgacatttctacattgtttattctgtacttttccttggagttaatgcaacacctcctgtcgcttagattttaaaaggaaaaaggagaaatgtgtctagtcataaaggggttgccgttaggaagtcagacttcagactgtgcgtctaagagtagaatccacttctcaagagactgggaatgtaaaatgaccactcaggttagaatttccaactgacagccaggaggaaaacttactctaaagttttttttgcctagtttaaattgcattttaaatcactgtttaagctattacagtattactgtaaaaagtttcaaagtaatttttagtcattacctacactgaaatttgaaagtgaagtcaacagcatgctttattctaactgctgttaaaactcaaaactattttttttaacaaattacaatattcctcttagattttcttctggacacctatacttcttcctactgtgtccagtattctccagcacatgtacctttgtgtttctctgcccatgtacatacccctgaaagttcaacaaaaaaagctataaaatagcagagagaacccaaaatatttcttatactgccaagttccctttaaaccttgggcacttgctctactacatggttgtattaatgctcataactaagctttcgatgaattagaccaatgtgttctatgttctaaatgatatttagatatctgaatccttctgttatagccaacaataaaaaaagttattaaaaatgttgaaaagtataaaatagtaattataaattagcaaatacccaatttaaaaaagcagttttccttatacagtacaagcaacagtaatttgaatattattcactttcagccaccatttgccctagatgtactttaaagtttttaagcttgtgtttttggagtgaaaatgtatatggatacttattctaataatgtaattcaggtatcaaaaaatacatatgcatgttaaaatgtgatgacagctcatattatagcaactcataacaggtaagtattatttccagaataacattaagtcacttttgtagctctaagtcaatgctgcacaaatggacacttaagattaaggcatcattctgctctggagtagtgcttctgtgaatcccaggaactgtacaaaggctttccgttttaaaaaatatatcttctgttatacttcagttatttcattccactgatcattttcttgcaaatgaaaattgaaaataccagtctataatgttttcatacaccttgctcttattcaaatggttagttatgaacaagtggtactcaattttctattgccactgttacatggttatttgtccctgatttgacgatgccttcttcagctccattctccagccactgagattcactgtccaacaagcggttttttgattcactaagtggtttgataggaaaaggttgatttgagccacttctggcatactcattctggtttgtaacagaagcttgttctggatccatccccacaaggcgagttggaaaactgcaaccatcacccaagcttgaaaatattggaagtagccaatatttcttttcatcaccaaagacttgtctccaatttttactgcatccaagagagaaaccatttccatcaggtccgtatgaaaacgtgggtgcgcggaatgattctattgttgttctattttttccaactagccagcagtggtagctgaaaagtgagaggacgctgatgaagaacattgcagacacaaagaaaagaaaaagtacgtggaattttgcacgtgtatctgtcagttcattcgtccaaaattttataaagtactctaaaactgttgcagccacgaaaaggcaatataatagggaatacaataaaaacagcaggaagaatttgtaattagaaaatcccacacagttattcacccaaggacagtgatgatccatcttaagaatacatgagtcacaggctgagcagtgatgcgcccgatcaggtttaatcagctgacatttttcacaatatctgatagtttttgaagctgatgtggtatagataggtaaagctcttgctgctcttctcaaaatttcttgttgtctttcttggctgaattctttttcataacgttccttttcagaattggacaagtagaactctttggagggggaagcgggagatgtgaaaattgtcatccaataggaccatacaaacataacaaagaacagatggaaagccacaaggtaaacaacggtctttccattttcttcatttccaaaaatagtaaacacgcagagctccaccacgtacgcgtagtaggaccagacgaccacgaaggtgatgaagagcaccggcacccagcccacgacgcgctggcagcagcgccacagcgtccagggcgccatgttccgctggcggctgccgagccccgcgtcccaccgttctggggagcgcgggagccccggcgacggtgactcggacgctccaggcggctgctggtccagctcccccgcctccgaggcaggacttgtgggagcaaaagt

SEQ ID NO: 13040 - RNA, 1834 nt, Homo sapiens
  source 1..1834: mol_type = other RNA
gctgggattacaggcatgagccaccacacccagccaaaaaaaggttttctgaggaagtatgatcagaagaaaatggaatgtgcttgaaagagatctaaagggccatggaagttaaaaggtttaactctatagaacagaacacgaagtatggaaaggttctttttaaaaacacttgtcttttggaacaaaatccaaattgtccccatgatttcgtcctttgacattatgttcatcttggttatcttagtcttttctcagacttcacagacaattatctaaaagcccctggctaagtgaatgcttatgactgtggtcacaaatggatggcttggattttatttgtcttgcagtgtttgtaaattttttgatgtatactgttattgccaacttacatactccatatgtatatggattgtatgtgtatgtgtgtgtgtgtgtgtgtatatatatatatatttgcattccccaaatttaaaaactacaatttggagatttttttccacacaaaaaatcagaaaattggcaacactctgccccatttccacatggcaacaatttagacaggccatgagctctccacatggctctgatcccaccactcttgtctcaaacaaatctagtcagttgtacgtatattatgaatgtatattgctgtgcttctccttcctgcctgactccggaagactcctgtctcagtctctctcaacatgtctgaaggacttaggggcaagtgtcagaggtgaaggccctagtctgagtttaatgtctggggccagcttgaaacagcagctagtattttgagctctaagctaacactctggactttcagtcatgttttctttccccagtgaaatagaaaagtttgatttcaaagaggaaaagtgtgcaatacctgcaacatacataaaacctatttaattttactcaggagtgggaatcaagaaacctgggttctgtttctgactcacttcggatagagaagggtagttaagctgtccttatgtttcttatcaaatgaggaaaatactgtggtagttcatagcaatttggggagttttagagtctatggaaaatggaagtgctatttgtaacttagattgaatgttgaaacttgtgtttgtttttcaggcacttacggaacttaactggatgttctatgtgtctagtaatcagctgatagtagatattattctactcctatattgggatgcaaaatagcagaaatcatacagtctatgctggtactttcagcaaagactttacaacagtaatcagttcatgaaactctgtgttctgaaagtggccacagtcagtgaatttgtgcaatttggtttccaacctatcggccacttcttgttgttccttccagggaaggaacgggtcgtcagtagagccaaactgcacaatgtaagggcagttggccttgatcttctcccactgccaggggcgggtgaagtatccacttgcacgctcattttcatcccccaagtctgatgtgtacgcagacactaatacaatagcatatactcgatgtgtttctgcatacctcatggccgcgatggccccagaactgtggccaatgatgatagtcttctcatcacagtgcagctctgtctccatgaagggcagccagatgctctctcgtgctgtaacttctccagctcctttttcacccagccataccagccgtgggtggtcacatccccgcctccgttcccgggaacaatcactgccttgctaggagaagccatgagtgcagcgaggccagagttccccagcgcgggtccagcggagctgagcccagcctgctcccgcagggagcctgcgccgcggc

SEQ ID NO: 13041 - RNA, 1852 nt, Homo sapiens
  source 1..1852: mol_type = other RNA
gctgggattacaggcatgagccaccacacccagccaaaaaaaggttttctgaggaagtatgatcagaagaaaatggaatgtgcttgaaagagatctaaagggccatggaagttaaaaggtttaactctatagaacagaacacgaagtatggaaaggttctttttaaaaacacttgtcttttggaacaaaatccaaattgtccccatgatttcgtcctttgacattatgttcatcttggttatcttagtcttttctcagacttcacagacaattatctaaaagcccctggctaagtgaatgcttatgactgtggtcacaaatggatggcttggattttatttgtcttgcagtgtttgtaaattttttgatgtatactgttattgccaacttacatactccatatgtatatggattgtatgtgtatgtgtgtgtgtgtgtgtgtatatatatatatatttgcattccccaaatttaaaaactacaatttggagatttttttccacacaaaaaatcagaaaattggcaacactctgccccatttccacatggcaacaatttagacaggccatgagctctccacatggctctgatcccaccactcttgtctcaaacaaatctagtcagttgtacgtatattatgaatgtatattgctgtgcttctccttcctgcctgactccggaagactcctgtctcagtctctctcaacatgtctgaaggacttaggggcaagtgtcagaggtgaaggccctagtctgagtttaatgtctggggccagcttgaaacagcagctagtattttgagctctaagctaacactctggactttcagtcatgttttctttccccagtgaaatagaaaagtttgatttcaaagaggaaaagtgtgcaatacctgcaacatacataaaacctatttaattttactcaggagtgggaatcaagaaacctgggttctgtttctgactcacttcggatagagaagggtagttaagctgtccttatgtttcttatcaaatgaggaaaatactgtggtagttcatagcaatttggggagttttagagtctatggaaaatggaagtgctatttgtaacttagattgaatgttgaaacttgtgtttgtttttcaggcacttacggaacttaactggatgttctatgtgtctagtaatcagctgatagtagatattattctactcctatattgggatgcaaaatagcagaaatcatacagtctatgctggtactttcagcaaagactttacaacagtaatcagttcatgaaactctgtgttctgaaagtggccacagtcagtgaatttgtgcaatttggtttccaacctatcggccacttcttgttgttccttccagggaaggaacgggtcgtcagtagagccaaactgcacaatgtaagggcagttggccttgatcttctcccactgccaggggcgggtgaagtatccacttgcacgctcattttcatcccccaagtctgatgtgtacgcagacactaatacaatagcatatactcgatgtgtttctgcatacctcatggccgcgatggccccagaactgtggccaatgatgatagtcttctcatcacagtgcagctctgtctccatgaagggcagccagatgctctctcgtgctgtaattgggtcgggcatgtttttagccaaacactggaaaccaggtatcttctccagctcctttttcacccagccataccagccgtgggtggtcacatccccgcctccgttcccgggaacaatcactgccttgctaggagaagccatgagtgcagcgaggccagagttccccagcgcgggtccagcggagctgagcccagcctgc

SEQ ID NO: 13042 - RNA, 4128 nt, Homo sapiens
  source 1..4128: mol_type = other RNA
gctgggattacaggcatgagccaccacacccagccaattttttgtatttttggttttgccaggttgcccagactggtctcaaactcctgagctcaagcaatctgcccacctcagcctccctagcagttgggactacaggtgcatgccaccacaccttgcaaatttttatttttgtagacatctgtatgttgcccaggctggtctcaaactcctggactcaagtgatcctcctgccttggtctcccaaagtgttgcgactacaggcatgagccgccgtgcctggcaagatatcattcttcagcaaaagcaggcagcaacagcagcggtttgcctgtagctgtggtcatggttaactgaggcctggtttcaagggaaccgagtgaatcagggttaacggcttgatatgctgccattctctggatgcaggatgacatgagaggtcgggagcagtctcttcggcaagccctgctgcagagagcccgcggtggacaggaagggcggggggggcgggcaggctgcgtgccaggccaggctctcagcctggtctttaaggtccatattctgttcctgaggcatccagaaccccagactccttctcataacacaggaacacatcactgggatgctgcacatcacctttgctatttcagatgacgctggaaagtgctgtggacctgaaggtgagtgggcagaaaggggtttgagagtatggacttcctgggcgttcccatggcttcatctgatgagaaaacctaggaaacgtcttccaagtgaacttcctggtttcccttccctagaaaccaggagcagggtgggagtaaagaaatggaggaaggggctgggctcggtggctcacgcctgtaatccgatactcaggaggctgaggcaggagaattgcttgaacctgggaggcggaggttgcagtgagccgagatcacgccactgcactccagcctgggtgacagagcgagactctgtctcaaaaaaaaaaaaaaaaaaaaaaaaaaaggacgggtggggcccacgtgtcaagagggtgtgactgccatggggaggctacatgagtcaagggcagctcagggacctatcctccactgctgcctctgcttcacgaaccagagatcacctaaatcgccctcttagagcccagcccttactcagcgtctccgattagggcaggaagtaagacagggcatgggagagactcagtaacaacccacatgtcccaggaagtttgaagaccgacgatgtgagagtgccggggagcacaggagaggttgggggcttctggggaacgggcgctgagggtctccagccaggagcaaagggccccttgctgctgctacagtctctttttaatgagtttctcgagcttgcggatgcgtgacgactcttgctctggtgttggcgccgtcagggacagtgagccggagctttctgcccccgagggcggtgcggggagccgctggcgcaggagttccagcatgctgctctgctcactcctcttcagccccttcatgtccagtatcttctgaaaggtttctgtgttgcagtctgtgagaagtttgatgtagttgtcaacaaacaccaccaacggttcatgaggggccatcactaccttgaggatcatctcagcccgggtcatgcctttgacaacgatcttggtgtagctggcgggtgccttcctcaccacctgcgagctgatggaggggagatcgagcaggaccatcttcagcgagtgggtgtccagcagcagctgttctgctcccaccatgctaattggcttgcacttgaagaggtgggtgatgaatttgggaatgaaggagtttgcaaatttaacgcagaactgagtgaagtacttgcgtgtggaagccaggttgtcacggatgatggggacgttctgcttgatgtgcagaatgacagaggtgacgtaggggctctggtcaccaacgtgctccacgttctgccactgcatcttgctcatggcagtcagggcaggatcacaggcagcatccagatcctgaaccagcagctgaatactgctggagatgacggtgctgaacgtgtccatctctccagtcagattgattcgttcaatcagacttacatccactttttctttgagtttttcttctagctgctgggtggtggccagacagtactctgccgtgctcaggatgttacagatgaggcagagctcctccagagtgaacttggctacttctgagccctccttttccttgaggaggctgctgatagtcagtcctccactgctggttgtggttttgggcaggttgccagagaggattttccaggcgtattctcggaggtacttctggaaaatggtggtcagggcgatcatgggctccccagtactgagctgagagcattgcaccatgcacttcttgtagtagacaaagaggtcggcgcagctggggagcacggcacccccttcatcagtgttgggcttaggtggcccctgggctttgaaatcagccacaaaccgatctatcagctctccgaggttcttgtcttgggattcgatatacacgtagagatgaggctcaaaacacttggaaacaatgccatgaaatggattgtctggggctttaggcttctttggtgaaggtcacatggtcagtcggttaatggccgacaagagtccagcattttcccagcacctgactctgctttaccccatgtactggtcagatgtcagtgttctgtgttcttagaatgagcaggtcttggtccttacaacagtaacttcaagttgatctaaatctcctttctccgttgccagttcctccatctctggtgttggctcatcttccaggaagggattggtagatgggggtggagactcaagctttttcagggtcccatcggtcagggtgcagccggagaagcgttttgcaagaaacccctcaaagttagttgttctttgaatagcaaaaagaagcaatttcacttcaatttccttcgctctggtacgcataatcttggcaagttctgcccttgtcacatggcaaaattccaccgcaatcctctcagccatgcaccactcacgtggaaacatgcggccgtatttctcctcatagtccacaagctggcgttttatccaggcatagcgtctgtcgattttgtccagccaggcaacatcttggttttcttgaaaaagtaccagatactctgacagatgctgtttaataaactttttgatgatttcctgtttgatcctgggatctagaatattagcaaccagacatgcatctcgtagaacattgctgggtcctcctggtctcttggtgccctgggaaggaaacgcttcttcaaaatctgccaggatttgctgtcctaactcagtctgtgcagccttcactctttcggaaagctgccggatctgcggaatccccatatacttgtggaagtgctccaggacattcatcacaccctgaaggagattagcaacttctccgtattgtcttcgcctggtcatggcttcgagggagtcgacacctcctgccagcatgtgcaggtggttcagtgtggtgattgaggtggtcaggtggcgtttggcgtgatctaattgcttaatatcacgggtgatttctttcaccatttgctctgatttttcagctttgtctttgatatctttgattttgccaaagagttgttggatagctttctgagcctcttcaagcgcttgccgtccatcctgccccacgttcgtctgacctcttacaacagttcgaatattgtcatccagtctccttattttcagcctaattttgttcacgacttcgtctatgttcgccagagattgctcggttgggaacagggtattgatatactcaacagcattgaaatctgctcgatctagagggtcctggcttggaaacacctgctcgatggccagctgcacctcgggcgtgagctgcagcacggcttccagctcctccacgaactccagttcctcctcctccatcattccgccacccggccccctgccgacccccgccgcgagcccaactcaggcctccagccgccacccaggccccagcacagcaactccctcgcggcagcgacctggtgagcccggctccgtcagccgctctgtcagccgct

SEQ ID NO: 13043 - RNA, 4229 nt, Homo sapiens
  source 1..4229: mol_type = other RNA
gctgggattacaggcatgagccaccacacccagccaattttttgtatttttggttttgccaggttgcccagactggtctcaaactcctgagctcaagcaatctgcccacctcagcctccctagcagttgggactacaggtgcatgccaccacaccttgcaaatttttatttttgtagacatctgtatgttgcccaggctggtctcaaactcctggactcaagtgatcctcctgccttggtctcccaaagtgttgcgactacaggcatgagccgccgtgcctggcaagatatcattcttcagcaaaagcaggcagcaacagcagcggtttgcctgtagctgtggtcatggttaactgaggcctggtttcaagggaaccgagtgaatcagggttaacggcttgatatgctgccattctctggatgcaggatgacatgagaggtcgggagcagtctcttcggcaagccctgctgcagagagcccgcggtggacaggaagggcggggggggcgggcaggctgcgtgccaggccaggctctcagcctggtctttaaggtccatattctgttcctgaggcatccagaaccccagactccttctcataacacaggaacacatcactgggatgctgcacatcacctttgctatttcagatgacgctggaaagtgctgtggacctgaaggtgagtgggcagaaaggggtttgagagtatggacttcctgggcgttcccatggcttcatctgatgagaaaacctaggaaacgtcttccaagtgaacttcctggtttcccttccctagaaaccaggagcagggtgggagtaaagaaatggaggaaggggctgggctcggtggctcacgcctgtaatccgatactcaggaggctgaggcaggagaattgcttgaacctgggaggcggaggttgcagtgagccgagatcacgccactgcactccagcctgggtgacagagcgagactctgtctcaaaaaaaaaaaaaaaaaaaaaaaaaaaggacgggtggggcccacgtgtcaagagggtgtgactgccatggggaggctacatgagtcaagggcagctcagggacctatcctccactgctgcctctgcttcacgaaccagagatcacctaaatcgccctcttagagcccagcccttactcagcgtctccgattagggcaggaagtaagacagggcatgggagagactcagtaacaacccacatgtcccaggaagtttgaagaccgacgatgtgagagtgccggggagcacaggagaggttgggggcttctggggaacgggcgctgagggtctccagccaggagcaaagggccccttgctgctgctacagtctctttttaatgagtttctcgagcttgcggatgcgtgacgactcttgctctggtgttggcgccgtcagggacagtgagccggagctttctgcccccgagggcggtgcggggagccgctggcgcaggagttccagcatgctgctctgctcactcctcttcagccccttcatgtccagtatcttctgaaaggtttctgtgttgcagtctgtgagaagtttgatgtagttgtcaacaaacaccaccaacggttcatgaggggccatcactaccttgaggatcatctcagcccgggtcatgcctttgacaacgatcttggtgtagctggcgggtgccttcctcaccacctgcgagctgatggaggggagatcgagcaggaccatcttcagcgagtgggtgtccagcagcagctgttctgctcccaccatgctaattggcttgcacttgaagaggtgggtgatgaatttgggaatgaaggagtttgcaaatttaacgcagaactgagtgaagtacttgcgtgtggaagccaggttgtcacggatgatggggacgttctgcttgatgtgcagaatgacagaggtgacgtaggggctctggtcaccaacgtgctccacgttctgccactgcatcttgctcatggcagtcagggcaggatcacaggcagcatccagatcctgaaccagcagctgaatactgctggagatgacggtgctgaacgtgtccatctctccagtcagattgattcgttcaatcagacttacatccactttttctttgagtttttcttctagctgctgggtggtggccagacagtactctgccgtgctcaggatgttacagatgaggcagagctcctccagagtgaacttggctacttctgagccctccttttccttgaggaggctgctgatagtcagtcctccactgctggttgtggttttgggcaggttgccagagaggattttccaggcgtattctcggaggtacttctggaaaatggtggtcagggcgatcatgggctccccagtactgagctgagagcattgcaccatgcacttcttgtagtagacaaagaggtcggcgcagctggggagcacggcacccccttcatcagtgttgggcttaggtggcccctgggctttgaaatcagccacaaaccgatctatcagctctccgaggttcttgtcttgggattcgatatacacgtagagatgaggctcaaaacacttggaaacaatgccatgaaatggattgtctggggctttaggcttctttggttgatctaaatctcctttctccgttgccagttcctccatctctggtgttggctcatcttccaggaagggattggtagatgggggtggagactcaagctttttcagggtcccatcggtcagggtgcagccggagaagcgttttgcaagaaacccctcaaagttagttgttctttgaatagcaaaaagaagcaatttcacttcaatttccttcgctctggtacgcataatcttggcaagttctgcccttgtcacatggcaaaattccaccgcaatcctctcagccatgcaccactcacgtggaaacatgcggccgtatttctcctcatagtccacaagctggcgttttatccaggcatagcgtctgtcgattttgtccagccaggcaacatcttggttttcttgaaaaagtaccagatactctgacagatgctgtttaataaactttttgatgatttcctgtttgatcctgggatctagaatattagcaaccagacatgcatctcgtagaacattgctgggtcctcctggtctcttggtgccctgggaaggaaacgcttcttcaaaatctgccaggatttgctgtcctaactcagtctgtgcagccttcactctttcggaaagctgccggatctgcggaatccccatatacttgtggaagtgctccaggacattcatcacaccctgaaggagattagcaacttctccgtattgtcttcgcctggtcatggcttcgagggagtcgacacctcctgccagcatgtgcaggtggttcagtgtggtgattgaggtggtcaggtggcgtttggcgtgatctaattgcttaatatcacgggtgatttctttcaccatttcacccgctgctctgtttggccgccagtctcttgtctctctcttcagcaatggtgaggcggataccctttcctcggggaagagaaatccatcgtttgttgcccttgccaatagtgaaaatgttggaaacttgagtgccaaagctgttgccactggtgtctttcacatgaaccacgtcagaagatcccgggtacctctctctgttggggatcacaccaactcttcccaggtgagcacctccagtcaccatatatggcttgccagtgtcgaacgtgatgaaatcggtcatcttgccagtctccaaatcaatctgaatggtgtcattcaccttgatgaggggtcagggtagcggatggtgcgagcatcatgagtcaccagatgagggattccttttgtgcccacaaagatttttctcactttgcacaacttgtacttggtctcctcaggtgtacagcaaagcaacctttggtgtcacggatcagatggaaattctctcctgtcttgtcaatgctgatgacatccatgaacccagcagggtatgttatatcagttcggaccgtgccatcgatcttaatgaaccgctgcatgcaaatcttcttaagtctgttccttaggaaaatgatgaggggaagacactctctcaacttgtggggactggtggacggacgaggagcaaacacaccggtcaatttatccagcatccaatgctttggagctgctacccgcttcagatgcttcttggcaccacgagccatgg

SEQ ID NO: 13044 - RNA, 4034 nt, Homo sapiens
  source 1..4034: mol_type = other RNA
gctgggattacaggcatgagccaccacacccagccaattttttgtatttttggttttgccaggttgcccagactggtctcaaactcctgagctcaagcaatctgcccacctcagcctccctagcagttgggactacaggtgcatgccaccacaccttgcaaatttttatttttgtagacatctgtatgttgcccaggctggtctcaaactcctggactcaagtgatcctcctgccttggtctcccaaagtgttgcgactacaggcatgagccgccgtgcctggcaagatatcattcttcagcaaaagcaggcagcaacagcagcggtttgcctgtagctgtggtcatggttaactgaggcctggtttcaagggaaccgagtgaatcagggttaacggcttgatatgctgccattctctggatgcaggatgacatgagaggtcgggagcagtctcttcggcaagccctgctgcagagagcccgcggtggacaggaagggcggggggggcgggcaggctgcgtgccaggccaggctctcagcctggtctttaaggtccatattctgttcctgaggcatccagaaccccagactccttctcataacacaggaacacatcactgggatgctgcacatcacctttgctatttcagatgacgctggaaagtgctgtggacctgaaggtgagtgggcagaaaggggtttgagagtatggacttcctgggcgttcccatggcttcatctgatgagaaaacctaggaaacgtcttccaagtgaacttcctggtttcccttccctagaaaccaggagcagggtgggagtaaagaaatggaggaaggggctgggctcggtggctcacgcctgtaatccgatactcaggaggctgaggcaggagaattgcttgaacctgggaggcggaggttgcagtgagccgagatcacgccactgcactccagcctgggtgacagagcgagactctgtctcaaaaaaaaaaaaaaaaaaaaaaaaaaaggacgggtggggcccacgtgtcaagagggtgtgactgccatggggaggctacatgagtcaagggcagctcagggacctatcctccactgctgcctctgcttcacgaaccagagatcacctaaatcgccctcttagagcccagcccttactcagcgtctccgattagggcaggaagtaagacagggcatgggagagactcagtaacaacccacatgtcccaggaagtttgaagaccgacgatgtgagagtgccggggagcacaggagaggttgggggcttctggggaacgggcgctgagggtctccagccaggagcaaagggccccttgctgctgctacagtctctttttaatgagtttctcgagcttgcggatgcgtgacgactcttgctctggtgttggcgccgtcagggacagtgagccggagctttctgcccccgagggcggtgcggggagccgctggcgcaggagttccagcatgctgctctgctcactcctcttcagccccttcatgtccagtatcttctgaaaggtttctgtgttgcagtctgtgagaagtttgatgtagttgtcaacaaacaccaccaacggttcatgaggggccatcactaccttgaggatcatctcagcccgggtcatgcctttgacaacgatcttggtgtagctggcgggtgccttcctcaccacctgcgagctgatggaggggagatcgagcaggaccatcttcagcgagtgggtgtccagcagcagctgttctgctcccaccatgctaattggcttgcacttgaagaggtgggtgatgaatttgggaatgaaggagtttgcaaatttaacgcagaactgagtgaagtacttgcgtgtggaagccaggttgtcacggatgatggggacgttctgcttgatgtgcagaatgacagaggtgacgtaggggctctggtcaccaacgtgctccacgttctgccactgcatcttgctcatggcagtcagggcaggatcacaggcagcatccagatcctgaaccagcagctgaatactgctggagatgacggtgctgaacgtgtccatctctccagtcagattgattcgttcaatcagacttacatccactttttctttgagtttttcttctagctgctgggtggtggccagacagtactctgccgtgctcaggatgttacagatgaggcagagctcctccagagtgaacttggctacttctgagccctccttttccttgaggaggctgctgatagtcagtcctccactgctggttgtggttttgggcaggttgccagagaggattttccaggcgtattctcggaggtacttctggaaaatggtggtcagggcgatcatgggctccccagtactgagctgagagcattgcaccatgcacttcttgtagtagacaaagaggtcggcgcagctggggagcacggcacccccttcatcagtgttgggcttaggtggcccctgggctttgaaatcagccacaaaccgatctatcagctctccgaggttcttgtcttgggattcgatatacacgtagagatgaggctcaaaacacttggaaacaatgccatgaaatggattgtctggggctttaggcttctttggttgatctaaatctcctttctccgttgccagttcctccatctctggtgttggctcatcttccaggaagggattggtagatgggggtggagactcaagctttttcagggtcccatcggtcagggtgcagccggagaagcgttttgcaagaaacccctcaaagttagttgttctttgaatagcaaaaagaagcaatttcacttcaatttccttcgctctggtacgcataatcttggcaagttctgcccttgtcacatggcaaaattccaccgcaatcctctcagccatgcaccactcacgtggaaacatgcggccgtatttctcctcatagtccacaagctggcgttttatccaggcatagcgtctgtcgattttgtccagccaggcaacatcttggttttcttgaaaaagtaccagatactctgacagatgctgtttaataaactttttgatgatttcctgtttgatcctgggatctagaatattagcaaccagacatgcatctcgtagaacattgctgggtcctcctggtctcttggtgccctgggaaggaaacgcttcttcaaaatctgccaggatttgctgtcctaactcagtctgtgcagccttcactctttcggaaagctgccggatctgcggaatccccatatacttgtggaagtgctccaggacattcatcacaccctgaaggagattagcaacttctccgtattgtcttcgcctggtcatggcttcgagggagtcgacacctcctgccagcatgtgcaggtggttcagtgtggtgattgaggtggtcaggtggcgtttggcgtgatctaattgcttaatatcacgggtgatttctttcaccatttgctctgatttttcagctttgtctttgatatctttgattttgccaaagagttgttggatagctttctgagcctcttcaagcgcacatggaaatggtgacggcacaaccacaacgctgaatctgtgctcttctaaatactgtttccgtggatgaaagagggaagaggaaaaaggaggccaagttcttccatgaagacagaaagccaaattcccatccattgtacaaacatatctcagtgacttcttgtatcaaggacctgaaatccagaaggctttgctctgttggcagtaattccgcaatttttctaatgcacagcctcaaactgaggatggaattttccttacacgatttctaactactagcaatcaaaagcaagagtgacctgggtactagccagagcagttacagtggtgatgaatggcattttcctcttgagacgcagagtctagtttaaacttgtgactgcctctaacatggaaataagcagatggtgagttacgcttgaccttctttcttggctcctgaagactgccagtttatatggagatggctcagaagaac

SEQ ID NO: 13045 - RNA, 3971 nt, Homo sapiens
  source 1..3971: mol_type = other RNA
gctgggattacaggcatgagccaccacacccagccaattttttgtatttttggttttgccaggttgcccagactggtctcaaactcctgagctcaagcaatctgcccacctcagcctccctagcagttgggactacaggtgcatgccaccacaccttgcaaatttttatttttgtagacatctgtatgttgcccaggctggtctcaaactcctggactcaagtgatcctcctgccttggtctcccaaagtgttgcgactacaggcatgagccgccgtgcctggcaagatatcattcttcagcaaaagcaggcagcaacagcagcggtttgcctgtagctgtggtcatggttaactgaggcctggtttcaagggaaccgagtgaatcagggttaacggcttgatatgctgccattctctggatgcaggatgacatgagaggtcgggagcagtctcttcggcaagccctgctgcagagagcccgcggtggacaggaagggcggggggggcgggcaggctgcgtgccaggccaggctctcagcctggtctttaaggtccatattctgttcctgaggcatccagaaccccagactccttctcataacacaggaacacatcactgggatgctgcacatcacctttgctatttcagatgacgctggaaagtgctgtggacctgaaggtgagtgggcagaaaggggtttgagagtatggacttcctgggcgttcccatggcttcatctgatgagaaaacctaggaaacgtcttccaagtgaacttcctggtttcccttccctagaaaccaggagcagggtgggagtaaagaaatggaggaaggggctgggctcggtggctcacgcctgtaatccgatactcaggaggctgaggcaggagaattgcttgaacctgggaggcggaggttgcagtgagccgagatcacgccactgcactccagcctgggtgacagagcgagactctgtctcaaaaaaaaaaaaaaaaaaaaaaaaaaaggacgggtggggcccacgtgtcaagagggtgtgactgccatggggaggctacatgagtcaagggcagctcagggacctatcctccactgctgcctctgcttcacgaaccagagatcacctaaatcgccctcttagagcccagcccttactcagcgtctccgattagggcaggaagtaagacagggcatgggagagactcagtaacaacccacatgtcccaggaagtttgaagaccgacgatgtgagagtgccggggagcacaggagaggttgggggcttctggggaacgggcgctgagggtctccagccaggagcaaagggccccttgctgctgctacagtctctttttaatgagtttctcgagcttgcggatgcgtgacgactcttgctctggtgttggcgccgtcagggacagtgagccggagctttctgcccccgagggcggtgcggggagccgctggcgcaggagttccagcatgctgctctgctcactcctcttcagccccttcatgtccagtatcttctgaaaggtttctgtgttgcagtctgtgagaagtttgatgtagttgtcaacaaacaccaccaacggttcatgaggggccatcactaccttgaggatcatctcagcccgggtcatgcctttgacaacgatcttggtgtagctggcgggtgccttcctcaccacctgcgagctgatggaggggagatcgagcaggaccatcttcagcgagtgggtgtccagcagcagctgttctgctcccaccatgctaattggcttgcacttgaagaggtgggtgatgaatttgggaatgaaggagtttgcaaatttaacgcagaactgagtgaagtacttgcgtgtggaagccaggttgtcacggatgatggggacgttctgcttgatgtgcagaatgacagaggtgacgtaggggctctggtcaccaacgtgctccacgttctgccactgcatcttgctcatggcagtcagggcaggatcacaggcagcatccagatcctgaaccagcagctgaatactgctggagatgacggtgctgaacgtgtccatctctccagtcagattgattcgttcaatcagacttacatccactttttctttgagtttttcttctagctgctgggtggtggccagacagtactctgccgtgctcaggatgttacagatgaggcagagctcctccagagtgaacttggctacttctgagccctccttttccttgaggaggctgctgatagtcagtcctccactgctggttgtggttttgggcaggttgccagagaggattttccaggcgtattctcggaggtacttctggaaaatggtggtcagggcgatcatgggctccccagtactgagctgagagcattgcaccatgcacttcttgtagtagacaaagaggtcggcgcagctggggagcacggcacccccttcatcagtgttgggcttaggtggcccctgggctttgaaatcagccacaaaccgatctatcagctctccgaggttcttgtcttgggattcgatatacacgtagagatgaggctcaaaacacttggaaacaatgccatgaaatggattgtctggggctttaggcttctttggttgatctaaatctcctttctccgttgccagttcctccatctctggtgttggctcatcttccaggaagggattggtagatgggggtggagactcaagctttttcagggtcccatcggtcagggtgcagccggagaagcgttttgcaagaaacccctcaaagttagttgttctttgaatagcaaaaagaagcaatttcacttcaatttccttcgctctggtacgcataatcttggcaagttctgcccttgtcacatggcaaaattccaccgcaatcctctcagccatgcaccactcacgtggaaacatgcggccgtatttctcctcatagtccacaagctggcgttttatccaggcatagcgtctgtcgattttgtccagccaggcaacatcttggttttcttgaaaaagtaccagatactctgacagatgctgtttaataaactttttgatgatttcctgtttgatcctgggatctagaatattagcaaccagacatgcatctcgtagaacattgctgggtcctcctggtctcttggtgccctgggaaggaaacgcttcttcaaaatctgccaggatttgctgtcctaactcagtctgtgcagccttcactctttcggaaagctgccggatctgcggaatccccatatacttgtggaagtgctccaggacattcatcacaccctgaaggagattagcaacttctccgtattgtcttcgcctggtcatggcttcgagggagtcgacacctcctgccagcatgtgcaggtggttcagtgtggtgattgaggtggtcaggtggcgtttggcgtgatctaattgcttaatatcacgggtgatttctttcaccatttgctctgatttttcagctttgtctttgatatctttgattttgccaaagagttgttggatagctttctgagcctcttcaagcgcttgccgtccatcctgccccacgttcgtctgacctcttacaacagttcgaatattgtcatccagtctccttattttcagcctaattttgttcacgacttcgtctatgttcgccagagattgctcggttgggaacagggtattgatatactcaacagcattgaaatctgctcgatctagagggtcctggcttggaaacacctgctcgatggccagctgcacctcgggcgtgagctgcagcacggcttccagctcctccacgaactccagttcctcctcctccatcattccgccacccggccccctgccgacccccgccgcgagcccaactcaggcctccagccgccacccaggccccagcacagcaactccctcgcggcagcgacctggtgagcccggctccgtcagccgctctgtc

SEQ ID NO: 13046 - RNA, 2761 nt, Homo sapiens
  source 1..2761: mol_type = other RNA
gctgggattacaggcatgagccaccacacccagccacatgagtgtatttttgacagcaatgtagtcaccaataaacgagtaacttcagttaaagtactgtagattataatacacagccctgtaatctaccctggagttcaacaaacggtattgaaaacagactgtgttccagatgcaataggaagagaataaataagataaacaatacataaatcctgcccagaagacgtttgcaattttttaagaggaaaaacatgaagacaaattgttttaagatgtttgctattttcaatagttgaaaaataaacaggagagaagggattatttaactgtgggtatgtagggctgagaaaggcacgcttgacaaaggaaacctgggcagtgttaccagaaagcgttgccaatcatgagtccatatagtgaagtgaaagcaagtttattaaagaagtaaagaaacaaaagaatggctactccataggcagagcagtggcttgggctgctggactgagtatatagtttttttgtgtgttgtttgtttgttttgacacggagtcttgctctgtcgcccaggctggagtgcagtggcgccatctcggctcactgcaagctccgcctcccgggttcacgccattctcctgcctcagcctcccgagtagctggaaatttattgtatttttagtagagacagggtttcaccgtgttagccaggatggtctcaatctactgacctggtgatcctcctggctcggcctcccaaagtgctgggattacaggcgtgagccaccgcgcccagccagttatttcttaattatatgttaaacaaggggtggattattcatgagttttcaaggaagggggcaggcaatttttggaacttagggttctaccctcttttagactgtatgacttctggatgttgccatggcatttgtaaactgtcatggtgctggtgggagtgtcttttagcatgctaatgcattataattcacgtataatgagaagtgaggatgaccagaggtcacttttgtcttcatcttggttttggtgggtttggcctgtcttctttacgacatcctgtttatcagcagggtctttgtgacctgtatcttgcgtggacctccaatcttctgtgactaagaatgcctaacctcctgggaatgcagctcagtaggtctcagcctcgttttacccagcacctgttcaagttggagtcactctggttcaaacgcctctgacaacaggactattggagtactgataggagtttatttgccttaatcacctggccaccctatccctttcttatttcctccctactcctccgtcctgggagactgaattcaaatagacaatggccagagaatatatacaaatagaacactaacctacaaccttcaacaaccagtccaggaaggcaacctactatgtccagtaaccagtccaagaaatcagattactatatttagcaaccagtccaggaagccaagcaataacccttgtagcaatctaccccaaatggccaggacgtgattaataacttacagcttctgtaagttttgtcagggcttccaactcaaggccagctagagagagccaaatatctacccacccctaaataattacataggatgccctgcttttagttagcccacctgcagcttctccatgccaacagccttgaattggcatacctgaagctttcccttttttccactctaaagctttctcactcctctgcctgccgttgagtctctgacaaatgcaagtgatgatggctgactcccttgctattgtaagctccaaataaatttggctttgcttgttctcatttagatggtctgcacttgtttctatactcctgaagaagattcctgctatctggacatgccttccctctggatagatatggcagaagagatgataatggtgtcttttagacctctgctcagcagggtctaggtcccggcttttcatatccaggaaagaactggaggaataggattggtatcaagatgctgacttcattagttgtatgcaatgccaaccacagcaacttcctaccaagacctgaccttctatggcatctttcccaatctgcctgtcaaaataaaatccacttctcagtggtccttttatcccaaaagctgctgcctcaacagtagagagcgtattgccctattagcttacctcctccacaagccatgatggaaaagaaagggttctaacccattggctcaccaatttctttttacttaagcagatgctatggtctgaatatgtttgtccctctcaaattcatgtgttgaaacctaaccctcaaagtgatggtactaagaagtggggcctttgagaggtgattacatcatggggatggagttctaatgatgggattagtgctcttgtaaaacaaggtcaaaggaaatgccttgcctatccactatgtgagtgtagaggtactgtctatgaggaagccggctatcatcagacactaaatttgtctgagccttgatcttggacttctggcctccaaaactgtgaggaatacagatgatcctcaacttacaatggggttatttcccaacaaacccatcagtaagttgaaaaatattgtaagtcaaaaatgcatttaatacacctaacctattgagccttatagcttatcctagactactgtaaacatagtcataacacttaggctacaattgggcaaagtcatgtaacacaaagcctatgtcagaataaagttataaagaatttttga

SEQ ID NO: 13047 - RNA, 3962 nt, Homo sapiens
  source 1..3962: mol_type = other RNA
gctgggattacaggcatgagccaccacacccagccagaagttttaataagagaatgctacagttattagacggcaatcatgtcaaagtctggatggaaatgtggaaagtcagaaatcaaataaattcaagggggctgataaaaatttggcattggcaactacttctgacactttaaaagtgttagagtaaacccctgccttaacattaatggattaaaaactcaattgtgtgatattcagtaaactcttgtcaggttaattaaatttttttcagtctgcactgtcagaaaaatcacaaaatatacttcaacttggccgggtgtggtggcttacgcctgtaatttaacactgggaggccaaggaggttggattgcttgagctcaggtgttcaagaccagcctgggcaatgtggtgaaaccctttctctaccaaacatacaaaaattagctgggtgtggtggcacgtgcccgtggtcccagctactcagagggagagatgggcagatggatggagcctgggaggacgaggctgcagtgagccatgattatgccactgcactccagcctcggtgacagagcgaggtcctgtctcaaaaataaaattaaaaataaaggtacttcaacttatgttttataaaacctttgggaaactagacaggctctcaataagaaccaaatttgagagaagagactacagagaggacaggtgtcaactgtaaaagagtaatatcatattaatattgtaggctgcagtatccagtggttttctgcatttcaacaaatgttcatttctgcaaataattttatttcgcaggtttcttcctttggatacaatgttcaaatattgtgcatttactccttttgattcagttaacaaacaagtattgagcacacctacaagcactagtcaatgttaaggttgtatagattcggtagcaaagttcctgcccccatggagcttacagtctaatggacatcaattctggcaccttcatcagtatacttttttaaagcccaggtcaaactcattttctaagtcctatttcctaggtaacatgtcataaatgtcaaagttttgacagaatgctttactgtaccacttaacaagggttctcagctgtgtggtcactggaccactgggatatgctgagctattgcttaaacactgacttaaataaaacaaatattttaaataagagaatgctactgtaattagaaggcaatcatttcaaagtctagatggaggccaggggcggtggctcatgcctgtaatcccagcactttgggaggccgaggtgggtggatcacatgaggtcaggagtttgagaccagcctggccagtatggtgaaactccatctctactaaaaatacaaaaattagccaggcgtggtggtgtgcacctgtaatccactgaggcaggagaatcacttgaacccgggaagtggaggttacagtgagctgagatagcaccactgcatccagcatgggcaacagagcgagattctgtttcaaaacaaaaaataaaaaacaaaaaaaagtctaggtggaaatgtggagcgttacaaatcaaataaattcaaagaggttgataaagaaaatttttccctcctatgaaatctaattacaagcattcaggttgtacatgagttctgtttttttttttttaatcaccttgtagaacttcctccctctgacaactctctgatgttcttactattctcatcattttcataaaatgtaccagcagcatgaattttgtgatgacttacaagatttgatcgccagctgaacctcttaccacatatctcacatttgtaaggtttttccccagtgtgaactcgcctatgatactgtaattgtgaagaccgactgaagactttaccacatacatcacatttgtatggtttctctcctgtgtggacactctgatgaagttggagacttgaggcctgactgaagtgcttcccacactccccacatgtatagggtttttctcctgtgtgcaccctctgatgcatgtcaaggttcaagctccacttgaagccctttccacactccccacatttgtatggcttttctccagtgtggactttttgatgggcttgaaggtgtgcactccgactgaagctcttcccacactcttcacatttaaatggtttttccccactgtgaactctctgatgggttagaagatgcgaggcctgactgaagaccttcccacactcctcacaattatatggtttctcccctgtgtggatcctacaatgaattttaagatctgctctacgactaaatccctttccgcactcttcacatttgtatggtttctcaccggtatggatcagctggtgaatctgaagtcgtgagctctgattgaagccctgcccacactcttcacacttaaaaggtttctgtacactatgtgctttcagatggattttaagatatgaactctgacggaaggctttaccacatacttcacatttatagggtttttcccctgtgtggactaccagatgcacttgataatgaattttcattctgaagctcttcccacactcattgcatttgtatggcttctctccagtgtggactccctgatgggcctgaaaacttgaactgtaaatgaaacccttaccacacactttacatacgtatggtttctctccagtgtggattctccgatgggcctgaaattgtgaaggctgaataaagcacttaccacattcttcacacttgtaaggtttctctcctgtgtggaccctttgatggatacgaaggtttgagctacaagtgaaacacttaccacagtcctcacatttgtatggtttctctcctgtgtggaccatgcaatgattattaagtgctgatctacgacggaagttcttaccacatgtatcacatttgaatggtttctccccagtatgaattctctgatgttcctgaagatgggaagcatgtatgaaggcccttccacattcctcacaattgtaaggtttctctcctgagtgtaatttgcaatgtacagtaagtgttgatctacgactgaagcctttcccacattccacacatttgaatggtttctctacagtgtggactctctgatgagtttgaagatgtgagctctgactaaattccttaccacacacgtcacacttatagcatttctctcccatgtggactctttgatgaatatgaagggctgagatgtaacagaagctttttccacactcatcacatgtatgagacttctctcctgagtgtaactgttgatgaagatcaaagttgaagacatcagtgaaggattttttgtactcatcacattggtaaaatttctgtcctgtgtgagttgtatatagtcctgccctaacctggcaggacaaatcaccttgtctggggaaccgagaaatacttatcatagagtcttcatacttgattaaatcacttgcaatctgtttccagatttgcccccagtaaagctcttcatgtcgtcctgcttctggaacagtctccacctcactttggatcttgtctgctgatttcccttttctttgagttgctgtcttcattatatcaagctttttttccttttctaaaaggaatacatcatgtttgaaggggtgatgccccactgacagcaggttcctgaagttctccagcatcacatcttggtacagattcctctggacagggtccagcagccccagctcctcctcagtgaagaccacagccacatccttgaaggtcagtccctccttgaatgtggtcatttttcctcctgtttctgggaatttgcagagtcctgagttatgccatttgagagaaggcagaatcgtgcctggaacagtggagctttgctttcagtagccaagaagtcagtccgcgcagtcctttttcaggcgtggaatgtgccgtgacaatcgccccctcttccctggagcggaagtgcccgcgactccact

SEQ ID NO: 13048 - RNA, 4080 nt, Homo sapiens
  source 1..4080: mol_type = other RNA
gctgggattacaggcatgagccaccacacccagccagaagttttaataagagaatgctacagttattagacggcaatcatgtcaaagtctggatggaaatgtggaaagtcagaaatcaaataaattcaagggggctgataaaaatttggcattggcaactacttctgacactttaaaagtgttagagtaaacccctgccttaacattaatggattaaaaactcaattgtgtgatattcagtaaactcttgtcaggttaattaaatttttttcagtctgcactgtcagaaaaatcacaaaatatacttcaacttggccgggtgtggtggcttacgcctgtaatttaacactgggaggccaaggaggttggattgcttgagctcaggtgttcaagaccagcctgggcaatgtggtgaaaccctttctctaccaaacatacaaaaattagctgggtgtggtggcacgtgcccgtggtcccagctactcagagggagagatgggcagatggatggagcctgggaggacgaggctgcagtgagccatgattatgccactgcactccagcctcggtgacagagcgaggtcctgtctcaaaaataaaattaaaaataaaggtacttcaacttatgttttataaaacctttgggaaactagacaggctctcaataagaaccaaatttgagagaagagactacagagaggacaggtgtcaactgtaaaagagtaatatcatattaatattgtaggctgcagtatccagtggttttctgcatttcaacaaatgttcatttctgcaaataattttatttcgcaggtttcttcctttggatacaatgttcaaatattgtgcatttactccttttgattcagttaacaaacaagtattgagcacacctacaagcactagtcaatgttaaggttgtatagattcggtagcaaagttcctgcccccatggagcttacagtctaatggacatcaattctggcaccttcatcagtatacttttttaaagcccaggtcaaactcattttctaagtcctatttcctaggtaacatgtcataaatgtcaaagttttgacagaatgctttactgtaccacttaacaagggttctcagctgtgtggtcactggaccactgggatatgctgagctattgcttaaacactgacttaaataaaacaaatattttaaataagagaatgctactgtaattagaaggcaatcatttcaaagtctagatggaggccaggggcggtggctcatgcctgtaatcccagcactttgggaggccgaggtgggtggatcacatgaggtcaggagtttgagaccagcctggccagtatggtgaaactccatctctactaaaaatacaaaaattagccaggcgtggtggtgtgcacctgtaatccactgaggcaggagaatcacttgaacccgggaagtggaggttacagtgagctgagatagcaccactgcatccagcatgggcaacagagcgagattctgtttcaaaacaaaaaataaaaaacaaaaaaaagtctaggtggaaatgtggagcgttacaaatcaaataaattcaaagaggttgataaagaaaatttttccctcctatgaaatctaattacaagcattcaggttgtacatgagttctgtttttttttttttaatcaccttgtagaacttcctccctctgacaactctctgatgttcttactattctcatcattttcataaaatgtaccagcagcatgaattttgtgatgacttacaagatttgatcgccagctgaacctcttaccacatatctcacatttgtaaggtttttccccagtgtgaactcgcctatgatactgtaattgtgaagaccgactgaagactttaccacatacatcacatttgtatggtttctctcctgtgtggacactctgatgaagttggagacttgaggcctgactgaagtgcttcccacactccccacatgtatagggtttttctcctgtgtgcaccctctgatgcatgtcaaggttcaagctccacttgaagccctttccacactccccacatttgtatggcttttctccagtgtggactttttgatgggcttgaaggtgtgcactccgactgaagctcttcccacactcttcacatttaaatggtttttccccactgtgaactctctgatgggttagaagatgcgaggcctgactgaagaccttcccacactcctcacaattatatggtttctcccctgtgtggatcctacaatgaattttaagatctgctctacgactaaatccctttccgcactcttcacatttgtatggtttctcaccggtatggatcagctggtgaatctgaagtcgtgagctctgattgaagccctgcccacactcttcacacttaaaaggtttctgtacactatgtgctttcagatggattttaagatatgaactctgacggaaggctttaccacatacttcacatttatagggtttttcccctgtgtggactaccagatgcacttgataatgaattttcattctgaagctcttcccacactcattgcatttgtatggcttctctccagtgtggactccctgatgggcctgaaaacttgaactgtaaatgaaacccttaccacacactttacatacgtatggtttctctccagtgtggattctccgatgggcctgaaattgtgaaggctgaataaagcacttaccacattcttcacacttgtaaggtttctctcctgtgtggaccctttgatggatacgaaggtttgagctacaagtgaaacacttaccacagtcctcacatttgtatggtttctctcctgtgtggaccatgcaatgattattaagtgctgatctacgacggaagttcttaccacatgtatcacatttgaatggtttctccccagtatgaattctctgatgttcctgaagatgggaagcatgtatgaaggcccttccacattcctcacaattgtaaggtttctctcctgagtgtaatttgcaatgtacagtaagtgttgatctacgactgaagcctttcccacattccacacatttgaatggtttctctacagtgtggactctctgatgagtttgaagatgtgagctctgactaaattccttaccacacacgtcacacttatagcatttctctcccatgtggactctttgatgaatatgaagggctgagatgtaacagaagctttttccacactcatcacatgtatgagacttctctcctgagtgtaactgttgatgaagatcaaagttgaagacatcagtgaaggattttttgtactcatcacattggtaaaatttctgtcctgtgtgagttgtatatagtcctgccctaacctggcaggacaaatcaccttgtctggggaaccgagaaatacttatcatagagtcttcatacttgattaaatcacttgcaatctgtttccagatttgcccccagtaaagctcttcatgtcgtcctgcttctggaacagtctccacctcactttggatcttgtctgctgatttcccttttctttgagttgctgtcttcattatatcaagctttttttccttttctaaaaggaatacatcatgtttgaaggggtgatgccccactgacagcaggttcctgaagttctccagcatcacatcttggtacagattcctctggacagggtccagcagccccagctcctcctcagtgaagaccacagccacatccttgaaggtcagtccctccttgaatgtggtcatttttcctcctgtttctgggaatttgcagagtcctgagttatgccatttgagagaaggcagaatcgtgcctggaacagtggagctttgctttcagtagccaagaagtcagtccgcgcagtcctttttcaggctctgctctcccacgaggcttcttttcccataaccggaccaccaggtcccagcgagccccaatcttaagtccctgacattaggaggggcccgcgagtcgcggaactggaagaaactaccgtggaatgtgccgtgacaatcgccccctcttccctggagcggaagtgcccgcgactccact

SEQ ID NO: 13049 - RNA, 3657 nt, Homo sapiens
  source 1..3657: mol_type = other RNA
gctgggattacaggcatgagccaccacacccagcccagacttactttttttaaaataagactaccagaggccgggtgcagtggctcagtttgggaggccaaggtgggaggattgcttgagtccaagagtttaagaccagtctgagcaacatagtgagaccccatttcattaaaaaaaaaaaaagataaaataagactatcatatagagctgtgtaatgtagtgagcctacattacaaaaatatatacaaccacacagagaatatgtaattacaccttgcctatatccataaatgatttgaagcaggtaacacatttgcttttaaatgccatttacaacatagactcttgaatgacatgaatttgaaaatgaagtattttttcagacttaaaacgttgatgtgctaatgtagcttactttaaaaaatgatttccaagtggggaaccaactacattgggaaaagacagtcagattcaaggacagtgtcataaaattgctggttttccttagtcaccctgactttatttttttgagacagagtctcgctctgtcactcaggttggaatgcagtggcgcgatctcggctcaccgcaatctctgcctcccgggttcaagcgattctcctgcctcagcctcccaagtagctgggactacaggcacatgccacagttcccagctaatttttgtaattttagtagagacagggtttcaccatattggtcaggctggtctggaactcctgacctcaggtgatccacctgcctcggcctctcaaagtgctgggattacaggcatgagccatcgtgcccagccactctcactttaatactatgaaaaatgctacttagatttttttctatactgcctacattccaagttattaaagtttaaaaccgtatgaaagcatttatgaagattctgaattgtatttctcattaaaagaaaagaaatgtgagtcatgtcccgaggcttatgtagaggagaaagcagaaggccattgtcagtcattttgaaagttaaaactcagcacttaatgtgaatttagatccatttaagagaggattcctcagttttatgggtttgtgctcctctgagcatcctcagggaagtgagaacacaagacttctgttcttctaagcaaaaatcattatcaaatgaatttattaaagagctatcccgagcaaattgcaattgtatgtatgtagctacataggcttccatgggaattgtaaatggctagctgagggcactttcaattgattcagagtaaaacaatctgaggcttgtaacaaatgtacaaaaaactaaaatcaatgagtaactctaataggaagaaactgtttgcattccttatgttacagtttgcttgtaaactgtatgtactttgtttcttttctcaacactgttttaaaactccagcattttcacctaaaagaaaacacaggctcttcataaatacctgtgaacaaataaatgaaatggtgactgaaggcgatttctgcagtagctttctctcagagataattatttttttttttgagacagagtctcgctctgtcgcccaggctggagtgcagtggcgcgatctcggctcactgcaagctccacctcctgggttcacgccactctcctgcctcagcctccagagtagctgggactacaggcgcccgccaccatgcccggctaattttttgtattttagtagagacgggctttcactgtgttagccaggatggtctcgatctcctgacctcatgatctgcccgcctcagcctcccaaagtgctgggattacaggcttgagccactgcgcccagctcaaagataatattttatcttgaagctagtgcatcgatttgtaaagctcatttaattttctacatactcaggatttgcatattgacttaaaatctgactttatcatccatgccgttatcaactagacaaaaaaatgtatcaagcacccacaggatgcacagatctatctctgaactggtgtagtggtattaatctgttctaagactagaattacatttttttttttaagaagctacagtccactgaaaaggaagtattatggtttttctgagaagaaaagttgctaaatactgcagcaaactcaggcttttcctgagaaaagccacaaacaaaatcatctctgaaattttttaagcaacaacttcctgaagcgtggaatttatggggccagtgagacactaaaatttcacaactctcacatacattatctatctaggactcagtgaagatgttcttcagatttttatttaagttaaattggtaaaatacaaaaagaaaatctggattgagtttcaaatcatcttaaatagcaatcctatgaacaattataactgcaatttcaaacactaagacttaaatatacaacttgatcatacaattatctcaaaacatatgatcaaaaactttggtcaagagcttctttcatgaattcttcaaggacagctatcacatttttggcttcaggcatttcttcatgttccactttaacaatcttcaaaagtatatctccactaccacagttctttaggaacatgtaacatttaaacaaagcataatgattcatttctgcctgtcggataaatctcttcaaattgtttgtgtcttgtatggcctttagtttaaagttctccagtacttgtcggaaaagaaaagggttacctcctttggcaccatttaaaaaagcttgcatccaatcctcacaaaaccggttacttcctgcattgcagaactgaggctgggagctgctgcaatcgatgaccacagacttatgctgctcctctgtcatggccatgcacaaagaagtcatggtgccttcatgaataagtccttgaagactggccacactcagaaacctgttaatgtctctctttgttttttcatctgattctttaacttcaacaggagtgtaactcaaagcagcatgtagcagaaaggtaagcttttcctgaaagagaagaacaaccctttggattgggcatacaacatcctcaaaccagctgctcagataggattttatgtgactctccaggccccttgcctcacaattcatgttatttttcagcccttgaatgtacttgtccaattcaagcctgaaaagctcaagtcctttttcagaccctcctaaaaaacagaccacatattctgaagggttacgttcagagtctatcgttactgtttcaggaagcagtttttcattttggaaaaggcagtaataacaaccaactcggtaacctggaatttttagctccacagatgcaacattacccagcccttcaaagactgcacctcttgaaagacgcttagcaatgaaactgcgcagctctggctccacttcggatggtagattagtatctgccaaggagaggctgaaatcatcaccagagggagtttctgcatttgtgccacttgggcttccgtcctcactgtcccctcgttgctgtgccaatctgcttccgcgatagctgtaaagacagtagtggctgctggacggcggctcgagtctccgctcctcggctgagcctccctcttcgctgctctctagttccttttcatctccatccatcgactcctgcaaagaggggagcattgcggcggcctctgagcggccctgtgtctccgcc

SEQ ID NO: 13050 - RNA, 1723 nt, Homo sapiens
  source 1..1723: mol_type = other RNA
gctgggattacaggcatgagccaccacacccagcccatgcattcaactttaatagtaaaaatcaaaactcagaaataatttttaatgtccactgataggagactattaggttgttatatatttgctcagaatagtatgctttcattgaaattaattatgaagtttatgaagcaaatttgaaaatgtatgttaaataaatctaagtttaaaaaagcatgctgtaaatttctgtggaataattgtaactatataacataatagaaaaaatgagtacaagtaaaataatattataatagtaactatgctaggaaagtgagattaaacaattttaacttttctatagccctgtggttaggagttgagtattattaatcacctgcattgaacaactcttttaatggaaatttctcagctcctgcatcacagttataatgtgaattttggaaactcgagtcaaaagttcataacttatttttcttcatttattgcaacataaacatctccaacataaagggatactctacttttatgctccactcttcattcacactttaactgacagagtcacctccaaaaaggcaggagttcctgggaagtatcctcaagcctcttatcatttgcaggagactgtatatgcttcaggttacacaaaacttgactcttcccctcattatgaagtttgccttcaagagccaatgtcaacagagctgggcgctcaggtagactttgaggcactcctcgcacacggccttcttgcagcaaggcaggggcttgatgggcttgtcttccaggcacacccggcacatcagcaccatgaggggcacatagggatcccctacaccgcccaggccagagtagggtggagctcccaacaggctgggcatggagaacggctcgggcgccaggtagaactccagctcgatgctgccgccgtcgggggagagggaatccgttgggagggacagtcgggggctggggaaggaagagcgggtgctgggagggttcaacactggcggagccccaggtggcgacgcgggcggcgagagctgctccgaggcgggggcctcgggcaggtcgctctccacgcagtacacggagcagaagacttgtctcttggcgagggacgggcgccgctgacccagcacgtccaggaccagtccgtcggcggcccccacgcgggtcctgggctccagctcttcgccggggggcgcctcctgctgttcatcccctccctcttttcgatccccagcttcctcctcttcctcctccagctccaactgcagtggcaaggtctggggattgagaggcccggtgagtgccagtcccgcaggctgcgccggtgctcggctcttactccagcccgggggccccaggctcctcgcgggctctggggcgctggtgtccgcgcagccccagtcgcttccgcagccaccgccgctcggctccgcggaggcggcgcgcagcgggggcgcccgggcgctgtccccctgaggcctcgggggctcagggtggcccgcagtgccactggccagggtctgcgactcctggggcccgccgccgccgctcaccgtgctctgctcctcgcccatcgccgcccgcggcccgcgccgccgctgcccatccagccgccgggacccccacccggcgcccgcgggcagcgggggcagtggctcggctcgactcgcggctccgcttctgcttccgggtccttcctcctgggctg

SEQ ID NO: 13051 - RNA, 928 nt, Homo sapiens
  source 1..928: mol_type = other RNA
gctgggattacaggcatgagccaccacacccagccccttaatttcttatatagtgcctagcacacagaagatgctctataaatagttactgaatggacaaatgactaaactttgaaacttctttgaccttactatgctcaaatatcacttctgatgttcttctccgactctctcacttatcttatatatgtctgcacacgttttttcctcattagactgtaaggtccattctgagcaggatctgttctacccagaccacaggtttctgcctttttttctggctcatcaagcaggcatgtttacccactctttttatcttcatgtttcccaggtcagcccaatgtgaggactttaagtagtagaaggaagtttcgatggtgacggacagtcactttctagagctcagatcactgctgcctccagcacttgtgggatggaaaaaatgaagaaattacagttgccctaaaaatgtcccccacttcaggaacctgaatattttacacagcaggagatacatcggaagtcctacagaatctcttgactttgggagatgcaactgcttttctattaggataacctaattttctgtgtccattttctcagaatgttgtgcccaacgcgttctgtttcctaaatacccagccttccttctggtagaggcaagaaaattatgctagcattcgctcactgcatgttttgagcgtttgagttcagagtacagctattctctctcctcgtaatgtaaacacaggttcccacggcggcaatgggagactcccctaaggggctcttgacgtacagggagacttccagatatggtacacagatgtcacattgctagaacgtctctagacggcaacgaaacattaaagcctaacctgaggtaatccctcaccggcagtgaagctcctctgctaggcactgtcgt

SEQ ID NO: 13052 - RNA, 1018 nt, Homo sapiens
  source 1..1018: mol_type = other RNA
gctgggattacaggcatgagccaccacacccagccctaaaagaaactttagttctcagcctccaatagccttcctaatcctccatcccccaaagtagtgggcatagaggacctgacagaaggagagtgtggctggctcagttcagccatccctgctgcaggaggagcagctcagagcccagaggcatctgcagaaggaaagactgacagctcctggcaagccttggcccttggcctcaccaaacctcagtgggtgctggtgcagttaacctgctgagaattccttcttggcactggtggttcatgatgttattcttcccatgcagacatccctgggcttgagtagggcttggtgggttccccttgttaggccaggtgaggtggctctcgcctgtaatcccagtgctctgagaggctgaggcaagaagattgctcgagcccacgagttggagaccagcctgggcaacacagtgagacctcgtctcaaaaaaatcttttttaattagccagacgcagctactcgggaggctgaggtgggaggatcacttgagttcaggaggtcggggctgtagtgaactgtgattgtaccactgcactccagcctgtgtgacggagcaagaccctctctctctaaaatgaaagtttgggctgaactttcatcccatctggactcagagtgacaaaggctgtaatgattccactaatcttgctccttctgtcttctctctttgaagatgacaccaagttgaatcccttggttctgatggctgctgaactccgacttcttcgctgagacatgactgtgggaacagcctccagctatctgctcatcagaggtgctttcctcaacctcctgcaccacctccaagagaaacagcatgcaaagcgtcggccgtgggtccagagctcagctcccacactagcaaggttttgtcactcttggtgggaaccgcaaaaggtagcagatccgccagcctcccttcgctgagcctgcgcggctaaggctcgcgcagtactgc

SEQ ID NO: 13053 - RNA, 1725 nt, Homo sapiens
  source 1..1725: mol_type = other RNA
gctgggattacaggcatgagccaccacacccagcctagctaaacctattcttaaggtgaccctagaaggctctgctgtcttctggaggctgaaacctccactttagcataactaaagtgacagtaacatcagtgtcctatgaggaaagaacaaggaaggtgctcagtaatgcagcactccctcctccagagcttggtaagcagggcctgagggagccagcagagccagctatagacaccatccccccagcagggccccaatgtctccactaggtggtgtctcctcatttcctccatggcctacaaacctccctgctaatgcacacagtggctgggccatgggttggcagtggctgactggtcagcaggtacgtgcctgagtgaggctggcctgtcagccactggggctcctccatctctggcccatggctaggccccccagcaggcaagggtaatcaactgtacttaaaaaagtgagcactgcacgaagggttgcctttggatttctgaaaaatacccccaaggaactgaacggaggggtgtacacactgccaaccacagacagtgctagccagactcaaccacagcagcccttatgttctccagagtagagcccagaggaagattcaaagccagcggagaccagtaaagggtcgcaggaccaaaacaggtgtcaacaggctgtggccttaacctctcaggcccaaagcctttctgctacacaggccttcctcttcactaggaccagatacacgccaagctgctattaggaagcgttttattgaccagcagagcagggatattcatttagcagctcagcttcagaccctcctctcccacatccttttacacaggtgtgtaaagtccttttaatgcaaaaggatttccagagtctccagggacagaaccaggggcttccctgggccaaagtaatcccattccaatctccccactggtcagacaccatcaccccagcccacagtgaccgtgggccttagtcctgggcatcggctttcagagcggctttgtacttccccctcatctccttgggtaatggcaccaggctggggcagggcacctgcccttccacttcacagatgcactcccgcaggcagtactttcgagggccgaagttggctgggtgagaaagctgctttttctcctcctcctcttccctgagggtttccctctcaacacccttcccacacacccctttcttcctcaaattctctgggctgagaagtttgttccttccaggtcaaaccaaacaactcactcattcttccccaagatttttctgatgtgctccatgatctccttattgctcttggtctccacatccaccaggacctgctccccagaatctaagtagaatcgcaggaagggtgacggcgtcatgttcttaaacatcatgatctgcacccaagggtttttgtattgaatctgaggtatgttgaaaaacacaaacttcctggcgccctcgcccagctccccatgcgtgttgtaattcactgtcatgaccttcacggagtccttgaacaccacgttcccctggctcagatattgcagggtgcggcggatggggaagcggcccttcatgggcatggcggcaacggtggcggggccgaccccacgggccgcgagccgagcagcgacgagaaaggactagctagcacccgcgcggatctcacgcggcttctccccagagccaggttccacttcccgc

SEQ ID NO: 13054 - RNA, 1625 nt, Homo sapiens
  source 1..1625: mol_type = other RNA
gctgggattacaggcatgagccaccacacccagcctagctaaacctattcttaaggtgaccctagaaggctctgctgtcttctggaggctgaaacctccactttagcataactaaagtgacagtaacatcagtgtcctatgaggaaagaacaaggaaggtgctcagtaatgcagcactccctcctccagagcttggtaagcagggcctgagggagccagcagagccagctatagacaccatccccccagcagggccccaatgtctccactaggtggtgtctcctcatttcctccatggcctacaaacctccctgctaatgcacacagtggctgggccatgggttggcagtggctgactggtcagcaggtacgtgcctgagtgaggctggcctgtcagccactggggctcctccatctctggcccatggctaggccccccagcaggcaagggtaatcaactgtacttaaaaaagtgagcactgcacgaagggttgcctttggatttctgaaaaatacccccaaggaactgaacggaggggtgtacacactgccaaccacagacagtgctagccagactcaaccacagcagcccttatgttctccagagtagagcccagaggaagattcaaagccagcggagaccagtaaagggtcgcaggaccaaaacaggtgtcaacaggctgtggccttaacctctcaggcccaaagcctttctgctacacaggccttcctcttcactaggaccagatacacgccaagctgctattaggaagcgttttattgaccagcagagcagggatattcatttagcagctcagcttcagaccctcctctcccacatccttttacacaggtgtgtaaagtccttttaatgcaaaaggatttccagagtctccagggacagaaccaggggcttccctgggccaaagtaatcccattccaatctccccactggtcagacaccatcaccccagcccacagtgaccgtgggccttagtcctgggcatcggctttcagagcggctttgtacttccccctcatctccttgggtaatggcaccaggctggggcagggcacctgcccttccacttcacagatgcactcccgcaggcagtactttcgagggccgaagttggctgggtgagaaagctgctttttctcctcctcctcttccctgagggtttcctcattcttccccaagatttttctgatgtgctccatgatctccttattgctcttggtctccacatccaccaggacctgctccccagaatctaagtagaatcgcaggaagggtgacggcgtcatgttcttaaacatcatgatctgcacccaagggtttttgtattgaatctgaggtatgttgaaaaacacaaacttcctggcgccctcgcccagctccccatgcgtgttgtaattcactgtcatgaccttcacggagtccttgaacaccacgttcccctggctcagatattgcagggtgcggcggatggggaagcggcccttcatgggcatggcggcaacggtggcggggccgaccccacgggccgcgagccgagcagcgacgagaaaggactagctagcacccgcgcggatctcacgcggcttctccccagagccaggtt

SEQ ID NO: 13055 - RNA, 1636 nt, Homo sapiens
  source 1..1636: mol_type = other RNA
gctgggattacaggcatgagccaccacacccagcctagctaaacctattcttaaggtgaccctagaaggctctgctgtcttctggaggctgaaacctccactttagcataactaaagtgacagtaacatcagtgtcctatgaggaaagaacaaggaaggtgctcagtaatgcagcactccctcctccagagcttggtaagcagggcctgagggagccagcagagccagctatagacaccatccccccagcagggccccaatgtctccactaggtggtgtctcctcatttcctccatggcctacaaacctccctgctaatgcacacagtggctgggccatgggttggcagtggctgactggtcagcaggtacgtgcctgagtgaggctggcctgtcagccactggggctcctccatctctggcccatggctaggccccccagcaggcaagggtaatcaactgtacttaaaaaagtgagcactgcacgaagggttgcctttggatttctgaaaaatacccccaaggaactgaacggaggggtgtacacactgccaaccacagacagtgctagccagactcaaccacagcagcccttatgttctccagagtagagcccagaggaagattcaaagccagcggagaccagtaaagggtcgcaggaccaaaacaggtgtcaacaggctgtggccttaacctctcaggcccaaagcctttctgctacacaggccttcctcttcactaggaccagatacacgccaagctgctattaggaagcgttttattgaccagcagagcagggatattcatttagcagctcagcttcagaccctcctctcccacatccttttacacaggtgtgtaaagtccttttaatgcaaaaggatttccagagtctccagggacagaaccaggggcttccctgggccaaagtaatcccattccaatctccccactggtcagacaccatcaccccagcccacagtgaccgtgggccttagtcctgggcatcggctttcagagcggctttgtacttccccctcatctccttgggtaatggcaccaggctggggcagggcacctgcccttccacttcacagatgcactcccgcaggcagtactttcgagggccgaagttggctgggtgagaaagctgctttttctcctcctcctcttccctgagggtttcctcattcttccccaagatttttctgatgtgctccatgatctccttattgctcttggtctccacatccaccaggacctgctccccagaatctaagtagaatcgcaggaagggtgacggcgtcatgttcttaaacatcatgatctgcacccaagggtttttgtattgaatctgaggtatgttgaaaaacacaaacttcctggcgccctcgcccagctccccatgcgtgttgtaattcactgtcatgaccttcacggagtccttgaacaccacgttcccctggctcagatattgcagggtgcggcggatggggaagcggcccttcatgggcatggcggcaacggtggcggggccgaccccacgggccgcgagccgagcagcgacgagaaaggactagctagcacccgcgcggatctcacgcggcttctccccagagccaggttccacttcccgc

SEQ ID NO: 13056 - RNA, 1374 nt, Homo sapiens
  source 1..1374: mol_type = other RNA
gctgggattacaggcatgagccaccacacccagcctataatttcttttgatcctaatgataacaccatggaagtaagattattatatcagattttcccaactgtccccaaaacgttgaaattaaaattttaaccaaaaactattatttttgagtgttaaaaaaagaagcaaccaccaccaccaacaacaacaaaagctaattcacacacatagtgtaaaagaatagagtaaaaaatcaaataggcattaactctagtatctatgagttattatatttaggaagtcagacaggccatgagctctcttgtagaaagctactcttctgagtgctatttgaaaagtgttaaagactaactttaaaccacaaaacaatgctaagaatattgcctgtatgaattaaagacaaataaattgctgtagatatagggagcactggttaacagaaagtcgtagggtcaaatgtatcaagaacctgataaacatctgagacatgcccattccagaaagtactgttgaaagcgttagacattctcctaattcctttctgtccatgaaaccatgccacttttcagagaagaggcagacgccgaaagtcccaacattagcccatatttgaagccagccctgaatacaatccacccaaagtaacttctggaaaaatatacctttatatttaacattaactgtaagaaaaaagatctcaactgtaatcaagatcatatgtttaaaataaatcatcaaatataaataactttatataaaataaagctcatagagaagtattaatatggggtagaaaaagtacattaatattagtgtatttattcattaaaatatgaatattgggtagaaaataactaatattattaaccaataaggaagacaacaaaaatcaatgaaagtagcattattggaacatgcagtgcaaatgaaaaaagttccaaacacattttctgctcatacttcctccagtaacatggccatctctgccatttcttactgttaacattaatctcattactggaagtgggggctgaggggaaggtagattaaaattatcaccatgatatagttacctccatagccattaagtaaactgttggtattttaataataagaaagaaaaacaactgggtgcagtggctcacacctataatcccagcactttaggaggctgaggcaggaggactgcttgagcccaggagttaaagaccagcccaggcaacatagggagatcctgtatctcaaaaataaaaaataaaagattagccaggcatagtggcacatgcctgtagttctagctactcggaaggctgaggcaggaggatcacttgagcccaggagttcaaggctacagtgagctggagttgcact

SEQ ID NO: 13057 - RNA, 1024 nt, Homo sapiens
  source 1..1024: mol_type = other RNA
gctgggattacaggcatgagccaccacacccagcctcattctcttattgaacctttatcaaatcacacttcctagtcgggagctttttgagacttcttccagcagccatggcaattcaacccactttagctgggaaatcaactctaattttgaaactggaaagtccagaaattctaggttcctgaggttttccagtagcacttccttatatagctccttttgaaaaggctccagcttcttccactctcctcttgaaaagttcacagctacatccttcaatgttatagattcacaggactcagtattgggacaaacagtgaccattttatcctcttttgagttctcctcttgggaaacagtagaatcttgagagactggatctttttcttcaagcatctgggtcaaatcttctattagggtcaccacttcctcactactctcaggatgttgtgactttacccaaatcctgatctccccaggcaaaatggtcaggaactgctcaaacaccagaagctctaaaatctgttctttcgtgtgaatgtctggtctcagccactgattgcagagctcccagagttgactcagagctttcctgggtccagctacttctgagtaacaaaaccacctaaacctctgtctgaaagactctgcatcagcagcatttcctcttaaaatagcttcttgttccccagaagtaaccactcttgggacctcattttgttcagtcgaggccagagtttgaggttctggtgagatggctgtcatcttgttcaagggcactacagcttgcattgtgtctcaggggcaggaatccagtcccttcacactctagttgagtatcagtacagtccaccaacaggcactatacacagccaggaatatcaaaggttccaggaatccagtttacagtcctgcagaaactgcatcagcatccgcaaacagcaccaacgccaccgcaaagagcttccagaagcttgtcccgcagcgagtgcgcgcgcaagcctgcgggaaccactgcgcctgc

SEQ ID NO: 13058 - RNA, 1645 nt, Homo sapiens
  source 1..1645: mol_type = other RNA
gctgggattacaggcatgagccaccacacccagcctccaacagctttttatgcacctcaatttatataacccattaatcctcaataagtaatacatctgaaaaacagatgatgtttttgaagacttaactcaagtgagcttgctgatgaagtgttttcaatggactaacagactcctgaaaatgctgtgtgggccatgcaggaagagacagctctggggtaccttccattcttccccatctgccactgctccaccactgccagctggcctcccagggcagcctgagcagcttcccatgggtctggccatggtccgctgtgcagggacaggtggtgggtcggggtagaggccccatcaaatatcgctctgtccagaaagtcgatggtggactccgtgtaaacaacctggaagacctggcctagcagacagcaaagctcctccgcagcgaccttgctctctgcagccaggatgaccaggcagcatgcctccacgggcccaactgcactctccgacagggagcctgcactgaggcctctggaactttccgcacacagactctggctgggggagatccctgggtcctgggctgtcttcaggaccaccaggtgtgcagcgtcatcccgaacataggagacggcggcgatgtcatggatgggcaccctgaggatgatatcctccccgtccctccaggccagcttgacgttgtacgcagacaggctgagcacagcatcgtgctcctgagtcaagtgtcccggaagctggtgggctctctttgcattgtctatgaaatgcaggatttcagtcctactggagggattcaggtatcctggtatggacgttaactgacctaaatactcattctccatggaataccctgtgtgaaattctgtttgaggaatttctttggagagattctggttcctcctctgccgacagctactatgcattctctactcacttctgaatttgttgaaaaatatggccagatgttagccctccctctgaaaaaaacatgactgaacaggaagaccagaaaccacagcttccttctgcaaagccactgaagctgtttacaattttttaaaagtttaaaaagcaggcagcacccagaaactgttggcaaaatccaaacagtctgcatgcacaaaaagacacaaagtaaaccagctcattttccctacttcccacagcacgcgaaccccacaagcagcctccctgcatttccagcagaaattctgcagtcaacagaaggacattaatttcaaagtccaccattctgcacattcaaatgccaaagctaaacaagcagacagaaagcactgtgaggggctaccatttcctggagacaacaggccgtgctgttggtgaagacccatggtacctgcctcatacgaagggtggaaacacgcgacaaggctgttccagttaccccatttgcagtgcttgctcaaaggcagcaagatctttacagagataactccattcccaggtggggcttgggcagggcacaccgggctctacgggtcctcagcctacaagtgcctctacctgcctccaggactcatgagtttgagtcagcagcactttgaaattaaacagcgtgcctctggccaagctcacttcttcaaggcaaatttcctaatct

SEQ ID NO: 13059 - RNA, 985 nt, Homo sapiens
  source 1..985: mol_type = other RNA
gctgggattacaggcatgagccaccacacccagcctccaacagctttttatgcacctcaatttatataacccattaatcctcaataagtaatacatctgaaaaacagatgatgtttttgaagacttaactcaagtgagcttgctgatgaagtgttttcaatggactaacagactcctgaaaatgctgtgtgggccatgcaggaagagacagctctggggtaccttccattcttccccatctgccactgctccaccactgccagctggcctcccagggcagcctgagcagcttcccatgggtctggccatggtccgctgtgcagggacaggtggtgggtcggggtagaggccccatcaaatatcgctctgtccagaaagtcgatggtggactccgtgtaaacaacctggaagacctggcctagcagacagcaaagctcctccgcagcgaccttgctctctgcagccaggatgaccaggcagcatgcctccacgggcccaactgcactctccgacagggagcctgcactgaggcctctggaactttccgcacacagactctggctgggggagatccctgggtcctgggctgtcttcaggaccaccaggtgtgcagcgtcatcccgaacataggagacggcggcgatgtcatggatgggcaccctgaggatgatatcctccccgtccctccaggccagcttgacgttgtacgcagacaggctgagcacagcatcgtgctcctgagtcaagtgtcccggaagctggtgggctctctttgcattgtctatgaaatgcaggatttcagtcctactggagggattcaggtatcctggtatggacgttaactgacctaaatacttcttgcccttcttgccctcctcttccatatcgccgcgtgcggctcccgcggcccgcccggcccgccccgggagccccgccgccagcagccgctacatgctcgacccgggcccgccgcccccgcgctccc

SEQ ID NO: 13060 - RNA, 1154 nt, Homo sapiens
  source 1..1154: mol_type = other RNA
gctgggattacaggcatgagccaccacacccagcctccaacagctttttatgcacctcaatttatataacccattaatcctcaataagtaatacatctgaaaaacagatgatgtttttgaagacttaactcaagtgagcttgctgatgaagtgttttcaatggactaacagactcctgaaaatgctgtgtgggccatgcaggaagagacagctctggggtaccttccattcttccccatctgccactgctccaccactgccagctggcctcccagggcagcctgagcagcttcccatgggtctggccatggtccgctgtgcagggacaggtggtgggtcggggtagaggccccatcaaatatcgctctgtccagaaagtcgatggtggactccgtgtaaacaacctggaagacctggcctagcagacagcaaagctcctccgcagcgaccttgctctctgcagccaggatgaccaggcagcatgcctccacgggcccaactgcactctccgacagggagcctgcactgaggcctctggaactttccgcacacagactctggctgggggagatccctgggtcctgggctgtcttcaggaccaccaggtgtgcagcgtcatcccgaacataggagacggcggcgatgtcatggatgggcaccctgaggatgatatcctccccgtccctccaggccagcttgacgttgtacgcagacaggctgagcacagcatcgtgctcctgagtcaagtgtcccggaagctggtgggctctctttgcattgtctatgaaatgcaggatttcagtcctactggagggattcaggtatcctggtatggacgttaactgacctaaatactttacctccttctcaatatagtcgctcagcagtctgtctggctcgacgcgctcaggcaatgacaacaccacagtgtgcagagggcgcctctctgtcaccttctcatgggctttcttatctctactcttttcaccttttaggaatactcgtttaaatggcgagacaattccaggctcattctccatggaataccctgtgtgaaattctgtttgaggaatttctttggagagattctggttcctcctctgccgacagctactatgcattctctactcacttctgaatttgttgaaaaatat

SEQ ID NO: 13061 - RNA, 2042 nt, Homo sapiens
  source 1..2042: mol_type = other RNA
gctgggattacaggcatgagccaccacacccagcctgaaatcaatttttaaaaattatagttgtggaggtttcaacaaaagagaatggtttaaaaaacaccccaaatagtggtagttgtcttgagatggagcaagttgccttatgaaggagtgaggtccctatcagaaaagatgacctgttagacatgttctagagcaaaggctggcatgctacagcccttggataaaatctgtctattgcctgttttttatatagatttattggaacacggccacgcccacttgtcaatggctgcatttgcaccataagggcaaaattgagtagttgcatagttgagactataaggcctacaaaacctaaaatactatttggcactttgcagaaagaaattatcacattgagttgaactaaatgagctctggttttctaaaagggggacagggtcagttggtagagactataggtgaaaatctgtacaacaatttcagattagtttttatacttaacccttactcaaaccaaaagattacttgccaatctaagacggattccatggttttgacttataaaaagaaatctagcacaatgtgtggcatagagacacccaagtatttactaaatgaatgaattgtatattcaagtgaccatgctttctactctcaccccaaagaagccgactgtcaacccctcttgctggccatagcagattggacaaggggtgggccctggatttgagcagcaatcctgtctacccagcaacctacagaacttctggatatgaaaagatgagctggacctttcacaatctctctcacagaaatttgaactaaaagtatccaggctaggagtattagctcatccctgtaatcccagcactttgggaagctgaggccacttgagcccaggagtccaagaccagcataggcaacagggtgaaaccccatctctacaaaaactacaaaaaaattagccgagcatggtgatgcaggctgagtagtcgcagctactcaggagacagaggtgggagaatcacctgagctcagggaagtcgaggctccagtgagccatgattgcaccactgcactccagcctgggcaacacagtgagaacctgtctcataaataaataaataaataaaggtatgcaaaaatagaggagttaatggttgtaatcagagctgaaaaatccaatatggagagaatggccttgaaatggctgtctttaccctcaagatgtcttagactaaccagaaaagcccttaggggggagacttatacatgcacctaacatatgtaaatccaactagaggccttgggcaaaatgaaacaaaaggtgagaatggtgtgggggattcaggccactgctaaaggttgaaatctacctggctgtggaccacaattcacacctttacacaaaggggggtgagggttgaggggttctccattgctagagactctccactctccgggggctcaagtggttcatactagaagcagccattaccacaggctcctttaggccacgttggaaggtggagatggacagcagggccaggtcttgctgctcctcagcgtagcgtaccaggtacacatagacaagcttcttcacctctatgttcttacaggccacgttcttcaccaccgcgggaaacaggtctgaagcattctttcctcgggcaatcatcgccacaatcctcttcatggcctccagcttgagagaatccttgttggtgtccagcatctccttcaggtcatcatgccgcttgtagtcggaggagaagatgccgccgctcgcggggtcgtggccgtactcgggctccccggggccagcggagccgcccttgtcttcgctgtaggcgggggcggccgacatggggcggccagggagacttcgccgaggaggaggttgcggggccggaggccggctggagcggaggaagggaaggcgggccggtccggtccgggctggcgaaggcggcggcgcggcaggggttcagcagaggctgcagtgtgcagcggcggaggctgcgcgcggatttctc

SEQ ID NO: 13062 - RNA, 3217 nt, Homo sapiens
  source 1..3217: mol_type = other RNA
gctgggattacaggcatgagccaccacacccagcctttttgttgtttcttctgagagatttcttcaactcaattttccaacccttctattaaattttttaaattccagatattctatttgcagccggcaaggactcttcctgcgctctgcttgttttccaaagcattccgttctagtttttatgggagcatcatcctttcatgtctctaaggataatcagagtggttaaaatgttcttgaagttttcttctgttccctgcagtagctctgtttcctccagtttcctctttcccaagtgattggtctgtctcatatacctagaggtcttgctttgcattcacatctaagggcaaaaggcgctaggatgcagtgcggaggtccattcgctttgtcgtaaggtttgtgcctttcttagtcctgcagtggttgagtaaaacctgaccatcccacaccctcaaatactaagtgcccctgggtagtgatgtggaggggccttcttattaatgtgaggaaatgcttgtgttataggttgtggtgagaaacgctggttacaaaactatatcaaagtaaaaatgtattaatgcacagtaaagacacctggaaaaaaaatgccctttaatgctcacagaaggtctctccgaggggcagccccaccaccctcctgtttcccttcctgcatttccacgtttttctgggcccagatgcagcctcccctcccacccctggtccctccgccttggcttccggctgtcgctttcatccctcctcctcatcagccccttgcagaactccagggtggggcttctgagtctcgctggcagtatgggctccataagtcttgctggacaccgaaattaagttctgcaggtgccgtcaatgtcaagggaaaccagaactggatagcagttgaaacacatattttgttcgggaccaggtaaaacgaagcttgctgacggcagacagggttagcagacacggcctggaggtggcagaggctaaggaacctgggactgctgggcctctgccccgtggggacctgtcctccaggaaacaaggccagacacaggagggcagggaggactcttctccagggccggtgcgccgtctcttcagccccatggcacttgacttaggcagagcctacagcaccctcaccccagtccctgcagccaccaggaggtggtccccctcatcccattagccatcaccgccattcacagaggtctcggactgaggctggcagggggagcaccatgacccaagatcagaaccctgttgtctgtgcctctggagaggtgggggcaggagctgagggagggtttgggtggagaggggagaagatgcagtagcaggagcagatgctggcaggtagagacaaacttttatgacctttgccttctgacctttgcctctggccactgctccaactaaaacagaatggccccctctgggaacagggcttcctatgggctgggaagcatggagcccccacagtgtggctatgcaggggagtgaggaccaggtgggggcaggcctgtgggggtcacagagctgggctaagcttcagagggaagtggcccctgggagggggaatggctggggttaagaccctgggttcccacgcccccaaaacagaagtagaattagggagaaaggacccccaagaccaaggacggcacctatcagaggagctctccacgggcaggaggtgtcccagggtgagggtggccaggacaggtctagggaaatgcaggtggagcaggacccagagatggattggagatgccggaggggaggcttcctagcgggagcggagacaggcactgcagacaagtgtcagcgggaggggctctgggtggggaagaagactgggacttggaggaagacctctccagggagaagggaggagggggaaggagaaggggaggaagtgggaggaggagagtgctcatcctggaagccacagcctcggagagaactttctagaaggaaggcatgaccatcagtgtcccaggatgctgagaggccaggaaaggtgaggcctcaaggcgccatggggttgtggtgaccccaagatcactgggcacagagcagggatggctgggggtggaaggggaggggcgcgggctgaggttctagggccccaaagccaggtgtgatgtggctctagggggagtgaggaaggggagaatgtccctctgagcgtgcctcttggggaaggcaggggttctggctggggcttctccactcccaggaaaggaggtggtgtggaaggagcgggtgggacggaggagagagcgccccgcggccgcaggaccagcaggtgggggaccagggtcagcgctgctggaggggccttagcgcgacaggactggccagagaccggggatgtggcacagaaagagttaaagggcaccccagggaccgccctgccggtccacccatgtcacccatgttggcccctactccagcccccgtctgctctgcaggggaaggaaccgggagccgcggtgggggcgactgggggtgtcggtctttccagaaaatcaggcaggcatcaggaaagaaggggcgagaacccggggacgcgagaggaagggggcgagggggcgcccagggaggcggagggagcgagaggaaggggggctgagccacggcccccacgcccgcgcgcccctccgcgtcccagggcgtcccctcccggagctgggacccaccgcgaccaccacctgctgggccagggtccgcgggctcaggggtctgcaggattagggtctgcggaaccaggacccgtgggacaaaggtctgtggggcgcgggtccgcggggtggaattcagcgcgccgagtctgcgtatggccggggtacgaggcgctcccagcgctgtctcccctcggtgggctcctgccccgaggactgcccggtggcaccggcgcggcccaggatggggtgaggggtgtctgcgccccgcctggccgctcctcttccgcggcccacactggcgactttgaccccggcaagcgggtcactgccctgcccggctccggcccccccggcgccccaccacccggccgactcggccaccgggcttatgctccgactctgaaccgactgaccccggccccctcggcgcccgcatcctccaaggaccggccagggctgctctctgcccttggtattggggacatcagggttggggggtctgggtgcacccacgc

SEQ ID NO: 13063 - RNA, 4013 nt, Homo sapiens
  source 1..4013: mol_type = other RNA
gctgggattacaggcatgagccaccacacccagcctttttgttgtttcttctgagagatttcttcaactcaattttccaacccttctattaaattttttaaattccagatattctatttgcagccggcaaggactcttcctgcgctctgcttgttttccaaagcattccgttctagtttttatgggagcatcatcctttcatgtctctaaggataatcagagtggttaaaatgttcttgaagttttcttctgttccctgcagtagctctgtttcctccagtttcctctttcccaagtgattggtctgtctcatatacctagaggtcttgctttgcattcacatctaagggcaaaaggcgctaggatgcagtgcggaggtccattcgctttgtcgtaaggtttgtgcctttcttagtcctgcagtggttgagtaaaacctgaccatcccacaccctcaaatactaagtgcccctgggtagtgatgtggaggggccttcttattaatgtgaggaaatgcttgtgttataggttgtggtgagaaacgctggttacaaaactatatcaaagtaaaaatgtattaatgcacagtaaagacacctggaaaaaaaatgccctttaatgctcacagaaggtctctccgaggggcagccccaccaccctcctgtttcccttcctgcatttccacgtttttctgggcccagatgcagcctcccctcccacccctggtccctccgccttggcttccggctgtcgctttcatccctcctcctcatcagccccttgcagaactccagggtggggcttctgagtctcgctggcagtatgggctccataagtcttgctggacaccgaaattaagttctgcaggtgccgtcaatgtcaagggaaaccagaactggatagcagttgaaacacatattttgttcgggaccaggtaaaatgaagcttgctgacggcagacagggttagcagacacggcctggaggtggcagaggctaaggaacctacccaggtaaaacgaagcttgctgacggcagacagggttagcagacacggcctggaggtggcagaggctaaggaacctaccaaggtaaaatgaagcttgctgaaggcagccagggtgagcagatattgcctgggggtggcggaaactgaggaccctacccaggtaaaaggaagcctgctgaaggcaggcagggtgagcagacattgcctgtgggtagcagaggctgaggactctacccaggtaacaggaatcttgcttaaggcaggcaaggtgagcagacatcgcctgggggtggcggaggctgaggactctacccagataacaggaatcttgctgcgggcagccagggtgagcagacgtcgcctgggggtggtggaagctgaggaccctacccaggtaaaaggaagcttgctgaaggcaggcaaggtaagcagacatcgcctgggggtggcggaggctgaggaccctgatcagatatggggggatggaggcttcttgccaaactgacttagcagagttcttgctgaatctggattttataaggcagaatgcagatgagcctgtgagaaggttctgaagccggactacagtttggtcaagcaaacaatcttgtcatggattcagtcatataaataagggtcacccagcccaggggaggtgccccaccccatctgttccctctccctccccacactgagtccgaacctttcaggctttgcccccttcacacactccaaatttattcttctacttctcttcctgcaggtaccagactccggccacccagcgcttacctgggactgctgggcctctgccccgtggggacctgtcctccaggaaacaaggccagacacaggagggcagggaggactcttctccagggccggtgcgccgtctcttcagccccatggcacttgacttaggcagagcctacagcaccctcaccccagtccctgcagccaccaggaggtggtccccctcatcccattagccatcaccgccattcacagaggtctcggactgaggctggcagggggagcaccatgacccaagatcagaaccctgttgtctgtgcctctggagaggtgggggcaggagctgagggagggtttgggtggagaggggagaagatgcagtagcaggagcagatgctggcaggtagagacaaacttttatgacctttgccttctgacctttgcctctggccactgctccaactaaaacagaatggccccctctgggaacagggcttcctatgggctgggaagcatggagcccccacagtgtggctatgcaggggagtgaggaccaggtgggggcaggcctgtgggggtcacagagctgggctaagcttcagagggaagtggcccctgggagggggaatggctggggttaagaccctgggttcccacgcccccaaaacagaagtagaattagggagaaaggacccccaagaccaaggacggcacctatcagaggagctctccacgggcaggaggtgtcccagggtgagggtggccaggacaggtctagggaaatgcaggtggagcaggacccagagatggattggagatgccggaggggaggcttcctagcgggagcggagacaggcactgcagacaagtgtcagcgggaggggctctgggtggggaagaagactgggacttggaggaagacctctccagggagaagggaggagggggaaggagaaggggaggaagtgggaggaggagagtgctcatcctggaagccacagcctcggagagaactttctagaaggaaggcatgaccatcagtgtcccaggatgctgagaggccaggaaaggtgaggcctcaaggcgccatggggttgtggtgaccccaagatcactgggcacagagcagggatggctgggggtggaaggggaggggcgcgggctgaggttctagggccccaaagccaggtgtgatgtggctctagggggagtgaggaaggggagaatgtccctctgagcgtgcctcttggggaaggcaggggttctggctggggcttctccactcccaggaaaggaggtggtgtggaaggagcgggtgggacggaggagagagcgccccgcggccgcaggaccagcaggtgggggaccagggtcagcgctgctggaggggccttagcgcgacaggactggccagagaccggggatgtggcacagaaagagttaaagggcaccccagggaccgccctgccggtccacccatgtcacccatgttggcccctactccagcccccgtctgctctgcaggggaaggaaccgggagccgcggtgggggcgactgggggtgtcggtctttccagaaaatcaggcaggcatcaggaaagaaggggcgagaacccggggacgcgagaggaagggggcgagggggcgcccagggaggcggagggagcgagaggaaggggggctgagccacggcccccacgcccgcgcgcccctccgcgtcccagggcgtcccctcccggagctgggacccaccgcgaccaccacctgctgggccagggtccgcgggctcaggggtctgcaggattagggtctgcggaaccaggacccgtgggacaaaggtctgtggggcgcgggtccgcggggtggaattcagcgcgccgagtctgcgtatggccggggtacgaggcgctcccagcgctgtctcccctcggtgggctcctgccccgaggactgcccggtggcaccggcgcggcccaggatggggtgaggggtgtctgcgccccgcctggccgctcctcttccgcggcccacactggcgactttgaccccggcaagcgggtcactgccctgcccggctccggcccccccggcgccccaccacccggccgactcggccaccgggcttatgctccgactctgaaccgactgaccccggccccctcggcgcccgcatcctccaaggaccggccagggctgctctctgcccttggtattggggacatcagggttggggggtctgggtgcacccacgc

SEQ ID NO: 13064 - RNA, 2143 nt, Homo sapiens
  source 1..2143: mol_type = other RNA
gctgggattacaggcatgagccaccacacccagctaacttcagtttttgatgagacagaaatgggaaaatgtagactggtttactactttatcttatgatacaatgttattgtagtataatatactatagactacccattaaagaaccaggaaggatattccgctagccttaagaagtaaatattgaatataaatataactttctacctcatctataacatattgatacattttattacaaagaaactcacacataaatgatttgtcctatttatcataataggccaccaatcactaggagccaagcttcatcagcttaagtcctaggtagcatgtctcaatgcatacatatttatatgttattaaccgtgtttcttttctttttttcgagacagagtgtccaggctggaggtgatctcggcttaccgcaacctccgcctccgggttcaagtgattctgccgcctcagccttcctgggtagctgggattacaggcacgcatcaccacgcccggctacttttgtatttttagtagagatagggtttctccgtgttggtcaggctggtctcgaactcccaacctcaggtgatccgcccgcctcagcctcccaaagtgctgggattacaggcatgagccaccatgcctggctattaaccttgtttctaacttcagcattgcacatctccttagtaaagcagtagccattaacaagtcaggtccaacaaccattttcctctggtcctcaagcagagactcagagccagttacacataaactatttcattataacatgaaaatagcaagccttgggctattgcaaaaggcttttcaaatgttgacctctaacttggagaaaatagagggaagcagaaatatagggtgctaatttgtgctataacctggtctcatgtcgtggtatattcccagttgcaacattttaaatttataagtgagaaagtaaaacaaagcttcatatctgtgaaagtgaaaaattgtccagaagtcttctattcaaagaccaattagctttttcttcccaataacttatcagaaagaaatgggtacttagaaacctaaggggttctttaaataggagtcagaaaaaatatataaaaataaaaaacaaagcaagaaagaacattgtataaaaataaaatgttctttaaagatgactgccctctcttgaaagatgagtgctatattaaaagggtagatgtatctctataactcatcgtgtttatatgtaaattctctggcagatataaacccatctttgtcttcatcttctttatcaaaaatatcctccaccaaagcatcatgatgactttcattcaccaccgcaccatgtttttcaaactccttctttaaatatgctttaacctcatctttagagagtttccagtcatcattaagatccatttcttggaatgattcatgggatcttggtccatttcgaatctccaggagatcaatattaaatatcagtgtactttctgggggaattttaccatttcagatctagacagagatgtgacatgcgctaggttgttgataaaactggtatctttccaaaagaggcatgcaagcatgtactaaaagacttttccttcttttccatagcccagagcaggaggaatgatgagctttctcttctctcctacacacattcctttcaagccctggtcccaacctttgagagcctccaggatgcccagggtaaaccaaatgggctgaccattgttatgtttgtgagtggagtgaaataaggagccgtccttttctaagtagccttcatagtggaccaacatcaaatcccctcctttggtcttgcgatggcagatgaatggcttctggagaacttcaattttcacttctggttcagggatcaaagccccaatcaaagaagtgacgaacagagtcaagaccgcgttccacaagaaaagcctcatgttgctgaagcaaggaaagaagtccctacaaaagcagcgaaaggtccctcgacttcatagatttaagaacgtagttcaaggcttacggacaagggcttcagacaagttcaggactcccccttcttagaagacgtggcacatttaccaccaactcttttctcaagggtcacgaacctacctttaaagagttaagc

SEQ ID NO: 13065 - RNA, 2051 nt, Homo sapiens
  source 1..2051: mol_type = other RNA
gctgggattacaggcatgagccaccacacccagctaacttcagtttttgatgagacagaaatgggaaaatgtagactggtttactactttatcttatgatacaatgttattgtagtataatatactatagactacccattaaagaaccaggaaggatattccgctagccttaagaagtaaatattgaatataaatataactttctacctcatctataacatattgatacattttattacaaagaaactcacacataaatgatttgtcctatttatcataataggccaccaatcactaggagccaagcttcatcagcttaagtcctaggtagcatgtctcaatgcatacatatttatatgttattaaccgtgtttcttttctttttttcgagacagagtgtccaggctggaggtgatctcggcttaccgcaacctccgcctccgggttcaagtgattctgccgcctcagccttcctgggtagctgggattacaggcacgcatcaccacgcccggctacttttgtatttttagtagagatagggtttctccgtgttggtcaggctggtctcgaactcccaacctcaggtgatccgcccgcctcagcctcccaaagtgctgggattacaggcatgagccaccatgcctggctattaaccttgtttctaacttcagcattgcacatctccttagtaaagcagtagccattaacaagtcaggtccaacaaccattttcctctggtcctcaagcagagactcagagccagttacacataaactatttcattataacatgaaaatagcaagccttgggctattgcaaaaggcttttcaaatgttgacctctaacttggagaaaatagagggaagcagaaatatagggtgctaatttgtgctataacctggtctcatgtcgtggtatattcccagttgcaacattttaaatttataagtgagaaagtaaaacaaagcttcatatctgtgaaagtgaaaaattgtccagaagtcttctattcaaagaccaattagctttttcttcccaataacttatcagaaagaaatgggtacttagaaacctaaggggttctttaaataggagtcagaaaaaatatataaaaataaaaaacaaagcaagaaagaacattgtataaaaataaaatgttctttaaagatgactgccctctcttgaaagatgagtgctatattaaaagggtagatgtatctctataactcatcgtgtttatatgtaaattctctggcagatataaacccatctttgtcttcatcttctttatcaaaaatatcctccaccaaagcatcatgatgactttcattcaccaccgcaccatgtttttcaaactccttctttaaatatgctttaacctcatctttagagagtttccagtcatcattaagatccatttcttggaatgattcatgggatcttggtccatttcgaatctccaggagatcaatattaaatatcagtgtactttctgggggaattttaccttttccttcttttccatagcccagagcaggaggaatgatgagctttctcttctctcctacacacattcctttcaagccctggtcccaacctttgagagcctccaggatgcccagggtaaaccaaatgggctgaccattgttatgtttgtgagtggagtgaaataaggagccgtccttttctaagtagccttcatagtggaccaacatcaaatcccctcctttggtcttgcgatggcagatgaatggcttctggagaacttcaattttcacttctggttcagggatcaaagccccaatcaaagaagtgacgaacagagtcaagaccgcgttccacaagaaaagcctcatgttgctgaagcaaggaaagaagtccctacaaaagcagcgaaaggtccctcgacttcatagatttaagaacgtagttcaaggcttacggacaagggcttcagacaagttcaggactcccccttcttagaagacgtggcacatttaccaccaactcttttctcaagggtcacgaacctacctttaaagagttaagc

SEQ ID NO: 13066 - RNA, 1899 nt, Homo sapiens
  source 1..1899: mol_type = other RNA
gctgggattacaggcatgagccaccacacccagctaacttcagtttttgatgagacagaaatgggaaaatgtagactggtttactactttatcttatgatacaatgttattgtagtataatatactatagactacccattaaagaaccaggaaggatattccgctagccttaagaagtaaatattgaatataaatataactttctacctcatctataacatattgatacattttattacaaagaaactcacacataaatgatttgtcctatttatcataataggccaccaatcactaggagccaagcttcatcagcttaagtcctaggtagcatgtctcaatgcatacatatttatatgttattaaccgtgtttcttttctttttttcgagacagagtgtccaggctggaggtgatctcggcttaccgcaacctccgcctccgggttcaagtgattctgccgcctcagccttcctgggtagctgggattacaggcacgcatcaccacgcccggctacttttgtatttttagtagagatagggtttctccgtgttggtcaggctggtctcgaactcccaacctcaggtgatccgcccgcctcagcctcccaaagtgctgggattacaggcatgagccaccatgcctggctattaaccttgtttctaacttcagcattgcacatctccttagtaaagcagtagccattaacaagtcaggtccaacaaccattttcctctggtcctcaagcagagactcagagccagttacacataaactatttcattataacatgaaaatagcaagccttgggctattgcaaaaggcttttcaaatgttgacctctaacttggagaaaatagagggaagcagaaatatagggtgctaatttgtgctataacctggtctcatgtcgtggtatattcccagttgcaacattttaaatttataagtgagaaagtaaaacaaagcttcatatctgtgaaagtgaaaaattgtccagaagtcttctattcaaagaccaattagctttttcttcccaataacttatcagaaagaaatgggtacttagaaacctaaggggttctttaaataggagtcagaaaaaatatataaaaataaaaaacaaagcaagaaagaacattgtataaaaataaaatgttctttaaagatgactgccctctcttgaaagatgagtgctatattaaaagggtagatgtatctctataactcatcgtgtttatatgtaaattctctggcagatataaacccatctttgtcttcatcttctttatcaaaaatatcctccaccaaagcatcatgatgactttcattcaccaccgcaccatgtttttcaaactccttctttaaatatgctttaacctcatctttagagagtttccagtcatcattaagatccatttcttggaatgattcatgggatcttggtccatttcgaatctccaggagatcaatattaaatatcagtgtactttctgggggaattttacgtggagtgaaataaggagccgtccttttctaagtagccttcatagtggaccaacatcaaatcccctcctttggtcttgcgatggcagatgaatggcttctggagaacttcaattttcacttctggttcagggatcaaagccccaatcaaagaagtgacgaacagagtcaagaccgcgttccacaagaaaagcctcatgttgctgaagcaaggaaagaagtccctacaaaagcagcgaaaggtccctcgacttcatagatttaagaacgtagttcaaggcttacggacaagggcttcagacaagttcaggactcccccttcttagaagacgtggcacatttaccaccaactcttttctcaagggtcacgaacctacctttaaagagttaagc
